European Patent Application EP 4 520 821 A1 - sequence listing, part 7

SEQ ID NO: 13067 - RNA, 9093 nt, Homo sapiens
  source 1..9093: mol_type = other RNA
gctgggattacaggcatgagccaccacacccagctggaaaatgtttaaaatttattaagtgaaaagtaactcatgctgcaatgaacgtactatgtaaaaatgtatgtatgtggaacagggaaaaatataaacagtcacagaaatgtgtttaggttggtagcattctttttcctcttaaaaattcctttttttggccgggcgctgtggctcacacctgtaatcccagcactttgggaagccgcggtggacagatcacaaggtcaggagatcaagaccatcctggctaacatggtgaaaccccgtctctactaaaaatacaaaaaattagctgggcatggaggcactcgcctgtagtcgcagctactcgggaggctgaggcaggagaatcgcttgaactggggagatggaggttgtagtgagcccagatcatgccactgcactcaagcctgggctgagacctccagagtctggctgagacctatggagtctcactctgtcacctaggctggagtacagtggtgcgatctcggcacactgcaacctccacctcccagacattctcctgcctcagcctctcaactagctgggattacattcgcccgcctccacacccactaatttttgtatttttagtagagatgcggtttccccatgttggccaggctgttcttgaactcctgacctcaagttatacgcccactttggactcccaaagtgctgggattacaggtgtgagccacggcaccagccaaaaatttctttaaatattagtggtatattattctctcaataagttttttttttttttttttttgagacagtcttgttttattgcctaagctggagtgcagtggcacaatctcaactcactgcaacctccacctcccaggtttattttttttctcatgcctcagcctcccaagaagctgggattacaggcatgtgccccaaaggccagttaagttttctttttctttttttcttttttcttggttgagacggattttcgctcgtcacccacactggagtgcaatggcgcgatctcggctcactgcaacctccgactcttgggttcaagcgattctcctgcctcagcctcccgagtagctgggattagaggcacctgtcaccacgcccgctacttttggtatttttagtagagatggagtttcaccacgttggccaggctgatctcaaactcctggcctcaagtgattcacctgccttggcctcccaaagtgctggaattacaggcccggcctatttttgcaataattatgaatagcacaccatttaaacctgttgattgagccctccttaaataactaaatacactactggccaacatggtgaaaacctgtctccactaaaaacacaaaaaaatggccgggcacagtggctcatgcctgtaatcccagcacttcaggaggccaaggggtgtgaatcacctgaggttaggagttcaagaccagcctggccaacatggtgaaaccctgtctctactaaaaaaaaatacaaaaattagctgagtgtagtggcacatacccgtagtctcagctactcaggaggctgaggcaggagaattgcttgaacctgggaggcaggggttgcagtgagccaagatcgtgccaccacactccagcctgggtgacacagcgagactccatctcaaaataaataaataaataaaaagaaagggaccgagcgcggtggctcatgcttgtaatcccagcactctgggaggctgagttgggcagatcacaaggtcaagagttcaggaccagcctgaccaacacggtaaaaccccatctctactaaaaatacaaaaatgagctgggtgtgatggcacgcgcctgtaaccccagttactcaaaaggctgaggcaagagaatcgcttgaacctgggaggcagaggttgcagtgagccgagatcacgccactgcattccagcctggtgacagtgagactctgtcacacacacacaaaaaagataaagaatgacaaaaatctgtgcctacattcagagtgacaagaatactaatgttctgcttgtagaaaagactattggttcagaatatgttaaatgcaaataatattttgtataatatatataaattacatatgcataaaaagagtatctatattagaatcttttgagacagggtcttgctctgtcaaccatgagggagtgcagtggcactaccacagctcactgtagccttgacttcctgagctcaagccatcctctcgcctcagcctcctgaatagttgggactgcaggtggtgccaccaaggctggctaagtttttatatttttttatagaaacaagcttttgccacgttgcccaggctggtctcaaacttctaaaagctcaagcaatctggccgccttgaactcccaaagtgcttgagttataggcatgagtcactgtgcccggcctacattagaatcttaacagtggggctgggcatggtgccccatgcctgtaatcccagcactttgggaggtcaaggtgggcagactacttgaggttgaggagttcgaggccagcctggccaacatggtgaaaccccatctgtactaaaaacacaaaaattagccaggtgtggtggcacatgtttgcaatcccagctacttgggaggctgaggcgggaggatcacttgaacctgggaagcagaggttgcagtgagccgagatggtgccatggcactccagcctgggcaatagacagcgggactcagtctcaaaacaaaaaaaaaaaaaaaaaaaaaagaatcttaacagtggttaacttcaaatagtgaaactatgactgttaactgagtttgacatttttgtgttttcctagatttttctacaataaacattattatttcataataaagcagtaaagactttttatacaaactattttaagataaacaaattttgacataggggttataagttaggtagaatctatttatataaaaaatggaactgtacttttgtgggccaaataagcactatgtaagtttttttaattttcccaaacacatgcacagaattaatattgccttaaattttgttagcacaagtttgagagagctctttagttcataaaaaaatgttttatggaccaggtgccgtggctcacacctgcaatctcaacactttgggaggcccaggtgggaggatcgcttgagcctaggagtttgagacaagactgggcgacgcagggagaccctgtctcaaaaaaacaaaaccaaaaacaagcaaacaaaaaaacagctgggcatggtggcatgcatatgtagtcccagctattctagaggctgaggtgagatcgctggagcccaggaggtggaggctacagtaagctgtgatcatgccaatgcactccagcttggtcaacaaagcaagactgtgcctcaaaaaaaaaaaagaaaagaaaagaaagaaagaaaagaaaaagaaaaaaagttatgtacgtatggtttttttttttttttggatagagtttcactcttcttgcccaggctggagtgcaatggtgcaatcttggctcaccacaaccttcccctactgggttcaagcgattctcctgtttcagcctccccagtagctgggattaaaggcatgtgccaccacgcccggctaattttgtatttttagtagagatgaagtttctccatgttggtcaggctggtcttgaactcctgacttcaggtgatctgcccgcctcagcctcccaaagtgctgggattacaggtgtgagccacctcgcctggccgttttttttttttttttttttttctgagacggagttttgctcttattgcccaggctggagtgcaatggcacgatctcggctcatcgcaacctctgcctcacgggttcaagcaattttcctgcctcagcgtctcaagtagctaggattacagggatgctccatcatgcccggctaattttgtatttttggtagagacagggtttctccatgttggtcaggctggtctcaaactcccaacctcaggtgatttacccgccttggcctcccaaagagctgggattacaggtgtgagccactgtgcccggccatgcttatgttttttaacaatacacttctgaactatcaaaaagaatataaatcaaaatcactgaagtagtttttaaaaactccaaaagctacaaaacttacttacttcaatatcaattaaaaacccatttgatagttcaataacttgagtcctgctagaatcattctataagccatcagtgacagtgaagtggccaaaatttgagtcacttgataagtacaaagaacacagatttttgtcattcttactgtgaagaaaaacagtgaatgaataacttagtttatatattaacagtacttttatttaaaaaattatctagagaataacttctttttaatcatttgttagtcatgtaactatggataaaacatactaatttagctgattcctctatgctctcttttccttgattccaatcattattagttattctacactgcctcatttattggcagttatgccaactggctgactctggttcaactgccctatttttgctttcatcattgtttatcatatctcacttgctttaaactccacctctttcatctcatctgatctgacacttggtttacatatcaattggctactctaaccttctaccgccagtttccaacccattcgaggtacttgggtaacaaaggaagatgctctatacacacaaaaccacagaaaataagtgggaagggataataaatttcacttaaagttttagaatttttcttttttttttgagacggagtttcactcttgttgcccaggctggagtgcaatggcgcgatcttggctcaccgcaacctctgcctcccaggttcaagcagttctcctgcttcagcctcccgagtagctggtattacaggcatgcaccaccaagcctggctaattttgtatttttagtagagacggggtttctccatgttggtcaggctggtcttgaacgcctgacctcaggtgatctgcctgcctcggcctcccaaagtgctgggattacaggcatgagccatcacgcccggccaaagttttagaatttaagttattccaaaaaaaattttttttttcaaaaatacagactgcatccaattaaattctatgttaactggtaatgactaggtctaaaatgttaggtatttaccaataaatgacataaaataactcaacaacaaagggatttttttttttaagagatagggtctcactttatcactcaggtttggctgagggcagtggtgtgatcacagctcactgaagcctccaactcctgggctcaagtgatcctcccgcctcagtctaccagagtatattcttgaaagtaaaattacaaatgaaattcagcagtgttaaaaataagcccacttgcagacaattatcatttttcttcctttctttcctcactatctgtacttggcatatttcctacagtggctgtcttaaagaaaaaaaggaatccttcacaaatagtgtagccaaaaaagttggactaatatacaatgctatcagtaaagtattatatataaaatttataagtgctaaagtgtaattttgaaagacacttaagatactccttttttttttgagacaaggtctcagccctgtcgcccaggctggagtgcactagcacaacatcagctcactgcaacctccgcctcccaggttcaagcgattctcctgcctcagcctcccaagtagctgagactacaggcgcacgccagcatgtccagataattttttgtatttttagtagagatggggtttcaccatgttggccaggatggtctcaaatctcttgacctcgtgatctgcccatgtcggcttcccaaagtgttaggataacaggcatgagctaccgtgcccagcctacttaaaatattcttgaaatagctctccccacctccttttttttttttttttgagaatgagtttcactcgacacccaggctggagtgcagtggtgcgatcttggctcactgcaacctctgcctcccaggttcaagcgattatcctgcctcagcctcctgagtagctgggattacaaatgtgcaccaccacatctggctaattttttttttttttttttgtatttttagtagagacggggtttcaccaagttggcctggctggtctcgaacacctgacctcaattgatccacctgcctcggcctcccaaagtattataggcatgagccaccgagcccggccttttttgttttttgtttttttaaaggcagggttttgctctgttgcccaggctggagtgcagtggtgtgatcacagatcactgcagccttgacctctcctggtctcaagtgatcctcccacctcagccttcagaacagctgggactacaggtgtgtgtcaccatgcccagtaatttttttgtatatttgtagaggcagggtctcccaatgttgcctgggctggtctcaaactcctgggctcaagcaatccaccagctttggccttccaaagttctaggattatacgcatgagccactgtgccctgccccaatattttgttacttactagtgagactaaacacttttctaaaagtttgttagccatactatcctataaaagctgtttgttcatgtcttttgtccatttatctttttttttgtttttcttgagacagagtcttgctctgtggcccaggctggagtgcaggggtgcaatctcggctcactgcaagctccgcctcccaggttcaaatgattctcctgcctcagcctcctgagtagctgggattacaggcatgtgccaccatgcccagctaatttttttgtgtgtgtttttcagtagagatggggtttcaccatgttggccaggctgatctcgaattcctgacctcaggtgctccacccgcctcagcctcccaaagtactgggattacaggggtgagccaccgcacccggccaattttctgtatttttaatagagacagggtttcatcctgttggccaggctggcctcgaacttcggacctcaggtgatccacccgcctcgacctcccaaagtgctgggattacaggtgtgggccaccacacccagccaatttttttgtatttttagtagagacagggtttcatcatgttggccaggctggtcgcaaactcctgacctcaggtgatccacccgcctcagcatcccaaagtgctgggattacaggcatgagccaccactcccggccaatgttttgtatttttagtagagatggggtttcatcatgttggccagactggtctcaaactctggacctcaggtgatccacctgcctcagcctcccaaagtgtagggattacaggtgtgagccaccgcgcccagcctatgtttctattttatacatattcaacaaacatgattccccaacttctgcaaaataatttctttttcaagaacattgattttagagctcacactaagaaaaagaatacaaaaataatggcatagaaagtgaaaaaacaaaaataaaaagtagaaagctaaagtttcccattaaaatgatcaatatactgtgcagtaagtcaaatgtgtacaatgaattaagaaaatatgatatataaaaatccaaatttacaaaattaagtacaaataggtgtttatattacaaagtgatactggtttataaaaggattcaacatagattttttttaaatggttgttttcctcaatcaatttaacaatgattttaaatgtataaaattttaatatctctttgagacagtgatccaagcttcttcccttgatgatgttaccagttcatactttgtttcaataacctgtccctccacagaaagtaggtgcagtctcttcaccaatacactaagaagtactgtggtcaccatatatgcaaacctcaactctggacactcctgtgtgcctgagaatccaagtgaggaaaaagttttcattactaattcatcatcaaaccgatctggatcaaacttgtgtggagatggccaagtattaggatcctgaagtaccacaccaagggcataaaggacgagggtctctctaggaataataaatcggtcaatttttccttcaatatcttgaagctgggcagaaactggagtcagtttggcagttcgaacagtttcacaaagcacatgctgacaatatattttgcagttattatgcaactggccagagaaaatatcatactgtcttctaggatctgttggtcattaaggttcccttgtactaaggagtcaatgaaaatatgttgactgaagttccttccttttcgttcttttatgatgttccttaaaacagactccagttgcatgagggcatcttcatattgttttttccgagtcatgtttttatcaagtgacccatctagaaagccttttccaatctcagaccaaactgtgccatgattcttctggaagcgaatgacttcctgatcatcttcaaatgtactacccattaccatctgtgtaacagacttcatagcaaaaccaagcatatgctggctgaggggcacgtgctgggtctctgggtaggagagccatttatctaataattcttctgaaagctttaggaggagggcaaagttactcttcagagaatcagtcacaccattttcatacaattttttcctcatgtggttttcactcacactgccaccaccagattgataccttaataatgacttcagcatggtttcaaaagggtccgatgtcttattgggattgatatgctgcttcagtacatcaacagtgcccaaactaaccacgaggcgcctgccaaaccagaaggagaccacaggcccatatctctcatgcaaattaaccaggaactcatgcaaacttccactattcacaatatctggaagattaccatctttttcttcagttggagtaatccctggaattcctgcagcttgtctggaagccggatagaggtagagcacggctcccaccaacgccagcaagaaggtaacggcgaagatcgcgaagtccaacatggttctgccgcccagggagccacgtctcggatcggccgctccagc

SEQ ID NO: 13068 - RNA, 9014 nt, Homo sapiens
  source 1..9014: mol_type = other RNA
gctgggattacaggcatgagccaccacacccagctggaaaatgtttaaaatttattaagtgaaaagtaactcatgctgcaatgaacgtactatgtaaaaatgtatgtatgtggaacagggaaaaatataaacagtcacagaaatgtgtttaggttggtagcattctttttcctcttaaaaattcctttttttggccgggcgctgtggctcacacctgtaatcccagcactttgggaagccgcggtggacagatcacaaggtcaggagatcaagaccatcctggctaacatggtgaaaccccgtctctactaaaaatacaaaaaattagctgggcatggaggcactcgcctgtagtcgcagctactcgggaggctgaggcaggagaatcgcttgaactggggagatggaggttgtagtgagcccagatcatgccactgcactcaagcctgggctgagacctccagagtctggctgagacctatggagtctcactctgtcacctaggctggagtacagtggtgcgatctcggcacactgcaacctccacctcccagacattctcctgcctcagcctctcaactagctgggattacattcgcccgcctccacacccactaatttttgtatttttagtagagatgcggtttccccatgttggccaggctgttcttgaactcctgacctcaagttatacgcccactttggactcccaaagtgctgggattacaggtgtgagccacggcaccagccaaaaatttctttaaatattagtggtatattattctctcaataagttttttttttttttttttttgagacagtcttgttttattgcctaagctggagtgcagtggcacaatctcaactcactgcaacctccacctcccaggtttattttttttctcatgcctcagcctcccaagaagctgggattacaggcatgtgccccaaaggccagttaagttttctttttctttttttcttttttcttggttgagacggattttcgctcgtcacccacactggagtgcaatggcgcgatctcggctcactgcaacctccgactcttgggttcaagcgattctcctgcctcagcctcccgagtagctgggattagaggcacctgtcaccacgcccgctacttttggtatttttagtagagatggagtttcaccacgttggccaggctgatctcaaactcctggcctcaagtgattcacctgccttggcctcccaaagtgctggaattacaggcccggcctatttttgcaataattatgaatagcacaccatttaaacctgttgattgagccctccttaaataactaaatacactactggccaacatggtgaaaacctgtctccactaaaaacacaaaaaaatggccgggcacagtggctcatgcctgtaatcccagcacttcaggaggccaaggggtgtgaatcacctgaggttaggagttcaagaccagcctggccaacatggtgaaaccctgtctctactaaaaaaaaatacaaaaattagctgagtgtagtggcacatacccgtagtctcagctactcaggaggctgaggcaggagaattgcttgaacctgggaggcaggggttgcagtgagccaagatcgtgccaccacactccagcctgggtgacacagcgagactccatctcaaaataaataaataaataaaaagaaagggaccgagcgcggtggctcatgcttgtaatcccagcactctgggaggctgagttgggcagatcacaaggtcaagagttcaggaccagcctgaccaacacggtaaaaccccatctctactaaaaatacaaaaatgagctgggtgtgatggcacgcgcctgtaaccccagttactcaaaaggctgaggcaagagaatcgcttgaacctgggaggcagaggttgcagtgagccgagatcacgccactgcattccagcctggtgacagtgagactctgtcacacacacacaaaaaagataaagaatgacaaaaatctgtgcctacattcagagtgacaagaatactaatgttctgcttgtagaaaagactattggttcagaatatgttaaatgcaaataatattttgtataatatatataaattacatatgcataaaaagagtatctatattagaatcttttgagacagggtcttgctctgtcaaccatgagggagtgcagtggcactaccacagctcactgtagccttgacttcctgagctcaagccatcctctcgcctcagcctcctgaatagttgggactgcaggtggtgccaccaaggctggctaagtttttatatttttttatagaaacaagcttttgccacgttgcccaggctggtctcaaacttctaaaagctcaagcaatctggccgccttgaactcccaaagtgcttgagttataggcatgagtcactgtgcccggcctacattagaatcttaacagtggggctgggcatggtgccccatgcctgtaatcccagcactttgggaggtcaaggtgggcagactacttgaggttgaggagttcgaggccagcctggccaacatggtgaaaccccatctgtactaaaaacacaaaaattagccaggtgtggtggcacatgtttgcaatcccagctacttgggaggctgaggcgggaggatcacttgaacctgggaagcagaggttgcagtgagccgagatggtgccatggcactccagcctgggcaatagacagcgggactcagtctcaaaacaaaaaaaaaaaaaaaaaaaaaagaatcttaacagtggttaacttcaaatagtgaaactatgactgttaactgagtttgacatttttgtgttttcctagatttttctacaataaacattattatttcataataaagcagtaaagactttttatacaaactattttaagataaacaaattttgacataggggttataagttaggtagaatctatttatataaaaaatggaactgtacttttgtgggccaaataagcactatgtaagtttttttaattttcccaaacacatgcacagaattaatattgccttaaattttgttagcacaagtttgagagagctctttagttcataaaaaaatgttttatggaccaggtgccgtggctcacacctgcaatctcaacactttgggaggcccaggtgggaggatcgcttgagcctaggagtttgagacaagactgggcgacgcagggagaccctgtctcaaaaaaacaaaaccaaaaacaagcaaacaaaaaaacagctgggcatggtggcatgcatatgtagtcccagctattctagaggctgaggtgagatcgctggagcccaggaggtggaggctacagtaagctgtgatcatgccaatgcactccagcttggtcaacaaagcaagactgtgcctcaaaaaaaaaaaagaaaagaaaagaaagaaagaaaagaaaaagaaaaaaagttatgtacgtatggtttttttttttttttggatagagtttcactcttcttgcccaggctggagtgcaatggtgcaatcttggctcaccacaaccttcccctactgggttcaagcgattctcctgtttcagcctccccagtagctgggattaaaggcatgtgccaccacgcccggctaattttgtatttttagtagagatgaagtttctccatgttggtcaggctggtcttgaactcctgacttcaggtgatctgcccgcctcagcctcccaaagtgctgggattacaggtgtgagccacctcgcctggccgttttttttttttttttttttttctgagacggagttttgctcttattgcccaggctggagtgcaatggcacgatctcggctcatcgcaacctctgcctcacgggttcaagcaattttcctgcctcagcgtctcaagtagctaggattacagggatgctccatcatgcccggctaattttgtatttttggtagagacagggtttctccatgttggtcaggctggtctcaaactcccaacctcaggtgatttacccgccttggcctcccaaagagctgggattacaggtgtgagccactgtgcccggccatgcttatgttttttaacaatacacttctgaactatcaaaaagaatataaatcaaaatcactgaagtagtttttaaaaactccaaaagctacaaaacttacttacttcaatatcaattaaaaacccatttgatagttcaataacttgagtcctgctagaatcattctataagccatcagtgacagtgaagtggccaaaatttgagtcacttgataagtacaaagaacacagatttttgtcattcttactgtgaagaaaaacagtgaatgaataacttagtttatatattaacagtacttttatttaaaaaattatctagagaataacttctttttaatcatttgttagtcatgtaactatggataaaacatactaatttagctgattcctctatgctctcttttccttgattccaatcattattagttattctacactgcctcatttattggcagttatgccaactggctgactctggttcaactgccctatttttgctttcatcattgtttatcatatctcacttgctttaaactccacctctttcatctcatctgatctgacacttggtttacatatcaattggctactctaaccttctaccgccagtttccaacccattcgaggtacttgggtaacaaaggaagatgctctatacacacaaaaccacagaaaataagtgggaagggataataaatttcacttaaagttttagaatttttcttttttttttgagacggagtttcactcttgttgcccaggctggagtgcaatggcgcgatcttggctcaccgcaacctctgcctcccaggttcaagcagttctcctgcttcagcctcccgagtagctggtattacaggcatgcaccaccaagcctggctaattttgtatttttagtagagacggggtttctccatgttggtcaggctggtcttgaacgcctgacctcaggtgatctgcctgcctcggcctcccaaagtgctgggattacaggcatgagccatcacgcccggccaaagttttagaatttaagttattccaaaaaaaattttttttttcaaaaatacagactgcatccaattaaattctatgttaactggtaatgactaggtctaaaatgttaggtatttaccaataaatgacataaaataactcaacaacaaagggatttttttttttaagagatagggtctcactttatcactcaggtttggctgagggcagtggtgtgatcacagctcactgaagcctccaactcctgggctcaagtgatcctcccgcctcagtctaccagagtatattcttgaaagtaaaattacaaatgaaattcagcagtgttaaaaataagcccacttgcagacaattatcatttttcttcctttctttcctcactatctgtacttggcatatttcctacagtggctgtcttaaagaaaaaaaggaatccttcacaaatagtgtagccaaaaaagttggactaatatacaatgctatcagtaaagtattatatataaaatttataagtgctaaagtgtaattttgaaagacacttaagatactccttttttttttgagacaaggtctcagccctgtcgcccaggctggagtgcactagcacaacatcagctcactgcaacctccgcctcccaggttcaagcgattctcctgcctcagcctcccaagtagctgagactacaggcgcacgccagcatgtccagataattttttgtatttttagtagagatggggtttcaccatgttggccaggatggtctcaaatctcttgacctcgtgatctgcccatgtcggcttcccaaagtgttaggataacaggcatgagctaccgtgcccagcctacttaaaatattcttgaaatagctctccccacctccttttttttttttttttgagaatgagtttcactcgacacccaggctggagtgcagtggtgcgatcttggctcactgcaacctctgcctcccaggttcaagcgattatcctgcctcagcctcctgagtagctgggattacaaatgtgcaccaccacatctggctaattttttttttttttttttgtatttttagtagagacggggtttcaccaagttggcctggctggtctcgaacacctgacctcaattgatccacctgcctcggcctcccaaagtattataggcatgagccaccgagcccggccttttttgttttttgtttttttaaaggcagggttttgctctgttgcccaggctggagtgcagtggtgtgatcacagatcactgcagccttgacctctcctggtctcaagtgatcctcccacctcagccttcagaacagctgggactacaggtgtgtgtcaccatgcccagtaatttttttgtatatttgtagaggcagggtctcccaatgttgcctgggctggtctcaaactcctgggctcaagcaatccaccagctttggccttccaaagttctaggattatacgcatgagccactgtgccctgccccaatattttgttacttactagtgagactaaacacttttctaaaagtttgttagccatactatcctataaaagctgtttgttcatgtcttttgtccatttatctttttttttgtttttcttgagacagagtcttgctctgtggcccaggctggagtgcaggggtgcaatctcggctcactgcaagctccgcctcccaggttcaaatgattctcctgcctcagcctcctgagtagctgggattacaggcatgtgccaccatgcccagctaatttttttgtgtgtgtttttcagtagagatggggtttcaccatgttggccaggctgatctcgaattcctgacctcaggtgctccacccgcctcagcctcccaaagtactgggattacaggggtgagccaccgcacccggccaattttctgtatttttaatagagacagggtttcatcctgttggccaggctggcctcgaacttcggacctcaggtgatccacccgcctcgacctcccaaagtgctgggattacaggtgtgggccaccacacccagccaatttttttgtatttttagtagagacagggtttcatcatgttggccaggctggtcgcaaactcctgacctcaggtgatccacccgcctcagcatcccaaagtgctgggattacaggcatgagccaccactcccggccaatgttttgtatttttagtagagatggggtttcatcatgttggccagactggtctcaaactctggacctcaggtgatccacctgcctcagcctcccaaagtgtagggattacaggtgtgagccaccgcgcccagcctatgtttctattttatacatattcaacaaacatgattccccaacttctgcaaaataatttctttttcaagaacattgattttagagctcacactaagaaaaagaatacaaaaataatggcatagaaagtgaaaaaacaaaaataaaaagtagaaagctaaagtttcccattaaaatgatcaatatactgtgcagtaagtcaaatgtgtacaatgaattaagaaaatatgatatataaaaatccaaatttacaaaattaagtacaaataggtgtttatattacaaagtgatactggtttataaaaggattcaacatagattttttttaaatggttgttttcctcaatcaatttaacaatgattttaaatgtataaaattttaatatctctttgagacagtgatccaagcttcttcccttgatgatgttaccagttcatactttgtttcaataacctgtccctccacagaaagtaggtgcagtctcttcaccaatacactaagaagtactgtggtcaccatatatgcaaacctcaactctggacactcctgtgtgcctgagaatccaagtgaggaaaaagttttcattactaattcatcatcaaaccgatctggatcaaacttgtgtggagatggccaagtattaggatcctgaagtaccacaccaagggcataaaggacgagggtctctctaggaataataaatcggtcaatttttccttcaatatcttgaagctgggcagaaactggagtcagtttggcagttcgaacagtttcacaaagcacatgctgacaatatattttgcagttattatgcaactggccagagaaaatatcatactgtcttctaggatctgttggtcattaaggttcccttgtactaaggagtcaatgaaaatatgttgactgaagttccttccttttcgttcttttatgatgttccttaaaacagactccagttgcatgagggtgtgccatgattcttctggaagcgaatgacttcctgatcatcttcaaatgtactacccattaccatctgtgtaacagacttcatagcaaaaccaagcatatgctggctgaggggcacgtgctgggtctctgggtaggagagccatttatctaataattcttctgaaagctttaggaggagggcaaagttactcttcagagaatcagtcacaccattttcatacaattttttcctcatgtggttttcactcacactgccaccaccagattgataccttaataatgacttcagcatggtttcaaaagggtccgatgtcttattgggattgatatgctgcttcagtacatcaacagtgcccaaactaaccacgaggcgcctgccaaaccagaaggagaccacaggcccatatctctcatgcaaattaaccaggaactcatgcaaacttccactattcacaatatctggaagattaccatctttttcttcagttggagtaatccctggaattcctgcagcttgtctggaagccggatagaggtagagcacggctcccaccaacgccagcaagaaggtaacggcgaagatcgcgaagtccaacatggttctgccgcccagggagccacgtctcggatcggccgctccagc

SEQ ID NO: 13069 - RNA, 8797 nt, Homo sapiens
  source 1..8797: mol_type = other RNA
gctgggattacaggcatgagccaccacacccagctggaaaatgtttaaaatttattaagtgaaaagtaactcatgctgcaatgaacgtactatgtaaaaatgtatgtatgtggaacagggaaaaatataaacagtcacagaaatgtgtttaggttggtagcattctttttcctcttaaaaattcctttttttggccgggcgctgtggctcacacctgtaatcccagcactttgggaagccgcggtggacagatcacaaggtcaggagatcaagaccatcctggctaacatggtgaaaccccgtctctactaaaaatacaaaaaattagctgggcatggaggcactcgcctgtagtcgcagctactcgggaggctgaggcaggagaatcgcttgaactggggagatggaggttgtagtgagcccagatcatgccactgcactcaagcctgggctgagacctccagagtctggctgagacctatggagtctcactctgtcacctaggctggagtacagtggtgcgatctcggcacactgcaacctccacctcccagacattctcctgcctcagcctctcaactagctgggattacattcgcccgcctccacacccactaatttttgtatttttagtagagatgcggtttccccatgttggccaggctgttcttgaactcctgacctcaagttatacgcccactttggactcccaaagtgctgggattacaggtgtgagccacggcaccagccaaaaatttctttaaatattagtggtatattattctctcaataagttttttttttttttttttttgagacagtcttgttttattgcctaagctggagtgcagtggcacaatctcaactcactgcaacctccacctcccaggtttattttttttctcatgcctcagcctcccaagaagctgggattacaggcatgtgccccaaaggccagttaagttttctttttctttttttcttttttcttggttgagacggattttcgctcgtcacccacactggagtgcaatggcgcgatctcggctcactgcaacctccgactcttgggttcaagcgattctcctgcctcagcctcccgagtagctgggattagaggcacctgtcaccacgcccgctacttttggtatttttagtagagatggagtttcaccacgttggccaggctgatctcaaactcctggcctcaagtgattcacctgccttggcctcccaaagtgctggaattacaggcccggcctatttttgcaataattatgaatagcacaccatttaaacctgttgattgagccctccttaaataactaaatacactactggccaacatggtgaaaacctgtctccactaaaaacacaaaaaaatggccgggcacagtggctcatgcctgtaatcccagcacttcaggaggccaaggggtgtgaatcacctgaggttaggagttcaagaccagcctggccaacatggtgaaaccctgtctctactaaaaaaaaatacaaaaattagctgagtgtagtggcacatacccgtagtctcagctactcaggaggctgaggcaggagaattgcttgaacctgggaggcaggggttgcagtgagccaagatcgtgccaccacactccagcctgggtgacacagcgagactccatctcaaaataaataaataaataaaaagaaagggaccgagcgcggtggctcatgcttgtaatcccagcactctgggaggctgagttgggcagatcacaaggtcaagagttcaggaccagcctgaccaacacggtaaaaccccatctctactaaaaatacaaaaatgagctgggtgtgatggcacgcgcctgtaaccccagttactcaaaaggctgaggcaagagaatcgcttgaacctgggaggcagaggttgcagtgagccgagatcacgccactgcattccagcctggtgacagtgagactctgtcacacacacacaaaaaagataaagaatgacaaaaatctgtgcctacattcagagtgacaagaatactaatgttctgcttgtagaaaagactattggttcagaatatgttaaatgcaaataatattttgtataatatatataaattacatatgcataaaaagagtatctatattagaatcttttgagacagggtcttgctctgtcaaccatgagggagtgcagtggcactaccacagctcactgtagccttgacttcctgagctcaagccatcctctcgcctcagcctcctgaatagttgggactgcaggtggtgccaccaaggctggctaagtttttatatttttttatagaaacaagcttttgccacgttgcccaggctggtctcaaacttctaaaagctcaagcaatctggccgccttgaactcccaaagtgcttgagttataggcatgagtcactgtgcccggcctacattagaatcttaacagtggggctgggcatggtgccccatgcctgtaatcccagcactttgggaggtcaaggtgggcagactacttgaggttgaggagttcgaggccagcctggccaacatggtgaaaccccatctgtactaaaaacacaaaaattagccaggtgtggtggcacatgtttgcaatcccagctacttgggaggctgaggcgggaggatcacttgaacctgggaagcagaggttgcagtgagccgagatggtgccatggcactccagcctgggcaatagacagcgggactcagtctcaaaacaaaaaaaaaaaaaaaaaaaaaagaatcttaacagtggttaacttcaaatagtgaaactatgactgttaactgagtttgacatttttgtgttttcctagatttttctacaataaacattattatttcataataaagcagtaaagactttttatacaaactattttaagataaacaaattttgacataggggttataagttaggtagaatctatttatataaaaaatggaactgtacttttgtgggccaaataagcactatgtaagtttttttaattttcccaaacacatgcacagaattaatattgccttaaattttgttagcacaagtttgagagagctctttagttcataaaaaaatgttttatggaccaggtgccgtggctcacacctgcaatctcaacactttgggaggcccaggtgggaggatcgcttgagcctaggagtttgagacaagactgggcgacgcagggagaccctgtctcaaaaaaacaaaaccaaaaacaagcaaacaaaaaaacagctgggcatggtggcatgcatatgtagtcccagctattctagaggctgaggtgagatcgctggagcccaggaggtggaggctacagtaagctgtgatcatgccaatgcactccagcttggtcaacaaagcaagactgtgcctcaaaaaaaaaaaagaaaagaaaagaaagaaagaaaagaaaaagaaaaaaagttatgtacgtatggtttttttttttttttggatagagtttcactcttcttgcccaggctggagtgcaatggtgcaatcttggctcaccacaaccttcccctactgggttcaagcgattctcctgtttcagcctccccagtagctgggattaaaggcatgtgccaccacgcccggctaattttgtatttttagtagagatgaagtttctccatgttggtcaggctggtcttgaactcctgacttcaggtgatctgcccgcctcagcctcccaaagtgctgggattacaggtgtgagccacctcgcctggccgttttttttttttttttttttttctgagacggagttttgctcttattgcccaggctggagtgcaatggcacgatctcggctcatcgcaacctctgcctcacgggttcaagcaattttcctgcctcagcgtctcaagtagctaggattacagggatgctccatcatgcccggctaattttgtatttttggtagagacagggtttctccatgttggtcaggctggtctcaaactcccaacctcaggtgatttacccgccttggcctcccaaagagctgggattacaggtgtgagccactgtgcccggccatgcttatgttttttaacaatacacttctgaactatcaaaaagaatataaatcaaaatcactgaagtagtttttaaaaactccaaaagctacaaaacttacttacttcaatatcaattaaaaacccatttgatagttcaataacttgagtcctgctagaatcattctataagccatcagtgacagtgaagtggccaaaatttgagtcacttgataagtacaaagaacacagatttttgtcattcttactgtgaagaaaaacagtgaatgaataacttagtttatatattaacagtacttttatttaaaaaattatctagagaataacttctttttaatcatttgttagtcatgtaactatggataaaacatactaatttagctgattcctctatgctctcttttccttgattccaatcattattagttattctacactgcctcatttattggcagttatgccaactggctgactctggttcaactgccctatttttgctttcatcattgtttatcatatctcacttgctttaaactccacctctttcatctcatctgatctgacacttggtttacatatcaattggctactctaaccttctaccgccagtttccaacccattcgaggtacttgggtaacaaaggaagatgctctatacacacaaaaccacagaaaataagtgggaagggataataaatttcacttaaagttttagaatttttcttttttttttgagacggagtttcactcttgttgcccaggctggagtgcaatggcgcgatcttggctcaccgcaacctctgcctcccaggttcaagcagttctcctgcttcagcctcccgagtagctggtattacaggcatgcaccaccaagcctggctaattttgtatttttagtagagacggggtttctccatgttggtcaggctggtcttgaacgcctgacctcaggtgatctgcctgcctcggcctcccaaagtgctgggattacaggcatgagccatcacgcccggccaaagttttagaatttaagttattccaaaaaaaattttttttttcaaaaatacagactgcatccaattaaattctatgttaactggtaatgactaggtctaaaatgttaggtatttaccaataaatgacataaaataactcaacaacaaagggatttttttttttaagagatagggtctcactttatcactcaggtttggctgagggcagtggtgtgatcacagctcactgaagcctccaactcctgggctcaagtgatcctcccgcctcagtctaccagagtatattcttgaaagtaaaattacaaatgaaattcagcagtgttaaaaataagcccacttgcagacaattatcatttttcttcctttctttcctcactatctgtacttggcatatttcctacagtggctgtcttaaagaaaaaaaggaatccttcacaaatagtgtagccaaaaaagttggactaatatacaatgctatcagtaaagtattatatataaaatttataagtgctaaagtgtaattttgaaagacacttaagatactccttttttttttgagacaaggtctcagccctgtcgcccaggctggagtgcactagcacaacatcagctcactgcaacctccgcctcccaggttcaagcgattctcctgcctcagcctcccaagtagctgagactacaggcgcacgccagcatgtccagataattttttgtatttttagtagagatggggtttcaccatgttggccaggatggtctcaaatctcttgacctcgtgatctgcccatgtcggcttcccaaagtgttaggataacaggcatgagctaccgtgcccagcctacttaaaatattcttgaaatagctctccccacctccttttttttttttttttgagaatgagtttcactcgacacccaggctggagtgcagtggtgcgatcttggctcactgcaacctctgcctcccaggttcaagcgattatcctgcctcagcctcctgagtagctgggattacaaatgtgcaccaccacatctggctaattttttttttttttttttgtatttttagtagagacggggtttcaccaagttggcctggctggtctcgaacacctgacctcaattgatccacctgcctcggcctcccaaagtattataggcatgagccaccgagcccggccttttttgttttttgtttttttaaaggcagggttttgctctgttgcccaggctggagtgcagtggtgtgatcacagatcactgcagccttgacctctcctggtctcaagtgatcctcccacctcagccttcagaacagctgggactacaggtgtgtgtcaccatgcccagtaatttttttgtatatttgtagaggcagggtctcccaatgttgcctgggctggtctcaaactcctgggctcaagcaatccaccagctttggccttccaaagttctaggattatacgcatgagccactgtgccctgccccaatattttgttacttactagtgagactaaacacttttctaaaagtttgttagccatactatcctataaaagctgtttgttcatgtcttttgtccatttatctttttttttgtttttcttgagacagagtcttgctctgtggcccaggctggagtgcaggggtgcaatctcggctcactgcaagctccgcctcccaggttcaaatgattctcctgcctcagcctcctgagtagctgggattacaggcatgtgccaccatgcccagctaatttttttgtgtgtgtttttcagtagagatggggtttcaccatgttggccaggctgatctcgaattcctgacctcaggtgctccacccgcctcagcctcccaaagtactgggattacaggggtgagccaccgcacccggccaattttctgtatttttaatagagacagggtttcatcctgttggccaggctggcctcgaacttcggacctcaggtgatccacccgcctcgacctcccaaagtgctgggattacaggtgtgggccaccacacccagccaatttttttgtatttttagtagagacagggtttcatcatgttggccaggctggtcgcaaactcctgacctcaggtgatccacccgcctcagcatcccaaagtgctgggattacaggcatgagccaccactcccggccaatgttttgtatttttagtagagatggggtttcatcatgttggccagactggtctcaaactctggacctcaggtgatccacctgcctcagcctcccaaagtgtagggattacaggtgtgagccaccgcgcccagcctatgtttctattttatacatattcaacaaacatgattccccaacttctgcaaaataatttctttttcaagaacattgattttagagctcacactaagaaaaagaatacaaaaataatggcatagaaagtgaaaaaacaaaaataaaaagtagaaagctaaagtttcccattaaaatgatcaatatactgtgcagtaagtcaaatgtgtacaatgaattaagaaaatatgatatataaaaatccaaatttacaaaattaagtacaaataggtgtttatattacaaagtgatactggtttataaaaggattcaacatagattttttttaaatggttgttttcctcaatcaatttaacaatgattttaaatgtataaaattttaatatctctttgagacagtgatccaagcttcttcccttgatgatgttaccagttcatactttgtttcaataacctgtccctccacagaaagtaggtgcagtctcttcaccaatacactaagaagtactgtggtcaccatatatgcaaacctcaactctggacactcctgtgtgcctgagaatccaagtgaggaaaaagttttcattactaattcatcatcaaaccgatctggatcaaacttgtgtggagatggccaagtattaggatcctgaagtaccacaccaagggcataaaggacgagggtctctctaggaataataaatcggtcaatttttccttcaatatcttgaagctgggcagaaactggagtcagtttggcagttcgaacagtttcacaaagcacatgctgacaatatattttgcagttattatgcaactggccagagaaaatatcatactgtcttctaggatctgttggtcattaaggttcccttgtactaaggagtcaatgaaaatatgttgactgaagttccttccttttcgttcttttatgatgttccttaaaacagactccagttgcatgagggtgtgccatgattcttctggaagcgaatgacttcctgatcatcttcaaatgtactacccattaccatctgtgtaacagacttcatagcaaaaccaagcatatgctggctgaggggcacgtgctgggtctctgggtaggagagccatttatctaataattcttctgaaagctttaggaggagggcaaagttactcttcagagaatcagtcacaccattttcatacaattttttcctcatgtggttttcactcacactgccaccaccagattgataccttaataatgacttcagcatggtttcaaaagggtccgcggatagaggtagagcacggctcccaccaacgccagcaagaaggtaacggcgaagatcgcgaagtccaacatggttctgccgcccagggagccacgtctcggatcggccgctccagc

SEQ ID NO: 13070 - RNA, 9238 nt, Homo sapiens
  source 1..9238: mol_type = other RNA
gctgggattacaggcatgagccaccacacccagctggaaaatgtttaaaatttattaagtgaaaagtaactcatgctgcaatgaacgtactatgtaaaaatgtatgtatgtggaacagggaaaaatataaacagtcacagaaatgtgtttaggttggtagcattctttttcctcttaaaaattcctttttttggccgggcgctgtggctcacacctgtaatcccagcactttgggaagccgcggtggacagatcacaaggtcaggagatcaagaccatcctggctaacatggtgaaaccccgtctctactaaaaatacaaaaaattagctgggcatggaggcactcgcctgtagtcgcagctactcgggaggctgaggcaggagaatcgcttgaactggggagatggaggttgtagtgagcccagatcatgccactgcactcaagcctgggctgagacctccagagtctggctgagacctatggagtctcactctgtcacctaggctggagtacagtggtgcgatctcggcacactgcaacctccacctcccagacattctcctgcctcagcctctcaactagctgggattacattcgcccgcctccacacccactaatttttgtatttttagtagagatgcggtttccccatgttggccaggctgttcttgaactcctgacctcaagttatacgcccactttggactcccaaagtgctgggattacaggtgtgagccacggcaccagccaaaaatttctttaaatattagtggtatattattctctcaataagttttttttttttttttttttgagacagtcttgttttattgcctaagctggagtgcagtggcacaatctcaactcactgcaacctccacctcccaggtttattttttttctcatgcctcagcctcccaagaagctgggattacaggcatgtgccccaaaggccagttaagttttctttttctttttttcttttttcttggttgagacggattttcgctcgtcacccacactggagtgcaatggcgcgatctcggctcactgcaacctccgactcttgggttcaagcgattctcctgcctcagcctcccgagtagctgggattagaggcacctgtcaccacgcccgctacttttggtatttttagtagagatggagtttcaccacgttggccaggctgatctcaaactcctggcctcaagtgattcacctgccttggcctcccaaagtgctggaattacaggcccggcctatttttgcaataattatgaatagcacaccatttaaacctgttgattgagccctccttaaataactaaatacactactggccaacatggtgaaaacctgtctccactaaaaacacaaaaaaatggccgggcacagtggctcatgcctgtaatcccagcacttcaggaggccaaggggtgtgaatcacctgaggttaggagttcaagaccagcctggccaacatggtgaaaccctgtctctactaaaaaaaaatacaaaaattagctgagtgtagtggcacatacccgtagtctcagctactcaggaggctgaggcaggagaattgcttgaacctgggaggcaggggttgcagtgagccaagatcgtgccaccacactccagcctgggtgacacagcgagactccatctcaaaataaataaataaataaaaagaaagggaccgagcgcggtggctcatgcttgtaatcccagcactctgggaggctgagttgggcagatcacaaggtcaagagttcaggaccagcctgaccaacacggtaaaaccccatctctactaaaaatacaaaaatgagctgggtgtgatggcacgcgcctgtaaccccagttactcaaaaggctgaggcaagagaatcgcttgaacctgggaggcagaggttgcagtgagccgagatcacgccactgcattccagcctggtgacagtgagactctgtcacacacacacaaaaaagataaagaatgacaaaaatctgtgcctacattcagagtgacaagaatactaatgttctgcttgtagaaaagactattggttcagaatatgttaaatgcaaataatattttgtataatatatataaattacatatgcataaaaagagtatctatattagaatcttttgagacagggtcttgctctgtcaaccatgagggagtgcagtggcactaccacagctcactgtagccttgacttcctgagctcaagccatcctctcgcctcagcctcctgaatagttgggactgcaggtggtgccaccaaggctggctaagtttttatatttttttatagaaacaagcttttgccacgttgcccaggctggtctcaaacttctaaaagctcaagcaatctggccgccttgaactcccaaagtgcttgagttataggcatgagtcactgtgcccggcctacattagaatcttaacagtggggctgggcatggtgccccatgcctgtaatcccagcactttgggaggtcaaggtgggcagactacttgaggttgaggagttcgaggccagcctggccaacatggtgaaaccccatctgtactaaaaacacaaaaattagccaggtgtggtggcacatgtttgcaatcccagctacttgggaggctgaggcgggaggatcacttgaacctgggaagcagaggttgcagtgagccgagatggtgccatggcactccagcctgggcaatagacagcgggactcagtctcaaaacaaaaaaaaaaaaaaaaaaaaaagaatcttaacagtggttaacttcaaatagtgaaactatgactgttaactgagtttgacatttttgtgttttcctagatttttctacaataaacattattatttcataataaagcagtaaagactttttatacaaactattttaagataaacaaattttgacataggggttataagttaggtagaatctatttatataaaaaatggaactgtacttttgtgggccaaataagcactatgtaagtttttttaattttcccaaacacatgcacagaattaatattgccttaaattttgttagcacaagtttgagagagctctttagttcataaaaaaatgttttatggaccaggtgccgtggctcacacctgcaatctcaacactttgggaggcccaggtgggaggatcgcttgagcctaggagtttgagacaagactgggcgacgcagggagaccctgtctcaaaaaaacaaaaccaaaaacaagcaaacaaaaaaacagctgggcatggtggcatgcatatgtagtcccagctattctagaggctgaggtgagatcgctggagcccaggaggtggaggctacagtaagctgtgatcatgccaatgcactccagcttggtcaacaaagcaagactgtgcctcaaaaaaaaaaaagaaaagaaaagaaagaaagaaaagaaaaagaaaaaaagttatgtacgtatggtttttttttttttttggatagagtttcactcttcttgcccaggctggagtgcaatggtgcaatcttggctcaccacaaccttcccctactgggttcaagcgattctcctgtttcagcctccccagtagctgggattaaaggcatgtgccaccacgcccggctaattttgtatttttagtagagatgaagtttctccatgttggtcaggctggtcttgaactcctgacttcaggtgatctgcccgcctcagcctcccaaagtgctgggattacaggtgtgagccacctcgcctggccgttttttttttttttttttttttctgagacggagttttgctcttattgcccaggctggagtgcaatggcacgatctcggctcatcgcaacctctgcctcacgggttcaagcaattttcctgcctcagcgtctcaagtagctaggattacagggatgctccatcatgcccggctaattttgtatttttggtagagacagggtttctccatgttggtcaggctggtctcaaactcccaacctcaggtgatttacccgccttggcctcccaaagagctgggattacaggtgtgagccactgtgcccggccatgcttatgttttttaacaatacacttctgaactatcaaaaagaatataaatcaaaatcactgaagtagtttttaaaaactccaaaagctacaaaacttacttacttcaatatcaattaaaaacccatttgatagttcaataacttgagtcctgctagaatcattctataagccatcagtgacagtgaagtggccaaaatttgagtcacttgataagtacaaagaacacagatttttgtcattcttactgtgaagaaaaacagtgaatgaataacttagtttatatattaacagtacttttatttaaaaaattatctagagaataacttctttttaatcatttgttagtcatgtaactatggataaaacatactaatttagctgattcctctatgctctcttttccttgattccaatcattattagttattctacactgcctcatttattggcagttatgccaactggctgactctggttcaactgccctatttttgctttcatcattgtttatcatatctcacttgctttaaactccacctctttcatctcatctgatctgacacttggtttacatatcaattggctactctaaccttctaccgccagtttccaacccattcgaggtacttgggtaacaaaggaagatgctctatacacacaaaaccacagaaaataagtgggaagggataataaatttcacttaaagttttagaatttttcttttttttttgagacggagtttcactcttgttgcccaggctggagtgcaatggcgcgatcttggctcaccgcaacctctgcctcccaggttcaagcagttctcctgcttcagcctcccgagtagctggtattacaggcatgcaccaccaagcctggctaattttgtatttttagtagagacggggtttctccatgttggtcaggctggtcttgaacgcctgacctcaggtgatctgcctgcctcggcctcccaaagtgctgggattacaggcatgagccatcacgcccggccaaagttttagaatttaagttattccaaaaaaaattttttttttcaaaaatacagactgcatccaattaaattctatgttaactggtaatgactaggtctaaaatgttaggtatttaccaataaatgacataaaataactcaacaacaaagggatttttttttttaagagatagggtctcactttatcactcaggtttggctgagggcagtggtgtgatcacagctcactgaagcctccaactcctgggctcaagtgatcctcccgcctcagtctaccagagtatattcttgaaagtaaaattacaaatgaaattcagcagtgttaaaaataagcccacttgcagacaattatcatttttcttcctttctttcctcactatctgtacttggcatatttcctacagtggctgtcttaaagaaaaaaaggaatccttcacaaatagtgtagccaaaaaagttggactaatatacaatgctatcagtaaagtattatatataaaatttataagtgctaaagtgtaattttgaaagacacttaagatactccttttttttttgagacaaggtctcagccctgtcgcccaggctggagtgcactagcacaacatcagctcactgcaacctccgcctcccaggttcaagcgattctcctgcctcagcctcccaagtagctgagactacaggcgcacgccagcatgtccagataattttttgtatttttagtagagatggggtttcaccatgttggccaggatggtctcaaatctcttgacctcgtgatctgcccatgtcggcttcccaaagtgttaggataacaggcatgagctaccgtgcccagcctacttaaaatattcttgaaatagctctccccacctccttttttttttttttttgagaatgagtttcactcgacacccaggctggagtgcagtggtgcgatcttggctcactgcaacctctgcctcccaggttcaagcgattatcctgcctcagcctcctgagtagctgggattacaaatgtgcaccaccacatctggctaattttttttttttttttttgtatttttagtagagacggggtttcaccaagttggcctggctggtctcgaacacctgacctcaattgatccacctgcctcggcctcccaaagtattataggcatgagccaccgagcccggccttttttgttttttgtttttttaaaggcagggttttgctctgttgcccaggctggagtgcagtggtgtgatcacagatcactgcagccttgacctctcctggtctcaagtgatcctcccacctcagccttcagaacagctgggactacaggtgtgtgtcaccatgcccagtaatttttttgtatatttgtagaggcagggtctcccaatgttgcctgggctggtctcaaactcctgggctcaagcaatccaccagctttggccttccaaagttctaggattatacgcatgagccactgtgccctgccccaatattttgttacttactagtgagactaaacacttttctaaaagtttgttagccatactatcctataaaagctgtttgttcatgtcttttgtccatttatctttttttttgtttttcttgagacagagtcttgctctgtggcccaggctggagtgcaggggtgcaatctcggctcactgcaagctccgcctcccaggttcaaatgattctcctgcctcagcctcctgagtagctgggattacaggcatgtgccaccatgcccagctaatttttttgtgtgtgtttttcagtagagatggggtttcaccatgttggccaggctgatctcgaattcctgacctcaggtgctccacccgcctcagcctcccaaagtactgggattacaggggtgagccaccgcacccggccaattttctgtatttttaatagagacagggtttcatcctgttggccaggctggcctcgaacttcggacctcaggtgatccacccgcctcgacctcccaaagtgctgggattacaggtgtgggccaccacacccagccaatttttttgtatttttagtagagacagggtttcatcatgttggccaggctggtcgcaaactcctgacctcaggtgatccacccgcctcagcatcccaaagtgctgggattacaggcatgagccaccactcccggccaatgttttgtatttttagtagagatggggtttcatcatgttggccagactggtctcaaactctggacctcaggtgatccacctgcctcagcctcccaaagtgtagggattacaggtgtgagccaccgcgcccagcctatgtttctattttatacatattcaacaaacatgattccccaacttctgcaaaataatttctttttcaagaacattgattttagagctcacactaagaaaaagaatacaaaaataatggcatagaaagtgaaaaaacaaaaataaaaagtagaaagctaaagtttcccattaaaatgatcaatatactgtgcagtaagtcaaatgtgtacaatgaattaagaaaatatgatatataaaaatccaaatttacaaaattaagtacaaataggtgtttatattacaaagtgatactggtttataaaaggattcaacatagattttttttaaatggttgttttcctcaatcaatttaacaatgattttaaatgtataaaattttaatatctctttgagacagtgatccaagcttcttcccttgatgatgttaccagttcatactttgtttcaataacctgtccctccacagaaagtaggtgcagtctcttcaccaatacactaagaagtactgtggtcaccatatatgcaaacctcaactctggacactcctgtgtgcctgagaatccaagtgaggaaaaagttttcattactaattcatcatcaaaccgatctggatcaaacttgtgtggagatggccaagtattaggatcctgaagtaccacaccaagggcataaaggacgagggtctctctaggaataataaatcggtcaatttttccttcaatatcttgaagctgggcagaaactggagtcagtttggcagttcgaacagtttcacaaagcacatgctgacaatatctgagctgctcaattttctctggagtaacaggaccatttccaaaaacttggtttatctcttcatataattttttttgaacttcttcagaggtggttaaaaaacagattgcccaggtacacaattttgcagttattatgcaactggccagagaaaatatcatactgtcttctaggatctgttggtcattaaggttcccttgtactaaggagtcaatgaaaatatgttgactgaagttccttccttttcgttcttttatgatgttccttaaaacagactccagttgcatgagggcatcttcatattgttttttccgagtcatgtttttatcaagtgacccatctagaaagccttttccaatctcagaccaaacctgaaaataggtaaatatacataatgtgccatgattcttctggaagcgaatgacttcctgatcatcttcaaatgtactacccattaccatctgtgtaacagacttcatagcaaaaccaagcatatgctggctgaggggcacgtgctgggtctctgggtaggagagccatttatctaataattcttctgaaagctttaggaggagggcaaagttactcttcagagaatcagtcacaccattttcatacaattttttcctcatgtggttttcactcacactgccaccaccagattgataccttaataatgacttcagcatggtttcaaaagggtccgatgtcttattgggattgatatgctgcttcagtacatcaacagtgcccaaactaaccacgaggcgcctgccaaaccagaaggagaccacaggcccatatctctcatgcaaattaaccaggaactcatgcaaacttccactattcacaatatctggaagattaccatctttttcttcagttggagtaatccctggaattcctgcagcttgtctggaagccggatagaggtagagcacggctcccaccaacgccagcaagaaggtaacggcgaagatcgcgaagtccaacatggttctgccgcccagggagccacgtctcggatcggccgctccagc

SEQ ID NO: 13071 - RNA, 8941 nt, Homo sapiens
  source 1..8941: mol_type = other RNA
gctgggattacaggcatgagccaccacacccagctggaaaatgtttaaaatttattaagtgaaaagtaactcatgctgcaatgaacgtactatgtaaaaatgtatgtatgtggaacagggaaaaatataaacagtcacagaaatgtgtttaggttggtagcattctttttcctcttaaaaattcctttttttggccgggcgctgtggctcacacctgtaatcccagcactttgggaagccgcggtggacagatcacaaggtcaggagatcaagaccatcctggctaacatggtgaaaccccgtctctactaaaaatacaaaaaattagctgggcatggaggcactcgcctgtagtcgcagctactcgggaggctgaggcaggagaatcgcttgaactggggagatggaggttgtagtgagcccagatcatgccactgcactcaagcctgggctgagacctccagagtctggctgagacctatggagtctcactctgtcacctaggctggagtacagtggtgcgatctcggcacactgcaacctccacctcccagacattctcctgcctcagcctctcaactagctgggattacattcgcccgcctccacacccactaatttttgtatttttagtagagatgcggtttccccatgttggccaggctgttcttgaactcctgacctcaagttatacgcccactttggactcccaaagtgctgggattacaggtgtgagccacggcaccagccaaaaatttctttaaatattagtggtatattattctctcaataagttttttttttttttttttttgagacagtcttgttttattgcctaagctggagtgcagtggcacaatctcaactcactgcaacctccacctcccaggtttattttttttctcatgcctcagcctcccaagaagctgggattacaggcatgtgccccaaaggccagttaagttttctttttctttttttcttttttcttggttgagacggattttcgctcgtcacccacactggagtgcaatggcgcgatctcggctcactgcaacctccgactcttgggttcaagcgattctcctgcctcagcctcccgagtagctgggattagaggcacctgtcaccacgcccgctacttttggtatttttagtagagatggagtttcaccacgttggccaggctgatctcaaactcctggcctcaagtgattcacctgccttggcctcccaaagtgctggaattacaggcccggcctatttttgcaataattatgaatagcacaccatttaaacctgttgattgagccctccttaaataactaaatacactactggccaacatggtgaaaacctgtctccactaaaaacacaaaaaaatggccgggcacagtggctcatgcctgtaatcccagcacttcaggaggccaaggggtgtgaatcacctgaggttaggagttcaagaccagcctggccaacatggtgaaaccctgtctctactaaaaaaaaatacaaaaattagctgagtgtagtggcacatacccgtagtctcagctactcaggaggctgaggcaggagaattgcttgaacctgggaggcaggggttgcagtgagccaagatcgtgccaccacactccagcctgggtgacacagcgagactccatctcaaaataaataaataaataaaaagaaagggaccgagcgcggtggctcatgcttgtaatcccagcactctgggaggctgagttgggcagatcacaaggtcaagagttcaggaccagcctgaccaacacggtaaaaccccatctctactaaaaatacaaaaatgagctgggtgtgatggcacgcgcctgtaaccccagttactcaaaaggctgaggcaagagaatcgcttgaacctgggaggcagaggttgcagtgagccgagatcacgccactgcattccagcctggtgacagtgagactctgtcacacacacacaaaaaagataaagaatgacaaaaatctgtgcctacattcagagtgacaagaatactaatgttctgcttgtagaaaagactattggttcagaatatgttaaatgcaaataatattttgtataatatatataaattacatatgcataaaaagagtatctatattagaatcttttgagacagggtcttgctctgtcaaccatgagggagtgcagtggcactaccacagctcactgtagccttgacttcctgagctcaagccatcctctcgcctcagcctcctgaatagttgggactgcaggtggtgccaccaaggctggctaagtttttatatttttttatagaaacaagcttttgccacgttgcccaggctggtctcaaacttctaaaagctcaagcaatctggccgccttgaactcccaaagtgcttgagttataggcatgagtcactgtgcccggcctacattagaatcttaacagtggggctgggcatggtgccccatgcctgtaatcccagcactttgggaggtcaaggtgggcagactacttgaggttgaggagttcgaggccagcctggccaacatggtgaaaccccatctgtactaaaaacacaaaaattagccaggtgtggtggcacatgtttgcaatcccagctacttgggaggctgaggcgggaggatcacttgaacctgggaagcagaggttgcagtgagccgagatggtgccatggcactccagcctgggcaatagacagcgggactcagtctcaaaacaaaaaaaaaaaaaaaaaaaaaagaatcttaacagtggttaacttcaaatagtgaaactatgactgttaactgagtttgacatttttgtgttttcctagatttttctacaataaacattattatttcataataaagcagtaaagactttttatacaaactattttaagataaacaaattttgacataggggttataagttaggtagaatctatttatataaaaaatggaactgtacttttgtgggccaaataagcactatgtaagtttttttaattttcccaaacacatgcacagaattaatattgccttaaattttgttagcacaagtttgagagagctctttagttcataaaaaaatgttttatggaccaggtgccgtggctcacacctgcaatctcaacactttgggaggcccaggtgggaggatcgcttgagcctaggagtttgagacaagactgggcgacgcagggagaccctgtctcaaaaaaacaaaaccaaaaacaagcaaacaaaaaaacagctgggcatggtggcatgcatatgtagtcccagctattctagaggctgaggtgagatcgctggagcccaggaggtggaggctacagtaagctgtgatcatgccaatgcactccagcttggtcaacaaagcaagactgtgcctcaaaaaaaaaaaagaaaagaaaagaaagaaagaaaagaaaaagaaaaaaagttatgtacgtatggtttttttttttttttggatagagtttcactcttcttgcccaggctggagtgcaatggtgcaatcttggctcaccacaaccttcccctactgggttcaagcgattctcctgtttcagcctccccagtagctgggattaaaggcatgtgccaccacgcccggctaattttgtatttttagtagagatgaagtttctccatgttggtcaggctggtcttgaactcctgacttcaggtgatctgcccgcctcagcctcccaaagtgctgggattacaggtgtgagccacctcgcctggccgttttttttttttttttttttttctgagacggagttttgctcttattgcccaggctggagtgcaatggcacgatctcggctcatcgcaacctctgcctcacgggttcaagcaattttcctgcctcagcgtctcaagtagctaggattacagggatgctccatcatgcccggctaattttgtatttttggtagagacagggtttctccatgttggtcaggctggtctcaaactcccaacctcaggtgatttacccgccttggcctcccaaagagctgggattacaggtgtgagccactgtgcccggccatgcttatgttttttaacaatacacttctgaactatcaaaaagaatataaatcaaaatcactgaagtagtttttaaaaactccaaaagctacaaaacttacttacttcaatatcaattaaaaacccatttgatagttcaataacttgagtcctgctagaatcattctataagccatcagtgacagtgaagtggccaaaatttgagtcacttgataagtacaaagaacacagatttttgtcattcttactgtgaagaaaaacagtgaatgaataacttagtttatatattaacagtacttttatttaaaaaattatctagagaataacttctttttaatcatttgttagtcatgtaactatggataaaacatactaatttagctgattcctctatgctctcttttccttgattccaatcattattagttattctacactgcctcatttattggcagttatgccaactggctgactctggttcaactgccctatttttgctttcatcattgtttatcatatctcacttgctttaaactccacctctttcatctcatctgatctgacacttggtttacatatcaattggctactctaaccttctaccgccagtttccaacccattcgaggtacttgggtaacaaaggaagatgctctatacacacaaaaccacagaaaataagtgggaagggataataaatttcacttaaagttttagaatttttcttttttttttgagacggagtttcactcttgttgcccaggctggagtgcaatggcgcgatcttggctcaccgcaacctctgcctcccaggttcaagcagttctcctgcttcagcctcccgagtagctggtattacaggcatgcaccaccaagcctggctaattttgtatttttagtagagacggggtttctccatgttggtcaggctggtcttgaacgcctgacctcaggtgatctgcctgcctcggcctcccaaagtgctgggattacaggcatgagccatcacgcccggccaaagttttagaatttaagttattccaaaaaaaattttttttttcaaaaatacagactgcatccaattaaattctatgttaactggtaatgactaggtctaaaatgttaggtatttaccaataaatgacataaaataactcaacaacaaagggatttttttttttaagagatagggtctcactttatcactcaggtttggctgagggcagtggtgtgatcacagctcactgaagcctccaactcctgggctcaagtgatcctcccgcctcagtctaccagagtatattcttgaaagtaaaattacaaatgaaattcagcagtgttaaaaataagcccacttgcagacaattatcatttttcttcctttctttcctcactatctgtacttggcatatttcctacagtggctgtcttaaagaaaaaaaggaatccttcacaaatagtgtagccaaaaaagttggactaatatacaatgctatcagtaaagtattatatataaaatttataagtgctaaagtgtaattttgaaagacacttaagatactccttttttttttgagacaaggtctcagccctgtcgcccaggctggagtgcactagcacaacatcagctcactgcaacctccgcctcccaggttcaagcgattctcctgcctcagcctcccaagtagctgagactacaggcgcacgccagcatgtccagataattttttgtatttttagtagagatggggtttcaccatgttggccaggatggtctcaaatctcttgacctcgtgatctgcccatgtcggcttcccaaagtgttaggataacaggcatgagctaccgtgcccagcctacttaaaatattcttgaaatagctctccccacctccttttttttttttttttgagaatgagtttcactcgacacccaggctggagtgcagtggtgcgatcttggctcactgcaacctctgcctcccaggttcaagcgattatcctgcctcagcctcctgagtagctgggattacaaatgtgcaccaccacatctggctaattttttttttttttttttgtatttttagtagagacggggtttcaccaagttggcctggctggtctcgaacacctgacctcaattgatccacctgcctcggcctcccaaagtattataggcatgagccaccgagcccggccttttttgttttttgtttttttaaaggcagggttttgctctgttgcccaggctggagtgcagtggtgtgatcacagatcactgcagccttgacctctcctggtctcaagtgatcctcccacctcagccttcagaacagctgggactacaggtgtgtgtcaccatgcccagtaatttttttgtatatttgtagaggcagggtctcccaatgttgcctgggctggtctcaaactcctgggctcaagcaatccaccagctttggccttccaaagttctaggattatacgcatgagccactgtgccctgccccaatattttgttacttactagtgagactaaacacttttctaaaagtttgttagccatactatcctataaaagctgtttgttcatgtcttttgtccatttatctttttttttgtttttcttgagacagagtcttgctctgtggcccaggctggagtgcaggggtgcaatctcggctcactgcaagctccgcctcccaggttcaaatgattctcctgcctcagcctcctgagtagctgggattacaggcatgtgccaccatgcccagctaatttttttgtgtgtgtttttcagtagagatggggtttcaccatgttggccaggctgatctcgaattcctgacctcaggtgctccacccgcctcagcctcccaaagtactgggattacaggggtgagccaccgcacccggccaattttctgtatttttaatagagacagggtttcatcctgttggccaggctggcctcgaacttcggacctcaggtgatccacccgcctcgacctcccaaagtgctgggattacaggtgtgggccaccacacccagccaatttttttgtatttttagtagagacagggtttcatcatgttggccaggctggtcgcaaactcctgacctcaggtgatccacccgcctcagcatcccaaagtgctgggattacaggcatgagccaccactcccggccaatgttttgtatttttagtagagatggggtttcatcatgttggccagactggtctcaaactctggacctcaggtgatccacctgcctcagcctcccaaagtgtagggattacaggtgtgagccaccgcgcccagcctatgtttctattttatacatattcaacaaacatgattccccaacttctgcaaaataatttctttttcaagaacattgattttagagctcacactaagaaaaagaatacaaaaataatggcatagaaagtgaaaaaacaaaaataaaaagtagaaagctaaagtttcccattaaaatgatcaatatactgtgcagtaagtcaaatgtgtacaatgaattaagaaaatatgatatataaaaatccaaatttacaaaattaagtacaaataggtgtttatattacaaagtgatactggtttataaaaggattcaacatagattttttttaaatggttgttttcctcaatcaatttaacaatgattttaaatgtataaaattttaatatctctttgagacagtgatccaagcttcttcccttgatgatgttaccagttcatactttgtttcaataacctgtccctccacagaaagtaggtgcagtctcttcaccaatacactaagaagtactgtggtcaccatatatgcaaacctcaactctggacactcctgtgtgcctgagaatccaagtgaggaaaaagttttcattactaattcatcatcaaaccgatctggatcaaacttgtgtggagatggccaagtattaggatcctgaagtaccacaccaagggcataaaggacgagggtctctctaggaataataaatcggtcaatttttccttcaatatcttgaagctgggcagaaactggagtcagtttggcagttcgaacagtttcacaaagcacatgctgacaatatctgagctgctcaattttctctggagtaacaggaccatttccaaaaacttggtttatctcttcatataattttttttgaacttcttcagaggtggttaaaaaacagattgcccaggtacacaattttgcagttattatgcaactggccagagaaaatatcatactgtcttctaggatctgttggtcattaaggttcccttgtactaaggagtcaatgaaaatatgttgactgaagttccttccttttcgttcttttatgatgttccttaaaacagactccagttgcatgagggcatcttcatattgttttttccgagtcatgtttttatcaagtgacccatctagaaagccttttccaatctcagaccaaactgtgccatgattcttctggaagcgaatgacttcctgatcatcttcaaatgtactacccattaccatctgtgtaacagacttcatagcaaaaccaagcatatgctggctgaggggcacgtgctgggtctctgggtaggagagccatttatctaataattcttctgaaagcttaataatgacttcagcatggtttcaaaagggtccgttttcttcagttggagtaatccctggaattcctgcagcttgtctggaagccggatagaggtagagcacggctcccaccaacgccagcaagaaggtaacggcgaagatcgcgaagtccaacatggttctgccgcccagggagccacgtctcggatcggccgctccagc

SEQ ID NO: 13072 - RNA, 9214 nt, Homo sapiens
  source 1..9214: mol_type = other RNA
gctgggattacaggcatgagccaccacacccagctggaaaatgtttaaaatttattaagtgaaaagtaactcatgctgcaatgaacgtactatgtaaaaatgtatgtatgtggaacagggaaaaatataaacagtcacagaaatgtgtttaggttggtagcattctttttcctcttaaaaattcctttttttggccgggcgctgtggctcacacctgtaatcccagcactttgggaagccgcggtggacagatcacaaggtcaggagatcaagaccatcctggctaacatggtgaaaccccgtctctactaaaaatacaaaaaattagctgggcatggaggcactcgcctgtagtcgcagctactcgggaggctgaggcaggagaatcgcttgaactggggagatggaggttgtagtgagcccagatcatgccactgcactcaagcctgggctgagacctccagagtctggctgagacctatggagtctcactctgtcacctaggctggagtacagtggtgcgatctcggcacactgcaacctccacctcccagacattctcctgcctcagcctctcaactagctgggattacattcgcccgcctccacacccactaatttttgtatttttagtagagatgcggtttccccatgttggccaggctgttcttgaactcctgacctcaagttatacgcccactttggactcccaaagtgctgggattacaggtgtgagccacggcaccagccaaaaatttctttaaatattagtggtatattattctctcaataagttttttttttttttttttttgagacagtcttgttttattgcctaagctggagtgcagtggcacaatctcaactcactgcaacctccacctcccaggtttattttttttctcatgcctcagcctcccaagaagctgggattacaggcatgtgccccaaaggccagttaagttttctttttctttttttcttttttcttggttgagacggattttcgctcgtcacccacactggagtgcaatggcgcgatctcggctcactgcaacctccgactcttgggttcaagcgattctcctgcctcagcctcccgagtagctgggattagaggcacctgtcaccacgcccgctacttttggtatttttagtagagatggagtttcaccacgttggccaggctgatctcaaactcctggcctcaagtgattcacctgccttggcctcccaaagtgctggaattacaggcccggcctatttttgcaataattatgaatagcacaccatttaaacctgttgattgagccctccttaaataactaaatacactactggccaacatggtgaaaacctgtctccactaaaaacacaaaaaaatggccgggcacagtggctcatgcctgtaatcccagcacttcaggaggccaaggggtgtgaatcacctgaggttaggagttcaagaccagcctggccaacatggtgaaaccctgtctctactaaaaaaaaatacaaaaattagctgagtgtagtggcacatacccgtagtctcagctactcaggaggctgaggcaggagaattgcttgaacctgggaggcaggggttgcagtgagccaagatcgtgccaccacactccagcctgggtgacacagcgagactccatctcaaaataaataaataaataaaaagaaagggaccgagcgcggtggctcatgcttgtaatcccagcactctgggaggctgagttgggcagatcacaaggtcaagagttcaggaccagcctgaccaacacggtaaaaccccatctctactaaaaatacaaaaatgagctgggtgtgatggcacgcgcctgtaaccccagttactcaaaaggctgaggcaagagaatcgcttgaacctgggaggcagaggttgcagtgagccgagatcacgccactgcattccagcctggtgacagtgagactctgtcacacacacacaaaaaagataaagaatgacaaaaatctgtgcctacattcagagtgacaagaatactaatgttctgcttgtagaaaagactattggttcagaatatgttaaatgcaaataatattttgtataatatatataaattacatatgcataaaaagagtatctatattagaatcttttgagacagggtcttgctctgtcaaccatgagggagtgcagtggcactaccacagctcactgtagccttgacttcctgagctcaagccatcctctcgcctcagcctcctgaatagttgggactgcaggtggtgccaccaaggctggctaagtttttatatttttttatagaaacaagcttttgccacgttgcccaggctggtctcaaacttctaaaagctcaagcaatctggccgccttgaactcccaaagtgcttgagttataggcatgagtcactgtgcccggcctacattagaatcttaacagtggggctgggcatggtgccccatgcctgtaatcccagcactttgggaggtcaaggtgggcagactacttgaggttgaggagttcgaggccagcctggccaacatggtgaaaccccatctgtactaaaaacacaaaaattagccaggtgtggtggcacatgtttgcaatcccagctacttgggaggctgaggcgggaggatcacttgaacctgggaagcagaggttgcagtgagccgagatggtgccatggcactccagcctgggcaatagacagcgggactcagtctcaaaacaaaaaaaaaaaaaaaaaaaaaagaatcttaacagtggttaacttcaaatagtgaaactatgactgttaactgagtttgacatttttgtgttttcctagatttttctacaataaacattattatttcataataaagcagtaaagactttttatacaaactattttaagataaacaaattttgacataggggttataagttaggtagaatctatttatataaaaaatggaactgtacttttgtgggccaaataagcactatgtaagtttttttaattttcccaaacacatgcacagaattaatattgccttaaattttgttagcacaagtttgagagagctctttagttcataaaaaaatgttttatggaccaggtgccgtggctcacacctgcaatctcaacactttgggaggcccaggtgggaggatcgcttgagcctaggagtttgagacaagactgggcgacgcagggagaccctgtctcaaaaaaacaaaaccaaaaacaagcaaacaaaaaaacagctgggcatggtggcatgcatatgtagtcccagctattctagaggctgaggtgagatcgctggagcccaggaggtggaggctacagtaagctgtgatcatgccaatgcactccagcttggtcaacaaagcaagactgtgcctcaaaaaaaaaaaagaaaagaaaagaaagaaagaaaagaaaaagaaaaaaagttatgtacgtatggtttttttttttttttggatagagtttcactcttcttgcccaggctggagtgcaatggtgcaatcttggctcaccacaaccttcccctactgggttcaagcgattctcctgtttcagcctccccagtagctgggattaaaggcatgtgccaccacgcccggctaattttgtatttttagtagagatgaagtttctccatgttggtcaggctggtcttgaactcctgacttcaggtgatctgcccgcctcagcctcccaaagtgctgggattacaggtgtgagccacctcgcctggccgttttttttttttttttttttttctgagacggagttttgctcttattgcccaggctggagtgcaatggcacgatctcggctcatcgcaacctctgcctcacgggttcaagcaattttcctgcctcagcgtctcaagtagctaggattacagggatgctccatcatgcccggctaattttgtatttttggtagagacagggtttctccatgttggtcaggctggtctcaaactcccaacctcaggtgatttacccgccttggcctcccaaagagctgggattacaggtgtgagccactgtgcccggccatgcttatgttttttaacaatacacttctgaactatcaaaaagaatataaatcaaaatcactgaagtagtttttaaaaactccaaaagctacaaaacttacttacttcaatatcaattaaaaacccatttgatagttcaataacttgagtcctgctagaatcattctataagccatcagtgacagtgaagtggccaaaatttgagtcacttgataagtacaaagaacacagatttttgtcattcttactgtgaagaaaaacagtgaatgaataacttagtttatatattaacagtacttttatttaaaaaattatctagagaataacttctttttaatcatttgttagtcatgtaactatggataaaacatactaatttagctgattcctctatgctctcttttccttgattccaatcattattagttattctacactgcctcatttattggcagttatgccaactggctgactctggttcaactgccctatttttgctttcatcattgtttatcatatctcacttgctttaaactccacctctttcatctcatctgatctgacacttggtttacatatcaattggctactctaaccttctaccgccagtttccaacccattcgaggtacttgggtaacaaaggaagatgctctatacacacaaaaccacagaaaataagtgggaagggataataaatttcacttaaagttttagaatttttcttttttttttgagacggagtttcactcttgttgcccaggctggagtgcaatggcgcgatcttggctcaccgcaacctctgcctcccaggttcaagcagttctcctgcttcagcctcccgagtagctggtattacaggcatgcaccaccaagcctggctaattttgtatttttagtagagacggggtttctccatgttggtcaggctggtcttgaacgcctgacctcaggtgatctgcctgcctcggcctcccaaagtgctgggattacaggcatgagccatcacgcccggccaaagttttagaatttaagttattccaaaaaaaattttttttttcaaaaatacagactgcatccaattaaattctatgttaactggtaatgactaggtctaaaatgttaggtatttaccaataaatgacataaaataactcaacaacaaagggatttttttttttaagagatagggtctcactttatcactcaggtttggctgagggcagtggtgtgatcacagctcactgaagcctccaactcctgggctcaagtgatcctcccgcctcagtctaccagagtatattcttgaaagtaaaattacaaatgaaattcagcagtgttaaaaataagcccacttgcagacaattatcatttttcttcctttctttcctcactatctgtacttggcatatttcctacagtggctgtcttaaagaaaaaaaggaatccttcacaaatagtgtagccaaaaaagttggactaatatacaatgctatcagtaaagtattatatataaaatttataagtgctaaagtgtaattttgaaagacacttaagatactccttttttttttgagacaaggtctcagccctgtcgcccaggctggagtgcactagcacaacatcagctcactgcaacctccgcctcccaggttcaagcgattctcctgcctcagcctcccaagtagctgagactacaggcgcacgccagcatgtccagataattttttgtatttttagtagagatggggtttcaccatgttggccaggatggtctcaaatctcttgacctcgtgatctgcccatgtcggcttcccaaagtgttaggataacaggcatgagctaccgtgcccagcctacttaaaatattcttgaaatagctctccccacctccttttttttttttttttgagaatgagtttcactcgacacccaggctggagtgcagtggtgcgatcttggctcactgcaacctctgcctcccaggttcaagcgattatcctgcctcagcctcctgagtagctgggattacaaatgtgcaccaccacatctggctaattttttttttttttttttgtatttttagtagagacggggtttcaccaagttggcctggctggtctcgaacacctgacctcaattgatccacctgcctcggcctcccaaagtattataggcatgagccaccgagcccggccttttttgttttttgtttttttaaaggcagggttttgctctgttgcccaggctggagtgcagtggtgtgatcacagatcactgcagccttgacctctcctggtctcaagtgatcctcccacctcagccttcagaacagctgggactacaggtgtgtgtcaccatgcccagtaatttttttgtatatttgtagaggcagggtctcccaatgttgcctgggctggtctcaaactcctgggctcaagcaatccaccagctttggccttccaaagttctaggattatacgcatgagccactgtgccctgccccaatattttgttacttactagtgagactaaacacttttctaaaagtttgttagccatactatcctataaaagctgtttgttcatgtcttttgtccatttatctttttttttgtttttcttgagacagagtcttgctctgtggcccaggctggagtgcaggggtgcaatctcggctcactgcaagctccgcctcccaggttcaaatgattctcctgcctcagcctcctgagtagctgggattacaggcatgtgccaccatgcccagctaatttttttgtgtgtgtttttcagtagagatggggtttcaccatgttggccaggctgatctcgaattcctgacctcaggtgctccacccgcctcagcctcccaaagtactgggattacaggggtgagccaccgcacccggccaattttctgtatttttaatagagacagggtttcatcctgttggccaggctggcctcgaacttcggacctcaggtgatccacccgcctcgacctcccaaagtgctgggattacaggtgtgggccaccacacccagccaatttttttgtatttttagtagagacagggtttcatcatgttggccaggctggtcgcaaactcctgacctcaggtgatccacccgcctcagcatcccaaagtgctgggattacaggcatgagccaccactcccggccaatgttttgtatttttagtagagatggggtttcatcatgttggccagactggtctcaaactctggacctcaggtgatccacctgcctcagcctcccaaagtgtagggattacaggtgtgagccaccgcgcccagcctatgtttctattttatacatattcaacaaacatgattccccaacttctgcaaaataatttctttttcaagaacattgattttagagctcacactaagaaaaagaatacaaaaataatggcatagaaagtgaaaaaacaaaaataaaaagtagaaagctaaagtttcccattaaaatgatcaatatactgtgcagtaagtcaaatgtgtacaatgaattaagaaaatatgatatataaaaatccaaatttacaaaattaagtacaaataggtgtttatattacaaagtgatactggtttataaaaggattcaacatagattttttttaaatggttgttttcctcaatcaatttaacaatgattttaaatgtataaaattttaatatctctttgagacagtgatccaagcttcttcccttgatgatgttaccagttcatactttgtttcaataacctgtccctccacagaaagtaggtgcagtctcttcaccaatacactaagaagtactgtggtcaccatatatgcaaacctcaactctggacactcctgtgtgcctgagaatccaagtgaggaaaaagttttcattactaattcatcatcaaaccgatctggatcaaacttgtgtggagatggccaagtattaggatcctgaagtaccacaccaagggcataaaggacgagggtctctctaggaataataaatcggtcaatttttccttcaatatcttgaagctgggcagaaactggagtcagtttggcagttcgaacagtttcacaaagcacatgctgacaatatctgagctgctcaattttctctggagtaacaggaccatttccaaaaacttggtttatctcttcatataattttttttgaacttcttcagaggtggttaaaaaacagattgcccaggtacacaattttgcagttattatgcaactggccagagaaaatatcatactgtcttctaggatctgttggtcattaaggttcccttgtactaaggagtcaatgaaaatatgttgactgaagttccttccttttcgttcttttatgatgttccttaaaacagactccagttgcatgagggcatcttcatattgttttttccgagtcatgtttttatcaagtgacccatctagaaagccttttccaatctcagaccaaactgtgccatgattcttctggaagcgaatgacttcctgatcatcttcaaatgtactacccattaccatctgtgtaacagacttcatagcaaaaccaagcatatgctggctgaggggcacgtgctgggtctctgggtaggagagccatttatctaataattcttctgaaagctttaggaggagggcaaagttactcttcagagaatcagtcacaccattttcatacaattttttcctcatgtggttttcactcacactgccaccaccagattgataccttaataatgacttcagcatggtttcaaaagggtccgatgtcttattgggattgatatgctgcttcagtacatcaacagtgcccaaactaaccacgaggcgcctgccaaaccagaaggagaccacaggcccatatctctcatgcaaattaaccaggaactcatgcaaacttccactattcacaatatctggaagattaccatctttttcttcagttggagtaatccctggaattcctgcagcttgtctggaagccggatagaggtagagcacggctcccaccaacgccagcaagaaggtaacggcgaagatcgcgaagtccaacatggttctgccgcccagggagccacgtctcggatcggccgctccagc

SEQ ID NO: 13073 - RNA, 8997 nt, Homo sapiens
  source 1..8997: mol_type = other RNA
gctgggattacaggcatgagccaccacacccagctggaaaatgtttaaaatttattaagtgaaaagtaactcatgctgcaatgaacgtactatgtaaaaatgtatgtatgtggaacagggaaaaatataaacagtcacagaaatgtgtttaggttggtagcattctttttcctcttaaaaattcctttttttggccgggcgctgtggctcacacctgtaatcccagcactttgggaagccgcggtggacagatcacaaggtcaggagatcaagaccatcctggctaacatggtgaaaccccgtctctactaaaaatacaaaaaattagctgggcatggaggcactcgcctgtagtcgcagctactcgggaggctgaggcaggagaatcgcttgaactggggagatggaggttgtagtgagcccagatcatgccactgcactcaagcctgggctgagacctccagagtctggctgagacctatggagtctcactctgtcacctaggctggagtacagtggtgcgatctcggcacactgcaacctccacctcccagacattctcctgcctcagcctctcaactagctgggattacattcgcccgcctccacacccactaatttttgtatttttagtagagatgcggtttccccatgttggccaggctgttcttgaactcctgacctcaagttatacgcccactttggactcccaaagtgctgggattacaggtgtgagccacggcaccagccaaaaatttctttaaatattagtggtatattattctctcaataagttttttttttttttttttttgagacagtcttgttttattgcctaagctggagtgcagtggcacaatctcaactcactgcaacctccacctcccaggtttattttttttctcatgcctcagcctcccaagaagctgggattacaggcatgtgccccaaaggccagttaagttttctttttctttttttcttttttcttggttgagacggattttcgctcgtcacccacactggagtgcaatggcgcgatctcggctcactgcaacctccgactcttgggttcaagcgattctcctgcctcagcctcccgagtagctgggattagaggcacctgtcaccacgcccgctacttttggtatttttagtagagatggagtttcaccacgttggccaggctgatctcaaactcctggcctcaagtgattcacctgccttggcctcccaaagtgctggaattacaggcccggcctatttttgcaataattatgaatagcacaccatttaaacctgttgattgagccctccttaaataactaaatacactactggccaacatggtgaaaacctgtctccactaaaaacacaaaaaaatggccgggcacagtggctcatgcctgtaatcccagcacttcaggaggccaaggggtgtgaatcacctgaggttaggagttcaagaccagcctggccaacatggtgaaaccctgtctctactaaaaaaaaatacaaaaattagctgagtgtagtggcacatacccgtagtctcagctactcaggaggctgaggcaggagaattgcttgaacctgggaggcaggggttgcagtgagccaagatcgtgccaccacactccagcctgggtgacacagcgagactccatctcaaaataaataaataaataaaaagaaagggaccgagcgcggtggctcatgcttgtaatcccagcactctgggaggctgagttgggcagatcacaaggtcaagagttcaggaccagcctgaccaacacggtaaaaccccatctctactaaaaatacaaaaatgagctgggtgtgatggcacgcgcctgtaaccccagttactcaaaaggctgaggcaagagaatcgcttgaacctgggaggcagaggttgcagtgagccgagatcacgccactgcattccagcctggtgacagtgagactctgtcacacacacacaaaaaagataaagaatgacaaaaatctgtgcctacattcagagtgacaagaatactaatgttctgcttgtagaaaagactattggttcagaatatgttaaatgcaaataatattttgtataatatatataaattacatatgcataaaaagagtatctatattagaatcttttgagacagggtcttgctctgtcaaccatgagggagtgcagtggcactaccacagctcactgtagccttgacttcctgagctcaagccatcctctcgcctcagcctcctgaatagttgggactgcaggtggtgccaccaaggctggctaagtttttatatttttttatagaaacaagcttttgccacgttgcccaggctggtctcaaacttctaaaagctcaagcaatctggccgccttgaactcccaaagtgcttgagttataggcatgagtcactgtgcccggcctacattagaatcttaacagtggggctgggcatggtgccccatgcctgtaatcccagcactttgggaggtcaaggtgggcagactacttgaggttgaggagttcgaggccagcctggccaacatggtgaaaccccatctgtactaaaaacacaaaaattagccaggtgtggtggcacatgtttgcaatcccagctacttgggaggctgaggcgggaggatcacttgaacctgggaagcagaggttgcagtgagccgagatggtgccatggcactccagcctgggcaatagacagcgggactcagtctcaaaacaaaaaaaaaaaaaaaaaaaaaagaatcttaacagtggttaacttcaaatagtgaaactatgactgttaactgagtttgacatttttgtgttttcctagatttttctacaataaacattattatttcataataaagcagtaaagactttttatacaaactattttaagataaacaaattttgacataggggttataagttaggtagaatctatttatataaaaaatggaactgtacttttgtgggccaaataagcactatgtaagtttttttaattttcccaaacacatgcacagaattaatattgccttaaattttgttagcacaagtttgagagagctctttagttcataaaaaaatgttttatggaccaggtgccgtggctcacacctgcaatctcaacactttgggaggcccaggtgggaggatcgcttgagcctaggagtttgagacaagactgggcgacgcagggagaccctgtctcaaaaaaacaaaaccaaaaacaagcaaacaaaaaaacagctgggcatggtggcatgcatatgtagtcccagctattctagaggctgaggtgagatcgctggagcccaggaggtggaggctacagtaagctgtgatcatgccaatgcactccagcttggtcaacaaagcaagactgtgcctcaaaaaaaaaaaagaaaagaaaagaaagaaagaaaagaaaaagaaaaaaagttatgtacgtatggtttttttttttttttggatagagtttcactcttcttgcccaggctggagtgcaatggtgcaatcttggctcaccacaaccttcccctactgggttcaagcgattctcctgtttcagcctccccagtagctgggattaaaggcatgtgccaccacgcccggctaattttgtatttttagtagagatgaagtttctccatgttggtcaggctggtcttgaactcctgacttcaggtgatctgcccgcctcagcctcccaaagtgctgggattacaggtgtgagccacctcgcctggccgttttttttttttttttttttttctgagacggagttttgctcttattgcccaggctggagtgcaatggcacgatctcggctcatcgcaacctctgcctcacgggttcaagcaattttcctgcctcagcgtctcaagtagctaggattacagggatgctccatcatgcccggctaattttgtatttttggtagagacagggtttctccatgttggtcaggctggtctcaaactcccaacctcaggtgatttacccgccttggcctcccaaagagctgggattacaggtgtgagccactgtgcccggccatgcttatgttttttaacaatacacttctgaactatcaaaaagaatataaatcaaaatcactgaagtagtttttaaaaactccaaaagctacaaaacttacttacttcaatatcaattaaaaacccatttgatagttcaataacttgagtcctgctagaatcattctataagccatcagtgacagtgaagtggccaaaatttgagtcacttgataagtacaaagaacacagatttttgtcattcttactgtgaagaaaaacagtgaatgaataacttagtttatatattaacagtacttttatttaaaaaattatctagagaataacttctttttaatcatttgttagtcatgtaactatggataaaacatactaatttagctgattcctctatgctctcttttccttgattccaatcattattagttattctacactgcctcatttattggcagttatgccaactggctgactctggttcaactgccctatttttgctttcatcattgtttatcatatctcacttgctttaaactccacctctttcatctcatctgatctgacacttggtttacatatcaattggctactctaaccttctaccgccagtttccaacccattcgaggtacttgggtaacaaaggaagatgctctatacacacaaaaccacagaaaataagtgggaagggataataaatttcacttaaagttttagaatttttcttttttttttgagacggagtttcactcttgttgcccaggctggagtgcaatggcgcgatcttggctcaccgcaacctctgcctcccaggttcaagcagttctcctgcttcagcctcccgagtagctggtattacaggcatgcaccaccaagcctggctaattttgtatttttagtagagacggggtttctccatgttggtcaggctggtcttgaacgcctgacctcaggtgatctgcctgcctcggcctcccaaagtgctgggattacaggcatgagccatcacgcccggccaaagttttagaatttaagttattccaaaaaaaattttttttttcaaaaatacagactgcatccaattaaattctatgttaactggtaatgactaggtctaaaatgttaggtatttaccaataaatgacataaaataactcaacaacaaagggatttttttttttaagagatagggtctcactttatcactcaggtttggctgagggcagtggtgtgatcacagctcactgaagcctccaactcctgggctcaagtgatcctcccgcctcagtctaccagagtatattcttgaaagtaaaattacaaatgaaattcagcagtgttaaaaataagcccacttgcagacaattatcatttttcttcctttctttcctcactatctgtacttggcatatttcctacagtggctgtcttaaagaaaaaaaggaatccttcacaaatagtgtagccaaaaaagttggactaatatacaatgctatcagtaaagtattatatataaaatttataagtgctaaagtgtaattttgaaagacacttaagatactccttttttttttgagacaaggtctcagccctgtcgcccaggctggagtgcactagcacaacatcagctcactgcaacctccgcctcccaggttcaagcgattctcctgcctcagcctcccaagtagctgagactacaggcgcacgccagcatgtccagataattttttgtatttttagtagagatggggtttcaccatgttggccaggatggtctcaaatctcttgacctcgtgatctgcccatgtcggcttcccaaagtgttaggataacaggcatgagctaccgtgcccagcctacttaaaatattcttgaaatagctctccccacctccttttttttttttttttgagaatgagtttcactcgacacccaggctggagtgcagtggtgcgatcttggctcactgcaacctctgcctcccaggttcaagcgattatcctgcctcagcctcctgagtagctgggattacaaatgtgcaccaccacatctggctaattttttttttttttttttgtatttttagtagagacggggtttcaccaagttggcctggctggtctcgaacacctgacctcaattgatccacctgcctcggcctcccaaagtattataggcatgagccaccgagcccggccttttttgttttttgtttttttaaaggcagggttttgctctgttgcccaggctggagtgcagtggtgtgatcacagatcactgcagccttgacctctcctggtctcaagtgatcctcccacctcagccttcagaacagctgggactacaggtgtgtgtcaccatgcccagtaatttttttgtatatttgtagaggcagggtctcccaatgttgcctgggctggtctcaaactcctgggctcaagcaatccaccagctttggccttccaaagttctaggattatacgcatgagccactgtgccctgccccaatattttgttacttactagtgagactaaacacttttctaaaagtttgttagccatactatcctataaaagctgtttgttcatgtcttttgtccatttatctttttttttgtttttcttgagacagagtcttgctctgtggcccaggctggagtgcaggggtgcaatctcggctcactgcaagctccgcctcccaggttcaaatgattctcctgcctcagcctcctgagtagctgggattacaggcatgtgccaccatgcccagctaatttttttgtgtgtgtttttcagtagagatggggtttcaccatgttggccaggctgatctcgaattcctgacctcaggtgctccacccgcctcagcctcccaaagtactgggattacaggggtgagccaccgcacccggccaattttctgtatttttaatagagacagggtttcatcctgttggccaggctggcctcgaacttcggacctcaggtgatccacccgcctcgacctcccaaagtgctgggattacaggtgtgggccaccacacccagccaatttttttgtatttttagtagagacagggtttcatcatgttggccaggctggtcgcaaactcctgacctcaggtgatccacccgcctcagcatcccaaagtgctgggattacaggcatgagccaccactcccggccaatgttttgtatttttagtagagatggggtttcatcatgttggccagactggtctcaaactctggacctcaggtgatccacctgcctcagcctcccaaagtgtagggattacaggtgtgagccaccgcgcccagcctatgtttctattttatacatattcaacaaacatgattccccaacttctgcaaaataatttctttttcaagaacattgattttagagctcacactaagaaaaagaatacaaaaataatggcatagaaagtgaaaaaacaaaaataaaaagtagaaagctaaagtttcccattaaaatgatcaatatactgtgcagtaagtcaaatgtgtacaatgaattaagaaaatatgatatataaaaatccaaatttacaaaattaagtacaaataggtgtttatattacaaagtgatactggtttataaaaggattcaacatagattttttttaaatggttgttttcctcaatcaatttaacaatgattttaaatgtataaaattttaatatctctttgagacagtgatccaagcttcttcccttgatgatgttaccagttcatactttgtttcaataacctgtccctccacagaaagtaggtgcagtctcttcaccaatacactaagaagtactgtggtcaccatatatgcaaacctcaactctggacactcctgtgtgcctgagaatccaagtgaggaaaaagttttcattactaattcatcatcaaaccgatctggatcaaacttgtgtggagatggccaagtattaggatcctgaagtaccacaccaagggcataaaggacgagggtctctctaggaataataaatcggtcaatttttccttcaatatcttgaagctgggcagaaactggagtcagtttggcagttcgaacagtttcacaaagcacatgctgacaatatctgagctgctcaattttctctggagtaacaggaccatttccaaaaacttggtttatctcttcatataattttttttgaacttcttcagaggtggttaaaaaacagattgcccaggtacacaattttgcagttattatgcaactggccagagaaaatatcatactgtcttctaggatctgttggtcattaaggttcccttgtactaaggagtcaatgaaaatatgttgactgaagttccttccttttcgttcttttatgatgttccttaaaacagactccagttgcatgagggcatcttcatattgttttttccgagtcatgtttttatcaagtgacccatctagaaagccttttccaatctcagaccaaactgtgccatgattcttctggaagcgaatgacttcctgatcatcttcaaatgtactacccattaccatctgtgtaacagacttcatagcaaaaccaagcatatgctggctgaggggcacgtgctgggtctctgggtaggagagccatttatctaataattcttctgaaagctttaggaggagggcaaagttactcttcagagaatcagtcacaccattttcatacaattttttcctcatgtggttttcactcacactgccaccaccagattgataccttaataatgacttcagcatggtttcaaaagggtccgcggatagaggtagagcacggctcccaccaacgccagcaagaaggtaacggcgaagatcgcgaagtccaacatggttctgccgcccagggagccacgtctcggatcggccgctccagc

SEQ ID NO: 13074 - RNA, 9766 nt, Homo sapiens
  source 1..9766: mol_type = other RNA
gctgggattacaggcatgagccaccacacccagctggaaaatgtttaaaatttattaagtgaaaagtaactcatgctgcaatgaacgtactatgtaaaaatgtatgtatgtggaacagggaaaaatataaacagtcacagaaatgtgtttaggttggtagcattctttttcctcttaaaaattcctttttttggccgggcgctgtggctcacacctgtaatcccagcactttgggaagccgcggtggacagatcacaaggtcaggagatcaagaccatcctggctaacatggtgaaaccccgtctctactaaaaatacaaaaaattagctgggcatggaggcactcgcctgtagtcgcagctactcgggaggctgaggcaggagaatcgcttgaactggggagatggaggttgtagtgagcccagatcatgccactgcactcaagcctgggctgagacctccagagtctggctgagacctatggagtctcactctgtcacctaggctggagtacagtggtgcgatctcggcacactgcaacctccacctcccagacattctcctgcctcagcctctcaactagctgggattacattcgcccgcctccacacccactaatttttgtatttttagtagagatgcggtttccccatgttggccaggctgttcttgaactcctgacctcaagttatacgcccactttggactcccaaagtgctgggattacaggtgtgagccacggcaccagccaaaaatttctttaaatattagtggtatattattctctcaataagttttttttttttttttttttgagacagtcttgttttattgcctaagctggagtgcagtggcacaatctcaactcactgcaacctccacctcccaggtttattttttttctcatgcctcagcctcccaagaagctgggattacaggcatgtgccccaaaggccagttaagttttctttttctttttttcttttttcttggttgagacggattttcgctcgtcacccacactggagtgcaatggcgcgatctcggctcactgcaacctccgactcttgggttcaagcgattctcctgcctcagcctcccgagtagctgggattagaggcacctgtcaccacgcccgctacttttggtatttttagtagagatggagtttcaccacgttggccaggctgatctcaaactcctggcctcaagtgattcacctgccttggcctcccaaagtgctggaattacaggcccggcctatttttgcaataattatgaatagcacaccatttaaacctgttgattgagccctccttaaataactaaatacactactggccaacatggtgaaaacctgtctccactaaaaacacaaaaaaatggccgggcacagtggctcatgcctgtaatcccagcacttcaggaggccaaggggtgtgaatcacctgaggttaggagttcaagaccagcctggccaacatggtgaaaccctgtctctactaaaaaaaaatacaaaaattagctgagtgtagtggcacatacccgtagtctcagctactcaggaggctgaggcaggagaattgcttgaacctgggaggcaggggttgcagtgagccaagatcgtgccaccacactccagcctgggtgacacagcgagactccatctcaaaataaataaataaataaaaagaaagggaccgagcgcggtggctcatgcttgtaatcccagcactctgggaggctgagttgggcagatcacaaggtcaagagttcaggaccagcctgaccaacacggtaaaaccccatctctactaaaaatacaaaaatgagctgggtgtgatggcacgcgcctgtaaccccagttactcaaaaggctgaggcaagagaatcgcttgaacctgggaggcagaggttgcagtgagccgagatcacgccactgcattccagcctggtgacagtgagactctgtcacacacacacaaaaaagataaagaatgacaaaaatctgtgcctacattcagagtgacaagaatactaatgttctgcttgtagaaaagactattggttcagaatatgttaaatgcaaataatattttgtataatatatataaattacatatgcataaaaagagtatctatattagaatcttttgagacagggtcttgctctgtcaaccatgagggagtgcagtggcactaccacagctcactgtagccttgacttcctgagctcaagccatcctctcgcctcagcctcctgaatagttgggactgcaggtggtgccaccaaggctggctaagtttttatatttttttatagaaacaagcttttgccacgttgcccaggctggtctcaaacttctaaaagctcaagcaatctggccgccttgaactcccaaagtgcttgagttataggcatgagtcactgtgcccggcctacattagaatcttaacagtggggctgggcatggtgccccatgcctgtaatcccagcactttgggaggtcaaggtgggcagactacttgaggttgaggagttcgaggccagcctggccaacatggtgaaaccccatctgtactaaaaacacaaaaattagccaggtgtggtggcacatgtttgcaatcccagctacttgggaggctgaggcgggaggatcacttgaacctgggaagcagaggttgcagtgagccgagatggtgccatggcactccagcctgggcaatagacagcgggactcagtctcaaaacaaaaaaaaaaaaaaaaaaaaaagaatcttaacagtggttaacttcaaatagtgaaactatgactgttaactgagtttgacatttttgtgttttcctagatttttctacaataaacattattatttcataataaagcagtaaagactttttatacaaactattttaagataaacaaattttgacataggggttataagttaggtagaatctatttatataaaaaatggaactgtacttttgtgggccaaataagcactatgtaagtttttttaattttcccaaacacatgcacagaattaatattgccttaaattttgttagcacaagtttgagagagctctttagttcataaaaaaatgttttatggaccaggtgccgtggctcacacctgcaatctcaacactttgggaggcccaggtgggaggatcgcttgagcctaggagtttgagacaagactgggcgacgcagggagaccctgtctcaaaaaaacaaaaccaaaaacaagcaaacaaaaaaacagctgggcatggtggcatgcatatgtagtcccagctattctagaggctgaggtgagatcgctggagcccaggaggtggaggctacagtaagctgtgatcatgccaatgcactccagcttggtcaacaaagcaagactgtgcctcaaaaaaaaaaaagaaaagaaaagaaagaaagaaaagaaaaagaaaaaaagttatgtacgtatggtttttttttttttttggatagagtttcactcttcttgcccaggctggagtgcaatggtgcaatcttggctcaccacaaccttcccctactgggttcaagcgattctcctgtttcagcctccccagtagctgggattaaaggcatgtgccaccacgcccggctaattttgtatttttagtagagatgaagtttctccatgttggtcaggctggtcttgaactcctgacttcaggtgatctgcccgcctcagcctcccaaagtgctgggattacaggtgtgagccacctcgcctggccgttttttttttttttttttttttctgagacggagttttgctcttattgcccaggctggagtgcaatggcacgatctcggctcatcgcaacctctgcctcacgggttcaagcaattttcctgcctcagcgtctcaagtagctaggattacagggatgctccatcatgcccggctaattttgtatttttggtagagacagggtttctccatgttggtcaggctggtctcaaactcccaacctcaggtgatttacccgccttggcctcccaaagagctgggattacaggtgtgagccactgtgcccggccatgcttatgttttttaacaatacacttctgaactatcaaaaagaatataaatcaaaatcactgaagtagtttttaaaaactccaaaagctacaaaacttacttacttcaatatcaattaaaaacccatttgatagttcaataacttgagtcctgctagaatcattctataagccatcagtgacagtgaagtggccaaaatttgagtcacttgataagtacaaagaacacagatttttgtcattcttactgtgaagaaaaacagtgaatgaataacttagtttatatattaacagtacttttatttaaaaaattatctagagaataacttctttttaatcatttgttagtcatgtaactatggataaaacatactaatttagctgattcctctatgctctcttttccttgattccaatcattattagttattctacactgcctcatttattggcagttatgccaactggctgactctggttcaactgccctatttttgctttcatcattgtttatcatatctcacttgctttaaactccacctctttcatctcatctgatctgacacttggtttacatatcaattggctactctaaccttctaccgccagtttccaacccattcgaggtacttgggtaacaaaggaagatgctctatacacacaaaaccacagaaaataagtgggaagggataataaatttcacttaaagttttagaatttttcttttttttttgagacggagtttcactcttgttgcccaggctggagtgcaatggcgcgatcttggctcaccgcaacctctgcctcccaggttcaagcagttctcctgcttcagcctcccgagtagctggtattacaggcatgcaccaccaagcctggctaattttgtatttttagtagagacggggtttctccatgttggtcaggctggtcttgaacgcctgacctcaggtgatctgcctgcctcggcctcccaaagtgctgggattacaggcatgagccatcacgcccggccaaagttttagaatttaagttattccaaaaaaaattttttttttcaaaaatacagactgcatccaattaaattctatgttaactggtaatgactaggtctaaaatgttaggtatttaccaataaatgacataaaataactcaacaacaaagggatttttttttttaagagatagggtctcactttatcactcaggtttggctgagggcagtggtgtgatcacagctcactgaagcctccaactcctgggctcaagtgatcctcccgcctcagtctaccagagtatattcttgaaagtaaaattacaaatgaaattcagcagtgttaaaaataagcccacttgcagacaattatcatttttcttcctttctttcctcactatctgtacttggcatatttcctacagtggctgtcttaaagaaaaaaaggaatccttcacaaatagtgtagccaaaaaagttggactaatatacaatgctatcagtaaagtattatatataaaatttataagtgctaaagtgtaattttgaaagacacttaagatactccttttttttttgagacaaggtctcagccctgtcgcccaggctggagtgcactagcacaacatcagctcactgcaacctccgcctcccaggttcaagcgattctcctgcctcagcctcccaagtagctgagactacaggcgcacgccagcatgtccagataattttttgtatttttagtagagatggggtttcaccatgttggccaggatggtctcaaatctcttgacctcgtgatctgcccatgtcggcttcccaaagtgttaggataacaggcatgagctaccgtgcccagcctacttaaaatattcttgaaatagctctccccacctccttttttttttttttttgagaatgagtttcactcgacacccaggctggagtgcagtggtgcgatcttggctcactgcaacctctgcctcccaggttcaagcgattatcctgcctcagcctcctgagtagctgggattacaaatgtgcaccaccacatctggctaattttttttttttttttttgtatttttagtagagacggggtttcaccaagttggcctggctggtctcgaacacctgacctcaattgatccacctgcctcggcctcccaaagtattataggcatgagccaccgagcccggccttttttgttttttgtttttttaaaggcagggttttgctctgttgcccaggctggagtgcagtggtgtgatcacagatcactgcagccttgacctctcctggtctcaagtgatcctcccacctcagccttcagaacagctgggactacaggtgtgtgtcaccatgcccagtaatttttttgtatatttgtagaggcagggtctcccaatgttgcctgggctggtctcaaactcctgggctcaagcaatccaccagctttggccttccaaagttctaggattatacgcatgagccactgtgccctgccccaatattttgttacttactagtgagactaaacacttttctaaaagtttgttagccatactatcctataaaagctgtttgttcatgtcttttgtccatttatctttttttttgtttttcttgagacagagtcttgctctgtggcccaggctggagtgcaggggtgcaatctcggctcactgcaagctccgcctcccaggttcaaatgattctcctgcctcagcctcctgagtagctgggattacaggcatgtgccaccatgcccagctaatttttttgtgtgtgtttttcagtagagatggggtttcaccatgttggccaggctgatctcgaattcctgacctcaggtgctccacccgcctcagcctcccaaagtactgggattacaggggtgagccaccgcacccggccaattttctgtatttttaatagagacagggtttcatcctgttggccaggctggcctcgaacttcggacctcaggtgatccacccgcctcgacctcccaaagtgctgggattacaggtgtgggccaccacacccagccaatttttttgtatttttagtagagacagggtttcatcatgttggccaggctggtcgcaaactcctgacctcaggtgatccacccgcctcagcatcccaaagtgctgggattacaggcatgagccaccactcccggccaatgttttgtatttttagtagagatggggtttcatcatgttggccagactggtctcaaactctggacctcaggtgatccacctgcctcagcctcccaaagtgtagggattacaggtgtgagccaccgcgcccagcctatgtttctattttatacatattcaacaaacatgattccccaacttctgcaaaataatttctttttcaagaacattgattttagagctcacactaagaaaaagaatacaaaaataatggcatagaaagtgaaaaaacaaaaataaaaagtagaaagctaaagtttcccattaaaatgatcaatatactgtgcagtaagtcaaatgtgtacaatgaattaagaaaatatgatatataaaaatccaaatttacaaaattaagtacaaataggtgtttatattacaaagtgatactggtttataaaaggattcaacatagattttttttaaatggttgttttcctcaatcaatttaacaatgattttaaatgtataaaattttaatatctctttgagacagtgatccaagcttcttcccttgatgatgttaccagttcatactttgtttcaataacctgtccctccacagaaagtaggtgcagtctcttcaccaatacactaagaagtactgtggtcaccatatatgcaaacctcaactctggacactcctgtgtgcctgagaatccaagtgaggaaaaagttttcattactaattcatcatcaaaccgatctggatcaaacttgtgtggagatggccaagtattaggatcctgaagtaccacaccaagggcataaaggacgagggtctctctaggaataataaatcggtcaatttttccttcaatatcttgaagctgggcagaaactggagtcagtttggcagttcgaacagtttcacaaagcacatgctgacaatatctgagctgctcaattttctctggagtaacaggaccatttccaaaaacttggtttatctcttcatataattttttttgaacttcttcagaggtggttaaaaaacagattgcccaggtacacaattttgcagttattatgcaactggccagagaaaatatcatactgtcttctaggatctgttggtcattaaggttcccttgtactaaggagtcaatgaaaatatgttgactgaagttccttccttttcgttcttttatgatgttccttaaaacagactccagttgcatgagggcatcttcatattgttttttccgagtcatgtttttatcaagtgacccatctagaaagccttttccaatctcagaccaaactgtgccatgattcttctggaagcgaatgacttcctgatcatcttcaaatgtactacccattaccatctgtgtaacagacttcatagcaaaaccaagcatatgctggctgaggggcacgtgctgggtctctgggtaggagagccatttatctaataattcttctgaaagctttaggaggagggcaaagttactcttcagagaatcagtcacaccattttcatacaattttttcctcatgtggttttcactcacactgccaccaccagattgataccttaataatgacttcagcatggtttcaaaagggtccgctgctcggaaaagaacatttaagaaggtgtatggtcaattccagcagttcagctacttttcaactttcactgtaaaaccaccaccttgctttgtagaacaggtgttttttgtttgtttgtttgtttgttttgagataagagtctggctctgtcgccaggctgcagtgcagtggtgcgatcttggctcactgcaagctccgcctcccaggttcaagcgattctcctgcctcagcctcctgagtagctgggattacaggcgcccgccaccacagccagctaatgtttgtatttttagtagagacggtgtgtcaccatgttggccaggatggtctcgatatcctgacctcgtgatccgcccgcctcagcctcccaaagtgtgtagaacaggttttaaagacggtcctcagtcatcaacacttttgttttcagaccctccctctctcgctgacggaggcaagtggagagaggaggaccggaggctcgcagaggcgtcagcggcagaggaaacctcgcacccgaacccgcagcgcggcgctctccccaaagaagcatttgcctggagcccctaagaggagcaagacctggacctcgagcactttggattccagtcaggatagatcgatggacagatggaaaagaggaatacacaagtgctgggagaatcctcaagaaaggagaaaggagtggcgcgcccaggagtctcgtcctgacacactgggaaatgaaatttgggtttggcgagttatggccaaaaagctgcccaaagtacttgagagccgccttggagagtggcgcggggtgcctggcaaggtgagaccggcctgcgggggcgcgggcttttcctcagcagctctacgcccgcctggcccggcgcctgaggggtagc

SEQ ID NO: 13075 - RNA, 9047 nt, Homo sapiens
  source 1..9047: mol_type = other RNA
gctgggattacaggcatgagccaccacacccagctggaaaatgtttaaaatttattaagtgaaaagtaactcatgctgcaatgaacgtactatgtaaaaatgtatgtatgtggaacagggaaaaatataaacagtcacagaaatgtgtttaggttggtagcattctttttcctcttaaaaattcctttttttggccgggcgctgtggctcacacctgtaatcccagcactttgggaagccgcggtggacagatcacaaggtcaggagatcaagaccatcctggctaacatggtgaaaccccgtctctactaaaaatacaaaaaattagctgggcatggaggcactcgcctgtagtcgcagctactcgggaggctgaggcaggagaatcgcttgaactggggagatggaggttgtagtgagcccagatcatgccactgcactcaagcctgggctgagacctccagagtctggctgagacctatggagtctcactctgtcacctaggctggagtacagtggtgcgatctcggcacactgcaacctccacctcccagacattctcctgcctcagcctctcaactagctgggattacattcgcccgcctccacacccactaatttttgtatttttagtagagatgcggtttccccatgttggccaggctgttcttgaactcctgacctcaagttatacgcccactttggactcccaaagtgctgggattacaggtgtgagccacggcaccagccaaaaatttctttaaatattagtggtatattattctctcaataagttttttttttttttttttttgagacagtcttgttttattgcctaagctggagtgcagtggcacaatctcaactcactgcaacctccacctcccaggtttattttttttctcatgcctcagcctcccaagaagctgggattacaggcatgtgccccaaaggccagttaagttttctttttctttttttcttttttcttggttgagacggattttcgctcgtcacccacactggagtgcaatggcgcgatctcggctcactgcaacctccgactcttgggttcaagcgattctcctgcctcagcctcccgagtagctgggattagaggcacctgtcaccacgcccgctacttttggtatttttagtagagatggagtttcaccacgttggccaggctgatctcaaactcctggcctcaagtgattcacctgccttggcctcccaaagtgctggaattacaggcccggcctatttttgcaataattatgaatagcacaccatttaaacctgttgattgagccctccttaaataactaaatacactactggccaacatggtgaaaacctgtctccactaaaaacacaaaaaaatggccgggcacagtggctcatgcctgtaatcccagcacttcaggaggccaaggggtgtgaatcacctgaggttaggagttcaagaccagcctggccaacatggtgaaaccctgtctctactaaaaaaaaatacaaaaattagctgagtgtagtggcacatacccgtagtctcagctactcaggaggctgaggcaggagaattgcttgaacctgggaggcaggggttgcagtgagccaagatcgtgccaccacactccagcctgggtgacacagcgagactccatctcaaaataaataaataaataaaaagaaagggaccgagcgcggtggctcatgcttgtaatcccagcactctgggaggctgagttgggcagatcacaaggtcaagagttcaggaccagcctgaccaacacggtaaaaccccatctctactaaaaatacaaaaatgagctgggtgtgatggcacgcgcctgtaaccccagttactcaaaaggctgaggcaagagaatcgcttgaacctgggaggcagaggttgcagtgagccgagatcacgccactgcattccagcctggtgacagtgagactctgtcacacacacacaaaaaagataaagaatgacaaaaatctgtgcctacattcagagtgacaagaatactaatgttctgcttgtagaaaagactattggttcagaatatgttaaatgcaaataatattttgtataatatatataaattacatatgcataaaaagagtatctatattagaatcttttgagacagggtcttgctctgtcaaccatgagggagtgcagtggcactaccacagctcactgtagccttgacttcctgagctcaagccatcctctcgcctcagcctcctgaatagttgggactgcaggtggtgccaccaaggctggctaagtttttatatttttttatagaaacaagcttttgccacgttgcccaggctggtctcaaacttctaaaagctcaagcaatctggccgccttgaactcccaaagtgcttgagttataggcatgagtcactgtgcccggcctacattagaatcttaacagtggggctgggcatggtgccccatgcctgtaatcccagcactttgggaggtcaaggtgggcagactacttgaggttgaggagttcgaggccagcctggccaacatggtgaaaccccatctgtactaaaaacacaaaaattagccaggtgtggtggcacatgtttgcaatcccagctacttgggaggctgaggcgggaggatcacttgaacctgggaagcagaggttgcagtgagccgagatggtgccatggcactccagcctgggcaatagacagcgggactcagtctcaaaacaaaaaaaaaaaaaaaaaaaaaagaatcttaacagtggttaacttcaaatagtgaaactatgactgttaactgagtttgacatttttgtgttttcctagatttttctacaataaacattattatttcataataaagcagtaaagactttttatacaaactattttaagataaacaaattttgacataggggttataagttaggtagaatctatttatataaaaaatggaactgtacttttgtgggccaaataagcactatgtaagtttttttaattttcccaaacacatgcacagaattaatattgccttaaattttgttagcacaagtttgagagagctctttagttcataaaaaaatgttttatggaccaggtgccgtggctcacacctgcaatctcaacactttgggaggcccaggtgggaggatcgcttgagcctaggagtttgagacaagactgggcgacgcagggagaccctgtctcaaaaaaacaaaaccaaaaacaagcaaacaaaaaaacagctgggcatggtggcatgcatatgtagtcccagctattctagaggctgaggtgagatcgctggagcccaggaggtggaggctacagtaagctgtgatcatgccaatgcactccagcttggtcaacaaagcaagactgtgcctcaaaaaaaaaaaagaaaagaaaagaaagaaagaaaagaaaaagaaaaaaagttatgtacgtatggtttttttttttttttggatagagtttcactcttcttgcccaggctggagtgcaatggtgcaatcttggctcaccacaaccttcccctactgggttcaagcgattctcctgtttcagcctccccagtagctgggattaaaggcatgtgccaccacgcccggctaattttgtatttttagtagagatgaagtttctccatgttggtcaggctggtcttgaactcctgacttcaggtgatctgcccgcctcagcctcccaaagtgctgggattacaggtgtgagccacctcgcctggccgttttttttttttttttttttttctgagacggagttttgctcttattgcccaggctggagtgcaatggcacgatctcggctcatcgcaacctctgcctcacgggttcaagcaattttcctgcctcagcgtctcaagtagctaggattacagggatgctccatcatgcccggctaattttgtatttttggtagagacagggtttctccatgttggtcaggctggtctcaaactcccaacctcaggtgatttacccgccttggcctcccaaagagctgggattacaggtgtgagccactgtgcccggccatgcttatgttttttaacaatacacttctgaactatcaaaaagaatataaatcaaaatcactgaagtagtttttaaaaactccaaaagctacaaaacttacttacttcaatatcaattaaaaacccatttgatagttcaataacttgagtcctgctagaatcattctataagccatcagtgacagtgaagtggccaaaatttgagtcacttgataagtacaaagaacacagatttttgtcattcttactgtgaagaaaaacagtgaatgaataacttagtttatatattaacagtacttttatttaaaaaattatctagagaataacttctttttaatcatttgttagtcatgtaactatggataaaacatactaatttagctgattcctctatgctctcttttccttgattccaatcattattagttattctacactgcctcatttattggcagttatgccaactggctgactctggttcaactgccctatttttgctttcatcattgtttatcatatctcacttgctttaaactccacctctttcatctcatctgatctgacacttggtttacatatcaattggctactctaaccttctaccgccagtttccaacccattcgaggtacttgggtaacaaaggaagatgctctatacacacaaaaccacagaaaataagtgggaagggataataaatttcacttaaagttttagaatttttcttttttttttgagacggagtttcactcttgttgcccaggctggagtgcaatggcgcgatcttggctcaccgcaacctctgcctcccaggttcaagcagttctcctgcttcagcctcccgagtagctggtattacaggcatgcaccaccaagcctggctaattttgtatttttagtagagacggggtttctccatgttggtcaggctggtcttgaacgcctgacctcaggtgatctgcctgcctcggcctcccaaagtgctgggattacaggcatgagccatcacgcccggccaaagttttagaatttaagttattccaaaaaaaattttttttttcaaaaatacagactgcatccaattaaattctatgttaactggtaatgactaggtctaaaatgttaggtatttaccaataaatgacataaaataactcaacaacaaagggatttttttttttaagagatagggtctcactttatcactcaggtttggctgagggcagtggtgtgatcacagctcactgaagcctccaactcctgggctcaagtgatcctcccgcctcagtctaccagagtatattcttgaaagtaaaattacaaatgaaattcagcagtgttaaaaataagcccacttgcagacaattatcatttttcttcctttctttcctcactatctgtacttggcatatttcctacagtggctgtcttaaagaaaaaaaggaatccttcacaaatagtgtagccaaaaaagttggactaatatacaatgctatcagtaaagtattatatataaaatttataagtgctaaagtgtaattttgaaagacacttaagatactccttttttttttgagacaaggtctcagccctgtcgcccaggctggagtgcactagcacaacatcagctcactgcaacctccgcctcccaggttcaagcgattctcctgcctcagcctcccaagtagctgagactacaggcgcacgccagcatgtccagataattttttgtatttttagtagagatggggtttcaccatgttggccaggatggtctcaaatctcttgacctcgtgatctgcccatgtcggcttcccaaagtgttaggataacaggcatgagctaccgtgcccagcctacttaaaatattcttgaaatagctctccccacctccttttttttttttttttgagaatgagtttcactcgacacccaggctggagtgcagtggtgcgatcttggctcactgcaacctctgcctcccaggttcaagcgattatcctgcctcagcctcctgagtagctgggattacaaatgtgcaccaccacatctggctaattttttttttttttttttgtatttttagtagagacggggtttcaccaagttggcctggctggtctcgaacacctgacctcaattgatccacctgcctcggcctcccaaagtattataggcatgagccaccgagcccggccttttttgttttttgtttttttaaaggcagggttttgctctgttgcccaggctggagtgcagtggtgtgatcacagatcactgcagccttgacctctcctggtctcaagtgatcctcccacctcagccttcagaacagctgggactacaggtgtgtgtcaccatgcccagtaatttttttgtatatttgtagaggcagggtctcccaatgttgcctgggctggtctcaaactcctgggctcaagcaatccaccagctttggccttccaaagttctaggattatacgcatgagccactgtgccctgccccaatattttgttacttactagtgagactaaacacttttctaaaagtttgttagccatactatcctataaaagctgtttgttcatgtcttttgtccatttatctttttttttgtttttcttgagacagagtcttgctctgtggcccaggctggagtgcaggggtgcaatctcggctcactgcaagctccgcctcccaggttcaaatgattctcctgcctcagcctcctgagtagctgggattacaggcatgtgccaccatgcccagctaatttttttgtgtgtgtttttcagtagagatggggtttcaccatgttggccaggctgatctcgaattcctgacctcaggtgctccacccgcctcagcctcccaaagtactgggattacaggggtgagccaccgcacccggccaattttctgtatttttaatagagacagggtttcatcctgttggccaggctggcctcgaacttcggacctcaggtgatccacccgcctcgacctcccaaagtgctgggattacaggtgtgggccaccacacccagccaatttttttgtatttttagtagagacagggtttcatcatgttggccaggctggtcgcaaactcctgacctcaggtgatccacccgcctcagcatcccaaagtgctgggattacaggcatgagccaccactcccggccaatgttttgtatttttagtagagatggggtttcatcatgttggccagactggtctcaaactctggacctcaggtgatccacctgcctcagcctcccaaagtgtagggattacaggtgtgagccaccgcgcccagcctatgtttctattttatacatattcaacaaacatgattccccaacttctgcaaaataatttctttttcaagaacattgattttagagctcacactaagaaaaagaatacaaaaataatggcatagaaagtgaaaaaacaaaaataaaaagtagaaagctaaagtttcccattaaaatgatcaatatactgtgcagtaagtcaaatgtgtacaatgaattaagaaaatatgatatataaaaatccaaatttacaaaattaagtacaaataggtgtttatattacaaagtgatactggtttataaaaggattcaacatagattttttttaaatggttgttttcctcaatcaatttaacaatgattttaaatgtataaaattttaatatctctttgagacagtgatccaagcttcttcccttgatgatgttaccagttcatactttgtttcaataacctgtccctccacagaaagtaggtgcagtctcttcaccaatacactaagaagtactgtggtcaccatatatgcaaacctcaactctggacactcctgtgtgcctgagaatccaagtgaggaaaaagttttcattactaattcatcatcaaaccgatctggatcaaacttgtgtggagatggccaagtattaggatcctgaagtaccacaccaagggcataaaggacgagggtctctctaggaataataaatcggtcaatttttccttcaatatcttgaagctgggcagaaactggagtcagtttggcagttcgaacagtttcacaaagcacatgctgacaatatctgagctgctcaattttctctggagtaacaggaccatttccaaaaacttggtttatctcttcatataattttttttgaacttcttcagaggtggttaaaaaacagattgcccaggtacacaattttgcagttattatgcaactggccagagaaaatatcatactgtcttctaggatctgttggtcattaaggttcccttgtactaaggagtcaatgaaaatatgttgactgaagttccttccttttcgttcttttatgatgttccttaaaacagactccagttgcatgagggcatcttcatattgttttttccgagtcatgtttttatcaagtgacccatctagaaagccttttccaatctcagaccaaactgtgccatgattcttctggaagcgaatgacttcctgatcatcttcaaatgtactacccattaccatctgtgtaacagacttcatagcaaaaccaagcatatgctggctgaggggcacgtgctgggtctctgggtaggagagccatttatctaataattcttctgaaagctttaggaggagggcaaagttactcttcagagaatcagtcacaccattttcatacaattttttcctcatgtggttttcactcacactgccaccaccagattgataccttaataatgacttcagcatggtttcaaaagggtccgttttcttcagttggagtaatccctggaattcctgcagcttgtctggaagccggatagaggtagagcacggctcccaccaacgccagcaagaaggtaacggcgaagatcgcgaagtccaacatggttctgccgcccagggagccacgtctcggatcggccgctccagc

SEQ ID NO: 13076 - RNA, 8862 nt, Homo sapiens
  source 1..8862: mol_type = other RNA
gctgggattacaggcatgagccaccacacccagctggaaaatgtttaaaatttattaagtgaaaagtaactcatgctgcaatgaacgtactatgtaaaaatgtatgtatgtggaacagggaaaaatataaacagtcacagaaatgtgtttaggttggtagcattctttttcctcttaaaaattcctttttttggccgggcgctgtggctcacacctgtaatcccagcactttgggaagccgcggtggacagatcacaaggtcaggagatcaagaccatcctggctaacatggtgaaaccccgtctctactaaaaatacaaaaaattagctgggcatggaggcactcgcctgtagtcgcagctactcgggaggctgaggcaggagaatcgcttgaactggggagatggaggttgtagtgagcccagatcatgccactgcactcaagcctgggctgagacctccagagtctggctgagacctatggagtctcactctgtcacctaggctggagtacagtggtgcgatctcggcacactgcaacctccacctcccagacattctcctgcctcagcctctcaactagctgggattacattcgcccgcctccacacccactaatttttgtatttttagtagagatgcggtttccccatgttggccaggctgttcttgaactcctgacctcaagttatacgcccactttggactcccaaagtgctgggattacaggtgtgagccacggcaccagccaaaaatttctttaaatattagtggtatattattctctcaataagttttttttttttttttttttgagacagtcttgttttattgcctaagctggagtgcagtggcacaatctcaactcactgcaacctccacctcccaggtttattttttttctcatgcctcagcctcccaagaagctgggattacaggcatgtgccccaaaggccagttaagttttctttttctttttttcttttttcttggttgagacggattttcgctcgtcacccacactggagtgcaatggcgcgatctcggctcactgcaacctccgactcttgggttcaagcgattctcctgcctcagcctcccgagtagctgggattagaggcacctgtcaccacgcccgctacttttggtatttttagtagagatggagtttcaccacgttggccaggctgatctcaaactcctggcctcaagtgattcacctgccttggcctcccaaagtgctggaattacaggcccggcctatttttgcaataattatgaatagcacaccatttaaacctgttgattgagccctccttaaataactaaatacactactggccaacatggtgaaaacctgtctccactaaaaacacaaaaaaatggccgggcacagtggctcatgcctgtaatcccagcacttcaggaggccaaggggtgtgaatcacctgaggttaggagttcaagaccagcctggccaacatggtgaaaccctgtctctactaaaaaaaaatacaaaaattagctgagtgtagtggcacatacccgtagtctcagctactcaggaggctgaggcaggagaattgcttgaacctgggaggcaggggttgcagtgagccaagatcgtgccaccacactccagcctgggtgacacagcgagactccatctcaaaataaataaataaataaaaagaaagggaccgagcgcggtggctcatgcttgtaatcccagcactctgggaggctgagttgggcagatcacaaggtcaagagttcaggaccagcctgaccaacacggtaaaaccccatctctactaaaaatacaaaaatgagctgggtgtgatggcacgcgcctgtaaccccagttactcaaaaggctgaggcaagagaatcgcttgaacctgggaggcagaggttgcagtgagccgagatcacgccactgcattccagcctggtgacagtgagactctgtcacacacacacaaaaaagataaagaatgacaaaaatctgtgcctacattcagagtgacaagaatactaatgttctgcttgtagaaaagactattggttcagaatatgttaaatgcaaataatattttgtataatatatataaattacatatgcataaaaagagtatctatattagaatcttttgagacagggtcttgctctgtcaaccatgagggagtgcagtggcactaccacagctcactgtagccttgacttcctgagctcaagccatcctctcgcctcagcctcctgaatagttgggactgcaggtggtgccaccaaggctggctaagtttttatatttttttatagaaacaagcttttgccacgttgcccaggctggtctcaaacttctaaaagctcaagcaatctggccgccttgaactcccaaagtgcttgagttataggcatgagtcactgtgcccggcctacattagaatcttaacagtggggctgggcatggtgccccatgcctgtaatcccagcactttgggaggtcaaggtgggcagactacttgaggttgaggagttcgaggccagcctggccaacatggtgaaaccccatctgtactaaaaacacaaaaattagccaggtgtggtggcacatgtttgcaatcccagctacttgggaggctgaggcgggaggatcacttgaacctgggaagcagaggttgcagtgagccgagatggtgccatggcactccagcctgggcaatagacagcgggactcagtctcaaaacaaaaaaaaaaaaaaaaaaaaaagaatcttaacagtggttaacttcaaatagtgaaactatgactgttaactgagtttgacatttttgtgttttcctagatttttctacaataaacattattatttcataataaagcagtaaagactttttatacaaactattttaagataaacaaattttgacataggggttataagttaggtagaatctatttatataaaaaatggaactgtacttttgtgggccaaataagcactatgtaagtttttttaattttcccaaacacatgcacagaattaatattgccttaaattttgttagcacaagtttgagagagctctttagttcataaaaaaatgttttatggaccaggtgccgtggctcacacctgcaatctcaacactttgggaggcccaggtgggaggatcgcttgagcctaggagtttgagacaagactgggcgacgcagggagaccctgtctcaaaaaaacaaaaccaaaaacaagcaaacaaaaaaacagctgggcatggtggcatgcatatgtagtcccagctattctagaggctgaggtgagatcgctggagcccaggaggtggaggctacagtaagctgtgatcatgccaatgcactccagcttggtcaacaaagcaagactgtgcctcaaaaaaaaaaaagaaaagaaaagaaagaaagaaaagaaaaagaaaaaaagttatgtacgtatggtttttttttttttttggatagagtttcactcttcttgcccaggctggagtgcaatggtgcaatcttggctcaccacaaccttcccctactgggttcaagcgattctcctgtttcagcctccccagtagctgggattaaaggcatgtgccaccacgcccggctaattttgtatttttagtagagatgaagtttctccatgttggtcaggctggtcttgaactcctgacttcaggtgatctgcccgcctcagcctcccaaagtgctgggattacaggtgtgagccacctcgcctggccgttttttttttttttttttttttctgagacggagttttgctcttattgcccaggctggagtgcaatggcacgatctcggctcatcgcaacctctgcctcacgggttcaagcaattttcctgcctcagcgtctcaagtagctaggattacagggatgctccatcatgcccggctaattttgtatttttggtagagacagggtttctccatgttggtcaggctggtctcaaactcccaacctcaggtgatttacccgccttggcctcccaaagagctgggattacaggtgtgagccactgtgcccggccatgcttatgttttttaacaatacacttctgaactatcaaaaagaatataaatcaaaatcactgaagtagtttttaaaaactccaaaagctacaaaacttacttacttcaatatcaattaaaaacccatttgatagttcaataacttgagtcctgctagaatcattctataagccatcagtgacagtgaagtggccaaaatttgagtcacttgataagtacaaagaacacagatttttgtcattcttactgtgaagaaaaacagtgaatgaataacttagtttatatattaacagtacttttatttaaaaaattatctagagaataacttctttttaatcatttgttagtcatgtaactatggataaaacatactaatttagctgattcctctatgctctcttttccttgattccaatcattattagttattctacactgcctcatttattggcagttatgccaactggctgactctggttcaactgccctatttttgctttcatcattgtttatcatatctcacttgctttaaactccacctctttcatctcatctgatctgacacttggtttacatatcaattggctactctaaccttctaccgccagtttccaacccattcgaggtacttgggtaacaaaggaagatgctctatacacacaaaaccacagaaaataagtgggaagggataataaatttcacttaaagttttagaatttttcttttttttttgagacggagtttcactcttgttgcccaggctggagtgcaatggcgcgatcttggctcaccgcaacctctgcctcccaggttcaagcagttctcctgcttcagcctcccgagtagctggtattacaggcatgcaccaccaagcctggctaattttgtatttttagtagagacggggtttctccatgttggtcaggctggtcttgaacgcctgacctcaggtgatctgcctgcctcggcctcccaaagtgctgggattacaggcatgagccatcacgcccggccaaagttttagaatttaagttattccaaaaaaaattttttttttcaaaaatacagactgcatccaattaaattctatgttaactggtaatgactaggtctaaaatgttaggtatttaccaataaatgacataaaataactcaacaacaaagggatttttttttttaagagatagggtctcactttatcactcaggtttggctgagggcagtggtgtgatcacagctcactgaagcctccaactcctgggctcaagtgatcctcccgcctcagtctaccagagtatattcttgaaagtaaaattacaaatgaaattcagcagtgttaaaaataagcccacttgcagacaattatcatttttcttcctttctttcctcactatctgtacttggcatatttcctacagtggctgtcttaaagaaaaaaaggaatccttcacaaatagtgtagccaaaaaagttggactaatatacaatgctatcagtaaagtattatatataaaatttataagtgctaaagtgtaattttgaaagacacttaagatactccttttttttttgagacaaggtctcagccctgtcgcccaggctggagtgcactagcacaacatcagctcactgcaacctccgcctcccaggttcaagcgattctcctgcctcagcctcccaagtagctgagactacaggcgcacgccagcatgtccagataattttttgtatttttagtagagatggggtttcaccatgttggccaggatggtctcaaatctcttgacctcgtgatctgcccatgtcggcttcccaaagtgttaggataacaggcatgagctaccgtgcccagcctacttaaaatattcttgaaatagctctccccacctccttttttttttttttttgagaatgagtttcactcgacacccaggctggagtgcagtggtgcgatcttggctcactgcaacctctgcctcccaggttcaagcgattatcctgcctcagcctcctgagtagctgggattacaaatgtgcaccaccacatctggctaattttttttttttttttttgtatttttagtagagacggggtttcaccaagttggcctggctggtctcgaacacctgacctcaattgatccacctgcctcggcctcccaaagtattataggcatgagccaccgagcccggccttttttgttttttgtttttttaaaggcagggttttgctctgttgcccaggctggagtgcagtggtgtgatcacagatcactgcagccttgacctctcctggtctcaagtgatcctcccacctcagccttcagaacagctgggactacaggtgtgtgtcaccatgcccagtaatttttttgtatatttgtagaggcagggtctcccaatgttgcctgggctggtctcaaactcctgggctcaagcaatccaccagctttggccttccaaagttctaggattatacgcatgagccactgtgccctgccccaatattttgttacttactagtgagactaaacacttttctaaaagtttgttagccatactatcctataaaagctgtttgttcatgtcttttgtccatttatctttttttttgtttttcttgagacagagtcttgctctgtggcccaggctggagtgcaggggtgcaatctcggctcactgcaagctccgcctcccaggttcaaatgattctcctgcctcagcctcctgagtagctgggattacaggcatgtgccaccatgcccagctaatttttttgtgtgtgtttttcagtagagatggggtttcaccatgttggccaggctgatctcgaattcctgacctcaggtgctccacccgcctcagcctcccaaagtactgggattacaggggtgagccaccgcacccggccaattttctgtatttttaatagagacagggtttcatcctgttggccaggctggcctcgaacttcggacctcaggtgatccacccgcctcgacctcccaaagtgctgggattacaggtgtgggccaccacacccagccaatttttttgtatttttagtagagacagggtttcatcatgttggccaggctggtcgcaaactcctgacctcaggtgatccacccgcctcagcatcccaaagtgctgggattacaggcatgagccaccactcccggccaatgttttgtatttttagtagagatggggtttcatcatgttggccagactggtctcaaactctggacctcaggtgatccacctgcctcagcctcccaaagtgtagggattacaggtgtgagccaccgcgcccagcctatgtttctattttatacatattcaacaaacatgattccccaacttctgcaaaataatttctttttcaagaacattgattttagagctcacactaagaaaaagaatacaaaaataatggcatagaaagtgaaaaaacaaaaataaaaagtagaaagctaaagtttcccattaaaatgatcaatatactgtgcagtaagtcaaatgtgtacaatgaattaagaaaatatgatatataaaaatccaaatttacaaaattaagtacaaataggtgtttatattacaaagtgatactggtttataaaaggattcaacatagattttttttaaatggttgttttcctcaatcaatttaacaatgattttaaatgtataaaattttaatatctctttgagacagtgatccaagcttcttcccttgatgatgttaccagttcatactttgtttcaataacctgtccctccacagaaagtaggtgcagtctcttcaccaatacactaagaagtactgtggtcaccatatatgcaaacctcaactctggacactcctgtgtgcctgagaatccaagtgaggaaaaagttttcattactaattcatcatcaaaccgatctggatcaaacttgtgtggagatggccaagtattaggatcctgaagtaccacaccaagggcataaaggacgagggtctctctaggaataataaatcggtcaatttttccttcaatatcttgaagctgggcagaaactggagtcagtttggcagttcgaacagtttcacaaagcacatgctgacaatatctgagctgctcaattttctctggagtaacaggaccatttccaaaaacttggtttatctcttcatataattttttttgaacttcttcagaggtggttaaaaaacagattgcccaggtacacaattttgcagttattatgcaactggccagagaaaatatcatactgtcttctaggatctgttggtcattaaggttcccttgtactaaggagtcaatgaaaatatgttgactgaagttccttccttttcgttcttttatgatgttccttaaaacagactccagttgcatgagggtgtgccatgattcttctggaagcgaatgacttcctgatcatcttcaaatgtactacccattaccatctgtgtaacagacttcatagcaaaaccaagcatatgctggctgaggggcacgtgctgggtctctgggtaggagagccatttatctaataattcttctgaaagcttaataatgacttcagcatggtttcaaaagggtccgttttcttcagttggagtaatccctggaattcctgcagcttgtctggaagccggatagaggtagagcacggctcccaccaacgccagcaagaaggtaacggcgaagatcgcgaagtccaacatggttctgccgcccagggagccacgtctcggatcggccgctccagc

SEQ ID NO: 13077 - RNA, 9135 nt, Homo sapiens
  source 1..9135: mol_type = other RNA
gctgggattacaggcatgagccaccacacccagctggaaaatgtttaaaatttattaagtgaaaagtaactcatgctgcaatgaacgtactatgtaaaaatgtatgtatgtggaacagggaaaaatataaacagtcacagaaatgtgtttaggttggtagcattctttttcctcttaaaaattcctttttttggccgggcgctgtggctcacacctgtaatcccagcactttgggaagccgcggtggacagatcacaaggtcaggagatcaagaccatcctggctaacatggtgaaaccccgtctctactaaaaatacaaaaaattagctgggcatggaggcactcgcctgtagtcgcagctactcgggaggctgaggcaggagaatcgcttgaactggggagatggaggttgtagtgagcccagatcatgccactgcactcaagcctgggctgagacctccagagtctggctgagacctatggagtctcactctgtcacctaggctggagtacagtggtgcgatctcggcacactgcaacctccacctcccagacattctcctgcctcagcctctcaactagctgggattacattcgcccgcctccacacccactaatttttgtatttttagtagagatgcggtttccccatgttggccaggctgttcttgaactcctgacctcaagttatacgcccactttggactcccaaagtgctgggattacaggtgtgagccacggcaccagccaaaaatttctttaaatattagtggtatattattctctcaataagttttttttttttttttttttgagacagtcttgttttattgcctaagctggagtgcagtggcacaatctcaactcactgcaacctccacctcccaggtttattttttttctcatgcctcagcctcccaagaagctgggattacaggcatgtgccccaaaggccagttaagttttctttttctttttttcttttttcttggttgagacggattttcgctcgtcacccacactggagtgcaatggcgcgatctcggctcactgcaacctccgactcttgggttcaagcgattctcctgcctcagcctcccgagtagctgggattagaggcacctgtcaccacgcccgctacttttggtatttttagtagagatggagtttcaccacgttggccaggctgatctcaaactcctggcctcaagtgattcacctgccttggcctcccaaagtgctggaattacaggcccggcctatttttgcaataattatgaatagcacaccatttaaacctgttgattgagccctccttaaataactaaatacactactggccaacatggtgaaaacctgtctccactaaaaacacaaaaaaatggccgggcacagtggctcatgcctgtaatcccagcacttcaggaggccaaggggtgtgaatcacctgaggttaggagttcaagaccagcctggccaacatggtgaaaccctgtctctactaaaaaaaaatacaaaaattagctgagtgtagtggcacatacccgtagtctcagctactcaggaggctgaggcaggagaattgcttgaacctgggaggcaggggttgcagtgagccaagatcgtgccaccacactccagcctgggtgacacagcgagactccatctcaaaataaataaataaataaaaagaaagggaccgagcgcggtggctcatgcttgtaatcccagcactctgggaggctgagttgggcagatcacaaggtcaagagttcaggaccagcctgaccaacacggtaaaaccccatctctactaaaaatacaaaaatgagctgggtgtgatggcacgcgcctgtaaccccagttactcaaaaggctgaggcaagagaatcgcttgaacctgggaggcagaggttgcagtgagccgagatcacgccactgcattccagcctggtgacagtgagactctgtcacacacacacaaaaaagataaagaatgacaaaaatctgtgcctacattcagagtgacaagaatactaatgttctgcttgtagaaaagactattggttcagaatatgttaaatgcaaataatattttgtataatatatataaattacatatgcataaaaagagtatctatattagaatcttttgagacagggtcttgctctgtcaaccatgagggagtgcagtggcactaccacagctcactgtagccttgacttcctgagctcaagccatcctctcgcctcagcctcctgaatagttgggactgcaggtggtgccaccaaggctggctaagtttttatatttttttatagaaacaagcttttgccacgttgcccaggctggtctcaaacttctaaaagctcaagcaatctggccgccttgaactcccaaagtgcttgagttataggcatgagtcactgtgcccggcctacattagaatcttaacagtggggctgggcatggtgccccatgcctgtaatcccagcactttgggaggtcaaggtgggcagactacttgaggttgaggagttcgaggccagcctggccaacatggtgaaaccccatctgtactaaaaacacaaaaattagccaggtgtggtggcacatgtttgcaatcccagctacttgggaggctgaggcgggaggatcacttgaacctgggaagcagaggttgcagtgagccgagatggtgccatggcactccagcctgggcaatagacagcgggactcagtctcaaaacaaaaaaaaaaaaaaaaaaaaaagaatcttaacagtggttaacttcaaatagtgaaactatgactgttaactgagtttgacatttttgtgttttcctagatttttctacaataaacattattatttcataataaagcagtaaagactttttatacaaactattttaagataaacaaattttgacataggggttataagttaggtagaatctatttatataaaaaatggaactgtacttttgtgggccaaataagcactatgtaagtttttttaattttcccaaacacatgcacagaattaatattgccttaaattttgttagcacaagtttgagagagctctttagttcataaaaaaatgttttatggaccaggtgccgtggctcacacctgcaatctcaacactttgggaggcccaggtgggaggatcgcttgagcctaggagtttgagacaagactgggcgacgcagggagaccctgtctcaaaaaaacaaaaccaaaaacaagcaaacaaaaaaacagctgggcatggtggcatgcatatgtagtcccagctattctagaggctgaggtgagatcgctggagcccaggaggtggaggctacagtaagctgtgatcatgccaatgcactccagcttggtcaacaaagcaagactgtgcctcaaaaaaaaaaaagaaaagaaaagaaagaaagaaaagaaaaagaaaaaaagttatgtacgtatggtttttttttttttttggatagagtttcactcttcttgcccaggctggagtgcaatggtgcaatcttggctcaccacaaccttcccctactgggttcaagcgattctcctgtttcagcctccccagtagctgggattaaaggcatgtgccaccacgcccggctaattttgtatttttagtagagatgaagtttctccatgttggtcaggctggtcttgaactcctgacttcaggtgatctgcccgcctcagcctcccaaagtgctgggattacaggtgtgagccacctcgcctggccgttttttttttttttttttttttctgagacggagttttgctcttattgcccaggctggagtgcaatggcacgatctcggctcatcgcaacctctgcctcacgggttcaagcaattttcctgcctcagcgtctcaagtagctaggattacagggatgctccatcatgcccggctaattttgtatttttggtagagacagggtttctccatgttggtcaggctggtctcaaactcccaacctcaggtgatttacccgccttggcctcccaaagagctgggattacaggtgtgagccactgtgcccggccatgcttatgttttttaacaatacacttctgaactatcaaaaagaatataaatcaaaatcactgaagtagtttttaaaaactccaaaagctacaaaacttacttacttcaatatcaattaaaaacccatttgatagttcaataacttgagtcctgctagaatcattctataagccatcagtgacagtgaagtggccaaaatttgagtcacttgataagtacaaagaacacagatttttgtcattcttactgtgaagaaaaacagtgaatgaataacttagtttatatattaacagtacttttatttaaaaaattatctagagaataacttctttttaatcatttgttagtcatgtaactatggataaaacatactaatttagctgattcctctatgctctcttttccttgattccaatcattattagttattctacactgcctcatttattggcagttatgccaactggctgactctggttcaactgccctatttttgctttcatcattgtttatcatatctcacttgctttaaactccacctctttcatctcatctgatctgacacttggtttacatatcaattggctactctaaccttctaccgccagtttccaacccattcgaggtacttgggtaacaaaggaagatgctctatacacacaaaaccacagaaaataagtgggaagggataataaatttcacttaaagttttagaatttttcttttttttttgagacggagtttcactcttgttgcccaggctggagtgcaatggcgcgatcttggctcaccgcaacctctgcctcccaggttcaagcagttctcctgcttcagcctcccgagtagctggtattacaggcatgcaccaccaagcctggctaattttgtatttttagtagagacggggtttctccatgttggtcaggctggtcttgaacgcctgacctcaggtgatctgcctgcctcggcctcccaaagtgctgggattacaggcatgagccatcacgcccggccaaagttttagaatttaagttattccaaaaaaaattttttttttcaaaaatacagactgcatccaattaaattctatgttaactggtaatgactaggtctaaaatgttaggtatttaccaataaatgacataaaataactcaacaacaaagggatttttttttttaagagatagggtctcactttatcactcaggtttggctgagggcagtggtgtgatcacagctcactgaagcctccaactcctgggctcaagtgatcctcccgcctcagtctaccagagtatattcttgaaagtaaaattacaaatgaaattcagcagtgttaaaaataagcccacttgcagacaattatcatttttcttcctttctttcctcactatctgtacttggcatatttcctacagtggctgtcttaaagaaaaaaaggaatccttcacaaatagtgtagccaaaaaagttggactaatatacaatgctatcagtaaagtattatatataaaatttataagtgctaaagtgtaattttgaaagacacttaagatactccttttttttttgagacaaggtctcagccctgtcgcccaggctggagtgcactagcacaacatcagctcactgcaacctccgcctcccaggttcaagcgattctcctgcctcagcctcccaagtagctgagactacaggcgcacgccagcatgtccagataattttttgtatttttagtagagatggggtttcaccatgttggccaggatggtctcaaatctcttgacctcgtgatctgcccatgtcggcttcccaaagtgttaggataacaggcatgagctaccgtgcccagcctacttaaaatattcttgaaatagctctccccacctccttttttttttttttttgagaatgagtttcactcgacacccaggctggagtgcagtggtgcgatcttggctcactgcaacctctgcctcccaggttcaagcgattatcctgcctcagcctcctgagtagctgggattacaaatgtgcaccaccacatctggctaattttttttttttttttttgtatttttagtagagacggggtttcaccaagttggcctggctggtctcgaacacctgacctcaattgatccacctgcctcggcctcccaaagtattataggcatgagccaccgagcccggccttttttgttttttgtttttttaaaggcagggttttgctctgttgcccaggctggagtgcagtggtgtgatcacagatcactgcagccttgacctctcctggtctcaagtgatcctcccacctcagccttcagaacagctgggactacaggtgtgtgtcaccatgcccagtaatttttttgtatatttgtagaggcagggtctcccaatgttgcctgggctggtctcaaactcctgggctcaagcaatccaccagctttggccttccaaagttctaggattatacgcatgagccactgtgccctgccccaatattttgttacttactagtgagactaaacacttttctaaaagtttgttagccatactatcctataaaagctgtttgttcatgtcttttgtccatttatctttttttttgtttttcttgagacagagtcttgctctgtggcccaggctggagtgcaggggtgcaatctcggctcactgcaagctccgcctcccaggttcaaatgattctcctgcctcagcctcctgagtagctgggattacaggcatgtgccaccatgcccagctaatttttttgtgtgtgtttttcagtagagatggggtttcaccatgttggccaggctgatctcgaattcctgacctcaggtgctccacccgcctcagcctcccaaagtactgggattacaggggtgagccaccgcacccggccaattttctgtatttttaatagagacagggtttcatcctgttggccaggctggcctcgaacttcggacctcaggtgatccacccgcctcgacctcccaaagtgctgggattacaggtgtgggccaccacacccagccaatttttttgtatttttagtagagacagggtttcatcatgttggccaggctggtcgcaaactcctgacctcaggtgatccacccgcctcagcatcccaaagtgctgggattacaggcatgagccaccactcccggccaatgttttgtatttttagtagagatggggtttcatcatgttggccagactggtctcaaactctggacctcaggtgatccacctgcctcagcctcccaaagtgtagggattacaggtgtgagccaccgcgcccagcctatgtttctattttatacatattcaacaaacatgattccccaacttctgcaaaataatttctttttcaagaacattgattttagagctcacactaagaaaaagaatacaaaaataatggcatagaaagtgaaaaaacaaaaataaaaagtagaaagctaaagtttcccattaaaatgatcaatatactgtgcagtaagtcaaatgtgtacaatgaattaagaaaatatgatatataaaaatccaaatttacaaaattaagtacaaataggtgtttatattacaaagtgatactggtttataaaaggattcaacatagattttttttaaatggttgttttcctcaatcaatttaacaatgattttaaatgtataaaattttaatatctctttgagacagtgatccaagcttcttcccttgatgatgttaccagttcatactttgtttcaataacctgtccctccacagaaagtaggtgcagtctcttcaccaatacactaagaagtactgtggtcaccatatatgcaaacctcaactctggacactcctgtgtgcctgagaatccaagtgaggaaaaagttttcattactaattcatcatcaaaccgatctggatcaaacttgtgtggagatggccaagtattaggatcctgaagtaccacaccaagggcataaaggacgagggtctctctaggaataataaatcggtcaatttttccttcaatatcttgaagctgggcagaaactggagtcagtttggcagttcgaacagtttcacaaagcacatgctgacaatatctgagctgctcaattttctctggagtaacaggaccatttccaaaaacttggtttatctcttcatataattttttttgaacttcttcagaggtggttaaaaaacagattgcccaggtacacaattttgcagttattatgcaactggccagagaaaatatcatactgtcttctaggatctgttggtcattaaggttcccttgtactaaggagtcaatgaaaatatgttgactgaagttccttccttttcgttcttttatgatgttccttaaaacagactccagttgcatgagggtgtgccatgattcttctggaagcgaatgacttcctgatcatcttcaaatgtactacccattaccatctgtgtaacagacttcatagcaaaaccaagcatatgctggctgaggggcacgtgctgggtctctgggtaggagagccatttatctaataattcttctgaaagctttaggaggagggcaaagttactcttcagagaatcagtcacaccattttcatacaattttttcctcatgtggttttcactcacactgccaccaccagattgataccttaataatgacttcagcatggtttcaaaagggtccgatgtcttattgggattgatatgctgcttcagtacatcaacagtgcccaaactaaccacgaggcgcctgccaaaccagaaggagaccacaggcccatatctctcatgcaaattaaccaggaactcatgcaaacttccactattcacaatatctggaagattaccatctttttcttcagttggagtaatccctggaattcctgcagcttgtctggaagccggatagaggtagagcacggctcccaccaacgccagcaagaaggtaacggcgaagatcgcgaagtccaacatggttctgccgcccagggagccacgtctcggatcggccgctccagc

SEQ ID NO: 13078 - RNA, 8918 nt, Homo sapiens
  source 1..8918: mol_type = other RNA
gctgggattacaggcatgagccaccacacccagctggaaaatgtttaaaatttattaagtgaaaagtaactcatgctgcaatgaacgtactatgtaaaaatgtatgtatgtggaacagggaaaaatataaacagtcacagaaatgtgtttaggttggtagcattctttttcctcttaaaaattcctttttttggccgggcgctgtggctcacacctgtaatcccagcactttgggaagccgcggtggacagatcacaaggtcaggagatcaagaccatcctggctaacatggtgaaaccccgtctctactaaaaatacaaaaaattagctgggcatggaggcactcgcctgtagtcgcagctactcgggaggctgaggcaggagaatcgcttgaactggggagatggaggttgtagtgagcccagatcatgccactgcactcaagcctgggctgagacctccagagtctggctgagacctatggagtctcactctgtcacctaggctggagtacagtggtgcgatctcggcacactgcaacctccacctcccagacattctcctgcctcagcctctcaactagctgggattacattcgcccgcctccacacccactaatttttgtatttttagtagagatgcggtttccccatgttggccaggctgttcttgaactcctgacctcaagttatacgcccactttggactcccaaagtgctgggattacaggtgtgagccacggcaccagccaaaaatttctttaaatattagtggtatattattctctcaataagttttttttttttttttttttgagacagtcttgttttattgcctaagctggagtgcagtggcacaatctcaactcactgcaacctccacctcccaggtttattttttttctcatgcctcagcctcccaagaagctgggattacaggcatgtgccccaaaggccagttaagttttctttttctttttttcttttttcttggttgagacggattttcgctcgtcacccacactggagtgcaatggcgcgatctcggctcactgcaacctccgactcttgggttcaagcgattctcctgcctcagcctcccgagtagctgggattagaggcacctgtcaccacgcccgctacttttggtatttttagtagagatggagtttcaccacgttggccaggctgatctcaaactcctggcctcaagtgattcacctgccttggcctcccaaagtgctggaattacaggcccggcctatttttgcaataattatgaatagcacaccatttaaacctgttgattgagccctccttaaataactaaatacactactggccaacatggtgaaaacctgtctccactaaaaacacaaaaaaatggccgggcacagtggctcatgcctgtaatcccagcacttcaggaggccaaggggtgtgaatcacctgaggttaggagttcaagaccagcctggccaacatggtgaaaccctgtctctactaaaaaaaaatacaaaaattagctgagtgtagtggcacatacccgtagtctcagctactcaggaggctgaggcaggagaattgcttgaacctgggaggcaggggttgcagtgagccaagatcgtgccaccacactccagcctgggtgacacagcgagactccatctcaaaataaataaataaataaaaagaaagggaccgagcgcggtggctcatgcttgtaatcccagcactctgggaggctgagttgggcagatcacaaggtcaagagttcaggaccagcctgaccaacacggtaaaaccccatctctactaaaaatacaaaaatgagctgggtgtgatggcacgcgcctgtaaccccagttactcaaaaggctgaggcaagagaatcgcttgaacctgggaggcagaggttgcagtgagccgagatcacgccactgcattccagcctggtgacagtgagactctgtcacacacacacaaaaaagataaagaatgacaaaaatctgtgcctacattcagagtgacaagaatactaatgttctgcttgtagaaaagactattggttcagaatatgttaaatgcaaataatattttgtataatatatataaattacatatgcataaaaagagtatctatattagaatcttttgagacagggtcttgctctgtcaaccatgagggagtgcagtggcactaccacagctcactgtagccttgacttcctgagctcaagccatcctctcgcctcagcctcctgaatagttgggactgcaggtggtgccaccaaggctggctaagtttttatatttttttatagaaacaagcttttgccacgttgcccaggctggtctcaaacttctaaaagctcaagcaatctggccgccttgaactcccaaagtgcttgagttataggcatgagtcactgtgcccggcctacattagaatcttaacagtggggctgggcatggtgccccatgcctgtaatcccagcactttgggaggtcaaggtgggcagactacttgaggttgaggagttcgaggccagcctggccaacatggtgaaaccccatctgtactaaaaacacaaaaattagccaggtgtggtggcacatgtttgcaatcccagctacttgggaggctgaggcgggaggatcacttgaacctgggaagcagaggttgcagtgagccgagatggtgccatggcactccagcctgggcaatagacagcgggactcagtctcaaaacaaaaaaaaaaaaaaaaaaaaaagaatcttaacagtggttaacttcaaatagtgaaactatgactgttaactgagtttgacatttttgtgttttcctagatttttctacaataaacattattatttcataataaagcagtaaagactttttatacaaactattttaagataaacaaattttgacataggggttataagttaggtagaatctatttatataaaaaatggaactgtacttttgtgggccaaataagcactatgtaagtttttttaattttcccaaacacatgcacagaattaatattgccttaaattttgttagcacaagtttgagagagctctttagttcataaaaaaatgttttatggaccaggtgccgtggctcacacctgcaatctcaacactttgggaggcccaggtgggaggatcgcttgagcctaggagtttgagacaagactgggcgacgcagggagaccctgtctcaaaaaaacaaaaccaaaaacaagcaaacaaaaaaacagctgggcatggtggcatgcatatgtagtcccagctattctagaggctgaggtgagatcgctggagcccaggaggtggaggctacagtaagctgtgatcatgccaatgcactccagcttggtcaacaaagcaagactgtgcctcaaaaaaaaaaaagaaaagaaaagaaagaaagaaaagaaaaagaaaaaaagttatgtacgtatggtttttttttttttttggatagagtttcactcttcttgcccaggctggagtgcaatggtgcaatcttggctcaccacaaccttcccctactgggttcaagcgattctcctgtttcagcctccccagtagctgggattaaaggcatgtgccaccacgcccggctaattttgtatttttagtagagatgaagtttctccatgttggtcaggctggtcttgaactcctgacttcaggtgatctgcccgcctcagcctcccaaagtgctgggattacaggtgtgagccacctcgcctggccgttttttttttttttttttttttctgagacggagttttgctcttattgcccaggctggagtgcaatggcacgatctcggctcatcgcaacctctgcctcacgggttcaagcaattttcctgcctcagcgtctcaagtagctaggattacagggatgctccatcatgcccggctaattttgtatttttggtagagacagggtttctccatgttggtcaggctggtctcaaactcccaacctcaggtgatttacccgccttggcctcccaaagagctgggattacaggtgtgagccactgtgcccggccatgcttatgttttttaacaatacacttctgaactatcaaaaagaatataaatcaaaatcactgaagtagtttttaaaaactccaaaagctacaaaacttacttacttcaatatcaattaaaaacccatttgatagttcaataacttgagtcctgctagaatcattctataagccatcagtgacagtgaagtggccaaaatttgagtcacttgataagtacaaagaacacagatttttgtcattcttactgtgaagaaaaacagtgaatgaataacttagtttatatattaacagtacttttatttaaaaaattatctagagaataacttctttttaatcatttgttagtcatgtaactatggataaaacatactaatttagctgattcctctatgctctcttttccttgattccaatcattattagttattctacactgcctcatttattggcagttatgccaactggctgactctggttcaactgccctatttttgctttcatcattgtttatcatatctcacttgctttaaactccacctctttcatctcatctgatctgacacttggtttacatatcaattggctactctaaccttctaccgccagtttccaacccattcgaggtacttgggtaacaaaggaagatgctctatacacacaaaaccacagaaaataagtgggaagggataataaatttcacttaaagttttagaatttttcttttttttttgagacggagtttcactcttgttgcccaggctggagtgcaatggcgcgatcttggctcaccgcaacctctgcctcccaggttcaagcagttctcctgcttcagcctcccgagtagctggtattacaggcatgcaccaccaagcctggctaattttgtatttttagtagagacggggtttctccatgttggtcaggctggtcttgaacgcctgacctcaggtgatctgcctgcctcggcctcccaaagtgctgggattacaggcatgagccatcacgcccggccaaagttttagaatttaagttattccaaaaaaaattttttttttcaaaaatacagactgcatccaattaaattctatgttaactggtaatgactaggtctaaaatgttaggtatttaccaataaatgacataaaataactcaacaacaaagggatttttttttttaagagatagggtctcactttatcactcaggtttggctgagggcagtggtgtgatcacagctcactgaagcctccaactcctgggctcaagtgatcctcccgcctcagtctaccagagtatattcttgaaagtaaaattacaaatgaaattcagcagtgttaaaaataagcccacttgcagacaattatcatttttcttcctttctttcctcactatctgtacttggcatatttcctacagtggctgtcttaaagaaaaaaaggaatccttcacaaatagtgtagccaaaaaagttggactaatatacaatgctatcagtaaagtattatatataaaatttataagtgctaaagtgtaattttgaaagacacttaagatactccttttttttttgagacaaggtctcagccctgtcgcccaggctggagtgcactagcacaacatcagctcactgcaacctccgcctcccaggttcaagcgattctcctgcctcagcctcccaagtagctgagactacaggcgcacgccagcatgtccagataattttttgtatttttagtagagatggggtttcaccatgttggccaggatggtctcaaatctcttgacctcgtgatctgcccatgtcggcttcccaaagtgttaggataacaggcatgagctaccgtgcccagcctacttaaaatattcttgaaatagctctccccacctccttttttttttttttttgagaatgagtttcactcgacacccaggctggagtgcagtggtgcgatcttggctcactgcaacctctgcctcccaggttcaagcgattatcctgcctcagcctcctgagtagctgggattacaaatgtgcaccaccacatctggctaattttttttttttttttttgtatttttagtagagacggggtttcaccaagttggcctggctggtctcgaacacctgacctcaattgatccacctgcctcggcctcccaaagtattataggcatgagccaccgagcccggccttttttgttttttgtttttttaaaggcagggttttgctctgttgcccaggctggagtgcagtggtgtgatcacagatcactgcagccttgacctctcctggtctcaagtgatcctcccacctcagccttcagaacagctgggactacaggtgtgtgtcaccatgcccagtaatttttttgtatatttgtagaggcagggtctcccaatgttgcctgggctggtctcaaactcctgggctcaagcaatccaccagctttggccttccaaagttctaggattatacgcatgagccactgtgccctgccccaatattttgttacttactagtgagactaaacacttttctaaaagtttgttagccatactatcctataaaagctgtttgttcatgtcttttgtccatttatctttttttttgtttttcttgagacagagtcttgctctgtggcccaggctggagtgcaggggtgcaatctcggctcactgcaagctccgcctcccaggttcaaatgattctcctgcctcagcctcctgagtagctgggattacaggcatgtgccaccatgcccagctaatttttttgtgtgtgtttttcagtagagatggggtttcaccatgttggccaggctgatctcgaattcctgacctcaggtgctccacccgcctcagcctcccaaagtactgggattacaggggtgagccaccgcacccggccaattttctgtatttttaatagagacagggtttcatcctgttggccaggctggcctcgaacttcggacctcaggtgatccacccgcctcgacctcccaaagtgctgggattacaggtgtgggccaccacacccagccaatttttttgtatttttagtagagacagggtttcatcatgttggccaggctggtcgcaaactcctgacctcaggtgatccacccgcctcagcatcccaaagtgctgggattacaggcatgagccaccactcccggccaatgttttgtatttttagtagagatggggtttcatcatgttggccagactggtctcaaactctggacctcaggtgatccacctgcctcagcctcccaaagtgtagggattacaggtgtgagccaccgcgcccagcctatgtttctattttatacatattcaacaaacatgattccccaacttctgcaaaataatttctttttcaagaacattgattttagagctcacactaagaaaaagaatacaaaaataatggcatagaaagtgaaaaaacaaaaataaaaagtagaaagctaaagtttcccattaaaatgatcaatatactgtgcagtaagtcaaatgtgtacaatgaattaagaaaatatgatatataaaaatccaaatttacaaaattaagtacaaataggtgtttatattacaaagtgatactggtttataaaaggattcaacatagattttttttaaatggttgttttcctcaatcaatttaacaatgattttaaatgtataaaattttaatatctctttgagacagtgatccaagcttcttcccttgatgatgttaccagttcatactttgtttcaataacctgtccctccacagaaagtaggtgcagtctcttcaccaatacactaagaagtactgtggtcaccatatatgcaaacctcaactctggacactcctgtgtgcctgagaatccaagtgaggaaaaagttttcattactaattcatcatcaaaccgatctggatcaaacttgtgtggagatggccaagtattaggatcctgaagtaccacaccaagggcataaaggacgagggtctctctaggaataataaatcggtcaatttttccttcaatatcttgaagctgggcagaaactggagtcagtttggcagttcgaacagtttcacaaagcacatgctgacaatatctgagctgctcaattttctctggagtaacaggaccatttccaaaaacttggtttatctcttcatataattttttttgaacttcttcagaggtggttaaaaaacagattgcccaggtacacaattttgcagttattatgcaactggccagagaaaatatcatactgtcttctaggatctgttggtcattaaggttcccttgtactaaggagtcaatgaaaatatgttgactgaagttccttccttttcgttcttttatgatgttccttaaaacagactccagttgcatgagggtgtgccatgattcttctggaagcgaatgacttcctgatcatcttcaaatgtactacccattaccatctgtgtaacagacttcatagcaaaaccaagcatatgctggctgaggggcacgtgctgggtctctgggtaggagagccatttatctaataattcttctgaaagctttaggaggagggcaaagttactcttcagagaatcagtcacaccattttcatacaattttttcctcatgtggttttcactcacactgccaccaccagattgataccttaataatgacttcagcatggtttcaaaagggtccgcggatagaggtagagcacggctcccaccaacgccagcaagaaggtaacggcgaagatcgcgaagtccaacatggttctgccgcccagggagccacgtctcggatcggccgctccagc

SEQ ID NO: 13079 - RNA, 9687 nt, Homo sapiens
  source 1..9687: mol_type = other RNA
gctgggattacaggcatgagccaccacacccagctggaaaatgtttaaaatttattaagtgaaaagtaactcatgctgcaatgaacgtactatgtaaaaatgtatgtatgtggaacagggaaaaatataaacagtcacagaaatgtgtttaggttggtagcattctttttcctcttaaaaattcctttttttggccgggcgctgtggctcacacctgtaatcccagcactttgggaagccgcggtggacagatcacaaggtcaggagatcaagaccatcctggctaacatggtgaaaccccgtctctactaaaaatacaaaaaattagctgggcatggaggcactcgcctgtagtcgcagctactcgggaggctgaggcaggagaatcgcttgaactggggagatggaggttgtagtgagcccagatcatgccactgcactcaagcctgggctgagacctccagagtctggctgagacctatggagtctcactctgtcacctaggctggagtacagtggtgcgatctcggcacactgcaacctccacctcccagacattctcctgcctcagcctctcaactagctgggattacattcgcccgcctccacacccactaatttttgtatttttagtagagatgcggtttccccatgttggccaggctgttcttgaactcctgacctcaagttatacgcccactttggactcccaaagtgctgggattacaggtgtgagccacggcaccagccaaaaatttctttaaatattagtggtatattattctctcaataagttttttttttttttttttttgagacagtcttgttttattgcctaagctggagtgcagtggcacaatctcaactcactgcaacctccacctcccaggtttattttttttctcatgcctcagcctcccaagaagctgggattacaggcatgtgccccaaaggccagttaagttttctttttctttttttcttttttcttggttgagacggattttcgctcgtcacccacactggagtgcaatggcgcgatctcggctcactgcaacctccgactcttgggttcaagcgattctcctgcctcagcctcccgagtagctgggattagaggcacctgtcaccacgcccgctacttttggtatttttagtagagatggagtttcaccacgttggccaggctgatctcaaactcctggcctcaagtgattcacctgccttggcctcccaaagtgctggaattacaggcccggcctatttttgcaataattatgaatagcacaccatttaaacctgttgattgagccctccttaaataactaaatacactactggccaacatggtgaaaacctgtctccactaaaaacacaaaaaaatggccgggcacagtggctcatgcctgtaatcccagcacttcaggaggccaaggggtgtgaatcacctgaggttaggagttcaagaccagcctggccaacatggtgaaaccctgtctctactaaaaaaaaatacaaaaattagctgagtgtagtggcacatacccgtagtctcagctactcaggaggctgaggcaggagaattgcttgaacctgggaggcaggggttgcagtgagccaagatcgtgccaccacactccagcctgggtgacacagcgagactccatctcaaaataaataaataaataaaaagaaagggaccgagcgcggtggctcatgcttgtaatcccagcactctgggaggctgagttgggcagatcacaaggtcaagagttcaggaccagcctgaccaacacggtaaaaccccatctctactaaaaatacaaaaatgagctgggtgtgatggcacgcgcctgtaaccccagttactcaaaaggctgaggcaagagaatcgcttgaacctgggaggcagaggttgcagtgagccgagatcacgccactgcattccagcctggtgacagtgagactctgtcacacacacacaaaaaagataaagaatgacaaaaatctgtgcctacattcagagtgacaagaatactaatgttctgcttgtagaaaagactattggttcagaatatgttaaatgcaaataatattttgtataatatatataaattacatatgcataaaaagagtatctatattagaatcttttgagacagggtcttgctctgtcaaccatgagggagtgcagtggcactaccacagctcactgtagccttgacttcctgagctcaagccatcctctcgcctcagcctcctgaatagttgggactgcaggtggtgccaccaaggctggctaagtttttatatttttttatagaaacaagcttttgccacgttgcccaggctggtctcaaacttctaaaagctcaagcaatctggccgccttgaactcccaaagtgcttgagttataggcatgagtcactgtgcccggcctacattagaatcttaacagtggggctgggcatggtgccccatgcctgtaatcccagcactttgggaggtcaaggtgggcagactacttgaggttgaggagttcgaggccagcctggccaacatggtgaaaccccatctgtactaaaaacacaaaaattagccaggtgtggtggcacatgtttgcaatcccagctacttgggaggctgaggcgggaggatcacttgaacctgggaagcagaggttgcagtgagccgagatggtgccatggcactccagcctgggcaatagacagcgggactcagtctcaaaacaaaaaaaaaaaaaaaaaaaaaagaatcttaacagtggttaacttcaaatagtgaaactatgactgttaactgagtttgacatttttgtgttttcctagatttttctacaataaacattattatttcataataaagcagtaaagactttttatacaaactattttaagataaacaaattttgacataggggttataagttaggtagaatctatttatataaaaaatggaactgtacttttgtgggccaaataagcactatgtaagtttttttaattttcccaaacacatgcacagaattaatattgccttaaattttgttagcacaagtttgagagagctctttagttcataaaaaaatgttttatggaccaggtgccgtggctcacacctgcaatctcaacactttgggaggcccaggtgggaggatcgcttgagcctaggagtttgagacaagactgggcgacgcagggagaccctgtctcaaaaaaacaaaaccaaaaacaagcaaacaaaaaaacagctgggcatggtggcatgcatatgtagtcccagctattctagaggctgaggtgagatcgctggagcccaggaggtggaggctacagtaagctgtgatcatgccaatgcactccagcttggtcaacaaagcaagactgtgcctcaaaaaaaaaaaagaaaagaaaagaaagaaagaaaagaaaaagaaaaaaagttatgtacgtatggtttttttttttttttggatagagtttcactcttcttgcccaggctggagtgcaatggtgcaatcttggctcaccacaaccttcccctactgggttcaagcgattctcctgtttcagcctccccagtagctgggattaaaggcatgtgccaccacgcccggctaattttgtatttttagtagagatgaagtttctccatgttggtcaggctggtcttgaactcctgacttcaggtgatctgcccgcctcagcctcccaaagtgctgggattacaggtgtgagccacctcgcctggccgttttttttttttttttttttttctgagacggagttttgctcttattgcccaggctggagtgcaatggcacgatctcggctcatcgcaacctctgcctcacgggttcaagcaattttcctgcctcagcgtctcaagtagctaggattacagggatgctccatcatgcccggctaattttgtatttttggtagagacagggtttctccatgttggtcaggctggtctcaaactcccaacctcaggtgatttacccgccttggcctcccaaagagctgggattacaggtgtgagccactgtgcccggccatgcttatgttttttaacaatacacttctgaactatcaaaaagaatataaatcaaaatcactgaagtagtttttaaaaactccaaaagctacaaaacttacttacttcaatatcaattaaaaacccatttgatagttcaataacttgagtcctgctagaatcattctataagccatcagtgacagtgaagtggccaaaatttgagtcacttgataagtacaaagaacacagatttttgtcattcttactgtgaagaaaaacagtgaatgaataacttagtttatatattaacagtacttttatttaaaaaattatctagagaataacttctttttaatcatttgttagtcatgtaactatggataaaacatactaatttagctgattcctctatgctctcttttccttgattccaatcattattagttattctacactgcctcatttattggcagttatgccaactggctgactctggttcaactgccctatttttgctttcatcattgtttatcatatctcacttgctttaaactccacctctttcatctcatctgatctgacacttggtttacatatcaattggctactctaaccttctaccgccagtttccaacccattcgaggtacttgggtaacaaaggaagatgctctatacacacaaaaccacagaaaataagtgggaagggataataaatttcacttaaagttttagaatttttcttttttttttgagacggagtttcactcttgttgcccaggctggagtgcaatggcgcgatcttggctcaccgcaacctctgcctcccaggttcaagcagttctcctgcttcagcctcccgagtagctggtattacaggcatgcaccaccaagcctggctaattttgtatttttagtagagacggggtttctccatgttggtcaggctggtcttgaacgcctgacctcaggtgatctgcctgcctcggcctcccaaagtgctgggattacaggcatgagccatcacgcccggccaaagttttagaatttaagttattccaaaaaaaattttttttttcaaaaatacagactgcatccaattaaattctatgttaactggtaatgactaggtctaaaatgttaggtatttaccaataaatgacataaaataactcaacaacaaagggatttttttttttaagagatagggtctcactttatcactcaggtttggctgagggcagtggtgtgatcacagctcactgaagcctccaactcctgggctcaagtgatcctcccgcctcagtctaccagagtatattcttgaaagtaaaattacaaatgaaattcagcagtgttaaaaataagcccacttgcagacaattatcatttttcttcctttctttcctcactatctgtacttggcatatttcctacagtggctgtcttaaagaaaaaaaggaatccttcacaaatagtgtagccaaaaaagttggactaatatacaatgctatcagtaaagtattatatataaaatttataagtgctaaagtgtaattttgaaagacacttaagatactccttttttttttgagacaaggtctcagccctgtcgcccaggctggagtgcactagcacaacatcagctcactgcaacctccgcctcccaggttcaagcgattctcctgcctcagcctcccaagtagctgagactacaggcgcacgccagcatgtccagataattttttgtatttttagtagagatggggtttcaccatgttggccaggatggtctcaaatctcttgacctcgtgatctgcccatgtcggcttcccaaagtgttaggataacaggcatgagctaccgtgcccagcctacttaaaatattcttgaaatagctctccccacctccttttttttttttttttgagaatgagtttcactcgacacccaggctggagtgcagtggtgcgatcttggctcactgcaacctctgcctcccaggttcaagcgattatcctgcctcagcctcctgagtagctgggattacaaatgtgcaccaccacatctggctaattttttttttttttttttgtatttttagtagagacggggtttcaccaagttggcctggctggtctcgaacacctgacctcaattgatccacctgcctcggcctcccaaagtattataggcatgagccaccgagcccggccttttttgttttttgtttttttaaaggcagggttttgctctgttgcccaggctggagtgcagtggtgtgatcacagatcactgcagccttgacctctcctggtctcaagtgatcctcccacctcagccttcagaacagctgggactacaggtgtgtgtcaccatgcccagtaatttttttgtatatttgtagaggcagggtctcccaatgttgcctgggctggtctcaaactcctgggctcaagcaatccaccagctttggccttccaaagttctaggattatacgcatgagccactgtgccctgccccaatattttgttacttactagtgagactaaacacttttctaaaagtttgttagccatactatcctataaaagctgtttgttcatgtcttttgtccatttatctttttttttgtttttcttgagacagagtcttgctctgtggcccaggctggagtgcaggggtgcaatctcggctcactgcaagctccgcctcccaggttcaaatgattctcctgcctcagcctcctgagtagctgggattacaggcatgtgccaccatgcccagctaatttttttgtgtgtgtttttcagtagagatggggtttcaccatgttggccaggctgatctcgaattcctgacctcaggtgctccacccgcctcagcctcccaaagtactgggattacaggggtgagccaccgcacccggccaattttctgtatttttaatagagacagggtttcatcctgttggccaggctggcctcgaacttcggacctcaggtgatccacccgcctcgacctcccaaagtgctgggattacaggtgtgggccaccacacccagccaatttttttgtatttttagtagagacagggtttcatcatgttggccaggctggtcgcaaactcctgacctcaggtgatccacccgcctcagcatcccaaagtgctgggattacaggcatgagccaccactcccggccaatgttttgtatttttagtagagatggggtttcatcatgttggccagactggtctcaaactctggacctcaggtgatccacctgcctcagcctcccaaagtgtagggattacaggtgtgagccaccgcgcccagcctatgtttctattttatacatattcaacaaacatgattccccaacttctgcaaaataatttctttttcaagaacattgattttagagctcacactaagaaaaagaatacaaaaataatggcatagaaagtgaaaaaacaaaaataaaaagtagaaagctaaagtttcccattaaaatgatcaatatactgtgcagtaagtcaaatgtgtacaatgaattaagaaaatatgatatataaaaatccaaatttacaaaattaagtacaaataggtgtttatattacaaagtgatactggtttataaaaggattcaacatagattttttttaaatggttgttttcctcaatcaatttaacaatgattttaaatgtataaaattttaatatctctttgagacagtgatccaagcttcttcccttgatgatgttaccagttcatactttgtttcaataacctgtccctccacagaaagtaggtgcagtctcttcaccaatacactaagaagtactgtggtcaccatatatgcaaacctcaactctggacactcctgtgtgcctgagaatccaagtgaggaaaaagttttcattactaattcatcatcaaaccgatctggatcaaacttgtgtggagatggccaagtattaggatcctgaagtaccacaccaagggcataaaggacgagggtctctctaggaataataaatcggtcaatttttccttcaatatcttgaagctgggcagaaactggagtcagtttggcagttcgaacagtttcacaaagcacatgctgacaatatctgagctgctcaattttctctggagtaacaggaccatttccaaaaacttggtttatctcttcatataattttttttgaacttcttcagaggtggttaaaaaacagattgcccaggtacacaattttgcagttattatgcaactggccagagaaaatatcatactgtcttctaggatctgttggtcattaaggttcccttgtactaaggagtcaatgaaaatatgttgactgaagttccttccttttcgttcttttatgatgttccttaaaacagactccagttgcatgagggtgtgccatgattcttctggaagcgaatgacttcctgatcatcttcaaatgtactacccattaccatctgtgtaacagacttcatagcaaaaccaagcatatgctggctgaggggcacgtgctgggtctctgggtaggagagccatttatctaataattcttctgaaagctttaggaggagggcaaagttactcttcagagaatcagtcacaccattttcatacaattttttcctcatgtggttttcactcacactgccaccaccagattgataccttaataatgacttcagcatggtttcaaaagggtccgctgctcggaaaagaacatttaagaaggtgtatggtcaattccagcagttcagctacttttcaactttcactgtaaaaccaccaccttgctttgtagaacaggtgttttttgtttgtttgtttgtttgttttgagataagagtctggctctgtcgccaggctgcagtgcagtggtgcgatcttggctcactgcaagctccgcctcccaggttcaagcgattctcctgcctcagcctcctgagtagctgggattacaggcgcccgccaccacagccagctaatgtttgtatttttagtagagacggtgtgtcaccatgttggccaggatggtctcgatatcctgacctcgtgatccgcccgcctcagcctcccaaagtgtgtagaacaggttttaaagacggtcctcagtcatcaacacttttgttttcagaccctccctctctcgctgacggaggcaagtggagagaggaggaccggaggctcgcagaggcgtcagcggcagaggaaacctcgcacccgaacccgcagcgcggcgctctccccaaagaagcatttgcctggagcccctaagaggagcaagacctggacctcgagcactttggattccagtcaggatagatcgatggacagatggaaaagaggaatacacaagtgctgggagaatcctcaagaaaggagaaaggagtggcgcgcccaggagtctcgtcctgacacactgggaaatgaaatttgggtttggcgagttatggccaaaaagctgcccaaagtacttgagagccgccttggagagtggcgcggggtgcctggcaaggtgagaccggcctgcgggggcgcgggcttttcctcagcagctctacgcccgcctggcccggcgcctgaggggtagc

SEQ ID NO: 13080 - RNA, 8968 nt, Homo sapiens
  source 1..8968: mol_type = other RNA
gctgggattacaggcatgagccaccacacccagctggaaaatgtttaaaatttattaagtgaaaagtaactcatgctgcaatgaacgtactatgtaaaaatgtatgtatgtggaacagggaaaaatataaacagtcacagaaatgtgtttaggttggtagcattctttttcctcttaaaaattcctttttttggccgggcgctgtggctcacacctgtaatcccagcactttgggaagccgcggtggacagatcacaaggtcaggagatcaagaccatcctggctaacatggtgaaaccccgtctctactaaaaatacaaaaaattagctgggcatggaggcactcgcctgtagtcgcagctactcgggaggctgaggcaggagaatcgcttgaactggggagatggaggttgtagtgagcccagatcatgccactgcactcaagcctgggctgagacctccagagtctggctgagacctatggagtctcactctgtcacctaggctggagtacagtggtgcgatctcggcacactgcaacctccacctcccagacattctcctgcctcagcctctcaactagctgggattacattcgcccgcctccacacccactaatttttgtatttttagtagagatgcggtttccccatgttggccaggctgttcttgaactcctgacctcaagttatacgcccactttggactcccaaagtgctgggattacaggtgtgagccacggcaccagccaaaaatttctttaaatattagtggtatattattctctcaataagttttttttttttttttttttgagacagtcttgttttattgcctaagctggagtgcagtggcacaatctcaactcactgcaacctccacctcccaggtttattttttttctcatgcctcagcctcccaagaagctgggattacaggcatgtgccccaaaggccagttaagttttctttttctttttttcttttttcttggttgagacggattttcgctcgtcacccacactggagtgcaatggcgcgatctcggctcactgcaacctccgactcttgggttcaagcgattctcctgcctcagcctcccgagtagctgggattagaggcacctgtcaccacgcccgctacttttggtatttttagtagagatggagtttcaccacgttggccaggctgatctcaaactcctggcctcaagtgattcacctgccttggcctcccaaagtgctggaattacaggcccggcctatttttgcaataattatgaatagcacaccatttaaacctgttgattgagccctccttaaataactaaatacactactggccaacatggtgaaaacctgtctccactaaaaacacaaaaaaatggccgggcacagtggctcatgcctgtaatcccagcacttcaggaggccaaggggtgtgaatcacctgaggttaggagttcaagaccagcctggccaacatggtgaaaccctgtctctactaaaaaaaaatacaaaaattagctgagtgtagtggcacatacccgtagtctcagctactcaggaggctgaggcaggagaattgcttgaacctgggaggcaggggttgcagtgagccaagatcgtgccaccacactccagcctgggtgacacagcgagactccatctcaaaataaataaataaataaaaagaaagggaccgagcgcggtggctcatgcttgtaatcccagcactctgggaggctgagttgggcagatcacaaggtcaagagttcaggaccagcctgaccaacacggtaaaaccccatctctactaaaaatacaaaaatgagctgggtgtgatggcacgcgcctgtaaccccagttactcaaaaggctgaggcaagagaatcgcttgaacctgggaggcagaggttgcagtgagccgagatcacgccactgcattccagcctggtgacagtgagactctgtcacacacacacaaaaaagataaagaatgacaaaaatctgtgcctacattcagagtgacaagaatactaatgttctgcttgtagaaaagactattggttcagaatatgttaaatgcaaataatattttgtataatatatataaattacatatgcataaaaagagtatctatattagaatcttttgagacagggtcttgctctgtcaaccatgagggagtgcagtggcactaccacagctcactgtagccttgacttcctgagctcaagccatcctctcgcctcagcctcctgaatagttgggactgcaggtggtgccaccaaggctggctaagtttttatatttttttatagaaacaagcttttgccacgttgcccaggctggtctcaaacttctaaaagctcaagcaatctggccgccttgaactcccaaagtgcttgagttataggcatgagtcactgtgcccggcctacattagaatcttaacagtggggctgggcatggtgccccatgcctgtaatcccagcactttgggaggtcaaggtgggcagactacttgaggttgaggagttcgaggccagcctggccaacatggtgaaaccccatctgtactaaaaacacaaaaattagccaggtgtggtggcacatgtttgcaatcccagctacttgggaggctgaggcgggaggatcacttgaacctgggaagcagaggttgcagtgagccgagatggtgccatggcactccagcctgggcaatagacagcgggactcagtctcaaaacaaaaaaaaaaaaaaaaaaaaaagaatcttaacagtggttaacttcaaatagtgaaactatgactgttaactgagtttgacatttttgtgttttcctagatttttctacaataaacattattatttcataataaagcagtaaagactttttatacaaactattttaagataaacaaattttgacataggggttataagttaggtagaatctatttatataaaaaatggaactgtacttttgtgggccaaataagcactatgtaagtttttttaattttcccaaacacatgcacagaattaatattgccttaaattttgttagcacaagtttgagagagctctttagttcataaaaaaatgttttatggaccaggtgccgtggctcacacctgcaatctcaacactttgggaggcccaggtgggaggatcgcttgagcctaggagtttgagacaagactgggcgacgcagggagaccctgtctcaaaaaaacaaaaccaaaaacaagcaaacaaaaaaacagctgggcatggtggcatgcatatgtagtcccagctattctagaggctgaggtgagatcgctggagcccaggaggtggaggctacagtaagctgtgatcatgccaatgcactccagcttggtcaacaaagcaagactgtgcctcaaaaaaaaaaaagaaaagaaaagaaagaaagaaaagaaaaagaaaaaaagttatgtacgtatggtttttttttttttttggatagagtttcactcttcttgcccaggctggagtgcaatggtgcaatcttggctcaccacaaccttcccctactgggttcaagcgattctcctgtttcagcctccccagtagctgggattaaaggcatgtgccaccacgcccggctaattttgtatttttagtagagatgaagtttctccatgttggtcaggctggtcttgaactcctgacttcaggtgatctgcccgcctcagcctcccaaagtgctgggattacaggtgtgagccacctcgcctggccgttttttttttttttttttttttctgagacggagttttgctcttattgcccaggctggagtgcaatggcacgatctcggctcatcgcaacctctgcctcacgggttcaagcaattttcctgcctcagcgtctcaagtagctaggattacagggatgctccatcatgcccggctaattttgtatttttggtagagacagggtttctccatgttggtcaggctggtctcaaactcccaacctcaggtgatttacccgccttggcctcccaaagagctgggattacaggtgtgagccactgtgcccggccatgcttatgttttttaacaatacacttctgaactatcaaaaagaatataaatcaaaatcactgaagtagtttttaaaaactccaaaagctacaaaacttacttacttcaatatcaattaaaaacccatttgatagttcaataacttgagtcctgctagaatcattctataagccatcagtgacagtgaagtggccaaaatttgagtcacttgataagtacaaagaacacagatttttgtcattcttactgtgaagaaaaacagtgaatgaataacttagtttatatattaacagtacttttatttaaaaaattatctagagaataacttctttttaatcatttgttagtcatgtaactatggataaaacatactaatttagctgattcctctatgctctcttttccttgattccaatcattattagttattctacactgcctcatttattggcagttatgccaactggctgactctggttcaactgccctatttttgctttcatcattgtttatcatatctcacttgctttaaactccacctctttcatctcatctgatctgacacttggtttacatatcaattggctactctaaccttctaccgccagtttccaacccattcgaggtacttgggtaacaaaggaagatgctctatacacacaaaaccacagaaaataagtgggaagggataataaatttcacttaaagttttagaatttttcttttttttttgagacggagtttcactcttgttgcccaggctggagtgcaatggcgcgatcttggctcaccgcaacctctgcctcccaggttcaagcagttctcctgcttcagcctcccgagtagctggtattacaggcatgcaccaccaagcctggctaattttgtatttttagtagagacggggtttctccatgttggtcaggctggtcttgaacgcctgacctcaggtgatctgcctgcctcggcctcccaaagtgctgggattacaggcatgagccatcacgcccggccaaagttttagaatttaagttattccaaaaaaaattttttttttcaaaaatacagactgcatccaattaaattctatgttaactggtaatgactaggtctaaaatgttaggtatttaccaataaatgacataaaataactcaacaacaaagggatttttttttttaagagatagggtctcactttatcactcaggtttggctgagggcagtggtgtgatcacagctcactgaagcctccaactcctgggctcaagtgatcctcccgcctcagtctaccagagtatattcttgaaagtaaaattacaaatgaaattcagcagtgttaaaaataagcccacttgcagacaattatcatttttcttcctttctttcctcactatctgtacttggcatatttcctacagtggctgtcttaaagaaaaaaaggaatccttcacaaatagtgtagccaaaaaagttggactaatatacaatgctatcagtaaagtattatatataaaatttataagtgctaaagtgtaattttgaaagacacttaagatactccttttttttttgagacaaggtctcagccctgtcgcccaggctggagtgcactagcacaacatcagctcactgcaacctccgcctcccaggttcaagcgattctcctgcctcagcctcccaagtagctgagactacaggcgcacgccagcatgtccagataattttttgtatttttagtagagatggggtttcaccatgttggccaggatggtctcaaatctcttgacctcgtgatctgcccatgtcggcttcccaaagtgttaggataacaggcatgagctaccgtgcccagcctacttaaaatattcttgaaatagctctccccacctccttttttttttttttttgagaatgagtttcactcgacacccaggctggagtgcagtggtgcgatcttggctcactgcaacctctgcctcccaggttcaagcgattatcctgcctcagcctcctgagtagctgggattacaaatgtgcaccaccacatctggctaattttttttttttttttttgtatttttagtagagacggggtttcaccaagttggcctggctggtctcgaacacctgacctcaattgatccacctgcctcggcctcccaaagtattataggcatgagccaccgagcccggccttttttgttttttgtttttttaaaggcagggttttgctctgttgcccaggctggagtgcagtggtgtgatcacagatcactgcagccttgacctctcctggtctcaagtgatcctcccacctcagccttcagaacagctgggactacaggtgtgtgtcaccatgcccagtaatttttttgtatatttgtagaggcagggtctcccaatgttgcctgggctggtctcaaactcctgggctcaagcaatccaccagctttggccttccaaagttctaggattatacgcatgagccactgtgccctgccccaatattttgttacttactagtgagactaaacacttttctaaaagtttgttagccatactatcctataaaagctgtttgttcatgtcttttgtccatttatctttttttttgtttttcttgagacagagtcttgctctgtggcccaggctggagtgcaggggtgcaatctcggctcactgcaagctccgcctcccaggttcaaatgattctcctgcctcagcctcctgagtagctgggattacaggcatgtgccaccatgcccagctaatttttttgtgtgtgtttttcagtagagatggggtttcaccatgttggccaggctgatctcgaattcctgacctcaggtgctccacccgcctcagcctcccaaagtactgggattacaggggtgagccaccgcacccggccaattttctgtatttttaatagagacagggtttcatcctgttggccaggctggcctcgaacttcggacctcaggtgatccacccgcctcgacctcccaaagtgctgggattacaggtgtgggccaccacacccagccaatttttttgtatttttagtagagacagggtttcatcatgttggccaggctggtcgcaaactcctgacctcaggtgatccacccgcctcagcatcccaaagtgctgggattacaggcatgagccaccactcccggccaatgttttgtatttttagtagagatggggtttcatcatgttggccagactggtctcaaactctggacctcaggtgatccacctgcctcagcctcccaaagtgtagggattacaggtgtgagccaccgcgcccagcctatgtttctattttatacatattcaacaaacatgattccccaacttctgcaaaataatttctttttcaagaacattgattttagagctcacactaagaaaaagaatacaaaaataatggcatagaaagtgaaaaaacaaaaataaaaagtagaaagctaaagtttcccattaaaatgatcaatatactgtgcagtaagtcaaatgtgtacaatgaattaagaaaatatgatatataaaaatccaaatttacaaaattaagtacaaataggtgtttatattacaaagtgatactggtttataaaaggattcaacatagattttttttaaatggttgttttcctcaatcaatttaacaatgattttaaatgtataaaattttaatatctctttgagacagtgatccaagcttcttcccttgatgatgttaccagttcatactttgtttcaataacctgtccctccacagaaagtaggtgcagtctcttcaccaatacactaagaagtactgtggtcaccatatatgcaaacctcaactctggacactcctgtgtgcctgagaatccaagtgaggaaaaagttttcattactaattcatcatcaaaccgatctggatcaaacttgtgtggagatggccaagtattaggatcctgaagtaccacaccaagggcataaaggacgagggtctctctaggaataataaatcggtcaatttttccttcaatatcttgaagctgggcagaaactggagtcagtttggcagttcgaacagtttcacaaagcacatgctgacaatatctgagctgctcaattttctctggagtaacaggaccatttccaaaaacttggtttatctcttcatataattttttttgaacttcttcagaggtggttaaaaaacagattgcccaggtacacaattttgcagttattatgcaactggccagagaaaatatcatactgtcttctaggatctgttggtcattaaggttcccttgtactaaggagtcaatgaaaatatgttgactgaagttccttccttttcgttcttttatgatgttccttaaaacagactccagttgcatgagggtgtgccatgattcttctggaagcgaatgacttcctgatcatcttcaaatgtactacccattaccatctgtgtaacagacttcatagcaaaaccaagcatatgctggctgaggggcacgtgctgggtctctgggtaggagagccatttatctaataattcttctgaaagctttaggaggagggcaaagttactcttcagagaatcagtcacaccattttcatacaattttttcctcatgtggttttcactcacactgccaccaccagattgataccttaataatgacttcagcatggtttcaaaagggtccgttttcttcagttggagtaatccctggaattcctgcagcttgtctggaagccggatagaggtagagcacggctcccaccaacgccagcaagaaggtaacggcgaagatcgcgaagtccaacatggttctgccgcccagggagccacgtctcggatcggccgctccagc

SEQ ID NO: 13081 - RNA, 8802 nt, Homo sapiens
  source 1..8802: mol_type = other RNA
gctgggattacaggcatgagccaccacacccagctggaaaatgtttaaaatttattaagtgaaaagtaactcatgctgcaatgaacgtactatgtaaaaatgtatgtatgtggaacagggaaaaatataaacagtcacagaaatgtgtttaggttggtagcattctttttcctcttaaaaattcctttttttggccgggcgctgtggctcacacctgtaatcccagcactttgggaagccgcggtggacagatcacaaggtcaggagatcaagaccatcctggctaacatggtgaaaccccgtctctactaaaaatacaaaaaattagctgggcatggaggcactcgcctgtagtcgcagctactcgggaggctgaggcaggagaatcgcttgaactggggagatggaggttgtagtgagcccagatcatgccactgcactcaagcctgggctgagacctccagagtctggctgagacctatggagtctcactctgtcacctaggctggagtacagtggtgcgatctcggcacactgcaacctccacctcccagacattctcctgcctcagcctctcaactagctgggattacattcgcccgcctccacacccactaatttttgtatttttagtagagatgcggtttccccatgttggccaggctgttcttgaactcctgacctcaagttatacgcccactttggactcccaaagtgctgggattacaggtgtgagccacggcaccagccaaaaatttctttaaatattagtggtatattattctctcaataagttttttttttttttttttttgagacagtcttgttttattgcctaagctggagtgcagtggcacaatctcaactcactgcaacctccacctcccaggtttattttttttctcatgcctcagcctcccaagaagctgggattacaggcatgtgccccaaaggccagttaagttttctttttctttttttcttttttcttggttgagacggattttcgctcgtcacccacactggagtgcaatggcgcgatctcggctcactgcaacctccgactcttgggttcaagcgattctcctgcctcagcctcccgagtagctgggattagaggcacctgtcaccacgcccgctacttttggtatttttagtagagatggagtttcaccacgttggccaggctgatctcaaactcctggcctcaagtgattcacctgccttggcctcccaaagtgctggaattacaggcccggcctatttttgcaataattatgaatagcacaccatttaaacctgttgattgagccctccttaaataactaaatacactactggccaacatggtgaaaacctgtctccactaaaaacacaaaaaaatggccgggcacagtggctcatgcctgtaatcccagcacttcaggaggccaaggggtgtgaatcacctgaggttaggagttcaagaccagcctggccaacatggtgaaaccctgtctctactaaaaaaaaatacaaaaattagctgagtgtagtggcacatacccgtagtctcagctactcaggaggctgaggcaggagaattgcttgaacctgggaggcaggggttgcagtgagccaagatcgtgccaccacactccagcctgggtgacacagcgagactccatctcaaaataaataaataaataaaaagaaagggaccgagcgcggtggctcatgcttgtaatcccagcactctgggaggctgagttgggcagatcacaaggtcaagagttcaggaccagcctgaccaacacggtaaaaccccatctctactaaaaatacaaaaatgagctgggtgtgatggcacgcgcctgtaaccccagttactcaaaaggctgaggcaagagaatcgcttgaacctgggaggcagaggttgcagtgagccgagatcacgccactgcattccagcctggtgacagtgagactctgtcacacacacacaaaaaagataaagaatgacaaaaatctgtgcctacattcagagtgacaagaatactaatgttctgcttgtagaaaagactattggttcagaatatgttaaatgcaaataatattttgtataatatatataaattacatatgcataaaaagagtatctatattagaatcttttgagacagggtcttgctctgtcaaccatgagggagtgcagtggcactaccacagctcactgtagccttgacttcctgagctcaagccatcctctcgcctcagcctcctgaatagttgggactgcaggtggtgccaccaaggctggctaagtttttatatttttttatagaaacaagcttttgccacgttgcccaggctggtctcaaacttctaaaagctcaagcaatctggccgccttgaactcccaaagtgcttgagttataggcatgagtcactgtgcccggcctacattagaatcttaacagtggggctgggcatggtgccccatgcctgtaatcccagcactttgggaggtcaaggtgggcagactacttgaggttgaggagttcgaggccagcctggccaacatggtgaaaccccatctgtactaaaaacacaaaaattagccaggtgtggtggcacatgtttgcaatcccagctacttgggaggctgaggcgggaggatcacttgaacctgggaagcagaggttgcagtgagccgagatggtgccatggcactccagcctgggcaatagacagcgggactcagtctcaaaacaaaaaaaaaaaaaaaaaaaaaagaatcttaacagtggttaacttcaaatagtgaaactatgactgttaactgagtttgacatttttgtgttttcctagatttttctacaataaacattattatttcataataaagcagtaaagactttttatacaaactattttaagataaacaaattttgacataggggttataagttaggtagaatctatttatataaaaaatggaactgtacttttgtgggccaaataagcactatgtaagtttttttaattttcccaaacacatgcacagaattaatattgccttaaattttgttagcacaagtttgagagagctctttagttcataaaaaaatgttttatggaccaggtgccgtggctcacacctgcaatctcaacactttgggaggcccaggtgggaggatcgcttgagcctaggagtttgagacaagactgggcgacgcagggagaccctgtctcaaaaaaacaaaaccaaaaacaagcaaacaaaaaaacagctgggcatggtggcatgcatatgtagtcccagctattctagaggctgaggtgagatcgctggagcccaggaggtggaggctacagtaagctgtgatcatgccaatgcactccagcttggtcaacaaagcaagactgtgcctcaaaaaaaaaaaagaaaagaaaagaaagaaagaaaagaaaaagaaaaaaagttatgtacgtatggtttttttttttttttggatagagtttcactcttcttgcccaggctggagtgcaatggtgcaatcttggctcaccacaaccttcccctactgggttcaagcgattctcctgtttcagcctccccagtagctgggattaaaggcatgtgccaccacgcccggctaattttgtatttttagtagagatgaagtttctccatgttggtcaggctggtcttgaactcctgacttcaggtgatctgcccgcctcagcctcccaaagtgctgggattacaggtgtgagccacctcgcctggccgttttttttttttttttttttttctgagacggagttttgctcttattgcccaggctggagtgcaatggcacgatctcggctcatcgcaacctctgcctcacgggttcaagcaattttcctgcctcagcgtctcaagtagctaggattacagggatgctccatcatgcccggctaattttgtatttttggtagagacagggtttctccatgttggtcaggctggtctcaaactcccaacctcaggtgatttacccgccttggcctcccaaagagctgggattacaggtgtgagccactgtgcccggccatgcttatgttttttaacaatacacttctgaactatcaaaaagaatataaatcaaaatcactgaagtagtttttaaaaactccaaaagctacaaaacttacttacttcaatatcaattaaaaacccatttgatagttcaataacttgagtcctgctagaatcattctataagccatcagtgacagtgaagtggccaaaatttgagtcacttgataagtacaaagaacacagatttttgtcattcttactgtgaagaaaaacagtgaatgaataacttagtttatatattaacagtacttttatttaaaaaattatctagagaataacttctttttaatcatttgttagtcatgtaactatggataaaacatactaatttagctgattcctctatgctctcttttccttgattccaatcattattagttattctacactgcctcatttattggcagttatgccaactggctgactctggttcaactgccctatttttgctttcatcattgtttatcatatctcacttgctttaaactccacctctttcatctcatctgatctgacacttggtttacatatcaattggctactctaaccttctaccgccagtttccaacccattcgaggtacttgggtaacaaaggaagatgctctatacacacaaaaccacagaaaataagtgggaagggataataaatttcacttaaagttttagaatttttcttttttttttgagacggagtttcactcttgttgcccaggctggagtgcaatggcgcgatcttggctcaccgcaacctctgcctcccaggttcaagcagttctcctgcttcagcctcccgagtagctggtattacaggcatgcaccaccaagcctggctaattttgtatttttagtagagacggggtttctccatgttggtcaggctggtcttgaacgcctgacctcaggtgatctgcctgcctcggcctcccaaagtgctgggattacaggcatgagccatcacgcccggccaaagttttagaatttaagttattccaaaaaaaattttttttttcaaaaatacagactgcatccaattaaattctatgttaactggtaatgactaggtctaaaatgttaggtatttaccaataaatgacataaaataactcaacaacaaagggatttttttttttaagagatagggtctcactttatcactcaggtttggctgagggcagtggtgtgatcacagctcactgaagcctccaactcctgggctcaagtgatcctcccgcctcagtctaccagagtatattcttgaaagtaaaattacaaatgaaattcagcagtgttaaaaataagcccacttgcagacaattatcatttttcttcctttctttcctcactatctgtacttggcatatttcctacagtggctgtcttaaagaaaaaaaggaatccttcacaaatagtgtagccaaaaaagttggactaatatacaatgctatcagtaaagtattatatataaaatttataagtgctaaagtgtaattttgaaagacacttaagatactccttttttttttgagacaaggtctcagccctgtcgcccaggctggagtgcactagcacaacatcagctcactgcaacctccgcctcccaggttcaagcgattctcctgcctcagcctcccaagtagctgagactacaggcgcacgccagcatgtccagataattttttgtatttttagtagagatggggtttcaccatgttggccaggatggtctcaaatctcttgacctcgtgatctgcccatgtcggcttcccaaagtgttaggataacaggcatgagctaccgtgcccagcctacttaaaatattcttgaaatagctctccccacctccttttttttttttttttgagaatgagtttcactcgacacccaggctggagtgcagtggtgcgatcttggctcactgcaacctctgcctcccaggttcaagcgattatcctgcctcagcctcctgagtagctgggattacaaatgtgcaccaccacatctggctaattttttttttttttttttgtatttttagtagagacggggtttcaccaagttggcctggctggtctcgaacacctgacctcaattgatccacctgcctcggcctcccaaagtattataggcatgagccaccgagcccggccttttttgttttttgtttttttaaaggcagggttttgctctgttgcccaggctggagtgcagtggtgtgatcacagatcactgcagccttgacctctcctggtctcaagtgatcctcccacctcagccttcagaacagctgggactacaggtgtgtgtcaccatgcccagtaatttttttgtatatttgtagaggcagggtctcccaatgttgcctgggctggtctcaaactcctgggctcaagcaatccaccagctttggccttccaaagttctaggattatacgcatgagccactgtgccctgccccaatattttgttacttactagtgagactaaacacttttctaaaagtttgttagccatactatcctataaaagctgtttgttcatgtcttttgtccatttatctttttttttgtttttcttgagacagagtcttgctctgtggcccaggctggagtgcaggggtgcaatctcggctcactgcaagctccgcctcccaggttcaaatgattctcctgcctcagcctcctgagtagctgggattacaggcatgtgccaccatgcccagctaatttttttgtgtgtgtttttcagtagagatggggtttcaccatgttggccaggctgatctcgaattcctgacctcaggtgctccacccgcctcagcctcccaaagtactgggattacaggggtgagccaccgcacccggccaattttctgtatttttaatagagacagggtttcatcctgttggccaggctggcctcgaacttcggacctcaggtgatccacccgcctcgacctcccaaagtgctgggattacaggtgtgggccaccacacccagccaatttttttgtatttttagtagagacagggtttcatcatgttggccaggctggtcgcaaactcctgacctcaggtgatccacccgcctcagcatcccaaagtgctgggattacaggcatgagccaccactcccggccaatgttttgtatttttagtagagatggggtttcatcatgttggccagactggtctcaaactctggacctcaggtgatccacctgcctcagcctcccaaagtgtagggattacaggtgtgagccaccgcgcccagcctatgtttctattttatacatattcaacaaacatgattccccaacttctgcaaaataatttctttttcaagaacattgattttagagctcacactaagaaaaagaatacaaaaataatggcatagaaagtgaaaaaacaaaaataaaaagtagaaagctaaagtttcccattaaaatgatcaatatactgtgcagtaagtcaaatgtgtacaatgaattaagaaaatatgatatataaaaatccaaatttacaaaattaagtacaaataggtgtttatattacaaagtgatactggtttataaaaggattcaacatagattttttttaaatggttgttttcctcaatcaatttaacaatgattttaaatgtataaaattttaatatctctttgagacagtgatccaagcttcttcccttgatgatgttaccagttcatactttgtttcaataacctgtccctccacagaaagtaggtgcagtctcttcaccaatacactaagaagtactgtggtcaccatatatgcaaacctcaactctggacactcctgtgtgcctgagaatccaagtgaggaaaaagttttcattactaattcatcatcaaaccgatctggatcaaacttgtgtggagatggccaagtattaggatcctgaagtaccacaccaagggcataaaggacgagggtctctctaggaataataaatcggtcaatttttccttcaatatcttgaagctgggcagaaactggagtcagtttggcagttcgaacagtttcacaaagcacatgctgacaatatctgagctgctcaattttctctggagtaacaggaccatttccaaaaacttggtttatctcttcatataattttttttgaacttcttcagaggtggttaaaaaacagattgcccaggtacacaattttgcagttattatgcaactggccagagaaaatatcatactgtcttctaggattgtgccatgattcttctggaagcgaatgacttcctgatcatcttcaaatgtactacccattaccatctgtgtaacagacttcatagcaaaaccaagcatatgctggctgaggggcacgtgctgggtctctgggtaggagagccatttatctaataattcttctgaaagctttaggaggagggcaaagttactcttcagagaatcagtcacaccattttcatacaattttttcctcatgtggttttcactcacactgccaccaccagattgataccttaataatgacttcagcatggtttcaaaagggtccgcggatagaggtagagcacggctcccaccaacgccagcaagaaggtaacggcgaagatcgcgaagtccaacatggttctgccgcccagggagccacgtctcggatcggccgctccagc

SEQ ID NO: 13082 - RNA, 8852 nt, Homo sapiens
  source 1..8852: mol_type = other RNA
gctgggattacaggcatgagccaccacacccagctggaaaatgtttaaaatttattaagtgaaaagtaactcatgctgcaatgaacgtactatgtaaaaatgtatgtatgtggaacagggaaaaatataaacagtcacagaaatgtgtttaggttggtagcattctttttcctcttaaaaattcctttttttggccgggcgctgtggctcacacctgtaatcccagcactttgggaagccgcggtggacagatcacaaggtcaggagatcaagaccatcctggctaacatggtgaaaccccgtctctactaaaaatacaaaaaattagctgggcatggaggcactcgcctgtagtcgcagctactcgggaggctgaggcaggagaatcgcttgaactggggagatggaggttgtagtgagcccagatcatgccactgcactcaagcctgggctgagacctccagagtctggctgagacctatggagtctcactctgtcacctaggctggagtacagtggtgcgatctcggcacactgcaacctccacctcccagacattctcctgcctcagcctctcaactagctgggattacattcgcccgcctccacacccactaatttttgtatttttagtagagatgcggtttccccatgttggccaggctgttcttgaactcctgacctcaagttatacgcccactttggactcccaaagtgctgggattacaggtgtgagccacggcaccagccaaaaatttctttaaatattagtggtatattattctctcaataagttttttttttttttttttttgagacagtcttgttttattgcctaagctggagtgcagtggcacaatctcaactcactgcaacctccacctcccaggtttattttttttctcatgcctcagcctcccaagaagctgggattacaggcatgtgccccaaaggccagttaagttttctttttctttttttcttttttcttggttgagacggattttcgctcgtcacccacactggagtgcaatggcgcgatctcggctcactgcaacctccgactcttgggttcaagcgattctcctgcctcagcctcccgagtagctgggattagaggcacctgtcaccacgcccgctacttttggtatttttagtagagatggagtttcaccacgttggccaggctgatctcaaactcctggcctcaagtgattcacctgccttggcctcccaaagtgctggaattacaggcccggcctatttttgcaataattatgaatagcacaccatttaaacctgttgattgagccctccttaaataactaaatacactactggccaacatggtgaaaacctgtctccactaaaaacacaaaaaaatggccgggcacagtggctcatgcctgtaatcccagcacttcaggaggccaaggggtgtgaatcacctgaggttaggagttcaagaccagcctggccaacatggtgaaaccctgtctctactaaaaaaaaatacaaaaattagctgagtgtagtggcacatacccgtagtctcagctactcaggaggctgaggcaggagaattgcttgaacctgggaggcaggggttgcagtgagccaagatcgtgccaccacactccagcctgggtgacacagcgagactccatctcaaaataaataaataaataaaaagaaagggaccgagcgcggtggctcatgcttgtaatcccagcactctgggaggctgagttgggcagatcacaaggtcaagagttcaggaccagcctgaccaacacggtaaaaccccatctctactaaaaatacaaaaatgagctgggtgtgatggcacgcgcctgtaaccccagttactcaaaaggctgaggcaagagaatcgcttgaacctgggaggcagaggttgcagtgagccgagatcacgccactgcattccagcctggtgacagtgagactctgtcacacacacacaaaaaagataaagaatgacaaaaatctgtgcctacattcagagtgacaagaatactaatgttctgcttgtagaaaagactattggttcagaatatgttaaatgcaaataatattttgtataatatatataaattacatatgcataaaaagagtatctatattagaatcttttgagacagggtcttgctctgtcaaccatgagggagtgcagtggcactaccacagctcactgtagccttgacttcctgagctcaagccatcctctcgcctcagcctcctgaatagttgggactgcaggtggtgccaccaaggctggctaagtttttatatttttttatagaaacaagcttttgccacgttgcccaggctggtctcaaacttctaaaagctcaagcaatctggccgccttgaactcccaaagtgcttgagttataggcatgagtcactgtgcccggcctacattagaatcttaacagtggggctgggcatggtgccccatgcctgtaatcccagcactttgggaggtcaaggtgggcagactacttgaggttgaggagttcgaggccagcctggccaacatggtgaaaccccatctgtactaaaaacacaaaaattagccaggtgtggtggcacatgtttgcaatcccagctacttgggaggctgaggcgggaggatcacttgaacctgggaagcagaggttgcagtgagccgagatggtgccatggcactccagcctgggcaatagacagcgggactcagtctcaaaacaaaaaaaaaaaaaaaaaaaaaagaatcttaacagtggttaacttcaaatagtgaaactatgactgttaactgagtttgacatttttgtgttttcctagatttttctacaataaacattattatttcataataaagcagtaaagactttttatacaaactattttaagataaacaaattttgacataggggttataagttaggtagaatctatttatataaaaaatggaactgtacttttgtgggccaaataagcactatgtaagtttttttaattttcccaaacacatgcacagaattaatattgccttaaattttgttagcacaagtttgagagagctctttagttcataaaaaaatgttttatggaccaggtgccgtggctcacacctgcaatctcaacactttgggaggcccaggtgggaggatcgcttgagcctaggagtttgagacaagactgggcgacgcagggagaccctgtctcaaaaaaacaaaaccaaaaacaagcaaacaaaaaaacagctgggcatggtggcatgcatatgtagtcccagctattctagaggctgaggtgagatcgctggagcccaggaggtggaggctacagtaagctgtgatcatgccaatgcactccagcttggtcaacaaagcaagactgtgcctcaaaaaaaaaaaagaaaagaaaagaaagaaagaaaagaaaaagaaaaaaagttatgtacgtatggtttttttttttttttggatagagtttcactcttcttgcccaggctggagtgcaatggtgcaatcttggctcaccacaaccttcccctactgggttcaagcgattctcctgtttcagcctccccagtagctgggattaaaggcatgtgccaccacgcccggctaattttgtatttttagtagagatgaagtttctccatgttggtcaggctggtcttgaactcctgacttcaggtgatctgcccgcctcagcctcccaaagtgctgggattacaggtgtgagccacctcgcctggccgttttttttttttttttttttttctgagacggagttttgctcttattgcccaggctggagtgcaatggcacgatctcggctcatcgcaacctctgcctcacgggttcaagcaattttcctgcctcagcgtctcaagtagctaggattacagggatgctccatcatgcccggctaattttgtatttttggtagagacagggtttctccatgttggtcaggctggtctcaaactcccaacctcaggtgatttacccgccttggcctcccaaagagctgggattacaggtgtgagccactgtgcccggccatgcttatgttttttaacaatacacttctgaactatcaaaaagaatataaatcaaaatcactgaagtagtttttaaaaactccaaaagctacaaaacttacttacttcaatatcaattaaaaacccatttgatagttcaataacttgagtcctgctagaatcattctataagccatcagtgacagtgaagtggccaaaatttgagtcacttgataagtacaaagaacacagatttttgtcattcttactgtgaagaaaaacagtgaatgaataacttagtttatatattaacagtacttttatttaaaaaattatctagagaataacttctttttaatcatttgttagtcatgtaactatggataaaacatactaatttagctgattcctctatgctctcttttccttgattccaatcattattagttattctacactgcctcatttattggcagttatgccaactggctgactctggttcaactgccctatttttgctttcatcattgtttatcatatctcacttgctttaaactccacctctttcatctcatctgatctgacacttggtttacatatcaattggctactctaaccttctaccgccagtttccaacccattcgaggtacttgggtaacaaaggaagatgctctatacacacaaaaccacagaaaataagtgggaagggataataaatttcacttaaagttttagaatttttcttttttttttgagacggagtttcactcttgttgcccaggctggagtgcaatggcgcgatcttggctcaccgcaacctctgcctcccaggttcaagcagttctcctgcttcagcctcccgagtagctggtattacaggcatgcaccaccaagcctggctaattttgtatttttagtagagacggggtttctccatgttggtcaggctggtcttgaacgcctgacctcaggtgatctgcctgcctcggcctcccaaagtgctgggattacaggcatgagccatcacgcccggccaaagttttagaatttaagttattccaaaaaaaattttttttttcaaaaatacagactgcatccaattaaattctatgttaactggtaatgactaggtctaaaatgttaggtatttaccaataaatgacataaaataactcaacaacaaagggatttttttttttaagagatagggtctcactttatcactcaggtttggctgagggcagtggtgtgatcacagctcactgaagcctccaactcctgggctcaagtgatcctcccgcctcagtctaccagagtatattcttgaaagtaaaattacaaatgaaattcagcagtgttaaaaataagcccacttgcagacaattatcatttttcttcctttctttcctcactatctgtacttggcatatttcctacagtggctgtcttaaagaaaaaaaggaatccttcacaaatagtgtagccaaaaaagttggactaatatacaatgctatcagtaaagtattatatataaaatttataagtgctaaagtgtaattttgaaagacacttaagatactccttttttttttgagacaaggtctcagccctgtcgcccaggctggagtgcactagcacaacatcagctcactgcaacctccgcctcccaggttcaagcgattctcctgcctcagcctcccaagtagctgagactacaggcgcacgccagcatgtccagataattttttgtatttttagtagagatggggtttcaccatgttggccaggatggtctcaaatctcttgacctcgtgatctgcccatgtcggcttcccaaagtgttaggataacaggcatgagctaccgtgcccagcctacttaaaatattcttgaaatagctctccccacctccttttttttttttttttgagaatgagtttcactcgacacccaggctggagtgcagtggtgcgatcttggctcactgcaacctctgcctcccaggttcaagcgattatcctgcctcagcctcctgagtagctgggattacaaatgtgcaccaccacatctggctaattttttttttttttttttgtatttttagtagagacggggtttcaccaagttggcctggctggtctcgaacacctgacctcaattgatccacctgcctcggcctcccaaagtattataggcatgagccaccgagcccggccttttttgttttttgtttttttaaaggcagggttttgctctgttgcccaggctggagtgcagtggtgtgatcacagatcactgcagccttgacctctcctggtctcaagtgatcctcccacctcagccttcagaacagctgggactacaggtgtgtgtcaccatgcccagtaatttttttgtatatttgtagaggcagggtctcccaatgttgcctgggctggtctcaaactcctgggctcaagcaatccaccagctttggccttccaaagttctaggattatacgcatgagccactgtgccctgccccaatattttgttacttactagtgagactaaacacttttctaaaagtttgttagccatactatcctataaaagctgtttgttcatgtcttttgtccatttatctttttttttgtttttcttgagacagagtcttgctctgtggcccaggctggagtgcaggggtgcaatctcggctcactgcaagctccgcctcccaggttcaaatgattctcctgcctcagcctcctgagtagctgggattacaggcatgtgccaccatgcccagctaatttttttgtgtgtgtttttcagtagagatggggtttcaccatgttggccaggctgatctcgaattcctgacctcaggtgctccacccgcctcagcctcccaaagtactgggattacaggggtgagccaccgcacccggccaattttctgtatttttaatagagacagggtttcatcctgttggccaggctggcctcgaacttcggacctcaggtgatccacccgcctcgacctcccaaagtgctgggattacaggtgtgggccaccacacccagccaatttttttgtatttttagtagagacagggtttcatcatgttggccaggctggtcgcaaactcctgacctcaggtgatccacccgcctcagcatcccaaagtgctgggattacaggcatgagccaccactcccggccaatgttttgtatttttagtagagatggggtttcatcatgttggccagactggtctcaaactctggacctcaggtgatccacctgcctcagcctcccaaagtgtagggattacaggtgtgagccaccgcgcccagcctatgtttctattttatacatattcaacaaacatgattccccaacttctgcaaaataatttctttttcaagaacattgattttagagctcacactaagaaaaagaatacaaaaataatggcatagaaagtgaaaaaacaaaaataaaaagtagaaagctaaagtttcccattaaaatgatcaatatactgtgcagtaagtcaaatgtgtacaatgaattaagaaaatatgatatataaaaatccaaatttacaaaattaagtacaaataggtgtttatattacaaagtgatactggtttataaaaggattcaacatagattttttttaaatggttgttttcctcaatcaatttaacaatgattttaaatgtataaaattttaatatctctttgagacagtgatccaagcttcttcccttgatgatgttaccagttcatactttgtttcaataacctgtccctccacagaaagtaggtgcagtctcttcaccaatacactaagaagtactgtggtcaccatatatgcaaacctcaactctggacactcctgtgtgcctgagaatccaagtgaggaaaaagttttcattactaattcatcatcaaaccgatctggatcaaacttgtgtggagatggccaagtattaggatcctgaagtaccacaccaagggcataaaggacgagggtctctctaggaataataaatcggtcaatttttccttcaatatcttgaagctgggcagaaactggagtcagtttggcagttcgaacagtttcacaaagcacatgctgacaatatctgagctgctcaattttctctggagtaacaggaccatttccaaaaacttggtttatctcttcatataattttttttgaacttcttcagaggtggttaaaaaacagattgcccaggtacacaattttgcagttattatgcaactggccagagaaaatatcatactgtcttctaggattgtgccatgattcttctggaagcgaatgacttcctgatcatcttcaaatgtactacccattaccatctgtgtaacagacttcatagcaaaaccaagcatatgctggctgaggggcacgtgctgggtctctgggtaggagagccatttatctaataattcttctgaaagctttaggaggagggcaaagttactcttcagagaatcagtcacaccattttcatacaattttttcctcatgtggttttcactcacactgccaccaccagattgataccttaataatgacttcagcatggtttcaaaagggtccgttttcttcagttggagtaatccctggaattcctgcagcttgtctggaagccggatagaggtagagcacggctcccaccaacgccagcaagaaggtaacggcgaagatcgcgaagtccaacatggttctgccgcccagggagccacgtctcggatcggccgctccagc

SEQ ID NO: 13083 - RNA, 9102 nt, Homo sapiens
  source 1..9102: mol_type = other RNA
gctgggattacaggcatgagccaccacacccagctggaaaatgtttaaaatttattaagtgaaaagtaactcatgctgcaatgaacgtactatgtaaaaatgtatgtatgtggaacagggaaaaatataaacagtcacagaaatgtgtttaggttggtagcattctttttcctcttaaaaattcctttttttggccgggcgctgtggctcacacctgtaatcccagcactttgggaagccgcggtggacagatcacaaggtcaggagatcaagaccatcctggctaacatggtgaaaccccgtctctactaaaaatacaaaaaattagctgggcatggaggcactcgcctgtagtcgcagctactcgggaggctgaggcaggagaatcgcttgaactggggagatggaggttgtagtgagcccagatcatgccactgcactcaagcctgggctgagacctccagagtctggctgagacctatggagtctcactctgtcacctaggctggagtacagtggtgcgatctcggcacactgcaacctccacctcccagacattctcctgcctcagcctctcaactagctgggattacattcgcccgcctccacacccactaatttttgtatttttagtagagatgcggtttccccatgttggccaggctgttcttgaactcctgacctcaagttatacgcccactttggactcccaaagtgctgggattacaggtgtgagccacggcaccagccaaaaatttctttaaatattagtggtatattattctctcaataagttttttttttttttttttttgagacagtcttgttttattgcctaagctggagtgcagtggcacaatctcaactcactgcaacctccacctcccaggtttattttttttctcatgcctcagcctcccaagaagctgggattacaggcatgtgccccaaaggccagttaagttttctttttctttttttcttttttcttggttgagacggattttcgctcgtcacccacactggagtgcaatggcgcgatctcggctcactgcaacctccgactcttgggttcaagcgattctcctgcctcagcctcccgagtagctgggattagaggcacctgtcaccacgcccgctacttttggtatttttagtagagatggagtttcaccacgttggccaggctgatctcaaactcctggcctcaagtgattcacctgccttggcctcccaaagtgctggaattacaggcccggcctatttttgcaataattatgaatagcacaccatttaaacctgttgattgagccctccttaaataactaaatacactactggccaacatggtgaaaacctgtctccactaaaaacacaaaaaaatggccgggcacagtggctcatgcctgtaatcccagcacttcaggaggccaaggggtgtgaatcacctgaggttaggagttcaagaccagcctggccaacatggtgaaaccctgtctctactaaaaaaaaatacaaaaattagctgagtgtagtggcacatacccgtagtctcagctactcaggaggctgaggcaggagaattgcttgaacctgggaggcaggggttgcagtgagccaagatcgtgccaccacactccagcctgggtgacacagcgagactccatctcaaaataaataaataaataaaaagaaagggaccgagcgcggtggctcatgcttgtaatcccagcactctgggaggctgagttgggcagatcacaaggtcaagagttcaggaccagcctgaccaacacggtaaaaccccatctctactaaaaatacaaaaatgagctgggtgtgatggcacgcgcctgtaaccccagttactcaaaaggctgaggcaagagaatcgcttgaacctgggaggcagaggttgcagtgagccgagatcacgccactgcattccagcctggtgacagtgagactctgtcacacacacacaaaaaagataaagaatgacaaaaatctgtgcctacattcagagtgacaagaatactaatgttctgcttgtagaaaagactattggttcagaatatgttaaatgcaaataatattttgtataatatatataaattacatatgcataaaaagagtatctatattagaatcttttgagacagggtcttgctctgtcaaccatgagggagtgcagtggcactaccacagctcactgtagccttgacttcctgagctcaagccatcctctcgcctcagcctcctgaatagttgggactgcaggtggtgccaccaaggctggctaagtttttatatttttttatagaaacaagcttttgccacgttgcccaggctggtctcaaacttctaaaagctcaagcaatctggccgccttgaactcccaaagtgcttgagttataggcatgagtcactgtgcccggcctacattagaatcttaacagtggggctgggcatggtgccccatgcctgtaatcccagcactttgggaggtcaaggtgggcagactacttgaggttgaggagttcgaggccagcctggccaacatggtgaaaccccatctgtactaaaaacacaaaaattagccaggtgtggtggcacatgtttgcaatcccagctacttgggaggctgaggcgggaggatcacttgaacctgggaagcagaggttgcagtgagccgagatggtgccatggcactccagcctgggcaatagacagcgggactcagtctcaaaacaaaaaaaaaaaaaaaaaaaaaagaatcttaacagtggttaacttcaaatagtgaaactatgactgttaactgagtttgacatttttgtgttttcctagatttttctacaataaacattattatttcataataaagcagtaaagactttttatacaaactattttaagataaacaaattttgacataggggttataagttaggtagaatctatttatataaaaaatggaactgtacttttgtgggccaaataagcactatgtaagtttttttaattttcccaaacacatgcacagaattaatattgccttaaattttgttagcacaagtttgagagagctctttagttcataaaaaaatgttttatggaccaggtgccgtggctcacacctgcaatctcaacactttgggaggcccaggtgggaggatcgcttgagcctaggagtttgagacaagactgggcgacgcagggagaccctgtctcaaaaaaacaaaaccaaaaacaagcaaacaaaaaaacagctgggcatggtggcatgcatatgtagtcccagctattctagaggctgaggtgagatcgctggagcccaggaggtggaggctacagtaagctgtgatcatgccaatgcactccagcttggtcaacaaagcaagactgtgcctcaaaaaaaaaaaagaaaagaaaagaaagaaagaaaagaaaaagaaaaaaagttatgtacgtatggtttttttttttttttggatagagtttcactcttcttgcccaggctggagtgcaatggtgcaatcttggctcaccacaaccttcccctactgggttcaagcgattctcctgtttcagcctccccagtagctgggattaaaggcatgtgccaccacgcccggctaattttgtatttttagtagagatgaagtttctccatgttggtcaggctggtcttgaactcctgacttcaggtgatctgcccgcctcagcctcccaaagtgctgggattacaggtgtgagccacctcgcctggccgttttttttttttttttttttttctgagacggagttttgctcttattgcccaggctggagtgcaatggcacgatctcggctcatcgcaacctctgcctcacgggttcaagcaattttcctgcctcagcgtctcaagtagctaggattacagggatgctccatcatgcccggctaattttgtatttttggtagagacagggtttctccatgttggtcaggctggtctcaaactcccaacctcaggtgatttacccgccttggcctcccaaagagctgggattacaggtgtgagccactgtgcccggccatgcttatgttttttaacaatacacttctgaactatcaaaaagaatataaatcaaaatcactgaagtagtttttaaaaactccaaaagctacaaaacttacttacttcaatatcaattaaaaacccatttgatagttcaataacttgagtcctgctagaatcattctataagccatcagtgacagtgaagtggccaaaatttgagtcacttgataagtacaaagaacacagatttttgtcattcttactgtgaagaaaaacagtgaatgaataacttagtttatatattaacagtacttttatttaaaaaattatctagagaataacttctttttaatcatttgttagtcatgtaactatggataaaacatactaatttagctgattcctctatgctctcttttccttgattccaatcattattagttattctacactgcctcatttattggcagttatgccaactggctgactctggttcaactgccctatttttgctttcatcattgtttatcatatctcacttgctttaaactccacctctttcatctcatctgatctgacacttggtttacatatcaattggctactctaaccttctaccgccagtttccaacccattcgaggtacttgggtaacaaaggaagatgctctatacacacaaaaccacagaaaataagtgggaagggataataaatttcacttaaagttttagaatttttcttttttttttgagacggagtttcactcttgttgcccaggctggagtgcaatggcgcgatcttggctcaccgcaacctctgcctcccaggttcaagcagttctcctgcttcagcctcccgagtagctggtattacaggcatgcaccaccaagcctggctaattttgtatttttagtagagacggggtttctccatgttggtcaggctggtcttgaacgcctgacctcaggtgatctgcctgcctcggcctcccaaagtgctgggattacaggcatgagccatcacgcccggccaaagttttagaatttaagttattccaaaaaaaattttttttttcaaaaatacagactgcatccaattaaattctatgttaactggtaatgactaggtctaaaatgttaggtatttaccaataaatgacataaaataactcaacaacaaagggatttttttttttaagagatagggtctcactttatcactcaggtttggctgagggcagtggtgtgatcacagctcactgaagcctccaactcctgggctcaagtgatcctcccgcctcagtctaccagagtatattcttgaaagtaaaattacaaatgaaattcagcagtgttaaaaataagcccacttgcagacaattatcatttttcttcctttctttcctcactatctgtacttggcatatttcctacagtggctgtcttaaagaaaaaaaggaatccttcacaaatagtgtagccaaaaaagttggactaatatacaatgctatcagtaaagtattatatataaaatttataagtgctaaagtgtaattttgaaagacacttaagatactccttttttttttgagacaaggtctcagccctgtcgcccaggctggagtgcactagcacaacatcagctcactgcaacctccgcctcccaggttcaagcgattctcctgcctcagcctcccaagtagctgagactacaggcgcacgccagcatgtccagataattttttgtatttttagtagagatggggtttcaccatgttggccaggatggtctcaaatctcttgacctcgtgatctgcccatgtcggcttcccaaagtgttaggataacaggcatgagctaccgtgcccagcctacttaaaatattcttgaaatagctctccccacctccttttttttttttttttgagaatgagtttcactcgacacccaggctggagtgcagtggtgcgatcttggctcactgcaacctctgcctcccaggttcaagcgattatcctgcctcagcctcctgagtagctgggattacaaatgtgcaccaccacatctggctaattttttttttttttttttgtatttttagtagagacggggtttcaccaagttggcctggctggtctcgaacacctgacctcaattgatccacctgcctcggcctcccaaagtattataggcatgagccaccgagcccggccttttttgttttttgtttttttaaaggcagggttttgctctgttgcccaggctggagtgcagtggtgtgatcacagatcactgcagccttgacctctcctggtctcaagtgatcctcccacctcagccttcagaacagctgggactacaggtgtgtgtcaccatgcccagtaatttttttgtatatttgtagaggcagggtctcccaatgttgcctgggctggtctcaaactcctgggctcaagcaatccaccagctttggccttccaaagttctaggattatacgcatgagccactgtgccctgccccaatattttgttacttactagtgagactaaacacttttctaaaagtttgttagccatactatcctataaaagctgtttgttcatgtcttttgtccatttatctttttttttgtttttcttgagacagagtcttgctctgtggcccaggctggagtgcaggggtgcaatctcggctcactgcaagctccgcctcccaggttcaaatgattctcctgcctcagcctcctgagtagctgggattacaggcatgtgccaccatgcccagctaatttttttgtgtgtgtttttcagtagagatggggtttcaccatgttggccaggctgatctcgaattcctgacctcaggtgctccacccgcctcagcctcccaaagtactgggattacaggggtgagccaccgcacccggccaattttctgtatttttaatagagacagggtttcatcctgttggccaggctggcctcgaacttcggacctcaggtgatccacccgcctcgacctcccaaagtgctgggattacaggtgtgggccaccacacccagccaatttttttgtatttttagtagagacagggtttcatcatgttggccaggctggtcgcaaactcctgacctcaggtgatccacccgcctcagcatcccaaagtgctgggattacaggcatgagccaccactcccggccaatgttttgtatttttagtagagatggggtttcatcatgttggccagactggtctcaaactctggacctcaggtgatccacctgcctcagcctcccaaagtgtagggattacaggtgtgagccaccgcgcccagcctatgtttctattttatacatattcaacaaacatgattccccaacttctgcaaaataatttctttttcaagaacattgattttagagctcacactaagaaaaagaatacaaaaataatggcatagaaagtgaaaaaacaaaaataaaaagtagaaagctaaagtttcccattaaaatgatcaatatactgtgcagtaagtcaaatgtgtacaatgaattaagaaaatatgatatataaaaatccaaatttacaaaattaagtacaaataggtgtttatattacaaagtgatactggtttataaaaggattcaacatagattttttttaaatggttgttttcctcaatcaatttaacaatgattttaaatgtataaaattttaatatctctttgagacagtgatccaagcttcttcccttgatgatgttaccagttcatactttgtttcaataacctgtccctccacagaaagtaggtgcagtctcttcaccaatacactaagaagtactgtggtcaccatatatgcaaacctcaactctggacactcctgtgtgcctgagaatccaagtgaggaaaaagttttcattactaattcatcatcaaaccgatctggatcaaacttgtgtggagatggccaagtattaggatcctgaagtaccacaccaagggcataaaggacgagggtctgagctgctcaattttctctggagtaacaggaccatttccaaaaacttggtttatctcttcatataattttttttgaacttcttcagaggtggttaaaaaacagattgcccaggtacacaattttgcagttattatgcaactggccagagaaaatatcatactgtcttctaggatctgttggtcattaaggttcccttgtactaaggagtcaatgaaaatatgttgactgaagttccttccttttcgttcttttatgatgttccttaaaacagactccagttgcatgagggcatcttcatattgttttttccgagtcatgtttttatcaagtgacccatctagaaagccttttccaatctcagaccaaactgtgccatgattcttctggaagcgaatgacttcctgatcatcttcaaatgtactacccattaccatctgtgtaacagacttcatagcaaaaccaagcatatgctggctgaggggcacgtgctgggtctctgggtaggagagccatttatctaataattcttctgaaagctttaggaggagggcaaagttactcttcagagaatcagtcacaccattttcatacaattttttcctcatgtggttttcactcacactgccaccaccagattgataccttaataatgacttcagcatggtttcaaaagggtccgatgtcttattgggattgatatgctgcttcagtacatcaacagtgcccaaactaaccacgaggcgcctgccaaaccagaaggagaccacaggcccatatctctcatgcaaattaaccaggaactcatgcaaacttccactattcacaatatctggaagattaccatctttttcttcagttggagtaatccctggaattcctgcagcttgtctggaagccggatagaggtagagcacggctcccaccaacgccagcaagaaggtaacggcgaagatcgcgaagtccaacatggttctgccgcccagggagccacgtctcggatcggccgctccagc

SEQ ID NO: 13084 - RNA, 8856 nt, Homo sapiens
  source 1..8856: mol_type = other RNA
gctgggattacaggcatgagccaccacacccagctggaaaatgtttaaaatttattaagtgaaaagtaactcatgctgcaatgaacgtactatgtaaaaatgtatgtatgtggaacagggaaaaatataaacagtcacagaaatgtgtttaggttggtagcattctttttcctcttaaaaattcctttttttggccgggcgctgtggctcacacctgtaatcccagcactttgggaagccgcggtggacagatcacaaggtcaggagatcaagaccatcctggctaacatggtgaaaccccgtctctactaaaaatacaaaaaattagctgggcatggaggcactcgcctgtagtcgcagctactcgggaggctgaggcaggagaatcgcttgaactggggagatggaggttgtagtgagcccagatcatgccactgcactcaagcctgggctgagacctccagagtctggctgagacctatggagtctcactctgtcacctaggctggagtacagtggtgcgatctcggcacactgcaacctccacctcccagacattctcctgcctcagcctctcaactagctgggattacattcgcccgcctccacacccactaatttttgtatttttagtagagatgcggtttccccatgttggccaggctgttcttgaactcctgacctcaagttatacgcccactttggactcccaaagtgctgggattacaggtgtgagccacggcaccagccaaaaatttctttaaatattagtggtatattattctctcaataagttttttttttttttttttttgagacagtcttgttttattgcctaagctggagtgcagtggcacaatctcaactcactgcaacctccacctcccaggtttattttttttctcatgcctcagcctcccaagaagctgggattacaggcatgtgccccaaaggccagttaagttttctttttctttttttcttttttcttggttgagacggattttcgctcgtcacccacactggagtgcaatggcgcgatctcggctcactgcaacctccgactcttgggttcaagcgattctcctgcctcagcctcccgagtagctgggattagaggcacctgtcaccacgcccgctacttttggtatttttagtagagatggagtttcaccacgttggccaggctgatctcaaactcctggcctcaagtgattcacctgccttggcctcccaaagtgctggaattacaggcccggcctatttttgcaataattatgaatagcacaccatttaaacctgttgattgagccctccttaaataactaaatacactactggccaacatggtgaaaacctgtctccactaaaaacacaaaaaaatggccgggcacagtggctcatgcctgtaatcccagcacttcaggaggccaaggggtgtgaatcacctgaggttaggagttcaagaccagcctggccaacatggtgaaaccctgtctctactaaaaaaaaatacaaaaattagctgagtgtagtggcacatacccgtagtctcagctactcaggaggctgaggcaggagaattgcttgaacctgggaggcaggggttgcagtgagccaagatcgtgccaccacactccagcctgggtgacacagcgagactccatctcaaaataaataaataaataaaaagaaagggaccgagcgcggtggctcatgcttgtaatcccagcactctgggaggctgagttgggcagatcacaaggtcaagagttcaggaccagcctgaccaacacggtaaaaccccatctctactaaaaatacaaaaatgagctgggtgtgatggcacgcgcctgtaaccccagttactcaaaaggctgaggcaagagaatcgcttgaacctgggaggcagaggttgcagtgagccgagatcacgccactgcattccagcctggtgacagtgagactctgtcacacacacacaaaaaagataaagaatgacaaaaatctgtgcctacattcagagtgacaagaatactaatgttctgcttgtagaaaagactattggttcagaatatgttaaatgcaaataatattttgtataatatatataaattacatatgcataaaaagagtatctatattagaatcttttgagacagggtcttgctctgtcaaccatgagggagtgcagtggcactaccacagctcactgtagccttgacttcctgagctcaagccatcctctcgcctcagcctcctgaatagttgggactgcaggtggtgccaccaaggctggctaagtttttatatttttttatagaaacaagcttttgccacgttgcccaggctggtctcaaacttctaaaagctcaagcaatctggccgccttgaactcccaaagtgcttgagttataggcatgagtcactgtgcccggcctacattagaatcttaacagtggggctgggcatggtgccccatgcctgtaatcccagcactttgggaggtcaaggtgggcagactacttgaggttgaggagttcgaggccagcctggccaacatggtgaaaccccatctgtactaaaaacacaaaaattagccaggtgtggtggcacatgtttgcaatcccagctacttgggaggctgaggcgggaggatcacttgaacctgggaagcagaggttgcagtgagccgagatggtgccatggcactccagcctgggcaatagacagcgggactcagtctcaaaacaaaaaaaaaaaaaaaaaaaaaagaatcttaacagtggttaacttcaaatagtgaaactatgactgttaactgagtttgacatttttgtgttttcctagatttttctacaataaacattattatttcataataaagcagtaaagactttttatacaaactattttaagataaacaaattttgacataggggttataagttaggtagaatctatttatataaaaaatggaactgtacttttgtgggccaaataagcactatgtaagtttttttaattttcccaaacacatgcacagaattaatattgccttaaattttgttagcacaagtttgagagagctctttagttcataaaaaaatgttttatggaccaggtgccgtggctcacacctgcaatctcaacactttgggaggcccaggtgggaggatcgcttgagcctaggagtttgagacaagactgggcgacgcagggagaccctgtctcaaaaaaacaaaaccaaaaacaagcaaacaaaaaaacagctgggcatggtggcatgcatatgtagtcccagctattctagaggctgaggtgagatcgctggagcccaggaggtggaggctacagtaagctgtgatcatgccaatgcactccagcttggtcaacaaagcaagactgtgcctcaaaaaaaaaaaagaaaagaaaagaaagaaagaaaagaaaaagaaaaaaagttatgtacgtatggtttttttttttttttggatagagtttcactcttcttgcccaggctggagtgcaatggtgcaatcttggctcaccacaaccttcccctactgggttcaagcgattctcctgtttcagcctccccagtagctgggattaaaggcatgtgccaccacgcccggctaattttgtatttttagtagagatgaagtttctccatgttggtcaggctggtcttgaactcctgacttcaggtgatctgcccgcctcagcctcccaaagtgctgggattacaggtgtgagccacctcgcctggccgttttttttttttttttttttttctgagacggagttttgctcttattgcccaggctggagtgcaatggcacgatctcggctcatcgcaacctctgcctcacgggttcaagcaattttcctgcctcagcgtctcaagtagctaggattacagggatgctccatcatgcccggctaattttgtatttttggtagagacagggtttctccatgttggtcaggctggtctcaaactcccaacctcaggtgatttacccgccttggcctcccaaagagctgggattacaggtgtgagccactgtgcccggccatgcttatgttttttaacaatacacttctgaactatcaaaaagaatataaatcaaaatcactgaagtagtttttaaaaactccaaaagctacaaaacttacttacttcaatatcaattaaaaacccatttgatagttcaataacttgagtcctgctagaatcattctataagccatcagtgacagtgaagtggccaaaatttgagtcacttgataagtacaaagaacacagatttttgtcattcttactgtgaagaaaaacagtgaatgaataacttagtttatatattaacagtacttttatttaaaaaattatctagagaataacttctttttaatcatttgttagtcatgtaactatggataaaacatactaatttagctgattcctctatgctctcttttccttgattccaatcattattagttattctacactgcctcatttattggcagttatgccaactggctgactctggttcaactgccctatttttgctttcatcattgtttatcatatctcacttgctttaaactccacctctttcatctcatctgatctgacacttggtttacatatcaattggctactctaaccttctaccgccagtttccaacccattcgaggtacttgggtaacaaaggaagatgctctatacacacaaaaccacagaaaataagtgggaagggataataaatttcacttaaagttttagaatttttcttttttttttgagacggagtttcactcttgttgcccaggctggagtgcaatggcgcgatcttggctcaccgcaacctctgcctcccaggttcaagcagttctcctgcttcagcctcccgagtagctggtattacaggcatgcaccaccaagcctggctaattttgtatttttagtagagacggggtttctccatgttggtcaggctggtcttgaacgcctgacctcaggtgatctgcctgcctcggcctcccaaagtgctgggattacaggcatgagccatcacgcccggccaaagttttagaatttaagttattccaaaaaaaattttttttttcaaaaatacagactgcatccaattaaattctatgttaactggtaatgactaggtctaaaatgttaggtatttaccaataaatgacataaaataactcaacaacaaagggatttttttttttaagagatagggtctcactttatcactcaggtttggctgagggcagtggtgtgatcacagctcactgaagcctccaactcctgggctcaagtgatcctcccgcctcagtctaccagagtatattcttgaaagtaaaattacaaatgaaattcagcagtgttaaaaataagcccacttgcagacaattatcatttttcttcctttctttcctcactatctgtacttggcatatttcctacagtggctgtcttaaagaaaaaaaggaatccttcacaaatagtgtagccaaaaaagttggactaatatacaatgctatcagtaaagtattatatataaaatttataagtgctaaagtgtaattttgaaagacacttaagatactccttttttttttgagacaaggtctcagccctgtcgcccaggctggagtgcactagcacaacatcagctcactgcaacctccgcctcccaggttcaagcgattctcctgcctcagcctcccaagtagctgagactacaggcgcacgccagcatgtccagataattttttgtatttttagtagagatggggtttcaccatgttggccaggatggtctcaaatctcttgacctcgtgatctgcccatgtcggcttcccaaagtgttaggataacaggcatgagctaccgtgcccagcctacttaaaatattcttgaaatagctctccccacctccttttttttttttttttgagaatgagtttcactcgacacccaggctggagtgcagtggtgcgatcttggctcactgcaacctctgcctcccaggttcaagcgattatcctgcctcagcctcctgagtagctgggattacaaatgtgcaccaccacatctggctaattttttttttttttttttgtatttttagtagagacggggtttcaccaagttggcctggctggtctcgaacacctgacctcaattgatccacctgcctcggcctcccaaagtattataggcatgagccaccgagcccggccttttttgttttttgtttttttaaaggcagggttttgctctgttgcccaggctggagtgcagtggtgtgatcacagatcactgcagccttgacctctcctggtctcaagtgatcctcccacctcagccttcagaacagctgggactacaggtgtgtgtcaccatgcccagtaatttttttgtatatttgtagaggcagggtctcccaatgttgcctgggctggtctcaaactcctgggctcaagcaatccaccagctttggccttccaaagttctaggattatacgcatgagccactgtgccctgccccaatattttgttacttactagtgagactaaacacttttctaaaagtttgttagccatactatcctataaaagctgtttgttcatgtcttttgtccatttatctttttttttgtttttcttgagacagagtcttgctctgtggcccaggctggagtgcaggggtgcaatctcggctcactgcaagctccgcctcccaggttcaaatgattctcctgcctcagcctcctgagtagctgggattacaggcatgtgccaccatgcccagctaatttttttgtgtgtgtttttcagtagagatggggtttcaccatgttggccaggctgatctcgaattcctgacctcaggtgctccacccgcctcagcctcccaaagtactgggattacaggggtgagccaccgcacccggccaattttctgtatttttaatagagacagggtttcatcctgttggccaggctggcctcgaacttcggacctcaggtgatccacccgcctcgacctcccaaagtgctgggattacaggtgtgggccaccacacccagccaatttttttgtatttttagtagagacagggtttcatcatgttggccaggctggtcgcaaactcctgacctcaggtgatccacccgcctcagcatcccaaagtgctgggattacaggcatgagccaccactcccggccaatgttttgtatttttagtagagatggggtttcatcatgttggccagactggtctcaaactctggacctcaggtgatccacctgcctcagcctcccaaagtgtagggattacaggtgtgagccaccgcgcccagcctatgtttctattttatacatattcaacaaacatgattccccaacttctgcaaaataatttctttttcaagaacattgattttagagctcacactaagaaaaagaatacaaaaataatggcatagaaagtgaaaaaacaaaaataaaaagtagaaagctaaagtttcccattaaaatgatcaatatactgtgcagtaagtcaaatgtgtacaatgaattaagaaaatatgatatataaaaatccaaatttacaaaattaagtacaaataggtgtttatattacaaagtgatactggtttataaaaggattcaacatagattttttttaaatggttgttttcctcaatcaatttaacaatgattttaaatgtataaaattttaatatctctttgagacagtgatccaagcttcttcccttgatgatgttaccagttcatactttgtttcaataacctgtccctccacagaaagtaggtgcagtctcttcaccaatacactaagaagtactgtggtcaccatatatgcaaacctcaactctggacactcctgtgtgcctgagaatccaagtgaggaaaaagttttcattactaattcatcatcaaaccgatctggatcaaacttgtgtggagatggccaagtattaggatcctgaagtaccacaccaagggcataaaggacgagggtctgagctgctcaattttctctggagtaacaggaccatttccaaaaacttggtttatctcttcatataattttttttgaacttcttcagaggtggttaaaaaacagattgcccaggtacacaattttgcagttattatgcaactggccagagaaaatatcatactgtcttctaggatctgttggtcattaaggttcccttgtactaaggagtcaatgaaaatatgttgactgaagttccttccttttcgttcttttatgatgttccttaaaacagactccagttgcatgagggtgtgccatgattcttctggaagcgaatgacttcctgatcatcttcaaatgtactacccattaccatctgtgtaacagacttcatagcaaaaccaagcatatgctggctgaggggcacgtgctgggtctctgggtaggagagccatttatctaataattcttctgaaagctttaggaggagggcaaagttactcttcagagaatcagtcacaccattttcatacaattttttcctcatgtggttttcactcacactgccaccaccagattgataccttaataatgacttcagcatggtttcaaaagggtccgttttcttcagttggagtaatccctggaattcctgcagcttgtctggaagccggatagaggtagagcacggctcccaccaacgccagcaagaaggtaacggcgaagatcgcgaagtccaacatggttctgccgcccagggagccacgtctcggatcggccgctccagc

SEQ ID NO: 13085 - RNA, 518 nt, Homo sapiens
  source 1..518: mol_type = other RNA
gctgggattacaggcatgagccaccacacccagctggcaatatatatatttttaatctgttgtacatgtaacagaaacttctggtcatccatcaaaatctatcttccctgtcttctatggtggtagagtttaagctgggtccccagcactccaggtataaacagcattactccggatcccttgcaattcaagttgactctgggacttactttaggccaatgggttatgggtgaaagttgactttccaggtcatctccaatctaagacataagccagtgttcttgagtccctttggttctttttttccatgagctgcaacatggacttctctgcaacccagccttgaccatacaaatgaggacattctatttttcagataattgttcccatataaaatttccctcgtcctcctctgcagttgatcttggatgagctgtaagttgaggcaataactgtcttctggccaggcgcagtggctcaagcctgtaatcccagcactttgggaggccgaggcgggc

SEQ ID NO: 13086 - RNA, 1230 nt, Homo sapiens
  source 1..1230: mol_type = other RNA
gctgggattacaggcatgagccaccacacccagctggcaatatatatatttttaatctgttgtacatgtaacagaaacttctggtcatccatcaaaatctatcttccctgtcttctatggtggtagagtttaagctgggtccccagcactccaggtataaacagcattactccggatcccttgcaattcaagttgactctgggacttactttaggccaatgggttatgggtgaaagttgactttccaggtcatctccaatctaagacataagccagtgttcttgagtccctttggttctttttttccatgagctgcaacatggacttctctgcaacccagccttgaccatacaaatgaggacattctatttttcagataattgttcccatataaaatttccctcgtcctcctctgcagttgatcttggatgagcttatatctcttcttgaagttctcattgctgcttctcctgtttagagtgaatttccgactctaccaagcaaaaagtgaaattgagttgtgtcattcacaaaacatgacaaataaatatccatgactgcttcatccgattgttcaaaaatattcctggacacttgcagatttccttatatagactttaaagcacataatactttgtacttctgtgtacttcctgagtttcctgagtttgaacggaaggaacaaaacatgccagagtatattttttaacactctgaaggagtgtgatttctgtgaccatgaactcattatgggttccattactttgagaagtgctattctttggaaaagatgaattggggagtttggagtcggacatagggtacaaactccagtgctgcctcttatatgctgtgtggtcttggacaagaagcttagtctctgaggatcttagagtcaaaacttataaagttggaataatatcttctcagcagtagttttgtaagaatcaaataagatagtacctaggaaggaggaatgaatctaacttcaatacacaggatacaagaaatgttgcatttgtttccctgaataaaatttaatctgctaacagtcttctgcatctcagcgataaacaaatacacaaatatataaaggaatagtctatgccgatcttcccaattccattgggatggcaggaaatacaataatggatctccctccaacttgtgaaggcactagaagtcttcccaagagcagaacttctgttcaggaggctcttggttcttact

SEQ ID NO: 13087 - RNA, 1484 nt, Homo sapiens
  source 1..1484: mol_type = other RNA
gctgggattacaggcatgagccaccacacccagctggcaatatatatatttttaatctgttgtacatgtaacagaaacttctggtcatccatcaaaatctatcttccctgtcttctatggtggtagagtttaagctgggtccccagcactccaggtataaacagcattactccggatcccttgcaattcaagttgactctgggacttactttaggccaatgggttatgggtgaaagttgactttccaggtcatctccaatctaagacataagccagtgttcttgagtccctttggttctttttttccatgagctgcaacatggacttctctgcaacccagccttgaccatacaaatgaggacattctctgggggaatggcagaaccgaaagatgtcagagcttgaatcgatgaatgactatttttcagataattgttcccatataaaatttccctcgtcctcctctgcagttgatcttggatgagcatggccttggctgaggctacttccagctagatgaaccagtgctgctttagaatccccctaaaatcagcaaaaacacacatttagctgaagaccaaaccccttgccaagaaaaggaaagctcatcgatgctcacatcctcaagctcgagctctgtaggggtgtttcccattgtttctgtatcttttcctgcagaataagagaaggaccctcaaaccagcatgagccgtcagtcaggatagcctcctcttagtaacagcttgtcttagcaacaccaagaagatggaaactggctagaacaaaggagagctctgcagagagacagatctgaactggaagccttctgcttctgctcttcaaaggctccttcactttccagcttcaattttccaatctatataaagggcacagtcatagttcattattagtcatgaacttcaagaactacatggagttcttgtgggaattatataaggtcacataaataaaggcacttagcgcagattcaggaacatattagtttttgttttggtaaatgccatttattattatcaataacaatagcacctagcagccccttccccagtagtttccctgccccagcagtccctgccctagcagtgcattctagtcaattgcagacactggttttcccctttagacctacagatgtttcctatgagactactgaaagcttctccaggactgaatttcttcccttattctctcccatttcccacccatggagaagttagacaacgttcagttacttgtaattatccatcaacccatcactcactatgcaccaagcattgggtcatgcattgagaatccataaatcaataagacccagcctctgccctctaagatctccccatttagagagggagctagtcatgtaaaaggataagtcaatataatgggatctgcataattatgaaggattatataaggaattaggtggacttttgttgaaatcttgtcttttttttttttttttc

SEQ ID NO: 13088 - RNA, 2058 nt, Homo sapiens
  source 1..2058: mol_type = other RNA
gctgggattacaggcatgagccaccacacccagctggcaatatatatatttttaatctgttgtacatgtaacagaaacttctggtcatccatcaaaatctatcttccctgtcttctatggtggtagagtttaagctgggtccccagcactccaggtataaacagcattactccggatcccttgcaattcaagttgactctgggacttactttaggccaatgggttatgggtgaaagttgactttccaggtcatctccaatctaagacataagccagtgttcttgagtccctttggttctttttttccatgagctgcaacatggacttctctgcaacccagccttgaccatacaaatgaggacattctctgggggaatggcagaaccgaaagatgtcagagcttgaatcgatgaatgactatttttcagataattgttcccatataaaatttccctcgtcctcctctgcagttgatcttggatgagctggagatgccttcatggagaaaggcaagtaaataaattgactataacctatcgtaatccagtatgaatgaatgtatcccttaggtttatatgtttccaatggcaggaagtagttaatctcaaaggctttacaaaagtggtgagctaagtccttatatctcttcttgaagttctcattgctgcttctcctgtttagagtgaatttccgactcttcaagagctggctaggaggaacaagatggagtgggtacagaagggaggaatacttctcggagtatatcctttatatagttttgacttctggaagcatgttaatgctccaccagacaggcatgatttcagctggggtcctagctgtttctcaacctccattgttccagcaggcatccaaagcagacttcccagtcatctgtgagctacccaacattctttcaattgatccctttccttaatatgttaaatcagtttcaagtaagaaccttcactggtgcaaaaaaaaaaaaaattaataccaaaggaagcacttatgtcaagtgaagagcaaatgagctccaggattgactttttgcagcagcatggccttggctgaggctacttccagctagatgaaccagtgctgctttagaatccccctaaaatcagcaaaaacacacatttagctgaagaccaaaccccttgccaagaaaaggaaagctcatcgatgctcacatcctcaagctcgagctctgtaggggtgtttcccattgtttctgtatcttttcctgcagaataagagaaggaccctcaaaccagcatgagccgtcagtcaggatagcctcctcttagtaacagcttgtcttagcaacaccaagaagatggaaactggctagaacaaaggagagctctgcagagagacagatctgaactggaagccttctgcttctgctcttcaaaggctccttcactttccagcttcaattttccaatctatataaagggcacagtcatagttcattattagtcatgaacttcaagaactacatggagttcttgtgggaattatataaggtcacataaataaaggcacttagcgcagattcaggaacatattagtttttgttttggtaaatgccatttattattatcaataacaatagcacctagcagccccttccccagtagtttccctgccccagcagtccctgccctagcagtgcattctagtcaattgcagacactggttttcccctttagacctacagatgtttcctatgagactactgaaagcttctccaggactgaatttcttcccttattctctcccatttcccacccatggagaagttagacaacgttcagttacttgtaattatccatcaacccatcactcactatgcaccaagcattgggtcatgcattgagaatccataaatcaataagacccagcctctgccctctaagatctccccatttagagagggagctagtcatgtaaaaggataagtcaatataatgggatctgcataattatgaaggattatataaggaattaggtggacttttgttgaaatcttgtcttttttttttttttttc

SEQ ID NO: 13089 - RNA, 570 nt, Homo sapiens
  source 1..570: mol_type = other RNA
gctgggattacaggcatgagccaccacacccagctggcaatatatatatttttaatctgttgtacatgtaacagaaacttctggtcatccatcaaaatctatcttccctgtcttctatggtggtagagtttaagctgggtccccagcactccaggtataaacagcattactccggatcccttgcaattcaagttgactctgggacttactttaggccaatgggttatgggtgaaagttgactttccaggtcatctccaatctaagacataagccagtgttcttgagtccctttggttctttttttccatgagctgcaacatggacttctctgcaacccagccttgaccatacaaatgaggacattctctgggggaatggcagaaccgaaagatgtcagagcttgaatcgatgaatgactatttttcagataattgttcccatataaaatttccctcgtcctcctctgcagttgatcttggatgagctgtaagttgaggcaataactgtcttctggccaggcgcagtggctcaagcctgtaatcccagcactttgggaggccgaggcgggc

SEQ ID NO: 13090 - RNA, 1795 nt, Homo sapiens
  source 1..1795: mol_type = other RNA
gctgggattacaggcatgagccaccacacccagctggcaatatatatatttttaatctgttgtacatgtaacagaaacttctggtcatccatcaaaatctatcttccctgtcttctatggtggtagagtttaagctgggtccccagcactccaggtataaacagcattactccggatcccttgcaattcaagttgactctgggacttactttaggccaatgggttatgggtgaaagttgactttccaggtcatctccaatctaagacataagccagtgttcttgagtccctttggttctttttttccatgagctgcaacatggacttctctgcaacccagccttgaccatacaaatgaggacattctctgggggaatggcagaaccgaaagatgtcagagcttgaatcgatgaatgactatttttcagataattgttcccatataaaatttccctcgtcctcctctgcagttgatcttggatgagcttatatctcttcttgaagttctcattgctgcttctcctgtttagagtgaatttccgactcagacaggcatgatttcagctggggtcctagctgtttctcaacctccattgttccagcaggcatccaaagcagacttcccagtcatctgtgagctacccaacattctttcaattgatccctttccttaatatgttaaatcagtttcaagtaagaaccttcactggtgcaaaaaaaaaaaaaattaataccaaaggaagcacttatgtcaagtgaagagcaaatgagctccaggattgactttttgcagcagcatggccttggctgaggctacttccagctagatgaaccagtgctgctttagaatccccctaaaatcagcaaaaacacacatttagctgaagaccaaaccccttgccaagaaaaggaaagctcatcgatgctcacatcctcaagctcgagctctgtaggggtgtttcccattgtttctgtatcttttcctgcagaataagagaaggaccctcaaaccagcatgagccgtcagtcaggatagcctcctcttagtaacagcttgtcttagcaacaccaagaagatggaaactggctagaacaaaggagagctctgcagagagacagatctgaactggaagccttctgcttctgctcttcaaaggctccttcactttccagcttcaattttccaatctatataaagggcacagtcatagttcattattagtcatgaacttcaagaactacatggagttcttgtgggaattatataaggtcacataaataaaggcacttagcgcagattcaggaacatattagtttttgttttggtaaatgccatttattattatcaataacaatagcacctagcagccccttccccagtagtttccctgccccagcagtccctgccctagcagtgcattctagtcaattgcagacactggttttcccctttagacctacagatgtttcctatgagactactgaaagcttctccaggactgaatttcttcccttattctctcccatttcccacccatggagaagttagacaacgttcagttacttgtaattatccatcaacccatcactcactatgcaccaagcattgggtcatgcattgagaatccataaatcaataagacccagcctctgccctctaagatctccccatttagagagggagctagtcatgtaaaaggataagtcaatataatgggatctgcataattatgaaggattatataaggaattaggtggacttttgttgaaatcttgtcttttttttttttttttc

SEQ ID NO: 13091 - RNA, 1282 nt, Homo sapiens
  source 1..1282: mol_type = other RNA
gctgggattacaggcatgagccaccacacccagctggcaatatatatatttttaatctgttgtacatgtaacagaaacttctggtcatccatcaaaatctatcttccctgtcttctatggtggtagagtttaagctgggtccccagcactccaggtataaacagcattactccggatcccttgcaattcaagttgactctgggacttactttaggccaatgggttatgggtgaaagttgactttccaggtcatctccaatctaagacataagccagtgttcttgagtccctttggttctttttttccatgagctgcaacatggacttctctgcaacccagccttgaccatacaaatgaggacattctctgggggaatggcagaaccgaaagatgtcagagcttgaatcgatgaatgactatttttcagataattgttcccatataaaatttccctcgtcctcctctgcagttgatcttggatgagcttatatctcttcttgaagttctcattgctgcttctcctgtttagagtgaatttccgactctaccaagcaaaaagtgaaattgagttgtgtcattcacaaaacatgacaaataaatatccatgactgcttcatccgattgttcaaaaatattcctggacacttgcagatttccttatatagactttaaagcacataatactttgtacttctgtgtacttcctgagtttcctgagtttgaacggaaggaacaaaacatgccagagtatattttttaacactctgaaggagtgtgatttctgtgaccatgaactcattatgggttccattactttgagaagtgctattctttggaaaagatgaattggggagtttggagtcggacatagggtacaaactccagtgctgcctcttatatgctgtgtggtcttggacaagaagcttagtctctgaggatcttagagtcaaaacttataaagttggaataatatcttctcagcagtagttttgtaagaatcaaataagatagtacctaggaaggaggaatgaatctaacttcaatacacaggatacaagaaatgttgcatttgtttccctgaataaaatttaatctgctaacagtcttctgcatctcagcgataaacaaatacacaaatatataaaggaatagtctatgccgatcttcccaattccattgggatggcaggaaatacaataatggatctccctccaacttgtgaaggcactagaagtcttcccaagagcagaacttctgttcaggaggctcttggttcttact

SEQ ID NO: 13092 - RNA, 1907 nt, Homo sapiens
  source 1..1907: mol_type = other RNA
gctgggattacaggcatgagccaccacacccagctggcaatatatatatttttaatctgttgtacatgtaacagaaacttctggtcatccatcaaaatctatcttccctgtcttctatggtggtagagtttaagctgggtccccagcactccaggtataaacagcattactccggatcccttgcaattcaagttgactctgggacttactttaggccaatgggttatgggtgaaagttgactttccaggtcatctccaatctaagacataagccagtgttcttgagtccctttggttctttttttccatgagctgcaacatggacttctctgcaacccagccttgaccatacaaatgaggacattctctgggggaatggcagaaccgaaagatgtcagagcttgaatcgatgaatgactatttttcagataattgttcccatataaaatttccctcgtcctcctctgcagttgatcttggatgagcttatatctcttcttgaagttctcattgctgcttctcctgtttagagtgaatttccgactcttcaagagctggctaggaggaacaagatggagtgggtacagaagggaggaatacttctcggagtatatcctttatatagttttgacttctggaagcatgttaatgctccaccagacaggcatgatttcagctggggtcctagctgtttctcaacctccattgttccagcaggcatccaaagcagacttcccagtcatctgtgagctacccaacattctttcaattgatccctttccttaatatgttaaatcagtttcaagtaagaaccttcactggtgcaaaaaaaaaaaaaattaataccaaaggaagcacttatgtcaagtgaagagcaaatgagctccaggattgactttttgcagcagcatggccttggctgaggctacttccagctagatgaaccagtgctgctttagaatccccctaaaatcagcaaaaacacacatttagctgaagaccaaaccccttgccaagaaaaggaaagctcatcgatgctcacatcctcaagctcgagctctgtaggggtgtttcccattgtttctgtatcttttcctgcagaataagagaaggaccctcaaaccagcatgagccgtcagtcaggatagcctcctcttagtaacagcttgtcttagcaacaccaagaagatggaaactggctagaacaaaggagagctctgcagagagacagatctgaactggaagccttctgcttctgctcttcaaaggctccttcactttccagcttcaattttccaatctatataaagggcacagtcatagttcattattagtcatgaacttcaagaactacatggagttcttgtgggaattatataaggtcacataaataaaggcacttagcgcagattcaggaacatattagtttttgttttggtaaatgccatttattattatcaataacaatagcacctagcagccccttccccagtagtttccctgccccagcagtccctgccctagcagtgcattctagtcaattgcagacactggttttcccctttagacctacagatgtttcctatgagactactgaaagcttctccaggactgaatttcttcccttattctctcccatttcccacccatggagaagttagacaacgttcagttacttgtaattatccatcaacccatcactcactatgcaccaagcattgggtcatgcattgagaatccataaatcaataagacccagcctctgccctctaagatctccccatttagagagggagctagtcatgtaaaaggataagtcaatataatgggatctgcataattatgaaggattatataaggaattaggtggacttttgttgaaatcttgtcttttttttttttttttc

SEQ ID NO: 13093 - RNA, 1153 nt, Homo sapiens
  source 1..1153: mol_type = other RNA
gctgggattacaggcatgagccaccacacccagctggcaatatatatatttttaatctgttgtacatgtaacagaaacttctggtcatccatcaaaatctatcttccctgtcttctatggtggtagagtttaagctgggtccccagcactccaggtataaacagcattactccggatcccttgcaattcaagttgactctgggacttactttaggccaatgggttatgggtgaaagttgactttccaggtcatctccaatctaagacataagccagtgttcttgagtccctttggttctttttttccatgagctgcaacatggacttctctgcaacccagccttgaccatacaaatgaggacattctctgggggaatggcagaaccgaaagatgtcagagcttgaatcgatgaatgactatttttcagataattgttcccatataaaatttccctcgtcctcctctgcagttgatcttggatgagcttatatctcttcttgaagttctcattgctgcttctcctgtttagagtgaatttccgactcttcaagagctggctaggaggaacaagatggagtgggtacagaagggaggaatacttctcggagtatatcctttatatagttttgacttctggaagcatgttaatgctccaccagacaggcatgatttcagctggggtcctagctgtttctcaacctccattgttccagcaggcatccaaagcagacttcccagtcatctgtgagctacccaacattctttcaattgatccctttccttaatatgttaaatcagtttcaagtaagaaccttcactggtgcaaaaaaaaaaaaaattaataccaaaggaagcacttatgtcaagtgaagagcaaatgagctccaggattgactttttgcagcagttctagaatgaagccgcggagccttgcggtcagtgttacagctcttaaggtgacgcgtctagagtttgttccttctgatgttcggatgtcttcggagtttctttcttctggtgggttcgtggtctcactggctcagaagtgaacccgtgaaccttcgcggtaagtgttaccgctcttaaggcagcgcgtctggagttgttcgtccctcccggtgagttcatggtctcgctggcttcaagagtgaa

SEQ ID NO: 13094 - RNA, 2008 nt, Homo sapiens
  source 1..2008: mol_type = other RNA
gctgggattacaggcatgagccaccacacccatcctatgaattttcttatgttgagtaagtcttgaagaccgggtaaaagctttggcacattcttcacatttgtaaggtttctctctagtatgaattttcttatgttgagtaagtcttgaggaccgattaaaagctttgccacattcttcacatttgtagggtttctctccactatgaattttcttatgactactaaggtttgaggagtgggtaaaagctttgtcacattgtttacatttgtagggtttctctccagtatgaattttcttatgttgagtaagtcttgaggaccggttaaaagctttgccacattcttcacatttgtaaggtttctctccagtatgaattttcttatgttgagtaagtcttgaggacaggataaaagctttgccacattcttcacatttgtagggtttctctccactatgaatttttttatgactgttaaggtttgaggactgcttaaaggctttgccacattcttcacatttgtagggtttctctccagtatgaattctcctatggctagtaaggtgtgaggaccggttaaaagctttgccacattcgttacatttatagggtttctcttcagtatgaattctcttatgtctagtaagtgtagaggaataggtaaaaactttgccacattcttcacaattgtagggtttctctccagtatgaattttcttgtcttgagtaagtgttgaggaacaggtaaaaactctgccacatttttcaaatttgtagggttcctctccagtatgaatttttttatgtcgagtaagtcttgaagactggttaaaagctttgccacattcttcacatttgtagggcttctctccagtatgaattaccttatgtttagtaagagttgaagaccagttaaaggctttgccacattcttcacatttgtagggtttctcaccagtatgtattctcttatggctagtaagggttgaggaccggttaaaggctttgccacattctttacatttgtagggtttctcttcagtatgaattatcttatgtttagtaaaggttgaggatatgctaaaggttttgccacattcatcacatttgtagggcttctctccagaatgaattctcttatgggtagtaagggttgagtacctgctaaaggctttgccacattctttacatttgtagggtttctctccagtatgaattctcttatggttagtaagggttgagtagtggttaaatgctttgccacattcttcacatctgtagtgtttctcaccaacataaattctcttatggttagtaagggctgaggactgattaaaggcattgccaaattctttacatctgtaggtattctctctaatatgaattttcttatgttgagttagttgtgaaagcatgcaaaatgatttgccacattttttacactggaaaggtttctttccagtatgtcttgtcttgtatctatctgcatttgaaaatgcataaaagacttttacatatatatcacagtgatacattttgctctgggtaagtgtcaaacattggttaagtccattataacctcctttgtatagcttacaatcacctacagttttatagccttttcttaattgtaagttctcatgtccacgtttatcatatctcctcagtgtcactttttggaaagaatcttttatgtcttgctctggccaaaagtcttcagcaaaatgagaacacacaactgggggttcatccaccatttcatgtcgcttcatcttgcagggttctttttctttctctagacaagtgattaggtctggcttagaaacagcaataccatttctaggcttccagggggtcctggagtcttagctgtgtatctcccaatatctgcgggtcacagggccacacaggctgggcctctaagaacaaaggacacagaaatgaagacgagacctggagctctggctgcagcaagagccaaacgccccgccatattccggaaaccgt

SEQ ID NO: 13095 - RNA, 2422 nt, Homo sapiens
  source 1..2422: mol_type = other RNA
gctgggattacaggcatgagccaccacacccatcctatgaattttcttatgttgagtaagtcttgaagaccgggtaaaagctttggcacattcttcacatttgtaaggtttctctctagtatgaattttcttatgttgagtaagtcttgaggaccgattaaaagctttgccacattcttcacatttgtagggtttctctccactatgaattttcttatgactactaaggtttgaggagtgggtaaaagctttgtcacattgtttacatttgtagggtttctctccagtatgaattttcttatgttgagtaagtcttgaggaccggttaaaagctttgccacattcttcacatttgtaaggtttctctccagtatgaattttcttatgttgagtaagtcttgaggacaggataaaagctttgccacattcttcacatttgtagggtttctctccactatgaatttttttatgactgttaaggtttgaggactgcttaaaggctttgccacattcttcacatttgtagggtttctctccagtatgaattctcctatggctagtaaggtgtgaggaccggttaaaagctttgccacattcgttacatttatagggtttctcttcagtatgaattctcttatgtctagtaagtgtagaggaataggtaaaaactttgccacattcttcacaattgtagggtttctctccagtatgaattttcttgtcttgagtaagtgttgaggaacaggtaaaaactctgccacatttttcaaatttgtagggttcctctccagtatgaatttttttatgtcgagtaagtcttgaagactggttaaaagctttgccacattcttcacatttgtagggcttctctccagtatgaattaccttatgtttagtaagagttgaagaccagttaaaggctttgccacattcttcacatttgtagggtttctcaccagtatgtattctcttatggctagtaagggttgaggaccggttaaaggctttgccacattctttacatttgtagggtttctcttcagtatgaattatcttatgtttagtaaaggttgaggatatgctaaaggttttgccacattcatcacatttgtagggcttctctccagaatgaattctcttatgggtagtaagggttgagtacctgctaaaggctttgccacattctttacatttgtagggtttctctccagtatgaattctcttatggttagtaagggttgagtagtggttaaatgctttgccacattcttcacatctgtagtgtttctcaccaacataaattctcttatggttagtaagggctgaggactgattaaaggcattgccaaattctttacatctgtaggtattctctctaatatgaattttcttatgttgagttagttgtgaaagcatgcaaaatgatttgccacattttttacactggaaaggtttctttccagtatgtcttgtcttgtatctatctgcatttgaaaatgcataaaagacttttacatatatatcacagtgatacattttgctctgggtaagtgtcaaacattggttaagtccattataacctcctttgtatagcttacaatcacctacagttttatagccttttcttaattgtaagttctcatgtccacgtttatcatatctcctcagtgtcactttttggaaagaatcttttatgtcttgctctggccaaaagtcttcagcaaaatgagaacacacaactgggggttcatccaccatttcatgtcgcttcatcttgcagggttctttttctttctctagacaagtgattaggtctggcttagaaacagcaatacccaggaagaccaagtttctgtagttctctaacatcacatttctatataagttctgttgtgctgtgtccaggcactgccactcctccagagagaattctatggccacatctgacgcccctcccatggttcttgcacaatctgggagagactgcggaattgcgcgtgcagagctccccagacagggctacacgtcaggcacagtcactgcggagggaagacaggacgcccggggcccggctgtcagcacagtcgccatcttatggctgaaggggactgaagccgagctgggcaaggagaattccgggcgcagattgtggagctgactgccgggagacctaagtccgccacggccacttctcacggttccgaccagcccctccccctctctggggatgtcagactcggcactctcaccatttctaggcttccagggggtcctggagtcttagctgtgtatctcccaatatctgcgggtcacagggccacacaggctgggcctctaagaacaaaggacacagaaatgaagacgagacctggagctctggctgcagcaagagccaaacgccccgccatattccggaaaccgt

SEQ ID NO: 13096 - RNA, 2224 nt, Homo sapiens
  source 1..2224: mol_type = other RNA
gctgggattacaggcatgagccaccacacccatcctatgaattttcttatgttgagtaagtcttgaagaccgggtaaaagctttggcacattcttcacatttgtaaggtttctctctagtatgaattttcttatgttgagtaagtcttgaggaccgattaaaagctttgccacattcttcacatttgtagggtttctctccactatgaattttcttatgactactaaggtttgaggagtgggtaaaagctttgtcacattgtttacatttgtagggtttctctccagtatgaattttcttatgttgagtaagtcttgaggaccggttaaaagctttgccacattcttcacatttgtaaggtttctctccagtatgaattttcttatgttgagtaagtcttgaggacaggataaaagctttgccacattcttcacatttgtagggtttctctccactatgaatttttttatgactgttaaggtttgaggactgcttaaaggctttgccacattcttcacatttgtagggtttctctccagtatgaattctcctatggctagtaaggtgtgaggaccggttaaaagctttgccacattcgttacatttatagggtttctcttcagtatgaattctcttatgtctagtaagtgtagaggaataggtaaaaactttgccacattcttcacaattgtagggtttctctccagtatgaattttcttgtcttgagtaagtgttgaggaacaggtaaaaactctgccacatttttcaaatttgtagggttcctctccagtatgaatttttttatgtcgagtaagtcttgaagactggttaaaagctttgccacattcttcacatttgtagggcttctctccagtatgaattaccttatgtttagtaagagttgaagaccagttaaaggctttgccacattcttcacatttgtagggtttctcaccagtatgtattctcttatggctagtaagggttgaggaccggttaaaggctttgccacattctttacatttgtagggtttctcttcagtatgaattatcttatgtttagtaaaggttgaggatatgctaaaggttttgccacattcatcacatttgtagggcttctctccagaatgaattctcttatgggtagtaagggttgagtacctgctaaaggctttgccacattctttacatttgtagggtttctctccagtatgaattctcttatggttagtaagggttgagtagtggttaaatgctttgccacattcttcacatctgtagtgtttctcaccaacataaattctcttatggttagtaagggctgaggactgattaaaggcattgccaaattctttacatctgtaggtattctctctaatatgaattttcttatgttgagttagttgtgaaagcatgcaaaatgatttgccacattttttacactggaaaggtttctttccagtatgtcttgtcttgtatctatctgcatttgaaaatgcataaaagacttttacatatatatcacagtgatacattttgctctgggtaagtgtcaaacattggttaagtccattataacctcctttgtatagcttacaatcacctacagttttatagccttttcttaattgtaagttctcatgtccacgtttatcatatctcctcagtgtcactttttggaaagaatcttttatgtcttgctctggccaaaagtcttcagcaaaatgagaacacacaactgggggttcatccaccatttcatgtcgcttcatcttgcagggttctttttctttctctagacaagtgattaggtctggcttagaaacagcaatacccaggaagaccaagtttctgtagttctctaacatcacatttctatataagttctgttgtgctgtgtccaggcactgccactcctccagagagaattctatggccacatctgtaaatgtcaatggtcccagtaatgccaatgtttttgatccaaaaagaatattttgtcaaacattcagtaaatgaaggaagctgtgtttttcccagtttttttgtccatttctaggcttccagggggtcctggagtcttagctgtgtatctcccaatatctgcgggtcacagggccacacaggctgggcctctaagaacaaaggacacagaaatgaagacgagacctggagctctggctgcagcaagagccaaacgccccgccatattccggaaaccgt

SEQ ID NO: 13097 - RNA, 2704 nt, Homo sapiens
  source 1..2704: mol_type = other RNA
gctgggattacaggcatgagccaccacacccatcctatgaattttcttatgttgagtaagtcttgaagaccgggtaaaagctttggcacattcttcacatttgtaaggtttctctctagtatgaattttcttatgttgagtaagtcttgaggaccgattaaaagctttgccacattcttcacatttgtagggtttctctccactatgaattttcttatgactactaaggtttgaggagtgggtaaaagctttgtcacattgtttacatttgtagggtttctctccagtatgaattttcttatgttgagtaagtcttgaggaccggttaaaagctttgccacattcttcacatttgtaaggtttctctccagtatgaattttcttatgttgagtaagtcttgaggacaggataaaagctttgccacattcttcacatttgtagggtttctctccactatgaatttttttatgactgttaaggtttgaggactgcttaaaggctttgccacattcttcacatttgtagggtttctctccagtatgaattctcctatggctagtaaggtgtgaggaccggttaaaagctttgccacattcgttacatttatagggtttctcttcagtatgaattctcttatgtctagtaagtgtagaggaataggtaaaaactttgccacattcttcacaattgtagggtttctctccagtatgaattttcttgtcttgagtaagtgttgaggaacaggtaaaaactctgccacatttttcaaatttgtagggttcctctccagtatgaatttttttatgtcgagtaagtcttgaagactggttaaaagctttgccacattcttcacatttgtagggcttctctccagtatgaattaccttatgtttagtaagagttgaagaccagttaaaggctttgccacattcttcacatttgtagggtttctcaccagtatgtattctcttatggctagtaagggttgaggaccggttaaaggctttgccacattctttacatttgtagggtttctcttcagtatgaattatcttatgtttagtaaaggttgaggatatgctaaaggttttgccacattcatcacatttgtagggcttctctccagaatgaattctcttatgggtagtaagggttgagtacctgctaaaggctttgccacattctttacatttgtagggtttctctccagtatgaattctcttatggttagtaagggttgagtagtggttaaatgctttgccacattcttcacatctgtagtgtttctcaccaacataaattctcttatggttagtaagggctgaggactgattaaaggcattgccaaattctttacatctgtaggtattctctctaatatgaattttcttatgttgagttagttgtgaaagcatgcaaaatgatttgccacattttttacactggaaaggtttctttccagtatgtcttgtcttgtatctatctgcatttgaaaatgcataaaagacttttacatatatatcacagtgatacattttgctctgggtaagtgtcaaacattggttaagtccattataacctcctttgtatagcttacaatcacctacagttttatagccttttcttaattgtaagttctcatgtccacgtttatcatatctcctcagtgtcactttttggaaagaatcttttatgtcttgctctggccaaaagtcttcagcaaaatgagaacacacaactgggggttcatccaccatttcatgtcgcttcatcttgcagggttctttttctttctctagacaagtgattaggtctggcttagaaacagcaatacccaggaagaccaagtttctgtagttctctaacatcacatttctatataagttctgttgtgctgtgtccaggcactgccactcctccagagagaattctatggccacatctgtaaatgtcaatggtcccagtaatgccaatgtttttgatccaaaaagaatattttgtcaaacattcagtaaatgaaggaagctgtgtttttcccagtttttttgtcctgacgcccctcccatggttcttgcacaatctgggagagactgcggaattgcgcgtgcagagctccccagacagggctacacgtcaggcacagtcactgcggagggaagacaggacgcccggggcccggctgtcagcacagtcgccatcttatggctgaaggggactgaagccgagctgggcaaggagaattccgggcgcagattgtggagctgactgccgggagacctaagtccgccacggccacttctcacggttccgaccagcccctccccctctctggggatgtcagactcggcactctcaccatttctaggcttccagggggtcctggagtcttagctgtgtatctcccaatatctgcgggtcacagggccacacaggctgggcctctaagaacaaaggacacagaaatgaagacgagacctggagctctggctgcagcaagagccaaacgccccgccatattccggaaaccgtcctgtcgctccagctgcgtgcctgattggataatgtttaagacccgccctctcaggccctgagtgacagagggtgatcagttgctgggcagaatgaagcgtgacagcctagctgcagccttttcaggcaggctttcctccgagctgagccaggcccaccctagagggtgtttgc

SEQ ID NO: 13098 - RNA, 2453 nt, Homo sapiens
  source 1..2453: mol_type = other RNA
gctgggattacaggcatgagccaccacacccatcctatgaattttcttatgttgagtaagtcttgaagaccgggtaaaagctttggcacattcttcacatttgtaaggtttctctctagtatgaattttcttatgttgagtaagtcttgaggaccgattaaaagctttgccacattcttcacatttgtagggtttctctccactatgaattttcttatgactactaaggtttgaggagtgggtaaaagctttgtcacattgtttacatttgtagggtttctctccagtatgaattttcttatgttgagtaagtcttgaggaccggttaaaagctttgccacattcttcacatttgtaaggtttctctccagtatgaattttcttatgttgagtaagtcttgaggacaggataaaagctttgccacattcttcacatttgtagggtttctctccactatgaatttttttatgactgttaaggtttgaggactgcttaaaggctttgccacattcttcacatttgtagggtttctctccagtatgaattctcctatggctagtaaggtgtgaggaccggttaaaagctttgccacattcgttacatttatagggtttctcttcagtatgaattctcttatgtctagtaagtgtagaggaataggtaaaaactttgccacattcttcacaattgtagggtttctctccagtatgaattttcttgtcttgagtaagtgttgaggaacaggtaaaaactctgccacatttttcaaatttgtagggttcctctccagtatgaatttttttatgtcgagtaagtcttgaagactggttaaaagctttgccacattcttcacatttgtagggcttctctccagtatgaattaccttatgtttagtaagagttgaagaccagttaaaggctttgccacattcttcacatttgtagggtttctcaccagtatgtattctcttatggctagtaagggttgaggaccggttaaaggctttgccacattctttacatttgtagggtttctcttcagtatgaattatcttatgtttagtaaaggttgaggatatgctaaaggttttgccacattcatcacatttgtagggcttctctccagaatgaattctcttatgggtagtaagggttgagtacctgctaaaggctttgccacattctttacatttgtagggtttctctccagtatgaattctcttatggttagtaagggttgagtagtggttaaatgctttgccacattcttcacatctgtagtgtttctcaccaacataaattctcttatggttagtaagggctgaggactgattaaaggcattgccaaattctttacatctgtaggtattctctctaatatgaattttcttatgttgagttagttgtgaaagcatgcaaaatgatttgccacattttttacactggaaaggtttctttccagtatgtcttgtcttgtatctatctgcatttgaaaatgcataaaagacttttacatatatatcacagtgatacattttgctctgggtaagtgtcaaacattggttaagtccattataacctcctttgtatagcttacaatcacctacagttttatagccttttcttaattgtaagttctcatgtccacgtttatcatatctcctcagtgtcactttttggaaagaatcttttatgtcttgctctggccaaaagtcttcagcaaaatgagaacacacaactgggggttcatccaccatttcatgtcgcttcatcttgcagggttctttttctttctctagacaagtgattaggtctggcttagaaacagcaatacccaggaagaccaagtttctgtagttctctaacatcacatttctatataagttctgttgtgctgtgtccaggcactgccactcctccagagagaattctatggccacatctgtaaatgtcaatggtcccagtaatgccaatgtttttgatccaaaaagaatattttgtcaaacattcagtaaatgaaggaagctgtgtttttcccagtttttttgtccttagaatcacatgaggcacttaattaaaacaacatggatgcttctatgcagaaccatttctaggcttccagggggtcctggagtcttagctgtgtatctcccaatatctgcgggtcacagggccacacaggctgggcctctaagaacaaaggacacagaaatgaagacgagacctggagctctggctgcagcaagagccaaacgccccgccatattccggaaaccgtcctgtcgctccagctgcgtgcctgattggataatgtttaagacccgccctctcaggccctgagtgacagagggtgatcagttgctgggcagaatgaagcgtgacagcctagctgcagccttttcaggcaggctttcctccgagctgagccaggcccaccctagagggtgtttgc

SEQ ID NO: 13099 - RNA, 4538 nt, Homo sapiens
  source 1..4538: mol_type = other RNA
gctgggattacaggcatgagccaccacacccatcctatgaattttcttatgttgagtaagtcttgaagaccgggtaaaagctttggcacattcttcacatttgtaaggtttctctctagtatgaattttcttatgttgagtaagtcttgaggaccgattaaaagctttgccacattcttcacatttgtagggtttctctccactatgaattttcttatgactactaaggtttgaggagtgggtaaaagctttgtcacattgtttacatttgtagggtttctctccagtatgaattttcttatgttgagtaagtcttgaggaccggttaaaagctttgccacattcttcacatttgtaaggtttctctccagtatgaattttcttatgttgagtaagtcttgaggacaggataaaagctttgccacattcttcacatttgtagggtttctctccactatgaatttttttatgactgttaaggtttgaggactgcttaaaggctttgccacattcttcacatttgtagggtttctctccagtatgaattctcctatggctagtaaggtgtgaggaccggttaaaagctttgccacattcgttacatttatagggtttctcttcagtatgaattctcttatgtctagtaagtgtagaggaataggtaaaaactttgccacattcttcacaattgtagggtttctctccagtatgaattttcttgtcttgagtaagtgttgaggaacaggtaaaaactctgccacatttttcaaatttgtagggttcctctccagtatgaatttttttatgtcgagtaagtcttgaagactggttaaaagctttgccacattcttcacatttgtagggcttctctccagtatgaattaccttatgtttagtaagagttgaagaccagttaaaggctttgccacattcttcacatttgtagggtttctcaccagtatgtattctcttatggctagtaagggttgaggaccggttaaaggctttgccacattctttacatttgtagggtttctcttcagtatgaattatcttatgtttagtaaaggttgaggatatgctaaaggttttgccacattcatcacatttgtagggcttctctccagaatgaattctcttatgggtagtaagggttgagtacctgctaaaggctttgccacattctttacatttgtagggtttctctccagtatgaattctcttatggttagtaagggttgagtagtggttaaatgctttgccacattcttcacatctgtagtgtttctcaccaacataaattctcttatggttagtaagggctgaggactgattaaaggcattgccaaattctttacatctgtaggtattctctctaatatgaattttcttatgttgagttagttgtgaaagcatgcaaaatgatttgccacattttttacactggaaaggtttctttccagtatgtcttgtcttgtatctatctgcatttgaaaatgcataaaagacttttacatatatatcacagtgatacattttgctctgggtaagtgtcaaacattggttaagtccattataacctcctttgtatagcttacaatcacctacagttttatagccttttcttaattgtaagttctcatgtccacgtttatcatatctcctcagtgtcactttttggaaagaatcttttatgtcttgctctggccaaaagtcttcagcaaaatgagaacacacaactgggggttcatccaccatttcatgtcgcttcatcttgcagggttctttttctttctctagacaagtgattaggtctggcttagaaacagcaatacccaggaagaccaagtttctgtagttctctaacatcacatttctatataagttctgttgtgctgtgtccaggcactgccactcctccagagagaattctatggccacatctgtaaatgtcaatggtcccagtaatgccaatgtttttgatccaaaaagaatattttgtcaaacattcagtaaatgaaggaagctgtgtttttcccagtttttttgtccttagaatcacatgaggcacttaattaaaacaacatggatgcttctatgcagaacttaaagagccaaagtggaatgggctcagtcatggtggatgggaggcaggactagattgcagctccgacttggacagagaagtgtgtggaggttcacagtgtgaattttagctccagattgactgcaagaacaaactagcaatcccaagaggacccacagaccatctgaaggaagcagactgctcctgcaggacctgagagacacccccaagtgggctgatacaaggttgtctgtcagaaattatttatttacaaaaaaaattgattattaattgggtatatatacatcgttaaggtttagagtatgggttatagtgcacagtgcagcactattaatttaatttatagccactggtggcaatagtaaacagtttcaagagataactacatagttcaaagaggaaagacgtaattgtgttctcattttaatgtctctctgagtttgacaactattaggttggtgcaaatgtaattctggtttttgccattacattaaaaggtaaaaccacaataacttttgccccgacctaacaagaggatttgcattcctcagataaaaggttttctgttctcactgatatgtgggagctaaactacgaaaacacaaaggcataggaatggtacaatggactttggggactttgggggaagagtgggagcagggcaagggatagaagactacaaatgggtgtagtgtaaactgcttgggtgatgggtgcacgaaaatctcacaaatcaccactaaagaacttatgcatgtaaccaaatactacctgtacaccagtgacttatggaaaaaaaaaagtcaaagtgaagaaacctctcttttcataacagattaaagtagcttctcaaaaacctgaaaaaaatagtaaaataaagtttacagaacaaacagaaggcagcaatgtctgaatgagtctgcatttgaaaaatagcatatgcacaggtactaatgcaatgtttgttaagcaggtactatgtgctcaagagtatgttacagagcactgtgctgggcataacatactgtgtgatttcatcctcataacaccctgggagttggtactaagtgtttaataattcccaggatttagataaaggacccagaattttaatttttctgtttctctgtcattgatttttaaaaaataaaatgtatagaataaaagctaaatatagacagatgagaggaatacagaaattaagagtttaatgtagtttagaggaatttttattgtgtttatatttaatttattgtgacttgtggagcaactactggatctgcaggaatagaaaacaagttgctaaatggaatgtcttggtaagcactgattttaataaaaaattaaaaatacgtatttttccacttatctgcttttgagtttcacgaaatcagagcaccagctctagaaaggtagcaaaatataccacccaaaactctgatctcttctaatcagttctgtgaggcaaggctccagagtggggccagaccaaaataaggcatccaaaaagggtgaatctgaacagaactgggccaaagagtggaccctgtgtagaattctgttctctatgccagtgggggtacttccagttctgtttttcctagacttacctaagaaaaacttaaattccagagtttgtgtaattttaattttttttagctactgtgctgtcaattttataacatatactaataagcaatttaagcaaatctcttaaggttttctagggtaattttattagaagataaatatatattcttaacaaggtaagaaaaatagaaataataataaaaattcttctgtccataaatatcccttcagctgatgacatcagaagttacaacaatgtaaagaaagtggcccaaataaagcccaagtttttttgcacacacgtattcattgtaccaaccatatgatgcttcattcaaccatttatccagttgatagtctaaaccaagagtttttggatggtagggaccatgactgcttcattttttttctaatggtcatattaatgaagcaattagtttatctgctttgagtctccagacctcctcctcgtcttttacccaaagtaccagaaaactagagaaactctcatctgggtaccaaccaaacacatctcttgtatgaggaaagaaacaaacacaagatgattcatttctcttacattgaaacagaagcggaattaaccactcttatcatcctgacacagttctgctctggacatcatcaaatgtctgaaatatacctagctaattgagagagggttcccagtgaccctgtgctgatggcccaataataagaaaggcagaagagactcaggctcattctaaatagaaaatggaactgccctggcagagctccagaacctggatcacccgtcctgatttgctagctcttgggtaagaggaaggacaagaatactcta

SEQ ID NO: 13100 - RNA, 2135 nt, Homo sapiens
  source 1..2135: mol_type = other RNA
gctgggattacaggcatgagccaccacacccatcctatgaattttcttatgttgagtaagtcttgaagaccgggtaaaagctttggcacattcttcacatttgtaaggtttctctctagtatgaattttcttatgttgagtaagtcttgaggaccgattaaaagctttgccacattcttcacatttgtagggtttctctccactatgaattttcttatgactactaaggtttgaggagtgggtaaaagctttgtcacattgtttacatttgtagggtttctctccagtatgaattttcttatgttgagtaagtcttgaggaccggttaaaagctttgccacattcttcacatttgtaaggtttctctccagtatgaattttcttatgttgagtaagtcttgaggacaggataaaagctttgccacattcttcacatttgtagggtttctctccactatgaatttttttatgactgttaaggtttgaggactgcttaaaggctttgccacattcttcacatttgtagggtttctctccagtatgaattctcctatggctagtaaggtgtgaggaccggttaaaagctttgccacattcgttacatttatagggtttctcttcagtatgaattctcttatgtctagtaagtgtagaggaataggtaaaaactttgccacattcttcacaattgtagggtttctctccagtatgaattttcttgtcttgagtaagtgttgaggaacaggtaaaaactctgccacatttttcaaatttgtagggttcctctccagtatgaatttttttatgtcgagtaagtcttgaagactggttaaaagctttgccacattcttcacatttgtagggcttctctccagtatgaattaccttatgtttagtaagagttgaagaccagttaaaggctttgccacattcttcacatttgtagggtttctcaccagtatgtattctcttatggctagtaagggttgaggaccggttaaaggctttgccacattctttacatttgtagggtttctcttcagtatgaattatcttatgtttagtaaaggttgaggatatgctaaaggttttgccacattcatcacatttgtagggcttctctccagaatgaattctcttatgggtagtaagggttgagtacctgctaaaggctttgccacattctttacatttgtagggtttctctccagtatgaattctcttatggttagtaagggttgagtagtggttaaatgctttgccacattcttcacatctgtagtgtttctcaccaacataaattctcttatggttagtaagggctgaggactgattaaaggcattgccaaattctttacatctgtaggtattctctctaatatgaattttcttatgttgagttagttgtgaaagcatgcaaaatgatttgccacattttttacactggaaaggtttctttccagtatgtcttgtcttgtatctatctgcatttgaaaatgcataaaagacttttacatatatatcacagtgatacattttgctctgggtaagtgtcaaacattggttaagtccattataacctcctttgtatagcttacaatcacctacagttttatagccttttcttaattgtaagttctcatgtccacgtttatcatatctcctcagtgtcactttttggaaagaatcttttatgtcttgctctggccaaaagtcttcagcaaaatgagaacacacaactgggggttcatccaccatttcatgtcgcttcatcttgcagggttctttttctttctctagacaagtgattaggtctggcttagaaacagcaatacccaggaagaccaagtttctgtagttctctaacatcacatttctatataagttctgttgtgctgtgtccaggcactgccactcctccagagagaattctatggccacatctgtaaatgtcaatggtcccatttctaggcttccagggggtcctggagtcttagctgtgtatctcccaatatctgcgggtcacagggccacacaggctgggcctctaagaacaaaggacacagaaatgaagacgagacctggagctctggctgcagcaagagccaaacgccccgccatattccggaaaccgt

SEQ ID NO: 13101 - RNA, 2158 nt, Homo sapiens
  source 1..2158: mol_type = other RNA
gctgggattacaggcatgagccaccacacccatcctatgaattttcttatgttgagtaagtcttgaagaccgggtaaaagctttggcacattcttcacatttgtaaggtttctctctagtatgaattttcttatgttgagtaagtcttgaggaccgattaaaagctttgccacattcttcacatttgtagggtttctctccactatgaattttcttatgactactaaggtttgaggagtgggtaaaagctttgtcacattgtttacatttgtagggtttctctccagtatgaattttcttatgttgagtaagtcttgaggaccggttaaaagctttgccacattcttcacatttgtaaggtttctctccagtatgaattttcttatgttgagtaagtcttgaggacaggataaaagctttgccacattcttcacatttgtagggtttctctccactatgaatttttttatgactgttaaggtttgaggactgcttaaaggctttgccacattcttcacatttgtagggtttctctccagtatgaattctcctatggctagtaaggtgtgaggaccggttaaaagctttgccacattcgttacatttatagggtttctcttcagtatgaattctcttatgtctagtaagtgtagaggaataggtaaaaactttgccacattcttcacaattgtagggtttctctccagtatgaattttcttgtcttgagtaagtgttgaggaacaggtaaaaactctgccacatttttcaaatttgtagggttcctctccagtatgaatttttttatgtcgagtaagtcttgaagactggttaaaagctttgccacattcttcacatttgtagggcttctctccagtatgaattaccttatgtttagtaagagttgaagaccagttaaaggctttgccacattcttcacatttgtagggtttctcaccagtatgtattctcttatggctagtaagggttgaggaccggttaaaggctttgccacattctttacatttgtagggtttctcttcagtatgaattatcttatgtttagtaaaggttgaggatatgctaaaggttttgccacattcatcacatttgtagggcttctctccagaatgaattctcttatgggtagtaagggttgagtacctgctaaaggctttgccacattctttacatttgtagggtttctctccagtatgaattctcttatggttagtaagggttgagtagtggttaaatgctttgccacattcttcacatctgtagtgtttctcaccaacataaattctcttatggttagtaagggctgaggactgattaaaggcattgccaaattctttacatctgtaggtattctctctaatatgaattttcttatgttgagttagttgtgaaagcatgcaaaatgatttgccacattttttacactggaaaggtttctttccagtatgtcttgtcttgtatctatctgcatttgaaaatgcataaaagacttttacatatatatcacagtgatacattttgctctgggtaagtgtcaaacattggttaagtccattataacctcctttgtatagcttacaatcacctacagttttatagccttttcttaattgtaagttctcatgtccacgtttatcatatctcctcagtgtcactttttggaaagaatcttttatgtcttgctctggccaaaagtcttcagcaaaatgagaacacacaactgggggttcatccaccatttcatgtcgcttcatcttgcagggttctttttctttctctagacaagtgattaggtctggcttagaaacagcaatacccaggaagaccaagtttctgtagttctctaacatcacatttctatataagttctgttgtgctgtgtccaggcactgccactcctccagagagaattctatggccacatctgtaaatgtcaatggtccctctcacattttaatgtgttcaatgaactgaagattttgttaatgcagattattttttcagaaaatctggaataaagtctgagttgctgaatttctaacaagctcaccagtaatgccaatgtttttgatccaaaaagaatattttgtcaaacattcagtaaatgaaggaagctgtgtttttcccagtttttttgtc

SEQ ID NO: 13102 - RNA, 2231 nt, Homo sapiens
  source 1..2231: mol_type = other RNA
gctgggattacaggcatgagccaccacacccatcctatgaattttcttatgttgagtaagtcttgaagaccgggtaaaagctttggcacattcttcacatttgtaaggtttctctctagtatgaattttcttatgttgagtaagtcttgaggaccgattaaaagctttgccacattcttcacatttgtagggtttctctccactatgaattttcttatgactactaaggtttgaggagtgggtaaaagctttgtcacattgtttacatttgtagggtttctctccagtatgaattttcttatgttgagtaagtcttgaggaccggttaaaagctttgccacattcttcacatttgtaaggtttctctccagtatgaattttcttatgttgagtaagtcttgaggacaggataaaagctttgccacattcttcacatttgtagggtttctctccactatgaatttttttatgactgttaaggtttgaggactgcttaaaggctttgccacattcttcacatttgtagggtttctctccagtatgaattctcctatggctagtaaggtgtgaggaccggttaaaagctttgccacattcgttacatttatagggtttctcttcagtatgaattctcttatgtctagtaagtgtagaggaataggtaaaaactttgccacattcttcacaattgtagggtttctctccagtatgaattttcttgtcttgagtaagtgttgaggaacaggtaaaaactctgccacatttttcaaatttgtagggttcctctccagtatgaatttttttatgtcgagtaagtcttgaagactggttaaaagctttgccacattcttcacatttgtagggcttctctccagtatgaattaccttatgtttagtaagagttgaagaccagttaaaggctttgccacattcttcacatttgtagggtttctcaccagtatgtattctcttatggctagtaagggttgaggaccggttaaaggctttgccacattctttacatttgtagggtttctcttcagtatgaattatcttatgtttagtaaaggttgaggatatgctaaaggttttgccacattcatcacatttgtagggcttctctccagaatgaattctcttatgggtagtaagggttgagtacctgctaaaggctttgccacattctttacatttgtagggtttctctccagtatgaattctcttatggttagtaagggttgagtagtggttaaatgctttgccacattcttcacatctgtagtgtttctcaccaacataaattctcttatggttagtaagggctgaggactgattaaaggcattgccaaattctttacatctgtaggtattctctctaatatgaattttcttatgttgagttagttgtgaaagcatgcaaaatgatttgccacattttttacactggaaaggtttctttccagtatgtcttgtcttgtatctatctgcatttgaaaatgcataaaagacttttacatatatatcacagtgatacattttgctctgggtaagtgtcaaacattggttaagtccattataacctcctttgtatagcttacaatcacctacagttttatagccttttcttaattgtaagttctcatgtccacgtttatcatatctcctcagtgtcactttttggaaagaatcttttatgtcttgctctggccaaaagtcttcagcaaaatgagaacacacaactgggggttcatccaccatttcatgtcgcttcatcttgcagggttctttttctttctctagacaagtgattaggtctggcttagaaacagcaatacccaggaagaccaagtttctgtagttctctaacatcacatttctatataagttctgttgtgctgtgtccaggcactgccactcctccagagagaattctatggccacatctgtaaatgtcaatggtccctgacgcccctcccatggttcttgcacaatctgggagagactgcggaattgcgcgtgcagagctccccagacagggctacacgtcaggcacagtcacatttctaggcttccagggggtcctggagtcttagctgtgtatctcccaatatctgcgggtcacagggccacacaggctgggcctctaagaacaaaggacacagaaatgaagacgagacctggagctctggctgcagcaagagccaaacgccccgccatattccggaaaccgt

SEQ ID NO: 13103 - RNA, 2441 nt, Homo sapiens
  source 1..2441: mol_type = other RNA
gctgggattacaggcatgagccaccacacccatcctatgaattttcttatgttgagtaagtcttgaagaccgggtaaaagctttggcacattcttcacatttgtaaggtttctctctagtatgaattttcttatgttgagtaagtcttgaggaccgattaaaagctttgccacattcttcacatttgtagggtttctctccactatgaattttcttatgactactaaggtttgaggagtgggtaaaagctttgtcacattgtttacatttgtagggtttctctccagtatgaattttcttatgttgagtaagtcttgaggaccggttaaaagctttgccacattcttcacatttgtaaggtttctctccagtatgaattttcttatgttgagtaagtcttgaggacaggataaaagctttgccacattcttcacatttgtagggtttctctccactatgaatttttttatgactgttaaggtttgaggactgcttaaaggctttgccacattcttcacatttgtagggtttctctccagtatgaattctcctatggctagtaaggtgtgaggaccggttaaaagctttgccacattcgttacatttatagggtttctcttcagtatgaattctcttatgtctagtaagtgtagaggaataggtaaaaactttgccacattcttcacaattgtagggtttctctccagtatgaattttcttgtcttgagtaagtgttgaggaacaggtaaaaactctgccacatttttcaaatttgtagggttcctctccagtatgaatttttttatgtcgagtaagtcttgaagactggttaaaagctttgccacattcttcacatttgtagggcttctctccagtatgaattaccttatgtttagtaagagttgaagaccagttaaaggctttgccacattcttcacatttgtagggtttctcaccagtatgtattctcttatggctagtaagggttgaggaccggttaaaggctttgccacattctttacatttgtagggtttctcttcagtatgaattatcttatgtttagtaaaggttgaggatatgctaaaggttttgccacattcatcacatttgtagggcttctctccagaatgaattctcttatgggtagtaagggttgagtacctgctaaaggctttgccacattctttacatttgtagggtttctctccagtatgaattctcttatggttagtaagggttgagtagtggttaaatgctttgccacattcttcacatctgtagtgtttctcaccaacataaattctcttatggttagtaagggctgaggactgattaaaggcattgccaaattctttacatctgtaggtattctctctaatatgaattttcttatgttgagttagttgtgaaagcatgcaaaatgatttgccacattttttacactggaaaggtttctttccagtatgtcttgtcttgtatctatctgcatttgaaaatgcataaaagacttttacatatatatcacagtgatacattttgctctgggtaagtgtcaaacattggttaagtccattataacctcctttgtatagcttacaatcacctacagttttatagccttttcttaattgtaagttctcatgtccacgtttatcatatctcctcagtgtcactttttggaaagaatcttttatgtcttgctctggccaaaagtcttcagcaaaatgagaacacacaactgggggttcatccaccatttcatgtcgcttcatcttgcagggttctttttctttctctagacaagtgattaggtctggcttagaaacagcaatacccaggaagaccaagtttctgtagttctctaacatcacatttctatataagttctgttgtgctgtgtccaggcactgccactcctccagagagaattctatggccacatctgtaaatgtcaatggtccctgacgcccctcccatggttcttgcacaatctgggagagactgcggaattgcgcgtgcagagctccccagacagggctacacgtcaggcacagtcactgcggagggaagacaggacgcccggggcccggctgtcagcacagtcgccatcttatggctgaaggggactgaagccgagctgggcaaggagaattccgggcgcagattgtggagctgactgccgggagacctaagtccgccacggccacttctcacggttccgaccagcccctccccctctctggggatgtcagactcggcactctcaccatttctaggcttccagggggtcctggagtcttagctgtgtatctcccaatatctgcgggtcacagggccacacaggctgggcctctaagaacaaaggacacagaaatgaagacgagacctggagctctggctgcagcaagagccaaacgccccgccatattccggaaaccgt

SEQ ID NO: 13104 - RNA, 2431 nt, Homo sapiens
  source 1..2431: mol_type = other RNA
gctgggattacaggcatgagccaccacacccatcctatgaattttcttatgttgagtaagtcttgaagaccgggtaaaagctttggcacattcttcacatttgtaaggtttctctctagtatgaattttcttatgttgagtaagtcttgaggaccgattaaaagctttgccacattcttcacatttgtagggtttctctccactatgaattttcttatgactactaaggtttgaggagtgggtaaaagctttgtcacattgtttacatttgtagggtttctctccagtatgaattttcttatgttgagtaagtcttgaggaccggttaaaagctttgccacattcttcacatttgtaaggtttctctccagtatgaattttcttatgttgagtaagtcttgaggacaggataaaagctttgccacattcttcacatttgtagggtttctctccactatgaatttttttatgactgttaaggtttgaggactgcttaaaggctttgccacattcttcacatttgtagggtttctctccagtatgaattctcctatggctagtaaggtgtgaggaccggttaaaagctttgccacattcgttacatttatagggtttctcttcagtatgaattctcttatgtctagtaagtgtagaggaataggtaaaaactttgccacattcttcacaattgtagggtttctctccagtatgaattttcttgtcttgagtaagtgttgaggaacaggtaaaaactctgccacatttttcaaatttgtagggttcctctccagtatgaatttttttatgtcgagtaagtcttgaagactggttaaaagctttgccacattcttcacatttgtagggcttctctccagtatgaattaccttatgtttagtaagagttgaagaccagttaaaggctttgccacattcttcacatttgtagggtttctcaccagtatgtattctcttatggctagtaagggttgaggaccggttaaaggctttgccacattctttacatttgtagggtttctcttcagtatgaattatcttatgtttagtaaaggttgaggatatgctaaaggttttgccacattcatcacatttgtagggcttctctccagaatgaattctcttatgggtagtaagggttgagtacctgctaaaggctttgccacattctttacatttgtagggtttctctccagtatgaattctcttatggttagtaagggttgagtagtggttaaatgctttgccacattcttcacatctgtagtgtttctcaccaacataaattctcttatggttagtaagggctgaggactgattaaaggcattgccaaattctttacatctgtaggtattctctctaatatgaattttcttatgttgagttagttgtgaaagcatgcaaaatgatttgccacattttttacactggaaaggtttctttccagtatgtcttgtcttgtatctatctgcatttgaaaatgcataaaagacttttacatatatatcacagtgatacattttgctctgggtaagtgtcaaacattggttaagtccattataacctcctttgtatagcttacaatcacctacagttttatagccttttcttaattgtaagttctcatgtccacgtttatcatatctcctcagtgtcactttttggaaagaatcttttatgtcttgctctggccaaaagtcttcagcaaaatgagaacacacaactgggggttcatccaccatttcatgtcgcttcatcttgcagggttctttttctttctctagacaagtgattaggtctggcttagaaacagcaatacccaggaagaccaagtttctgtagttctctaacatcacatttctatataagttctgttgtgctgtgtccaggcactgccactcctccagagagaattctatggccacatctgtaaatgtcaatggtccctttagtgcaaaggtggaactctcatgaatgtgtcttgaagctttcatacttgattctggcctcaccttagaatcacatgaggcacttaattaaaacaacatggatgcttctatgcagaaccatttctaggcttccagggggtcctggagtcttagctgtgtatctcccaatatctgcgggtcacagggccacacaggctgggcctctaagaacaaaggacacagaaatgaagacgagacctggagctctggctgcagcaagagccaaacgccccgccatattccggaaaccgtcctgtcgctccagctgcgtgcctgattggataatgtttaagacccgccctctcaggccctgagtgacagagggtgatcagttgctgggcagaatgaagcgtgacagcctagctgcagccttttcaggcaggctttcctccgagctgagccaggcccaccctagagggtgtttgca

SEQ ID NO: 13105 - RNA, 4515 nt, Homo sapiens
  source 1..4515: mol_type = other RNA
gctgggattacaggcatgagccaccacacccatcctatgaattttcttatgttgagtaagtcttgaagaccgggtaaaagctttggcacattcttcacatttgtaaggtttctctctagtatgaattttcttatgttgagtaagtcttgaggaccgattaaaagctttgccacattcttcacatttgtagggtttctctccactatgaattttcttatgactactaaggtttgaggagtgggtaaaagctttgtcacattgtttacatttgtagggtttctctccagtatgaattttcttatgttgagtaagtcttgaggaccggttaaaagctttgccacattcttcacatttgtaaggtttctctccagtatgaattttcttatgttgagtaagtcttgaggacaggataaaagctttgccacattcttcacatttgtagggtttctctccactatgaatttttttatgactgttaaggtttgaggactgcttaaaggctttgccacattcttcacatttgtagggtttctctccagtatgaattctcctatggctagtaaggtgtgaggaccggttaaaagctttgccacattcgttacatttatagggtttctcttcagtatgaattctcttatgtctagtaagtgtagaggaataggtaaaaactttgccacattcttcacaattgtagggtttctctccagtatgaattttcttgtcttgagtaagtgttgaggaacaggtaaaaactctgccacatttttcaaatttgtagggttcctctccagtatgaatttttttatgtcgagtaagtcttgaagactggttaaaagctttgccacattcttcacatttgtagggcttctctccagtatgaattaccttatgtttagtaagagttgaagaccagttaaaggctttgccacattcttcacatttgtagggtttctcaccagtatgtattctcttatggctagtaagggttgaggaccggttaaaggctttgccacattctttacatttgtagggtttctcttcagtatgaattatcttatgtttagtaaaggttgaggatatgctaaaggttttgccacattcatcacatttgtagggcttctctccagaatgaattctcttatgggtagtaagggttgagtacctgctaaaggctttgccacattctttacatttgtagggtttctctccagtatgaattctcttatggttagtaagggttgagtagtggttaaatgctttgccacattcttcacatctgtagtgtttctcaccaacataaattctcttatggttagtaagggctgaggactgattaaaggcattgccaaattctttacatctgtaggtattctctctaatatgaattttcttatgttgagttagttgtgaaagcatgcaaaatgatttgccacattttttacactggaaaggtttctttccagtatgtcttgtcttgtatctatctgcatttgaaaatgcataaaagacttttacatatatatcacagtgatacattttgctctgggtaagtgtcaaacattggttaagtccattataacctcctttgtatagcttacaatcacctacagttttatagccttttcttaattgtaagttctcatgtccacgtttatcatatctcctcagtgtcactttttggaaagaatcttttatgtcttgctctggccaaaagtcttcagcaaaatgagaacacacaactgggggttcatccaccatttcatgtcgcttcatcttgcagggttctttttctttctctagacaagtgattaggtctggcttagaaacagcaatacccaggaagaccaagtttctgtagttctctaacatcacatttctatataagttctgttgtgctgtgtccaggcactgccactcctccagagagaattctatggccacatctgtaaatgtcaatggtccctttagtgcaaaggtggaactctcatgaatgtgtcttgaagctttcatacttgattctggcctcaccttagaatcacatgaggcacttaattaaaacaacatggatgcttctatgcagaacttaaagagccaaagtggaatgggctcagtcatggtggatgggaggcaggactagattgcagctccgacttggacagagaagtgtgtggaggttcacagtgtgaattttagctccagattgactgcaagaacaaactagcaatcccaagaggacccacagaccatctgaaggaagcagactgctcctgcaggacctgagagacacccccaagtgggctgatacaaggttgtctgtcagaaattatttatttacaaaaaaaattgattattaattgggtatatatacatcgttaaggtttagagtatgggttatagtgcacagtgcagcactattaatttaatttatagccactggtggcaatagtaaacagtttcaagagataactacatagttcaaagaggaaagacgtaattgtgttctcattttaatgtctctctgagtttgacaactattaggttggtgcaaatgtaattctggtttttgccattacattaaaaggtaaaaccacaataacttttgccccgacctaacaagaggatttgcattcctcagataaaaggttttctgttctcactgatatgtgggagctaaactacgaaaacacaaaggcataggaatggtacaatggactttggggactttgggggaagagtgggagcagggcaagggatagaagactacaaatgggtgtagtgtaaactgcttgggtgatgggtgcacgaaaatctcacaaatcaccactaaagaacttatgcatgtaaccaaatactacctgtacaccagtgacttatggaaaaaaaaaagtcaaagtgaagaaacctctcttttcataacagattaaagtagcttctcaaaaacctgaaaaaaatagtaaaataaagtttacagaacaaacagaaggcagcaatgtctgaatgagtctgcatttgaaaaatagcatatgcacaggtactaatgcaatgtttgttaagcaggtactatgtgctcaagagtatgttacagagcactgtgctgggcataacatactgtgtgatttcatcctcataacaccctgggagttggtactaagtgtttaataattcccaggatttagataaaggacccagaattttaatttttctgtttctctgtcattgatttttaaaaaataaaatgtatagaataaaagctaaatatagacagatgagaggaatacagaaattaagagtttaatgtagtttagaggaatttttattgtgtttatatttaatttattgtgacttgtggagcaactactggatctgcaggaatagaaaacaagttgctaaatggaatgtcttggtaagcactgattttaataaaaaattaaaaatacgtatttttccacttatctgcttttgagtttcacgaaatcagagcaccagctctagaaaggtagcaaaatataccacccaaaactctgatctcttctaatcagttctgtgaggcaaggctccagagtggggccagaccaaaataaggcatccaaaaagggtgaatctgaacagaactgggccaaagagtggaccctgtgtagaattctgttctctatgccagtgggggtacttccagttctgtttttcctagacttacctaagaaaaacttaaattccagagtttgtgtaattttaattttttttagctactgtgctgtcaattttataacatatactaataagcaatttaagcaaatctcttaaggttttctagggtaattttattagaagataaatatatattcttaacaaggtaagaaaaatagaaataataataaaaattcttctgtccataaatatcccttcagctgatgacatcagaagttacaacaatgtaaagaaagtggcccaaataaagcccaagtttttttgcacacacgtattcattgtaccaaccatatgatgcttcattcaaccatttatccagttgatagtctaaaccaagagtttttggatggtagggaccatgactgcttcattttttttctaatggtcatattaatgaagcaattagtttatctgctttgagtctccagacctcctcctcgtcttttacccaaagtaccagaaaactagagaaactctcatctgggtaccaaccaaacacatctcttgtatgaggaaagaaacaaacacaagatgattcatttctcttacattgaaacagaagcggaattaaccactcttatcatcctgacacagttctgctctggacatcatcaaatgtctgaaatatacctagctaattgagagagggttcccagtgaccctgtgctgatggcccaataataagaaaggcagaagagactcaggctcattctaaatagaaaatggaactgccctggcagagctccagaacctggatcacccgtcctgatttgctagctcttgggtaagaggaaggacaagaatactcta

SEQ ID NO: 13106 - RNA, 1672 nt, Homo sapiens
  source 1..1672: mol_type = other RNA
gctgggattacaggcatgagccaccacaccccgcccttatgtttgaaatatttttaaaataaagtttaaaatattaaataaacaaaaataaagatcaaatgaaagacagtcaagttcctgggaagcccactgcagatgcagatagcagaggcctggatggacctgcagtatcttggcagggcctatggcaaaccagaaagggctagcgttgaaacccaggttctaaatggctttattttttccatgactttttcctcctaatattcaatgtccttgcaagactgatggatcctagggtttgaatccacaaagaatcaaaaatgcagtttatggtctgaccaagggactgaagaaagcctgcggttgatcctggtgaccccccgattggcgtttacagtgcagccatgccatggctgggggacatggctcaagatggagtccctcctctcatgatccagccacaaaggcttgcctgagtccttgggaaggttccagatcaggcttcccgtcagacgctgtcctcacctccgatgatctgctccaatggcatctgtgactccgccaaagccctgctctttcagaagggcctccagttcccgcttgactttgcccacaacgggtggcccccagaaggtgagggccgtgtacagctgcaccagggaggcccctgcccggatcttctccagcgcgtcctgcccgctgctcacaccaccaaccccaattatgggaactcggccttgggtgagtgcatacatctcccgaatggtttgagttgataaatcccggaggggcttcccactcagccctcctgtttcagagcgcagggcaccctggaggcccgcagggcgactcacggtggtgttcgtaacaatcagcccatcgatgcccaactctttgaccacactggcaatgtcctccttatcctggctggtgaggtcaggagcgatcttcaccaggactgccggcctgtgcactctccgcaagccatccctctcctgcagcaccttggtcagcaggcggcgcagctcggcctttccctgaaggctccgcagcccggcagtgttggggctggacacattcaccaccaggtagtcggccagggggcccagtacgcgcaccccttctgcgtagtcctccgcggcgtccactgaggtcttgttcttccccaagttgacccccagaggcagtccatcttctgtgagcttggcctgcttctgctgtctggcccgtaacctgtgttccaccactgaaagcccgtgactgttaaatccataccacatgccacacaaccaggaggccgcacacacagggctcagagcaggatctcacacccctgctcacctataggattcaccaagtaccatcatcccagcacctgcagttatctgtagcagctgaatgttaagcaaatatattttgcctggccaattctgaagatattgatccccacctgttaatgacagcttggtcctcagggaggcggaagactctgggtctagggtttccttcctgaggttttggagtcacacttcctatctcaacaaaaccaaagcccatcttataaagtccgtccacggcttccccatgcttgtcaaatcctgcagcaattcctactggatttcggaatttatggcccagaactctcacttcctgggaagaggaagacaaagtc

SEQ ID NO: 13107 - RNA, 2035 nt, Homo sapiens
  source 1..2035: mol_type = other RNA
gctgggattacaggcatgagccaccacaccccgcccttatgtttgaaatatttttaaaataaagtttaaaatattaaataaacaaaaataaagatcaaatgaaagacagtcaagttcctgggaagcccactgcagatgcagatagcagaggcctggatggacctgcagtatcttggcagggcctatggcaaaccagaaagggctagcgttgaaacccaggttctaaatggctttattttttccatgactttttcctcctaatattcaatgtccttgcaagactgatggatcctagggtttgaatccacaaagaatcaaaaatgcagtttatggtctgaccaagggactgaagaaagcctgcggttgatcctggtgaccccccgattggcgtttacagtgcagccatgccatggctgggggacatggctcaagatggagtccctcctctcatgatccagccacaaaggcttgcctgagtccttgggaaggttccagatcaggcttcccgtcagacgctgtcctcacctccgatgatctgctccaatggcatctgtgactccgccaaagccctgctctttcagaagggcctccagttcccgcttgactttgcccacaacgggtggcccccagaaggtgagggccgtgtacagctgcaccagggaggcccctgcccggatcttctccagcgcgtcctgcccgctgctcacaccaccaaccccaattatgggaactcggccttgggtgagtgcatacatctcccgaatggtttgagttgataaatcccggaggggcttcccactcagccctcctgtttcagagcgcagggcaccctggaggcccgcagggcgactcacggtggtgttcgtaacaatcagcccatcgatgcccaactctttgaccacactggcaatgtcctccttatcctggctggtgaggtcaggagcgatcttcaccaggactgccggcctgtgcactctccgcaagccatccctctcctgcagcaccttggtcagcaggcggcgcagctcggcctttccctgaaggctccgcagcccggcagtgttggggctggacacattcaccaccaggtagtcggccagggggcccagtacgcgcaccccttctgcgtagtcctccgcggcgtccactgaggtcttgttcttccccaagttgacccccagaggcagtccatcttctgtgagcttggcctgcttctgctgtctggcccgtaacctgtgttccaccactgaaagcccgtgactgttaaatccatacctgttaatgacagcttggtcctcagggaggcggaagactctgggtctagggtttccttcctgaggttttggagtcacacttcctatctcaacaaaaccaaagcccatcttataaagtccgtccacggcttccccatgcttgtcaaatcctgcagcaattcctactggatttcggaatttatggcccagaactctcacttccagcatgtcagagtcttgaaatctggcccgtggaaggagccccagggaggtgaagcgaacagccagtctgtgggctgactccgggtccagcagcccctgcagagtcggcatcaggtgttcagcatagaaacgctcatctcccgtggccatcaggtaggaggcgaagagaagtcctcctccccccaggatgatcacagcatcctgggcccgcttctaaaagggttgggagcatgtcctactctagtttcattccccgttggatccggcacacaacgctaggcggtcatgtgttcactaagcacccctgtgccaggctcaaaaacatggcccaggcgcagacactcagatcagcacccacccagacctgcaggcgctgtctgcacacgcctgaccgagtccacgtgcaaatgcacacgcacgagcatttgcaggagaccccggaaacacgcacacgtcccaggggggcccacactcccggagccgccttcggtccatgcctcgcccggcctgactctccgttctcgccctccccggtccctggtcccccatccacactgctc

SEQ ID NO: 13108 - RNA, 1730 nt, Homo sapiens
  source 1..1730: mol_type = other RNA
gctgggattacaggcatgagccaccacaccccgcccttatgtttgaaatatttttaaaataaagtttaaaatattaaataaacaaaaataaagatcaaatgaaagacagtcaagttcctgggaagcccactgcagatgcagatagcagaggcctggatggacctgcagtatcttggcagggcctatggcaaaccagaaagggctagcgttgaaacccaggttctaaatggctttattttttccatgactttttcctcctaatattcaatgtccttgcaagactgatggatcctagggtttgaatccacaaagaatcaaaaatgcagtttatggtctgaccaagggactgaagaaagcctgcggttgatcctggtgaccccccgattggcgtttacagtgcagccatgccatggctgggggacatggctcaagatggagtccctcctctcatgatccagccacaaaggcttgcctgagtccttgggaaggttccagatcaggcttcccgtcagacgctgtcctcacctccgatgatctgctccaatggcatctgtgactccgccaaagccctgctctttcagaagggcctccagttcccgcttgactttgcccacaacgggtggcccccagaaggtgagggccgtgtacagctgcaccagggaggcccctgcccggatcttctccagcgcgtcctgcccgctgctcacaccaccaaccccaattatgggaactcggccttgggtgagtgcatacatctcccgaatggtttgagttgataaatcccggaggggcttcccactcagccctcctgtttcagagcgcagggcaccctggaggcccgcagggcgactcacggtggtgttcgtaacaatcagcccatcgatgcccaactctttgaccacactggcaatgtcctccttatcctggctggtgaggtcaggagcgatcttcaccaggactgccggcctgtgcactctccgcaagccatccctctcctgcagcaccttggtcagcaggcggcgcagctcggcctttccctgaaggctccgcagcccggcagtgttggggctggacacattcaccaccaggtagtcggccagggggcccagtacgcgcaccccttctgcgtagtcctccgcggcgtccactgaggtcttgttcttccccaagttgacccccagaggcagtccatcttctgtgagcttggcctgcttctgctgtctggcccgtaacctgtgttccaccactgaaagcccgtgactgttaaatccatacctgttaatgacagcttggtcctcagggaggcggaagactctgggtctagggtttccttcctgaggttttggagtcacacttcctatctcaacaaaaccaaagcccatcttataaagtccgtccacggcttccccatgcttgtcaaatcctgcagcaattcctactggatttcggaatttatggcccagaactctcacttccagcatgtcagagtcttgaaatctggcccgtggaaggagccccagggaggtgaagcgaacagccagtctgtgggctgactccgggtccagcagcccctgcagagtcggcatcaggtgttcagcatagaaacgctcatctcccgtggccatcaggtaggaggcgaagagaagtcctcctccccccaggatgatcacagcatcctgggcccgctttttcaggtgtctccacgccatgctccttccgtcattaagccc

SEQ ID NO: 13109 - RNA, 1810 nt, Homo sapiens
  source 1..1810: mol_type = other RNA
gctgggattacaggcatgagccaccacaccccgcccttatgtttgaaatatttttaaaataaagtttaaaatattaaataaacaaaaataaagatcaaatgaaagacagtcaagttcctgggaagcccactgcagatgcagatagcagaggcctggatggacctgcagtatcttggcagggcctatggcaaaccagaaagggctagcgttgaaacccaggttctaaatggctttattttttccatgactttttcctcctaatattcaatgtccttgcaagactgatggatcctagggtttgaatccacaaagaatcaaaaatgcagtttatggtctgaccaagggactgaagaaagcctgcggttgatcctggtgaccccccgattggcgtttacagtgcagccatgccatggctgggggacatggctcaagatggagtccctcctctcatgatccagccacaaaggcttgcctgagtccttgggaaggttccagatcaggcttcccgtcagacgctgtcctcacctccgatgatctgctccaatggcatctgtgactccgccaaagccctgctctttcagaagggcctccagttcccgcttgactttgcccacaacgggtggcccccagaaggtgagggccgtgtacagctgcaccagggaggcccctgcccggatcttctccagcgcgtcctgcccgctgctcacaccaccaaccccaattatgggaactcggccttgggtgagtgcatacatctcccgaatggtttgagttgataaatcccggaggggcttcccactcagccctcctgtttcagagcgcagggcaccctggaggcccgcagggcgactcacggtggtgttcgtaacaatcagcccatcgatgcccaactctttgaccacactggcaatgtcctccttatcctggctggtgaggtcaggagcgatcttcaccaggactgccggcctgtgcactctccgcaagccatccctctcctgcagcaccttggtcagcaggcggcgcagctcggcctttccctgaaggctccgcagcccggcagtgttggggctggacacattcaccaccaggtagtcggccagggggcccagtacgcgcaccccttctgcgtagtcctccgcggcgtccactgaggtcttgttcttccccaagttgacccccagaggcagtccatcttctgtgagcttggcctgcttctgctgtctggcccgtaacctgtgttccaccactgaaagcccgtgactgttaaatccatacctgttaatgacagcttggtcctcagggaggcggaagactctgggtctagggtttccttcctgaggttttggagtcacacttcctatctcaacaaaaccaaagcccatcttataaagtccgtccacggcttccccatgcttgtcaaatcctgcagcaattcctactggatttcggaatttatggcccagaactctcacttcttggggttctggttttcaaaaagatcagtcccagctgagaagtttaggggactgcagccttcgcctttgtatttaatgtatagggtgtctgggagcactaccagcatgtcagagtcttgaaatctggcccgtggaaggagccccagggaggtgaagcgaacagccagtctgtgggctgactccgggtccagcagcccctgcagagtcggcatcaggtgttcagcatagaaacgctcatctcccgtggccatcaggtaggaggcgaagagaagtcctcctccccccaggatgatcacagcatcctgggcccgctttttcaggtgtctccacgccat

SEQ ID NO: 13110 - RNA, 1580 nt, Homo sapiens
  source 1..1580: mol_type = other RNA
gctgggattacaggcatgagccaccacaccccgctaggagttcacactttagttggggaaaatatacaataagcaagccaatttttaaaatgagaacttcagagttaaatgctacaaagacaatctcacaggaagttgcgatgtagaatgatagggctctcagaatagtaagagaaactattatttcttacgatgtttgtctttctttgtatcggtgctcagctgagtctgcagtgcttcggaggcagctttcattttataaaaatctatgatttctccttccagttgttttttctcttcctcgagcttccttatctcctcctgttgaatcattttaagatgctcgaacttgtcctgcagctctttttcagcttctttaaatgttgcttctttctccttgactcgctgcataaatctctgtttcaactcttcttcttccctctgacattgatcatagaactcttgtcttttggcttcaaagatttcttgaaaactaactggctggttgtttggacccacatctgtaaagcccattttctgcagtttttggtacctataacattcatagtgctgagtgtgggttttttcttttagattttccatattggtacaaagaagcatatctcggagcttaacgaagtcacagtgattttcattttccacttgcaaaactccccaagggtagtgacggcctctgaccatcctttttccaactttcacttcatctgtactccctaccacagcaaagggtaacagcccactaactgaggagttcgcttgagcagcagtttcttcatctgttgggagctgatatatctggatgccattgctaatcaattcactcattatcttattcttaaacgtctgtaaatcatttttagaaatagtgtctgctttggcaatcagtggtataatattcaccttactgtcaaggttcttcattgttaatagatcaagagacttcagggaatgtcctgtaggtgaaatgaagtaaagacacacgtggacgcgagaatcatggtactcaaacaaggaacgtttaatcttcagttcttcttgaagataggcctcaaattgggcatctatgtagtcaactattggttggtagctggcttctttgtctatttgatcaccataccctactgtctccacaacagtcaatttcaactgaacattgctttcctgaagttcatatgtctgaatttgaagtccaacatttgagtaaaaatgtgaggatttgttatctttcaagttagtattaaacaatgtgtctatcagtgtcgattttccaattccagtctcccccacacagagaatattaaaagtgaatccttgtcggatagatctgctcaccaactgattgggcaaacattcaaaaccaaaatgtccaatcgtagttaaacaacgaatattattttctttttgtgtatctccatcagcaggtatttgtgtgggcatagccattgttctttctgccatgctacactaaaagagctctgttagtcctcatagtagatctgagatgtatgtattttcattgccatatgccaggtgaaaaaattcagactcagaaagattaa

SEQ ID NO: 13111 - RNA, 1559 nt, Homo sapiens
  source 1..1559: mol_type = other RNA
gctgggattacaggcatgagccaccacaccccgctaggagttcacactttagttggggaaaatatacaataagcaagccaatttttaaaatgagaacttcagagttaaatgctacaaagacaatctcacaggaagttgcgatgtagaatgatagggctctcagaatagtaagagaaactattatttcttacgatgtttgtctttctttgtatcggtgctcagctgagtctgcagtgcttcggaggcagctttcattttataaaaatctatgatttctccttccagttgttttttctcttcctcgagcttccttatctcctcctgttgaatcattttaagatgctcgaacttgtcctgcagctctttttcagcttctttaaatgttgcttctttctccttgactcgctgcataaatctctgtttcaactcttcttcttccctctgacattgatcatagaactcttgtcttttggcttcaaagatttcttgaaaactaactggctggttgtttggacccacatctgtaaagcccattttctgcagtttttggtacctataacattcatagtgctgagtgtgggttttttcttttagattttccatattggtacaaagaagcatatctcggagcttaacgaagtcacagtgattttcattttccacttgcaaaactccccaagggtagtgacggcctctgaccatcctttttccaactttcacttcatctgtactccctaccacagcaaagggtaacagcccactaactgaggagttcgcttgagcagcagtttcttcatctgttgggagctgatatatctggatgccattgctaatcaattcactcattatcttattcttaaacgtctgtaaatcatttttagaaatagtgtctgctttggcaatcagtggtataatattcaccttactgtcaaggttcttcattgttaatagatcaagagacttcagggaatgtcctgtaggtgaaatgaagtaaagacacacgtggacgcgagaatcatggtactcaaacaaggaacgtttaatcttcagttcttcttgaagataggcctcaaattgggcatctatgtagtcaactattggttggtagctggcttctttgtctatttgatcaccataccctactgtctccacaacagtcaatttcaactgaacattgctttcctgaagttcatatgtctgaatttgaagtccaacatttgagtaaaaatgtgaggatttgttatctttcaagttagtattaaacaatgtgtctatcagtgtcgattttccaattccagtctcccccacacagagaatattaaaagtgaatccttgtcggatagatctgctcaccaactgattgggcaaacattcaaaaccaaaatgtccaatcgtagttaaacaacgaatattattttctttttgtgtatctccatcagcaggtatttgtgtgggcatagccattgttctttctgccatgctacactaaaagagtttcccagggattcagctgtgcagcagacacaggtccgaactgattccaagctggtgtcctttct

SEQ ID NO: 13112 - RNA, 4082 nt, Homo sapiens
  source 1..4082: mol_type = other RNA
gctgggattacaggcatgagccaccacacccggcaatttcctggttttgataaactacagtatggctttgtaggatgtaatcattgggagatgctagatgaaagatacatgggaattttctactatttctgcaactttctctaagtctaaaattatttcaaaacaaaaagtaaaaaacaatgaaaagcaggccgggtccagtggctcatgcctgtaatcccagcactttgggaggccgaggcaggcagatcacaaggtcaggagattgagaccatcctggctaacatggtgaaaccctgtctctactaaaaatacaaaaaggtagccgggcgtggtggtgggcacctgtagtcccagctactcgggaggctgaggcaggagaatggcgtgaacctgggaggcagggcttgcagtgagccgagatcgcgccactgcactccagcttgggggacagagtgagactctgtctcaaaaaaaaaaaaaaaaaaaaaaaggcagtcagtgaggtagggagcagcagcccctgaggggtagacagtgatccaagcatctgctggagctcacaccctggattctgactgcctcatacccaccatactgttaggacatgcttccattacccaagggactttgattcctggccccattctctgcttcctgaaagactagctaacactacgcgagggttccatgaagggcctgtgggggaaggtgggtggactgcttatcagcagtggctactgtagatggtgcccaaggatgcaccaggccttactgtgcctggctaaggtgggcttgaaacattggctggtctgtgaaatgcccttgggggacggtgtccagaccctctgctttgtgactaacatgcagactgaataaactgcatgtttattccaggctcgtttagctggacgagcagtacagacagggctgaggctgactccatggccatgtgggcagaggtcaaacccatgatctctcttcctacagcttcctaatgtctgcgatgttggtcttttgaaggaggcccccacagagctgagcttgcttggttatctgggactgctgctcagtctgagtaggggagggtaatgaaccagtcaggcctcctcctggaggtgcccaacactggcctagtccccaaggctgacgaaacatggtctggcctgaccccaggacgtggggtgaggaggaacactgggcataatatagtagcggaaacaggcaagcctctatgggtcccttccccttagaattttagggtagggaacgaggaggctacagactaaattgcagaactatctgcacctgggcctctgagctcttcctccactcccagtggagccattctggggactgagttgcatgaggactagcagagggtggcagttcagtctggtccctgtcttcttccagccagctgtgttcttagctgccatacttctgagcttcctgggaacatgagaaagtctggcgactatgggggatggggatcattctgaaggaaataagggacctccatccctccttgccttgaagggggtggaaaggcagctcctctcctgaaggcttgttagcaggttatgggcccacaacaaaggggccagagtagggcgaaattcctccttcaggttttggggctgagaaggggtcttcatgggctgtgaggaggtaagcaggcctgagactgggtagagatgggagcggcatgaggggaaggtaagtcagttgccatgccacagccaaggggcctttattggatggtgagggcacataggagcaggcaggtggctgctagatggtgttgcacaccttctcagggtgcagtggtgcccggatgtccagtctgcgagtcttgctgtccttgtcgatgatctccagacgcagcttggggaggcgcttctcagcctggggtgagggcagttctgggcttttgagtagctgcttgtctgagtcctccaccgtgatgcgcaaagtacagccccctggcagcaggtcctgctcataggctgctgccagctggttcaccacacggcgttctacctcatgtttgatggagcgggcgccatagtgcacattgtagccgtcgaccagcacatctgccacctcgcggtcccagagcagcgtgatgttgtgcctttgcttggctctcttggcccagaagtttagttccttgttgacgagttggatgagctccgagtggcagaaggggaggaagtagacgatctcattgatccgtcccagaaactcatccctccggaagtgagctttcaggatagggcgaatcacattctccttgaagttctttgagatggtgatcttgtcacttatctggacatcccccaggttttcggcaatacggttacggctcatctccaaagcttcctgcctcagctgcagcgcgtgctgtgcgatctcgtcgctggccacattggaggtcatgatgaagatggcgtccttgcaatcaatggtcttcccttttccatctgtcagccggccctcatcaaacagctgcagcatgatggtgagcacatctggatgggccttgtctacttcatcaaagagcaccacagcattggggcactgcttcaacttcttggtcagctggccaccctcctcatggccaacgtagcctggtggagacccaataaacttggccacctcgtgtcgctcctggaactcggacatgtccagcctgatgaagccctttttagcatctttgtgcatatatttggctgtctgcttggccagctctgtttttcctattccagatgatcccaagaagaggaagaccagagggtgttcttcatcgtaccagccattctccttcctccggatcgcagcacccactgtggcgatggcgctctcctggccaatgatgtgctcctttagtcgctgctccagggggaagcggcgccgctcctcagcctcacgcttccgctgcttctcttggtacttggcttcagaagtcctcagaagcttcatcacttccccttctcgggcataatccaagggtgtgtgtcccatttcattcctctgcagggggttggctcctccatcaagcagctccttgacagtgcggtagtcatcagcaagaacagcatagtgcaaggccgtgcagcccttgaaactggcgcggttgttcagcctgttgttgaagtcatcctctcgggtgatcaggacgccagcggggagtcctagccatctcctgaactccagggcacttgtccactggtttgtgatgtgccggcttgcaccgtcctgtcccccatcttccaaagaatggattccctgttccttggcagtcttgtaaacactgctgaaatcatctccaaggtttggatcagccccagcagcaagcaggacctgtaccacactgttgtttcggttgatggctgccaccatgagtgctgtccagccaagtctgtgctttgcattgacatctgcaccttctgacaacagcctgaggggccattcagaggaggaaatcttggtgttcttcagtgagactccagcattcagccctgcccagcttcttgactgagcatcattctttgcagtctcttggggctgctgacttcttgcatattgttggcacgggcagcttccaacagggctgcatccttgttggacggactcttgctgtagcaatgaaccaccagcgctgcggccagggcgcacatgcccagtccggccctgctggggaccccgttccagctgtcctgtcctgggagtgtttcttcgggaccaggaaggcgtccccaagtggcagccgcgaggcatttggtatcgaagcgtcctccctggcgccccccggtggctgccccacgtccggagaacaaggccggcgatgttccagggcgccccccggtggctaccctcagccactgcggctccccgagactcccagtagtcacattccggccggaagcacctccatggccccggagcgttggggacctgagcagccggaggagtagccgtggcgccagtgcttttctcctcaacaccagggaccccagcatcttgacagctgcttcgataaccccgtggtgccggcccctgtgctgaccacgtccaac

SEQ ID NO: 13113 - RNA, 3975 nt, Homo sapiens
  source 1..3975: mol_type = other RNA
gctgggattacaggcatgagccaccacacccggcaatttcctggttttgataaactacagtatggctttgtaggatgtaatcattgggagatgctagatgaaagatacatgggaattttctactatttctgcaactttctctaagtctaaaattatttcaaaacaaaaagtaaaaaacaatgaaaagcaggccgggtccagtggctcatgcctgtaatcccagcactttgggaggccgaggcaggcagatcacaaggtcaggagattgagaccatcctggctaacatggtgaaaccctgtctctactaaaaatacaaaaaggtagccgggcgtggtggtgggcacctgtagtcccagctactcgggaggctgaggcaggagaatggcgtgaacctgggaggcagggcttgcagtgagccgagatcgcgccactgcactccagcttgggggacagagtgagactctgtctcaaaaaaaaaaaaaaaaaaaaaaaggcagtcagtgaggtagggagcagcagcccctgaggggtagacagtgatccaagcatctgctggagctcacaccctggattctgactgcctcatacccaccatactgttaggacatgcttccattacccaagggactttgattcctggccccattctctgcttcctgaaagactagctaacactacgcgagggttccatgaagggcctgtgggggaaggtgggtggactgcttatcagcagtggctactgtagatggtgcccaaggatgcaccaggccttactgtgcctggctaaggtgggcttgaaacattggctggtctgtgaaatgcccttgggggacggtgtccagaccctctgctttgtgactaacatgcagactgaataaactgcatgtttattccaggctcgtttagctggacgagcagtacagacagggctgaggctgactccatggccatgtgggcagaggtcaaacccatgatctctcttcctacagcttcctaatgtctgcgatgttggtcttttgaaggaggcccccacagagctgagcttgcttggttatctgggactgctgctcagtctgagtaggggagggtaatgaaccagtcaggcctcctcctggaggtgcccaacactggcctagtccccaaggctgacgaaacatggtctggcctgaccccaggacgtggggtgaggaggaacactgggcataatatagtagcggaaacaggcaagcctctatgggtcccttccccttagaattttagggtagggaacgaggaggctacagactaaattgcagaactatctgcacctgggcctctgagctcttcctccactcccagtggagccattctggggactgagttgcatgaggactagcagagggtggcagttcagtctggtccctgtcttcttccagccagctgtgttcttagctgccatacttctgagcttcctgggaacatgagaaagtctggcgactatgggggatggggatcattctgaaggaaataagggacctccatccctccttgccttgaagggggtggaaaggcagctcctctcctgaaggcttgttagcaggttatgggcccacaacaaaggggccagagtagggcgaaattcctccttcaggttttggggctgagaaggggtcttcatgggctgtgaggaggtaagcaggcctgagactgggtagagatgggagcggcatgaggggaaggtaagtcagttgccatgccacagccaaggggcctttattggatggtgagggcacataggagcaggcaggtggctgctagatggtgttgcacaccttctcagggtgcagtggtgcccggatgtccagtctgcgagtcttgctgtccttgtcgatgatctccagacgcagcttggggaggcgcttctcagcctggggtgagggcagttctgggcttttgagtagctgcttgtctgagtcctccaccgtgatgcgcaaagtacagccccctggcagcaggtcctgctcataggctgctgccagctggttcaccacacggcgttctacctcatgtttgatggagcgggcgccatagtgcacattgtagccgtcgaccagcacatctgccacctcgcggtcccagagcagcgtgatgttgtgcctttgcttggctctcttggcccagaagtttagttccttgttgacgagttggatgagctccgagtggcagaaggggaggaagtagacgatctcattgatccgtcccagaaactcatccctccggaagtgagctttcaggatagggcgaatcacattctccttgaagttctttgagatggtgatcttgtcacttatctggacatcccccaggttttcggcaatacggttacggctcatctccaaagcttcctgcctcagctgcagcgcgtgctgtgcgatctcgtcgctggccacattggaggtcatgatgaagatggcgtccttgcaatcaatggtcttcccttttccatctgtcagccggccctcatcaaacagctgcagcatgatggtgagcacatctggatgggccttgtctacttcatcaaagagcaccacagcattggggcactgcttcaacttcttggtcagctggccaccctcctcatggccaacgtagcctggtggagacccaataaacttggccacctcgtgtcgctcctggaactcggacatgtccagcctgatgaagccctttttagcatctttgtgcatatatttggctgtctgcttggccagctctgtttttcctattccagatgatcccaagaagaggaagaccagagggtgttcttcatcgtaccagccattctccttcctccggatcgcagcacccactgtggcgatggcgctctcctggccaatgatgtgctcctttagtcgctgctccagggggaagcggcgccgctcctcagcctcacgcttccgctgcttctcttggtacttggcttcagaagtcctcagaagcttcatcacttccccttctcgggcataatccaagggtgtgtgtcccatttcattcctctgcagggggttggctcctccatcaagcagctccttgacagtgcggtagtcatcagcaagaacagcatagtgcaaggccgtgcagcccttgaaactggcgcggttgttcagcctgttgttgaagtcatcctctcgggtgatcaggacgccagcggggagtcctagccatctcctgaactccagggcacttgtccactggtttgtgatgtgccggcttgcaccgtcctgtcccccatcttccaaagaatggattccctgttccttggcagtcttgtaaacactgctgaaatcatctccaaggtttggatcagccccagcagcaagcaggacctgtaccacactgttgtttcggttgatggctgccaccatgagtgctgtccagccaagtctgtgctttgcattgacatctgcaccttctgacaacagcctgctgacttcttgcatattgttggcacgggcagcttccaacagggctgcatccttgttggacggactcttgctgtagcaatgaaccaccagcgctgcggccagggcgcacatgcccagtccggccctgctggggaccccgttccagctgtcctgtcctgggagtgtttcttcgggaccaggaaggcgtccccaagtggcagccgcgaggcatttggtatcgaagcgtcctccctggcgccccccggtggctgccccacgtccggagaacaaggccggcgatgttccagggcgccccccggtggctaccctcagccactgcggctccccgagactcccagtagtcacattccggccggaagcacctccatggccccggagcgttggggacctgagcagccggaggagtagccgtggcgccagtgcttttctcctcaacaccagggaccccagcatcttgacagctgcttcgataaccccgtggtgccggcccctgtgctgaccacgtccaac

SEQ ID NO: 13114 - RNA, 3798 nt, Homo sapiens
  source 1..3798: mol_type = other RNA
gctgggattacaggcatgagccaccacacccggcaatttcctggttttgataaactacagtatggctttgtaggatgtaatcattgggagatgctagatgaaagatacatgggaattttctactatttctgcaactttctctaagtctaaaattatttcaaaacaaaaagtaaaaaacaatgaaaagcaggccgggtccagtggctcatgcctgtaatcccagcactttgggaggccgaggcaggcagatcacaaggtcaggagattgagaccatcctggctaacatggtgaaaccctgtctctactaaaaatacaaaaaggtagccgggcgtggtggtgggcacctgtagtcccagctactcgggaggctgaggcaggagaatggcgtgaacctgggaggcagggcttgcagtgagccgagatcgcgccactgcactccagcttgggggacagagtgagactctgtctcaaaaaaaaaaaaaaaaaaaaaaaggcagtcagtgaggtagggagcagcagcccctgaggggtagacagtgatccaagcatctgctggagctcacaccctggattctgactgcctcatacccaccatactgttaggacatgcttccattacccaagggactttgattcctggccccattctctgcttcctgaaagactagctaacactacgcgagggttccatgaagggcctgtgggggaaggtgggtggactgcttatcagcagtggctactgtagatggtgcccaaggatgcaccaggccttactgtgcctggctaaggtgggcttgaaacattggctggtctgtgaaatgcccttgggggacggtgtccagaccctctgctttgtgactaacatgcagactgaataaactgcatgtttattccaggctcgtttagctggacgagcagtacagacagggctgaggctgactccatggccatgtgggcagaggtcaaacccatgatctctcttcctacagcttcctaatgtctgcgatgttggtcttttgaaggaggcccccacagagctgagcttgcttggttatctgggactgctgctcagtctgagtaggggagggtaatgaaccagtcaggcctcctcctggaggtgcccaacactggcctagtccccaaggctgacgaaacatggtctggcctgaccccaggacgtggggtgaggaggaacactgggcataatatagtagcggaaacaggcaagcctctatgggtcccttccccttagaattttagggtagggaacgaggaggctacagactaaattgcagaactatctgcacctgggcctctgagctcttcctccactcccagtggagccattctggggactgagttgcatgaggactagcagagggtggcagttcagtctggtccctgtcttcttccagccagctgtgttcttagctgccatacttctgagcttcctgggaacatgagaaagtctggcgactatgggggatggggatcattctgaaggaaataagggacctccatccctccttgccttgaagggggtggaaaggcagctcctctcctgaaggcttgttagcaggttatgggcccacaacaaaggggccagagtagggcgaaattcctccttcaggttttggggctgagaaggggtcttcatgggctgtgaggaggtaagcaggcctgagactgggtagagatgggagcggcatgaggggaaggtaagtcagttgccatgccacagccaaggggcctttattggatggtgagggcacataggagcaggcaggtggctgctagatggtgttgcacaccttctcagggtgcagtggtgcccggatgtccagtctgcgagtcttgctgtccttgtcgatgatctccagacgcagcttggggaggcgcttctcagcctggggtgagggcagttctgggcttttgagtagctgcttgtctgagtcctccaccgtgatgcgcaaagtacagccccctggcagcaggtcctgctcataggctgctgccagctggttcaccacacggcgttctacctcatgtttgatggagcgggcgccatagtgcacattgtagccgtcgaccagcacatctgccacctcgcggtcccagagcagcgtgatgttgtgcctttgcttggctctcttggcccagaagtttagttccttgttgacgagttggatgagctccgagtggcagaaggggaggaagtagacgatctcattgatccgtcccagaaactcatccctccggaagtgagctttcaggatagggcgaatcacattctccttgaagttctttgagatggtgatcttgtcacttatctggacatcccccaggttttcggcaatacggttacggctcatctccaaagcttcctgcctcagctgcagcgcgtgctgtgcgatctcgtcgctggccacattggaggtcatgatgaagatggcgtccttgcaatcaatggtcttcccttttccatctgtcagccggccctcatcaaacagctgcagcatgatggtgagcacatctggatgggccttgtctacttcatcaaagagcaccacagcattggggcactgcttcaacttcttggtcagctggccaccctcctcatggccaacgtagcctggtggagacccaataaacttggccacctcgtgtcgctcctggaactcggacatgtccagcctgatgaagccctttttagcatctttgtgcatatatttggctgtctgcttggccagctctgtttttcctattccagatgatcccaagaagaggaagaccagagggtgttcttcatcgtaccagccattctccttcctccggatcgcagcacccactgtggcgatggcgctctcctggccaatgatgtgctcctttagtcgctgctccagggggaagcggcgccgctcctcagcctcacgcttccgctgcttctcttggtacttggcttcagaagtcctcagaagcttcatcacttccccttctcgggcataatccaagggtgtgtgtcccatttcattcctctgcagggggttggctcctccatcaagcagctccttgacagtgcggtagtcatcagcaagaacagcatagtgcaaggccgtgcagcccttgaaactggcgcggttgttcagcctgttgttgaagtcatcctctcgggtgatcaggacttccaaagaatggattccctgttccttggcagtcttgtaaacactgctgaaatcatctccaaggtttggatcagccccagcagcaagcaggacctgtaccacactgctgacttcttgcatattgttggcacgggcagcttccaacagggctgcatccttgttggacggactcttgctgtagcaatgaaccaccagcgctgcggccagggcgcacatgcccagtccggccctgctggggaccccgttccagctgtcctgtcctgggagtgtttcttcgggaccaggaaggcgtccccaagtggcagccgcgaggcatttggtatcgaagcgtcctccctggcgccccccggtggctgccccacgtccggagaacaaggccggcgatgttccagggcgccccccggtggctaccctcagccactgcggctccccgagactcccagtagtcacattccggccggaagcacctccatggccccggagcgttggggacctgagcagccggaggagtagccgtggcgccagtgcttttctcctcaacaccagggaccccagcatcttgacagctgcttcgataaccccgtggtgccggcccctgtgctgaccacgtccaac

SEQ ID NO: 13115 - RNA, 3885 nt, Homo sapiens
  source 1..3885: mol_type = other RNA
gctgggattacaggcatgagccaccacacccggcaatttcctggttttgataaactacagtatggctttgtaggatgtaatcattgggagatgctagatgaaagatacatgggaattttctactatttctgcaactttctctaagtctaaaattatttcaaaacaaaaagtaaaaaacaatgaaaagcaggccgggtccagtggctcatgcctgtaatcccagcactttgggaggccgaggcaggcagatcacaaggtcaggagattgagaccatcctggctaacatggtgaaaccctgtctctactaaaaatacaaaaaggtagccgggcgtggtggtgggcacctgtagtcccagctactcgggaggctgaggcaggagaatggcgtgaacctgggaggcagggcttgcagtgagccgagatcgcgccactgcactccagcttgggggacagagtgagactctgtctcaaaaaaaaaaaaaaaaaaaaaaaggcagtcagtgaggtagggagcagcagcccctgaggggtagacagtgatccaagcatctgctggagctcacaccctggattctgactgcctcatacccaccatactgttaggacatgcttccattacccaagggactttgattcctggccccattctctgcttcctgaaagactagctaacactacgcgagggttccatgaagggcctgtgggggaaggtgggtggactgcttatcagcagtggctactgtagatggtgcccaaggatgcaccaggccttactgtgcctggctaaggtgggcttgaaacattggctggtctgtgaaatgcccttgggggacggtgtccagaccctctgctttgtgactaacatgcagactgaataaactgcatgtttattccaggctcgtttagctggacgagcagtacagacagggctgaggctgactccatggccatgtgggcagaggtcaaacccatgatctctcttcctacagcttcctaatgtctgcgatgttggtcttttgaaggaggcccccacagagctgagcttgcttggttatctgggactgctgctcagtctgagtaggggagggtaatgaaccagtcaggcctcctcctggaggtgcccaacactggcctagtccccaaggctgacgaaacatggtctggcctgaccccaggacgtggggtgaggaggaacactgggcataatatagtagcggaaacaggcaagcctctatgggtcccttccccttagaattttagggtagggaacgaggaggctacagactaaattgcagaactatctgcacctgggcctctgagctcttcctccactcccagtggagccattctggggactgagttgcatgaggactagcagagggtggcagttcagtctggtccctgtcttcttccagccagctgtgttcttagctgccatacttctgagcttcctgggaacatgagaaagtctggcgactatgggggatggggatcattctgaaggaaataagggacctccatccctccttgccttgaagggggtggaaaggcagctcctctcctgaaggcttgttagcaggttatgggcccacaacaaaggggccagagtagggcgaaattcctccttcaggttttggggctgagaaggggtcttcatgggctgtgaggaggtaagcaggcctgagactgggtagagatgggagcggcatgaggggaaggtaagtcagttgccatgccacagccaaggggcctttattggatggtgagggcacataggagcaggcaggtggctgctagatggtgttgcacaccttctcagggtgcagtggtgcccggatgtccagtctgcgagtcttgctgtccttgtcgatgatctccagacgcagcttggggaggcgcttctcagcctggggtgagggcagttctgggcttttgagtagctgcttgtctgagtcctccaccgtgatgcgcaaagtacagccccctggcagcaggtcctgctcataggctgctgccagctggttcaccacacggcgttctacctcatgtttgatggagcgggcgccatagtgcacattgtagccgtcgaccagcacatctgccacctcgcggtcccagagcagcgtgatgttgtgcctttgcttggctctcttggcccagaagtttagttccttgttgacgagttggatgagctccgagtggcagaaggggaggaagtagacgatctcattgatccgtcccagaaactcatccctccggaagtgagctttcaggatagggcgaatcacattctccttgaagttctttgagatggtgatcttgtcacttatctggacatcccccaggttttcggcaatacggttacggctcatctccaaagcttcctgcctcagctgcagcgcgtgctgtgcgatctcgtcgctggccacattggaggtcatgatgaagatggcgtccttgcaatcaatggtcttcccttttccatctgtcagccggccctcatcaaacagctgcagcatgatggtgagcacatctggatgggccttgtctacttcatcaaagagcaccacagcattggggcactgcttcaacttcttggtcagctggccaccctcctcatggccaacgtagcctggtggagacccaataaacttggccacctcgtgtcgctcctggaactcggacatgtccagcctgatgaagccctttttagcatctttgtgcatatatttggctgtctgcttggccagctctgtttttcctattccagatgatcccaagaagaggaagaccagagggtgttcttcatcgtaccagccattctccttcctccggatcgcagcacccactgtggcgatggcgctctcctggccaatgatgtgctcctttagtcgctgctccagggggaagcggcgccgctcctcagcctcacgcttccgctgcttctcttggtacttggcttcagaagtcctcagaagcttcatcacttccccttctcgggcataatccaagggtgtgtgtcccatttcattcctctgcagggggttggctcctccatcaagcagctccttgacagtgcggtagtcatcagcaagaacagcatagtgcaaggccgtgcagcccttgaaactggcgcggttgttcagcctgttgttgaagtcatcctctcgggtgatcaggacttccaaagaatggattccctgttccttggcagtcttgtaaacactgctgaaatcatctccaaggtttggatcagccccagcagcaagcaggacctgtaccacactgttgtttcggttgatggctgccaccatgagtgctgtccagccaagtctgtgctttgcattgacatctgcaccttctgacaacagcctgctgacttcttgcatattgttggcacgggcagcttccaacagggctgcatccttgttggacggactcttgctgtagcaatgaaccaccagcgctgcggccagggcgcacatgcccagtccggccctgctggggaccccgttccagctgtcctgtcctgggagtgtttcttcgggaccaggaaggcgtccccaagtggcagccgcgaggcatttggtatcgaagcgtcctccctggcgccccccggtggctgccccacgtccggagaacaaggccggcgatgttccagggcgccccccggtggctaccctcagccactgcggctccccgagactcccagtagtcacattccggccggaagcacctccatggccccggagcgttggggacctgagcagccggaggagtagccgtggcgccagtgcttttctcctcaacaccagggaccccagcatcttgacagctgcttcgataaccccgtggtgccggcccctgtgctgaccacgtccaac

SEQ ID NO: 13116 - RNA, 2020 nt, Homo sapiens
  source 1..2020: mol_type = other RNA
gctgggattacaggcatgagccaccacacccggccaagttctttaccatcttcagaaggcttagcttgcacttttggaagaagaatagactcccaggaagactgtgagagagatttggggcccaaattgatattatcaaatacactgaacttgactgtattcaccatgttctggctcttgagaaatgagagtgctagtgaggctggtgccactttgtgtatcttctgtaccttgaagtccctcagaaaccttgcccctggtcttctctggtcttctcattctaaggacataacaggttctctttttctctggagatgaaatctagatctttgattttggaaccaaatttggactcttgactctgaagcaccaatttcttcagcaagttgttctctggaatcaatcccagggtatgggtttttcataaatgcatggatgactgtgtgtaattgaaaggtgctataggtggtacaacaccatctggcttctctattttgaaactccacaccaggttaatcttgtccatggctgtggcttaaatctaaagtcaggttctggtgttttctggaatccatgcctagctctttgattctgaaaccaaatctggattctggactcttctgcattgattgctaaagcaagtttttgtttggtagcataacctgggtaaggtttttgagtgaaggtattgatgaggattttcaattgatcttctgtgaatttggtgcaattgcacctatgatttgttgctaccatcttgtgtgaagaggggtcttcaactatgcagaaagagagttctggaggctgagctactgtctgggagactgcttacagctcattttttaaaaagaaaggtcacatataatacaatataaaattcacaaatctaaagcttatggttttctgggttttgacaaatgaaaactcctgtgcaacttcaagccttaccaggatatggatgagggtttctatccaaaagcaccagtattctaacaaacaactttacgttttttgaattgtccagtgcctgtgaggattccttactccaagtttatgacaaacatattcagaaggcatagtctacaattagtgtttgggtaagtattttcatcaattgtctgattatttgctgtgaatttgaagtatgctgattcttatgtaattgtcttctgagaaacattgtgccatttttcttgtggaaaccacctttatcttgtttcctgcaaaatcatggaggtttgggaagttcctttagacccattctcgtatggaggtttgttttcttcttttttctttcctgggcgtggtggcgggtgcctgtaatcccagctactcaggaggctgaggcaggagaatggcgtgaacccaggaagcagagcttgcagtgagctgagatcatgccactgcactccagcctgggcaatacagcgagactccatcctgcccatccacagatgaagggataaagtaactgtggtggacatacacaaagagaatagtcttcagccagaaaatcagaatgaaatttcatcatttggagccatactgttgaacctggaggacagcatggtaaatgacctgttcaaacacagctgcagggatgaggaaactgctgtacagatacaccacggaatatgtttcagccagaaacctttgggaaatcctgccatctgcagccacatgaagaaaccagaggctgctggggaagtggaggcagtctcagaaggaatcagtgatgggtacaaagttactctcagatgagactgatcaattctggccttctattccacagcagggtgactagcctgttcatccacagataaagagatcaagaaactctcatatacatacactaggaaatattctccagccatcaaaataatgaagcagtgtcatttagagcaacacagatgaaccgcggagacctgcctcctactccaccatcacatggaacccaccactgcttctccgaagctcgctctgaccacgccgctgctgctgcaggggcctcgcaggaagt

SEQ ID NO: 13117 - RNA, 1523 nt, Homo sapiens
  source 1..1523: mol_type = other RNA
gctgggattacaggcatgagccaccacacccggccaagttctttaccatcttcagaaggcttagcttgcacttttggaagaagaatagactcccaggaagactgtgagagagatttggggcccaaattgatattatcaaatacactgaacttgattgtattcaccatgttctggctcttgagaaatgagagtgctagtgaggctggtgccactttgtgtatcttctgtaccttgaagtccctcagaaaccttgcccctggtcttctctggtcttctcattctaaggacataacaggttctctttttctctggagatgaaatctagatcttcgattttggaaccaaatttggactcttgactctgaagcaccaatttcttcagcaagttgttctctggaatcaatcccagggtatgggtttttcataaatgcatggatgactgtgtgtaattgaaaggtgctataggtggtacaacaccatctggcttctctattttgaaactccacaccaggttaatcttgtccatggctgtggcttaaatctaaagtcaggttctggtgttttctggaatccatgcctagctctttgattctgaaaccaaatctggattctggactcttctgcattgattgctaaagcaagtttttgtttggtagcataacctgggtaaggtttttgagtgaaggtattgatgaggattttcaattgatcttctgtgaatttggtgcaattgcacctatgatttgttgctaccatcttgtgtgaagaggggtcttcaactatgcagaaagagagttctggaggctgagctactgtctgggagactgcttacagctcattttttaaaaagaaaggtcacatataatacaatataaaattcacaaatctaaagcttatggttttctgggttttgacaaatgaaaactcctgtgcaacttcaagccttaccaggatatggatgagggtttctacccaaaagcaccagtattctaacaaacaactttacgttttttgaattgtccagtgcctgtgaggattccttactccaagtttatgacaaacatattcagaaggcatagtctacaattagtgtttgggtaagtattttcatcaattgtctgattatttgctgtgaatttgaagtatgctgattcttatgtaattgtcttctgagaaacattgtgccatttttcttgtggaaaccacctttatcttgtttcctgcaaaatcatggaggtttgggaagttcctttagacccattctcgtatggaggtttgttttcttcttttttctttcctgggcgtggtggcgggtgcctgtaatcccagctactcaggaggctgaggcaggagaatggcgtgaacccaggaagcagagcttgcagtgagctgagatcatgccactgcactccagcctgggcaatacagcgagacgcggagacctgcctcctactccaccatcacatggaacccaccactgcttctccgaagctcgctctgaccacgccgctgctgctgcaggg

SEQ ID NO: 13118 - RNA, 4943 nt, Homo sapiens
  source 1..4943: mol_type = other RNA
gctgggattacaggcatgagccaccacacccggccaagttctttaccatcttcagaaggcttagcttgcacttttggaagaagaatagactcccaggaagactgtgagagagatttggggcccaaattgatattatcaaatacactgaacttgattgtattcaccatgttctggctcttgagaaatgagagtgctagtgaggctggtgccactttgtgtatcttctgtaccttgaagtccctcagaaaccttgcccctggtcttctctggtcttctcattctaaggacataacaggttctctttttctctggagatgaaatctagatcttcgattttggaaccaaatttggactcttgactctgaagcaccaatttcttcagcaagttgttctctggaatcaatcccagggtatgggtttttcataaatgcatggatgactgtgtgtaattgaaaggtgctataggtggtacaacaccatctggcttctctattttgaaactccacaccaggttaatcttgtccatggctgtggcttaaatctaaagtcaggttctggtgttttctggaatccatgcctagctctttgattctgaaaccaaatctggattctggactcttctgcattgattgctaaagcaagtttttgtttggtagcataacctgggtaaggtttttgagtgaaggtattgatgaggattttcaattgatcttctgtgaatttggtgcaattgcacctatgatttgttgctaccatcttgtgtgaagaggggtcttcaactatgcagaaagagagttctggaggctgagctactgtctgggagactgcttacagctcattttttaaaaagaaaggtcacatataatacaatataaaattcacaaatctaaagcttatggttttctgggttttgacaaatgaaaactcctgtgcaacttcaagccttaccaggatatggatgagggtttctacccaaaagcaccagtattctaacaaacaactttacgttttttgaattgtccagtgcctgtgaggattccttactccaagtttatgacaaacatattcagaaggcatagtctacaattagtgtttgggtaagtattttcatcaattgtctgattatttgctgtgaatttgaagtatgctgattcttatgtaattgtcttctgagaaacattgtgccatttttcttgtggaaaccacctttatcttgtttcctgcaaaatcatggaggtttgggaagttcctttagacccattctcgtatggaggtttgttttcttcttttttctttcctgggcgtggtggcgggtgcctgtaatcccagctactcaggaggctgaggcaggagaatggcgtgaacccaggaagcagagcttgcagtgagctgagatcatgccactgcactccagcctgggcaatacagcgagactgcccatccacagatgaagggataaagtaactgtggtggacatacacaaagagaatagtcttcagccagaaaatcagaatgaaatttcatcctttggagccatactgttgaacctggaggacagcatggtaaatgacctgttcaaacacagctgcagggatgaggaaactgctgtacagatacaccacggaatatgtttcagccagaaacctttgggaaatcctgccatctgcagccacatgaagaaaccagaggctgctggggaagtggaggcagtctcagaaggaatcagtgatgggtacaaagttactctcagatgagactgatcaattctggccttctattccacagcagggtgactagccttaacacaaatgtaccatatgtttcaaagtagccataaattcattgccaagtgcaaagtccagacgaatatttcctaggttttcttccaggatttttatagtcagaggatgtaatcttatgccaacgggtcttaataatcaaatgactccacagtgagaatcattactctgaaaaattgattttgttagaatgatggaaatttaaatatttgaaagtaaaaacacatgccacctttttcctagaactctgcaaggcaaattgctgtaagacaggcagaggaagcacaatatatatatatatccaaaatataatttgcagtgaaataaatgaaagcaaattataaataaacttacctgattttacaaactaacctttaaagggatttctactaatttttctattgcctgaattgccctttcttctagatccaatttatatttttgtacttcaccaatgtgtcttcaccaatgtgtactttccatatgttttttaagatttaatattactttttccaacatcttcttatcctcttcaagttttttatattcctgttgtatttttttcatagataataactcctgttgaataacttctttttagtcaaatagacatattttgaagatacagctttcagctttgctgtaagatcatcgaactacattaataaaataatatagcttgataatgaagtaggctgagaataatctcatacaaaaccaataacaaattttgaaatacatttacttgcaataaaatgttatctataatgtagattctttaaatgttaacccgtactcagaaatgcaagaacaaagtaaaagccaccatgagtcacaaacatatattctttactctcatcatctttgccacagaacttttgcacttgatcttacttttgtttttctgataatttgtgttttttcctttcttaaatggctctaagttaactcttattagaaagtttcaaacccccttctctcatcatcatgccccaaaatttgtcaaaaaaaagtttcagagatattatattgagttatttaggccaaaggcaataaatggctcttacaataagactttgaaaataatgtaatactctacaataggcatggtgtatcatgcatataatcctagcacttaaggaggctgtggcagaaagatcccttgaggtcaaacatttgagatcagccagagcaacatagtgataccataatctcgacaaaaaaaaaaaaaaaaaaaaaaaaacgtgaaaaaattagccacgcatgatgccttatgcttgtagatccaactggttgggagattaaggcaaaaggatggcttgcactcaagagttcagggctgtggtgaattatgatcaaaccacggcacttctgcctcgatgacaaagaccatatctcaaaaaaacacaaaataatcctataaataaggattctaatgccacaagcctttccataggctgtaaatgttttatgctaatttgaattgcattttaaaaagtaatgattcttggggtaaaggccatagaatacagtcccaagaaataaatccacatatttaccttacaagaaataaatccacattcttgtgttacaagagctcctgaaggagacactaaacgtagaaaggaaaaaccagtaccagccactacaaaaacatatcgaattgtaaagaccattgacactataaagaaactgcaaactaatgggaaaaataaaaagctagcaacatcatgacaggataaatttcacctgtagcaatactaaacttaaatgtaaatgggctaaatgccccagttaaaagacacagactggcaagttggataaagagtaaagacccattgttgtcctgtattcaggagacccatctcatgtgcaaagacacacataggcttaaaataaagggatggaggaatatttaccaagcaaatggaaagcaaaaaagagcagggtttgcaatcctagtctctgataaaacagacattaactgaaaaagatcaagagagacaaagaagagcaccacaaagcagtgccatctgcttttcctcaggcctctgctccatcagctggcagccacccaggatgttggaacctggccatccctgcttctttcagtgggtgaggttggtggctgctccacctgctccaggcacacccttaacagaggtggctgcttgctctttaagccagcttggccttgcctggcatgcacaggccccggggaccgacatgctgctctgactgagaccgtcctgactttgtcaaattctacgtctggcctgggccacagaagcacaagtcccctgggtggtaccactggctgctttctggactggaacataaagtcctcctcaagatgacctgtggtctgcctcttggcaaccaacaagcccgcagtgtcatacgacccatgagacatggactgaaggcccaaagggagtgcacaccatgttccagagccagctgctcctttcctctatatggccccatttgcagcacagttgttgcactgaggcttgtgcatgctgggcaagggcaagctggctcaaagggcaaccagctatctttgcacggatgtgccagcagcaggcagaccagccatcaacctcacacgctgccagtcaggctaaatcagctcttctaccataaaggtagggccacagtgccatctggttttcctaaggcctctgtttcttcagccattaggtggcacccactcaggctttgggaacctggctaccccggcttcctggagtgggtgagctggtggctgctccacctgctctaggtgcacccttgcagaggtggctggttgctctttgagccagcttggccttgcctggcatgcacagaccccagctacagacacgctactccaagtgagcttgtcctgtctacggccaaattctaagtttggccagggccacagaaggcagagtcccgagggtggtaatcctggctgctttctgcacttgaacataaagtccttctcaagacggcctatggtctgcctcttggcaaccaagaagcccacagtgacataagacccttgaggcaaggactggagcccccaaaggcagcatacaccttgctcctgagatggctgctcgtttcccctatatggctccacttgtagcacagtagtag

SEQ ID NO: 13119 - RNA, 2037 nt, Homo sapiens
  source 1..2037: mol_type = other RNA
gctgggattacaggcatgagccaccacacccggccaagttctttaccatcttcagaaggcttagcttgcacttttggaagaagaatagactcccaggaagactgtgagagagatttggggcccaaattgatattatcaaatacactgaacttgattgtattcaccatgttctggctcttgagaaatgagagtgctagtgaggctggtgccactttgtgtatcttctgtaccttgaagtccctcagaaaccttgcccctggtcttctctggtcttctcattctaaggacataacaggttctctttttctctggagatgaaatctagatcttcgattttggaaccaaatttggactcttgactctgaagcaccaatttcttcagcaagttgttctctggaatcaatcccagggtatgggtttttcataaatgcatggatgactgtgtgtaattgaaaggtgctataggtggtacaacaccatctggcttctctattttgaaactccacaccaggttaatcttgtccatggctgtggcttaaatctaaagtcaggttctggtgttttctggaatccatgcctagctctttgattctgaaaccaaatctggattctggactcttctgcattgattgctaaagcaagtttttgtttggtagcataacctgggtaaggtttttgagtgaaggtattgatgaggattttcaattgatcttctgtgaatttggtgcaattgcacctatgatttgttgctaccatcttgtgtgaagaggggtcttcaactatgcagaaagagagttctggaggctgagctactgtctgggagactgcttacagctcattttttaaaaagaaaggtcacatataatacaatataaaattcacaaatctaaagcttatggttttctgggttttgacaaatgaaaactcctgtgcaacttcaagccttaccaggatatggatgagggtttctacccaaaagcaccagtattctaacaaacaactttacgttttttgaattgtccagtgcctgtgaggattccttactccaagtttatgacaaacatattcagaaggcatagtctacaattagtgtttgggtaagtattttcatcaattgtctgattatttgctgtgaatttgaagtatgctgattcttatgtaattgtcttctgagaaacattgtgccatttttcttgtggaaaccacctttatcttgtttcctgcaaaatcatggaggtttgggaagttcctttagacccattctcgtatggaggtttgttttcttcttttttctttcctgggcgtggtggcgggtgcctgtaatcccagctactcaggaggctgaggcaggagaatggcgtgaacccaggaagcagagcttgcagtgagctgagatcatgccactgcactccagcctgggcaatacagcgagactgcccatccacagatgaagggataaagtaactgtggtggacatacacaaagagaatagtcttcagccagaaaatcagaatgaaatttcatcctttggagccatactgttgaacctggaggacagcatggtaaatgacctgttcaaacacagctgcagggatgaggaaactgctgtacagatacaccacggaatatgtttcagccagaaacctttgggaaatcctgccatctgcagccacatgaagaaaccagaggctgctggggaagtggaggcagtctcagaaggaatcagtgatgggtacaaagttactctcagatgagactgatcaattctggccttctattccacagcagggtgactagccttaacacaaatgtaccatatgtttcaaagtagctgttcatccacagataaagagatcaagaaactctcatatacatacactaggaaatattctccagccatcaaaataatgaaacagtgtcatttagagcaacacagatgaaccgcggagacctgcctcctactccaccatcacatggaacccaccactgcttctccgaagctcgctctgaccacgccgctgctgctgcaggggcctc

SEQ ID NO: 13120 - RNA, 5381 nt, Homo sapiens
  source 1..5381: mol_type = other RNA
gctgggattacaggcatgagccaccacacccggccacaagctgtttcttaactaagcttctgaagcaggaactcctaaagtgtcaataggcagttttacttacagtagtagttatatactaatgctgcttgcagaattttttttccctttagagttcacagaagtactaccacatggagacaaaacaaaacagtaaaaatagtataggtagtaaaaaggccaaaactaagaaatttggggccataacattagaaaagtttgaaaatatactttacatatttgcttaaaaaattaagtgtagtactgccttaatgcttggttcctctaccattaaatggcatttcattcagtttatgctgaactcttagatcaacttattattactgaatacaaagctaagcaaacctagacattttagctgctgccactgtgtattatcacagtacataaggaatctgtcacaaggtttgtctccccttctccattatactgttcttaaaggtagagggcaggtctcatgcacctttgcatcccctgcatataagcacagtggctggcatacagtgggtgaataggtatttactgatgcattgctgagtagtggcttataacatggagaaaagcccaacattgtcctgttctatcagcattacttaggtatcctcactcctaataggcagaaagcagttttgaagtaaagttaaattcctcacttgctaaacacagcagacctgtcaagtgttggacaagacttaaaccactttctttaaatgtgttcataaagcattttgagaaatcaagagatgaaaggcgctatgtaagtacaaaatattcaagacagtttagcaaaagtgctacttttctacgatgatggaatggttgtgctagtttgaggggaacatcccctgaggctactcttcttgctgtcattattaacacaacaatggaattttgacaaagatgccatcactttatatagtttttattcagctaactactttctataaaccatgtgacagaaaatgaaattaagccacttattccacataaaccaatactttatcaaagttccgcattttacaagtcatgttcaaaaaacacacacaaattagcattttgtacacaaatgtttatttctcaattaaacattccctttaaacacaaggaatgagttctaaatcttcataaagatgaattaaaaatgaaatccctccagtatagtgtatataatcactgtgttcttggtcactactggcatttactgtttaacatcaaaaacaaagacaggttatttaaaaatcatgctactggatttctagctcttcctctatgaccagttctacactgatctgcaatgtttaaaagtttacatcaccaaatcaaagcaagtttaaggtgtgaagtagctgtgcattaaacacaaaataaacaataaaattataagatatagtcaagttcataacgaatataggtgttcttatcatcgttgtagattcttgggtaatgtgctatgagagcgtcctgggaaccaatgtagatggagttgtaaattttccaatatacatctctgactttccgggctgggtgaaacagaccctgtaaacaatattgcaacattctacatggtccaatagcaactctcaggccctctagggctcccataactgcctgaattacatgaggagatgtctcaaatacattgggccatacatagttcaacaagtgattcagcgaatcttcacaaccaaatccataaaccccaagtgacatgtgctgtaccactgcactagccgtctgtctgtgtacaaggtctctatccattaaagcatcttcaagtaacggtgttacggcataaatgtagtcttttcccatttcaccaatatattcaaacaagaaggaaagcgattttaacactccattttgaacattcagttcaggaactctgtattcattcattaaggcagggagtactgtaaagggtgaacatgtttctgcaacaatagctattgctacagtggtacaaactctgttctgcctttcttgaactttgaggttgttcagaagtgtagccaatacatcatgagggccaatggcctttgcaatataaccaaatgtgttgactgtggctctacgaatagcctttttgtgggcttttaagagctctaaaagctcaaagcaaatcctcatccactctcttgcagatacatattcagctcccctgtcagcaatacgaccaacaagatcaatacaattctcttgtactttttcatgtctgttctttaagatgggggtgagtctaggcagcagatctttaattggtggagtcatcttatgcatacctatgacatttacaatggccttcagtgctccaagaatgctgcccaatacttcagggtactcttcacccaaatactcatacaatacaacacccaagtgtcccatcaatttttcctcttgacaagtcttcatgacaacagcagttcgagaaatcaagtcagctgcctgttgcctaactttagcagatttgttatttaaacgccacaaaactgtaccacagatctgaggcaagtatggtttgactcgtttgccaagagcattaaccactgtgccaaagccgttcaacattactgagtcctctgtagtctgttcttggaaagcataaagaataccatcaatcagttgttcttcaagtttatgatcaatatctgctgctcccaaattacccataattttctcaattgtctccatcaccatttttctgtactgttcggcttcatctttcagatcatccacaatcctggatataatttctgctgcacctactttgtttgccaactccacagtagtatcaactaactgtcggtaatttcttctatccaaagccatcctgtgctgccagaagtgtttaaaaaagggaggaagaatctctgttttaatgtagtttgcttctacaccatctgtcccacaacactgttttaccaccttcagcacaatttttttcatttcctcatcaggagactggaattctcgaataaggattaacatcacttctctagtatagtagttggcatattctgcatccataagaggaataagatacccaatagccttcaagaaagcagccaaaccctttcctctgtgttggcggatacccttccataaaggctttaacacagaatcaaaagattcgataccataaggagttgctgcttcagccaaggcagcaatggccaaagcactgatggtccgaactttctgctgctcatccacaagaccatgttcaatgatttcaactaaacttctaagatgtggcaagatggcacagcccataagaatagctatctgttgtacaatcttaataccagtgtgtctcgcttgccaggacttcttgcttttgcacacagcttttaagaagggcaataaagaaggaatgcccagggcagaggctacaacagcaaaagctctagctgttgtgttacggacatactcatccatgttatctatatcaggtctcatggtagagatcatagtagccagaccagcagcctttgccaaattagaaatgatctctcggccttccactctagcatagtaatcttcatcaatcaatagcggttcaatgaccacgaggatcttatgcacatatggacgaactaagtcatcaagtttgtacagtatcctatcaataactttcacaagtaaatgacgctcttgatcctcaagtgtaggagacatcagcagaggaagaatctgattaaacaaaggaccagctccaaattcacgagctttatcagtaatctgacgcaatgcagcctttctcattggtggtgttccattcttaatttttaaaagcaacttcattatttttctctctttttgctcttctggactaagtgttgattcatcaacatcaaccaatagtttatcaaagtattgaatatcatcaggttttaaaaatggaagatttccagatggctggtcattaacacttttcatagttcgatcttcagtttgcatgtggaaaccagtcataccacccaaaggtgttggagtagctgtcagctttcgagctggagttcgaataggaacataaccagctggaggaggaagtaccttatatccttctgggaacatagcatctaattcctcatcagaaagtgggcgatttctctcatcaatttctctttcccaccgccaagcctgaagctgttcaggagtcatactcattatgtgacctggagtaggggtagccatgttcatggctggtgtgccaattggtgtctttccaggggtcagaactggagtgcttccacccatctgactagctggtgtttcatcccaccgtgattttcttttactggctccaggagtcggtgtttcaccaatagaatctccacctcgatctgttcgaggagtctcagcccatccacttccatgcccaggagtatctctctctgttttgggggtttcatcccatctgtttttacgagcactggaagttgcgcctccatggcctggtgtcgcatggcctggtgtatcacctcgtccaggagtagcagctcccgctggtgtgtggctaggtgtaggatcccatatttttgagcctggggttgctccaggagtctcgcttccctttgcacgacctggtgtctcatcccatcttaaggaaggagtatgcccaggggtctctgcctgatcccaacttgatagttttttgggagtggcaccaggagtctgatcagctgtttgatcccaacgccgttttcgttttgatggaggctgggacgctgctgctccattgacgacttttagttctccagctttagctttttctgctagctgttgcctaatttctcgttcttctttagtcaagtgttgttctcgcattacatccatgtaagtcctagcattcattttaggatcaggggttttccctccatctgcaaaaggatcaagacgctctggggaaattatcatggtccgcctatgctttttgtattcatcttcccggtctgcaatctttggaggtctgtgctcagcaaatggatcatactgttctgttgactgtggtatatcattaagcaatgccacaggggcatgatatcctggcttcttctgaccaagcaaactcgtagatgatgaatagtcatcgtcatcatcttcaagttcagttgcagcaattgatgtcacgtatccagcaaatctgctgtcacttccaccataaatttcctggtcataataacctgtagaatcgaggcccactccttgagcttcatcaagagctgccttcttgccttgaatttctcgaatctgtgcttcaatatcttcgtgagtcttggcgatcttcgccattttgtccactcgaacacacagacggaact

SEQ ID NO: 13121 - RNA, 424 nt, Homo sapiens
  source 1..424: mol_type = other RNA
gctgggattacaggcatgagccaccacacccggccacagggttttctgtgaaaggaacactctctgtcgttttcaaagcataggcagtaaggcacgtgagtctggagcagcttggggtcatctttgccatcactggaacagaggcctagaataaaggcaacacagaaaacaaaaacaaaaacaggcagtcaagagatgaagagggaccgtttcttgatgacatcgtgcctgaagttagatgtatccctgaacttttttattacacaagtcaatgaattccttttttaaaaattaagctaatttgaggtttatcacttgcaacagaaagcagactgaccaatatatcaactagtaagaaatacaagacaaaaccaactggatttggaaccagattttggttcaacctgtccatcatcaacgaaag

SEQ ID NO: 13122 - RNA, 10763 nt, Homo sapiens
  source 1..10763: mol_type = other RNA
gctgggattacaggcatgagccaccacacccggcccacatttttggtttttactttttggaaaaagcaatataagaaataattccactaccttgtacatctagtattagtccaggtaggatatctattttattgtgaacaaaacttatttgtactataaagtaaaaactgcttatttcttccatctaaaaagcagcatagtaaaacatcataaacttaggcattttttctaattatctaagttttagaaaacttataagcatccaaaataattttcaaatccagtattaagtaatcttaaaaatgaaggcatttttacatcaaaatctctggataaataacaaaataaaacttagtaggttttgatttagaaaaagtttctaaaaaaatcagtattttaaaaactaaaaatcaatcatgttagttctgccgacttgaaatctcctaaaaaactgtaagataaaaaaaaagatagccacggtggcaccacgggtgaagcactggattgaaacctcccatcaccccaaaaaagaataaaataaatgaatagatgccagtctcatttatgcatcataattattgctacttaacttgagactttgttcaatacaaattcctgaagtcttaagaaaagacaccttgacatttaaatatgttctattttacaattgttgtaccagtttatttcagagttatttacctaaaacatagctattttttccttaataaaacagaggatttttacttattggaaagaaaattcttctatagctttttattagccctgactcacatcaaatcaaatctattcaaaagtttccctaaacagaatcctttatttcttaaaatttttttactcactcaaaagattataaagaaaagggcactggatactgtggtcaacaggaaagcgaaattgcaaaagaaaaatttctctaagattcaactgagaagacaattggatttaaggacatctatgatttgtggaacaaaaaagaatactattactggaaacagatccctttaaagaaagccatgtaaccattccttcctgaaaatgcatttaacatacaaagtctctgcacaatttcagagggattcacaagttctcccaaacacatgaaatctcagattaataacactggtagttgtaaaagctctctgacctaactcaaaagataatcttacaaaaaaatctaagtttaacaatgtctttgaattccaaattaaataaatcagacttttactttaagatcttaataatcaaccacaacatttaacactatataataaaattagctataatcctaaaacatgaaatagaaatttttaaattactatatataaatgattattttaagttatacatatcttttcaattcattcatcaatcacacagatatcctaagtaaaaattcaacatatttgggtactactaactcttaattattagagtaaaacagtatttgcttagtgaagaaagagtcaagaaattcggaactttgcaaatgcaaattgtgctgcaaatgctacttaaaaggcccaactgtcaaaatcacaattagcacttttgcttaattatattattaaggaaatacatctgtaaaatgtatctctagttccacttttttctactcaatttttattaaggacagtaatagatttcagtaacttctcattagaaacacgctaagtagtaatagaattagctaatgtaccagtttcaatattcttattttattcttaccatgcaaacttgtaactttcaccgagttttgaaaatccaagtgtgcaacagatacctttaaaatattatccccaatcaggagttccataaataaattgatatattttcattacagtggtcagtaaataggaaaatgattacttaagaatgtatttaaagccatctctctcaactgtcccattatctgtactcttttattagaaaaatcttaaattttatcatttggaataataagaaaattgaacctaatgttctcattttagtttgttttaaaaatggatacaatgacctttaggaatgggccacaaaatcaaatcaaatgtattttctcaaatacatcttagtatagaccaagaattagtttatataccacagcaaattgtggttatctgtaaatgattttcagggataaaagccttgcaacattgcagagagttgagagatgtggttaaagtgacaaagcaataaatcaggtttcagtaatcataacagaaaatggaaataacaatcacttggaatcttgagtattatattcagtttctccagctgaaatctggctgagccgcttgctcgatccccaaaattttcgagaaagctgacctgaacgcatctcagcaggcttgccaacacccactacaatcaatttgccatcttctaaacctacaagaatatggctgtattctttggtgacacaaacacaatggataggcagtcgcatggctaatgggttgatgctgagattcaagctgtggagatctcttatagacaggaatccttgtatgctgcctgtgacaatgtgttctccgattatacatatatctgatacttgttccttcaggatttgagaccctagatacttgccatttatagaaaacagatgtaatgcattcttatccttgagggtggtcttttcttcagtgctggagtagacaacaatatgtccttcccaagatatagccaaattaggaatggtcaggaacagagaactctcacaaggtggtcgtaaagtcctcatgtactgacctttctgaatggtatgtataatcaccgttccatcccttgatcctgacactgccatgtctagctcagtgctgatgccgacactcagtacctcgttggtgtgtccataaagaatctgaaaaggtttagatgctaagcccacaggaacacctccctgttgtgttatttgccatatcatacatgtagtatctctggaaccagaaatcaaatgtattccacagtaatctgtagctaagcaagtcacaatatccatatgccggatgatgtgtgagataattttgccttttgtaagtgacatcacttgaatgctattatcccagtatccagcactgaagagcaactttgcatcatgtgatactacaaatagcttagaagtgatctctagcccgggagcaaaagaaccatttatactgcgctgagtttttggatttgtcacagtttgatccttgatgaatgtaaagtaattagaaatgtttctgtcataaggcaaccatccatgggttccaataacataattcatgcttattgttatcagtaactcagggctgccttgagacataaaagaacgatactgatttttggggatggtggcctttaatagtggaataccatcactaatcccctctataaaaaatgacttgagttcaggaaggtgttgaaacaggtttagggttgaagtgtctattttggttggcttctgcactgcttcttctgctgataatcttggagggtgtggttcctttaataattgacagggtgtttgcccaaaattattaatcatcccttctaaggcttttctttctttctcatctgttaaggcatccagatccacagctccttcataactacaataatagaaaacgttgagtgcctctactgcagctggtcccctctgtttatagccaaagatcagatctatccattcatgaagatgagctgaaacatattcagactccaaagctttcctatgtttatagatgaaatcttcagctgatttagcccatttcgggagaatgacatcatttactaattctttggaaatctgtagacgacccaagttaaattgattttgattttccaaaaactctgggaaatagaagaattcaggaataagttctttaacatcatatggattatccataagagcttgccaggtagcaggaatagaatggaactgtcgatctgcacagtcaaaccttccactctgaagttggatgtggagggtggtgaacggttctacacgaatgagatagtgcatgacccccgcagaatttgaatagtgagtaccatagtgaaacttatcaatagttcccataggatcctcaaaattttcatatttttctctcatagctttggcgtttttttcattaactaccccaattggtttggaaagatctcgaaatacagcagggttattaaggtccaactcttccgaagtataatcttgtaaaatccagggaaacacaggatactgtgcaaggtcattataggttcgtcctgccattgtatttatttgaatgaggtagtcaaaatttgatatctctctgtttacccatttctgtgtcaatcctgatgctttgaataactcctgtggtgatctgcttccataataactatttggggaatgaagtgacaacagtcggctatatattttgtttctaacctcttttttgaaattgagaaagtagttggattggtcaacatgaaaaatctcaagggctgatcttcttaaattgtaacgccggagatgaatctctcgaatttgagaatgaggccacttgaaatcaaagcctactccatcttctttttcaatgctgccatcatagaagtaaatgtgttgagtagtgatttctaatctgccaggaattacatcaattattgtaatgagttcacagtcttccatcaataccaatttttctttttgatcctgttcttctttctcatcaacatttactctagctgttatatcctcttcaggaaggtctaatttatcctccaccatatcactaacttttacttgtttcactacttccaaaagcaatgtatcactggaaggctgtgagtgttggatacccagattatctctcaaggcactagcttcctcatgggttttgaaattataattcggtaccagcttaagtctcatgcgggaataattctctacattagctagcttccagtgaattggattctgtttccttttagcccaaggtcccctttcacatgtaagatagagctgtattgctttccagcgtctaagagtggctaactgttgactgctaagttgtttaagcatattattatacctcaggttctcttggcgtgcttttcgattaaatggctccacaaacagctcctgaaatttgagcttgctttcccctccttcccggtctcgtttatgcatatttaccattaaagcttcataacaatccttccaataaagtgccatgttctcatgaccatcgtaaaatgtatgagcttcatactgcttcatataaggtacaatatatttttcaatgtaaacttgccattcatttgaattacaatattcttgaaaatcttcaaaaaatgaggagctaccattggtaaaaggtaaagaaggtaggtgcaagttcatgaagagaagctcataaattttggaaaccagggtacgaacaaggggaatcagaaatgagtagatttcagtctgttccttgattgattgacttagaacatgttccagcttccctaaaatgtaacatgcttcatcctgattttcaatcactttggtctgaagaagggtatttagcttagctgatgccattgcacaaacctgcaaattaccccttccaatgaatcctagaagcaactggatctgaatttgagagagttttacccatactggactttcagaatagcagactgacagacagtcaaagagcagcatcatatcctctaaaagcttctcggtccacatgtttgaattaactagtccctctgactgaagaaagtcctgtatgatcagcactagtcggaaggcgttttcagcagttactggattagtttttgcttctctgttttctgagattgcccattctaacatcttttgtagcaaagttagttttatttcatctgatggtcgaagtagttcactggatattcctggtttacttagtgctgaaaacacttgtcctcgttcaatccaagtatcatcatcagacttttctagtcccttacacattacataattcaaaatatgtgtcagtaattgaagaagctcctcctcacatctctcttggctttcaagtaaagagaagtcatcactaaagcccatatcatttgtgatgctgctttctctgtcagagtgcacagaaaacgatttagtagactctactggggatggtgtgctaggcagactgtctggcacttgacttccactatcactcatttcacatgagtcaattccactgaggtctaaactcaaatgtgaagggttactatgccagaattcctcttgattctctgatttgaaagacaattctcccacagagctatcttctggaaataatggtgtgtttgagtctaaagagtgtctatcctccaaactccactgatccgaagacacattagctgaggcaaaagaggtgattttttcctcatctgttttttcatcagagttcttcttggtatcttcagttgacatatttttatcattgtctttcattaaaacagctctactgtgcttatgaagagtatttccgttttcaaattttgcttttaaaaaaagcctaactaaggtgtcttgccaacccacttgctgtgatatttgatgtgctgcatctggctggaactgcaaaatttgcaaaacctttctgcagatggccactctaacatttatatgtgctctgtgagatatatataccacagatagtagatctttgaaattaataacaggatctgtatttatgatttgatgggtgaggtttttaataagagaagtattaacaagtgcttcattaagaaggagtcccagtcccgagtagccaacttctctgagtcgaatatgttgtttactacgctcataaacgttcgtgcatttcaacatttgttccataatcttaaaaatgatttctcttagtctgtcagagtacttctgatttaagagcaatgcgtacagtatgtcagcatttcctggttcaaaaagcagtaagaaaagctgacctctggttgggctggtacgtaggagactgaagagcacgtccaaaattccaaagagctgttcttcttcattagtagcagctatgtaccccataatactttgtatctcttcatgagatccacctttgcacagaaaatatttaattagtccatacaaagaagtccttattgttcgaatatcatctagagatagttcattatatttacaaccattcccataataaatcctaagtgtatctaggagaaactgcacaccatacttctttcggaaaactctcctgctgtctttaatgatggttgaaagatactgtatgtgaccgattcgaaagggaaaatctccacggttccaaatacgaaagtcaaagagtaaatattgatacatttgttgcaggagctgcatatttttctctaatgatacttgttcaattagtaactgaactgccatcaacacattaacatccatcaaggtgcttggcaccttctgaagtaaagcaccaagagttgcaactccatgggagtgaataagattgccctggttgataggatgtctctgaataaaatgtttcacaattaagataaatgttgcaactaggtttctctctagtcttgactctgaggcctttgtggaagtccatacgagccaatctccttcaacaggtgttactgattcaggaactgtgctttcattcttttcttcaggaatctgtccttcactaaagtggctgatttgttccaataaaggaaagagtacatttaacccacctatgcagtttatgatatccttaatgtcccagttcactactttgtttcctgttaatcttccatgcaaacaattagtagataaatcaagacagattgaatttttgcaggcctttgctgtgtagtaaagaaggatgttaccaggcaggtcggccatgtcagactcttgacacttccaagggcttaaacaatttggacctgctaaatataatgccttcacctgaggaggttgtagtggttcataaaagatgataacagatcctagctgaccctccagagatgtgggacacccccattcactgtcttgggttccagctgatatcaatttggtaatcaattttgatttttcaattgttcctccccaggaggctgatgacagaattccaccaaatgatgtccgatgaggggtaatgggagaagagaaaggtggatctgggatttgggatggtggaggagtggtggttctttgcccagctgaaccaatgcaacaggaagtaaagggttcattcatggcaggaaatctgagaggggcagaaaccttctgttgtccattgtcatagatatagacgaagctctgaccaaaaggcctttttccaggcatgtggacaacagttatgttgtgccagagggaatcacagaaactgtggtcaggaagcataaccgttgcatattctctttttgtgcacactgccacgaccaacatacctgaatgggtaataaaggcttcaaaacccatgccacttcctgtaaaaaaactgtacaattgtttccttttccctcctttgttagcaatgccaagagtcaactgatcctggtctaagcaaaaccaagcactgaaagaaaaggcagaccctggccatttctgtatgggaggcacagaaattcctgccatactatgtgacaaattgaaatactggagggcactctctagacttagttttcgggccattgtcaggattgctcgagtcacgggagtgacataagggtgaacagactcagattcatccactctcagcaatctcagtagtcgacggatttcttctgagctcactgactgactccccaaggaaccatggattgcaatcaagttctcagcacaagtttgatggagggaagaatgcaagtcaagggtttcaatgattctaatccccatgtttgcattgacacaagtagttcgactctgtctattaatacaacaaattcttttcagccaatcagagatgaagatttgcaggtcatgggattgtagttctggaagccactggataagaagcaagagaggttggacattactaatgcccaaaatcccaactgaagtgtggtcaccctctacagccatattcataagttctttaagtaattccagtggtggctgacccagggattttaatacttcaagcatatgtgtataaccaattctttctttaaatacttccttagcagctggagatttgttcattactgcggtcaaagcctgaatggttgatatggccaaacaatccaattgtccctgaaacacctggtcctcattcatttctgtcagtaatttgttggcaaggtctttctcgttcttgtctgccaccttattgttagcatttaaaaatagcttgcagttctgtagcagtcgtatgagatgttcaaagcaattgctgttaagaaaaatggcctgaagaacaggtctatctgtacaatctaacatggctgtgatggtattcagcattttgatctgtagagcaataaatcggttttcccactgtctggacctcctttgattaggtaaagctgaatgatctgaatttagcaatttaaaatagttctccagaatagtactggtttccacttgacgctgatcagagttgctactgagaaggatatgtaccacttctgtaaggcacttcagagttagttctgccttcctacccacttcttcaggatctccatcctcccaggaatcacaatctgccaatactcgcataagaacttccatagtggctggagaaattgcttgcaaagcattcctctgcccaccggctacaatggctccaaagagatgcaataagcaacatttaagactttccttgagatgttcactttcctgaaaacattgataaaagaaagggacgaattccactgtgagagaagctggtttatatttctgtctgctcttttccacagtactaaggattcgtcctgaaattctatgtctccaattccgatatggatcatataagctttcacaaaatgccaatgcgtggatcacaaattcttcaatacatgtctgatctgccatttccttctctttttttttgctttttaattgctgaatatagagtgttgtcatggtgatgacataattaatgtacgagcaagtcccaatttcttccacatttgatagatttctgcaaagaataatgaagaacttgacaagcaaaattgacaaggcttgctgttgttcctctaacccatctgccattttctgaacacactgtagaagctggatcctcagaacctgcagaatattatcaggaagcagagatattcctggaggcatatcatctaccctggtaggcagcttttcaaagtcaacgtctaaaaattgttcatagctagaaacaaaagtgtccaaccacagcttcaggtaatctggatctttctttgtacaataaagcatccaaagttcaaagagcctctctctggatgccattctggctttcactctggcactttaagttttccttaaaaaaattatgttcaagactacagcatgtccattttattttccaagtttttcagccgttcagtaaagctcatagcagtaaagaaagcaaaaagaagtgaaacaaatggactgtcctctggttaaaaacaaaaaggcaatttcagcagtcactccaatatatcttcatcagtggtagttgggcaattaaataaatattgtgtgccgcgcggcagccgccgcccggcagccgtctaactgcttccctcgaccccttcccaaggcgaagccccgtgtcaccccgcagccaggcagacgagcgggc

SEQ ID NO: 13123 - RNA, 10676 nt, Homo sapiens
  source 1..10676: mol_type = other RNA
gctgggattacaggcatgagccaccacacccggcccacatttttggtttttactttttggaaaaagcaatataagaaataattccactaccttgtacatctagtattagtccaggtaggatatctattttattgtgaacaaaacttatttgtactataaagtaaaaactgcttatttcttccatctaaaaagcagcatagtaaaacatcataaacttaggcattttttctaattatctaagttttagaaaacttataagcatccaaaataattttcaaatccagtattaagtaatcttaaaaatgaaggcatttttacatcaaaatctctggataaataacaaaataaaacttagtaggttttgatttagaaaaagtttctaaaaaaatcagtattttaaaaactaaaaatcaatcatgttagttctgccgacttgaaatctcctaaaaaactgtaagataaaaaaaaagatagccacggtggcaccacgggtgaagcactggattgaaacctcccatcaccccaaaaaagaataaaataaatgaatagatgccagtctcatttatgcatcataattattgctacttaacttgagactttgttcaatacaaattcctgaagtcttaagaaaagacaccttgacatttaaatatgttctattttacaattgttgtaccagtttatttcagagttatttacctaaaacatagctattttttccttaataaaacagaggatttttacttattggaaagaaaattcttctatagctttttattagccctgactcacatcaaatcaaatctattcaaaagtttccctaaacagaatcctttatttcttaaaatttttttactcactcaaaagattataaagaaaagggcactggatactgtggtcaacaggaaagcgaaattgcaaaagaaaaatttctctaagattcaactgagaagacaattggatttaaggacatctatgatttgtggaacaaaaaagaatactattactggaaacagatccctttaaagaaagccatgtaaccattccttcctgaaaatgcatttaacatacaaagtctctgcacaatttcagagggattcacaagttctcccaaacacatgaaatctcagattaataacactggtagttgtaaaagctctctgacctaactcaaaagataatcttacaaaaaaatctaagtttaacaatgtctttgaattccaaattaaataaatcagacttttactttaagatcttaataatcaaccacaacatttaacactatataataaaattagctataatcctaaaacatgaaatagaaatttttaaattactatatataaatgattattttaagttatacatatcttttcaattcattcatcaatcacacagatatcctaagtaaaaattcaacatatttgggtactactaactcttaattattagagtaaaacagtatttgcttagtgaagaaagagtcaagaaattcggaactttgcaaatgcaaattgtgctgcaaatgctacttaaaaggcccaactgtcaaaatcacaattagcacttttgcttaattatattattaaggaaatacatctgtaaaatgtatctctagttccacttttttctactcaatttttattaaggacagtaatagatttcagtaacttctcattagaaacacgctaagtagtaatagaattagctaatgtaccagtttcaatattcttattttattcttaccatgcaaacttgtaactttcaccgagttttgaaaatccaagtgtgcaacagatacctttaaaatattatccccaatcaggagttccataaataaattgatatattttcattacagtggtcagtaaataggaaaatgattacttaagaatgtatttaaagccatctctctcaactgtcccattatctgtactcttttattagaaaaatcttaaattttatcatttggaataataagaaaattgaacctaatgttctcattttagtttgttttaaaaatggatacaatgacctttaggaatgggccacaaaatcaaatcaaatgtattttctcaaatacatcttagtatagaccaagaattagtttatataccacagcaaattgtggttatctgtaaatgattttcagggataaaagccttgcaacattgcagagagttgagagatgtggttaaagtgacaaagcaataaatcaggtttcagtaatcataacagaaaatggaaataacaatcacttggaatcttgagtattatattcagtttctccagctgaaatctggctgagccgcttgctcgatccccaaaattttcgagaaagctgacctgaacgcatctcagcaggcttgccaacacccactacaatcaatttgccatcttctaaacctacaagaatatggctgtattctttggtgacacaaacacaatggataggcagtcgcatggctaatgggttgatgctgagattcaagctgtggagatctcttatagacaggaatccttgtatgctgcctgtgacaatgtgttctccgattatacatatatctgatacttgttccttcaggatttgagaccctagatacttgccatttatagaaaacagatgtaatgcattcttatccttgagggtggtcttttcttcagtgctggagtagacaacaatatgtccttcccaagatatagccaaattaggaatggtcaggaacagagaactctcacaaggtggtcgtaaagtcctcatgtactgacctttctgaatggtatgtataatcaccgttccatcccttgatcctgacactgccatgtctagctcagtgctgatgccgacactcagtacctcgttggtgtgtccataaagaatctgaaaaggtttagatgctaagcccacaggaacacctccctgttgtgttatttgccatatcatacatgtagtatctctggaaccagaaatcaaatgtattccacagtaatctgtagctaagcaagtcacaatatccatatgccggatgatgtgtgagataattttgccttttgtaagtgacatcacttgaatgctattatcccagtatccagcactgaagagcaactttgcatcatgtgatactacaaatagcttagaagtgatctctagcccgggagcaaaagaaccatttatactgcgctgagtttttggatttgtcacagtttgatccttgatgaatgtaaagtaattagaaatgtttctgtcataaggcaaccatccatgggttccaataacataattcatgcttattgttatcagtaactcagggctgccttgagacataaaagaacgatactgatttttggggatggtggcctttaatagtggaataccatcactaatcccctctataaaaaatgacttgagttcaggaaggtgttgaaacaggtttagggttgaagtgtctattttggttggcttctgcactgcttcttctgctgataatcttggagggtgtggttcctttaataattgacagggtgtttgcccaaaattattaatcatcccttctaaggcttttctttctttctcatctgttaaggcatccagatccacagctccttcataactacaataatagaaaacgttgagtgcctctactgcagctggtcccctctgtttatagccaaagatcagatctatccattcatgaagatgagctgaaacatattcagactccaaagctttcctatgtttatagatgaaatcttcagctgatttagcccatttcgggagaatgacatcatttactaattctttggaaatctgtagacgacccaagttaaattgattttgattttccaaaaactctgggaaatagaagaattcaggaataagttctttaacatcatatggattatccataagagcttgccaggtagcaggaatagaatggaactgtcgatctgcacagtcaaaccttccactctgaagttggatgtggagggtggtgaacggttctacacgaatgagatagtgcatgacccccgcagaatttgaatagtgagtaccatagtgaaacttatcaatagttcccataggatcctcaaaattttcatatttttctctcatagctttggcgtttttttcattaactaccccaattggtttggaaagatctcgaaatacagcagggttattaaggtccaactcttccgaagtataatcttgtaaaatccagggaaacacaggatactgtgcaaggtcattataggttcgtcctgccattgtatttatttgaatgaggtagtcaaaatttgatatctctctgtttacccatttctgtgtcaatcctgatgctttgaataactcctgtggtgatctgcttccataataactatttggggaatgaagtgacaacagtcggctatatattttgtttctaacctcttttttgaaattgagaaagtagttggattggtcaacatgaaaaatctcaagggctgatcttcttaaattgtaacgccggagatgaatctctcgaatttgagaatgaggccacttgaaatcaaagcctactccatcttctttttcaatgctgccatcatagaagtaaatgtgttgagtagtgatttctaatctgccaggaattacatcaattattgtaatgagttcacagtcttccatcaataccaatttttctttttgatcctgttcttctttctcatcaacatttactctagctgttatatcctcttcaggaaggtctaatttatcctccaccatatcactaacttttacttgtttcactacttccaaaagcaatgtatcactggaaggctgtgagtgttggatacccagattatctctcaaggcactagcttcctcatgggttttgaaattataattcggtaccagcttaagtctcatgcgggaataattctctacattagctagcttccagtgaattggattctgtttccttttagcccaaggtcccctttcacatgtaagatagagctgtattgctttccagcgtctaagagtggctaactgttgactgctaagttgtttaagcatattattatacctcaggttctcttggcgtgcttttcgattaaatggctccacaaacagctcctgaaatttgagcttgctttcccctccttcccggtctcgtttatgcatatttaccattaaagcttcataacaatccttccaataaagtgccatgttctcatgaccatcgtaaaatgtatgagcttcatactgcttcatataaggtacaatatatttttcaatgtaaacttgccattcatttgaattacaatattcttgaaaatcttcaaaaaatgaggagctaccattggtaaaaggtaaagaaggtaggtgcaagttcatgaagagaagctcataaattttggaaaccagggtacgaacaaggggaatcagaaatgagtagatttcagtctgttccttgattgattgacttagaacatgttccagcttccctaaaatgtaacatgcttcatcctgattttcaatcactttggtctgaagaagggtatttagcttagctgatgccattgcacaaacctgcaaattaccccttccaatgaatcctagaagcaactggatctgaatttgagagagttttacccatactggactttcagaatagcagactgacagacagtcaaagagcagcatcatatcctctaaaagcttctcggtccacatgtttgaattaactagtccctctgactgaagaaagtcctgtatgatcagcactagtcggaaggcgttttcagcagttactggattagtttttgcttctctgttttctgagattgcccattctaacatcttttgtagcaaagttagttttatttcatctgatggtcgaagtagttcactggatattcctggtttacttagtgctgaaaacacttgtcctcgttcaatccaagtatcatcatcagacttttctagtcccttacacattacataattcaaaatatgtgtcagtaattgaagaagctcctcctcacatctctcttggctttcaagtaaagagaagtcatcactaaagcccatatcatttgtgatgctgctttctctgtcagagtgcacagaaaacgatttagtagactctactggggatggtgtgctaggcagactgtctggcacttgacttccactatcactcatttcacatgagtcaattccactgaggtctaaactcaaatgtgaagggttactatgccagaattcctcttgattctctgatttgaaagacaattctcccacagagctatcttctggaaataatggtgtgtttgagtctaaagagtgtctatcctccaaactccactgatccgaagacacattagctgaggcaaaagaggtgattttttcctcatctgttttttcatcagagttcttcttggtatcttcagttgacatatttttatcattgtctttcattaaaacagctctactgtgcttatgaagagtatttccgttttcaaattttgcttttaaaaaaagcctaactaaggtgtcttgccaacccacttgctgtgatatttgatgtgctgcatctggctggaactgcaaaatttgcaaaacctttctgcagatggccactctaacatttatatgtgctctgtgagatatatataccacagatagtagatctttgaaattaataacaggatctgtatttatgatttgatgggtgaggtttttaataagagaagtattaacaagtgcttcattaagaaggagtcccagtcccgagtagccaacttctctgagtcgaatatgttgtttactacgctcataaacgttcgtgcatttcaacatttgttccataatcttaaaaatgatttctcttagtctgtcagagtacttctgatttaagagcaatgcgtacagtatgtcagcatttcctggttcaaaaagcagtaagaaaagctgacctctggttgggctggtacgtaggagactgaagagcacgtccaaaattccaaagagctgttcttcttcattagtagcagctatgtaccccataatactttgtatctcttcatgagatccacctttgcacagaaaatatttaattagtccatacaaagaagtccttattgttcgaatatcatctagagatagttcattatatttacaaccattcccataataaatcctaagtgtatctaggagaaactgcacaccatacttctttcggaaaactctcctgctgtctttaatgatggttgaaagatactgtatgtgaccgattcgaaagggaaaatctccacggttccaaatacgaaagtcaaagagtaaatattgatacatttgttgcaggagctgcatatttttctctaatgatacttgttcaattagtaactgaactgccatcaacacattaacatccatcaaggtgcttggcaccttctgaagtaaagcaccaagagttgcaactccatgggagtgaataagattgccctggttgataggatgtctctgaataaaatgtttcacaattaagataaatgttgcaactaggtttctctctagtcttgactctgaggcctttgtggaagtccatacgagccaatctccttcaacaggtgttactgattcaggaactgtgctttcattcttttcttcaggaatctgtccttcactaaagtggctgatttgttccaataaaggaaagagtacatttaacccacctatgcagtttatgatatccttaatgtcccagttcactactttgtttcctgttaatcttccatgcaaacaattagtagataaatcaagacagattgaatttttgcaggcctttgctgtgtagtaaagaaggatgttaccaggcaggtcggccatgtcagactcttgacacttccaagggcttaaacaatttggacctgctaaatataatgccttcacctgaggaggttgtagtggttcataaaagatgataacagatcctagctgaccctccagagatgtgggacacccccattcactgtcttgggttccagctgatatcaatttggtaatcaattttgatttttcaattgttcctccccaggaggctgatgacagaattccaccaaatgatgtccgatgaggggtaatgggagaagagaaaggtggatctgggatttgggatggtggaggagtggtggttctttgcccagctgaaccaatgcaacaggaagtaaagggttcattcatggcaggaaatctgagaggggcagaaaccttctgttgtccattgtcatagatatagacgaagctctgaccaaaaggcctttttccaggcatgtggacaacagttatgttgtgccagagggaatcacagaaactgtggtcaggaagcataaccgttgcatattctctttttgtgcacactgccacgaccaacatacctgaatgggtaataaaggcttcaaaacccatgccacttcctgtaaaaaaactgtacaattgtttccttttccctcctttgttagcaatgccaagagtcaactgatcctggtctaagcaaaaccaagcactgaaagaaaaggcagaccctggccatttctgtatgggaggcacagaaattcctgccatactatgtgacaaattgaaatactggagggcactctctagacttagttttcgggccattgtcaggattgctcgagtcacgggagtgacataagggtgaacagactcagattcatccactctcagcaatctcagtagtcgacggatttcttctgagctcactgactgactccccaaggaaccatggattgcaatcaagttctcagcacaagtttgatggagggaagaatgcaagtcaagggtttcaatgattctaatccccatgtttgcattgacacaagtagttcgactctgtctattaatacaacaaattcttttcagccaatcagagatgaagatttgcaggtcatgggattgtagttctggaagccactggataagaagcaagagaggttggacattactaatgcccaaaatcccaactgaagtgtggtcaccctctacagccatattcataagttctttaagtaattccagtggtggctgacccagggattttaatacttcaagcatatgtgtataaccaattctttctttaaatacttccttagcagctggagatttgttcattactgcggtcaaagcctgaatggttgatatggccaaacaatccaattgtccctgaaacaccttgcagttctgtagcagtcgtatgagatgttcaaagcaattgctgttaagaaaaatggcctgaagaacaggtctatctgtacaatctaacatggctgtgatggtattcagcattttgatctgtagagcaataaatcggttttcccactgtctggacctcctttgattaggtaaagctgaatgatctgaatttagcaatttaaaatagttctccagaatagtactggtttccacttgacgctgatcagagttgctactgagaaggatatgtaccacttctgtaaggcacttcagagttagttctgccttcctacccacttcttcaggatctccatcctcccaggaatcacaatctgccaatactcgcataagaacttccatagtggctggagaaattgcttgcaaagcattcctctgcccaccggctacaatggctccaaagagatgcaataagcaacatttaagactttccttgagatgttcactttcctgaaaacattgataaaagaaagggacgaattccactgtgagagaagctggtttatatttctgtctgctcttttccacagtactaaggattcgtcctgaaattctatgtctccaattccgatatggatcatataagctttcacaaaatgccaatgcgtggatcacaaattcttcaatacatgtctgatctgccatttccttctctttttttttgctttttaattgctgaatatagagtgttgtcatggtgatgacataattaatgtacgagcaagtcccaatttcttccacatttgatagatttctgcaaagaataatgaagaacttgacaagcaaaattgacaaggcttgctgttgttcctctaacccatctgccattttctgaacacactgtagaagctggatcctcagaacctgcagaatattatcaggaagcagagatattcctggaggcatatcatctaccctggtaggcagcttttcaaagtcaacgtctaaaaattgttcatagctagaaacaaaagtgtccaaccacagcttcaggtaatctggatctttctttgtacaataaagcatccaaagttcaaagagcctctctctggatgccattctggctttcactctggcactttaagttttccttaaaaaaattatgttcaagactacagcatgtccattttattttccaagtttttcagccgttcagtaaagctcatagcagtaaagaaagcaaaaagaagtgaaacaaatggactgtcctctggttaaaaacaaaaaggcaatttcagcagtcactccaatatatcttcatcagtggtagttgggcaattaaataaatattgtgtgccgcgcggcagccgccgcccggcagccgtctaactgcttccctcgaccccttcccaaggcgaagccccgtgtcaccccgcagccaggcagacgagcgggc

SEQ ID NO: 13124 - RNA, 15931 nt, Homo sapiens
  source 1..15931: mol_type = other RNA
gctgggattacaggcatgagccaccacacccggcccagaatgttcgtaatttcatataaacattttatttgcctttctttttcttttcctgaagatgttttgttgcttacttttcagtttatactggctttttaaaacagatttcctttagagtaattacttccatagtgacagctatatttactgaaataaaatgtttcaaacatgtctcgaagtttgaatttctgtcactaaagaaaattagttaagattaataagaatgttttttgttttttttttttttttttctgcaggtgacttcacctttgattttcctacatttaggcaatgttagtgatgttctttaaactgccaggtagaatttcaatgtttgcaatacaaataccattaaatacttttattatagttactttgataaattcttttaaaaatactattttggtcctttatagaggtagcataatatttaaaactaactttaaaacaaattattttactaatctgcttgcattttattaaattccctttacagaattaatgaacttttaaagatttcataacaaagaactaattaatgagaagcataaataacagcttatgaaagaacaggtaatgataccttaatctgagtcccaaggaccactttccaattacacaattacaagccattaatttaaaatatcaatcattagactattatcaattattggaagtgtgtattatataaaaattatataaacatctttaataaagcaatgttgattacattcaggtgtatgatgtgatgaaataaagctagtgttcactggcagatattcttaggtaaccgctttaaagactaaacattttgaaatgaacatttcattgttagctgctaagtagtggttttataaaagtattgaaggtctgggaaagaagaatttcctaattattctaaaaagttttcatctttcttttttttaaaccataattgtatgtttgttcaaggttcagataaaagtggcagggatcagggttaaaatctgttctattccatcaaaaataaaccacatttattatttaatattttctagctattctcataattctttctctgtcaaatattagggtttaatagctgttatataatggcttgaaaacataaaatatttaatattttaataaacaattttttatacaatttttattgtacgacactctatctttgataattttgacttaaataaagtgttttattaatagtctacttagtaatatagtttgtatttccttgttttgagggagaagtggttgaactaatgagttttgttttcacttgcttctctttctattcatttgtaatttttcagccataatgggtttgaatatatgccaaccactgaagtgaagatgatataaattatctcatcaaatccttaaaagtattagtacctcatttcatatatgaggaaactgaggcttagggacattaaataatatcacacagatacaaagtcacagttctttgtgattctgtagctcctgattttaatggttatgcaggttgcttccctaacatatcaagtttaaggttattataactaatgagaaacatgttagtctttatacttaagtcaatgaaactgagtgtttatatgtttgctttatctatcctagtcacatcttcctgaattttaaaagcacacagaacacaaatcagtccaatgaaccaaatctaaactacatagaaaatgaacaaccataaaacagaatttaaggtccaaagtaacttgggagatcaactaaattcctgcgcttttgactataagaaacaagcccgagagagaagtggtcttatccaagatacaaaggagatttgagttatatagcccaactttttgcacactaattccatatattttcagaaagtagctggcatttattgagcactttatatgtgtcaggcactgtgcagtatggttactgttgaggtgagtgttgttattaacccatgtacagatgagaaaattgaagcatatacatgcccaaggaccaaggttagtatgagccaggatttaaatttagatgtagacagcattggactcagaatttaaaagattcatcatgttttcataatataacttcccatccaataggctacagtcttatagacacagttgctgttagatataattggcctccattacaaaacagctcacttcctgcttcctccttacttcagatacactagtaaagcatgctatattccaactaatgagggcagttatgtaaaatacttagcaataggatagctgaggcctaccagtcaaaacagacactagtccaaacagaatagagattggcagcagaccacaggaatgccagtacccattgatactacttgccaaataactgtcctgaaaccaattaaatcatgcagtcaaggactgaaaaagtatatttcccccctcatcaaatgtctgaacttctgcatttattaagcaaggaaagacataaatagaaaggaaaataatgctaatacagaccgtagtgagtgaattgctttgagactattaactaccacaaagtgtacagaaagaaaacaacgtgatccagctgaagaggatgcatgcctgttaataacaaccagcttccaaacttaataatgatatcgattgcaaaaagtaaccacatgacaggtggtagactattgcacctgcattgtagagacattaaaatgttcttccatttgactgctaccatccccactatcagcaaacccagtgtggatttaaatgccgtaattggtggtgtactagcatcaaataaaactatgtcttactagaaattatagatttttgaaacaatatcagaaatttattactttttttttttttttgagacagggtcttgctcagttgcctaagctggagtgcagtggcacaatcagagctcaatgtaatcttgatctcctgggctcaagtgaccctcctgcttcaacctcccaagtagctgggactataggcacatgccaccactcctggctaatttttttttttttttttagagatagggtctcactgcattgcccaggctggtctggaaatcctgacctcaagcaatcctcccaccttggcctcccaaagtactgcgattataggcatgagccactgtgctcagcttatcttgattttgtttttagtattttgatttccaatgccttctgaatgctcattcctggggctcttttgacacccacatattctgaattaattttcagcaataactacatctatgtgtactctagcaaccagatagaatatatgctacattataaagaagtctgttctctttctgttcaaccatgttgttcaatgatcccacacaccatgagaaaaaaggcctgccatggttgtgtgttatcccatggcacctcatcttcccaatttttttcccccagaaagaatacagaataatgaaaacctttctgacagacccatcttgataatagctgtgcaaattattgagtgttttgaggaattttgaatgctaattacctttaaatagatcatctctacatgtaattcttaccccaatacacaagaaatttgattttcatcataaaaagctggcaatttgtcaccatgtgcttgtgaattacatctgcatgaaaaatacatggtgcttcatgtcatttattcaatgtatactcagtaccagatactctgtcaactactatatatgcctttaattctgacaaccaccatatgtgttagacatcattgtccccattttaggaaaagtacactgataaccctaaagtgcaagttattgccaaggcaaattggcaggtcagtggttgaagcaggattccaaagtaagtcagcttgatttcaaactgatttcttaataactaccactctccactcccttctttacaagcatatcatttctaggaaagactattctcatggcaataaccaagataacacaatgtgaacctttaaatgatatatgctgtatttttatatgggatatgacatagtgaataatgactgtcttttttaattttgctgatgaagatgaaaaaaaaaaaatctctgcttttcacatgcaaagaattcattttgactagccgactgtcgaaatgtttaactttgtgtctacttgtgctttgtggacttttcatgatggcgatattttgttgcaaggtgatttttttttttttttttttgagtctcactctgtcaccaggctggagtgcaatggcatgatcttggctcactgcaacctccacctcctaggttcaagcaattctcctgcctcagcctcctgagtagctgggactacaggcacgcaccaccaagcccggctaaattttttgtatttttagtagagacagggtttcaccatgttggccaggatggtcttgatttcttgacctcgtgatctgcccacctcggcctcccaaagtgctgggattaaggtgatttttaaagatacctctttgtatgcttttctgcaagctggttcagttttgagtttgtctgtaatatataaaaaggatgttcttggctgggcgcagtggctcacacctgtaatcccagcactttgggaggcctaggtggggggatcacctgaggtcaggagttcgagactagcctggccaatgtggcaaaacccatctctactaaaaatacaaaaaattagccaggcatggtggtgcacgcctgtagtcccagctacgcaggaggctgaggcaggagaattgcttgaacccgggaggcggaggttgcagtgagccgagcttgtgccactgcactccaatctggtgacagagtgagactccaactcaaaaaaaaataaataaataaaataaaaagatgttcttcaggtctttttaattgttatctcagcacatcctatgaatgtagacatactgattccatctaaagctttcaaatcagatgcatggccaccaaataatcataaaaacaaaatttcttttaaaaatgttgatgagtaatcaagagattttaaggaaaatatatatgtttgtttgttcttgtaaaacgcatactgtggtctttgagcaaggctaattttgcacaagtcagaactccacagctctttctggggctattaaaaaaagagccatctggccataagcaactgacagagtggctcttcccctgtagctgggcacccaccagggcctgggcatggctcttaacactggatgaggtacaacaatttacagaatatgttttctgtttccaggggccccattgtataggcatgaagcagactcacaaaaaattacaatatataggtgctaaaaataaatgtattttaaagttatattaaccgcacaaagcggtcagataattggcaggtgtgattccagcggctttggaagagaggtctttgacttgtatcttaaaggacaaatatgtcatcaggcaaaggggaatgtcacaggatgaaagaccttgagcacatatatagtggtttgaaggaacttgagatcccaggaagataaactgaaagcattttgtttgctcatttcatatatatatatatataaaatctagattatatatgtaattatatatatataatctagagcatgtaatgaaggaggaggcaatattggtaagaaatgtcagggagcaacatgtagtaggatacataagtcacacaaagagtttgaattctatcttgcaagcaataaaaacgcatgttttgcaagcactgcagtatcgtactcaggcattccttatagattatgattaccctttgtccttcaatgtgttggaaaggctaaattagaaaaagactaaaggaagggtcttaaccaagtcagagtcagggaaccaagaggagaaaacacatttgagaggccactctggtgctggaactagcagaatcctaggctgattatttaaatgcagtggtgtggctcatgcctgtaatcccagcactttgggaggcctaggtgggtggatcacctaagatcaggagtttgagaccagcctggccatattctgctcaaaaaaagcaaagaggcagaaagagcccaggctgacggttaaaaaccagcagcttccaagaaagatttttgatgagcaaaatttaactctcctggaaaacattcttattctgcaccagaacttaccaggcctcggtaaatatttgctgaatgaaatcaaaactaaaccaacaaaggcccatcctatcccaactagggagtttagaagactttttgagccagcatagttttttatattaggaaaagagtgacccaatactgaggtttattatgtcattgaagtaataagaattcccctaaggatatattgaggttttcgtctagtttagacttcataccaaaaaaaaaaaaaaaaaaaaaagacagatatgatcacccattggtatgtgtgtgctaaaatgacatatagtttgggttattaccattaaaaacttttgtatccttaactttcagtagagccagtgaaaataaagcttatataatatcccctaaagcacacatttttatctatgttatgggaaaaaaaaagagcataaattcagaagccagtttactaatgccctaatagattgtgacatacgtgctttttcagcggaatctacaaaatacttagagcaacatctcaagtacgaaacaaattcattcctaaaaataacccaactgaagaccttttagtagctctttcagctcaccctatgggtacagacatatcttgattccatctgaaaccttcaaatcagataaatgtgcagccatcaaataatcacaaaaagaatttttataaaaaataggaatggatgaccaagggctttaaaagacaagaattttgaggcttctaaaatgttccctttatttgccataaatgataatatatgtatccactgagaagttatgatagctccatcatgaaaaatctgaaggctagtcagtctcaaggatggtcaatttattaagaggcaggaaaacaattaagagtccatggagtcatgctcagtggtaattcctgactctgccatttacaggatttgtagctatagactaatcacttaatttctcttgaagctaagttttaaaatctaaaaattaaaataacgcaccttacagggttattttaaagacagaatgcaaacatacgttatcacacagtttgcacaaggtcttatataaacaaaggttgttagtaattatcaggtgccattattcctttagattgagttccatcgtggtgcttaataaaaatttaaatgtctgcatgtgtaattacgaaatacaatttctaagttttcaaatacttggtggaaacttgaaaatttaattcaaattaagttctgactttagcaatgtactctctcattgctgcatctattaaaaaccaagaacatctaattatgacagttgcatcaaccttaccaacaggtagaaacatctcttttgtcaccttagatgtcctgtcaatttaatgaagtagtataaagtgattatgcaggctctgagacactggaatgcattagaaaaagtgtttattacctgatctgtgagtttcttaatggctcacagacacttttctctgaatccccggaagaccctaacatagtgctgtagaaagtagatgaatagtaaatatatcagatgaagagatttcttcagggacatagtgagggagaagatttgcctgatttggctaagaacgcatttcactattctgtgaggcctctgaactcagcctagtgtttggaacagagtaggaggacattaatgaattattttgaatgaatggtattttttgactaatggtttagtctgtatagaataaggtctgtaactcttggcaaaagtacccaagaatagcatagatgttactttacataaaatccccaaaagtaatatgaattacttgttagcactgtctttcatagtcaatgttccaacagagattctacaaacaggtaatactagttaactgaaatgtcatgaatttatttcctgattcaatctctgtcaaatacattattaatgaaatggccaagaggggttagcaaaaggggttctgaaaaatcatatgagactaatcaattgaagttgagcatatgaatagatacatttccttgagtgcctattgaaaggatggacagatgtgctataaattctgcggcagaaaagtactatgagaattcttaaagaaatctgacatttaaaaccaatagcgtggctgggcatggtgtcctctgcctgtactcccagcactttgggtgatcgaggtgggatgattgcttgcatctaggagtttgagaccagcctgggcaacatggtaagaccgtgtttaaaaaaaatttaaaaataaaaaataaagccaatagcatctattttgaaataggggaaaagcctattctgataggataaatacaatgacattatctgtatcctaaacaacatagatttcaccagtataaaataagatgctctgtgtatgtgtgcatacctaaaaggtattcgtaggaacacacaatttagttgggaaatttaaaagaacatgaggatttcatataaactcctcacacaaaaaggatcaaatggcctttagaaatgcaagtcatattcatgataggagaatacgaaagtcctattacctcttttattcctgccctcctgcgtcatttcttctacattaacagcacaagtattgactgtatcccaatgaacttactcagataaacacaatgtggttttcttttaaaataagactttactgaatatatcaacaaggtactgtatagtgtagagtgaagtttgtcattaacaaagtgtgcgacatggtaggtctcagaggatgtgtgatgcagaatctttcagccccttatcagagagaacacactaaacagaaaccagaagcaaatcagcatatggttcaaacaataacaaatcatcaggttaactttcagtgaatatacactagtcctatgagcgacacacacttggcaatgccttcaccttgccttaaacattataaatcttacattccagggacacctttacaaatgcccctgtttgtgtgtgtgtgtgtgtgtgtgtacaagcatgtgcatgtttgataataatttttaaatgcctgttgcaatggccttgctttgtgctcttctggtgggtgtgcaggtagaaaacaaaaaactatagtaaaaaaatttgttttgttataacaacggtatcagacatatacaaaactctttctccacagtgacaagcattccccattgctagtaactgtcttttgaccctgctgaagaaatcagagaaggatgtaggttatgccttcttagcattcatattttgactttagaaagagcatcaggcaaggtttgacaagaccaagaacaagaccaagaactgttttgttctgtgtgagtatcttttttccatttggggcactgttttctgctttgctttcccatgcagctggaatggtaagtcatgagcaaaactgctattctcatgttctaaagtaaaatgtaatgtctccttgttataggttagagaaaaatgctataagcaaagacaccaatgggaattaaccccttcacttttcaaaagctgcgatggcctctgcagccaaggtccggagatcaagtgaagcatccattccctgtggactgcaatattgcctcgtgttctgaatggatgcttcaatcacagcatgaagatgttgtcctccctggtggggaaggaagttctgatttgtgtgaaatgactaagaccattatgataggtgctagtagaaaatgaagctgtaatattagctacttcattaatacttcttaccagactggtcacgtactttttgtttttaacctcagggagaatgtctaatatattttcaacgaacatccagataattagaaattgcattatttctcacaggggagaatgttttccatttgttacacaaggaaaataggcaggggatacattcctcgtatctgcctgcgattgtcccatgcagtgggctgctaatgcatctgacggtgtttgagggtggcccagagtctctctataatcaaacatatctccccaaacaagcaggtattaacaactaccctggctatagataactgtcaatatatccttttgatcatgactatgcctcttccttttcaatgtcttctgtacagtgacatttaccaagctctgaatgggatcagattctatctgagtcacctcatttggccaggcagcatcaagctctttattggccagtgagcatggctttttttcccatggtcttggcctgtactcgcaaccttgactcttgactaatcatctcaaaatacatcataatgacagcaagagaggcccaaacacagagcagatatatcagcaaatatacattcccatgactaaaaatgccaatcaaagcagaatccccagggacagttgtttggcaattttcataagacacattagacatcacagattccatcacgtgctttctatcctggtgcaggtgaggctgtaacaaatgggagacggattttaatcttagcagtctttgccatgttgtacacaaggtgaaaataaagcctgttactaggttcaatctcttcaggaacacctccagcaaaagggaccctgtcagaccatcttaagcattgcacatgactgtctccattgtaccatttaagccccaaataattctgtgaaccccataagaaatgacaggaacctcttcatccttgttcttcctggcccaaagtggtttcagcagccagaaatcccactgggggttaaacatacaatatacataaatgagaatgagtattttgtgaataacagaaataaaaaccctcaaaagtcaaagtaccatcatttgaatgcacaattttatctacacagccaaggggaagaggacagtagaagggaattatccagctaagtacacaaagcccccatgtcattgtcttgattttagatgtcttactgctacactgatcaccttcacagactcttttcccttcactgtgtggacctaactttaaaaaaagcaacagccaaaaccctctagctaatagactaaaatggaaaccagagtcactttagaattaatttaaattaattcatagctaagttcagctctactgactgcacagtttcaattcttgtgtctacgacatacagctgcagttatattttctgcttattctgagggacaagggagattaaaacatataagttgggctatattattaaagaaaataaagctcttactataaagaaaaagttgcatagcattttatacctaaacttttacaaagaagacacatcacagttttattttgctgagagagagagagctagtaagatgattgtgacatttacttcatgggtccctataataatggtcaatggtaaaagaaatatgcagcacagagtgaaatgtttaaatttgattttcgaaagatattttttccaagggagtagtttttgataacgtatgtgatctatagcccttctctatctaaggatggcaaagattaaattatgtgttttctgaaggtgttgtctcaaaagtatctagaattaagcacggacatcctctcttttctacgccctgctctgccaggattaggggaaaaagccttcactctctgacttgtttttcatgggttgtcctgctaacataagattgattagccctccacaattgccaaagtagaggaacatccacgatggaaaaggaacaaataaaatttcaaaagtggaacaggatcaaagtcagtccaaggtggaaaccaggtattgctttttaaaaaaaattcattattttggccagctttgatgtgtccttacagaattattagcagtgaaaattagtactcattttaaaatgtataagtacgtaatggatatcttgtgcagccaagactggcatccataattttccttgaaatactgaacagagggagaaaaacaaaggtgtcataaacaactaattatgaaaatatatgggagatgattggaagacaagaatttgcaaggggataaaagatattacttcaagctatttcaacatgatactaacaaagtcagctgacataacagaaccactgatcagttgtttttgtctaaatagcaggaagggtaatttttaaataagtcattgttgtattttccaaacattgatcacctgttggtctaaatatcatgttgacatagcctcagtgaatctacccaaataattctcattatcaaaaataattccattcaatataattcttccctttattagcctcttctaaaaaagtattctagaatatatctctgttgaatgtgattcaacctgatatatgatttgaacagtaacacttttaaagggagtcttcttgctacaacatcagactggtccctgaagatgactgaaatcagactcaagtctctaactctgttatcacataggaccagggaagcatgaagagtgatttttaagttcccagtcagaaagccaacccctgcattttcgggtcctttcaaatctcatctcaattttcttgattctgtcaggccgggttaacttatctcacgggaaccggcttcctcctggtgctttcagcatttcccacacagggtcaaatcagggtaactacctccattcttacattatagaattttttacctgtcttccggacctggaggtataggaatagtgtgaaactatcgggccatttcttgttttacccatattattcctcttaccctgatgagtccatttaatctgccctttcatctgaccaccaggaatttattctgacagcttcaacagcaaagtggttgatgtgtatcctaaggaaaaatcactcgttctttttgccttggcattgggttctcattgtacaaccctgtacagtacttcagcaacttttttttttttaagatttaaaaagcaaagagttacaaaactgtttgtaattaacttgaaatagaaaagatagcactttttttaaatcccattatatagtacaccgtataaattacagagtattcaaatgcacaaatgcatctgtgtaacatttatcaaatgtaatctgcgtgtctttatgtgcacacacgagtgtgttctcaagagtctaattgtccgccttgataacgctgggcctctggctgtcacgtatggcagtgctccaggtctggcacgctgctgttgcagtatcgcatgttgttggggatatggcagtctgtgtaattaatgcccccatttggggtgtaaatgggctgcagtctgaaatctcctttaaggagttgatcgttatttaaggagacgatctgaaaactggtttctgtcatctccaggatggagttgtccttcttggtgcctgcctcgcaataatcatctttccgccggccccggttgtatttccacttctgggaggtgtagcgcccctttttgtgcatatgccagcaaaagacgctgagcaagaccaccagcacaaatatcaccgcgcccccgatcaagcccgccagcagaaagggggagcccatgctgtgggacgtcgtctgctcatggctggacgctgtgttgctgccgttgttcagataggaggcatgggtggtggcctctgaacaaatggtgtcttctaccgcgcggtagttaaaagcatccagtggcactaaacaaatccgataggtggatcggggctctaagttaaccaggctcaggtgttgcttctcaccgctgactatgcgctcctgaacgatgccccctactaaactgtggcccattttcacccatgtgagtttgtatgccatcacggtgaagagagagagccagctgacttgaatggaagtatcattcacaaaatggatagagagctggatccgttcagaaataggtggggtcactctttctctgccatcccagtcaggaatcgtgggaagtttcgatgtggtaggagttggaggcgtgtagcttctgctagggtttggaatagagagggtgggaggctgagtggtcggagaagctgtacttggggctggggtgaagagaggcaggccgggggtcgtggtgggacaggacaaaagattcatatttaattccctgacggccatcccccggacttgttcaggaccttggcacatgaaaccccgcacgttgagagatgaagggatatatttgagccattctgtgacccatttaatactgcagtcacaaaaccaagggttattccgagcagtgagctgcttcaggttggagagattatcaaaaaccccttgagtcagcatccgcagttggttgttggatatatccagccgttccagcttacgcagatttgagaaggctgtcaaaggaatgtggtttatctggttgtcctgcaaatagagcctgatcagatgcgtacctgggagatcgggaggagggtgggacagcgaattacgtacaattgaaaattccttgagcttggtgagatggctgaaggtgccctcggcgatacccttgttggtcaggaggttcccgtccacaataagacgctccaagctcgtgagattctggaaggccatgtcggatatgacagcaattcgattttcatccactctcagctcttgcaagtccacaggaagcccaacaggcacactgctcaggtgattcttagacaaaaacaacaatttgaggctaatagcctcccggaaggccccgtcttccacccccactgtggatatggagttgtcatccaggtgcagctcttcaagcttcaagagctgggcaagagcagcccgtgaaatggtctgaatattgttttcctgcaaatggagaactctgacattcttgggaaggttcatggggaattcgtccagttggttgccatacaggtagaccgtgtgcaccgactgtacattgtgcagttctgcaggaaatccagcattattaatttggttgttgtggaggtagagtacagttacgccctccgggatcccaagaggcactgaggtcaagcttcgctcattacagtagacaaagttcctgtcgcagcggcacacactagggcaggccaggagtttggacacctgtgagtagagccccagggaaatgataagccaagacttcaggaaaaaagccccatggctgggccactttgtggtctgtaggcccatttctgaagtacggaaataaaatacaatgtggtgggaaaaagaaaaagaaaaaaaaaataaacagcaaaatcaaaatgactggatggggttctgttgaagtccagaactccagctagagggaacgtcctgagggcgtatggtaaaataatctccctgctgtctctggtcttatcagcctgtgttgccctctttgctgctgtcctccatgtgcaaaaaattcaacagggagaatttttccacactggcaacaggtgatggcaagttatcagccgtgtcaacacaagcccaagtgggcaggcagaactctcttcttcttttgtaggtcaagccagccttgattagcctacgaacttcttggttaagctcaatctgcaatatttacatagcccatcttctccccacagtatgtgactaatacgtatcccggggaggagggagcgcggctgggggtgctaatcggaagggaacagacagtgagtgccatcttgctgggaggttccagaagcaaagcgccaacgacgacagtagcggtggcctcagctccaccagtaactgccgctggcaggagcaccacacgctctaggagtttcccgggtatcaagtatgggtccagcccgtcccagttatcctcttcccctatggcttcattcccgttgtcagtaccccgacctcagcttgcaaccttgatcttgggcttgattataaatgacgaaagaccgcggcagccttcaaagtgcgggagcgagccccgtactggtcagcgcggcg

SEQ ID NO: 13125 - RNA, 15675 nt, Homo sapiens
  source 1..15675: mol_type = other RNA
gctgggattacaggcatgagccaccacacccggcccagaatgttcgtaatttcatataaacattttatttgcctttctttttcttttcctgaagatgttttgttgcttacttttcagtttatactggctttttaaaacagatttcctttagagtaattacttccatagtgacagctatatttactgaaataaaatgtttcaaacatgtctcgaagtttgaatttctgtcactaaagaaaattagttaagattaataagaatgttttttgttttttttttttttttttctgcaggtgacttcacctttgattttcctacatttaggcaatgttagtgatgttctttaaactgccaggtagaatttcaatgtttgcaatacaaataccattaaatacttttattatagttactttgataaattcttttaaaaatactattttggtcctttatagaggtagcataatatttaaaactaactttaaaacaaattattttactaatctgcttgcattttattaaattccctttacagaattaatgaacttttaaagatttcataacaaagaactaattaatgagaagcataaataacagcttatgaaagaacaggtaatgataccttaatctgagtcccaaggaccactttccaattacacaattacaagccattaatttaaaatatcaatcattagactattatcaattattggaagtgtgtattatataaaaattatataaacatctttaataaagcaatgttgattacattcaggtgtatgatgtgatgaaataaagctagtgttcactggcagatattcttaggtaaccgctttaaagactaaacattttgaaatgaacatttcattgttagctgctaagtagtggttttataaaagtattgaaggtctgggaaagaagaatttcctaattattctaaaaagttttcatctttcttttttttaaaccataattgtatgtttgttcaaggttcagataaaagtggcagggatcagggttaaaatctgttctattccatcaaaaataaaccacatttattatttaatattttctagctattctcataattctttctctgtcaaatattagggtttaatagctgttatataatggcttgaaaacataaaatatttaatattttaataaacaattttttatacaatttttattgtacgacactctatctttgataattttgacttaaataaagtgttttattaatagtctacttagtaatatagtttgtatttccttgttttgagggagaagtggttgaactaatgagttttgttttcacttgcttctctttctattcatttgtaatttttcagccataatgggtttgaatatatgccaaccactgaagtgaagatgatataaattatctcatcaaatccttaaaagtattagtacctcatttcatatatgaggaaactgaggcttagggacattaaataatatcacacagatacaaagtcacagttctttgtgattctgtagctcctgattttaatggttatgcaggttgcttccctaacatatcaagtttaaggttattataactaatgagaaacatgttagtctttatacttaagtcaatgaaactgagtgtttatatgtttgctttatctatcctagtcacatcttcctgaattttaaaagcacacagaacacaaatcagtccaatgaaccaaatctaaactacatagaaaatgaacaaccataaaacagaatttaaggtccaaagtaacttgggagatcaactaaattcctgcgcttttgactataagaaacaagcccgagagagaagtggtcttatccaagatacaaaggagatttgagttatatagcccaactttttgcacactaattccatatattttcagaaagtagctggcatttattgagcactttatatgtgtcaggcactgtgcagtatggttactgttgaggtgagtgttgttattaacccatgtacagatgagaaaattgaagcatatacatgcccaaggaccaaggttagtatgagccaggatttaaatttagatgtagacagcattggactcagaatttaaaagattcatcatgttttcataatataacttcccatccaataggctacagtcttatagacacagttgctgttagatataattggcctccattacaaaacagctcacttcctgcttcctccttacttcagatacactagtaaagcatgctatattccaactaatgagggcagttatgtaaaatacttagcaataggatagctgaggcctaccagtcaaaacagacactagtccaaacagaatagagattggcagcagaccacaggaatgccagtacccattgatactacttgccaaataactgtcctgaaaccaattaaatcatgcagtcaaggactgaaaaagtatatttcccccctcatcaaatgtctgaacttctgcatttattaagcaaggaaagacataaatagaaaggaaaataatgctaatacagaccgtagtgagtgaattgctttgagactattaactaccacaaagtgtacagaaagaaaacaacgtgatccagctgaagaggatgcatgcctgttaataacaaccagcttccaaacttaataatgatatcgattgcaaaaagtaaccacatgacaggtggtagactattgcacctgcattgtagagacattaaaatgttcttccatttgactgctaccatccccactatcagcaaacccagtgtggatttaaatgccgtaattggtggtgtactagcatcaaataaaactatgtcttactagaaattatagatttttgaaacaatatcagaaatttattactttttttttttttttgagacagggtcttgctcagttgcctaagctggagtgcagtggcacaatcagagctcaatgtaatcttgatctcctgggctcaagtgaccctcctgcttcaacctcccaagtagctgggactataggcacatgccaccactcctggctaatttttttttttttttttagagatagggtctcactgcattgcccaggctggtctggaaatcctgacctcaagcaatcctcccaccttggcctcccaaagtactgcgattataggcatgagccactgtgctcagcttatcttgattttgtttttagtattttgatttccaatgccttctgaatgctcattcctggggctcttttgacacccacatattctgaattaattttcagcaataactacatctatgtgtactctagcaaccagatagaatatatgctacattataaagaagtctgttctctttctgttcaaccatgttgttcaatgatcccacacaccatgagaaaaaaggcctgccatggttgtgtgttatcccatggcacctcatcttcccaatttttttcccccagaaagaatacagaataatgaaaacctttctgacagacccatcttgataatagctgtgcaaattattgagtgttttgaggaattttgaatgctaattacctttaaatagatcatctctacatgtaattcttaccccaatacacaagaaatttgattttcatcataaaaagctggcaatttgtcaccatgtgcttgtgaattacatctgcatgaaaaatacatggtgcttcatgtcatttattcaatgtatactcagtaccagatactctgtcaactactatatatgcctttaattctgacaaccaccatatgtgttagacatcattgtccccattttaggaaaagtacactgataaccctaaagtgcaagttattgccaaggcaaattggcaggtcagtggttgaagcaggattccaaagtaagtcagcttgatttcaaactgatttcttaataactaccactctccactcccttctttacaagcatatcatttctaggaaagactattctcatggcaataaccaagataacacaatgtgaacctttaaatgatatatgctgtatttttatatgggatatgacatagtgaataatgactgtcttttttaattttgctgatgaagatgaaaaaaaaaaaatctctgcttttcacatgcaaagaattcattttgactagccgactgtcgaaatgtttaactttgtgtctacttgtgctttgtggacttttcatgatggcgatattttgttgcaaggtgatttttttttttttttttttgagtctcactctgtcaccaggctggagtgcaatggcatgatcttggctcactgcaacctccacctcctaggttcaagcaattctcctgcctcagcctcctgagtagctgggactacaggcacgcaccaccaagcccggctaaattttttgtatttttagtagagacagggtttcaccatgttggccaggatggtcttgatttcttgacctcgtgatctgcccacctcggcctcccaaagtgctgggattaaggtgatttttaaagatacctctttgtatgcttttctgcaagctggttcagttttgagtttgtctgtaatatataaaaaggatgttcttggctgggcgcagtggctcacacctgtaatcccagcactttgggaggcctaggtggggggatcacctgaggtcaggagttcgagactagcctggccaatgtggcaaaacccatctctactaaaaatacaaaaaattagccaggcatggtggtgcacgcctgtagtcccagctacgcaggaggctgaggcaggagaattgcttgaacccgggaggcggaggttgcagtgagccgagcttgtgccactgcactccaatctggtgacagagtgagactccaactcaaaaaaaaataaataaataaaataaaaagatgttcttcaggtctttttaattgttatctcagcacatcctatgaatgtagacatactgattccatctaaagctttcaaatcagatgcatggccaccaaataatcataaaaacaaaatttcttttaaaaatgttgatgagtaatcaagagattttaaggaaaatatatatgtttgtttgttcttgtaaaacgcatactgtggtctttgagcaaggctaattttgcacaagtcagaactccacagctctttctggggctattaaaaaaagagccatctggccataagcaactgacagagtggctcttcccctgtagctgggcacccaccagggcctgggcatggctcttaacactggatgaggtacaacaatttacagaatatgttttctgtttccaggggccccattgtataggcatgaagcagactcacaaaaaattacaatatataggtgctaaaaataaatgtattttaaagttatattaaccgcacaaagcggtcagataattggcaggtgtgattccagcggctttggaagagaggtctttgacttgtatcttaaaggacaaatatgtcatcaggcaaaggggaatgtcacaggatgaaagaccttgagcacatatatagtggtttgaaggaacttgagatcccaggaagataaactgaaagcattttgtttgctcatttcatatatatatatatataaaatctagattatatatgtaattatatatatataatctagagcatgtaatgaaggaggaggcaatattggtaagaaatgtcagggagcaacatgtagtaggatacataagtcacacaaagagtttgaattctatcttgcaagcaataaaaacgcatgttttgcaagcactgcagtatcgtactcaggcattccttatagattatgattaccctttgtccttcaatgtgttggaaaggctaaattagaaaaagactaaaggaagggtcttaaccaagtcagagtcagggaaccaagaggagaaaacacatttgagaggccactctggtgctggaactagcagaatcctaggctgattatttaaatgcagtggtgtggctcatgcctgtaatcccagcactttgggaggcctaggtgggtggatcacctaagatcaggagtttgagaccagcctggccatattctgctcaaaaaaagcaaagaggcagaaagagcccaggctgacggttaaaaaccagcagcttccaagaaagatttttgatgagcaaaatttaactctcctggaaaacattcttattctgcaccagaacttaccaggcctcggtaaatatttgctgaatgaaatcaaaactaaaccaacaaaggcccatcctatcccaactagggagtttagaagactttttgagccagcatagttttttatattaggaaaagagtgacccaatactgaggtttattatgtcattgaagtaataagaattcccctaaggatatattgaggttttcgtctagtttagacttcataccaaaaaaaaaaaaaaaaaaaaaagacagatatgatcacccattggtatgtgtgtgctaaaatgacatatagtttgggttattaccattaaaaacttttgtatccttaactttcagtagagccagtgaaaataaagcttatataatatcccctaaagcacacatttttatctatgttatgggaaaaaaaaagagcataaattcagaagccagtttactaatgccctaatagattgtgacatacgtgctttttcagcggaatctacaaaatacttagagcaacatctcaagtacgaaacaaattcattcctaaaaataacccaactgaagaccttttagtagctctttcagctcaccctatgggtacagacatatcttgattccatctgaaaccttcaaatcagataaatgtgcagccatcaaataatcacaaaaagaatttttataaaaaataggaatggatgaccaagggctttaaaagacaagaattttgaggcttctaaaatgttccctttatttgccataaatgataatatatgtatccactgagaagttatgatagctccatcatgaaaaatctgaaggctagtcagtctcaaggatggtcaatttattaagaggcaggaaaacaattaagagtccatggagtcatgctcagtggtaattcctgactctgccatttacaggatttgtagctatagactaatcacttaatttctcttgaagctaagttttaaaatctaaaaattaaaataacgcaccttacagggttattttaaagacagaatgcaaacatacgttatcacacagtttgcacaaggtcttatataaacaaaggttgttagtaattatcaggtgccattattcctttagattgagttccatcgtggtgcttaataaaaatttaaatgtctgcatgtgtaattacgaaatacaatttctaagttttcaaatacttggtggaaacttgaaaatttaattcaaattaagttctgactttagcaatgtactctctcattgctgcatctattaaaaaccaagaacatctaattatgacagttgcatcaaccttaccaacaggtagaaacatctcttttgtcaccttagatgtcctgtcaatttaatgaagtagtataaagtgattatgcaggctctgagacactggaatgcattagaaaaagtgtttattacctgatctgtgagtttcttaatggctcacagacacttttctctgaatccccggaagaccctaacatagtgctgtagaaagtagatgaatagtaaatatatcagatgaagagatttcttcagggacatagtgagggagaagatttgcctgatttggctaagaacgcatttcactattctgtgaggcctctgaactcagcctagtgtttggaacagagtaggaggacattaatgaattattttgaatgaatggtattttttgactaatggtttagtctgtatagaataaggtctgtaactcttggcaaaagtacccaagaatagcatagatgttactttacataaaatccccaaaagtaatatgaattacttgttagcactgtctttcatagtcaatgttccaacagagattctacaaacaggtaatactagttaactgaaatgtcatgaatttatttcctgattcaatctctgtcaaatacattattaatgaaatggccaagaggggttagcaaaaggggttctgaaaaatcatatgagactaatcaattgaagttgagcatatgaatagatacatttccttgagtgcctattgaaaggatggacagatgtgctataaattctgcggcagaaaagtactatgagaattcttaaagaaatctgacatttaaaaccaatagcgtggctgggcatggtgtcctctgcctgtactcccagcactttgggtgatcgaggtgggatgattgcttgcatctaggagtttgagaccagcctgggcaacatggtaagaccgtgtttaaaaaaaatttaaaaataaaaaataaagccaatagcatctattttgaaataggggaaaagcctattctgataggataaatacaatgacattatctgtatcctaaacaacatagatttcaccagtataaaataagatgctctgtgtatgtgtgcatacctaaaaggtattcgtaggaacacacaatttagttgggaaatttaaaagaacatgaggatttcatataaactcctcacacaaaaaggatcaaatggcctttagaaatgcaagtcatattcatgataggagaatacgaaagtcctattacctcttttattcctgccctcctgcgtcatttcttctacattaacagcacaagtattgactgtatcccaatgaacttactcagataaacacaatgtggttttcttttaaaataagactttactgaatatatcaacaaggtactgtatagtgtagagtgaagtttgtcattaacaaagtgtgcgacatggtaggtctcagaggatgtgtgatgcagaatctttcagccccttatcagagagaacacactaaacagaaaccagaagcaaatcagcatatggttcaaacaataacaaatcatcaggttaactttcagtgaatatacactagtcctatgagcgacacacacttggcaatgccttcaccttgccttaaacattataaatcttacattccagggacacctttacaaatgcccctgtttgtgtgtgtgtgtgtgtgtgtgtacaagcatgtgcatgtttgataataatttttaaatgcctgttgcaatggccttgctttgtgctcttctggtgggtgtgcaggtagaaaacaaaaaactatagtaaaaaaatttgttttgttataacaacggtatcagacatatacaaaactctttctccacagtgacaagcattccccattgctagtaactgtcttttgaccctgctgaagaaatcagagaaggatgtaggttatgccttcttagcattcatattttgactttagaaagagcatcaggcaaggtttgacaagaccaagaacaagaccaagaactgttttgttctgtgtgagtatcttttttccatttggggcactgttttctgctttgctttcccatgcagctggaatggtaagtcatgagcaaaactgctattctcatgttctaaagtaaaatgtaatgtctccttgttataggttagagaaaaatgctataagcaaagacaccaatgggaattaaccccttcacttttcaaaagctgcgatggcctctgcagccaaggtccggagatcaagtgaagcatccattccctgtggactgcaatattgcctcgtgttctgaatggatgcttcaatcacagcatgaagatgttgtcctccctggtggggaaggaagttctgatttgtgtgaaatgactaagaccattatgataggtgctagtagaaaatgaagctgtaatattagctacttcattaatacttcttaccagactggtcacgtactttttgtttttaacctcagggagaatgtctaatatattttcaacgaacatccagataattagaaattgcattatttctcacaggggagaatgttttccatttgttacacaaggaaaataggcaggggatacattcctcgtatctgcctgcgattgtcccatgcagtgggctgctaatgcatctgacggtgtttgagggtggcccagagtctctctataatcaaacatatctccccaaacaagcaggtattaacaactaccctggctatagataactgtcaatatatccttttgatcatgactatgcctcttccttttcaatgtcttctgtacagtgacatttaccaagctctgaatgggatcagattctatctgagtcacctcatttggccaggcagcatcaagctctttattggccagtgagcatggctttttttcccatggtcttggcctgtactcgcaaccttgactcttgactaatcatctcaaaatacatcataatgacagcaagagaggcccaaacacagagcagatatatcagcaaatatacattcccatgactaaaaatgccaatcaaagcagaatccccagggacagttgtttggcaattttcataagacacattagacatcacagattccatcacgtgctttctatcctggtgcaggtgaggctgtaacaaatgggagacggattttaatcttagcagtctttgccatgttgtacacaaggtgaaaataaagcctgttactaggttcaatctcttcaggaacacctccagcaaaagggaccctgtcagaccatcttaagcattgcacatgactgtctccattgtaccatttaagccccaaataattctgtgaaccccataagaaatgacaggaacctcttcatccttgttcttcctggcccaaagtggtttcagcagccagaaatcccactgggggttaaacatacaatatacataaatgagaatgagtattttgtgaataacagaaataaaaaccctcaaaagtcaaagtaccatcatttgaatgcacaattttatctacacagccaaggggaagaggacagtagaagggaattatccagctaagtacacaaagcccccatgtcattgtcttgattttagatgtcttactgctacactgatcaccttcacagactcttttcccttcactgtgtggacctaactttaaaaaaagcaacagccaaaaccctctagctaatagactaaaatggaaaccagagtcactttagaattaatttaaattaattcatagctaagttcagctctactgactgcacagtttcaattcttgtgtctacgacatacagctgcagttatattttctgcttattctgagggacaagggagattaaaacatataagttgggctatattattaaagaaaataaagctcttactataaagaaaaagttgcatagcattttatacctaaacttttacaaagaagacacatcacagttttattttgctgagagagagagagctagtaagatgattgtgacatttacttcatgggtccctataataatggtcaatggtaaaagaaatatgcagcacagagtgaaatgtttaaatttgattttcgaaagatattttttccaagggagtagtttttgataacgtatgtgatctatagcccttctctatctaaggatggcaaagattaaattatgtgttttctgaaggtgttgtctcaaaagtatctagaattaagcacggacatcctctcttttctacgccctgctctgccaggattaggggaaaaagccttcactctctgacttgtttttcatgggttgtcctgctaacataagattgattagccctccacaattgccaaagtagaggaacatccacgatggaaaaggaacaaataaaatttcaaaagtggaacaggatcaaagtcagtccaaggtggaaaccaggtattgctttttaaaaaaaattcattattttggccagctttgatgtgtccttacagaattattagcagtgaaaattagtactcattttaaaatgtataagtacgtaatggatatcttgtgcagccaagactggcatccataattttccttgaaatactgaacagagggagaaaaacaaaggtgtcataaacaactaattatgaaaatatatgggagatgattggaagacaagaatttgcaaggggataaaagatattacttcaagctatttcaacatgatactaacaaagtcagctgacataacagaaccactgatcagttgtttttgtctaaatagcaggaagggtaatttttaaataagtcattgttgtattttccaaacattgatcacctgttggtctaaatatcatgttgacatagcctcagtgaatctacccaaataattctcattatcaaaaataattccattcaatataattcttccctttattagcctcttctaaaaaagtattctagaatatatctctgttgaatgtgattcaacctgatatatgatttgaacagtaacacttttaaagggagtcttcttgctacaacatcagactggtccctgaagatgactgaaatcagactcaagtctctaactctgttatcacataggaccagggaagcatgaagagtgatttttaagttcccagtcagaaagccaacccctgcattttcgggtcctttcaaatctcatctcaattttcttgattctgtcaggccgggttaacttatctcacgggaaccggcttcctcctggtgctttcagcatttcccacacagggtcaaatcagggtaactacctccattcttacattatagaattttttacctgtcttccggacctggaggtataggaatagtgtgaaactatcgggccatttcttgttttacccatattattcctcttaccctgatgagtccatttaatctgccctttcatctgaccaccaggaatttattctgacagcttcaacagcaaagtggttgatgtgtatcctaaggaaaaatcactcgttctttttgccttggcattgggttctcattgtacaaccctgtacagtacttcagcaacttttttttttttaagatttaaaaagcaaagagttacaaaactgtttgtaattaacttgaaatagaaaagatagcactttttttaaatcccattatatagtacaccgtataaattacagagtattcaaatgcacaaatgcatctgtgtaacatttatcaaatgtaatctgcgtgtctttatgtgcacacacgagtgtgttctcaagagtctaattgtccgccttgataacgctgggcctctggctgtcacgtatggcagtgctccaggtctggcacgctgctgttgcagtatcgcatgttgttggggatatggcagtctgtgtaattaatgcccccatttggggtgtaaatgggctgcagtctgaaatctcctttaaggagttgatcgttatttaaggagacgatctgaaaactggtttctgtcatctccaggatggagttgtccttcttggtgcctgcctcgcaataatcatctttccgccggccccggttgtatttccacttctgggaggtgtagcgcccctttttgtgcatatgccagcaaaagacgctgagcaagaccaccagcacaaatatcaccgcgcccccgatcaagcccgccagcagaaagggggagcccatgctgtgggacgtcgtctgctcatggctggacgctgtgttgctgccgttgttcagataggaggcatgggtggtggcctctgaacaaatggtgtcttctaccgcgcggtagttaaaagcatccagtggcactaaacaaatccgataggtggatcggggctctaagttaaccaggctcaggtgttgcttctcaccgctgactatgcgctcctgaacgatgccccctactaaactgtggcccattttcacccatgtgagtttgtatgccatcacggtgaagagagagagccagctgacttgaatggaagtatcattcacaaaatggatagagagctggatccgttcagaaataggtggggtcactctttctctgccatcccagtcaggaatcgtgggaagtttcgatgtggtaggagttggaggcgtgtagcttctgctagggtttggaatagagagggtgggaggctgagtggtcggagaagctgtacttggggctggggtgaagagaggcaggccgggggtcgtggtgggacaggacaaaagattcatatttaattccctgacggccatcccccggacttgttcaggaccttggcacatgaaaccccgcacgttgagagatgaagggatatatttgagccattctgtgacccatttaatactgcagtcacaaaaccaagggttattccgagcagtgagctgcttcaggttggagagattatcaaaaaccccttgagtcagcatccgcagttggttgttggatatatccagccgttccagcttacgcagatttgagaaggctgtcaaaggaatgtggtttatctggttgtcctgcaaatagagcctgatcagatgcgtacctgggagatcgggaggagggtgggacagcgaattacgtacaattgaaaattccttgagcttggtgagatggctgaaggtgccctcggcgatacccttgttggtcaggaggttcccgtccacaataagacgctccaagctcgtgagattctggaaggccatgtcggatatgacagcaattcgattttcatccactctcagctcttgcaagtccacaggaagcccaacaggcacactgctcaggtgattcttagacaaaaacaacaatttgaggctaatagcctcccggaaggccccgtcttccacccccactgtggatatggagttgtcatccaggtgcagctcttcaagcttcaagagctgggcaagagcagcccgtgaaatggtctgaatattgttttcctgcaaatggagaactctgacattcttgggaaggttcatggggaattcgtccagttggttgccatacaggtagaccgtgtgcaccgactgtacattgtgcagttctgcaggaaatccagcattattaatttggttgttgtggaggtagagtacagttacgccctccgggatcccaagaggcactgaggtcaagcttcgctcattacagtagacaaagttcctgtcgcagcggcacacactagggcaggccaggagtttggacacctgtgagtagagccccagggaaatgataagccaagacttcaggaaaaaagccccatggctgggccactttgtggtctgtaggcccatttctgaagtacggaaataaaatacaatgtggtgggaaaaagaaaaagaaaaaaaaaataaacagcaaaatcaaaatgactggatggggttctgttgaagtccagaactccagctagagggaacgtcctgagggcgtatggtaaaataatctccctgctgtctctggtcttatcagcctgtgttgccctctttgctgctgtcctccatgtgcaaaaaattcaacagggagaatttttccacactggcaacaggtgatggcaagttatcagccgtgtcaacacaagcccaagtgggcaggcagaactctcttcttcttttgtaggtcaagccagccttgattagcctacgaacttcttggttaagctcaatctgcaatctcggaaaggagtagctcagcgccttggcgcggagatttgcgggcactgatgatatctcgagcgctcgttcctccgcggtgacaatggataatgccaaacgcgcaagtgacggcgacaggtttcgaacgtacaact

SEQ ID NO: 13126 - RNA, 15930 nt, Homo sapiens
  source 1..15930: mol_type = other RNA
gctgggattacaggcatgagccaccacacccggcccagaatgttcgtaatttcatataaacattttatttgcctttctttttcttttcctgaagatgttttgttgcttacttttcagtttatactggctttttaaaacagatttcctttagagtaattacttccatagtgacagctatatttactgaaataaaatgtttcaaacatgtctcgaagtttgaatttctgtcactaaagaaaattagttaagattaataagaatgttttttgttttttttttttttttttctgcaggtgacttcacctttgattttcctacatttaggcaatgttagtgatgttctttaaactgccaggtagaatttcaatgtttgcaatacaaataccattaaatacttttattatagttactttgataaattcttttaaaaatactattttggtcctttatagaggtagcataatatttaaaactaactttaaaacaaattattttactaatctgcttgcattttattaaattccctttacagaattaatgaacttttaaagatttcataacaaagaactaattaatgagaagcataaataacagcttatgaaagaacaggtaatgataccttaatctgagtcccaaggaccactttccaattacacaattacaagccattaatttaaaatatcaatcattagactattatcaattattggaagtgtgtattatataaaaattatataaacatctttaataaagcaatgttgattacattcaggtgtatgatgtgatgaaataaagctagtgttcactggcagatattcttaggtaaccgctttaaagactaaacattttgaaatgaacatttcattgttagctgctaagtagtggttttataaaagtattgaaggtctgggaaagaagaatttcctaattattctaaaaagttttcatctttcttttttttaaaccataattgtatgtttgttcaaggttcagataaaagtggcagggatcagggttaaaatctgttctattccatcaaaaataaaccacatttattatttaatattttctagctattctcataattctttctctgtcaaatattagggtttaatagctgttatataatggcttgaaaacataaaatatttaatattttaataaacaattttttatacaatttttattgtacgacactctatctttgataattttgacttaaataaagtgttttattaatagtctacttagtaatatagtttgtatttccttgttttgagggagaagtggttgaactaatgagttttgttttcacttgcttctctttctattcatttgtaatttttcagccataatgggtttgaatatatgccaaccactgaagtgaagatgatataaattatctcatcaaatccttaaaagtattagtacctcatttcatatatgaggaaactgaggcttagggacattaaataatatcacacagatacaaagtcacagttctttgtgattctgtagctcctgattttaatggttatgcaggttgcttccctaacatatcaagtttaaggttattataactaatgagaaacatgttagtctttatacttaagtcaatgaaactgagtgtttatatgtttgctttatctatcctagtcacatcttcctgaattttaaaagcacacagaacacaaatcagtccaatgaaccaaatctaaactacatagaaaatgaacaaccataaaacagaatttaaggtccaaagtaacttgggagatcaactaaattcctgcgcttttgactataagaaacaagcccgagagagaagtggtcttatccaagatacaaaggagatttgagttatatagcccaactttttgcacactaattccatatattttcagaaagtagctggcatttattgagcactttatatgtgtcaggcactgtgcagtatggttactgttgaggtgagtgttgttattaacccatgtacagatgagaaaattgaagcatatacatgcccaaggaccaaggttagtatgagccaggatttaaatttagatgtagacagcattggactcagaatttaaaagattcatcatgttttcataatataacttcccatccaataggctacagtcttatagacacagttgctgttagatataattggcctccattacaaaacagctcacttcctgcttcctccttacttcagatacactagtaaagcatgctatattccaactaatgagggcagttatgtaaaatacttagcaataggatagctgaggcctaccagtcaaaacagacactagtccaaacagaatagagattggcagcagaccacaggaatgccagtacccattgatactacttgccaaataactgtcctgaaaccaattaaatcatgcagtcaaggactgaaaaagtatatttcccccctcatcaaatgtctgaacttctgcatttattaagcaaggaaagacataaatagaaaggaaaataatgctaatacagaccgtagtgagtgaattgctttgagactattaactaccacaaagtgtacagaaagaaaacaacgtgatccagctgaagaggatgcatgcctgttaataacaaccagcttccaaacttaataatgatatcgattgcaaaaagtaaccacatgacaggtggtagactattgcacctgcattgtagagacattaaaatgttcttccatttgactgctaccatccccactatcagcaaacccagtgtggatttaaatgccgtaattggtggtgtactagcatcaaataaaactatgtcttactagaaattatagatttttgaaacaatatcagaaatttattactttttttttttttttgagacagggtcttgctcagttgcctaagctggagtgcagtggcacaatcagagctcaatgtaatcttgatctcctgggctcaagtgaccctcctgcttcaacctcccaagtagctgggactataggcacatgccaccactcctggctaatttttttttttttttttagagatagggtctcactgcattgcccaggctggtctggaaatcctgacctcaagcaatcctcccaccttggcctcccaaagtactgcgattataggcatgagccactgtgctcagcttatcttgattttgtttttagtattttgatttccaatgccttctgaatgctcattcctggggctcttttgacacccacatattctgaattaattttcagcaataactacatctatgtgtactctagcaaccagatagaatatatgctacattataaagaagtctgttctctttctgttcaaccatgttgttcaatgatcccacacaccatgagaaaaaaggcctgccatggttgtgtgttatcccatggcacctcatcttcccaatttttttcccccagaaagaatacagaataatgaaaacctttctgacagacccatcttgataatagctgtgcaaattattgagtgttttgaggaattttgaatgctaattacctttaaatagatcatctctacatgtaattcttaccccaatacacaagaaatttgattttcatcataaaaagctggcaatttgtcaccatgtgcttgtgaattacatctgcatgaaaaatacatggtgcttcatgtcatttattcaatgtatactcagtaccagatactctgtcaactactatatatgcctttaattctgacaaccaccatatgtgttagacatcattgtccccattttaggaaaagtacactgataaccctaaagtgcaagttattgccaaggcaaattggcaggtcagtggttgaagcaggattccaaagtaagtcagcttgatttcaaactgatttcttaataactaccactctccactcccttctttacaagcatatcatttctaggaaagactattctcatggcaataaccaagataacacaatgtgaacctttaaatgatatatgctgtatttttatatgggatatgacatagtgaataatgactgtcttttttaattttgctgatgaagatgaaaaaaaaaaaatctctgcttttcacatgcaaagaattcattttgactagccgactgtcgaaatgtttaactttgtgtctacttgtgctttgtggacttttcatgatggcgatattttgttgcaaggtgatttttttttttttttttttgagtctcactctgtcaccaggctggagtgcaatggcatgatcttggctcactgcaacctccacctcctaggttcaagcaattctcctgcctcagcctcctgagtagctgggactacaggcacgcaccaccaagcccggctaaattttttgtatttttagtagagacagggtttcaccatgttggccaggatggtcttgatttcttgacctcgtgatctgcccacctcggcctcccaaagtgctgggattaaggtgatttttaaagatacctctttgtatgcttttctgcaagctggttcagttttgagtttgtctgtaatatataaaaaggatgttcttggctgggcgcagtggctcacacctgtaatcccagcactttgggaggcctaggtggggggatcacctgaggtcaggagttcgagactagcctggccaatgtggcaaaacccatctctactaaaaatacaaaaaattagccaggcatggtggtgcacgcctgtagtcccagctacgcaggaggctgaggcaggagaattgcttgaacccgggaggcggaggttgcagtgagccgagcttgtgccactgcactccaatctggtgacagagtgagactccaactcaaaaaaaaataaataaataaaataaaaagatgttcttcaggtctttttaattgttatctcagcacatcctatgaatgtagacatactgattccatctaaagctttcaaatcagatgcatggccaccaaataatcataaaaacaaaatttcttttaaaaatgttgatgagtaatcaagagattttaaggaaaatatatatgtttgtttgttcttgtaaaacgcatactgtggtctttgagcaaggctaattttgcacaagtcagaactccacagctctttctggggctattaaaaaaagagccatctggccataagcaactgacagagtggctcttcccctgtagctgggcacccaccagggcctgggcatggctcttaacactggatgaggtacaacaatttacagaatatgttttctgtttccaggggccccattgtataggcatgaagcagactcacaaaaaattacaatatataggtgctaaaaataaatgtattttaaagttatattaaccgcacaaagcggtcagataattggcaggtgtgattccagcggctttggaagagaggtctttgacttgtatcttaaaggacaaatatgtcatcaggcaaaggggaatgtcacaggatgaaagaccttgagcacatatatagtggtttgaaggaacttgagatcccaggaagataaactgaaagcattttgtttgctcatttcatatatatatatatataaaatctagattatatatgtaattatatatatataatctagagcatgtaatgaaggaggaggcaatattggtaagaaatgtcagggagcaacatgtagtaggatacataagtcacacaaagagtttgaattctatcttgcaagcaataaaaacgcatgttttgcaagcactgcagtatcgtactcaggcattccttatagattatgattaccctttgtccttcaatgtgttggaaaggctaaattagaaaaagactaaaggaagggtcttaaccaagtcagagtcagggaaccaagaggagaaaacacatttgagaggccactctggtgctggaactagcagaatcctaggctgattatttaaatgcagtggtgtggctcatgcctgtaatcccagcactttgggaggcctaggtgggtggatcacctaagatcaggagtttgagaccagcctggccatattctgctcaaaaaaagcaaagaggcagaaagagcccaggctgacggttaaaaaccagcagcttccaagaaagatttttgatgagcaaaatttaactctcctggaaaacattcttattctgcaccagaacttaccaggcctcggtaaatatttgctgaatgaaatcaaaactaaaccaacaaaggcccatcctatcccaactagggagtttagaagactttttgagccagcatagttttttatattaggaaaagagtgacccaatactgaggtttattatgtcattgaagtaataagaattcccctaaggatatattgaggttttcgtctagtttagacttcataccaaaaaaaaaaaaaaaaaaaaaagacagatatgatcacccattggtatgtgtgtgctaaaatgacatatagtttgggttattaccattaaaaacttttgtatccttaactttcagtagagccagtgaaaataaagcttatataatatcccctaaagcacacatttttatctatgttatgggaaaaaaaaagagcataaattcagaagccagtttactaatgccctaatagattgtgacatacgtgctttttcagcggaatctacaaaatacttagagcaacatctcaagtacgaaacaaattcattcctaaaaataacccaactgaagaccttttagtagctctttcagctcaccctatgggtacagacatatcttgattccatctgaaaccttcaaatcagataaatgtgcagccatcaaataatcacaaaaagaatttttataaaaaataggaatggatgaccaagggctttaaaagacaagaattttgaggcttctaaaatgttccctttatttgccataaatgataatatatgtatccactgagaagttatgatagctccatcatgaaaaatctgaaggctagtcagtctcaaggatggtcaatttattaagaggcaggaaaacaattaagagtccatggagtcatgctcagtggtaattcctgactctgccatttacaggatttgtagctatagactaatcacttaatttctcttgaagctaagttttaaaatctaaaaattaaaataacgcaccttacagggttattttaaagacagaatgcaaacatacgttatcacacagtttgcacaaggtcttatataaacaaaggttgttagtaattatcaggtgccattattcctttagattgagttccatcgtggtgcttaataaaaatttaaatgtctgcatgtgtaattacgaaatacaatttctaagttttcaaatacttggtggaaacttgaaaatttaattcaaattaagttctgactttagcaatgtactctctcattgctgcatctattaaaaaccaagaacatctaattatgacagttgcatcaaccttaccaacaggtagaaacatctcttttgtcaccttagatgtcctgtcaatttaatgaagtagtataaagtgattatgcaggctctgagacactggaatgcattagaaaaagtgtttattacctgatctgtgagtttcttaatggctcacagacacttttctctgaatccccggaagaccctaacatagtgctgtagaaagtagatgaatagtaaatatatcagatgaagagatttcttcagggacatagtgagggagaagatttgcctgatttggctaagaacgcatttcactattctgtgaggcctctgaactcagcctagtgtttggaacagagtaggaggacattaatgaattattttgaatgaatggtattttttgactaatggtttagtctgtatagaataaggtctgtaactcttggcaaaagtacccaagaatagcatagatgttactttacataaaatccccaaaagtaatatgaattacttgttagcactgtctttcatagtcaatgttccaacagagattctacaaacaggtaatactagttaactgaaatgtcatgaatttatttcctgattcaatctctgtcaaatacattattaatgaaatggccaagaggggttagcaaaaggggttctgaaaaatcatatgagactaatcaattgaagttgagcatatgaatagatacatttccttgagtgcctattgaaaggatggacagatgtgctataaattctgcggcagaaaagtactatgagaattcttaaagaaatctgacatttaaaaccaatagcgtggctgggcatggtgtcctctgcctgtactcccagcactttgggtgatcgaggtgggatgattgcttgcatctaggagtttgagaccagcctgggcaacatggtaagaccgtgtttaaaaaaaatttaaaaataaaaaataaagccaatagcatctattttgaaataggggaaaagcctattctgataggataaatacaatgacattatctgtatcctaaacaacatagatttcaccagtataaaataagatgctctgtgtatgtgtgcatacctaaaaggtattcgtaggaacacacaatttagttgggaaatttaaaagaacatgaggatttcatataaactcctcacacaaaaaggatcaaatggcctttagaaatgcaagtcatattcatgataggagaatacgaaagtcctattacctcttttattcctgccctcctgcgtcatttcttctacattaacagcacaagtattgactgtatcccaatgaacttactcagataaacacaatgtggttttcttttaaaataagactttactgaatatatcaacaaggtactgtatagtgtagagtgaagtttgtcattaacaaagtgtgcgacatggtaggtctcagaggatgtgtgatgcagaatctttcagccccttatcagagagaacacactaaacagaaaccagaagcaaatcagcatatggttcaaacaataacaaatcatcaggttaactttcagtgaatatacactagtcctatgagcgacacacacttggcaatgccttcaccttgccttaaacattataaatcttacattccagggacacctttacaaatgcccctgtttgtgtgtgtgtgtgtgtgtgtgtacaagcatgtgcatgtttgataataatttttaaatgcctgttgcaatggccttgctttgtgctcttctggtgggtgtgcaggtagaaaacaaaaaactatagtaaaaaaatttgttttgttataacaacggtatcagacatatacaaaactctttctccacagtgacaagcattccccattgctagtaactgtcttttgaccctgctgaagaaatcagagaaggatgtaggttatgccttcttagcattcatattttgactttagaaagagcatcaggcaaggtttgacaagaccaagaacaagaccaagaactgttttgttctgtgtgagtatcttttttccatttggggcactgttttctgctttgctttcccatgcagctggaatggtaagtcatgagcaaaactgctattctcatgttctaaagtaaaatgtaatgtctccttgttataggttagagaaaaatgctataagcaaagacaccaatgggaattaaccccttcacttttcaaaagctgcgatggcctctgcagccaaggtccggagatcaagtgaagcatccattccctgtggactgcaatattgcctcgtgttctgaatggatgcttcaatcacagcatgaagatgttgtcctccctggtggggaaggaagttctgatttgtgtgaaatgactaagaccattatgataggtgctagtagaaaatgaagctgtaatattagctacttcattaatacttcttaccagactggtcacgtactttttgtttttaacctcagggagaatgtctaatatattttcaacgaacatccagataattagaaattgcattatttctcacaggggagaatgttttccatttgttacacaaggaaaataggcaggggatacattcctcgtatctgcctgcgattgtcccatgcagtgggctgctaatgcatctgacggtgtttgagggtggcccagagtctctctataatcaaacatatctccccaaacaagcaggtattaacaactaccctggctatagataactgtcaatatatccttttgatcatgactatgcctcttccttttcaatgtcttctgtacagtgacatttaccaagctctgaatgggatcagattctatctgagtcacctcatttggccaggcagcatcaagctctttattggccagtgagcatggctttttttcccatggtcttggcctgtactcgcaaccttgactcttgactaatcatctcaaaatacatcataatgacagcaagagaggcccaaacacagagcagatatatcagcaaatatacattcccatgactaaaaatgccaatcaaagcagaatccccagggacagttgtttggcaattttcataagacacattagacatcacagattccatcacgtgctttctatcctggtgcaggtgaggctgtaacaaatgggagacggattttaatcttagcagtctttgccatgttgtacacaaggtgaaaataaagcctgttactaggttcaatctcttcaggaacacctccagcaaaagggaccctgtcagaccatcttaagcattgcacatgactgtctccattgtaccatttaagccccaaataattctgtgaaccccataagaaatgacaggaacctcttcatccttgttcttcctggcccaaagtggtttcagcagccagaaatcccactgggggttaaacatacaatatacataaatgagaatgagtattttgtgaataacagaaataaaaaccctcaaaagtcaaagtaccatcatttgaatgcacaattttatctacacagccaaggggaagaggacagtagaagggaattatccagctaagtacacaaagcccccatgtcattgtcttgattttagatgtcttactgctacactgatcaccttcacagactcttttcccttcactgtgtggacctaactttaaaaaaagcaacagccaaaaccctctagctaatagactaaaatggaaaccagagtcactttagaattaatttaaattaattcatagctaagttcagctctactgactgcacagtttcaattcttgtgtctacgacatacagctgcagttatattttctgcttattctgagggacaagggagattaaaacatataagttgggctatattattaaagaaaataaagctcttactataaagaaaaagttgcatagcattttatacctaaacttttacaaagaagacacatcacagttttattttgctgagagagagagagctagtaagatgattgtgacatttacttcatgggtccctataataatggtcaatggtaaaagaaatatgcagcacagagtgaaatgtttaaatttgattttcgaaagatattttttccaagggagtagtttttgataacgtatgtgatctatagcccttctctatctaaggatggcaaagattaaattatgtgttttctgaaggtgttgtctcaaaagtatctagaattaagcacggacatcctctcttttctacgccctgctctgccaggattaggggaaaaagccttcactctctgacttgtttttcatgggttgtcctgctaacataagattgattagccctccacaattgccaaagtagaggaacatccacgatggaaaaggaacaaataaaatttcaaaagtggaacaggatcaaagtcagtccaaggtggaaaccaggtattgctttttaaaaaaaattcattattttggccagctttgatgtgtccttacagaattattagcagtgaaaattagtactcattttaaaatgtataagtacgtaatggatatcttgtgcagccaagactggcatccataattttccttgaaatactgaacagagggagaaaaacaaaggtgtcataaacaactaattatgaaaatatatgggagatgattggaagacaagaatttgcaaggggataaaagatattacttcaagctatttcaacatgatactaacaaagtcagctgacataacagaaccactgatcagttgtttttgtctaaatagcaggaagggtaatttttaaataagtcattgttgtattttccaaacattgatcacctgttggtctaaatatcatgttgacatagcctcagtgaatctacccaaataattctcattatcaaaaataattccattcaatataattcttccctttattagcctcttctaaaaaagtattctagaatatatctctgttgaatgtgattcaacctgatatatgatttgaacagtaacacttttaaagggagtcttcttgctacaacatcagactggtccctgaagatgactgaaatcagactcaagtctctaactctgttatcacataggaccagggaagcatgaagagtgatttttaagttcccagtcagaaagccaacccctgcattttcgggtcctttcaaatctcatctcaattttcttgattctgtcaggccgggttaacttatctcacgggaaccggcttcctcctggtgctttcagcatttcccacacagggtcaaatcagggtaactacctccattcttacattatagaattttttacctgtcttccggacctggaggtataggaatagtgtgaaactatcgggccatttcttgttttacccatattattcctcttaccctgatgagtccatttaatctgccctttcatctgaccaccaggaatttattctgacagcttcaacagcaaagtggttgatgtgtatcctaaggaaaaatcactcgttctttttgccttggcattgggttctcattgtacaaccctgtacagtacttcagcaacttttttttttttaagatttaaaaagcaaagagttacaaaactgtttgtaattaacttgaaatagaaaagatagcactttttttaaatcccattatatagtacaccgtataaattacagagtattcaaatgcacaaatgcatctgtgtaacatttatcaaatgtaatctgcgtgtctttatgtgcacacacgagtgtgttctcaagagtctaattgtccgccttgataacgctgggcctctggctgtcacgtatggcagtgctccaggtctggcacgctgctgttgcagtatcgcatgttgttggggatatggcagtctgtgtaattaatgcccccatttggggtgtaaatgggctgcagtctgaaatctcctttaaggagttgatcgttatttaaggagacgatctgaaaactggtttctgtcatctccaggatggagttgtccttcttggtgcctgcctcgcaataatcatctttccgccggccccggttgtatttccacttctgggaggtgtagcgcccctttttgtgcatatgccagcaaaagacgctgagcaagaccaccagcacaaatatcaccgcgcccccgatcaagcccgccagcagaaagggggagcccatgctgtgggacgtcgtctgctcatggctggacgctgtgttgctgccgttgttcagataggaggcatgggtggtggcctctgaacaaatggtgtcttctaccgcgcggtagttaaaagcatccagtggcactaaacaaatccgataggtggatcggggctctaagttaaccaggctcaggtgttgcttctcaccgctgactatgcgctcctgaacgatgccccctactaaactgtggcccattttcacccatgtgagtttgtatgccatcacggtgaagagagagagccagctgacttgaatggaagtatcattcacaaaatggatagagagctggatccgttcagaaataggtggggtcactctttctctgccatcccagtcaggaatcgtgggaagtttcgatgtggtaggagttggaggcgtgtagcttctgctagggtttggaatagagagggtgggaggctgagtggtcggagaagctgtacttggggctggggtgaagagaggcaggccgggggtcgtggtgggacaggacaaaagattcatatttaattccctgacggccatcccccggacttgttcaggaccttggcacatgaaaccccgcacgttgagagatgaagggatatatttgagccattctgtgacccatttaatactgcagtcacaaaaccaagggttattccgagcagtgagctgcttcaggttggagagattatcaaaaaccccttgagtcagcatccgcagttggttgttggatatatccagccgttccagcttacgcagatttgagaaggctgtcaaaggaatgtggtttatctggttgtcctgcaaatagagcctgatcagatgcgtacctgggagatcgggaggagggtgggacagcgaattacgtacaattgaaaattccttgagcttggtgagatggctgaaggtgccctcggcgatacccttgttggtcaggaggttcccgtccacaataagacgctccaagctcgtgagattctggaaggccatgtcggatatgacagcaattcgattttcatccactctcagctcttgcaagtccacaggaagcccaacaggcacactgctcaggtgattcttagacaaaaacaacaatttgaggctaatagcctcccggaaggccccgtcttccacccccactgtggatatggagttgtcatccaggtgcagctcttcaagcttcaagagctgggcaagagcagcccgtgaaatggtctgaatattgttttcctgcaaatggagaactctgacattcttgggaaggttcatggggaattcgtccagttggttgccatacaggtagaccgtgtgcaccgactgtacattgtgcagttctgcaggaaatccagcattattaatttggttgttgtggaggtagagtacagttacgccctccgggatcccaagaggcactgaggtcaagcttcgctcattacagtagacaaagttcctgtcgcagcggcacacactagggcaggccaggagtttggacacctgtgagtagagccccagggaaatgataagccaagacttcaggaaaaaagccccatggctgggccactttgtggtctgtaggcccatttctgaagtacggaaataaaatacaatgtggtgggaaaaagaaaaagaaaaaaaaaataaacagcaaaatcaaaatgactggatggggttctgttgaagtccagaactccagctagagggaacgtcctgagggcgtatggtaaaataatctccctgctgtctctggtcttatcagcctgtgttgccctctttgctgctgtcctccatgtgcaaaaaattcaacagggagaatttttccacactggcaacaggtgatggcaagttatcagccgtgtcaacacaagcccaagtgggcaggcagaactctcttcttcttttgtaggtcaagccagccttgattagcctacgaacttcttggttaagctcaatctgcaatctgacggctgcgtcttctccttgcaatgggctcatccgaatccgacagggtcagggaggtggaaagggaagacgctggcgcggcagcagcggggatcccggggcatggtattgttttaggggtcgccgccgaggtccctcctgcccatcgttgagaactgccaccctgatcccagggctcggtggacacggcggcgggagcggagatgccgcctcgccgctgctgggcaccagggacggaggaccagaggcgcacctcggaaaggagtagctcagcgccttggcgcggagatttgcgggcactgatgatatctcgagcgctcgttcctccgcggtgacaatggataatgccaaacgcgcaagtgacggcgacaggtttcgaacgtacaact

SEQ ID NO: 13127 - RNA, 16184 nt, Homo sapiens
  source 1..16184: mol_type = other RNA
gctgggattacaggcatgagccaccacacccggcccagaatgttcgtaatttcatataaacattttatttgcctttctttttcttttcctgaagatgttttgttgcttacttttcagtttatactggctttttaaaacagatttcctttagagtaattacttccatagtgacagctatatttactgaaataaaatgtttcaaacatgtctcgaagtttgaatttctgtcactaaagaaaattagttaagattaataagaatgttttttgttttttttttttttttttctgcaggtgacttcacctttgattttcctacatttaggcaatgttagtgatgttctttaaactgccaggtagaatttcaatgtttgcaatacaaataccattaaatacttttattatagttactttgataaattcttttaaaaatactattttggtcctttatagaggtagcataatatttaaaactaactttaaaacaaattattttactaatctgcttgcattttattaaattccctttacagaattaatgaacttttaaagatttcataacaaagaactaattaatgagaagcataaataacagcttatgaaagaacaggtaatgataccttaatctgagtcccaaggaccactttccaattacacaattacaagccattaatttaaaatatcaatcattagactattatcaattattggaagtgtgtattatataaaaattatataaacatctttaataaagcaatgttgattacattcaggtgtatgatgtgatgaaataaagctagtgttcactggcagatattcttaggtaaccgctttaaagactaaacattttgaaatgaacatttcattgttagctgctaagtagtggttttataaaagtattgaaggtctgggaaagaagaatttcctaattattctaaaaagttttcatctttcttttttttaaaccataattgtatgtttgttcaaggttcagataaaagtggcagggatcagggttaaaatctgttctattccatcaaaaataaaccacatttattatttaatattttctagctattctcataattctttctctgtcaaatattagggtttaatagctgttatataatggcttgaaaacataaaatatttaatattttaataaacaattttttatacaatttttattgtacgacactctatctttgataattttgacttaaataaagtgttttattaatagtctacttagtaatatagtttgtatttccttgttttgagggagaagtggttgaactaatgagttttgttttcacttgcttctctttctattcatttgtaatttttcagccataatgggtttgaatatatgccaaccactgaagtgaagatgatataaattatctcatcaaatccttaaaagtattagtacctcatttcatatatgaggaaactgaggcttagggacattaaataatatcacacagatacaaagtcacagttctttgtgattctgtagctcctgattttaatggttatgcaggttgcttccctaacatatcaagtttaaggttattataactaatgagaaacatgttagtctttatacttaagtcaatgaaactgagtgtttatatgtttgctttatctatcctagtcacatcttcctgaattttaaaagcacacagaacacaaatcagtccaatgaaccaaatctaaactacatagaaaatgaacaaccataaaacagaatttaaggtccaaagtaacttgggagatcaactaaattcctgcgcttttgactataagaaacaagcccgagagagaagtggtcttatccaagatacaaaggagatttgagttatatagcccaactttttgcacactaattccatatattttcagaaagtagctggcatttattgagcactttatatgtgtcaggcactgtgcagtatggttactgttgaggtgagtgttgttattaacccatgtacagatgagaaaattgaagcatatacatgcccaaggaccaaggttagtatgagccaggatttaaatttagatgtagacagcattggactcagaatttaaaagattcatcatgttttcataatataacttcccatccaataggctacagtcttatagacacagttgctgttagatataattggcctccattacaaaacagctcacttcctgcttcctccttacttcagatacactagtaaagcatgctatattccaactaatgagggcagttatgtaaaatacttagcaataggatagctgaggcctaccagtcaaaacagacactagtccaaacagaatagagattggcagcagaccacaggaatgccagtacccattgatactacttgccaaataactgtcctgaaaccaattaaatcatgcagtcaaggactgaaaaagtatatttcccccctcatcaaatgtctgaacttctgcatttattaagcaaggaaagacataaatagaaaggaaaataatgctaatacagaccgtagtgagtgaattgctttgagactattaactaccacaaagtgtacagaaagaaaacaacgtgatccagctgaagaggatgcatgcctgttaataacaaccagcttccaaacttaataatgatatcgattgcaaaaagtaaccacatgacaggtggtagactattgcacctgcattgtagagacattaaaatgttcttccatttgactgctaccatccccactatcagcaaacccagtgtggatttaaatgccgtaattggtggtgtactagcatcaaataaaactatgtcttactagaaattatagatttttgaaacaatatcagaaatttattactttttttttttttttgagacagggtcttgctcagttgcctaagctggagtgcagtggcacaatcagagctcaatgtaatcttgatctcctgggctcaagtgaccctcctgcttcaacctcccaagtagctgggactataggcacatgccaccactcctggctaatttttttttttttttttagagatagggtctcactgcattgcccaggctggtctggaaatcctgacctcaagcaatcctcccaccttggcctcccaaagtactgcgattataggcatgagccactgtgctcagcttatcttgattttgtttttagtattttgatttccaatgccttctgaatgctcattcctggggctcttttgacacccacatattctgaattaattttcagcaataactacatctatgtgtactctagcaaccagatagaatatatgctacattataaagaagtctgttctctttctgttcaaccatgttgttcaatgatcccacacaccatgagaaaaaaggcctgccatggttgtgtgttatcccatggcacctcatcttcccaatttttttcccccagaaagaatacagaataatgaaaacctttctgacagacccatcttgataatagctgtgcaaattattgagtgttttgaggaattttgaatgctaattacctttaaatagatcatctctacatgtaattcttaccccaatacacaagaaatttgattttcatcataaaaagctggcaatttgtcaccatgtgcttgtgaattacatctgcatgaaaaatacatggtgcttcatgtcatttattcaatgtatactcagtaccagatactctgtcaactactatatatgcctttaattctgacaaccaccatatgtgttagacatcattgtccccattttaggaaaagtacactgataaccctaaagtgcaagttattgccaaggcaaattggcaggtcagtggttgaagcaggattccaaagtaagtcagcttgatttcaaactgatttcttaataactaccactctccactcccttctttacaagcatatcatttctaggaaagactattctcatggcaataaccaagataacacaatgtgaacctttaaatgatatatgctgtatttttatatgggatatgacatagtgaataatgactgtcttttttaattttgctgatgaagatgaaaaaaaaaaaatctctgcttttcacatgcaaagaattcattttgactagccgactgtcgaaatgtttaactttgtgtctacttgtgctttgtggacttttcatgatggcgatattttgttgcaaggtgatttttttttttttttttttgagtctcactctgtcaccaggctggagtgcaatggcatgatcttggctcactgcaacctccacctcctaggttcaagcaattctcctgcctcagcctcctgagtagctgggactacaggcacgcaccaccaagcccggctaaattttttgtatttttagtagagacagggtttcaccatgttggccaggatggtcttgatttcttgacctcgtgatctgcccacctcggcctcccaaagtgctgggattaaggtgatttttaaagatacctctttgtatgcttttctgcaagctggttcagttttgagtttgtctgtaatatataaaaaggatgttcttggctgggcgcagtggctcacacctgtaatcccagcactttgggaggcctaggtggggggatcacctgaggtcaggagttcgagactagcctggccaatgtggcaaaacccatctctactaaaaatacaaaaaattagccaggcatggtggtgcacgcctgtagtcccagctacgcaggaggctgaggcaggagaattgcttgaacccgggaggcggaggttgcagtgagccgagcttgtgccactgcactccaatctggtgacagagtgagactccaactcaaaaaaaaataaataaataaaataaaaagatgttcttcaggtctttttaattgttatctcagcacatcctatgaatgtagacatactgattccatctaaagctttcaaatcagatgcatggccaccaaataatcataaaaacaaaatttcttttaaaaatgttgatgagtaatcaagagattttaaggaaaatatatatgtttgtttgttcttgtaaaacgcatactgtggtctttgagcaaggctaattttgcacaagtcagaactccacagctctttctggggctattaaaaaaagagccatctggccataagcaactgacagagtggctcttcccctgtagctgggcacccaccagggcctgggcatggctcttaacactggatgaggtacaacaatttacagaatatgttttctgtttccaggggccccattgtataggcatgaagcagactcacaaaaaattacaatatataggtgctaaaaataaatgtattttaaagttatattaaccgcacaaagcggtcagataattggcaggtgtgattccagcggctttggaagagaggtctttgacttgtatcttaaaggacaaatatgtcatcaggcaaaggggaatgtcacaggatgaaagaccttgagcacatatatagtggtttgaaggaacttgagatcccaggaagataaactgaaagcattttgtttgctcatttcatatatatatatatataaaatctagattatatatgtaattatatatatataatctagagcatgtaatgaaggaggaggcaatattggtaagaaatgtcagggagcaacatgtagtaggatacataagtcacacaaagagtttgaattctatcttgcaagcaataaaaacgcatgttttgcaagcactgcagtatcgtactcaggcattccttatagattatgattaccctttgtccttcaatgtgttggaaaggctaaattagaaaaagactaaaggaagggtcttaaccaagtcagagtcagggaaccaagaggagaaaacacatttgagaggccactctggtgctggaactagcagaatcctaggctgattatttaaatgcagtggtgtggctcatgcctgtaatcccagcactttgggaggcctaggtgggtggatcacctaagatcaggagtttgagaccagcctggccatattctgctcaaaaaaagcaaagaggcagaaagagcccaggctgacggttaaaaaccagcagcttccaagaaagatttttgatgagcaaaatttaactctcctggaaaacattcttattctgcaccagaacttaccaggcctcggtaaatatttgctgaatgaaatcaaaactaaaccaacaaaggcccatcctatcccaactagggagtttagaagactttttgagccagcatagttttttatattaggaaaagagtgacccaatactgaggtttattatgtcattgaagtaataagaattcccctaaggatatattgaggttttcgtctagtttagacttcataccaaaaaaaaaaaaaaaaaaaaaagacagatatgatcacccattggtatgtgtgtgctaaaatgacatatagtttgggttattaccattaaaaacttttgtatccttaactttcagtagagccagtgaaaataaagcttatataatatcccctaaagcacacatttttatctatgttatgggaaaaaaaaagagcataaattcagaagccagtttactaatgccctaatagattgtgacatacgtgctttttcagcggaatctacaaaatacttagagcaacatctcaagtacgaaacaaattcattcctaaaaataacccaactgaagaccttttagtagctctttcagctcaccctatgggtacagacatatcttgattccatctgaaaccttcaaatcagataaatgtgcagccatcaaataatcacaaaaagaatttttataaaaaataggaatggatgaccaagggctttaaaagacaagaattttgaggcttctaaaatgttccctttatttgccataaatgataatatatgtatccactgagaagttatgatagctccatcatgaaaaatctgaaggctagtcagtctcaaggatggtcaatttattaagaggcaggaaaacaattaagagtccatggagtcatgctcagtggtaattcctgactctgccatttacaggatttgtagctatagactaatcacttaatttctcttgaagctaagttttaaaatctaaaaattaaaataacgcaccttacagggttattttaaagacagaatgcaaacatacgttatcacacagtttgcacaaggtcttatataaacaaaggttgttagtaattatcaggtgccattattcctttagattgagttccatcgtggtgcttaataaaaatttaaatgtctgcatgtgtaattacgaaatacaatttctaagttttcaaatacttggtggaaacttgaaaatttaattcaaattaagttctgactttagcaatgtactctctcattgctgcatctattaaaaaccaagaacatctaattatgacagttgcatcaaccttaccaacaggtagaaacatctcttttgtcaccttagatgtcctgtcaatttaatgaagtagtataaagtgattatgcaggctctgagacactggaatgcattagaaaaagtgtttattacctgatctgtgagtttcttaatggctcacagacacttttctctgaatccccggaagaccctaacatagtgctgtagaaagtagatgaatagtaaatatatcagatgaagagatttcttcagggacatagtgagggagaagatttgcctgatttggctaagaacgcatttcactattctgtgaggcctctgaactcagcctagtgtttggaacagagtaggaggacattaatgaattattttgaatgaatggtattttttgactaatggtttagtctgtatagaataaggtctgtaactcttggcaaaagtacccaagaatagcatagatgttactttacataaaatccccaaaagtaatatgaattacttgttagcactgtctttcatagtcaatgttccaacagagattctacaaacaggtaatactagttaactgaaatgtcatgaatttatttcctgattcaatctctgtcaaatacattattaatgaaatggccaagaggggttagcaaaaggggttctgaaaaatcatatgagactaatcaattgaagttgagcatatgaatagatacatttccttgagtgcctattgaaaggatggacagatgtgctataaattctgcggcagaaaagtactatgagaattcttaaagaaatctgacatttaaaaccaatagcgtggctgggcatggtgtcctctgcctgtactcccagcactttgggtgatcgaggtgggatgattgcttgcatctaggagtttgagaccagcctgggcaacatggtaagaccgtgtttaaaaaaaatttaaaaataaaaaataaagccaatagcatctattttgaaataggggaaaagcctattctgataggataaatacaatgacattatctgtatcctaaacaacatagatttcaccagtataaaataagatgctctgtgtatgtgtgcatacctaaaaggtattcgtaggaacacacaatttagttgggaaatttaaaagaacatgaggatttcatataaactcctcacacaaaaaggatcaaatggcctttagaaatgcaagtcatattcatgataggagaatacgaaagtcctattacctcttttattcctgccctcctgcgtcatttcttctacattaacagcacaagtattgactgtatcccaatgaacttactcagataaacacaatgtggttttcttttaaaataagactttactgaatatatcaacaaggtactgtatagtgtagagtgaagtttgtcattaacaaagtgtgcgacatggtaggtctcagaggatgtgtgatgcagaatctttcagccccttatcagagagaacacactaaacagaaaccagaagcaaatcagcatatggttcaaacaataacaaatcatcaggttaactttcagtgaatatacactagtcctatgagcgacacacacttggcaatgccttcaccttgccttaaacattataaatcttacattccagggacacctttacaaatgcccctgtttgtgtgtgtgtgtgtgtgtgtgtacaagcatgtgcatgtttgataataatttttaaatgcctgttgcaatggccttgctttgtgctcttctggtgggtgtgcaggtagaaaacaaaaaactatagtaaaaaaatttgttttgttataacaacggtatcagacatatacaaaactctttctccacagtgacaagcattccccattgctagtaactgtcttttgaccctgctgaagaaatcagagaaggatgtaggttatgccttcttagcattcatattttgactttagaaagagcatcaggcaaggtttgacaagaccaagaacaagaccaagaactgttttgttctgtgtgagtatcttttttccatttggggcactgttttctgctttgctttcccatgcagctggaatggtaagtcatgagcaaaactgctattctcatgttctaaagtaaaatgtaatgtctccttgttataggttagagaaaaatgctataagcaaagacaccaatgggaattaaccccttcacttttcaaaagctgcgatggcctctgcagccaaggtccggagatcaagtgaagcatccattccctgtggactgcaatattgcctcgtgttctgaatggatgcttcaatcacagcatgaagatgttgtcctccctggtggggaaggaagttctgatttgtgtgaaatgactaagaccattatgataggtgctagtagaaaatgaagctgtaatattagctacttcattaatacttcttaccagactggtcacgtactttttgtttttaacctcagggagaatgtctaatatattttcaacgaacatccagataattagaaattgcattatttctcacaggggagaatgttttccatttgttacacaaggaaaataggcaggggatacattcctcgtatctgcctgcgattgtcccatgcagtgggctgctaatgcatctgacggtgtttgagggtggcccagagtctctctataatcaaacatatctccccaaacaagcaggtattaacaactaccctggctatagataactgtcaatatatccttttgatcatgactatgcctcttccttttcaatgtcttctgtacagtgacatttaccaagctctgaatgggatcagattctatctgagtcacctcatttggccaggcagcatcaagctctttattggccagtgagcatggctttttttcccatggtcttggcctgtactcgcaaccttgactcttgactaatcatctcaaaatacatcataatgacagcaagagaggcccaaacacagagcagatatatcagcaaatatacattcccatgactaaaaatgccaatcaaagcagaatccccagggacagttgtttggcaattttcataagacacattagacatcacagattccatcacgtgctttctatcctggtgcaggtgaggctgtaacaaatgggagacggattttaatcttagcagtctttgccatgttgtacacaaggtgaaaataaagcctgttactaggttcaatctcttcaggaacacctccagcaaaagggaccctgtcagaccatcttaagcattgcacatgactgtctccattgtaccatttaagccccaaataattctgtgaaccccataagaaatgacaggaacctcttcatccttgttcttcctggcccaaagtggtttcagcagccagaaatcccactgggggttaaacatacaatatacataaatgagaatgagtattttgtgaataacagaaataaaaaccctcaaaagtcaaagtaccatcatttgaatgcacaattttatctacacagccaaggggaagaggacagtagaagggaattatccagctaagtacacaaagcccccatgtcattgtcttgattttagatgtcttactgctacactgatcaccttcacagactcttttcccttcactgtgtggacctaactttaaaaaaagcaacagccaaaaccctctagctaatagactaaaatggaaaccagagtcactttagaattaatttaaattaattcatagctaagttcagctctactgactgcacagtttcaattcttgtgtctacgacatacagctgcagttatattttctgcttattctgagggacaagggagattaaaacatataagttgggctatattattaaagaaaataaagctcttactataaagaaaaagttgcatagcattttatacctaaacttttacaaagaagacacatcacagttttattttgctgagagagagagagctagtaagatgattgtgacatttacttcatgggtccctataataatggtcaatggtaaaagaaatatgcagcacagagtgaaatgtttaaatttgattttcgaaagatattttttccaagggagtagtttttgataacgtatgtgatctatagcccttctctatctaaggatggcaaagattaaattatgtgttttctgaaggtgttgtctcaaaagtatctagaattaagcacggacatcctctcttttctacgccctgctctgccaggattaggggaaaaagccttcactctctgacttgtttttcatgggttgtcctgctaacataagattgattagccctccacaattgccaaagtagaggaacatccacgatggaaaaggaacaaataaaatttcaaaagtggaacaggatcaaagtcagtccaaggtggaaaccaggtattgctttttaaaaaaaattcattattttggccagctttgatgtgtccttacagaattattagcagtgaaaattagtactcattttaaaatgtataagtacgtaatggatatcttgtgcagccaagactggcatccataattttccttgaaatactgaacagagggagaaaaacaaaggtgtcataaacaactaattatgaaaatatatgggagatgattggaagacaagaatttgcaaggggataaaagatattacttcaagctatttcaacatgatactaacaaagtcagctgacataacagaaccactgatcagttgtttttgtctaaatagcaggaagggtaatttttaaataagtcattgttgtattttccaaacattgatcacctgttggtctaaatatcatgttgacatagcctcagtgaatctacccaaataattctcattatcaaaaataattccattcaatataattcttccctttattagcctcttctaaaaaagtattctagaatatatctctgttgaatgtgattcaacctgatatatgatttgaacagtaacacttttaaagggagtcttcttgctacaacatcagactggtccctgaagatgactgaaatcagactcaagtctctaactctgttatcacataggaccagggaagcatgaagagtgatttttaagttcccagtcagaaagccaacccctgcattttcgggtcctttcaaatctcatctcaattttcttgattctgtcaggccgggttaacttatctcacgggaaccggcttcctcctggtgctttcagcatttcccacacagggtcaaatcagggtaactacctccattcttacattatagaattttttacctgtcttccggacctggaggtataggaatagtgtgaaactatcgggccatttcttgttttacccatattattcctcttaccctgatgagtccatttaatctgccctttcatctgaccaccaggaatttattctgacagcttcaacagcaaagtggttgatgtgtatcctaaggaaaaatcactcgttctttttgccttggcattgggttctcattgtacaaccctgtacagtacttcagcaacttttttttttttaagatttaaaaagcaaagagttacaaaactgtttgtaattaacttgaaatagaaaagatagcactttttttaaatcccattatatagtacaccgtataaattacagagtattcaaatgcacaaatgcatctgtgtaacatttatcaaatgtaatctgcgtgtctttatgtgcacacacgagtgtgttctcaagagtctaattgtccgccttgataacgctgggcctctggctgtcacgtatggcagtgctccaggtctggcacgctgctgttgcagtatcgcatgttgttggggatatggcagtctgtgtaattaatgcccccatttggggtgtaaatgggctgcagtctgaaatctcctttaaggagttgatcgttatttaaggagacgatctgaaaactggtttctgtcatctccaggatggagttgtccttcttggtgcctgcctcgcaataatcatctttccgccggccccggttgtatttccacttctgggaggtgtagcgcccctttttgtgcatatgccagcaaaagacgctgagcaagaccaccagcacaaatatcaccgcgcccccgatcaagcccgccagcagaaagggggagcccatgctgtgggacgtcgtctgctcatggctggacgctgtgttgctgccgttgttcagataggaggcatgggtggtggcctctgaacaaatggtgtcttctaccgcgcggtagttaaaagcatccagtggcactaaacaaatccgataggtggatcggggctctaagttaaccaggctcaggtgttgcttctcaccgctgactatgcgctcctgaacgatgccccctactaaactgtggcccattttcacccatgtgagtttgtatgccatcacggtgaagagagagagccagctgacttgaatggaagtatcattcacaaaatggatagagagctggatccgttcagaaataggtggggtcactctttctctgccatcccagtcaggaatcgtgggaagtttcgatgtggtaggagttggaggcgtgtagcttctgctagggtttggaatagagagggtgggaggctgagtggtcggagaagctgtacttggggctggggtgaagagaggcaggccgggggtcgtggtgggacaggacaaaagattcatatttaattccctgacggccatcccccggacttgttcaggaccttggcacatgaaaccccgcacgttgagagatgaagggatatatttgagccattctgtgacccatttaatactgcagtcacaaaaccaagggttattccgagcagtgagctgcttcaggttggagagattatcaaaaaccccttgagtcagcatccgcagttggttgttggatatatccagccgttccagcttacgcagatttgagaaggctgtcaaaggaatgtggtttatctggttgtcctgcaaatagagcctgatcagatgcgtacctgggagatcgggaggagggtgggacagcgaattacgtacaattgaaaattccttgagcttggtgagatggctgaaggtgccctcggcgatacccttgttggtcaggaggttcccgtccacaataagacgctccaagctcgtgagattctggaaggccatgtcggatatgacagcaattcgattttcatccactctcagctcttgcaagtccacaggaagcccaacaggcacactgctcaggtgattcttagacaaaaacaacaatttgaggctaatagcctcccggaaggccccgtcttccacccccactgtggatatggagttgtcatccaggtgcagctcttcaagcttcaagagctgggcaagagcagcccgtgaaatggtctgaatattgttttcctgcaaatggagaactctgacattcttgggaaggttcatggggaattcgtccagttggttgccatacaggtagaccgtgtgcaccgactgtacattgtgcagttctgcaggaaatccagcattattaatttggttgttgtggaggtagagtacagttacgccctccgggatcccaagaggcactgaggtcaagcttcgctcattacagtagacaaagttcctgtcgcagcggcacacactagggcaggccaggagtttggacacctgtgagtagagccccagggaaatgataagccaagacttcaggaaaaaagccccatggctgggccactttgtggtctgtaggcccatttctgaagtacggaaataaaatacaatgtggtgggaaaaagaaaaagaaaaaaaaaataaacagcaaaatcaaaatgactggatggggttctgttgaagtccagaactccagctagagggaacgtcctgagggcgtatggtaaaataatctccctgctgtctctggtcttatcagcctgtgttgccctctttgctgctgtcctccatgtgcaaaaaattcaacagggagaatttttccacactggcaacaggtgatggcaagttatcagccgtgtcaacacaagcccaagtgggcaggcagaactctcttcttcttttgtaggtcaagccagccttgattagcctacgaacttcttggttaagctcaatctgcaatctgcaaaggttctcgaggtctccttccagccctggtggtaatcccgctcagcgccgcgccctcccccagatccaaacttttgctgggtcctccgggtggcggcggcggcgacggcggcggctgctggagccaagccctgtcgcccgcagcgtcggggcgcgggggtgcggaggccggagcctcagagcggcgcgcgcctccccgcagcgggccggggccggggcgcccagctcgcctcgcttgctctcgcctacgtcccctacggagctgcggcatcgtcttcccccgtcctccgccaccaccgcctccagggttcgggcatgccactttctcttggcttcggccgccgcgacccccgccttctctcctcctccgcctccccctctccgcttcgccaagccaacgaaccccaaaagaagtacagcgagcggggaaggcggcagaaagctgccccgcggcgccggagctcctcggatttggaggatcccgggactcggcgggagagctaggcgggctctcctccgacgcgtgtgtgcggacagctcggagccgggcgtgcggcgctgcgcgggggcgggcgcagggctcgctccaagtgctgcgcccgcccggcgtgggtctggaggctgctcagaccacactact

SEQ ID NO: 13128 - RNA, 15952 nt, Homo sapiens
  source 1..15952: mol_type = other RNA
gctgggattacaggcatgagccaccacacccggcccagaatgttcgtaatttcatataaacattttatttgcctttctttttcttttcctgaagatgttttgttgcttacttttcagtttatactggctttttaaaacagatttcctttagagtaattacttccatagtgacagctatatttactgaaataaaatgtttcaaacatgtctcgaagtttgaatttctgtcactaaagaaaattagttaagattaataagaatgttttttgttttttttttttttttttctgcaggtgacttcacctttgattttcctacatttaggcaatgttagtgatgttctttaaactgccaggtagaatttcaatgtttgcaatacaaataccattaaatacttttattatagttactttgataaattcttttaaaaatactattttggtcctttatagaggtagcataatatttaaaactaactttaaaacaaattattttactaatctgcttgcattttattaaattccctttacagaattaatgaacttttaaagatttcataacaaagaactaattaatgagaagcataaataacagcttatgaaagaacaggtaatgataccttaatctgagtcccaaggaccactttccaattacacaattacaagccattaatttaaaatatcaatcattagactattatcaattattggaagtgtgtattatataaaaattatataaacatctttaataaagcaatgttgattacattcaggtgtatgatgtgatgaaataaagctagtgttcactggcagatattcttaggtaaccgctttaaagactaaacattttgaaatgaacatttcattgttagctgctaagtagtggttttataaaagtattgaaggtctgggaaagaagaatttcctaattattctaaaaagttttcatctttcttttttttaaaccataattgtatgtttgttcaaggttcagataaaagtggcagggatcagggttaaaatctgttctattccatcaaaaataaaccacatttattatttaatattttctagctattctcataattctttctctgtcaaatattagggtttaatagctgttatataatggcttgaaaacataaaatatttaatattttaataaacaattttttatacaatttttattgtacgacactctatctttgataattttgacttaaataaagtgttttattaatagtctacttagtaatatagtttgtatttccttgttttgagggagaagtggttgaactaatgagttttgttttcacttgcttctctttctattcatttgtaatttttcagccataatgggtttgaatatatgccaaccactgaagtgaagatgatataaattatctcatcaaatccttaaaagtattagtacctcatttcatatatgaggaaactgaggcttagggacattaaataatatcacacagatacaaagtcacagttctttgtgattctgtagctcctgattttaatggttatgcaggttgcttccctaacatatcaagtttaaggttattataactaatgagaaacatgttagtctttatacttaagtcaatgaaactgagtgtttatatgtttgctttatctatcctagtcacatcttcctgaattttaaaagcacacagaacacaaatcagtccaatgaaccaaatctaaactacatagaaaatgaacaaccataaaacagaatttaaggtccaaagtaacttgggagatcaactaaattcctgcgcttttgactataagaaacaagcccgagagagaagtggtcttatccaagatacaaaggagatttgagttatatagcccaactttttgcacactaattccatatattttcagaaagtagctggcatttattgagcactttatatgtgtcaggcactgtgcagtatggttactgttgaggtgagtgttgttattaacccatgtacagatgagaaaattgaagcatatacatgcccaaggaccaaggttagtatgagccaggatttaaatttagatgtagacagcattggactcagaatttaaaagattcatcatgttttcataatataacttcccatccaataggctacagtcttatagacacagttgctgttagatataattggcctccattacaaaacagctcacttcctgcttcctccttacttcagatacactagtaaagcatgctatattccaactaatgagggcagttatgtaaaatacttagcaataggatagctgaggcctaccagtcaaaacagacactagtccaaacagaatagagattggcagcagaccacaggaatgccagtacccattgatactacttgccaaataactgtcctgaaaccaattaaatcatgcagtcaaggactgaaaaagtatatttcccccctcatcaaatgtctgaacttctgcatttattaagcaaggaaagacataaatagaaaggaaaataatgctaatacagaccgtagtgagtgaattgctttgagactattaactaccacaaagtgtacagaaagaaaacaacgtgatccagctgaagaggatgcatgcctgttaataacaaccagcttccaaacttaataatgatatcgattgcaaaaagtaaccacatgacaggtggtagactattgcacctgcattgtagagacattaaaatgttcttccatttgactgctaccatccccactatcagcaaacccagtgtggatttaaatgccgtaattggtggtgtactagcatcaaataaaactatgtcttactagaaattatagatttttgaaacaatatcagaaatttattactttttttttttttttgagacagggtcttgctcagttgcctaagctggagtgcagtggcacaatcagagctcaatgtaatcttgatctcctgggctcaagtgaccctcctgcttcaacctcccaagtagctgggactataggcacatgccaccactcctggctaatttttttttttttttttagagatagggtctcactgcattgcccaggctggtctggaaatcctgacctcaagcaatcctcccaccttggcctcccaaagtactgcgattataggcatgagccactgtgctcagcttatcttgattttgtttttagtattttgatttccaatgccttctgaatgctcattcctggggctcttttgacacccacatattctgaattaattttcagcaataactacatctatgtgtactctagcaaccagatagaatatatgctacattataaagaagtctgttctctttctgttcaaccatgttgttcaatgatcccacacaccatgagaaaaaaggcctgccatggttgtgtgttatcccatggcacctcatcttcccaatttttttcccccagaaagaatacagaataatgaaaacctttctgacagacccatcttgataatagctgtgcaaattattgagtgttttgaggaattttgaatgctaattacctttaaatagatcatctctacatgtaattcttaccccaatacacaagaaatttgattttcatcataaaaagctggcaatttgtcaccatgtgcttgtgaattacatctgcatgaaaaatacatggtgcttcatgtcatttattcaatgtatactcagtaccagatactctgtcaactactatatatgcctttaattctgacaaccaccatatgtgttagacatcattgtccccattttaggaaaagtacactgataaccctaaagtgcaagttattgccaaggcaaattggcaggtcagtggttgaagcaggattccaaagtaagtcagcttgatttcaaactgatttcttaataactaccactctccactcccttctttacaagcatatcatttctaggaaagactattctcatggcaataaccaagataacacaatgtgaacctttaaatgatatatgctgtatttttatatgggatatgacatagtgaataatgactgtcttttttaattttgctgatgaagatgaaaaaaaaaaaatctctgcttttcacatgcaaagaattcattttgactagccgactgtcgaaatgtttaactttgtgtctacttgtgctttgtggacttttcatgatggcgatattttgttgcaaggtgatttttttttttttttttttgagtctcactctgtcaccaggctggagtgcaatggcatgatcttggctcactgcaacctccacctcctaggttcaagcaattctcctgcctcagcctcctgagtagctgggactacaggcacgcaccaccaagcccggctaaattttttgtatttttagtagagacagggtttcaccatgttggccaggatggtcttgatttcttgacctcgtgatctgcccacctcggcctcccaaagtgctgggattaaggtgatttttaaagatacctctttgtatgcttttctgcaagctggttcagttttgagtttgtctgtaatatataaaaaggatgttcttggctgggcgcagtggctcacacctgtaatcccagcactttgggaggcctaggtggggggatcacctgaggtcaggagttcgagactagcctggccaatgtggcaaaacccatctctactaaaaatacaaaaaattagccaggcatggtggtgcacgcctgtagtcccagctacgcaggaggctgaggcaggagaattgcttgaacccgggaggcggaggttgcagtgagccgagcttgtgccactgcactccaatctggtgacagagtgagactccaactcaaaaaaaaataaataaataaaataaaaagatgttcttcaggtctttttaattgttatctcagcacatcctatgaatgtagacatactgattccatctaaagctttcaaatcagatgcatggccaccaaataatcataaaaacaaaatttcttttaaaaatgttgatgagtaatcaagagattttaaggaaaatatatatgtttgtttgttcttgtaaaacgcatactgtggtctttgagcaaggctaattttgcacaagtcagaactccacagctctttctggggctattaaaaaaagagccatctggccataagcaactgacagagtggctcttcccctgtagctgggcacccaccagggcctgggcatggctcttaacactggatgaggtacaacaatttacagaatatgttttctgtttccaggggccccattgtataggcatgaagcagactcacaaaaaattacaatatataggtgctaaaaataaatgtattttaaagttatattaaccgcacaaagcggtcagataattggcaggtgtgattccagcggctttggaagagaggtctttgacttgtatcttaaaggacaaatatgtcatcaggcaaaggggaatgtcacaggatgaaagaccttgagcacatatatagtggtttgaaggaacttgagatcccaggaagataaactgaaagcattttgtttgctcatttcatatatatatatatataaaatctagattatatatgtaattatatatatataatctagagcatgtaatgaaggaggaggcaatattggtaagaaatgtcagggagcaacatgtagtaggatacataagtcacacaaagagtttgaattctatcttgcaagcaataaaaacgcatgttttgcaagcactgcagtatcgtactcaggcattccttatagattatgattaccctttgtccttcaatgtgttggaaaggctaaattagaaaaagactaaaggaagggtcttaaccaagtcagagtcagggaaccaagaggagaaaacacatttgagaggccactctggtgctggaactagcagaatcctaggctgattatttaaatgcagtggtgtggctcatgcctgtaatcccagcactttgggaggcctaggtgggtggatcacctaagatcaggagtttgagaccagcctggccatattctgctcaaaaaaagcaaagaggcagaaagagcccaggctgacggttaaaaaccagcagcttccaagaaagatttttgatgagcaaaatttaactctcctggaaaacattcttattctgcaccagaacttaccaggcctcggtaaatatttgctgaatgaaatcaaaactaaaccaacaaaggcccatcctatcccaactagggagtttagaagactttttgagccagcatagttttttatattaggaaaagagtgacccaatactgaggtttattatgtcattgaagtaataagaattcccctaaggatatattgaggttttcgtctagtttagacttcataccaaaaaaaaaaaaaaaaaaaaaagacagatatgatcacccattggtatgtgtgtgctaaaatgacatatagtttgggttattaccattaaaaacttttgtatccttaactttcagtagagccagtgaaaataaagcttatataatatcccctaaagcacacatttttatctatgttatgggaaaaaaaaagagcataaattcagaagccagtttactaatgccctaatagattgtgacatacgtgctttttcagcggaatctacaaaatacttagagcaacatctcaagtacgaaacaaattcattcctaaaaataacccaactgaagaccttttagtagctctttcagctcaccctatgggtacagacatatcttgattccatctgaaaccttcaaatcagataaatgtgcagccatcaaataatcacaaaaagaatttttataaaaaataggaatggatgaccaagggctttaaaagacaagaattttgaggcttctaaaatgttccctttatttgccataaatgataatatatgtatccactgagaagttatgatagctccatcatgaaaaatctgaaggctagtcagtctcaaggatggtcaatttattaagaggcaggaaaacaattaagagtccatggagtcatgctcagtggtaattcctgactctgccatttacaggatttgtagctatagactaatcacttaatttctcttgaagctaagttttaaaatctaaaaattaaaataacgcaccttacagggttattttaaagacagaatgcaaacatacgttatcacacagtttgcacaaggtcttatataaacaaaggttgttagtaattatcaggtgccattattcctttagattgagttccatcgtggtgcttaataaaaatttaaatgtctgcatgtgtaattacgaaatacaatttctaagttttcaaatacttggtggaaacttgaaaatttaattcaaattaagttctgactttagcaatgtactctctcattgctgcatctattaaaaaccaagaacatctaattatgacagttgcatcaaccttaccaacaggtagaaacatctcttttgtcaccttagatgtcctgtcaatttaatgaagtagtataaagtgattatgcaggctctgagacactggaatgcattagaaaaagtgtttattacctgatctgtgagtttcttaatggctcacagacacttttctctgaatccccggaagaccctaacatagtgctgtagaaagtagatgaatagtaaatatatcagatgaagagatttcttcagggacatagtgagggagaagatttgcctgatttggctaagaacgcatttcactattctgtgaggcctctgaactcagcctagtgtttggaacagagtaggaggacattaatgaattattttgaatgaatggtattttttgactaatggtttagtctgtatagaataaggtctgtaactcttggcaaaagtacccaagaatagcatagatgttactttacataaaatccccaaaagtaatatgaattacttgttagcactgtctttcatagtcaatgttccaacagagattctacaaacaggtaatactagttaactgaaatgtcatgaatttatttcctgattcaatctctgtcaaatacattattaatgaaatggccaagaggggttagcaaaaggggttctgaaaaatcatatgagactaatcaattgaagttgagcatatgaatagatacatttccttgagtgcctattgaaaggatggacagatgtgctataaattctgcggcagaaaagtactatgagaattcttaaagaaatctgacatttaaaaccaatagcgtggctgggcatggtgtcctctgcctgtactcccagcactttgggtgatcgaggtgggatgattgcttgcatctaggagtttgagaccagcctgggcaacatggtaagaccgtgtttaaaaaaaatttaaaaataaaaaataaagccaatagcatctattttgaaataggggaaaagcctattctgataggataaatacaatgacattatctgtatcctaaacaacatagatttcaccagtataaaataagatgctctgtgtatgtgtgcatacctaaaaggtattcgtaggaacacacaatttagttgggaaatttaaaagaacatgaggatttcatataaactcctcacacaaaaaggatcaaatggcctttagaaatgcaagtcatattcatgataggagaatacgaaagtcctattacctcttttattcctgccctcctgcgtcatttcttctacattaacagcacaagtattgactgtatcccaatgaacttactcagataaacacaatgtggttttcttttaaaataagactttactgaatatatcaacaaggtactgtatagtgtagagtgaagtttgtcattaacaaagtgtgcgacatggtaggtctcagaggatgtgtgatgcagaatctttcagccccttatcagagagaacacactaaacagaaaccagaagcaaatcagcatatggttcaaacaataacaaatcatcaggttaactttcagtgaatatacactagtcctatgagcgacacacacttggcaatgccttcaccttgccttaaacattataaatcttacattccagggacacctttacaaatgcccctgtttgtgtgtgtgtgtgtgtgtgtgtacaagcatgtgcatgtttgataataatttttaaatgcctgttgcaatggccttgctttgtgctcttctggtgggtgtgcaggtagaaaacaaaaaactatagtaaaaaaatttgttttgttataacaacggtatcagacatatacaaaactctttctccacagtgacaagcattccccattgctagtaactgtcttttgaccctgctgaagaaatcagagaaggatgtaggttatgccttcttagcattcatattttgactttagaaagagcatcaggcaaggtttgacaagaccaagaacaagaccaagaactgttttgttctgtgtgagtatcttttttccatttggggcactgttttctgctttgctttcccatgcagctggaatggtaagtcatgagcaaaactgctattctcatgttctaaagtaaaatgtaatgtctccttgttataggttagagaaaaatgctataagcaaagacaccaatgggaattaaccccttcacttttcaaaagctgcgatggcctctgcagccaaggtccggagatcaagtgaagcatccattccctgtggactgcaatattgcctcgtgttctgaatggatgcttcaatcacagcatgaagatgttgtcctccctggtggggaaggaagttctgatttgtgtgaaatgactaagaccattatgataggtgctagtagaaaatgaagctgtaatattagctacttcattaatacttcttaccagactggtcacgtactttttgtttttaacctcagggagaatgtctaatatattttcaacgaacatccagataattagaaattgcattatttctcacaggggagaatgttttccatttgttacacaaggaaaataggcaggggatacattcctcgtatctgcctgcgattgtcccatgcagtgggctgctaatgcatctgacggtgtttgagggtggcccagagtctctctataatcaaacatatctccccaaacaagcaggtattaacaactaccctggctatagataactgtcaatatatccttttgatcatgactatgcctcttccttttcaatgtcttctgtacagtgacatttaccaagctctgaatgggatcagattctatctgagtcacctcatttggccaggcagcatcaagctctttattggccagtgagcatggctttttttcccatggtcttggcctgtactcgcaaccttgactcttgactaatcatctcaaaatacatcataatgacagcaagagaggcccaaacacagagcagatatatcagcaaatatacattcccatgactaaaaatgccaatcaaagcagaatccccagggacagttgtttggcaattttcataagacacattagacatcacagattccatcacgtgctttctatcctggtgcaggtgaggctgtaacaaatgggagacggattttaatcttagcagtctttgccatgttgtacacaaggtgaaaataaagcctgttactaggttcaatctcttcaggaacacctccagcaaaagggaccctgtcagaccatcttaagcattgcacatgactgtctccattgtaccatttaagccccaaataattctgtgaaccccataagaaatgacaggaacctcttcatccttgttcttcctggcccaaagtggtttcagcagccagaaatcccactgggggttaaacatacaatatacataaatgagaatgagtattttgtgaataacagaaataaaaaccctcaaaagtcaaagtaccatcatttgaatgcacaattttatctacacagccaaggggaagaggacagtagaagggaattatccagctaagtacacaaagcccccatgtcattgtcttgattttagatgtcttactgctacactgatcaccttcacagactcttttcccttcactgtgtggacctaactttaaaaaaagcaacagccaaaaccctctagctaatagactaaaatggaaaccagagtcactttagaattaatttaaattaattcatagctaagttcagctctactgactgcacagtttcaattcttgtgtctacgacatacagctgcagttatattttctgcttattctgagggacaagggagattaaaacatataagttgggctatattattaaagaaaataaagctcttactataaagaaaaagttgcatagcattttatacctaaacttttacaaagaagacacatcacagttttattttgctgagagagagagagctagtaagatgattgtgacatttacttcatgggtccctataataatggtcaatggtaaaagaaatatgcagcacagagtgaaatgtttaaatttgattttcgaaagatattttttccaagggagtagtttttgataacgtatgtgatctatagcccttctctatctaaggatggcaaagattaaattatgtgttttctgaaggtgttgtctcaaaagtatctagaattaagcacggacatcctctcttttctacgccctgctctgccaggattaggggaaaaagccttcactctctgacttgtttttcatgggttgtcctgctaacataagattgattagccctccacaattgccaaagtagaggaacatccacgatggaaaaggaacaaataaaatttcaaaagtggaacaggatcaaagtcagtccaaggtggaaaccaggtattgctttttaaaaaaaattcattattttggccagctttgatgtgtccttacagaattattagcagtgaaaattagtactcattttaaaatgtataagtacgtaatggatatcttgtgcagccaagactggcatccataattttccttgaaatactgaacagagggagaaaaacaaaggtgtcataaacaactaattatgaaaatatatgggagatgattggaagacaagaatttgcaaggggataaaagatattacttcaagctatttcaacatgatactaacaaagtcagctgacataacagaaccactgatcagttgtttttgtctaaatagcaggaagggtaatttttaaataagtcattgttgtattttccaaacattgatcacctgttggtctaaatatcatgttgacatagcctcagtgaatctacccaaataattctcattatcaaaaataattccattcaatataattcttccctttattagcctcttctaaaaaagtattctagaatatatctctgttgaatgtgattcaacctgatatatgatttgaacagtaacacttttaaagggagtcttcttgctacaacatcagactggtccctgaagatgactgaaatcagactcaagtctctaactctgttatcacataggaccagggaagcatgaagagtgatttttaagttcccagtcagaaagccaacccctgcattttcgggtcctttcaaatctcatctcaattttcttgattctgtcaggccgggttaacttatctcacgggaaccggcttcctcctggtgctttcagcatttcccacacagggtcaaatcagggtaactacctccattcttacattatagaattttttacctgtcttccggacctggaggtataggaatagtgtgaaactatcgggccatttcttgttttacccatattattcctcttaccctgatgagtccatttaatctgccctttcatctgaccaccaggaatttattctgacagcttcaacagcaaagtggttgatgtgtatcctaaggaaaaatcactcgttctttttgccttggcattgggttctcattgtacaaccctgtacagtacttcagcaacttttttttttttaagatttaaaaagcaaagagttacaaaactgtttgtaattaacttgaaatagaaaagatagcactttttttaaatcccattatatagtacaccgtataaattacagagtattcaaatgcacaaatgcatctgtgtaacatttatcaaatgtaatctgcgtgtctttatgtgcacacacgagtgtgttctcaagagtctaattgtccgccttgataacgctgggcctctggctgtcacgtatggcagtgctccaggtctggcacgctgctgttgcagtatcgcatgttgttggggatatggcagtctgtgtaattaatgcccccatttggggtgtaaatgggctgcagtctgaaatctcctttaaggagttgatcgttatttaaggagacgatctgaaaactggtttctgtcatctccaggatggagttgtccttcttggtgcctgcctcgcaataatcatctttccgccggccccggttgtatttccacttctgggaggtgtagcgcccctttttgtgcatatgccagcaaaagacgctgagcaagaccaccagcacaaatatcaccgcgcccccgatcaagcccgccagcagaaagggggagcccatgctgtgggacgtcgtctgctcatggctggacgctgtgttgctgccgttgttcagataggaggcatgggtggtggcctctgaacaaatggtgtcttctaccgcgcggtagttaaaagcatccagtggcactaaacaaatccgataggtggatcggggctctaagttaaccaggctcaggtgttgcttctcaccgctgactatgcgctcctgaacgatgccccctactaaactgtggcccattttcacccatgtgagtttgtatgccatcacggtgaagagagagagccagctgacttgaatggaagtatcattcacaaaatggatagagagctggatccgttcagaaataggtggggtcactctttctctgccatcccagtcaggaatcgtgggaagtttcgatgtggtaggagttggaggcgtgtagcttctgctagggtttggaatagagagggtgggaggctgagtggtcggagaagctgtacttggggctggggtgaagagaggcaggccgggggtcgtggtgggacaggacaaaagattcatatttaattccctgacggccatcccccggacttgttcaggaccttggcacatgaaaccccgcacgttgagagatgaagggatatatttgagccattctgtgacccatttaatactgcagtcacaaaaccaagggttattccgagcagtgagctgcttcaggttggagagattatcaaaaaccccttgagtcagcatccgcagttggttgttggatatatccagccgttccagcttacgcagatttgagaaggctgtcaaaggaatgtggtttatctggttgtcctgcaaatagagcctgatcagatgcgtacctgggagatcgggaggagggtgggacagcgaattacgtacaattgaaaattccttgagcttggtgagatggctgaaggtgccctcggcgatacccttgttggtcaggaggttcccgtccacaataagacgctccaagctcgtgagattctggaaggccatgtcggatatgacagcaattcgattttcatccactctcagctcttgcaagtccacaggaagcccaacaggcacactgctcaggtgattcttagacaaaaacaacaatttgaggctaatagcctcccggaaggccccgtcttccacccccactgtggatatggagttgtcatccaggtgcagctcttcaagcttcaagagctgggcaagagcagcccgtgaaatggtctgaatattgttttcctgcaaatggagaactctgacattcttgggaaggttcatggggaattcgtccagttggttgccatacaggtagaccgtgtgcaccgactgtacattgtgcagttctgcaggaaatccagcattattaatttggttgttgtggaggtagagtacagttacgccctccgggatcccaagaggcactgaggtcaagcttcgctcattacagtagacaaagttcctgtcgcagcggcacacactagggcaggccaggagtttggacacctgtgagtagagccccagggaaatgataagccaagacttcaggaaaaaagccccatggctgggccactttgtggtctgtaggcccatttctgaagtacggaaataaaatacaatgtggtgggaaaaagaaaaagaaaaaaaaaataaacagcaaaatcaaaatgactggatggggttctgttgaagtccagaactccagctagagggaacgtcctgagggcgtatggtaaaataatctccctgctgtctctggtcttatcagcctgtgttgccctctttgctgctgtcctccatgtgcaaaaaattcaacagggagaatttttccacactggcaacaggtgatggcaagttatcagccgtgtcaacacaagcccaagtgggcaggcagaactctcttcttcttttgtaggtcaagccagccttgattagcctacgaacttcttggttaagctcaatctgcaatctggcaacgcagccccttttacctgacggctgcgtcttctccttgcaatgggctcatccgaatccgacagggtcagggaggtggaaagggaagacgctggcgcggcagcagcggggatcccggggcatggtattgttttaggggtcgccgccgaggtccctcctgcccatcgttgagaactgccaccctgatcccagggctcggtggacacggcggcgggagcggagatgccgcctcgccgctgctgggcaccagggacggaggaccagaggcgcacctcggaaaggagtagctcagcgccttggcgcggagatttgcgggcactgatgatatctcgagcgctcgttcctccgcggtgacaatggataatgccaaacgcgcaagtgacggcgacaggtttcgaacgtacaact

SEQ ID NO: 13129 - RNA, 3242 nt, Homo sapiens
  source 1..3242: mol_type = other RNA
gctgggattacaggcatgagccaccacacccggcctgaaaatggggtactttaaaaatagatgaatagtggctgcctgagtagtggagagggtcttctggattccttttccaatactctcctgccctcaagaagctccagctcaatatgttcttagttctggtaaaatagcaatgtcagaatatcaaattaacattaggcacatctcatcacagtgactcccatatattgaggctatgccaaagccccatgctcaagacctttggaaaccgtctgtaatttgactctgaaaatacaaagtagctaaattgatcttgccacctggctagcccttttggcctagagaatgcgctgatctgttcatagtggtccttttgaaaaggcagaacacgagcagtgagagaggtaagaggattcatgttgaccttagaaacttcacccagaaggtgaagctcatttaaactggtagattttctatagcaaaagaaaggagaacaagtaattacatggtttcattaagctacttaatttaggcccagtcagatctgcagttctctctggtctggggttaagactagcagcgttggattatttgtctttcctggctaagaaacattgtgctttcctcctgccccccaagttcttgaaatgcaccttttctttcaccaaaaagacagctatcgggtatttaccccatcctctaacacaccttcaaatgaaggttcctgattgagtcaatttgctgtggatgaagttagctgtttaatgcgaaagcagtctaacttctagtagcctagctaaatcctactgggagccttatacacgtagactaaactcttgctggtatcttcagatagtaatgcatttgtgtatttcagatgagttcatcttaattcacttccattttttgccttctattgccttgcttggcaggtagctgcattccatagtgtggcattcagtatggtggatttaaaagtgagggtgggagggtaaagtaggggttaggaacttttgcccaaggatcaggtttagtcttgcttatgggtaaactggtggggttccggaaaccgacatgggtcttccagtaggagtgggaacacatgaaggacccccaacaattcctttaattagtgcttattctagtttgagcactgcctgtattaaagtcagacgcagcccacggtggaaccttcttgaatacgagttaatacacgaatagctcagagctagagatccatcttctatttgtttgacaggcaacagctggaatgggctttcctccactaggaaccctgaaattgagtaatctagggtgaattaatactgctgtcttcccttcctccctttgatcttaatatcataaacgtttttaaagaactggaagagggtgagtgtgtagagaaaatgccaagtaggaaagttacaggtgagattaatgaattcatactgttactgtataaatacacaatttttttaaacagcaccatttccaagttatacacaatatgattatgacttggcacaacttttaaaggtggaaaaggctagttgctagttcagtaataaaatacctggtacatagaacgataaggagctgtattctacctgctacacattgtgcattttacacctccagctaggacagaaacaagccacaagcggggaatacccgcccaaattaatactggaaagtttacaaaaccttcacttctcataagggtgatgctaccagcggcttgcttcacctggaattagagtaactgatttttaaagacaactgagaatattaactcgcttcaaacaataaaatagtcattttgccgacatttcataaaatcgccagttttaagctcagttcagaggcttttaaaaaaatattctagacctagtaaagtgcctccattcataaaatgaaacatccaagattgagacaatttcatactgatgcgcatctaaaataggtcgacgtatacagtaaataaacagcgcctctaagttgccatatttcagttagtggaatacacacccagccttcgccgttctggatgtgcaaactagaaactgaagacaaatggggatttcagcgtctagtcccaatcgttcagcacggaagtactccacacggtcggctgcttttcaaaaaccaccaggacgacgtcccatgtcgagccgaccgctgagccgcacgcctccccacggcgggggcgagatggtgcgcagacctagcggtgcgaggggcggcggcgaccctgggcggccgggagcccgggccttcagcgcagcttcttgccaggcgggccgtccctggcgctgcggggcggcgggcgggcgggcggcggcggcactttggagagcgggcagtacttgatggtgtgcgcgttgtcgccgctggcgccgcacaggggacacgtgtagcggcgcagcacgggacacagcactcgcccgtcggggcccttgaggatatgggtggtgtagagcgccatcgcctccttgttgttccggcagaacacgcacacctgcagctcgggcttcagcagccgggcggccgccgccccggaggccgcgtgcagccggggctcggccgcccacgccggggcccgctcctcgcgcggcgtcgcctcgctggtggtggtggcggcggcggcggcggcgggcgcgcagcccagcagcacggcggcggcacgacccgcgaacgggctcagctcggcgaagcgctcctccagcagcccggcctcggcggggcccgcgcacagctccagcgcgcgcaattccagcgcgctccccaggtagcggccccgggaccccggctcgtcgctgtcgtcgtcgtcgtcctcgtcgtagtcgggcggccccagcgccggccccagcgccccaggcccggcccccgtgtggggggagcagcaggacgacgaggaggaggagggcggggagccgccgccgccgttcccaccgcgggcgcagccgaagcgcggctcgccgtccaccgctttggtgatgagcgtggcgagccccaggtagtcgttccaggagctgaagggctgcgggtgcgccgggcccggggcgctcacgtagcgggcgctgggcacgagcgccatgggcgggggggcgcggccgcggcggggcgagcggggcgcccaggggaaagcctccatgggcgggctgcgggccgcgcgccgcctccccgccgccggcgcgggccggacggaagggacacgccgagcctgcccgccggcctgccgc

SEQ ID NO: 13130 - RNA, 1428 nt, Homo sapiens
  source 1..1428: mol_type = other RNA
gctgggattacaggcatgagccaccacacccggcctgagatcaggccatttaaccagtaccctcagttacatcaaatatcaacttttttcttgccattcacacaaacttggcaatgcaatatgaaagatttgccactgtctatgctatggcatgagggtccaggttaatggcactcacaaaggagaaccttggctgtctcaagtgagccagcttacagcatttctagccatcagccatacagtagtaagtaacttgacagtcagatttcaagccctgtgatactcaaatttactctgaggcaagagaataaaaatgttttgccattaagtaaaaaatacgaggatgtctaatttggtatttaaaagtataaaatggctgggtacagccagctcatgcttataattgcaatacctcgggaggcccaggcaggaagattgcttgagctcaggagtttgagagcagcctgggcagcatagtgagagctcatctcttggtgaaagagtgacgacttttcaggtacatctgtggaagcatcccagtgccagagggatccatcttcagagcaggtaaaaagatgttctgggttggatgggtgaaagtgaacttcccacatttcagcttcatgagccttcagcagagatacaggcatagtaccttgtctaacatcccaaatactcaacattccatcttggccaccagtagctacaacatgctgttggttgggatgtctatcaacacagtggagtggcactcggtcaccagtcagtgacaatatctgagaaggctcatttccttgttgtctgaaatcccatattttcaactgtccaattgaatttacagtaagaatctcaggagttcgaagaaaggttacagcatggagtgtactactatctgcattgtctatggttcttacagcttccttgtgatcagctctgaagagatttattcgaccatcctctccaactgtaacgatttctgggttgttgcacacaacacctgtacatggtgcactgctataggaaggactgccagggcctgtgtggtagtgagctgtagtccactgctggttgactgacagagtctggttatttggatggtgaaggaaaactgttacacatcctgttgatgaagcagcgacaattctttcctggtcaaaaaactgtaaatccattacatcaccatggtgtctgatatcacacaataactgatggtctccttcaaaccctccatcagagtccaagtttccaaaatctccaatagaccacagtgaaatataattttcctcattgtcccaagatcctgtagcgaacgtctccgcggtctgtaaacttcccggaggcagcggtcgccagcgggttttgctgattttctgggacacaaacttcgcataaatttcctccatgccgaaagcggccgcagcaggtact

SEQ ID NO: 13131 - RNA, 2078 nt, Homo sapiens
  source 1..2078: mol_type = other RNA
gctgggattacaggcatgagccaccacacccggcctggacttcttatatatgaggtcttatatataatcttacatataaatatatatatctatgtataaaatctatctatgtatatctatctatctataaagaaagagacagagacagatacagggtctcacttcgttgcccaggctggtctcaaactcctgggctcaagtgttcctcctgcctcaaccttccaaagcgctgggattacaggcgtgagccaccaagcccagctaccatcagcaatttttattattgttcttccttgtggattttgtttttaatgatttggtccatcaatacatctttctcatgtacttgctggacaaagcgcacaactgcagatcagctctcctgatcagcaaaggaaattaattttattttctttaataaattactataacttgacctgaagatgtaaaaatatattattagcttttgaaactttaatatagatgtaatttctgacaagcttttacaaatactgaaaatagcttccaagtcctctttcttcttttaaggatctttggagattcataaaaactactgaatttgctgattatttaagttattagaggaagatgaaaattcagtgacttctcaaaaattataattcacatttaattacaagtcatgatttttctttactttttcaacaaaatggtaaatatagtctttaaaagatgtaaaaaaaaaattttttttacatttaaataagcatttaaaaatctaaggtaagactacaaagcagcataacaggttttctgtcacttgtaaactggattagaaggcaatccccagaattccagaaccgttgtggagatatgatttttaatttacaatctagaaaaactgcattcaacaagtagtccaaggatttgggttctagttgccagcttgcatggtacaatcttgagtaagtctctcaacttctggatataggaaatcaaaggccccccaacagaatgaaaggtgttaaatcaggtcatcttgaatattcttcccagctctgttattttacaacgccatgaaatcagagtaacatgttccaggctgtttggggtttgggattttagaacctgatgcaatgtatagcactttttaaatttctactttttggagtcttattcgaatatatacatatatatatgtcccccatgttcttctgtgcatgtagtatatttttctatttaacagcctcttcaccattagcaataaaaaagtttctcaaggatgtattttttatttcttttttttcggggggagagagtttcactcttgttgcccaggctggagtgcaacggcgcgatctcggcttactgcaacctccgccccccaggttcaagtgattctcctgcctcagcctcctgagtaactgggattacaggcatgcgccatcacatctggctaattttgtatttttcgtagagatggggtttcaccatgttggtcaggctggtctcgaactcctgacctcaggtgatccgcccaccacggcctcccaaagtgctgggattacaggcatgagccactgcgcccggcctcatttcttgcttttatgtttttttggcttccttttttaatttctccaagatctcttctggagttgtagaagccaaaagcttcaccaccttttcacgagatttaccacccttatccaaaaccacatcactcttcctgagttctaggaccttggaaagataccgacagagctcagcattagcctctccctctgatggaggtgctgcaatagctacatttacagcctctgctgtcaaatctgttacagcattttgtttggagccaggttttgcatggatggctatggtgacgcatcctttaggatcaactgccacaggacctaagggaggaagtggtctctctggttccttgctctggcttttacccttggtcgtcgcaccagccttcttaggcatctcggcgcaaagaagccgagcggagccccgagtattgggtgttgcccgaaggtgcctcagcccgctgcggagccgcagcatccccgcctgggaaggcgccggaagagccctct

SEQ ID NO: 13132 - RNA, 3793 nt, Homo sapiens
  source 1..3793: mol_type = other RNA
gctgggattacaggcatgagccaccacacccggctaattttgtatttttagtagaggcagggtttcaccatgttggccaggctggtcttgaactcctgactttgggtgatccacccgcctcggcctcccaaagtgctgggatgacaggcatgagccaccatgcccggcacctcgcctggctttttaatttttgagatgtctggctctgttgcccaggctggagggcagtgttgcgatcttggctcactgcaaccttcgcctcccaggttcaagcgattctcctgcctcggcctcccaagtagctgggactgcaggcgcaaaccaccatgccagactaattggctgtttaatttttaatagagatggggtcttgctttgttgtccaggctggttgaactcctggccttaattgatcctcctgccttggcctcccaaagtatcgggattgcaggagtgagccaacatgctcagcctgatgttgcatttctaaccagcatccacgtgatgccacagatgctgctgctgctccagcgggaatgtgggaaaagcacaggctcaggagtcagatggacatgggtggacatgggctctaaacctgactctgcccttggttgctgtgtgatgttgggcaagttgctgaacctctctgaattttggatttctcatgtgcaaaatagggatcacttctgccttttaggttctttgaagatttataataacgtacatgcataggttttcttcttgctcccagaggggcagggtgaggtcactctcctgcatgctctcactacaggttcagctgagaccgtttttcttctctaaagtacttggctttcttcttccaagtcaggatttctccgcctcggcgctactcacattttgggctggatcattttgtgttgtgggggatgctccgtgattaccgcattatagaacgttcagcagcatctctggcctcacccactggatactggtggcacccgtctcccctacttgtgaccaccgaaaatgtctccaggcactgccaaatgttcctggaggcaaaatcactcacaaataggaaataatgacctaattagtaacttacattagcaattcattcaacaatatgtgttgagcatctactgtttgccagaccatacagcagggatgtagtgatatttaagacaaacaaggtccctgacctcatggagactttttcctttttggacctcagtcttctccgctgtaatgtgggtatcacaaggctgcggacctcctaaatttgttgggaagatgaagttagacttgcaagtgcctggcccctggcatgagggattagccaatgccaggggtatgatgggcctagggatggaacctgggagcttggggagaagcgagtgtgggcagggacagtgcatggagaagccaggaaacctgagctgcaagggaggcggaaaggggccatgaaaggccctggtgcaaagtgtgcggcagcagcaaggcaggggaaaggggctgcagggagggccaagggtagcaggaagatgggaccaaaactggagagaaggagagagacagtgggacatagaggatgacaggaaggggtggagatgggaggagagaggcacagatggagaagataaaaaaccagacagacagacatgtacacacgtgataagacagagagaccaaggggcggagggaaaatgagtccaggcggaagggaacacctctgaggaagatcactgcacaaaccctggtcagctgcacatgaccccaaagagtggctcttaggtttattccaaacgtacctgatttgggtgataaagagttaaaattaaatacaaaggccaatgccagtccattcctggcgccagctcctgcctcttccttctcatggggccctcaccagagtgatggggtggagcatacccaaccctgggaggaaatgaggcttttgtgccgagcggcaatatgatggcaatactggcagtggtagtcaacccatctgtaaacagctgacagagggcagtacaagaatccacctcacagccagggccgcaaccgcaagtaaagcacacagctgaaatgactgacgtgggtggaactgagctgagaaggaacgtggctcggcttgaccctggagcacacatcacaaccatgagaaacaggcaactaaagtgacctccagcccacagcaacaaccttctctggctacaactgggaggcagggacagaccccagaaaaccatcttgggtcatctaaggtacgtgtaaccatatttttaaaatgacaaaatctcaagcatgttgctttggtgagcttctgattttactagaaatacactctaagaacagtcgagacgccgcgccttgtggaggcgatgggtcatgttactggttctgcgatgatcttccagagctccagttgctggaggcgctcgtaaaccaggagctgtgggaaggaggcctccacgggctccaccacgaagcgcagcttgccatctgcgagctgctccagcgcgtgcaggcaggagcggaagtgatcgtaggcttcacatgtgacgtccaagtgtctcaatgtgaagttgagcctcttctccaccgacagtatggctgtgcaggcatttttcaatctgtgggcgagtcgggagagcgttttaaacacagcatcagtcaagtcgtcgtcgtaaaacacttcggctgcaaacaggatggtggtgtgatcgtacaagtcagaaatttcctcttgtgaccaactgaaggggaccttgggatctgtgcagaggtcgtccttcagccagtccagttctttgaccctaactataccacctccagtggcagccaggtggctgttgagggcaatgtttcgctggcacatggacaagagatctgcaccgacatctgtacaataaacggtccgtgccatggtggctgcgatgatgctagcgagccccgtgccggccccgagctccagcgctgtacatcctcggaagaggtcctgtcggaacaggatgtagtctgccaggagcagggcgccccgccacacctattctgatgatatcgtgcgggctgccttgtgcttcctctcccaggacgtcgtcttcttcctgtgctagaatcatgggatgtaccttgtctctcagaggccctgctgggttggaatcagaggcggctcgtggtcttctcaccacgtccaaatccccatcctcatccagctgagcttcagccacttcctggccagtggtgtcagtcccggcctggagggagaaaccctcattaccatggccacttcctggaggggaccctgtgctgcctgtctcagcagaaggaggctcctttgtgtgaacatctctgtgactgccacccttggctcctgaatctgtccaagagtcttggctccatagaagcttgaattgggacaggaaaactggctgccccacgctgttcagccgtaccatgagatgtctatggttcggggtatagaggtggacatctgacagcacagtgtcgctcctaaaggtgacctcgtccatggctgccgcaggagccagctgtaccatggcccaggctccaccttagtcctaggacaggagtccctcagaggtgagaatgggtcctcagcatggcaggtcccagaggagatactgcagacaggtccaagctggtagcgagtagctttgcatcgccctgggagaagatctcagagacttggccagggaagagaatccagccgccgcggggcccagcctgggatcccacccgactcccgtctctgtgggacttaggcggccgccataacaggcggtct

SEQ ID NO: 13133 - RNA, 3834 nt, Homo sapiens
  source 1..3834: mol_type = other RNA
gctgggattacaggcatgagccaccacacccggctaattttgtatttttagtagaggcagggtttcaccatgttggccaggctggtcttgaactcctgactttgggtgatccacccgcctcggcctcccaaagtgctgggatgacaggcatgagccaccatgcccggcacctcgcctggctttttaatttttgagatgtctggctctgttgcccaggctggagggcagtgttgcgatcttggctcactgcaaccttcgcctcccaggttcaagcgattctcctgcctcggcctcccaagtagctgggactgcaggcgcaaaccaccatgccagactaattggctgtttaatttttaatagagatggggtcttgctttgttgtccaggctggttgaactcctggccttaattgatcctcctgccttggcctcccaaagtatcgggattgcaggagtgagccaacatgctcagcctgatgttgcatttctaaccagcatccacgtgatgccacagatgctgctgctgctccagcgggaatgtgggaaaagcacaggctcaggagtcagatggacatgggtggacatgggctctaaacctgactctgcccttggttgctgtgtgatgttgggcaagttgctgaacctctctgaattttggatttctcatgtgcaaaatagggatcacttctgccttttaggttctttgaagatttataataacgtacatgcataggttttcttcttgctcccagaggggcagggtgaggtcactctcctgcatgctctcactacaggttcagctgagaccgtttttcttctctaaagtacttggctttcttcttccaagtcaggatttctccgcctcggcgctactcacattttgggctggatcattttgtgttgtgggggatgctccgtgattaccgcattatagaacgttcagcagcatctctggcctcacccactggatactggtggcacccgtctcccctacttgtgaccaccgaaaatgtctccaggcactgccaaatgttcctggaggcaaaatcactcacaaataggaaataatgacctaattagtaacttacattagcaattcattcaacaatatgtgttgagcatctactgtttgccagaccatacagcagggatgtagtgatatttaagacaaacaaggtccctgacctcatggagactttttcctttttggacctcagtcttctccgctgtaatgtgggtatcacaaggctgcggacctcctaaatttgttgggaagatgaagttagacttgcaagtgcctggcccctggcatgagggattagccaatgccaggggtatgatgggcctagggatggaacctgggagcttggggagaagcgagtgtgggcagggacagtgcatggagaagccaggaaacctgagctgcaagggaggcggaaaggggccatgaaaggccctggtgcaaagtgtgcggcagcagcaaggcaggggaaaggggctgcagggagggccaagggtagcaggaagatgggaccaaaactggagagaaggagagagacagtgggacatagaggatgacaggaaggggtggagatgggaggagagaggcacagatggagaagataaaaaaccagacagacagacatgtacacacgtgataagacagagagaccaaggggcggagggaaaatgagtccaggcggaagggaacacctctgaggaagatcactgcacaaaccctggtcagctgcacatgaccccaaagagtggctcttaggtttattccaaacgtacctgatttgggtgataaagagttaaaattaaatacaaaggccaatgccagtccattcctggcgccagctcctgcctcttccttctcatggggccctcaccagagtgatggggtggagcatacccaaccctgggaggaaatgaggcttttgtgccgagcggcaatatgatggcaatactggcagtggtagtcaacccatctgtaaacagctgacagagggcagtacaagaatccacctcacagccagggccgcaaccgcaagtaaagcacacagctgaaatgactgacgtgggtggaactgagctgagaaggaacgtggctcggcttgaccctggagcacacatcacaaccatgagaaacaggcaactaaagtgacctccagcccacagcaacaaccttctctggctacaactgggaggcagggacagaccccagaaaaccatcttgggtcatctaaggtacgtgtaaccatatttttaaaatgacaaaatctcaagcatgttgctttggtgagcttctgattttactagaaatacactctaagaacagtcgagacgccgcgccttgtggaggcgatgggtcatgttactggttctgcgatgatcttccagagctccagttgctggaggcgctcgtaaaccaggagctgtgggaaggaggcctccacgggctccaccacgaagcgcagcttgccatctgcgagctgctccagcgcgtgcaggcaggagcggaagtgatcgtaggcttcacatgtgacgtccaagtgtctcaatgtgaagttgagcctcttctccaccgacagtatggctgtgcaggcatttttcaatctgtgggcgagtcgggagagcgttttaaacacagcatcagtcaagtcgtcgtcgtaaaacacttcggctgcaaacaggatggtggtgtgatcgtacaagtcagaaatttcctcttgtgaccaactgaaggggaccttgggatctgtgcagaggtcgtccttcagccagtccagttctttgaccctaactataccacctccagtggcagccaggtggctgttgagggcaatgtttcgctggcacatggacaagagatctgcaccgacatctgtacaataaacggtccgtgccatggtggctgcgatgatgctagcgagccccgtgccggccccgagctccagcgctgtacatcctcggaagaggtcctgtcggaacaggatgtagtctgccaggagcagggcgccccgccacacctgcttgccaacatcctccaggggcgtggccatggtgtgctctattctgatgatatcgtgcgggctgccttgtgcttcctctcccaggacgtcgtcttcttcctgtgctagaatcatgggatgtaccttgtctctcagaggccctgctgggttggaatcagaggcggctcgtggtcttctcaccacgtccaaatccccatcctcatccagctgagcttcagccacttcctggccagtggtgtcagtcccggcctggagggagaaaccctcattaccatggccacttcctggaggggaccctgtgctgcctgtctcagcagaaggaggctcctttgtgtgaacatctctgtgactgccacccttggctcctgaatctgtccaagagtcttggctccatagaagcttgaattgggacaggaaaactggctgccccacgctgttcagccgtaccatgagatgtctatggttcggggtatagaggtggacatctgacagcacagtgtcgctcctaaaggtgacctcgtccatggctgccgcaggagccagctgtaccatggcccaggctccaccttagtcctaggacaggagtccctcagaggtgagaatgggtcctcagcatggcaggtcccagaggagatactgcagacaggtccaagctggtagcgagtagctttgcatcgccctgggagaagatctcagagacttggccagggaagagaatccagccgccgcggggcccagcctgggatcccacccgactcccgtctctgtgggacttaggcggccgccataacaggcggtct

SEQ ID NO: 13134 - RNA, 3849 nt, Homo sapiens
  source 1..3849: mol_type = other RNA
gctgggattacaggcatgagccaccacacccggctaattttgtatttttagtagaggcagggtttcaccatgttggccaggctggtcttgaactcctgactttgggtgatccacccgcctcggcctcccaaagtgctgggatgacaggcatgagccaccatgcccggcacctcgcctggctttttaatttttgagatgtctggctctgttgcccaggctggagggcagtgttgcgatcttggctcactgcaaccttcgcctcccaggttcaagcgattctcctgcctcggcctcccaagtagctgggactgcaggcgcaaaccaccatgccagactaattggctgtttaatttttaatagagatggggtcttgctttgttgtccaggctggttgaactcctggccttaattgatcctcctgccttggcctcccaaagtatcgggattgcaggagtgagccaacatgctcagcctgatgttgcatttctaaccagcatccacgtgatgccacagatgctgctgctgctccagcgggaatgtgggaaaagcacaggctcaggagtcagatggacatgggtggacatgggctctaaacctgactctgcccttggttgctgtgtgatgttgggcaagttgctgaacctctctgaattttggatttctcatgtgcaaaatagggatcacttctgccttttaggttctttgaagatttataataacgtacatgcataggttttcttcttgctcccagaggggcagggtgaggtcactctcctgcatgctctcactacaggttcagctgagaccgtttttcttctctaaagtacttggctttcttcttccaagtcaggatttctccgcctcggcgctactcacattttgggctggatcattttgtgttgtgggggatgctccgtgattaccgcattatagaacgttcagcagcatctctggcctcacccactggatactggtggcacccgtctcccctacttgtgaccaccgaaaatgtctccaggcactgccaaatgttcctggaggcaaaatcactcacaaataggaaataatgacctaattagtaacttacattagcaattcattcaacaatatgtgttgagcatctactgtttgccagaccatacagcagggatgtagtgatatttaagacaaacaaggtccctgacctcatggagactttttcctttttggacctcagtcttctccgctgtaatgtgggtatcacaaggctgcggacctcctaaatttgttgggaagatgaagttagacttgcaagtgcctggcccctggcatgagggattagccaatgccaggggtatgatgggcctagggatggaacctgggagcttggggagaagcgagtgtgggcagggacagtgcatggagaagccaggaaacctgagctgcaagggaggcggaaaggggccatgaaaggccctggtgcaaagtgtgcggcagcagcaaggcaggggaaaggggctgcagggagggccaagggtagcaggaagatgggaccaaaactggagagaaggagagagacagtgggacatagaggatgacaggaaggggtggagatgggaggagagaggcacagatggagaagataaaaaaccagacagacagacatgtacacacgtgataagacagagagaccaaggggcggagggaaaatgagtccaggcggaagggaacacctctgaggaagatcactgcacaaaccctggtcagctgcacatgaccccaaagagtggctcttaggtttattccaaacgtacctgatttgggtgataaagagttaaaattaaatacaaaggccaatgccagtccattcctggcgccagctcctgcctcttccttctcatggggccctcaccagagtgatggggtggagcatacccaaccctgggaggaaatgaggcttttgtgccgagcggcaatatgatggcaatactggcagtggtagtcaacccatctgtaaacagctgacagagggcagtacaagaatccacctcacagccagggccgcaaccgcaagtaaagcacacagctgaaatgactgacgtgggtggaactgagctgagaaggaacgtggctcggcttgaccctggagcacacatcacaaccatgagaaacaggcaactaaagtgacctccagcccacagcaacaaccttctctggctacaactgggaggcagggacagaccccagaaaaccatcttgggtcatctaaggtacgtgtaaccatatttttaaaatgacaaaatctcaagcatgttgctttggtgagcttctgattttactagaaatacactctaagaacagtcgagacgccgcgccttgtggaggcgatgggtcatgttactggttctgcgatgatcttccagagctccagttgctggaggcgctcgtaaaccaggagctgtgggaaggaggcctccacgggctccaccacgaagcgcagcttgccatctgcgagctgctccagcgcgtgcaggcaggagcggaagtgatcgtaggcttcacatgtgacgtccaagtgtctcaatgtgaagttgagcctgcaaaccagccagtcggacgcacaaactcttctccaccgacagtatggctgtgcaggcatttttcaatctgtgggcgagtcgggagagcgttttaaacacagcatcagtcaagtcgtcgtcgtaaaacacttcggctgcaaacaggatggtggtgtgatcgtacaagtcagaaatttcctcttgtgaccaactgaaggggaccttgggatctgtgcagaggtcgtccttcagccagtccagttctttgaccctaactataccacctccagtggcagccaggtggctgttgagggcaatgtttcgctggcacatggacaagagatctgcaccgacatctgtacaataaacggtccgtgccatggtggctgcgatgatgctagcgagccccgtgccggccccgagctccagcgctgtacatcctcggaagaggtcctgtcggaacaggatgtagtctgccaggagcagggcgccccgccacacctattctgatgatatcgtgcgggctgccttgtgcttcctctcccaggacgtcgtcttcttcctgtgctagaatcatgggatgtaccttgtctctcagaggccctgctgggttggaatcagaggcggctcgtggtcttctcaccacgtccaaatccccatcctcatccagctgagcttcagccacttcctggccagtggtgtcagtcccggcctggagggagaaaccctcattaccatggccacttcctggaggggaccctgtgctgcctgtctcagcagaaggaggctcctttgtgtgaacatctctgtgactgccacccttggctcctgaatctgtccaagagtcttggctccatagaagcttgaattgggacaggaaaactggctgccccacgctgttcagccgtaccatgagatgtctatggttcggggtatagaggtggacatctgacagcacagtgtcgctcctaaaggtgacctcgtccatggctgccgcaggagccagctgtaccatggcccaggctccaccttagtcctaggacaggagtccctcagaggtgagaatgggtcctcagcatggcaggtcccagaggagatactgcagacaggtccaagctggtagcgagtagctttgcatcgccctgggagaagatctcagagacttggccagggaagagaatccagccgccgcggggcccagcctgggatcccacccgactcccgtctctgtgggacttaggcggccgccataacaggcggtctgcgcaggcgcggccccgcccccgcgtgc

SEQ ID NO: 13135 - RNA, 3890 nt, Homo sapiens
  source 1..3890: mol_type = other RNA
gctgggattacaggcatgagccaccacacccggctaattttgtatttttagtagaggcagggtttcaccatgttggccaggctggtcttgaactcctgactttgggtgatccacccgcctcggcctcccaaagtgctgggatgacaggcatgagccaccatgcccggcacctcgcctggctttttaatttttgagatgtctggctctgttgcccaggctggagggcagtgttgcgatcttggctcactgcaaccttcgcctcccaggttcaagcgattctcctgcctcggcctcccaagtagctgggactgcaggcgcaaaccaccatgccagactaattggctgtttaatttttaatagagatggggtcttgctttgttgtccaggctggttgaactcctggccttaattgatcctcctgccttggcctcccaaagtatcgggattgcaggagtgagccaacatgctcagcctgatgttgcatttctaaccagcatccacgtgatgccacagatgctgctgctgctccagcgggaatgtgggaaaagcacaggctcaggagtcagatggacatgggtggacatgggctctaaacctgactctgcccttggttgctgtgtgatgttgggcaagttgctgaacctctctgaattttggatttctcatgtgcaaaatagggatcacttctgccttttaggttctttgaagatttataataacgtacatgcataggttttcttcttgctcccagaggggcagggtgaggtcactctcctgcatgctctcactacaggttcagctgagaccgtttttcttctctaaagtacttggctttcttcttccaagtcaggatttctccgcctcggcgctactcacattttgggctggatcattttgtgttgtgggggatgctccgtgattaccgcattatagaacgttcagcagcatctctggcctcacccactggatactggtggcacccgtctcccctacttgtgaccaccgaaaatgtctccaggcactgccaaatgttcctggaggcaaaatcactcacaaataggaaataatgacctaattagtaacttacattagcaattcattcaacaatatgtgttgagcatctactgtttgccagaccatacagcagggatgtagtgatatttaagacaaacaaggtccctgacctcatggagactttttcctttttggacctcagtcttctccgctgtaatgtgggtatcacaaggctgcggacctcctaaatttgttgggaagatgaagttagacttgcaagtgcctggcccctggcatgagggattagccaatgccaggggtatgatgggcctagggatggaacctgggagcttggggagaagcgagtgtgggcagggacagtgcatggagaagccaggaaacctgagctgcaagggaggcggaaaggggccatgaaaggccctggtgcaaagtgtgcggcagcagcaaggcaggggaaaggggctgcagggagggccaagggtagcaggaagatgggaccaaaactggagagaaggagagagacagtgggacatagaggatgacaggaaggggtggagatgggaggagagaggcacagatggagaagataaaaaaccagacagacagacatgtacacacgtgataagacagagagaccaaggggcggagggaaaatgagtccaggcggaagggaacacctctgaggaagatcactgcacaaaccctggtcagctgcacatgaccccaaagagtggctcttaggtttattccaaacgtacctgatttgggtgataaagagttaaaattaaatacaaaggccaatgccagtccattcctggcgccagctcctgcctcttccttctcatggggccctcaccagagtgatggggtggagcatacccaaccctgggaggaaatgaggcttttgtgccgagcggcaatatgatggcaatactggcagtggtagtcaacccatctgtaaacagctgacagagggcagtacaagaatccacctcacagccagggccgcaaccgcaagtaaagcacacagctgaaatgactgacgtgggtggaactgagctgagaaggaacgtggctcggcttgaccctggagcacacatcacaaccatgagaaacaggcaactaaagtgacctccagcccacagcaacaaccttctctggctacaactgggaggcagggacagaccccagaaaaccatcttgggtcatctaaggtacgtgtaaccatatttttaaaatgacaaaatctcaagcatgttgctttggtgagcttctgattttactagaaatacactctaagaacagtcgagacgccgcgccttgtggaggcgatgggtcatgttactggttctgcgatgatcttccagagctccagttgctggaggcgctcgtaaaccaggagctgtgggaaggaggcctccacgggctccaccacgaagcgcagcttgccatctgcgagctgctccagcgcgtgcaggcaggagcggaagtgatcgtaggcttcacatgtgacgtccaagtgtctcaatgtgaagttgagcctgcaaaccagccagtcggacgcacaaactcttctccaccgacagtatggctgtgcaggcatttttcaatctgtgggcgagtcgggagagcgttttaaacacagcatcagtcaagtcgtcgtcgtaaaacacttcggctgcaaacaggatggtggtgtgatcgtacaagtcagaaatttcctcttgtgaccaactgaaggggaccttgggatctgtgcagaggtcgtccttcagccagtccagttctttgaccctaactataccacctccagtggcagccaggtggctgttgagggcaatgtttcgctggcacatggacaagagatctgcaccgacatctgtacaataaacggtccgtgccatggtggctgcgatgatgctagcgagccccgtgccggccccgagctccagcgctgtacatcctcggaagaggtcctgtcggaacaggatgtagtctgccaggagcagggcgccccgccacacctgcttgccaacatcctccaggggcgtggccatggtgtgctctattctgatgatatcgtgcgggctgccttgtgcttcctctcccaggacgtcgtcttcttcctgtgctagaatcatgggatgtaccttgtctctcagaggccctgctgggttggaatcagaggcggctcgtggtcttctcaccacgtccaaatccccatcctcatccagctgagcttcagccacttcctggccagtggtgtcagtcccggcctggagggagaaaccctcattaccatggccacttcctggaggggaccctgtgctgcctgtctcagcagaaggaggctcctttgtgtgaacatctctgtgactgccacccttggctcctgaatctgtccaagagtcttggctccatagaagcttgaattgggacaggaaaactggctgccccacgctgttcagccgtaccatgagatgtctatggttcggggtatagaggtggacatctgacagcacagtgtcgctcctaaaggtgacctcgtccatggctgccgcaggagccagctgtaccatggcccaggctccaccttagtcctaggacaggagtccctcagaggtgagaatgggtcctcagcatggcaggtcccagaggagatactgcagacaggtccaagctggtagcgagtagctttgcatcgccctgggagaagatctcagagacttggccagggaagagaatccagccgccgcggggcccagcctgggatcccacccgactcccgtctctgtgggacttaggcggccgccataacaggcggtctgcgcaggcgcggccccgcccccgcgtgc

SEQ ID NO: 13136 - RNA, 3652 nt, Homo sapiens
  source 1..3652: mol_type = other RNA
gctgggattacaggcatgagccaccacacccggctaattttgtatttttagtagaggcagggtttcaccatgttggccaggctggtcttgaactcctgactttgggtgatccacccgcctcggcctcccaaagtgctgggatgacaggcatgagccaccatgcccggcacctcgcctggctttttaatttttgagatgtctggctctgttgcccaggctggagggcagtgttgcgatcttggctcactgcaaccttcgcctcccaggttcaagcgattctcctgcctcggcctcccaagtagctgggactgcaggcgcaaaccaccatgccagactaattggctgtttaatttttaatagagatggggtcttgctttgttgtccaggctggttgaactcctggccttaattgatcctcctgccttggcctcccaaagtatcgggattgcaggagtgagccaacatgctcagcctgatgttgcatttctaaccagcatccacgtgatgccacagatgctgctgctgctccagcgggaatgtgggaaaagcacaggctcaggagtcagatggacatgggtggacatgggctctaaacctgactctgcccttggttgctgtgtgatgttgggcaagttgctgaacctctctgaattttggatttctcatgtgcaaaatagggatcacttctgccttttaggttctttgaagatttataataacgtacatgcataggttttcttcttgctcccagaggggcagggtgaggtcactctcctgcatgctctcactacaggttcagctgagaccgtttttcttctctaaagtacttggctttcttcttccaagtcaggatttctccgcctcggcgctactcacattttgggctggatcattttgtgttgtgggggatgctccgtgattaccgcattatagaacgttcagcagcatctctggcctcacccactggatactggtggcacccgtctcccctacttgtgaccaccgaaaatgtctccaggcactgccaaatgttcctggaggcaaaatcactcacaaataggaaataatgacctaattagtaacttacattagcaattcattcaacaatatgtgttgagcatctactgtttgccagaccatacagcagggatgtagtgatatttaagacaaacaaggtccctgacctcatggagactttttcctttttggacctcagtcttctccgctgtaatgtgggtatcacaaggctgcggacctcctaaatttgttgggaagatgaagttagacttgcaagtgcctggcccctggcatgagggattagccaatgccaggggtatgatgggcctagggatggaacctgggagcttggggagaagcgagtgtgggcagggacagtgcatggagaagccaggaaacctgagctgcaagggaggcggaaaggggccatgaaaggccctggtgcaaagtgtgcggcagcagcaaggcaggggaaaggggctgcagggagggccaagggtagcaggaagatgggaccaaaactggagagaaggagagagacagtgggacatagaggatgacaggaaggggtggagatgggaggagagaggcacagatggagaagataaaaaaccagacagacagacatgtacacacgtgataagacagagagaccaaggggcggagggaaaatgagtccaggcggaagggaacacctctgaggaagatcactgcacaaaccctggtcagctgcacatgaccccaaagagtggctcttaggtttattccaaacgtacctgatttgggtgataaagagttaaaattaaatacaaaggccaatgccagtccattcctggcgccagctcctgcctcttccttctcatggggccctcaccagagtgatggggtggagcatacccaaccctgggaggaaatgaggcttttgtgccgagcggcaatatgatggcaatactggcagtggtagtcaacccatctgtaaacagctgacagagggcagtacaagaatccacctcacagccagggccgcaaccgcaagtaaagcacacagctgaaatgactgacgtgggtggaactgagctgagaaggaacgtggctcggcttgaccctggagcacacatcacaaccatgagaaacaggcaactaaagtgacctccagcccacagcaacaaccttctctggctacaactgggaggcagggacagaccccagaaaaccatcttgggtcatctaaggtacgtgtaaccatatttttaaaatgacaaaatctcaagcatgttgctttggtgagcttctgattttactagaaatacactctaagaacagtcgagacgccgcgccttgtggaggcgatgggtcatgttactggttctgcgatgatcttccagagctcctcttctccaccgacagtatggctgtgcaggcatttttcaatctgtgggcgagtcgggagagcgttttaaacacagcatcagtcaagtcgtcgtcgtaaaacacttcggctgcaaacaggatggtggtgtgatcgtacaagtcagaaatttcctcttgtgaccaactgaaggggaccttgggatctgtgcagaggtcgtccttcagccagtccagttctttgaccctaactataccacctccagtggcagccaggtggctgttgagggcaatgtttcgctggcacatggacaagagatctgcaccgacatctgtacaataaacggtccgtgccatggtggctgcgatgatgctagcgagccccgtgccggccccgagctccagcgctgtacatcctcggaagaggtcctgtcggaacaggatgtagtctgccaggagcagggcgccccgccacacctattctgatgatatcgtgcgggctgccttgtgcttcctctcccaggacgtcgtcttcttcctgtgctagaatcatgggatgtaccttgtctctcagaggccctgctgggttggaatcagaggcggctcgtggtcttctcaccacgtccaaatccccatcctcatccagctgagcttcagccacttcctggccagtggtgtcagtcccggcctggagggagaaaccctcattaccatggccacttcctggaggggaccctgtgctgcctgtctcagcagaaggaggctcctttgtgtgaacatctctgtgactgccacccttggctcctgaatctgtccaagagtcttggctccatagaagcttgaattgggacaggaaaactggctgccccacgctgttcagccgtaccatgagatgtctatggttcggggtatagaggtggacatctgacagcacagtgtcgctcctaaaggtgacctcgtccatggctgccgcaggagccagctgtaccatggcccaggctccaccttagtcctaggacaggagtccctcagaggtgagaatgggtcctcagcatggcaggtcccagaggagatactgcagacaggtccaagctggtagcgagtagctttgcatcgccctgggagaagatctcagagacttggccagggaagagaatccagccgccgcggggcccagcctgggatcccacccgactcccgtctctgtgggacttaggcggccgccataacaggcggtctgcgcaggcgcggccccgcccccgcgtgc

SEQ ID NO: 13137 - RNA, 3693 nt, Homo sapiens
  source 1..3693: mol_type = other RNA
gctgggattacaggcatgagccaccacacccggctaattttgtatttttagtagaggcagggtttcaccatgttggccaggctggtcttgaactcctgactttgggtgatccacccgcctcggcctcccaaagtgctgggatgacaggcatgagccaccatgcccggcacctcgcctggctttttaatttttgagatgtctggctctgttgcccaggctggagggcagtgttgcgatcttggctcactgcaaccttcgcctcccaggttcaagcgattctcctgcctcggcctcccaagtagctgggactgcaggcgcaaaccaccatgccagactaattggctgtttaatttttaatagagatggggtcttgctttgttgtccaggctggttgaactcctggccttaattgatcctcctgccttggcctcccaaagtatcgggattgcaggagtgagccaacatgctcagcctgatgttgcatttctaaccagcatccacgtgatgccacagatgctgctgctgctccagcgggaatgtgggaaaagcacaggctcaggagtcagatggacatgggtggacatgggctctaaacctgactctgcccttggttgctgtgtgatgttgggcaagttgctgaacctctctgaattttggatttctcatgtgcaaaatagggatcacttctgccttttaggttctttgaagatttataataacgtacatgcataggttttcttcttgctcccagaggggcagggtgaggtcactctcctgcatgctctcactacaggttcagctgagaccgtttttcttctctaaagtacttggctttcttcttccaagtcaggatttctccgcctcggcgctactcacattttgggctggatcattttgtgttgtgggggatgctccgtgattaccgcattatagaacgttcagcagcatctctggcctcacccactggatactggtggcacccgtctcccctacttgtgaccaccgaaaatgtctccaggcactgccaaatgttcctggaggcaaaatcactcacaaataggaaataatgacctaattagtaacttacattagcaattcattcaacaatatgtgttgagcatctactgtttgccagaccatacagcagggatgtagtgatatttaagacaaacaaggtccctgacctcatggagactttttcctttttggacctcagtcttctccgctgtaatgtgggtatcacaaggctgcggacctcctaaatttgttgggaagatgaagttagacttgcaagtgcctggcccctggcatgagggattagccaatgccaggggtatgatgggcctagggatggaacctgggagcttggggagaagcgagtgtgggcagggacagtgcatggagaagccaggaaacctgagctgcaagggaggcggaaaggggccatgaaaggccctggtgcaaagtgtgcggcagcagcaaggcaggggaaaggggctgcagggagggccaagggtagcaggaagatgggaccaaaactggagagaaggagagagacagtgggacatagaggatgacaggaaggggtggagatgggaggagagaggcacagatggagaagataaaaaaccagacagacagacatgtacacacgtgataagacagagagaccaaggggcggagggaaaatgagtccaggcggaagggaacacctctgaggaagatcactgcacaaaccctggtcagctgcacatgaccccaaagagtggctcttaggtttattccaaacgtacctgatttgggtgataaagagttaaaattaaatacaaaggccaatgccagtccattcctggcgccagctcctgcctcttccttctcatggggccctcaccagagtgatggggtggagcatacccaaccctgggaggaaatgaggcttttgtgccgagcggcaatatgatggcaatactggcagtggtagtcaacccatctgtaaacagctgacagagggcagtacaagaatccacctcacagccagggccgcaaccgcaagtaaagcacacagctgaaatgactgacgtgggtggaactgagctgagaaggaacgtggctcggcttgaccctggagcacacatcacaaccatgagaaacaggcaactaaagtgacctccagcccacagcaacaaccttctctggctacaactgggaggcagggacagaccccagaaaaccatcttgggtcatctaaggtacgtgtaaccatatttttaaaatgacaaaatctcaagcatgttgctttggtgagcttctgattttactagaaatacactctaagaacagtcgagacgccgcgccttgtggaggcgatgggtcatgttactggttctgcgatgatcttccagagctcctcttctccaccgacagtatggctgtgcaggcatttttcaatctgtgggcgagtcgggagagcgttttaaacacagcatcagtcaagtcgtcgtcgtaaaacacttcggctgcaaacaggatggtggtgtgatcgtacaagtcagaaatttcctcttgtgaccaactgaaggggaccttgggatctgtgcagaggtcgtccttcagccagtccagttctttgaccctaactataccacctccagtggcagccaggtggctgttgagggcaatgtttcgctggcacatggacaagagatctgcaccgacatctgtacaataaacggtccgtgccatggtggctgcgatgatgctagcgagccccgtgccggccccgagctccagcgctgtacatcctcggaagaggtcctgtcggaacaggatgtagtctgccaggagcagggcgccccgccacacctgcttgccaacatcctccaggggcgtggccatggtgtgctctattctgatgatatcgtgcgggctgccttgtgcttcctctcccaggacgtcgtcttcttcctgtgctagaatcatgggatgtaccttgtctctcagaggccctgctgggttggaatcagaggcggctcgtggtcttctcaccacgtccaaatccccatcctcatccagctgagcttcagccacttcctggccagtggtgtcagtcccggcctggagggagaaaccctcattaccatggccacttcctggaggggaccctgtgctgcctgtctcagcagaaggaggctcctttgtgtgaacatctctgtgactgccacccttggctcctgaatctgtccaagagtcttggctccatagaagcttgaattgggacaggaaaactggctgccccacgctgttcagccgtaccatgagatgtctatggttcggggtatagaggtggacatctgacagcacagtgtcgctcctaaaggtgacctcgtccatggctgccgcaggagccagctgtaccatggcccaggctccaccttagtcctaggacaggagtccctcagaggtgagaatgggtcctcagcatggcaggtcccagaggagatactgcagacaggtccaagctggtagcgagtagctttgcatcgccctgggagaagatctcagagacttggccagggaagagaatccagccgccgcggggcccagcctgggatcccacccgactcccgtctctgtgggacttaggcggccgccataacaggcggtctgcgcaggcgcggccccgcccccgcgtgc

SEQ ID NO: 13138 - RNA, 3966 nt, Homo sapiens
  source 1..3966: mol_type = other RNA
gctgggattacaggcatgagccaccacacccggctaattttgtatttttagtagaggcagggtttcaccatgttggccaggctggtcttgaactcctgactttgggtgatccacccgcctcggcctcccaaagtgctgggatgacaggcatgagccaccatgcccggcacctcgcctggctttttaatttttgagatgtctggctctgttgcccaggctggagggcagtgttgcgatcttggctcactgcaaccttcgcctcccaggttcaagcgattctcctgcctcggcctcccaagtagctgggactgcaggcgcaaaccaccatgccagactaattggctgtttaatttttaatagagatggggtcttgctttgttgtccaggctggttgaactcctggccttaattgatcctcctgccttggcctcccaaagtatcgggattgcaggagtgagccaacatgctcagcctgatgttgcatttctaaccagcatccacgtgatgccacagatgctgctgctgctccagcgggaatgtgggaaaagcacaggctcaggagtcagatggacatgggtggacatgggctctaaacctgactctgcccttggttgctgtgtgatgttgggcaagttgctgaacctctctgaattttggatttctcatgtgcaaaatagggatcacttctgccttttaggttctttgaagatttataataacgtacatgcataggttttcttcttgctcccagaggggcagggtgaggtcactctcctgcatgctctcactacaggttcagctgagaccgtttttcttctctaaagtacttggctttcttcttccaagtcaggatttctccgcctcggcgctactcacattttgggctggatcattttgtgttgtgggggatgctccgtgattaccgcattatagaacgttcagcagcatctctggcctcacccactggatactggtggcacccgtctcccctacttgtgaccaccgaaaatgtctccaggcactgccaaatgttcctggaggcaaaatcactcacaaataggaaataatgacctaattagtaacttacattagcaattcattcaacaatatgtgttgagcatctactgtttgccagaccatacagcagggatgtagtgatatttaagacaaacaaggtccctgacctcatggagactttttcctttttggacctcagtcttctccgctgtaatgtgggtatcacaaggctgcggacctcctaaatttgttgggaagatgaagttagacttgcaagtgcctggcccctggcatgagggattagccaatgccaggggtatgatgggcctagggatggaacctgggagcttggggagaagcgagtgtgggcagggacagtgcatggagaagccaggaaacctgagctgcaagggaggcggaaaggggccatgaaaggccctggtgcaaagtgtgcggcagcagcaaggcaggggaaaggggctgcagggagggccaagggtagcaggaagatgggaccaaaactggagagaaggagagagacagtgggacatagaggatgacaggaaggggtggagatgggaggagagaggcacagatggagaagataaaaaaccagacagacagacatgtacacacgtgataagacagagagaccaaggggcggagggaaaatgagtccaggcggaagggaacacctctgaggaagatcactgcacaaaccctggtcagctgcacatgaccccaaagagtggctcttaggtttattccaaacgtacctgatttgggtgataaagagttaaaattaaatacaaaggccaatgccagtccattcctggcgccagctcctgcctcttccttctcatggggccctcaccagagtgatggggtggagcatacccaaccctgggaggaaatgaggcttttgtgccgagcggcaatatgatggcaatactggcagtggtagtcaacccatctgtaaacagctgacagagggcagtacaagaatccacctcacagccagggccgcaaccgcaagtaaagcacacagctgaaatgactgacgtgggtggaactgagctgagaaggaacgtggctcggcttgaccctggagcacacatcacaaccatgagaaacaggcaactaaagtgacctccagcccacagcaacaaccttctctggctacaactgggaggcagggacagaccccagaaaaccatcttgggtcatctaaggtacgtgtaaccatatttttaaaatgacaaaatctcaagcatgttgctttggtgagcttctgattttactagaaatacactctaagaacagtcgagacgccgcgccttgtggaggcgatgggtcatgttactggttctgcgatgatcttccagagctcctcttctccaccgacagtatggctgtgcaggcatttttcaatctgtgggcgagtcgggagagcgttttaaacacagcatcagtcaagtcgtcgtcgtaaaacacttcggctgcaaacaggatggtggtgtgatcgtacaagtcagaaatttcctcttgtgaccaactgaaggggaccttgggatctgtgcagaggtcgtccttcagccagtccagttctttgaccctaactataccacctgtgagtgagtcctggccgtgctggatgcagggctggaaaggagactgtcaggaggaggcaaggagagcaggccggggctgggccagggaggcctgggaattcaaggagctcagacttcaccccacaggtgatgacgcccctgggaggttttcagcagcaagtgaagtggactggcttgcatctgagaaagggcactctggatgtttcatgaggacatcttggacgggtcaactaaggagctggggagaccagctcaggggccgccgccagtgtccgggagagaaagagctggagtaggatgacgcagtggatctccagtggcagccaggtggctgttgagggcaatgtttcgctggcacatggacaagagatctgcaccgacatctgtacaataaacggtccgtgccatggtggctgcgatgatgctagcgagccccgtgccggccccgagctccagcgctgtacatcctcggaagaggtcctgtcggaacaggatgtagtctgccaggagcagggcgccccgccacacctattctgatgatatcgtgcgggctgccttgtgcttcctctcccaggacgtcgtcttcttcctgtgctagaatcatgggatgtaccttgtctctcagaggccctgctgggttggaatcagaggcggctcgtggtcttctcaccacgtccaaatccccatcctcatccagctgagcttcagccacttcctggccagtggtgtcagtcccggcctggagggagaaaccctcattaccatggccacttcctggaggggaccctgtgctgcctgtctcagcagaaggaggctcctttgtgtgaacatctctgtgactgccacccttggctcctgaatctgtccaagagtcttggctccatagaagcttgaattgggacaggaaaactggctgccccacgctgttcagccgtaccatgagatgtctatggttcggggtatagaggtggacatctgacagcacagtgtcgctcctaaaggtgacctcgtccatggctgccgcaggagccagctgtaccatggcccaggctccaccttagtcctaggacaggagtccctcagaggtgagaatgggtcctcagcatggcaggtcccagaggagatactgcagacaggtccaagctggtagcgagtagctttgcatcgccctgggagaagatctcagagacttggccagggaagagaatccagccgccgcggggcccagcctgggatcccacccgactcccgtctctgtgggacttaggcggccgccataacaggcggtctgcgcaggcgcggccccgcccccgcgtgc

SEQ ID NO: 13139 - RNA, 4007 nt, Homo sapiens
  source 1..4007: mol_type = other RNA
gctgggattacaggcatgagccaccacacccggctaattttgtatttttagtagaggcagggtttcaccatgttggccaggctggtcttgaactcctgactttgggtgatccacccgcctcggcctcccaaagtgctgggatgacaggcatgagccaccatgcccggcacctcgcctggctttttaatttttgagatgtctggctctgttgcccaggctggagggcagtgttgcgatcttggctcactgcaaccttcgcctcccaggttcaagcgattctcctgcctcggcctcccaagtagctgggactgcaggcgcaaaccaccatgccagactaattggctgtttaatttttaatagagatggggtcttgctttgttgtccaggctggttgaactcctggccttaattgatcctcctgccttggcctcccaaagtatcgggattgcaggagtgagccaacatgctcagcctgatgttgcatttctaaccagcatccacgtgatgccacagatgctgctgctgctccagcgggaatgtgggaaaagcacaggctcaggagtcagatggacatgggtggacatgggctctaaacctgactctgcccttggttgctgtgtgatgttgggcaagttgctgaacctctctgaattttggatttctcatgtgcaaaatagggatcacttctgccttttaggttctttgaagatttataataacgtacatgcataggttttcttcttgctcccagaggggcagggtgaggtcactctcctgcatgctctcactacaggttcagctgagaccgtttttcttctctaaagtacttggctttcttcttccaagtcaggatttctccgcctcggcgctactcacattttgggctggatcattttgtgttgtgggggatgctccgtgattaccgcattatagaacgttcagcagcatctctggcctcacccactggatactggtggcacccgtctcccctacttgtgaccaccgaaaatgtctccaggcactgccaaatgttcctggaggcaaaatcactcacaaataggaaataatgacctaattagtaacttacattagcaattcattcaacaatatgtgttgagcatctactgtttgccagaccatacagcagggatgtagtgatatttaagacaaacaaggtccctgacctcatggagactttttcctttttggacctcagtcttctccgctgtaatgtgggtatcacaaggctgcggacctcctaaatttgttgggaagatgaagttagacttgcaagtgcctggcccctggcatgagggattagccaatgccaggggtatgatgggcctagggatggaacctgggagcttggggagaagcgagtgtgggcagggacagtgcatggagaagccaggaaacctgagctgcaagggaggcggaaaggggccatgaaaggccctggtgcaaagtgtgcggcagcagcaaggcaggggaaaggggctgcagggagggccaagggtagcaggaagatgggaccaaaactggagagaaggagagagacagtgggacatagaggatgacaggaaggggtggagatgggaggagagaggcacagatggagaagataaaaaaccagacagacagacatgtacacacgtgataagacagagagaccaaggggcggagggaaaatgagtccaggcggaagggaacacctctgaggaagatcactgcacaaaccctggtcagctgcacatgaccccaaagagtggctcttaggtttattccaaacgtacctgatttgggtgataaagagttaaaattaaatacaaaggccaatgccagtccattcctggcgccagctcctgcctcttccttctcatggggccctcaccagagtgatggggtggagcatacccaaccctgggaggaaatgaggcttttgtgccgagcggcaatatgatggcaatactggcagtggtagtcaacccatctgtaaacagctgacagagggcagtacaagaatccacctcacagccagggccgcaaccgcaagtaaagcacacagctgaaatgactgacgtgggtggaactgagctgagaaggaacgtggctcggcttgaccctggagcacacatcacaaccatgagaaacaggcaactaaagtgacctccagcccacagcaacaaccttctctggctacaactgggaggcagggacagaccccagaaaaccatcttgggtcatctaaggtacgtgtaaccatatttttaaaatgacaaaatctcaagcatgttgctttggtgagcttctgattttactagaaatacactctaagaacagtcgagacgccgcgccttgtggaggcgatgggtcatgttactggttctgcgatgatcttccagagctcctcttctccaccgacagtatggctgtgcaggcatttttcaatctgtgggcgagtcgggagagcgttttaaacacagcatcagtcaagtcgtcgtcgtaaaacacttcggctgcaaacaggatggtggtgtgatcgtacaagtcagaaatttcctcttgtgaccaactgaaggggaccttgggatctgtgcagaggtcgtccttcagccagtccagttctttgaccctaactataccacctgtgagtgagtcctggccgtgctggatgcagggctggaaaggagactgtcaggaggaggcaaggagagcaggccggggctgggccagggaggcctgggaattcaaggagctcagacttcaccccacaggtgatgacgcccctgggaggttttcagcagcaagtgaagtggactggcttgcatctgagaaagggcactctggatgtttcatgaggacatcttggacgggtcaactaaggagctggggagaccagctcaggggccgccgccagtgtccgggagagaaagagctggagtaggatgacgcagtggatctccagtggcagccaggtggctgttgagggcaatgtttcgctggcacatggacaagagatctgcaccgacatctgtacaataaacggtccgtgccatggtggctgcgatgatgctagcgagccccgtgccggccccgagctccagcgctgtacatcctcggaagaggtcctgtcggaacaggatgtagtctgccaggagcagggcgccccgccacacctgcttgccaacatcctccaggggcgtggccatggtgtgctctattctgatgatatcgtgcgggctgccttgtgcttcctctcccaggacgtcgtcttcttcctgtgctagaatcatgggatgtaccttgtctctcagaggccctgctgggttggaatcagaggcggctcgtggtcttctcaccacgtccaaatccccatcctcatccagctgagcttcagccacttcctggccagtggtgtcagtcccggcctggagggagaaaccctcattaccatggccacttcctggaggggaccctgtgctgcctgtctcagcagaaggaggctcctttgtgtgaacatctctgtgactgccacccttggctcctgaatctgtccaagagtcttggctccatagaagcttgaattgggacaggaaaactggctgccccacgctgttcagccgtaccatgagatgtctatggttcggggtatagaggtggacatctgacagcacagtgtcgctcctaaaggtgacctcgtccatggctgccgcaggagccagctgtaccatggcccaggctccaccttagtcctaggacaggagtccctcagaggtgagaatgggtcctcagcatggcaggtcccagaggagatactgcagacaggtccaagctggtagcgagtagctttgcatcgccctgggagaagatctcagagacttggccagggaagagaatccagccgccgcggggcccagcctgggatcccacccgactcccgtctctgtgggacttaggcggccgccataacaggcggtctgcgcaggcgcggccccgcccccgcgtgc

SEQ ID NO: 13140 - RNA, 2062 nt, Homo sapiens
  source 1..2062: mol_type = other RNA
gctgggattacaggcatgagccaccacacccggctaattttttgtatttttagtacagacagggtttctccatgttggtcaggctggtctcgaacccccaacctcaggtgatccgcccccctcggcctcccaaagtgctgggattacaggcatgagccaccacgcctggccaatttaatttattgaattgtaaaaaggtatgttttaaccctatataaatgtatgactatatggagataattattattcacctgaataaaaaacagcaatataaagacacaaataggtaacagtacaatattaaatactataacatctaatccaatattaaaattatatatatacacatagatacaggtagggctgccaacaaatggtcttcatgtctaaaattgtggtaattgttgcagagacttctgtgactatattggaaaccttggaactgtacactgtgtgggggtgaaatttacggcattttaattatatctcaaagttctgttaaaaagtgagtggcttaatattctgtgaagtaaggaatggttttatttaaaacataaattaataatttccagtggattcccttaaaaagattacagcagggatttccagatcacacccacccccacctctagagtttttggctgttttctaaagtcttgaattcaatgaggtgaaggaggaagaaagtgtttaggaagtcagtgggttccagaagagctggtgctgggtggggcagagtggggagagatgctcctttcaaatggaaggctctggaacccgccaaaagggagtgcaagctggggcaatcttcctggacagccaccagagaaaggcttcagaccccacgctcccgctgacatccacagacagggacatctcactggcttttaaaatcatcaactctttttatatcgacacaaagaaataatgaaaaggggaattctggtttacagtcatttcattaaattatccaaaacaacttttgaaacaaaagttataaaagtgaaactcaaaattattctctgcttaataaatactctcagtggctcagatatagttcaggcaaactagccatggatgcagccaaagccagggggtggagggggtcccggcgtgctccaggaggcctctccggtgagtccggcagctgttccctcggcgctgcagccctctctttgctcagctgggggcctctattttgtaaacctcagaataagtcataagccccgtgaagacatccaagatattccttagggttatacctgtatcaggaacaggtttggatgcaggggaaattccaaggatgacgggtatggatcggaaaagacagtgatgtccaagtacaggcggtgcactccacaggtcatctcggacagtcactggaagctaggcaaagtctgtggtctcatggccacaagcccaatgatttgacctcagagggtatccttccacctctaaggagttctcttgtgctcttttactccagtgttggctccaggaccttgggtagagggtgctggtgatatgaggtggtccaggagcaggcccgtaatgctccttcccaaaggaacccagaatcaggtttccgtacactagatccagcaagtttgttcctcaggaagtgagccatttcagggtaaatactcccctctgaggttgatggcatattgccagcatcttcttttttgcagatgtctcctacagcaccctcaggaggagctaggagaacacagagtaagggtcagtgccctggtggtggcaactgtgtcacccagagagctttgcttggtgtggtgcatggaggtagctgatcacagcatgcgccaacctgatgctgggccatgctccaggtggaaggaggagggcaacagagagagcaggagggaactgagacaaggaggcctaggccttgtccttgtcctaaggcatcatgaagcagcacaaaggagtaaacccaaaatggacctaaaatgcacaccaaggttcaacagaagggtcccttcatcactcacatgatttgaaactcttctacacaaacaagactttcttaacgtattcaaga

SEQ ID NO: 13141 - RNA, 6360 nt, Homo sapiens
  source 1..6360: mol_type = other RNA
gctgggattacaggcatgagccaccacacccggctggctatttcttaaaaaagaaaaagaaaaaaaaagtacaaacatgtgcttcacaggagaacaaaatttcgtgaagatgaaacactccctaaataagattgtgtggcagaagaagatgaagaatagaaacatgaacacaatttccaagatggaaaggatctggaagactggtcccatccatatatgttgtctttcttgcatttgaatgataagcattgtgatgcagattgcccagcctgcagattagtgcctagcacaccaaaggcattcaacaatatttattgaacaaacaaatgaatctcctctgcccacaagtttgtacagctgtggagaccacctaccaaaaagtccctagaagcctaagatggttgggcttctttgatacctgttttgatagctgttaacagctgaaaccactaggttaacagcttaaaccactaggttccccagatgaagagattaaatcaacattaatatttggtccatattctaatatccaggtaaatatatagaccatgaactgctggttttgaaagtcctcagactttggtctttttagttctgaactgaaatctcaaaattcaagaaaaaaggcatcagtactcaaaaaatcttatattttatgctatatattagattctgttgttattaaataatgatacatacgaatacctcagtctgttgatatctattgaatctgttgaacctggcaagacctactttaacattaaggactaaatctctaaaattaatcatgcatgtgaccttggacaagccccattcctgtagtggcataatgagaataccggactagatcaatggttctcaaactttgctgcctgttagaatcactttgggagctttaaaaaaatcttgatgtgcaggctgcaccccagaccaatttaatcaggctttctggacacacgaactgggcatcataggttataaatcaccttcaggtgataccaatgaacagcctgcagtgaaaactactggattaggggccctctaaagttccttgctcttctcaaagctgggattctttagttccaaaaaggtgagatgacctctcctggaactagaatttctctccttaatatgtagtctatctttttcaaccaacttggattaaactgcctaagcactccgatatatcacacattcatgcccaaactgctcttcagcaatgctggggcttggaggttctggcttctgataatgcagggtttaaggaactagatttttgctactggtcaaaagctcccacttagtccctgagggtgtatgcaccaggagtatgtgacggaaagtttttctgctcctgtaattttgtcagaccttcagatgggtttgcctaaaggaccaagtagaaaagtgtacatattcaccattctcccttctcctttctcctatacacacgtgctttgaaaacagaaataggcaaagtgctttacctattcagtttccttcccctgctttgcttttctaatgtgaaatcatgtctcctattgccaggagaggagtttcttgaacttgtccatgacaagctggatgattaagttaattaactgttctgaattggtaagggcaagagtattcatacttaacaggctcccacagtactgtgcttagaacgacttgcccatcctccccaatacccctgcccctgcaatgtaagaggttcttacattagtgcatgagagtaggagagcagggtccagaggcttgatttattgacagccatcaaatgccaggtactttgtatcaccttgtttcaacctaggatgctggagctgtccctgttttacaatgaagaaaacctggcctctgagaggccccctgatttgcctaaaggcatacagttggtcaatggaaatgcctagatttgaacccaggtgtaagtgagcaaaatttcactctgctgagcacatcgtgaatgaggaacagataaagcaagaacatggctgggagagagagttcatttctattatctgttcacctacacttaaattaggaagcaggagagtgtacccaaaagctcagagagaggacagccaactaactgtgcagcagttcagaaagaagtttcaggacttcctgaaagacaggagcaggccattcaactccttccctcctttttccttcacattctaactcaacacaaccctaggctcaggaaccagcgcacccctccttccatctacccttttatagtcagtccacaatccttattccaaaaataaatcctcctgatgagatgatgagaggcaacaaaaagcaaagctaaaaagttttatgcttttgttatgggacattatttggacagaattattatcatgtttttacaaatttccctaaaacaaataattctggatatacccaaattactccagcctcctggcccaatatgtttttgcaattacttggcactccaactctatgcaacttaaattagttaacagtcaccaagttatttttaggccatagcaacacacacactctactatacctagcttgttatttgtactccttaggaacaaaatttgcctttgtactggcactatcatttcctttcaatcaatatcaataaaaacattctaccatatttatggagtgcttaccatgtatgtgtataaagttctgaacactttacacacattaattcatttatttcagaaactaacactttgagatagctattgttatatcctctttttgttaatgaggtaactaaggaactgaaggattcagttccttccccaagggcacatacctagttagaggggagccaaggctagcattcaggctgactagatccgaagttctgccttgatttctccatcatttgctacaaggctaatgtttgacattttagccttggatgttaaccagaggctcagaataacaacagcacgtttatgaatgtagatatgtctttatttcaggtattttttaaaatcctcataacatctctgagagaaaaggggagacttttattcccttccccaccccacccccgaaaaaagggcagaaacagaatatttttcacaggtctctgatttctgagcctagccatccactttgtcatagaactctattgccaataagagtatatttcagaattcttttcaactagggaaaagtgtgcaatgtatggtgctcaattctaaggagtgatgaagttttatagtataaaggcctaactgcctgcatgatcaaatcctccccatggatcatccttttaaaccatttccctcttcttctcacattcccccagtaaaggcctttggtacagagcagtcctataaagattgtagcagttggtcattccttgttttacaacagcatagagcaagtagaggcatgggctctgacataccagggaggaagggggacacacagaccccaaggaggcacctggagccctcctactcccagggagggaagctcctctgtagacctgactgccagtcagtcacagagggattcgaagttgaaaagcacttaaaaatgggtacatgacactcaagtgtttacgagtgaaaatgttcatagtatactataaaatatttccagctttattgaatttgaaacattaatttacacattaaacatacttaaatacattaaaacattatctatatttttaaatatttcaacagaaaagagaaagcaaataggaaaaatataattgtttaatctggttgataggtgtatggatgttcattacacacttttctgcttttctatatgcttgaaaatgtttataataacatttttgaaggcatatactgtctttaagaaaaaggggcagtagactatttcttcctacctaagtaaatgacaaattatttccctggacccagctttactgaaaagaaagggagcctgaaaaactttatagcaaaaacggtagctctcgttatggatggtctagaattgttcaactttcttactcagtttgactagaaagcaagttttagttgattaaaaatcagctttgagtaaaacaatataattctttcaaagacctcacaaatccctaaatatttattcatttggatcattttcaccaggttgaagagaagcacaggtctgatgccatttattctttagaagatgagactaaaacatagattctagcataggtcacaacagggagggcactgtaaattagaacagtaacttaatcccaggggctgccatgcctctgatcggtttcttcccaacctgacacagcattactaaaatggcaagttagcagccgctctacttgacagacagcaccaaaaatggagagtatggcatggagacagggggacaaggatcttggacagggagggtagcaaccagtgtttacaaacataaaccagagcatcagatgggccagccataaattacccaagattgtactgaaatctctgaaaataaactaacaagcctttagaagtttcctccttatgttctaactatgcccccctcccaccaacttccctgcaaaaattactccttccgaaatggtaccactaccactcttgctgaaacacaatcttatcaccaagggaggggattactcaaataaatctgagaggagaagccagaccagaatggtctgcttgacccactcaagaatctgagagaagtctgctggtcatgcctttggggaatgcccaccccgtctttcaccacagtggtgctatggtattaatctctggtttaccaagttgaaaggataacgaagggcattctaatattgacccattcctttcccttcttttccatcttggtcccaattttaggccattctcccaaaagataccaaaatgataatgataattataaagtagaatatagaccccttcactcctgaactacatattttcaatgaaattcccagatatttgaagaaaaggcccccaaaactacaaataatctaacctctaccaccagagcatcttccaagtcgactgccgcggtgtctcaccaactcgaaaatgacgaggcctcgcagtggctgcccagggcgcccagtggtgaggtcagcagtgtgtcctgccccgccccattgaggcaatcttactctgacactgaggaagaagtctaggctgtccagaatctcagctgcatccacaggaaagggagagaggatcctcactttcacaagtagcacccaggagattcatttctcaatgactgatgggtcacccctatccacaactccacccactgcaaaatagagagtagggtctgcaactccttgtaatcatccccatgattaggaggtctaggatcatcttgatccgtgttgtttcctctcttcagatcatgaagacacaaaagacttgctttttatcatgaacacctttcaacaccagaggttctttgccttctctcttcagggactcgaggactatgtgaagtggctgggagggcatcactcggcttggttcattggtattctcatcataaactataatttctttggaaaagatcctcttgaaagagtccttgccttccctacaggaaatcaagtctaggacagtgatcttgccctgctgcagtctccgccggctgatcttatcggcacagttaatgtggacagctccttggatgtgactcttgttgtactccatgaagggcctgcagtcaatgatgacagggccctgactcggcaggtgactcttgctgcatttggtcatcttctttgccaagtcattggggtagattattttgatgctggctagctgcttgggggtccctgacacagggctgcccaccccacttgatggacttagagagcctgtattctcattattgttgaccatctggttagcagggcaggtggtagaggttccgatggcagtggtggtggtgccagcggcaatggcttgggtttgggcctgattgtccttgtcgtaggttgccacagtgcagcagctggcactgctgcatccacaattcagcgagcgggcagagccgctggatgagggcatatacgtcagattcgcagccttgagggacacaacggtggtggcgatgacaggagggtggctgttactgcctgggttggcagagccaaggtaactagagtctaaacaaaggttgagatcctgaggtcggacgggcctagatagtgccactactaccctgtcgtctaaaggagacggaggcatgaggaggctgaaaactggcaattcaagaagaactcaagacagtttcataaataagtgtattcctccaccatctggcgctcctcttcagctatggactcgcacattcagcccccattcactcggcttcattgatctccagcagcaacatagttac

SEQ ID NO: 13142 - RNA, 2129 nt, Homo sapiens
  source 1..2129: mol_type = other RNA
gctgggattacaggcatgagccaccacaccctagattcttaagaggattataggatcacatagctcaggtaaagttcaaaattatcaaggtattatatttatttggttattttgagtgttttgtagtgaaaacatctttagcatatctcatattccattttaccacaaaccccaggaagcctaatgattttgtgtttgagtcatctctagttcagctctgatggggaggctgaagaacaaacacaggccaatttaattctatcttgtttgctttctctgggattcagtgtgataggacacctaagtcttgccctcaacaagttcacttttgagggtacagagatggttgttgctagcattttggaggaaggcattgtatgtcacttctgcatataagagctggtttcccctcttggtgcctggatagaaagctgcacaaaaaggctttattatatgctgttctaaattaggagtttaggagataataaagggaaaatcagttacattaaagcctagtaaaggaggctgatcacagagcccttttctgatgttcatcctactctaatccagacacaaatgagagtggcttactttaccaagatgtgattgatttctttggtcaggctgagtctgccatccccatcttctcctgcagtgcttagtgcccctcattctgcttccttcagtgtgttctccctttccaggcatctgaagaagggtgtccactttcggtaagccttgtcataatcactccatgggatgattcttctccagaaatactcttcatgtcaaaaatagtcttccttggtatttctttctccattatccatctttttttcttactctccaacttaaggctctcaaatggtttggaaagtagatgtgctgtggtttgcctgttcgtgagccagctttcattttctccttgatgctccccatctgcagggcagagtccttgcagggcatatcttcatcttcaagcatttcaatcacatcttctatgagggtcaccatatctttactgttgtttggatgttgtaaattcacccaagtcctgacttcttcaggcaggattgccaggaattgttccagcaccaacagttctataatctgcttctttgtatgaatctctggtctcagccattgaagacagagctcccagagttggctcagggcttcatggggcccagacactttcaaatactggaaatgtctgaacttttgacgagatgcctcagagtcatgtgtctccacgacggggttggtttcctgctgccaagacatatctgctctcagaacctctctttgttcacgtagagacaggtttcgaggttttgagatagccatcaacttgctcagaggctgcatcttcctaaatagaactcccacagtagttcaaatccgccttactagattgcagtaattctcaggcttgagctaagcacctgtgtactatatgcagtgtgatttaagccaagttatttcacggtaaggaggaaagttccagaaactttagacacaaagccaatattcaggtacctgagcaatgtaaacagttacagagctaggacagggagagacgttcaggatggcatgctgcatttaggtaagatttccgaggtggaatagttttgatgatagagatccaaggtgtgacgtgactgcaagtagcttaagtggcaaatgatgaacacttggagggcagcgtggaaactgggtaactgcaagcaagctgaggtaagctgcacgttccgcatggacgccctcaagcgtgattcccaattccaagaccccgcgtccccaccgcccgctgacgagaacgatacccgtgagcaccgctcctctccagtggcccgttcagtcactcacaagcgccagttctcagaggagccgcggaatcgctgtcttggacagtgaagggagctggcgttggtaatcacgctgcaactaggaatccctgacctcgccgaaccctcaactcactgccggctccgagtttcataaattgccgcggaacaacctcgacgcactcttgcgcacgcgcaccagctgtggaaggaaccccctaggagcccccgcgacccggatcggtgaggtagaccaggcctttgccagccccgtccctttct

SEQ ID NO: 13143 - RNA, 2049 nt, Homo sapiens
  source 1..2049: mol_type = other RNA
gctgggattacaggcatgagccaccacaccctagattcttaagaggattataggatcacatagctcaggtaaagttcaaaattatcaaggtattatatttatttggttattttgagtgttttgtagtgaaaacatctttagcatatctcatattccattttaccacaaaccccaggaagcctaatgattttgtgtttgagtcatctctagttcagctctgatggggaggctgaagaacaaacacaggccaatttaattctatcttgtttgctttctctgggattcagtgtgataggacacctaagtcttgccctcaacaagttcacttttgagggtacagagatggttgttgctagcattttggaggaaggcattgtatgtcacttctgcatataagagctggtttcccctcttggtgcctggatagaaagctgcacaaaaaggctttattatatgctgttctaaattaggagtttaggagataataaagggaaaatcagttacattaaagcctagtaaaggaggctgatcacagagcccttttctgatgttcatcctactctaatccagacacaaatgagagtggcttactttaccaagatgtgattgatttctttggtcaggctgagtctgccatccccatcttctcctgcagtgcttagtgcccctcattctgcttccttcagtgtgttctccctttccaggcatctgaagaagggtgtccactttcggtaagccttgtcataatcactccatgggatgattcttctccagaaatactcttcatgtcaaaaatagtcttccttggtatttctttctccattatccatctttttttcttactctccaacttaaggctctcaaatggtttggaaagtagatgtgctttacgcaatgaattcaggttcctaaagttttccagcatcacattcctgtacaggttctttacagcagagtccagttgcccccactcttccttgctgaattccacaaccacatctttgaatgtcactggttcctgtggtttgcctgttcgtgagccagctttcattttctccttgatgctccccatctgcagggcagagtccttgcagggcatatcttcatcttcaagcatttcaatcacatcttctatgagggtcaccatatctttactgttgtttggatgttgtaaattcacccaagtcctgacttcttcaggcaggattgccaggaattgttccagcaccaacagttctataatctgcttctttgtatgaatctctggtctcagccattgaagacagagctcccagagttggctcagggcttcatggggcccagacactttcaaatactggaaatgtctgaacttttgacgagatgcctcagagtcatgtgtctccacgacggggttggtttcctgctgccaagacatatctgctctcagaacctctctttgttcacgtagagacaggtttcgaggttttgagatagccatcaacttgctcagaggctgcatcttcctaaatagaactcccacagtagttcaaatccgccttactagattgcagtaattctcaggcttgagctaagcacctgtgtactatatgcagtgtgatttaagccaagttatttcacggtaaggaggaaagttccagaaactttagacacaaagccaatattcaggtacctgagcaatgtaaacagttacagagctaggacagggagagacgttcaggatggcatgctgcatttaggtaagatttccgaggtggaatagttttgatgatagagatccaaggtgtgacgtgactgcaagtagcttaagtggcaaatgatgaacaaagcgccagttctcagaggagccgcggaatcgctgtcttggacagtgaagggagctggcgttggtaatcacgctgcaactaggaatccctgacctcgccgaaccctcaactcactgccggctccgagtttcataaattgccgcggaacaacctcgacgcactcttgcgcacgcgcaccagctgtggaaggaaccccctaggagcccccgcgacccggatcggt

SEQ ID NO: 13144 - RNA, 788 nt, Homo sapiens
  source 1..788: mol_type = other RNA
gctgggattacaggcatgagccaccacaccgggccccagggttattttatgtgacaaactccaccacgtgactctcctgaacccttctgggcagccctcactgtaacatcacagaagatggacatgacctccaaagccccctcggtcaggttcctgcctcgccccctccagggccccgcacccaccctggtctggcagcactccaaaagtgctctgagcctttgcactggctatctatcctcctcagattatccttccccacctgctctgcctggcaaacacctctccttcatctctcgacacttccttgagcatcgtggtttgagggtcttttcaagagcagcttctttcttccttcctctgggtcctgctgtgtccaccacatacatctgtcacaggacaccttacagcttttctgtgttcactgtccacctccttctgtctagatctgatggttgtgaagttctggataacataatctagcctgttcttttctcatacttgttcggtggcactggtttgctggtgtcttgagcatctatgaaacagtctcgcagaggcctggctgtgtgcactgggatgacaggtcctgaggaacacggatggtggtggtgagagaggaggaggcagcatgaatctcaagccgctttctgacttgggcagctggctgggtgggagtctctttcacagaggcaggaaacacaggaggcaagccagggttggggtggaaacatgtaatcagcgtcctagggctgccatgacaaagccccacagactggcagcttaga

SEQ ID NO: 13145 - RNA, 9806 nt, Homo sapiens
  source 1..9806: mol_type = other RNA
gctgggattacaggcatgagccaccacacctagatatacctcgcttctcagagatttcctggggctgggagtcctatgaatgagagatgagaagcagaacttctgtaaatggtgacatggcttcatgtgtttctatacacgattcctagagcaggtgagggaatcaagatcgaatagagccttcaaagggatttatagggtaactgagcctaagaaccaaaaggggaaggttgcctcagaattctccttttttaacttccattggctttactgctatctctacaggattgcggatacacaaagatatggccttctaggacttaaggctcgggcatttctgggagcaacaggcaggagggaacccctctgccctatagaagacagaattttagcttttatctaaaagattctcttgaccctcaacctcaactctgttcctcttctccacatccatctcccttttctctacccactcatgtccaggtggcagcctacatccctcagctggccaagtcaaacccagacctgtggggtgtctccctgtgcactgtggatggtcaacggtgagatgctgggcaagaggaaggggaggcagggcacaggtgccgaacacaggccaacccctttcatggcatctgtctgcctccaggcactctgtgggccacacaaagatccccttctgcctgcagtcctgtgtgaagcccctcacctatgccatctccataagcaccctaggcactgactacgtgcacaagtttgtgggcaaagagccaagtggcctgcgctacaacaagctctccctcaatgaggaaggtgagcactaccaaggctcagaccgtacttacagctgtccccttctccttatccccaccccatctcccagccttttttgtttctctgcccttcctgattagccctgtcatgcctttctccctagcagtctttcttgtctaacccacaaagtgagcgggctgtcagggaggctttgttcagtggctaagactcttggtggtttgtatttccccaggaatcccccataaccccatggtcaatgctggtgccattgttgtcagctccctgatcaaggtcagtgccaccttaaccttctgataggtattatcctctaagctcctgtgttcctgtatccctcatatttgttcagctctccagggagactggtggggctctgattcctttgagggtccccagaaggcacatgaggcacagcagggacccacatgttatgctgacaatgtcagtataagagactgcaccacctccgtcatccccactcagtactgttccctgcccccacccatgagtctagagcctagagctttctgacccttagagaagtgagcaggtcctgacccctgcctaggaccaagggccaaatgccagagacaaggggaggacagcactattgggcactgattggccacttctgggtgtgggacacctgcaggcaagggtgaatggccaggccagggcagttattcacgtcacctggaactgtgagttggccttgaacagggtgtcagactagcccatcagctgtaggtctcccagggcttgagcaagaacctgggagcagctgggcagcaacaccctggagccaatcacagcccctcctggggaaggtggtgttaggaatcctcccctcagggactcaggtatcagagtccctgtggtattgactctgtagttgacacatgagtaagcaatgagtctgggtgaggaaaagaggctgagtctctccccttgttctgtgatggctccatctacaaacctgtatctgggacctgcctcatcccattcccatctaagtaggaccttttttaaaaaatatagaggccaggcgcggtggctcacgcctgtaatcccaacactttgggaggccgaggtgggcaaatcacgaggtcaggagatcgagaccatcctggctagcacggtgaaaccccgtctctactaaaaatacaaaaaattagccaggcttggtggtgggcacctgtggtcccagctgctcgggaggctaaggcaggagaatggtatgaacccgggaggcggagcttgcagttgagccgagatcctgccactgcactccagcctgggcgacagagcaagactccatctcaaaaaaaaaaaaaaaaaaaaattgaggcagggtctctcctatgttgcctaggctggtctcaaacccctggtctcaagcgatcctcctgcctcagccccccaaattgctgagattacaggcatgaaccatcatgctggccaatgggatggagtaaagctccagcatggggtgtaaggaatggggatggagatcagggatagggtggggctaggagacaggattcgagtcaggaaaatgaacgtgggagtcagggatgagggtttggattgagaatggaagtgggatggcccagcaagctggctcatgcctgtaatccgagctacttggaggctgaagtgggaggatcgcttgagcctgggaggtcaaagctgcagtgagccatgatcgtgccactgcactccagcctgggtgacaagggtgacaaagcaagactgtctcaaaaaaaagaaagagaaagagaggagccaatggaagtgcggtgttttcagaaggataaaaaaagggccattataaaattgaacacatttgcagcagcaggaccagactaacactagaactccactagatccttctgacccttccctctgtcatcctcctacacttagaatgctgacatctctctctttctctgcagatggactgtaacaaagcagagaagtttgattttgtaagttcccttgctacttagcccctggctgcatttcgccatggcatgctgtcctctccagctgccccagtggctctctaaccccactaccaggtgcaccagcccatactagaagccttatttccagaaatgtggaaatctgctggcctcagagaggaaagcctcttgacaagacctgagttcagaagggctagtcaacctgtgaggtattaatagagcttcttaaccaagtggagcctcaatgtccctttttctcttccaggtgttgcagtatctcaacaaaatggctgggaatgaatacatgggtttcagcaatgccacgtaagtccctactcagaggactgactgaaagcattgtggtgtatgtgtgtgtacttaggatggggacaagaggaatgggggagagagaatcttaggaggaagaaatcccaggggaactttggccctccagcttcctctgagtcccttcataaacatttgtttatcttgtaaaataatttgttccatttctaattagtacataatgagagaggcagtgtgatggtttgtgcctaagccctttcttgccaagactttcaaagccaaaaacttcaccagttttcctagatgactagacagtttggggtgtttggtttgggtttactttataacaaaactatgctgagtgtttgctcaggttcagaaatttcctctaatattactgtgagaagttataaaggggttcatttagtttgtggtgtgatgtagttctgtctctccagggaaggtaatttttccccttctcccaacacccactcctccaacttcaagtactaaattgggtgtttgcttcagattccagtcagagaaggaaacaggggatcggaattatgccatcggctattatctcaaggaaaagaaggtaaccagaagaggccggaagagaaagtccctgggaattctgctgctagtggaagggcagtaggggttgggggcttcagctgagaccctgacagtgtgaaagggctgatgtcctgaagagaaatgctctcccctctcttccttgcagtgctttcctaagggggtggacatgatggctgcccttgatctctacttccaggtaagaaaacactgctcagggccgagggaacaggacagactgtccttgcccttgccctttccctacacccgagggtcccatgtgcaggttcacgtcacatcttcacctattctttgttttcatagctgtgttctgtggaggtcacttgtgaatcaggcagtgtcatggcagccaccctcgccaacggtgggatctgccccatcacaggcgagagtgtgctgagtgctgaagcagtgcgcaacaccctcagcctcatgcattcctgcggcatgtatgacttctctggccagtttgccttccacgtgagtttctggctctgctatccatctgtcatgagcccagtgctaagaagagagaacactgactctctcaagatagaggtggaagcttgttcctgcctctcattcactaacttccaggaaggcaattaggttgagactccttagacgagtttctcaaaaacaccaagttcctcgaatatataaagagatgtctttgggaggccgaggcaggtggatcacctgaggtcaggagttcgagaccagcctgacctacatggtgaaaccccatctctactaaatacaaaaaattagccgggggtggtggtgtgcacctgtaatcccagctacttgggaggctgaggcagaagtgcttgaacctgggaggcagaggttgcactgagccgagattgtgccattgcactgtagcctgggcaacaagagcaaaactccatctcaaaaaaaaagaaaaaaagaaaaagaaaaacaaccagaggtgttgcagctcctgaattgtgcttcacattgctggctcttctccttggggtctcagcttagatgtcatttccaaagaaagacttttctgaccaccctatctcatgtggcccccctctacctctatttacagcaccctacttctcactatttatcacaattactttaaacattacgtgtctatttatttacctgtttattacctatctcctaacaccagaatggaagttcctagttctagcacagcatctagcacagaatgctgtaagtatttcaaaaaatattttctagctgaatcaatgaatttaagggaaggaaaggacaggagtaataaaagaagctaattaacaagccaaaaggttgaggtggattgtggtcatgcagtcatttgtaaacttgttaagagtacagcctaacttgtttattttctgatttggggcacacccactttatcctcagcttcagttctgttccccaggtgggcctgccagccaagtcagctgtatcaggagccatcctcctggtggtacccaatgtcatgggaatgatgtgcctgtcacccccattggacaagctggggaacagccatagggggaccagcttctgccaggtgagatgctttgcatatagtacttactatttttgaagcaataaatttgtttaatggtaccacttttactataataaagcaattttgagctcctactaagtgtaaggagtaaataaacaatatatttggcttacaattctagaagttggtgtctctcttcaatttccacaactatgacaacctgaggcactgtgctcggaagttagacccacggcgtgaaggggcagaaattcgggtaaggaaaactccaggtggcttgtaagaatatttcaaaggccaggtgcggtggctcacgcctgtaatccctgcactttgagaggccaaggcgggcggatcacaaggtcaggagatcaagaccatcctggctaacacggtgaaacctggtctctattgaaaatacaaaaaattagccagacgtggtggcacgcgcctgtggtcccagctacttgggaggctgaggcaggagaatcgcttgaaaccgggaggcagaggttgcagtgagccaagaccgcgcgccactacacttcagcctgaacgacagagcgagactccgtctcaaaaaaaaaaaaaaaaaaaagaatatttcagagtagcacattccataacacttcagcaatacccttggactaagcatccatggaggagggtcacagggcacagctggcataggtgagttcaattaatgtcatgtgggtatgatttgtgttccagaacaagactgtggtcaacctgttatttgctgcctatagtggcgatgtctcagctcttcgaaggtaatgctactgtgaccaaatatacacaataaaatactcctggtcagagattttactaggaggcagcgtaacaaaatagttaagtgcttcagctttggaattagaatggatatagattgcatttaaatgaaatttttttaaaaaaggagattttttttaaaaaaagtaaactgtctgctctatgataattaatgttagccattgttattgagtgttaagagcagtgtcctaggaagtaggtaccctgcctcaaatgggcacttaccacaggtaggcagtgagtgatatttctggaaggatcacattcccatctctctaatatgagtataacagtctcatctggatatggaaaaaagattattcagagccaacaaatctggctataggctgtttcactttctctgaaactcatccagtctgacaccagttcacaaagaacacctgtgattccagtctgatctaggcaactctagctgctttcccactaccctcaggtttgccttgtcagccatggatatggaacagaaagactatgactcgcgcacagctctgcatgttgctgcagctgaaggtactgaagggttaaggaggggaggaggagggtaatcataagaccctttctttttcaccaaaagtaccttcattatatgtgccctcaaggttataggggcagcaactagttttatctagacacccttcggtttgcagctagactatgactgagtgctgcagggtacaaaatgggaagaggccttttcccctcccctcttggtaaagacttcagtggctaagtgtctgcaccaaagggttcaagacctgcgccttctcattttccttctgcccatattcctaggacacatcgaagttgttaaattcctgatcgaggcttgcaaagtgaatccttttgccaaggacaggtgaggaataggctaaaagtggaggagggtgggcacagcttctccacctaccctccagccaccatgcaaatatatacaaccaccactctccacgtctcctttgcctgatcatatcattattcctctcaggtggggcaacattcccctggatgatgctgtgcagttcaaccatctggaggtggtcaaactgcttcaagattaccaggactcctacacactctctgaaactcaggctgaggcagcagctgaggccctgtccaaagagaacttagaaagcatggtatgagcacaggtcatggacagcccctgctcaagaaaaagcatgagctggccacacatgtaatccataaccaccaaaaatactatggagagctacactgcttcagtggggaccaagcagtcatttggtgacttaggctagtgctttctatgggagtcaaaataccccattccctcagcagacagagtacagagaagggcctcagaggacacctgcagtacagctatccagagagactgggcttcaaggtacagcctaatggcttgccccactcaaaaccatcccagctcttcacccaggtctcctcttcctctccctgaagaaaccatcatgagagagatactctggtggagggactctagctaccatgcacatgtacatatccacagaatatgggaagtgggaatggctatatacatggctttagtagtctggagaaatctactccccttggccaggacatgctgctgctactgctaacagccaattttatagacagagaaagtattttgtgttcaaataaactttaattaccaaatcatttttgctaaacccagtccttctttcttccctaggggtatctagcttcatcaccatcatagaaggtagaaaaagatggaatcacagggtcaaagcacagcttctctacctaccctaccaaacagtacatattcacttaccccaccaggtttttctcaactccaaatactgctttaggttaagtgtattctgctgccaagggaagcataggtttgagtctaaacaggctctgaaacagattgtgcaaaacctcaggcctccttccttcctcgggaagttccaactgtggcagaaatgaagatggaacttctcaagaataaacagttttggccgggtgtggtggctcacgcctgaaatcccagcactttgggaggccaaggtgggctgatcacatgaggccaggagttcgagaccagcctggccaatatggcaaaaccccatctctactaaaaatataaaaatgagacgggcatggtggcacacacctgtaatcctagctactcaggaggctgaggcacgagagtcgcttgaacccaaaaggcagagtttgcagtgagccaagatcatgccactgcactccagcctgggtgacagagtgagactctgtctcaaaaataaataaatagtttctagcactcatcccctagatatcccccaagtgtctctcttcccctttggtcaaggttataactgggataatgattatgacagactggctgggtgtcagaggtacagatttaaggtagatggactcagggtaaggatagctacagctgtgtggggctgaaggtctgtggcactgagctactggggaaggagggctctgttttcattttgacacactgagttaataaagcacttactgagggagccagagcccaaactctaaatgtgctgtagaaaaagggccaagtcattgactgcaccactccttcagccagaggtagaaaggatttactcttcagccatctggtagagccccaagaacaagttacatgtggacaaagggagggagaggtatcatggtgattaataaattcaaacaaagctgaatgataagaccccaggatggaatacagtctgagaaaggcctgggcaaagggaggcagagggactgaaggaagcaggtcaaggaagatacacccatggtagcctaggaaattggcagtagttggtgggtggggaaaaggagggtttggctgtatgcctagctttcacaaggtaggggatgaggaagatgatcatgatattgcacagaggacccaacactgaattgtgggagctagaggttgcttgaggcaaagtaaaaaggcttcggacactttcaaaaggaggctggccaaaggcgtgattagggactccagtaatggacatactagaggccctcgggcacctcaagccctgaatgggtcagcagctccccatcccagagagcaaaggcaggcaccactggaccccggaaatctgtctgtagcgtgtgaaccacagagacctggctcacatccaccaggctcagcttctgggcctcatactccagcaacagccccaccttctctggctgcccaataccctcaactggggctttctcgttggccaacatggtgtaccacttgcgctgggcataggtgaacacccaggaacgatcatcaacaccaatgcagctatcccgggacatgtccacatctgccactcctatccggaactgctgggagcgcttcactgtcacttcccagtagtgtctgccactggtgaccgctgtgtctgccagcaccactgcccactcccggaagcgctccacattcaaggccaccttggtgggctccaatcccaccaagccatatttgacacccgtatcatctctgaagagtgccaggctgctgtgggcggttttttcttccagtttgaaactgacgcctctctgggcctctgtggaggcaactcccaatcgtttggctccccagcggcacaagcgcaaagaacgtgcaaaaagcagcgccatcttgcgccttggat

SEQ ID NO: 13146 - RNA, 3632 nt, Homo sapiens
  source 1..3632: mol_type = other RNA
gctgggattacaggcatgagccaccacacctagcttgtttattcttttaaaactgcctattttgccatgaaataggtacccttgctgtgaaagcctgtgaacacccctggatgtgtgtaccttcatttaaaaactgccttagagggcatgaaatgtcatcagggaagatctattccgagctgggtgtgagctctagccctctccctgaccatcggtttgctctggggtatgaggttctgagtgtgaggcgcccactggggcctggcgtcagggccgacttgcttctcttaggctctgcgttcaggggctacctcttccaaagactacacagctgcaggcccagcctcagagcagaggtgatatgggtattaccaggctctaatggaaagtgtgctctctcgatatctacttgcagggaagcttctgaaattggtaagggagcacctattgcaaggctcagtgaacaaatggttttggtatttccctttttcatggggcaccagaagggtattttctcctacacaggatcgcatctgaagactttgctgaactgtgttttcctgaagtgaggagatgaaagacctcagataggaaaaacagagagtgagagagagagacagacactgagccaggttcccacacagtttattgagggagccaaagccagtgagaggacgaaggagtcctacttcaacctacttccttaaagctgtgtgcctccagcatgaagggaccttcccagagggcagggcctgccctataaggggccacatgaagccttgtggagactcctgcctctcataccacagcctgtcctaccctaaagacccagacatgacagcagacataatccccaccccaggagggtgctgaggaaacacccttacccatgcccctcccctagagacctcaggaagaaaggccaggacacctgtcctgtgattggccagttgaatcctcaacgtgaagacctggcaggcctggctgacaggtctgttcagatgtggcctcaggcatctactctaggatccaacccctaacattcaaacatgattaaaaacacccaggacacttctcttgctggcagaggccacaccccagataatggcagtcctgccaaactctggccagagatagggacccaagctgactgggtgtgagcacgtaaggagaccactctgccccatggggagaatcttccagggctcagctgaggctcagagcccaggcttatgttattccccatcaaatgccagtgattcctccaaacattccccacaagggagaaagggaggaggaggcagagagcttatcaagaggttcaccctatatggggctggaggttggatctactggggtgaggaaaagggtgtagaggattggggcactggggcaggggcgctggcacattcctcagattctggcatgtcatcctggaagtactcagcctggcggtactgccacagacgcaggttcccgtcccacgaactgctgacaatcttctcttcaaaggggtgccaactgacgtcacgcacacaggccttgtggttggtcagcttcttcacaatgtggccacttagaaggtcgtacacaaccactttgccagtggagcagccactgtagatgaactgctggccagtgctatgaatgggggagaaccggcagcggatgagggtgtgcagcactccgtggccccggtaggtcatcaaggagctgtcccctgggagcttcagcttccgccaggcttttttgggcacttgctgccaccgatagtcccagttttgctgtgtggcagcctggcgtgaagcttccatgccttcccggctggaaaagcgtcggatatcccagagtttgatggtctggtctttagagttggagatcagataccgggcatcacccttgctgtcaatgaaggtgatgccatcctggtgtccagccagtgcacccacaggcttggggtcatcctcccgcatggtgcgtcgatcccacactttgcagatggcatcatctcccccagagaacaggatttgggagcttatatcagcaaaggccactgcattcacatcatcctcatgggactcaatctgaagggtgcgccggttctgttctcggtcaaagacatacaggcagccatcattggcccctcctagtacttctcgtccatctgaggagacagcaatggagaagacagcaaagcgacgctcatctggcctgagatccagggcagtgtgtgtatctccctcaccatagatattgcagatatgaatgtaatcagaccagctagagtagaggaagtggttcccatcaggggtgaaggccacatccaagacgctccagcctacgtcgcgggccttgatgctcttgaatttacggaaacggccatatcggcagtcatagagtcggattgtctggtcttggcaagcagacatgaatatttgaccatctttgctgtagatgccacagaaagccttctgagagtagctatcagtgaagcccagatcattgggcaagaagctggtgcaacattcgaggaaagctgtgcttctgggcggcccgcctaagccccagctgccctgtggccagttccacttgtgtcttgatctcattgaattccagctcccgggtgtcaggggtagcatccacaggtgggttgtatcgatccccaagacgaccatcccaagctctgtcattctcttcctctgagtccaagagggcctgaatgaattgtaaatttgctgcacctcctccctgcaccaacctcacttggcctctgggccagatccacatcttcatcctcttcttcctcttcctcactccgacgcaggccagcccctcttcggggcaagccctcggaggggtctccggacccggatcctgcactgctgctgttccgcgatcccatcttctggtcacagcattcttaggtcctgtgcgggggctcctcctgtcacctccttgggtttggtgaaagcaaagcgtgctctagaaataccagggtctcctgagacggggtagtagctatctctaggagggtgacccttcctcggggctgagatcccttttctttagcctatgccaactaccaaggcgtcgggaacacaaaccttctccaatcctatcgaagtccccggactggggagcgggaggggtgttgggcggtgttggatttccaggtaacctctctgaccgaccaatcgaaatccctctcggaagaaagcgcttcactagcttatctcatctaaccaattagaagccttaggactcaaagaccctcgacgcccccaccttatcgaccaatcagagcgcccccttacaaaggccggcagcagtgacagccaatgaaaatagaatttggcctaacacccctccttcctcgcctcacgcccacgtggtgcgccgggggtgtgtacgccatgagggggaggaagccgagaagcacctcccactgaagccggcggtaaccgccccacgcgagaccacccaccagccaggagcggtcgcaggacccgcagcggcgcgaggccttgtttacaccgactgccgccactgcgttggccaaccgctcctccgtcacgcgcttcgctcgtcacgcatctcgcggcttcctggccggcgggctgcaaacgtcacac

SEQ ID NO: 13147 - RNA, 3190 nt, Homo sapiens
  source 1..3190: mol_type = other RNA
gctgggattacaggcatgagccaccacacctagcttgtttattcttttaaaactgcctattttgccatgaaataggtacccttgctgtgaaagcctgtgaacacccctggatgtgtgtaccttcatttaaaaactgccttagagggcatgaaatgtcatcagggaagatctattccgagctgggtgtgagctctagccctctccctgaccatcggtttgctctggggtatgaggttctgagtgtgaggcgcccactggggcctggcgtcagggccgacttgcttctcttaggctctgcgttcaggggctacctcttccaaagactacacagctgcaggcccagcctcagagcagaggtgatatgggtattaccaggctctaatggaaagtgtgctctctcgatatctacttgcagggaagcttctgaaattggtaagggagcacctattgcaaggctcagtgaacaaatggttttggtatttccctttttcatggggcaccagaagggtattttctcctacacaggatcgcatctgaagactttgctgaactgtgttttcctgaagtgaggagatgaaagacctcagataggaaaaacagagagtgagagagagagacagacactgagccaggttcccacacagtttattgagggagccaaagccagtgagaggacgaaggagtcctacttcaacctacttccttaaagctgtgtgcctccagcatgaagggaccttcccagagggcagggcctgccctataaggggccacatgaagccttgtggagactcctgcctctcataccacagcctgtcctaccctaaagacccagacatgacagcagacataatccccaccccaggagggtgctgaggaaacacccttacccatgcccctcccctagagacctcaggaagaaaggccaggacacctgtcctgtgattggccagttgaatcctcaacgtgaagacctggcaggcctggctgacaggtctgttcagatgtggcctcaggcatctactctaggatccaacccctaacattcaaacatgattaaaaacacccaggacacttctcttgctggcagaggccacaccccagataatggcagtcctgccaaactctggccagagatagggacccaagctgactgggtgtgagcacgtaaggagaccactctgccccatggggagaatcttccagggctcagctgaggctcagagcccaggcttatgttattccccatcaaatgccagtgattcctccaaacattccccacaagggagaaagggaggaggaggcagagagcttatcaagaggttcaccctatatggggctggaggttggatctactggggtgaggaaaagggtgtagaggattggggcactggggcaggggcgctggcacattcctcagattctggcatgtcatcctggaagtactcagcctggcggtactgccacagacgcaggttcccgtcccacgaactgctgacaatcttctcttcaaaggggtgccaactgacgtcacgcacacaggccttgtggttggtcagcttcttcacaatgtggccacttagaaggtcgtacacaaccactttgccagtggagcagccactgtagatgaactgctggccagtgctatgaatgggggagaaccggcagcggatgagggtgtgcagcactccgtggccccggtaggtcatcaaggagctgtcccctgggagcttcagcttccgccaggcttttttgggcacttgctgccaccgatagtcccagttttgctgtgtggcagcctggcgtgaagcttccatgccttcccggctggaaaagcgtcggatatcccagagtttgatggtctggtctttagagttggagatcagataccgggcatcacccttgctgtcaatgaaggtgatgccatcctggtgtccagccagtgcacccacaggcttggggtcatcctcccgcatggtgcgtcgatcccacactttgcagatggcatcatctcccccagagaacaggatttgggagcttatatcagcaaaggccactgcattcacatcatcctcatgggactcaatctgaagggtgcgccggttctgttctcggtcaaagacatacaggcagccatcattggcccctcctagtacttctcgtccatctgaggagacagcaatggagaagacagcaaagcgacgctcatctggcctgagatccagggcagtgtgtgtatctccctcaccatagatattgcagatatgaatgtaatcagaccagctagagtagaggaagtggttcccatcaggggtgaaggccacatccaagacgctccagcctacgtcgcgggccttgatgctcttgaatttacggaaacggccatatcggcagtcatagagtcggattgtctggtcttggcaagcagacatgaatatttgaccatctttgctgtagatgccacagaaagccttctgagagtagctatcagtgaagcccagatcattgggcaagaagtgagatatcactcgagactgttctccaagggagaagcttccccgatggcagaggccccgttctctctggtgcaacattcgaggaaagctgtgcttctgggcggcccgcctaagccccagctgccctgtggccagttccacttgtgtcttgatctcattgaattccagctcccgggtgtcaggggtagcatccacaggtgggttgtatcgatccccaagacgaccatcccaagctctgtcattctcttcctctgagtccaagagggcctgaatgaattgtaaatttgctgcacctcctccctgcaccaacctcacttggcctctgcggaggagataggccagtacctgggccagatccacatcttcatcctcttcttcctcttcctcactccgacgcaggccagcccctcttcggggcaagccctcggaggggtctccggacccggatcctgcactgctgctgttccgcgatcccatcttctggtcacagcattcttaggtcctgtgcgggggctcctcctgtcacctccagccaggagcggtcgcaggacccgcagcggcgcgaggccttgtttacaccgactgccgccactgcgttggccaaccgctcctccgtcacgcgcttcgctcgtcacgcatctcgcggcttcctggccggcgggctgcaaacgtcacac

SEQ ID NO: 13148 - RNA, 3720 nt, Homo sapiens
  source 1..3720: mol_type = other RNA
gctgggattacaggcatgagccaccacacctagcttgtttattcttttaaaactgcctattttgccatgaaataggtacccttgctgtgaaagcctgtgaacacccctggatgtgtgtaccttcatttaaaaactgccttagagggcatgaaatgtcatcagggaagatctattccgagctgggtgtgagctctagccctctccctgaccatcggtttgctctggggtatgaggttctgagtgtgaggcgcccactggggcctggcgtcagggccgacttgcttctcttaggctctgcgttcaggggctacctcttccaaagactacacagctgcaggcccagcctcagagcagaggtgatatgggtattaccaggctctaatggaaagtgtgctctctcgatatctacttgcagggaagcttctgaaattggtaagggagcacctattgcaaggctcagtgaacaaatggttttggtatttccctttttcatggggcaccagaagggtattttctcctacacaggatcgcatctgaagactttgctgaactgtgttttcctgaagtgaggagatgaaagacctcagataggaaaaacagagagtgagagagagagacagacactgagccaggttcccacacagtttattgagggagccaaagccagtgagaggacgaaggagtcctacttcaacctacttccttaaagctgtgtgcctccagcatgaagggaccttcccagagggcagggcctgccctataaggggccacatgaagccttgtggagactcctgcctctcataccacagcctgtcctaccctaaagacccagacatgacagcagacataatccccaccccaggagggtgctgaggaaacacccttacccatgcccctcccctagagacctcaggaagaaaggccaggacacctgtcctgtgattggccagttgaatcctcaacgtgaagacctggcaggcctggctgacaggtctgttcagatgtggcctcaggcatctactctaggatccaacccctaacattcaaacatgattaaaaacacccaggacacttctcttgctggcagaggccacaccccagataatggcagtcctgccaaactctggccagagatagggacccaagctgactgggtgtgagcacgtaaggagaccactctgccccatggggagaatcttccagggctcagctgaggctcagagcccaggcttatgttattccccatcaaatgccagtgattcctccaaacattccccacaagggagaaagggaggaggaggcagagagcttatcaagaggttcaccctatatggggctggaggttggatctactggggtgaggaaaagggtgtagaggattggggcactggggcaggggcgctggcacattcctcagattctggcatgtcatcctggaagtactcagcctggcggtactgccacagacgcaggttcccgtcccacgaactgctgacaatcttctcttcaaaggggtgccaactgacgtcacgcacacaggccttgtggttggtcagcttcttcacaatgtggccacttagaaggtcgtacacaaccactttgccagtggagcagccactgtagatgaactgctggccagtgctatgaatgggggagaaccggcagcggatgagggtgtgcagcactccgtggccccggtaggtcatcaaggagctgtcccctgggagcttcagcttccgccaggcttttttgggcacttgctgccaccgatagtcccagttttgctgtgtggcagcctggcgtgaagcttccatgccttcccggctggaaaagcgtcggatatcccagagtttgatggtctggtctttagagttggagatcagataccgggcatcacccttgctgtcaatgaaggtgatgccatcctggtgtccagccagtgcacccacaggcttggggtcatcctcccgcatggtgcgtcgatcccacactttgcagatggcatcatctcccccagagaacaggatttgggagcttatatcagcaaaggccactgcattcacatcatcctcatgggactcaatctgaagggtgcgccggttctgttctcggtcaaagacatacaggcagccatcattggcccctcctagtacttctcgtccatctgaggagacagcaatggagaagacagcaaagcgacgctcatctggcctgagatccagggcagtgtgtgtatctccctcaccatagatattgcagatatgaatgtaatcagaccagctagagtagaggaagtggttcccatcaggggtgaaggccacatccaagacgctccagcctacgtcgcgggccttgatgctcttgaatttacggaaacggccatatcggcagtcatagagtcggattgtctggtcttggcaagcagacatgaatatttgaccatctttgctgtagatgccacagaaagccttctgagagtagctatcagtgaagcccagatcattgggcaagaagtgagatatcactcgagactgttctccaagggagaagcttccccgatggcagaggccccgttctctctggtgcaacattcgaggaaagctgtgcttctgggcggcccgcctaagccccagctgccctgtggccagttccacttgtgtcttgatctcattgaattccagctcccgggtgtcaggggtagcatccacaggtgggttgtatcgatccccaagacgaccatcccaagctctgtcattctcttcctctgagtccaagagggcctgaatgaattgtaaatttgctgcacctcctccctgcaccaacctcacttggcctctgcggaggagataggccagtacctgggccagatccacatcttcatcctcttcttcctcttcctcactccgacgcaggccagcccctcttcggggcaagccctcggaggggtctccggacccggatcctgcactgctgctgttccgcgatcccatcttctggtcacagcattcttaggtcctgtgcgggggctcctcctgtcacctccttgggtttggtgaaagcaaagcgtgctctagaaataccagggtctcctgagacggggtagtagctatctctaggagggtgacccttcctcggggctgagatcccttttctttagcctatgccaactaccaaggcgtcgggaacacaaaccttctccaatcctatcgaagtccccggactggggagcgggaggggtgttgggcggtgttggatttccaggtaacctctctgaccgaccaatcgaaatccctctcggaagaaagcgcttcactagcttatctcatctaaccaattagaagccttaggactcaaagaccctcgacgcccccaccttatcgaccaatcagagcgcccccttacaaaggccggcagcagtgacagccaatgaaaatagaatttggcctaacacccctccttcctcgcctcacgcccacgtggtgcgccgggggtgtgtacgccatgagggggaggaagccgagaagcacctcccactgaagccggcggtaaccgccccacgcgagaccacccaccagccaggagcggtcgcaggacccgcagcggcgcgaggccttgtttacaccgactgccgccactgcgttggccaaccgctcctccgtcacgcgcttcgctcgtcacgcatctcgcggcttcctggccggcgggctgcaaacgtcacac

SEQ ID NO: 13149 - RNA, 3247 nt, Homo sapiens
  source 1..3247: mol_type = other RNA
gctgggattacaggcatgagccaccacacctagcttgtttattcttttaaaactgcctattttgccatgaaataggtacccttgctgtgaaagcctgtgaacacccctggatgtgtgtaccttcatttaaaaactgccttagagggcatgaaatgtcatcagggaagatctattccgagctgggtgtgagctctagccctctccctgaccatcggtttgctctggggtatgaggttctgagtgtgaggcgcccactggggcctggcgtcagggccgacttgcttctcttaggctctgcgttcaggggctacctcttccaaagactacacagctgcaggcccagcctcagagcagaggtgatatgggtattaccaggctctaatggaaagtgtgctctctcgatatctacttgcagggaagcttctgaaattggtaagggagcacctattgcaaggctcagtgaacaaatggttttggtatttccctttttcatggggcaccagaagggtattttctcctacacaggatcgcatctgaagactttgctgaactgtgttttcctgaagtgaggagatgaaagacctcagataggaaaaacagagagtgagagagagagacagacactgagccaggttcccacacagtttattgagggagccaaagccagtgagaggacgaaggagtcctacttcaacctacttccttaaagctgtgtgcctccagcatgaagggaccttcccagagggcagggcctgccctataaggggccacatgaagccttgtggagactcctgcctctcataccacagcctgtcctaccctaaagacccagacatgacagcagacataatccccaccccaggagggtgctgaggaaacacccttacccatgcccctcccctagagacctcaggaagaaaggccaggacacctgtcctgtgattggccagttgaatcctcaacgtgaagacctggcaggcctggctgacaggtctgttcagatgtggcctcaggcatctactctaggatccaacccctaacattcaaacatgattaaaaacacccaggacacttctcttgctggcagaggccacaccccagataatggcagtcctgccaaactctggccagagatagggacccaagctgactgggtgtgagcacgtaaggagaccactctgccccatggggagaatcttccagggctcagctgaggctcagagcccaggcttatgttattccccatcaaatgccagtgattcctccaaacattccccacaagggagaaagggaggaggaggcagagagcttatcaagaggttcaccctatatggggctggaggttggatctactggggtgaggaaaagggtgtagaggattggggcactggggcaggggcgctggcacattcctcagattctggcatgtcatcctggaagtactcagcctggcggtactgccacagacgcaggttcccgtcccacgaactgctgacaatcttctcttcaaaggggtgccaactgacgtcacgcacacaggccttgtggttggtcagcttcttcacaatgtggccacttagaaggtcgtacacaaccactttgccagtggagcagccactgtagatgaactgctggccagtgctatgaatgggggagaaccggcagcggatgagggtgtgcagcactccgtggccccggtaggtcatcaaggagctgtcccctgggagcttcagcttccgccaggcttttttgggcacttgctgccaccgatagtcccagttttgctgtgtggcagcctggcgtgaagcttccatgccttcccggctggaaaagcgtcggatatcccagagtttgatggtctggtctttagagttggagatcagataccgggcatcacccttgctgtcaatgaaggtgatgccatcctggtgtccagccagtgcacccacaggcttggggtcatcctcccgcatggtgcgtcgatcccacactttgcagatggcatcatctcccccagagaacaggatttgggagcttatatcagcaaaggccactgcattcacatcatcctcatgggactcaatctgaagggtgcgccggttctgttctcggtcaaagacatacaggcagccatcattggcccctcctagtacttctcgtccatctgaggagacagcaatggagaagacagcaaagcgacgctcatctggcctgagatccagggcagtgtgtgtatctccctcaccatagatattgcagatatgaatgtaatcagaccagctagagtagaggaagtggttcccatcaggggtgaaggccacatccaagacgctccagcctacgtcgcgggccttgatgctcttgaatttacggaaacggccatatcggcagtcatagagtcggattgtctggtcttggcaagcagacatgaatatttgaccatctttgctgtagatgccacagaaagccttctgagagtagctatcagtgaagcccagatcattgggcaagaagtgagatatcactcgagactgttctccaagggagaagcttccccgatggcagaggccccgttctctctggtgcaacattcgaggaaagctgtgcttctgggcggcccgcctaagccccagctgccctgtggccagttccacttgtgtcttgatctcattgaattccagctcccgggtgtcaggggtagcatccacaggtgggttgtatcgatccccaagacgaccatcccaagctctgtcattctcttcctctgagtccaagagggcctgcggaggagataggccagtacctgggccagatccacatcttcatcctcttcttcctcttcctcactccgacgcaggccagcccctcttcggggcaagccctcggaggggtctccggacccggatcctgcactgctgctgttccgcgatcccatcttctggtcacagcattcttaggtcctgtgcgggggctcctcctgtcacctccttgggtttggtgaaagcaaagcgtgctctagaaataccagggtctcctgagacggggtagtagctatctctaggagggtgacccttcctcggggctgagatcccttttctttagcctatgccaactaccaaggcgtcgggaacacaaaccttctccaatcctgtgaagcaaagaaagcaagagtgaaccgtagtgcgctaccctagctcaccaactgaagaaagatttgttttctacaccaaactcacctatcgaagtc

SEQ ID NO: 13150 - RNA, 3072 nt, Homo sapiens
  source 1..3072: mol_type = other RNA
gctgggattacaggcatgagccaccacacctagcttgtttattcttttaaaactgcctattttgccatgaaataggtacccttgctgtgaaagcctgtgaacacccctggatgtgtgtaccttcatttaaaaactgccttagagggcatgaaatgtcatcagggaagatctattccgagctgggtgtgagctctagccctctccctgaccatcggtttgctctggggtatgaggttctgagtgtgaggcgcccactggggcctggcgtcagggccgacttgcttctcttaggctctgcgttcaggggctacctcttccaaagactacacagctgcaggcccagcctcagagcagaggtgatatgggtattaccaggctctaatggaaagtgtgctctctcgatatctacttgcagggaagcttctgaaattggtaagggagcacctattgcaaggctcagtgaacaaatggttttggtatttccctttttcatggggcaccagaagggtattttctcctacacaggatcgcatctgaagactttgctgaactgtgttttcctgaagtgaggagatgaaagacctcagataggaaaaacagagagtgagagagagagacagacactgagccaggttcccacacagtttattgagggagccaaagccagtgagaggacgaaggagtcctacttcaacctacttccttaaagctgtgtgcctccagcatgaagggaccttcccagagggcagggcctgccctataaggggccacatgaagccttgtggagactcctgcctctcataccacagcctgtcctaccctaaagacccagacatgacagcagacataatccccaccccaggagggtgctgaggaaacacccttacccatgcccctcccctagagacctcaggaagaaaggccaggacacctgtcctgtgattggccagttgaatcctcaacgtgaagacctggcaggcctggctgacaggtctgttcagatgtggcctcaggcatctactctaggatccaacccctaacattcaaacatgattaaaaacacccaggacacttctcttgctggcagaggccacaccccagataatggcagtcctgccaaactctggccagagatagggacccaagctgactgggtgtgagcacgtaaggagaccactctgccccatggggagaatcttccagggctcagctgaggctcagagcccaggcttatgttattccccatcaaatgccagtgattcctccaaacattccccacaagggagaaagggaggaggaggcagagagcttatcaagaggttcaccctatatggggctggaggttggatctactggggtgaggaaaagggtgtagaggattggggcactggggcaggggcgctggcacattcctcagattctggcatgtcatcctggaagtactcagcctggcggtactgccacagacgcaggttcccgtcccacgaactgctgacaatcttctcttcaaaggggtgccaactgacgtcacgcacacaggccttgtggttggtcagcttcttcacaatgtggccacttagaaggtcgtacacaaccactttgccagtggagcagccactgtagatgaactgctggccagtgctatgaatgggggagaaccggcagcggatgagggtgtgcagcactccgtggccccggtaggtcatcaaggagctgtcccctgggagcttcagcttccgccaggcttttttgggcacttgctgccaccgatagtcccagttttgctgtgtggcagcctggcgtgaagcttccatgccttcccggctggaaaagcgtcggatatcccagagtttgatggtctggtctttagagttggagatcagataccgggcatcacccttgctgtcaatgaaggtgatgccatcctggtgtccagccagtgcacccacaggcttggggtcatcctcccgcatggtgcgtcgatcccacactttgcagatggcatcatctcccccagagaacaggatttgggagcttatatcagcaaaggccactgcattcacatcatcctcatgggactcaatctgaagggtgcgccggttctgttctcggtcaaagacatacaggcagccatcattggcccctcctagtacttctcgtccatctgaggagacagcaatggagaagacagcaaagcgacgctcatctggcctgagatccagggcagtgtgtgtatctccctcaccatagatattgcagatatgaatgtaatcagaccagctagagtagaggaagtggttcccatcaggggtgaaggccacatccaagacgctccagcctacgtcgcgggccttgatgctcttgaatttacggaaacggccatatcggcagtcatagagtcggattgtctggtcttggcaagcagacatgaatatttgaccatctttgctgtagatgccacagaaagccttctgagagtagctatcagtgaagcccagatcattgggcaagaagtgagatatcactcgagactgttctccaagggagaagcttccccgatggcagaggccccgttctctctggtgcaacattcgaggaaagctgtgcttctgggcggcccgcctaagccccagctgccctgtggccagttccacttgtgtcttgatctcattgaattccagctcccgggtgtcaggggtagcatccacaggtgggttgtatcgatccccaagacgaccatcccaagctctgtcattctcttcctctgagtccaagagggcctgggccagatccacatcttcatcctcttcttcctcttcctcactccgacgcaggccagcccctcttcggggcaagccctcggaggggtctccggacccggatcctgcactgctgctgttccgcgatcccatcttctggtcacagcattcttaggtcctgtgcgggggctcctcctgtcacctccttctccaatcctgtgaagcaaagaaagcaagagtgaaccgtagtgcgctaccctagctcaccaactgaagaaagatttgttttctacaccaaactcacctatcgaag

SEQ ID NO: 13151 - RNA, 5153 nt, Homo sapiens
  source 1..5153: mol_type = other RNA
gctgggattacaggcatgagccaccacacctgacccacattgggaaatcttgttaatatcagattacaattaagtgggaatagtggtgaggctgagactatttctaataagttccctggtgatactgaggctgctgttcctcaaatcatacttgggagtagcaatgttctagagatgatctagtgggtttttttgagacagagttactctatcgcccaggctggaatgcagtggaaatctcggctcactgcaacctctgcctcccaggttcaagtgattctcctgcctcagcctcccaactagctgggattacacgcacccaccaccatgcccggctaatttttgtatttttagtagatacagggtttcgccatgttggccatgcttgtcttgaactcctgacttcacgtggtccacctgccttggcctcccaaagtgctgggataacaggcataaaccaccacgcctggcaagatttgattatgacttatcagatctaaacagagttcctgaactagtcaagtagcaatctaattctacattagaacaaaacgcaagagataggccaatggttagaactgagggtataatagggtttacctgtatgaaattcactgtttattaagtcacttttatgtacagaaagacctgccctagttaccatatcacttttagggtttcaaggcttcatctcacattcttcagctgaaaacaggtaaatctggtgaaggtattatctgaactgcccgtcacagagctagagagaagtttttcttttgttttttttttttttgagacagtctctcactctcaccctggctggagtgcattggtgtgatctcaactcactgcaacctccaccttccaggttcaagcaattctcctgcctcagtctcccgagtacctgggattacaggcgcctgccaccaagcccagctaattttttttagtagagacggggttttgccaccttgcccaggctggtctcgaactcctgagctcctgcaatccactcacctcagcctccctaaatgctgggattataggcatgaggaaccgcacccagcctaaagagaagtttttcttttttttttttttttgagacggagtctcgctctgtcacccaggctggagtgcagtggcgcgctctcggctcactgcaagctccgcctcccgggttcacaccattctcctgcctcagcctcccgagtagctgggactacaggcgcctgccaccgcacccggctaatttttttttgtattttttagtagagacggggtttcaccgtggtctcgatctcctgaccttgtgatccgcccgcctcggcctcccaaagtgctgggattgcaggcgtgagccactgcgcccggccaagagaagtttttcttaaaatcctttttttgggggggccaggatcggtggctaacatctgtaatcccagcaactttgggaggtcgaggcaggcggatcatgaggtcaagcaatcgagaccatcctggccaacatggtgaaacctcatctctattaaaaatacaaaaattagctgagtgtggtagcacgtgcctgtagtcccagctacttgggaggctgaggcaggagaattgcttgaacccaggagacggaggttgcggtgagctgagaacgcaccactgcattctagcctgacgacagagggagactccgtctcaaaaataaaaaataaaaataaaaataatcccttttttttttttaactatgcaagtctcattacatttaaaacccttttttaaacttggtcccttttctgtgccaactttatgtttgtttttgttcttgtttttgtttgagatggagtctcgctctgttgcccaggctggagtgcggtggcgcgatctcagctcactccaacctctgcctcctgggttcaagtgattctcctgccttagcctcctgagtagctgggattacaggcgtgcaccaccacgcctggataattttttttgtaattttagtagagatggggtttcaccatattggtctgaaactcctgacctcgtgatctgcccgccttggcctcccaaagtgctggcattacaggtatgagccactgtgcctggcccctattttttattttctgagatgaagtctcgctctgttgcccaggctggagcgcactagcatgatctcagctcaatgcaacctccgcctccaaggttaaagcaattcttctgcctcagcctctaagtagctgggatcacaggtgcctggaacgtgcctggctaatttttctatttttagtagagatggttttgccatgttggccaggctggtctcaaactcctgacctcaggtgatctgtctgcctcggcctcccaaagtgttaggattacaggcgtgagccattgtacccggccgagttacataatttgaatacattgttattaatctgcaataatctgtaaggtattatctccattttacagatgagaatgtgaagaaaatgacttgttcaaggccctcattgcaataaccagagctaagtttgcaaccacgtctcttagactccaaggcccacacactttttactttatgacactgcctccctaaatgctaaagattaaaaactctggtaggatgaatttttacatctctgtcagcagtgggattagaatccatgcctgtgaagagatgggaccgtaactcagcacctaaatggattattttttgtattaaaaatttcataattccctttctcagggaaatctgtaaagataaaatattaaagataaagatctgtaaagataaaaaatattaaatcctacaggcaagcctgagggcagcactaatgtgttaatggcttaaaaaatgattccaatgtttgcatgccctcaggcctggggcgtttattagtgcaggccaaagggctcttgggatttcttttgccttgatgagatacggcagaaacaacctgggggtttgaagagtggggctgcaaaaaggatttctgcaactccaatgcaaaatgatagtccatgtgttctggcatatcccataccggtaccagggagccacacttctcacagggcacttggtcctcagcagctagaagacttggatttggggttgctttctgagtcacctccagcacagatttggaagctgaagaggcgtgcatgctttggctgttgtgggccaaatccatctctgcaggagttgctttagaggattcttctagcttcgacaccccttcacaaacagggacacaccctggatactctgttggtaaagagtttggtaatgctttacagttggaccatgggttttgttggggggaagaaactgaagaattattaagctgtttctgctttagaagcagacttttctgcttaaagaagggctcagttcctgtactttgactggtttgaaaaggtaatgagggcttggatggtgaattgctcatgggagcctgagtgggagcagtaagagatgaaagcgaagcttctttaactttctgcctttctgcagctttttggaagaatgattccagagacgtggttgctttcttagtggctgtcaccgctgggccacttccctgggtcttagcttctgagctggtaactggcacctttggcagagaacttgggtcactgctcaagaagctggtgatgtcattctgtctggattccagaagtattacagttcttgatgacagtaaatgcatcatggctcatcttgtgagcatcatagcgggtaagggcacagcagcggcgcaggctgctgaggcgtttgtctccttgtacacgaatgctcacaaccagctgggtggctaccctgtcattatcatttcggtctttagtcagtctctcctctagttcctgggctaattgcaacagccaccattgtacctgttcccgagtagcaagagctgtttttcctgggaagttcttactacagccaatggttttgggtagttgcctgggtttaactggatcatgttcaatccctcggcacatggcatatagccaagacccattcttctccccaaaatgactctggagctgggattcagtgaactgggtcagttcacccatgtattctatccctaggatctcaatgacagaggcccctagctttcctccaagactacggattttgcgaatgggcatttggctgaagagctgtgggactgacccatgtgaaaccagggtttggcggttgggcttgtttagtccacaggccagttttgccaggaccttattgtgtgaaattccagctgaacactgaaaaccagtctccctctctatggctgctctcatttcctccacaatcactgctcccacggtgagctgcaggtctggagaggtgaggttatcaatctgaagagaatcgagccattgaaataagccttgttttcgcatcccctctttctgaacagtctcttctgccgttgtagggccttggggcaacccttcaatgtaagtgcttggcaacaagtctgccgagataggctgaccttgtagcttttgtagtctctcttgtacagcactggtcagatctacgtaagcctcatcaatgctggcacgttcaatcacagcaaaacgagacattatctccatcacttcaacactggcttcccggtacttggtgaggttagctttcccacgggactcacgaacttgtgccagtagaagatctggacataacttcttagcatcatctgcccacatacttctagtgactccaaatgcacgagcttcataactcactgcaattattccaccacccttccatgatttgtactgtacaactgcacaaggtttattcctcaaatgaggattttgccgctgctccacttgaacaaaaaaacagtccatgtccacgagagcaaccactcgatcctgtccagtagccatttttcaaggtaacaaacacctggcaaaactgccagcagcggttgccgaaaatgctgggttcggtgcctactggaaggaaaatggaagggctcctgaatatcttttcgcctttctaggagcggtccagtgagtttcgagcgagatttattccctgtgacgacggagaaaccgagaagggatcgtaaaggatcctgcccgggcaaccgtccccagcagggatcagacgagagcggcgcgcccagcaatgcagccgccagact

SEQ ID NO: 13152 - RNA, 5224 nt, Homo sapiens
  source 1..5224: mol_type = other RNA
gctgggattacaggcatgagccaccacacctgacccacattgggaaatcttgttaatatcagattacaattaagtgggaatagtggtgaggctgagactatttctaataagttccctggtgatactgaggctgctgttcctcaaatcatacttgggagtagcaatgttctagagatgatctagtgggtttttttgagacagagttactctatcgcccaggctggaatgcagtggaaatctcggctcactgcaacctctgcctcccaggttcaagtgattctcctgcctcagcctcccaactagctgggattacacgcacccaccaccatgcccggctaatttttgtatttttagtagatacagggtttcgccatgttggccatgcttgtcttgaactcctgacttcacgtggtccacctgccttggcctcccaaagtgctgggataacaggcataaaccaccacgcctggcaagatttgattatgacttatcagatctaaacagagttcctgaactagtcaagtagcaatctaattctacattagaacaaaacgcaagagataggccaatggttagaactgagggtataatagggtttacctgtatgaaattcactgtttattaagtcacttttatgtacagaaagacctgccctagttaccatatcacttttagggtttcaaggcttcatctcacattcttcagctgaaaacaggtaaatctggtgaaggtattatctgaactgcccgtcacagagctagagagaagtttttcttttgttttttttttttttgagacagtctctcactctcaccctggctggagtgcattggtgtgatctcaactcactgcaacctccaccttccaggttcaagcaattctcctgcctcagtctcccgagtacctgggattacaggcgcctgccaccaagcccagctaattttttttagtagagacggggttttgccaccttgcccaggctggtctcgaactcctgagctcctgcaatccactcacctcagcctccctaaatgctgggattataggcatgaggaaccgcacccagcctaaagagaagtttttcttttttttttttttttgagacggagtctcgctctgtcacccaggctggagtgcagtggcgcgctctcggctcactgcaagctccgcctcccgggttcacaccattctcctgcctcagcctcccgagtagctgggactacaggcgcctgccaccgcacccggctaatttttttttgtattttttagtagagacggggtttcaccgtggtctcgatctcctgaccttgtgatccgcccgcctcggcctcccaaagtgctgggattgcaggcgtgagccactgcgcccggccaagagaagtttttcttaaaatcctttttttgggggggccaggatcggtggctaacatctgtaatcccagcaactttgggaggtcgaggcaggcggatcatgaggtcaagcaatcgagaccatcctggccaacatggtgaaacctcatctctattaaaaatacaaaaattagctgagtgtggtagcacgtgcctgtagtcccagctacttgggaggctgaggcaggagaattgcttgaacccaggagacggaggttgcggtgagctgagaacgcaccactgcattctagcctgacgacagagggagactccgtctcaaaaataaaaaataaaaataaaaataatcccttttttttttttaactatgcaagtctcattacatttaaaacccttttttaaacttggtcccttttctgtgccaactttatgtttgtttttgttcttgtttttgtttgagatggagtctcgctctgttgcccaggctggagtgcggtggcgcgatctcagctcactccaacctctgcctcctgggttcaagtgattctcctgccttagcctcctgagtagctgggattacaggcgtgcaccaccacgcctggataattttttttgtaattttagtagagatggggtttcaccatattggtctgaaactcctgacctcgtgatctgcccgccttggcctcccaaagtgctggcattacaggtatgagccactgtgcctggcccctattttttattttctgagatgaagtctcgctctgttgcccaggctggagcgcactagcatgatctcagctcaatgcaacctccgcctccaaggttaaagcaattcttctgcctcagcctctaagtagctgggatcacaggtgcctggaacgtgcctggctaatttttctatttttagtagagatggttttgccatgttggccaggctggtctcaaactcctgacctcaggtgatctgtctgcctcggcctcccaaagtgttaggattacaggcgtgagccattgtacccggccgagttacataatttgaatacattgttattaatctgcaataatctgtaaggtattatctccattttacagatgagaatgtgaagaaaatgacttgttcaaggccctcattgcaataaccagagctaagtttgcaaccacgtctcttagactccaaggcccacacactttttactttatgacactgcctccctaaatgctaaagattaaaaactctggtaggatgaatttttacatctctgtcagcagtgggattagaatccatgcctgtgaagagatgggaccgtaactcagcacctaaatggattattttttgtattaaaaatttcataattccctttctcagggaaatctgtaaagataaaatattaaagataaagatctgtaaagataaaaaatattaaatcctacaggcaagcctgagggcagcactaatgtgttaatggcttaaaaaatgattccaatgtttgcatgccctcaggcctggggcgtttattagtgcaggccaaagggctcttgggatttcttttgccttgatgagatacggcagaaacaacctgggggtttgaagagtggggctgcaaaaaggatttctgcaactccaatgcaaaatgatagtccatgtgttctggcatatcccataccggtaccagggagccacacttctcacagggcacttggtcctcagcagctagaagacttggatttggggttgctttctgagtcacctccagcacagatttggaagctgaagaggcgtgcatgctttggctgttgtgggccaaatccatctctgcaggagttgctttagaggattcttctagcttcgacaccccttcacaaacagggacacaccctggatactctgttggtaaagagtttggtaatgctttacagttggaccatgggttttgttggggggaagaaactgaagaattattaagctgtttctgctttagaagcagacttttctgcttaaagaagggctcagttcctgtactttgactggtttgaaaaggtaatgagggcttggatggtgaattgctcatgggagcctgagtgggagcagtaagagatgaaagcgaagcttctttaactttctgcctttctgcagctttttggaagaatgattccagagacgtggttgctttcttagtggctgtcaccgctgggccacttccctgggtcttagcttctgagctggtaactggcacctttggcagagaacttgggtcactgctcaagaagctggtgatgtctgtagaagatgaaggggcagaggcagaaaattttgtagcacagaggaaaagcattgtgagaggaggagaccattctgtctggattccagaagtattacagttcttgatgacagtaaatgcatcatggctcatcttgtgagcatcatagcgggtaagggcacagcagcggcgcaggctgctgaggcgtttgtctccttgtacacgaatgctcacaaccagctgggtggctaccctgtcattatcatttcggtctttagtcagtctctcctctagttcctgggctaattgcaacagccaccattgtacctgttcccgagtagcaagagctgtttttcctgggaagttcttactacagccaatggttttgggtagttgcctgggtttaactggatcatgttcaatccctcggcacatggcatatagccaagacccattcttctccccaaaatgactctggagctgggattcagtgaactgggtcagttcacccatgtattctatccctaggatctcaatgacagaggcccctagctttcctccaagactacggattttgcgaatgggcatttggctgaagagctgtgggactgacccatgtgaaaccagggtttggcggttgggcttgtttagtccacaggccagttttgccaggaccttattgtgtgaaattccagctgaacactgaaaaccagtctccctctctatggctgctctcatttcctccacaatcactgctcccacggtgagctgcaggtctggagaggtgaggttatcaatctgaagagaatcgagccattgaaataagccttgttttcgcatcccctctttctgaacagtctcttctgccgttgtagggccttggggcaacccttcaatgtaagtgcttggcaacaagtctgccgagataggctgaccttgtagcttttgtagtctctcttgtacagcactggtcagatctacgtaagcctcatcaatgctggcacgttcaatcacagcaaaacgagacattatctccatcacttcaacactggcttcccggtacttggtgaggttagctttcccacgggactcacgaacttgtgccagtagaagatctggacataacttcttagcatcatctgcccacatacttctagtgactccaaatgcacgagcttcataactcactgcaattattccaccacccttccatgatttgtactgtacaactgcacaaggtttattcctcaaatgaggattttgccgctgctccacttgaacaaaaaaacagtccatgtccacgagagcaaccactcgatcctgtccagtagccatttttcaaggtaacaaacacctggcaaaactgccagcagcggttgccgaaaatgctgggttcggtgcctactggaaggaaaatggaagggctcctgaatatcttttcgcctttctaggagcggtccagtgagtttcgagcgagatttattccctgtgacgacggagaaaccgagaagggatcgtaaaggatcctgcccgggcaaccgtccccagcagggatcagacgagagcggcgcgcccagcaatgcagccgccagact

SEQ ID NO: 13153 - RNA, 4865 nt, Homo sapiens
  source 1..4865: mol_type = other RNA
gctgggattacaggcatgagccaccacacctgacccacattgggaaatcttgttaatatcagattacaattaagtgggaatagtggtgaggctgagactatttctaataagttccctggtgatactgaggctgctgttcctcaaatcatacttgggagtagcaatgttctagagatgatctagtgggtttttttgagacagagttactctatcgcccaggctggaatgcagtggaaatctcggctcactgcaacctctgcctcccaggttcaagtgattctcctgcctcagcctcccaactagctgggattacacgcacccaccaccatgcccggctaatttttgtatttttagtagatacagggtttcgccatgttggccatgcttgtcttgaactcctgacttcacgtggtccacctgccttggcctcccaaagtgctgggataacaggcataaaccaccacgcctggcaagatttgattatgacttatcagatctaaacagagttcctgaactagtcaagtagcaatctaattctacattagaacaaaacgcaagagataggccaatggttagaactgagggtataatagggtttacctgtatgaaattcactgtttattaagtcacttttatgtacagaaagacctgccctagttaccatatcacttttagggtttcaaggcttcatctcacattcttcagctgaaaacaggtaaatctggtgaaggtattatctgaactgcccgtcacagagctagagagaagtttttcttttgttttttttttttttgagacagtctctcactctcaccctggctggagtgcattggtgtgatctcaactcactgcaacctccaccttccaggttcaagcaattctcctgcctcagtctcccgagtacctgggattacaggcgcctgccaccaagcccagctaattttttttagtagagacggggttttgccaccttgcccaggctggtctcgaactcctgagctcctgcaatccactcacctcagcctccctaaatgctgggattataggcatgaggaaccgcacccagcctaaagagaagtttttcttttttttttttttttgagacggagtctcgctctgtcacccaggctggagtgcagtggcgcgctctcggctcactgcaagctccgcctcccgggttcacaccattctcctgcctcagcctcccgagtagctgggactacaggcgcctgccaccgcacccggctaatttttttttgtattttttagtagagacggggtttcaccgtggtctcgatctcctgaccttgtgatccgcccgcctcggcctcccaaagtgctgggattgcaggcgtgagccactgcgcccggccaagagaagtttttcttaaaatcctttttttgggggggccaggatcggtggctaacatctgtaatcccagcaactttgggaggtcgaggcaggcggatcatgaggtcaagcaatcgagaccatcctggccaacatggtgaaacctcatctctattaaaaatacaaaaattagctgagtgtggtagcacgtgcctgtagtcccagctacttgggaggctgaggcaggagaattgcttgaacccaggagacggaggttgcggtgagctgagaacgcaccactgcattctagcctgacgacagagggagactccgtctcaaaaataaaaaataaaaataaaaataatcccttttttttttttaactatgcaagtctcattacatttaaaacccttttttaaacttggtcccttttctgtgccaactttatgtttgtttttgttcttgtttttgtttgagatggagtctcgctctgttgcccaggctggagtgcggtggcgcgatctcagctcactccaacctctgcctcctgggttcaagtgattctcctgccttagcctcctgagtagctgggattacaggcgtgcaccaccacgcctggataattttttttgtaattttagtagagatggggtttcaccatattggtctgaaactcctgacctcgtgatctgcccgccttggcctcccaaagtgctggcattacaggtatgagccactgtgcctggcccctattttttattttctgagatgaagtctcgctctgttgcccaggctggagcgcactagcatgatctcagctcaatgcaacctccgcctccaaggttaaagcaattcttctgcctcagcctctaagtagctgggatcacaggtgcctggaacgtgcctggctaatttttctatttttagtagagatggttttgccatgttggccaggctggtctcaaactcctgacctcaggtgatctgtctgcctcggcctcccaaagtgttaggattacaggcgtgagccattgtacccggccgagttacataatttgaatacattgttattaatctgcaataatctgtaaggtattatctccattttacagatgagaatgtgaagaaaatgacttgttcaaggccctcattgcaataaccagagctaagtttgcaaccacgtctcttagactccaaggcccacacactttttactttatgacactgcctccctaaatgctaaagattaaaaactctggtaggatgaatttttacatctctgtcagcagtgggattagaatccatgcctgtgaagagatgggaccgtaactcagcacctaaatggattattttttgtattaaaaatttcataattccctttctcagggaaatctgtaaagataaaatattaaagataaagatctgtaaagataaaaaatattaaatcctacaggcaagcctgagggcagcactaatgtgttaatggcttaaaaaatgattccaatgtttgcatgccctcaggcctggggcgtttattagtgcaggccaaagggctcttgggatttcttttgccttgatgagatacggcagaaacaacctgggggtttgaagagtggggctgcaaaaaggatttctgcaactccaatgcaaaatgatagtccatgtgttctggcatatcccataccggtaccagggagccacacttctcacagggcacttggtcctcagcagctagaagacttggatttggggttgctttctgagtcacctccagcacagatttggaagctgaagaggcgtgcatgctttggctgttgtgggccaaatccatctctgcaggagttgctttagaggattcttctagcttcgacaccccttcacaaacagggacacaccctggatactctgttggtaaagagtttggtaatgctttacagttggaccatgggttttgttggggggaagaaactgaagaattattaagctgtttctgctttagaagcagacttttctgcttaaagaagggctcagttcctgtactttgactggtttgaaaaggtaatgagggcttggatggtgaattgctcatgggagcctgagtgggagcagtaagagatgaaagcgaagcttctttaactttctgcctttctgcagctttttggaagaatgattccagagacgtggttgctttcttagtggctgtcaccgctgggccacttccctgggtcttagcttctgagctggtaactggcacctttggcagagaacttgggtcactgctcaagaagctggtgatgtctgtagaagatgaaggggcagaggcagaaaattttgtagcacagaggaaaagcattgtgagaggaggagaccattctgtctggattccagaagtattacagttcttgatgacagtaaatgcatcatggctcatcttgtgagcatcatagcgggtaagggcacagcagcggcgcaggctgctgaggcgtttgtctccttgtacacgaatgctcacaaccagctgggtggctaccctgtcattatcatttcggtctttagtcagtctctcctctagttcctgggctaattgcaacagccaccattgtacctgttcccgagtagcaagagctgtttttcctgggaagttcttactacagccaatggttttgggtagttgcctgggtttaactggatcatgttcaatccctcggcacatggcatatagccaagacccattcttctccccaaaatgactctggagctgggattcagtgaactgggtcagttcacccatgtattctatccctaggatctcaatgacagaggcccctagctttcctccaagactacggattttgcgaatgggcatttggctgaagagctgtgggactgacccatgtgaaaccagggtttggcggttgggcttgtttagtccacaggccagttttgccaggaccttattgtgtgaaattccagctgaacactgaaaaccagtctccctctctatggctgctctcatttcctccacaatcactgctcccacggtgagctgcaggtctggagaggtgaggttatcaatctgaagagaatcgagccattgaaataagccttgttttcgcatcccctttggtgaggttagctttcccacgggactcacgaacttgtgccagtagaagatctggacataacttcttagcatcatctgcccacatacttctagtgactccaaatgcacgagcttcataactcactgcaattattcaaggtaacaaacacctggcaaaactgccagcagcggttgccgaaaatgctgggttcggtgcctactggaaggaaaatggaagggctcctgaatatcttttcgcctttctaggagcggtccagtgagtttcgagcgagatttattccctgtgacgacggagaaaccgagaagggatcgtaaaggatcctgcccgggcaaccgtccccagcagggatcagacgagagcggcgcgcccagcaatgcagccgccagact

SEQ ID NO: 13154 - RNA, 5117 nt, Homo sapiens
  source 1..5117: mol_type = other RNA
gctgggattacaggcatgagccaccacacctggccagaatgtatcatttcttgatctgagtctggttacagagatgtattcactttgccaatatcaatgatgttacatactcatgatttgtgtacttttctttatgtatgtgtgagcaaagagttaatagcaggtctgtaccatttttctcccagaactatgcctgcttgggaaattttaggtttgtcttatcccagcacgagtttcttgtaaatgacccaaattaagataaatttggaatattgggtaccagggacagacatccattttgtgcactgtgaaacctacaatctatgggacagtacatggggctgggagacctgtgaaccgtaggcctatatgactggtgggaaacccacatagaagcttctttgcatcaaggcaaacccccacataccacaacctcatccaaataccacaagctcatgcacgctctttaggcaggtgaggagggacccaagcatcatgcatgcttaatttcctgtcctgtatcctactataaagctaagcaaatttagtgctaggctaaatgctattgtatctcatcagtttgcttgccagtccaaacatgttcccaataccatggtggtaccatgtattgcacttcaataaaaagtttactaaattcctttatctattcttgccaaaaggttattttcactgattatatattccgcttggcctccaaattccttccatttttctgagcctcctcgctgtctgttgacctcctatattctcctttttaggactctacaattgacccctaaacctcctattcatttttttatgcagagctgtttaaatattgcactatctcacctcaaatgacccagagaaccctcatatcaataactaatattaagattggttgcaaaacatagttcctttccaggagaacttgtataactatctcttttttttttgacagagtctcactctgtcacccaggatagagggcagtagcacagtctcagctcaccgcaacttccacctcctgggttcaagcaattctcctgcctcagcctcccgagtagctgggattacaggcacgtgccaccacgcctggctaacttttcgtatttttagtagagacagggtttcaccatgttggccaggctgatctctaactcctgacctcagatgatccacccgcctcggcctcccaaagtgctggattacaggcatgagccattgtgcctggctgactacctcttaaggaaacttttttgtttagttagacaaagaatggtaaatctctttccacgcacattcaaaattcacacattatctggactcttagttacctaggacatacccccagttattcttgtacctaatttggtacctcaaattttcccgaggtgttaaaacaaaaggaatagagcttgcctagcaccttagaagtgctgcaccctcttagaagtgccaggcactgtcatagttgttgccctcttagaatgatttgcctctgggtgtcactctttgctctgtacctggtacaactatagtgatggcagatgctccatactcagtcctagcttttcagtgtttggctttgctgggttttttctttctttctttttgagagaaatggggacttccaagctgagtaaaacctggaaagggcaacttactgcagccatatattgatactacattatttcctatgtcataatattaacctcccttccatctgcttttgctgtttagtagtctcatgtcttcttgagctagactatcttatgtaaattcatgttatgtgaattgaggtctcagtaataacagccttctgtctttcctcaccgtaacaggagtcataggaaagggggtgtgatagtctcagaaacagcctagcatctcatacaaacttgtttctgtttttgagacagggtctcgctctatcacccaggctggagtgcagtggcacaatcatggctcactgcagccttgatctcctgggctcctgtctcagcctcccaagtagctgggactacgtgcatgcatgcaccactacacctagctttttttttcttttttcttttttcttgtaatagagataggatctcactttgttgcccaggctggtctcaaactgggctcaagttatcttcccaccttggcctcccaaagtgctgggattataggcatgagccaccacattcagcccaaacatttctgagaccactacttgaactatcaagtctcctcttgtaactgattctcattagaaataatacacatttattgaatgtcattgatatataaagataccattctttgagtgggggaaatataatttaaaagtcgcaactactgacaatcaacaaataaactctaatgagaatcataaagcttgttcccagagaaccatgatacagggtgggacagtacgcaaataatgggctcctgttgtcagacttcatggtgattacattagtgctttctccagtatctttcttcctattgtactcctgaagcactcagaatgataaagataaatttctgatcattcctacaaagagtgcaggcaaagttaagatttaactgtgattgctggttgtttcatctcgaattcaaaatcctggatttccgaaacaatggagcttgatgtcacatttggctatcttgcttttgtctcctcttctggaaagaacaaatcatcttcctgaaaattacaggagacacttagtatgacaaaataaggcctctgaaactgtccaatctcacatgtaaaaagtgtaaaatcacagaactaaaatcaggttccggattttcctggaaatagaatgtcaccgggatctgttcaaaggtgagctttggctacattttataacagtgtttaaaactcgaatgcaaaaaactgctttcaatataatcagatatgtgcaaaaacaatttgttaaataacatgggaagattatattaacaaaagacatttccagaatactaacattcatgtgatttataaaggtgcattttctgtaaagagctatacagcccaaaaacatgaaattcttcaagggagtcccctttatcccatgagttggaagaatttattttcatattctatgcatggatcactgaagtgatgaatgtcactcgtcttcaagaaggaagcactctcagccttgtgaagaagaacctcaagggttcctggggctatgatcatgaagagcaccacaatgaagactgctgcgaagtctttttcacttcttcacatttgggatgtgaaatattttacagaaaaataagagtgtgcaaatccctctcacacatagaaaaacgattgtgtgaatattcttaaatttttaaaacttttaaaaactgtgatctttgcactgttttcaagagtcagcaactctgaagaaagatattcaccataagtgaccccatatggtgaagatattcacaataaatgacagttttgcaagatgactctttgggttggcattctgtttccggtcaccaggtttccgcaatctctgtgacagcccgcagcagctcggcaaatgtagggcggccttcaggtttctcatgccagcagctgtacatgacttcatatatggacattggtgccaggtgagggcgatatagcctgaagccttcagaaatagcttccacgacttgcaaatttgacttattttcaaaaggcatttttccttctgtaaaaacttcccacattaaaactccaaatgaccagacatcagatttactgctgtacttattgaaaagaaaaacttcaggaggggaccacttgattgggaacttggctccaaaagaactgacatactcatcatccaaaacgtaccttgtcattccaaagtctgaaatttttactatgcatgttgaactgaccaaacaattccttgccgccaaatccctatgaatatagccattcctctccagatattccattccttcacatatatcctggcatacactcagtagcatttccttcctaagctttcctttattctccctgagatagttaagcaggcagccattttccatgaactctgtcacaatgtaaaggggcttccgctgtatacagactccataaagttgcactagctttgaatgagataatttcatcatcactttggcctcttcaatgaaatcctcttcagacatggagccttcattgatggccttgatagctacctggatatgtgaccgccattcacctaaatggaccactccaaactgaccgcttccaatctcctttataaaagccaactcagatggatctatctcccacttttcgtagctaaacccagctgtggctggtaaacaactgcccatcagcccaactggatatcggagacgagtcatgagaccggctgcattgtgctggtgataccagattaactcagggattgattgaaaggcgtgtctttcagccacataccactgtcctgagtcattcttttttatctgataatgttttatggcagcctccgtacttcttctagctcccataaatacggaaattgtgtaggatcctaaatgtcttgaatctctgacaataaatgcaccttctttagactcttgtctcaatagatgttctgcctgatttctggtaatgtttctatggtaccaccccaaacggtctcttgccttccaccagtgaggattgtatttctccagtatcaggtattcttctgctctccttaaggctaaattacagggttctctgggcagaaaatcataaagtgccttgacttggatcttctcttcagcaacctcagagggtgggaggggaggcagtggctttcgttttgacggctgcacacggcccgtgttggattgcttcttatttgacaattggctgagccacggcctgcgacgctgggtgtatttttctggaagctcttcatctgtgctcaggcttatctgtgttctcatttgtctcatttgatggtgtctttttgttataaatagacatggtatagtgattaggaacaagagtttgaatcccagctccaccatttcatagtgtggccttgggtaagcaatgtaacctctctaatcttcaatttcctcatcgcttctgcactgaacagcaacagcagcaacagaaaacc

SEQ ID NO: 13155 - RNA, 6176 nt, Homo sapiens
  source 1..6176: mol_type = other RNA
gctgggattacaggcatgagccaccacacctggccagaatgtatcatttcttgatctgagtctggttacagagatgtattcactttgccaatatcaatgatgttacatactcatgatttgtgtacttttctttatgtatgtgtgagcaaagagttaatagcaggtctgtaccatttttctcccagaactatgcctgcttgggaaattttaggtttgtcttatcccagcacgagtttcttgtaaatgacccaaattaagataaatttggaatattgggtaccagggacagacatccattttgtgcactgtgaaacctacaatctatgggacagtacatggggctgggagacctgtgaaccgtaggcctatatgactggtgggaaacccacatagaagcttctttgcatcaaggcaaacccccacataccacaacctcatccaaataccacaagctcatgcacgctctttaggcaggtgaggagggacccaagcatcatgcatgcttaatttcctgtcctgtatcctactataaagctaagcaaatttagtgctaggctaaatgctattgtatctcatcagtttgcttgccagtccaaacatgttcccaataccatggtggtaccatgtattgcacttcaataaaaagtttactaaattcctttatctattcttgccaaaaggttattttcactgattatatattccgcttggcctccaaattccttccatttttctgagcctcctcgctgtctgttgacctcctatattctcctttttaggactctacaattgacccctaaacctcctattcatttttttatgcagagctgtttaaatattgcactatctcacctcaaatgacccagagaaccctcatatcaataactaatattaagattggttgcaaaacatagttcctttccaggagaacttgtataactatctcttttttttttgacagagtctcactctgtcacccaggatagagggcagtagcacagtctcagctcaccgcaacttccacctcctgggttcaagcaattctcctgcctcagcctcccgagtagctgggattacaggcacgtgccaccacgcctggctaacttttcgtatttttagtagagacagggtttcaccatgttggccaggctgatctctaactcctgacctcagatgatccacccgcctcggcctcccaaagtgctggattacaggcatgagccattgtgcctggctgactacctcttaaggaaacttttttgtttagttagacaaagaatggtaaatctctttccacgcacattcaaaattcacacattatctggactcttagttacctaggacatacccccagttattcttgtacctaatttggtacctcaaattttcccgaggtgttaaaacaaaaggaatagagcttgcctagcaccttagaagtgctgcaccctcttagaagtgccaggcactgtcatagttgttgccctcttagaatgatttgcctctgggtgtcactctttgctctgtacctggtacaactatagtgatggcagatgctccatactcagtcctagcttttcagtgtttggctttgctgggttttttctttctttctttttgagagaaatggggacttccaagctgagtaaaacctggaaagggcaacttactgcagccatatattgatactacattatttcctatgtcataatattaacctcccttccatctgcttttgctgtttagtagtctcatgtcttcttgagctagactatcttatgtaaattcatgttatgtgaattgaggtctcagtaataacagccttctgtctttcctcaccgtaacaggagtcataggaaagggggtgtgatagtctcagaaacagcctagcatctcatacaaacttgtttctgtttttgagacagggtctcgctctatcacccaggctggagtgcagtggcacaatcatggctcactgcagccttgatctcctgggctcctgtctcagcctcccaagtagctgggactacgtgcatgcatgcaccactacacctagctttttttttcttttttcttttttcttgtaatagagataggatctcactttgttgcccaggctggtctcaaactgggctcaagttatcttcccaccttggcctcccaaagtgctgggattataggcatgagccaccacattcagcccaaacatttctgagaccactacttgaactatcaagtctcctcttgtaactgattctcattagaaataatacacatttattgaatgtcattgatatataaagataccattctttgagtgggggaaatataatttaaaagtcgcaactactgacaatcaacaaataaactctaatgagaatcataaagcttgttcccagagaaccatgatacagggtgggacagtacgcaaataatgggctcctgttgtcagacttcatggtgattacattagtgctttctccagtatctttcttcctattgtactcctgaagcactcagaatgataaagataaatttctgatcattcctacaaagagtgcaggcaaagttaagatttaactgtgattgctggttgtttcatctcgaattcaaaatcctggatttccgaaacaatggagcttgatgtcacatttggctatcttgcttttgtctcctcttctggaaagaacaaatcatcttcctgaaaattacaggagacacttagtatgacaaaataaggcctctgaaactgtccaatctcacatgtaaaaagtgtaaaatcacagaactaaaatcaggttccggattttcctggaaatagaatgtcaccgggatctgttcaaaggtgagctttggctacattttataacagtgtttaaaactcgaatgcaaaaaactgctttcaatataatcagatatgtgcaaaaacaatttgttaaataacatgggaagattatattaacaaaagacatttccagaatactaacattcatgtgatttataaaggtgcattttctgtaaagagctatacagcccaaaaacatgaaattcttcaagggagtcccctttatcccatgagttggaagaatttattttcatattctatgcatggatcactgaagtgatgaatgtcactcgtcttcaagaaggaagcactctcagccttgtgaagaagaacctcaagggttcctggggctatgatcatgaagagcaccacaatgaagactgctgcgaagtctttttcacttcttcacatttgggatgtgaaatattttacagaaaaataagagtgtgcaaatccctctcacacatagaaaaacgattgtgtgaatattcttaaatttttaaaacttttaaaaactgtgatctttgcactgttttcaagagtcagcaactctgaagaaagatattcaccataagtgaccccatatggtgaagatattcacaataaatgacagttttgcaagatgactctttgggttggcattctgtttccggtcaccaggtttccgcaatctctgtgacagcccgcagcagctcggcaaatgtagggcggccttcaggtttctcatgccagcagctgtacatgacttcatatatggacattggtgccaggtgagggcgatatagcctgaagccttcagaaatagcttccacgacttgcaaatttgacttattttcaaaaggcatttttccttctgtaaaaacttcccacattaaaactccaaatgaccagacatcagatttactgctgtacttattgaaaagaaaaacttcaggaggggaccacttgattgggaacttggctccaaaagaactgacatactcatcatccaaaacgtaccttgtcattccaaagtctgaaatttttactatgcatgttgaactgaccaaacaattccttgccgccaaatccctatgaatatagccattcctctccagatattccattccttcacatatatcctggcatacactcagtagcatttccttcctaagctttcctttattctccctgagatagttaagcaggcagccattttccatgaactctgtcacaatgtaaaggggcttccgctgtatacagactccataaagttgcactagctttgaatgagataatttcatcatcactttggcctcttcaatgaaatcctcttcagacatggagccttcattgatggccttgatagctacctggatatgtgaccgccattcacctaaatggaccactccaaactgaccgcttccaatctcctttataaaagccaactcagatggatctatctcccacttttcgtagctaaacccagctgtggctggtaaacaactgcccatcagcccaactggatatcggagacgagtcatgagaccggctgcattgtgctggtgataccagattaactcagggattgattgaaaggcgtgtctttcagccacataccactgtcctgagtcattcttttttatctgataatgttttatggcagcctccgtacttcttctagctcccataaatacggaaattgtgtaggatcctaaatgtcttgaatctctgacaataaatgcaccttctttagactcttgtctcaatagatgttctgcctgatttctggtaatgtttctatggtaccactcatatatttctaaattagttattttgttttcagtcacatagttgcttgggattaagccttcattccccaaacggtctcttgccttccaccagtgaggattgtatttctccagtatcaggtattcttctgctctccttaaggctaaattacagggttctctgggcagaaaatcataaagtgccttgacttggatcttctcttcagcaacctcagagggtgggaggggaggcagtggctttcgttttgacggctgcacacggcccgtgttggattgcttcttatttgacaattggctgagccacggcctgcgacgctgggtgtatttttctggaagctcttcatctgtgctcaggcttatctgtgttctcatttgtaggaggaaaggatcatggtagccccttctgcggggagcacacaacagtcttcagttcttctgcggtgctctactcacaaaaacacatctttcaactgaaatcatagttcgctcaagatgtttctcacgggcagagttaaccccacctattttcctgttctgaaaacctcagaagagtataaatgacaaccaatggcatatataagaaagctcagtaatctccatcccaatctctgagggtatctgctattagtctctcatccccaaaggtgtgggtgactcgcaaacatcattttcaagaaatcacaaaattttggtaaaaggcacctttaaaattatcaaatcaaactgccctctctggactgggaaggaaatgaaggcacagacagaataagggacttgcccaaggccacaccgtgagtggcagaaacaattagattctaggctctggaatattgagtttagaatgttccatcctcccactcagcagacactttatttgggggaagtcaatctagtaataaccctaaaatgtgattgggggatggctgagaaatataaaaacaccaacaatacaaaacacacttgggagtttcacttcatcccactggaaagcataaccatgtgtcaactaattaacagagcaactttaatgaagacacagcatattctaatcgcccttccaatttcctggtttagattaaggtctccttagcattctgggtgatgactgttatttttacttcaccttttgcctttgttatgctttcgtataaaactttttttctaagtcttagtgaaaaatatttaaagatttttgaaggaaatgttgacaaatgttgccaggtgctatctatcttgttttcccataaaaagcatacactgaccattaggacagggactctatcttctcctcactctctttcataccacctagtacttcccgtagctcctcaaggtgaaaagggaagtatgggatgggaggagggaaggtcaggaaggaaggagaaaaggctgacagtgatagtaaggtagagtgtgccaggaccgactccttcaatgagctacaagtcagttaaaagttgtgcatggttagcaaccaaaatgcccatcaatgataggctggataaagaaaatgtggtacatatacaccgtggaatattatgcag

SEQ ID NO: 13156 - RNA, 5182 nt, Homo sapiens
  source 1..5182: mol_type = other RNA
gctgggattacaggcatgagccaccacacctggccagaatgtatcatttcttgatctgagtctggttacagagatgtattcactttgccaatatcaatgatgttacatactcatgatttgtgtacttttctttatgtatgtgtgagcaaagagttaatagcaggtctgtaccatttttctcccagaactatgcctgcttgggaaattttaggtttgtcttatcccagcacgagtttcttgtaaatgacccaaattaagataaatttggaatattgggtaccagggacagacatccattttgtgcactgtgaaacctacaatctatgggacagtacatggggctgggagacctgtgaaccgtaggcctatatgactggtgggaaacccacatagaagcttctttgcatcaaggcaaacccccacataccacaacctcatccaaataccacaagctcatgcacgctctttaggcaggtgaggagggacccaagcatcatgcatgcttaatttcctgtcctgtatcctactataaagctaagcaaatttagtgctaggctaaatgctattgtatctcatcagtttgcttgccagtccaaacatgttcccaataccatggtggtaccatgtattgcacttcaataaaaagtttactaaattcctttatctattcttgccaaaaggttattttcactgattatatattccgcttggcctccaaattccttccatttttctgagcctcctcgctgtctgttgacctcctatattctcctttttaggactctacaattgacccctaaacctcctattcatttttttatgcagagctgtttaaatattgcactatctcacctcaaatgacccagagaaccctcatatcaataactaatattaagattggttgcaaaacatagttcctttccaggagaacttgtataactatctcttttttttttgacagagtctcactctgtcacccaggatagagggcagtagcacagtctcagctcaccgcaacttccacctcctgggttcaagcaattctcctgcctcagcctcccgagtagctgggattacaggcacgtgccaccacgcctggctaacttttcgtatttttagtagagacagggtttcaccatgttggccaggctgatctctaactcctgacctcagatgatccacccgcctcggcctcccaaagtgctggattacaggcatgagccattgtgcctggctgactacctcttaaggaaacttttttgtttagttagacaaagaatggtaaatctctttccacgcacattcaaaattcacacattatctggactcttagttacctaggacatacccccagttattcttgtacctaatttggtacctcaaattttcccgaggtgttaaaacaaaaggaatagagcttgcctagcaccttagaagtgctgcaccctcttagaagtgccaggcactgtcatagttgttgccctcttagaatgatttgcctctgggtgtcactctttgctctgtacctggtacaactatagtgatggcagatgctccatactcagtcctagcttttcagtgtttggctttgctgggttttttctttctttctttttgagagaaatggggacttccaagctgagtaaaacctggaaagggcaacttactgcagccatatattgatactacattatttcctatgtcataatattaacctcccttccatctgcttttgctgtttagtagtctcatgtcttcttgagctagactatcttatgtaaattcatgttatgtgaattgaggtctcagtaataacagccttctgtctttcctcaccgtaacaggagtcataggaaagggggtgtgatagtctcagaaacagcctagcatctcatacaaacttgtttctgtttttgagacagggtctcgctctatcacccaggctggagtgcagtggcacaatcatggctcactgcagccttgatctcctgggctcctgtctcagcctcccaagtagctgggactacgtgcatgcatgcaccactacacctagctttttttttcttttttcttttttcttgtaatagagataggatctcactttgttgcccaggctggtctcaaactgggctcaagttatcttcccaccttggcctcccaaagtgctgggattataggcatgagccaccacattcagcccaaacatttctgagaccactacttgaactatcaagtctcctcttgtaactgattctcattagaaataatacacatttattgaatgtcattgatatataaagataccattctttgagtgggggaaatataatttaaaagtcgcaactactgacaatcaacaaataaactctaatgagaatcataaagcttgttcccagagaaccatgatacagggtgggacagtacgcaaataatgggctcctgttgtcagacttcatggtgattacattagtgctttctccagtatctttcttcctattgtactcctgaagcactcagaatgataaagataaatttctgatcattcctacaaagagtgcaggcaaagttaagatttaactgtgattgctggttgtttcatctcgaattcaaaatcctggatttccgaaacaatggagcttgatgtcacatttggctatcttgcttttgtctcctcttctggaaagaacaaatcatcttcctgaaaattacaggagacacttagtatgacaaaataaggcctctgaaactgtccaatctcacatgtaaaaagtgtaaaatcacagaactaaaatcaggttccggattttcctggaaatagaatgtcaccgggatctgttcaaaggtgagctttggctacattttataacagtgtttaaaactcgaatgcaaaaaactgctttcaatataatcagatatgtgcaaaaacaatttgttaaataacatgggaagattatattaacaaaagacatttccagaatactaacattcatgtgatttataaaggtgcattttctgtaaagagctatacagcccaaaaacatgaaattcttcaagggagtcccctttatcccatgagttggaagaatttattttcatattctatgcatggatcactgaagtgatgaatgtcactcgtcttcaagaaggaagcactctcagccttgtgaagaagaacctcaagggttcctggggctatgatcatgaagagcaccacaatgaagactgctgcgaagtctttttcacttcttcacatttgggatgtgaaatattttacagaaaaataagagtgtgcaaatccctctcacacatagaaaaacgattgtgtgaatattcttaaatttttaaaacttttaaaaactgtgatctttgcactgttttcaagagtcagcaactctgaagaaagatattcaccataagtgaccccatatggtgaagatattcacaataaatgacagttttgcaagatgactctttgggttggcattctgtttccggtcaccaggtttccgcaatctctgtgacagcccgcagcagctcggcaaatgtagggcggccttcaggtttctcatgccagcagctgtacatgacttcatatatggacattggtgccaggtgagggcgatatagcctgaagccttcagaaatagcttccacgacttgcaaatttgacttattttcaaaaggcatttttccttctgtaaaaacttcccacattaaaactccaaatgaccagacatcagatttactgctgtacttattgaaaagaaaaacttcaggaggggaccacttgattgggaacttggctccaaaagaactgacatactcatcatccaaaacgtaccttgtcattccaaagtctgaaatttttactatgcatgttgaactgaccaaacaattccttgccgccaaatccctatgaatatagccattcctctccagatattccattccttcacatatatcctggcatacactcagtagcatttccttcctaagctttcctttattctccctgagatagttaagcaggcagccattttccatgaactctgtcacaatgtaaaggggcttccgctgtatacagactccataaagttgcactagctttgaatgagataatttcatcatcactttggcctcttcaatgaaatcctcttcagacatggagccttcattgatggccttgatagctacctggatatgtgaccgccattcacctaaatggaccactccaaactgaccgcttccaatctcctttataaaagccaactcagatggatctatctcccacttttcgtagctaaacccagctgtggctggtaaacaactgcccatcagcccaactggatatcggagacgagtcatgagaccggctgcattgtgctggtgataccagattaactcagggattgattgaaaggcgtgtctttcagccacataccactgtcctgagtcattcttttttatctgataatgttttatggcagcctccgtacttcttctagctcccataaatacggaaattgtgtaggatcctaaatgtcttgaatctctgacaataaatgcaccttctttagactcttgtctcaatagatgttctgcctgatttctggtaatgtttctatggtaccactcatatatttctaaattagttattttgttttcagtcacatagttgcttgggattaagccttcattccccaaacggtctcttgccttccaccagtgaggattgtatttctccagtatcaggtattcttctgctctccttaaggctaaattacagggttctctgggcagaaaatcataaagtgccttgacttggatcttctcttcagcaacctcagagggtgggaggggaggcagtggctttcgttttgacggctgcacacggcccgtgttggattgcttcttatttgacaattggctgagccacggcctgcgacgctgggtgtatttttctggaagctcttcatctgtgctcaggcttatctgtgttctcatttgtctcatttgatggtgtctttttgttataaatagacatggtatagtgattaggaacaagagtttgaatcccagctccaccatttcatagtgtggccttgggtaagcaatgtaacctctctaatcttcaatttcctcatcgcttctgcactgaacagcaacagcagcaacagaaaac

SEQ ID NO: 13157 - RNA, 4600 nt, Homo sapiens
  source 1..4600: mol_type = other RNA
gctgggattacaggcatgagccaccacacctggccagaatgtatcatttcttgatctgagtctggttacagagatgtattcactttgccaatatcaatgatgttacatactcatgatttgtgtacttttctttatgtatgtgtgagcaaagagttaatagcaggtctgtaccatttttctcccagaactatgcctgcttgggaaattttaggtttgtcttatcccagcacgagtttcttgtaaatgacccaaattaagataaatttggaatattgggtaccagggacagacatccattttgtgcactgtgaaacctacaatctatgggacagtacatggggctgggagacctgtgaaccgtaggcctatatgactggtgggaaacccacatagaagcttctttgcatcaaggcaaacccccacataccacaacctcatccaaataccacaagctcatgcacgctctttaggcaggtgaggagggacccaagcatcatgcatgcttaatttcctgtcctgtatcctactataaagctaagcaaatttagtgctaggctaaatgctattgtatctcatcagtttgcttgccagtccaaacatgttcccaataccatggtggtaccatgtattgcacttcaataaaaagtttactaaattcctttatctattcttgccaaaaggttattttcactgattatatattccgcttggcctccaaattccttccatttttctgagcctcctcgctgtctgttgacctcctatattctcctttttaggactctacaattgacccctaaacctcctattcatttttttatgcagagctgtttaaatattgcactatctcacctcaaatgacccagagaaccctcatatcaataactaatattaagattggttgcaaaacatagttcctttccaggagaacttgtataactatctcttttttttttgacagagtctcactctgtcacccaggatagagggcagtagcacagtctcagctcaccgcaacttccacctcctgggttcaagcaattctcctgcctcagcctcccgagtagctgggattacaggcacgtgccaccacgcctggctaacttttcgtatttttagtagagacagggtttcaccatgttggccaggctgatctctaactcctgacctcagatgatccacccgcctcggcctcccaaagtgctggattacaggcatgagccattgtgcctggctgactacctcttaaggaaacttttttgtttagttagacaaagaatggtaaatctctttccacgcacattcaaaattcacacattatctggactcttagttacctaggacatacccccagttattcttgtacctaatttggtacctcaaattttcccgaggtgttaaaacaaaaggaatagagcttgcctagcaccttagaagtgctgcaccctcttagaagtgccaggcactgtcatagttgttgccctcttagaatgatttgcctctgggtgtcactctttgctctgtacctggtacaactatagtgatggcagatgctccatactcagtcctagcttttcagtgtttggctttgctgggttttttctttctttctttttgagagaaatggggacttccaagctgagtaaaacctggaaagggcaacttactgcagccatatattgatactacattatttcctatgtcataatattaacctcccttccatctgcttttgctgtttagtagtctcatgtcttcttgagctagactatcttatgtaaattcatgttatgtgaattgaggtctcagtaataacagccttctgtctttcctcaccgtaacaggagtcataggaaagggggtgtgatagtctcagaaacagcctagcatctcatacaaacttgtttctgtttttgagacagggtctcgctctatcacccaggctggagtgcagtggcacaatcatggctcactgcagccttgatctcctgggctcctgtctcagcctcccaagtagctgggactacgtgcatgcatgcaccactacacctagctttttttttcttttttcttttttcttgtaatagagataggatctcactttgttgcccaggctggtctcaaactgggctcaagttatcttcccaccttggcctcccaaagtgctgggattataggcatgagccaccacattcagcccaaacatttctgagaccactacttgaactatcaagtctcctcttgtaactgattctcattagaaataatacacatttattgaatgtcattgatatataaagataccattctttgagtgggggaaatataatttaaaagtcgcaactactgacaatcaacaaataaactctaatgagaatcataaagcttgttcccagagaaccatgatacagggtgggacagtacgcaaataatgggctcctgttgtcagacttcatggtgattacattagtgctttctccagtatctttcttcctattgtactcctgaagcactcagaatgataaagataaatttctgatcattcctacaaagagtgcaggcaaagttaagatttaactgtgattgctggttgtttcatctcgaattcaaaatcctggatttccgaaacaatggagcttgatgtcacatttggctatcttgcttttgtctcctcttctggaaagaacaaatcatcttcctgaaaattacaggagacacttagtatgacaaaataaggcctctgaaactgtccaatctcacatgtaaaaagtgtaaaatcacagaactaaaatcaggttccggattttcctggaaatagaatgtcaccgggatctgttcaaaggtgagctttggctacattttataacagtgtttaaaactcgaatgcaaaaaactgctttcaatataatcagatatgtgcaaaaacaatttgttaaataacatgggaagattatattaacaaaagacatttccagaatactaacattcatgtgatttataaaggtgcattttctgtaaagagctatacagcccaaaaacatgaaattcttcaagggagtcccctttatcccatgagttggaagaatttattttcatattctatgcatggatcactgaagtgatgaatgtcactcgtcttcaagaaggaagcactctcagccttgtgaagaagaacctcaagggttcctggggctatgatcatgaagagcaccacaatgaagactgctgcgaagtctttttcacttcttcacatttgggatgtgaaatattttacagaaaaataagagtgtgcaaatccctctcacacatagaaaaacgattgtgtgaatattcttaaatttttaaaacttttaaaaactgtgatctttgcactgttttcaagagtcagcaactctgaagaaagatattcaccataagtgaccccatatggtgaagatattcacaataaatgacagttttgcaagatgactctttgggttggcattctgtttccggtcaccaggtttccgcaatctctgtgacagcccgcagcagctcggcaaatgtagggcggccttcaggtttctcatgccagcagctgtacatgacttcatatatggacattggtgccaggtgagggcgatatagcctgaagccttcagaaatagcttccacgacttgcaaatttgacttattttcaaaaggcatttttccttctgtaaaaacttcccacattaaaactccaaatgaccagacatcagatttactgctgtacttattgaaaagaaaaacttcaggaggggaccacttgattgggaacttggctccaaaagaactgacatactcatcatccaaaacgtaccttgtcattccaaagtctgaaatttttactatgcatgttgaactgaccaaacaattccttgccgccaaatccctatgaatatagccattcctctccagatattccattccttcacatatatcctggcatacactcagtagcatttccttcctaagctttcctttattctccctgagatagttaagcaggcagccattttccatgaactctgtcacaatgtaaaggggcttccgctgtatacagactccataaagttgcactagctttgaatgagataatttcatcatcactttggcctcttcaatgaaatcctcttcagacatggagccttcattgatggccttgatagctacctggatatgtgaccgccattcacctaaatggaccactccaaactgaccgcttccaatctcctttataaaagccaactcagatggatctatctcccacttttcgtagctaaacccagctgtggctggtaaacaactgcccatcagcccaactggatatcggagacgagtcatgagaccggctgcattgtgctggtgataccagattaactcagggattgattgaaaggcgtgtctttcagccacataccactgtcctgagtcattcttttttatctgataatgttttatggcagcctccgtacttcttctagctcccataaatacggaaattgtgtaggatcctaaatgtcttgaatctctgacaataaatgcaccttctttagactgtagtcccagctactcagag

SEQ ID NO: 13158 - RNA, 4453 nt, Homo sapiens
  source 1..4453: mol_type = other RNA
gctgggattacaggcatgagccaccacacctggccagaatgtatcatttcttgatctgagtctggttacagagatgtattcactttgccaatatcaatgatgttacatactcatgatttgtgtacttttctttatgtatgtgtgagcaaagagttaatagcaggtctgtaccatttttctcccagaactatgcctgcttgggaaattttaggtttgtcttatcccagcacgagtttcttgtaaatgacccaaattaagataaatttggaatattgggtaccagggacagacatccattttgtgcactgtgaaacctacaatctatgggacagtacatggggctgggagacctgtgaaccgtaggcctatatgactggtgggaaacccacatagaagcttctttgcatcaaggcaaacccccacataccacaacctcatccaaataccacaagctcatgcacgctctttaggcaggtgaggagggacccaagcatcatgcatgcttaatttcctgtcctgtatcctactataaagctaagcaaatttagtgctaggctaaatgctattgtatctcatcagtttgcttgccagtccaaacatgttcccaataccatggtggtaccatgtattgcacttcaataaaaagtttactaaattcctttatctattcttgccaaaaggttattttcactgattatatattccgcttggcctccaaattccttccatttttctgagcctcctcgctgtctgttgacctcctatattctcctttttaggactctacaattgacccctaaacctcctattcatttttttatgcagagctgtttaaatattgcactatctcacctcaaatgacccagagaaccctcatatcaataactaatattaagattggttgcaaaacatagttcctttccaggagaacttgtataactatctcttttttttttgacagagtctcactctgtcacccaggatagagggcagtagcacagtctcagctcaccgcaacttccacctcctgggttcaagcaattctcctgcctcagcctcccgagtagctgggattacaggcacgtgccaccacgcctggctaacttttcgtatttttagtagagacagggtttcaccatgttggccaggctgatctctaactcctgacctcagatgatccacccgcctcggcctcccaaagtgctggattacaggcatgagccattgtgcctggctgactacctcttaaggaaacttttttgtttagttagacaaagaatggtaaatctctttccacgcacattcaaaattcacacattatctggactcttagttacctaggacatacccccagttattcttgtacctaatttggtacctcaaattttcccgaggtgttaaaacaaaaggaatagagcttgcctagcaccttagaagtgctgcaccctcttagaagtgccaggcactgtcatagttgttgccctcttagaatgatttgcctctgggtgtcactctttgctctgtacctggtacaactatagtgatggcagatgctccatactcagtcctagcttttcagtgtttggctttgctgggttttttctttctttctttttgagagaaatggggacttccaagctgagtaaaacctggaaagggcaacttactgcagccatatattgatactacattatttcctatgtcataatattaacctcccttccatctgcttttgctgtttagtagtctcatgtcttcttgagctagactatcttatgtaaattcatgttatgtgaattgaggtctcagtaataacagccttctgtctttcctcaccgtaacaggagtcataggaaagggggtgtgatagtctcagaaacagcctagcatctcatacaaacttgtttctgtttttgagacagggtctcgctctatcacccaggctggagtgcagtggcacaatcatggctcactgcagccttgatctcctgggctcctgtctcagcctcccaagtagctgggactacgtgcatgcatgcaccactacacctagctttttttttcttttttcttttttcttgtaatagagataggatctcactttgttgcccaggctggtctcaaactgggctcaagttatcttcccaccttggcctcccaaagtgctgggattataggcatgagccaccacattcagcccaaacatttctgagaccactacttgaactatcaagtctcctcttgtaactgattctcattagaaataatacacatttattgaatgtcattgatatataaagataccattctttgagtgggggaaatataatttaaaagtcgcaactactgacaatcaacaaataaactctaatgagaatcataaagcttgttcccagagaaccatgatacagggtgggacagtacgcaaataatgggctcctgttgtcagacttcatggtgattacattagtgctttctccagtatctttcttcctattgtactcctgaagcactcagaatgataaagataaatttctgatcattcctacaaagagtgcaggcaaagttaagatttaactgtgattgctggttgtttcatctcgaattcaaaatcctggatttccgaaacaatggagcttgatgtcacatttggctatcttgcttttgtctcctcttctggaaagaacaaatcatcttcctgaaaattacaggagacacttagtatgacaaaataaggcctctgaaactgtccaatctcacatgtaaaaagtgtaaaatcacagaactaaaatcaggttccggattttcctggaaatagaatgtcaccgggatctgttcaaaggtgagctttggctacattttataacagtgtttaaaactcgaatgcaaaaaactgctttcaatataatcagatatgtgcaaaaacaatttgttaaataacatgggaagattatattaacaaaagacatttccagaatactaacattcatgtgatttataaaggtgcattttctgtaaagagctatacagcccaaaaacatgaaattcttcaagggagtcccctttatcccatgagttggaagaatttattttcatattctatgcatggatcactgaagtgatgaatgtcactcgtcttcaagaaggaagcactctcagccttgtgaagaagaacctcaagggttcctggggctatgatcatgaagagcaccacaatgaagactgctgcgaagtctttttcacttcttcacatttgggatgtgaaatattttacagaaaaataagagtgtgcaaatccctctcacacatagaaaaacgattgtgtgaatattcttaaatttttaaaacttttaaaaactgtgatctttgcactgttttcaagagtcagcaactctgaagaaagatattcaccataagtgaccccatatggtgaagatattcacaataaatgacagttttgcaagatgactctttgggttggcattctgtttccggtcaccaggtttccgcaatctctgtgacagcccgcagcagctcggcaaatgtagggcggccttcaggtttctcatgccagcagctgtacatgacttcatatatggacattggtgccaggtgagggcgatatagcctgaagccttcagaaatagcttccacgacttgcaaatttgacttattttcaaaaggcatttttccttctgtaaaaacttcccacattaaaactccaaatgaccagacatcagatttactgctgtacttattgaaaagaaaaacttcaggaggggaccacttgattgggaacttggctccaaaagaactgacatactcatcatccaaaacgtaccttgtcattccaaagtctgaaatttttactatgcatgttgaactgaccaaacaattccttgccgccaaatccctatgaatatagccattcctctccagatattccattccttcacatatatcctggcatacactcagtagcatttccttcctaagctttcctttattctccctgagatagttaagcaggcagccattttccatgaactctgtcacaatgtaaaggggcttccgctgtatacagactccataaagttgcactagctttgaatgagataatttcatcatcactttggcctcttcaatgaaatcctcttcagacatggagccttcattgatggccttgatagctacctggatatgtgaccgccattcacctaaatggaccactccaaactgaccgcttccaatctcctttataaaagccaactcagatggatctatctcccacttttcgtagctaaacccagctgtggctggtaaacaactgcccatcagcccaactggatatcggagacgagtcatgagaccttctagctcccataaatacggaaattgtgtaggatcctaaatgtcttgaatctctgacaataaatgcaccttctttagactg

SEQ ID NO: 13159 - RNA, 5070 nt, Homo sapiens
  source 1..5070: mol_type = other RNA
gctgggattacaggcatgagccaccacacctggccagaatgtatcatttcttgatctgagtctggttacagagatgtattcactttgccaatatcaatgatgttacatactcatgatttgtgtacttttctttatgtatgtgtgagcaaagagttaatagcaggtctgtaccatttttctcccagaactatgcctgcttgggaaattttaggtttgtcttatcccagcacgagtttcttgtaaatgacccaaattaagataaatttggaatattgggtaccagggacagacatccattttgtgcactgtgaaacctacaatctatgggacagtacatggggctgggagacctgtgaaccgtaggcctatatgactggtgggaaacccacatagaagcttctttgcatcaaggcaaacccccacataccacaacctcatccaaataccacaagctcatgcacgctctttaggcaggtgaggagggacccaagcatcatgcatgcttaatttcctgtcctgtatcctactataaagctaagcaaatttagtgctaggctaaatgctattgtatctcatcagtttgcttgccagtccaaacatgttcccaataccatggtggtaccatgtattgcacttcaataaaaagtttactaaattcctttatctattcttgccaaaaggttattttcactgattatatattccgcttggcctccaaattccttccatttttctgagcctcctcgctgtctgttgacctcctatattctcctttttaggactctacaattgacccctaaacctcctattcatttttttatgcagagctgtttaaatattgcactatctcacctcaaatgacccagagaaccctcatatcaataactaatattaagattggttgcaaaacatagttcctttccaggagaacttgtataactatctcttttttttttgacagagtctcactctgtcacccaggatagagggcagtagcacagtctcagctcaccgcaacttccacctcctgggttcaagcaattctcctgcctcagcctcccgagtagctgggattacaggcacgtgccaccacgcctggctaacttttcgtatttttagtagagacagggtttcaccatgttggccaggctgatctctaactcctgacctcagatgatccacccgcctcggcctcccaaagtgctggattacaggcatgagccattgtgcctggctgactacctcttaaggaaacttttttgtttagttagacaaagaatggtaaatctctttccacgcacattcaaaattcacacattatctggactcttagttacctaggacatacccccagttattcttgtacctaatttggtacctcaaattttcccgaggtgttaaaacaaaaggaatagagcttgcctagcaccttagaagtgctgcaccctcttagaagtgccaggcactgtcatagttgttgccctcttagaatgatttgcctctgggtgtcactctttgctctgtacctggtacaactatagtgatggcagatgctccatactcagtcctagcttttcagtgtttggctttgctgggttttttctttctttctttttgagagaaatggggacttccaagctgagtaaaacctggaaagggcaacttactgcagccatatattgatactacattatttcctatgtcataatattaacctcccttccatctgcttttgctgtttagtagtctcatgtcttcttgagctagactatcttatgtaaattcatgttatgtgaattgaggtctcagtaataacagccttctgtctttcctcaccgtaacaggagtcataggaaagggggtgtgatagtctcagaaacagcctagcatctcatacaaacttgtttctgtttttgagacagggtctcgctctatcacccaggctggagtgcagtggcacaatcatggctcactgcagccttgatctcctgggctcctgtctcagcctcccaagtagctgggactacgtgcatgcatgcaccactacacctagctttttttttcttttttcttttttcttgtaatagagataggatctcactttgttgcccaggctggtctcaaactgggctcaagttatcttcccaccttggcctcccaaagtgctgggattataggcatgagccaccacattcagcccaaacatttctgagaccactacttgaactatcaagtctcctcttgtaactgattctcattagaaataatacacatttattgaatgtcattgatatataaagataccattctttgagtgggggaaatataatttaaaagtcgcaactactgacaatcaacaaataaactctaatgagaatcataaagcttgttcccagagaaccatgatacagggtgggacagtacgcaaataatgggctcctgttgtcagacttcatggtgattacattagtgctttctccagtatctttcttcctattgtactcctgaagcactcagaatgataaagataaatttctgatcattcctacaaagagtgcaggcaaagttaagatttaactgtgattgctggttgtttcatctcgaattcaaaatcctggatttccgaaacaatggagcttgatgtcacatttggctatcttgcttttgtctcctcttctggaaagaacaaatcatcttcctgaaaattacaggagacacttagtatgacaaaataaggcctctgaaactgtccaatctcacatgtaaaaagtgtaaaatcacagaactaaaatcaggttccggattttcctggaaatagaatgtcaccgggatctgttcaaaggtgagctttggctacattttataacagtgtttaaaactcgaatgcaaaaaactgctttcaatataatcagatatgtgcaaaaacaatttgttaaataacatgggaagattatattaacaaaagacatttccagaatactaacattcatgtgatttataaaggtgcattttctgtaaagagctatacagcccaaaaacatgaaattcttcaagggagtcccctttatcccatgagttggaagaatttattttcatattctatgcatggatcactgaagtgatgaatgtcactcgtcttcaagaaggaagcactctcagccttgtgaagaagaacctcaagggttcctggggctatgatcatgaagagcaccacaatgaagactgctgcgaagtctttttcacttcttcacatttgggatgtgaaatattttacagaaaaataagagtgtgcaaatccctctcacacatagaaaaacgattgtgtgaatattcttaaatttttaaaacttttaaaaactgtgatctttgcactgttttcaagagtcagcaactctgaagaaagatattcaccataagtgaccccatatggtgaagatattcacaataaatgacagttttgcaagatgactctttgggttggcattctgtttccggtcaccaggtttccgcaatctctgtgacagcccgcagcagctcggcaaatgtagggcggccttcaggtttctcatgccagcagctgtacatgacttcatatatggacattggtgccaggtgagggcgatatagcctgaagccttcagaaatagcttccacgacttgcaaatttgacttattttcaaaaggcatttttccttctgtaaaaacttcccacattaaaactccttgtcattccaaagtctgaaatttttactatgcatgttgaactgaccaaacaattccttgccgccaaatccctatgaatatagccattcctctccagatattccattccttcacatatatcctggcatacactcagtagcatttccttcctaagctttcctttattctccctgagatagttaagcaggcagccattttccatgaactctgtcacaatgtaaaggggcttccgctgtatacagactccataaagttgcactagctttgaatgagataatttcatcatcactttggcctcttcaatgaaatcctcttcagacatggagccttcattgatggccttgatagctacctggatatgtgaccgccattcacctaaatggaccactccaaactgaccgcttccaatctcctttataaaagccaactcagatggatctatctcccacttttcgtagctaaacccagctgtggctggtaaacaactgcccatcagcccaactggatatcggagacgagtcatgagaccggctgcattgtgctggtgataccagattaactcagggattgattgaaaggcgtgtctttcagccacataccactgtcctgagtcattcttttttatctgataatgttttatggcagcctccgtacttcttctagctcccataaatacggaaattgtgtaggatcctaaatgtcttgaatctctgacaataaatgcaccttctttagactcttgtctcaatagatgttctgcctgatttctggtaatgtttctatggtaccactcatatatttctaaattagttattttgttttcagtcacatagttgcttgggattaagccttcattccccaaacggtctcttgccttccaccagtgaggattgtatttctccagtatcaggtattcttctgctctccttaaggctaaattacagggttctctgggcagaaaatcataaagtgccttgacttggatcttctcttcagcaacctcagagggtgggaggggaggcagtggctttcgttttgacggctgcacacggcccgtgttggattgcttcttatttgacaattggctgagccacggcctgcgacgctgggtgtatttttctggaagctcttcatctgtgctcaggcttatctgtgttctcatttgtctcatttgatggtgtctttttgttataaatagacatggtatagtgattaggaacaagagtttgaatcccagctccaccatttcatagtgtggccttgggtaagcaatgtaacctctctaatcttcaatttcctcatcgcttctgcactgaacagcaacagcagcaacagaaaaccgactgg

SEQ ID NO: 13160 - RNA, 2112 nt, Homo sapiens
  source 1..2112: mol_type = other RNA
gctgggattacaggcatgagccaccacacctggccagctcttgggttttctacttgaacagatagtctctgatttgttacaccttccagggacctcagccttcccctcatctgtccgcccaggtttcaagtaacgggagagattcctgcaaaactttcctgagaattgacggaatgacagaggtggagaccaggaggtggactcaggaccttcctatggtcctgggtcccctccccaccaagggtggagggccgaggacacaaaaaggcctgctcccaagaccccacttgcaaaggagcagatgcacggtcacacacacatagacccaagcagaggctctgtggggagaggggtgtgccaggcatgcgcaggtggtgtgggcaggggaaggctgggagaagcagcaaataaattccccaggaatcttccccagggctggactcagcccagcaagtagactggggtgcctgggcgttgggtggacctacctgtagcttcctcattccctcccaccccaccccatccccgccaagtcccagaggatcaacccactcagggcaccccacccaagaaataaaatcttccccagtacaaaaggctcctaagccacggtaagtggcacctaggagagggacagagggaggaagggtatggagtggacaagggggcctgatcccctccctggccagaagcaaggtccaggcatgggcaagggtgtcatctgggttcccttggctcctctcagatctcagtcagggcgtcgactggcaccaggccccgcttcttgccactgctgacgcggatgaagccgtcagcatccttgcttctgcccacgcccacgcagatctggttctccttgaggctcatgtaaccctgttccttgttcccggagaagggttggcagcagcgccaaacattctcgcctggcctcacccgttgcacaaaattagctgggaagaagccaacccggtcgccgatcttgccctgctgtccaggactcttctcctctggtcctggcccttcactctctgctggggctgtgaatactggagatgcactgtcaccaggcccctcctcagagctgcggatgctgccttccccatcctcggtcagctcatcccgctcactcaggctccttgtcggggactcagaggtgctgctgaaactggagcggttcatcagtgccagggaggtgccatagcgcagggtctcgtagacagggtccaccttcccactgtccccagtgggtggggactctttgcttgtggcacagactggtggcggctcatgcaccaggagaggggaactgaagttgcggcggaaggaggtggacgtcttgcctgggcattgctggtgggagatctcctcagagcaccagaggtggacgctgactttgcacatcttacatcgcaagccctgtttggagtttcctacgatgagctggtggcacagctcacaagggctagctcgcttgaagacatgttcctggaagctgtgcagcctcactggtttgagcgctgccagggggcgtgggactgggcatggggagggggatggggtagccaggcccctgtccgaggctgtgggtggtggggagggagggggcagtggggttgggggcgtcagcagcacctcggtggggcacttgagctcagagcccgagcgaaggaagaagttctccaagctcttacttcggaggatggtcttgagggagagggagcgcttgaatcgctggagcttggtttcctggagggcggagacggtccctggggggctgtgggtggccgcgtcatccggttcgttctccttctcgctcatctcggtcatggttcggggagaggggaggagagggtgccgagatccgacggcaggcccaccgcgggcaggctgcgggtggcgggcgtctccgggactctgaagccgttctccagaggctgcccccagttagcccccggcacggcagcccccaacccgcgggagcgggcagagaaagttgccggggtggcgggcgaggggaggccaccacgctgagccgcaggagcgggacgaccccgggcgcgaggaccgagggtctgcagaggatgctgctcgcagcgcggggaggagggaagt

SEQ ID NO: 13161 - RNA, 2277 nt, Homo sapiens
  source 1..2277: mol_type = other RNA
gctgggattacaggcatgagccaccacacctggccagctcttgggttttctacttgaacagatagtctctgatttgttacaccttccagggacctcagccttcccctcatctgtccgcccaggtttcaagtaacgggagagattcctgcaaaactttcctgagaattgacggaatgacagaggtggagaccaggaggtggactcaggaccttcctatggtcctgggtcccctccccaccaagggtggagggccgaggacacaaaaaggcctgctcccaagaccccacttgcaaaggagcagatgcacggtcacacacacatagacccaagcagaggctctgtggggagaggggtgtgccaggcatgcgcaggtggtgtgggcaggggaaggctgggagaagcagcaaataaattccccaggaatcttccccagggctggactcagcccagcaagtagactggggtgcctgggcgttgggtggacctacctgtagcttcctcattccctcccaccccaccccatccccgccaagtcccagaggatcaacccactcagggcaccccacccaagaaataaaatcttccccagtacaaaaggctcctaagccacggtaagtggcacctaggagagggacagagggaggaagggtatggagtggacaagggggcctgatcccctccctggccagaagcaaggtccaggcatgggcaagggtgtcatctgggttcccttggctcctctcagatctcagtcagggcgtcgactggcaccaggccccgcttcttgccactgctgacgcggatgaagccgtcagcatccttgcttctgcccacgcccacgcagatctggttctccttgaggctcatgtaaccctgttccttgttcccggagaagggttggcagcagcgccaaacattctcgcctggcctcacccgttgcacaaaattagctgggaagaagccaacccggtcgccgatcttgcccttccaccagtcctcgttagagtcatccaccagcatgatccgatctccaggcctggggaggacagagtgcagagccagatcattgttctcctggggcagaaacttgtagagtgcaacgtaggagtacatgggccccacatccttccgcagggtggctttggggagctgctgtccaggactcttctcctctggtcctggcccttcactctctgctggggctgtgaatactggagatgcactgtcaccaggcccctcctcagagctgcggatgctgccttccccatcctcggtcagctcatcccgctcactcaggctccttgtcggggactcagaggtgctgctgaaactggagcggttcatcagtgccagggaggtgccatagcgcagggtctcgtagacagggtccaccttcccactgtccccagtgggtggggactctttgcttgtggcacagactggtggcggctcatgcaccaggagaggggaactgaagttgcggcggaaggaggtggacgtcttgcctgggcattgctggtgggagatctcctcagagcaccagaggtggacgctgactttgcacatcttacatcgcaagccctgtttggagtttcctacgatgagctggtggcacagctcacaagggctagctcgcttgaagacatgttcctggaagctgtgcagcctcactggtttgagcgctgccagggggcgtgggactgggcatggggagggggatggggtagccaggcccctgtccgaggctgtgggtggtggggagggagggggcagtggggttgggggcgtcagcagcacctcggtggggcacttgagctcagagcccgagcgaaggaagaagttctccaagctcttacttcggaggatggtcttgagggagagggagcgcttgaatcgctggagcttggtttcctggagggcggagacggtccctggggggctgtgggtggccgcgtcatccggttcgttctccttctcgctcatctcggtcatggttcggggagaggggaggagagggtgccgagatccgacggcaggcccaccgcgggcaggctgcgggtggcgggcgtctccgggactctgaagccgttctccagaggctgcccccagttagcccccggcacggcagcccccaacccgcgggagcgggcagagaaagttgccggggtggcgggcgaggggaggccaccacgctgagccgcaggagcgggacgaccccgggcgcgaggaccgagggtctgcagaggatgctgctcgcagcgcggggaggagggaagt

SEQ ID NO: 13162 - RNA, 2420 nt, Homo sapiens
  source 1..2420: mol_type = other RNA
gctgggattacaggcatgagccaccacacctggccagctcttgggttttctacttgaacagatagtctctgatttgttacaccttccagggacctcagccttcccctcatctgtccgcccaggtttcaagtaacgggagagattcctgcaaaactttcctgagaattgacggaatgacagaggtggagaccaggaggtggactcaggaccttcctatggtcctgggtcccctccccaccaagggtggagggccgaggacacaaaaaggcctgctcccaagaccccacttgcaaaggagcagatgcacggtcacacacacatagacccaagcagaggctctgtggggagaggggtgtgccaggcatgcgcaggtggtgtgggcaggggaaggctgggagaagcagcaaataaattccccaggaatcttccccagggctggactcagcccagcaagtagactggggtgcctgggcgttgggtggacctacctgtagcttcctcattccctcccaccccaccccatccccgccaagtcccagaggatcaacccactcagggcaccccacccaagaaataaaatcttccccagtacaaaaggctcctaagccacggtaagtggcacctaggagagggacagagggaggaagggtatggagtggacaagggggcctgatcccctccctggccagaagcaaggtccaggcatgggcaagggtgtcatctgggttcccttggctcctctcagatctcagtcagggcgtcgactggcaccaggccccgcttcttgccactgctgacgcggatgaagccgtcagcatccttgcttctgcccacgcccacgcagatctggttctccttgaggctcatgtaaccctgttccttgttcccggagaagggttggcagcagcgccaaacattctcgcctggcctcacccgttgcacaaaattagctgggaagaagccaacccggtcgccgatcttgcccttccaccagtcctcgttagagtcatccaccagcatgatccgatctccaggctgcagagccagatcattgttctcctggggcagaaacttgtagagtgcaacgtaggagtacatgggccccacatccttccgcagggtggctttggggagctgctgtccaggactcttctcctctggtcctggcccttcactctctgctggggctgtgaatactggagatgcactgtcaccaggcccctcctcagagctgcggatgctgccttccccatcctcggtcagctcatcccgctcactcaggctccttgtcggggactcagaggtgctgctgaaactggagcggttcatcagtgccagggaggtgccatagcgcagggtctcgtagacagggtccaccttcccactgtccccagtgggtggggactctttgcttgtggcacagactggtggcggctcatgcaccaggagaggggaactgaagttgcggcggaaggaggtggacgtcttgcctgggcattgctggtgggagatctcctcagagcaccagaggtggacgctgactttgcacatcttacatcgcaagccctgtttggagtttcctacgatgagctggtggcacagctcacaagggctagctcgcttgaagacatgttcctggaagctgtgcagcctcactggtttgagcgctgccagggggcgtgggactgggcatggggagggggatggggtagccaggcccctgtccgaggctgtgggtggtggggagggagggggcagtggggttgggggcgtcagcagcacctcggtggggcacttgagctcagagcccgagcgaaggaagaagttctccaagctcttacttcggaggatggtcttgagggagagggagcgcttgaatcgctggagcttggtttcctggagggcggagacggtccctggggggctgtgggtggccgcgtcatccggttcgttctccttctcgctcatctcggtcatggttcggggagaggggaggagagggtgccgagatccgacggcaggcccaccgcgggcaggctgcgggtggcgggcgtctccgggactctgaagccgttctccagaggctgcccccagttagcccccggcacggcagcccccaacccgcgggagcgggcagagaaagttgccggggtggcgggcgaggggaggccaccacgctgagccgcaggagcgggacgaccccgggcgcgaggaccgagggtctgcagaggatgctgctcgcagcgcggggaggagggaagtggggccgcggggatgagccgagggagggagccaaggagctgtccgtgtccagccggctccgccgtccgctgcgcccgccccccatcccctcccctcccccgccggccccagcccggcacccggcggcccctccgcccagtcctcgccgcccaactttg

SEQ ID NO: 13163 - RNA, 2218 nt, Homo sapiens
  source 1..2218: mol_type = other RNA
gctgggattacaggcatgagccaccacacctggccagctcttgggttttctacttgaacagatagtctctgatttgttacaccttccagggacctcagccttcccctcatctgtccgcccaggtttcaagtaacgggagagattcctgcaaaactttcctgagaattgacggaatgacagaggtggagaccaggaggtggactcaggaccttcctatggtcctgggtcccctccccaccaagggtggagggccgaggacacaaaaaggcctgctcccaagaccccacttgcaaaggagcagatgcacggtcacacacacatagacccaagcagaggctctgtggggagaggggtgtgccaggcatgcgcaggtggtgtgggcaggggaaggctgggagaagcagcaaataaattccccaggaatcttccccagggctggactcagcccagcaagtagactggggtgcctgggcgttgggtggacctacctgtagcttcctcattccctcccaccccaccccatccccgccaagtcccagaggatcaacccactcagggcaccccacccaagaaataaaatcttccccagtacaaaaggctcctaagccacggtaagtggcacctaggagagggacagagggaggaagggtatggagtggacaagggggcctgatcccctccctggccagaagcaaggtccaggcatgggcaagggtgtcatctgggttcccttggctcctctcagatctcagtcagggcgtcgactggcaccaggccccgcttcttgccactgctgacgcggatgaagccgtcagcatccttgcttctgcccacgcccacgcagatctggttctccttgaggctcatgtaaccctgttccttgttcccggagaagggttggcagcagcgccaaacattctcgcctggcctcacccgttgcacaaaattagctgggaagaagccaacccggtcgccgatcttgcccttccaccagtcctcgttagagtcatccaccagcatgatccgatctccaggctgcagagccagatcattgttctcctggggcagaaacttgtagagtgcaacgtaggagtacatgggccccacatccttccgcagggtggctttggggagctgctgtccaggactcttctcctctggtcctggcccttcactctctgctggggctgtgaatactggagatgcactgtcaccaggcccctcctcagagctgcggatgctgccttccccatcctcggtcagctcatcccgctcactcaggctccttgtcggggactcagaggtgctgctgaaactggagcggttcatcagtgccagggaggtgccatagcgcagggtctcgtagacagggtccaccttcccactgtccccagtgggtggggactctttgcttgtggcacagactggtggcggctcatgcaccaggagaggggaactgaagttgcggcggaaggaggtggacgtcttgcctgggcattgctggtgggagatctcctcagagcaccagaggtggacgctgactttgcacatcttacatcgcaagccctgtttggagtttcctcggtggggcacttgagctcagagcccgagcgaaggaagaagttctccaagctcttacttcggaggatggtcttgagggagagggagcgcttgaatcgctggagcttggtttcctggagggcggagacggtccctggggggctgtgggtggccgcgtcatccggttcgttctccttctcgctcatctcggtcatggttcggggagaggggaggagagggtgccgagatccgacggcaggcccaccgcgggcaggctgcgggtggcgggcgtctccgggactctgaagccgttctccagaggctgcccccagttagcccccggcacggcagcccccaacccgcgggagcgggcagagaaagttgccggggtggcgggcgaggggaggccaccacgctgagccgcaggagcgggacgaccccgggcgcgaggaccgagggtctgcagaggatgctgctcgcagcgcggggaggagggaagtggggccgcggggatgagccgagggagggagccaaggagctgtccgtgtccagccggctccgccgtccgctgcgcccgccccccatcccctcccctcccccgccggccccagcccggcacccggcggcccctccgcccagtcctcgccgcccaactttg

SEQ ID NO: 13164 - RNA, 2210 nt, Homo sapiens
  source 1..2210: mol_type = other RNA
gctgggattacaggcatgagccaccacacctggccagctcttgggttttctacttgaacagatagtctctgatttgttacaccttccagggacctcagccttcccctcatctgtccgcccaggtttcaagtaacgggagagattcctgcaaaactttcctgagaattgacggaatgacagaggtggagaccaggaggtggactcaggaccttcctatggtcctgggtcccctccccaccaagggtggagggccgaggacacaaaaaggcctgctcccaagaccccacttgcaaaggagcagatgcacggtcacacacacatagacccaagcagaggctctgtggggagaggggtgtgccaggcatgcgcaggtggtgtgggcaggggaaggctgggagaagcagcaaataaattccccaggaatcttccccagggctggactcagcccagcaagtagactggggtgcctgggcgttgggtggacctacctgtagcttcctcattccctcccaccccaccccatccccgccaagtcccagaggatcaacccactcagggcaccccacccaagaaataaaatcttccccagtacaaaaggctcctaagccacggtaagtggcacctaggagagggacagagggaggaagggtatggagtggacaagggggcctgatcccctccctggccagaagcaaggtccaggcatgggcaagggtgtcatctgggttcccttggctcctctcagatctcagtcagggcgtcgactggcaccaggccccgcttcttgccactgctgacgcggatgaagccgtcagcatccttgcttctgcccacgcccacgcagatctggttctccttgaggctcatgtaaccctgttccttgttcccggagaagggttggcagcagcgccaaacattctcgcctggcctcacccgttgcacaaaattagctgggaagaagccaacccggtcgccgatcttgcctgcagagccagatcattgttctcctggggcagaaacttgtagagtgcaacgtaggagtacatgggccccacatccttccgcagggtggctttggggagctgctgtccaggactcttctcctctggtcctggcccttcactctctgctggggctgtgaatactggagatgcactgtcaccaggcccctcctcagagctgcggatgctgccttccccatcctcggtcagctcatcccgctcactcaggctccttgtcggggactcagaggtgctgctgaaactggagcggttcatcagtgccagggaggtgccatagcgcagggtctcgtagacagggtccaccttcccactgtccccagtgggtggggactctttgcttgtggcacagactggtggcggctcatgcaccaggagaggggaactgaagttgcggcggaaggaggtggacgtcttgcctgggcattgctggtgggagatctcctcagagcaccagaggtggacgctgactttgcacatcttacatcgcaagccctgtttggagtttcctacgatgagctggtggcacagctcacaagggctagctcgcttgaagacatgttcctggaagctgtgcagcctcactggtttgagcgctgccagggggcgtgggactgggcatggggagggggatggggtagccaggcccctgtccgaggctgtgggtggtggggagggagggggcagtggggttgggggcgtcagcagcacctcggtggggcacttgagctcagagcccgagcgaaggaagaagttctccaagctcttacttcggaggatggtcttgagggagagggagcgcttgaatcgctggagcttggtttcctggagggcggagacggtccctggggggctgtgggtggccgcgtcatccggttcgttctccttctcgctcatctcggtcatggttcggggagaggggaggagagggtgccgagatccgacggcaggcccaccgcgggcaggctgcgggtggcgggcgtctccgggactctgaagccgttctccagaggctgcccccagttagcccccggcacggcagcccccaacccgcgggagcgggcagagaaagttgccggggtggcgggcgaggggaggccaccacgctgagccgcaggagcgggacgaccccgggcgcgaggaccgagggtctgcagaggatgctgctcgcagcgcggggaggagggaagt

SEQ ID NO: 13165 - RNA, 5524 nt, Homo sapiens
  source 1..5524: mol_type = other RNA
gctgggattacaggcatgagccaccacacctggccaggaattagatctcagatttcaaaatacttccaacttctataaagaactcaatagctaattgttgacttgtaagtcaaggaagtagaattatatacaagatttaaaaacatacacacagagggttcaataatctggtatggatgggacacagaaaacagaattgtagatcgggcgcagtggctcatgcctgtaatcccagcactttaggaggccgaggtgggcggaacacgagatcaagagatcgagaccatcctggccaacatggtgaaaccctgtctctactaaaaatgcaaaaattagccgggcgtggtggcgctcacctattaaaaaaggtaattgtatcttttctgaaaaatgtttaaaaaaagaaaaaattgtttttttacccttttcatttattcttggcaaataatgccacgtggcaattttactttcacatcttcaccagtgcatcattttaaaaaagcaataatcagcctctcaaaataatggcataaataaaaatgtataggcatagtgcaaatcccacaactttaacccaactacttcctctatatttatgggaacaaaactaagtgacactttacaaagccaaacaatgagaagagaatcatctgggtagcttgattctcttgctgaaggagaccacagcatggactctggattccaattctgatttgccactcactagctatgagtcctgaataagttctctatacctgttttcttaacatgggaagaaagtatacattttgtacgattcttcgggagattgaagaggcaaatgtacacaaaagtatctggtgcatgccaattagtattaagtttcctgttcttttctcatttggcactgttgttttctcttctccagttccttccgataccaatttcaaaaaagtattcctctcacttttttcccactagttttcttcttcttcttcttttttttttttaaatttgagatggagtgtcgctttgtcgcccaggctggagtgtaatggtgcgatcttggctcactgcaacctctgcctcccaggttcaagccattcccctgcctcagcctctgagtagctgggattacaggtgcacgccaccacacccaggtaatttttgtatttttagtagagacggggtttcaccatgttgctcaggctggcctcgatctcctgaccttaggtgatctgcccacctccgcctcccaaagtgttgggattacaggcatgagccaccgcgcccggccttcctggtagtttccattccatctccctgtatttttctcttatcactctcgaagtctatctttcttgttcttttcctccctagctttttttttttaaacactcctttcaagctgtgtccaacacccacaaggaatgactatttttaactaatcttactgacctcatttaatctattcaataaaacctctgccctaaggagcaaagaaacttgcagaggaagtaaggcaaactggaagaagcatactgtcagcggattaaattcttgagcaaggcaatactccttatggattcttcccatgtacaatccgtaactcttcccatgggcctttatatcaaccctaagataattacactcctgcctcaaaataaaataaaataaaacccaccacatcttgtattgtagacatcccagctgcatgttaagctgagtgaaagtaccatgctgtcttttaaatcactttatatctacttaatcatcccacagtaacccgagttgaagaagttactttggtttctcataaatgaatatgcacgtgctgaacatatcggaaagaaccacaccctctcactgatgaacacgttggcagttctcccaactgttttatcaagagaagctagaaggtaaagaaaaggaaacagagccctataggaaaaatgattgacttcacacgtttgagcgatttgggcttcagctatgactttgctggagtacagatgggtgccatcagagcacaaagctgagcaaacctctcttcttaccctgtgccctccctgaatttttggatttctgagcttgtctactaccaacaaatgttttaccctccagtgcacctttgacagtatacagctctatttttcaaacggcaagtatgttatccaagttcagagatgcaactgaggaattaacatgaaaaccatctttcactcaataaatcagaagctgctagttaagtaagcctcaagaacctaagaaaaaacaccaaagtgtaagtattactcagtcaccaatctaaagacagaactttgactcaaggtagaaatgaaaccgtaattatataaatatatttataaatatttatacaattatatacttatacataagcacttacacagacttagaaaaaaatttaagaacattaattcaaaaggactcactgaagaataaacagatttttccatgatttccttgaggagatataaaactcattctttagggagagttcctcaaaattcaaccattagaaaccatatcctataactgtgtactagcaacacatggcatctttttttcttcttttcccaaatcccctaattgccaagagagcaatcttaaagtagatgaaaacctaaaggtctctacgcaacatctgaggaacatacgctcctcagataaaagaatcaatctaaatcctcaactgacaaaaaggtccatttaatatttttcattttacaagttaaaagttctagttttgccaccagaatcacgactacccccccttcagaggactccatttaagctcaaaatacgaaatgagcatagggtgaagttgatgtgtaaatggtattctacagattcaagatggcctcttctaaaaacactgaagaaagctttcaccaactctaatttgattttgggttttgttggcagaaaaagcccaagacatctgaaaattactagtaacctccgccatcctccttactaaatgttgtcttctgaatggagttgaaaggtcttccccttagagaggctttccgttttgataccttttgaaagaaaacagcatgcggactcatgttcaattcagtcaccagagccttttagagactattccaaccaggggcaaaaaatgaaccattatttctaaccaaaagaacatggttagcaactctcagctgaatggttttctttttccccagggacatacctaagtatgcctgaaacaacacaggacaatcaataaccatagtggttacaattccaagccattgtactacatgattattgaccagctgccttcctacagatcactgcagactcagacaatggagggctccaaaggaactaatatgctgtgctggcaaaaatagcaagcaccttcctatcccagtcaccacgataggttcacttcatgtccattcttggactagcaggatcaatacagagtaataaggaaaactgtctcaggttaggacaatgaaagtcaccccatgctatatgctccatatttaacactcattctgccaataacacatgtcatggaaatagtccttatagctgggaacatgaaaatcctttgaaaaaggtttttaagtatgatgagcaatcattacaagggatgctttttccacgtaaacaaaagcctggatattttgttaagcgacatttccacatgaagaacacaacaaaaccaaacccatgttagagaatttcttctccctgctaaacacggggacttacaaaaaagggagggttgttcttactctgaatctagccattcctttgcccgaagagtctggggagtaacgttaacatttgatcccaaaaaagtgccgtgcaagagaccacttactggaacacacaattcctgctgctagtactaggagaggtcttatccttacacttcagtttggtcaccagattaggtaagaaagaaaagtgtggggggagggggaggcagaagggtacggagtggggagcgagaaaacagaagaggagaaagaaacaaagggggagaaagagactgattataggagagatcaagaaataagagaaggaaggtgacttgcttgcccaactttggctctgtggtcctatgagccaaaatgcatacttagtgacatgtatctcacaggaaaagggaaaaaaggggtaagctgagagaggtcaagccatggtgttaatttctttcctgtacaaagacagtctcttgaggacaaaggcctgcctcttgcaatgtaatatcatagtccagatgagataatttccttcgaggaaagttggtgagaagttcaaaacgttcatttgggtatcctttagactgcacgtgcttcaccaaagctagcagtttagcttgctctggaagagtgatctgttccctttttccatctggataccgcaacatcagctgtgcttttggtccatttacatctatcccctccactactccatctgctttttcaggtggcatctccagtatctctgaatccacagctggcaatccttggtggtttgtggctgttccaggatcagttctgactggtggctcagtcagcggccttctattctcctcttttctatgccccaaatctttgtggggagactttctggacttggcaagattctctacctcttcttcttcatcagagccacaaacggatatgaactcctcactgccagaaaaaagttcagattcagattcttcatctgagcggctatcctgttttgtctgtgttgaatcaaaatgtgtttcttgtaaggaggctctgatggcagcttctagctggctgtcttcacttgcatctataaggctctctgaacgggcacattttttggggggactgctagaaagtccatccagttgtccatgttcacccagaaatcccgtcacttggtccaagaaagaagatacatctaactggtgccattctactagcttctgacctgtccgtgggtccaatatggaaacataggggaaatcccctaacttataaaactgtatgtatctctgaccttcctcactgtcatgataaacctgccagaaaatgaaatgttcccggataatattcttcacagcttcgttgctccacacatcgcggttgaggcactgacatgcaaagtcttgaacattttgaatgtttatcatcagccacttattttgcatctggccacactctttggctgtttcaaagctgcctttatgcatcaaatcaatgggtggccggaatagatctgcaagggtagttaatttcttatcgatagctcctccatttcttaattcttgttcttgccgaatagtttcagtctgaaaatcccggaaaccatcaaaaattgaacgtgcaggccgtcgtcttttaggagcaccaaataatggttctggttccaccagtatttcctgcttttgaggaattggggcacgaacttcttctcggtaatggtggtgaactgttgaattaaccccttcagcgccgaggacgccgcggagcccccgtgggcagccatcttaccgccgccgccgccgccgaacaac

SEQ ID NO: 13166 - RNA, 5667 nt, Homo sapiens
  source 1..5667: mol_type = other RNA
gctgggattacaggcatgagccaccacacctggccaggaattagatctcagatttcaaaatacttccaacttctataaagaactcaatagctaattgttgacttgtaagtcaaggaagtagaattatatacaagatttaaaaacatacacacagagggttcaataatctggtatggatgggacacagaaaacagaattgtagatcgggcgcagtggctcatgcctgtaatcccagcactttaggaggccgaggtgggcggaacacgagatcaagagatcgagaccatcctggccaacatggtgaaaccctgtctctactaaaaatgcaaaaattagccgggcgtggtggcgctcacctattaaaaaaggtaattgtatcttttctgaaaaatgtttaaaaaaagaaaaaattgtttttttacccttttcatttattcttggcaaataatgccacgtggcaattttactttcacatcttcaccagtgcatcattttaaaaaagcaataatcagcctctcaaaataatggcataaataaaaatgtataggcatagtgcaaatcccacaactttaacccaactacttcctctatatttatgggaacaaaactaagtgacactttacaaagccaaacaatgagaagagaatcatctgggtagcttgattctcttgctgaaggagaccacagcatggactctggattccaattctgatttgccactcactagctatgagtcctgaataagttctctatacctgttttcttaacatgggaagaaagtatacattttgtacgattcttcgggagattgaagaggcaaatgtacacaaaagtatctggtgcatgccaattagtattaagtttcctgttcttttctcatttggcactgttgttttctcttctccagttccttccgataccaatttcaaaaaagtattcctctcacttttttcccactagttttcttcttcttcttcttttttttttttaaatttgagatggagtgtcgctttgtcgcccaggctggagtgtaatggtgcgatcttggctcactgcaacctctgcctcccaggttcaagccattcccctgcctcagcctctgagtagctgggattacaggtgcacgccaccacacccaggtaatttttgtatttttagtagagacggggtttcaccatgttgctcaggctggcctcgatctcctgaccttaggtgatctgcccacctccgcctcccaaagtgttgggattacaggcatgagccaccgcgcccggccttcctggtagtttccattccatctccctgtatttttctcttatcactctcgaagtctatctttcttgttcttttcctccctagctttttttttttaaacactcctttcaagctgtgtccaacacccacaaggaatgactatttttaactaatcttactgacctcatttaatctattcaataaaacctctgccctaaggagcaaagaaacttgcagaggaagtaaggcaaactggaagaagcatactgtcagcggattaaattcttgagcaaggcaatactccttatggattcttcccatgtacaatccgtaactcttcccatgggcctttatatcaaccctaagataattacactcctgcctcaaaataaaataaaataaaacccaccacatcttgtattgtagacatcccagctgcatgttaagctgagtgaaagtaccatgctgtcttttaaatcactttatatctacttaatcatcccacagtaacccgagttgaagaagttactttggtttctcataaatgaatatgcacgtgctgaacatatcggaaagaaccacaccctctcactgatgaacacgttggcagttctcccaactgttttatcaagagaagctagaaggtaaagaaaaggaaacagagccctataggaaaaatgattgacttcacacgtttgagcgatttgggcttcagctatgactttgctggagtacagatgggtgccatcagagcacaaagctgagcaaacctctcttcttaccctgtgccctccctgaatttttggatttctgagcttgtctactaccaacaaatgttttaccctccagtgcacctttgacagtatacagctctatttttcaaacggcaagtatgttatccaagttcagagatgcaactgaggaattaacatgaaaaccatctttcactcaataaatcagaagctgctagttaagtaagcctcaagaacctaagaaaaaacaccaaagtgtaagtattactcagtcaccaatctaaagacagaactttgactcaaggtagaaatgaaaccgtaattatataaatatatttataaatatttatacaattatatacttatacataagcacttacacagacttagaaaaaaatttaagaacattaattcaaaaggactcactgaagaataaacagatttttccatgatttccttgaggagatataaaactcattctttagggagagttcctcaaaattcaaccattagaaaccatatcctataactgtgtactagcaacacatggcatctttttttcttcttttcccaaatcccctaattgccaagagagcaatcttaaagtagatgaaaacctaaaggtctctacgcaacatctgaggaacatacgctcctcagataaaagaatcaatctaaatcctcaactgacaaaaaggtccatttaatatttttcattttacaagttaaaagttctagttttgccaccagaatcacgactacccccccttcagaggactccatttaagctcaaaatacgaaatgagcatagggtgaagttgatgtgtaaatggtattctacagattcaagatggcctcttctaaaaacactgaagaaagctttcaccaactctaatttgattttgggttttgttggcagaaaaagcccaagacatctgaaaattactagtaacctccgccatcctccttactaaatgttgtcttctgaatggagttgaaaggtcttccccttagagaggctttccgttttgataccttttgaaagaaaacagcatgcggactcatgttcaattcagtcaccagagccttttagagactattccaaccaggggcaaaaaatgaaccattatttctaaccaaaagaacatggttagcaactctcagctgaatggttttctttttccccagggacatacctaagtatgcctgaaacaacacaggacaatcaataaccatagtggttacaattccaagccattgtactacatgattattgaccagctgccttcctacagatcactgcagactcagacaatggagggctccaaaggaactaatatgctgtgctggcaaaaatagcaagcaccttcctatcccagtcaccacgataggttcacttcatgtccattcttggactagcaggatcaatacagagtaataaggaaaactgtctcaggttaggacaatgaaagtcaccccatgctatatgctccatatttaacactcattctgccaataacacatgtcatggaaatagtccttatagctgggaacatgaaaatcctttgaaaaaggtttttaagtatgatgagcaatcattacaagggatgctttttccacgtaaacaaaagcctggatattttgttaagcgacatttccacatgaagaacacaacaaaaccaaacccatgttagagaatttcttctccctgctaaacacggggacttacaaaaaagggagggttgttcttactctgaatctagccattcctttgcccgaagagtctggggagtaacgttaacatttgatcccaaaaaagtgccgtgcaagagaccacttactggaacacacaattcctgctgctagtactaggagaggtcttatccttacacttcagtttggtcaccagattaggtaagaaagaaaagtgtggggggagggggaggcagaagggtacggagtggggagcgagaaaacagaagaggagaaagaaacaaagggggagaaagagactgattataggagagatcaagaaataagagaaggaaggtgacttgcttgcccaactttggctctgtggtcctatgagccaaaatgcatacttagtgacatgtatctcacaggaaaagggaaaaaaggggtaagctgagagaggtcaagccatggtgttaatttctttcctgtacaaagacagtctcttgaggacaaaggcctgcctcttgcaatgtaatatcatagtccagatgagataatttccttcgaggaaagttggtgagaagttcaaaacgttcatttgggtatcctttagactgcacgtgcttcaccaaagctagcagtttagcttgctctggaagagtgatctgttccctttttccatctggataccgcaacatcagctgtgcttttggtccatttacatctatcccctccactactccatctgctttttcaggtggcatctccagtatctctgaatccacagctggcaatccttggtggtttgtggctgttccaggatcagttctgactggtggctcagtcagcggccttctattctcctcttttctatgccccaaatctttgtggggagactttctggacttggcaagattctctacctcttcttcttcatcagagccacaaacggatatgaactcctcactgccagaaaaaagttcagattcagattcttcatctgagcggctatcctgttttgtctgtgttgaatcaaaatgtgtttcttgtaaggaggctctgatggcagcttctagctggctgtcttcacttgcatctataaggctctctgaacgggcacattttttggggggactgctagaaagtccatccagttgtccatgttcacccagaaatcccgtcacttggtccaagaaagaagatacatctaactggtgccattctactagcttctgacctgtccgtgggtccaatatggaaacataggggaaatcccctaacttataaaactgtatgtatctctgaccttcctcactgtcatgataaacctgccagaaaatgaaatgttcccggataatattcttcacagcttcgttgctccacacatcgcggttgaggcactgacatgcaaagtcttgaacattttgaatgtttatcatcagccacttattttgcatctggccacactctttggctgtttcaaagctgcctttatgcatcaaatcaatgggtggccggaatagatctgcaagggtagttaatttcttatcgatagctcctccatttcttaattcttgttcttgccgaatagtttcagtctgaaaatcccggaaaccatcaaaaattgaacgtgcaggccgtcgtcttttaggagcaccaaataatggttctggttccaccagtatttcctgcttttgaggaattggggcacgaacttcttcttctgtgtgtggtctgacagtagagacacttgctgaactggtactgggctcttcagcgattcctccaccatccaaaaacatagtgactgccatttccagattattgttgcacgcttcaagcatatgttttcctacactttcacttgcacaaatctattttcttgtgttgagttcgttctgtttctctctgaaaggtagatttttgaaatgcaaaagcatgaaactaacttctttttctcccaggt

SEQ ID NO: 13167 - RNA, 5672 nt, Homo sapiens
  source 1..5672: mol_type = other RNA
gctgggattacaggcatgagccaccacacctggccaggaattagatctcagatttcaaaatacttccaacttctataaagaactcaatagctaattgttgacttgtaagtcaaggaagtagaattatatacaagatttaaaaacatacacacagagggttcaataatctggtatggatgggacacagaaaacagaattgtagatcgggcgcagtggctcatgcctgtaatcccagcactttaggaggccgaggtgggcggaacacgagatcaagagatcgagaccatcctggccaacatggtgaaaccctgtctctactaaaaatgcaaaaattagccgggcgtggtggcgctcacctattaaaaaaggtaattgtatcttttctgaaaaatgtttaaaaaaagaaaaaattgtttttttacccttttcatttattcttggcaaataatgccacgtggcaattttactttcacatcttcaccagtgcatcattttaaaaaagcaataatcagcctctcaaaataatggcataaataaaaatgtataggcatagtgcaaatcccacaactttaacccaactacttcctctatatttatgggaacaaaactaagtgacactttacaaagccaaacaatgagaagagaatcatctgggtagcttgattctcttgctgaaggagaccacagcatggactctggattccaattctgatttgccactcactagctatgagtcctgaataagttctctatacctgttttcttaacatgggaagaaagtatacattttgtacgattcttcgggagattgaagaggcaaatgtacacaaaagtatctggtgcatgccaattagtattaagtttcctgttcttttctcatttggcactgttgttttctcttctccagttccttccgataccaatttcaaaaaagtattcctctcacttttttcccactagttttcttcttcttcttcttttttttttttaaatttgagatggagtgtcgctttgtcgcccaggctggagtgtaatggtgcgatcttggctcactgcaacctctgcctcccaggttcaagccattcccctgcctcagcctctgagtagctgggattacaggtgcacgccaccacacccaggtaatttttgtatttttagtagagacggggtttcaccatgttgctcaggctggcctcgatctcctgaccttaggtgatctgcccacctccgcctcccaaagtgttgggattacaggcatgagccaccgcgcccggccttcctggtagtttccattccatctccctgtatttttctcttatcactctcgaagtctatctttcttgttcttttcctccctagctttttttttttaaacactcctttcaagctgtgtccaacacccacaaggaatgactatttttaactaatcttactgacctcatttaatctattcaataaaacctctgccctaaggagcaaagaaacttgcagaggaagtaaggcaaactggaagaagcatactgtcagcggattaaattcttgagcaaggcaatactccttatggattcttcccatgtacaatccgtaactcttcccatgggcctttatatcaaccctaagataattacactcctgcctcaaaataaaataaaataaaacccaccacatcttgtattgtagacatcccagctgcatgttaagctgagtgaaagtaccatgctgtcttttaaatcactttatatctacttaatcatcccacagtaacccgagttgaagaagttactttggtttctcataaatgaatatgcacgtgctgaacatatcggaaagaaccacaccctctcactgatgaacacgttggcagttctcccaactgttttatcaagagaagctagaaggtaaagaaaaggaaacagagccctataggaaaaatgattgacttcacacgtttgagcgatttgggcttcagctatgactttgctggagtacagatgggtgccatcagagcacaaagctgagcaaacctctcttcttaccctgtgccctccctgaatttttggatttctgagcttgtctactaccaacaaatgttttaccctccagtgcacctttgacagtatacagctctatttttcaaacggcaagtatgttatccaagttcagagatgcaactgaggaattaacatgaaaaccatctttcactcaataaatcagaagctgctagttaagtaagcctcaagaacctaagaaaaaacaccaaagtgtaagtattactcagtcaccaatctaaagacagaactttgactcaaggtagaaatgaaaccgtaattatataaatatatttataaatatttatacaattatatacttatacataagcacttacacagacttagaaaaaaatttaagaacattaattcaaaaggactcactgaagaataaacagatttttccatgatttccttgaggagatataaaactcattctttagggagagttcctcaaaattcaaccattagaaaccatatcctataactgtgtactagcaacacatggcatctttttttcttcttttcccaaatcccctaattgccaagagagcaatcttaaagtagatgaaaacctaaaggtctctacgcaacatctgaggaacatacgctcctcagataaaagaatcaatctaaatcctcaactgacaaaaaggtccatttaatatttttcattttacaagttaaaagttctagttttgccaccagaatcacgactacccccccttcagaggactccatttaagctcaaaatacgaaatgagcatagggtgaagttgatgtgtaaatggtattctacagattcaagatggcctcttctaaaaacactgaagaaagctttcaccaactctaatttgattttgggttttgttggcagaaaaagcccaagacatctgaaaattactagtaacctccgccatcctccttactaaatgttgtcttctgaatggagttgaaaggtcttccccttagagaggctttccgttttgataccttttgaaagaaaacagcatgcggactcatgttcaattcagtcaccagagccttttagagactattccaaccaggggcaaaaaatgaaccattatttctaaccaaaagaacatggttagcaactctcagctgaatggttttctttttccccagggacatacctaagtatgcctgaaacaacacaggacaatcaataaccatagtggttacaattccaagccattgtactacatgattattgaccagctgccttcctacagatcactgcagactcagacaatggagggctccaaaggaactaatatgctgtgctggcaaaaatagcaagcaccttcctatcccagtcaccacgataggttcacttcatgtccattcttggactagcaggatcaatacagagtaataaggaaaactgtctcaggttaggacaatgaaagtcaccccatgctatatgctccatatttaacactcattctgccaataacacatgtcatggaaatagtccttatagctgggaacatgaaaatcctttgaaaaaggtttttaagtatgatgagcaatcattacaagggatgctttttccacgtaaacaaaagcctggatattttgttaagcgacatttccacatgaagaacacaacaaaaccaaacccatgttagagaatttcttctccctgctaaacacggggacttacaaaaaagggagggttgttcttactctgaatctagccattcctttgcccgaagagtctggggagtaacgttaacatttgatcccaaaaaagtgccgtgcaagagaccacttactggaacacacaattcctgctgctagtactaggagaggtcttatccttacacttcagtttggtcaccagattaggtaagaaagaaaagtgtggggggagggggaggcagaagggtacggagtggggagcgagaaaacagaagaggagaaagaaacaaagggggagaaagagactgattataggagagatcaagaaataagagaaggaaggtgacttgcttgcccaactttggctctgtggtcctatgagccaaaatgcatacttagtgacatgtatctcacaggaaaagggaaaaaaggggtaagctgagagaggtcaagccatggtgttaatttctttcctgtacaaagacagtctcttgaggacaaaggcctgcctcttgcaatgtaatatcatagtccagatgagataatttccttcgaggaaagttggtgagaagttcaaaacgttcatttgggtatcctttagactgcacgtgcttcaccaaagctagcagtttagcttgctctggaagagtgatctgttccctttttccatctggataccgcaacatcagctgtgcttttggtccatttacatctatcccctccactactccatctgctttttcaggtggcatctccagtatctctgaatccacagctggcaatccttggtggtttgtggctgttccaggatcagttctgactggtggctcagtcagcggccttctattctcctcttttctatgccccaaatctttgtggggagactttctggacttggcaagattctctacctcttcttcttcatcagagccacaaacggatatgaactcctcactgccagaaaaaagttcagattcagattcttcatctgagcggctatcctgttttgtctgtgttgaatcaaaatgtgtttcttgtaaggaggctctgatggcagcttctagctggctgtcttcacttgcatctataaggctctctgaacgggcacattttttggggggactgctagaaagtccatccagttgtccatgttcacccagaaatcccgtcacttggtccaagaaagaagatacatctaactggtgccattctactagcttctgacctgtccgtgggtccaatatggaaacataggggaaatcccctaacttataaaactgtatgtatctctgaccttcctcactgtcatgataaacctgccagaaaatgaaatgttcccggataatattcttcacagcttcgttgctccacacatcgcggttgaggcactgacatgcaaagtcttgaacattttgaatgtttatcatcagccacttattttgcatctggccacactctttggctgtttcaaagctgcctttatgcatcaaatcaatgggtggccggaatagatctgcaagggtagttaatttcttatcgatagctcctccatttcttaattcttgttcttgccgaatagtttcagtctgaaaatcccggaaaccatcaaaaattgaacgtgcaggccgtcgtcttttaggagcaccaaataatggttctggttccaccagtatttcctgcttttgaggaattggggcacgaacttcttcttctgtgtgtggtctgacagtagagacacttgctgaactggtactgggctcttcagcgattcctccaccatccaaaaacatagtgactgccatttccagattattgttgcacgcttcaagcatatgttttcctacactttcacttgcaccggtaatggtggtgaactgttgaattaaccccttcagcgccgaggacgccgcggagcccccgtgggcagccatcttaccgccgccgccgccgccgaacaac

SEQ ID NO: 13168 - RNA, 8916 nt, Homo sapiens
  source 1..8916: mol_type = other RNA
gctgggattacaggcatgagccaccacacctggccataatatatttccgattgcttaacattttctctagcttactttttacagtatataatacacataacatacaaagtgtgtgttaaatgacttattggtaaagtttccacagtaggctgtcaagttttgggggaatcagcttatacatagatttgactgaaggaagctggggcccctagcccctgcattatgaaagagctaactgtatacacaatccagctttgtttcattggttttctcaatctacaggaatatgacaactacaaaagaccttagagactgaactactgagaatcaatcattcgacttgctacacagtcccacacaggattatggttggtacattgaatgggtctagataaatcctaactgacctatacatccaaaacttttctgtacacttaccaagttccaagcacagtgctggaaattaggaaactcattaataagcaagtgtttctagagtattttgaactggttcaaaaccagttcagatttatagaaccaaagagtaggtactgatgaaaaggagatcctatgttgaactagtaaaacacatgcacaaaagcccagtggcagaagtaaaagaaaaggcagccaagcagagctgaaatagtgcaaatgcaggttaaatacagtgggctattcatctccaagttgccgtgaagtggctaagtccactcaccaagccaaatgaatagcaaagacaacagttccagcctccagttttgaaatccatagttaagtgcggcagctcccacttgtaagcatagcacctcaggaggttgaggtgagacaaccacttgagcccaggagttagacactagtccaggcaacatagtgagaatcatctcaaagataataaaaataaaactttgttgactggcctaatccaagtctaaaatcacatctgatctcaagacagacacccatgtcacatccacaccagtgtcaaggctccaggtaaatgttgggagatagaagggataacctgaataatgacaatttgggtattctgaagcatgagaaatccaaatatatagcgatacctcatttcgttttaccctagatcatttctgggttctgccaaaggccaaagaaagtaaacagcatatgaaaacacatgtattaaaataaaacaagaaaggaatgagatgagattttcaaacctagctcactttaggttaaggtcaattttttttttgttttttacacataaaatcttcaaaacgaggcatatgtttaattttattatccagtcttagtctcagtgttcttatgtacactgagtaatgcatcccttacacctaggaggaattttgcctttgaaccaagaaaaccccaactagttcagaaataaagttctaaaaccaatttaaaaagtaatcccaatcacaaattttaggttttcttatgtttaggaagtgctcataggctctaagtacttttgtttccttattaatgttcaccacgatctttcgcaatacagatgaaaagactgatgctgaaccaacaggtggtagacagactctaaagcctgtgtttaaagacactacccaaagacactacttgtattctcacacatatccattaaaatttggtagcagagacatttgtttaggggctgaaaagttttagtctaaaattagatctccatttttattcatggattcttattcctatagagcaacctcatctactttcctagttggatcaactgattccacttatttgaaaataattacaaatacggacggcagtagcagtaggaaaaataacattgtttgattcaacttcaaagtatccactgtgcgttcagtttttatgatacatgtacaaattttctttcacctgaaaggccctagaaataccctgtaaagagcatattcagcaactggacttaagtttctaagtaatactccctattctaagaagccagcaatccttggagaaatggcccattccagggctgaaatagaaaacgcctgtaagactagaaaactttttgagccaaaaagtatgttgatcagagtaaagaatataccggaattctttcaactattttcagagttgaaggaaagctgtaatattgataagttaccccaaaacaccaatctggagtttgactaaggggattcactgcagataaaactttattcagcaatttttttaaataaagcttttgttcttggctaagtaaattatcttaacagctaacagcgtcttgttcactgctgctgccacgtcatttaacttactttttcagttgcatatatatgaccctgaagcctttactggcccctggggcccacctacctcaaatgttctgaccttcaaatggctgacttggtctatcaatcatgtcttcctttaaaaattatctttcagccaggtgcagtggctaacgtctgtaatcccagcactttgggagaccaagatgggtggattacctgagtccaggagttcgaaaccagcctggccaacatggtgaaacacctctcaacaaatgtaaaaattagctgggcgtggtggcacgtgcctgtgataccagctactcgagaggctgattgcagcagtacactccaacctgggcaaatgaagtaagaccctgtctcagaaaaaaaaaaaaaaaaaaaaatttctacatggaatggtcatcctcatcctcacttgaaatactcttgtaacaggtggttccagtgttttaaacccattaagaggacttccacagctaaactttctatggactggccacttgtatttctacctgtatttccaggtatctcaattccttgaatgtagcctcaattgttctgttctgggacctttgcctgtatttcctcctgttcctccacctgaactgctcaccgttcagaggttcttcctctcacttcacaaattcctacagattctcaaaatctcagctaaaagctcatacaaattttgagccttctggtagcaactattttacaacctcatgaaatttaccagagccgcaattgcctaatacattatgaatgataaaattatgaataagaccttcaactctggatatgagatctgtcgacttctggcactcacgtttaatcacacattcctagttccttctttttggctttaagtttaaaacatgtaagaaactggctgggcgtggtggctcatgcttgtaatcccagcacttttgagaggccagcactttgagaggctgaggtgggaggatcactggaggtcaggaggtcgagaccagcctggccaacatggtgaaaacccatctctactaaaagtacaaaaatcagctgggctcagtggcacacgcctgtaatcccgactacttggaatgctgaggcacgagaatcgcttgaacccgggagatgacagctgtagtgagccgagatcatgccactgcactccagcctgggcaacagagcaagactctatctcaaaaataaaaataaatggataaaacatgtaagaaactaaaaagcaatgcttttatgtaatattttatcctgggtttcaaaataataaaactcagtttgttctaggatccacaaaacttaaaatgcccaatttcccataggaaaattaaacaaccagactgacttatttcccgccagtaatctattatttctaaataccccatttcttcttttattcagactcttggcttgaggatgacatggtcgggcctcaataagcccactgtaagtcaaaaatatcataagtagaagatgtgtttaatactccaataaactcataaagctgaagtcttaagtcaaaccattataagtcagggactgtctgtactaagattttagtgaataacttaatttttgtaaactggaaaacctgacaatatgatgtcaaaaggaagaaacacaagatacaaagcatactgtatttttgaaaatatacatcaatcaaaatttcttatgaatacttatccttgagtaaaataatttcatataccaacaaggatgtttccatttctgtaaagtcatgtaagtgatcctcaatcagtccaagaacttggctttttatccaggttatattttaatatctggagttttaatccagcatacaaaaatcaccagtatacatctattaagttaactgcagtattatttcaccatcaccatttacatgtacttttcaggtatcagagacttagtgctttaagtagcaaattacctaaattatgaacacatatttccaaaaacaaaatcaagctcataattaccaagtatatatgtacagtgcagattaaaaaaaaactgaattagcacatatttctcttttctaaagctcctatgaagaacttacactcttctgcactaccaatctattctgtacatttaaaataacatttgttttgatttaaagtcaaaaatataaaggcttaaatttttgtaagactaacccataaaaaaggactccaattttaaaccaatccctgaaaccaaagcattcaaatatttgaatattagttcaatatttctacatagcacgataagattttcagttacttcaagttttgtctttatttttaataatgggaatggcctacaattacaataaacaattaattcagttattttaggggccttaccatatcattaacctattcacacaacaaaaatatttttatgaaagttaatatatcctttcctgattaagtgtgctaaaacagaaatagaggtagaatcccatttttcttaagtaccactctacaagccagttccacacaattaaggtatttttgcaatctaaaatagtgatgctaatactgcttcagtaagctagatttactaatttaagaatcctaagaaattatatatgtggctttcagacatccatgttaaactatcaacttgtggaatttgtggaacacttaccctacttgagtgaccataaagcaaacaactctaaaattttttcatatcagttttctttataagtgattatatgatatttcaccatttctaacaggaaaaaatgagacttacttggcagtgtgcatgggctgctggaaactacaatcagagtgtaaagacaaatctcaaaaatgtttgtagataactcagaataataacccagaatataacctatcaggaactatggaattccattttagtcttcaaataataaactccacttagcagggattgtgaggttgctcttaaaattatatatttacagaacatagtggcctcagcacaaaatagctccctctagacatcactactctccactcttcaaaaaaaaagtatatacattcatttaaaaaaaaacacccaaaatatcaccagtacattttataaaattaaatccaaattttattaaggatttcaggttacatacttcaaatttctagaatggaatggaatcattttggaactggaaaaatggcataaacactgacgtcccttaaaacttcaattttataaagaaaattcttctgcaaaccacatcccctttatgtaacaagactaggtattatctacaccttcactttggcaatagctatttcctaaagaatgaaaaagatgattttgctacttcagttcattaaaaatgggattctatctttgaagttcagaaaaagctgcatttcgatgaactatggttaaaaaaaaaaagcacatagtgtctaatcaaagcaaaggaaatcattttgaaaataaagaaaaaaagctattataattggttaaggatttccagtagtaagttaaaatctcaggagaggaatggatagcactacaaacaatgtgttcacattccaagaccttaacactaacttctcagaaaggaagttttcattacctctaaaaatcaattcaatgtaattttattaagagcaggaaatctagaccttcctctaatgacaatccaataatccaccctcactgtcaaaaaaaagttcaaccccaaaattaacagtaattagcctgaggtattgtaaatgtggctctacagtctgaaatttaatggcatcttttgtcaaaaatagtcttatttccactttaagtctcatgactacaatactatagtgctatccctgtagtatttacaatacagtcatcaaaaatatctgaaaacaaatcttggaccttgtgaaatagtgcatccctccacttctataaaaataggagccacacaaagatctaaaaagagtgctgactgcccagatccagaacagaggtacttaacacctttgttttccagtttagttatcaaagcgtggtgtgaacaaaatgcttagtgtcacactggcattacaaataggcccaaaattttgagcttttaacaagattgagaaacattatatgagatttaactcaatatgccttaacacatccatgaggtagttaggtaaacagtactacccattttaattacacagtaaacagaagcacgggtaagtgacatactcatactttaagcaataagaattagaagaaaccatagaagcttggggccttctctctagctctaacccaaagaaaatgaatttttttttttttttttaaaagaaaacagcatcaatcacttaagattttcttcctcttttttttttttttttacacttgcttattagtatagcatctcgttccaaagctggtaccttttcttcaacaatgtgttaaaaactgagtataacccttaattcaaggtaggcctctacttctacctgaattggtacaaaattaagacattatcttgtaagaactaaaattgtatttgaaatttttattttagctgcaaaaacaaaaacaagcaaacaaacaacaaataacttgaaaataggcttgtcaaatgatgtaaattcatcctttccagggaagcagaaggtagaccctaccacaaagaaaagatgcttagttaatggaggttaaatttaaaaatacagttaaattcaggctaacttctgaaaatcccgttttattcacctcactgtggtaccagtaactatactgagtcaggttactttacagttaactatgtcacctaaaacacaataatccattaacactctaataacagttattgggtgtggtcatactggaaattcttaaccatatagttgtcttgccaattttttttttaaacaataaattgtcttagtataagtcactgcatttctgtaacaaagtaatgaaaggcacagctaatccaagcggacttaaccctattcaacaaccagctgaaaaaatactttggttcttcaaggaaaaaattacaaaaaaaaaaaaaaggtatttcctttaacagttgttaattttcatagctgtactccaagagctacataaaaatattccagaagaaccaaattatgtagcaatgaatgaacatgcgtgacagaatttgtgcattcaacatagctggcagaaaaactagttaaaatgctaggtagaacaaattggtctttaaaatatcagtttcctgtcctttaaaaaaaaattacctagtctaccaagaaaatacaaaaacataaggctgtaagtaaataagagttgtgtttaggctattacagtgcaggttatcctcaaggccacatacatcctgcttcactgctgcttgcactctgctgggttttgatccttctttgggtcatagtctggatcattttcctcatctccttcttcttccccttcctcatccgcttcttcaccttcttcatcataatcatcatcatcatcttcaatagcttctccagtaaaatataacactgatcttgggattatacgctcacgtaaaaagtgaccaatttcgaagtctgcagcaaggatagcttcagcatcatcatccagatctccactctcaggaacttcaggaggggcaaaaaagttaaagaaagagtcattggaaactgttttagtcacagtacgaactgtcccacgtcccttgtgtttctgcttcttcttaatagttttcaaagtgacattctttccttttttccaatctatctggcaccctgtacaacccataatttctggtccatcaaaagaaaagggatcagaatcatctggttctgacctcatcctgtatgtctttgtcagcacttcatttgtaaaatattcattgggttcaaagtgaaattctaagacaaaactcataggctggccagcatctgagaacttcactttaatatctttcaagtgcttcagaataggttcatcgtgttcctgaaccatatcactgagcaagtcaacattcttaaaaacagttaaccaaaattcaggaattcctttggggtcttctttttcttcatcttttttctcatcttcaatcttggccttttctttcaattcctccgaaatctcatcttcttcatctggtttccattcacattcttcttccgtaggttcataaattgcattaataatttcaaatcgcttatcaaatagaggctgatagagaacagcatacttcctttcaagatcgtgaacttcctcatagaatttggcttctatctgtgcacatttaacttgcaggtttttgagagcattcactcgtcttttaactaccctaggcaggctttcaatgtatcctgttggtgtttctaccagaccatcaagtctttcttgaagggctgcaagaatctgaggattttgcatcatctgaacagttagctgacgtgctttgagttttgtttcttcaccagtttcctcttcttctacttcttcaacatcatccaaatcttgatcaagttcagactgttctttgttgtcaatgtctgccatgttgtaagaactccaaatatcggcgactagtatggggagccaggcggccggagctgcgcaggcagtgactcagggcggcagcggcagcagcagcgggaggagcaggaggcggcgccgcgagcagatggcgctaaaaaag

SEQ ID NO: 13169 - RNA, 3900 nt, Homo sapiens
  source 1..3900: mol_type = other RNA
gctgggattacaggcatgagccaccacacctggcccgctttttgaactttactgaagcttatatacaattctgccagagttgttttccaaaatcatccaactctaaaacatattcttttatctaaaaaaatcaattggtttccataccactcattaaataaattattaacataattggttaactaattggttaacacaacccctcctcaattctggggataagattatgcctcattttgaggaaggtgaaaggcttgacggtgaaattgaaatgcaaagaacagagttcaaggctcatggttaggttgttattcccagatcctaatacaaaccagcaatggtgctattctgagcccttatccacaggaggttagatgccaaaaaggactctgaggtcagccaaggtgagcttggtgacagattctccagaccctgatagaacttgtttggccaaatctttctttttttcttggagctgtaagatcttttcttctactgttccctcacaaacaaatctgtgtatgacaacatctttctgctgccctactcggtaaattcggtcacaagcttgatcttcaagtgatggattccagtgcatgtccaaaagaaagaggtgatttcctccagtcaggtttagaccaacacctccggccaagagagagattagcattacctgagggcctctggagtggttaaatgcctctaccaagtccattctctgcttgggattgacagagccatcgatggtggcataagtcagtccatgcttcttcaggtgcaatgctacaactttcagcatgttggtccactgagagacaatgacactcttttgggatgctgaatttctttgaattgcctccaattctgccaacagagatgaaatcttggtgctctctcgcatgccttcaaaaagctccatcttgaagaaggtgccgttaagggaaacagtggaagatggctctgagtcacggagttctgacaaggtcaaagcactgagctgttcttccagggaaaggacaagaccttcacccttcagttccattggatccagggccgacttcagtaaagaaagatgacagcaacactggcggagtctcagcaactgggacagtatgtggacggtgctggatctcggtgagtctgctgcctccgagtgtctaggctcctcagacccaaactccagtgccactctactgaatggattattagggcttcttccagattggttgcctctactttcatgtctttttagataggattgcagagctgaccttgatcttgcaaaaaacacattgtaaacagtctcttcatcttcagaaagctttaaatggtgcaactgaaatttacgctggggcagtatcaccaaaggtctgccagtagagtccagctggtcttttgttctcctcagcaaaaggctcttggttaaaatacttaaccgttctcctcctttctttgagccattgtcaacctgactcctccacagattgaactcatcaaatggagagcaacggagaaacttcagcagcgaatacatatccaataagttgttttgaatgggggttccagtgacagcccaacgggcacaggcttgtagcttacacacagctatggaagtctgcactcggggattcttaacattgtgagcttcatccaatatgattcgagcccaggctattcgaagcaaaggtgttgaggtgccctccacattgaggtttgcacctgggatctctgcctcttgcttgtttgtgggaatctccttggccacgaggctataggtagtgatcacgatgtcatatgtagagaggactctggcacgtgaatcccggtttggcccatggtagagatagactcttagtttgttgctgttcacccgtttctccacctcatttttccaatgatggatcagggaggcaggacagatgattagtgttccatgggaagtaaagtcacaagagtcatctttggagagccacgtcaaagctgtgcttttctccttttcttcctttttctcttgattcttctgggtcaggatgagcgcaatcattgtcagggtttttcctaagcccatatcatccagaattcctccttgtggcttctgactttctcgccatagtaaccaagccaatgcctgcttctggtgtagtagcaaagggaccttcagcccggcgggatcttctgccacaaccgtctcaccaggacatgactcaagtgagcgatgcagttgaccgatggcttcacttgtgattttccacactgcatgaacgtgatcttggtttgtatggcctcgatagcactgactggatcctccagcagtcacctggcaggcagactttagttctagagaacccacaggttgggtaccacgacgaggaaggggttggggaggcaccaggtggggagggccagtggtagttttggtgaagtgactctgctgtggtacttgactgttactcttctcattagttccttgctctggggaaagggtaagaccactgagtacttcctccagctcctggatttgtttgatcaacttctgacccttgtctggaagagcctggatgttcactgatgccagtgtgctcttcttttgtttcagttgtgttgtaaggtagacacgccgggctactgggtctgagggttctaccttcttggaaacacctgaggcaggagacacctttctttgcacacttcgatcagggaattggaggttttccttcgtctctaagtccagagtcgagtcaaagagtagggggctcccaggcttagaggaaacaaaaacaacatcatcttcctcctcgtcgtcactgcttgtggcagcttcacggccctcacccagggaaagccctggtgctgctggtgcagcctgagccgctggtcctccaggagcaggcacactgtgggtctccggccgctcttggaaatgcccctgaggcaggcttttctgggtggcctgtatgctagggccatcctttgcctttgtttctttagcctcccagttcgtgtactccttgttgaggggtccccctttctggggcttgcttattgagttgtgactgtgaacattttgaggcaaaagctgggtaaccttttctctcagaggttctgattctctttggacatcttgactcttaccacttgatttctcctgagaagatgcagatggtcttgtaagctcattaccttggcactgttgagatttaatttcagaaaagtctcttttgtgtgtgcctccagtctctgcctcacactgaatctctgctccctcttcttgcttcttctcttgaactacagattgttttttctttggtaccaggccagatgagaggtctttctccatcatttcaggcttctgttctttcttttgatcgaaaagctgatctcccttttctctttgcttcttatcagccttcttttcctcaccttcacctttgatgagctgtttccagagagctggttcttgattcttgtcaagtaccttgaatggatttctcagccagttggaagaatgatgaaatgtctcagatgcatgctgagacttattggatacagaatgttctttggaatcaggatcctgccatggaatacttccacaccagcgtttcccctctgccttacttctaatgcatcggaagaacaatctgtattctttcttgtcctgtggcagaagcaaaccctgaagctctaccacaaagtcctcatgcaataagcaatgggaaacaggaatgtcggtggcccgcacgaagctgcacgtgtctgcccggcacacgtagaagctctttcctttattcgggccatcgcggacgccggtcttaagaaagcagaaagtcccgtgctctggacacctaacttcttccatttcgctgggtcccccaagttccacaaagccccgcccccaattct

SEQ ID NO: 13170 - RNA, 3880 nt, Homo sapiens
  source 1..3880: mol_type = other RNA
gctgggattacaggcatgagccaccacacctggcccgctttttgaactttactgaagcttatatacaattctgccagagttgttttccaaaatcatccaactctaaaacatattcttttatctaaaaaaatcaattggtttccataccactcattaaataaattattaacataattggttaactaattggttaacacaacccctcctcaattctggggataagattatgcctcattttgaggaaggtgaaaggcttgacggtgaaattgaaatgcaaagaacagagttcaaggctcatggttaggttgttattcccagatcctaatacaaaccagcaatggtgctattctgagcccttatccacaggaggttagatgccaaaaaggactctgaggtcagccaaggtgagcttggtgacagattctccagaccctgatagaacttgtttggccaaatctttctttttttcttggagctgtaagatcttttcttctactgttccctcacaaacaaatctgtgtatgacaacatctttctgctgccctactcggtaaattcggtcacaagcttgatcttcaagtgatggattccagtgcatgtccaaaagaaagaggtgatttcctccagtcaggtttagaccaacacctccggccaagagagagattagcattacctgagggcctctggagtggttaaatgcctctaccaagtccattctctgcttgggattgacagagccatcgatggtggcataagtcagtccatgcttcttcaggtgcaatgctacaactttcagcatgttggtccactgagagacaatgacactcttttgggatgctgaatttctttgaattgcctccaattctgccaacagagatgaaatcttggtgctctctcgcatgccttcaaaaagctccatcttgaagaaggtgccgttaagggaaacagtggaagatggctctgagtcacggagttctgacaaggtcaaagcactgagctgttcttccagggaaaggacaagaccttcacccttcagttccattggatccagggccgacttcagtaaagaaagatgacagcaacactggcggagtctcagcaactgggacagtatgtggacggtgctggatctcggtgagtctgctgcctccgagtgtctaggctcctcagacccaaactccagtgccactctactgaatggattattagggcttcttccagattggttgcctctactttcatgtctttttagataggattgcagagctgaccttgatcttgcaaaaaacacattgtaaacagtctcttcatcttcagaaagctttaaatggtgcaactgaaatttacgctggggcagtatcaccaaaggtctgccagtagagtccagctggtcttttgttctcctcagcaaaaggctcttggttaaaatacttaaccgttctcctcctttctttgagccattgtcaacctgactcctccacagattgaactcatcaaatggagagcaacggagaaacttcagcagcgaatacatatccaataagttgttttgaatgggggttccagtgacagcccaacgggcacaggcttgtagcttacacacagctatggaagtctgcactcggggattcttaacattgtgagcttcatccaatatgattcgagcccaggctattcgaagcaaaggtgttgaggtgccctccacattgaggtttgcacctgggatctctgcctcttgcttgtttgtgggaatctccttggccacgaggctataggtagtgatcacgatgtcatatgtagagaggactctggcacgtgaatcccggtttggcccatggtagagatagactcttagtttgttgctgttcacccgtttctccacctcatttttccaatgatggatcagggaggcaggacagatgattagtgttccatgggaagtaaagtcacaagagtcatctttggagagccacgtcaaagctgtgcttttctccttttcttcctttttctcttgattcttctgggtcaggatgagcgcaatcattgtcagggtttttcctaagcccatatcatctgccagaattcctccttgtggcttctgactttctcgccatagtaaccaagccaatgcctgcttctggtgtagtagcaaagggaccttcagcccggcgggatcttctgccacaaccgtctcaccaggacatgactcaagtgagcgatgcagttgaccgatggcttcacttgtgattttccacactgcatgaacgtgatcttggtttgtatggcctcgatagcactgactggatcctccagcagtcacctggcaggcagactttagttctagagaacccacaggttgggtaccacgacgaggaaggggttggggaggcaccaggtggggagggccagtggtagttttggtgaagtgactctgctgtggtacttgactgttactcttctcattagttccttgctctggggaaagggtaagaccactgagtacttcctccagctcctggatttgtttgatcaacttctgacccttgtctggaagagcctggatgttcactgatgccagtgtgctcttcttttgtttcagttgtgttgtaaggtagacacgccgggctactgggtctgagggttctaccttcttggaaacacctgaggcaggagacacctttctttgcacacttcgatcagggaattggaggttttccttcgtctctaagtccagagtcgagtcaaagagtagggggctcccaggcttagaggaaacaaaaacaacatcatcttcctcctcgtcgtcactgcttgtggcagcttcacggccctcacccagggaaagccctggtgctgctggtgcagcctgagccgctggtcctccaggagcaggcacactgtgggtctccggccgctcttggaaatgcccctgaggcaggcttttctgggtggcctgtatgctagggccatcctttgcctttgtttctttagcctcccagttcgtgtactccttgttgaggggtccccctttctggggcttgcttattgagttgtgactgtgaacattttgaggcaaaagctgggtaaccttttctctcagaggttctgattctctttggacatcttgactcttaccacttgatttctcctgagaagatgcagatggtcttgtaagctcattaccttggcactgttgagatttaatttcagaaaagtctcttttgtgtgtgcctccagtctctgcctcacactgaatctctgctccctcttcttgcttcttctcttgaactacagattgttttttctttggtaccaggccagatgagaggtctttctccatcatttcaggcttctgttctttcttttgatcgaaaagctgatctcccttttctctttgcttcttatcagccttcttttcctcaccttcacctttgatgagctgtttccagagagctggttcttgattcttgtcaagtaccttgaatggatttctcagccagttggaagaatgatgaaatgtctcagatgcatgctgagacttattggatacagaatgttctttggaatcaggatcctgccatggaatacttccacaccagcgtttcccctctgccttacttctaatgcatcggaagaacaatctgtattctttcttgtcctgtggcagaagcaaaccctgaagctctaccacaaagtcctcatgcaataagcaatgggaaacaggaatgtcggtggcccgcacgaagctgcacgtgtctgcccggcacacgtagaagctctttcctttattcgggccatcgcggacgccggtcttaagaaagcagaaagtcccgtgctctggacacctaacttcttccatttcgctgggtcccccaagttc

SEQ ID NO: 13171 - RNA, 3924 nt, Homo sapiens
  source 1..3924: mol_type = other RNA
gctgggattacaggcatgagccaccacacctggcccgctttttgaactttactgaagcttatatacaattctgccagagttgttttccaaaatcatccaactctaaaacatattcttttatctaaaaaaatcaattggtttccataccactcattaaataaattattaacataattggttaactaattggttaacacaacccctcctcaattctggggataagattatgcctcattttgaggaaggtgaaaggcttgacggtgaaattgaaatgcaaagaacagagttcaaggctcatggttaggttgttattcccagatcctaatacaaaccagcaatggtgctattctgagcccttatccacaggaggttagatgccaaaaaggactctgaggtcagccaaggtgagcttggtgacagattctccagaccctgatagaacttgtttggccaaatctttctttttttcttggagctgtaagatcttttcttctactgttccctcacaaacaaatctgtgtatgacaacatctttctgctgccctactcggtaaattcggtcacaagcttgatcttcaagtgatggattccagtgcatgtccaaaagaaagaggtgatttcctccagtcaggtttagaccaacacctccggccaagagagagattagcattacctgagggcctctggagtggttaaatgcctctaccaagtccattctctgcttgggattgacagagccatcgatggtggcataagtcagtccatgcttcttcaggtgcaatgctacaactttcagcatgttggtccactgagagacaatgacactcttttgggatgctgaatttctttgaattgcctccaattctgccaacagagatgaaatcttggtgctctctcgcatgccttcaaaaagctccatcttgaagaaggtgccgttaagggaaacagtggaagatggctctgagtcacggagttctgacaaggtcaaagcactgagctgttcttccagggaaaggacaagaccttcacccttcagttccattggatccagggccgacttcagtaaagaaagatgacagcaacactggcggagtctcagcaactgggacagtatgtggacggtgctggatctcggtgagtctgctgcctccgagtgtctaggctcctcagacccaaactccagtgccactctactgaatggattattagggcttcttccagattggttgcctctactttcatgtctttttagataggattgcagagctgaccttgatcttgcaaaaaacacattgtaaacagtctcttcatcttcagaaagctttaaatggtgcaactgaaatttacgctggggcagtatcaccaaaggtctgccagtagagtccagctggtcttttgttctcctcagcaaaaggctcttggttaaaatacttaaccgttctcctcctttctttgagccattgtcaacctgactcctccacagattgaactcatcaaatggagagcaacggagaaacttcagcagcgaatacatatccaataagttgttttgaatgggggttccagtgacagcccaacgggcacaggcttgtagcttacacacagctatggaagtctgcactcggggattcttaacattgtgagcttcatccaatatgattcgagcccaggctattcgaagcaaaggtgttgaggtgccctccacattgaggtttgcacctgggatctctgcctcttgcttgtttgtgggaatctccttggccacgaggctataggtagtgatcacgatgtcatatgtagagaggactctggcacgtgaatcccggtttggcccatggtagagatagactcttagtttgttgctgttcacccgtttctccacctcatttttccaatgatggatcagggaggcaggacagatgattagtgttccatgggaagtaaagtcacaagagtcatctttggagagccacgtcaaagctgtgcttttctccttttcttcctttttctcttgattcttctgggtcaggatgagcgcaatcattgtcagggtttttcctaagcccatatcatctgccagaattcctccttgtggcttctgactttctcgccatagtaaccaagccaatgcctgcttctggtgtagtagcaaagggaccttcagcccggcgggatcttctgccacaaccgtctcaccaggacatgactcaagtgagcgatgcagttgaccgatggcttcacttgtgattttccacactgcatgaacgtgatcttggtttgtatggcctgcatacaaataggtgttacctcgatagcactgactggatcctccagcagtcacctggcaggcagactttagttctagagaacccacaggttgggtaccacgacgaggaaggggttggggaggcaccaggtggggagggccagtggtagttttggtgaagtgactctgctgtggtacttgactgttactcttctcattagttccttgctctggggaaagggtaagaccactgagtacttcctccagctcctggatttgtttgatcaacttctgacccttgtctggaagagcctggatgttcactgatgccagtgtgctcttcttttgtttcagttgtgttgtaaggtagacacgccgggctactgggtctgagggttctaccttcttggaaacacctgaggcaggagacacctttctttgcacacttcgatcagggaattggaggttttccttcgtctctaagtccagagtcgagtcaaagagtagggggctcccaggcttagaggaaacaaaaacaacatcatcttcctcctcgtcgtcactgcttgtggcagcttcacggccctcacccagggaaagccctggtgctgctggtgcagcctgagccgctggtcctccaggagcaggcacactgtgggtctccggccgctcttggaaatgcccctgaggcaggcttttctgggtggcctgtatgctagggccatcctttgcctttgtttctttagcctcccagttcgtgtactccttgttgaggggtccccctttctggggcttgcttattgagttgtgactgtgaacattttgaggcaaaagctgggtaaccttttctctcagaggttctgattctctttggacatcttgactcttaccacttgatttctcctgagaagatgcagatggtcttgtaagctcattaccttggcactgttgagatttaatttcagaaaagtctcttttgtgtgtgcctccagtctctgcctcacactgaatctctgctccctcttcttgcttcttctcttgaactacagattgttttttctttggtaccaggccagatgagaggtctttctccatcatttcaggcttctgttctttcttttgatcgaaaagctgatctcccttttctctttgcttcttatcagccttcttttcctcaccttcacctttgatgagctgtttccagagagctggttcttgattcttgtcaagtaccttgaatggatttctcagccagttggaagaatgatgaaatgtctcagatgcatgctgagacttattggatacagaatgttctttggaatcaggatcctgccatggaatacttccacaccagcgtttcccctctgccttacttctaatgcatcggaagaacaatctgtattctttcttgtcctgtggcagaagcaaaccctgaagctctaccacaaagtcctcatgcaataagcaatgggaaacaggaatgtcggtggcccgcacgaagctgcacgtgtctgcccggcacacgtagaagctctttcctttattcgggccatcgcggacgccggtcttaagaaagcagaaagtcccgtgctctggacacctaacttcttccatttcgctgggtcccccaagttccacaaagccccgcccccaattct

SEQ ID NO: 13172 - RNA, 3963 nt, Homo sapiens
  source 1..3963: mol_type = other RNA
gctgggattacaggcatgagccaccacacctggcccgctttttgaactttactgaagcttatatacaattctgccagagttgttttccaaaatcatccaactctaaaacatattcttttatctaaaaaaatcaattggtttccataccactcattaaataaattattaacataattggttaactaattggttaacacaacccctcctcaattctggggataagattatgcctcattttgaggaaggtgaaaggcttgacggtgaaattgaaatgcaaagaacagagttcaaggctcatggttaggttgttattcccagatcctaatacaaaccagcaatggtgctattctgagcccttatccacaggaggttagatgccaaaaaggactctgaggtcagccaaggtgagcttggtgacagattctccagaccctgatagaacttgtttggccaaatctttctttttttcttggagctgtaagatcttttcttctactgttccctcacaaacaaatctgtgtatgacaacatctttctgctgccctactcggtaaattcggtcacaagcttgatcttcaagtgatggattccagtgcatgtccaaaagaaagaggtgatttcctccagtcaggtttagaccaacacctccggccaagagagagattagcattacctgagggcctctggagtggttaaatgcctctaccaagtccattctctgcttgggattgacagagccatcgatggtggcataagtcagtccatgcttcttcaggtgcaatgctacaactttcagcatgttggtccactgagagacaatgacactcttttgggatgctgaatttctttgaattgcctccaattctgccaacagagatgaaatcttggtgctctctcgcatgccttcaaaaagctccatcttgaagaaggtgccgttaagggaaacagtggaagatggctctgagtcacggagttctgacaaggtcaaagcactgagctgttcttccagggaaaggacaagaccttcacccttcagttccattggatccagggccgacttcagtaaagaaagatgacagcaacactggcggagtctcagcaactgggacagtatgtggacggtgctggatctcggtgagtctgctgcctccgagtgtctaggctcctcagacccaaactccagtgccactctactgaatggattattagggcttcttccagattggttgcctctactttcatgtctttttagataggattgcagagctgaccttgatcttgcaaaaaacacattgtaaacagtctcttcatcttcagaaagctttaaatggtgcaactgaaatttacgctggggcagtatcaccaaaggtctgccagtagagtccagctggtcttttgttctcctcagcaaaaggctcttggttaaaatacttaaccgttctcctcctttctttgagccattgtcaacctgactcctccacagattgaactcatcaaatggagagcaacggagaaacttcagcagcgaatacatatccaataagttgttttgaatgggggttccagtgacagcccaacgggcacaggcttgtagcttacacacagctatggaagtctgcactcggggattcttaacattgtgagcttcatccaatatgattcgagcccaggctattcgaagcaaaggtgttgaggtgccctgaagtgggaatctggctgctcttgacgaaacagcacctgacccatagtggatactcaacgtctccacattgaggtttgcacctgggatctctgcctcttgcttgtttgtgggaatctccttggccacgaggctataggtagtgatcacgatgtcatatgtagagaggactctggcacgtgaatcccggtttggcccatggtagagatagactcttagtttgttgctgttcacccgtttctccacctcatttttccaatgatggatcagggaggcaggacagatgattagtgttccatgggaagtaaagtcacaagagtcatctttggagagccacgtcaaagctgtgcttttctccttttcttcctttttctcttgattcttctgggtcaggatgagcgcaatcattgtcagggtttttcctaagcccatatcatccagaattcctccttgtggcttctgactttctcgccatagtaaccaagccaatgcctgcttctggtgtagtagcaaagggaccttcagcccggcgggatcttctgccacaaccgtctcaccaggacatgactcaagtgagcgatgcagttgaccgatggcttcacttgtgattttccacactgcatgaacgtgatcttggtttgtatggcctcgatagcactgactggatcctccagcagtcacctggcaggcagactttagttctagagaacccacaggttgggtaccacgacgaggaaggggttggggaggcaccaggtggggagggccagtggtagttttggtgaagtgactctgctgtggtacttgactgttactcttctcattagttccttgctctggggaaagggtaagaccactgagtacttcctccagctcctggatttgtttgatcaacttctgacccttgtctggaagagcctggatgttcactgatgccagtgtgctcttcttttgtttcagttgtgttgtaaggtagacacgccgggctactgggtctgagggttctaccttcttggaaacacctgaggcaggagacacctttctttgcacacttcgatcagggaattggaggttttccttcgtctctaagtccagagtcgagtcaaagagtagggggctcccaggcttagaggaaacaaaaacaacatcatcttcctcctcgtcgtcactgcttgtggcagcttcacggccctcacccagggaaagccctggtgctgctggtgcagcctgagccgctggtcctccaggagcaggcacactgtgggtctccggccgctcttggaaatgcccctgaggcaggcttttctgggtggcctgtatgctagggccatcctttgcctttgtttctttagcctcccagttcgtgtactccttgttgaggggtccccctttctggggcttgcttattgagttgtgactgtgaacattttgaggcaaaagctgggtaaccttttctctcagaggttctgattctctttggacatcttgactcttaccacttgatttctcctgagaagatgcagatggtcttgtaagctcattaccttggcactgttgagatttaatttcagaaaagtctcttttgtgtgtgcctccagtctctgcctcacactgaatctctgctccctcttcttgcttcttctcttgaactacagattgttttttctttggtaccaggccagatgagaggtctttctccatcatttcaggcttctgttctttcttttgatcgaaaagctgatctcccttttctctttgcttcttatcagccttcttttcctcaccttcacctttgatgagctgtttccagagagctggttcttgattcttgtcaagtaccttgaatggatttctcagccagttggaagaatgatgaaatgtctcagatgcatgctgagacttattggatacagaatgttctttggaatcaggatcctgccatggaatacttccacaccagcgtttcccctctgccttacttctaatgcatcggaagaacaatctgtattctttcttgtcctgtggcagaagcaaaccctgaagctctaccacaaagtcctcatgcaataagcaatgggaaacaggaatgtcggtggcccgcacgaagctgcacgtgtctgcccggcacacgtagaagctctttcctttattcgggccatcgcggacgccggtcttaagaaagcagaaagtcccgtgctctggacacctaacttcttccatttcgctgggtcccccaagttccacaaagccccgcccccaattct

SEQ ID NO: 13173 - RNA, 3984 nt, Homo sapiens
  source 1..3984: mol_type = other RNA
gctgggattacaggcatgagccaccacacctggcccgctttttgaactttactgaagcttatatacaattctgccagagttgttttccaaaatcatccaactctaaaacatattcttttatctaaaaaaatcaattggtttccataccactcattaaataaattattaacataattggttaactaattggttaacacaacccctcctcaattctggggataagattatgcctcattttgaggaaggtgaaaggcttgacggtgaaattgaaatgcaaagaacagagttcaaggctcatggttaggttgttattcccagatcctaatacaaaccagcaatggtgctattctgagcccttatccacaggaggttagatgccaaaaaggactctgaggtcagccaaggtgagcttggtgacagattctccagaccctgatagaacttgtttggccaaatctttctttttttcttggagctgtaagatcttttcttctactgttccctcacaaacaaatctgtgtatgacaacatctttctgctgccctactcggtaaattcggtcacaagcttgatcttcaagtgatggattccagtgcatgtccaaaagaaagaggtgatttcctccagtcaggtttagaccaacacctccggccaagagagagattagcattacctgagggcctctggagtggttaaatgcctctaccaagtccattctctgcttgggattgacagagccatcgatggtggcataagtcagtccatgcttcttcaggtgcaatgctacaactttcagcatgttggtccactgagagacaatgacactcttttgggatgctgaatttctttgaattgcctccaattctgccaacagagatgaaatcttggtgctctctcgcatgccttcaaaaagctccatcttgaagaaggtgccgttaagggaaacagtggaagatggctctgagtcacggagttctgacaaggtcaaagcactgagctgttcttccagggaaaggacaagaccttcacccttcagttccattggatccagggccgacttcagtaaagaaagatgacagcaacactggcggagtctcagcaactgggacagtatgtggacggtgctggatctcggtgagtctgctgcctccgagtgtctaggctcctcagacccaaactccagtgccactctactgaatggattattagggcttcttccagattggttgcctctactttcatgtctttttagataggattgcagagctgaccttgatcttgcaaaaaacacattgtaaacagtctcttcatcttcagaaagctttaaatggtgcaactgaaatttacgctggggcagtatcaccaaaggtctgccagtagagtccagctggtcttttgttctcctcagcaaaaggctcttggttaaaatacttaaccgttctcctcctttctttgagccattgtcaacctgactcctccacagattgaactcatcaaatggagagcaacggagaaacttcagcagcgaatacatatccaataagttgttttgaatgggggttccagtgacagcccaacgggcacaggcttgtagcttacacacagctatggaagtctgcactcggggattcttaacattgtgagcttcatccaatatgattcgagcccaggctattcgaagcaaaggtgttgaggtgccctgaagtgggaatctggctgctcttgacgaaacagcacctgacccatagtggatactcaacgtctccacattgaggtttgcacctgggatctctgcctcttgcttgtttgtgggaatctccttggccacgaggctataggtagtgatcacgatgtcatatgtagagaggactctggcacgtgaatcccggtttggcccatggtagagatagactcttagtttgttgctgttcacccgtttctccacctcatttttccaatgatggatcagggaggcaggacagatgattagtgttccatgggaagtaaagtcacaagagtcatctttggagagccacgtcaaagctgtgcttttctccttttcttcctttttctcttgattcttctgggtcaggatgagcgcaatcattgtcagggtttttcctaagcccatatcatccagaattcctccttgtggcttctgactttctcgccatagtaaccaagccaatgcctgcttctggtgtagtagcaaagggaccttcagcccggcgggatcttctgccacaaccgtctcaccaggacatgactcaagtgagcgatgcagttgaccgatggcttcacttgtgattttccacactgcatgaacgtgatcttggtttgtatggcctgcatacaaataggtgttacctcgatagcactgactggatcctccagcagtcacctggcaggcagactttagttctagagaacccacaggttgggtaccacgacgaggaaggggttggggaggcaccaggtggggagggccagtggtagttttggtgaagtgactctgctgtggtacttgactgttactcttctcattagttccttgctctggggaaagggtaagaccactgagtacttcctccagctcctggatttgtttgatcaacttctgacccttgtctggaagagcctggatgttcactgatgccagtgtgctcttcttttgtttcagttgtgttgtaaggtagacacgccgggctactgggtctgagggttctaccttcttggaaacacctgaggcaggagacacctttctttgcacacttcgatcagggaattggaggttttccttcgtctctaagtccagagtcgagtcaaagagtagggggctcccaggcttagaggaaacaaaaacaacatcatcttcctcctcgtcgtcactgcttgtggcagcttcacggccctcacccagggaaagccctggtgctgctggtgcagcctgagccgctggtcctccaggagcaggcacactgtgggtctccggccgctcttggaaatgcccctgaggcaggcttttctgggtggcctgtatgctagggccatcctttgcctttgtttctttagcctcccagttcgtgtactccttgttgaggggtccccctttctggggcttgcttattgagttgtgactgtgaacattttgaggcaaaagctgggtaaccttttctctcagaggttctgattctctttggacatcttgactcttaccacttgatttctcctgagaagatgcagatggtcttgtaagctcattaccttggcactgttgagatttaatttcagaaaagtctcttttgtgtgtgcctccagtctctgcctcacactgaatctctgctccctcttcttgcttcttctcttgaactacagattgttttttctttggtaccaggccagatgagaggtctttctccatcatttcaggcttctgttctttcttttgatcgaaaagctgatctcccttttctctttgcttcttatcagccttcttttcctcaccttcacctttgatgagctgtttccagagagctggttcttgattcttgtcaagtaccttgaatggatttctcagccagttggaagaatgatgaaatgtctcagatgcatgctgagacttattggatacagaatgttctttggaatcaggatcctgccatggaatacttccacaccagcgtttcccctctgccttacttctaatgcatcggaagaacaatctgtattctttcttgtcctgtggcagaagcaaaccctgaagctctaccacaaagtcctcatgcaataagcaatgggaaacaggaatgtcggtggcccgcacgaagctgcacgtgtctgcccggcacacgtagaagctctttcctttattcgggccatcgcggacgccggtcttaagaaagcagaaagtcccgtgctctggacacctaacttcttccatttcgctgggtcccccaagttccacaaagccccgcccccaattct

SEQ ID NO: 13174 - RNA, 3966 nt, Homo sapiens
  source 1..3966: mol_type = other RNA
gctgggattacaggcatgagccaccacacctggcccgctttttgaactttactgaagcttatatacaattctgccagagttgttttccaaaatcatccaactctaaaacatattcttttatctaaaaaaatcaattggtttccataccactcattaaataaattattaacataattggttaactaattggttaacacaacccctcctcaattctggggataagattatgcctcattttgaggaaggtgaaaggcttgacggtgaaattgaaatgcaaagaacagagttcaaggctcatggttaggttgttattcccagatcctaatacaaaccagcaatggtgctattctgagcccttatccacaggaggttagatgccaaaaaggactctgaggtcagccaaggtgagcttggtgacagattctccagaccctgatagaacttgtttggccaaatctttctttttttcttggagctgtaagatcttttcttctactgttccctcacaaacaaatctgtgtatgacaacatctttctgctgccctactcggtaaattcggtcacaagcttgatcttcaagtgatggattccagtgcatgtccaaaagaaagaggtgatttcctccagtcaggtttagaccaacacctccggccaagagagagattagcattacctgagggcctctggagtggttaaatgcctctaccaagtccattctctgcttgggattgacagagccatcgatggtggcataagtcagtccatgcttcttcaggtgcaatgctacaactttcagcatgttggtccactgagagacaatgacactcttttgggatgctgaatttctttgaattgcctccaattctgccaacagagatgaaatcttggtgctctctcgcatgccttcaaaaagctccatcttgaagaaggtgccgttaagggaaacagtggaagatggctctgagtcacggagttctgacaaggtcaaagcactgagctgttcttccagggaaaggacaagaccttcacccttcagttccattggatccagggccgacttcagtaaagaaagatgacagcaacactggcggagtctcagcaactgggacagtatgtggacggtgctggatctcggtgagtctgctgcctccgagtgtctaggctcctcagacccaaactccagtgccactctactgaatggattattagggcttcttccagattggttgcctctactttcatgtctttttagataggattgcagagctgaccttgatcttgcaaaaaacacattgtaaacagtctcttcatcttcagaaagctttaaatggtgcaactgaaatttacgctggggcagtatcaccaaaggtctgccagtagagtccagctggtcttttgttctcctcagcaaaaggctcttggttaaaatacttaaccgttctcctcctttctttgagccattgtcaacctgactcctccacagattgaactcatcaaatggagagcaacggagaaacttcagcagcgaatacatatccaataagttgttttgaatgggggttccagtgacagcccaacgggcacaggcttgtagcttacacacagctatggaagtctgcactcggggattcttaacattgtgagcttcatccaatatgattcgagcccaggctattcgaagcaaaggtgttgaggtgccctgaagtgggaatctggctgctcttgacgaaacagcacctgacccatagtggatactcaacgtctccacattgaggtttgcacctgggatctctgcctcttgcttgtttgtgggaatctccttggccacgaggctataggtagtgatcacgatgtcatatgtagagaggactctggcacgtgaatcccggtttggcccatggtagagatagactcttagtttgttgctgttcacccgtttctccacctcatttttccaatgatggatcagggaggcaggacagatgattagtgttccatgggaagtaaagtcacaagagtcatctttggagagccacgtcaaagctgtgcttttctccttttcttcctttttctcttgattcttctgggtcaggatgagcgcaatcattgtcagggtttttcctaagcccatatcatctgccagaattcctccttgtggcttctgactttctcgccatagtaaccaagccaatgcctgcttctggtgtagtagcaaagggaccttcagcccggcgggatcttctgccacaaccgtctcaccaggacatgactcaagtgagcgatgcagttgaccgatggcttcacttgtgattttccacactgcatgaacgtgatcttggtttgtatggcctcgatagcactgactggatcctccagcagtcacctggcaggcagactttagttctagagaacccacaggttgggtaccacgacgaggaaggggttggggaggcaccaggtggggagggccagtggtagttttggtgaagtgactctgctgtggtacttgactgttactcttctcattagttccttgctctggggaaagggtaagaccactgagtacttcctccagctcctggatttgtttgatcaacttctgacccttgtctggaagagcctggatgttcactgatgccagtgtgctcttcttttgtttcagttgtgttgtaaggtagacacgccgggctactgggtctgagggttctaccttcttggaaacacctgaggcaggagacacctttctttgcacacttcgatcagggaattggaggttttccttcgtctctaagtccagagtcgagtcaaagagtagggggctcccaggcttagaggaaacaaaaacaacatcatcttcctcctcgtcgtcactgcttgtggcagcttcacggccctcacccagggaaagccctggtgctgctggtgcagcctgagccgctggtcctccaggagcaggcacactgtgggtctccggccgctcttggaaatgcccctgaggcaggcttttctgggtggcctgtatgctagggccatcctttgcctttgtttctttagcctcccagttcgtgtactccttgttgaggggtccccctttctggggcttgcttattgagttgtgactgtgaacattttgaggcaaaagctgggtaaccttttctctcagaggttctgattctctttggacatcttgactcttaccacttgatttctcctgagaagatgcagatggtcttgtaagctcattaccttggcactgttgagatttaatttcagaaaagtctcttttgtgtgtgcctccagtctctgcctcacactgaatctctgctccctcttcttgcttcttctcttgaactacagattgttttttctttggtaccaggccagatgagaggtctttctccatcatttcaggcttctgttctttcttttgatcgaaaagctgatctcccttttctctttgcttcttatcagccttcttttcctcaccttcacctttgatgagctgtttccagagagctggttcttgattcttgtcaagtaccttgaatggatttctcagccagttggaagaatgatgaaatgtctcagatgcatgctgagacttattggatacagaatgttctttggaatcaggatcctgccatggaatacttccacaccagcgtttcccctctgccttacttctaatgcatcggaagaacaatctgtattctttcttgtcctgtggcagaagcaaaccctgaagctctaccacaaagtcctcatgcaataagcaatgggaaacaggaatgtcggtggcccgcacgaagctgcacgtgtctgcccggcacacgtagaagctctttcctttattcgggccatcgcggacgccggtcttaagaaagcagaaagtcccgtgctctggacacctaacttcttccatttcgctgggtcccccaagttccacaaagccccgcccccaattct

SEQ ID NO: 13175 - RNA, 3936 nt, Homo sapiens
  source 1..3936: mol_type = other RNA
gctgggattacaggcatgagccaccacacctggcccgctttttgaactttactgaagcttatatacaattctgccagagttgttttccaaaatcatccaactctaaaacatattcttttatctaaaaaaatcaattggtttccataccactcattaaataaattattaacataattggttaactaattggttaacacaacccctcctcaattctggggataagattatgcctcattttgaggaaggtgaaaggcttgacggtgaaattgaaatgcaaagaacagagttcaaggctcatggttaggttgttattcccagatcctaatacaaaccagcaatggtgctattctgagcccttatccacaggaggttagatgccaaaaaggactctgaggtcagccaaggtgagcttggtgacagattctccagaccctgatagaacttgtttggccaaatctttctttttttcttggagctgtaagatcttttcttctactgttccctcacaaacaaatctgtgtatgacaacatctttctgctgccctactcggtaaattcggtcacaagcttgatcttcaagtgatggattcctctttaaaatcttggataacatttctctatctcagtgcatgtccaaaagaaagaggtgatttcctccagtcaggtttagaccaacacctccggccaagagagagattagcattacctgagggcctctggagtggttaaatgcctctaccaagtccattctctgcttgggattgacagagccatcgatggtggcataagtcagtccatgcttcttcaggtgcaatgctacaactttcagcatgttggtccactgagagacaatgacactcttttgggatgctgaatttctttgaattgcctccaattctgccaacagagatgaaatcttggtgctctctcgcatgccttcaaaaagctccatcttgaagaaggtgccgttaagggaaacagtggaagatggctctgagtcacggagttctgacaaggtcaaagcactgagctgttcttccagggaaaggacaagaccttcacccttcagttccattggatccagggccgacttcagtaaagaaagatgacagcaacactggcggagtctcagcaactgggacagtatgtggacggtgctggatctcggtgagtctgctgcctccgagtgtctaggctcctcagacccaaactccagtgccactctactgaatggattattagggcttcttccagattggttgcctctactttcatgtctttttagataggattgcagagctgaccttgatcttgcaaaaaacacattgtaaacagtctcttcatcttcagaaagctttaaatggtgcaactgaaatttacgctggggcagtatcaccaaaggtctgccagtagagtccagctggtcttttgttctcctcagcaaaaggctcttggttaaaatacttaaccgttctcctcctttctttgagccattgtcaacctgactcctccacagattgaactcatcaaatggagagcaacggagaaacttcagcagcgaatacatatccaataagttgttttgaatgggggttccagtgacagcccaacgggcacaggcttgtagcttacacacagctatggaagtctgcactcggggattcttaacattgtgagcttcatccaatatgattcgagcccaggctattcgaagcaaaggtgttgaggtgccctccacattgaggtttgcacctgggatctctgcctcttgcttgtttgtgggaatctccttggccacgaggctataggtagtgatcacgatgtcatatgtagagaggactctggcacgtgaatcccggtttggcccatggtagagatagactcttagtttgttgctgttcacccgtttctccacctcatttttccaatgatggatcagggaggcaggacagatgattagtgttccatgggaagtaaagtcacaagagtcatctttggagagccacgtcaaagctgtgcttttctccttttcttcctttttctcttgattcttctgggtcaggatgagcgcaatcattgtcagggtttttcctaagcccatatcatctgccagaattcctccttgtggcttctgactttctcgccatagtaaccaagccaatgcctgcttctggtgtagtagcaaagggaccttcagcccggcgggatcttctgccacaaccgtctcaccaggacatgactcaagtgagcgatgcagttgaccgatggcttcacttgtgattttccacactgcatgaacgtgatcttggtttgtatggcctcgatagcactgactggatcctccagcagtcacctggcaggcagactttagttctagagaacccacaggttgggtaccacgacgaggaaggggttggggaggcaccaggtggggagggccagtggtagttttggtgaagtgactctgctgtggtacttgactgttactcttctcattagttccttgctctggggaaagggtaagaccactgagtacttcctccagctcctggatttgtttgatcaacttctgacccttgtctggaagagcctggatgttcactgatgccagtgtgctcttcttttgtttcagttgtgttgtaaggtagacacgccgggctactgggtctgagggttctaccttcttggaaacacctgaggcaggagacacctttctttgcacacttcgatcagggaattggaggttttccttcgtctctaagtccagagtcgagtcaaagagtagggggctcccaggcttagaggaaacaaaaacaacatcatcttcctcctcgtcgtcactgcttgtggcagcttcacggccctcacccagggaaagccctggtgctgctggtgcagcctgagccgctggtcctccaggagcaggcacactgtgggtctccggccgctcttggaaatgcccctgaggcaggcttttctgggtggcctgtatgctagggccatcctttgcctttgtttctttagcctcccagttcgtgtactccttgttgaggggtccccctttctggggcttgcttattgagttgtgactgtgaacattttgaggcaaaagctgggtaaccttttctctcagaggttctgattctctttggacatcttgactcttaccacttgatttctcctgagaagatgcagatggtcttgtaagctcattaccttggcactgttgagatttaatttcagaaaagtctcttttgtgtgtgcctccagtctctgcctcacactgaatctctgctccctcttcttgcttcttctcttgaactacagattgttttttctttggtaccaggccagatgagaggtctttctccatcatttcaggcttctgttctttcttttgatcgaaaagctgatctcccttttctctttgcttcttatcagccttcttttcctcaccttcacctttgatgagctgtttccagagagctggttcttgattcttgtcaagtaccttgaatggatttctcagccagttggaagaatgatgaaatgtctcagatgcatgctgagacttattggatacagaatgttctttggaatcaggatcctgccatggaatacttccacaccagcgtttcccctctgccttacttctaatgcatcggaagaacaatctgtattctttcttgtcctgtggcagaagcaaaccctgaagctctaccacaaagtcctcatgcaataagcaatgggaaacaggaatgtcggtggcccgcacgaagctgcacgtgtctgcccggcacacgtagaagctctttcctttattcgggccatcgcggacgccggtcttaagaaagcagaaagtcccgtgctctggacacctaacttcttccatttcgctgggtcccccaagttccacaaagccccgcccccaattct

SEQ ID NO: 13176 - RNA, 4020 nt, Homo sapiens
  source 1..4020: mol_type = other RNA
gctgggattacaggcatgagccaccacacctggcccgctttttgaactttactgaagcttatatacaattctgccagagttgttttccaaaatcatccaactctaaaacatattcttttatctaaaaaaatcaattggtttccataccactcattaaataaattattaacataattggttaactaattggttaacacaacccctcctcaattctggggataagattatgcctcattttgaggaaggtgaaaggcttgacggtgaaattgaaatgcaaagaacagagttcaaggctcatggttaggttgttattcccagatcctaatacaaaccagcaatggtgctattctgagcccttatccacaggaggttagatgccaaaaaggactctgaggtcagccaaggtgagcttggtgacagattctccagaccctgatagaacttgtttggccaaatctttctttttttcttggagctgtaagatcttttcttctactgttccctcacaaacaaatctgtgtatgacaacatctttctgctgccctactcggtaaattcggtcacaagcttgatcttcaagtgatggattcctctttaaaatcttggataacatttctctatctcagtgcatgtccaaaagaaagaggtgatttcctccagtcaggtttagaccaacacctccggccaagagagagattagcattacctgagggcctctggagtggttaaatgcctctaccaagtccattctctgcttgggattgacagagccatcgatggtggcataagtcagtccatgcttcttcaggtgcaatgctacaactttcagcatgttggtccactgagagacaatgacactcttttgggatgctgaatttctttgaattgcctccaattctgccaacagagatgaaatcttggtgctctctcgcatgccttcaaaaagctccatcttgaagaaggtgccgttaagggaaacagtggaagatggctctgagtcacggagttctgacaaggtcaaagcactgagctgttcttccagggaaaggacaagaccttcacccttcagttccattggatccagggccgacttcagtaaagaaagatgacagcaacactggcggagtctcagcaactgggacagtatgtggacggtgctggatctcggtgagtctgctgcctccgagtgtctaggctcctcagacccaaactccagtgccactctactgaatggattattagggcttcttccagattggttgcctctactttcatgtctttttagataggattgcagagctgaccttgatcttgcaaaaaacacattgtaaacagtctcttcatcttcagaaagctttaaatggtgcaactgaaatttacgctggggcagtatcaccaaaggtctgccagtagagtccagctggtcttttgttctcctcagcaaaaggctcttggttaaaatacttaaccgttctcctcctttctttgagccattgtcaacctgactcctccacagattgaactcatcaaatggagagcaacggagaaacttcagcagcgaatacatatccaataagttgttttgaatgggggttccagtgacagcccaacgggcacaggcttgtagcttacacacagctatggaagtctgcactcggggattcttaacattgtgagcttcatccaatatgattcgagcccaggctattcgaagcaaaggtgttgaggtgccctgaagtgggaatctggctgctcttgacgaaacagcacctgacccatagtggatactcaacgtctccacattgaggtttgcacctgggatctctgcctcttgcttgtttgtgggaatctccttggccacgaggctataggtagtgatcacgatgtcatatgtagagaggactctggcacgtgaatcccggtttggcccatggtagagatagactcttagtttgttgctgttcacccgtttctccacctcatttttccaatgatggatcagggaggcaggacagatgattagtgttccatgggaagtaaagtcacaagagtcatctttggagagccacgtcaaagctgtgcttttctccttttcttcctttttctcttgattcttctgggtcaggatgagcgcaatcattgtcagggtttttcctaagcccatatcatctgccagaattcctccttgtggcttctgactttctcgccatagtaaccaagccaatgcctgcttctggtgtagtagcaaagggaccttcagcccggcgggatcttctgccacaaccgtctcaccaggacatgactcaagtgagcgatgcagttgaccgatggcttcacttgtgattttccacactgcatgaacgtgatcttggtttgtatggcctgcatacaaataggtgttacctcgatagcactgactggatcctccagcagtcacctggcaggcagactttagttctagagaacccacaggttgggtaccacgacgaggaaggggttggggaggcaccaggtggggagggccagtggtagttttggtgaagtgactctgctgtggtacttgactgttactcttctcattagttccttgctctggggaaagggtaagaccactgagtacttcctccagctcctggatttgtttgatcaacttctgacccttgtctggaagagcctggatgttcactgatgccagtgtgctcttcttttgtttcagttgtgttgtaaggtagacacgccgggctactgggtctgagggttctaccttcttggaaacacctgaggcaggagacacctttctttgcacacttcgatcagggaattggaggttttccttcgtctctaagtccagagtcgagtcaaagagtagggggctcccaggcttagaggaaacaaaaacaacatcatcttcctcctcgtcgtcactgcttgtggcagcttcacggccctcacccagggaaagccctggtgctgctggtgcagcctgagccgctggtcctccaggagcaggcacactgtgggtctccggccgctcttggaaatgcccctgaggcaggcttttctgggtggcctgtatgctagggccatcctttgcctttgtttctttagcctcccagttcgtgtactccttgttgaggggtccccctttctggggcttgcttattgagttgtgactgtgaacattttgaggcaaaagctgggtaaccttttctctcagaggttctgattctctttggacatcttgactcttaccacttgatttctcctgagaagatgcagatggtcttgtaagctcattaccttggcactgttgagatttaatttcagaaaagtctcttttgtgtgtgcctccagtctctgcctcacactgaatctctgctccctcttcttgcttcttctcttgaactacagattgttttttctttggtaccaggccagatgagaggtctttctccatcatttcaggcttctgttctttcttttgatcgaaaagctgatctcccttttctctttgcttcttatcagccttcttttcctcaccttcacctttgatgagctgtttccagagagctggttcttgattcttgtcaagtaccttgaatggatttctcagccagttggaagaatgatgaaatgtctcagatgcatgctgagacttattggatacagaatgttctttggaatcaggatcctgccatggaatacttccacaccagcgtttcccctctgccttacttctaatgcatcggaagaacaatctgtattctttcttgtcctgtggcagaagcaaaccctgaagctctaccacaaagtcctcatgcaataagcaatgggaaacaggaatgtcggtggcccgcacgaagctgcacgtgtctgcccggcacacgtagaagctctttcctttattcgggccatcgcggacgccggtcttaagaaagcagaaagtcccgtgctctggacacctaacttcttccatttcgctgggtcccccaagttccacaaagccccgcccccaattct

SEQ ID NO: 13177 - RNA, 4614 nt, Homo sapiens
  source 1..4614: mol_type = other RNA
gctgggattacaggcatgagccaccacacctggcccgctttttgaactttactgaagcttatatacaattctgccagagttgttttccaaaatcatccaactctaaaacatattcttttatctaaaaaaatcaattggtttccataccactcattaaataaattattaacataattggttaactaattggttaacacaacccctcctcaattctggggataagattatgcctcattttgaggaaggtgaaaggcttgacggtgaaattgaaatgcaaagaacagagttcaaggctcatggttaggttgttattcccagatcctaatacaaaccagcaatggtgctattctgagcccttatccacaggaggttagatgccaaaaaggactctgaggtcagccaaggtgagcttggtgacagattctccagaccctgatagaacttgtttggccaaatctttctttttttcttggagctgtaagatcttttcttctactgttccctcacaaacaaatctgtgtatgacaacatctttctgctgccctactcggtaaattcggtcacaagcttgatcttcaagtgatggattcctgttagaagacagctaaagctcaaaggaactgacatactagatcagaaatggcaaactatgggccatgggccaaatccagcccacagcttgtttttgtagctaaaaattattgttacagttttaaagggatttaagaaaagaaagcaaagcaaaacaaaacacacacatcatgtgacagagaactatgtggcctgaaaagcctcaaagaaaaaaaatctgtcgatccctgtcctaagctatactggcctaagacaagctggtgccagataccttcttgcctagtttctagtgagaaactagggtcagactgttaataatagctcttagcactatcatcagttgacaactcttaagtaacagaggtgaaaccaaaactcaggtctggtctctaggtagctagatgtccttgggcaagttatttaacctcagtcctctaggcttcagattgctacttggaaattgaagggccagctaatgatcttgactagctgcctttttcaacttgaatattctgtgattcgattaaggagacttaatttgtttccttctttattgattcccattgtaactccaaattagtttctcatcttacctctttaaaatcttggataacatttctctatctcagtgcatgtccaaaagaaagaggtgatttcctccagtcaggtttagaccaacacctccggccaagagagagattagcattacctgagggcctctggagtggttaaatgcctctaccaagtccattctctgcttgggattgacagagccatcgatggtggcataagtcagtccatgcttcttcaggtgcaatgctacaactttcagcatgttggtccactgagagacaatgacactcttttgggatgctgaatttctttgaattgcctccaattctgccaacagagatgaaatcttggtgctctctcgcatgccttcaaaaagctccatcttgaagaaggtgccgttaagggaaacagtggaagatggctctgagtcacggagttctgacaaggtcaaagcactgagctgttcttccagggaaaggacaagaccttcacccttcagttccattggatccagggccgacttcagtaaagaaagatgacagcaacactggcggagtctcagcaactgggacagtatgtggacggtgctggatctcggtgagtctgctgcctccgagtgtctaggctcctcagacccaaactccagtgccactctactgaatggattattagggcttcttccagattggttgcctctactttcatgtctttttagataggattgcagagctgaccttgatcttgcaaaaaacacattgtaaacagtctcttcatcttcagaaagctttaaatggtgcaactgaaatttacgctggggcagtatcaccaaaggtctgccagtagagtccagctggtcttttgttctcctcagcaaaaggctcttggttaaaatacttaaccgttctcctcctttctttgagccattgtcaacctgactcctccacagattgaactcatcaaatggagagcaacggagaaacttcagcagcgaatacatatccaataagttgttttgaatgggggttccagtgacagcccaacgggcacaggcttgtagcttacacacagctatggaagtctgcactcggggattcttaacattgtgagcttcatccaatatgattcgagcccaggctattcgaagcaaaggtgttgaggtgccctgaagtgggaatctggctgctcttgacgaaacagcacctgacccatagtggatactcaacgtctccacattgaggtttgcacctgggatctctgcctcttgcttgtttgtgggaatctccttggccacgaggctataggtagtgatcacgatgtcatatgtagagaggactctggcacgtgaatcccggtttggcccatggtagagatagactcttagtttgttgctgttcacccgtttctccacctcatttttccaatgatggatcagggaggcaggacagatgattagtgttccatgggaagtaaagtcacaagagtcatctttggagagccacgtcaaagctgtgcttttctccttttcttcctttttctcttgattcttctgggtcaggatgagcgcaatcattgtcagggtttttcctaagcccatatcatctgccagaattcctccttgtggcttctgactttctcgccatagtaaccaagccaatgcctgcttctggtgtagtagcaaagggaccttcagcccggcgggatcttctgccacaaccgtctcaccaggacatgactcaagtgagcgatgcagttgaccgatggcttcacttgtgattttccacactgcatgaacgtgatcttggtttgtatggcctgcatacaaataggtgttacctcgatagcactgactggatcctccagcagtcacctggcaggcagactttagttctagagaacccacaggttgggtaccacgacgaggaaggggttggggaggcaccaggtggggagggccagtggtagttttggtgaagtgactctgctgtggtacttgactgttactcttctcattagttccttgctctggggaaagggtaagaccactgagtacttcctccagctcctggatttgtttgatcaacttctgacccttgtctggaagagcctggatgttcactgatgccagtgtgctcttcttttgtttcagttgtgttgtaaggtagacacgccgggctactgggtctgagggttctaccttcttggaaacacctgaggcaggagacacctttctttgcacacttcgatcagggaattggaggttttccttcgtctctaagtccagagtcgagtcaaagagtagggggctcccaggcttagaggaaacaaaaacaacatcatcttcctcctcgtcgtcactgcttgtggcagcttcacggccctcacccagggaaagccctggtgctgctggtgcagcctgagccgctggtcctccaggagcaggcacactgtgggtctccggccgctcttggaaatgcccctgaggcaggcttttctgggtggcctgtatgctagggccatcctttgcctttgtttctttagcctcccagttcgtgtactccttgttgaggggtccccctttctggggcttgcttattgagttgtgactgtgaacattttgaggcaaaagctgggtaaccttttctctcagaggttctgattctctttggacatcttgactcttaccacttgatttctcctgagaagatgcagatggtcttgtaagctcattaccttggcactgttgagatttaatttcagaaaagtctcttttgtgtgtgcctccagtctctgcctcacactgaatctctgctccctcttcttgcttcttctcttgaactacagattgttttttctttggtaccaggccagatgagaggtctttctccatcatttcaggcttctgttctttcttttgatcgaaaagctgatctcccttttctctttgcttcttatcagccttcttttcctcaccttcacctttgatgagctgtttccagagagctggttcttgattcttgtcaagtaccttgaatggatttctcagccagttggaagaatgatgaaatgtctcagatgcatgctgagacttattggatacagaatgttctttggaatcaggatcctgccatggaatacttccacaccagcgtttcccctctgccttacttctaatgcatcggaagaacaatctgtattctttcttgtcctgtggcagaagcaaaccctgaagctctaccacaaagtcctcatgcaataagcaatgggaaacaggaatgtcggtggcccgcacgaagctgcacgtgtctgcccggcacacgtagaagctctttcctttattcgggccatcgcggacgccggtcttaagaaagcagaaagtcccgtgctctggacacctaacttcttccatttcgctgggtcccccaagttccacaaagccccgcccccaattct

SEQ ID NO: 13178 - RNA, 2103 nt, Homo sapiens
  source 1..2103: mol_type = other RNA
gctgggattacaggcatgagccaccacacctggccgatgcttttaaatttacaatatgtaaaaatgttaaaatatatggtgctctcttcagtgtgaattttctgatattgaggaaatagcaaaagtgaagatcctaggtgctgcaatgacaagcattacggtattttctttttaaaatgctctccagtatgtctcgaaaatattcgtaaatcagcagcaatgaattttttttctaagtgggagagatcacagaagcttcttttttgcccacttttctgtctcaatttctctaaaatgaacatgcactgcttttgatttaagaaaagaggtttgtttaatgagaaacgtcctttcactctgtgaaaacatcgtgtggataatacataaagggcagagtcaggtgccgggggcgcatgcaggaagtgctcagctggactctgccctcggacaccgcgccactgttacatggagaagtcctcccggaggtgaatccgctgatgctgacacatgttggaactgtgccggaaggccttcccacactcgctgcacttgtagggcttctccccggtgtggatcctccggtgctgaatcaagtacgtgctctggctgaaggctttcttgcaatcgctgcatctgtagggtttctctccgtggtgcagcctctggtggtggatgagtctggaactgttgtggaaggccttcccacactcgctgcacttgtagggcttctctcctgtgtggattctctggtgctggatgaggtgtgtgctttggctgaaaactttgccacagtcattgcattcatagggcttctctccagtgtggcttctctgatgttccacgagtttggttttttgaatgaaagctttctcacattcattacatttatagggtttctctccagtgtgaattctctgatgttggataaggttagaactttgtgtaaagcctttgccacattccttgcactcaaatggcttctctccggtgtgagtccgacgatgtcggataaggattgagccatcactgaaggctttcccgcagtcattacatttatagggtttctctccggtgtggattctctggtgataaatcagggaagagtaggcgctaaagtgcttcccacactccccacacttgtagggtttctccccagtgtgaatcctctggtgcttcatgaggttgggcctccgggtgaatgtcttcccacactcgtcacaccggtagggaatctctcctgagtgcatccttcggtgattgatgaactcgcagctctggctgaaggctttcccacactcatcacatttgtagggcttctcttcagtgtgaagccgctgatgcttgacaaggttggcactgtacctgaatgttttcccacagtaactgcaataatgcaattttttcccagtaggaattttctgatcttctttaacaactaagtttgcactgaagatttccccagagttacgaactgtatttgttttttttgacctgtgtacacgcttatggttgttgagatatgatctctgttcaaaactttgctcacatatatcacatttgtgaggtctctgatcaggaacaggtcttgacagcaacctgaggtttcccccagactccctgctgctctccccgttggtcagtgtgactgccctggggcctctctgctccactagcttttccaggctcccctctgacttactgatgtggtcacaggcttctactggctcagatccctggggatcttcctcaccaaatgtctcctgtgaagtcaactccttgtactcagttctggtcccaagagccagtgagactaggttcccgtaggtctccagcatcacgtccctgtagaggcccctctgagcagggcccaggcggccccattcctcccgggagaggtacacagccacgtcctcgaaggtcacctcggcctggggtggggcagacaggaacaaggccgccattgcctgagggttgggctttctgagggcagtgagcaggagctggtcactgaggagcagaagcatgagactctcggattagatacatgtgatgcaactatttggcctcagcgccgccgagcagcacggcagcccaacctcgccc

SEQ ID NO: 13179 - RNA, 2107 nt, Homo sapiens
  source 1..2107: mol_type = other RNA
gctgggattacaggcatgagccaccacacctggccgatgcttttaaatttacaatatgtaaaaatgttaaaatatatggtgctctcttcagtgtgaattttctgatattgaggaaatagcaaaagtgaagatcctaggtgctgcaatgacaagcattacggtattttctttttaaaatgctctccagtatgtctcgaaaatattcgtaaatcagcagcaatgaattttttttctaagtgggagagatcacagaagcttcttttttgcccacttttctgtctcaatttctctaaaatgaacatgcactgcttttgatttaagaaaagaggtttgtttaatgagaaacgtcctttcactctgtgaaaacatcgtgtggataatacataaagggcagagtcaggtgccgggggcgcatgcaggaagtgctcagctggactctgccctcggacaccgcgccactgttacatggagaagtcctcccggaggtgaatccgctgatgctgacacatgttggaactgtgccggaaggccttcccacactcgctgcacttgtagggcttctccccggtgtggatcctccggtgctgaatcaagtacgtgctctggctgaaggctttcttgcaatcgctgcatctgtagggtttctctccgtggtgcagcctctggtggtggatgagtctggaactgttgtggaaggccttcccacactcgctgcacttgtagggcttctctcctgtgtggattctctggtgctggatgaggtgtgtgctttggctgaaaactttgccacagtcattgcattcatagggcttctctccagtgtggcttctctgatgttccacgagtttggttttttgaatgaaagctttctcacattcattacatttatagggtttctctccagtgtgaattctctgatgttggataaggttagaactttgtgtaaagcctttgccacattccttgcactcaaatggcttctctccggtgtgagtccgacgatgtcggataaggattgagccatcactgaaggctttcccgcagtcattacatttatagggtttctctccggtgtggattctctggtgataaatcagggaagagtaggcgctaaagtgcttcccacactccccacacttgtagggtttctccccagtgtgaatcctctggtgcttcatgaggttgggcctccgggtgaatgtcttcccacactcgtcacaccggtagggaatctctcctgagtgcatccttcggtgattgatgaactcgcagctctggctgaaggctttcccacactcatcacatttgtagggcttctcttcagtgtgaagccgctgatgcttgacaaggttggcactgtacctgaatgttttcccacagtaactgcaataatgcaattttttcccagtaggaattttctgatcttctttaacaactaagtttgcactgaagatttccccagagttacgaactgtatttgttttttttgacctgtgtacacgcttatggttgttgagatatgatctctgttcaaaactttgctcacatatatcacatttgtgaggtctctgatcaggaacaggtcttgacagcaacctgaggtttcccccagactccctgctgctctccccgttggtcagtgtgactgccctggggcctctctgctccactagcttttccaggctcccctctgacttactgatgtggtcacaggcttctactggctcagatccctggggatcttcctcaccaaatgtctcctgtgaagtcaactccttgtactcagttctggtcccaagagccagtgagactaggttcccgtaggtctccagcatcacgtccctgtagaggcccctctgagcagggcccaggcggccccattcctcccgggagaggtacacagccacgtcctcgaaggtcacctcggcctggggtggggcagacaggaacaaggccgccattgcctgagggttgggctttctgagggcagtgagcaggagctggtcactgaggagctaccagaagcatgagactctcggattagatacatgtgatgcaactatttggcctcagcgccgccgagcagcacggcagcccaacctcgccc

SEQ ID NO: 13180 - RNA, 2223 nt, Homo sapiens
  source 1..2223: mol_type = other RNA
gctgggattacaggcatgagccaccacacctggccgatgcttttaaatttacaatatgtaaaaatgttaaaatatatggtgctctcttcagtgtgaattttctgatattgaggaaatagcaaaagtgaagatcctaggtgctgcaatgacaagcattacggtattttctttttaaaatgctctccagtatgtctcgaaaatattcgtaaatcagcagcaatgaattttttttctaagtgggagagatcacagaagcttcttttttgcccacttttctgtctcaatttctctaaaatgaacatgcactgcttttgatttaagaaaagaggtttgtttaatgagaaacgtcctttcactctgtgaaaacatcgtgtggataatacataaagggcagagtcaggtgccgggggcgcatgcaggaagtgctcagctggactctgccctcggacaccgcgccactgttacatggagaagtcctcccggaggtgaatccgctgatgctgacacatgttggaactgtgccggaaggccttcccacactcgctgcacttgtagggcttctccccggtgtggatcctccggtgctgaatcaagtacgtgctctggctgaaggctttcttgcaatcgctgcatctgtagggtttctctccgtggtgcagcctctggtggtggatgagtctggaactgttgtggaaggccttcccacactcgctgcacttgtagggcttctctcctgtgtggattctctggtgctggatgaggtgtgtgctttggctgaaaactttgccacagtcattgcattcatagggcttctctccagtgtggcttctctgatgttccacgagtttggttttttgaatgaaagctttctcacattcattacatttatagggtttctctccagtgtgaattctctgatgttggataaggttagaactttgtgtaaagcctttgccacattccttgcactcaaatggcttctctccggtgtgagtccgacgatgtcggataaggattgagccatcactgaaggctttcccgcagtcattacatttatagggtttctctccggtgtggattctctggtgataaatcagggaagagtaggcgctaaagtgcttcccacactccccacacttgtagggtttctccccagtgtgaatcctctggtgcttcatgaggttgggcctccgggtgaatgtcttcccacactcgtcacaccggtagggaatctctcctgagtgcatccttcggtgattgatgaactcgcagctctggctgaaggctttcccacactcatcacatttgtagggcttctcttcagtgtgaagccgctgatgcttgacaaggttggcactgtacctgaatgttttcccacagtaactgcaataatgcaattttttcccagtaggaattttctgatcttctttaacaactaagtttgcactgaagatttccccagagttacgaactgtatttgttttttttgacctgtgtacacgcttatggttgttgagatatgatctctgttcaaaactttgctcacatatatcacatttgtgaggtctctgatcaggaacaggtcttgacagcaacctgaggtttcccccagactccctgctgctctccccgttggtcagtgtgactgccctggggcctctctgctccactagcttttccaggctcccctctgacttactgatgtggtcacaggcttctactggctcagatccctggggatcttcctcaccaaatgtctcctgtgaagtcaactccttgtactcagttctggtcccaagagctgggctgttgactctcaggtgctctttcccagaggtgccctgaacatccaggacccagggctcatcccctcgctccaactgcgagatcactccaggcttggggcctgcaggtcctactcccagtgagactaggttcccgtaggtctccagcatcacgtccctgtagaggcccctctgagcagggcccaggcggccccattcctcccgggagaggtacacagccacgtcctcgaaggtcacctcggcctggggtggggcagacaggaacaaggccgccattgcctgagggttgggctttctgagggcagtgagcaggagctggtcactgaggagcagaagcatgagactctcggattagatacatgtgatgcaactatttggcctcagcgccgccgagcagcacggcagcccaacctcgccc

SEQ ID NO: 13181 - RNA, 2274 nt, Homo sapiens
  source 1..2274: mol_type = other RNA
gctgggattacaggcatgagccaccacacctggccgatgcttttaaatttacaatatgtaaaaatgttaaaatatatggtgctctcttcagtgtgaattttctgatattgaggaaatagcaaaagtgaagatcctaggtgctgcaatgacaagcattacggtattttctttttaaaatgctctccagtatgtctcgaaaatattcgtaaatcagcagcaatgaattttttttctaagtgggagagatcacagaagcttcttttttgcccacttttctgtctcaatttctctaaaatgaacatgcactgcttttgatttaagaaaagaggtttgtttaatgagaaacgtcctttcactctgtgaaaacatcgtgtggataatacataaagggcagagtcaggtgccgggggcgcatgcaggaagtgctcagctggactctgccctcggacaccgcgccactgttacatggagaagtcctcccggaggtgaatccgctgatgctgacacatgttggaactgtgccggaaggccttcccacactcgctgcacttgtagggcttctccccggtgtggatcctccggtgctgaatcaagtacgtgctctggctgaaggctttcttgcaatcgctgcatctgtagggtttctctccgtggtgcagcctctggtggtggatgagtctggaactgttgtggaaggccttcccacactcgctgcacttgtagggcttctctcctgtgtggattctctggtgctggatgaggtgtgtgctttggctgaaaactttgccacagtcattgcattcatagggcttctctccagtgtggcttctctgatgttccacgagtttggttttttgaatgaaagctttctcacattcattacatttatagggtttctctccagtgtgaattctctgatgttggataaggttagaactttgtgtaaagcctttgccacattccttgcactcaaatggcttctctccggtgtgagtccgacgatgtcggataaggattgagccatcactgaaggctttcccgcagtcattacatttatagggtttctctccggtgtggattctctggtgataaatcagggaagagtaggcgctaaagtgcttcccacactccccacacttgtagggtttctccccagtgtgaatcctctggtgcttcatgaggttgggcctccgggtgaatgtcttcccacactcgtcacaccggtagggaatctctcctgagtgcatccttcggtgattgatgaactcgcagctctggctgaaggctttcccacactcatcacatttgtagggcttctcttcagtgtgaagccgctgatgcttgacaaggttggcactgtacctgaatgttttcccacagtaactgcaataatgcaattttttcccagtaggaattttctgatcttctttaacaactaagtttgcactgaagatttccccagagttacgaactgtatttgttttttttgacctgtgtacacgcttatggttgttgagatatgatctctgttcaaaactttgctcacatatatcacatttgtgaggtctctgatcaggaacaggtcttgacagcaacctgaggtttcccccagactccctgctgctctccccgttggtcagtgtgactgccctggggcctctctgctccactagcttttccaggctcccctctgacttactgatgtggtcacaggcttctactggctcagatccctggggatcttcctcaccaaatgtctcctgtgaagtcaactccttgtactcagttctggtcccaagagctgggctgttgactctcaggtgctctttcccagaggtgccctgaacatccaggacccagggctcatcccctcgctccaactgcgagatcactccaggcttggggcctgcaggtcctactcccagtgagactaggttcccgtaggtctccagcatcacgtccctgtagaggcccctctgagcagggcccaggcggccccattcctcccgggagaggtacacagccacgtcctcgaaggtcacctcggcctggggtggggcagacaggaacaaggccgccattgcctgagggttgggctttctgagggcagtgagcaggagctggtcactgaggagctaccagaagcatgagactctcggattagatacatgtgatgcaactatttggcctaaagaaaattgtgcatccttaatagactcattttaacaggaaagcctcagcgccgccgagcagcacggcagcccaacctcgccc

SEQ ID NO: 13182 - RNA, 2227 nt, Homo sapiens
  source 1..2227: mol_type = other RNA
gctgggattacaggcatgagccaccacacctggccgatgcttttaaatttacaatatgtaaaaatgttaaaatatatggtgctctcttcagtgtgaattttctgatattgaggaaatagcaaaagtgaagatcctaggtgctgcaatgacaagcattacggtattttctttttaaaatgctctccagtatgtctcgaaaatattcgtaaatcagcagcaatgaattttttttctaagtgggagagatcacagaagcttcttttttgcccacttttctgtctcaatttctctaaaatgaacatgcactgcttttgatttaagaaaagaggtttgtttaatgagaaacgtcctttcactctgtgaaaacatcgtgtggataatacataaagggcagagtcaggtgccgggggcgcatgcaggaagtgctcagctggactctgccctcggacaccgcgccactgttacatggagaagtcctcccggaggtgaatccgctgatgctgacacatgttggaactgtgccggaaggccttcccacactcgctgcacttgtagggcttctccccggtgtggatcctccggtgctgaatcaagtacgtgctctggctgaaggctttcttgcaatcgctgcatctgtagggtttctctccgtggtgcagcctctggtggtggatgagtctggaactgttgtggaaggccttcccacactcgctgcacttgtagggcttctctcctgtgtggattctctggtgctggatgaggtgtgtgctttggctgaaaactttgccacagtcattgcattcatagggcttctctccagtgtggcttctctgatgttccacgagtttggttttttgaatgaaagctttctcacattcattacatttatagggtttctctccagtgtgaattctctgatgttggataaggttagaactttgtgtaaagcctttgccacattccttgcactcaaatggcttctctccggtgtgagtccgacgatgtcggataaggattgagccatcactgaaggctttcccgcagtcattacatttatagggtttctctccggtgtggattctctggtgataaatcagggaagagtaggcgctaaagtgcttcccacactccccacacttgtagggtttctccccagtgtgaatcctctggtgcttcatgaggttgggcctccgggtgaatgtcttcccacactcgtcacaccggtagggaatctctcctgagtgcatccttcggtgattgatgaactcgcagctctggctgaaggctttcccacactcatcacatttgtagggcttctcttcagtgtgaagccgctgatgcttgacaaggttggcactgtacctgaatgttttcccacagtaactgcaataatgcaattttttcccagtaggaattttctgatcttctttaacaactaagtttgcactgaagatttccccagagttacgaactgtatttgttttttttgacctgtgtacacgcttatggttgttgagatatgatctctgttcaaaactttgctcacatatatcacatttgtgaggtctctgatcaggaacaggtcttgacagcaacctgaggtttcccccagactccctgctgctctccccgttggtcagtgtgactgccctggggcctctctgctccactagcttttccaggctcccctctgacttactgatgtggtcacaggcttctactggctcagatccctggggatcttcctcaccaaatgtctcctgtgaagtcaactccttgtactcagttctggtcccaagagctgggctgttgactctcaggtgctctttcccagaggtgccctgaacatccaggacccagggctcatcccctcgctccaactgcgagatcactccaggcttggggcctgcaggtcctactcccagtgagactaggttcccgtaggtctccagcatcacgtccctgtagaggcccctctgagcagggcccaggcggccccattcctcccgggagaggtacacagccacgtcctcgaaggtcacctcggcctggggtggggcagacaggaacaaggccgccattgcctgagggttgggctttctgagggcagtgagcaggagctggtcactgaggagctaccagaagcatgagactctcggattagatacatgtgatgcaactatttggcctcagcgccgccgagcagcacggcagcccaacctcgccc

SEQ ID NO: 13183 - RNA, 2471 nt, Homo sapiens
  source 1..2471: mol_type = other RNA
gctgggattacaggcatgagccaccacacctggccgatgcttttaaatttacaatatgtaaaaatgttaaaatatatggtgctctcttcagtgtgaattttctgatattgaggaaatagcaaaagtgaagatcctaggtgctgcaatgacaagcattacggtattttctttttaaaatgctctccagtatgtctcgaaaatattcgtaaatcagcagcaatgaattttttttctaagtgggagagatcacagaagcttcttttttgcccacttttctgtctcaatttctctaaaatgaacatgcactgcttttgatttaagaaaagaggtttgtttaatgagaaacgtcctttcactctgtgaaaacatcgtgtggataatacataaagggcagagtcaggtgccgggggcgcatgcaggaagtgctcagctggactctgccctcggacaccgcgccactgttacatggagaagtcctcccggaggtgaatccgctgatgctgacacatgttggaactgtgccggaaggccttcccacactcgctgcacttgtagggcttctccccggtgtggatcctccggtgctgaatcaagtacgtgctctggctgaaggctttcttgcaatcgctgcatctgtagggtttctctccgtggtgcagcctctggtggtggatgagtctggaactgttgtggaaggccttcccacactcgctgcacttgtagggcttctctcctgtgtggattctctggtgctggatgaggtgtgtgctttggctgaaaactttgccacagtcattgcattcatagggcttctctccagtgtggcttctctgatgttccacgagtttggttttttgaatgaaagctttctcacattcattacatttatagggtttctctccagtgtgaattctctgatgttggataaggttagaactttgtgtaaagcctttgccacattccttgcactcaaatggcttctctccggtgtgagtccgacgatgtcggataaggattgagccatcactgaaggctttcccgcagtcattacatttatagggtttctctccggtgtggattctctggtgataaatcagggaagagtaggcgctaaagtgcttcccacactccccacacttgtagggtttctccccagtgtgaatcctctggtgcttcatgaggttgggcctccgggtgaatgtcttcccacactcgtcacaccggtagggaatctctcctgagtgcatccttcggtgattgatgaactcgcagctctggctgaaggctttcccacactcatcacatttgtagggcttctcttcagtgtgaagccgctgatgcttgacaaggttggcactgtacctgaatgttttcccacagtaactgcaataatgcaattttttcccagtaggaattttctgatcttctttaacaactaagtttgcactgaagatttccccagagttacgaactgtatttgttttttttgacctgtgtacacgcttatggttgttgagatatgatctctgttcaaaactttgctcacatatatcacatttgtgaggtctctgatcaggaacaggtcttgacagcaacctgaggtttcccccagactccctgctgctctccccgttggtcagtgtgactgccctggggcctctctgctccactagcttttccaggctcccctctgacttactgatgtggtcacaggcttctactggctcagatccctggggatcttcctcaccaaatgtctcctgtgaagtcaactccttgtactcagttctggtcccaagagctgggctgttgactctcaggtgctctttcccagaggtgccctgaacatccaggacccagggctcatcccctcgctccaactgcgagatcactccaggcttggggcctgcaggtcctactcccagtgagactaggttcccgtaggtctccagcatcacgtccctgtagaggcccctctgagcagggcccaggcggccccattcctcccgggagaggtacacagccacgtcctcgaaggtcacctcggcctggggtggggcagacaggaacaaggccgccattgcctgagggttgggctttctgagggcagtgagcaggagctggtcactgaggagctaccagaagcatgagactctcggattagatacatgtgatgcaactatttggcctggtagaactgaaaccctgcaaaactctcagtggggaaaccccactcgaagtatgtactttatggagactcttgtcggggccttgtccggggggtccctcgaacaggaagtgccgctgatggcgggacggacccacgcctgcagcaccgcgagaggaccgggcacaggggcaacgcgcaggggagggtctgcgccgggagggtctgcgccccgcgcgcccgcccccgccgggctcacactcacctcagcgccgccgagcagcacggcagcccaacctcgccc

SEQ ID NO: 13184 - RNA, 3020 nt, Homo sapiens
  source 1..3020: mol_type = other RNA
gctgggattacaggcatgagccaccacacctggcctaaaatacgcattcttttaaactgtgtatggtacactcaccatgacagacaacatattgggtcataaaacgagtctcaataaaactaagaggattgaaatcataaagaggatattttctgacctcaatggaattaaagtagaaatcagcaacaagaagatattaagaggaaaaaaaacaaatgtttgctgatcagacaacccacttctgataatccatgggtcaaagaagaactgagggaggaaattagaaaataatcagaggctgggcatggtggctcacacctgtaatcccagcactttgggaggccaaagtgggtggatcacctgaggtcaggagttcgagaccagcctggccaatgtggtgaaaccccatctctactaaaaatacaaaaatcagccaggtatggtggctggagcctgtaatcccagctactgaggaggctgaggcaggagaatcgcttgaacccaggaggcagaggttgcagtgagctgagatcgtaccattgcactctagcctgggcaacaaaagcgaaattccatctcaaaaagaaaaaaaaaagaaaattagaactgaataataaaaatacgacataataaaattgtaaagtcgcaactaaagtaatgcttaaaagaaaatgtatagctttaaatatgtattttaaataacgtctaagatcaatgacctaaggcttatcttaaggaactaaagaaaaaagatcaaaggagactcaagctaaatagaagaaagaaaataacagaaattaattatataaacaattgagaaaaataaaaccaaaggttggttctttaaaagttatatcgtcggccaggcacggtggctcacgcctgtaatcccagcactctgggaggctgaggcgggtggaccacgaggtaaagagatcgagaccatcctggctaacacagtgaaacccagtctccactaaaaatataaaaaattagccgggcgtggtggtgggagcctgtagtcccagctactggggaggctgaggcaggagaatggcatgaacccggaaggcagagcttgcagtaagccgagatcgcgccactgcactccagcctgggagacagtgtaagactgtctcaaaaaaaataaaataaaataaaaagtcagatcagtaaaactgataaacccctacccaacctgattaggaaagtgagaacagaaattaccagtatcataatgaaaaggaaattatcaacacagctcctaaagacattaaaagggtaagaagggaccattataaataaccttatgtctacaaatttgataacctgggtcaaaaggatagatttcttggatagattcattacctaaatgacaccaagatcaaaccaaaaaatgtgaatagccctatatttattaaatacactatagaaaaccagacaaagaaaatttaaggcccagatggtttcagacattaattctacagccctgacaaggaaaaaggggatagttagaattgggttactaaaaagttagcttttaatatcaacaggaatactggtcaagagtccacattatgcaggttgtaaatggtagacactataaacaaataggaatcagctctgatgatactcattttttcttccctttcaaaggcttggcaaataaagccgggtcaatttgctcctttgccagtcctctgacagagaagagtcttgctgcccgctcctgcagagtgcccccacatttcagtccaagggccatcagttcacatttgagcttctccaaacccagcaactccagttctgcaacagaggtgaacgccaataaatctatagtttccttatcaataactgcgtttcctggctggctttcctgcagtttggcaacggcaacgttttccctttcttcaggtgctacctcagcaactctttccccatcagtcctttcttctgtctctttatccttattcagtccagccccagtgggctcctcttctatgggttctttactctctgccttcttctcctgggtctcttctgtttctgtaaccatcctgctttccatgtgctctttggactcccccagctcagcacatgagtcttctaaaatatgcctcccagagtcagtcaccgggatctgcagttgttctggtgatccatggtctgtattcactactctcgccctctgagaaccactgggaaatttggctgccatctcgacaccattgctaccaatttttggagcatggaaacccattcctgaagtgcttggtgcttcttcactgtcatcatctgaactctcagagttggacccttctgcagtctctagtccctccatgcccaaccagaagcatctcctctttcccgcactggctcctctgtctgtttgagatttagtaggccattgccgtttccgattctcactgatttctgctgaaaccatcttgctggaggcagcctgcatacctttgaggacggaatcctccagacgctcagccatctcatggcactgctgctggtagtcggggctggtgaagcagtgcttgggttctacaagcttccgctgcagtcgctccagccgcttctgctccttttcagcctctcgctcggcttgttgttttacccattcagccattgctttttcatgattgacatcgcgtagtctccttccactgagatcccgacaagcttctcgattggttgtcttctcaatctgagcaccaagtgctcggagcatagatccaaaacctccttttccaccgcaaagtctgggttccaaactataaacagctccatgctgcactgtgtcactggtgttaatgagtgctccattgcatttcacaaagaagttttccactggaacattctgatcttggcagtgccggtggataaaatcccggacggtgcaccgacccgaggcacaccgcaccgccttgcacccgaagccagggccgcgaatccacaccagcgccgcggcctccgccatgtcaccgactacccgaacctcaagcctctct

SEQ ID NO: 13185 - RNA, 5184 nt, Homo sapiens
  source 1..5184: mol_type = other RNA
gctgggattacaggcatgagccaccacacctggcctaaacctcttctttcttaatggtactggtgggaataagctaatttatgtgtcaatgctgaagggtttcccgtatcccaggagtcctgggatgaaggtatgaggaagaatccctatctcttttttcccctcagttaaaggaggttctatctcagcttctcccctaactctatccaaaagaaaggctttgcaaagcgggtagaacctaaaaaggcgaaaggatgtgggtatgctgtctgtaggattgtcaggaagggttttatacactgaatattagatgtcatgttgcaaatacaccacctaaaactagaactgaattatatttgccccaactcccctaaaagagtttaatcttataactttgtaaaaatccttgcctaggacttttaagtctcccttccttaaagagggaaagtggggcatagacaatgacttttattgttacctagttatctcagaaagaggttaaggagattttccctactggaagccccactcttggaaaggatacagttttcatcaccctcagggtttcggggtggccctggcatattcaataaaaccagctttgcttcatgggacttgttaactataacctcgttgagtttcactgctgtatgcatccgcctcacattggactggtccggacgcatgttaagcaggtcctggaatccttccattgacttcgctttttgtccccgggatgccatgtacttgtcttttgtccaagtcatgtgcaccttctcctgataggtttctgtctcttcgtcctcatcagagccaatgctggtcaatcgtagcattgagtttcggtctttcaccaattgtgcctctctgtctcgctctgttttggatagccgcatgtgccggagcatctgggacctttgttccatcatcaaagtgcgctcgtaagtatatgctgatatatcactgtcatgctcttgtatctcaaactcagctttctcaccatctccaccacttctacctccgcctcaatgcgtaagtgatataggaaggtggctaggtccttcttcatttggatactgttgtcttctaattgggctactgtgaagatccgtatgctgcactttcgccacaccttgtgctgtttcagtaggaatggtagtagcataagcatccccccatcatgcacaatccaccacacatcaatgttgccctcagaaaattgctccacattgctgggaaagaaggagatgtttttagccaccagcagtgcaagatgggcagcagttgtcactcgaactgtgccaataaaagtcttccaagcgcgggcatcttcgctttgacgccagccattaggccagcccatcaccaccgtgttgtgcttcatgcccccaaggccacatgactggatgaggtgggaaatgccctctctcagcttggcggccaccaccagctggcagaatccttttaccttctctgcctccattaggtgctttatggtctgctcagcagctaaagcttcaccgtagttctctaggaagttccccacgatgacagagcccacaatagtgagaccttttcctgctttgagctgtgaggcaaaggtgaggaggcgaggatgcttgacatgtaagtcttcatctagtttcagtaatacaagcaactgaggcctccagtttttagtgtgtggaggtccttcctccaatcgaagcaaagcaaaccgggctgcactgagggacagcccacggataccatcaccccattctttctcagctccttggtattcaatgtacttgtagatcataccagctattaccatggctacaatggcataataccaggaagaaatgaacatcagagccagacagatactcattcccatgaaagaaagggcccaatggtagtagcggaatcggggtctccagttgggtgttcgaagtaatgtttgcaaggcacatgccaagtttacaaagaggtaacacatgagaaaaaacatggaaagaattggggccacaagatccagggaggcaatgagtattccaagctctgcaatggcagcagttagaagtaaagcccaggtaggttccccattggctttgctgtggccaaaaaccctcagaaacggtatgatgttatccttggcaatagcttgtagcagcctcggtgcacctgtgaggctctgaagtccagccccacatgttgaaaagaaggagccaataacaatcacccatggggatggccaagataaggtgcctaccaccaaattacctttcacagcatcaccgaacttgtctctgagaacaaccccttcaatacatgcaccaaaaaggacaacattgcttaaataaacaaaggaggtggtcaggatggcaaggatagtaccaatcggaatagacttctgagcatctttcagatctccagatctgtttgatccagccatgatacctgtaacagagggaaagaagattcccaccagaagcgtgaaggaggtggtgatgtcaacaagaacatattcatggtttaagctgcctaagacatcagaagatttggctgaaggcttttcgatgatctctcccttgggtaggtaattactccaaagattctctgtaattataccactagccaatccaggaatgccctggattgaagtgacgttattgtgaacaaagtattcatcacaggtggcattgaaaaattgactcgagttacagaagaatccccataactttgatgggactgtcatgttgttaatttccttggtcttagagcaaacgtcaatgtgtcttgatgaaagggtgcggttacccagcatgcagaccgggaagtgtggaggagcaaaagaagacttgatggctccagcatagatggccaagatggacacaatgacacaggccaggaaaagtgaggcaaacttgttcacatagcgtacgccgataaataccactaataccataaggaccaagaaagctgtgccgtagacacgcatgttatttagcatggctgctgattccttgagtgcgtcatcactgtgaaagatggcagctcgggggacgatatagaccagaaagatttcaatggcaccaaggatgtacatggctgctgcaaatgtggtaccaagataaaagcagaggccaacagccccaccaaactctgggcccagtgcccgggaaatcataaagtatgagcccccagctggcaccactccattagtggcaatggcactcatggagatagcagtcaacattgtacagcagcagcagataaggacaattgcaaaagcctgaagaactccagctgtgcccaccacccatgtaaggcgtaaaaaaaggatcactccaaaaatattttgtagacatgggaggtagacacccatgaaggtacccatttggggggtcttggtgggcttctttttcccttcagtgatgttttctgcctcttcatgttcctttgctccttgagtcagattagtgtaattggccatgcggttgaggagggaagacaccttcggtctggtgtccatttcttcctcaaagagtgccaaatttttatcaaaatattcatctccttcttcataattggaattattgagataagcatttcgagctttcttatgtccgtcgtctaacagttggctgtgttcccctgtgatggagttctgactcaggtcctcgatgacatcctgggggtgagaagtccggtcactgggtggatccagtgcaacagttgccagcgaagtggtggccccagacatctcactcataggctcactccggcttgtttcaggcacgctttcccgggagctaaatcttactcgggaactagatcgagagctgaggtccggactggtgtctgacaaacctggaatgtcatcgatctttgtcggtgtcaccatgaaccgaactgaagccatcttggtggtggtttctggaggatgcattttgttctttttaagaacaaaaaaagtggggggaacctcgcaaaatcttcctcttacgctagctacttttgactgcaatacaaaagataacttgaaaaataacacatttcaataaccttgattcacaccacacaaaaagccccaactaagaatacttctactcagaattcaagccgactgtcctagaaagtgcatcaccaataggtgaatatattttttaagagagaaaaaaacaaaaaacaaaaagacaaaacaatgccaatcttgtgtgacttctttccttcagaatgaagagctacctagctaacccctctggtccggggctgaaggctcagtgccatggtctcagggcagcagatgaagcctccctcccctcagcccccagtttcctgtcgaggtagtcctttatctggtgagtgtcccacggttctagttgggcgaagtgcgtgcaggcaaacctttatcaggcgactatagcgtggatcagattgctaaaaggtgtacacccggccacctgttgtgtatcaggtgaataccccacaggtctggctggggggaggtgtatgcaaagccacccggtgtttttgatgtcgacaatccacttgggtctggtgggaaaggtgcacatgcataacgggaaaaataacccacactactgagagaagggtgagcagaggaggatgcaggggcagagcggattcctgtctccgagaggtcggtgggggtggcgcgcccgctcttctcctagcagaaaggtcctcggggtctgggaggaggttagcggatcaagacacctcggactgcagctcagagtcgtggcaagtcgtagctagtccactgagccacggtccgctcgctaggtttctcctgcgtgtgacaggacgagccaccccctttgccggaggcgcgttctcccctacccccgccccggcgcaggtcaccccctcgtcgttcttcctcagggtcccagtagaggaggagacggccacgcaggctggcctgactgggcagcagggtgagggagaaggaggtcgcaggtgcagtatcccggcgccagctgatgcgggtgcgcgcgcagctgttgtttactagccggtaactgtttcagagccgcggcgcgcgcagggttcgcgctgccggggctggcgccccctccccggcccgacgccagagcagcagttacgtgacctggcctcccccagccccgggcccgacggggtgcgcccgcgccgccgcagcccttcccttcc

SEQ ID NO: 13186 - RNA, 5082 nt, Homo sapiens
  source 1..5082: mol_type = other RNA
gctgggattacaggcatgagccaccacacctggcctaggatttcaatcacaaaagatttttttttttttttttttgagacggagtctcactctgtcgcccaggctggagtgcagtggcgtgatctcggctcactgcaagctccgcctcccaggttcatgtcattctcctgcctcagcctcctgagtagctgggactacagatgcccatcaccacgcccagctaatttttgtatttttagtagagacggagtttcaccatgttagccaggatggtctcgatctcctgaccttgtgatccgcccgcctcagcctcccaaagtgctgggattataggcgtgagccaccgcgcctggacacacaaaagatttttaaaattcctaaagtgtgttttctccacaatgttatctatacatttagttaggctattattcaagttatttggcttttagcctgcatttctgatatgtgggaacaaactactttatcttccttttgtctttcaagttctaggatgataggagttttgtttaccaaaaggaatcctccatgaatttataattgttgatcatagccactgctcttcctctagcctaactttgtatggcttcctaactctaatcccataccttcttaaccatttcaggtatgctttcatagatctgcaccaatgtgtttctttttgtgtcatattctgctacagtaaaaggagatactaaggcatgaggagtaacagcttcagaaatgagagtggcctattaatactatccactaaagtgtagaggaagcagatatggtaatgctacatgccacacaaaacagattaataagaagttgttgtagtttctagtaccaatattacaaacggtgtaatttgagtatatgaaaaaaaagtgaagtttctatgtataataaaaacaatataatagtctttttcaaagctgcagagaatgctatagtttgggattttataattcctgtgaagaggaatataagggaaggcaactctgtcaacaaattttgtatgtctttactgtattcaaaacccttgccgaaaaaataaaagcaacaatgagaccatgtctcatattaattttgccctgttttccttttgtaaatacatgatcactgggtaaagcacaagtgtaatttctgctccataataccttcttaaaattaattagatctctaatgcctcatgtgtcctataggcttatctataggaagtactacaggcttatctataagaagtattacagaagtgacttaggaaactaggagaaagtgaattgggttattatatccaaagaagtttcagagtaaaatttataatatttaatagaaagaaatgtaccaggtcctaggatgccaactggaaatctattccatgtataatatccagtctaatcttaatcaacagagtcagcatcttttcccttcaaaactcttactgaagatgtaaataagtagaaaacttgacccatgcaaacaattcccttcatattgcaagtgttagcatgaaagaaactggctgaaagagaggcccaaaatatagatgcttggtttattttcaagtatgatccactctaatcataccatttggataagatgaatttattaagagaaggataaatttggaaaattagtaaagtggtcaaatatcaataaggagtagatggaaataaacagctatttaacgacttactttcaaaataaaaagaagttaatgtatgtttttgtgtttttaaattttcatcttcccagctcccaaaagaccaagaattgaacgacaaccagggtctctggttcctggaatttattacgtattcattctcatgaagtaggtttgtctccacattactaggtggaaatctgggcaccaagtagttaagtgaacctctcagagtcaccctagaaatgaataatgacaaaaccaaagcaaaaacccaaaatattatactggtctgtattgatacctttactccaaattattttttatttatcagcttgccattaagaagctgaatcagggtaacaccaatatgtattagaatttgcctctggtactgaaaatgaaggaaggaaaccaagactatttacacttttttttttttttttttttttgagacagagtctcactctgtcacccaggctggagtgcagtggtgtgatcttggctcaccgcaacctctgcctcccgggttcaagcgattctcctgcctcagcctcccaagtagctcggattacaggtgtgtgccaccatgcccagctaatttttgtatttttagtataggtggggtttcaccatgttgcacaggctggtctcaaattcctgacctcaggtgatctgcccgcctcagcctcccaaagtgctgggattacaggtgttagccaccacgcccagcccatttacgctttatgttgcaaatattggcagtgttacctttaggtaatacaaagctggaatgcccaatatttttcctctgataattgtgatggtatcttttgagtctgcattggtcagcttcatccaatacaagggcttggccattctcctcttaatcattcttaccctattgatagaagaaatggcctctcctttgactctcaataaagatctccgaggactcttgctgcatttcagaaaactctggcccaccaacctttctttccgagggtaggacagaagttttcttcactccttctcctgtggggatttgcccattgatgttaagagttcggaagggtgagtgagtggataagcgtttatcccattcactaggccgtggttctggtacagactccatgaagttctttttcagctcactgatgctggcatgatgttttttgatctcctcttgactcttgtctaaatcctccaacattaaattgctatgtctgatataaatgttttcaccatctagtctttctctctttttcttcctcattcttatcagatcttcagttttttctgcaagcttctgtgtttggtcaccatttgaggtgggtactgtcacctcgatgtgggttttttccaccttccatgcttctgtgggctctggctcagcttgctcaggtggctcgtcttcctttttcacttcagccttcactgtttccttctgtgctttagggaccactgtttttttagcagaggcatctaggacgccaccttctgcaacctgaccctgagtaatggcaggtgcagaagtgggccgaggacttcggtctgccgaatcgacagctgctgctccatcgaggctccgggacgcccgtttacttgctgtacgctcgaagtgtggggcaggcctgtcaattagagcactagcttgcctggtctgagcttgagtccggccactgtatcgaaatttggatcctagcgcaagaaatttgcttttgggaatggtgtctgtagatgtcaatctgaaaaacgtgtgatgttctacacagactttccataatttcttagctgctcggtaactgggaagtttgaatccgatggtactttcatactgctcttgctctccaggccgaatcttgatgaaaaagctactacgtttataagaaatcttcagcactttgggccaagggaagcggttaattctcagcttatctttgtaaaccagaaggccactagagcagacacctaggatgatatctactccttccaagtcctttgctttatgaagatcaactccatacatagacaactttttggcattctcaagaaactccaagtcagcctgagctggagtcatggacctgtatgacttatgcagttccatgaccttctcttcaagttccttggtctgattcggggccagtttaaaatcactaacataatccacgccatggagttctgggtcgtagtctcccagttcagactggatggtgtaagaacctaataatgctaaggttgcaaaggaacagggcagacgtcctgcaactatgtcctgccgaagctgaagacataaataatatcttgttatgtcttctgttaactgtgctgggtcaggtggataaaactttacattaaatgtaaaattccaagggacaccacgaacctgcttttttatttctttggcggaatccagccatgtcttagaggttgcgttatcccaaatggctagaccaaaatagtcttcttccaaaagattgagatgctcacatactcgtttaagcaaatcttgtcccttagcatgtttctccacaacacattcataaactgtgtcatccaacaaagaaaccttgcagtgcatgttcctgtgttttctgattggtttttgggaagcttttaattctgtttctgcttttgattgagggctttcttcttttacttctattttggagcactcttcaagtccttctccttccttaatttcaaaatctggatcttctctgagttcttcctgagcaggctgtgtttctgcactgcttaatgaatgaagatccaaagatgggtctgttttgagttccggttcaggagctgcaattggggcctttaaaatgatctcttcatcaagactggttccaaattctatctctttctgacctccttcacctttttctttatctgactctacttctttgccttcttcctcggacacctgagatttgggccttttgagaaacgaggagaatagtcgtgaaagtcctctgctttctgatgtccgctccttgttcttggtcaagtcttcatgtgtaggagtgtctccattagaagctttcagcttctgttcacaccaattatctccttcagctgctgtttgacaagattcctcctgctgaggttcttgttggcctgagtttatggcttcctcaccctcttccttctgttggtgctgtgaattttcggcctcagtcactaaactcttctctgttgtcatgatgttgcggtggctccggggccgggctcctgcgcccgccactgctgcagcccgacgaacaatggcaggaggaggcgccggcgtccgaggctcgggccctctgcggctcgcgggcccgccggctgctgctggctgactgactaaacgcaccagcggagggagggagcgagcgagcgaccctggcgcgcgccctcccgccttc

SEQ ID NO: 13187 - RNA, 8338 nt, Homo sapiens
  source 1..8338: mol_type = other RNA
gctgggattacaggcatgagccaccacacctggcctaggatttcaatcacaaaagatttttttttttttttttttgagacggagtctcactctgtcgcccaggctggagtgcagtggcgtgatctcggctcactgcaagctccgcctcccaggttcatgtcattctcctgcctcagcctcctgagtagctgggactacagatgcccatcaccacgcccagctaatttttgtatttttagtagagacggagtttcaccatgttagccaggatggtctcgatctcctgaccttgtgatccgcccgcctcagcctcccaaagtgctgggattataggcgtgagccaccgcgcctggacacacaaaagatttttaaaattcctaaagtgtgttttctccacaatgttatctatacatttagttaggctattattcaagttatttggcttttagcctgcatttctgatatgtgggaacaaactactttatcttccttttgtctttcaagttctaggatgataggagttttgtttaccaaaaggaatcctccatgaatttataattgttgatcatagccactgctcttcctctagcctaactttgtatggcttcctaactctaatcccataccttcttaaccatttcaggtatgctttcatagatctgcaccaatgtgtttctttttgtgtcatattctgctacagtaaaaggagatactaaggcatgaggagtaacagcttcagaaatgagagtggcctattaatactatccactaaagtgtagaggaagcagatatggtaatgctacatgccacacaaaacagattaataagaagttgttgtagtttctagtaccaatattacaaacggtgtaatttgagtatatgaaaaaaaagtgaagtttctatgtataataaaaacaatataatagtctttttcaaagctgcagagaatgctatagtttgggattttataattcctgtgaagaggaatataagggaaggcaactctgtcaacaaattttgtatgtctttactgtattcaaaacccttgccgaaaaaataaaagcaacaatgagaccatgtctcatattaattttgccctgttttccttttgtaaatacatgatcactgggtaaagcacaagtgtaatttctgctccataataccttcttaaaattaattagatctctaatgcctcatgtgtcctataggcttatctataggaagtactacaggcttatctataagaagtattacagaagtgacttaggaaactaggagaaagtgaattgggttattatatccaaagaagtttcagagtaaaatttataatatttaatagaaagaaatgtaccaggtcctaggatgccaactggaaatctattccatgtataatatccagtctaatcttaatcaacagagtcagcatcttttcccttcaaaactcttactgaagatgtaaataagtagaaaacttgacccatgcaaacaattcccttcatattgcaagtgttagcatgaaagaaactggctgaaagagaggcccaaaatatagatgcttggtttattttcaagtatgatccactctaatcataccatttggataagatgaatttattaagagaaggataaatttggaaaattagtaaagtggtcaaatatcaataaggagtagatggaaataaacagctatttaacgacttactttcaaaataaaaagaagttaatgtatgtttttgtgtttttaaattttcatcttcccagctcccaaaagaccaagaattgaacgacaaccagggtctctggttcctggaatttattacgtattcattctcatgaagtaggtttgtctccacattactaggtggaaatctgggcaccaagtagttaagtgaacctctcagagtcaccctagaaatgaataatgacaaaaccaaagcaaaaacccaaaatattatactggtctgtattgatacctttactccaaattattttttatttatcagcttgccattaagaagctgaatcagggtaacaccaatatgtattagaatttgcctctggtactgaaaatgaaggaaggaaaccaagactatttacacttttttttttttttttttttttgagacagagtctcactctgtcacccaggctggagtgcagtggtgtgatcttggctcaccgcaacctctgcctcccgggttcaagcgattctcctgcctcagcctcccaagtagctcggattacaggtgtgtgccaccatgcccagctaatttttgtatttttagtataggtggggtttcaccatgttgcacaggctggtctcaaattcctgacctcaggtgatctgcccgcctcagcctcccaaagtgctgggattacaggtgttagccaccacgcccagcccatttacgctttatgttgcaaatattggcagtgttacctttaggtaatacaaagctggaatgcccaatatttttcctctgataattgtgatggtatcttttgagtctgcattggtcagcttcatccaatacaagggcttggccattctcctcttaatcattcttaccctattgatagaagaaatggcctctcctttgactctcaataaagatctccgaggactcttgctgcatttcagaaaactgaaaagtatcattggcttagacttttaatggacttggaataactccaatacaaagagaaataaaattcagggtgaagtttacaatagtaattaataaaaagctgtgtataaggatgaaaactggaaattcaggaattataatctgaaacagttataaaagtataaataaagttctgattatttccttttaattccttaaaaaaagatttaaaataatctaaccaattctatagtccaatttgttatttcattaagggaaactcttgtatctttatttcccagataaaagagagtactcatgattattactttctgtggtagagaacagctttgtaatatttcaggtccctcttattatgagtgaatcaataaatatacttatttacaaaatatatattataaatagacatagcctgtgacataaaagatatatacgcacaccaaattttaaattttaacctggtccttgcttctttttccatttcttgggaaagcctataatgacagcgtagcagttttcaggaaataacagataattatttctacatgtctccagagacaagagaacaatattggtagatgttgaaggacaaaagattcttgtctttactgttctctttttttgctctaagaggccatcttctcaaaaacaaaaagtcttgtttagaagtttcatcaactgaaaagcattgagaagtaaaacaaagtataataatcttagtttgataaccctataaactcagatttcaaaacaaatatttgagacattaaccaaatcatccatattggtacattcaagtgccataaaaagcaagctacatgcaaggtttcttcaatattgaggtaaaaaataacaggttaggcatgtgagttgtcctgaagagagagagagtgcccacatttacttcaggtaagtcttagaagtcaacatgcaaacagaggacacatacttgtcacaagtgaacttgaggtcacaaagccattgattaaaaacaattgatttcaacacaagtacacgaacaaacaggtctgaagtatatcaggaaaacaaagtatatcaatatatattttaagcttagcaatggctaactattgctgctagcaatataattagtaaagccataaagaagtaacacagtatcttaattcagagaagggtttatgtacagatcttgagtaaatctgtgttccagacttttaaggataggtagagtagtctgagaatttcagtcctggctggaggctaaggggcaccagcaccattttccttaaaccatatcaacactctacttgtgaaaagatggcatttaatctttgaagatctcttctatacaccaggcaggaaaaagttgtctgtccctgtacagctcagaaatactcataaaaaggccacagaagtcaaaagcccttttccagaaaagacttttgtttatactggtttgatatcctaagaaaaggagtggttatggatttgtagattaaaacgttatcattttaaggcttctgaaaggttagcgagttgaaattttttcttaaactatgaagcccatgccaaacaaatgactatagaggattaggaaaatattccatcaaatgtatctagagagtatcctggtttgtgtgagatattggataggaagacataacaatagtaaacagtaaacatgcaggataaaagagttaaagcttttgggaagattaccaacctgccatatgcttaattctgatttgtttaaatttgttaaacttcaatgcagaaaagctggctttgggcagtccattgctactcctttgtaccccacaatacatactctacaaagagtaacatttgacagaaaaatgatcacaagagctcccctaggatagtgaactatcaagatcagagggcatcatacagcaataacacagttgaagccaaggacagaagttcaatggtcttgacatttcagatgagcaccctgttttctgatcacagaaagaccaaccaccaaacagccaacacaaggatcacgagaaaagacatcatgaaaggaatacgaggagatggaaaagtactaaagtagaggtggcactttttgagagacttgtgatcctcagggattggaatagaaaccttgggaagaatttcttcattttcttgctggggcaaggctctttcagtagatctttcttgccttttaattttctcttcatcctgtactaacagagcacgttcctgtgtctgctttcacagtagaagatcaagaaagacagaataagatgaacaaaatgacagatggaaaatgctcaaaaatgatacttggggatgtgcaaaggatttggaagtatcttttagacactcttcattttagctttactttattttggcaatttatcctggcaaagtttctgtaacacaatagggtgctcaatagatacctttttgagtgagtgaacattagaacggaaagttcaaggaatcactggctttccccttgctatgttatttattcttcctttgaggatattcacatatgaattttaggtcattttctattactttggtgctgccaatcactaattgggcaatgccaataatgaagcattctccttgccatcataaaagttatttttggctgagcgcagtggctcacgcctgtaattccagcactttgggaggccgaggtgggcggatcacgaggtcaggagtttgagaccagcctggccaacatggtgaaaccccgtctctactaaaaatacaaaaattagctgggcgtggtggcacatgcctgttatcctagctactcaggaggctgaggccggagaattgcttgaacccgggaggcagaggttgcagtgagctgagatcgcgccactgcactccagcctgggggacagaacaacagtctgtctcagacaaaaaaaaaaagttacttttattacaaatataatggcagaatataaaaagtaatccttatatctcttcatatagactttaaaaacaacagttttaaaagcaacagttcattcagtatagcaattagtttttgctccagaaataaaaaatcttaatcttatacattttaaagattgcaaaagaaaaacaaaaagtataaaagtttataatgtccctccaaggttcaccaaaacaaataaataataatgaccatcatgaaggtttatacattactttaagcaaatgctttagacacttttaaagaaagttttttctccccaattgtccaattgagaagtttttattccccctgcaatttctgtactctgctatccatagtcaagacagatgttatctatgaaaggaaaaacttggctctaagttctctcagttgagctagccttctctgatcagtttggaagttcaacactggttctttgcacacccctaagtgatatgtatcagggagaaagtagctaggggactctggcccaccaacctttctttccgagggtaggacagaagttttcttcactccttctcctgtggggatttgcccattgatgttaagagttcggaagggtgagtgagtggataagcgtttatcccattcactaggccgtggttctggtacagactccatgaagttctttttcagctcactgatgctggcatgatgttttttgatctcctcttgactcttgtctaaatccttccatgcttctgtgggctctggctcagcttgctcaggtggctcgtcttcctttttcacttcagccttcactgtttccttctgtgctttagggaccactgtttttttagcagaggcatctaggacgccaccttctgcaacctgaccctgagtaatggcaggtgcagaagtgggccgaggacttcggtctgccgaatcgacagctgctccatcgaggctccgggacgcccgtttacttgctgtacgctcgaagtgtggggcaggcctgtcaattagagcactagcttgcctggtctgagcttgagtccggccactgtatcgaaatttggatcctagcgcaagaaatttgcttttgggaatggtgtctgtagatgtcaatctgaaaaacgtgtgatgttctacacagactttccataatttcttagctgctcggtaactgggaagtttgaatccgatggtactttcatactgctcttgctctccaggccgaatcttgatgaaaaagctactacgtttataagaaatcttcagcactttgggccaagggaagcggttaattctcagcttatctttgtaaaccagaaggccactagagcagacacctaggatgatatctactccttccaagtcctttgctttatgaagatcaactccatacatagacaactttttggcattctcaagaaactccaagtcagcctgagctggagtcatggacctgtatgacttatgcagttccatgaccttctcttcaagttccttggtctgattcggggccagtttaaaatcactaacataatccacgccatggagttctgggtcgtagtctcccagttcagactggatggtgtaagaacctaataatgctaaggttgcaaaggaacagggcagacgtcctgcaactatgtcctgccgaagctgaagacataaataatatcttgttatgtcttctgttaactgtgctgggtcaggtggataaaactttacattaaatgtaaaattccaagggacaccacgaacctgcttttttatttctttggcggaatccagccatgtcttagaggttgcgttatcccaaatggctagaccaaaatagtcttcttccaaaagattgagatgctcacatactcgtttaagcaaatcttgtcccttagcatgtttctccacaacacattcataaactgtgtcatccaacaaagaaaccttgcagtgcatgttcctgtgttttctgattggtttttgggaagcttttaattctgtttctgcttttgattgagggctttcttcttttacttctattttggagcactcttcaagtccttctccttccttaatttcaaaatctggatcttctctgagttcttcctgagcaggctgtgtttctgcactgcttaatgaatgaagatccaaagatgggtctgttttgagttccggttcaggagctgcaattggggcctttaaaatgatctcttcatcaagactggttccaaattctatctctttctgacctccttcacctttttctttatctgactctacttctttgccttcttcctcggacacctgagatttgggccttttgagaaacgaggagaatagtcgtgaaagtcctctgctttctgatgtccgctccttgttcttggtcaagtcttcatgtgtaggagtgtctccattagaagctttcagcttctgttcacaccaattatctccttcagctgctgtttgacaagattcctcctgctgaggttcttgttggcctgagtttatggcttcctcaccctcttccttctgttggtgctgtgaattttcggcctcagtcactaaactcttctctgttgtcatgatgttgcggtggctccggggccgggctcctgcgcccgccactgctgcagcccgacgaacaatggcaggaggaggcgccggcgtccgaggctcgggccctctgcggctcgcgggcccgccggctgctgctggctgactgactaaacgcaccagcggagggagggagcgagcgagcgaccctggcgcgcgccctcccgccttc

SEQ ID NO: 13188 - RNA, 7108 nt, Homo sapiens
  source 1..7108: mol_type = other RNA
gctgggattacaggcatgagccaccacacctggcctattctttagtctttcaaaaggattgtgagcagttttagactatgccactaaaaaaatgaaaaggaagttacttttcttttcagcacttcacagcaaatattacattctggcaagtgctagttccaaacacagccaatcctatttgaaccagtctctgttgcaactactaaattcttatcatttgtagtgcaaaagctgctctagacagtatgtaaatcaatgggtgcagctgtgtttcagttaaactgtacttacaaaaacaggcagggaccagatttggccagcaaactgtagtttgctgacccctgatctataggcaatgggaatatgaatagttggatagtagcatacaacataaataacaactataaaacaatatacatcagaaaggtctgtcagttatatataatatatataaatataaacatatataatatatatataatatatatatatatacatgctcatatgagaaacgctgggggctgagcacagtggctcatacctgtaatcccagcactttggaggccgagacaggtggatcacctgaggtcaggagttcgagaccagcctggccgtctctactaaaaatacaaaaatgagccaggcatggtggcatatgcctgtaatcccggctacttaggaggctgaggcaggagaactgcttgaacctaagaggcagaggttgcagtgagccaagatcatgccactgcactccagcctgggtgacagagcgagactcctcaaaaacaaaacaaaacaaaacaaaacaaaacaaaacccctccagggctgagacaatgtgtccactgtgattttaaggtaaatgaaagcactggggaatcgctggtaaatacgcaaatagaaacaggagtacaagtggggattctcctttgaggaggtgataagctcaaaaccacagatgatacatcctgccagatggcagaggagcagccagacctattaggacattaaattcaatgcctgaccaacagtgttaagaccatgttactaggatttaccacagcccaagcagcgcgtacatctcactgccgagttgtctctccccacaaatactccaaccctcacccaaggagtctgagtaagagaaaaaccatagagcaggtctaagaggacatgcctgtgatacaggacttcaagtgggtgatgtaagaaacgagctctgcctgtagaaaggaagccctggtgtggattttctggtgatgaagatggggcagacctgttccagctggagggcctgggtgtgaatgagggccaggctacatccctcgaacatccttcttcccaagtcactcacttaggagagggaagactggcactaaaatcaaagtctgtcaccctctctgcctcagaagtgtgtgatacaggtcattcataagaacacgaaaccagggcattttattttaaatgctgaaattcttgaggaaattagatttgctatggactgaattgtgtcccccatcctaaattcctatgttgaagccctcaccccgaatgtgatatttgcagatggagcatttggggagggaattaggttagatgtggtcatgagggtggggcctcatgatgggattagagcctttataagaagaaactcgggtgcttgctgccctctgccctctctccactcacatgcatgtggaaaggccatgtgagaacacagcaagaagggagctacaaggaaccagaggagaggccctccccagacactgatcctgctaacaccttgatctgggacttacagtctccagaagtaaattcctgttgttgaagccacccagtgtatggtattttactgtggcagcccaagctaagacaatacttaaattttgtcatagtcttaggcctaccactccttttttggatgctacaaaaaaaaaagaataaagtcctcaccagtttcaggtcggcattttctttctgtcactgccttttctcttgctggtctttgaggacaggcagcattgtcctctcccttttggaatattcagggtttagcaccaagaggtctttaataaaggtttgttgagtaaatattgaaatcaaaggaatgtaaatatggaatcaagactttttctaaagtggtgtggtggctcacgcctatagtcccagcactttgggaagctgaggcaggaggatctcttaagtccaggagttcgaagctgcagttagctatgcttgtgccactgcactccagcctgggtgacagagtaagaccctctctctctaaaaacaataccaacaacaaaaccttttgctatcattgggagcaaaaaatgtgtgggtggaaatgaaaagtgttgtttcactgagatgagataggaaggacaggcatttcccctgtcatgcctcatttcttcatcctctctcctcctccctctctaatgcattgattaacttaacttttctgattatctcctaatatattgtatagggaaagaaaagaagagccagggaggacaaaaacctagatcttaacatttcaataagttctgaataatcagaatggtagaaggccatggtaaaacaaaacaaaacacaaaaaacaggtattagacttcttaatagttccttcacatagggcattttaattttttgaaagctcttgcatatatatcatgtaactttatttagacttcaacttccaattagcgaaaagtctgtcttgtactccctgcttctgaggtactaaagcagttctcaactggggggtgattttgccccccagggaacacctggcaggtctggaggcatttttagttgtcataactgggtaggatgctactggcatctaatgggcagaggccaggaatgctgctaaatattctacaatgcacaagacagccccacacaatcaagaattatcccactccaaatgttgatagtactgaggttgaaaaattctgcactaaaggaaagagatgaaagacagggtggactcttcttaggaattttttttaaaacatcaaatcctagagtcataaacggcttgtttctaaatcacattactggtatcttggaacagcaagggtggtgaaaatatagcaaagcccgatttatctgaagagtttagaggttgaacaattctcctcaactagtttgttttagaaatgctttcttcccaggagaagcacaagggggcgcaagaatcccacatcacttcagtgttcttagccttcttgccactctgctgccaagtcagaaaaaagaaaaacactgaccaggtgtgagttaatgctcctgtcctgcagaacactgtcagctatgagggcaaaaatcgtgtctgtttaactcgcttgcacaatgcctggcttaatattatgctgttacctgtacttaataattattttcagagccaaatagagttctctatttttcttctctttagtattcagaggttgaaatgaggactttacatcttcaatggcaaaatcattcccacttaaaagctgagtacaattcaatcctactcaggagagaggctttacccatttaggtataaaccaaaccaacagatcaatggaaacagaattccaatatgcagatggcatgaaatacagatctttagttcagcccatctctgctctcacctacacatctggactctgtgcaaatgcataacatgccaagtcagacaccctggaaagacaaggcccgggagggcagtatggcagattgaaacctgccctgagttgggaagggaatatgtacaggaaactatctactaaccattttgaagttttacagctaacgctaggactactgctgggatcttttacctataattataaaggtgcctccagggaagtttttagtggtacaaaatgttcagagacattctgggagaaaagtctcaggtcagtggttttgaacctttcattaatttttccccaatggactaatgttttgaaaaattttgcctatcaaattccatgttaaaaataattttttccatgtgtgtgactgctgatccagattttatccaaagattggtaattttaagtaggttcataatagtatcactcttgcagttgtgatgctgataagcaacaaagttaagtaactgtacagacactcattgctttctgctactgatcactaattctggccatctctctgtatatattcagaacacagctatatgacagatggcttcataacattatttcattaccaataatgttctccaaaattctgtatcatagcaccgattagagcctctgaatagctgagctgttttactacactgaatcgatataattctagtcaaaggccaaaagcctcaaatcttcccaaactgttaatattctatttggaagtattgaggaaatatataaaatatagttaaggatttttatggacttcggaaatatagaaaatactgttaaggactcacgatcttaagaaattttgtagaaacatttttccctctagtgtattatgtatttggatatacaaataacccacttggaatcttacttgaatagtttagaagtatccaatatacctcaattagaattaaaaacaaaacaaaaccaaaaaaataacacttgttcttgagagtttagaaactcacagaaattcaggctggaaagaaacttggggaacatctaactcccctatttttcacttgaaaatataacctctttggaccttaaatgactaaatcatttgaagagcaataaagcccatttttcccaattctgagcttattctatcatacccccatgctttctggtgatccataagagtttagtatacatagtaaataatgataaataacatatttatatatttatacttatctaaacccatgatttaaaatttgtttgaataccacccacagtaagaaatatgcaatccagtacttactcatacacaagcaaagttttatgcaacaaaactgatccttataacatattgcaatacacttccacaaaactgatttcatgacccaatattgtctcagctcaaattctgaaaacacatggtgccctctggctgtgttaattttgggttgattatatattcttacataattctctagttgtttcatttggattaacattgccactcctccctcctgacaaggttgtaacttaataatagcatgtcttatagcagatgccccataaagacttgttaaagtacacttatgcctcactgctttatactgctgaaaaacatctaatttctgtattgcagtggcagaaaacgaaagaaaccttgacagaactcccattctccctctaattctcatcactaagccctttctgcttgacatggagaaggcatatatttggggtggggaagcaatgggtagaacactgattaaaacagaatgaagggcggtttctttttttcttacatctagaggtttaagatctaagtgagaaaatatcacactcctagttgctccaagaagggtttctgagaagcaatttatgatgaatatcattcaggaatatccggagattcctcataaaagcaagtgtgcaggaatcatcttggccattagaagcaatcaatactctcctgtcagtttgttttgaaatttgtgcatgtcctctctccttttatcatatgctctagtgacttcatcaagacagtctaaaggaagatgggcccggtgcagtggctcacgcctgtaatctcagcactttgggaagctgaggtgggaggattgcttgaggctagaagtttgagaccagcctgggaaagaaagggagaccctgtctctcatacaaaaaaaaaaaaaggaagaaagaaaaatgatgtgaaacttacccttatgaattccattctttgctaacaattattctattcattcttttttcattccaaaaacacttgttgagtgccaactatgtaccaagcaagatgctttaggagtgagtgatactgtggtgggtggggatgccagacctggtctgcctgtatggaaggttacaatctagagcagaatgtgtaaaagaggaatctgtacttttttttttttccacatgattgttttctcaccatttttcatattgaaaatgacagatttataaaaattgcagcttattcttaccaagcagtgttgacaaaattcagagtagggaatatcagcacaattcaccaacacttgaataaattctttgagatggaaaggattgcatagggactcacacaccttgaagtatacggttcccttctctttgacaatggcagcctgctccaatttttctttggtatccatctcccaggattctttggccttggtccaagatataaaatacattgttcttcccgctgcattttctccagagctttgtcaattccaattggaatgtcgtggtcttctccttcgcccacagtgaatgccacatctctgcagtcaaacatccttccaccacagcggccttccaggtggatttctactgttgctccttcgtttggatttgaatatccctctcctttccgtttggttctccggataatgcctccatcttcaaataaatcctctcctttgaaatcaaggagctcaatctcaaaaaagagagttgcattcgagggaattttagggagactgccagccgagccatatgcatattctggtttgcacagtaaatggcatatctctcctttcttcatggtagccaccccaatgtcccatgccttgatgacttggcctttgccaagactaaagacaaatggttcatttctatcatgactggaatcaaacttctttccatttgacaattttcctttgtaatggacataaactttgtctccaatcatcggcgtttcctcaccattccccactcttttgacaatctttaatactcccctgtcttttttggaggtaatatcctctccctgctcagcaacagtggctgtggggctttcttcattgttcttggcaccttcatcagtagtcattgtcttttaagtagagaacctgtcgccgcgggggctcgccgactccgtcactctccgccttgcccgtgctccgctaacccttcagcccgcccagcaggccgcccgcgcgccggacaccgccgcccgagact

SEQ ID NO: 13189 - RNA, 1682 nt, Homo sapiens
  source 1..1682: mol_type = other RNA
gctgggattacaggcatgagccaccacacctggcctcaattataatttctaatagctgaatttggttattttcaaatctgattgtttcatgcctatattttcaagcatttttctttctttaaaacttaaaatatattatactttatctcataatactaatatctaacatttgtgcaggtctgcttccacatctgttatctctgcaagttctcattcacagtgcttgcttgtgcattagtagtattttggctgtgaagcactcattttccttcaaacttcatatgttgaaattccttgaagcctgggatgaatgtctggtcctctcaaaaaaactatttacatttgcttcagcctcacacatgagagcattaccagtctaaggcaaccttgaacaaaattacttacttaagatttgtccaacttcccagttagtataatgctggccacactaggagaacagcccatcattataaacactcaaggctttattcactgtcccccaccccactcccttagccccaaagctcaggatgggcaattctccttgccattctgtaggggggattttaggtgtattttgagttcacccttacattgctggtatagccatccaggtcccgctccatgagatactattcgtatagagagtcctgactttgtctcaagttctcctgattccataataacactggtttaaatattccactcaactcttaaaattttggacctgagtatctttatttctttgccaattcatcaacgtatttactatgtttttctctatcacccacatttattttgttgttggctggaggaaagtctgtcaaggtatttaatctgcaatattgctagaaacagaagtcattttcttcatttctttcttcatccttgccccctttattcttttacttttcttcttcaccaccccattcaggaaaatacccaggaaaacttccattgttgaaataaactcaatcttgccatctgtatttgtagttaagacattgaaaaacttctttaacttttcattcattgtaaaattcttcacggagaggctccacttatggaaattggcagtcagaggttctactgctaatgacagcaacaactcagtaggaaaattctggaacattctgctgtgcaattgacctccagtgaagttcagcggcattgccacgtcaacagtatctgtggcagttaataagcactctccactaatcagcagtgaaagctcttcaaatccaaggcatgtgccccacacaggaaaatagtctccatcatcaaaactctgtatggacaagttataaaatattttggccactttagcataatctgagcgtctgaggtcaacacttcctccagggaaaaggattccattaatagatttgaaaagtatttcatagtctttctctgtaagatccagccttactggtacaactctcgcacctgcagactccaagtactttacataggacgcagcaatatagtatcttccatagtttttcatgactttattacggcatttttgcattaatattccgatgatgggcttcttggcggtgtcgccgtggggtctagacagctcgaggctcgccgccccgcagagtagcaggcccagcacgcacagcaggcagcccggactggccatggcgctcgccgcctcccgccgcctttcaaaagct

SEQ ID NO: 13190 - RNA, 685 nt, Homo sapiens
  source 1..685: mol_type = other RNA
gctgggattacaggcatgagccaccacacctggcctcagctcctcattttatacaggaggaaattaagcccacaaaaggaagggacttgcttttctagagtacagagaaagggcctctgagcacctgtgtaggtgcttggtgaatccagccaggaggcctgattatccttcattgactatccatgtgatcttgggtgaggttcagagtaacagtcaagccagtgctcagctgggtgtgtccacacctccctggtactcacatgcactccgctcttcttctggctgtcaagtccctagatgacccaggccacctcgttttccctcaggtcaagcagctgaggtgggggttcaggcctctccagggctgtagctcaggcctcaggaggtgcaggagacacctcttccctgcagcccctccaggcaatgctgtcctgagtcctcagctcttatgttgtatatatgtcctatttcccagctgggtggtgttcttctgtcttcaacaaagcttccacagcatggaacagggacccaggaggttgcctgctggctgaggttgggtgggcttagggggtggctagctttattccctgattgtcccctcccatgttctgtttctgtcctatcagagtgcccttttttcaatcctccccgcaattggctacttttagaatcctgctgattggtg

SEQ ID NO: 13191 - RNA, 687 nt, Homo sapiens
  source 1..687: mol_type = other RNA
gctgggattacaggcatgagccaccacacctggcctcagctcctcattttatacaggaggaaattaagcccacaaaaggaagggacttgcttttctagagtacagagaaagggcctctgagcacctgtgtaggtgcttggtgaatccagccaggaggcctgattatccttcattgactatccatgtgatcttgggtgaggttcagagtaacagtcaagccagtgctcagctgggtgtgtccacacctccctggtactcacatgcactccgctcttcttctggctgtcaagtccctagatgacccaggccacctcgttttccctcaggtcaagcagctgaggtgggggttcaggcctctccagggctgtagctcaggcctcaggaggtgcaggagacacctcttccctgcagcccctccaggcaatgctgtcctgagtcctcagctcttatgttgtatatatgtcctatttcccagctgggtggtgttcttctgtcttcaacaaagcttccacagcatggaacagggacccaggaggttgcctgctggctgaggttgggtgggcttagggggtggctagctttattccctgattgtcccctcccatgttctgtttctgtcctatcagagtgcccttttttcaatcctccccgcaattggctacttttagaatcctgctgattggtgca

SEQ ID NO: 13192 - RNA, 2424 nt, Homo sapiens
  source 1..2424: mol_type = other RNA
gctgggattacaggcatgagccaccacacctggcctctctggtgattttcttaatggcatctgggaactcatctgctgcctcttggtcagctaaagctactcctcctgttatctagatatttttacaacccaagtcactttctaaaactatcaaatcatcttttgttggcattaaattctccagctttagaaccttcaccttctttctgctttgtcatataatgacttcaccttttctcaaatcatattagagtctgtatgtatgcttttcttgtagcaatcctgcaaccatatcaaagctgcattctaaatatgagatgaatacacccgcctgctggtgtacctgcagtgacagtttcacaaatttctttccctctcttgcttttttttttttttttaacaacagttcttacactggattcatttatcttgaaatggtgggcaactgcagctgcagactgaaatctataagacatatcaaggaactcagccttttcttctaatgccgtaacttttctctgcttcttgggagacttccagcatcaccagtggcattgtgtatgggtcctgcagtgctactcgaggtttacagtattgcaccaaacacgttgaaaaataccagagatcacgtttcactaggctatgcaactgactggaggaatgagctggtgccacagaggtgatcggtgtcacacagcattttaattgggcacttgaaacacttgggctcactgcagtaggaacgagcagtgaccaggaaattttacagtagcactgaatggactacagttagtttcatgcaattatgattcaatactgcatctttacatttgcgtttctcttgacagagaatgacaccacatacagtctgggtttgtgtaagttttgatagattttaacttcttataatagatttgtatgtatttcatggttgtaaatggtaaaatagactagtatgtacgtatatttaatgcattcaggacatatctaactttttctgaatttttttcaatatttctaggttatgcatttcatctgtcagttttttcaaattgttgcaaatttccaataaaattttccaatgtatttattgaaaaaaatctgtataaaactggcccacaaagttcaatcccgtgttgttcaagggccagctgtacttgtgttgttgttacctctaactgagtttgtggtccatacatgtcccagatttttcttcttcggacatcaatccctctgcctggatgcccctcactgctcaggatgtggaccaggaggccatttccacatcccaggtccacaaaggactgcctggcagttagtctcctctcagccctttcttcttcccatagaatcagcaggtatgctgcgatagccacatcttcatacacgaacttctcaggatcagtgacttcaggccacaccttaaccatttccttatacttctctttaagttcctggtaagccttgctatacttcataatggagatgagggaaagggtgcttttaaagtcactcttcttgttctctacagaccacttggccaacttggccagcaactcttctccaagccacgtgggtttgggatacacgattccatctgaatgccatctttctggacagaaaattaaaacagatatgaaccattcttctttgctatgactgagctgaatttgatacacattgctcatcttaacctttaggttcccctcatcatcttcttccaaaggcaaaaacgttatggttccattgaggacatcttgcacgactatttccctcctgggagttgtaagggggcaatgtgggctagttttcgggatgacggttctgagaaccacgtcgagctcacgctgcgcctctggctgcgatcccgccccggagctggtgaggaaggccagcaactccgaattgccacgggcgagactttgggagaaatcctcccaaagcgaatccagatctgcggcggggaagtcgccctcccttccttcagcatggccggggtgcccggagtccctcaggggcactgaggcggcttccctctgtgcctcctcttgctggcactggccctgggcctcctcaagttcgcaacatgccgtgccctgctcgggtcctgatagcgacctgggacccgggccccctccgggggaaccctggccgggtcccggaccccgctccttctgctccgagcctgcgctagtcccggggccgcgggcctccgcgcagggcagggcggcgctccagcgggcctccaggcgggcgccgcaaagccgtttgtttgccacctgcggcctctccagccacacttcgaccgcagcccagaagccctgtgggagaagcgcgcctgggtagctgatcccggtacggcccacctcagccatggcagccagcaggtgtacagccctggcagcggcgcgccgagatgacgca

SEQ ID NO: 13193 - RNA, 4044 nt, Homo sapiens
  source 1..4044: mol_type = other RNA
gctgggattacaggcatgagccaccacacctggcctggattagtaatttcggatttccaaattcaggtcaagaagtggaatttattatgtggttcttgtgaaaaaaatataaatgtggccttttaaatatatttagtcttttttttaaacaaaggctactcaaaccattaccttcctgccccccttgaaaagaaaaaaaaaatctatccatcccatttgctttctctaattttgaaaagtcagaaagatctcaaaggtttcttactaccgtacttacatgcaaaggcgaaagcacatccaattagatttgagggtatcatttattccgtgcagagccaaggactactgtgaaaaaaaggcatagatacagaaagaaaaaagaaaagcagcaataacaaactaaacagggctagggagcagtggcagaaaaaagttcagaagcaatacattttttaaaaaaaaaagcttctatttgtttcttttgactttttattccctgactcgccatatgatttattttgctgggaaaaatttaatgcaaaaaagtcaatccaatcaataatcttggaatcaaaaagtcagctggatgcctttcgttgttatgctcattttaaaaaaattttagtgatgcaagagacaatttaaaagtgtactttctgtacaagccacaaaaatgctcacacaagcggtggttggaacaagcatacaacacaaatattcaagcttttgtctgatgcacagcctatgagcaaattcagcccatggtttgaatcaacatgccagctactatttggctgctccacagttagctccagactagaattatttaaaaaaacaaaagcaaaaacaagaatgttggtccagtagctcctaaacctgtgaagactatgactactgctgtgtctagtgtgtagtttctattccagctttgtttaggcttccatgaaactaatttccttactttgcttaattaagcataatcagttcatggaagaccattccttctttcctctaagtatggttgaggacaaagaaaaggagaaaaaatctttgctgaaatcaaaatggagacttgctcattcaaaaaagaaagtgtgtgtcaggggagacgcagcatattctatcctatttacttaatctctaaccagtgaggaaaatgcagaggggcagtgggttcatgagaaatgttatcctttctacatgtagagagaaagctgggaggatcttgttagtagaggggaaaaaacaatcacacagatgaaaggataagcatcagaaaggagcagtatagaaaagagattaaatatgcactcttccatacaaattaggcatttagtacaggttctggcatatgggccagttctaatccctgatgaggcaagggccttagacaaagagcaggtggagctagccaaggtgaggaaaattccagacaatgatttgagacttcagctgttctatttcttctttcttttattgccaaatactgaaaggagactaagcaaggaagctggatatgaaatgtctaccttcttgacttacgggtcatgttgtggtccttcctatttccaccttaaaattgacaaggcctcgctcaaatttgtgctaccaatgatacagagtttatagcaaattttctaagggaagtatctgtggaaattttctcatgattcatgaaaaatgttattagaagtacaagtatcctggaatcagtcatcaggtcctccctctaagcccactgggaacaaactgaggtgtgtttatgaaagattccttactgttagtggtaagcaggctgtagaaagcccatcatccttagaagaagattcttctactaagcaatgttacatgatccaacctttaagacctctatctgtgagaggatcaaggatgcaccagtaaatgtgaactaatcatagttttctcataccagtctactccaacttggccaggattgaaggcaggcattcagatgcagtttcaaaccatgagaggagacagtctgaacagacccacaagctcaggccaaataatgttattgattaaaatgaaaatgtcatgcaagggtaaaaataaaatataatgcttgctcaccagtctgtctacgtacaaatctaccttggcttaggacaagtgtggagaaaagacagtgagttcagggattgtgcactcatggagatgaatcatcaagaaaatgcaaactcttgtcatggctattcaggtttttagttcagctgctgaggcggtgagaagttttcatgtcagacgtacaggtagcattttaccccactttcctctgtccaaagcgacatacaagtaacaggcctgcttcgtgctgccattcagaacaggcataaaaagcaaatcatttactttccggaaacagagtccagctgcacagagcattcgcggttattcccttgttctatcattttctaccacccaacaacattcagcaaaacgagttaataatagttactggtgtttgaggaagggtaaaaaaataaaataaaataaaataaaactaaagaacacacatggcagagatacgatattactgcaaaagcaggtgaatgcgggaacatccttggcttgccaggctttatgtgaagcttgcatttttcttatccttgtctttcttggtttgctgggccccagattgctgggcctgggactgtagtaactgagccgctgctttcttcttctggaagttgttcacctcctcctcaagctccttcttcttgtcttccactttcttcttttcttcttggtgtgtccgctttagaaggtcaaacttctcgtgaagctctttctctgcctccttaagttcagcttctttctccttcactctcataacaaacatttgtctcatttcttcttctttcttctgcagttctcccaggaattcattcctttttgcttcatatgtctcctgaagactgaagggtttgctgtcagggtcagtgtccttgaaccccatctcttcaagcttacagcgtcggtacaattcatagtggcgggtgtgagtctgctctcgcaagtcctccatgttcacgcggatcagcatctctcgaagtttcacaaaatcgcaatgattttcattctcaacctgcaccacaccccaggggtactgcctggcctttgccatcttgttgccaatcttcacctcttcggtgctgccaaccactgcaaatgggagatggacactcattgttgcgttaatctctgccaccgtttcttcatcagtgggaaactgatatatctggaccccattgctgaccagttcactcatgatcttactcttgaatttgtgcagttcattcttggcaatggtgtcagcttttgcaattattggaatgatgttcaccttactgtccagctttttcatggtgaccagatccagggactttagtgaatgtccagtaggggcaataaagtagaggcaggcatggatcctcgtgtcatggtagttgaagagagaacgtttaatcttcaattcctcttgcaggtaggcctcgaactgggcatcaatatattctactatcggcttatagctgtcatctttatttatctggtctccaaatcccacggtgtcaacaatggttaacttcagccgtacattgctttcctgaagctcataacttctggcttttaaccgaacacctggttcattgtgagtagctgggtcactttcaaatttggtgttgaacaaagtgtccattaacgtggatttgccaatgcctgtctcaccaacacaaaggatgttgaaacagaatccttgagaagtagacttgttgaccagctggtcagggaggctgtcaaatcccacatggccagacaaagacaagtttcgaagctcttcattagacggtctccccacggccacggccatcgcagctgcggcaccggctccggctgcgcccgggtgctttacgccgactccggctgctgctagtgctcgggctccggctcgcctccctcgcgcctccctcgcggctgcgctctgctcgccggcgtcccgctggcagccagcggcatctgctc

SEQ ID NO: 13194 - RNA, 4264 nt, Homo sapiens
  source 1..4264: mol_type = other RNA
gctgggattacaggcatgagccaccacacctggcctggattagtaatttcggatttccaaattcaggtcaagaagtggaatttattatgtggttcttgtgaaaaaaatataaatgtggccttttaaatatatttagtcttttttttaaacaaaggctactcaaaccattaccttcctgccccccttgaaaagaaaaaaaaaatctatccatcccatttgctttctctaattttgaaaagtcagaaagatctcaaaggtttcttactaccgtacttacatgcaaaggcgaaagcacatccaattagatttgagggtatcatttattccgtgcagagccaaggactactgtgaaaaaaaggcatagatacagaaagaaaaaagaaaagcagcaataacaaactaaacagggctagggagcagtggcagaaaaaagttcagaagcaatacattttttaaaaaaaaaagcttctatttgtttcttttgactttttattccctgactcgccatatgatttattttgctgggaaaaatttaatgcaaaaaagtcaatccaatcaataatcttggaatcaaaaagtcagctggatgcctttcgttgttatgctcattttaaaaaaattttagtgatgcaagagacaatttaaaagtgtactttctgtacaagccacaaaaatgctcacacaagcggtggttggaacaagcatacaacacaaatattcaagcttttgtctgatgcacagcctatgagcaaattcagcccatggtttgaatcaacatgccagctactatttggctgctccacagttagctccagactagaattatttaaaaaaacaaaagcaaaaacaagaatgttggtccagtagctcctaaacctgtgaagactatgactactgctgtgtctagtgtgtagtttctattccagctttgtttaggcttccatgaaactaatttccttactttgcttaattaagcataatcagttcatggaagaccattccttctttcctctaagtatggttgaggacaaagaaaaggagaaaaaatctttgctgaaatcaaaatggagacttgctcattcaaaaaagaaagtgtgtgtcaggggagacgcagcatattctatcctatttacttaatctctaaccagtgaggaaaatgcagaggggcagtgggttcatgagaaatgttatcctttctacatgtagagagaaagctgggaggatcttgttagtagaggggaaaaaacaatcacacagatgaaaggataagcatcagaaaggagcagtatagaaaagagattaaatatgcactcttccatacaaattaggcatttagtacaggttctggcatatgggccagttctaatccctgatgaggcaagggccttagacaaagagcaggtggagctagccaaggtgaggaaaattccagacaatgatttgagacttcagctgttctatttcttctttcttttattgccaaatactgaaaggagactaagcaaggaagctggatatgaaatgtctaccttcttgacttacgggtcatgttgtggtccttcctatttccaccttaaaattgacaaggcctcgctcaaatttgtgctaccaatgatacagagtttatagcaaattttctaagggaagtatctgtggaaattttctcatgattcatgaaaaatgttattagaagtacaagtatcctggaatcagtcatcaggtcctccctctaagcccactgggaacaaactgaggtgtgtttatgaaagattccttactgttagtggtaagcaggctgtagaaagcccatcatccttagaagaagattcttctactaagcaatgttacatgatccaacctttaagacctctatctgtgagaggatcaaggatgcaccagtaaatgtgaactaatcatagttttctcataccagtctactccaacttggccaggattgaaggcaggcattcagatgcagtttcaaaccatgagaggagacagtctgaacagacccacaagctcaggccaaataatgttattgattaaaatgaaaatgtcatgcaagggtaaaaataaaatataatgcttgctcaccagtctgtctacgtacaaatctaccttggcttaggacaagtgtggagaaaagacagtgagttcagggattgtgcactcatggagatgaatcatcaagaaaatgcaaactcttgtcatggctattcaggtttttagttcagctgctgaggcggtgagaagttttcatgtcagacgtacaggtagcattttaccccactttcctctgtccaaagcgacatacaagtaacaggcctgcttcgtgctgccattcagaacaggcataaaaagcaaatcatttactttccggaaacagagtccagctgcacagagcattcgcggttattcccttgttctatcattttctaccacccaacaacattcagcaaaacgagttaataatagttactggtgtttgaggaagggtaaaaaaataaaataaaataaaataaaactaaagaacacacatggcagagatacgatattactgcaaaagcaggtgaatgcgggaacatccttggcttgccaggctttatgtgaagcttgcatttttcttatccttgtctttcttggtttgctgggccccagattgctgggcctgggactgtagtaactgagccgctgctttcttcttctggaagttgttcacctcctcctcaagctccttcttcttgtcttccactttcttcttttcttcttggtgtgtccgctttagaaggtcaaacttctcgtgaagctctttctctgcctccttaagttcagcttctttctccttcactctcataacaaacatttgtctcatttcttcttctttcttctgcagttctcccaggaattcattcctttttgcttcatatgtctcctgaagactgaagggtttgctgtcagggtcagtgtccttgaaccccatctcttcaagcttacagcgtcggtacaattcatagtggcgggtgtgagtctgctctcgcaagtcctccatgttcacgcggatcagcatctctcgaagtttcacaaaatcgcaatgattttcattctcaacctgcaccacaccccaggggtactgcctggcctttgccatcttgttgccaatcttcacctcttcggtgctgccaaccactgcaaatgggagatggacactcattgttgcgttaatctctgccaccgtttcttcatcagtgggaaactgatatatctggaccccattgctgaccagttcactcatgatcttactcttgaatttgtgcagttcattcttggcaatggtgtcagcttttgcaattattggaatgatgttcaccttactgtccagctttttcatggtgaccagatccagggactttagtgaatgtccagtaggggcaataaagtagaggcaggcatggatcctcgtgtcatggtagttgaagagagaacgtttaatcttcaattcctcttgcaggtaggcctcgaactgggcatcaatatattctactatcggcttatagctgtcatctttatttatctggtctccaaatcccacggtgtcaacaatggttaacttcagccgtacattgctttcctgaagctcataacttctggcttttaaccgaacacctggttcattgtgagtagctgggtcactttcaaatttggtgttgaacaaagtgtccattaacgtggatttgccaatgcctgtctcaccaacacaaaggatgttgaaacagaatccttgagaagtagacttgttgaccagctggtcagggaggctgtcaaatcccacatggccagacaaagacaagtttcgaagctcttcattcataaatgcagcatatttaaaacttctcagcacatgagctggtttcctctcctccattagttttacaggtttcttgagtcttcttccccctcttcaccctgtagctcctagcacaggctctgtaactgctggagttttgcagagtttaccgatgtagacccttcatcttaggtcatgtctttttctgaggtcctatttcagtagtacagacgcctctgagagacggtctccccacggccacggccatcgcagctgcggcaccggctccggctgcgcccgggtgctttacgccgactccggctgctgctagtgctcgggctccggctcgcctccctcgcgcctccctcgcggctgcgctctgctcgccggcgtcccgctggcagccagcggcatctgctc

SEQ ID NO: 13195 - RNA, 4095 nt, Homo sapiens
  source 1..4095: mol_type = other RNA
gctgggattacaggcatgagccaccacacctggcctggattagtaatttcggatttccaaattcaggtcaagaagtggaatttattatgtggttcttgtgaaaaaaatataaatgtggccttttaaatatatttagtcttttttttaaacaaaggctactcaaaccattaccttcctgccccccttgaaaagaaaaaaaaaatctatccatcccatttgctttctctaattttgaaaagtcagaaagatctcaaaggtttcttactaccgtacttacatgcaaaggcgaaagcacatccaattagatttgagggtatcatttattccgtgcagagccaaggactactgtgaaaaaaaggcatagatacagaaagaaaaaagaaaagcagcaataacaaactaaacagggctagggagcagtggcagaaaaaagttcagaagcaatacattttttaaaaaaaaaagcttctatttgtttcttttgactttttattccctgactcgccatatgatttattttgctgggaaaaatttaatgcaaaaaagtcaatccaatcaataatcttggaatcaaaaagtcagctggatgcctttcgttgttatgctcattttaaaaaaattttagtgatgcaagagacaatttaaaagtgtactttctgtacaagccacaaaaatgctcacacaagcggtggttggaacaagcatacaacacaaatattcaagcttttgtctgatgcacagcctatgagcaaattcagcccatggtttgaatcaacatgccagctactatttggctgctccacagttagctccagactagaattatttaaaaaaacaaaagcaaaaacaagaatgttggtccagtagctcctaaacctgtgaagactatgactactgctgtgtctagtgtgtagtttctattccagctttgtttaggcttccatgaaactaatttccttactttgcttaattaagcataatcagttcatggaagaccattccttctttcctctaagtatggttgaggacaaagaaaaggagaaaaaatctttgctgaaatcaaaatggagacttgctcattcaaaaaagaaagtgtgtgtcaggggagacgcagcatattctatcctatttacttaatctctaaccagtgaggaaaatgcagaggggcagtgggttcatgagaaatgttatcctttctacatgtagagagaaagctgggaggatcttgttagtagaggggaaaaaacaatcacacagatgaaaggataagcatcagaaaggagcagtatagaaaagagattaaatatgcactcttccatacaaattaggcatttagtacaggttctggcatatgggccagttctaatccctgatgaggcaagggccttagacaaagagcaggtggagctagccaaggtgaggaaaattccagacaatgatttgagacttcagctgttctatttcttctttcttttattgccaaatactgaaaggagactaagcaaggaagctggatatgaaatgtctaccttcttgacttacgggtcatgttgtggtccttcctatttccaccttaaaattgacaaggcctcgctcaaatttgtgctaccaatgatacagagtttatagcaaattttctaagggaagtatctgtggaaattttctcatgattcatgaaaaatgttattagaagtacaagtatcctggaatcagtcatcaggtcctccctctaagcccactgggaacaaactgaggtgtgtttatgaaagattccttactgttagtggtaagcaggctgtagaaagcccatcatccttagaagaagattcttctactaagcaatgttacatgatccaacctttaagacctctatctgtgagaggatcaaggatgcaccagtaaatgtgaactaatcatagttttctcataccagtctactccaacttggccaggattgaaggcaggcattcagatgcagtttcaaaccatgagaggagacagtctgaacagacccacaagctcaggccaaataatgttattgattaaaatgaaaatgtcatgcaagggtaaaaataaaatataatgcttgctcaccagtctgtctacgtacaaatctaccttggcttaggacaagtgtggagaaaagacagtgagttcagggattgtgcactcatggagatgaatcatcaagaaaatgcaaactcttgtcatggctattcaggtttttagttcagctgctgaggcggtgagaagttttcatgtcagacgtacaggtagcattttaccccactttcctctgtccaaagcgacatacaagtaacaggcctgcttcgtgctgccattcagaacaggcataaaaagcaaatcatttactttccggaaacagagtccagctgcacagagcattcgcggttattcccttgttctatcattttctaccacccaacaacattcagcaaaacgagttaataatagttactggtgtttgaggaagggtaaaaaaataaaataaaataaaataaaactaaagaacacacatggcagagatacgatattactgcaaaagcaggtgaatgcgggaacatccttggcttgccaggctttatgtgaagcttgcatttttcttatccttgtctttcttggtttgctgggccccagattgctgggcctgggactgtagtaactgagccgctgctttcttcttctggaagttgttcacctcctcctcaagctccttcttcttgtcttccactttcttcttttcttcttggtgtgtccgctttagaaggtcaaacttctcgtgaagctctttctctgcctccttaagttcagcttctttctccttcactctcataacaaacatttgtctcatttcttcttctttcttctgcagttctcccaggaattcattcctttttgcttcatatgtctcctgaagactgaagggtttgctgtcagggtcagtgtccttgaaccccatctcttcaagcttacagcgtcggtacaattcatagtggcgggtgtgagtctgctctcgcaagtcctccatgttcacgcggatcagcatctctcgaagtttcacaaaatcgcaatgattttcattctcaacctgcaccacaccccaggggtactgcctggcctttgccatcttgttgccaatcttcacctcttcggtgctgccaaccactgcaaatgggagatggacactcattgttgcgttaatctctgccaccgtttcttcatcagtgggaaactgatatatctggaccccattgctgaccagttcactcatgatcttactcttgaatttgtgcagttcattcttggcaatggtgtcagcttttgcaattattggaatgatgttcaccttactgtccagctttttcatggtgaccagatccagggactttagtgaatgtccagtaggggcaataaagtagaggcaggcatggatcctcgtgtcatggtagttgaagagagaacgtttaatcttcaattcctcttgcaggtaggcctcgaactgggcatcaatatattctactatcggcttatagctgtcatctttatttatctggtctccaaatcccacggtgtcaacaatggttaacttcagccgtacattgctttcctgaagctcataacttctggcttttaaccgaacacctggttcattgtgagtagctgggtcactttcaaatttggtgttgaacaaagtgtccattaacgtggatttgccaatgcctgtctcaccaacacaaaggatgttgaaacagaatccttgagaagtagacttgttgaccagctggtcagggaggctgtcaaatcccacatggccagacaaagacaagtttcgaagctcttcattcataaatgcagcatatttaaaacttctcagcacatgagctggtttcctctcctccattagttttacaggtttcttgagtcttcttccccctcttcaccctgtagctcctagcacaggctctgtaactgctggagttttgcagagtttaccgatgtagacccttcatcttaggtcatgtctttttctgaggtcctatttcagtagtacagacgcctctgagctgaagagag

SEQ ID NO: 13196 - RNA, 3948 nt, Homo sapiens
  source 1..3948: mol_type = other RNA
gctgggattacaggcatgagccaccacacctggcctggattagtaatttcggatttccaaattcaggtcaagaagtggaatttattatgtggttcttgtgaaaaaaatataaatgtggccttttaaatatatttagtcttttttttaaacaaaggctactcaaaccattaccttcctgccccccttgaaaagaaaaaaaaaatctatccatcccatttgctttctctaattttgaaaagtcagaaagatctcaaaggtttcttactaccgtacttacatgcaaaggcgaaagcacatccaattagatttgagggtatcatttattccgtgcagagccaaggactactgtgaaaaaaaggcatagatacagaaagaaaaaagaaaagcagcaataacaaactaaacagggctagggagcagtggcagaaaaaagttcagaagcaatacattttttaaaaaaaaaagcttctatttgtttcttttgactttttattccctgactcgccatatgatttattttgctgggaaaaatttaatgcaaaaaagtcaatccaatcaataatcttggaatcaaaaagtcagctggatgcctttcgttgttatgctcattttaaaaaaattttagtgatgcaagagacaatttaaaagtgtactttctgtacaagccacaaaaatgctcacacaagcggtggttggaacaagcatacaacacaaatattcaagcttttgtctgatgcacagcctatgagcaaattcagcccatggtttgaatcaacatgccagctactatttggctgctccacagttagctccagactagaattatttaaaaaaacaaaagcaaaaacaagaatgttggtccagtagctcctaaacctgtgaagactatgactactgctgtgtctagtgtgtagtttctattccagctttgtttaggcttccatgaaactaatttccttactttgcttaattaagcataatcagttcatggaagaccattccttctttcctctaagtatggttgaggacaaagaaaaggagaaaaaatctttgctgaaatcaaaatggagacttgctcattcaaaaaagaaagtgtgtgtcaggggagacgcagcatattctatcctatttacttaatctctaaccagtgaggaaaatgcagaggggcagtgggttcatgagaaatgttatcctttctacatgtagagagaaagctgggaggatcttgttagtagaggggaaaaaacaatcacacagatgaaaggataagcatcagaaaggagcagtatagaaaagagattaaatatgcactcttccatacaaattaggcatttagtacaggttctggcatatgggccagttctaatccctgatgaggcaagggccttagacaaagagcaggtggagctagccaaggtgaggaaaattccagacaatgatttgagacttcagctgttctatttcttctttcttttattgccaaatactgaaaggagactaagcaaggaagctggatatgaaatgtctaccttcttgacttacgggtcatgttgtggtccttcctatttccaccttaaaattgacaaggcctcgctcaaatttgtgctaccaatgatacagagtttatagcaaattttctaagggaagtatctgtggaaattttctcatgattcatgaaaaatgttattagaagtacaagtatcctggaatcagtcatcaggtcctccctctaagcccactgggaacaaactgaggtgtgtttatgaaagattccttactgttagtggtaagcaggctgtagaaagcccatcatccttagaagaagattcttctactaagcaatgttacatgatccaacctttaagacctctatctgtgagaggatcaaggatgcaccagtaaatgtgaactaatcatagttttctcataccagtctactccaacttggccaggattgaaggcaggcattcagatgcagtttcaaaccatgagaggagacagtctgaacagacccacaagctcaggccaaataatgttattgattaaaatgaaaatgtcatgcaagggtaaaaataaaatataatgcttgctcaccagtctgtctacgtacaaatctaccttggcttaggacaagtgtggagaaaagacagtgagttcagggattgtgcactcatggagatgaatcatcaagaaaatgcaaactcttgtcatggctattcaggtttttagttcagctgctgaggcggtgagaagttttcatgtcagacgtacaggtagcattttaccccactttcctctgtccaaagcgacatacaagtaacaggcctgcttcgtgctgccattcagaacaggcataaaaagcaaatcatttactttccggaaacagagtccagctgcacagagcattcgcggttattcccttgttctatcattttctaccacccaacaacattcagcaaaacgagttaataatagttactggtgtttgaggaagggtaaaaaaataaaataaaataaaataaaactaaagaacacacatggcagagatacgatattactgcaaaagcaggtgaatgcgggaacatccttggcttgccaggctttatgtgaagcttgcatttttcttatccttgtctttcttggtttgctgggccccagattgctgggcctgggactgtagtaactgagccgctgctttcttcttctggaagttgttcacctcctcctcaagctccttcttcttgtcttccactttcttcttttcttcttggtgtgtccgctttagaaggtcaaacttctcgtgaagctctttctctgcctccttaagttcagcttctttctccttcactctcataacaaacatttgtctcatttcttcttctttcttctgcagttctcccaggaattcattcctttttgcttcatatgtctcctgaagactgaagggtttgctgtcagggtcagtgtccttgaaccccatctcttcaagcttacagcgtcggtacaattcatagtggcgggtgtgagtctgctctcgcaagtcctccatgttcacgcggatcagcatctctcgaagtttcacaaaatcgcaatgattttcattctcaacctgcaccacaccccaggggtactgcctggcctttgccatcttgttgccaatcttcacctcttcggtgctgccaaccactgcaaatgggagatggacactcattgttgcgttaatctctgccaccgtttcttcatcagtgggaaactgatatatctggaccccattgctgaccagttcactcatgatcttactcttgaatttgtgcagttcattcttggcaatggtgtcagcttttgcaattattggaatgatgttcaccttactgtccagctttttcatggtgaccagatccagggactttagtgaatgtccagtaggggcaataaagtagaggcaggcatggatcctcgtgtcatggtagttgaagagagaacgtttaatcttcaattcctcttgcaggtaggcctcgaactgggcatcaatatattctactatcggcttatagctgtcatctttatttatctggtctccaaatcccacggtgtcaacaatggttaacttcagccgtacattgctttcctgaagctcataacttctggcttttaaccgaacacctggttcattgtgagtagctgggtcactttcaaatttggtgttgaacaaagtgtccattaacgtggatttgccaatgcctgtctcaccaacacaaaggatgttgaaacagaatccttgagaagtagacttgttgaccagctggtcagggaggctgtcaaatcccacatggccagacaaagacaagtttcgaagctcttcattcccttcatcttaggtcatgtctttttctgaggtcctatttcagtagtacagacgcctctgagctgaagagaggtaaagaaaag

SEQ ID NO: 13197 - RNA, 1128 nt, Homo sapiens
  source 1..1128: mol_type = other RNA
gctgggattacaggcatgagccaccacacctggccttcagatgctaatctcttacagaaacaccctcacagacacctccagaaataacgtttaatcagatacctgggcattctataagctcagtcaagttgacatgcaaaattaatcactagtcatgaaattcaaagcttaaatgtagttatgatttgtggtaaacttttaggctatacttaatcaatctacattgttttattataaagagatggtaccaccctaatagtttgttgattcatatttctaacccttacatgttgtttaacttaatgttggtaagccagcttcttgctttccaaaaaataaaatacgtcgatgctgcctaactgcaattaaccaacattcttaaagcatttgccaaaatggattgtttatgagaactcatggtgctcagcactcactttcttcaataaaatcaattgaaaaggtctaactgttggtgagtgaagactgtggcggctttagctgccttctgattgcttgggcagatgtgtgtcagcatgctttctcttcttctggggagtgaaggaagtccctttatgtgtgtgcccaggactggctcctgttcctggaataaataccatcatgttgtgcagtcttgcagtttctagtaagtgctgtgcatgattggcatgtccttcagaaagcagcgagcctgagtgtttacaatgctcgtgaggtgcctccctgatagtaagtgctgctctttcttaacattcttttttcctttaaaatttgtttcaatccatgaggtaaaaaataatgacgatatagatagacgaacagttcatgttgtttttcccccaggttcaggttaaaacaaatacttcttcgtaagtaggttggtaccagttcctattgagaggtgacagcttgctggcagccctcgctggctctgggcgcctcctcggccttggcgcccactctggccgcgcttgaggaacccttcagctcaccgctgcactgtgggagcccctttctgggctggccaaggccagagccggctccctcagcttgcggggaggtgaggagggagaggagcggcggcaacggcgcggcgggaaccgaggatgcgcgcggcgcttgccagacaga

SEQ ID NO: 13198 - RNA, 1222 nt, Homo sapiens
  source 1..1222: mol_type = other RNA
gctgggattacaggcatgagccaccacacctggccttgagggctttttaaggaggtagaatcagcagaatcaggcagattggatgcgaatgtgagggagagagaggggattctcagtttgggttcctccagaagctgatcctgaggcaaacatttaagtacaaatcatttatttcagaggtgatccagggaaaagaagaaagccatggtggctgccgagcaggtcatcactgtgggtcagtcctgtggggaacccgtgggagactgcgcagaacctgccacagggaggtcccacccaaaaggcaaggaaactggagcagttggtcaccaactccagctgtcatcggttaaaggctgatcctcaaactttctggcacttctggccaagtgtgctccaaaggccagagaaaccccagggcagaaacccagggtcccacagtgagaagctgcagaggtgtggggatgagagtgctaagtggcacaggcagcccccagccttggtgtccctgtgggtcctctcagggccggggctgctctttcagccccagccatagccctagaacccccagcccccttcctgaggcccaggaggggcgtaggaggcacagcatctgctgcaggatgaaaggagccctgtctgttccctgtaggctgagctctggttctcccagctgggtggaggagggactctgtgtaggagttggggaagtgggggtgggtttcaacctgatggccctgcctgcaccccagtgttctctcctcagcactccacctttctcactggtcctcctgctgtccctgggtcctcctgggtatgcagagccctggtttccatggagactgtgctctgacctctggaaatgctccctctgaccagcttagccaggccgcctgatccccatactcacatcaaggcaaaggaacttggcagctctttaataaaaccaaatcctgttgcccaggagcttcatgtttgggcctctaggccatagggtgggtgaagtcacttctactctctttaagatggagccatcagttaaaggagggaagagatgcccaggagtggaactgtagggggcagccagagcagtaagagcaggagcaggtcagtgccgtgtcactcaggccaagggaagatgggctttgggcttctggcaattcgcagactgggcttctggcaattcgcagactgtggtcccagctacttgggaggctgagccagg

SEQ ID NO: 13199 - RNA, 903 nt, Homo sapiens
  source 1..903: mol_type = other RNA
gctgggattacaggcatgagccaccacacctggcctttcttttcattttaacagcccctgtcttggttcagatgttcagaattttctctccttaatgactgcatagtttttctgcctctcattttgcctttttcaaactcctgctagagtgcccttcttaaatgccagtctggtcaggtcactctcctgcagaaagttcttcagtgtgcctgtgctggttgagcagagcctgaggtctagagagatgcatgccttcacagatgatctccaagtgagcaggcactttccgctctgcctgccacaatatgacacagccacctcactcacttccagccaatgctgacatttgccttctcatcctccacaaagtaggaaagctcctcaaatccagaggtaacagtctgtttcacccaaacataaggacaggctagagggagcctagcttttggggggcaaccaagagtaacagctcacctatctaggacactgtctacagttttcgataccatactcctcatggaggcctggttcatcctcaggctgagggaaaaagagcaagctctggtttgtatgagaggactgctgagtgctggaagggtgtggactccagggccatactgcctggtttgaagcctgactttccatgttacctcaaataagttatttagcttccataagtcagttgcctcttctgaacaggaataaaaaattttacttcccccctaaggctgccatgaggattaaatgggctagcacatgtgaaatggtagaacagtatctgacccaccatacctgttctgtacatatagttactattacatgaccagggagaagtctccatgcctggccccaccaatacctcaaaaggagattaaattgacaacagtctacaggtacctgtaa

SEQ ID NO: 13200 - RNA, 1518 nt, Homo sapiens
  source 1..1518: mol_type = other RNA
gctgggattacaggcatgagccaccacacctggcctttcttttcattttaacagcccctgtcttggttcagatgttcagaattttctctccttaatgactgcatagtttttctgcctctcattttgcctttttcaaactcctgctagagtgcccttcttaaatgccagtctggtcaggtcactctcctgcagaaagttcttcagtgtgcctgtgctggttgagcagagcctgaggtctagagagatgcatgccttcacagatgatctccaagtgagcaggcactttccgctctgcctgccacaatatgacacagccacctcactcacttccagccaatgctgacatttgccttctcatcctccacaaagtaggaaagctcctcaaatccagaggtaacagtctgtttcacccaaacataaggacaggctagagggagcctagcttttggggggcaaccaagagtaacagctcacctatctaggacactgtctacagttttcgataccatactcctcatggaggcctggttcatcctcaggctgagggaaaaagagcaagctctggtttgtatgagaggactgctgagtgctggaagggtgtggactccagggccatactgcctggtttgaagcctgactttccatgttacctcaaataagttatttagcttccataagtcagttgcctcttctgaacaggaataaaaaattttacttcccccctaaggctgccatgaggattaaatgggctagcacatgtgaaatggtagaacagtatctgacccaccatacctgttctgtacatatagttactattacatgaccagggagaagtctccatgcctggccccaccaatacctcaaaaggagattaaattgacaacagtctacaggtacctgtaaatgaggctaaaaaggaagatgaagaacaatacccatttcatccacaggagcaatgagtatttcattccctaaatctgtggcccagatggaagtgacatcaaccttaagcttctcccacgcatatatttgtttagcactgtacagattataaattgagaatcctttggctcctccaataaacacatagtcttgggaaacagccatacaatttggcattttgttgagctggatttctccaagtggagggtagacggtgggctggatctggctgctctcagcttccctcagtgcgtttctctcttcaataatttcccaagactggtcaaacagaaggttcaccagcttgttgatcattcgataaggctgaggcaaggaatccagctcctcatctggatccacgaggacatgatcctgttcatcgtctttaggccagtccttctctgttgggggtggcacctccaatggtccctttcgtgtaccaatggggtgctttattttctgggtctgacttcctcttgggaatgacatcacagaaggtggcactgggaacctctatgaaactgaaaagctggccgggcggcgttgcgtcgccttggtaaccacaacttccggctt

SEQ ID NO: 13201 - RNA, 13048 nt, Homo sapiens
  source 1..13048: mol_type = other RNA
gctgggattacaggcatgagccaccacacctggcgatgttgaactcttgccactcaccaatcagaaacataaattctcttttttccaaagaaataataaccttatagaaatgtgagaatagagttccctttgtcattgagcataccaattagttttaaaaaccatttcttttatttcttcttgagttattttctctattattttgcctatttaatttggattttccctttcataatgattttctccatgcatctaggatgcctagtggtctatttagttttagggaaagatgatactaaaacatttactgaagaagctgagtgtgtaggtgaagctcctctggtaggctctactctgggcagtagccagcaaacttttttctgtaaagggccagaaaatattttaggctttgcaggccgtaaggtctatgttgcaactttgcaattctaccatagataatatgtaaatgaatagacaggatgcatttcaataaaaccttatttgtaagaagagggattgagccactttgcagacctctgctctaaggcgaatcagatgagaagttggacccttgcttggggtataggtgctaggaattctttgcagaagtttgcagagatgaagagttgcagccagtctacatatggaataataaaccatggttgtctcatggtttattagtgcatatgtagaacagctgcatgcccctgttcaaaaagctggtatgcccctttttgtgcttatcagctctgagtctcaagttcacttttcatcactatcctcttttgcataaattatatcatggctttctccaccctgttacgtctgttgctgctgcttttgtcttctgtcttctgaaaatttgttgaaatctttcatctagaattgtctcttttccaattctctttgtttgcattgatttatatatttttaaaatttattatcctttcacttgggtcttaagagacagacagaataaaaaatatttatgaatacactatatcaagaaacttgtgtgtgtgtgtgtgtctttttttttttttttttttttttttgagacagggtctcgctctgttacccaggctggggtgaagtggcatgatcatggctcactgcaaccttgacctctcaggctcaagtgatcctcccacctcagcctcccaagtagctgggactacaggcacacaccaacacacctggctaatttttaaattttttttgtagagacagggtctcactatattgcctaaactgatcttgatctcctggactcaagcgatcctcccaccttggcctcccaaagtgctgggattacaggtgtaaaccgccgtgcccagcaatttttaattttttgtagagatgggatctccctttgtttgttgcccaagctggtctcaaactcctgggctcaagcgatcctcctgcgtcagcctcccaaagtgagattacaggtagaaaccactaaaaaacaattttttatcttcagcttttaaggggtacatatgcaggatgtgcaggtttgttacataggtaaatgtgtggtgtggtggtttgctgtacagatcatcccatcacctagatgttaagcccagcatccattagctattcttcctgattctctccctcccctcctcaacaggccccagtggcgtgttgttccccctatgtgtccatgtgttctcaccattcagctcccacttataagtgagaatatgcactgtttggttttccgttcctgccttagtttgctaaggataacggcctccagctccatgcatatccatgcaaatgacaagatcttgttcttttttatggctgcatagtatttcatggtgtgtatatatatgtgtacagtattttatttgtccagtctatgatggacatttggatggattccacatatttgctattgtgaatagtgctgcagtgaacatacgcatccatgtatctttataatagaatgatttatattcctttggatatatacccagcaatggtattgctgggtcaaatggtatttctgcttttagatctttggggaattgccacactgtcttccacaatggttaaactaatttacactcccagcaacagtgtaaaggtgttccttttcctccacaacctcggaagcatctgttattttttttttttttgacattttaataattgccattctgactggtgtgagatggtatttcattgtggttttgattaggatttctctaatgatcagtgatgttgagcttcttttcataggtttgttggccatatgcatgtcttcttttgagaagtgtctgttcatgtcctttgcccactttttaatggggttttttcttgtaaatttgtttaagttatttgtagactctggatattagacttttgtcagatggacagattgcaaaaatgttctcccattctgtaagttgtctacttgctctggtgatagtttcttttgctgtgcagaagctctttagttcaattagatcccagtcgtcaatttttgcttgtgttgcaagtgattttggtatttgcattataaaatctttgcctgtgcctatgtcccagatagtattgcctagattttcttctagggattttatagttttgggttttacatttaagtctttaatccatctggaactaatttttgtatgaaggtgtaaggaaagggttcagtttcaattttctgcatacggctagccagttctcccagcaccattgattaaatagggagtcctttccccattgcttgtttttgtcaggtttgttgaagatcagatggttgtaggtgtgctaaattcttaatactggggtaatattaattagtttatttttactttcactagctttgaacctatttaaaatgttgtttgtttttaaattagtatcatctttttaaatcctatgtaaaaagtttcccttcaggtaggcaactcactcctaccacagaagttgattgcaggcccacatatataggcacaagctgggtcattcccaatttccaaaccaatcttacctaaaagtcttttttcctctaaggtgttccctagattgaatattttcatgaaaacagaaacattagctttcatcagggtctctacgtcacaaggccaagttcagatgctgaacacacatgaatggtcagtgtgtgaacagtgtctgaatgcagtagagctctggtgggtgccactaggacttctgcccaattaagtgttttcctcttctcaataaggtccaaagttttcttgtagaagggaattgtgactctcatgaagaatcttatggatttctgaaggtatcgtccagggactcaccacagtctcctctctttcatactctacacacacctgcttggtttgaggtgcaagcccagcacttccatgtttttttgtatgctgcagactatgacacggagcattagagcctttttggaaggtaactggagactgcgtagcctttcttactgctgctttggctccaccagcttttttctgtatggtgaaagtggcagttccatgtggccaaggtgagccttgaggttgcccaaaagacttcctcttatggatataactcggtttggacatatatttgacttttccaggtcgatttattagaaaactgtgaccatgttgattctctcctcttggagaagggcagtgttgacaactggaagactgagtagggctgggtttgttaggcaatggtttctgtggtagagttggtagctgtactgactcagataacagttcattcatcagaccgtacgcttgtgagattcgacgactatagtgttcagagagcagcaatctgtctttttcatgcttcatcttttgtctcagccttatttcccttgaagtcatgtaaagtggattgcttctgggacagaaaggatcatgttcttgccctctcttttctgccagctcatttaagtactttgccattctttcttttcgttttcttttcatccaggcttgaatctctcttctttccttgtcagttctttgtgaatgtctgccagaataatgctgaattctggaggtgcccatagcttgttctgttaagccaagttcttcactggaaactccgtctttaattataaggtcatcaataatgtctgcaatatcagtcaatccagtcatctggagcggatgtactgaaacactctcacacaattcatcactgctattcataccaggagaagtagtattctgatcactggaactggaaaggctgacagctgaatcggcagtaggaaacacacaggttttctgaccagaataattttctgttattgaaaattcaggttctgaagtctcctttttgtcactttgatcttcttcatccatatgggtcaaaaaacgcacttcttcagaaatgctaatggtttttgaagctaatgtttttttgaattcagggccagaagagaattcaatgtgatccactggtccaatcttatcacaatgtagatctagcatttcaggcttggggaaatcctgttctatgttttcagcaatgttctgtattgctagcaactgctcgtcaattttctgaagcttagcactgagatgctctagttggtgagctgcagagcttggtgcagggcaagctgcagagacaccttgcagccgtttccacaatagataatcttctgcagagtctgactttgtgctctgtcctttgaatcggaactctggttttggcagacctttgttctgctgtatgtctgatggtgtaggtgaggtgacactaggctccttcacttctgtaatgcctgctctcaagctttttccatccagacaagctggagttacttcttgactcttaaaattatgtgggggaacagcattagtaactgaagctgccatataatgtaactctgcagacgatggaactgctagatgatcgctttgctgtttgataacattatcatttgaaggctcttctctcacaggtaattcctgtagaagatcattagcttcaatgtcaatcacatttatataagtatgtccaaccaagtttgttactgtatgaggtattgagggtgaccaaggtttctctgacatttcactggaaagcttcagatttagatagacatctgggaccaagagctgaggagcagtcaaaggctcatgttctgggtctgtatttgtacttgcatcttgacttcctatagctttcttttttacagaggccatgaaatgcaatccagctgaagtattatcatcttgtagcatttcaaaaggaacgtcgaagtcatccaaaggatgggaaccacaatgttcttgttgttccttgggtttcttaatgatttctgaatcatcattattaattatggaattctctggtcgaaaagtcacatttggttttctcctcagtttctcacatcttttttcttgcagctctttctcagctcttcttctttgcctttttttactgtcctttccttgtcttacttcaggtggttctattttgacctttagaagttgaaggtgtccagcatcaccttgttcaaataaattatgtgttagtttctgttggctttgtttaaacgcaatgaggttttcaagtgggataagttgtgtttttttgcacctattttctggggacaaatgtgaatgaagtaatgacaatcttgggtattttctttcttctgctataggttggataggtgttgagggaactgtaatagatgctcttgaggttgatggaaacatattaggaggtttaagtggcaggtatagtaacggaagtccaaaggaatggtgaggagatatctcaagggtccctggcttaacatcaaatagtttttctggttttataaacactgaagagtcctgttgaggtgtcaaattttcttgtccaacatattgatccaagttcacatgattaggaatttctgtaattacagtttctgcccacgtcttctgctcaacttctttttttctggcttcagtgttatactggcttacattcaaatgggatgctggagtagtttgtgctgctctctgtggcagagcaggttggaaggagtcagataatccccaagcctctcttggttgtggcaaaggcctgaagggaacttgtggaatacttcctgtatgtaagaaaaggggctggaattcttgtttagacttaaattgaagcaaaggaaagccatcaccaggactaaatgtttttgcatgtgggataagtctaggtgccttctgaacaacagaaggtgtggacaaaaggtagaggtgagtatttccagcaggagctggataaaacgaagtggatggtaagttttgagatgatggaattggtccttttttccggggctggccatttaattgacataaaggaatactcccatgtggaacattctgtacgtttccagtactattttgaccagatgggatagttccttcatggcagtgtgggctgttcttgcgaggctctctggcgttctctcccattgactgtggtttaataaaaaatctctccttaagatttttgttgctgtcttcaacatcaccacatcctcttaggtttgattcttggctttcccctaaatgcacagactgagactgctgtacaagttgttgtgtatctgggagattagcaaaggatgatcctactatttgcattaggctcatgaagttgatctgttgcagctgaactaatttaaacatttcatcttgcagcatctgcctaacggactccgaacaatctggtaactgagccgtgaattcatttctctgggtcttctgaggtgttggagcaggtggttgtgaagcaacattgactccatttgatatcagaagtggaactgaggaagatttttctttatatgtagaaatctgtgcactagaaatttctgaactcgtatctacttgcattgattgaggagtggtatgcccaggatgtgaaaaggcttcgatcatacctttttgttcagtcgatttttcctccataattgtctccagtggttcttccctttgacactgaacctcttctgtgaactcttcttctaactgctgtggtaaagtcatcatgcaaatggcaagactgggacttctgaaacctccaacagattcttcaatgtcttcttcatagtctgatatgtgcatatccatttcctcttctgtaaatgcttctacttctaaaagattctcatcaatatctataaattcttttttagtattatgagtgatggaaataatatcatcattgatttcttttatatcaggattttttgcttcagttggcattctattcaagatattttgacaagatttattctgaccatttctttcctcagttccacctggagttgctactgcaactgaaccgccagcatctgatttgctctccctctcaatattgggtccaatctgacacccagtgtcacgattctctaccatcttaataatggcattttttgccttatatgtagcaaaatagggttgttccaaaagccataatgatgtaagaatggcagctgtagaggtctttacacgaattactggactgtactcagaggatgactcagttataccagaatcacagagtagccttctattagaccaccttatcatccattccagcagtcttcctatactgccaaaagtgtttagtgctaaaggaagatcttcttgagggttaatatcattgcactgaatagctttgaaaatacatcttctagttttaatggacttgggagtccaaaaaatgtggtttgatgatctctggattagacatttctctctagtgtcatcttgtattttgtaaattgacctttgttttaaaccaaataatccactcattccttcattcttattgacttcattcgaaggatattgtaaaaaaggtttgatcccttgattaaccagtactgatgatgaaagtttctggttttctaaatgcatgccatattcatcatttaaagaggatgatttttctgattcataggactcaggagcaacaacaaagcaagaaccagctctaaacacattctggcttttagttttgctctgatgtcgttttaatgttgtatgtacatcaaaaagtaaagaattaagttcatgttctctaagctttccagaaaaactagttagaaatggaatgtcagcatccctggaataaggtaggtctctttcaagaatgtaactcaaaaacagatcaaggaatttaatatattcatcatcatcacgttcaaattcccaaacacctattacaggaagtgtattttgtgataacttttcatgatcttctttctttgtaggattttctttctgattacacattttccttttatcagttggcttatgaattgatgttaattccatgtgatttggggcatttctttgatagatatttatcctacttttttcttcaaccgacaaagcttcagagaacgtatctgcatcactgtgaaccacagaatctcctagttctgtgagtgtacttctgctcaaactagtccccagggaatatctgtcaacacctggagcctcatctggtttctcttcttcaattggttcccatatattcacttcaaaagagcctatatttctctgcacacgttttagagctttcaccctcactttctggatagaatgcatgacaacagacatcatttcctcagtctggggtcctttcacaacacagtgtctgagtctctggtgaagagagtgatatttgtctcttaaaggaaccctcacgtcctcaggatagggaaatgctttcacgaaaatttctgctacctttctgattggtggcagttctccaataaggctcaaaattatatcctgaataagttcttccatattaaaaaaccgagagaaaggcagcattctataagcccattccactgcactaagacagtgctcaatcatacaagaatcaaactccacttcaaggtccttttctccttttacattttctcttgctttctgatattgcctgcaactataggataacttatcacggacatgcagcatccaacacagagcacaaagttctctgaagcaacctattgctctaatggaaacttcatcaagcttgtggtctccagctgctccaggtctaaaaaatgcgatacctcctttacagtaattaagtaatgactgaggaaaaggactcagtgaaggaagggatcctttcattcgaatcttctgcatgacttttcttgcccacctcaactgcaatatataccactgtgctacaggaaaagaacactgagccgcccggaaaagcaggagaacacgctgaaggattccagataccttctggcgattatttttttcagcttttaaaagaagatcatcaccatcttcttcactaagaatagctggctggggacagtacaatggaggagctggaagatacaagccgaatggcactaagccccacagtcttttactgaagtccttggcagagtctatcagaagttgaaatgtctccgaaagaatatctgcatcggccataactgatgctttcagtacttcttgtactgaaccaaatagcagatttgcatcttcctcttcaatgggatctgtaaactgtttatattttgagcccatttcattttttgcttccaaagaggctggttgacctaaaacacactgcagtttttcctgaaaaatctgtgctggagtcatacggagtggtagattcagactctttttcttggacctcatgaaattgctatcacgtttacagaacagctggaaagccacaccaattgaaacagacgtcttccagtctccaagtttatatgccaaccacacagcctctggaaccaggccaccaataaatagtaattcaagtgcatattcaactgtccacacattagagagattctgatctctaacaacactggccaccttagagtgttgcagaggaataagtcgaaaggactgctctgttttaatatgaagtgggggaagaacattcacatgatgagggggcaaaatgcaaagctgctgattggtgaaataggcagccatgaaacgagccatggactggacgactctcactgctgcctcaggatgaacaccgcccaccattccacactcaaaatgagactttgcagcacctgaaaaatctttattttcttttacaggtagttgggaccatctcaggatttctcttgctagctgatcacacaatccttgagcatcatttaaattatagctatagaggtggcagtataagagagaaagataatagcgtatctgaagaaaatacgtccttcttcctcctttctcttcgatttcttgtagagcttttttccacagctgaacagacttttcatatgatcctaataaaaaacattcttccccattgatagatttaagttctaaggtttgattcaagcaatctccagtactctgtaggttagcctgcaaatgacataacagggacttgacagtagatgcttcatgtgtcatcttttcagttaactgactatcagcttcaggaactcttcgatttaattgtgcttgataccataaagtttttttgtacagtattctccagagaataagcaatctgtgtcctggctgttgcacaggatttactacttgaggatgaatcttgaaaaatgagttccaagaccagtttttctgaaaaccactatcttgaaacatctgaaaaataggtaccaccaatgagtcttgagctgttattttacttccatcagctgatgctgaaataacttcaggttgaagaatgtatacaccatttaaattgtcagctaccattttgagtaaataaaaacaagctaaaagtttctctgagaataactgacccttttgttgctgagtcagcaaaagttttacagtatttgaggtcagctttatcaaatgccccacatcttgtttgtatcttatatcccaataatggattgataaacactgatgaaaaagttgaaagatacaaagtatccatgcattatgtcttgagcttttgcttaaaacaagatcaagtttaggaaaaggacattttataaattgaagaatgtaaaaaaaatgagtgatacaaactactatgtaatttaacattaaatttttttctgtcacagtttttgaaattcctatagtccacgctgcaagtagacttttctggatagaatgcagttctgtaatggttctatctgtctcctcactatcatcctttgcatgtatcgtatcaaacatagatgcaaattccaatcttccttccttcatactactacacagcacatcatctcttttgttccaaaaaggacataagttgtctggaaagtgtctgccttcgttagtttcttctgcttcaaaatcctgaaaatctgctgcattttcatttattgtttcttctgcctgcaagaatttggggacagtgaaatcggctgaactttcatttccttggtgttctaacaggctagaccttagggaattcagtgatcgcaagttcagtcctttgccttttggcttagacaatatcacactttgatatattttctcaagcctctgggttgaatcaagtagaagtgatctcatgtgtactgatggagataggctatcaagaaatcgaagggttgtgaccatatatccatcagatataacgaggtagggtaaccgtgagtgtgcttttatagaaaatctctgtctcatagggtcactatcagaagctgatgaatcaacagaattatttgaatcttgaaacgtaaactgctgtggtctatacgttattagtggatgaagaggaataaattctgctgggccaaattctatagagcaaccaaatgtaattaatgttagcaattcaccttggcaggtcaataaaaccagagagccacgttttaacatacaagccagaaaaagactatcatgcgtccagctgatatcacctacccagtaggacctaataagtgtagctggaaccacgggactcttgttactacatcctttaaggctaccacagagagtaacaaaattcagtgtgtttataaataatacctgagttgccttggggtctttctgattaagagttactgccagggtaaggccatctcttgaaaaggcagaaattagagctcctcttgactttactgattcacatttaggaattaaactacagagatgacagtcttgttgagcccaatgaacatggtatggcaatgatcttacagatgtaaatacattctcatgccaccgaattgctagaaatgttaacttcaggcattccccagaataaaaagtaaatgaacacaggcagcagtctccaaataactcattttttataaaaacagcattcactacagcttctttatcttcggtggaaggcaagagaactgcttcttcaggtatgacctgggaccaccgacccgccaatgaaaggcttttagaagataagatattctttaattccaaatattcccaaagaaatatgcatccagaaggtgttatgagcacaattcttttcccatttccagatacatacaagtacagtctcaaagagcttgcgactgtagctttgatcatttccttaggcttttcagttattggtatagttttcaaacaatcttgatctttgttccaaaggaaaagctctcctgtagttagtaccccagccagccaggcatcattactggatgttgttaggacaataacatccttcaagaaaggctgcagactaggaattttcttctttatctttcctgatagcaaattaatttcatttatgaatttatcatccaaaagaaaaacggcttctttttcctttcccaaccaggagacacgtggccatggttttttctgcttaatacctgttgatgtcaagatttctaatcttatctccatgtttgttaagctatcaatgaccaattaagtaaaacagtcccaagattctccgccaggggcagggtccggccagtcaggcgcgagaaggctaggcgaggccgactgcgcggggtgaagacgccaggccgacagctgcgggccctaccgccagccctgacgcgagcctgcgtcctggcgacggcggagggcgggcagggggcgcgggcgctgccacggcgcctgct

SEQ ID NO: 13202 - RNA, 2483 nt, Homo sapiens
  source 1..2483: mol_type = other RNA
gctgggattacaggcatgagccaccacacctggctaaatgtatcgtgttctaaacctgcttcattcactttggctgtgactggagacaacaaacattttgggaaataaatcatgctcatgtcatagacatgtggagtctcagcatggaccccaatctctttccactttaaggttttggagatactagatctgcagccttcattagccagccaagggggttccctagtggagaaagagattggctgtaaaaatgccgtgagtcactagtttgactgtgtcaaagcctgtgaggcagcttttgttttcaccttttcctccaaatgtttgcttcttgtctgattgacaggaggccctaaaactcatgactggtggtcactgagctctcaccctgcttggctattgtagataggcaatactaaactggggaatgcagctacagggcaatagtattacttacctggtatagatccagccttcatgtttttctgacatgtaccaagttaacattagagaaacattccaaaaggtattaataaaatgaaaagttttaccaaaagcaatgaaagttcactgctatggtctaaatgtttgtcctccccaccccaaaatgcatatgtcgaaacctaatccccaaggtgatggtattaggaggtaaggccattgggaggcgattaggtcatgagaccagagccctcatgaatgagattagtgcccttgtaaaagagaccccagaggactagctcaccctttctatcatatgaggacacagcaagaaggtactatctatgagccagaaggctggccctcagcagacactgaacctgccagcaccctgcgcttggacttcccagcctccagaactgtaagaaatgaattcctattgtttataagccattctgtttatggcgttttgttatagcagcctgaacaggctaagacactcacatcatgtctgtattttatgattgatttgagggcatccttagaaaactaaatataattgactaaaattgaatgtggactaaatgttaataatattttatcagtgttaaattctgtgagtttggtatttgtgttgtggttgttagacaacatccttgaccttagaagatacatgctgaggtatgtaggtatacaggtgtaaagggttacaatatctgccactcactctcaaagagttcagcaaaatggtaactgtaatattgtgagagagagaaagtttgaacaaatattaacaatgatagaatctatgtgaaggatatgcaggtgtttgttgtacaattcttgcaacttttatgtaaatgtgaaagttttcaaaatataaagttttaaaaaagcaaagcacaacacttcctcataagggtcaaacactggatttagaacagtcacatgacaaaaaacatcaactggaaaagggtcgccagagtgcagtcagcacatgttttgtgggcctgtttatgctcaggattgtcttggaaagtccaaagcaccagaaaggtgtagcatgtgcattaagggcactgctggctgccagttgtcaagctcctcaacctcttgtatctcatttttcaaactgttggccttctccttcacccagaaaggcaagttgggaatttgtggaagaggctcaagtggaataaatgtatcaaatttcttttcataaggcactattgaaaaattcactggtgggagcattgatcctgctttgtggaagcctttactctgttctgggtacatatatggattgtcgcctggagttaactttgggattccattcctgggatcaatatcgtatttctttctcccaaagcacttgtccaccgtcctctctgatagagacctcttgttgccgaggaagactccattaaagaagcactgctttccgacgtggtaggtgtggatgttgctgctaaaccttgggtaaaatgtccactcaggacgatgcccatctttcgtctgcaacttaagcaggctgaattcctcaggatatttatccttttggacttcaggcaacgacatttcagaggagtgatcagaatgtgagaaggagagtttccgatccaagtcagcagtggtgtctacgtaagcagacactctggggaggccaggaggctcactgacacttgggcctgtttccacagaagatgaggaactgacacttttgccagagggtgttgtgttggcaaaacatcccttagattccagaaaatcactgcaattagcactgtaggtcctctccacctcggtcatgccagagtcccttttttctggaaccttctccagctgtctgccgcaggtcgtgcttgagatggaggggagacggcagccccgtggactgtttccagtgagcatggatggactcatcaacgaaccaactggcaactgaactgccgaacgcacgccgcacgccgaggcctgagaaccgagagcctagggcaaaagggacaccgcagccgcctgcttctcccacagaggcgcgttcc

SEQ ID NO: 13203 - RNA, 2475 nt, Homo sapiens
  source 1..2475: mol_type = other RNA
gctgggattacaggcatgagccaccacacctggctaaatgtatcgtgttctaaacctgcttcattcactttggctgtgactggagacaacaaacattttgggaaataaatcatgctcatgtcatagacatgtggagtctcagcatggaccccaatctctttccactttaaggttttggagatactagatctgcagccttcattagccagccaagggggttccctagtggagaaagagattggctgtaaaaatgccgtgagtcactagtttgactgtgtcaaagcctgtgaggcagcttttgttttcaccttttcctccaaatgtttgcttcttgtctgattgacaggaggccctaaaactcatgactggtggtcactgagctctcaccctgcttggctattgtagataggcaatactaaactggggaatgcagctacagggcaatagtattacttacctggtatagatccagccttcatgtttttctgacatgtaccaagttaacattagagaaacattccaaaaggtattaataaaatgaaaagttttaccaaaagcaatgaaagttcactgctatggtctaaatgtttgtcctccccaccccaaaatgcatatgtcgaaacctaatccccaaggtgatggtattaggaggtaaggccattgggaggcgattaggtcatgagaccagagccctcatgaatgagattagtgcccttgtaaaagagaccccagaggactagctcaccctttctatcatatgaggacacagcaagaaggtactatctatgagccagaaggctggccctcagcagacactgaacctgccagcaccctgcgcttggacttcccagcctccagaactgtaagaaatgaattcctattgtttataagccattctgtttatggcgttttgttatagcagcctgaacaggctaagacactcacatcatgtctgtattttatgattgatttgagggcatccttagaaaactaaatataattgactaaaattgaatgtggactaaatgttaataatattttatcagtgttaaattctgtgagtttggtatttgtgttgtggttgttagacaacatccttgaccttagaagatacatgctgaggtatgtaggtatacaggtgtaaagggttacaatatctgccactcactctcaaagagttcagcaaaatggtaactgtaatattgtgagagagagaaagtttgaacaaatattaacaatgatagaatctatgtgaaggatatgcaggtgtttgttgtacaattcttgcaacttttatgtaaatgtgaaagttttcaaaatataaagttttaaaaaagcaaagcacaacacttcctcataagggtcaaacactggatttagaacagtcacatgacaaaaaacatcaactggaaaagggtcgccagagtgcagtcagcacatgttttgtgggcctgtttatgctcaggattgtcttggaaagtccaaagcaccagaaaggtgtagcatgtgcattaagggcactgctggctgccagttgtcaagctcctcaacctcttgtatctcatttttcaaactgttggccttctccttcacccagaaaggcaagttgggaatttgtggaagaggctcaagtggaataaatgtatcaaatttcttttcataaggcactattgaaaaattcactggtgggagcattgatcctgctttgtggaagcctttactctgttctgggtacatatatggattgtcgcctggagttaactttgggattccattcctgggatcaatatcgtatttctttctcccaaagcacttgtccaccgtcctctctgatagagacctcttgttgccgaggaagactccattaaagaagcactgctttccgacgtggtaggtgtggatgttgctgctaaaccttgggtaaaatgtccactcaggacgatgcccatctttcgtctgcaacttaagcaggctgaattcctcaggatatttatccttttggacttcaggcaacgacatttcagaggagtgatcagaatgtgagaaggagagtttccgatccaagtcagcagtggtgtctacgtaagcagacactctggggaggccaggaggctcactgacacttgggcctgtttccacagaagatgaggaactgacacttttgccagagggtgttgtgttggcaaaacatcccttagattccagaaaatcactgcaattagcactgtaggtcctctccacctcggtcatgccagagtcccttttttctggaaccttctccagctgtctgccgcaggtcgtgcttgagatggaggggagacggcagccccgtggactgtttccagtgagcatggatggactcatcaactggcaactgaactgccgaacgcacgccgcacgccgaggcctgagaaccgagagcctagggcaaaagggacaccgcagccgcctgcttctcccacagaggcgcgttcc

SEQ ID NO: 13204 - RNA, 284 nt, Homo sapiens
  source 1..284: mol_type = other RNA
gctgggattacaggcatgagccaccacacctggctgatatactataatttctgcatctcttagtttaacctctgtccttcctttatcttcttgcatgatggcatatcaggtaacagctggccaggcatctctttctgtgtgatctctccacctggctagcttgggttttctgtcatcatgacagtctcagcatagtccgacttcttacaatgtggccagcttcccctaaatacaagaggagaagcttcctgatcttggtgcctggactcaggagtcccagaaat

SEQ ID NO: 13205 - RNA, 4947 nt, Homo sapiens
  source 1..4947: mol_type = other RNA
gctgggattacaggcatgagccaccacacctggcttccaaatgagtatgttggagccataacccccaatgtgactgtatttggagacagggcctttaaagtggtaatcaaggtgaaatgcagccataagggtggctaatccaatgtgactgatgtcttcagaagaggaagaacacagttacaaatgcataatcacagaggataggccactatgggcaaaagtccagagcgggcacaactggtagctatcagttgttaacactcccaggaagtgaaggaataaatgcttctgtcttgaaagggggtggttctgggtgccgtgccacagagtccactatgctgtcattgttcatggaccacacaattgtgtactgagataatttaaaagaacctggataactgtagcagtctcctaaatggtttcaaggacttcggctttcttcttctccaccccattcttcacattactgctagaatgatctttctcattcacagggatcagaatactgaattgttgcctgttcatctggtaggtagtagtcatagaccttgatggttgctggtttcaagttggtgaccagcacactttggctgatggtgaaggtgtaagtctgagtgttcttaatgagctcatccaagtaaatgttaagtgtgtcagttccaaattcaaccttcttcaccaggggttgctggagaagtaactgattggtgccctccatgggactgaacccagatagcatcttcacttccacaatagccatattggaagagctacggctccccacataactggtgtgaatagtgagagtcaaggatcgaggtgaagtcggttgctcacatctagcttttcctatttccacactaagactaaaggtcttcatatttgtgggagggagaatattgtatctcaacaccgtctgcacatagacacagccctggcctgaggcctccaacgtgtacattccagggacattgggcagggtatcctgctgaaataccaatctgttaactgactgtatgttgaatgtgcgctggaaattctcagtggattttacaaccaggttgatctcctcagatggcatgtaggcggtagtggcatatttggcaagagcttggagagcaactacagtatcctgagtagaagagaagcccccatatgcattgtgttgcttggccaaccaagccactatgctagtggccttcgctatctccttttgagtcaggctgggcttggtaagctgggccaacaatgcatatgctgtgagttccacatctacagccgcaggctcagaccaagggctggcgttcgatgatggagtaggtttctggctccagtaaatggattctcctgagatgatagcctgttgatctaactgtttaaggagaatgtttctgatgtccatttccccagccagggagaaaatgtaagccaacagggcctgtgtgtagaggttggtcgtggaggtggccgaattcttgagacaccgtagaccctgactcaccattgggtcatctacatcctttcccatctccagcaatgcagctgtgacatacgcagtcaaggagacctcatcatcaacaccacccttcatagctgtgtgaaggagatttcccacgttggcatagcagccactggggagctggtttcctgccatccacttgagagcatcctggatgttcttgggatcaatgaagatgaatttctgagcttggccaaagcattttgtgacaaacgctgtcagccatgtgtttccatttccatctcgctccccaaaggcactgtatgagccattgctgtgtttgtacatcagctccttctggtaccctatttccaggaaacccactgcccgagacctgatctcctccgtcagcagccctgccttctccaggtactgcaagacatagatgatgggagcaaacaagaccatgttctgctcgccacagccactgggcatctgcaccagaccatccaggttctgcagggctgtgcccataatgtctcccagaaccgtaacataagccttggtcgagtcaggaacaatgtccactgggagctccagggagacagattcagatgccacctttccttttgggcacagcaatgagctgtgtgtcttctccaccaggactccctcaggtttgacgagaactggcttgatgagcgtgtcacttcggcccttttggggaacaaaccccttctggcccccacatggttcattgctgtccagaatctttgtactaatagtaaagttaatgtgacccaatttgacagctgtgatgttccagtggtgggtttttgcgtcatcagcacagagacaactggaggtctgagaatctgcccatgattctagctggtactcatgcgatttagccaggtcagtctgaaccctgatgcaatcctttaggtaattgaagatggtggcagtaagacgaaaggattccccacggactactgagtaagggagagtcaggtcaacaaagaacggcttgaaagcagttagtccaacagtgggtgaaagcccgaagcctcttgactgggaagtgcagaaactcatcgccttccactcggtgatggcgtcaggaactgtgacgtggaccgcctccttccccgagttaccaataggaaacagatcccagagccaggtctctgggaagtactggcggacctgagaatcctctgcttgatgtaaaggagttgatgactcaaaagcctctggatgaccaccgcctgcacccatagcagtgctgtattctggagatctgtgactgcaatctactggcttcttgattttggcattggacagtattttcaggcccacgtcccggaaaaagctgaaaaggtccgtgccttcagagaacgagggcctccagataatggaacgctggctcgaatgcccttggggcattgggtcaatgaggggctgaggaaagtcccatgggccagacactggacactgatcatactcagccacttgataggggtagtgaccataccagaatggaaacatcccatagacagagcggttgctcagctctctgtctggcctaagcagtaagacactctcatccaccgcccggagcgcacacagggatccgggagctgcctgcagctgcagctccacttctgctcctggaagctgctgggagggggagaagccaagggaaacctgattgtcaaagcacatctcgactgagaactgaattttgtcagctacaacacctccactgggaaaaatggcatagatcaccagggaaggatcaggggccagtctcgaagtgaaggtcagtgagagagagaaggaggctttcagtcctttcttcttagagttcaggtgtttctgcccctccatcaccaaacttcctttccctattaaatagtaggagaagctgatctcttggtcagggcttgcatcggccgggtcgatgtaataatccaccagcacttcctggggctggccacatttcaaggggccgtttagccggtggatgccaaggaagctgcgggttgtgctgtagaagggtcgcaggtgcaggtaggcattttggtagtaacgtggcacttgttccggattatatactaagtcttccatttgaaactttccctccagagaaacgtctgtcccattccaaccggatgtctccaaggtaaagggagctaggccattgttatcagtaaccagggtctggttgaaggttccatttgtgccataaatcaccagaaacactagatggttcttgaggaaggagtcatcatggcccctaactcttatcttcccactgaaggggaaatttggatggtaaaaattgctggtgtcttcaaaggtcattgatcccatttgtggagaaatgtagatattctgagtggcattggcctccacacctgtcccttcctccacaacagtagccacaatattgatttgatggctgtacgcatatccaatgaggtcaaaggtggccatgtccacaggtgctgagaaacatcctgttttgtcagtctgtccagagaggttcctgcatttgtcaggaagctgttcccgttccacctctcgataccagtaagtatttgccttctgacacacagatacctgcactgcccctagcatgggctttccataggtgtacctacaacaaatttttactaagaaagattcctgcaccgttgataactccttgggttccaccacttccaccttaaacttcggcagcacatattcctccacactgaaagtaccaaaggtcttgccctcagccactgccacagtgtaggtgcccagcattgcctctggtgccagttggaaggacaggtctacaatgccttgctcaggtaccacttccagccactgtgcaatcctgttgctatttggatcctgtagttccaccatggagtacttgtcattcactggaacgaagttgctatccatggtgacaatgcggaaatacacttgctgccctggggtgtagagaggtttgtcagtctgtacaaaggtgccgttcccctgcctctgaattagaacctttttcttctcctcaaagctgatgttatttccaactcccgacacccggattgtggccacttcttctgtgccaccagcaggaggtggtacaagaaaggagatacaatgtaagtgcctcttcttcagtccagagtattctagcaacttctgggtcttgtccttggtctccagagtaaccgtgaatttaacatcactgtacccagggctcaggtccaaacaaaccttctgaacggaggggaaatttagccgggctggtaatgtcaccaggtagtttggaagttcttctgcaatggctggtgatagggccaacattcctagaaggagctgagcccacatctttgtgggtgagacagatttttccagggtcaggggcagagatcgctccgcgtagctttatatactaattccaggtagggtgtgcagtgatgactgat

SEQ ID NO: 13206 - RNA, 4986 nt, Homo sapiens
  source 1..4986: mol_type = other RNA
gctgggattacaggcatgagccaccacacctggcttccaaatgagtatgttggagccataacccccaatgtgactgtatttggagacagggcctttaaagtggtaatcaaggtgaaatgcagccataagggtggctaatccaatgtgactgatgtcttcagaagaggaagaacacagttacaaatgcataatcacagaggataggccactatgggcaaaagtccagagcgggcacaactggtagctatcagttgttaacactcccaggaagtgaaggaataaatgcttctgtcttgaaagggggtggttctgggtgccgtgccacagagtccactatgctgtcattgttcatggaccacacaattgtgtactgagataatttaaaagaacctggataactgtagcagtctcctaaatggtttcaaggacttcggctttcttcttctccaccccattcttcacattactgctagaatgatctttctcattcacagggatcagaatactgaattgttgcctgttcatctggtaggtagtagtcatagaccttgatggttgctggtttcaagttggtgaccagcacactttggctgatggtgaaggtgtaagtctgagtgttcttaatgagctcatccaagtaaatgttaagtgtgtcagttccaaattcaaccttcttcaccaggggttgctggagaagtaactgattggtgccctccatgggactgaacccagatagcatcttcacttccacaatagccatattggaagagctacggctccccacataactggtgtgaatagtgagagtcaaggatcgaggtgaagtcggttgctcacatctagcttttcctatttccacactaagactaaaggtcttcatatttgtgggagggagaatattgtatctcaacaccgtctgcacatagacacagccctggcctgaggcctccaacgtgtacattccagggacattgggcagggtatcctgctgaaataccaatctgttaactgactgtatgttgaatgtgcgctggaaattctcagtggattttacaaccaggttgatctcctcagatggcatgtaggcggtagtggcatatttggcaagagcttggagagcaactacagtatcctgagtagaagagaagcccccatatgcattgtgttgcttggccaaccaagccactatgctagtggccttcgctatctccttttgagtcaggctgggcttggtaagctgggccaacaatgcatatgctgtgagttccacatctacagccgcaggctcagaccaagggctggcgttcgatgatggagtaggtttctggctccagtaaatggattctcctgagatgatagcctgttgatctaactgtttaaggagaatgtttctgatgtccatttccccagccagggagaaaatgtaagccaacagggcctgtgtgtagaggttggtcgtggaggtggccgaattcttgagacaccgtagaccctgactcaccattgggtcatctacatcctttcccatctccagcaatgcagctgtgacatacgcagtcaaggagacctcatcatcaacaccacccttcatagctgtgtgaaggagatttcccacgttggcatagcagccactggggagctggtttcctgccatccacttgagagcatcctggatgttcttgggatcaatgaagatgaatttctgagcttggccaaagcattttgtgacaaacgctgtcagccatgtgtttccatttccatctcgctccccaaaggcactgtatgagccattgctgtgtttgtacatcagctccttctggtaccctatttccaggaaacccactgcccgagacctgatctcctccgtcagcagccctgccttctccaggtactgcaagacatagatgatgggagcaaacaagaccatgttctgctcgccacagccactgggcatctgcaccagaccatccaggttctgcagggctgtgcccataatgtctcccagaaccgtaacataagccttggtcgagtcaggaacaatgtccactgggagctccagggagacagattcagatgccacctttccttttgggcacagcaatgagctgtgtgtcttctccaccaggactccctcaggtttgacgagaactggcttgatgagcgtgtcacttcggcccttttggggaacaaaccccttctggcccccacatggttcattgctgtccagaatctttgtactaatagtaaagttaatgtgacccaatttgacagctgtgatgttccagtggtgggtttttgcgtcatcagcacagagacaactggaggtctgagaatctgcccatgattctagctggtactcatgcgatttagccaggtcagtctgaaccctgatgcaatcctttaggtaattgaagatggtggcagtaagacgaaaggattccccacggactactgagtaagggagagtcaggtcaacaaagaacggcttgaaagcagttagtccaacagtgggtgaaagcccgaagcctcttgactgggaagtgcagaaactcatcgccttccactcggtgatggcgtcaggaactgtgacgtggaccgcctccttccccgagttaccaataggaaacagatcccagagccaggtctctgggaagtactggcggacctgagaatcctctgcttgatgtaaaggagttgatgactcaaaagcctctggatgaccaccgcctgcacccatagcagtgctgtattctggagatctgtgactgcaatctactggcttcttgattttggcattggacagtattttcaggcccacgtcccggaaaaagctgaaaaggtccgtgccttcagagaacgagggcctccagataatggaacgctggctcgaatgcccttggggcattgggtcaatgaggggctgaggaaagtcccatgggccagacactggacactgatcatactcagccacttgataggggtagtgaccataccagaatggaaacatcccatagacagagcggttgctcagctctctgtctggcctaagcagtaagacactctcatccaccgcccggagcgcacacagggatccgggagctgcctgcagctgcagctccacttctgctcctggaagctgctgggagggggagaagccaagggaaacctggggaagggaaaggtataacttggggatcaggtcagcctgattgtcaaagcacatctcgactgagaactgaattttgtcagctacaacacctccactgggaaaaatggcatagatcaccagggaaggatcaggggccagtctcgaagtgaaggtcagtgagagagagaaggaggctttcagtcctttcttcttagagttcaggtgtttctgcccctccatcaccaaacttcctttccctattaaatagtaggagaagctgatctcttggtcagggcttgcatcggccgggtcgatgtaataatccaccagcacttcctggggctggccacatttcaaggggccgtttagccggtggatgccaaggaagctgcgggttgtgctgtagaagggtcgcaggtgcaggtaggcattttggtagtaacgtggcacttgttccggattatatactaagtcttccatttgaaactttccctccagagaaacgtctgtcccattccaaccggatgtctccaaggtaaagggagctaggccattgttatcagtaaccagggtctggttgaaggttccatttgtgccataaatcaccagaaacactagatggttcttgaggaaggagtcatcatggcccctaactcttatcttcccactgaaggggaaatttggatggtaaaaattgctggtgtcttcaaaggtcattgatcccatttgtggagaaatgtagatattctgagtggcattggcctccacacctgtcccttcctccacaacagtagccacaatattgatttgatggctgtacgcatatccaatgaggtcaaaggtggccatgtccacaggtgctgagaaacatcctgttttgtcagtctgtccagagaggttcctgcatttgtcaggaagctgttcccgttccacctctcgataccagtaagtatttgccttctgacacacagatacctgcactgcccctagcatgggctttccataggtgtacctacaacaaatttttactaagaaagattcctgcaccgttgataactccttgggttccaccacttccaccttaaacttcggcagcacatattcctccacactgaaagtaccaaaggtcttgccctcagccactgccacagtgtaggtgcccagcattgcctctggtgccagttggaaggacaggtctacaatgccttgctcaggtaccacttccagccactgtgcaatcctgttgctatttggatcctgtagttccaccatggagtacttgtcattcactggaacgaagttgctatccatggtgacaatgcggaaatacacttgctgccctggggtgtagagaggtttgtcagtctgtacaaaggtgccgttcccctgcctctgaattagaacctttttcttctcctcaaagctgatgttatttccaactcccgacacccggattgtggccacttcttctgtgccaccagcaggaggtggtacaagaaaggagatacaatgtaagtgcctcttcttcagtccagagtattctagcaacttctgggtcttgtccttggtctccagagtaaccgtgaatttaacatcactgtacccagggctcaggtccaaacaaaccttctgaacggaggggaaatttagccgggctggtaatgtcaccaggtagtttggaagttcttctgcaatggctggtgatagggccaacattcctagaaggagctgagcccacatctttgtgggtgagacagatttttccagggtcaggggcagagatcgctccgcgtagctttatatactaattccaggtagggtgtgcagtgatgactgat

SEQ ID NO: 13207 - RNA, 6833 nt, Homo sapiens
  source 1..6833: mol_type = other RNA
gctgggattacaggcatgagccaccacacctggtgggacagggattttaagttttaaaaaactcttctgtggagcttatgttaggtaatttgcctaagagagttgtaaagcagtgcaagactaactaggcaagggggtatgtgtagctattgaggattaagggatagtgaaatgaactttaggaacattctcagccataagcaagagctggattcacacaaccaatttttgaaaaaaatcaagatacccataatttgggcacctttataattcatgatgagaaagagcatgttaactacatgtttaaatatattttatttcaagttaatataacagccatgatttgttcatttaagtgaaatgcttcgataaaaacctcggtgtcacttggttaaaatattggagacagattaaatgttaagccactatagtagtgactctggttctttagactattgcatgtaccttgttaatgaactacaggaatgcacattgatataatgcacaatgtcttcacatgtctcaatcctcattcctcttcctttcatgcctccctaatgcctcagtatccaatataaaactacaaaaactactgttcttttcgtttgagtggtatttaattaaaacttcaattctatgttatttccacagtccagtaatttattttaaatttgagtaatttcaaattccacaaacaaaactgaagaacagcaatattttgtttgaatttctctcttctgtacactcagtgatctaaaacaccacaatatccaacatacacaaacctcagggaagggttagtaaacacacacaagattggaatcatggtgctctttgctcctgaatggaatggtcccacagaaaaagcacaggatacagcacaacataagggcacctgttacatatgaagtgagcaaaacatactagcattttctatatgcataatggggaaacctgcataggttagagggccttttacgctcatttaaaaatcaggcaagttgtctgtaacatttttcaataatctgggaagcactgcaatccagtgtacgatgtgctgattagtgttgtctttgttggcactgacagtcttgcatggtcatatgccagtgtttttgctttagcttttctttgaataaaacagatttaaatgcatttagacaatacgtatttgtaagctgtttacatacactaaatttaagagattcaatattagagtttctttgtttctttaaacactacagagtgcaaatcaggttcttcacaacagattgaatattgagcagttctttaaagaaagagggggaagaaaaaaagcccaagtgaataaaacattgaaactattccccttcgaaaataaattctaaaatgatgtggaatgtgaaataaggttttaacataggtgatccaagtttatagttagaaacaaaaagaagtccttcatgaaataaaggttacaagaacacgttgcctgttttcccccattataaactgagaagtgggtaaagacgatgtttcagtacgaaaataggtgactacaggatcagcgcttcatctcacatgctgtacccaaagccaggctgtggctgtccatacggtggtgcggtataaccataaccaaaaggtgcctggggagggacggcaacactgggtcctgctgtcagcatcaactggggctgaccataaacaatgggttgtgtctctgtagcttgttcttcttcttttctcagtgattctgaagcatctaatttatccacctttgtcaagtactccttcatgacctggatgaaatagggcatggcaaaatccatgatattgtgcctccatgcagtttctaggacgacatctggccttaaaagatcgtaacaggtaaacagacaagctccaaagcactctcttttttcttcctgcaaaaaccactgcaggagttcttcagccaattcagtatctttagattcagaagcatactgcattgcatccttgtaaaggctgtctttcttgcacagctctacactctgtttccagcgattgttgcctttgaagagataagcagcaattctcctgaactcaatgagttcatgtttttccaaacgctgagcaagcgagatattgtcaaagttgtcataagcatctattgatgttcgcagagcctgataatcttcttctgtaataaaaagattgttcaatgattcattcacagatttgttgttatggttctgaactgaacgcaaatacggtttcaccagtggtagctgtttaaccttgctgaaataattgactgcacgagtgtgatccaaccgtggagacagcaccatcagcaaatcatttaacaacagaggcttgaattctaagtagaactgtattgctctgtagtatagttccacattggcaaccttggtaatgatatctttgaattgcccttctttccaggcatcagttggatgattcatcatggtaattatggcattatcatattcttcatacttgtcatacaaaaacaccagttctgcccaaagatgagcttgttctgcagctcttagcaccttgggaatattcactctagaccagaacagctccaggtgctccctcattttctgaggcttaaatttagagtatagaatagctaattcagtaaacattcccatgtgagctcgctcaagtcccagtgctgcttccaacatggtgatcagctcttcaaaatagccacgatcctgatagtagttgataagttcttctaattcatctgcatgtacaacaatatgaagtccacacatctgagcaagacggaattctttcccatctacacaggcgaagcagacctctttccatgttcgagtactgttagctttcctagccccatcaacagctgcctgatattcacccaggtgaaccagggtagatgccaaacgtccaaaattggaaacattattgtacaacaacttagcagcatcatacattttttcatcataacaacggtcaccaacttgttggatatgagcattatttggtccattgataaattcttctaactctgcaaggcggtttgttttagccagtgcgaatatcagttctgtctccacataggactctcgagccttcttacgggccatctgcaagtacttcaccagttcttcccagtttccactagtattggcagcctgaacaacttccatgtaggaggaaggatcatctgctttgatataagaatcaatggcttctttcaccattcctttctgcaactgggcttttgcaagttgactccagaccgcaggttcattgcaacgttcagcaaactcatatgcccgatccaagtttccaatatgctcaattaagacctgaactgctgaagtattgacatcaaatttccggaaaatggcaaatgcttcttcaaacagctcattgctgatggcgatattggcaatatctggggcatcataattatccaggcggttaatatactccataacacgtgtacggtcagccttaattgcagtgaggataaggaggttttgcagattcctgtgttcactgaatacagagttatcaaggacaattttctccagcagttcaatgagttcattaggaaggtctgcagtcatgaaagcctttacagttactgacacttcttcagggtcctgagtctcagacaaagctgtttgtacaacctggtcaattaggggtctcctgtaaggattgctttccagcagcacgctgccccacaattctggatcctttcgacgtaccaggtagcgagaaagacttttgaagagggaattctcattgcaaacattaataagttccagatcacattggccacgttcataagcaacacaggccagatgtggatctctcttctcacaatactttccaacaacgcgactgtcatagtagggattttcacgaagaaatctctccgggttgttattactgtctatgtagattttggctaaggcattgtgagtagcaggctcctcacagccctcatgaattctggcctctagccaaggcagaagcagtttcaatctgtttcttttttcaacctcagcaacaagctcatcagtagagaattgacctcttacaacaagaatcaagttttttatgacatcttcagaacagtcaacatcaagtaatcctccaataactacaggaagtcgacttggattcaccttctgtacatatatctctatatacttttgaagattatttctatataaatagagcaccaaatcatggacaaagtcaaatcgatcacacacaatgataagtggtagctgatctgttagttttgcttccttaagaaaattcttgactcgctcaggatcgtagcagttgctttctctacagattctttctacttctttgatttgcccagtcttgcaagctgcctgaatatatttaaagtgcacatctgggtcctggctaaagttaacaatggatcccagaaaataaaagagaccttcaaaactcttgaaagattcaaaaagttcaatcagagactgagttgacagttgttcatgatatttagaagccacctgaacacaaatctgcagattctgacggatgttggcagacagcatggctctgagacattctagggagtcttctactgataaggaaccaaagtagttgactaaccactcagggttaagaagatgggtgtgaaccactgcacgttttatatcatataaatcagtgaaatgttctaatgcacgctgcagtaggccagccttttcacacagttgagcaatatgagcccggtcataatgtgtgaacatctgattgcctagaatagcatctgcaacttgaggcgcatgcataaggttcatctcaagtaaccgcgtctgtaaaggaccttcagatgggcgattattcttcagagcatcaagcaagaatgcagtacactgctgaattagattgtattccataaagacatctacaatctgtgtgatgtcagcaagaggctcttcatcttgaactaacatttgggcaaactgctgtccctgatctggactgattcgcattacatttctcagcagaaatatccaatctggagtgtatccaacttttttagcatataaaacaatcttttggacttgacctgtttctgcaaagcactgaatgactttatttgggacgttagcccttaggtacacactaagtgccaatgtagggtccacagatttcacaagatcacccagttcttcagaacattccagcttatcttcttttaaccatttctccaaaagctgttttcgcccttgctgaagtacaggcctacaaagctctaaggattcgtatttgttgagctgtccctggtccaaaaggataccaaagtactgaagtagaggagaagtttgacctggctgggctgggacactctggaaccgacggatagtgtctggagtacgaagaattccctttggtgcattagcagccacctttgctgcctccgagtaatttccctgggcaaaaagagcattaaatttccgggcaaagagttcttcagcaccggctaagttattacgtacagccattctcagagccaaatcaggattttgtagaacattggtgatgtaaggaattatgttttcttcttccacacacactgacagaacttgtccctttctgtttactccaattattccagctgtggcttcatgaggtgcagtaacaaaaattgtttctccactgattctattcatgtagatgcaggtaccagtctcaagatcatagaggtggatataaccatacttggttatcaagaacaccacatcatgcttttcactgatctgcattgcaacaggaaaatcattttgtgcttctggaggaaagaagacatccactgccttctttggaaagggctggttccctgtaggtggtgtgccaacttcaataatatgtaacttccctccagcttggccccgaactgcaaaacaaaataacgttgattcttctgcatttccttccatcttaaactgtgcaaagctagctgcatgtccttcaatgggctgagacactttcctatctacagaatatagctgcatagctcccaccacacgattttgctgtgcagatataccagtcagaagtaaccacttttgttttgcatctgtacggtaattgataatctggcaccctgcaaggctagaatggcgatcaaacattttcactggctgagactctccttccatactccagtgataaactgcattatccgtaacaagagcaaccgtattcaaagagatccatttccaaaaggtgacatcatcagtcatggtatgagccttcattttacttttcatttcaatgttaaaaatctgaagagttttcccagattcttttatacctttcagtgcaattactttgctagctggattcatgatggcgctgtctgctgaaattggtcttcgaattggattacttgggtcattcatatcaatgattaccacctgggcctgctctcctactttttctctaatgcagatgaatttgtcagactccatagtcagggtactgaagccaatgtttgctgggttgatacccaggttctggagctggagatgctcctgaaaacgaattggcagaatctgggccatggcgctgtcgggggttatggtctcctcctgtcactggggctgcggggcagtggctgcccgggctctccaagggagaggaggagaaggggaggggggaggctgggctcagcaggatcctctccggggacgcaggaaactggcaggcagacgaaagagctcgggtcgggggcggaggctccaggggccaggagagccgcaatggcggaaccgggcgcagcgcagactccggaaacggct

SEQ ID NO: 13208 - RNA, 6821 nt, Homo sapiens
  source 1..6821: mol_type = other RNA
gctgggattacaggcatgagccaccacacctggtgggacagggattttaagttttaaaaaactcttctgtggagcttatgttaggtaatttgcctaagagagttgtaaagcagtgcaagactaactaggcaagggggtatgtgtagctattgaggattaagggatagtgaaatgaactttaggaacattctcagccataagcaagagctggattcacacaaccaatttttgaaaaaaatcaagatacccataatttgggcacctttataattcatgatgagaaagagcatgttaactacatgtttaaatatattttatttcaagttaatataacagccatgatttgttcatttaagtgaaatgcttcgataaaaacctcggtgtcacttggttaaaatattggagacagattaaatgttaagccactatagtagtgactctggttctttagactattgcatgtaccttgttaatgaactacaggaatgcacattgatataatgcacaatgtcttcacatgtctcaatcctcattcctcttcctttcatgcctccctaatgcctcagtatccaatataaaactacaaaaactactgttcttttcgtttgagtggtatttaattaaaacttcaattctatgttatttccacagtccagtaatttattttaaatttgagtaatttcaaattccacaaacaaaactgaagaacagcaatattttgtttgaatttctctcttctgtacactcagtgatctaaaacaccacaatatccaacatacacaaacctcagggaagggttagtaaacacacacaagattggaatcatggtgctctttgctcctgaatggaatggtcccacagaaaaagcacaggatacagcacaacataagggcacctgttacatatgaagtgagcaaaacatactagcattttctatatgcataatggggaaacctgcataggttagagggccttttacgctcatttaaaaatcaggcaagttgtctgtaacatttttcaataatctgggaagcactgcaatccagtgtacgatgtgctgattagtgttgtctttgttggcactgacagtcttgcatggtcatatgccagtgtttttgctttagcttttctttgaataaaacagatttaaatgcatttagacaatacgtatttgtaagctgtttacatacactaaatttaagagattcaatattagagtttctttgtttctttaaacactacagagtgcaaatcaggttcttcacaacagattgaatattgagcagttctttaaagaaagagggggaagaaaaaaagcccaagtgaataaaacattgaaactattccccttcgaaaataaattctaaaatgatgtggaatgtgaaataaggttttaacataggtgatccaagtttatagttagaaacaaaaagaagtccttcatgaaataaaggttacaagaacacgttgcctgttttcccccattataaactgagaagtgggtaaagacgatgtttcagtacgaaaataggtgactacaggatcagcgcttcatctcacatgctgtacccaaagccaggctgtggctgtccatacggtggtgcggtataaccataaccaaaaggtgcctggggagggacggcaacactgggtcctgctgtcagcatcaactggggctgaccataaacaatgggttgtgtctctgtagcttgttcttcttcttttctcagtgattctgaagcatctaatttatccacctttgtcaagtactccttcatgacctggatgaaatagggcatggcaaaatccatgatattgtgcctccatgcagtttctaggacgacatctggccttaaaagatcgtaacaggtaaacagacaagctccaaagcactctcttttttcttcctgcaaaaaccactgcaggagttcttcagccaattcagtatctttagattcagaagcatactgcattgcatccttgtaaaggctgtctttcttgcacagctctacactctgtttccagcgattgttgcctttgaagagataagcagcaattctcctgaactcaatgagttcatgtttttccaaacgctgagcaagcgagatattgtcaaagttgtcataagcatctattgatgttcgcagagcctgataatcttcttctgtaataaaaagattgttcaatgattcattcacagatttgttgttatggttctgaactgaacgcaaatacggtttcaccagtggtagctgtttaaccttgctgaaataattgactgcacgagtgtgatccaaccgtggagacagcaccatcagcaaatcatttaacaacagaggcttgaattctaagtagaactgtattgctctgtagtatagttccacattggcaaccttggtaatgatatctttgaattgcccttctttccaggcatcagttggatgattcatcatggtaattatggcattatcatattcttcatacttgtcatacaaaaacaccagttctgcccaaagatgagcttgttctgcagctcttagcaccttgggaatattcactctagaccagaacagctccaggtgctccctcattttctgaggcttaaatttagagtatagaatagctaattcagtaaacattcccatgtgagctcgctcaagtcccagtgctgcttccaacatggtgatcagctcttcaaaatagccacgatcctgatagtagttgataagttcttctaattcatctgcatgtacaacaatatgaagtccacacatctgagcaagacggaattctttcccatctacacaggcgaagcagacctctttccatgttcgagtactgttagctttcctagccccatcaacagctgcctgatattcacccaggtgaaccagggtagatgccaaacgtccaaaattggaaacattattgtacaacaacttagcagcatcatacattttttcatcataacaacggtcaccaacttgttggatatgagcattatttggtccattgataaattcttctaactctgcaaggcggtttgttttagccagtgcgaatatcagttctgtctccacataggactctcgagccttcttacgggccatctgcaagtacttcaccagttcttcccagtttccactagtattggcagcctgaacaacttccatgtaggaggaaggatcatctgctttgatataagaatcaatggcttctttcaccattcctttctgcaactgggcttttgcaagttgactccagaccgcaggttcattgcaacgttcagcaaactcatatgcccgatccaagtttccaatatgctcaattaagacctgaactgctgaagtattgacatcaaatttccggaaaatggcaaatgcttcttcaaacagctcattgctgatggcgatattggcaatatctggggcatcataattatccaggcggttaatatactccataacacgtgtacggtcagccttaattgcagtgaggataaggaggttttgcagattcctgtgttcactgaatacagagttatcaaggacaattttctccagcagttcaatgagttcattaggaaggtctgcagtcatgaaagcctttacagttactgacacttcttcagggtcctgagtctcagacaaagctgtttgtacaacctggtcaattaggggtctcctgtaaggattgctttccagcagcacgctgccccacaattctggatcctttcgacgtaccaggtagcgagaaagacttttgaagagggaattctcattgcaaacattaataagttccagatcacattggccacgttcataagcaacacaggccagatgtggatctctcttctcacaatactttccaacaacgcgactgtcatagtagggattttcacgaagaaatctctccgggttgttattactgtctatgtagattttggctaaggcattgtgagtagcaggctcctcacagccctcatgaattctggcctctagccaaggcagaagcagtttcaatctgtttcttttttcaacctcagcaacaagctcatcagtagagaattgacctcttacaacaagaatcaagttttttatgacatcttcagaacagtcaacatcaagtaatcctccaataactacaggaagtcgacttggattcaccttctgtacatatatctctatatacttttgaagattatttctatataaatagagcaccaaatcatggacaaagtcaaatcgatcacacacaatgataagtggtagctgatctgttagttttgcttccttaagaaaattcttgactcgctcaggatcgtagcagttgctttctctacagattctttctacttctttgatttgcccagtcttgcaagctgcctgaatatatttaaagtgcacatctgggtcctggctaaagttaacaatggatcccagaaaataaaagagaccttcaaaactcttgaaagattcaaaaagttcaatcagagactgagttgacagttgttcatgatatttagaagccacctgaacacaaatctgcagattctgacggatgttggcagacagcatggctctgagacattctagggagtcttctactgataaggaaccaaagtagttgactaaccactcagggttaagaagatgggtgtgaaccactgcacgttttatatcatataaatcagtgaaatgttctaatgcacgctgcagtaggccagccttttcacacagttgagcaatatgagcccggtcataatgtgtgaacatctgattgcctagaatagcatctgcaacttgaggcgcatgcataaggttcatctcaagtaaccgcgtctgtaaaggaccttcagatgggcgattattcttcagagcatcaagcaagaatgcagtacactgctgaattagattgtattccataaagacatctacaatctgtgtgatgtcagcaagaggctcttcatcttgaactaacatttgggcaaactgctgtccctgatctggactgattcgcattacatttctcagcagaaatatccaatctggagtgtatccaacttttttagcatataaaacaatcttttggacttgacctgtttctgcaaagcactgaatgactttatttgggacgttagcccttaggtacacactaagtgccaatgtagggtccacagatttcacaagatcacccagttcttcagaacattccagcttatcttcttttaaccatttctccaaaagctgttttcgcccttgctgaagtacaggcctacaaagctctaaggattcgtatttgttgagctgtccctggtccaaaaggataccaaagtactgaagtagaggagaagtttgacctggctgggctgggacactctggaaccgacggatagtgtctggagtacgaagaattccctttggtgcattagcagccacctttgctgcctccgagtaatttccctgggcaaaaagagcattaaatttccgggcaaagagttcttcagcaccggctaagttattacgtacagccattctcagagccaaatcaggattttgtagaacattggtgatgtaaggaattatgttttcttcttccacacacactgacagaacttgtccctttctgtttactccaattattccagctgtggcttcatgaggtgcagtaacaaaaattgtttctccactgattctattcatgtagatgcaggtaccagtctcaagatcatagaggtggatataaccatacttggttatcaagaacaccacatcatgcttttcactgatctgcattgcaacaggaaaatcattttgtgcttctggaggaaagaagacatccactgccttctttggaaagggctggttccctgtaggtggtgtgccaacttcaataatatgtaacttccctccagcttggccccgaactgcaaaacaaaataacgttgattcttctgcatttccttccatcttaaactgtgcaaagctagctgcatgtccttcaatgggctgagacactttcctatctacagaatatagctgcatagctcccaccacacgattttgctgtgcagatataccagtcagaagtaaccacttttgttttgcatctgtacggtaattgataatctggcaccctgcaaggctagaatggcgatcaaacattttcactggctgagactctccttccatactccagtgataaactgcattatccgtaacaagagcaaccgtattcaaagagatccatttccaaaaggtgacatcatcagtcatggtatgagccttcattttacttttcatttcaatgttaaaaatctgaagagttttcccagctttcagtgcaattactttgctagctggattcatgatggcgctgtctgctgaaattggtcttcgaattggattacttgggtcattcatatcaatgattaccacctgggcctgctctcctactttttctctaatgcagatgaatttgtcagactccatagtcagggtactgaagccaatgtttgctgggttgatacccaggttctggagctggagatgctcctgaaaacgaattggcagaatctgggccatggcgctgtcgggggttatggtctcctcctgtcactggggctgcggggcagtggctgcccgggctctccaagggagaggaggagaaggggaggggggaggctgggctcagcaggatcctctccggggacgcaggaaactggcaggcagacgaaagagctcgggtcgggggcggaggctccaggggccaggagagccgcaatggcggaaccgggcgcagcgcagactccggaaacggct

SEQ ID NO: 13209 - RNA, 1145 nt, Homo sapiens
  source 1..1145: mol_type = other RNA
gctgggattacaggcatgagccaccacacctggtgtcacatagacatttttatcctatgtagactgaatatatggaatcctgactttatagtaccactataatagcaacttaaataccactcaggaaaatctgaggatgcaatacaatatctctgattctagtttataatgaaaaaatgacagcctaggtgaagtgtattagacattgtaaatctcagacaaacccaggtgcagtacagagctccaggagtcccacgtgggaacctgggagtcctccatgagtggtgaaagttaggggaaatgctgagtactacaaaagcagccacaaactgttggaggaggaagcactccataggttcagctccctggctcaaccacacctcacatgccagtaccaagggtggccttcttagttcctctctcacccaaaatgtttcagtccagtctagcagagtctgcagatccagatatcttccaatgttccagtgtttccgatcaacatcttcatctgcatcccacttgcgagttaagaaagggtgttttttgctgattatttctccttcgaagaaggttgtaagggttggatactcctcagtaaggcctttaatcttcaagtacccacaaaggtaagagttccccgtgtccacgtgctgcagcaccacctctacgtcgtacgagttccccttgctcttctggtggccgcggaacttggagccgctgtagagcaggctggtggccacgccgggctgctgggtgttgatgggcggcggcgggatgagtgaggccgcggaggcagcggaggcaccggccggcgggggacactcggtgcggaccggcatcgcggggtcccccggagccagggctggggggagtgggagaggaaccgccgccgccgcgcgggagccgaggagggtggcggggagggagaggccggggcgcgcacgcgcggggtgggggcgggaggggcgaccacccgcccgctgcctgcggagcaagcgctccggccgccaccgggacccagggacctgcgagcagggcctcccagtcctgagctgggtccccctcccgacttgccctcgcgcacacatacacacacacagacactcacagacacacaacacacaaacacacacagacacacacac

SEQ ID NO: 13210 - RNA, 4863 nt, Homo sapiens
  source 1..4863: mol_type = other RNA
gctgggattacaggcatgagccaccacacctgtggtttttttattttattattttattatttttattttttaaaccatttatatttttattttttaaaccatttaaaacaaacagccttcagtggagaacgtgaggacacagcaattaaatgaaataaaattactgaaacaatttgataaagtttgatttttaaatttgatttgttactgaaaaggacactttttgttggttggttggttggttggttggtttttttttttttttttgagacagagtctcgctctgtcgcccaggctggagtgcagtggcgcgatctcagctcactgcaacctctgcctcccgggttcatgccatgctcctgcctcagcctctccgaatagctgggactacaggtgcccgccaccacgcccggctaatttatttgtatttttagtagagacggggtttcactgtggtctcaatctcctgacctcgtgatacacccgcctcagcctcccaaggtgctgggattacaagcctgagcgaccgcgcctggcctgaaaaggacactagtaaggaaactatgtaattcagtgtttctcatttgaaacattttgaactgattagtcttttgttattagaattgattatctacagtgttttgttgttacaattgaacattcctagagtttgcttgctttttgtaaattactccagatagcaatttaggaaactcctcattatttttgtttagggctaaaatgattctcctggagacagagcagttgtacttggggtacaaggaagagctgtgctgaacgtcagccagggaaccttctaagtcaccgctgtgggctgtgtcctgctgtttatttccttaggttggagcccaagtttcagcataggtcacctgttaacatctttctctttgataagtcatcaaagagacttgggctggaatatcctgccaccagggggaatgttcaaaagtacatctgctccagaggtcctccagtgttgacaggcacattgtagcaaattattgggttatacagttaacaaataccttttgtttggagctgtaagacccaattataaagcactagtagtttttgtctttttaatgcattaacaaacatatattgcatgtttatggtgtgttctgcattcactaggcagtggaagctggagctaactagagcacagttcctgtcttcagaggtcagtagcatactggaggagatggaaaagattgaatgaatcacagcctcatggggtacttgagggatgatatgactatttctctgcatagcatatctccattagagcactagtccactgtgtaacaataaccttgcatacatgcctgccacttctaactagtgagtccttcctgggcatgaagcacgtatcattcctctgtgtactgcagagttgtagacactgtgcttgacacatagattttagtaaatgtttatgggtggaactaatgagagaactagaagagggagtgaattgaatgttcttgagttaatgggaaggagttaatgaaggcctcacagaggggcaaatgagctggatcttgtaggatctgtaggagtttaccaggtagagaagagtgactccaccagcaaggtgtttgggatttctatagttaattgttaagaatttattcctgttccccagatccttatgactaatgccaacactaaacataaaacaggatgttactctttctacaatgagctttggtgtttttgtttttgaaaaatattttcggtatatggtttttgtttctgataggaattctcctttaggctattgtcaatttgttttcctgtaatgatttgaaacaattatattaacttaaaatgatgtcacaatgagtgaaataatgaaaaaaagttatagttattgagggtagtctcatgatgagataaagtgcatacagctgcactcatgtcgccaggtgattaagaacagaattggtattaaggtcaacggattagcaaaaagggaggagattattgtcttttcattattttgaaagaagtaccatctgcccttgattgttttggtttaggttttattcagcccaaattagaatccgctgtggtgttgattgttccttgttggtgatagccctagaactgtgtttcccatcgttgatacttgcattcacgtttgctagttctctcttctcctgtgaagacatgaacgtagctgctcctttaattacatttagctagttttaattcagagatggctattggccctttgttttcttaccatcttttattgtgttcattttcctagttgatttttaatggtgacatcactaacagctctaaagactcaaagcttaccagacagcacgcttccctgggtcagaagatgagagtcctctcctctctcattcagtaccagggtgtaccagtgagaggcttgtgaagggattgtttcggcgactccttatctaagaaatgaagataatttttatgaggtgcattttggtctgtgggagtggaagggaaaatgacggtttctttcctatactgtcctttgtttggaatggtgaaaatgttttgaatctgtttctggtgtgatcgttaggtccaagatttcacgtgacgttgtgtgccgggtgttgtggtcaacacacaggaatgctcctttattctctgtacggcctttgggtgcatcatttgagtggatgttcatttgcttgagacgattgtcagagggaatcttgtgtgccctttgctctctgtgcctgtcattgcgagggtttctttgagccggtctgctgaccgtcaggcacttgagattgactcggtgaacaatgccgccagcctttctgatgcggctcctgccctctctgactcctacacaggatcagaatcactcagatatcacttctgttggtggaggcgagagaagaatatttatccagtttctgcctttctgcccccattagctctttaccaaaaaaaaaaaaaaaaaaaaaaaaaaaaaaaaaaaaaaaaaaaaaaaaaaagcaaaaccagttattctgtgaaaatatgcaaagcagagttttggccttgaggatgcgtatttgtgacttgctttcctgtacagtaagtgctgccgcctcaggagcgggcgcagtcgcttatggtgccggtgagcctgcgcggcgctggcttttgctcctctggtgccaatgcagctcgttgacagctccaagatatttggatatctcactcttccggctatttcagctgccaaactagaatcccaaccttctgagagtctgttctcttttggatttgttcatagatgtctattctctcctgatctggttcatgaacactctggaagccaagttcattgaagacactctggatgtgtaatttggaagaggagactggagcatggaggctttgttcctggtgccatgctagagcgggagaggagtgactgcaaacctaggcctctgtcctgtcacctttcctccagctggtgaaccaccttgtctactcccttgccccaacacagccgacaggtggacagccagacacatgcagagccattgttttttcaaagacctcttttctgaactatagatgggaagctgctgcaaaaaagcaaggtgcagcccctttcttgtatgagggaagctactgtttaccatccatggctgcttgagtttttagagctgcgtcagatgaataacttgttggtatcactcgtcaatcttagaggcactttcagagattaggaattgtgaccaacaggagagactatctggcattaggaacaccagggcctattttggatcatgctgtactgcttacggtcatgccctgtccaatctgggatgactgtggcatacaagtcaccatggccattgtgaagcccttgttcttggagaccctgtgctccaggtgtggctggttggttccctgtggcaggacccccagaggccccaggggttgtgagagtcaggggtgtgcaggttctgagggctttgctgggtgggccgaggttgagtgggctggttgcagaatcctggtgcccagagggttcttctttgcctgttgctggggactcacgccttgtgaggggacctttctttattaccctgatgaggacagaagagttcctgagaggaagccacaagccgcctccctgacctggcagctgcctgtgtgccctggtgtgtgggttcctcccttcctgggttcatgcagcagactcttggcagtgcaggcctccttccaggggctctcagggctcagttctcatctctctgggtcacactgagccctgctgatccccctcctgtgtggctgcctctctgatgcctgaaacaccttcagctgttagtcccacggcctctcatcacctcgatatccttttctgcttgctttctggttttcagtggctgccagcagaggctgtaatgctcccctgggacctgaccagtagagaacaaatgctatgaagaccagaggcccctcactgctccacgcgtatacagggtgcgtctgtctggacagccgaaggcccatgggtggttttgttttcaaaacacaatgaaaaatgactagtcatgccatattgttagcacctttcgattttttttactgtaaaaatcaaaacagaaatatttggctccagagctctgtgaaccccgaaaatttgagacgggtctcagttaatcttgaaagtttactttgccaaggttgaggatgtgcgctcattaacacagcctcaggagatctaacaacatgtgcccgaggtggcctgagcacagcttggtacgttttagggagacatgagacaccaatcaatacatgtaaaataaacattggttaggtccagaaaggcaggaccac

SEQ ID NO: 13211 - RNA, 533 nt, Homo sapiens
  source 1..533: mol_type = other RNA
gctgggattacaggcatgagccaccacaccttctgcagcgcccattccttcacccacaatatgccctgaactccctgtatgactctgccccttccctcctttccatgagaagtcagatgtgtcaacctgaagaatccccagatgcccaggcagtgctgaatggtcaccaccaccacgttttcatgggctgcgagtacccgcccatcagaggttgatgcggtgcccaccatcagcccccctctgtggatccacaccatcaccagcagcctgtttttcttggtcaagtcagcaggagtgtaaatattgaggtaaagacagtcttcagaaagcttgaaaggaatgttctcctttcggttggtcaatagttctgagagaaactgccctaccttgggatcttgggtgcacctgcggagggggaaagaagaaccccagaaggcaggcctcatggcccccactaggtacatgaggaaactgaggcactcaggctctgggatgacacagatgaaagcagggccagccttgatcaccgtcat

SEQ ID NO: 13212 - RNA, 1323 nt, Homo sapiens
  source 1..1323: mol_type = other RNA
gctgggattacaggcatgagccaccacacgcagccacctgagactttttaaacagcaccagcacttctggctggtttgaaccttaaatgccaccacccaccagagaggaggctctcactagattctaaatctgttatttaattacttttcaattgaaaaacaaaacagacagaagaaacttattagaataaggccacctaggaatgttcttaacttttccattcagcttttggctgatatatgaaaatacaaataaatacatcctttccccaggtgcaaggctaaaccagcagctccaagggcttggtctacagtgctcagaaagacacactgccttaaaagtcaggctagtgccctagctccggtggcctctgcaaatgaggccttgacagtcgtcagtggacagacacatagtatccagcaccaggtcttgggccttcctgcttcccagagtttcacaggtaggacgcatgtgaggggagcagtccgtacttctgttggaggatggctgtagtactttccagggcacagcctggacgaatgatgccaaactttccgggcacagacaaatcaaccacagttgagccaaggcgacactcggggctctggccatccccaatttgtcccccatcaataaccaaggacaactgaggccagagatcctggaactcctcgacattcagagaactggcctgggagctgaggttggcactagtgagagcaagcggaccctcaaacatctgagccaagtcttgcataaaagcatgatcaggaatccgaatgcctacaagaggcgtaaaagggtttaggtccttgttgagctcctccgagcgttccatcaccagggtcactggtcctggcagtaggtctttcaggagcccctcaggtactctcacacggcagtatctgtagacgtcggccacgcggccgaggcatacggccagaggcttggcctcgctgcgacccttgaggcggtacacagcgcgcagagccgccgagcagctcgccgcgcaggccaggccgtacagcgtatcggtggggacggccaccacggcgccggcgcgcagctcggccacggcggcccgcagcgcctcggtccagccggcgcgctccgggctcgcggcctgcacggccccgctccccgggagccgcaacagccgggcgccgggggccgccggagcgggactcggcgggcggaagaggcgaccgctccgggagccagcaggcccctcgctcaaccccacgctggcagccaccgcggccctcatccccctgcaccgacgcgccggagacatccgcccaggcccgcttccgggaggaagt

SEQ ID NO: 13213 - RNA, 3235 nt, Homo sapiens
  source 1..3235: mol_type = other RNA
gctgggattacaggcatgagccaccacacgcagctggaacaagtatacttttaatgtaattacaatgcttccaaaaatctgcttttaaagttatacacaaataaatttttttttttcctggagacagagtttcactcttattgcccaggctggagtgcaatgatctcgactcaccacaacctctgcctccagggttcaagcctcctgagtagctgggattacaggcatgtgccaccatgcatggctaattttatattttcagtagagactgggtttctccgttttggtcagtctgatctcaaactcccgacatcaggtgatcctcccaccttggcctcccaaagtgctgggattacaggcatgagccactgtgcccagccacaaataatttatctaagaagtgtttccaaactcattacatttgcaggaatcttcttcaatatacattccctgatgttgcacaaagtttggcaaccgctttagggtttccttctaatacaaaacgcgggcaataagatctgtaatacaagcaaaggtactacaaacctctttatatttgtaatgcttgtcttcagaatcaatactcttcttcaccttaaaggcttatattttctgaaagatttttgtcacagtaattgctcttttatgaaccttcttctgttgagtaagatgtgatggacattaatggcttttccatattctttatatttgtacaatttttctcaaggataatagctttcctgtgaaatacggtgtaagcactgattaaaagttttgccacattcttcatacttgtaggtattttggaagtatgaattacctacaataaagtgtggcaaccatataaaggctttgtcacatttcatacatttctatggtgtagtataattttttttatgcatagaaaagttggaggtgttgggaaaagcactgtcacatctttcaggtttgtaaagttcctcttcaccatgaattatcgccatgtctcttaagaattaagagcttatggctgggaattgaggctcatgcctgtcatcccagcactttaggaagccgaggcgagtggatcacctgaggtcaggagtttgagaccagcctggcaaatatggcaaaagcccatctctactaaaaatacaaaaattagctgggaatggtggtggcacctgtaatcccagctacttgggaggctgaggcaggagaatggcttgaacccaggaggcagaggtcacagtaagccaagatcatgccattgcactacagcccgggtcacaagagtgaaactgcatctcaaaaaataaataaacaaataaaaataaaagaattgagaacttgttacaggcttgccacattcttcacacttgtagggtttctgtccagtatgaattatgtgtaataagggttgagaacttccttaaaaagctttgtcagccaggcacagtggctcatgcctgtaaccccaacactttgggaggccaaagcaggcagaccacctgaggttaggagattgagaccagcctgaccaacatggagaaaccccatctctactaaaaatacaaaattagccaggtgtggtggtgcagccctgtaatcctagctactaaggagagttacttgaacccagaaggtggaggttgtggtgagccaaaattatgccattgcactccagcctgggaaacaacagcagaattacctctcaaaaaaataataataataaaataatcctttgtcacgttcttggtttctgtccaatatgaattctcttatgtttattaaggtctgaggaccagttaaaagctttgccacattctttacatttgtaaggtttctctccagtatgagttgtcttatgttcagttagatttgaggatgtagtatacgctttgccacattcttcacatttgtagggtttctctccagtatgagttctcctatgtttatggaggcctgcagaccatgtaaaggctttgccacattcttcacatttgtatggtttctctccagtatgaattatcttatgcatagtaaggtgtgaggagcgggtgaaggctttgccacattcttcacatttgtagggtttctctcccgtatgaatcttctcatgtttactaaggatcgaggatgaaataaaggctttgccacatttatcacacgtgtacggtttctctccagtatgaattttcttatgtgaagaaagagttgcaggatggttaaaagctttgtcacattctttacatttgtagggttgctctccagtatggattatcttatgtgtagtaagggtataggggtacataaaggctttgccacattcttcacaaatgtagggtttctctccactatgaattttcttatgtgtagtaaagctagagaagtacttaaagactttgccacattcttcacatttgtagggtttctctctagtatgagttatcttatgtgtagtaaggtgtgaggaccggttgaaggctttgccacattcttcacatttgtatggtttctctccagtatcaatttttttatgtgtagtatgggttgaggactggttaaaagctttgtcaccttctatatatttcaaaggttttttttcagtatgtcttcttttatgtctctttgaatttgaaaattgatgaaagactttcacatatttaccacattgaaatattttgctctgggtagttgtcaaacattggttaagtccattataacctcttttgtgtaacttacactcatccacactttcacagccttttttaaagtgtaaattgccatgtccacatttttcaaattttctcagtatcactttttggtaagaatcttttatgctctgctctggccaaaggtcttgggcaaaatgagaacacacaactgggggtttggcaatcatctcatgtctcttcatagtcagaggttttattccttgctccagacaggtgatcaggtctggcttagagacaataataccaaggaagaccaggtgtctgtagttctctaacatcacatccctatataaattctgctgtgcagtgtccaggcaatgccactcctccagagagaattctacagccacatctctaaattgcaatgattccatttctaggcttctaaggggtcccggcatcttggctgtggatctcccaatacctacaggacacagggccacagagggtgggcctctaggagcagaggacacagagtagcgaagaggcgacctagagctccagatgcagcgagagac

SEQ ID NO: 13214 - RNA, 3549 nt, Homo sapiens
  source 1..3549: mol_type = other RNA
gctgggattacaggcatgagccaccacacgccaccttcacctctccttcttgcatccctctaaccaaaggagtgctcctagagaaatcaagtttattttctaaacaccagtgaaagcaaaatccagtaggaaataccttgcttcagcgtggcatatcttaagtggaccaaaaggggtggtaggataatttttttacaaatttgctttaaattctactttgaaatttagaatttgatttttttcccctccatttgcagaatttaacaccatttaacacgaacccaaggcaggttgagagcggagatgtaaacattttcaacagtagcgtggactttacggctttctacatccccatgtgggttgaggctgcaactggttttggggagtggggggcagagcagggagaaggcgttaactgccagatgggacagggcagcagccaagccccacagcccagctgcaaagggctgttcacggggcacacgtgggaggtacccagtttggctctttcccatccctgatctgaaaaaggaactccactgactgataaaattcttcatcgctattagggcaaaatctactccccaaggcactgtgtgcatggtcccaagatggaaattctccacgtgttacttcctaggcagtagcaccactcaaaagaatccaggcctgcgcctcctcggtaagatgcaccacgctgaccgtgatgggtggcggcaggtcaggacccggctcactgaaatgcaaacatacatgagcttcctgctcatttttaaagacaagctccggtgagggctccaaatcagagacagtgcagctcgtctcgtcggtattcccttgcacggcagcctggcagagcaccaaatggcacagctagggaaaacgggcttgtattttctctgagcggcaatctgactcggcacacaccatttcagaaagcgaggctgcgaagcctgtgttctcgggtgacgcagagcagacaaggatgcagaatggcttctggagaggggtcttccgactcgggcatgagggtccaggtcagacctcagccgcagggccctagcagataggcctggctcttgtcacatgcagtgagaagctgtgacatgagaattaatggttgggacaagacagggacaaagactggagacatgcttccctagactgcacagggaaacacaggagatgagattcagtcaaaacacacatagatcacgttacctgaagtgcctgagttaaaaggctgatgcagaaataagtcctaggatgaaggtaggatttatcccaaacacctgccccacaagtcgccaaatgctgcctatcaagggcttctaagtgctgaccggggaaggcaggcattcacatcactcacaaccagggaaggaagcagtctcagcaggtttatgcccagtcaccccaattctactgggctccaccaccctccagcgggcgagatcctgccacccagcatgtgtgcgtgtgtgtacacagcaagagaaaataggccagggccagatctctggtcctggaattttggggaaagacaaaggaaaaaggcacatgaaggtggctgattgaatttaaaagaaaaaaaaaggtagctgcaagtgacatatcattattttgatttttttaacgtaccttttttcccccatgaaaagagaaattcaaaatataaactttattattttacattcaagtgaaacttccatctggaggggctaaacacagctgccggccacattcactgatttattactttgttgcctttttcgttcacctgatggaagaattcaaccctcttaaaaacataacaacaacaaaaacagctggagagtcccagccgtaatactaggtgtagacacgcacaagcacacacacaaattcaaaaacttctacatagaaaaataaaggataaacattatccatctattttgtactgtgtaatgcaacttttatatacataaatttttttttttttttttttttttttttttttttttttttttttttactgttttcagtcactgcaaattttcttccctcctctgggatctaaggatccagggaggaggctgccacagtgaagcagaaaagctacattctgcccagggaggaagagaaaaagcaatttctcgctccccttcccaagtccttcctgtccaccaccacctcggatgtccccgcacacagccttccggtgagcggccgtgccgtcccctcctctctctaaggcattggggagcagagggcccataggcagcaccctgcaaaaaaaaaatgatctacgtgtgaggagagggcaaggggctggatgcaggcagagaatgactttaagaaaagattctatgatcccttcctttagtatggagctcgattttccagctggcgcttggtgagaaagtacttgaagaactcatagacagaccaagaaatggcggtggagggcatctggtagatgacacgcgcctggatgcctttgaagtagccggccaggccgttgagctggtacaccgtccggaaggcattggccatacccgacagccggccgctgatgttggccagcgagagggccacgttctcctgagtgttcagaagggtcttacagacgtccaggggggtcgtggcggccgcggcgagggccccggccagcccgcctgagatgatgtgggactgcgggttgtaggtccggtgggggttgacctgctcctgcaggaactcataggtgatgaagtggatggactggaaggggatgttcatggtcagctgcgtggtgtagctccggtagaaggcccccaacccctcggtcctccacaccgtccggatgcagctgattgctgaccggtgctgcgagttgtacatctgcaagcgctgcttcaccacttctgctggattcattaccgcatcgtggagcagggtggccatactcccagctatcccgttggctaggtggctgtttccttggtggtggaaaacgtcatttaaagtccttttcatgttttcatagcaggcaaaatacatggcatgggccggccctgcacccatgatcatgacgttgacgcctcgcaagggcctccagaagccttcggtccgcatgattttcttgagggctccgtagatacttgtgtactgggctttgggatctggactcaaactctgcattcgtgtctgtaatcccagctactcaggaggctgaggagggaggattccttgtacccaggagttcgaggctgcagtaaactatgatctcaacactgcactccagcctaggcgacaaggcaagaccctgtctcttcaccgagtccaccgggtacatgaccgagtgctccaggatcccggccatcgctcctgctgtcatgtgggtggacacggaggcgctagtcggcaggttctcgtagtcctccgacccggtggcgtccttgccgccgccgccatctcggctgtccccatccatcctccgcgccaccgcctggctgcccacgctcccgctgcgcagctccatccgccagctcggcggggcgcaggaggctgcaggaggtgggcagggag

SEQ ID NO: 13215 - RNA, 3425 nt, Homo sapiens
  source 1..3425: mol_type = other RNA
gctgggattacaggcatgagccaccacacgccaccttcacctctccttcttgcatccctctaaccaaaggagtgctcctagagaaatcaagtttattttctaaacaccagtgaaagcaaaatccagtaggaaataccttgcttcagcgtggcatatcttaagtggaccaaaaggggtggtaggataatttttttacaaatttgctttaaattctactttgaaatttagaatttgatttttttcccctccatttgcagaatttaacaccatttaacacgaacccaaggcaggttgagagcggagatgtaaacattttcaacagtagcgtggactttacggctttctacatccccatgtgggttgaggctgcaactggttttggggagtggggggcagagcagggagaaggcgttaactgccagatgggacagggcagcagccaagccccacagcccagctgcaaagggctgttcacggggcacacgtgggaggtacccagtttggctctttcccatccctgatctgaaaaaggaactccactgactgataaaattcttcatcgctattagggcaaaatctactccccaaggcactgtgtgcatggtcccaagatggaaattctccacgtgttacttcctaggcagtagcaccactcaaaagaatccaggcctgcgcctcctcggtaagatgcaccacgctgaccgtgatgggtggcggcaggtcaggacccggctcactgaaatgcaaacatacatgagcttcctgctcatttttaaagacaagctccggtgagggctccaaatcagagacagtgcagctcgtctcgtcggtattcccttgcacggcagcctggcagagcaccaaatggcacagctagggaaaacgggcttgtattttctctgagcggcaatctgactcggcacacaccatttcagaaagcgaggctgcgaagcctgtgttctcgggtgacgcagagcagacaaggatgcagaatggcttctggagaggggtcttccgactcgggcatgagggtccaggtcagacctcagccgcagggccctagcagataggcctggctcttgtcacatgcagtgagaagctgtgacatgagaattaatggttgggacaagacagggacaaagactggagacatgcttccctagactgcacagggaaacacaggagatgagattcagtcaaaacacacatagatcacgttacctgaagtgcctgagttaaaaggctgatgcagaaataagtcctaggatgaaggtaggatttatcccaaacacctgccccacaagtcgccaaatgctgcctatcaagggcttctaagtgctgaccggggaaggcaggcattcacatcactcacaaccagggaaggaagcagtctcagcaggtttatgcccagtcaccccaattctactgggctccaccaccctccagcgggcgagatcctgccacccagcatgtgtgcgtgtgtgtacacagcaagagaaaataggccagggccagatctctggtcctggaattttggggaaagacaaaggaaaaaggcacatgaaggtggctgattgaatttaaaagaaaaaaaaaggtagctgcaagtgacatatcattattttgatttttttaacgtaccttttttcccccatgaaaagagaaattcaaaatataaactttattattttacattcaagtgaaacttccatctggaggggctaaacacagctgccggccacattcactgatttattactttgttgcctttttcgttcacctgatggaagaattcaaccctcttaaaaacataacaacaacaaaaacagctggagagtcccagccgtaatactaggtgtagacacgcacaagcacacacacaaattcaaaaacttctacatagaaaaataaaggataaacattatccatctattttgtactgtgtaatgcaacttttatatacataaatttttttttttttttttttttttttttttttttttttttttttttactgttttcagtcactgcaaattttcttccctcctctgggatctaaggatccagggaggaggctgccacagtgaagcagaaaagctacattctgcccagggaggaagagaaaaagcaatttctcgctccccttcccaagtccttcctgtccaccaccacctcggatgtccccgcacacagccttccggtgagcggccgtgccgtcccctcctctctctaaggcattggggagcagagggcccataggcagcaccctgcaaaaaaaaaatgatctacgtgtgaggagagggcaaggggctggatgcaggcagagaatgactttaagaaaagattctatgatcccttcctttagtatggagctcgattttccagctggcgcttggtgagaaagtacttgaagaactcatagacagaccaagaaatggcggtggagggcatctggtagatgacacgcgcctggatgcctttgaagtagccggccaggccgttgagctggtacaccgtccggaaggcattggccatacccgacagccggccgctgatgttggccagcgagagggccacgttctcctgagtgttcagaagggtcttacagacgtccaggggggtcgtggcggccgcggcgagggccccggccagcccgcctgagatgatgtgggactgcgggttgtaggtccggtgggggttgacctgctcctgcaggaactcataggtgatgaagtggatggactggaaggggatgttcatggtcagctgcgtggtgtagctccggtagaaggcccccaacccctcggtcctccacaccgtccggatgcagctgattgctgaccggtgctgcgagttgtacatctgcaagcgctgcttcaccacttctgctggattcattaccgcatcgtggagcagggtggccatactcccagctatcccgttggctaggtggctgtttccttggtggtggaaaacgtcatttaaagtccttttcatgttttcatagcaggcaaaatacatggcatgggccggccctgcacccatgatcatgacgttgacgcctcgcaagggcctccagaagccttcggtccgcatgattttcttgagggctccgtagatacttgtgtactgggctttgggatctggactcaaactctgcattcgtgtcttcaccgagtccaccgggtacatgaccgagtgctccaggatcccggccatcgctcctgctgtcatgtgggtggacacggaggcgctagtcggcaggttctcgtagtcctccgacccggtggcgtccttgccgccgccgccatctcggctgtccccatccatcctccgcgccaccgcctggctgcccacgctcccgctgcgcagctccatccgccagctcggcggggcgcaggaggctgcaggaggtgggcagggag

SEQ ID NO: 13216 - RNA, 3496 nt, Homo sapiens
  source 1..3496: mol_type = other RNA
gctgggattacaggcatgagccaccacacgccaccttcacctctccttcttgcatccctctaaccaaaggagtgctcctagagaaatcaagtttattttctaaacaccagtgaaagcaaaatccagtaggaaataccttgcttcagcgtggcatatcttaagtggaccaaaaggggtggtaggataatttttttacaaatttgctttaaattctactttgaaatttagaatttgatttttttcccctccatttgcagaatttaacaccatttaacacgaacccaaggcaggttgagagcggagatgtaaacattttcaacagtagcgtggactttacggctttctacatccccatgtgggttgaggctgcaactggttttggggagtggggggcagagcagggagaaggcgttaactgccagatgggacagggcagcagccaagccccacagcccagctgcaaagggctgttcacggggcacacgtgggaggtacccagtttggctctttcccatccctgatctgaaaaaggaactccactgactgataaaattcttcatcgctattagggcaaaatctactccccaaggcactgtgtgcatggtcccaagatggaaattctccacgtgttacttcctaggcagtagcaccactcaaaagaatccaggcctgcgcctcctcggtaagatgcaccacgctgaccgtgatgggtggcggcaggtcaggacccggctcactgaaatgcaaacatacatgagcttcctgctcatttttaaagacaagctccggtgagggctccaaatcagagacagtgcagctcgtctcgtcggtattcccttgcacggcagcctggcagagcaccaaatggcacagctagggaaaacgggcttgtattttctctgagcggcaatctgactcggcacacaccatttcagaaagcgaggctgcgaagcctgtgttctcgggtgacgcagagcagacaaggatgcagaatggcttctggagaggggtcttccgactcgggcatgagggtccaggtcagacctcagccgcagggccctagcagataggcctggctcttgtcacatgcagtgagaagctgtgacatgagaattaatggttgggacaagacagggacaaagactggagacatgcttccctagactgcacagggaaacacaggagatgagattcagtcaaaacacacatagatcacgttacctgaagtgcctgagttaaaaggctgatgcagaaataagtcctaggatgaaggtaggatttatcccaaacacctgccccacaagtcgccaaatgctgcctatcaagggcttctaagtgctgaccggggaaggcaggcattcacatcactcacaaccagggaaggaagcagtctcagcaggtttatgcccagtcaccccaattctactgggctccaccaccctccagcgggcgagatcctgccacccagcatgtgtgcgtgtgtgtacacagcaagagaaaataggccagggccagatctctggtcctggaattttggggaaagacaaaggaaaaaggcacatgaaggtggctgattgaatttaaaagaaaaaaaaaggtagctgcaagtgacatatcattattttgatttttttaacgtaccttttttcccccatgaaaagagaaattcaaaatataaactttattattttacattcaagtgaaacttccatctggaggggctaaacacagctgccggccacattcactgatttattactttgttgcctttttcgttcacctgatggaagaattcaaccctcttaaaaacataacaacaacaaaaacagctggagagtcccagccgtaatactaggtgtagacacgcacaagcacacacacaaattcaaaaacttctacatagaaaaataaaggataaacattatccatctattttgtactgtgtaatgcaacttttatatacataaatttttttttttttttttttttttttttttttttttttttttttttactgttttcagtcactgcaaattttcttccctcctctgggatctaaggatccagggaggaggctgccacagtgaagcagaaaagctacattctgcccagggaggaagagaaaaagcaatttctcgctccccttcccaagtccttcctgtccaccaccacctcggatgtccccgcacacagccttccggtgagcggccgtgccgtcccctcctctctctaaggcattggggagcagagggcccataggcagcaccctgcaaaaaaaaaatgatctacgtgtgaggagagggcaaggggctggatgcaggcagagaatgactttaagaaaagattctatgatcccttcctttagtatggagctcgattttccagctggcgcttggtgagaaagtacttgaagaactcatagacagaccaagaaatggcggtggagggcatctggtagatgacacgcgcctggatgcctttgaagtagccggccaggccgttgagctggtacaccgtccggaaggcattggccatacccgacagccggccgctgatgttggccagcgagagggccacgttctcctgagtgttcagaagggtcttacagacgtccaggggggtcgtggcggccgcggcgagggccccggccagcccgcctgagatgatgtgggactgcgggttgtaggtccggtgggggttgacctgctcctgcaggaactcataggtgatgaagtggatggactggaaggggatgttcatggtcagctgcgtggtgtagctccggtagaaggcccccaacccctcggtcctccacaccgtccggatgcagctgattgctgaccggtgctgcgagttgtacatctgcaagcgctgcttcaccacttctgctggattcattaccgcatcgtggagcagggtggccatactcccagctatcccgttggctaggtggctgtttccttggtggtggaaaacgtcatttaaagtccttttcatgttttcatagcaggcaaaatacatggcatgggccggccctgcacccatgatcatgacgttgacgcctcgcaagggcctccagaagccttcggtccgcatgattttcttgagggctccgtagatacttgtgtactgggctttgggatctggactcaaactctgcattcgtgtttttaacttgggcagtctgggatctcaaggaagaggagacatccaggtccctgaaccaaggcagtaagtagcttcaccgagtccaccgggtacatgaccgagtgctccaggatcccggccatcgctcctgctgtcatgtgggtggacacggaggcgctagtcggcaggttctcgtagtcctccgacccggtggcgtccttgccgccgccgccatctcggctgtccccatccatcctccgcgccaccgcctggctgcccacgctcccgctgcgcagctccatccgccagctcggcggggcgcaggaggctgcaggaggtgggcagggag

SEQ ID NO: 13217 - RNA, 3902 nt, Homo sapiens
  source 1..3902: mol_type = other RNA
gctgggattacaggcatgagccaccacacgccaccttcacctctccttcttgcatccctctaaccaaaggagtgctcctagagaaatcaagtttattttctaaacaccagtgaaagcaaaatccagtaggaaataccttgcttcagcgtggcatatcttaagtggaccaaaaggggtggtaggataatttttttacaaatttgctttaaattctactttgaaatttagaatttgatttttttcccctccatttgcagaatttaacaccatttaacacgaacccaaggcaggttgagagcggagatgtaaacattttcaacagtagcgtggactttacggctttctacatccccatgtgggttgaggctgcaactggttttggggagtggggggcagagcagggagaaggcgttaactgccagatgggacagggcagcagccaagccccacagcccagctgcaaagggctgttcacggggcacacgtgggaggtacccagtttggctctttcccatccctgatctgaaaaaggaactccactgactgataaaattcttcatcgctattagggcaaaatctactccccaaggcactgtgtgcatggtcccaagatggaaattctccacgtgttacttcctaggcagtagcaccactcaaaagaatccaggcctgcgcctcctcggtaagatgcaccacgctgaccgtgatgggtggcggcaggtcaggacccggctcactgaaatgcaaacatacatgagcttcctgctcatttttaaagacaagctccggtgagggctccaaatcagagacagtgcagctcgtctcgtcggtattcccttgcacggcagcctggcagagcaccaaatggcacagctagggaaaacgggcttgtattttctctgagcggcaatctgactcggcacacaccatttcagaaagcgaggctgcgaagcctgtgttctcgggtgacgcagagcagacaaggatgcagaatggcttctggagaggggtcttccgactcgggcatgagggtccaggtcagacctcagccgcagggccctagcagataggcctggctcttgtcacatgcagtgagaagctgtgacatgagaattaatggttgggacaagacagggacaaagactggagacatgcttccctagactgcacagggaaacacaggagatgagattcagtcaaaacacacatagatcacgttacctgaagtgcctgagttaaaaggctgatgcagaaataagtcctaggatgaaggtaggatttatcccaaacacctgccccacaagtcgccaaatgctgcctatcaagggcttctaagtgctgaccggggaaggcaggcattcacatcactcacaaccagggaaggaagcagtctcagcaggtttatgcccagtcaccccaattctactgggctccaccaccctccagcgggcgagatcctgccacccagcatgtgtgcgtgtgtgtacacagcaagagaaaataggccagggccagatctctggtcctggaattttggggaaagacaaaggaaaaaggcacatgaaggtggctgattgaatttaaaagaaaaaaaaaggtagctgcaagtgacatatcattattttgatttttttaacgtaccttttttcccccatgaaaagagaaattcaaaatataaactttattattttacattcaagtgaaacttccatctggaggggctaaacacagctgccggccacattcactgatttattactttgttgcctttttcgttcacctgatggaagaattcaaccctcttaaaaacataacaacaacaaaaacagctggagagtcccagccgtaatactaggtgtagacacgcacaagcacacacacaaattcaaaaacttctacatagaaaaataaaggataaacattatccatctattttgtactgtgtaatgcaacttttatatacataaatttttttttttttttttttttttttttttttttttttttttttttactgttttcagtcactgcaaattttcttccctcctctgggatctaaggatccagggaggaggctgccacagtgaagcagaaaagctacattctgcccagggaggaagagaaaaagcaatttctcgctccccttcccaagtccttcctgtccaccaccacctcggatgtccccgcacacagccttccggtgagcggccgtgccgtcccctcctctctctaaggcattggggagcagagggcccataggcagcaccctgcaaaaaaaaaatgatctacgtgtgaggagagggcaaggggctggatgcaggcagagaatgactttaagaaaagattctatgatcccttcctttagtatggagctcgattttccagctggcgcttggtgagaaagtacttgaagaactcatagacagaccaagaaatggcggtggagggcatctggtagatgacacgcgcctggatgcctttgaagtagccggccaggccgttgagctggtacaccgtccggaaggcattggccatacccgacagccggccgctgatgttggccagcgagagggccacgttctcctgagtgttcagaagggtcttacagacgtccaggggggtcgtggcggccgcggcgagggccccggccagcccgcctgagatgatgtgggactgcgggttgtaggtccggtgggggttgacctgctcctgcaggaactcataggtgatgaagtggatggactggaaggggatgttcatggtcagctgcgtggtgtagctccggtagaaggcccccaacccctcggtcctccacaccgtccggatgcagctgattgctgaccggtgctgcgagttgtacatctgcaagcgctgcttcaccacttctgctggattcattaccgcatcgtggagcagggtggccatactcccagctatcccttttaaagcttagttagatcttggcgttgtagagacctgttgtaccagtttttaaatagtctcaaagaagctgtccagataacttttttttttttttgaatccagcattcaaaagttttgtttctattcagggtttctcctatgtctgatcattaattgcttttgaatgtttaaaaacaaaacaaacaaaaaaaaatacaaaagaaaacccacataacaataaaaccaaaacacctctgtcactgatttctccccaggcttcagaaagcggaggggaacagaaaaaagcatgtgtgtgcgcgcgcgtgtgtgtgcgtgcgtgtgtctgggtgtgcattgcacacacaactctgagttctttattcgtgagcaagcgggccgaagtcgaggcggctgggtcacagggaggaacaccctggggagggacgtgttgaagaagagaactttctaactccagacaaacgctttcaaaataccgttggctaggtggctgtttccttggtggtggaaaacgtcatttaaagtccttttcatgttttcatagcaggcaaaatacatggcatgggccggccctgcacccatgatcatgacgttgacgcctcgcaagggcctccagaagccttcggtccgcatgattttcttgagggctccgtagatacttgtgtactgggctttgggatctggactcaaactctgcattcgtgtcttcaccgagtccaccgggtacatgaccgagtgctccaggatcccggccatcgctcctgctgtcatgtgggtggacacggaggcgctagtcggcaggttctcgtagtcctccgacccggtggcgtccttgccgccgccgccatctcggctgtccccatccatcctccgcgccaccgcctggctgcccacgctcccgctgcgcagctccatccgccagctcggcggggcgcaggaggctgcaggaggtgggcagggag

SEQ ID NO: 13218 - RNA, 1368 nt, Homo sapiens
  source 1..1368: mol_type = other RNA
gctgggattacaggcatgagccaccacactcagcccaatgccaaatgtatccaatagtctttgattccagaattacttatgatagaacactgcatcatctacagaaatcttgatcaataacctagataacctagtttctaggttattgatcaagatttctgtagatgatgtagtatgtacatttctgtgtatgttattaatcaagatttctgtataagatctagaaacaaaaatgcacattaagaaattaaaacttacatctcataaccaattatctttctaaacaatttacaaacataaaatatacaatattatttaaaataaatatacatataatatatagtttctacattctcatacaggcttaaaaatgaggtaataaaaactgattaaaccttttaccattctggaaatggcttagggaaatgatcatgaaatatttttttcttaggtcttcattttttccttcaatacttctaagtacctctttttctatgctgaaaagttatgtaaaaaatccctaagctttgttggatagtctgtcatcaccccagttgctcccaaatcaaaagctcttttgtattcttgttcttcatttaatacccaaatatacacttgaatgcctcgagcagttaggtggtcaaacaaagctttcctcattagtaagagatcagaaagccagatgagaaacttttgacttctggacatggtgtgtggttcttttagcttcagtataatagaaggcattgggatttcaaaaaactgttctcgaatgggcacaaagggcaagaggccagtgaagaaaaggccaagaatgagcaggacacgttgtagactgaagagtataggaatatctgaattctctttgaaatgagacatccagtttgccaaggtaaggtgggagctcacagtatttgagatcagagatgtttacattgaccccagttgctctctttagattctcatcatgtgacactacaacttgttcatcttttgtgatatggcagtccaattctagcatatcagttccgattttaaccgcatgctgaaaggctgccattgtattctccaaattttctccagcacctccgcggtgagagatgtgtttactgaggaatcgctgcttctttctctggtgcagcaaggtcgggtatttaagcaacaagaatgaggtcaccaagtatcctcctagcgtagagagaaggtaaaaagccgcagtggacgacatctcagtcaccgtgtgggaagtctcccacctccgggccctctgaactccgctgcggcagtagcaacgacggcggcggcggcggctgctcgaggtcggctcgcccccagccggtgccactggtgcagcgcacttgtcggtgc

SEQ ID NO: 13219 - RNA, 1536 nt, Homo sapiens
  source 1..1536: mol_type = other RNA
gctgggattacaggcatgagccaccacactcagcccaatgccaaatgtatccaatagtctttgattccagaattacttatgatagaacactgcatcatctacagaaatcttgatcaataacctagataacctagtttctaggttattgatcaagatttctgtagatgatgtagtatgtacatttctgtgtatgttattaatcaagatttctgtataagatctagaaacaaaaatgcacattaagaaattaaaacttacatctcataaccaattatctttctaaacaatttacaaacataaaatatacaatattatttaaaataaatatacatataatatatagtttctacattctcatacaggcttaaaaatgaggtaataaaaactgattaaaccttttaccattctggaaatggcttagggaaatgatcatgaaatatttttttcttaggtcttcattttttccttcaatacttctaagtacctctttttctatgctgaaaagttatgtaaaaaatccctaagctttgttggatagtctgtcatcaccccagttgctcccaaatcaaaagctcttttgtattcttgttcttcatttaatacccaaatatacacttgaatgcctcgagcagttaggtggtcaaacaaagctttcctcattagtaagagatcagaaagccagatgagaaacttttgacttctggacatggtgtgtggttcttttagcttcagtataatagaaggcattgggatttcaaaaaactgttctcgaatgggcacaaagggcaagaggccagtgaagaaaaggccaagaatgagcaggacacgttgtagactgaagagtataggaatatctgaattctctttgtagcacttttctacaatttcataattggcattaccccacactgttaagtgttctcgattataccgcttcaccaactctgaaaccttcttaatcagcacattgttgttgactttgatatcgatgttaatgggagtgttaggaaaggcctcaaaaacttccttcagtaatggaattcggttatcttttccttcacactggcatgctctttgaaatgagacatccagtttgccaaggtaaggtgggagctcacagtatttgagatcagagatgtttacattgaccccagttgctctctttagattctcatcatgtgacactacaacttgttcatcttttgtgatatggcagtccaattctagcatatcagttccgattttaaccgcatgctgaaaggctgccattgtattctccaaattttctccagcacctccgcggtgagagatgtgtttactgaggaatcgctgcttctttctctggtgcagcaaggtcgggtatttaagcaacaagaatgaggtcaccaagtatcctcctagcgtagagagaaggtaaaaagccgcagtggacgacatctcagtcaccgtgtgggaagtctcccacctccgggccctctgaactccgctgcggcagtagcaacgacggcggcggcggcggctgctcgaggtcggctc

SEQ ID NO: 13220 - RNA, 1384 nt, Homo sapiens
  source 1..1384: mol_type = other RNA
gctgggattacaggcatgagccaccacactcagcccaatgccaaatgtatccaatagtctttgattccagaattacttatgatagaacactgcatcatctacagaaatcttgatcaataacctagataacctagtttctaggttattgatcaagatttctgtagatgatgtagtatgtacatttctgtgtatgttattaatcaagatttctgtataagatctagaaacaaaaatgcacattaagaaattaaaacttacatctcataaccaattatctttctaaacaatttacaaacataaaatatacaatattatttaaaataaatatacatataatatatagtttctacattctcatacaggcttaaaaatgaggtaataaaaactgattaaaccttttaccattctggaaatggcttagggaaatgatcatgaaatatttttttcttaggtcttcattttttccttcaatacttctaagtacctctttttctatgctgaaaagttatgtaaaaaatccctaagctttgttggatagtctgtcatcaccccagttgctcccaaatcaaaagctcttttgtattcttgttcttcatttaatacccaaatatacacttgaatgcctcgagcagttaggtggtcaaacaaagctttcctcattagtaagagatcagaaagccagatgagaaacttttgacttctggacatggtgtgtggttcttttagcttcagtataatagaaggcattgggatttcaaaaaactgttctcgaatgggcacaaagggcaagaggccagtgaagaaaaggccaagaatgagcaggacacgttgtagactgaagagtataggaatatctgaattctctttgtagcacttttctacaatttcataattggcattaccccacactgttaagtgttctcgattataccgcttcaccaactctgaaaccttcttaatcagcacattgttgttgactttgatatcgatgttaatgggagtgttaggaaaggcctcaaaaacttccttcagtaatggaattcggttatcttttccttcacactggcatgctgttaagcataacaatatggacactgggagagaagcctcttgaaatcctttgctgaacggatcatgtacaagctgccaagagttcatctctgtggaaagggtgtccctaaaagcaaagctaacacaaatgaaagcaaaagcaagaaacggagatagagagagaccaattactgcttgagcaactggaatcagtcatgtctgagggcatataacccctggactttctaattatgaaaaccaatatattcatttttaatttttttcttaagctatcttgagatgtgcatctaacacttataactgaaagagttta

SEQ ID NO: 13221 - RNA, 14536 nt, Homo sapiens
  source 1..14536: mol_type = other RNA
gctgggattacaggcatgagccaccacactcagcctggacagtgttgttcttctagttggttttcctaaacatctacagcaacataaatcttcccatgccttagttagcctgatttagttgagaaacactgaagggacaatcagagacatatatcaccaatcaagtatatatcattctatttcatccttttctctctcctttactgtccctcataatttctacatgagccgaacacacacacttctttttgaaagtgaatgtatatattcactcacttcaaaaatacttactgaaccccaattctatgctaggtcttacatcaggcggtgaggatacaaagtccctgccctcacagagcttcctttctagcagcctcagccacttttagcttgttttcatgaatggagccctgatgtgggaagtgcacctcccagcgtggctgcatctggtccaggctgaatgattaacccttatagtgagtctaagttgaatgaaaacttggattttcagagtcgccattaataccatgttgtcaagggagatggcaaacgatgttgttattcacaagtcgggagccttcaatgatgtaaatttgtatttctcttcccatttttatggagccatatttcagaattcagaaatggaactatggaaatatggctctccccgtccccaaaaagagtccttcttctagacttcttgacaatatgtgtgaggaagcctctggattcagttgttttgtttttttaagtaactttttaaatgaagtataatatgtaaacaaaaaagtgtgtacatcgtagtgtatagctccatgaactttctcactgagcacacatgtaaccagcacccagattaagaaacataacattaatagcgcccatggaagctcctccttcctgtcatgaccccatcccacccctccaccctcatcccaaaggtaactaactactatctggacttctacaaccatggattagttttgcctgtttttgaactttatataaatggagtcatatagcaggttctctttggtactattttcttttactcaatgttatgtttatgaagtttattcatgctgttttattaacccatagaaaatatagatagctcccaagaagaaacataaaaattataatcctactacattaatatgtcagtgtttgtccttctagccacttttctatgtatatacttatgttaactttttttccaaaattagaccatagtgtgcatactactttgtgatttgctttgttgtttgatatatcagatctaccaatgtgttctaaatgttggtcgttgtaatgaggctatattctgaattgactaataggtaatacagaaaagtagaaaattattttttaagtacccataagtatttatattaatcattttgtccgatgtagatttgatccgtctcagtcaggcttccaaaagacttccaaataaaggtagcgaacaaatggatcactgattgctagggaaatctggtaatcaagaccaagttgggcctcttgtttctcaatgaatcttctaaatcactctctactgttttaaacctaggtattctgcgaatatgtaacagattaggaactgaataattctgagaatggcttgttagagtctctgttcaactcttggcttactctataatctgagacaagtctgtaaaatgttccttatttctcagacgaagagcctcatctccacatctgtttgggatcataagaaataatacttacataacattttggaatccttgaatgaaaagttttttggagttgctgactgttcctaaaatttcctcaactaacattgtggaaatccattgttgtggatatagttgctgagctaggtcataactagattgcaaatcttgagtagtggaaaaatctacgcctcgaagttctggtcatttattttaaaagctattcatttattcctagatgttcatactgtgagcttagcctgttatcattttggtttacttgctaaatattcacatttggggtcttcatccttacccatttaggattgtatctattggcatatgccattggatttgtctgagtgaggtcacctggaacactagtgttctgacattgagtttacactgcagggatgagagaagtaaatattcctattagtcagtaaggtttgaatttatagcctgagactcctcagacactgactgtctgggacccttggagacagaccagcattgaatgaaactgaaaggtagagaatatactgtggctgggaaaagtgatggagcaaatctatgcagagatacaatagtaggatatttaagagttggaagggatattagaggccctgtggtcatacttcatttttcagttggggaaactgaggcttaaggaggtcacagaatgagttagtcacagagctgggttagaagcttactttagtgtttcaccaactactcagatgtctgcactactgagatacatagagaaagagcgtcagaggaaggattagggtgtcctctagacctcattacactaatgcagtccctggtaggatctaaagacgtacttgtctccaagacacctgacaagctgagagtattgattcattctttcccaacttgggattgcaatggtgaaaggaatttggcattttatctaatcagcattggaaacttggctttcttttggagaattcaaaagttcagtttaggatatgttcacaagatactttcctccagaattaggtgggagataaattattaaatttatgagacttgtctttctttctttctttctttctttctttctttctttctttctttcttctttcctttcttctttcttttcatgtagcatttctttttcacattgtttctgatgacccttaacccctgctttttaaattcagtttcatttgtgttgtcacatatatatcagttgttgagtctttagtatgcggagatgctgagcttgcccttccaagatgttggaaggtcaactcactttatggtctaggtccaggaaacaagaatatttccaactcgctggggaccatcttggccttgagcagaaatgggatctgaattattacctaagagacctttgtagattgtcacagttggcagcctcaggacttgagctaatcctggaaattctttaacttcccagaaagaaggttccacaagggcaggctgaggtcctcagagagagcagatggaatagagcttacaaccagttgcctttacaactggacttggagataaataataacattatacccattttttttttatcatgaagcctttgactttcaggggatatctattctttattccttttaccctgtatgtggaaaaaaaatgctctgtatgaaagaaaagcaagcaaacttgttgactcagttcccatggtgaatgcaaggcagaccaggccaatagaaacaactcagatattacaaaaatgtgtttctttctggcagctgcacagtcagtcctttatatccagtcactgcaatcgccccatcacacaaaaccatttccaaggtcattattctggttgcgggggctgcttcccctacaaataaatgttggttttactaaatgtcctctctctccaactcactttatggcaaatgaggagtagcaaagcatcatttaggaagagaaagtgtagaaaatcagagagatgaaatactacaggttttctaaaggctcaggtttatctggctcaagcaatacaaattacaaactatggcaccacctgtataatctggttttaattaacttgaggaaggtacatcaatgttatttcattaaaatcaaattctgtttaaatggaaaaccaccactacagggtacattggggcattgttcacttgggttttggggttggcaagtaaatcctgtatttagaaaaacccaagcaaaccctgtttttttggaatcttcttatgcttcggaaggcttgtcataggttccttggaatgtagggggtgccctggtgaggaccaaggcacagctcaagatgttgtttgccaattcttccttttatgacccttctagtcttctgtcttcctgctccctgcctgtctccatatctctttagtgcttggccttgatgccctataggactctctctcccatttgccactttgaactgaatgatttgatccccactgggtggacagtggatgacatagggcactctataaacaaagatgctatttcaggcttacaagaggaatgaggcccacgtgatcacaaggggctggtgaataatagaaccctcttttgaaactctcacttcaccaattacctaagagctgggaggaacctgaaagatcctataatctacacacctccttttccgaggaggacactgagattcggaggtaaagaaactggtccatactagtgaaggctgtttgagtggggcctccccatttcgactcatgccctttcccctccagcctggtgccccagttctgcagacctgttgattacaacacagcccacgccgagaaaatcctgccctgtcagcagaacagctttacaagctgacataggacatgtgtgtgtttggagtcaggagaatggctgagttttagttccagttctgcctctgctttgctggcttcagcgagtcacttctccttcctttgtctatttcccctattgggaaggagaagataattaacctttccacctatcaggctcacttgagtgttataaagaataatgaggtgatatttgtaaagtgctttgagctgctgggaaagaggagggggtgagctccgtggaaaacattattagctggaaggacttatcaattgagctatttaacaatagcagagagtaaggatactcagaaatgaattccagggactagccctgctttgaatttaggaggaggattagtgggaacctaataggtattccgcttctccagtttcttcagtgcaccgtcaaactaggaaaggtaattacattcttctatgtcggattcagcccggagtttcaattgggatgtcaaagtgtgcttgtcctctattctcatactgaggctgtgttatggtgtgattgttaaagccttgggcatcttctatcccctggggtaatttcgcttaggagctatacaaagtaatttctatgcagtggctgggctgctgtttataaggttgattagtagagcttctaaatctaaagcgcctggggagcaatttggttgaagcagggaaataaaaggcaaggtctttatcatggttgatctttttttattgagccgctccatgggaattttctcagtgactcagatgcatctacagtgcaaaacgtggggcttggtggctctttgacatggcaatggaggcctagccccaggtaaaggtgaacttgccaggtcactaaatatatttagggcccccttttaacttcctttactctcacagagggtgatgtttttggggccctgaaatgtgtgggaatgtttccaaaagattgttctgatgagggatctgtttctgcaaactcctgccccactgtttgaaagaccgtctgccccaaattcaggtctttctcatttttagggccagggaagaagacagaggaagagaagaactgggggaattttgttttgaacttgtgcagtctctgtgggctgactgaacagtgagccaggcagaaggtggctccctctttagtcggcaggagcagggctgaattttatcaacatcttctgcaggtgtagggagaggtcaagatgtcatttggaatgataatttctctgatcaaagttaagttaaggaaattacagtgattgcatctttgtcccctaaagtttatgagcctctttgtaatcgctgcttccgcaaacccttccccaccttcccaagttctcaggcctccatctgcaggggctgctgggcttttccctccaggaaggacgggctcgccagctggccagaggttcctgtattagtgctgccctgtactgacttgtgagtctccagtaacaatcctccggtgtggcacagctacaagcaatgaccagggaggcccaccttgaatcctgaacctctttgggggctgactcagtcctctgaaactgactcttggattccttcctgggtttgccaccaactcatttttgtttttctcagcaaatcacttctctgccttgagactccatgaaataatataaggtttccttggcaggattctctgacctttttcagagacccagatttcttgtttattttaatttgaatgtctcaatcctctgaaagcatttggaatattttcttcatttccctctcccaaggtatctactttatcccagacagggctcccccagtgggttttgaggggaaggatgctgaggctttgggcccgggctcctgtcctttacttcacctctgccagggcaaagaccagcactgggctgacctccctgggctgggccaaaagagaaggctgtggaagccgcacgtctccgatgctgcccactgtcctttccctctgcagccacagctgcctccagcccccctcacccccgcctgctctttttctcagtgagcctcagcgccagtgccccagtgagctgctgggaacagaggtccgtcccctgcactggcctcggctccccgcaccagaacattcaggcatcaatgggaaacagcaagatctgtcggcatccccccctttcttcaggctttgagggccacattctccacggccatctgttccctttcacctctctggacaatgttgctttttaaagccagcgattcttcctcctttatcccctcctctcccgcctccccttcttctgtgctcccaccctttctacctctcctctctttgcccgattcctatgaaattagcctctcttaagataagatttgcccttcctccatacaaagctgttttgcaaacactatgggtttttgaatttttatttttacattttgtttgaagtgagggcttgctacttttaaagtttgtgattgtcttgtggagggggtagtcttttgatagggataggaagggggaggatagaaaaactttttagtcatgaaaaaagaaaatacagaataataatgagttttaggttcctgctggcaggcacttgcctctttaaagaaggaatcctccctttcctttccttgatgatcagtttaaggaaatttttatgctctcgaggtcttcccaccttttattgtattactattttgttgttgctgcaatgttgttgttgtgctgtttttaatttagagccagggcttctgtggatctggtacagcggattcctttgtcttggacagagccatatacaactccagaggttcctggattcaggcagagtgcccatggtgccttctagatgaagcaatcatcctgactcaagggctggacatcaaggggtgtttgccccaggactgaccagtgactaagtgtgtgaccttgggtacatcactttctttaagaataatgatgacagaatcatttacttcaaaaaatttttaacacatgattcttctgtttttactattacttggtttcacaagcaagacgagtccgtggtaatgtcatgaaaacttatgggttatccttgggtaaggatgtaccaagaatccaccgttagggtctagttgagcagcagacatgggaaatatctaaaacaaggacggactcctggctgtggctgcctgtcaggatcacagagcagggacacgggcaccggcagagttgggctgacagattgaatcctgtctctcctacttactagctatacagatatcagtaaggttttgtcatctataaaataggggcaacactagagatatacttcgtatggtcgttgagacaattaagagatttttatcacgtaaagcacttggaatagtttctggaacctggtcggtactatgtcgttgtccctcttcctatcccacatccacattacagatgaaaacatgggctaacgggttttctgcagggctcttcttagtctttcacattcaccttctgctggttcattttttcattgcagagtgaacaccaaagttggtagtcttgatcactttgcggatgctggtcatttgcagtaaacccatagttctgtctcatttctggataagcattggcccagaaagagtgactggtaaaggacatgccactttgcacccttcccagctctctccaaaggcagctggctgaatgcacacttctgagggtgatgttttttccagcactcagggatatacccagtgtgagatcagaatcagcagctgtattcattctgcctcagccagtgccatctgaaacaaacatcaagtggtcaaaaaatgagatggtgaccatgtataatacacaagacttattagaattcaactctggtatccgcctgctgcctctgactctacaatgggagcaggaaagcaaagctcataccaggacagctgaaaggtgtggtctgaggatttcatggtgaacagatagaacacactgtgggggaaaaaaaacatattttatgcaagcatctttctggcttgtcttgaatgaagctaaatttaaagagaaagtgccacagatttctttaaatggttaggtttttgttttctttgttttattttgctagtatttacttaagggtaatatgtgttttctgtaatgagtgaatttatttttaattaaaaacttatttgcaaaggtcaagagatttcactacaagtcaccattcaggattttttttttcctttccttaagtagaaggtagcaaggggaaagctgtattggagaaaaggttcaggggcatggcctcctggagaatgttgggagttgagctgatgggaggagattgcttctttttattcagacaatctagttctgttcttcttatgcctactattgttttccttgccatctttgagaccttgatgatcgacactgcagacacagcagagaatcctagtacagactgaagcttttcgtataaagtgagcatgctcactgtgattctggacagttcctacatagtatctctgtaggataacatatgtcttggttttctcagggcaagctcagtttatctctgttatcccagtataactattaaaatgtccccatttcattttcaaaaatgtcctggttggataagaacttaaagtattttgttaagactctgggaaactgaaggtattttctccctgtccatgagccagtggagttgttgagtgatttgtgctggtgcataccagtctctagcctagtggatggctcacccccgcttctcccctaccttgtgctatggaggatccatccctaactcttgcattccagaggttctgattgcctcacttcttcctgtcttctgcttcacatttcttacctttctcagtaacgagtttgctgagacttgcatcagcctaggtatgttgtgcaagtaaagcctctggactgcattcactcctttcacctccagccaagagacatcaggaatgaaattttctgctttactaaagtgaagcagcccattctttaccagccaaatgccttcctcggtgggtaaatggtattagttgaagcagttattacatagttttatgcctcagatcctgtatttataaatctgaaagacgactaatagctttaaagtattttgagaatctcaaagctcagaagattataaataacaaaagatatattttttcgtatctaaaatggtagcacaaatactgcggttgcttacttaatagatagcgtgtggtccctgagccattgcagctgatgggttttttccagtgctctatttatagagctaggtcagaaatatcacttccgttggaacctgacctatagaccattgtcaattttagagacccaaggaagtagaatgcaccctaaatacagctggttcacagattcagttagtgaaccacaagccctcaaggaaattaattttgctggaagataaatgtctgagcctatcccagtctcttttctttgacacctttgtcctgtggtctcacagagcttgtaggtcatcttgaatctttattctaaaaataacctattataggcagtttcccagctttaataacttactcatcctcttcgccttttgttgctaaaattctgcattgaatggaacaagaactgatgacctgccaagagaggtaaccaagattctcagtcccttccccagttcaaatggatggtccaataaagaaccatgctcagcaagtgccaggggcctagttttaaacaggagaagctgaattgaatggatgatgaattgaatgaatgaattgaatccttctgatccctagtctcgcactcagactcccgtctttaagctttgttactatgaagttgtgtttgctgggacttggccactggtcagcacaggtttacccatcataaagtcttactaagtagggtagactaagaaaatctctagtctggagagaaatctgctatcagcaaaagaacccatgcctgtgctcttttcaagcacaaacgggtgctgggtagggcacagcgattcaaagacagcgcatggagtggtgcattctcaaacttcctggaacaagtgaggttctcgatgaggaactcattcatatcatcaaaataccaaagactcaaagttttttaataaggcaggaactattgaggtcatttaccccttcttgtcatggatgaggaaactgaggctcagtgaggttaggtaactgctcattaccaaggcctactctgaggttctttgttacactactctccttctcccacctggtctcatcaaaagcccagacggagtcagaaatagaactgcagggtcctgctttctagccagcagctggccacaggctatcatgcattacatggaatgtgcttcaggacgtgaggacaagagatatgaacgagaatgcagttccagtggtaacataccatcttcttccctggatttatttcaatcctgaaaacatttgtaggtattgttattcctttatttttttaaatttcctctttctactctaaataaatgggctttcatctgcagggactggagggaccaaatatccagaatatccagtccgctaaggccatgaacttttccttcccctctgttcctattttgggagtcattgctttgtttttttgacttttttttttttaacatggaaaagcattcttttaaagttgacccttttgctgcagggcaaatgcttttctgttatgcactagagattcagtttgatctcctagaaatgcttagcacaggagtcataaattgaaatgttttcagagaaggagctttctcattaagagctttccaacaggcctcttctaaatactgacacgggttggtaccagaagcccatcacctttttggaaatcaaggctacatagcaacctggttatcctcctccagtctgattgcacgagggctacaccccatgtatacagagcagagagacagctccttgccttgtgagaaattcgtcttcataaccaactcccacaccaaatgagtaaggaattggatccaaaagatagtcatgaaagatattccagaatccaaatcatgtgttttaaccactttgcaactaagatttactatcttgcctcattgttaacagaataaaaaatgcaggagataatgattaaacttctttcctccctagaatttcatcttcagtgtttgatcatcattgttcctgtcacttatacatatcaagtatcttcatctaagggtcatcaagaacctctggttgcctggaggccagaattattattcacattttacagatgggttagcaatcacagaaagagaacatgctttgacttacctaaaagagtctctgagagagtggagaatgaatgttcccacagtcttttacagagccctgacttcagtgtgagtagattagatttgctctatgtagcttacacagagacttctacaggctcaatcccataacaatgaaaatcctcaaaaatgaaaatattttcaaagctcagttcacgtatttgatttttgtatttgcattggaattaaccaaattccagacaatgaagttatactgctttggcaggtctaaatatcacaatcatcaaaaaggagagagagggagtgagcacctcaatttttagaacttcctcttaaagtgaacatagagaaggttcacttatctgtttcctaaccaattaggtcatcttgcaggaaatcaccttttcttaaaagccagtaggcagattcctcctactttaaatttcccatcaacagcattaacaatcatttatgccagccctctcacaggaatgcttgaaagtcaaaagacataagagaccactaagttttctagtttaaaataaggtcacaactttatagtaacttacagtttccctacctccctctctcaagtgattctatcactgcaatcacccttcaattgctttcctatacttgaggccctattaagtaaactatctttccaatccttgccagatttttaattctacaaccagagaggatcagttccaggccacctgacttgcgtgaatccagctgctgggccagttgagtgagattaagtaacttgctgagccagagtatgtgctgtctttctggaaaccccttgccctgggttatcactgtacatcagaacagaggaagccgagtatggagcctgagtgacatgcagagctcagatgagtgataagatcctcatgacacacttccatcggtatcctcccagagatgggcctttgagctctcaagactcttgtgggctggcagaataacacgttatttgacatgagagacatgataagcccagagaaagctaattggagtagtggttaaaactcagttggcctggtttcgaaccctggctgtgtcagtaactaaccatgtgaactggagtgacttagtttctcatagcctcattctgtcaatagggatgttaatattactcacttcataggattgttgtaaggatcaaaagagatgtagctaagatatgaagctcagcaagatttaagcttacatagtgcctagcacatagtaccttaaaaaatattgcctttccaccttgggcaacatagtgagaccctgtctctacagaaaaataaaaataagttagccaatcattgtggcatgtgcctgtggtcccagctactcggtaggctgaggtgggaggattgcttgagcatgggaattcaaggttacagtgggctatgatcatactactgcattccagcctgggcaataagggagaccctttctctaaaaaaaaatttaaaaattgcctttcattatcattaactttcaaggccttgctgttattacttttatggtggattaatatttgtaagaactcctaaaaatacaaatggatatttttaaagtctatagtagactacagtcaagcttgctcactcagggtttcctttggaaacttttctgtggtcatctgtactcatggcccttacttaagacttgggtttacctgtccagaaaacaaccaaatacatgggtacttttttatactattcttattgttttagcgacgcggagtcctttaaatagttgctcctggcccaaatgtggctccaatctctgaagacatcctgtgtcttcctttagacccgagaaactcctacagtttatcaccaaaaaaaaaaaaaaaaaaaaaaagtttgagtgcttaactagcaactcctaattattcacatgtagctttttcttgacaaactttagagcttagcctcccttgatcccatcacttagcaggcatctaagcaactaatttctagagtttacttgaaaaatgtaaacctgttaattttagctaagcaagatagaattaaggatgtaaatctgctgccaaaacaaggatacaatatgattcaaaatttagtggaaataactttttaattagtcatttagtcagtattataagcatcctctgtgtctcagaccttgtgttaagtaactcaggcatgctgacatacatcaggcgtgggtttggcctctttataatatacagtcatatgtcacttaacaatgaagatgggttctgagaaatgcatcattaagcaattttgacattgtgtgaacatcatagaatgtatttacacaaactgagatggtatagcctactacaaacccaggctgtatagtatagcccattgctcctagtctacagacccattcagcatgttgctgtactgaatactataggcaattggaacacagtagtaagtatttgtgtatctaaacacatctaaacagaaaaggtacaataaaaatggtaaaaggattaaaaatggtacacctgtgtagggcacttactatgactgcagcttataggactggagttgctctgggtccgttggtgagtgcacctactgatgaatgaacatgaaggcctaggacactgctgtacactactgtagacttcataaaccccgtatccttaggctatattcattgatagagacatttttctttcttcaataataaattaacctttgat

SEQ ID NO: 13222 - RNA, 14597 nt, Homo sapiens
  source 1..14597: mol_type = other RNA
gctgggattacaggcatgagccaccacactcagcctggacagtgttgttcttctagttggttttcctaaacatctacagcaacataaatcttcccatgccttagttagcctgatttagttgagaaacactgaagggacaatcagagacatatatcaccaatcaagtatatatcattctatttcatccttttctctctcctttactgtccctcataatttctacatgagccgaacacacacacttctttttgaaagtgaatgtatatattcactcacttcaaaaatacttactgaaccccaattctatgctaggtcttacatcaggcggtgaggatacaaagtccctgccctcacagagcttcctttctagcagcctcagccacttttagcttgttttcatgaatggagccctgatgtgggaagtgcacctcccagcgtggctgcatctggtccaggctgaatgattaacccttatagtgagtctaagttgaatgaaaacttggattttcagagtcgccattaataccatgttgtcaagggagatggcaaacgatgttgttattcacaagtcgggagccttcaatgatgtaaatttgtatttctcttcccatttttatggagccatatttcagaattcagaaatggaactatggaaatatggctctccccgtccccaaaaagagtccttcttctagacttcttgacaatatgtgtgaggaagcctctggattcagttgttttgtttttttaagtaactttttaaatgaagtataatatgtaaacaaaaaagtgtgtacatcgtagtgtatagctccatgaactttctcactgagcacacatgtaaccagcacccagattaagaaacataacattaatagcgcccatggaagctcctccttcctgtcatgaccccatcccacccctccaccctcatcccaaaggtaactaactactatctggacttctacaaccatggattagttttgcctgtttttgaactttatataaatggagtcatatagcaggttctctttggtactattttcttttactcaatgttatgtttatgaagtttattcatgctgttttattaacccatagaaaatatagatagctcccaagaagaaacataaaaattataatcctactacattaatatgtcagtgtttgtccttctagccacttttctatgtatatacttatgttaactttttttccaaaattagaccatagtgtgcatactactttgtgatttgctttgttgtttgatatatcagatctaccaatgtgttctaaatgttggtcgttgtaatgaggctatattctgaattgactaataggtaatacagaaaagtagaaaattattttttaagtacccataagtatttatattaatcattttgtccgatgtagatttgatccgtctcagtcaggcttccaaaagacttccaaataaaggtagcgaacaaatggatcactgattgctagggaaatctggtaatcaagaccaagttgggcctcttgtttctcaatgaatcttctaaatcactctctactgttttaaacctaggtattctgcgaatatgtaacagattaggaactgaataattctgagaatggcttgttagagtctctgttcaactcttggcttactctataatctgagacaagtctgtaaaatgttccttatttctcagacgaagagcctcatctccacatctgtttgggatcataagaaataatacttacataacattttggaatccttgaatgaaaagttttttggagttgctgactgttcctaaaatttcctcaactaacattgtggaaatccattgttgtggatatagttgctgagctaggtcataactagattgcaaatcttgagtagtggaaaaatctacgcctcgaagttctggtcatttattttaaaagctattcatttattcctagatgttcatactgtgagcttagcctgttatcattttggtttacttgctaaatattcacatttggggtcttcatccttacccatttaggattgtatctattggcatatgccattggatttgtctgagtgaggtcacctggaacactagtgttctgacattgagtttacactgcagggatgagagaagtaaatattcctattagtcagtaaggtttgaatttatagcctgagactcctcagacactgactgtctgggacccttggagacagaccagcattgaatgaaactgaaaggtagagaatatactgtggctgggaaaagtgatggagcaaatctatgcagagatacaatagtaggatatttaagagttggaagggatattagaggccctgtggtcatacttcatttttcagttggggaaactgaggcttaaggaggtcacagaatgagttagtcacagagctgggttagaagcttactttagtgtttcaccaactactcagatgtctgcactactgagatacatagagaaagagcgtcagaggaaggattagggtgtcctctagacctcattacactaatgcagtccctggtaggatctaaagacgtacttgtctccaagacacctgacaagctgagagtattgattcattctttcccaacttgggattgcaatggtgaaaggaatttggcattttatctaatcagcattggaaacttggctttcttttggagaattcaaaagttcagtttaggatatgttcacaagatactttcctccagaattaggtgggagataaattattaaatttatgagacttgtctttctttctttctttctttctttctttctttctttctttctttcttctttcctttcttctttcttttcatgtagcatttctttttcacattgtttctgatgacccttaacccctgctttttaaattcagtttcatttgtgttgtcacatatatatcagttgttgagtctttagtatgcggagatgctgagcttgcccttccaagatgttggaaggtcaactcactttatggtctaggtccaggaaacaagaatatttccaactcgctggggaccatcttggccttgagcagaaatgggatctgaattattacctaagagacctttgtagattgtcacagttggcagcctcaggacttgagctaatcctggaaattctttaacttcccagaaagaaggttccacaagggcaggctgaggtcctcagagagagcagatggaatagagcttacaaccagttgcctttacaactggacttggagataaataataacattatacccattttttttttatcatgaagcctttgactttcaggggatatctattctttattccttttaccctgtatgtggaaaaaaaatgctctgtatgaaagaaaagcaagcaaacttgttgactcagttcccatggtgaatgcaaggcagaccaggccaatagaaacaactcagatattacaaaaatgtgtttctttctggcagctgcacagtcagtcctttatatccagtcactgcaatcgccccatcacacaaaaccatttccaaggtcattattctggttgcgggggctgcttcccctacaaataaatgttggttttactaaatgtcctctctctccaactcactttatggcaaatgaggagtagcaaagcatcatttaggaagagaaagtgtagaaaatcagagagatgaaatactacaggttttctaaaggctcaggtttatctggctcaagcaatacaaattacaaactatggcaccacctgtataatctggttttaattaacttgaggaaggtacatcaatgttatttcattaaaatcaaattctgtttaaatggaaaaccaccactacagggtacattggggcattgttcacttgggttttggggttggcaagtaaatcctgtatttagaaaaacccaagcaaaccctgtttttttggaatcttcttatgcttcggaaggcttgtcataggttccttggaatgtagggggtgccctggtgaggaccaaggcacagctcaagatgttgtttgccaattcttccttttatgacccttctagtcttctgtcttcctgctccctgcctgtctccatatctctttagtgcttggccttgatgccctataggactctctctcccatttgccactttgaactgaatgatttgatccccactgggtggacagtggatgacatagggcactctataaacaaagatgctatttcaggcttacaagaggaatgaggcccacgtgatcacaaggggctggtgaataatagaaccctcttttgaaactctcacttcaccaattacctaagagctgggaggaacctgaaagatcctataatctacacacctccttttccgaggaggacactgagattcggaggtaaagaaactggtccatactagtgaaggctgtttgagtggggcctccccatttcgactcatgccctttcccctccagcctggtgccccagttctgcagacctgttgattacaacacagcccacgccgagaaaatcctgccctgtcagcagaacagctttacaagctgacataggacatgtgtgtgtttggagtcaggagaatggctgagttttagttccagttctgcctctgctttgctggcttcagcgagtcacttctccttcctttgtctatttcccctattgggaaggagaagataattaacctttccacctatcaggctcacttgagtgttataaagaataatgaggtgatatttgtaaagtgctttgagctgctgggaaagaggagggggtgagctccgtggaaaacattattagctggaaggacttatcaattgagctatttaacaatagcagagagtaaggatactcagaaatgaattccagggactagccctgctttgaatttaggaggaggattagtgggaacctaataggtattccgcttctccagtttcttcagtgcaccgtcaaactaggaaaggtaattacattcttctatgtcggattcagcccggagtttcaattgggatgtcaaagtgtgcttgtcctctattctcatactgaggctgtgttatggtgtgattgttaaagccttgggcatcttctatcccctggggtaatttcgcttaggagctatacaaagtaatttctatgcagtggctgggctgctgtttataaggttgattagtagagcttctaaatctaaagcgcctggggagcaatttggttgaagcagggaaataaaaggcaaggtctttatcatggttgatctttttttattgagccgctccatgggaattttctcagtgactcagatgcatctacagtgcaaaacgtggggcttggtggctctttgacatggcaatggaggcctagccccaggtaaaggtgaacttgccaggtcactaaatatatttagggcccccttttaacttcctttactctcacagagggtgatgtttttggggccctgaaatgtgtgggaatgtttccaaaagattgttctgatgagggatctgtttctgcaaactcctgccccactgtttgaaagaccgtctgccccaaattcaggtctttctcatttttagggccagggaagaagacagaggaagagaagaactgggggaattttgttttgaacttgtgcagtctctgtgggctgactgaacagtgagccaggcagaaggtggctccctctttagtcggcaggagcagggctgaattttatcaacatcttctgcaggtgtagggagaggtcaagatgtcatttggaatgataatttctctgatcaaagttaagttaaggaaattacagtgattgcatctttgtcccctaaagtttatgagcctctttgtaatcgctgcttccgcaaacccttccccaccttcccaagttctcaggcctccatctgcaggggctgctgggcttttccctccaggaaggacgggctcgccagctggccagaggttcctgtattagtgctgccctgtactgacttgtgagtctccagtaacaatcctccggtgtggcacagctacaagcaatgaccagggaggcccaccttgaatcctgaacctctttgggggctgactcagtcctctgaaactgactcttggattccttcctgggtttgccaccaactcatttttgtttttctcagcaaatcacttctctgccttgagactccatgaaataatataaggtttccttggcaggattctctgacctttttcagagacccagatttcttgtttattttaatttgaatgtctcaatcctctgaaagcatttggaatattttcttcatttccctctcccaaggtatctactttatcccagacagggctcccccagtgggttttgaggggaaggatgctgaggctttgggcccgggctcctgtcctttacttcacctctgccagggcaaagaccagcactgggctgacctccctgggctgggccaaaagagaaggctgtggaagccgcacgtctccgatgctgcccactgtcctttccctctgcagccacagctgcctccagcccccctcacccccgcctgctctttttctcagtgagcctcagcgccagtgccccagtgagctgctgggaacagaggtccgtcccctgcactggcctcggctccccgcaccagaacattcaggcatcaatgggaaacagcaagatctgtcggcatccccccctttcttcaggctttgagggccacattctccacggccatctgttccctttcacctctctggacaatgttgctttttaaagccagcgattcttcctcctttatcccctcctctcccgcctccccttcttctgtgctcccaccctttctacctctcctctctttgcccgattcctatgaaattagcctctcttaagataagatttgcccttcctccatacaaagctgttttgcaaacactatgggtttttgaatttttatttttacattttgtttgaagtgagggcttgctacttttaaagtttgtgattgtcttgtggagggggtagtcttttgatagggataggaagggggaggatagaaaaactttttagtcatgaaaaaagaaaatacagaataataatgagttttaggttcctgctggcaggcacttgcctctttaaagaaggaatcctccctttcctttccttgatgatcagtttaaggaaatttttatgctctcgaggtcttcccaccttttattgtattactattttgttgttgctgcaatgttgttgttgtgctgtttttaatttagagccagggcttctgtggatctggtacagcggattcctttgtcttggacagagccatatacaactccagaggttcctggattcaggcagagtgcccatggtgccttctagatgaagcaatcatcctgactcaagggctggacatcaaggggtgtttgccccaggactgaccagtgactaagtgtgtgaccttgggtacatcactttctttaagaataatgatgacagaatcatttacttcaaaaaatttttaacacatgattcttctgtttttactattacttggtttcacaagcaagacgagtccgtggtaatgtcatgaaaacttatgggttatccttgggtaaggatgtaccaagaatccaccgttagggtctagttgagcagcagacatgggaaatatctaaaacaaggacggactcctggctgtggctgcctgtcaggatcacagagcagggacacgggcaccggcagagttgggctgacagattgaatcctgtctctcctacttactagctatacagatatcagtaaggttttgtcatctataaaataggggcaacactagagatatacttcgtatggtcgttgagacaattaagagatttttatcacgtaaagcacttggaatagtttctggaacctggtcggtactatgtcgttgtccctcttcctatcccacatccacattacagatgaaaacatgggctaacgggttttctgcagggctcttcttagtctttcacattcaccttctgctggttcattttttcattgcagagtgaacactcataattctttactgtaatgtcttatatcaactgacatctgagatgtgggacacattacccaaagttggtagtcttgatcactttgcggatgctggtcatttgcagtaaacccatagttctgtctcatttctggataagcattggcccagaaagagtgactggtaaaggacatgccactttgcacccttcccagctctctccaaaggcagctggctgaatgcacacttctgagggtgatgttttttccagcactcagggatatacccagtgtgagatcagaatcagcagctgtattcattctgcctcagccagtgccatctgaaacaaacatcaagtggtcaaaaaatgagatggtgaccatgtataatacacaagacttattagaattcaactctggtatccgcctgctgcctctgactctacaatgggagcaggaaagcaaagctcataccaggacagctgaaaggtgtggtctgaggatttcatggtgaacagatagaacacactgtgggggaaaaaaaacatattttatgcaagcatctttctggcttgtcttgaatgaagctaaatttaaagagaaagtgccacagatttctttaaatggttaggtttttgttttctttgttttattttgctagtatttacttaagggtaatatgtgttttctgtaatgagtgaatttatttttaattaaaaacttatttgcaaaggtcaagagatttcactacaagtcaccattcaggattttttttttcctttccttaagtagaaggtagcaaggggaaagctgtattggagaaaaggttcaggggcatggcctcctggagaatgttgggagttgagctgatgggaggagattgcttctttttattcagacaatctagttctgttcttcttatgcctactattgttttccttgccatctttgagaccttgatgatcgacactgcagacacagcagagaatcctagtacagactgaagcttttcgtataaagtgagcatgctcactgtgattctggacagttcctacatagtatctctgtaggataacatatgtcttggttttctcagggcaagctcagtttatctctgttatcccagtataactattaaaatgtccccatttcattttcaaaaatgtcctggttggataagaacttaaagtattttgttaagactctgggaaactgaaggtattttctccctgtccatgagccagtggagttgttgagtgatttgtgctggtgcataccagtctctagcctagtggatggctcacccccgcttctcccctaccttgtgctatggaggatccatccctaactcttgcattccagaggttctgattgcctcacttcttcctgtcttctgcttcacatttcttacctttctcagtaacgagtttgctgagacttgcatcagcctaggtatgttgtgcaagtaaagcctctggactgcattcactcctttcacctccagccaagagacatcaggaatgaaattttctgctttactaaagtgaagcagcccattctttaccagccaaatgccttcctcggtgggtaaatggtattagttgaagcagttattacatagttttatgcctcagatcctgtatttataaatctgaaagacgactaatagctttaaagtattttgagaatctcaaagctcagaagattataaataacaaaagatatattttttcgtatctaaaatggtagcacaaatactgcggttgcttacttaatagatagcgtgtggtccctgagccattgcagctgatgggttttttccagtgctctatttatagagctaggtcagaaatatcacttccgttggaacctgacctatagaccattgtcaattttagagacccaaggaagtagaatgcaccctaaatacagctggttcacagattcagttagtgaaccacaagccctcaaggaaattaattttgctggaagataaatgtctgagcctatcccagtctcttttctttgacacctttgtcctgtggtctcacagagcttgtaggtcatcttgaatctttattctaaaaataacctattataggcagtttcccagctttaataacttactcatcctcttcgccttttgttgctaaaattctgcattgaatggaacaagaactgatgacctgccaagagaggtaaccaagattctcagtcccttccccagttcaaatggatggtccaataaagaaccatgctcagcaagtgccaggggcctagttttaaacaggagaagctgaattgaatggatgatgaattgaatgaatgaattgaatccttctgatccctagtctcgcactcagactcccgtctttaagctttgttactatgaagttgtgtttgctgggacttggccactggtcagcacaggtttacccatcataaagtcttactaagtagggtagactaagaaaatctctagtctggagagaaatctgctatcagcaaaagaacccatgcctgtgctcttttcaagcacaaacgggtgctgggtagggcacagcgattcaaagacagcgcatggagtggtgcattctcaaacttcctggaacaagtgaggttctcgatgaggaactcattcatatcatcaaaataccaaagactcaaagttttttaataaggcaggaactattgaggtcatttaccccttcttgtcatggatgaggaaactgaggctcagtgaggttaggtaactgctcattaccaaggcctactctgaggttctttgttacactactctccttctcccacctggtctcatcaaaagcccagacggagtcagaaatagaactgcagggtcctgctttctagccagcagctggccacaggctatcatgcattacatggaatgtgcttcaggacgtgaggacaagagatatgaacgagaatgcagttccagtggtaacataccatcttcttccctggatttatttcaatcctgaaaacatttgtaggtattgttattcctttatttttttaaatttcctctttctactctaaataaatgggctttcatctgcagggactggagggaccaaatatccagaatatccagtccgctaaggccatgaacttttccttcccctctgttcctattttgggagtcattgctttgtttttttgacttttttttttttaacatggaaaagcattcttttaaagttgacccttttgctgcagggcaaatgcttttctgttatgcactagagattcagtttgatctcctagaaatgcttagcacaggagtcataaattgaaatgttttcagagaaggagctttctcattaagagctttccaacaggcctcttctaaatactgacacgggttggtaccagaagcccatcacctttttggaaatcaaggctacatagcaacctggttatcctcctccagtctgattgcacgagggctacaccccatgtatacagagcagagagacagctccttgccttgtgagaaattcgtcttcataaccaactcccacaccaaatgagtaaggaattggatccaaaagatagtcatgaaagatattccagaatccaaatcatgtgttttaaccactttgcaactaagatttactatcttgcctcattgttaacagaataaaaaatgcaggagataatgattaaacttctttcctccctagaatttcatcttcagtgtttgatcatcattgttcctgtcacttatacatatcaagtatcttcatctaagggtcatcaagaacctctggttgcctggaggccagaattattattcacattttacagatgggttagcaatcacagaaagagaacatgctttgacttacctaaaagagtctctgagagagtggagaatgaatgttcccacagtcttttacagagccctgacttcagtgtgagtagattagatttgctctatgtagcttacacagagacttctacaggctcaatcccataacaatgaaaatcctcaaaaatgaaaatattttcaaagctcagttcacgtatttgatttttgtatttgcattggaattaaccaaattccagacaatgaagttatactgctttggcaggtctaaatatcacaatcatcaaaaaggagagagagggagtgagcacctcaatttttagaacttcctcttaaagtgaacatagagaaggttcacttatctgtttcctaaccaattaggtcatcttgcaggaaatcaccttttcttaaaagccagtaggcagattcctcctactttaaatttcccatcaacagcattaacaatcatttatgccagccctctcacaggaatgcttgaaagtcaaaagacataagagaccactaagttttctagtttaaaataaggtcacaactttatagtaacttacagtttccctacctccctctctcaagtgattctatcactgcaatcacccttcaattgctttcctatacttgaggccctattaagtaaactatctttccaatccttgccagatttttaattctacaaccagagaggatcagttccaggccacctgacttgcgtgaatccagctgctgggccagttgagtgagattaagtaacttgctgagccagagtatgtgctgtctttctggaaaccccttgccctgggttatcactgtacatcagaacagaggaagccgagtatggagcctgagtgacatgcagagctcagatgagtgataagatcctcatgacacacttccatcggtatcctcccagagatgggcctttgagctctcaagactcttgtgggctggcagaataacacgttatttgacatgagagacatgataagcccagagaaagctaattggagtagtggttaaaactcagttggcctggtttcgaaccctggctgtgtcagtaactaaccatgtgaactggagtgacttagtttctcatagcctcattctgtcaatagggatgttaatattactcacttcataggattgttgtaaggatcaaaagagatgtagctaagatatgaagctcagcaagatttaagcttacatagtgcctagcacatagtaccttaaaaaatattgcctttccaccttgggcaacatagtgagaccctgtctctacagaaaaataaaaataagttagccaatcattgtggcatgtgcctgtggtcccagctactcggtaggctgaggtgggaggattgcttgagcatgggaattcaaggttacagtgggctatgatcatactactgcattccagcctgggcaataagggagaccctttctctaaaaaaaaatttaaaaattgcctttcattatcattaactttcaaggccttgctgttattacttttatggtggattaatatttgtaagaactcctaaaaatacaaatggatatttttaaagtctatagtagactacagtcaagcttgctcactcagggtttcctttggaaacttttctgtggtcatctgtactcatggcccttacttaagacttgggtttacctgtccagaaaacaaccaaatacatgggtacttttttatactattcttattgttttagcgacgcggagtcctttaaatagttgctcctggcccaaatgtggctccaatctctgaagacatcctgtgtcttcctttagacccgagaaactcctacagtttatcaccaaaaaaaaaaaaaaaaaaaaaaagtttgagtgcttaactagcaactcctaattattcacatgtagctttttcttgacaaactttagagcttagcctcccttgatcccatcacttagcaggcatctaagcaactaatttctagagtttacttgaaaaatgtaaacctgttaattttagctaagcaagatagaattaaggatgtaaatctgctgccaaaacaaggatacaatatgattcaaaatttagtggaaataactttttaattagtcatttagtcagtattataagcatcctctgtgtctcagaccttgtgttaagtaactcaggcatgctgacatacatcaggcgtgggtttggcctctttataatatacagtcatatgtcacttaacaatgaagatgggttctgagaaatgcatcattaagcaattttgacattgtgtgaacatcatagaatgtatttacacaaactgagatggtatagcctactacaaacccaggctgtatagtatagcccattgctcctagtctacagacccattcagcatgttgctgtactgaatactataggcaattggaacacagtagtaagtatttgtgtatctaaacacatctaaacagaaaaggtacaataaaaatggtaaaaggattaaaaatggtacacctgtgtagggcacttactatgactgcagcttataggactggagttgctctgggtccgttggtgagtgcacctactgatgaatgaacatgaaggcctaggacactgctgtacactactgtagacttcataaaccccgtatccttaggctatattcattgatagagacatttttctttcttcaataataaattaacctttgat

SEQ ID NO: 13223 - RNA, 11768 nt, Homo sapiens
  source 1..11768: mol_type = other RNA
gctgggattacaggcatgagccaccacactcagcctggacagtgttgttcttctagttggttttcctaaacatctacagcaacataaatcttcccatgccttagttagcctgatttagttgagaaacactgaagggacaatcagagacatatatcaccaatcaagtatatatcattctatttcatccttttctctctcctttactgtccctcataatttctacatgagccgaacacacacacttctttttgaaagtgaatgtatatattcactcacttcaaaaatacttactgaaccccaattctatgctaggtcttacatcaggcggtgaggatacaaagtccctgccctcacagagcttcctttctagcagcctcagccacttttagcttgttttcatgaatggagccctgatgtgggaagtgcacctcccagcgtggctgcatctggtccaggctgaatgattaacccttatagtgagtctaagttgaatgaaaacttggattttcagagtcgccattaataccatgttgtcaagggagatggcaaacgatgttgttattcacaagtcgggagccttcaatgatgtaaatttgtatttctcttcccatttttatggagccatatttcagaattcagaaatggaactatggaaatatggctctccccgtccccaaaaagagtccttcttctagacttcttgacaatatgtgtgaggaagcctctggattcagttgttttgtttttttaagtaactttttaaatgaagtataatatgtaaacaaaaaagtgtgtacatcgtagtgtatagctccatgaactttctcactgagcacacatgtaaccagcacccagattaagaaacataacattaatagcgcccatggaagctcctccttcctgtcatgaccccatcccacccctccaccctcatcccaaaggtaactaactactatctggacttctacaaccatggattagttttgcctgtttttgaactttatataaatggagtcatatagcaggttctctttggtactattttcttttactcaatgttatgtttatgaagtttattcatgctgttttattaacccatagaaaatatagatagctcccaagaagaaacataaaaattataatcctactacattaatatgtcagtgtttgtccttctagccacttttctatgtatatacttatgttaactttttttccaaaattagaccatagtgtgcatactactttgtgatttgctttgttgtttgatatatcagatctaccaatgtgttctaaatgttggtcgttgtaatgaggctatattctgaattgactaataggtaatacagaaaagtagaaaattattttttaagtacccataagtatttatattaatcattttgtccgatgtagatttgatccgtctcagtcaggcttccaaaagacttccaaataaaggtagcgaacaaatggatcactgattgctagggaaatctggtaatcaagaccaagttgggcctcttgtttctcaatgaatcttctaaatcactctctactgttttaaacctaggtattctgcgaatatgtaacagattaggaactgaataattctgagaatggcttgttagagtctctgttcaactcttggcttactctataatctgagacaagtctgtaaaatgttccttatttctcagacgaagagcctcatctccacatctgtttgggatcataagaaataatacttacataacattttggaatccttgaatgaaaagttttttggagttgctgactgttcctaaaatttcctcaactaacattgtggaaatccattgttgtggatatagttgctgagctaggtcataactagattgcaaatcttgagtagtggaaaaatctacgcctcgaagttctggtcatttattttaaaagctattcatttattcctagatgttcatactgtgagcttagcctgttatcattttggtttacttgctaaatattcacatttggggtcttcatccttacccatttaggattgtatctattggcatatgccattggatttgtctgagtgaggtcacctggaacactagtgttctgacattgagtttacactgcagggatgagagaagtaaatattcctattagtcagtaaggtttgaatttatagcctgagactcctcagacactgactgtctgggacccttggagacagaccagcattgaatgaaactgaaaggtagagaatatactgtggctgggaaaagtgatggagcaaatctatgcagagatacaatagtaggatatttaagagttggaagggatattagaggccctgtggtcatacttcatttttcagttggggaaactgaggcttaaggaggtcacagaatgagttagtcacagagctgggttagaagcttactttagtgtttcaccaactactcagatgtctgcactactgagatacatagagaaagagcgtcagaggaaggattagggtgtcctctagacctcattacactaatgcagtccctggtaggatctaaagacgtacttgtctccaagacacctgacaagctgagagtattgattcattctttcccaacttgggattgcaatggtgaaaggaatttggcattttatctaatcagcattggaaacttggctttcttttggagaattcaaaagttcagtttaggatatgttcacaagatactttcctccagaattaggtgggagataaattattaaatttatgagacttgtctttctttctttctttctttctttctttctttctttctttctttcttctttcctttcttctttcttttcatgtagcatttctttttcacattgtttctgatgacccttaacccctgctttttaaattcagtttcatttgtgttgtcacatatatatcagttgttgagtctttagtatgcggagatgctgagcttgcccttccaagatgttggaaggtcaactcactttatggtctaggtccaggaaacaagaatatttccaactcgctggggaccatcttggccttgagcagaaatgggatctgaattattacctaagagacctttgtagattgtcacagttggcagcctcaggacttgagctaatcctggaaattctttaacttcccagaaagaaggttccacaagggcaggctgaggtcctcagagagagcagatggaatagagcttacaaccagttgcctttacaactggacttggagataaataataacattatacccattttttttttatcatgaagcctttgactttcaggggatatctattctttattccttttaccctgtatgtggaaaaaaaatgctctgtatgaaagaaaagcaagcaaacttgttgactcagttcccatggtgaatgcaaggcagaccaggccaatagaaacaactcagatattacaaaaatgtgtttctttctggcagctgcacagtcagtcctttatatccagtcactgcaatcgccccatcacacaaaaccatttccaaggtcattattctggttgcgggggctgcttcccctacaaataaatgttggttttactaaatgtcctctctctccaactcactttatggcaaatgaggagtagcaaagcatcatttaggaagagaaagtgtagaaaatcagagagatgaaatactacaggttttctaaaggctcaggtttatctggctcaagcaatacaaattacaaactatggcaccacctgtataatctggttttaattaacttgaggaaggtacatcaatgttatttcattaaaatcaaattctgtttaaatggaaaaccaccactacagggtacattggggcattgttcacttgggttttggggttggcaagtaaatcctgtatttagaaaaacccaagcaaaccctgtttttttggaatcttcttatgcttcggaaggcttgtcataggttccttggaatgtagggggtgccctggtgaggaccaaggcacagctcaagatgttgtttgccaattcttccttttatgacccttctagtcttctgtcttcctgctccctgcctgtctccatatctctttagtgcttggccttgatgccctataggactctctctcccatttgccactttgaactgaatgatttgatccccactgggtggacagtggatgacatagggcactctataaacaaagatgctatttcaggcttacaagaggaatgaggcccacgtgatcacaaggggctggtgaataatagaaccctcttttgaaactctcacttcaccaattacctaagagctgggaggaacctgaaagatcctataatctacacacctccttttccgaggaggacactgagattcggaggtaaagaaactggtccatactagtgaaggctgtttgagtggggcctccccatttcgactcatgccctttcccctccagcctggtgccccagttctgcagacctgttgattacaacacagcccacgccgagaaaatcctgccctgtcagcagaacagctttacaagctgacataggacatgtgtgtgtttggagtcaggagaatggctgagttttagttccagttctgcctctgctttgctggcttcagcgagtcacttctccttcctttgtctatttcccctattgggaaggagaagataattaacctttccacctatcaggctcacttgagtgttataaagaataatgaggtgatatttgtaaagtgctttgagctgctgggaaagaggagggggtgagctccgtggaaaacattattagctggaaggacttatcaattgagctatttaacaatagcagagagtaaggatactcagaaatgaattccagggactagccctgctttgaatttaggaggaggattagtgggaacctaataggtattccgcttctccagtttcttcagtgcaccgtcaaactaggaaaggtaattacattcttctatgtcggattcagcccggagtttcaattgggatgtcaaagtgtgcttgtcctctattctcatactgaggctgtgttatggtgtgattgttaaagccttgggcatcttctatcccctggggtaatttcgcttaggagctatacaaagtaatttctatgcagtggctgggctgctgtttataaggttgattagtagagcttctaaatctaaagcgcctggggagcaatttggttgaagcagggaaataaaaggcaaggtctttatcatggttgatctttttttattgagccgctccatgggaattttctcagtgactcagatgcatctacagtgcaaaacgtggggcttggtggctctttgacatggcaatggaggcctagccccaggtaaaggtgaacttgccaggtcactaaatatatttagggcccccttttaacttcctttactctcacagagggtgatgtttttggggccctgaaatgtgtgggaatgtttccaaaagattgttctgatgagggatctgtttctgcaaactcctgccccactgtttgaaagaccgtctgccccaaattcaggtctttctcatttttagggccagggaagaagacagaggaagagaagaactgggggaattttgttttgaacttgtgcagtctctgtgggctgactgaacagtgagccaggcagaaggtggctccctctttagtcggcaggagcagggctgaattttatcaacatcttctgcaggtgtagggagaggtcaagatgtcatttggaatgataatttctctgatcaaagttaagttaaggaaattacagtgattgcatctttgtcccctaaagtttatgagcctctttgtaatcgctgcttccgcaaacccttccccaccttcccaagttctcaggcctccatctgcaggggctgctgggcttttccctccaggaaggacgggctcgccagctggccagaggttcctgtattagtgctgccctgtactgacttgtgagtctccagtaacaatcctccggtgtggcacagctacaagcaatgaccagggaggcccaccttgaatcctgaacctctttgggggctgactcagtcctctgaaactgactcttggattccttcctgggtttgccaccaactcatttttgtttttctcagcaaatcacttctctgccttgagactccatgaaataatataaggtttccttggcaggattctctgacctttttcagagacccagatttcttgtttattttaatttgaatgtctcaatcctctgaaagcatttggaatattttcttcatttccctctcccaaggtatctactttatcccagacagggctcccccagtgggttttgaggggaaggatgctgaggctttgggcccgggctcctgtcctttacttcacctctgccagggcaaagaccagcactgggctgacctccctgggctgggccaaaagagaaggctgtggaagccgcacgtctccgatgctgcccactgtcctttccctctgcagccacagctgcctccagcccccctcacccccgcctgctctttttctcagtgagcctcagcgccagtgccccagtgagctgctgggaacagaggtccgtcccctgcactggcctcggctccccgcaccagaacattcaggcatcaatgggaaacagcaagatctgtcggcatccccccctttcttcaggctttgagggccacattctccacggccatctgttccctttcacctctctggacaatgttgctttttaaagccagcgattcttcctcctttatcccctcctctcccgcctccccttcttctgtgctcccaccctttctacctctcctctctttgcccgattcctatgaaattagcctctcttaagataagatttgcccttcctccatacaaagctgttttgcaaacactatgggtttttgaatttttatttttacattttgtttgaagtgagggcttgctacttttaaagtttgtgattgtcttgtggagggggtagtcttttgatagggataggaagggggaggatagaaaaactttttagtcatgaaaaaagaaaatacagaataataatgagttttaggttcctgctggcaggcacttgcctctttaaagaaggaatcctccctttcctttccttgatgatcagtttaaggaaatttttatgctctcgaggtcttcccaccttttattgtattactattttgttgttgctgcaatgttgttgttgtgctgtttttaatttagagccagggcttctgtggatctggtacagcggattcctttgtcttggacagagccatatacaactccagaggttcctggattcaggcagagtgcccatggtgccttctagatgaagcaatcatcctgactcaagggctggacatcaaggggtgtttgccccaggactgaccagtgactaagtgtgtgaccttgggtacatcactttctttaagaataatgatgacagaatcatttacttcaaaaaatttttaacacatgattcttctgtttttactattacttggtttcacaagcaagacgagtccgtggtaatgtcatgaaaacttatgggttatccttgggtaaggatgtaccaagaatccaccgttagggtctagttgagcagcagacatgggaaatatctaaaacaaggacggactcctggctgtggctgcctgtcaggatcacagagcagggacacgggcaccggcagagttgggctgacagattgaatcctgtctctcctacttactagctatacagatatcagtaaggttttgtcatctataaaataggggcaacactagagatatacttcgtatggtcgttgagacaattaagagatttttatcacgtaaagcacttggaatagtttctggaacctggtcggtactatgtcgttgtccctcttcctatcccacatccacattacagatgaaaacatgggctaacgggttttctgcagggctcttcttagtctttcacattcaccttctgctggttcattttttcattgcagagtgaacactgataaaataaataatgtaattatcagattataatgatgattaacacagcgattctatttagaaatgtcataaaatagtgaaacatcctaagatacagaaagatatatgatcatgtacttctggcaaagaaggtgaaccagatgtggagatgatagtcatagaaggaaagccagtcatgattttggcaactgggatcaccttacatattttcagttggagaaaacctggagatttatttttcttttggtatcaatttctagaaacctgtcgtatgactaagagtttcccaacaatagggagagaacattattaaaatatgcttttctagaaaggcccaaatgactctgaataagaaactgaatattataatttaatgaggaaaagaaaatgaatgggatgtccagaaaattggggcggggagggggtagtttccatgcattttccctcctagaaagggagattaatggccattcttgtaatatctaaatggccaaaagaaacaatgaaaagaaaaataatgaatcagactctggggtttaaatcctgactctgccacttgccaggtggccttgggcaaatcactttctttgtagcgcagcttccttcactagaaaattggtatgataatggtacctccctcacagagataatgtatgtaaggtgtttagcctggaaaacaataattatcccaaagtgttacctcataattctttactgtaatgtcttatatcaactgacatctgagatgtgggacacattacccaaagttggtagtcttgatcactttgcggatgctggtcatttgcagtaaacccatagttctgtctcatttctggataagcattggcccagaaagagtgactggtaaaggacatgccactttgcacccttcccagctctctccaaaggcagctggctgaatgcacacttctgagggtgatgttttttccagcactcagggatatacccagtgtgagatcagaatcagcagctgtattcattctgcctcagccagtgccatctaaaagagtctctgagagagtggagaatgaatgttcccacagtcttttacagagccctgacttcagtgtgagtagattagatttgctctatgtagcttacacagagacttctacaggctcaatcccataacaatgaaaatcctcaaaaatgaaaatattttcaaagctcagttcacgtatttgatttttgtatttgcattggaattaaccaaattccagacaatgaagttatactgctttggcaggtctaaatatcacaatcatcaaaaaggagagagagggagtgagcacctcaatttttagaacttcctcttaaagtgaacatagagaaggttcacttatctgtttcctaaccaattaggtcatcttgcaggaaatcaccttttcttaaaagccagtaggcagattcctcctactttaaatttcccatcaacagcattaacaatcatttatgccagccctctcacaggaatgcttgaaagtcaaaagacataagagaccactaagttttctagtttaaaataaggtcacaactttatagtaacttacagtttccctacctccctctctcaagtgattctatcactgcaatcacccttcaattgctttcctatacttgaggccctattaagtaaactatctttccaatccttgccagatttttaattctacaaccagagaggatcagttccaggccacctgacttgcgtgaatccagctgctgggccagttgagtgagattaagtaacttgctgagccagagtatgtgctgtctttctggaaaccccttgccctgggttatcactgtacatcagaacagaggaagccgagtatggagcctgagtgacatgcagagctcagatgagtgataagatcctcatgacacacttccatcggtatcctcccagagatgggcctttgagctctcaagactcttgtgggctggcagaataacacgttatttgacatgagagacatgataagcccagagaaagctaattggagtagtggttaaaactcagttggcctggtttcgaaccctggctgtgtcagtaactaaccatgtgaactggagtgacttagtttctcatagcctcattctgtcaatagggatgttaatattactcacttcataggattgttgtaaggatcaaaagagatgtagctaagatatgaagctcagcaagatttaagcttacatagtgcctagcacatagtaccttaaaaaatattgcctttccaccttgggcaacatagtgagaccctgtctctacagaaaaataaaaataagttagccaatcattgtggcatgtgcctgtggtcccagctactcggtaggctgaggtgggaggattgcttgagcatgggaattcaaggttacagtgggctatgatcatactactgcattccagcctgggcaataagggagaccctttctctaaaaaaaaatttaaaaattgcctttcattatcattaactttcaaggccttgctgttattacttttatggtggattaatatttgtaagaactcctaaaaatacaaatggatatttttaaagtctatagtagactacagtcaagcttgctcactcagggtttcctttggaaacttttctgtggtcatctgtactcatggcccttacttaagacttgggtttacctgtccagaaaacaaccaaatacatgggtacttttttatactattcttattgttttagcgacgcggagtcctttaaatagttgctcctggcccaaatgtggctccaatctctgaagacatcctgtgtcttcctttagacccgagaaactcctacagtttatcaccaaaaaaaaaaaaaaaaaaaaaaagtttgagtgcttaactagcaactcctaattattcacatgtagctttttcttgacaaactttagagcttagcctcccttgatcccatcacttagcaggcatctaagcaactaatttctagagtttacttgaaaaatgtaaacctgttaattttagctaagcaagatagaattaaggatgtaaatctgctgccaaaacaaggatacaatatgattcaaaatttagtggaaataactttttaattagtcatttagtcagtattataagcatcctctgtgtctcagaccttgtgttaagtaactcaggcatgctgacatacatcaggcgtgggtttggcctctttataatatacagtcatatgtcacttaacaatgaagatgggttctgagaaatgcatcattaagcaattttgacattgtgtgaacatcatagaatgtatttacacaaactgagatggtatagcctactacaaacccaggctgtatagtatagcccattgctcctagtctacagacccattcagcatgttgctgtactgaatactataggcaattggaacacagtagtaagtatttgtgtatctaaacacatctaaacagaaaaggtacaataaaaatggtaaaaggattaaaaatggtacacctgtgtagggcacttactatgactgcagcttataggactggagttgctctgggtccgttggtgagtgcacctactgatgaatgaacatgaaggcctaggacactgctgtacactactgtagacttcataaaccccgtatccttaggctatattcattgatagagacatttttctttcttcaataataaattaacctttgat

SEQ ID NO: 13224 - RNA, 4209 nt, Homo sapiens
  source 1..4209: mol_type = other RNA
gctgggattacaggcatgagccaccacactcagccttaaatgaagattttgtaaggaattgagcattcaactaaactcgtttttgtgagatggtcattttgttttaacctaacatggtttagagattattttatgaactctaagcattctggttcctcagttttctcaaagaaagagaactttagcaagtagcaggacaagctaccccacaccaatgccaccaggcgacaatactatgaataagtcaggaggcctcctagaatgcagccaaataggaaactgttccaaacagaatcagtcttgcatacttctgctcagaaggctcctctcgctttggaaactggaatgaggatcaccaacaggatcctcattttacacaggagttatgagagttacatcctctagcagagatgcttggtcattacctgtggtacatgagattaccgagctaaaagggaaaaaaaacgatcttaatgttctcccatgaactcaacttaagctttttatggaggcactgaggccatgcagctccttttccaaaagacacagataaaagccaaataaggtagaggactttggaaattttctctgaaaagttaaattccacataatagtaagactgtttgctgagagaaaactgacaagtaaaaactggtttaagagacagacattcaagacaaactgtattggaaatacaataatgaattttggcctgatagccctcatgctgtcttatagcaaaacactaaaattcatgcaacagagaaattggtgacatgaggactttttctccagacttcctggggaaaaactgtgagaatatacttttttcttctgtttgctttcgaaatgcattctttcttttgctgactttcccaaactttcccagtcgtttctgatgaaaaattcttcaataggaaaagaccaggtaaacttacatgaaagacatcaagtatcttttgagctccttctctctgccagaggagcaatcaactggattacacaaaactaccttcacaactaaaacaggtagaattggaacaggaattagttgtcattaatatactcgtaataaaataaagcttgttctgaaaccacaaggggtggtaagaagagactgtataaaagctactgggttctctagaaaatggatacagtatacagaatgtgagaagatacagaactcacactccagttataaaaatagacatggttctcagacaaaaagcaaatgagtacaaaagaattctccaaacgtgaactatttttaaaagatacatctatataaaacaacaagatgtcatctcagagctccaaagagtagtttgttgaaatggctgaaaaggggagatgaattggagacagataggtcaagaacccagaacagatgtgtcctactcttgtgtttggcagtgtacattggaggtcacaggcagatagactgcttttggtaatacatatataaataataatggctgactggttgatggtgcttgatggatgaatgagaaaacccaggttatcaaataatctcggtagttgaactgttagcttcttcacttgacaatgttgcacatcagaaatgattctaggttttttttacccagaatgatccctgccattcacaactcatgctccacgccccatggtttctattgtgccctaaaagatcagcctagactaatacataaatagaaaataactctggccttgaaatgaggggcagacaagtacttcatgctcagtacttataaatcacaaagaaatgctgaaattaatggtctgtctccttttactacaaaggagatgccatgagttaaagtcatgaaacaaagaaagtcaaaaagatatgggtagcagcacctttccatacccgcctggattttcaaggagcttttcactccttatgcctttcaaacaaaagttcatcagtttgaagaaaaagaaatggctctaaagttaaagagtccccagagaaaactaacagtacatgaaataggccctatgtgggcaaaaggacaagctgcagaaccagttaagacagaagaggcagcccaaggtcttactaaattacagttttagcatagtgtagcacaacatgggcagccctttttccatccaagcaacaattcagcaccatccacgtctggttcaaaagattactgaagtctgggctttcatctttggtaccacctcatgagttattcttggtttgcagtaggttcaaagaaacagaaaagctggtacctttgccttgtctgtgagtacaaacgctgggactctgattgctgcaaccattgaggccaattaaaataatactgtaacacacaggaatgatgcatccaattcctaatttccagataatagcagccatgcccctacagaggcgggatcatccatccccatcgtttaaggccttcggtttgttgtcctcagagtagaatagaacactgtgttcccacggacaaggaactccagatgaacccatggtctacatttggacagaattttaagtaccagatatgccaggcacagaaagaggactgacctgtggccatcatgcttggagaagcttctgttttggcacacaaactagaaacttcttagtgtattctggttttagttccctttcctgagtgaagcagccagggagtgaccaggttccataagccctcaatctgatacttggcattaattctctccatggtcttcttccacccaagctacaattttcccttcccatccagggatggcatcatcatcatggaaaatctcctctttgacagtgccaaactcaggatccagtgctttgaagtgataccggtgatttccttcccgatcaatagctgctttaaaatcctttaacgtcacctcctccaacctctttggtatattgaccatgaagggcgtaagtgaccggtcagtgaaatagagcactttagtacaggtgctgctgacagttggagagctctgtgagtgaggcaactttgagttagggggccaggactcccggtattcactacctacttgagttctgggtgacttgacccgaacctttctttcttgtttcttctgcgtctccataacatgcaggcgctccatgaggctagaaatgccctgctccaagctgtcaatagtgtggtgctgaggatcgtggccactgaagctgttgcgcaggctgcggagagcatctcgaacaagctgcaggtcgctggtccctctgttgctgactgaagtagctccttttcctgccgttggaaggagaaaaccattgctttgagagttgtgactgttgtagttggtcgcctcatctgcctctcttttcatacagtgagccaagaggacatctttgtgttctagctctcgctctagatccacctggtggtaactgacatcagagagtttccggagtgcttcttctaacttggcctggtgctgctgaagaaggcgatccttctgccccagctcttttttatattctcccaagagccggttcctctcatctagcttcctctgcagatccacattctggttgtgcagctcatctttgtccatatttgccctcagtagctcttgtttgagctgaagaacagatgtgtcctgctgagtcaatctctgctgcaaggcatcctttatcccctgtaagtttctggcttcttgtttacatttcagcagttccttctttaagtcctgattctcctccatactctgatccagacgactttggattataatcagttgttcctcgggattgacacctggttcacagagggccaagggcctctcctgttcatcttcaggtaaggatccattgagcagtaaggccctgggactagttcctttcgttaggtccatgctctggctctttcagctctctggacacctgactgctctgcttcaaggtgccttggccccagaagaaaatctgtagtcctgatatcattttctttgcttcctccatttctttttctaaatattcttgttgttccaacagctgttcttcccatgaggtctccagataggttccagggctccctggccgccagtctcgagataatggagaatctgtcccttctgttctgttctctattccttcagcgggaataatcacaaaatctgccttctcttctgactgggttataatggactcgctctttgcactgtggattggactgggtgaagtcaggcatttgacttgcgtccctccca

SEQ ID NO: 13225 - RNA, 4537 nt, Homo sapiens
  source 1..4537: mol_type = other RNA
gctgggattacaggcatgagccaccacactcagccttaaatgaagattttgtaaggaattgagcattcaactaaactcgtttttgtgagatggtcattttgttttaacctaacatggtttagagattattttatgaactctaagcattctggttcctcagttttctcaaagaaagagaactttagcaagtagcaggacaagctaccccacaccaatgccaccaggcgacaatactatgaataagtcaggaggcctcctagaatgcagccaaataggaaactgttccaaacagaatcagtcttgcatacttctgctcagaaggctcctctcgctttggaaactggaatgaggatcaccaacaggatcctcattttacacaggagttatgagagttacatcctctagcagagatgcttggtcattacctgtggtacatgagattaccgagctaaaagggaaaaaaaacgatcttaatgttctcccatgaactcaacttaagctttttatggaggcactgaggccatgcagctccttttccaaaagacacagataaaagccaaataaggtagaggactttggaaattttctctgaaaagttaaattccacataatagtaagactgtttgctgagagaaaactgacaagtaaaaactggtttaagagacagacattcaagacaaactgtattggaaatacaataatgaattttggcctgatagccctcatgctgtcttatagcaaaacactaaaattcatgcaacagagaaattggtgacatgaggactttttctccagacttcctggggaaaaactgtgagaatatacttttttcttctgtttgctttcgaaatgcattctttcttttgctgactttcccaaactttcccagtcgtttctgatgaaaaattcttcaataggaaaagaccaggtaaacttacatgaaagacatcaagtatcttttgagctccttctctctgccagaggagcaatcaactggattacacaaaactaccttcacaactaaaacaggtagaattggaacaggaattagttgtcattaatatactcgtaataaaataaagcttgttctgaaaccacaaggggtggtaagaagagactgtataaaagctactgggttctctagaaaatggatacagtatacagaatgtgagaagatacagaactcacactccagttataaaaatagacatggttctcagacaaaaagcaaatgagtacaaaagaattctccaaacgtgaactatttttaaaagatacatctatataaaacaacaagatgtcatctcagagctccaaagagtagtttgttgaaatggctgaaaaggggagatgaattggagacagataggtcaagaacccagaacagatgtgtcctactcttgtgtttggcagtgtacattggaggtcacaggcagatagactgcttttggtaatacatatataaataataatggctgactggttgatggtgcttgatggatgaatgagaaaacccaggttatcaaataatctcggtagttgaactgttagcttcttcacttgacaatgttgcacatcagaaatgattctaggttttttttacccagaatgatccctgccattcacaactcatgctccacgccccatggtttctattgtgccctaaaagatcagcctagactaatacataaatagaaaataactctggccttgaaatgaggggcagacaagtacttcatgctcagtacttataaatcacaaagaaatgctgaaattaatggtctgtctccttttactacaaaggagatgccatgagttaaagtcatgaaacaaagaaagtcaaaaagatatgggtagcagcacctttccatacccgcctggattttcaaggagcttttcactccttatgcctttcaaacaaaagttcatcagtttgaagaaaaagaaatggctctaaagttaaagagtccccagagaaaactaacagtacatgaaataggccctatgtgggcaaaaggacaagctgcagaaccagttaagacagaagaggcagcccaaggtcttactaaattacagttttagcatagtgtagcacaacatgggcagccctttttccatccaagcaacaattcagcaccatccacgtctggttcaaaagattactgaagtctgggctttcatctttggtaccacctcatgagttattcttggtttgcagtaggttcaaagaaacagaaaagctggtacctttgccttgtctgtgagtacaaacgctgggactctgattgctgcaaccattgaggccaattaaaataatactgtaacacacaggaatgatgcatccaattcctaatttccagataatagcagccatgcccctacagaggcgggatcatccatccccatcgtttaaggccttcggtttgttgtcctcagagtagaatagaacactgtgttcccacggacaaggaactccagatgaacccatggtctacatttggacagaattttaagtaccagatatgccaggcacagaaagaggactgacctgtggccatcatgcttggagaagcttctgttttggcacacaaactagaaacttcttagtgtattctggttttagttccctttcctgagtgaagcagccagggagtgaccaggttccataagccctcaatctgatacttggcattaattctctccatggtcttcttccacccaagctacaattttcccttcccatccagggatggcatcatcatcatggaaaatctcctctttgacagtgccaaactcaggatccagtgctttgaagtgataccggtgatttccttcccgatcaatagctgctttaaaatcctttaacgtcacctcctccaacctctttggtatattgaccatgaagggcgtaagtgaccggtcagtgaaatagagcactttagtacaggtgctgctgacagttggagagctctgtgagtgaggcaactttgagttagggggccaggactcccggtattcactacctacttgagttctgggtgacttgacccgaacctttctttcttgtttcttctgcgtctccataacatgcaggcgctccatgaggctagaaatgccctgctccaagctgtcaatagtgtggtgctgaggatcgtggccactgaagctgttgcgcaggctgcggagagcatctcgaacaagctgcaggtcgctggtccctctgttgctgactgaagtagctccttttcctgccgttggaaggagaaaaccattgctttgagagttgtgactgttgtagttggtcgcctcatctgcctctcttttcatacagtgagccaagaggacatctttgtgttctagctctcgctctagatccacctggtggtaactgacatcagagagtttccggagtgcttcttctaacttggcctggtgctgctgaagaaggcgatccttctgccccagctcttttttatattctcccaagagccggttcctctcatctagcttcctctgcagatccacattctggttgtgcagctcatctttgtccatatttgccctcagtagctcttgtttgagctgaagaacagatgtgtcctgctgagtcaatctctgctgcaaggcatcctttatcccctgtaagtttctggcttcttgtttacatttcagcagttccttctttaagtcctgattctcctccatactctgatccagacgactttggattataatcagttgttcctcgggattgacacctggttcacagagggccaagggcctctcctgttcatcttcaggtaaggatccattgagcagtaaggcctgtagtcctgatatcattttctttgcttcctccatttctttttctaaatattcttgttgttccaacagctgttcttcccatgaggtctccagataggttccagggctccctggccgccagtctcgagataatggagaatctgtcccttctgttctgttctctattccttcagcgggaataatcacaaaatctgccttctcttctgactgggttataatggactcgctctttgcactgtggattggactgggtgaagtcaggcatttgacttgcgtccctcccatggtccccctcctgtctcgggcttcagcaagcctgcgtccccgggtgaagtgggaggctgagagtcacatcgctcccaaattcaggcatgtctccccgcgctggggctggaaaacgcctccacgggaaggccagctagcaaagctactggcccggctcgcgggagaaagcgggaacggcggcggcggcggcgtctcggccccagcgactgggatgctccaggctctgaagcgcgcagtcccggccgctcagactgtgcagcagcccggccccggcggaagctgcctcccctcgcaggctgccggcccctggccgctgcatcttggcctccgcggacgcacggtgccgggcatcccccctggcgggggcatctcaacccatctcccactgggagggaggctcccggcggcgcaggctgcgcctcgagtc

SEQ ID NO: 13226 - RNA, 4887 nt, Homo sapiens
  source 1..4887: mol_type = other RNA
gctgggattacaggcatgagccaccacactcagccttaaatgaagattttgtaaggaattgagcattcaactaaactcgtttttgtgagatggtcattttgttttaacctaacatggtttagagattattttatgaactctaagcattctggttcctcagttttctcaaagaaagagaactttagcaagtagcaggacaagctaccccacaccaatgccaccaggcgacaatactatgaataagtcaggaggcctcctagaatgcagccaaataggaaactgttccaaacagaatcagtcttgcatacttctgctcagaaggctcctctcgctttggaaactggaatgaggatcaccaacaggatcctcattttacacaggagttatgagagttacatcctctagcagagatgcttggtcattacctgtggtacatgagattaccgagctaaaagggaaaaaaaacgatcttaatgttctcccatgaactcaacttaagctttttatggaggcactgaggccatgcagctccttttccaaaagacacagataaaagccaaataaggtagaggactttggaaattttctctgaaaagttaaattccacataatagtaagactgtttgctgagagaaaactgacaagtaaaaactggtttaagagacagacattcaagacaaactgtattggaaatacaataatgaattttggcctgatagccctcatgctgtcttatagcaaaacactaaaattcatgcaacagagaaattggtgacatgaggactttttctccagacttcctggggaaaaactgtgagaatatacttttttcttctgtttgctttcgaaatgcattctttcttttgctgactttcccaaactttcccagtcgtttctgatgaaaaattcttcaataggaaaagaccaggtaaacttacatgaaagacatcaagtatcttttgagctccttctctctgccagaggagcaatcaactggattacacaaaactaccttcacaactaaaacaggtagaattggaacaggaattagttgtcattaatatactcgtaataaaataaagcttgttctgaaaccacaaggggtggtaagaagagactgtataaaagctactgggttctctagaaaatggatacagtatacagaatgtgagaagatacagaactcacactccagttataaaaatagacatggttctcagacaaaaagcaaatgagtacaaaagaattctccaaacgtgaactatttttaaaagatacatctatataaaacaacaagatgtcatctcagagctccaaagagtagtttgttgaaatggctgaaaaggggagatgaattggagacagataggtcaagaacccagaacagatgtgtcctactcttgtgtttggcagtgtacattggaggtcacaggcagatagactgcttttggtaatacatatataaataataatggctgactggttgatggtgcttgatggatgaatgagaaaacccaggttatcaaataatctcggtagttgaactgttagcttcttcacttgacaatgttgcacatcagaaatgattctaggttttttttacccagaatgatccctgccattcacaactcatgctccacgccccatggtttctattgtgccctaaaagatcagcctagactaatacataaatagaaaataactctggccttgaaatgaggggcagacaagtacttcatgctcagtacttataaatcacaaagaaatgctgaaattaatggtctgtctccttttactacaaaggagatgccatgagttaaagtcatgaaacaaagaaagtcaaaaagatatgggtagcagcacctttccatacccgcctggattttcaaggagcttttcactccttatgcctttcaaacaaaagttcatcagtttgaagaaaaagaaatggctctaaagttaaagagtccccagagaaaactaacagtacatgaaataggccctatgtgggcaaaaggacaagctgcagaaccagttaagacagaagaggcagcccaaggtcttactaaattacagttttagcatagtgtagcacaacatgggcagccctttttccatccaagcaacaattcagcaccatccacgtctggttcaaaagattactgaagtctgggctttcatctttggtaccacctcatgagttattcttggtttgcagtaggttcaaagaaacagaaaagctggtacctttgccttgtctgtgagtacaaacgctgggactctgattgctgcaaccattgaggccaattaaaataatactgtaacacacaggaatgatgcatccaattcctaatttccagataatagcagccatgcccctacagaggcgggatcatccatccccatcgtttaaggccttcggtttgttgtcctcagagtagaatagaacactgtgttcccacggacaaggaactccagatgaacccatggtctacatttggacagaattttaagtaccagatatgccaggcacagaaagaggactgacctgtggccatcatgcttggagaagcttctgttttggcacacaaactagaaacttcttagtgtattctggttttagttccctttcctgagtgaagcagccagggagtgaccaggttccataagccctcaatctgatacttggcattaattctctccatggtcttcttccacccaagctacaattttcccttcccatccagggatggcatcatcatcatggaaaatctcctctttgacagtgccaaactcaggatccagtgctttgaagtgataccggtgatttccttcccgatcaatagctgctttaaaatcctttaacgtcacctcctccaacctctttggtatattgaccatgaagggcgtaagtgaccggtcagtgaaatagagcactttagtacaggtgctgctgacagttggagagctctgtgagtgaggcaactttgagttagggggccaggactcccggtattcactacctacttgagttctgggtgacttgacccgaacctttctttcttgtttcttctgcgtctccataacatgcaggcgctccatgaggctagaaatgccctgctccaagctgtcaatagtgtggtgctgaggatcgtggccactgaagctgttgcgcaggctgcggagagcatctcgaacaagctgcaggtcgctggtccctctgttgctgactgaagtagctccttttcctgccgttggaaggagaaaaccattgctttgagagttgtgactgttgtagttggtcgcctcatctgcctctcttttcatacagtgagccaagaggacatctttgtgttctagctctcgctctagatccacctggtggtaactgacatcagagagtttccggagtgcttcttctaacttggcctggtgctgctgaagaaggcgatccttctgccccagctcttttttatattctcccaagagccggttcctctcatctagcttcctctgcagatccacattctggttgtgcagctcatctttgtccatatttgccctcagtagctcttgtttgagctgaagaacagatgtgtcctgctgagtcaatctctgctgcaaggcatcctttatcccctgtaagtttctggcttcttgtttacatttcagcagttccttctttaagtcctgattctcctccatactctgatccagacgactttggattataatcagttgttcctcgggattgacacctggttcacagagggccaagggcctctcctgttcatcttcaggtaaggatccattgagcagtaaggcctgtagtcctgatatcattttctttgcttcctccatttctttttctaaatattcttgttgttccaacagctgttcttcccatgaggtctccagataggttccagggctccctggccgccagtctcgagataatggagaatctgtcccttctgttctgttctctattccttcagcgggaataatcacaaaatctgccttctcttctgactgggttataatggactcgctctttgcactgtggattggactgggtgaagtcaggctctgtctatatcgaaagacatcccgtcctgatcgggacatgtcatgacacacatcggccagagcagcagctgctccctgggcaacagcagtggcacagtgtggtcggtgactttgcagaggggctctggagtcccgtccttggttcaccgtcctgctggagccaggtttgaaatgagctgccaaggcaaggaccagcctcatgatagacttcaggtttccatccacaatatctttagccgaagtctggtgcatacgaatctttttagaggccacaaactgtagcactttctccacattattcttcatctcctgttggttaccgggactcagctgtaccccactcagcttttctcctgcaacaatctcgatgagatatgccaggatcaccccatcccggagatcttgtcgcaggtcctgcacaggcttcactgctggcctcttcttcagctgtgcattcacccaggccacataggcctgcagctgttgagaaggctctgttggcagcaaggagttattgaatctcataaccacttgggtccccatcttcaagagtccctagaagagacgaatcagggccatctcttaaatgatgggtccgtctggttcagcatctctgtccccagccctcctgagctcggcctgccagtgctctggctttgccgcggtttcccgctgccatggtgatgcgggggccggccacaagccccgcccgactccagccagccagagccagcccctgccggccttggtcccgcctctggcccgccggatcccgcctcctgcaggcccagaccgcgc

SEQ ID NO: 13227 - RNA, 5189 nt, Homo sapiens
  source 1..5189: mol_type = other RNA
gctgggattacaggcatgagccaccacactcagccttaaatgaagattttgtaaggaattgagcattcaactaaactcgtttttgtgagatggtcattttgttttaacctaacatggtttagagattattttatgaactctaagcattctggttcctcagttttctcaaagaaagagaactttagcaagtagcaggacaagctaccccacaccaatgccaccaggcgacaatactatgaataagtcaggaggcctcctagaatgcagccaaataggaaactgttccaaacagaatcagtcttgcatacttctgctcagaaggctcctctcgctttggaaactggaatgaggatcaccaacaggatcctcattttacacaggagttatgagagttacatcctctagcagagatgcttggtcattacctgtggtacatgagattaccgagctaaaagggaaaaaaaacgatcttaatgttctcccatgaactcaacttaagctttttatggaggcactgaggccatgcagctccttttccaaaagacacagataaaagccaaataaggtagaggactttggaaattttctctgaaaagttaaattccacataatagtaagactgtttgctgagagaaaactgacaagtaaaaactggtttaagagacagacattcaagacaaactgtattggaaatacaataatgaattttggcctgatagccctcatgctgtcttatagcaaaacactaaaattcatgcaacagagaaattggtgacatgaggactttttctccagacttcctggggaaaaactgtgagaatatacttttttcttctgtttgctttcgaaatgcattctttcttttgctgactttcccaaactttcccagtcgtttctgatgaaaaattcttcaataggaaaagaccaggtaaacttacatgaaagacatcaagtatcttttgagctccttctctctgccagaggagcaatcaactggattacacaaaactaccttcacaactaaaacaggtagaattggaacaggaattagttgtcattaatatactcgtaataaaataaagcttgttctgaaaccacaaggggtggtaagaagagactgtataaaagctactgggttctctagaaaatggatacagtatacagaatgtgagaagatacagaactcacactccagttataaaaatagacatggttctcagacaaaaagcaaatgagtacaaaagaattctccaaacgtgaactatttttaaaagatacatctatataaaacaacaagatgtcatctcagagctccaaagagtagtttgttgaaatggctgaaaaggggagatgaattggagacagataggtcaagaacccagaacagatgtgtcctactcttgtgtttggcagtgtacattggaggtcacaggcagatagactgcttttggtaatacatatataaataataatggctgactggttgatggtgcttgatggatgaatgagaaaacccaggttatcaaataatctcggtagttgaactgttagcttcttcacttgacaatgttgcacatcagaaatgattctaggttttttttacccagaatgatccctgccattcacaactcatgctccacgccccatggtttctattgtgccctaaaagatcagcctagactaatacataaatagaaaataactctggccttgaaatgaggggcagacaagtacttcatgctcagtacttataaatcacaaagaaatgctgaaattaatggtctgtctccttttactacaaaggagatgccatgagttaaagtcatgaaacaaagaaagtcaaaaagatatgggtagcagcacctttccatacccgcctggattttcaaggagcttttcactccttatgcctttcaaacaaaagttcatcagtttgaagaaaaagaaatggctctaaagttaaagagtccccagagaaaactaacagtacatgaaataggccctatgtgggcaaaaggacaagctgcagaaccagttaagacagaagaggcagcccaaggtcttactaaattacagttttagcatagtgtagcacaacatgggcagccctttttccatccaagcaacaattcagcaccatccacgtctggttcaaaagattactgaagtctgggctttcatctttggtaccacctcatgagttattcttggtttgcagtaggttcaaagaaacagaaaagctggtacctttgccttgtctgtgagtacaaacgctgggactctgattgctgcaaccattgaggccaattaaaataatactgtaacacacaggaatgatgcatccaattcctaatttccagataatagcagccatgcccctacagaggcgggatcatccatccccatcgtttaaggccttcggtttgttgtcctcagagtagaatagaacactgtgttcccacggacaaggaactccagatgaacccatggtctacatttggacagaattttaagtaccagatatgccaggcacagaaagaggactgacctgtggccatcatgcttggagaagcttctgttttggcacacaaactagaaacttcttagtgtattctggttttagttccctttcctgagtgaagcagccagggagtgaccaggttccataagccctcaatctgatacttggcattaattctctccatggtcttcttccacccaagctacaattttcccttcccatccagggatggcatcatcatcatggaaaatctcctctttgacagtgccaaactcaggatccagtgctttgaagtgataccggtgatttccttcccgatcaatagctgctttaaaatcctttaacgtcacctcctccaacctctttggtatattgaccatgaagggcgtaagtgaccggtcagtgaaatagagcactttagtacaggtgctgctgacagttggagagctctgtgagtgaggcaactttgagttagggggccaggactcccggtattcactacctacttgagttctgggtgacttgacccgaacctttctttcttgtttcttctgcgtctccataacatgcaggcgctccatgaggctagaaatgccctgctccaagctgtcaatagtgtggtgctgaggatcgtggccactgaagctgttgcgcaggctgcggagagcatctcgaacaagctgcaggtcgctggtccctctgttgctgactgaagtagctccttttcctgccgttggaaggagaaaaccattgctttgagagttgtgactgttgtagttggtcgcctcatctgcctctcttttcatacagtgagccaagaggacatctttgtgttctagctctcgctctagatccacctggtggtaactgacatcagagagtttccggagtgcttcttctaacttggcctggtgctgctgaagaaggcgatccttctgccccagctcttttttatattctcccaagagccggttcctctcatctagcttcctctgcagatccacattctggttgtgcagctcatctttgtccatatttgccctcagtagctcttgtttgagctgaagaacagatgtgtcctgctgagtcaatctctgctgcaaggcatcctttatcccctgtaagtttctggcttcttgtttacatttcagcagttccttctttaagtcctgattctcctccatactctgatccagacgactttggattataatcagttgttcctcgggattgacacctggttcacagagggccaagggcctctcctgttcatcttcaggtaaggatccattgagcagtaaggcctgtagtcctgatatcattttctttgcttcctccatttctttttctaaatattcttgttgttccaacagctgttcttcccatgaggtctccagataggttccagggctccctggccgccagtctcgagataatggagaatctgtcccttctgttctgttctctattccttcagcgggaataatcacaaaatctgccttctcttctgactgggttataatggactcgctctttgcactgtggattggactgggtgaagtcaggctctgtctatatcgaaagacatcccgtcctgatcgggacatgtcatgacacacatcggccagagcagcagctgctccctgggcaacagcagtggcacagtgtggtcggtgactttgcagaggggctctggagtcccgtccttggttcaccgtcctgctggagccaggtttgaaatgagctgccaaggcaaggaccagcctcatgatagacttcaggtttccatccacaatatctttagccgaagtctggtgcatacgaatctttttagaggccacaaactgtagcactttctccacattattcttcatctcctgttggttaccgggactcagctgtaccccactcagcttttctcctgcaacaatctcgatgagatatgccaggatcaccccatcccggagatcttgtcgcaggtcctgcacaggcttcactgctggcctcttcttcagctgtgcattcacccaggccacataggcctgcagctgttgctcattgaagccctcctgcaggacgtccagtaagttccctcgggtcaggcaggctagcattgttcctgctgggggctccccgggcggggtctccagcccggcggccgccgccgcctcctcctcctccctctgcacacaaaggctctcggctcagctcattgggatccctccggagtcccgcatgccacttactggaaacctagactggagccaaactagcggcttgcactgggcatgctcgcacgggggcctccgctggaggggcccggcgcggtcgcggttcctatggaaacaactgggcgcgcactaggttgagcggcgctgccgggctgcccccagccccgctttcctgcgggaaagccgcacggccaggcgggctggcgagggcgcgcgctgcacgcccgcacgcacgcgcacaccccccccccgcccgggccgcagcacgggcgtgtgtgcgtgcgctacacacacacacactcacacggcttttaggcaaacgtgctgctgtatgtgcgcgctgtgtgcatacacacacacacacacatacacacatacacacatacacacacacacgttgacaaacaggcggcccggctggcgtatgcatgcgcttg

SEQ ID NO: 13228 - RNA, 4995 nt, Homo sapiens
  source 1..4995: mol_type = other RNA
gctgggattacaggcatgagccaccacactcagccttaaatgaagattttgtaaggaattgagcattcaactaaactcgtttttgtgagatggtcattttgttttaacctaacatggtttagagattattttatgaactctaagcattctggttcctcagttttctcaaagaaagagaactttagcaagtagcaggacaagctaccccacaccaatgccaccaggcgacaatactatgaataagtcaggaggcctcctagaatgcagccaaataggaaactgttccaaacagaatcagtcttgcatacttctgctcagaaggctcctctcgctttggaaactggaatgaggatcaccaacaggatcctcattttacacaggagttatgagagttacatcctctagcagagatgcttggtcattacctgtggtacatgagattaccgagctaaaagggaaaaaaaacgatcttaatgttctcccatgaactcaacttaagctttttatggaggcactgaggccatgcagctccttttccaaaagacacagataaaagccaaataaggtagaggactttggaaattttctctgaaaagttaaattccacataatagtaagactgtttgctgagagaaaactgacaagtaaaaactggtttaagagacagacattcaagacaaactgtattggaaatacaataatgaattttggcctgatagccctcatgctgtcttatagcaaaacactaaaattcatgcaacagagaaattggtgacatgaggactttttctccagacttcctggggaaaaactgtgagaatatacttttttcttctgtttgctttcgaaatgcattctttcttttgctgactttcccaaactttcccagtcgtttctgatgaaaaattcttcaataggaaaagaccaggtaaacttacatgaaagacatcaagtatcttttgagctccttctctctgccagaggagcaatcaactggattacacaaaactaccttcacaactaaaacaggtagaattggaacaggaattagttgtcattaatatactcgtaataaaataaagcttgttctgaaaccacaaggggtggtaagaagagactgtataaaagctactgggttctctagaaaatggatacagtatacagaatgtgagaagatacagaactcacactccagttataaaaatagacatggttctcagacaaaaagcaaatgagtacaaaagaattctccaaacgtgaactatttttaaaagatacatctatataaaacaacaagatgtcatctcagagctccaaagagtagtttgttgaaatggctgaaaaggggagatgaattggagacagataggtcaagaacccagaacagatgtgtcctactcttgtgtttggcagtgtacattggaggtcacaggcagatagactgcttttggtaatacatatataaataataatggctgactggttgatggtgcttgatggatgaatgagaaaacccaggttatcaaataatctcggtagttgaactgttagcttcttcacttgacaatgttgcacatcagaaatgattctaggttttttttacccagaatgatccctgccattcacaactcatgctccacgccccatggtttctattgtgccctaaaagatcagcctagactaatacataaatagaaaataactctggccttgaaatgaggggcagacaagtacttcatgctcagtacttataaatcacaaagaaatgctgaaattaatggtctgtctccttttactacaaaggagatgccatgagttaaagtcatgaaacaaagaaagtcaaaaagatatgggtagcagcacctttccatacccgcctggattttcaaggagcttttcactccttatgcctttcaaacaaaagttcatcagtttgaagaaaaagaaatggctctaaagttaaagagtccccagagaaaactaacagtacatgaaataggccctatgtgggcaaaaggacaagctgcagaaccagttaagacagaagaggcagcccaaggtcttactaaattacagttttagcatagtgtagcacaacatgggcagccctttttccatccaagcaacaattcagcaccatccacgtctggttcaaaagattactgaagtctgggctttcatctttggtaccacctcatgagttattcttggtttgcagtaggttcaaagaaacagaaaagctggtacctttgccttgtctgtgagtacaaacgctgggactctgattgctgcaaccattgaggccaattaaaataatactgtaacacacaggaatgatgcatccaattcctaatttccagataatagcagccatgcccctacagaggcgggatcatccatccccatcgtttaaggccttcggtttgttgtcctcagagtagaatagaacactgtgttcccacggacaaggaactccagatgaacccatggtctacatttggacagaattttaagtaccagatatgccaggcacagaaagaggactgacctgtggccatcatgcttggagaagcttctgttttggcacacaaactagaaacttcttagtgtattctggttttagttccctttcctgagtgaagcagccagggagtgaccaggttccataagccctcaatctgatacttggcattaattctctccatggtcttcttccacccaagctacaattttcccttcccatccagggatggcatcatcatcatggaaaatctcctctttgacagtgccaaactcaggatccagtgctttgaagtgataccggtgatttccttcccgatcaatagctgctttaaaatcctttaacgtcacctcctccaacctctttggtatattgaccatgaagggcgtaagtgaccggtcagtgaaatagagcactttagtacaggtgctgctgacagttggagagctctgtgagtgaggcaactttgagttagggggccaggactcccggtattcactacctacttgagttctgggtgacttgacccgaacctttctttcttgtttcttctgcgtctccataacatgcaggcgctccatgaggctagaaatgccctgctccaagctgtcaatagtgtggtgctgaggatcgtggccactgaagctgttgcgcaggctgcggagagcatctcgaacaagctgcaggtcgctggtccctctgttgctgactgaagtagctccttttcctgccgttggaaggagaaaaccattgctttgagagttgtgactgttgtagttggtcgcctcatctgcctctcttttcatacagtgagccaagaggacatctttgtgttctagctctcgctctagatccacctggtggtaactgacatcagagagtttccggagtgcttcttctaacttggcctggtgctgctgaagaaggcgatccttctgccccagctcttttttatattctcccaagagccggttcctctcatctagcttcctctgcagatccacattctggttgtgcagctcatctttgtccatatttgccctcagtagctcttgtttgagctgaagaacagatgtgtcctgctgagtcaatctctgctgcaaggcatcctttatcccctgtaagtttctggcttcttgtttacatttcagcagttccttctttaagtcctgattctcctccatactctgatccagacgactttggattataatcagttgttcctcgggattgacacctggttcacagagggccaagggcctctcctgttcatcttcaggtaaggatccattgagcagtaaggcctgtagtcctgatatcattttctttgcttcctccatttctttttctaaatattcttgttgttccaacagctgttcttcccatgaggtctccagataggttccagggctccctggccgccagtctcgagataatggagaatctgtcccttctgttctgttctctattccttcagcgggaataatcacaaaatctgccttctcttctgactgggttataatggactcgctctttgcactgtggattggactgggtgaagtcaggctggagcagctggattcagacggggacctttgttgcccttcgtactgctgcactagggcccgcacactccagtatggattctcaatttcctcatccatgctgctgttcctctgtctatatcgaaagacatcccgtcctgatcgggacatgtcatgacacacatcggccagagcagcagctgctccctgggcaacagcagtggcacagtgtggtcggtgactttgcagaggggctctggagtcccgtccttggttcaccgtcctgctggagccaggtttgaaatgagctgccaaggcaaggaccagcctcatgatagacttcaggtttccatccacaatatctttagccgaagtctggtgcatacgaatctttttagaggccacaaactgtagcactttctccacattattcttcatctcctgttggttaccgggactcagctgtaccccactcagcttttctcctgcaacaatctcgatgagatatgccaggatcaccccatcccggagatcttgtcgcaggtcctgcacaggcttcactgctggcctcttcttcagctgtgcattcacccaggccacataggcctgcagctgttgagaaggctctgttggcagcaaggagttattgaatctcataaccacttgggtccccatcttcaagagtccctagaagagacgaatcagggccatctcttaaatgatgggtccgtctggttcagcatctctgtccccagccctcctgagctcggcctgccagtgctctggctttgccgcggtttcccgctgccatggtgatgcgggggccggccacaagccccgcccgactccagccagccagagccagcccctgccggccttggtcccgcctctggcccgccggatcccgcctcctgcaggcccagaccgcgc

SEQ ID NO: 13229 - RNA, 4868 nt, Homo sapiens
  source 1..4868: mol_type = other RNA
gctgggattacaggcatgagccaccacactcagccttaaatgaagattttgtaaggaattgagcattcaactaaactcgtttttgtgagatggtcattttgttttaacctaacatggtttagagattattttatgaactctaagcattctggttcctcagttttctcaaagaaagagaactttagcaagtagcaggacaagctaccccacaccaatgccaccaggcgacaatactatgaataagtcaggaggcctcctagaatgcagccaaataggaaactgttccaaacagaatcagtcttgcatacttctgctcagaaggctcctctcgctttggaaactggaatgaggatcaccaacaggatcctcattttacacaggagttatgagagttacatcctctagcagagatgcttggtcattacctgtggtacatgagattaccgagctaaaagggaaaaaaaacgatcttaatgttctcccatgaactcaacttaagctttttatggaggcactgaggccatgcagctccttttccaaaagacacagataaaagccaaataaggtagaggactttggaaattttctctgaaaagttaaattccacataatagtaagactgtttgctgagagaaaactgacaagtaaaaactggtttaagagacagacattcaagacaaactgtattggaaatacaataatgaattttggcctgatagccctcatgctgtcttatagcaaaacactaaaattcatgcaacagagaaattggtgacatgaggactttttctccagacttcctggggaaaaactgtgagaatatacttttttcttctgtttgctttcgaaatgcattctttcttttgctgactttcccaaactttcccagtcgtttctgatgaaaaattcttcaataggaaaagaccaggtaaacttacatgaaagacatcaagtatcttttgagctccttctctctgccagaggagcaatcaactggattacacaaaactaccttcacaactaaaacaggtagaattggaacaggaattagttgtcattaatatactcgtaataaaataaagcttgttctgaaaccacaaggggtggtaagaagagactgtataaaagctactgggttctctagaaaatggatacagtatacagaatgtgagaagatacagaactcacactccagttataaaaatagacatggttctcagacaaaaagcaaatgagtacaaaagaattctccaaacgtgaactatttttaaaagatacatctatataaaacaacaagatgtcatctcagagctccaaagagtagtttgttgaaatggctgaaaaggggagatgaattggagacagataggtcaagaacccagaacagatgtgtcctactcttgtgtttggcagtgtacattggaggtcacaggcagatagactgcttttggtaatacatatataaataataatggctgactggttgatggtgcttgatggatgaatgagaaaacccaggttatcaaataatctcggtagttgaactgttagcttcttcacttgacaatgttgcacatcagaaatgattctaggttttttttacccagaatgatccctgccattcacaactcatgctccacgccccatggtttctattgtgccctaaaagatcagcctagactaatacataaatagaaaataactctggccttgaaatgaggggcagacaagtacttcatgctcagtacttataaatcacaaagaaatgctgaaattaatggtctgtctccttttactacaaaggagatgccatgagttaaagtcatgaaacaaagaaagtcaaaaagatatgggtagcagcacctttccatacccgcctggattttcaaggagcttttcactccttatgcctttcaaacaaaagttcatcagtttgaagaaaaagaaatggctctaaagttaaagagtccccagagaaaactaacagtacatgaaataggccctatgtgggcaaaaggacaagctgcagaaccagttaagacagaagaggcagcccaaggtcttactaaattacagttttagcatagtgtagcacaacatgggcagccctttttccatccaagcaacaattcagcaccatccacgtctggttcaaaagattactgaagtctgggctttcatctttggtaccacctcatgagttattcttggtttgcagtaggttcaaagaaacagaaaagctggtacctttgccttgtctgtgagtacaaacgctgggactctgattgctgcaaccattgaggccaattaaaataatactgtaacacacaggaatgatgcatccaattcctaatttccagataatagcagccatgcccctacagaggcgggatcatccatccccatcgtttaaggccttcggtttgttgtcctcagagtagaatagaacactgtgttcccacggacaaggaactccagatgaacccatggtctacatttggacagaattttaagtaccagatatgccaggcacagaaagaggactgacctgtggccatcatgcttggagaagcttctgttttggcacacaaactagaaacttcttagtgtattctggttttagttccctttcctgagtgaagcagccagggagtgaccaggttccataagccctcaatctgatacttggcattaattctctccatggtcttcttccacccaagctacaattttcccttcccatccagggatggcatcatcatcatggaaaatctcctctttgacagtgccaaactcaggatccagtgctttgaagtgataccggtgatttccttcccgatcaatagctgctttaaaatcctttaacgtcacctcctccaacctctttggtatattgaccatgaagggcgtaagtgaccggtcagtgaaatagagcactttagtacaggtgctgctgacagttggagagctctgtgagtgaggcaactttgagttagggggccaggactcccggtattcactacctacttgagttctgggtgacttgacccgaacctttctttcttgtttcttctgcgtctccataacatgcaggcgctccatgaggctagaaatgccctgctccaagctgtcaatagtgtggtgctgaggatcgtggccactgaagctgttgcgcaggctgcggagagcatctcgaacaagctgcaggtcgctggtccctctgttgctgactgaagtagctccttttcctgccgttggaaggagaaaaccattgctttgagagttgtgactgttgtagttggtcgcctcatctgcctctcttttcatacagtgagccaagaggacatctttgtgttctagctctcgctctagatccacctggtggtaactgacatcagagagtttccggagtgcttcttctaacttggcctggtgctgctgaagaaggcgatccttctgccccagctcttttttatattctcccaagagccggttcctctcatctagcttcctctgcagatccacattctggttgtgcagctcatctttgtccatatttgccctcagtagctcttgtttgagctgaagaacagatgtgtcctgctgagtcaatctctgctgcaaggcatcctttatcccctgtaagtttctggcttcttgtttacatttcagcagttccttctttaagtcctgattctcctccatactctgatccagacgactttggattataatcagttgttcctcgggattgacacctggttcacagagggccaagggcctctcctgttcatcttcaggtaaggatccattgagcagtaaggcctgtagtcctgatatcattttctttgcttcctccatttctttttctaaatattcttgttgttccaacagctgttcttcccatgaggtctccagataggttccagggctccctggccgccagtctcgagataatggagaatctgtcccttctgttctgttctctattccttcagcgggaataatcacaaaatctgccttctcttctgactgggttataatggactcgctctttgcactgtggattggactgggtgaagtcaggctggagcagctggattcagacggggacctttgttgcccttcgtactgctgcactagggcccgcacactccagtatggattctcaatttcctcatccatgctgctgttcctctgtctatatcgaaagacatcccgtcctgatcgggacatgtcatgacacacatcggccagagcagcagctgctccctgggcaacagcagtggcacagtgtggtcggtgactttgcagaggggctctggagtcccgtccttggttcaccgtcctgctggagccaggtttgaaatgagctgccaaggcaaggaccagcctcatgatagacttcaggtttccatccacaatatctttagccgaagtctggtgcatacgaatctttttagaggccacaaactgtagcactttctccacattattcttcatctcctgttggttaccgggactcagctgtaccccactcagcttttctcctgcaacaatctcgatgagatatgccaggatcaccccatcccggagatcttgtcgcaggtcctgcacaggcttcactgctggcctcttcttcagctgtgcattcacccaggccacataggcctgcagctgttgagaaggctctgttggcagcaaggagttattgaatctcataaccacttgggtccccatcttcaagagtccctcttaaatgatgggtccgtctggttcagcatctctgtccccagccctcctgagctcggcctgccagtgctctggctttgccgcggtttcccgctgccatggtgatgcgggggccg

SEQ ID NO: 13230 - RNA, 4900 nt, Homo sapiens
  source 1..4900: mol_type = other RNA
gctgggattacaggcatgagccaccacactcagccttaaatgaagattttgtaaggaattgagcattcaactaaactcgtttttgtgagatggtcattttgttttaacctaacatggtttagagattattttatgaactctaagcattctggttcctcagttttctcaaagaaagagaactttagcaagtagcaggacaagctaccccacaccaatgccaccaggcgacaatactatgaataagtcaggaggcctcctagaatgcagccaaataggaaactgttccaaacagaatcagtcttgcatacttctgctcagaaggctcctctcgctttggaaactggaatgaggatcaccaacaggatcctcattttacacaggagttatgagagttacatcctctagcagagatgcttggtcattacctgtggtacatgagattaccgagctaaaagggaaaaaaaacgatcttaatgttctcccatgaactcaacttaagctttttatggaggcactgaggccatgcagctccttttccaaaagacacagataaaagccaaataaggtagaggactttggaaattttctctgaaaagttaaattccacataatagtaagactgtttgctgagagaaaactgacaagtaaaaactggtttaagagacagacattcaagacaaactgtattggaaatacaataatgaattttggcctgatagccctcatgctgtcttatagcaaaacactaaaattcatgcaacagagaaattggtgacatgaggactttttctccagacttcctggggaaaaactgtgagaatatacttttttcttctgtttgctttcgaaatgcattctttcttttgctgactttcccaaactttcccagtcgtttctgatgaaaaattcttcaataggaaaagaccaggtaaacttacatgaaagacatcaagtatcttttgagctccttctctctgccagaggagcaatcaactggattacacaaaactaccttcacaactaaaacaggtagaattggaacaggaattagttgtcattaatatactcgtaataaaataaagcttgttctgaaaccacaaggggtggtaagaagagactgtataaaagctactgggttctctagaaaatggatacagtatacagaatgtgagaagatacagaactcacactccagttataaaaatagacatggttctcagacaaaaagcaaatgagtacaaaagaattctccaaacgtgaactatttttaaaagatacatctatataaaacaacaagatgtcatctcagagctccaaagagtagtttgttgaaatggctgaaaaggggagatgaattggagacagataggtcaagaacccagaacagatgtgtcctactcttgtgtttggcagtgtacattggaggtcacaggcagatagactgcttttggtaatacatatataaataataatggctgactggttgatggtgcttgatggatgaatgagaaaacccaggttatcaaataatctcggtagttgaactgttagcttcttcacttgacaatgttgcacatcagaaatgattctaggttttttttacccagaatgatccctgccattcacaactcatgctccacgccccatggtttctattgtgccctaaaagatcagcctagactaatacataaatagaaaataactctggccttgaaatgaggggcagacaagtacttcatgctcagtacttataaatcacaaagaaatgctgaaattaatggtctgtctccttttactacaaaggagatgccatgagttaaagtcatgaaacaaagaaagtcaaaaagatatgggtagcagcacctttccatacccgcctggattttcaaggagcttttcactccttatgcctttcaaacaaaagttcatcagtttgaagaaaaagaaatggctctaaagttaaagagtccccagagaaaactaacagtacatgaaataggccctatgtgggcaaaaggacaagctgcagaaccagttaagacagaagaggcagcccaaggtcttactaaattacagttttagcatagtgtagcacaacatgggcagccctttttccatccaagcaacaattcagcaccatccacgtctggttcaaaagattactgaagtctgggctttcatctttggtaccacctcatgagttattcttggtttgcagtaggttcaaagaaacagaaaagctggtacctttgccttgtctgtgagtacaaacgctgggactctgattgctgcaaccattgaggccaattaaaataatactgtaacacacaggaatgatgcatccaattcctaatttccagataatagcagccatgcccctacagaggcgggatcatccatccccatcgtttaaggccttcggtttgttgtcctcagagtagaatagaacactgtgttcccacggacaaggaactccagatgaacccatggtctacatttggacagaattttaagtaccagatatgccaggcacagaaagaggactgacctgtggccatcatgcttggagaagcttctgttttggcacacaaactagaaacttcttagtgtattctggttttagttccctttcctgagtgaagcagccagggagtgaccaggttccataagccctcaatctgatacttggcattaattctctccatggtcttcttccacccaagctacaattttcccttcccatccagggatggcatcatcatcatggaaaatctcctctttgacagtgccaaactcaggatccagtgctttgaagtgataccggtgatttccttcccgatcaatagctgctttaaaatcctttaacgtcacctcctccaacctctttggtatattgaccatgaagggcgtaagtgaccggtcagtgaaatagagcactttagtacaggtgctgctgacagttggagagctctgtgagtgaggcaactttgagttagggggccaggactcccggtattcactacctacttgagttctgggtgacttgacccgaacctttctttcttgtttcttctgcgtctccataacatgcaggcgctccatgaggctagaaatgccctgctccaagctgtcaatagtgtggtgctgaggatcgtggccactgaagctgttgcgcaggctgcggagagcatctcgaacaagctgcaggtcgctggtccctctgttgctgactgaagtagctccttttcctgccgttggaaggagaaaaccattgctttgagagttgtgactgttgtagttggtcgcctcatctgcctctcttttcatacagtgagccaagaggacatctttgtgttctagctctcgctctagatccacctggtggtaactgacatcagagagtttccggagtgcttcttctaacttggcctggtgctgctgaagaaggcgatccttctgccccagctcttttttatattctcccaagagccggttcctctcatctagcttcctctgcagatccacattctggttgtgcagctcatctttgtccatatttgccctcagtagctcttgtttgagctgaagaacagatgtgtcctgctgagtcaatctctgctgcaaggcatcctttatcccctgtaagtttctggcttcttgtttacatttcagcagttccttctttaagtcctgattctcctccatactctgatccagacgactttggattataatcagttgttcctcgggattgacacctggttcacagagggccaagggcctctcctgttcatcttcaggtaaggatccattgagcagtaaggcctgtagtcctgatatcattttctttgcttcctccatttctttttctaaatattcttgttgttccaacagctgttcttcccatgaggtctccagataggttccagggctccctggccgccagtctcgagataatggagaatctgtcccttctgttctgttctctattccttcagcgggaataatcacaaaatctgccttctcttctgactgggttataatggactcgctctttgcactgtggattggactgggtgaagtcaggctggagcagctggattcagacggggacctttgttgcccttcgtactgctgcactagggcccgcacactccagtatggattctcaatttcctcatccatgctgctgttcctctgtctatatcgaaagacatcccgtcctgatcgggacatgtcatgacacacatcggccagagcagcagctgctccctgggcaacagcagtggcacagtgtggtcggtgactttgcagaggggctctggagtcccgtccttggttcaccgtcctgctggagccaggtttgaaatgagctgccaaggcaaggaccagcctcatgatagacttcaggtttccatccacaatatctttagccgaagtctggtgcatacgaatctttttagaggccacaaactgtagcactttctccacattattcttcatctcctgttggttaccgggactcagctgtaccccactcagcttttctcctgcaacaatctcgatgagatatgccaggatcaccccatcccggagatcttgtcgcaggtcctgcacaggcttcactgctggcctcttcttcagctgtgcattcacccaggccacataggcctgcagctgttgctcattgaagccctcctgcaggacgtccagtaagttccctcgggtcaggcaggctagcattgttcctgctgggggctccccgggcggggtctccagcccggcggccgccgccgcctcctcctcctccctctgcacacaaaggctctcggctcagctcattgggatccctccggagtcccgcatgccacttactggaaacctagactggagccaaact

SEQ ID NO: 13231 - RNA, 4184 nt, Homo sapiens
  source 1..4184: mol_type = other RNA
gctgggattacaggcatgagccaccacactcagccttaaatgaagattttgtaaggaattgagcattcaactaaactcgtttttgtgagatggtcattttgttttaacctaacatggtttagagattattttatgaactctaagcattctggttcctcagttttctcaaagaaagagaactttagcaagtagcaggacaagctaccccacaccaatgccaccaggcgacaatactatgaataagtcaggaggcctcctagaatgcagccaaataggaaactgttccaaacagaatcagtcttgcatacttctgctcagaaggctcctctcgctttggaaactggaatgaggatcaccaacaggatcctcattttacacaggagttatgagagttacatcctctagcagagatgcttggtcattacctgtggtacatgagattaccgagctaaaagggaaaaaaaacgatcttaatgttctcccatgaactcaacttaagctttttatggaggcactgaggccatgcagctccttttccaaaagacacagataaaagccaaataaggtagaggactttggaaattttctctgaaaagttaaattccacataatagtaagactgtttgctgagagaaaactgacaagtaaaaactggtttaagagacagacattcaagacaaactgtattggaaatacaataatgaattttggcctgatagccctcatgctgtcttatagcaaaacactaaaattcatgcaacagagaaattggtgacatgaggactttttctccagacttcctggggaaaaactgtgagaatatacttttttcttctgtttgctttcgaaatgcattctttcttttgctgactttcccaaactttcccagtcgtttctgatgaaaaattcttcaataggaaaagaccaggtaaacttacatgaaagacatcaagtatcttttgagctccttctctctgccagaggagcaatcaactggattacacaaaactaccttcacaactaaaacaggtagaattggaacaggaattagttgtcattaatatactcgtaataaaataaagcttgttctgaaaccacaaggggtggtaagaagagactgtataaaagctactgggttctctagaaaatggatacagtatacagaatgtgagaagatacagaactcacactccagttataaaaatagacatggttctcagacaaaaagcaaatgagtacaaaagaattctccaaacgtgaactatttttaaaagatacatctatataaaacaacaagatgtcatctcagagctccaaagagtagtttgttgaaatggctgaaaaggggagatgaattggagacagataggtcaagaacccagaacagatgtgtcctactcttgtgtttggcagtgtacattggaggtcacaggcagatagactgcttttggtaatacatatataaataataatggctgactggttgatggtgcttgatggatgaatgagaaaacccaggttatcaaataatctcggtagttgaactgttagcttcttcacttgacaatgttgcacatcagaaatgattctaggttttttttacccagaatgatccctgccattcacaactcatgctccacgccccatggtttctattgtgccctaaaagatcagcctagactaatacataaatagaaaataactctggccttgaaatgaggggcagacaagtacttcatgctcagtacttataaatcacaaagaaatgctgaaattaatggtctgtctccttttactacaaaggagatgccatgagttaaagtcatgaaacaaagaaagtcaaaaagatatgggtagcagcacctttccatacccgcctggattttcaaggagcttttcactccttatgcctttcaaacaaaagttcatcagtttgaagaaaaagaaatggctctaaagttaaagagtccccagagaaaactaacagtacatgaaataggccctatgtgggcaaaaggacaagctgcagaaccagttaagacagaagaggcagcccaaggtcttactaaattacagttttagcatagtgtagcacaacatgggcagccctttttccatccaagcaacaattcagcaccatccacgtctggttcaaaagattactgaagtctgggctttcatctttggtaccacctcatgagttattcttggtttgcagtaggttcaaagaaacagaaaagctggtacctttgccttgtctgtgagtacaaacgctgggactctgattgctgcaaccattgaggccaattaaaataatactgtaacacacaggaatgatgcatccaattcctaatttccagataatagcagccatgcccctacagaggcgggatcatccatccccatcgtttaaggccttcggtttgttgtcctcagagtagaatagaacactgtgttcccacggacaaggaactccagatgaacccatggtctacatttggacagaattttaagtaccagatatgccaggcacagaaagaggactgacctgtggccatcatgcttggagaagcttctgttttggcacacaaactagaaacttcttagtgtattctggttttagttccctttcctgagtgaagcagccagggagtgaccaggttccataagccctcaatctgatacttggcattaattctctccatggtcttcttccacccaagctacaattttcccttcccatccagggatggcatcatcatcatggaaaatctcctctttgacagtgccaaactcaggatccagtgctttgaagtgataccggtgatttccttcccgatcaatagctgctttaaaatcctttaacgtcacctcctccaacctctttggtatattgaccatgaagggcgtaagtgaccggtcagtgaaatagagcactttagtacaggtgctgctgacagttggagagctctgtgagtgaggcaactttgagttagggggccaggactcccggtattcactacctacttgagttctgggtgacttgacccgaacctttctttcttgtttcttctgcgtctccataacatgcaggcgctccatgaggctagaaatgccctgctccaagctgtcaatagtgtggtgctgaggatcgtggccactgaagctgttgcgcaggctgcggagagcatctcgaacaagctgcaggtcgctggtccctctgttgctgactgaagtagctccttttcctgccgttggaaggagaaaaccattgctttgagagttgtgactgttgtagttggtcgcctcatctgcctctcttttcatacagtgagccaagaggacatctttgtgttctagctctcgctctagatccacctggtggtaactgacatcagagagtttccggagtgcttcttctaacttggcctggtgctgctgaagaaggcgatccttctgccccagctcttttttatattctcccaagagccggttcctctcatctagcttcctctgcagatccacattctggttgtgcagctcatctttgtccatatttgccctcagtagctcttgtttgagctgaagaacagatgtgtcctgctgagtcaatctctgctgcaaggcatcctttatcccctgtaagtttctggcttcttgtttacatttcagcagttccttctttaagtcctgattctcctccatactctgatccagacgactttggattataatcagttgttcctcgggattgacacctggttcacagagggccaagggcctctcctgttcatcttcaggtaaggatccattgagcagtaaggcctgtagtcctgatatcattttctttgcttcctccatttctttttctaaatattcttgttgttccaacagctgttcttcccatgaggtctccagataggttccagggctccctggccgccagtctcgagataatggagaatctgtcccttctgttctgttctctattccttcagcgggaataatcacaaaatctgccttctcttctgactgggttataatggactcgctctttgcactgtggattggactgggtgaagtcaggcttctccactctgagccctcccttggtggacgaggggtcggtcggacaggtcaggcccgcatggggctctggccgctcctcggggtggagactctga

SEQ ID NO: 13232 - RNA, 4645 nt, Homo sapiens
  source 1..4645: mol_type = other RNA
gctgggattacaggcatgagccaccacactgggcctgcattctattttgaccttcactaaaaagcttgccctgtgttgccccatcagtggcttcctctccttagaaacctggctgtgtgaaggtcaaggtctgttaacacggccaaagggacatttaatatttgcagtgtctcagcaccaaacaagtatacaacttcccgtgacagggcaggtaagaccttggagagactgtagacaggtcatttgaaccaattctctggggtaagatgtaggaaatggagcttttgccatctttcattggttccaagatatacatttttggatctctgaagtcaggaggcatctcccagatgatggtatcatattcttactgttggcccggacagaaggcaggtgctccgggagaggatagtactgtttttgccagccatccagggccacccagcctcagactgttggacattacactctctgcttgatgttcttttggatcacactgatagtgcaaattcagaaagcaaacctgcatgagtaccaccggcttgggactcctgttctcagggaaggatttttcacccccatttagtgtcaaggttgagatgcatgggtttccttgctccccctttctgcatggtggctctatttctcatttaccctctcattgagggcatcacagctttatgtggtgggggtagagagagtttcctattagacgccccatcttgggccttttttcttagtggtccataaaatgatgatgcatcttatcaccacggtttctcatagctgatgaagtaagtttctgttacaaatattgtatatgatatttgaaatgatccttcatgcatatagaaaaggagacaggattctgaagaaatggtttcatgagatgaagctttcctgtcttgtcctaaaccacttcctgtctgagctgttcacggggcattccctccccagcacctggaacccgctggcttctcatgactttcgggataagggcagagctcttccacatggccaaagccctgctgctcctgcttgttctccggtcatttccgcactgtattcctattctctcccctccagctttcagtcctcacattctcaaccttccacaccgcctctcatcacagagctctggtatgatggctctgttgggaaacttctctctccctggttggcttagctgacctccgttccagtgtcactgcttcaggacgcttcccccgatgctgtcagaccctgacggcaggcccctgcagtgctatgtgcttctctcccagcatgaacacaagctgcagctctatctctctgtgattcttggtcaatgttcaaatccttcgctggactgagcactccgtgagacaggaatcaggcctatttttactaaacattgtatccccagagtcaagccgggcatctggaagttggttggtgcctaagtataatttataaatggatggatgaatccaggtgtgagctgcccccacaagcagggagtaaacttctggagcctggcgcagccaggggaagcagaaagagcaacagacttgtcattagaaggtctctacttttgccataatgatgtgaccttgggaaaatcccatcctctccctgtttcctcagctctaaattgggaatatcgtttagtctgcctctaagatagggatgttttgtgaggccatgaagacactttgaactatacaagttatgcccctacccacaagcttctagctcagcactaggctcatatgccatgctctgttgacatgagttggttgactgtcccctcccccagagaaagggagatgagatcttataatccttggggaggggtgctcaaagctttgggtcatgaaacgaccatgtggccttgcgcttccccatctttatgtttgcccttttcaaaaaccctcacggaacttcttaggccttcaaggcccaatggcctaggtacataagaaaaggaacctcctgttgaggaccttctggcctttattctcgacacagagttggggccgttagccagaagaggagaaagggtggagaatgggaagactccttccttccttctctcctgcttgcaggctggtcttcagacagagacagggatgggtagggacaatgactttgccttctgggacagagctcctgggacaatcatctgcaggtgtatgcattccacctacacctggcagaatacatgaagttgcttactttacctctgggacctggactttaatattaaggtagatatttacagcaaagccttactactttctcccatatacctcatcttagagatgggcatcctgggtttctgtttcatctgtactgattgactatatcattttccctctctgagtcaattttctcatcagttacatgtaaataataataataataatgccacccaccttcctatctcactgagttcttttaaggaccaagtgaggtcatttgtcagacatgagtgcttggtaagtgaaaaatcaatgcaaacgaaaggcaatattattttctctatgcattgtaaatccctgcttctgtagcaggaaagcaccatgctgacttagttattcctaattaactcaaatattacccaagatctacagtccataaggtatgtaggcagaaagtgagatatgaacaaatccttcatcacaaatcaattctcaagcatttccccagggccagccatcctccctctgcagaaggggaccctgaggggtactcactctctaattgttttaacagcttggctgccctgccagagccctcccagaaaaccagattggtgaggggaggtgcagaatgaagaattaactggcacctcagcaattctggattctgtggaggggctggaaggctatactacagacacacacccctgcaggataattctagctggaggccgcagcagggtggatgagaacatgcttctgcaaacctcttgggatgcatcactgactggattctggcgattagagcttccagcctgccagaaattcctcagtgcatgatctgctgagcagctctgacagggattcactggtgtcctggtagaatgtggagcccaggccctcagagctcccactctccagctggaagctgcccaccagctcctgaatccactgcaggtctgcggagagctcctgcctcagaatctcaaactgggcttgcagatggtccagtttcctggccatgcttccgaggctacatcccgtggcctggatgtcttctcgcagcagcttcttcaatgactccaccttgcggaactcatacctgagctgggacaggtcatgccgggcgctctcattctcctctcggtaccaagcttccttctcattgaagatggagaccagggcctccacatcgtcctggatggtatcgtgggcctccaccagggcacggcatcccaggtcgacccgagccacgtcttccaccacacaggcaaaacgctcgaagttgacataggagttgttgggaggcatgcttgagtggcatttgagagtgtactctctcaggtgcttggtcttcagctgggtgggctctgtcttccgctgttcaggggctctgccttctccttttgacgtgatccaggggtgtctgagagcctcttggattgtgagccgtttccgggtctctttaaccagaagcttccgaataaagtccttggccagctcgctcgtctggctgaagaattcctcatcaaagtcgtaactcactgctgtgatatttgccagtgtttcctgcttcgtgtctcccaggaaaggggatgctccacttaagaggatgtaggtgatgacgcctatgctccacatgtcagcctccagacccaggggctcgtagttcacaatttctggagcaacaaattccggcgtcccaaaaatattcttaaattcaactccatcttctatttcgtgagccagaccaaagtcaatcagcttgatgtgtggaatgggaatattcttgtctaacaacataatgttttctggcttgagatcaaagtgagcaattttctttgtgtgaaggtagttcaccccatccaggatctgcttaatgaagctggtggcctcctcctcactcagtgactccttctgggccaggaaatcgaagagctctcctccagacactagctcaaggatgagcaccacgtcggtgcggttctcatagacgtcgtgcagcgtgatgacattgtggtgcagcacctgccgcaggatgctcacctcccgctcgatctcctcccggctcacaccgcgccggctcgcccggctctgccgcttcttgatgaacttggctgcatactcaagccccgtgctcttctcccggcacttcttcacgatggcaaactggccactccccagctcctctccgatgtcataaaagtcctccaccttctgctgcttgaatggctccatgtttggactcctcattgaggcctggaacatacaatcggcgggaggctgagctgccgcggtcgcggccgcggcaggcgcggcgggagcggcgggcgcggcgggcgcggcgggcgcggcgggcgcggcgggaacgggggacgcggcggggtgcgctgggctcggccctgcagtcctctcctcccagagcgcccggcacccgcccgccgagcagcctaggagccgag

SEQ ID NO: 13233 - RNA, 11161 nt, Homo sapiens
  source 1..11161: mol_type = other RNA
gctgggattacaggcatgagccaccacacttggcctaaaactggatttttttttttttttttttttttttttttttttgagatgaagtctcgctctgtcgcccaggctggaatgcagtggcacgatctcggctcactgcaagcttcacctcctgggttcatgccattctcctgcctcagcctccggagtagctgggactataggcgcctgccaccatgcccggctaattttttgtatttttgtagagatgaggtttcaccgtgttggccaggatagtcttgatctcctgacctcgtgatccgcccccctcggcctccccaagtgctgagattatagacgtgagccatcgcgcctggctagaactggatatttaaaatccagtaaatatttggtaaatttactacatcccatatatttcaactagtaataaattcggatttacttgtcgtcatcttcttttgtgtttatgttagccttatttttctaattcggcagtccccaaccttgttggcaccagggactgatttttgtggaagacaatttttccactgatgcggtttttttcccatggatgggggccggggcgggcatggttttgggattaaactgttccacctcagaaaatcaggcagtagattctcataaggagcacgcaacctagatccctcacatgcgcagttcacaatagagtttgtgctgctgtgagaatctaatgcagcagctgatctgacaggaggcggtgctcagggtaggtttgccgctcgcttcctgctgtgcagccaggtcctgaacaggtcagggacaggcagcctgggggggttggggacctctgctgtgttgttttcccctgttgttcttgctgctactaaactgataaagctttctttattttccctctacaactttggaagttacacattttgattctttagtaattatgctaaaaaacgacagctttcatacttaaagcctaaagttaatcaagatctttatactctgctcccaaagaaatggaaagctcttagaacactgtaattctgatcactgaactactgttttcagcatcttttgtttttgagacagggtctcactctgttgcccagactggagtgcactagtgcaatgaatcatagctcactacagttttgaactctgggcttaagggatcctcctgcctctgcctgccaagtagctgggactacaggcatgctactgtgcatggccaacttttttattttttttagagaccaggtctcactatgttgcccaggctggtctcaaactcctgggctcaaacgatcctcctgccttggccttccaaagtgctgggattacaggtgtgaaccaccatgcccagccggtttttaattttttaatatgcctccaaaggagacattatcatggttttctactgttcatattgggttatatttgcccggatcttcatcagtcttttttgttaatcactgtctattatgtatcacttcttccttcattgagtttttaaaattcatgtggcatatatttcagtaggcttttcagtgagggtctgttatcctgaagtctctcagtctttgagaagtctttaattcactttcattcttggatgataactagaaatcaaattccagattgacagttatttttctctattattttgaagctactgtattgtctctgatttctatggctgctatggagaacttctaccagcaggttagattcttgtgggtaaactctctttttctttctggttgcttttaagctttttctctttgtctctgttgttctgcagtattatttttatttatccctggctcgctgcatttcctaaatgtgaagattcatgtctcattaatcattttcagccattatcacttttaatattgccttgctcccctactcgattctctcctcctagaacttctacaggacatacgctgaatattctcattcaatttttcatgcctcttaacacgtattctccatcactactccattcttgctaatttccccaacttcattttatagtttattcttttttttttttttttgagatggagtctcactctgtcacccacactggagtgcaatggcacgatcttggctcactgcaacctccacctcccgggttcaagcgattctcctgcttcagcctctcaagtagctgggattacaggtgcacgccaccaggcccagctaattttttttgttttttttaatagagacagggtttcaccatgtgtaccaggttggtcttgaactcctgacctcatggtccacccgcctcagcctcccaaagtgctaggattacaggcatgagccaccgcgcccagtccggtttattcattttctgtgtcctaatatcttcattaagttaatttccagtacagttgtacctcagtatctgcagggagttggttccaggatccctttgactatcaaaatccacagatgctcaagggccctatataaaatggtgtcttttctggtgttttttgtttttgttttttgagacaaggtctcattctgttgccaggctggagagcagtggctcagtcacagctcactgtagcctcgacctcctgggctcaggtgattctcccacctcaacctaccaagtagctgggactataggcacgtgccactatgcctggtcaatttttgtattttgtgtagacagggttttgccatgttgcccaggctggtctacaactcctgggctcaagcagtctgcccacctccatcccccaaaaacgttgggattacacgtgtgagccaccatgccaggcctggagtagtatttgcatgtaacctatgcacatcctcccatatactttaagtcatctctggattacttataatatctaatacaatataaatactatgtaaatagttgttacactgtattttaaaatatgtatatttttattgttgtattattttttcaaatctttcccatcacattagttgattctgaagatgcagagcccgtaaatatggacggccaactatgttgtatttctcatttctgaaaattctatttagtttctaaagtttgtttccttcttctaaatatatttaaatatactttatttgtagcctctgcttaataattctattatctaaagtccttgggggtttaaatcttattgccttctgactcttatgataaattgtttccttgcatgttctattattttgaattgtgatctcaacttcattggggtttcatatgtggatatcctgttaggtctgagttaacatgcaacaatctagaaattctgtttccttctggcaactgccctagaaatacttttcatattaagttcacaggattcgcagaccacacaggtagtataaatttgaatcccaaactggtgaaaaggtaggtctatggtgacaaattcccaggaatgacttttattctctgtaccatgagtccaagctaacacaagcactagagggtggattttgttttttaatccttccattgagggtgaatgtctttaaaggtcctggctttgtatgtggatctcaatccaacttctcaccttgtaggggggcctaagactttacctcgagtgtccttgcgtgacctttaaaacccgagcatactggttacagaaactagggactgtctttacgcccaggcagtcacaaagcataaaccacacaccatactgttgttaaatttcctgtttagggctccgcccaggctggaatgcaatggcatgatctcagctcactgcaacctccatctcccaggttcaaatgattctgcctcagcctcccaagtagctgggattaccggcatgcgccaccatgcccagctaatttttatatttttagaagagatggattttcaccatgttggccaggctagtctcaaactcctgacctcaagtgatccgcctgcctcagcctcccaaagtgctgggattacaggcgtgagccaccaggcctggcggaaccttgatcttttaaatgtgaatttcagatatttctattacctgtaaggagagaggtggggaagacgaaggttgaagggaatattgaataaataactcctgtgtactagccctcaatacatgagatatttgataacagctatacaaaacaagccatgttaatagatgagaaattaaagctcagaaaggtcaaataatttcgctaaggtcacaatgtactattacacccgaattcacgttggaattaactagtcagatccattttcattctggacatggtggtgtatgcctgtagtcccagctatttgggggcctgaagtgagaggactgcttgtgcctaggaattcatgtacagcctgggcaacatagcaagaaactgcttctaaaaataaataggctgggtgcagtggctcacgcctgtaatcccagcactttgggaggtggaggcaggtggatcacttgaggtcaggagttcaagaccagcctggccaacacggcgaaaccccatctctactaaaaatacaaaaaattagctgggtgtggtggtgcgtgcctgtaatcccagttacttgggaggctgaggcaggagaagagctttaacccaggaagcagaggttgtggtgagctgagatcacgtcactgcactccagcctgggcaacagagcaagactctgtctcaaataaaaataaataactttgggaggccgaagtgggaggatcccgaggtcgagatcgagaccatcctggctaacacagtgaaaccccatctctactaaaaatacaaaaaattagctgggcatggtggcaggcacctgtagtctcccagctacttggaaggctgaggcagaagaattgcttgaacctgggaggcggaggttgcagtgagccgagatcgtgccactgcattccagcctgggcaacagagagagactccatctcaaaaaattaaaaataagttaacaaataatcaattttcttcctctacagcagaggtcagcaaacttattctgttaaaggccaaacagtaaatattttaggcctcataagccatatggtattggctgcaactattcagttttactgttgtatcattaaagcagccactgaaaagtgtaaacaaatgagcatgactgtgttcccataaaactttaaggacattgacatttgaatttcataaaattttcacatataacaatactattattacttggatcttttccccaaccatataaaaatttaaaacccgttgctaatgcatgggtcttacaaaaacagcctggagttgacccacgggccgtggtttgctgacccttatcatacaccataacacctccttggaagtacacctctctaatgcctttgttccaaacaatactgggttaggaaagacatggaaaaaggaaaatgagatacattattttttgtaccctatgggggattgaggggttgttgctacatagccccctcaatttgtgctgtagcaatatgcagttaagatccttattctaatgttaaatgtctcttctgtggcttatcctaactttaaaaaaaaaaaaaagaagccatcttacgtaaatgaacttacaattttaagacagggtctcactctgtcacccaggctggagtgcagtggtacaatcacggctcattgcagcctcgacctctcaggctcgagagatcctcccaccccaacttcccaagtagctgggactacaggtgtgcaccactatgcctagctcatcttttttttttttttttttttcctttaaaagatatggagtctcgctattttgcccaggctggtcttgaactcctggactcaagcaatccacctgcctcagcctcccagagtgttgggattacaggtgtgagccactgtgcccggcctgaattatcttcttattgtaaaatttcctttaatgcttaatagttgatgtatattaagtgctaactaaatgttcactgataaacattaatcagatgctgctaaatattgtctttctttattcacagatgatagtcaatgggcacaacatataagtagttacaatgaaatgagaagcaatatagcagtcaggctatatgcatgatttaacaacaaaattatcacttccttttaatttagaataagggacaatttaaaaagcatctcttggccctatcatttctgttccagtagttagtgttcatatgtgaatactaagtttgacattcctttctcccatagaaccattttggtgatttggatggtggccactacactgctttctgcaagaattcagtcacccaggcctgatatagctttgataacacacgagtcagtgagattccagatacttctgttcaaaatgctatggatctcctgttctatagctgccagcccttttccataccaatacaaaagcgttaagagccaggaaaatggtgtttcctgaacactgcaaaacaagcagtcagcatctggtggtagagttttgcttggtcattaaactcttagaacttacttgcatcattaacatttttatgccttgtgggcatgttatacaacctttcatcttaagataaatctgtcgtccagaagatgggtcttggttcactaaaaaaggcagtgtgaatataatgcaatgctaatggatgcaggccttcaaaacactgcaattatatagtgagttcaggtttcaaaattcagtgtttatcagaaaatatctcataatcatatatattcaacaaattattttccaaagatactcatgaagctaaacaaaaataatttttgttcaaatggctcgatgagtttaagaatatgatttgaatatatttgatataataatttagccaagaagtggtctcttagactaattgtaaaacatgaaaagttgtcagcttcacaatttgaaccccatcctttcatcttctccctgagagcctgctaatggtggtctctttctgaagcacttttagaatcttatttttatatggagtgttttactgactatatatatagcaactgagtccctcggttaaataaattataagctcctttaaccctcttaatacatcactctgtaaagatgtagtttataatgcagttcactttgcaatcatgcctgactcccggcatttttactttaatatttagaatgaatattctcaatatgtgagaatactagtcttgaaagaatgactctgggtgttattatatagcacgtgtgtatataaaatctatggttttactgtcctatatttgataatacaatattaaagacagaacacccacagggttataaattatttttctcattaagattttaatgtagctgtaaatgaaattctcgttttaaaaaaattaaagtttccatttttttttttagaataaagatttagtgcacaaatacagcccaaagccaacagaaaaattgctttgccctgtcatttccctaagaaagcactgaagttaactcaaaataggctgaaagaaaaaaagcaatcctctgagttctaggtttcacaaaaggaccacgtgttaaactatgtacatcgatttgatgtgcaagtatgcaataaatatgtacacatacattcctatctgctttacatcattctagagtattcatagtatatcaagatgggatttagaaatgtgaaaaggccataacagtgaaaaggaaaaaaaaaagataacaatagtttttagaccagtcgaataataatgcttagctagttaattattttaactttggagcagactaaaaaagttgttttgaaataaatggtacctgtaagtgatgattactgcaatacttgttaaatgttatttgtcagcactgaccggaattatatagtgctagtaacacagctcccactgtcctagaattcctctaaatggccagctatagctaccattatcctgataagcatttcaagagttgtgttgctgagccttttaaaagataactagtttataacctatgtctccttatgtggctacatcagttactcgtggtcccaatgaagtataaaagaggatataagctgctgaagatttcacagaagaaacggagatatcagaaacttcatgatcatcaaacttaaaccaccgttgtcttgctgcatttttacaataggctgtgtagtggcctccatccagcccaccgtagtgatttgaaacagaaaacaaattatatttcttcaaattgttctttggaccaataacatactgtgacaagtcaagattttctaacgggaagtccacagatgtctgtaatttttgtttccacctgccatcgtaggaaaaacgtttcagatgcactaaaagcacaggtggtaacttccagatttctatcttttttagagaatcccgtcgagctctgcaatgactgcagtaaaatctgttgttatctgtgagtttttcttctttggaaaataatctaaggcaatcctgtaatgtacatttacttgtggatgctagtggtagagacaaatacatgaaggcctcaaatgtcctagactttttgtgacatgtgaggcactgtactgtagatttgaattgaccctgaaaaagtgcaacaataatagactcattgagctgcttgtgtttctgccaggcatgttctgcagctttaaagtcatcgagatgatcattattttcttctttatatctcttccgattatcagctttatttagatcttcatggagaccatccattaggaacagaagcaattcttgtgaatcttgctgactgtatcctgcaaactggtcattgatcttcccaatggtgattttaaagtcctttggactgatatatctatactgtcctgtccacagggctttcatgattataccaaattcttctgccacttcacctttatgccccaacaaatttgacctgttaatatcatcctgataacagtttcggttgaaataatcagccaaatgtggagcgttacataggcactgcaatattgagttcatataacaagtatttcctaagttacgaagtccagtaagagctggtccagaacctccaaaaacaggattgaggttccgaatctgagaagcagaaagccttgagatctcagctttaggataacatgttggcttgttttcccgattaactgttggagttactgttggcttcctcttctcttcctcttgaatagcctgggttatatctggggaggagtaggagcgcttcagtttggaaggttccctatcccgctcagcaggaatctgtggcttggctttatgagttggaggggtggaaggaggtgcagatgaaggagccatttccggtgggtacatatgaacagtgttggtgggtgaatgataataacgaaaggttccagtgattgggtcaagaaacttggcccagcctgaaggcagtcctggtacgatcctccccatttcttcacttcgtgctcttgtcaaaggttctcgttgagccttgcctgaacctgaatcccctgtcacagatgtatggggcacatctcctgttgactttttctgtatttctggggttggacaccttttccccctatcttctacagatttcttggcatcagaagtttcatgttcacttttactttgtctttttactcctgttatttctttgcccctctttgctgaggtttctttatcttctttcttggcctgttcactttctttcttctccatttcttcttttgctttttgttgcttctctgtaatttcattttcttcagcttcttgtttctttttggctttttgttcttgttcttccttcctcagtttctctttctgttcctcttgctgcctttcccgaagttctttttcttgtttgtttttttccattagaagagcagtttctgcatgaatacgagccttttcttcatctgttaacatgagagttggagaaaaaactactggcttggtggaacgatcaggaataacttttccactctgaggagattgttgctcatggtttgtactttcagattttattctatgctcttcaggcaatttgactgctggttttttagtacgatcaatctgtggaacattctttatactaggcactggctgaattatgggtgaaacatcagatttagaagcagcaactggttcaactggagttgatatattcagtggtcccattctctcattttgaccacttatcaattctatattttcatctacttctatagatgcaggtggcgtctgggcagcaggtttagaaggaattgattcttccaatgagggataagtaaaatccaatgagatagacacctcttcattctggcgtcgtgggggtggagtgaccttagcatttgttgtatactggggataacaaaggagccagttttcatagcctccctctaaaaccaaaggctcattgcgcaggacagttttactttcccacttgaaaagtgcatctttcagactccggagagttgttccaatctgtaaatctttggcagaactaaaccagtcaagaagtaccacatactccacattccccctcttcttccatgtgtctttagaatcatctggcaggtgtgcttcaatccaactagcagtgactcctggactgatggcttcttcaggaacactgagagaatgtaaaatacaggaatcctgataatcctgcattcttcgagcatccattataatcaagctgatgtttttatccgtcatcattgtgtatagttcctttgctgtgattgctcctttctctttggtctcacatttttcattcttttcaccattgctcttttgggttttgtctttggaatccaaaacattctccaaagagcctttagccaatgtgccaccatcctctcttcctgtttcctgccttttttgttgtagccgctgtgcttcctcctgcctgtctttttcctcaagttttttccggacttcagcttcttcatatctcttagtgcttattttctctggtttaacttctgtcttcttattaaggtcttttagtgaagaactgaggtagagttctttaggaactgaagccacagcaggcatgatgaattatctttacttttccactttcacaatggatgctatatttccttacaagtgcttctttccgtgacgccgggcgcgcttcactaacgccagccttctcgccaaatgcccatctcccaagaactcgagggagaattagccttggctaccaggacggaagccagcccagctc

SEQ ID NO: 13234 - RNA, 11479 nt, Homo sapiens
  source 1..11479: mol_type = other RNA
gctgggattacaggcatgagccaccacacttggcctaaaactggatttttttttttttttttttttttttttttttttgagatgaagtctcgctctgtcgcccaggctggaatgcagtggcacgatctcggctcactgcaagcttcacctcctgggttcatgccattctcctgcctcagcctccggagtagctgggactataggcgcctgccaccatgcccggctaattttttgtatttttgtagagatgaggtttcaccgtgttggccaggatagtcttgatctcctgacctcgtgatccgcccccctcggcctccccaagtgctgagattatagacgtgagccatcgcgcctggctagaactggatatttaaaatccagtaaatatttggtaaatttactacatcccatatatttcaactagtaataaattcggatttacttgtcgtcatcttcttttgtgtttatgttagccttatttttctaattcggcagtccccaaccttgttggcaccagggactgatttttgtggaagacaatttttccactgatgcggtttttttcccatggatgggggccggggcgggcatggttttgggattaaactgttccacctcagaaaatcaggcagtagattctcataaggagcacgcaacctagatccctcacatgcgcagttcacaatagagtttgtgctgctgtgagaatctaatgcagcagctgatctgacaggaggcggtgctcagggtaggtttgccgctcgcttcctgctgtgcagccaggtcctgaacaggtcagggacaggcagcctgggggggttggggacctctgctgtgttgttttcccctgttgttcttgctgctactaaactgataaagctttctttattttccctctacaactttggaagttacacattttgattctttagtaattatgctaaaaaacgacagctttcatacttaaagcctaaagttaatcaagatctttatactctgctcccaaagaaatggaaagctcttagaacactgtaattctgatcactgaactactgttttcagcatcttttgtttttgagacagggtctcactctgttgcccagactggagtgcactagtgcaatgaatcatagctcactacagttttgaactctgggcttaagggatcctcctgcctctgcctgccaagtagctgggactacaggcatgctactgtgcatggccaacttttttattttttttagagaccaggtctcactatgttgcccaggctggtctcaaactcctgggctcaaacgatcctcctgccttggccttccaaagtgctgggattacaggtgtgaaccaccatgcccagccggtttttaattttttaatatgcctccaaaggagacattatcatggttttctactgttcatattgggttatatttgcccggatcttcatcagtcttttttgttaatcactgtctattatgtatcacttcttccttcattgagtttttaaaattcatgtggcatatatttcagtaggcttttcagtgagggtctgttatcctgaagtctctcagtctttgagaagtctttaattcactttcattcttggatgataactagaaatcaaattccagattgacagttatttttctctattattttgaagctactgtattgtctctgatttctatggctgctatggagaacttctaccagcaggttagattcttgtgggtaaactctctttttctttctggttgcttttaagctttttctctttgtctctgttgttctgcagtattatttttatttatccctggctcgctgcatttcctaaatgtgaagattcatgtctcattaatcattttcagccattatcacttttaatattgccttgctcccctactcgattctctcctcctagaacttctacaggacatacgctgaatattctcattcaatttttcatgcctcttaacacgtattctccatcactactccattcttgctaatttccccaacttcattttatagtttattcttttttttttttttttgagatggagtctcactctgtcacccacactggagtgcaatggcacgatcttggctcactgcaacctccacctcccgggttcaagcgattctcctgcttcagcctctcaagtagctgggattacaggtgcacgccaccaggcccagctaattttttttgttttttttaatagagacagggtttcaccatgtgtaccaggttggtcttgaactcctgacctcatggtccacccgcctcagcctcccaaagtgctaggattacaggcatgagccaccgcgcccagtccggtttattcattttctgtgtcctaatatcttcattaagttaatttccagtacagttgtacctcagtatctgcagggagttggttccaggatccctttgactatcaaaatccacagatgctcaagggccctatataaaatggtgtcttttctggtgttttttgtttttgttttttgagacaaggtctcattctgttgccaggctggagagcagtggctcagtcacagctcactgtagcctcgacctcctgggctcaggtgattctcccacctcaacctaccaagtagctgggactataggcacgtgccactatgcctggtcaatttttgtattttgtgtagacagggttttgccatgttgcccaggctggtctacaactcctgggctcaagcagtctgcccacctccatcccccaaaaacgttgggattacacgtgtgagccaccatgccaggcctggagtagtatttgcatgtaacctatgcacatcctcccatatactttaagtcatctctggattacttataatatctaatacaatataaatactatgtaaatagttgttacactgtattttaaaatatgtatatttttattgttgtattattttttcaaatctttcccatcacattagttgattctgaagatgcagagcccgtaaatatggacggccaactatgttgtatttctcatttctgaaaattctatttagtttctaaagtttgtttccttcttctaaatatatttaaatatactttatttgtagcctctgcttaataattctattatctaaagtccttgggggtttaaatcttattgccttctgactcttatgataaattgtttccttgcatgttctattattttgaattgtgatctcaacttcattggggtttcatatgtggatatcctgttaggtctgagttaacatgcaacaatctagaaattctgtttccttctggcaactgccctagaaatacttttcatattaagttcacaggattcgcagaccacacaggtagtataaatttgaatcccaaactggtgaaaaggtaggtctatggtgacaaattcccaggaatgacttttattctctgtaccatgagtccaagctaacacaagcactagagggtggattttgttttttaatccttccattgagggtgaatgtctttaaaggtcctggctttgtatgtggatctcaatccaacttctcaccttgtaggggggcctaagactttacctcgagtgtccttgcgtgacctttaaaacccgagcatactggttacagaaactagggactgtctttacgcccaggcagtcacaaagcataaaccacacaccatactgttgttaaatttcctgtttagggctccgcccaggctggaatgcaatggcatgatctcagctcactgcaacctccatctcccaggttcaaatgattctgcctcagcctcccaagtagctgggattaccggcatgcgccaccatgcccagctaatttttatatttttagaagagatggattttcaccatgttggccaggctagtctcaaactcctgacctcaagtgatccgcctgcctcagcctcccaaagtgctgggattacaggcgtgagccaccaggcctggcggaaccttgatcttttaaatgtgaatttcagatatttctattacctgtaaggagagaggtggggaagacgaaggttgaagggaatattgaataaataactcctgtgtactagccctcaatacatgagatatttgataacagctatacaaaacaagccatgttaatagatgagaaattaaagctcagaaaggtcaaataatttcgctaaggtcacaatgtactattacacccgaattcacgttggaattaactagtcagatccattttcattctggacatggtggtgtatgcctgtagtcccagctatttgggggcctgaagtgagaggactgcttgtgcctaggaattcatgtacagcctgggcaacatagcaagaaactgcttctaaaaataaataggctgggtgcagtggctcacgcctgtaatcccagcactttgggaggtggaggcaggtggatcacttgaggtcaggagttcaagaccagcctggccaacacggcgaaaccccatctctactaaaaatacaaaaaattagctgggtgtggtggtgcgtgcctgtaatcccagttacttgggaggctgaggcaggagaagagctttaacccaggaagcagaggttgtggtgagctgagatcacgtcactgcactccagcctgggcaacagagcaagactctgtctcaaataaaaataaataactttgggaggccgaagtgggaggatcccgaggtcgagatcgagaccatcctggctaacacagtgaaaccccatctctactaaaaatacaaaaaattagctgggcatggtggcaggcacctgtagtctcccagctacttggaaggctgaggcagaagaattgcttgaacctgggaggcggaggttgcagtgagccgagatcgtgccactgcattccagcctgggcaacagagagagactccatctcaaaaaattaaaaataagttaacaaataatcaattttcttcctctacagcagaggtcagcaaacttattctgttaaaggccaaacagtaaatattttaggcctcataagccatatggtattggctgcaactattcagttttactgttgtatcattaaagcagccactgaaaagtgtaaacaaatgagcatgactgtgttcccataaaactttaaggacattgacatttgaatttcataaaattttcacatataacaatactattattacttggatcttttccccaaccatataaaaatttaaaacccgttgctaatgcatgggtcttacaaaaacagcctggagttgacccacgggccgtggtttgctgacccttatcatacaccataacacctccttggaagtacacctctctaatgcctttgttccaaacaatactgggttaggaaagacatggaaaaaggaaaatgagatacattattttttgtaccctatgggggattgaggggttgttgctacatagccccctcaatttgtgctgtagcaatatgcagttaagatccttattctaatgttaaatgtctcttctgtggcttatcctaactttaaaaaaaaaaaaaagaagccatcttacgtaaatgaacttacaattttaagacagggtctcactctgtcacccaggctggagtgcagtggtacaatcacggctcattgcagcctcgacctctcaggctcgagagatcctcccaccccaacttcccaagtagctgggactacaggtgtgcaccactatgcctagctcatcttttttttttttttttttttcctttaaaagatatggagtctcgctattttgcccaggctggtcttgaactcctggactcaagcaatccacctgcctcagcctcccagagtgttgggattacaggtgtgagccactgtgcccggcctgaattatcttcttattgtaaaatttcctttaatgcttaatagttgatgtatattaagtgctaactaaatgttcactgataaacattaatcagatgctgctaaatattgtctttctttattcacagatgatagtcaatgggcacaacatataagtagttacaatgaaatgagaagcaatatagcagtcaggctatatgcatgatttaacaacaaaattatcacttccttttaatttagaataagggacaatttaaaaagcatctcttggccctatcatttctgttccagtagttagtgttcatatgtgaatactaagtttgacattcctttctcccatagaaccattttggtgatttggatggtggccactacactgctttctgcaagaattcagtcacccaggcctgatatagctttgataacacacgagtcagtgagattccagatacttctgttcaaaatgctatggatctcctgttctatagctgccagcccttttccataccaatacaaaagcgttaagagccaggaaaatggtgtttcctgaacactgcaaaacaagcagtcagcatctggtggtagagttttgcttggtcattaaactcttagaacttacttgcatcattaacatttttatgccttgtgggcatgttatacaacctttcatcttaagataaatctgtcgtccagaagatgggtcttggttcactaaaaaaggcagtgtgaatataatgcaatgctaatggatgcaggccttcaaaacactgcaattatatagtgagttcaggtttcaaaattcagtgtttatcagaaaatatctcataatcatatatattcaacaaattattttccaaagatactcatgaagctaaacaaaaataatttttgttcaaatggctcgatgagtttaagaatatgatttgaatatatttgatataataatttagccaagaagtggtctcttagactaattgtaaaacatgaaaagttgtcagcttcacaatttgaaccccatcctttcatcttctccctgagagcctgctaatggtggtctctttctgaagcacttttagaatcttatttttatatggagtgttttactgactatatatatagcaactgagtccctcggttaaataaattataagctcctttaaccctcttaatacatcactctgtaaagatgtagtttataatgcagttcactttgcaatcatgcctgactcccggcatttttactttaatatttagaatgaatattctcaatatgtgagaatactagtcttgaaagaatgactctgggtgttattatatagcacgtgtgtatataaaatctatggttttactgtcctatatttgataatacaatattaaagacagaacacccacagggttataaattatttttctcattaagattttaatgtagctgtaaatgaaattctcgttttaaaaaaattaaagtttccatttttttttttagaataaagatttagtgcacaaatacagcccaaagccaacagaaaaattgctttgccctgtcatttccctaagaaagcactgaagttaactcaaaataggctgaaagaaaaaaagcaatcctctgagttctaggtttcacaaaaggaccacgtgttaaactatgtacatcgatttgatgtgcaagtatgcaataaatatgtacacatacattcctatctgctttacatcattctagagtattcatagtatatcaagatgggatttagaaatgtgaaaaggccataacagtgaaaaggaaaaaaaaaagataacaatagtttttagaccagtcgaataataatgcttagctagttaattattttaactttggagcagactaaaaaagttgttttgaaataaatggtacctgtaagtgatgattactgcaatacttgttaaatgttatttgtcagcactgaccggaattatatagtgctagtaacacagctcccactgtcctagaattcctctaaatggccagctatagctaccattatcctgataagcatttcaagagttgtgttgctgagccttttaaaagataactagtttataacctatgtctccttatgtggctacatcagttactcgtggtcccaatgaagtataaaagaggatataagctgctgaagatttcacagaagaaacggagatatcagaaacttcatgatcatcaaacttaaaccaccgttgtcttgctgcatttttacaataggctgtgtagtggcctccatccagcccaccgtagtgatttgaaacagaaaacaaattatatttcttcaaattgttctttggaccaataacatactgtgacaagtcaagattttctaacgggaagtccacagatgtctgtaatttttgtttccacctgccatcgtaggaaaaacgtttcagatgcactaaaagcacaggtggtaacttccagatttctatcttttttagagaatcccgtcgagctctgcaatgactgcagtaaaatctgttgttatctgtgagtttttcttctttggaaaataatctaaggcaatcctgtaatgtacatttacttgtggatgctagtggtagagacaaatacatgaaggcctcaaatgtcctagactttttgtgacatgtgaggcactgtactgtagatttgaattgaccctgaaaaagtgcaacaataatagactcattgagctgcttgtgtttctgccaggcatgttctgcagctttaaagtcatcgagatgatcattattttcttctttatatctcttccgattatcagctttatttagatcttcatggagaccatccattaggaacagaagcaattcttgtgaatcttgctgactgtatcctgcaaactggtcattgatcttcccaatggtgattttaaagtcctttggactgatatatctatactgtcctgtccacagggctttcatgattataccaaattcttctgccacttcacctttatgccccaacaaatttgacctgttaatatcatcctgataacagtttcggttgaaataatcagccaaatgtggagcgttacataggcactgcaatattgagttcatataacaagtatttcctaagttacgaagtccagtaagagctggtccagaacctccaaaaacaggattgaggttccgaatctgagaagcagaaagccttgagatctcagctttaggataacatgttggcttgttttcccgattaactgttggagttactgttggcttcctcttctcttcctcttgaatagcctgggttatatctggggaggagtaggagcgcttcagtttggaaggttccctatcccgctcagcaggaatctgtggcttggctttatgagttggaggggtggaaggaggtgcagatgaaggagccatttccggtgggtacatatgaacagtgttggtgggtgaatgataataacgaaaggttccagtgattgggtcaagaaacttggcccagcctgaaggcagtcctggtacgatcctccccatttcttcacttcgtgctcttgtcaaaggttctcgttgagctttatttctttcggtatcgtctgtatcctctctaaaagttcctgtccttagaattccactttctggttgtcctttaatcttaaatggcttgcctgaacctgaatcccctgtcacagatgtatggggcacatctcctgttgactttttctgtatttctggggttggacaccttttccccctatcttctacagatttcttggcatcagaagtttcatgttcacttttactttgtctttttactcctgttatttctttgcccctctttgctgaggtttctttatcttctttcttggcctgttcactttctttcttctccatttcttcttttgctttttgttgcttctctgtaatttcattttcttcagcttcttgtttctttttggctttttgttcttgttcttccttcctcagtttctctttctgttcctcttgctgcctttcccgaagttctttttcttgtttgtttttttccattagaagagcagtttctgcatgaatacgagccttttcttcatctgttaacatgagagttggagaaaaaactactggcttggtggaacgatcaggaataacttttccactctgaggagattgttgctcatggtttgtactttcagattttattctatgctcttcaggcaatttgactgctggttttttagtacgatcaatctgtggaacattctttatactaggcactggctgaattatgggtgaaacatcagatttagaagcagcaactggttcaactggagttgatatattcagtggtcccattctctcattttgaccacttatcaattctatattttcatctacttctatagatgcaggtggcgtctgggcagcaggtttagaaggaattgattcttccaatgagggataagtaaaatccaatgagatagacacctcttcattctggcgtcgtgggggtggagtgaccttagcatttgttgtatactggggataacaaaggagccagttttcatagcctccctctaaaaccaaaggctcattgcgcaggacagttttactttcccacttgaaaagtgcatctttcagactccggagagttgttccaatctgtaaatctttggcagaactaaaccagtcaagaagtaccacatactccacattccccctcttcttccatgtgtctttagaatcatctggcaggtgtgcttcaatccaactagcagtgactcctggactgatggcttcttcaggaacactgagagaatgtaaaatacaggaatcctgataatcctgcattcttcgagcatccattataatcaagctgatgtttttatccgtcatcattgtgtatagttcctttgctgtgattgctcctttctctttggtctcacatttttcattcttttcaccattgctcttttgggttttgtctttggaatccaaaacattctccaaagagcctttagccaatgtgccaccatcctctcttcctgtttcctgccttttttgttgtagccgctgtgcttcctcctgcctgtctttttcctcaagttttttccggacttcagcttcttcatatcttaatttaaggctttcagagagtctttcagcttcttcgacagcttttttgatgtttccaggtccaagtattgaatggaaataatcctgctgttgcttgaaatcaggtctttttttgataagattataaacagtcacgtatttcatatatagtacataggccctttcctcatcacgatctaatctgcattcttctgctgtcttaaagatcttcagggcactgtgcacataactcttagtgcttattttctctggtttaacttctgtcttcttattaaggtcttttagtgaagaactgaggtagagttctttaggaactgaagccacagcaggcatgatgaattatctttacttttccactttcacaatggatgctatatttccttacaagtgcttctttccgtgacgccgggcgcgcttcactaacgccagccttctcgccaaatgcccatctcccaagaactcgagggagaattagccttggctaccaggacggaagccagcccagctc

SEQ ID NO: 13235 - RNA, 11619 nt, Homo sapiens
  source 1..11619: mol_type = other RNA
gctgggattacaggcatgagccaccacacttggcctaaaactggatttttttttttttttttttttttttttttttttgagatgaagtctcgctctgtcgcccaggctggaatgcagtggcacgatctcggctcactgcaagcttcacctcctgggttcatgccattctcctgcctcagcctccggagtagctgggactataggcgcctgccaccatgcccggctaattttttgtatttttgtagagatgaggtttcaccgtgttggccaggatagtcttgatctcctgacctcgtgatccgcccccctcggcctccccaagtgctgagattatagacgtgagccatcgcgcctggctagaactggatatttaaaatccagtaaatatttggtaaatttactacatcccatatatttcaactagtaataaattcggatttacttgtcgtcatcttcttttgtgtttatgttagccttatttttctaattcggcagtccccaaccttgttggcaccagggactgatttttgtggaagacaatttttccactgatgcggtttttttcccatggatgggggccggggcgggcatggttttgggattaaactgttccacctcagaaaatcaggcagtagattctcataaggagcacgcaacctagatccctcacatgcgcagttcacaatagagtttgtgctgctgtgagaatctaatgcagcagctgatctgacaggaggcggtgctcagggtaggtttgccgctcgcttcctgctgtgcagccaggtcctgaacaggtcagggacaggcagcctgggggggttggggacctctgctgtgttgttttcccctgttgttcttgctgctactaaactgataaagctttctttattttccctctacaactttggaagttacacattttgattctttagtaattatgctaaaaaacgacagctttcatacttaaagcctaaagttaatcaagatctttatactctgctcccaaagaaatggaaagctcttagaacactgtaattctgatcactgaactactgttttcagcatcttttgtttttgagacagggtctcactctgttgcccagactggagtgcactagtgcaatgaatcatagctcactacagttttgaactctgggcttaagggatcctcctgcctctgcctgccaagtagctgggactacaggcatgctactgtgcatggccaacttttttattttttttagagaccaggtctcactatgttgcccaggctggtctcaaactcctgggctcaaacgatcctcctgccttggccttccaaagtgctgggattacaggtgtgaaccaccatgcccagccggtttttaattttttaatatgcctccaaaggagacattatcatggttttctactgttcatattgggttatatttgcccggatcttcatcagtcttttttgttaatcactgtctattatgtatcacttcttccttcattgagtttttaaaattcatgtggcatatatttcagtaggcttttcagtgagggtctgttatcctgaagtctctcagtctttgagaagtctttaattcactttcattcttggatgataactagaaatcaaattccagattgacagttatttttctctattattttgaagctactgtattgtctctgatttctatggctgctatggagaacttctaccagcaggttagattcttgtgggtaaactctctttttctttctggttgcttttaagctttttctctttgtctctgttgttctgcagtattatttttatttatccctggctcgctgcatttcctaaatgtgaagattcatgtctcattaatcattttcagccattatcacttttaatattgccttgctcccctactcgattctctcctcctagaacttctacaggacatacgctgaatattctcattcaatttttcatgcctcttaacacgtattctccatcactactccattcttgctaatttccccaacttcattttatagtttattcttttttttttttttttgagatggagtctcactctgtcacccacactggagtgcaatggcacgatcttggctcactgcaacctccacctcccgggttcaagcgattctcctgcttcagcctctcaagtagctgggattacaggtgcacgccaccaggcccagctaattttttttgttttttttaatagagacagggtttcaccatgtgtaccaggttggtcttgaactcctgacctcatggtccacccgcctcagcctcccaaagtgctaggattacaggcatgagccaccgcgcccagtccggtttattcattttctgtgtcctaatatcttcattaagttaatttccagtacagttgtacctcagtatctgcagggagttggttccaggatccctttgactatcaaaatccacagatgctcaagggccctatataaaatggtgtcttttctggtgttttttgtttttgttttttgagacaaggtctcattctgttgccaggctggagagcagtggctcagtcacagctcactgtagcctcgacctcctgggctcaggtgattctcccacctcaacctaccaagtagctgggactataggcacgtgccactatgcctggtcaatttttgtattttgtgtagacagggttttgccatgttgcccaggctggtctacaactcctgggctcaagcagtctgcccacctccatcccccaaaaacgttgggattacacgtgtgagccaccatgccaggcctggagtagtatttgcatgtaacctatgcacatcctcccatatactttaagtcatctctggattacttataatatctaatacaatataaatactatgtaaatagttgttacactgtattttaaaatatgtatatttttattgttgtattattttttcaaatctttcccatcacattagttgattctgaagatgcagagcccgtaaatatggacggccaactatgttgtatttctcatttctgaaaattctatttagtttctaaagtttgtttccttcttctaaatatatttaaatatactttatttgtagcctctgcttaataattctattatctaaagtccttgggggtttaaatcttattgccttctgactcttatgataaattgtttccttgcatgttctattattttgaattgtgatctcaacttcattggggtttcatatgtggatatcctgttaggtctgagttaacatgcaacaatctagaaattctgtttccttctggcaactgccctagaaatacttttcatattaagttcacaggattcgcagaccacacaggtagtataaatttgaatcccaaactggtgaaaaggtaggtctatggtgacaaattcccaggaatgacttttattctctgtaccatgagtccaagctaacacaagcactagagggtggattttgttttttaatccttccattgagggtgaatgtctttaaaggtcctggctttgtatgtggatctcaatccaacttctcaccttgtaggggggcctaagactttacctcgagtgtccttgcgtgacctttaaaacccgagcatactggttacagaaactagggactgtctttacgcccaggcagtcacaaagcataaaccacacaccatactgttgttaaatttcctgtttagggctccgcccaggctggaatgcaatggcatgatctcagctcactgcaacctccatctcccaggttcaaatgattctgcctcagcctcccaagtagctgggattaccggcatgcgccaccatgcccagctaatttttatatttttagaagagatggattttcaccatgttggccaggctagtctcaaactcctgacctcaagtgatccgcctgcctcagcctcccaaagtgctgggattacaggcgtgagccaccaggcctggcggaaccttgatcttttaaatgtgaatttcagatatttctattacctgtaaggagagaggtggggaagacgaaggttgaagggaatattgaataaataactcctgtgtactagccctcaatacatgagatatttgataacagctatacaaaacaagccatgttaatagatgagaaattaaagctcagaaaggtcaaataatttcgctaaggtcacaatgtactattacacccgaattcacgttggaattaactagtcagatccattttcattctggacatggtggtgtatgcctgtagtcccagctatttgggggcctgaagtgagaggactgcttgtgcctaggaattcatgtacagcctgggcaacatagcaagaaactgcttctaaaaataaataggctgggtgcagtggctcacgcctgtaatcccagcactttgggaggtggaggcaggtggatcacttgaggtcaggagttcaagaccagcctggccaacacggcgaaaccccatctctactaaaaatacaaaaaattagctgggtgtggtggtgcgtgcctgtaatcccagttacttgggaggctgaggcaggagaagagctttaacccaggaagcagaggttgtggtgagctgagatcacgtcactgcactccagcctgggcaacagagcaagactctgtctcaaataaaaataaataactttgggaggccgaagtgggaggatcccgaggtcgagatcgagaccatcctggctaacacagtgaaaccccatctctactaaaaatacaaaaaattagctgggcatggtggcaggcacctgtagtctcccagctacttggaaggctgaggcagaagaattgcttgaacctgggaggcggaggttgcagtgagccgagatcgtgccactgcattccagcctgggcaacagagagagactccatctcaaaaaattaaaaataagttaacaaataatcaattttcttcctctacagcagaggtcagcaaacttattctgttaaaggccaaacagtaaatattttaggcctcataagccatatggtattggctgcaactattcagttttactgttgtatcattaaagcagccactgaaaagtgtaaacaaatgagcatgactgtgttcccataaaactttaaggacattgacatttgaatttcataaaattttcacatataacaatactattattacttggatcttttccccaaccatataaaaatttaaaacccgttgctaatgcatgggtcttacaaaaacagcctggagttgacccacgggccgtggtttgctgacccttatcatacaccataacacctccttggaagtacacctctctaatgcctttgttccaaacaatactgggttaggaaagacatggaaaaaggaaaatgagatacattattttttgtaccctatgggggattgaggggttgttgctacatagccccctcaatttgtgctgtagcaatatgcagttaagatccttattctaatgttaaatgtctcttctgtggcttatcctaactttaaaaaaaaaaaaaagaagccatcttacgtaaatgaacttacaattttaagacagggtctcactctgtcacccaggctggagtgcagtggtacaatcacggctcattgcagcctcgacctctcaggctcgagagatcctcccaccccaacttcccaagtagctgggactacaggtgtgcaccactatgcctagctcatcttttttttttttttttttttcctttaaaagatatggagtctcgctattttgcccaggctggtcttgaactcctggactcaagcaatccacctgcctcagcctcccagagtgttgggattacaggtgtgagccactgtgcccggcctgaattatcttcttattgtaaaatttcctttaatgcttaatagttgatgtatattaagtgctaactaaatgttcactgataaacattaatcagatgctgctaaatattgtctttctttattcacagatgatagtcaatgggcacaacatataagtagttacaatgaaatgagaagcaatatagcagtcaggctatatgcatgatttaacaacaaaattatcacttccttttaatttagaataagggacaatttaaaaagcatctcttggccctatcatttctgttccagtagttagtgttcatatgtgaatactaagtttgacattcctttctcccatagaaccattttggtgatttggatggtggccactacactgctttctgcaagaattcagtcacccaggcctgatatagctttgataacacacgagtcagtgagattccagatacttctgttcaaaatgctatggatctcctgttctatagctgccagcccttttccataccaatacaaaagcgttaagagccaggaaaatggtgtttcctgaacactgcaaaacaagcagtcagcatctggtggtagagttttgcttggtcattaaactcttagaacttacttgcatcattaacatttttatgccttgtgggcatgttatacaacctttcatcttaagataaatctgtcgtccagaagatgggtcttggttcactaaaaaaggcagtgtgaatataatgcaatgctaatggatgcaggccttcaaaacactgcaattatatagtgagttcaggtttcaaaattcagtgtttatcagaaaatatctcataatcatatatattcaacaaattattttccaaagatactcatgaagctaaacaaaaataatttttgttcaaatggctcgatgagtttaagaatatgatttgaatatatttgatataataatttagccaagaagtggtctcttagactaattgtaaaacatgaaaagttgtcagcttcacaatttgaaccccatcctttcatcttctccctgagagcctgctaatggtggtctctttctgaagcacttttagaatcttatttttatatggagtgttttactgactatatatatagcaactgagtccctcggttaaataaattataagctcctttaaccctcttaatacatcactctgtaaagatgtagtttataatgcagttcactttgcaatcatgcctgactcccggcatttttactttaatatttagaatgaatattctcaatatgtgagaatactagtcttgaaagaatgactctgggtgttattatatagcacgtgtgtatataaaatctatggttttactgtcctatatttgataatacaatattaaagacagaacacccacagggttataaattatttttctcattaagattttaatgtagctgtaaatgaaattctcgttttaaaaaaattaaagtttccatttttttttttagaataaagatttagtgcacaaatacagcccaaagccaacagaaaaattgctttgccctgtcatttccctaagaaagcactgaagttaactcaaaataggctgaaagaaaaaaagcaatcctctgagttctaggtttcacaaaaggaccacgtgttaaactatgtacatcgatttgatgtgcaagtatgcaataaatatgtacacatacattcctatctgctttacatcattctagagtattcatagtatatcaagatgggatttagaaatgtgaaaaggccataacagtgaaaaggaaaaaaaaaagataacaatagtttttagaccagtcgaataataatgcttagctagttaattattttaactttggagcagactaaaaaagttgttttgaaataaatggtacctgtaagtgatgattactgcaatacttgttaaatgttatttgtcagcactgaccggaattatatagtgctagtaacacagctcccactgtcctagaattcctctaaatggccagctatagctaccattatcctgataagcatttcaagagttgtgttgctgagccttttaaaagataactagtttataacctatgtctccttatgtggctacatcagttactcgtggtcccaatgaagtataaaagaggatataagctgctgaagatttcacagaagaaacggagatatcagaaacttcatgatcatcaaacttaaaccaccgttgtcttgctgcatttttacaataggctgtgtagtggcctccatccagcccaccgtagtgatttgaaacagaaaacaaattatatttcttcaaattgttctttggaccaataacatactgtgacaagtcaagattttctaacgggaagtccacagatgtctgtaatttttgtttccacctgccatcgtaggaaaaacgtttcagatgcactaaaagcacaggtggtaacttccagatttctatcttttttagagaatcccgtcgagctctgcaatgactgcagtaaaatctgttgttatctgtgagtttttcttctttggaaaataatctaaggcaatcctgtaatgtacatttacttgtggatgctagtggtagagacaaatacatgaaggcctcaaatgtcctagactttttgtgacatgtgaggcactgtactgtagatttgaattgaccctgaaaaagtgcaacaataatagactcattgagctgcttgtgtttctgccaggcatgttctgcagctttaaagtcatcgagatgatcattattttcttctttatatctcttccgattatcagctttatttagatcttcatggagaccatccattaggaacagaagcaattcttgtgaatcttgctgactgtatcctgcaaactggtcattgatcttcccaatggtgattttaaagtcctttggactgatatatctatactgtcctgtccacagggctttcatgattataccaaattcttctgccacttcacctttatgccccaacaaatttgacctgttaatatcatcctgataacagtttcggttgaaataatcagccaaatgtggagcgttacataggcactgcaatattgagttcatataacaagtatttcctaagttacgaagtccagtaagagctggtccagaacctccaaaaacaggattgaggttccgaatctgagaagcagaaagccttgagatctcagctttaggataacatgttggcttgttttcccgattaactgttggagttactgttggcttcctcttctcttcctcttgaatagcctgggttatatctggggaggagtaggagcgcttcagtttggaaggttccctatcccgctcagcaggaatctgtggcttggctttatgagttggaggggtggaaggaggtgcagatgaaggagccatttccggtgggtacatatgaacagtgttggtgggtgaatgataataacgaaaggttccagtgattgggtcaagaaacttggcccagcctgaaggcagtcctggtacgatcctccccatttcttcacttcgtgctcttgtcaaaggttctcgttgagctttatttctttcggtatcgtctgtatcctctctaaaagttcctgtccttagaattccactttctggttgtcctttaatcttaaatggcttgcctgaacctgaatcccctgtcacagatgtatggggcacatctcctgttgactttttctgtatttctggggttggacaccttttccccctatcttctacagatttcttggcatcagaagtttcatgttcacttttactttgtctttttactcctgttatttctttgcccctctttgctgaggtttctttatcttctttcttggcctgttcactttctttcttctccatttcttcttttgctttttgttgcttctctgtaatttcattttcttcagcttcttgtttctttttggctttttgttcttgttcttccttcctcagtttctctttctgttcctcttgctgcctttcccgaagttctttttcttgtttgtttttttccattagaagagcagtttctgcatgaatacgagccttttcttcatctgttaacatgagagttggagaaaaaactactggcttggtggaacgatcaggaataacttttccactctgaggagattgttgctcatggtttgtactttcagattttattctatgctcttcaggcaatttgactgctggttttttagtacgatcaatctgtggaacattctttatactaggcactggctgaattatgggtgaaacatcagatttagaagcagcaactggttcaactggagttgatatattcagtggtcccattctctcattttgaccacttatcaattctatattttcatctacttctatagatgcaggtggcgtctgggcagcaggtttagaaggaattgattcttccaatgagggataagtaaaatccaatgagatagacacctcttcattctggcgtcgtgggggtggagtgaccttagcatttgttgtatactggggataacaaaggagccagttttcatagcctccctctaaaaccaaaggctcattgcgcaggacagttttactttcccacttgaaaagtgcatctttcagactccggagagttgttccaatctgtaaatctttggcagaactaaaccagtcaagaagtaccacatactccacattccccctcttcttccatgtgtctttagaatcatctggcaggtgtgcttcaatccaactagcagtgactcctggactgatggcttcttcaggaacactgagagaatgtaaaatacaggaatcctgataatcctgcattcttcgagcatccattataatcaagctgatgtttttatccgtcatcattgtgtatagttcctttgctgtgattgctcctttctctttggtctcacatttttcattcttttcaccattgctcttttgggttttgtctttggaatccaaaacattctccaaagagcctttagccaatgtgccaccatcctctcttcctgtttcctgccttttttgttgtagccgctgtgcttcctcctgcctgtctttttcctcaagttttttccggacttcagcttcttcatatcttaatttaaggctttcagagagtctttcagcttcttcgacagcttttttgatgtttccaggtccaagtattgaatggaaataatcctgctgttgcttgaaatcaggtctttttttgataagattataaacagtcacgtatttcatatatagtacataggccctttcctcatcacgatctaatctgcattcttctgctgtcttaaagatcttcagggcactgtgcacataactcttagtgcttattttctctggtttaacttctgtcttcttattaaggtcttttagtgaagaactgaggtagagttctttaggaactgaagccacagcaggcatgatgaattatctttacttttccactttcacaatggatgctatatttccttacaagtgcttctttcctttaggagttgtcccactcctctccgcggacagagcttgtctccggggtaaccagcagctggtggaaggaaaggcgttcatcgttcacagcggacgacttcccagagaacaggtgctagggcccaagacccgcactcaccgtgacgccgggcgcgcttcactaacgccagccttctcgccaaatgcccatctcccaagaactcgagggagaattagccttggctaccaggacggaagccagcccagctc

SEQ ID NO: 13236 - RNA, 4713 nt, Homo sapiens
  source 1..4713: mol_type = other RNA
gctgggattacaggcatgagccaccacacttggcctaaattctcataataggaaaacaataaactatggaacactcctcgacagaattttttataattaagagcatttatccaggctacataccaacagggaaaacatgatacactattaagtaaaacactaggacattaaattgtatatattacatgattaaaactatgtaaatatttgtatctttgaaaaagactgaaaaataattacatatgttcagaatctaatcatttcccacctccttcaatgcaatggcctttgtctcttgggagaggagggcactggagtcctagtctaggggagcccagcaccccagtctctcgcctgcaaccctgttaacagccctgcactggtctctctgctttcaccctttctctctccaacctcctcagcactggccagctagagaggtccttcagaatgtgaatcagctcatgcccctcttctgctcagaaccctaggaggcttcctgtatctctccaactaaaagcttcctgccatggccgtccaggctgcagaatgtcagctcgcctgctctgacctgctgctcggttccctgcctatgcctgcctctccagccatgctggcctcctggctgctcttcaggaacacactccagtctcggggcctttgcacgtgctgttttctctgccaggaatgtgctccctccctccttcatgacagctcttcagagaggtcttacctgggctcatctaaaatagatccactccctctttttgctcccaaaccctttatatttctttatagcacttattaacatgtcccacagtacatttattacatcttctactttctagaatgcaaattccttgagaacaaagactttacgcttgattctctcctgtatccccagtacctagcatagagcctgacacatagtaggtgatgaacaaacacctgctgaatgcaagactgttgtactgagcaaccatccaacgggggctgtaagcggcatgtaggctttgtttcttgggtaacctcccctccttaatccttctggcataggcagactcacagcaggtacccagtagaaggtaaggtggctgatcatttttccataggaggtctccatggcacacagggtagaaagtgcattctgtgaattagaggcagcagagcatggcagctaatggaaactggctctgggaggtcaaattctggcttaacaccaccagctgggcagccttgggaaaattatgacaattctcagggcattaatttttccttgtgcagaaagagaaggataatgacagctcctatttcccagggctggggaataaataagagaatgcccccataaagcaattagcaagcacagtgcctggcatggaggtgacgagcaacgagaagcagtcaaattaatcaacagccacatttgtgcctttgtctctttcaagtttacaacgtgctcttatatacatgctttagctgatctgggcctttgaacaacctgtcggtttttatcaccattttataggtaagaaaattgggtcagaggaaaaagtgctagctcacagaacacaactgaattttgctagaacttctggtgccctttctttcagaacacaagtgattattactgctgatatgaatcaaggtgatttggagctgggcatgcagtctcagctaccagagaggctgaggcagaaggatcgcttgagcctgggagatcaaggctgcagtaagccatgatcatgccactgcactccagcctgggagacagagcaaggccctgtcttggggggaaaaaaaattaggcgggccccactggagccccagactctaaagtgtgtgcctagtgtaaggctgtggatggcaaatgaattccaaaatgaaatcagccagccagctacaggcttacaacctagtggtggcagggagtgtacgggctccctcatctgcagctccttctctggatgaggcttgagagcaagtctggacaggcaaaccatctctcagtccacccaggacttaaaacacttcattgttttcccaaaagggaaaaatagcaaagccctttctgtacagtttctcctgcttagagttgggtggcagctctatacagcaaatgctgactttgctgtttgagatctttgatacagtgtgacctctgagctctgaaccaggctgcccctgacaaaaaaagtgtttcctcccacaggtaaacaaggaagaaggcactgcaaggagctctgggcctggctcagtggaggctctgccacctttccaggatcaaaggccaagggaggtgacatggcaaggaaaagatctacaggggtcagacaaggaattttagaaccacaaggtcaaaaaaccatgggctctcaggagtcacagattattaaaactgcagcatttgagaccaaaacactcatgacttagagcaccttaagcctcatggtgttggcagagattacattggaagggaagagtcaaaaggtgcttctccactgataattctgatggcttctgggccctgggcatcttctgtgaggtcagagccttggcaaacgttccctcgtgagaatacggcctgaaggctccagctgcaggaggacggctgggagaacaggctttggatatcaaccgaatgccaacattctaccaaccaggccccactggggcaagagatcagaagagatctgatggtgccaggtttgcagtggccatcaaccaccaaaagactgtgagaacaataccatgatagtgtggcttgatggtatgtgctccttgccaggaacatgctgcgtgagtggcacttagtcgcccacagagcgctgcacagcaccacaaccgataacttccatttgcatagtgtttacagcacaggacagcattcatcccccaagccccagaaatggcctaggaagtaggggacaacaatggctctggccaggcagtggggatggctcttgagggccacattgggggacaccttgaaaagcagccaaaagacccacaccagccccagcctcatccacattcagttaaggtcactttaggtacctacattaatagaattcaatgattttcaaaaaccacagagagttctaggatagtcatgaccttgtatcaaaattatagaaatctctctataaaaaaatctctctgaagagttcagcatcccaggctgctcagagcagagtggaccagaagacggaggctggactgctttgccagtgtgagaaattcccagaagagcagaaagcacgtgcgatgggagatgctcctgctcctaggaacctgcaagtcctatgccctgggatatggagcgtctccctccttgaggggtccctggcactcttctccatctttggcaggtgagaagaggagtttgcaatcccggagcacctctggctgccaggcctggctggaaggaccagctcagactctggtccctccaggatcagagggtctggtgctccggccagaatcagaactcgtcccgcagcttagggggcctgtccatgccgaagaaagaagacggcctcccctggaggtcccgctcccgcttcacaaaggcagtgaaggaggagacacagttgccaataaagtggtcggcttggccgaggatgtacaggtcgacctgggccacctcaggcttcaggctcaccaccttcaccttccctttgaagagctgttggagctcaggcacataactctcggaatcagtagcaacgtagaccgactgggcatccagcgacctcacccagagcttcacagccctctggatctccttcaggtcaggcaggcacatagtcatcgtgaggggggccgctgtgctgcggctgtagcccacacactgcggagaggccatgaagtgcgagcctgcagtcccgtccttcagcatggcacaggcgttcttccagtcagagccaatgcgcagatgaatgcccacatagggccggacaaggtgggcatgaatctgggcctctcccgtcttcaccatttcgtctgaccataccatgtacttctgtagtggcctgtgttcctctaggacggggaactgggctggggctcctggcagggcaagcaccggatgttcctttggagaaaatctctggctccattgttctctgtaggaagcactgaaggaaatgcctgtaaaaagctccgacttgttgaaactcacatgaaactgatcccagaatgggccaaaggggtttccttccttcatggggcacgtcttcttatctgggcttcgctgggctgccacctcaaagcagtatgccacccgcttctcagggggccagtgggtgggtgccagcttctccatgaaatcctccaagctgatgacccgatggtaagcctggaggggctccagcttgaagtacttctggtaggacacatggaggttggtgaaaggaggcttgtgatgctggtactcaatccaaggagggacagccaaggtacggtttagcagctttgcaaatgccagagagcccaagaagtgatcggcctggttcccaaagcgccccatgcaggggcagtagagcaggtaaccggccgggtcccaggagcccgcaggcatccccgggagcggcagaagcagcagcaggaaagacacgctcagcggccgtgcccacgcggcggcgcccatgtcggcccgggaacccgagccagccgcggcgcacagtcggggagggaaggagggacgcgagc

SEQ ID NO: 13237 - RNA, 4905 nt, Homo sapiens
  source 1..4905: mol_type = other RNA
gctgggattacaggcatgagccaccacacttggcctaaattctcataataggaaaacaataaactatggaacactcctcgacagaattttttataattaagagcatttatccaggctacataccaacagggaaaacatgatacactattaagtaaaacactaggacattaaattgtatatattacatgattaaaactatgtaaatatttgtatctttgaaaaagactgaaaaataattacatatgttcagaatctaatcatttcccacctccttcaatgcaatggcctttgtctcttgggagaggagggcactggagtcctagtctaggggagcccagcaccccagtctctcgcctgcaaccctgttaacagccctgcactggtctctctgctttcaccctttctctctccaacctcctcagcactggccagctagagaggtccttcagaatgtgaatcagctcatgcccctcttctgctcagaaccctaggaggcttcctgtatctctccaactaaaagcttcctgccatggccgtccaggctgcagaatgtcagctcgcctgctctgacctgctgctcggttccctgcctatgcctgcctctccagccatgctggcctcctggctgctcttcaggaacacactccagtctcggggcctttgcacgtgctgttttctctgccaggaatgtgctccctccctccttcatgacagctcttcagagaggtcttacctgggctcatctaaaatagatccactccctctttttgctcccaaaccctttatatttctttatagcacttattaacatgtcccacagtacatttattacatcttctactttctagaatgcaaattccttgagaacaaagactttacgcttgattctctcctgtatccccagtacctagcatagagcctgacacatagtaggtgatgaacaaacacctgctgaatgcaagactgttgtactgagcaaccatccaacgggggctgtaagcggcatgtaggctttgtttcttgggtaacctcccctccttaatccttctggcataggcagactcacagcaggtacccagtagaaggtaaggtggctgatcatttttccataggaggtctccatggcacacagggtagaaagtgcattctgtgaattagaggcagcagagcatggcagctaatggaaactggctctgggaggtcaaattctggcttaacaccaccagctgggcagccttgggaaaattatgacaattctcagggcattaatttttccttgtgcagaaagagaaggataatgacagctcctatttcccagggctggggaataaataagagaatgcccccataaagcaattagcaagcacagtgcctggcatggaggtgacgagcaacgagaagcagtcaaattaatcaacagccacatttgtgcctttgtctctttcaagtttacaacgtgctcttatatacatgctttagctgatctgggcctttgaacaacctgtcggtttttatcaccattttataggtaagaaaattgggtcagaggaaaaagtgctagctcacagaacacaactgaattttgctagaacttctggtgccctttctttcagaacacaagtgattattactgctgatatgaatcaaggtgatttggagctgggcatgcagtctcagctaccagagaggctgaggcagaaggatcgcttgagcctgggagatcaaggctgcagtaagccatgatcatgccactgcactccagcctgggagacagagcaaggccctgtcttggggggaaaaaaaattaggcgggccccactggagccccagactctaaagtgtgtgcctagtgtaaggctgtggatggcaaatgaattccaaaatgaaatcagccagccagctacaggcttacaacctagtggtggcagggagtgtacgggctccctcatctgcagctccttctctggatgaggcttgagagcaagtctggacaggcaaaccatctctcagtccacccaggacttaaaacacttcattgttttcccaaaagggaaaaatagcaaagccctttctgtacagtttctcctgcttagagttgggtggcagctctatacagcaaatgctgactttgctgtttgagatctttgatacagtgtgacctctgagctctgaaccaggctgcccctgacaaaaaaagtgtttcctcccacaggtaaacaaggaagaaggcactgcaaggagctctgggcctggctcagtggaggctctgccacctttccaggatcaaaggccaagggaggtgacatggcaaggaaaagatctacaggggtcagacaaggaattttagaaccacaaggtcaaaaaaccatgggctctcaggagtcacagattattaaaactgcagcatttgagaccaaaacactcatgacttagagcaccttaagcctcatggtgttggcagagattacattggaagggaagagtcaaaaggtgcttctccactgataattctgatggcttctgggccctgggcatcttctgtgaggtcagagccttggcaaacgttccctcgtgagaatacggcctgaaggctccagctgcaggaggacggctgggagaacaggctttggatatcaaccgaatgccaacattctaccaaccaggccccactggggcaagagatcagaagagatctgatggtgccaggtttgcagtggccatcaaccaccaaaagactgtgagaacaataccatgatagtgtggcttgatggtatgtgctccttgccaggaacatgctgcgtgagtggcacttagtcgcccacagagcgctgcacagcaccacaaccgataacttccatttgcatagtgtttacagcacaggacagcattcatcccccaagccccagaaatggcctaggaagtaggggacaacaatggctctggccaggcagtggggatggctcttgagggccacattgggggacaccttgaaaagcagccaaaagacccacaccagccccagcctcatccacattcagttaaggtcactttaggtacctacattaatagaattcaatgattttcaaaaaccacagagagttctaggatagtcatgaccttgtatcaaaattatagaaatctctctataaaaaaatctctctgaagagttcagcatcccaggctgctcagagcagagtggaccagaagacggaggctggactgctttgccagtgtgagaaattcccagaagagcagaaagcacgtgcgatgggagatgctcctgctcctaggaacctgcaagtcctatgccctgggatatggagcgtctccctccttgaggggtccctggcactcttctccatctttggcaggtgagaagaggagtttgcaatcccggagcacctctggctgccaggcctggctggaaggaccagctcagactctggtccctccaggatcagagggtctggtgctccggccagaatcagaactcgtcccgcagcttagggggcctgtccatgccgaagaaagaagacggcctcccctggaggtcccgctcccgcttcacaaaggcagtgaaggaggagacacagttgccaataaagtggtcggcttggccgaggatgtacaggtcgacctgggccacctcaggcttcaggctcaccaccttcaccttccctttgaagagctgttggagctcaggcacataactctcggaatcagtagcaacgtagaccgactgggcatccagcgacctcacccagagcttcacagccctctggatctccttcaggtcaggcaggcacatagtcatcgtgaggggggccgctgtgctgcggctgtagcccacacactgcggagaggccatgaagtgcgagcctgcagtcccgtccttcagcatggcacaggcgttcttccagtcagagccaatgcgcagatgaatgcccacatagggccggacaaggtgggcatgaatctgggcctctcccgtcttcaccatttcgtctgaccataccatgtacttctgtagtggcctgtgttcctctaggacggggaactgggctggggctcctggcagggcaagcaccggatgttcctttggagaaaatctgagaatggtttggcacgatggtgcattgccttccaatagtcaatgtgcagtaagcgtcagctgaattagagctgtgccaggctattcacaggctcagaacgagcagagctggaaggatcctcagaaatcacgtggtaaagaagaaatacctcttatcctctttccctcgaacccagttttcagctggatacgtggcagcctctggctccattgttctctgtaggaagcactgaaggaaatgcctgtaaaaagctccgacttgttgaaactcacatgaaactgatcccagaatgggccaaaggggtttccttccttcatggggcacgtcttcttatctgggcttcgctgggctgccacctcaaagcagtatgccacccgcttctcagggggccagtgggtgggtgccagcttctccatgaaatcctccaagctgatgacccgatggtaagcctggaggggctccagcttgaagtacttctggtaggacacatggaggttggtgaaaggaggcttgtgatgctggtactcaatccaaggagggacagccaaggtacggtttagcagctttgcaaatgccagagagcccaagaagtgatcggcctggttcccaaagcgccccatgcaggggcagtagagcaggtaaccggccgggtcccaggagcccgcaggcatccccgggagcggcagaagcagcagcaggaaagacacgctcagcggccgtgcccacgcggcggcgcccatgtcggcccgggaacccgagccagccgcggcgcacagtcggggagggaaggagg

SEQ ID NO: 13238 - RNA, 5070 nt, Homo sapiens
  source 1..5070: mol_type = other RNA
gctgggattacaggcatgagccaccacagacagcctctacatcccctttgaatgtacataactagactctttgcctgagtcccacccatttctctgagcttcttgcgttctgggaaatgactaatctttgacctccttcaatggttcattggaaaaattcaacccgatgggtcctctttactccccttcttctttttcaagagaagttccctatctaccgttcccacctccttgctagtcatttcacattttctctccttcttttacattgttaacttaaaacatactcactgtcttctgggccacaagacccaacaccttaaaccagatgtcaaagaaagaagccacgggaagtaaacactttgcttatccacactttctaaataatacatgttcaaattctaaatatggcatatcttaaaagttttttctcacagattccctctaaactgctctcttcatataaaatgatagccacacctcagaactgcagcaaccaaagctctctctatactgacttgcagacaataaaactgccaggtggtaccaaaaaaaaaaaaaaaagaaagaaagaaaccccacaaaaacctcatcattaaatggaatgttgttaagaaatagctgttttatttaacagctattcatttttattgaataaacattttctagtatgcattctgttaattgacctgacagcatatgctgtatatggagaaacttctaaacattatgctctatgtaatatgcttatctgaaaaagctctcatttgcagcaatatggaaataaaattctgctttctaaaattcaagacttttaaaatgcattaatccacacagtttatgaaattgttctggacattttaaaatcctttctttaaggaaaaaaaaaactttagtaattgctaatagtatttgttgctgagtttcataatggagcagtgcacatccaatacaacttttacagacatagaaatggtgcagggataataggaaataaaaagcagttatggtatcgggtaaagaattactcaacagataaaagaaaatgttcagaaactctatcaaattatattattagaaaactattgttataatagtttcatggctcagacataaatagagttgaaacattacagagataatacatttagtcttgaggaagaaagacagtttgtgagtgtgttggcgggctctaccagctaatggcagcacctctcttgggctgatggcttctgagtgatgagtctaccttccagcccagaatcgccaactccgctacctagaggcataaatgagcaatgctgctggtgggaacgagagcaggctggagggctccctgtcttcaatagcaattcatctcccaacaattgttgccgttgtgggactatcagcccaaggttaccagatattctaatttttcaaaagaagatggaaaagccagatttgccccatttctctaggttgtcaactaactaatttttagaaatgacaataccatttgaacgcaattaagccaacctataaacaaaactcactatggaactagtgcactccatagtgaatctttgtcagggccctcccattctgaaaacggcatttgctgtaatttgtaattatctttgataatatgaagcaaacatggaaaggtttgcatttatttattttatatcctggcactgagtaaaaactctccccgtatcctcaatgatggtattggtgcaactggaaaatcctccaacattcaatataacacacagcgtaattaactcgtttttataccaggcccttttaagccagatctttgtgttccatggacttctaacatattttacagttctaattctcttccactgtcctacattaatcaaagctgtaacccctgttgtctttgtactacggaatctgaatgtgcccctggcgaggaatgggggaaaagtcaacaggaattaaatttcagtgcaactgtttactcaactgtggcctgcagttattgaaattttatccgtggttttgtgtgactaccgcagtaatgaattcagcatggctatgattttctcactgctggtattctcacttcaagtaaaaacctgtagaataaaaatgatgaaaacaaccatagtccattgtagaatgctcacatttctccaaactgtctaattgtcgcagttttcagtctggaagaaaactctgataactctagtcctgtagaaatattttcaggcctgtagtttttcttatttcatctacagatttcccttttccccaacaacctgttaaaagccttatcatatacttaggggagttgaacagctgtcaatgttatattttaaaagacttcaaaaggctttgctaatcacaatacagggggttttagccacagtgatagaccccactgctttgtttcttcccaaaatgtgtcaacgacatacggagaaaaaactgtcataaaaacatttaaaaacagtataaaagtctaatcataatacatttcttgacctttgtgtcaataacccataacaacaaattttccaaagtggacacagccaaaggaagatgtggataaatatgtttgcaactgatactttttaaggaagatgttggtgaaatatgcttttataattttattctatgtagccaatttgttatcactgttgtgtgtgtgggcgcatgtgtgtgtgcacatgttttgatggtttatatgtaaagttttttggctggcttactactttgagatcctgaatgatttttagctcctcaaaaaaaatcagaatttcccatttatgtaattaatgtactctaaatattaattatttagtatcacatcagtcagtagtagccccatatcaagtgctcaagtgcttcataaagaaatgggcaatcttgacacttgtctggtaagggcacagaagatagcattcagcaacattaactatttgttctgaataaaatggctgagaacatcacatgaacatgtacttgcacaaatacacggagacccttttactatctactgctgggttttgctaacaacctcactggttggaatttggccatctgcactaacttaaatgcacaaagtttatacacaacaagcatcacaaattccagctgaagtgagccagtggtgcaggcacaaatgggtttgggctgccaatgaaagaaagatcaaatcacttgcaggaagtcctctgaattaagacttttgctggtctgttacttttcctttctttcgctttgttgcatctttctcccaacaggttccacaggctcatgttggttccaccaccttgtaaggagctaacagtctaatcattccttattccttaaaaaactcttcgcaaggagaaaataaaacatgctttatagcttgtctccaagttgcatcccaaacaagcttagcttctctgacacagattccaagaaaatggtttgagcactttgtccctatcttcttcctccccacaagagttcctgcagctttcagaaaggcccaaagatacttcattctttttaattcacctgtttctgagtggcgccataactatgttttgaataagtaaatcaagaacaaaaccggtcataaaccatctattattattaacaaagcctaataatatttcctgattccgaggaatcaggaaaggcgggaaaaccaaagccagtcttcaagcaaatgttgtttacttatttgaatatttatcaacactttgacaacagaacactatttcttgggtcgcctgtaccattcggaaatattttaccagtcactcacaggtacccaggtccatacctgtaaaaagtataactaacaggaatgagtacatcccaacttatgtacattttggggaggcaccaataagagctaatttaaagcagtaagacttagccacaaacccagtgctgcatgaatacagggaacatatgtaaatactctatacccccaaatcctactcgtagagggaagcagcttcctacagtgatgcccgtgttctagatgttttggctgttatctcgccatctccgcctgtctttctatgtatttatttcaactctccttactcatctactctttttctctcttttattccttagctcttatttccttcttcacaggcttaagcctgtttttcgtttaatttttatttttgcatgaaagcagtgggaaccatttctccaaagaataattttattcaaaatggggaagggttaggctgacacacaggtccactcatcttcgtctcagcaactgctccccacaaggggacctgcaggacttccaactcccaagggcttgaaattagtctcttaagccaactgctgggactcctagagggctgatggtttatgagatgccactgttgctgctgctgctgggcgtgggcgaggtcagctgccccgatgtccacggccggcgtctctccgttggaccgcccctcccgaagaccgccgcactctagtaagtggttgctgccgcccgacccattctggatggctgaaccgttactttttgtctcagtcccagattcttgcatcatgactcaaaaaccttttttggcttctgtaaagcaatcttcagttatagtcacctcaaaaggtcacgtcttacccctgaaattttaacgtgtctcacagccataaaaagcctggggtcactgggagggggcatgcataatgccacaggactgcaacacacagagggaagccttttggctagcaggcatcacatccatccgttcatggctgacagcaaatcagagaagggatcgaagccctcaccattgccgaaatgttttgttcggaaactggaattgtcaacaaaagcttctgggacaccgcggagtccggggagggagtaggagcgccgccttcacgcccgcggaggaggcgccggcagcaccatggtccccggcgccgctgccgctgcccccggcccgctcgctcgctcgccgcgcgctctcttcctcttacaaactttcgggttccgctgcaaatggtctctcggtgcaaactaaggtgttttcgggcctttccccgcgcgcgcccactcccgcccgcgcgcgcaccccgcgc

SEQ ID NO: 13239 - RNA, 1446 nt, Homo sapiens
  source 1..1446: mol_type = other RNA
gctgggattacaggcatgagccaccacatccaacctcatttgactctcctgacagtctgggaagtttaagcagggaacccagctgcaactatctaatgaataatggacagtttagcatcttaactaataaggaatcttgggcttaagatattcccaactttattactgggttgtgactaagtttcctctcccacttccccccaacaaaaggctatatatactctattagcttttatatttaaatgaaggcagattgattttttttaaaagacattgaagacacccctcaaacaaatggaagcactctgggttttggtaaagctggtgttaatcatatctttagcttcttaacaaggggaagaaattacttgtgggcactttgggtttttttgtgccatcagtaatccccaggggaaaatgatacgtatatgtttttccacaatcagttcaggataccaggatattaatggtatacctaaatcaacataccaacaaactagctaatgaggtattaatagtatacctattaataggtaaacagaagtaaaatcatgtaccaacaaaacaaagcagtgattgtttagagaggtgaatgggatttgtgctaatttgtaaagtgtactaccttaggcaagcactagaaacaaatattgaacaccttaatatttagttgtatatcaacttacagtttacaaagttttccatacacaggatctcatttgattattataaaatccctgccgcccgcgcttcgacgcgtcctttcctggcttgtgcaatttccccttctccatagcactgagcctcctctgcagggccgcctgcctgcgtagccagcagtaccgaaccacgtagaaaagcagcagcagcaacagcaccaccccgaggacacccccgatcacagctcccagaacgaccccgtacctagttggcactttttcaaagacatacagcgtgacctgagaggtcttgcccactatgtctggagggtttttgacgtcacaagtgaacgtgccattgtcactgtagtctaggttgtgtatgacaatggagccatccttccagcgagggtcccctacccactggatgcgctctttgaaggtccccacctcgtcaatgtagggttgtcccttggcatagtggaagatcgaaatggcatctctgcccccttcgggctggtagcgccaggtgaaggagatgtcatctgagacccactcactggaccagaaggagcagtgcagggtcacccgggagcccacagcaccatggacctccctgtcggtgtaaaccacgatggcctgggccggggacagcaccaaagaagagaagagcagcacagccaggatagggctggggctggatgagggagccccaggagccatagctggggcaggggcaggggcccggagcatctgtggggttgagaaagtgggggaccaggaactg

SEQ ID NO: 13240 - RNA, 2470 nt, Homo sapiens
  source 1..2470: mol_type = other RNA
gctgggattacaggcatgagccaccacatcccccttaatacacatcttgaaggaatggatgaatcagtgaattaatgaagctggacgcggctgggcctcaaggcagagttttggggaggtggtggtgagagaaggctgcagtaatttcactccctcccaggaaaacagcactttccttgcagtgtcctgggtaaatgtccccagccatgaccctctggagctatgcttccttaccagggatagctgctctcggagctggatgaccacccgtttgtgtgctccagctaaggcaatgaagtaaaacatgatgaggcaaataatcatgaagaaaggaactgcaaaggcttcggatgtgacaccatggatgaaggactgcagcgagctggggaaggtgctcaccgtcttggggatgacctcccaggtggtgttgaagttggtgaacggcccacaggctttcgaggaagggatgcgtgatatgctgattgtcagaggtattattgccaaacacagcccgatcaacaacaccaacaggaagaagaaattagaattggatgctctgaacggcctgggggagggtctgcaggtgtaaagcagactccactctttcacatagaagatgataatgaatttcagggttgcaattgcagggagaaggggtgagaaaaaggctccgatccagcagatggtttgcccgtaaactatccccaggacgttatcaggaatggcaaactcctgctgcccccagcactgaatcagcttgcaagaggaacagtaggtcaccaggagctttctaggaaaatccacgaagagtgtcacagccaagatgatgatgaagtcgaagatcatcagcttgtacatttcctgcccaacttgggtctcccagcacgggtagagtttctggttgtagccgcaaaggtcacatgtgtcatcatcacaggatgtgatcttggagcccagcgtgaacaccaggacacatatggtggccagccgcataaagacacacctaaggattgtcagacggatctcaaagcctggagaataatcctcatagcggatgatcttggcaaagatcattggggtgataaaattggccagcgtgatcacaatagacggtagatacaatatgaagaggttctctccaaaaaccatcttgtcgatttcctttttcatgtgctcttgcgagaagacagttgctacgtatattgcataaaagcatgcccctaaaacagccagaacaatacagttcaaaaacagtctcaaagagtaaatgcgtattgtttcttctgaggtcctttctgctattttctgccgcattctttcttcctccagatctgctcggagctcgtaccgcaagctgctgtgcttcagatccgccatgctgcggttagtgatgcagaagtcccagccggcaaatatcttgttgcagtaactctgaaagtgctcctcactccgaatcaggttgattttgaatccttccaccgaccttttcactatccaaagaaggctcagggccagggaggcgattgtgcttaacaaatacgccaggggcagatcataggtgaagttctgaaatttcaccccatcaatggtgtaatgtccgtaaaagaggctagtttcctccaggaaaccagtgccagaaagcaagtctatgatataactgtaaaagtaaatgagtccagaactgcttactggatagactgtacattgtttatccatgtctttgaaaggaatgagcacgaagctgctgttggtgatcttgtatttcgtgagtaagactgggagcaaaaccagcataaagatgatcagaaatatcaccaaattcagcaacaccaggaatctcaagaaggagaaataggactgaatcccagtgccaaatttcccttctatgctgcggatgtcctcccgccacagctccaggtgggtcgtcatctctcgagccttctctaggaacctcttccaagacttgctgctataccgcttccactggtcccattcggagagatacttcatttgtgtctcttgaatgtcccttagtctccgcttctcagagatgttcagtgcataatttcgaagagaatggctgctgaggttttcagcgattctgtcctccagctgggagctgtaagagtcggttggctttagcaaagttccgctttgcttgtcccgggaatggacagtcgttctcctacgtgcaatggaccggtagcttggcaattcttggaggaagttcacaggtggagaagagaagcaactggagtctagagagaggttctctggatggaccgccggctgccggctgggcctgccgggctggagcgcactgccgctggactcgctcatggccgcgccccgcgctcctcagaggctgccgaggaccctctccagccgccgccgccgccgccgcctccccggccttccctcgcggagccgggattccaggttccggcgctgacatcacagaagccggagt

SEQ ID NO: 13241 - RNA, 5855 nt, Homo sapiens
  source 1..5855: mol_type = other RNA
gctgggattacaggcatgagccaccacatccggccataaacccagtaattttgtatggcagataaaacattttatggaatattctttatgatagccaacttactgtagtagtcacatctgacctttgataatttttttaaattaagttctgatgacaggaaaagatagaccaaaatatttcccaacctggcagatatatacttaatctgttcagctcacaacagagagaaatggtcatattgagatggataaaaattcagatttgagacttccatgtatataggcatacctgtgtctgcaaatgagcacattttggaacgtaggagttagcatacagtatgaaagttgaaagcaaacaatgctggtttctaaaagtggatcccttttcttcactgaacatcatccttagacaccacaatttccaatatacttaaaaaccatcaacccctaaaaagttataatgatttgcctattgatataaaaattttcacaaaactagcgagaaagaaaaaccccttgactccaggaaaaccttttcataatgcatcccccaagttgggggattaaatcgctgaaatgtttatttagcactagagaagtaaattcaaagttgcctgtgggtagacgtacaatagaattggttgacaaagtttggtttataaaatatacttacatattgtttcttaggcaaaaatcggcagcaatctggaataattcagattttttatgagattaattgccaatctttttatctgtgacgataatgccaaaaatgactcagagccaataaccttcatctgtcatatggaagaaacaatcctagggcaatagttttttcaaaagcggaactgacaaagataagcgtttaaaagggtcttgatcaattagttacaggaacatgaaagaaagtgttccacagagaactgtgtctcctaaaatctctttcttctatcatctaccttacccaaaatttctcaatccaaccacatctacctgctggtccatcagataccagatgcctttacatccaaaattctcttaatgctttttttcccccaccaaagttctcattacaaataatatagattggaagtttggaggatggaggggaataaaaaggaaaagtaaaacaaagtcactttccccaatccatatataaaactacaaaagagttttcctgtattgaaattaacatgcttttgtaatgagcaacgccttagtggtagggtattcagtgaatttaaactaagttaacagaatctgagaggcaaagaactaaaaacaggatatacagttaccccttaaaatgtcatttctgttaccaaaaagcctgcttcagtaccaagttccaacatatctgagttatgctacttcacttttagccaattccaactttgatactttaagaaaaaatcattttattgttaaaaaagaaaaaaaaacttagatcttatagttcatgaacttctaggacaagataaattcctctgttttagacacaaaatagatcacgtcagttaaatagactttgttttaattcactcactgaaacatctccaactactagcaaaaattccgaatgtctgaatgcacactactcttcctaatgtggggagacaactgtgtgctttgtatctttcccactcaaattggcttataaaatgaaattattttaactatccaatggaaggtacataatttaaaacatcctatagaaatgacatgttactagtaatttacaattttaaaaaacagccacaaaaaagtcaaagctaaaaacaagatttttactatgaatcagtgcttctattatccttctgaaagaagttatattttaatgtgatgtaaaggcaacattgaaatttcttctttaaattaaccacctaatttatccctaaaattacaaagaatcagtcttttacaggtcaagtgcagtaaactaaaatgttctctcagcacaaagcagcactagaaaaagtaacagttatagatgggagttgactagttttgcagtggctgcgccatcaataacaaacagacatcagacggtatccatcccagagcacagacactactacagactagatgcgaagaatgcgtcacactcttggctgataaatgtcctttgtctttgactctttctagtttgaatgaagtggattttttaaaagtttaaatcaggtcacataagttggctgcttaaataacatcatgatgaggtatgaaaagctctgaatatcccttacattcagcaggatttaccagagatgtataatagcttgtcaggggcaacttccaaatagtttttacactttggggttataatgaattctagaagaggacaagtctaaaaaggtttaaaagggtatgctctgaaacagaggtgagcaaccttttccttcagaattcactttgaacagcacatcaacaaaaaaatcttctctggtagtgtatcccaacattgagtcaagatggccaactagcaccgagaagtcgtattgaactcatttgcagttgtcttggcaattaagcgtattttttcattccagtccaagcacaaatgtggatcactgaacacagtactggaagcgccatttgcaggtacagattgcagtcatcattaaatgagccagaaggcagatactgtttttattttgtgtggggggagggggaagcggcacagtactagcaggagatgaaataaaatgattaggaaacaatgaggttataagatcactgttcttatttgggttaagcaggtcatgttgagaagatggttatttctttcagataaggatgctacattaaaggaatcgtgtgcagcatgaaaagattagaatcgagctgcacctaagaaaaaaatcccaaagttactttcaaaagtatgtgttatctgccagtcacagaggggaaaagcacctagggtgaactccaattttttaatgaggaccttgatcaggaccacaaagcctgaaacatttattttaatgcagaaacacagcccctagttacactgattgcatttgggaaaattggagggttttttcgtccttagttttttttattaaattacaggatatggttttcgattactaagtattcgaaatcctcataccagcaacagaaatgaaccacttccaaattctaagacacaaaagaccaaagagaagcaaaagcgatacaaattaatatgtgcccctctcctttctgctctaagggaatctacaaaccagtatcacatttaggagtcaaagtgttaattcttcagcattcctgacaactagaaagcacattcactgaaggctgaaggtgagggagtggatggtttaactttaatatctgaagaatggcgccaatagaggaaagaaaaccatccaatctcagtaaggattaatgcaaatctggctagaaaaagccaccaggtaatccaagggttcactgtggaagaactcatgaaaagtactctgaagtatacacaacaggtctaaacatctcccttgtcgtaagtagttgtgtaaaattcaagataaagatttagtctcatcttttaatgtcagttttttcccccatgttaaagggaatgaggaggagtcctcttttattcccccacaagaaaaagggagccacattaatatgtgtatattcccataactctaatgtaagtgcggatctccaaagcctagggatttttccgtaaaagagagtgggccgttctggttacccttttattagaagggtattccaccacagagagccggaggttttccagatgtgtgtaagagagcaggtgcgcaaggcaagcaaatgagcgcaaacagtattatggaaaacatttgagaagttagctccatgaggactgtgggctccacaagaggactcgactgggtagcctggtctgacacaggtacgtgaaagcagagtattgcttcaaagctggaaaccttccataggagcctcacactgttggaagatgtactgctgctggttaaggtcaacctggggtgcaatgctgctgtcttcatcttcggtcccgaagtaatgctcaataagatcaaaggccttttggtagatctcctggttttcatgactctgtaagaactcaattttatccagaccataagcttcttcaatcaaagcacagtaagggttaatgccagtgccattccttttggcttcctgttctccaagcctcaggatattttccaagccatttagggcaacctgtacaatcttagagtccatgaccgtgaggagatcacagagcggcttgatacaacccagttctactaggtacttgatctgttcagctgatcctccagaagttgcatttgtgatggcccaagctgcttcttttcttgtccgaaattcagcagtttgtaaaatactaatgagggctgggaaaatgttggcatctatcacagtctggatctgtgccctatttccagctgtaatattagatatcgtccaacatgcttcctttttgatagattcctttgggctactcagcaaatgcaataaactctgcagagctgagcaattcagaattacctgtgtctgaatatcatcccctgtgacaatgtttcccacagctcgcaaagcaggagaaaccactttataatcattatgcatcagcagttccacaagtctcctacatactcccgcatcgatgaccgcttgaattttatcattgggtccatctgatagatatgagagggcccagcaggcatcagccagtacatcagtgtcactgacaaacagcaaccaggaaagcacattcagacatggagaaacctttgcaaattctggaggtggacttttccctctacagagattagacaaagcccatactgcattccgggtcatggtcaggcggttttgctttgaaaataactgcaaaagagggggaaggatattgcagtctaagacatagtccctgcacatggtactatctccagcaatgttgccaagagcccagactgcctgttcctggacatcttcaaactctgagctgagcaactctatgaagatgggcacagctcctgcctgaatcacaattcgggtctgaagagaatttcctgaagcaatatttgtcagtacccaagctgattcaaactcctatcaagtttcccactccaggttgaggtacgcctggttccctttctccatttggatcaggactctgttgctggccactttgccggttccactctggttcctagcaaatgccaggctcacctgcagtgtacaattctcttttcgtttgaggaactccacaaacctggccactactcctggtgtgctgataacttcatcaataggagggttaggttcttttgaaagcagcttcctgaatttctgtgttgctgaaagctgttgctctgggcttttggaaaatatcatttcaatcatgtcagaagtgatgacaccacctggtgccatctccatgttactaatctgagcctcatgaaagcctccatctgacataacttcttcttctgtttcttcttctgctgtagcaacatttctccgcttgaataactgctcttctcttttctgctttcgtaactgcagtccttcttcctccctcctcctgcgcatctcatcgggattcagagatttgttcttgtaacttttcaggcgaaagttctcttttcctggggtggtcatgatttcaggctcaaggcaaccgatcccggtgccaccgctgaagttagcccctcgctcgcccgcccgccgtgccactcccgcgcacaacctcgaagagctggcccgcgcctcggcggtgctcaccaggcctcgctctccgccgcctcgcaccgagcagcgagactcagctcagccggcgttcgcagtgc

SEQ ID NO: 13242 - RNA, 5732 nt, Homo sapiens
  source 1..5732: mol_type = other RNA
gctgggattacaggcatgagccaccacatccggccataaacccagtaattttgtatggcagataaaacattttatggaatattctttatgatagccaacttactgtagtagtcacatctgacctttgataatttttttaaattaagttctgatgacaggaaaagatagaccaaaatatttcccaacctggcagatatatacttaatctgttcagctcacaacagagagaaatggtcatattgagatggataaaaattcagatttgagacttccatgtatataggcatacctgtgtctgcaaatgagcacattttggaacgtaggagttagcatacagtatgaaagttgaaagcaaacaatgctggtttctaaaagtggatcccttttcttcactgaacatcatccttagacaccacaatttccaatatacttaaaaaccatcaacccctaaaaagttataatgatttgcctattgatataaaaattttcacaaaactagcgagaaagaaaaaccccttgactccaggaaaaccttttcataatgcatcccccaagttgggggattaaatcgctgaaatgtttatttagcactagagaagtaaattcaaagttgcctgtgggtagacgtacaatagaattggttgacaaagtttggtttataaaatatacttacatattgtttcttaggcaaaaatcggcagcaatctggaataattcagattttttatgagattaattgccaatctttttatctgtgacgataatgccaaaaatgactcagagccaataaccttcatctgtcatatggaagaaacaatcctagggcaatagttttttcaaaagcggaactgacaaagataagcgtttaaaagggtcttgatcaattagttacaggaacatgaaagaaagtgttccacagagaactgtgtctcctaaaatctctttcttctatcatctaccttacccaaaatttctcaatccaaccacatctacctgctggtccatcagataccagatgcctttacatccaaaattctcttaatgctttttttcccccaccaaagttctcattacaaataatatagattggaagtttggaggatggaggggaataaaaaggaaaagtaaaacaaagtcactttccccaatccatatataaaactacaaaagagttttcctgtattgaaattaacatgcttttgtaatgagcaacgccttagtggtagggtattcagtgaatttaaactaagttaacagaatctgagaggcaaagaactaaaaacaggatatacagttaccccttaaaatgtcatttctgttaccaaaaagcctgcttcagtaccaagttccaacatatctgagttatgctacttcacttttagccaattccaactttgatactttaagaaaaaatcattttattgttaaaaaagaaaaaaaaacttagatcttatagttcatgaacttctaggacaagataaattcctctgttttagacacaaaatagatcacgtcagttaaatagactttgttttaattcactcactgaaacatctccaactactagcaaaaattccgaatgtctgaatgcacactactcttcctaatgtggggagacaactgtgtgctttgtatctttcccactcaaattggcttataaaatgaaattattttaactatccaatggaaggtacataatttaaaacatcctatagaaatgacatgttactagtaatttacaattttaaaaaacagccacaaaaaagtcaaagctaaaaacaagatttttactatgaatcagtgcttctattatccttctgaaagaagttatattttaatgtgatgtaaaggcaacattgaaatttcttctttaaattaaccacctaatttatccctaaaattacaaagaatcagtcttttacaggtcaagtgcagtaaactaaaatgttctctcagcacaaagcagcactagaaaaagtaacagttatagatgggagttgactagttttgcagtggctgcgccatcaataacaaacagacatcagacggtatccatcccagagcacagacactactacagactagatgcgaagaatgcgtcacactcttggctgataaatgtcctttgtctttgactctttctagtttgaatgaagtggattttttaaaagtttaaatcaggtcacataagttggctgcttaaataacatcatgatgaggtatgaaaagctctgaatatcccttacattcagcaggatttaccagagatgtataatagcttgtcaggggcaacttccaaatagtttttacactttggggttataatgaattctagaagaggacaagtctaaaaaggtttaaaagggtatgctctgaaacagaggtgagcaaccttttccttcagaattcactttgaacagcacatcaacaaaaaaatcttctctggtagtgtatcccaacattgagtcaagatggccaactagcaccgagaagtcgtattgaactcatttgcagttgtcttggcaattaagcgtattttttcattccagtccaagcacaaatgtggatcactgaacacagtactggaagcgccatttgcaggtacagattgcagtcatcattaaatgagccagaaggcagatactgtttttattttgtgtggggggagggggaagcggcacagtactagcaggagatgaaataaaatgattaggaaacaatgaggttataagatcactgttcttatttgggttaagcaggtcatgttgagaagatggttatttctttcagataaggatgctacattaaaggaatcgtgtgcagcatgaaaagattagaatcgagctgcacctaagaaaaaaatcccaaagttactttcaaaagtatgtgttatctgccagtcacagaggggaaaagcacctagggtgaactccaattttttaatgaggaccttgatcaggaccacaaagcctgaaacatttattttaatgcagaaacacagcccctagttacactgattgcatttgggaaaattggagggttttttcgtccttagttttttttattaaattacaggatatggttttcgattactaagtattcgaaatcctcataccagcaacagaaatgaaccacttccaaattctaagacacaaaagaccaaagagaagcaaaagcgatacaaattaatatgtgcccctctcctttctgctctaagggaatctacaaaccagtatcacatttaggagtcaaagtgttaattcttcagcattcctgacaactagaaagcacattcactgaaggctgaaggtgagggagtggatggtttaactttaatatctgaagaatggcgccaatagaggaaagaaaaccatccaatctcagtaaggattaatgcaaatctggctagaaaaagccaccaggtaatccaagggttcactgtggaagaactcatgaaaagtactctgaagtatacacaacaggtctaaacatctcccttgtcgtaagtagttgtgtaaaattcaagataaagatttagtctcatcttttaatgtcagttttttcccccatgttaaagggaatgaggaggagtcctcttttattcccccacaagaaaaagggagccacattaatatgtgtatattcccataactctaatgtaagtgcggatctccaaagcctagggatttttccgtaaaagagagtgggccgttctggttacccttttattagaagggtattccaccacagagagccggaggttttccagatgtgtgtaagagagcaggtgcgcaaggcaagcaaatgagcgcaaacagtattatggaaaacatttgagaagttagctccatgaggactgtgggctccacaagaggactcgactgggtagcctggtctgacacaggtacgtgaaagcagagtattgcttcaaagctggaaaccttccataggagcctcacactgttggaagatgtactgctgctggttaaggtcaacctggggtgcaatgctgctgtcttcatcttcggtcccgaagtaatgctcaataagatcaaaggccttttggtagatctcctggttttcatgactctgtaagaactcaattttatccagaccataagcttcttcaatcaaagcacagtaagggttaatgccagtgccattccttttggcttcctgttctccaagcctcaggatattttccaagccatttagggcaacctgtacaatcttagagtccatgaccgtgaggagatcacagagcggcttgatacaacccagttctactaggtacttgatctgttcagctgatcctccagaagttgcatttgtgatggcccaagctgcttcttttcttgtccgaaattcagcagtttgtaaaatactaatgagggctgggaaaatgttggcatctatcacagtctggatctgtgccctatttccagctgtaatattagatatcgtccaacatgcttcctttttgatagattcctttgggctactcagcaaatgcaataaactctgcagagctgagcaattcagaattacctgtgtctgaatatcatcccctgtgacaatgtttcccacagctcgcaaagcaggagaaaccactttataatcattatgcatcagcagttccacaagtctcctacatactcccgcatcgatgaccgcttgaattttatcattgggtccatctgatagatatgagagggcccagcaggcatcagccagtacatcagtgtcactgacaaacagcaaccaggaaagcacattcagacatggagaaacctttgcaaattctggaggtggacttttccctctacagagattagacaaagcccatactgcattccgggtcatggtcaggcggttttgctttgaaaataactgcaaaagagggggaaggatattgcagtctaagacatagtccctgcacatggtactatctccagcaatgttgccaagagcccagactgcctgttcctggacatcttcaaactctgagctgagcaactctatgaagatgggcacagctcctgcctgaatcacaattcgggtctgaagagaatttcctgaagcaatatttgtcagtacccaagctgattcaaactgcagtgtacaattctcttttcgtttgaggaactccacaaacctggccactactcctggtgtgctgataacttcatcaataggagggttaggttcttttgaaagcagcttcctgaatttctgtgttgctgaaagctgttgctctgggcttttggaaaatatcatttcaatcatgtcagaagtgatgacaccacctggtgccatctccatgttactaatctgagcctcatgaaagcctccatctgacataacttcttcttctgtttcttcttctgctgtagcaacatttctccgcttgaataactgctcttctcttttctgctttcgtaactgcagtccttcttcctccctcctcctgcgcatctcatcgggattcagagatttgttcttgtaacttttcaggcgaaagttctcttttcctggggtggtcatgatttcaggctcaaggcaaccgatcccggtgccaccgctgaagttagcccctcgctcgcccgcccgccgtgccactcccgcgcacaacctcgaagagctggcccgcgcctcggcggtgctcaccaggcctcgctctccgccgcctcgcaccgagcagcgagactcagctcagccggcgttcgcagtgc

SEQ ID NO: 13243 - RNA, 1821 nt, Homo sapiens
  source 1..1821: mol_type = other RNA
gctgggattacaggcatgagccaccacatccggcctaaaaggcacttttttttttttgagacggagtttccctcttgttgcccaggctggaatgcaatggtgcaatctcactgcaacctctgccttccagattgaagcaattctcctgcctcagctttccccagtagctgggattacaggcacctgctaccatgcctggctaatttttgtatttttagtagagacagggtttcaccatgttggccaggctggtcttgaactcctgacctcaggtgatccacccaccttggcctcccaaagtgctgggattacaagcgtgagccaccatgcccagcctctaaaaggcactttttaagggaccttggagtttgtcctcaaacagctcaaccccacaggcgaggctggtcctagcacccctaccagacagctagtcagtgagaggggtccaacctcccccagcttttccctggaagtggggcagggtcagcagggaattctgggggtgaagctcatggtccaggagccttctggtgcccagagggtagaggagtggaaggcctgggggtgctcagccccactgtatcctggacaggctgggccggcttgcaggctggtctccatggaggctcagaaggaaagtgtgcaagagcaggttaggaagggaaaccaagtcagggaagggccccagccggggctagtggtctgttcactgcccagcgggcactctcagcagcaccccgcagcactccgcttcacatggcatggcttgcagaagagatggttgttcagggggtagcagccttggtccgtgggctcgacagacaggaggatcctgcagtcctcacacctgtagcaattttcatggaagtttcttcccatgcattcgattttgaaggcatctttcccatcccgagggatgatgggattttcacagatgctgcagacgggggcgaatttcctgtagaagtcgtccaggcagtacacctcgttctggctgcccagggcaaagctctcatccccaatgcaccgggcgcaggtcacacacgtgaagcaggaggggtggaaggcctggcccagggccctgatgatgtggtcccggaccacctcgccacacttgccgcacctctccagtgtgtcctggtagcagggttcgcagaggggtcgcccatccttctggtagaagctctgcccagccagctggcggcggcaggtgcggcacgtgaagcactgggcatggtactgcctcttcatggcctccacagccagctctcggggggacacggtcttgtggcagaaggcacagatgtctccattgaagagctgcataggtgcagccggcactgtggctgcagctctgccaggggttgtccaggggctgggcctccccgccaagccagcctcgggtgtcttcatgggggcaggagcctcccaggggcggccacgccgggcctcacaaactgcctgcctcacttcctccgccacggccacatcgcggcgcgggggtgccagggtgataaagacagacgatgccaccctcttctcaggctttgaggccatggcttcagctcctggtgtggcaatgatcactcttccttgtctcacacccgcgaggaaggaacagatgcttcagctcccagccccagcagggctgacttccgttcccagtctggagtcccgcctgcctgctgggccacaccccaagtgacctccctcacctgggatcagattctcctagaagggctgaagtcctggaggttcaggccagctctgggccgcccgcgccccggcggctccgatccgacgcccgagccagcggagccc

SEQ ID NO: 13244 - RNA, 2358 nt, Homo sapiens
  source 1..2358: mol_type = other RNA
gctgggattacaggcatgagccaccacatccggcctaaaaggcacttttttttttttgagacggagtttccctcttgttgcccaggctggaatgcaatggtgcaatctcactgcaacctctgccttccagattgaagcaattctcctgcctcagctttccccagtagctgggattacaggcacctgctaccatgcctggctaatttttgtatttttagtagagacagggtttcaccatgttggccaggctggtcttgaactcctgacctcaggtgatccacccaccttggcctcccaaagtgctgggattacaagcgtgagccaccatgcccagcctctaaaaggcactttttaagggaccttggagtttgtcctcaaacagctcaaccccacaggcgaggctggtcctagcacccctaccagacagctagtcagtgagaggggtccaacctcccccagcttttccctggaagtggggcagggtcagcagggaattctgggggtgaagctcatggtccaggagccttctggtgcccagagggtagaggagtggaaggcctgggggtgctcagccccactgtatcctggacaggctgggccggcttgcaggctggtctccatggaggctcagaaggaaagtgtgcaagagcaggttaggaagggaaaccaagtcagggaagggccccagccggggctagtggtctgttcactgcccagcgggcactctcagcagcaccccgcagcactccgcttcacatggcatggcttgcagaagagatggttgttcagggggtagcagccttggtccgtgggctcgacagacaggaggatcctgcagtcctcacacctgtagcaattttcatggaagtttcttcccatgcattcgattttgaaggcatctttcccatcccgagggatgatgggattttcacagatgctgcagacgggggcgaatttcctgtagaagtcgtccaggcagtacacctcgttctggctgcccagggcaaagctctcatccccaatgcaccgggcgcaggtcacacacgtgaagcaggaggggtggaaggcctggcccagggccctgatgatgtggtcccggaccacctcgccacacttgccgcacctctccagtgtgtcctggtagcagggttcgcagaggggtcgcccatccttctggtagaagctctgcccagccagctggcggcggcaggtgcggcacgtgaagcactgggcatggtactgcctcttcatggcctccacagccagctctcggggggacacggtcttgtggcagaaggcacagatgtctgtggatgcccctttctcaacaggttctgccgggggaggtggcagctcttcctccatgggcctgaggggaccgggctggactgaaggtccctccgctggggcctgtggtgggggcgggggcggggacaggtgcagctgctctaagtctgcaatgagtgaggcccccattggagcaggagcctcctcttcagaaggcagaagcactggagggggcggtggagggggtgggaggaggtccaggtcaggaagcacgtcctcaccatccaggacaggaggagggggtgggcatcctccattgaagagctgcataggtgcagccggcactgtggctgcagctctgccaggggttgtccaggggctgggcctccccgccaagccagcctcgggtgtcttcatgggggcaggagcctcccaggggcggccacgccgggcctcacaaactgcctgcctcacttcctccgccacggccacatcgcggcgcgggggtgccagggtgataaagacagacgatgccaccctcttctcaggctttgaggccatggcttcagctcctggtgtggcaatgatcactcttccttgtctcacacccgcgaggaaggaacagatgcttcagctcccagccccagcagggctgacttccgttcccagtctggagtcccgcctgcctgctgggccacaccccaagtgacctccctcacctgggatcagattctcctagaagggctgaagtcctggaggttcaggccagctcctgtccggcggaggtgagcgcttactttggctctgggatccgccagggtcttgcgtcaaaccgaccagggttctgcggccgtttactaagcgtgagacccggagcagtcacgccacctcctgagcctcagtgtcttcatctgtaaagtggaggtagccactgcctacctctccaggttggcctgcctccagcaccccaggccacctgttccaccgccaccactgctcccggatggagggattcgtcctggcccgcagcagctcgggtgtcgatgtcaccgatcggcaggtgccaaactt

SEQ ID NO: 13245 - RNA, 2381 nt, Homo sapiens
  source 1..2381: mol_type = other RNA
gctgggattacaggcatgagccaccacatccggcctaaaaggcacttttttttttttgagacggagtttccctcttgttgcccaggctggaatgcaatggtgcaatctcactgcaacctctgccttccagattgaagcaattctcctgcctcagctttccccagtagctgggattacaggcacctgctaccatgcctggctaatttttgtatttttagtagagacagggtttcaccatgttggccaggctggtcttgaactcctgacctcaggtgatccacccaccttggcctcccaaagtgctgggattacaagcgtgagccaccatgcccagcctctaaaaggcactttttaagggaccttggagtttgtcctcaaacagctcaaccccacaggcgaggctggtcctagcacccctaccagacagctagtcagtgagaggggtccaacctcccccagcttttccctggaagtggggcagggtcagcagggaattctgggggtgaagctcatggtccaggagccttctggtgcccagagggtagaggagtggaaggcctgggggtgctcagccccactgtatcctggacaggctgggccggcttgcaggctggtctccatggaggctcagaaggaaagtgtgcaagagcaggttaggaagggaaaccaagtcagggaagggccccagccggggctagtggtctgttcactgcccagcgggcactctcagcagcaccccgcagcactccgcttcacatggcatggcttgcagaagagatggttgttcagggggtagcagccttggtccgtgggctcgacagacaggaggatcctgcagtcctcacacctgtagcaattttcatggaagtttcttcccatgcattcgattttgaaggcatctttcccatcccgagggatgatgggattttcacagatgctgcagacgggggcgaatttcctgtagaagtcgtccaggcagtacacctcgttctggctgcccagggcaaagctctcatccccaatgcaccgggcgcaggtcacacacgtgaagcaggaggggtggaaggcctggcccagggccctgatgatgtggtcccggaccacctcgccacacttgccgcacctctccagtgtgtcctggtagcagggttcgcagaggggtcgcccatccttctggtagaagctctgcccagccagctggcggcggcaggtgcggcacgtgaagcactgggcatggtactgcctcttcatggcctccacagccagctctcggggggacacggtcttgtggcagaaggcacagatgtctgtggatgcccctttctcaacaggttctgccgggggaggtggcagctcttcctccatgggcctgaggggaccgggctggactgaaggtccctccgctggggcctgtggtgggggcgggggcggggacaggtgcagctgctctaagtctgcaatgagtgaggcccccattggagcaggagcctcctcttcagaaggcagaagcactggagggggcggtggagggggtgggaggaggtccaggtcaggaagcacgtcctcaccatccaggacaggaggagggggtgggcatcctccattgaagagctgcataggtgcagccggcactgtggctgcagctctgccaggggttgtccaggggctgggcctccccgccaagccagcctcgggtgtcttcatgggggcaggagcctcccaggggcggccacgccgggcctcacaaactgcctgcctcacttcctccgccacggccacatcgcggcgcgggggtgccagggtgataaagacagacgatgccaccctcttctcaggctttgaggccatggcttcagctcctggtgtggcaatgatcactcttccttgtctcacacccgcgaggaaggaacagatgcttcagctcccagccccagcagggctgacttccgttcccagtctggagtcccgcctgcctgctgggccacaccccaagtgacctccctcacctgggatcagattctcctagaagggctgaagtcctggaggttcaggccagctctgcctgtccggcggaggtgagcgcttactttggctctgggatccgccagggtcttgcgtcaaaccgaccagggttctgcggccgtttactaagcgtgagacccggagcagtcacgccacctcctgagcctcagtgtcttcatctgtaaagtggaggtagccactgcctacctctccaggttggccttgttctgctctcctgagcggtaagccctctgcaggtgggtcccggtgtcccgggggacaggccgctccaggagctctggaaggcagggcccggctggccctgtggctgaacccctccctccacatccagtgaccct

SEQ ID NO: 13246 - RNA, 2112 nt, Homo sapiens
  source 1..2112: mol_type = other RNA
gctgggattacaggcatgagccaccacatccggcctaaaaggcacttttttttttttgagacggagtttccctcttgttgcccaggctggaatgcaatggtgcaatctcactgcaacctctgccttccagattgaagcaattctcctgcctcagctttccccagtagctgggattacaggcacctgctaccatgcctggctaatttttgtatttttagtagagacagggtttcaccatgttggccaggctggtcttgaactcctgacctcaggtgatccacccaccttggcctcccaaagtgctgggattacaagcgtgagccaccatgcccagcctctaaaaggcactttttaagggaccttggagtttgtcctcaaacagctcaaccccacaggcgaggctggtcctagcacccctaccagacagctagtcagtgagaggggtccaacctcccccagcttttccctggaagtggggcagggtcagcagggaattctgggggtgaagctcatggtccaggagccttctggtgcccagagggtagaggagtggaaggcctgggggtgctcagccccactgtatcctggacaggctgggccggcttgcaggctggtctccatggaggctcagaaggaaagtgtgcaagagcaggttaggaagggaaaccaagtcagggaagggccccagccggggctagtggtctgttcactgcccagcgggcactctcagcagcaccccgcagcactccgcttcacatggcatggcttgcagaagagatggttgttcagggggtagcagccttggtccgtgggctcgacagacaggaggatcctgcagtcctcacacctgtagcaattttcatggaagtttcttcccatgcattcgattttgaaggcatctttcccatcccgagggatgatgggattttcacagatgctgcagacgggggcgaatttcctgtagaagtcgtccaggcagtacacctcgttctggctgcccagggcaaagctctcatccccaatgcaccgggcgcaggtcacacacgtgaagcaggaggggtggaaggcctggcccagggccctgatgatgtggtcccggaccacctcgccacacttgccgcacctctccagtgtgtcctggtagcagggttcgcagaggggtcgcccatccttctggtagaagctctgcccagccagctggcggcggcaggtgcggcacgtgaagcactgggcatggtactgcctcttcatggcctccacagccagctctcggggggacacggtcttgtggcagaaggcacagatgtctgtggatgcccctttctcaacaggttctgccgggggaggtggcagctcttcctccatgggcctgaggggaccgggctggactgaaggtccctccgctggggcctgtggtgggggcgggggcggggacaggtgcagctgctctaagtctgcaatgagtgaggcccccattggagcaggagcctcctcttcagaaggcagaagcactggagggggcggtggagggggtgggaggaggtccaggtcaggaagcacgtcctcaccatccaggacaggaggagggggtgggcatcctccattgaagagctgcataggtgcagccggcactgtggctgcagctctgccaggggttgtccaggggctgggcctccccgccaagccagcctcgggtgtcttcatgggggcaggagcctcccaggggcggccacgccgggcctcacaaactgcctgcctcacttcctccgccacggccacatcgcggcgcgggggtgccagggtgataaagacagacgatgccaccctcttctcaggctttgaggccatggcttcagctcctggtgtggcaatgatcactcttccttgtctcacacccgcgaggaaggaacagatgcttcagctcccagccccagcagggctgacttccgttcccagtctggagtcccgcctgcctgctgggccacaccccaagtgacctccctcacctgggatcagattctcctagaagggctgaagtcctggaggttcaggccagctctgggccgcccgcgccccggcggctccgatccgacgcccgagccagcggagccc

SEQ ID NO: 13247 - RNA, 2312 nt, Homo sapiens
  source 1..2312: mol_type = other RNA
gctgggattacaggcatgagccaccacatccggcctaaaaggcacttttttttttttgagacggagtttccctcttgttgcccaggctggaatgcaatggtgcaatctcactgcaacctctgccttccagattgaagcaattctcctgcctcagctttccccagtagctgggattacaggcacctgctaccatgcctggctaatttttgtatttttagtagagacagggtttcaccatgttggccaggctggtcttgaactcctgacctcaggtgatccacccaccttggcctcccaaagtgctgggattacaagcgtgagccaccatgcccagcctctaaaaggcactttttaagggaccttggagtttgtcctcaaacagctcaaccccacaggcgaggctggtcctagcacccctaccagacagctagtcagtgagaggggtccaacctcccccagcttttccctggaagtggggcagggtcagcagggaattctgggggtgaagctcatggtccaggagccttctggtgcccagagggtagaggagtggaaggcctgggggtgctcagccccactgtatcctggacaggctgggccggcttgcaggctggtctccatggaggctcagaaggaaagtgtgcaagagcaggttaggaagggaaaccaagtcagggaagggccccagccggggctagtggtctgttcactgcccagcgggcactctcagcagcaccccgcagcactccgcttcacatggcatggcttgcagaagagatggttgttcagggggtagcagccttggtccgtgggctcgacagacaggaggatcctgcagtcctcacacctgtagcaattttcatggaagtttcttcccatgcattcgattttgaaggcatctttcccatcccgagggatgatgggattttcacagatgctgcagacgggggcgaatttcctgtagaagtcgtccaggcagtacacctcgttctggctgcccagggcaaagctctcatccccaatgcaccgggcgcaggtcacacacgtgaagcaggaggggtggaaggcctggcccagggccctgatgatgtggtcccggaccacctcgccacacttgccgcacctctccagtgtgtcctggtagcagggttcgcagaggggtcgcccatccttctggtagaagctctgcccagccagctggcggcggcaggtgcggcacgtgaagcactgggcatggtactgcctcttcatggcctccacagccagctctcggggggacacggtcttgtggcagaaggcacagatgtctgtggatgcccctttctcaacaggttctgccgggggaggtggcagctcttcctccatgggcctgaggggaccgggctggactgaaggtccctccgctggggcctgtggtgggggcgggggcggggacaggtgcagctgctctaagtctgcaatgagtgaggcccccattggagcaggagcctcctcttcagaaggcagaagcactggagggggcggtggagggggtgggaggaggtccaggtcaggaagcacgtcctcaccatccaggacaggaggagggggtgggcatcctccattgaagagctgcataggtgcagccggcactgtggctgcagctctgccaggggttgtccaggggctgggcctccccgccaagccagcctcgggtgtcttcatgggggcaggagcctcccaggggcggccacgccgggcctcacaaactgcctgcctcacttcctccgccacggccacatcgcggcgcgggggtgccagggtgataaagacagacgatgccaccctcttctcaggctttgaggccatggcttcagctcctggtgtggcaatgatcactcttccttgtctcacacccgcgaggaaggaacagatgcttcagctcccagccccagcagggctgacttccgttcccagtctggagtcccgcctgcctgctgggccacaccccaagtgacctccctcacctgggatcagattctcctagaagggctgaagtcctggaggttcaggccagctctgtttggctctgggatccgccagggtcttgcgtcaaaccgaccagggttctgcggccgtttactaagcgtgagacccggagcagtcacgccacctcctgagcctcagtgtcttcatctgtaaagtggaggtagccactgcctacctctccaggttggcctgcctccagcaccccaggccacctgttccaccgccaccactgctcccggatggagggattcgtcctggcccgcagcagctcgggtgtcgatgtc

SEQ ID NO: 13248 - RNA, 2820 nt, Homo sapiens
  source 1..2820: mol_type = other RNA
gctgggattacaggcatgagccaccacatctagcctataatgcttttgttaagtataaactttctgatattgagtaagatgtgaacagacattaatggcttttcacattctttatatttttacaatttttctctagtataaaaggcttcctgtgcaataagatgggaaaatttgttaaaagttttgccacatttttcatatttgcctgagttttcttcagtataaattatcttacctaccataacatgcaactaccatttaaaggacttacctcatttaacacatttctagagtttttcaccagtatgatttctctattttagaaaaatgtcaggtgtggttaaatgctgtcacattttttatgtatgtagagtttctctccagtataaaatattttaattaataaagatggagaaccagttaaaagctttgccacatttttttttttttttacaattgcaggggttctctccagtatcaattattttacatttattcaaacaaaaagtttgaggacttttaaaagacatttccatattccttattgtagggtttttcttcagtatcaattcttttagtgtataataagggttcaagactaggtaaaagctttaccacattgtttttgtagggtttgtctctagaatgaattatctgatattgtgtaaggcctgagatgtgcttaaatgttttgtcacatttttgacctttgtagagtctctctaatataaattctcttaggctttgggaggctgaggcaggtggttcacctgaagtcaggagtttgagaccagcctggtcaaaatggtgaaaccccatctctactaaaaatacaaaactcagccagtgtggttgcacgtgcctgtaattccagctactcaggaggctgaggcaggagaatcgcttgaacccaggaggcagaggttgcagtgagctgacatcgtgccactgcactccagcctgggtgacaaagtgagactctgtctcaaaaaaatttttttaaataaattctcttgggttcattaaggtttgaggggtggttaaaggctgttacttttttttttacatttataagacttttgtccaatatgaattatcttatggacagcagtggtttggaactggttaaagaattggccacattctccacacttgtagtgattttttccagtataaattattttatgtattataaggcctgagggctggactttaccacattattcatatttgtagggtttctctccagtatgcatattcttatgattagcaagacttgaatgccacttaaaagtttggtcacattcttcacatttgtagggtttctctccagtatgaatcctcttatgagtatttagagttgaggagaaggtaaaggctttcccacattctttacatttgtagagtttctctccagtatgaattatcttatgtttcttaagggttgaggagcagttaaaggctttgccacattcttcacatttgtagggtttctctccagtatgagttctcttgtggtaagtgaaggttgagggtaagctaaaggctttgccacattcttcacaagtgtagggtttctctccagtatgaatcctcttatgagtatttagagttgaggagaaggtaaaggctttcccacattcttcacatgtgtagagtttctccccagtatgaactatcttatgtttcttaagggttgaggataagctaaaggctttgccacattcttcacatttgtagggtctctctccagtatgaattctcttgtggttagtaagtgttgaagagcggctaaaggctttgccacattcttcacatgtgtagggtttctctccagtatgaattctcttgtagttagtaagtgttgagcggctaaagactttgccacgttcttcacatgtgtaaggtttctctccagtatgaattctcttatgtttagtaagggatgcagaccagctaaaagctttgccacattcctcacatctgtagggtttctctccagtatgaattcttttatgtctagtaagggttgaagagcagttaaaggatttgccacattcttcacatttgtaagacttctccctagtatgaattatctgatgttgatttaggcgtgaaagcatgcaaaatgatttgccatcgtttttacatttgaaatgtttctttccagtatgtcttgtcttgtgtctattggaatttgaaaatttaccaaagactttgacgcatttatgagtctgaaatgttttgttttgggtagctgacaaacattggttaacataattataacctcctttgtgcacctcacactcacctacacttttacagcatttttttacttgtaaatcctcctgtccacattttccatatcttctcagtatcactttttggagtgaatcttttatgccctgctctgactgaaggtcttgggtgaaatgagaacatgtaactgggtgtttggctaccatctcatttctctttatattctggggctctttattttgctccagacaggtgatcaagtctggcttagagacagcaatacccagggagaccaggtttctgtagttctctaacatcacatctctatataaattctgctgagcatgatccaggcattgccattccgccagagaaaattctatagctatgtctctgaatgtcaacagtcccatttctcggcttccagggggtcccggtcttttagccataaatctgcgaatacttgcaggacacaaggccacagaggcttggcctccaggagcagaggacgcagagcagtgaagagaaggactggagctctgggcgcagagaagcaaaaag

SEQ ID NO: 13249 - RNA, 2013 nt, Homo sapiens
  source 1..2013: mol_type = other RNA
gctgggattacaggcatgagccaccacatctggccaacattcactcttaagcctttctaaattattccaatattacaaggacaaatgctaatctgatgagtttcaatctacgttgaatgaatgctaaagttgaatgaaatgctaaactgatgagtttcaatctatgttgactgtttcatcacagtaacataaatgaagtttttatttttcataaatgaaatgtaatgatgttaacagtggattggaaaatcttctggaagtttttgggtttttttttcaagacagagtctggagagcagttgtagcgcccaggctggagagcagtggcaccacctcagctcattgcaacctctgctttccaggttcaagtgatcctctcacctcagcctgagtagctgggactacgggtgcgtgccaccacgtctggctaattttttgtagagataaggtctcatcatgttgcccaggctggtctcgaactcctgggttcaagtgatccacccgccctggcctcccaaaatgttgggattataggtgtgagccaccatgccatgtttttaatgcattttaaaattatgttaaaagaaaattcttacaaagatattttaagattacatcacagcaagcaactgtttaattgggacaaagaagatacactaaaagccaaatgaattactgtaattaaatttgtacagtttattgacttttttttcctttttatttatttgagatggagttttgctcttgtcacccaggctggagggcaatggagcgatcttggctcactgcaacctccccctcccaggttcaagtgattctcctgccttagcctcccgagtagctgggattacaggcacccactaccacgcctgactaatttttgtgtttttagtggagacaggatttcaccatgttggccaggctggtctcgaactcctgacctcaggtgatccacccgccttggcctcctaaagtgctgggattacaggcgtgagccactatgcctggctattgacatttttttttttaagcaaagaggtggggcacatccactgcagtccaggcattctggcaccacctctgttattaactggaatcaaattttaaaaatttctgtgatcttgaaggtcttgttgaagttttagaggtcttttgtttttcttttagccactagatttttcaggaaaaattcacctgctttatatgaagaacgcaccaaagggccacttgcagtataatgaaatccaagttcatttcctactttttcccagtatttgaatttttcaggagtaatatattcttcaaccttaaggtgacgccttgttggctgcatatattgtcctaaagtcaagcagtctacatctgcctcacgaagtgctttcattgttgcatatacttgctcatcattctcgcctaaacccaacattatagatgttttagaaataacatcaggctgaaccttcttggcatgtttcagtacacgtagggactgatcaaaattggcccgaggatcacgaaccttactctgtaattccgggactgtttctacattatgtgcatacacatctaatcctgacagagcaactttttctattgctttgagatcacctcgaaaatcaggagtaagacactccacaaggatttttggattccatgatcgtggctgtggcggtggcatattctccacctccccaacactctccaatattgggacatcgagcttcctcacatacctttctcctttctggcgttttaggtttcctttatattcatcccaggtgctcctgtctgcaagatcaccagatacaaaatcttgaaggtctggtccattctgtaggagttccttttttttatctggcaaggagcttaacggtctgactgggctgcaaaaatatctcccaaatacccggggccccagggtgcgggctgcatccccgcagcgtagagacatttcctctttaggactagcgcagtgcaggggttgagggatcgctaactcccgggaaaggacag

SEQ ID NO: 13250 - RNA, 2322 nt, Homo sapiens
  source 1..2322: mol_type = other RNA
gctgggattacaggcatgagccaccacatctggccaacattcactcttaagcctttctaaattattccaatattacaaggacaaatgctaatctgatgagtttcaatctacgttgaatgaatgctaaagttgaatgaaatgctaaactgatgagtttcaatctatgttgactgtttcatcacagtaacataaatgaagtttttatttttcataaatgaaatgtaatgatgttaacagtggattggaaaatcttctggaagtttttgggtttttttttcaagacagagtctggagagcagttgtagcgcccaggctggagagcagtggcaccacctcagctcattgcaacctctgctttccaggttcaagtgatcctctcacctcagcctgagtagctgggactacgggtgcgtgccaccacgtctggctaattttttgtagagataaggtctcatcatgttgcccaggctggtctcgaactcctgggttcaagtgatccacccgccctggcctcccaaaatgttgggattataggtgtgagccaccatgccatgtttttaatgcattttaaaattatgttaaaagaaaattcttacaaagatattttaagattacatcacagcaagcaactgtttaattgggacaaagaagatacactaaaagccaaatgaattactgtaattaaatttgtacagtttattgacttttttttcctttttatttatttgagatggagttttgctcttgtcacccaggctggagggcaatggagcgatcttggctcactgcaacctccccctcccaggttcaagtgattctcctgccttagcctcccgagtagctgggattacaggcacccactaccacgcctgactaatttttgtgtttttagtggagacaggatttcaccatgttggccaggctggtctcgaactcctgacctcaggtgatccacccgccttggcctcctaaagtgctgggattacaggcgtgagccactatgcctggctattgacatttttttttttaagcaaagaggtggggcacatccactgcagtccaggcattctggcaccacctctgttattaactggaatcaaattttaaaaatttctgtgatcttgaaggtcttgttgaagttttagaggtcttttgtttttcttttagccactagatttttcaggaaaaattcacctgctttatatgaagaacgcaccaaagggccacttgcagtataatgaaatccaagttcatttcctactttttcccagtatttgaatttttcaggagtaatatattcttcaaccttaaggtgacgccttgttggctgcatatattgtcctaaagtcaagcagtctacatctgcctcacgaagtgctttcattgttgcatatacttgctcatcattctcgcctaaacccaacattatagatgttttagaaataacatcaggctgaaccttcttggcatgtttcagtacacgtagggactgatcaaaattggcccgaggatcacgaaccttactctgtaattccgggactgtttctacattatgtgcatacacatctaatcctgacagagcaactttttctattgctttgagatcacctcgaaaatcaggagtaagacactccacaaggatttttggattcctttcctttaaatatgatacggtctttgcaatgtgttcagctcccccatcaggcatatcatctcgatccacagatgtcaggacaacataatccagaccccattctgcaattgcctttgcagtattgtagggctcactggcatccagtggaggaggatttcttgcagtcttaacagaacaaaatctgcaacctcttgtacatgtgtcacccatcaacatgatcgtggctgtggcggtggcatattctccacctccccaacactctccaatattgggacatcgagcttcctcacatactgtatggagatttaaattccgcaaagtatttttcagtttattgtaatttttccccatgggaatctctgtctttagccatggaggtagtcttaacctttctcctttctggcgttttaggtttcctttatattcatcccaggtgctcctgtctgcaagatcaccagatacaaaatcttgaaggtctggtccattctgtaggagttccttttttttatctggcaaggagcttaacggtctgactgggctgcaaaaatatctcccaaatacccggggccccagggtgcgggctgcatccccgcagcgtagagacatttcctctttaggactagcgcagtgcaggggttgagggatcgctaactcccgggaaaggacag

SEQ ID NO: 13251 - RNA, 2193 nt, Homo sapiens
  source 1..2193: mol_type = other RNA
gctgggattacaggcatgagccaccacatctggccaacattcactcttaagcctttctaaattattccaatattacaaggacaaatgctaatctgatgagtttcaatctacgttgaatgaatgctaaagttgaatgaaatgctaaactgatgagtttcaatctatgttgactgtttcatcacagtaacataaatgaagtttttatttttcataaatgaaatgtaatgatgttaacagtggattggaaaatcttctggaagtttttgggtttttttttcaagacagagtctggagagcagttgtagcgcccaggctggagagcagtggcaccacctcagctcattgcaacctctgctttccaggttcaagtgatcctctcacctcagcctgagtagctgggactacgggtgcgtgccaccacgtctggctaattttttgtagagataaggtctcatcatgttgcccaggctggtctcgaactcctgggttcaagtgatccacccgccctggcctcccaaaatgttgggattataggtgtgagccaccatgccatgtttttaatgcattttaaaattatgttaaaagaaaattcttacaaagatattttaagattacatcacagcaagcaactgtttaattgggacaaagaagatacactaaaagccaaatgaattactgtaattaaatttgtacagtttattgacttttttttcctttttatttatttgagatggagttttgctcttgtcacccaggctggagggcaatggagcgatcttggctcactgcaacctccccctcccaggttcaagtgattctcctgccttagcctcccgagtagctgggattacaggcacccactaccacgcctgactaatttttgtgtttttagtggagacaggatttcaccatgttggccaggctggtctcgaactcctgacctcaggtgatccacccgccttggcctcctaaagtgctgggattacaggcgtgagccactatgcctggctattgacatttttttttttaagcaaagaggtggggcacatccactgcagtccaggcattctggcaccacctctgttattaactggaatcaaattttaaaaatttctgtgatcttgaaggtcttgttgaagttttagaggtcttttgtttttcttttagccactagatttttcaggaaaaattcacctgctttatatgaagaacgcaccaaagggccacttgcagtataatgaaatccaagttcatttcctactttttcccagtatttgaatttttcaggagtaatatattcttcaaccttaaggtgacgccttgttggctgcatatattgtcctaaagtcaagcagtctacatctgcctcacgaagtgctttcattgttgcatatacttgctcatcattctcgcctaaacccaacattatagatgttttagaaataacatcaggctgaaccttcttggcatgtttcagtacacgtagggactgatcaaaattggcccgaggatcacgaaccttactttcctttaaatatgatacggtctttgcaatgtgttcagctcccccatcaggcatatcatctcgatccacagatgtcaggacaacataatccagaccccattctgcaattgcctttgcagtattgtagggctcactggcatccagtggaggaggatttcttgcagtcttaacagaacaaaatctgcaacctcttgtacatgtgtcacccatcaacatgatcgtggctgtggcggtggcatattctccacctccccaacactctccaatattgggacatcgagcttcctcacatactgtatggagatttaaattccgcaaagtatttttcagtttattgtaatttttccccatgggaatctctgtctttagccatggaggtagtcttaacctttctcctttctggcgttttaggtttcctttatattcatcccaggtgctcctgtctgcaagatcaccagatacaaaatcttgaaggtctggtccattctgtaggagttccttttttttatctggcaaggagcttaacggtctgactgggctgcaaaaatatctcccaaatacccggggccccagggtgcgggctgcatccccgcagcgtagagacatttcctctttaggactagcgcagtgcaggggttgagggatcgctaactcccgggaaaggacag

SEQ ID NO: 13252 - RNA, 2210 nt, Homo sapiens
  source 1..2210: mol_type = other RNA
gctgggattacaggcatgagccaccacatctggccaacattcactcttaagcctttctaaattattccaatattacaaggacaaatgctaatctgatgagtttcaatctacgttgaatgaatgctaaagttgaatgaaatgctaaactgatgagtttcaatctatgttgactgtttcatcacagtaacataaatgaagtttttatttttcataaatgaaatgtaatgatgttaacagtggattggaaaatcttctggaagtttttgggtttttttttcaagacagagtctggagagcagttgtagcgcccaggctggagagcagtggcaccacctcagctcattgcaacctctgctttccaggttcaagtgatcctctcacctcagcctgagtagctgggactacgggtgcgtgccaccacgtctggctaattttttgtagagataaggtctcatcatgttgcccaggctggtctcgaactcctgggttcaagtgatccacccgccctggcctcccaaaatgttgggattataggtgtgagccaccatgccatgtttttaatgcattttaaaattatgttaaaagaaaattcttacaaagatattttaagattacatcacagcaagcaactgtttaattgggacaaagaagatacactaaaagccaaatgaattactgtaattaaatttgtacagtttattgacttttttttcctttttatttatttgagatggagttttgctcttgtcacccaggctggagggcaatggagcgatcttggctcactgcaacctccccctcccaggttcaagtgattctcctgccttagcctcccgagtagctgggattacaggcacccactaccacgcctgactaatttttgtgtttttagtggagacaggatttcaccatgttggccaggctggtctcgaactcctgacctcaggtgatccacccgccttggcctcctaaagtgctgggattacaggcgtgagccactatgcctggctattgacatttttttttttaagcaaagaggtggggcacatccactgcagtccaggcattctggcaccacctctgttattaactggaatcaaattttaaaaatttctgtgatcttgaaggtcttgttgaagttttagaggtcttttgtttttcttttagccactagatttttcaggaaaaattcaccttaaggtgacgccttgttggctgcatatattgtcctaaagtcaagcagtctacatctgcctcacgaagtgctttcattgttgcatatacttgctcatcattctcgcctaaacccaacattatagatgttttagaaataacatcaggctgaaccttcttggcatgtttcagtacacgtagggactgatcaaaattggcccgaggatcacgaaccttactctgtaattccgggactgtttctacattatgtgcatacacatctaatcctgacagagcaactttttctattgctttgagatcacctcgaaaatcaggagtaagacactccacaaggatttttggattcctttcctttaaatatgatacggtctttgcaatgtgttcagctcccccatcaggcatatcatctcgatccacagatgtcaggacaacataatccagaccccattctgcaattgcctttgcagtattgtagggctcactggcatccagtggaggaggatttcttgcagtcttaacagaacaaaatctgcaacctcttgtacatgtgtcacccatcaacatgatcgtggctgtggcggtggcatattctccacctccccaacactctccaatattgggacatcgagcttcctcacatactgtatggagatttaaattccgcaaagtatttttcagtttattgtaatttttccccatgggaatctctgtctttagccatggaggtagtcttaacctttctcctttctggcgttttaggtttcctttatattcatcccaggtgctcctgtctgcaagatcaccagatacaaaatcttgaaggtctggtccattctgtaggagttccttttttttatctggcaaggagcttaacggtctgactgggctgcaaaaatatctcccaaatacccggggccccagggtgcgggctgcatccccgcagcgtagagacatttcctctttaggactagcgcagtgcaggggttgagggatcgctaactcccgggaaaggacag

SEQ ID NO: 13253 - RNA, 2645 nt, Homo sapiens
  source 1..2645: mol_type = other RNA
gctgggattacaggcatgagccaccacccccagcccttatgtttctttattactggtgttcagaaatggtattaattttgtaggttgatcatgtggctggaaaatatgctaacttgtcattctaaaagtttgactctttattttgtgagttttgcaagtttatcatctcaccttcaaaaatctgtttttatttcttcctgtgatagtttttacacctcttattatgtctggaccattgtactatatatatatatattattttttcattgtactatattaaaactagtggtgacagtaatttcccctcaaattaggactgaaagtctcattttaaaaaaacccaaattcagcctgggcaacaaggcgaaaccccatctccactaaaaatacaaaaattagccagacatggtggcgcatgtctgtagtctcagctactcagaaggctgaggtgggaggactgtttgagcccaggaggcagaggctgcagtgagccaagatggtgccactgcactccagcctgggtgacagagtgctgtctacaaaaaacaaataacaaacaaaaaatgaaaaattggaaacaaaatgtaagtttataactttctgtcattaaaagtggatgatagtgtactcacttccacaacacatatactaaaatcagaatgatacagagagaaaagtggatgatggtttcttcggtttccttgaaaaaaagtgtttttaaactagataacccagccgggtgcgatggtgcactcctgtattcctagcactttgggaggctgtggcaggtggatggcgttaagtccaggagttggagaccagcctgggcaacatggcaaaacctcgtctctacaaaaaacacaaaaattggccaggctcggtggctcatgtctgtaatcccagcactttgggaggtcaaggcaggcggatcactggaggtcaggagttcaagaccagcctgggcaacgtggtgaaaccccgtctctactaaaaatacaaaagttagccaggcatggtggcacacgcctgtaatcccagctactcaggaggctgacacaggagaatcacttgaaccccaggaggtggaggttgcactgagctgagatcccgccactgcactccaccctgggtgacagtgcgagactcagtctcaaaaaaaaaaaattagccaggtgtggtggcgagcatctgtagtcctagctactcaggaggctgaggtgggaggatcacctgagcccaggaggtcaaggcttttgtgagccgtgactgtaccactgtattccagcctgggtgacagaatgagagctagtttcaaaaaaataaaagtggataacccccaaaaccactgtcctacttttagaaaatccaagatagttttgggaagggaattttggagtctcattggccatgaaagggactaggcaggcttctcagggagacttgtggggctgattacgtagtgcccagctctacttggaaaactctttttgcaacatttacatggaaatcagagacacagacccagatgttgggttaaaatgagacaaaggaaaaaaacagtcatgtacaagaggcaagaagaccacttttctaaatgatctatatttattagtactctggtcagagaaatcccaagtctaccatattggaggttttctggaattccaggctatctgttagactgtaggcttcaaaggcttggcttgtcatattgggccaggtttgtgcaggagataggcctacagctggaccagcaaagatgctgagagaggaaccctgtcctcctacctggtactttgtgggtgagagatactgatacagacagtggaaagaagagctggatatctcattctcatcaggaagattgtacagttctatgatttggaatatgtcataggcatcagagtacaaagcaggaaccgaggccaccagcctctcccactgagtatcttgcatttggaagtcactggtagaactctcagtgaaggtagagttccatgcccaattggaagggtctaagggctgagatggaagggagctgtagaaatctgaaatcacaggagaaaaagcataaggactgggggatgttctgggggaggtgggcacattcttcttggatggaaggatctggtttcgttgctttgctgattgctgctgctgctgcttcttcaatttgaatcgccggttcctgaaccaaacctttactgttgactccggtaggtcgagtctcaaagctagtttctcctgaagatttctatctgggaacatggtctggctaaacagagcttctagctcctcatactgttggtgggtgaaagaagtacgttctttatgccttctccgtattgctgtagtcgcagctactcgggaggctgaggtgggaggatcagttgaacctgggaggttgaggctgcagtaagccgagaccgtgccactgcactccagcttggataacagagtgaaactgggactagctggatcctgtggtggtatcaccttcatgttggaataattcctattgatgaaagggtctggctggggattctctggggccattctgttcctcatggtttctgaaatctgtcacgaatccccttagagtaaccattttcagtcctacgtggtgtgtctctctctggaaatgc

SEQ ID NO: 13254 - RNA, 6248 nt, Homo sapiens
  source 1..6248: mol_type = other RNA
gctgggattacaggcatgagccaccacccccggcaacttttttaatttatattttattttttattgaaataggtggcccaaaacttgtgaaacagaactcatgctgaaggacgacattaatcataataattaaagagacagatattgcttatgtaaaccgtataaagaattaaaaacaaatccaattctgactttcaatgttgtttcaacaccgaaaaaatatgatggcttattctttggtatgagaagtcattttgatggtatttttaccctattaaacaaaaatgggatttaaaaatctggttcgggatgttcaaagataattgctaaggcaaattttgcaatttgagaaaacctaactgtaatgatccatttattcagttatttgttaatactcaaattagtaattttcactctgaatggtaaataaaatgttaataaaaaataacaagacatataaactttccctaatgagatgcagttaataaaaacggttgtttacttcagagtatttactataaacatgtccacttatgttattttattgctatctatatactctttcagtttactgtattactgtacttttctctaaaactttaaaaatctgttatctaaaatcaattctctaatgctaattttgcaggaaaactgtatttcacattattaatctcattaatataactttcctataaataagcatgaaacatttggaggatgcatatataatgagtgcttggttactatagtagcgaatgtcaaactaattgctaaaaaaagtctaaaggttttcacactttgaaaaatctagtatatcatctatcattattctccaatattgtggcaagaatagtcaccgcaagtaaaaattaagatactgttgtagagattaaggcaattttattataaattcctgatatattccacccctgcctgttcttaatctaaatgtaatttagcactgcaaaccatttatgaaaataaatttattttaaaaggcataaaagttattagtgtaaaaagaaaaaatatctatacctacaaaaaaggccaaagacactaatgaagttacctcagtaaagatactgtaacatgtaacttggccagccaagttacaacacattcctcacaactgtattatgtctcaaggttctgaggatctgaaaggtcttttgatccacctaaaagtggccaccaaccaaattaatttctctgaaagacatctttaagcaattatttcagcctaacctcgcttcatatggactcactcagatggctcatgttttattagggacttgaaggtttaaaaatatgtagtcaatccagggcaaagttatgttgtttgcctatttgtaaaattaacacatacagaaaataagattcaaactgatattgaaaaagactaacatattcatctaattttaaaaaaaaacctaccaatagaacaaaatatattttattttaattataccagcacagtaaggcccagaaagaccatggagttgcacaaagaatgttcagcaccagcaagataaaacagatactggcagtcagtgctaacggctagcacacaagcccctgccgcatttgtatgatctggagcagagcctcctgaacatcttcatccatgtgaccctgtgcagcactaagaaggtgtgtccgataaattgcaattacttcttggtgctgtctgtcagcatcggccagctgttgctccagagatttcacttggtgctgcagagtgtcaatcagctggctctgcctcttggtggggttcccacttgtgtaggtgagttgggaaaggccattgagtgcctgttttaatctttccacatcattaagcagttcagttatcttattatcttttgcttctatttgtttagcagattcttgtattcttctttgtaactctgtgattgttgttaaggacttatcacatcgttccttctgatccttaatttcttgctcaatgctgaaatgcagtaattccttctcatcttttgcagatatttccttctttttggcatgcaaaacttcctcacatacttcctcatactttctattcagattggccaatttttcatttaagctagaaatctgtgtctccaaatcactttttgttgctttatatttagacaagtcaactacctctctagtctctaatttttttaatgcttgtttagtattctgaacctccgactgaagtttggagacttcttccattttgttttggctttcttcttccttttctctcaagctggcttttatgattccaacttctttctcaaatgcttctttaatctgcaaatgctctgccaggggtacagaagagttcttttgattctccaacaattgatgcagtttggtcactgtctgctgctctttctcgtaacacctttgcatactcttcagttcttcctttagattttcaattgtgccattaagagattttttcagagcctcaacctgttccaatggaacatgttgtttttgcaaaagattttgcactgcaagtatctcagaagtctgtttggcattttcttctactagcttctctttcacattctttacttccgtgtatttctgtgacaagtcttttaactgtttgtttagctcgtctgtttttctgcttaatgctctttccatttcatgagacttctcaatgagaactgtcttatctctcaaatctttctgaagggtaaaaatctccttctttaacttgtcattctcttgcttgtttttcttgacttcttcttcactgacactatacttttgtgtctgctctgataactggtcttttagttctttctctgttgctttaaattttctctcgcactcctcaaagctgacaattggggcgtattttaccttaatgcattcttgtattgtgtcgagctccttcttctgggctttaatttcggcatgcagtgtcacaatctcttcttggccttttctgtagttggccaagatttcagcattactatcctgcacctttctcatgctctgacttagcgagctcatctttgcctcgtgctctgccaggctgatgtactcagcttttatttggttctgagtgttttccaggtttctttttaatatttcattcttatcttttatttttacaaattcctgatttatatcttcaaattttttcttcacatctaataattctctgttagttttggctaacgtgtcattcagtgtcattttaacctcttcatgggttttaactggcacatactgattactcatcatcttcttcaagttagtgttttcagatgtgagagcgtgtattttctcctggtcttcaccacattttttcttaagttcagacagctgtttcttaagttcaacaatattggatttcagagctattatctctttttcatgtttctcaggaggtacaaacacagtttctaggcggcttacatccttacttaagctgtcattttccagtagcaatttctccatttccaacttcttttctgtatatttttgtgttacatctaaaagctttctattaagatcatcaataattgcatcatgtgactttttcatgtcttcacttacttttaaaggaacataatgatttttcatttcaattgttaagttatgtgcttgctccttgaggagcttattatccaaataaactttttcaatttccttttgtagtgtctgatttttcaatgttaactcagtgatcttcttcccaagttctcctgatttctgttctaatctgctcttaacctgttcatgttcctctggtttgacgtgctgagcaagcttggccttaacattctcaagttctctctttaactgtctaatttcactaagtgatttttcatgttctctttccatttctactaatttttttgctttctcattcacttcatttgataatgagctcttcatgttttcaaatttttcagctggaatggaaagggccaacttcgctgacaattcttttgcctggccttccatctctgtgacctttcttcctttcttctctcgctccatttcacacatactaagttccttctgtaatcgcttattttcttctatcagcttgccttcatccctcttaaactcttctactatcatctcattttgtttgatttggtttcttaatttccccacttctgctgaagcaccttcatattttactttcaagtctttcaactgatccttcagttcctcggttagtctgtgattccctgaggctgcttcacttgttaagtgttctttaagggcaagaaaatgggtctgcatttgtttaactttaccttctgactcatacatcctcttctgcacatcttttaatgcatcttctaattgctttatctgttcatctgaatcctccttgaccctttcacattctaatgctaaagctttgcattctgccactttgtgtgccagttcattttggagcttcagtcggtcttgttttgctgactcacagaaagttcgcattgcttctaactctttctttaaaatttcattttcagagtatgacgtttgactgggtaaagatagttccagaggtcttaacatagatctgctttgcatatgggctggtatacctggggaagtacactgtgagtctgccatatacatctgaccttgtttaagaagcatatcttcttttcggttactgaaatgacttcctgatcctaaatgatcactctcaaaatatttaaatctatttttcagagcctcaatagtccttaagctttcttcatgttgcttttctttagctgccaaaagggacttcagcttttctctctcgctttccagatcatcagcaaccataacttcctcattcagctgtaactgtaaaccattgactttatccaaaagtattctttgttcttgctgaatttttctcaacctctctttcaaatcttcattttcaatctccaaatcctgaatattttgatgctccctctgatgtgacttcacatttacttcatcttgcatgtgtgtcaaatttcgctgttgcaaagatggccctttcttccaaagttctctccctttgttggtattttccgatgcagtcttcaacaaggttagaatgtccagattgtcaccaattcttgcatagtaagaactatcatggccaagcgcatccagcaagcttatatcagcaccatttttaattaagacttctactgcatctctgcaaccatattcgcaacctagcatgagggcagttctgttttgtttgtctctggaattaacatccgctcctctatctatcagcagttgacatattgttggcctactcatctgagtagccagaacaagtggtgtccgcccgtctacatctttggcattcacagaggccccatggtcacaaagcagctgtatgctagaaggacaatctgccattgcggcatcgtgaagtgcagttcttccctgcaggtctgcatgctcagtgggacaattgtactgtagaagtttttgtaggcacaatgcatgtccatacttagcagccaggtgaagagcatttctccctgcagtgtcactggttgtaatatcaactccatgtataaggatggcattcaaacactcaagattcccctttgaggtcacaacatggaagacagatctgccttccacatctagtttgcctggattgaccccctttttagcaaggattgaggtcactttttctacatcccccctttctgctgctttcatcaatcggtcatcatatttattccaatctgctgcatgatcacttattttccagttgcattccaaatttccttctcccttctgtgctaacttcattaggagagcagagttataaaatcttcccaaaacacatgatatacaagaaacatttaaaattatacttttgagggaaagcatgtttcttttgttctctgtccagttctctttgcctttgaggcaaaaaaggaaatcaataactactgaacacctaccctgtaccaggcactaaagtcccaatcaaccctagtaaactaaaattatcatctccatttagcagataagaaaagccaaggccccagagacagtaaatgtcttaagtgttcaaaagcccaaccatgacttctatagttccaaaatcagtgtgcttttcccataccctttcagatttcaaatcacacttttagatttggctctggttacatagctcctaggactcttagatgcagtggaattctacatacattttaagaaactacccccccccaacacagacatttatttaaaaagtactg

SEQ ID NO: 13255 - RNA, 5965 nt, Homo sapiens
  source 1..5965: mol_type = other RNA
gctgggattacaggcatgagccaccacccccggcaacttttttaatttatattttattttttattgaaataggtggcccaaaacttgtgaaacagaactcatgctgaaggacgacattaatcataataattaaagagacagatattgcttatgtaaaccgtataaagaattaaaaacaaatccaattctgactttcaatgttgtttcaacaccgaaaaaatatgatggcttattctttggtatgagaagtcattttgatggtatttttaccctattaaacaaaaatgggatttaaaaatctggttcgggatgttcaaagataattgctaaggcaaattttgcaatttgagaaaacctaactgtaatgatccatttattcagttatttgttaatactcaaattagtaattttcactctgaatggtaaataaaatgttaataaaaaataacaagacatataaactttccctaatgagatgcagttaataaaaacggttgtttacttcagagtatttactataaacatgtccacttatgttattttattgctatctatatactctttcagtttactgtattactgtacttttctctaaaactttaaaaatctgttatctaaaatcaattctctaatgctaattttgcaggaaaactgtatttcacattattaatctcattaatataactttcctataaataagcatgaaacatttggaggatgcatatataatgagtgcttggttactatagtagcgaatgtcaaactaattgctaaaaaaagtctaaaggttttcacactttgaaaaatctagtatatcatctatcattattctccaatattgtggcaagaatagtcaccgcaagtaaaaattaagatactgttgtagagattaaggcaattttattataaattcctgatatattccacccctgcctgttcttaatctaaatgtaatttagcactgcaaaccatttatgaaaataaatttattttaaaaggcataaaagttattagtgtaaaaagaaaaaatatctatacctacaaaaaaggccaaagacactaatgaagttacctcagtaaagatactgtaacatgtaacttggccagccaagttacaacacattcctcacaactgtattatgtctcaaggttctgaggatctgaaaggtcttttgatccacctaaaagtggccaccaaccaaattaatttctctgaaagacatctttaagcaattatttcagcctaacctcgcttcatatggactcactcagatggctcatgttttattagggacttgaaggtttaaaaatatgtagtcaatccagggcaaagttatgttgtttgcctatttgtaaaattaacacatacagaaaataagattcaaactgatattgaaaaagactaacatattcatctaattttaaaaaaaaacctaccaatagaacaaaatatattttattttaattataccagcacagtaaggcccagaaagaccatggagttgcacaaagaatgttcagcaccagcaagataaaacagatactggcagtcagtgctaacggctagcacacaagcccctgccgcatttgtatgatctggagcagagcctcctgaacatcttcatccatgtgaccctgtgcagcactaagaaggtgtgtccgataaattgcaattacttcttggtgctgtctgtcagcatcggccagctgttgctccagagatttcacttggtgctgcagagtgtcaatcagctggctctgcctcttggtggggttcccacttgtgtaggtgagttgggaaaggccattgagtgcctgttttaatctttccacatcattaagcagttcagttatcttattatcttttgcttctatttgtttagcagattcttgtattcttctttgtaactctgtgattgttgttaaggacttatcacatcgttccttctgatccttaatttcttgctcaatgctgaaatgcagtaattccttctcatcttttgcagatatttccttctttttggcatgcaaaacttcctcacatacttcctcatactttctattcagattggccaatttttcatttaagctagaaatctgtgtctccaaatcactttttgttgctttatatttagacaagtcaactacctctctagtctctaatttttttaatgcttgtttagtattctgaacctccgactgaagtttggagacttcttccattttgttttggctttcttcttccttttctctcaagctggcttttatgattccaacttctttctcaaatgcttctttaatctgcaaatgctctgccaggggtacagaagagttcttttgattctccaacaattgatgcagtttggtcactgtctgctgctctttctcgtaacacctttgcatactcttcagttcttcctttagattttcaattgtgccattaagagattttttcagagcctcaacctgttccaatggaacatgttgtttttgcaaaagattttgcactgcaagtatctcagaagtctgtttggcattttcttctactagcttctctttcacattctttacttccgtgtatttctgtgacaagtcttttaactgtttgtttagctcgtctgtttttctgcttaatgctctttccatttcatgagacttctcaatgagaactgtcttatctctcaaatctttctgaagggtaaaaatctccttctttaacttgtcattctcttgcttgtttttcttgacttcttcttcactgacactatacttttgtgtctgctctgataactggtcttttagttctttctctgttgctttaaattttctctcgcactcctcaaagctgacaattggggcgtattttaccttaatgcattcttgtattgtgtcgagctccttcttctgggctttaatttcggcatgcagtgtcacaatctcttcttggccttttctgtagttggccaagatttcagcattactatcctgcacctttctcatgctctgacttagcgagctcatctttgcctcgtgctctgccaggctgatgtactcagcttttatttggttctgagtgttttccaggtttctttttaatatttcattcttatcttttatttttacaaattcctgatttatatcttcaaattttttcttcacatctaataattctctgttagttttggctaacgtgtcattcagtgtcattttaacctcttcatgggttttaactggcacatactgattactcatcatcttcttcaagttagtgttttcagatgtgagagcgtgtattttctcctggtcttcaccacattttttcttaagttcagacagctgtttcttaagttcaacaatattggatttcagagctattatctctttttcatgtttctcaggaggtacaaacacagtttctaggcggcttacatccttacttaagctgtcattttccagtagcaatttctccatttccaacttcttttctgtatatttttgtgttacatctaaaagctttctattaagatcatcaataattgcatcatgtgactttttcatgtcttcacttacttttaaaggaacataatgatttttcatttcaattgttaagttatgtgcttgctccttgaggagcttattatccaaataaactttttcaatttccttttgtagtgtctgatttttcaatgttaactcagtgatcttcttcccaagttctcctgatttctgttctaatctgctcttaacctgttcatgttcctctggtttgacgtgctgagcaagcttggccttaacattctcaagttctctctttaactgtctaatttcactaagtgatttttcatgttctctttccatttctactaatttttttgctttctcattcacttcatttgataatgagctcttcatgttttcaaatttttcagctggaatggaaagggccaacttcgctgacaattcttttgcctggccttccatctctgtgacctttcttcctttcttctctcgctccatttcacacatactaagttccttctgtaatcgcttattttcttctatcagcttgccttcatccctcttaaactcttctactatcatctcattttgtttgatttggtttcttaatttccccacttctgctgaagcaccttcatattttactttcaagtctttcaactgatccttcagttcctcggttagtctgtgattccctgaggctgcttcacttgttaagtgttctttaagggcaagaaaatgggtctgcatttgtttaactttaccttctgactcatacatcctcttctgcacatcttttaatgcatcttctaattgctttatctgttcatctgaatcctccttgaccctttcacattctaatgctaaagctttgcattctgccactttgtgtgccagttcattttggagcttcagtcggtcttgttttgctgactcacagaaagttcgcattgcttctaactctttctttaaaatttcattttcagagtatgacgtttgactgggtaaagatagttccagaggtcttaacatagatctgctttgcatatgggctggtatacctggggaagtacactgtgagtctgccatatacatctgaccttgtttaagaagcatatcttcttttcggttactgaaatgacttcctgatcctaaatgatcactctcaaaatatttaaatctatttttcagagcctcaatagtccttaagctttcttcatgttgcttttctttagctgccaaaagggacttcagcttttctctctcgctttccagatcatcagcaaccataacttcctcattcagctgtaactgtaaaccattgactttatccaaaagtattctttgttcttgctgaatttttctcaacctctctttcaaatcttcattttcaatctccaaatcctgaatattttgatgctccctctgatgtgacttcacatttacttcatcttgcatgtgtgtcaaatttcgctgttgcaaagatggccctttcttccaaagttctctccctttgttggtattttccgatgcagtcttcaacaaggttagaatgtccagattgtcaccaattcttgcatagtaagaactatcatggccaagcgcatccagcaagcttatatcagcaccatttttaattaagacttctactgcatctctgcaaccatattcgcaacctagcatgagggcagttctgttttgtttgtctctggaattaacatccgctcctctatctatcagcagttgacatattgttggcctactcatctgagtagccagaacaagtggtgtccgcccgtctacatctttggcattcacagaggccccatggtcacaaagcagctgtatgctagaaggacaatctgccattgcggcatcgtgaagtgcagttcttccctgcaggtctgcatgctcagtgggacaattgtactgtagaagtttttgtaggcacaatgcatgtccatacttagcagccaggtgaagagcatttctccctgcagtgtcactggttgtaatatcaactccatgtataaggatggcattcaaacactcaagattcccctttgaggtcacaacatggaagacagatctgccttccacatctagtttgcctggattgaccccctttttagcaaggattgaggtcactttttctacatcccccctttctgctgctttcatcaatcggtcatcatatttattccaatctgctgcatgcgcgctggcggcggcggcgccagacgacgcggggccgggcacgtcctgcctcctcaggcgggacttgaggctcttcatggctaactcttgcctggcccccgcgcgaaccttaaaggctgcggagtgccagcgcgcaaggagtagacggcagcggctgcagcagaggcggcgcgggctgtaccagccccacctgcctgccacctgcgggccccgggcagcagacgtcgac

SEQ ID NO: 13256 - RNA, 6142 nt, Homo sapiens
  source 1..6142: mol_type = other RNA
gctgggattacaggcatgagccaccacccccggcaacttttttaatttatattttattttttattgaaataggtggcccaaaacttgtgaaacagaactcatgctgaaggacgacattaatcataataattaaagagacagatattgcttatgtaaaccgtataaagaattaaaaacaaatccaattctgactttcaatgttgtttcaacaccgaaaaaatatgatggcttattctttggtatgagaagtcattttgatggtatttttaccctattaaacaaaaatgggatttaaaaatctggttcgggatgttcaaagataattgctaaggcaaattttgcaatttgagaaaacctaactgtaatgatccatttattcagttatttgttaatactcaaattagtaattttcactctgaatggtaaataaaatgttaataaaaaataacaagacatataaactttccctaatgagatgcagttaataaaaacggttgtttacttcagagtatttactataaacatgtccacttatgttattttattgctatctatatactctttcagtttactgtattactgtacttttctctaaaactttaaaaatctgttatctaaaatcaattctctaatgctaattttgcaggaaaactgtatttcacattattaatctcattaatataactttcctataaataagcatgaaacatttggaggatgcatatataatgagtgcttggttactatagtagcgaatgtcaaactaattgctaaaaaaagtctaaaggttttcacactttgaaaaatctagtatatcatctatcattattctccaatattgtggcaagaatagtcaccgcaagtaaaaattaagatactgttgtagagattaaggcaattttattataaattcctgatatattccacccctgcctgttcttaatctaaatgtaatttagcactgcaaaccatttatgaaaataaatttattttaaaaggcataaaagttattagtgtaaaaagaaaaaatatctatacctacaaaaaaggccaaagacactaatgaagttacctcagtaaagatactgtaacatgtaacttggccagccaagttacaacacattcctcacaactgtattatgtctcaaggttctgaggatctgaaaggtcttttgatccacctaaaagtggccaccaaccaaattaatttctctgaaagacatctttaagcaattatttcagcctaacctcgcttcatatggactcactcagatggctcatgttttattagggacttgaaggtttaaaaatatgtagtcaatccagggcaaagttatgttgtttgcctatttgtaaaattaacacatacagaaaataagattcaaactgatattgaaaaagactaacatattcatctaattttaaaaaaaaacctaccaatagaacaaaatatattttattttaattataccagcacagtaaggcccagaaagaccatggagttgcacaaagaatgttcagcaccagcaagataaaacagatactggcagtcagtgctaacggctagcacacaagcccctgccgcatttgtatgatctggagcagagcctcctgaacatcttcatccatgtgaccctgtgcagcactaagaaggtgtgtccgataaattgcaattacttcttggtgctgtctgtcagcatcggccagctgttgctccagagatttcacttggtgctgcagagtgtcaatcagctggctctgcctcttggtggggttcccacttgtgtaggtgagttgggaaaggccattgagtgcctgttttaatctttccacatcattaagcagttcagttatcttattatcttttgcttctatttgtttagcagattcttgtattcttctttgtaactctgtgattgttgttaaggacttatcacatcgttccttctgatccttaatttcttgctcaatgctgaaatgcagtaattccttctcatcttttgcagatatttccttctttttggcatgcaaaacttcctcacatacttcctcatactttctattcagattggccaatttttcatttaagctagaaatctgtgtctccaaatcactttttgttgctttatatttagacaagtcaactacctctctagtctctaatttttttaatgcttgtttagtattctgaacctccgactgaagtttggagacttcttccattttgttttggctttcttcttccttttctctcaagctggcttttatgattccaacttctttctcaaatgcttctttaatctgcaaatgctctgccaggggtacagaagagttcttttgattctccaacaattgatgcagtttggtcactgtctgctgctctttctcgtaacacctttgcatactcttcagttcttcctttagattttcaattgtgccattaagagattttttcagagcctcaacctgttccaatggaacatgttgtttttgcaaaagattttgcactgcaagtatctcagaagtctgtttggcattttcttctactagcttctctttcacattctttacttccgtgtatttctgtgacaagtcttttaactgtttgtttagctcgtctgtttttctgcttaatgctctttccatttcatgagacttctcaatgagaactgtcttatctctcaaatctttctgaagggtaaaaatctccttctttaacttgtcattctcttgcttgtttttcttgacttcttcttcactgacactatacttttgtgtctgctctgataactggtcttttagttctttctctgttgctttaaattttctctcgcactcctcaaagctgacaattggggcgtattttaccttaatgcattcttgtattgtgtcgagctccttcttctgggctttaatttcggcatgcagtgtcacaatctcttcttggccttttctgtagttggccaagatttcagcattactatcctgcacctttctcatgctctgacttagcgagctcatctttgcctcgtgctctgccaggctgatgtactcagcttttatttggttctgagtgttttccaggtttctttttaatatttcattcttatcttttatttttacaaattcctgatttatatcttcaaattttttcttcacatctaataattctctgttagttttggctaacgtgtcattcagtgtcattttaacctcttcatgggttttaactggcacatactgattactcatcatcttcttcaagttagtgttttcagatgtgagagcgtgtattttctcctggtcttcaccacattttttcttaagttcagacagctgtttcttaagttcaacaatattggatttcagagctattatctctttttcatgtttctcaggaggtacaaacacagtttctaggcggcttacatccttacttaagctgtcattttccagtagcaatttctccatttccaacttcttttctgtatatttttgtgttacatctaaaagctttctattaagatcatcaataattgcatcatgtgactttttcatgtcttcacttacttttaaaggaacataatgatttttcatttcaattgttaagttatgtgcttgctccttgaggagcttattatccaaataaactttttcaatttccttttgtagtgtctgatttttcaatgttaactcagtgatcttcttcccaagttctcctgatttctgttctaatctgctcttaacctgttcatgttcctctggtttgacgtgctgagcaagcttggccttaacattctcaagttctctctttaactgtctaatttcactaagtgatttttcatgttctctttccatttctactaatttttttgctttctcattcacttcatttgataatgagctcttcatgttttcaaatttttcagctggaatggaaagggccaacttcgctgacaattcttttgcctggccttccatctctgtgacctttcttcctttcttctctcgctccatttcacacatactaagttccttctgtaatcgcttattttcttctatcagcttgccttcatccctcttaaactcttctactatcatctcattttgtttgatttggtttcttaatttccccacttctgctgaagcaccttcatattttactttcaagtctttcaactgatccttcagttcctcggttagtctgtgattccctgaggctgcttcacttgttaagtgttctttaagggcaagaaaatgggtctgcatttgtttaactttaccttctgactcatacatcctcttctgcacatcttttaatgcatcttctaattgctttatctgttcatctgaatcctccttgaccctttcacattctaatgctaaagctttgcattctgccactttgtgtgccagttcattttggagcttcagtcggtcttgttttgctgactcacagaaagttcgcattgcttctaactctttctttaaaatttcattttcagagtatgacgtttgactgggtaaagatagttccagaggtcttaacatagatctgctttgcatatgggctggtatacctggggaagtacactgtgagtctgccatatacatctgaccttgtttaagaagcatatcttcttttcggttactgaaatgacttcctgatcctaaatgatcactctcaaaatatttaaatctatttttcagagcctcaatagtccttaagctttcttcatgttgcttttctttagctgccaaaagggacttcagcttttctctctcgctttccagatcatcagcaaccataacttcctcattcagctgtaactgtaaaccattgactttatccaaaagtattctttgttcttgctgaatttttctcaacctctctttcaaatcttcattttcaatctccaaatcctgaatattttgatgctccctctgatgtgacttcacatttacttcatcttgcatgtgtgtcaaatttcgctgttgcaaagatggccctttcttccaaagttctctccctttgttggtattttccgatgcagtcttcaacaaggttagaatgtccagattgtcaccaattcttgcatagtaagaactatcatggccaagcgcatccagcaagcttatatcagcaccatttttaattaagacttctactgcatctctgcaaccatattcgcaacctagcatgagggcagttctgttttgtttgtctctggaattaacatccgctcctctatctatcagcagttgacatattgttggcctactcatctgagtagccagaacaagtggtgtccgcccgtctacatctttggcattcacagaggccccatggtcacaaagcagctgtatgctagaaggacaatctgccattgcggcatcgtgaagtgcagttcttccctgcaggtctgcatgctcagtgggacaattgtactgtagaagtttttgtaggcacaatgcatgtccatacttagcagccaggtgaagagcatttctccctgcagtgtcactggttgtaatatcaactccatgtataaggatggcattcaaacactcaagattcccctttgaggtcacaacatggaagacagatctgccttccacatctagtttgcctggattgaccccctttttagcaaggattgaggtcactttttctacatcccccctttctgctgctttcatcaatcggtcatcatatttattccaatctgctgcatgtctgttcttaggagtacaagaaaaccaacagttcatcatagacaggatttagtttcttgttgctaatggcaaactactttgcattaagttacaaatctctgtaagctcacaaagcaaactctcagacaaactcctgacaagtgactcagtccctcacatgctgtgctacacttagcttggatctctaacgatattttcttcgtcttcaggatccttctccgccttcataacgctcgaatattatcttccttgcaatgcagaacttgattaagagcagccccaagtcaggtacagtaactctatctatttcttattctttggaagctagctatctttcaaagttgtccctttgagggaccccactggaaaacttgaacagcactctgcatcctgctgcctcaacact

SEQ ID NO: 13257 - RNA, 5985 nt, Homo sapiens
  source 1..5985: mol_type = other RNA
gctgggattacaggcatgagccaccaccccctgccaagcctgggtctttctatcgtgtctctgcttgggacttctgcaggtcaacttgtgccaataaaagtggtgctcagggtgggagcttttctggcatcctgcatatgaagtacatttttttccctgaattaattctgtcctcatgcattcaataaagctttcactataaagggcaaaagactttgctcaaaagactgactttatattcttatattcttttattttgaggtcaaagggattggaaaaagtttattccacagctgctatcacttgcttgtttgtcaaagggttaatataaactgcagtgtcataaccaaataattagatctaggtctgaatgcaagtttgtaaacagggctatagatatactgacagggatggtggtatttggagggagctgttactgaaggacagtgagggcattgccgggaggggagtgggctgaggggaatgaagaggagaagagaaaataagaaggcagtgagaggaagtcttgttgacagaggaacaaaagtctcggttcttgttcatcagctacacactgaattctcatgtcttctaatatccaccacaataagtaactacagcaaagacaaggctaggacctaccttagagaagaatgcttgataaaacacactactggatttcaaatctgtgttcatatgagtgatgcgagtgtgtgtgcatgtgctgctgtaactatcatcaccaccaccttcacaccattgtcttcatcgtggtcttccgaactttccgactctaccctctcccagaaatccacccagcccagttagagaaccagcatgggactcctgggcttaaactcctcccatcttcactggtgaactcttgtgtctttgtctggttttggtgtcagggtaatattgaccttatagaatgagctatgaagtgttctctctttttctattttttggaagagtttgtgaaaattggtattaatttttctttgcatgtttggcaggaatcaccagcttaattgtttttgtaaaccattgcacctagttcacagttgatattcattaaaggttctgcattgaaatgaatctgtttctataatgttgtatcttacctgatataatttaatgatgaatatttaacttaaaattttaaaagaggcttctatctgatatatcatagaatactacaaaagtccagactgaagtccaaatttcagactatttataccagatcttgaattttataggtgtgacctactagtcactcctaaaaatagattccttcaaatttctctgggtaccaggtaatattcattcaactaagccctgaactgagttccagcttcctatctgtatctccctaaactcattactaattaaaggaagccatagctacattttaaatacaaaatgcttaacttacaaaggctcgttaaaaggtaatgattcaagtgttttgttaataacaaggacttattaccttttaagaacaattgtccaaatgtatcatagaatttgttaataatgaaaattccactgttcttacccttgtggtgaagccctggaatctgtattttaacaagttccttgggtgattctaatgcagttggtcagaggagcatactttgaaaaacaccactttaaagttatcatgactttgtggataaaggtgatgaataaagtaaattgtgtctataataaagtgccgggcacaccacttggctcaaggtggcatgctgtgggtgccaatgtgactggtttaagaagcataattcaaattaccttaaagagggttacagctgggtaaaaacttaattgttgataggactgcaggcatatctaggtatttttggtcactctcccacagtctccactcattctcagcaataacaaagcatggactatgagaaagggcttatgtttggaatcccaattatgctgtgtatcagttgtgtaacttcaagaactaccctccctaagcctcagcttcctcatctgtaaacagggataatgtcatctaccttgctgtggtggtgtgcagatttaatgaaatacagtagactttttttttcttaattgccctttgccctttgcccaaccctctcccactcccctcctccagatgggctcatgtaacacagggccagcaggagacggtacaaatgcacttgcacagctacagtgatggatggctgtcaagtggctgtctcagctaaggaaactcaaacatgaaaagggaagaaaaggaagcagattcaaaggctggtgatgagatgatcaagtgcttgcttcagaacacaaatctcaacatgagaccagtgaaattcaattgaagcagagcacacttatatcctcgggtgctttgatatatttaggaggaaatgagggaatatcaaggtcaggtctaaaaggagatcaatgaaaagtgataatttctgctgtcgcaggagataggcactgggtgtacaaatatttcacgtagatggaatgatccaatttcatccagcaaataccacctgtgaacacatttctggtatattttgctgaatggacaccaagtttgtgagtaagtgaatttctagcaatggtgaaattatctctgcgagccccatacagacattccttactttaaatccatcaatttaatcaacggagagtgtaaaattataggagtctcttttgattcctttcatattcatttcctactatggctttgggattcaaatgattagctctgtgacattagaggcaagttactttacctcaccgagccttcttgcttaatcctcacttcaaccctattagctctattctatttccaggaacatgggggtagagggtgccttaccgaaggtcacccagctagtaagaagtagaccaagcccagggcaggcttcctctgtgttccattccaactctggggacttgcccagggacagcaaattagggggccaagatcactttttcagatgttattctgggtctttccatgttcagccatcagagtttataatccaccaaagggaagattcaatgtctgtataaggtctctcacaaacagacaggcatggtgaagtggactgcatgaactactttgtatgccttcctgatgcttggttgtaagttaatacatccatcttcctctttcctttctcacagaataaatacccttcagttaccaccacttttgttttgcgtgattctataatctactggcttctaactgttcactgttcaaagaagatagatacaaggacctaagggtaagggatgtacataacctcagataaagggtagtattctctggactagggaattgtgggaagagcatgataagaacagattagaactaaccactattgttatgactgcgtaatgtggaaattagagtcatctatccatccagccagccagccagtaattcatagaaccctagaattttagaactggcagacaatcatagagataatttaattcaatatgttaatttttacagatggaaaaaaattagatggagagagaggaaataactccattaaagtcacatagcaactgatggcagagctggaaccagcattccagcttctcatttcctggtccagttttgttgttgttgctgttgtttcttttctttttttcttttttctttttttttttttggcatcagaagagacagtattttaaaggtactaatagcatattgttattaaaaacaacagtagacaatgtctccacaaaacctaactgcttgtaacatatcttcacttaagtatttcatgtgagtcaccatgtacagggcattagaaattattccattaagtatatgctctgaattgcttgggtttgctcataaatcccaatcccacaggacttacgaaggcaaatgatcttcccaaaaggtccatgtgccttttgttctttaggctaatcctcatataacttgaaaataaatctcactcctctgacggatactctgggcaaacttaggatttttctgtcaagtaagtatttcatgaggacatgctagtgagagatgctaaaaaattcactcattaatttgtttaacatatattaacttaggtgctgtgggaagacattgggatacaacagaggacagaggatacaaagtccctgccctcttggagagcagtgacttacattccaatgaagggagagggaccataagccaataagctggtatgtcaggtggtgggaagttccaacaagaataataaaggtgacagagagtcacatgtgctgtgtgtgtgtatgtgtgcttacctagggtcaacaacagcctctctgatcaagtgagagttgaacagagacctggaggaagtgagccttgtgggcttctgcagggagagtgcaaagaccctaaggccggaggatgtgtctgaggaatgctgaagaggccagtgaggctgaatgggagctaacgaggagtaggagaagagatcagagaagggcgagcagagtggggagggccttggataacagagagagggatttggtttaatcttctgtgcgatggggagcggctggaggatttgagcagacctgatgtagctccgagtggcacgatttgactcttggtttatgtttacttcagctgctgcattcagaacagacactagatgtttctcactctattaatgtcacgctccagggtcaatacagcattttacatctgaatgctcttttcaaaaatatctgtaggagctgctcactgcactcgccacctcctcgcggatttgccggttgagggcgtccgccgcggcgcgccccctgccagcctcggggccggtggcctggacctgggcctgggccgcgggcagcggcgtctgctcgtgccccaggccctcggcgcggcgcacaatccaggcaggcccggccttcctgcgcgtgtcgcgctcgtccgccccggacgcctttccggccgccaggccacccgctccgccgggggccgcctcctgctcccgggcctcagcggcggcctgcactggccagcgctcctggctctgcggccggcgcttgggcgccccgagaatgggcgccgacgcctgggaggccgcagagatctgcacgggcttggggatccacgggtggtccccgcggcgcggcagcggccaggcgcggaagtccttctggtactgggtctcgcgctcgaagggagcgtcggagggctggtattcgctgcgcggccggcagctgggctcgggccgctgcaccttccaggctcggtaatcctgccgcatcaccgagtccgcggggccggaggtggagccggagcccaggcccgggcccggcccgctccggccggggcccgccgccggctcgcgctcgccggtaggcccaggcgctggccccgttgcccgggcaactgcatccaactcgccctgggctggctgcgtctctatggcaaccgcgcgcgccgaggggggcgcgagcgccggctgcgcctgctgctgcggcggcggtggctgcggcggggcgcccgggtgctcggtggcctccgagtacttggtgaaaaccagcggcacagcgatgtccgctttgtccaactggttccagaagcgggcgatgcagcaggccctcgtgatgcacggccacgccatgatgctagctgaaaagccggcctcctctttcttcttgtggttctaaagcaagtctctataatcttccttcagcctccgatcctgaccggccaatgtggttcccaccgttttctacccccgatcagccggagctagttcgccctcctccctcagcgagcacccggggagagctgtcctaggagagtctgtagagtccctcgattaccggtcgcaaacgcctttgggagcgcagtctgctgcgagcgccgaagggtgagacgcacggcgttcccgagtccccggcgagggtgtctgggacgcgcccctccctgcggctgcggcggcgcacagacctcggtcgagcgaggcgacgtga

SEQ ID NO: 13258 - RNA, 1762 nt, Homo sapiens
  source 1..1762: mol_type = other RNA
gctgggattacaggcatgagccaccacctggcctcatattggctttcaatgcttttgggagcagattctgcccatgccctcaatgtgcacaaactttctagcacctgacctctccctcctttgtacgtcttccaggtttcctacccttcaaagaaagctaagttcaaggtgagttccttccttctgggaaccctggccacctcttggtctatcagtgtttctcagcctgaggctgcacctcttcaacggggcagaaagaaacatactgggacatctctgtagtcacaagctggggaatactggtatgcaactcccatttggtgagcagggcaaggttgccaactgtttgtaatacatgggatagtcctgcagaatggagaactggcctgtccaaaataaaagtagcaaccccctctaatgaaccactctccccactgaaaggacacgagcatgtggcagtttgagttagggtagcagtgggaagaggatgggctctggagccacacctgggtttgaatcctggctctgttgcttattagtggtgtgatcctagcaaatttcttaacctctctgggcttcagtttccatgactatcatacaggtgtgaaagcaaaagcaacccatataaggttgtctggcaggttaacacagataatgacagtaacagctaatagttactgaacactttaaatcaccagatactgtgctaaaagctttccacatgaccccatgggaagggcactattatttttctccacattcaccaggaaattgaggccagagagattaagtaacttgcccaagatcacagagctattaagtggcagagtctggactcaaagtaaggtagtcaaatgccagagcccacgctcctaacttttcactatgctgcctctggctccttacgaaacacgatcatgtgtgaggagcccaacatggcacttagcacacagctaggccacaacacccggcaggtggtactggtgttactcacctgagtactgtcacaactaacatgacattactgctcacaaatcactttcccaacagctgtggtggtggaaacacccaccagatcctcatcatgtctataaggaaactgtggcccagagaggtcattgttcttgtcctagtcatctacagtgtgcaggggaaagagtcccttgagttttatagccaggattcaaacctggctctgaatgatgccaaaagtcatgttctcatccaagaccctgtactggttcccgagaaagctgcttcaaatgttgcagagagatgccttctgacctgatggtgtgggacagggccaggattcccagcacgaagaaatacatggacagcaggaggttgatgtactcctgggagaatattttgaaaaagaggtagagccccaagagtgtgcagctggcgatgatggggaagcgggcggcatcccggctggtgattgtttcaggcatgtctgaagcattcttgccgcgggcgcagcgtacggagcgcagggcgccgaagaagatgggcagcagcgccatgagcaggaggctgccgtaggccagcgcgatgccctcgggcgtggaaggcggccgcgtagtgctgttggtggggccgcctgcctcggcactgccgttatgcggatcgctgagggccgagtccatggcgagggtgcgttcgggatccgactccagctccggttgctgcagcagggacgcaggcggagacaccggctctgcagggaaagccacgttcccctaaggcaacaggaagt

SEQ ID NO: 13259 - RNA, 996 nt, Homo sapiens
  source 1..996: mol_type = other RNA
gctgggattacaggcatgagccaccacgacaggccctcaccccaagtttctgattcagtagttctgggttggggcccaagaatgtgcgttactgacaagttccctgatgctgatgctataggcccagggggaatggggaagcacacttcgaaaacccctggtggagagtaaagcatcagcagcaggcagacgttgaatcatttccagagtgaatggatgaaaagaggcgtcttcttcaggaagagaggtcttcctgtagtcaaagactaggctgacggtaaggccacatcggataacttaaggtggtaggcagagccgaacttcagagtctggattcagagacgaagcaatttggggggacaaggtcgaggactgaccctgccaggggaatgataggagatcaaggaattgggtgttacaagggtattcaaaatgaattatttctggcagaggctacagtctagaggacagttccaacaggaagtgaagatctgaagggttggaagtagctacgccgggcctgaattctgtagcgctgaccgtgggcaggccctacagacagcaagcagtccatccacgttagtgcaccagaactagcaacaaaatctacgggaagtgtgcgatccctcagcaacaacgctgcacgctgtgtagcctcccttacagctttataggaaccacggcgagcacaccctcctcatgcctcaggtttcccgcttaaaaatgcgctaatagcagtaatagtaaaccacacaacctcagcgagatgacacagtgaggtggttaacgtaaagctctggacacacagtgcgcacctatacatcagttattaagtgtcctgttggctactacaggtcctggccaatgctcagagttgcgtgtggcctatgagcctcacgttgcggcgggcgcgcgtccccgcacatctgcaggacggcgccatcctcctccttaacccgcccagctctgggatgttgttgcctgggcgggactaga

SEQ ID NO: 13260 - RNA, 5548 nt, Homo sapiens
  source 1..5548: mol_type = other RNA
gctgggattacaggcatgagccaccacgaccagcagttaatcttaatgtatcttaaatatatgagaggccacttgctcagtgtcagaggtcggcatgtcattaaaccagctttaaatattgtttttattgtttattttttgagacagactcttactctgtcacccaagctggagtgcagtggcacaacctgggctcactgcaacctccacctcccgggttcaagtgagcctcggcctctcaattagctgggactacagtggactacagacatgcaccaccacgcccagctaatttttgtatttttagcagagacagggttttaacatgttggccaggctggtctccaacttttggcctcatgtgatctgcccaccccagcctcccaaagtgctgggattacaagcatgagccaccatgcccagcttcacctttaaatattctaaatgaaaacttttgcagcctggctttatgggggttagaatttggggcataattactcctgtgggtagagacaactccaggttgtgtttggaggaaactgttggccccattcacaggtatatgcccagccaaccactggcaaaggaagacgacttcatcaacctgttttgctttctctgaagtcattcttacttgtctcttggccggatggtctgcccaatagctacccttctaagggacaataacctagacctcctggttcctagattcacatcaaaccctccactgagaacactattgatggaaaactgaccgaaggaccaacagcccgttagtcttctagggattctaaacccatctagaccagcccctttcagtcctcttcatccacttatttgactagtcctttgggggttatatctatgttaagctatattatcagaaacaatgctttgatacttgtgtttattattggtaaaactgttaagtttgccatgttgtagtgttctctttatgggaactagagggaaaggttccttagatctccagattaggggtagctgcctcaggtttatcgcatggagtctgaacttgatcttgtttccttctttacactgacaactaggaagcaaaatctgttatttatccttaagtgtataagacctgctgtaatgcagtttgtgtggataagattattttcctggcctcaacttttattttcctttagcccaatttccctacttaaaatcgtgtaatttttgtatttttgtaagttgtccttaaacttttttggggagaattttaaaaatagaagaaaaactactctctggtgttagacttcagaatagaggatatccttgtggggacagtgactggaacgagacacaggggtggcgtgggttctggggtgccagtcatgctggacgcgtcatacaggtatgttcactctgtgatgtcagtgagctaaatacttatgatttgtgcacttttctgtatgtatgttaagcttctatgttcaaaaaatgaggactgagggaaatgatactcacgtgccatatatatgtacttcctttaatcctctgaacacttttaagttagtagttatccccattataaaaacgaggaatgtgaggttcaaacaggttaaggaatgaggccaaaattccaaatgacttctgataacaaaagcacaggcttatcctactacactacactgctccttgctctttttttttttttttttcaattggacacggggtctcgctctgcacccatgctgtagtgcagtggtgtgataatggctcactccatcgctacagcctccaactcctgggctcatgggatccttcaacctcagtctcccaagtaggtgggactacaggcatataccaccatacctggctaattttcttatttttttcatagagatggggtcttgctacatcacccaggatcccactttcctactttaaatggcctgtctttatccagcttagccaataaaatccaagaaacattggtcagacctagtagagacacaggtgaaaggacttctacggagggggcagtgggcagcatctgaggctgaagctggctgtgggattcatttggcggagggggctttgggagacagcactggactgaaagtgcggagcttgaggctgcttctggacagggctggattctcactgtgagaaggcccatgaagccccctaaaggtccaccatctctacaagttccatcagcccctcccaagaagttgaggacagatggcagaatcacaacacccagcacgcacagtgtgagccctgctgcctgcccctcttctcttcaggagccaggatttattctgattgtacagaaccactatgactattatccaaccccttcacactgggacccctcctccagatgtagttggagttgaagggcccaggcctgctgcatgtgcagtccagtcatgtactcaagacagggttctcacaaacagctttctgcagaaaggcaaacagaaaggcttacaggctcaactcgtgagcagaacaaaataacctggattttacttcataaaggaaaagtcattaaaaggcaatgattgggaaagaggtcagcagaccaatttagggatttccccatattctgcaacactagctacgtgattttggactcatcatttaccccttgctactgcttcctcatttcccaatagggagttggaatgtccattctaaagcccctctcaactctgaaattctaactctaaactagacaccagtcatcttctccgagaaacagcactggacaaatggggcagaggggaggacaggtgatggccattccctctctcccccccagggcaaacaatgtggcaaggaactggcccagtgataaggggtctcaacaatcagatatggagccatggagggttcttgagcacagacagagcaaaagtggtatttgtggaacactggttttgaagaaatacataactgaactaaaggggagaccaatgggcaaatatgacactcgaaaaagaagaaaacagaacactcctttaggctagaaatatatatgagtgtcttattttagtctacttggcctcatttttccccatggttgtctgacatgttgcctgggggaacacttacagtcacatgagtaatgacaagaatctctttacgtgctacagggtccttaggcttttctttgtggaattttacagtgaacaatatggctaaattatgttattctataaaactttgactacttttcaggccttgaaattttatttacatgtctctaacacacacacatacacttcctattttttaatacaaaaagtacatagtagccccccgtatctgcgggtggtatgtttcaagacccccagtggttgcctgaaaccaagatggtaccaaactctaaaaaaaaaagaacaactttaacaatataccgtaataaaagttatgtgaatgtgatctttcaaattttttttgttttttttgagacagacttttgctctgtcgcccaggctggagtgcagtagcgtgatctcgacttactgcaacctccaccttccaggctcaagctaacctcccaccccagctgggactacaggcacatgccaccacatttggctaatttttgtattttctgtagagacagagtttcaccatgttgcccacactggtcttgaactcctgggctcaagggatctgctggccttggcctctcaaagtgctggggttataggcatgagcctataaccctcaaaatatcttaagaaaagtaactgactgcagttgaaaacaggtaattgaaattgtggtaagtgaaaccatggataaagcgggactactgtacatgctcattaaaaaaaattaagggccaggcatggtggcttacacctgtagtcctagctactcaggaggctgaggcaggaagactgcttgagcccaggggaggtcgaggctacaatgagctgtgatcacacaccactgcactccagcctgcgtaccacaagatcctgtctcaaaaaatatataaagtaaaaagagtgattttatttatttatgaaacagggtctcactctgtcgcccaggctggagtgcaatggcatgatcttggctcactgcagtctccgcctcttgggttcaagcgattctcttgcctcagcctcctgagtagctgggattacaggcactcgccactatgcccagctaatttttttgtatttttagtagagatggggtctcaccatgttggccaggctggtctcaaactcctgacctcagatgatcccccaacctcggcctcccgaagtgctgggattacaggcatgagccaccgcacccagacgaaagagtgattttaaattttcctcttcaagggaaggtataaatgccaacctcatgaaaggtcaggacttaggatccaggcccaggaccacaggagatgggttcttaggaggctttagaaatttgctctgaaggaaaactcttggcacacacaggccttcttttttattcaccgtctctcgaaacacatactcgtttaccacttcttcataacctgtgtccataaagagctgagccaggaagtcatcagtaaaaaaatatgatctggtcccatcttgtctaacataaaagttttctccaagtttgctgctggctttaaacctaagcatggcatgatcatacagtccgtagtcacgaaacaagacacttttgcctggttttaataccttatagcaggactccatggatcccaggtaactgcaaaatcatccttgtcccagggctggcgaagctctgaagagcagccatggcacttgtaaatgttttgtaagacaaggtgcatcttatcaggatgaacagctgacagcacaaatatcaacataacaacatccacagactctggcggtacatgatccagaagatcatctttagtcagatcacactggaataccttgcatctttctgtatcatataaaggattttgcttaacatattcaatggctcttggagaaaaatcacaggcataggcaaagatattcggatcttcttctaaaagtgggaataaacagtttccaaccccacagccagcttcaagcattgttaacttttgatcttcaaactctctacatgatcttagctcctcaaactctctggtggtccagtgtctgtctttgaagaaattagtgctatttcttttgtaaaaaagatcccaatttttctgagcctcttgttccaatttctgctgtttaaaatcagacaccaaagtttggtctcttttcagtttctcctcttcttcagaggtgagaatccttgcctgcagccctttcctttgcaaagaagccatctctgaaactgacggtaacacttaacacagctgaagattctccatcaccaaataatatgaatccacgctaatggatcagatacatttcctgaggtgagtttcacgcctcaaacagcacagggggcccacagccagccccactgggcctcggaggcagaatacgggaagaaccgcgaaacaaccctaaaccaattctgaggaccacgaattcggattatccgggagttcttttgccatggcaccgcc

SEQ ID NO: 13261 - RNA, 5320 nt, Homo sapiens
  source 1..5320: mol_type = other RNA
gctgggattacaggcatgagccaccacgaccagcagttaatcttaatgtatcttaaatatatgagaggccacttgctcagtgtcagaggtcggcatgtcattaaaccagctttaaatattgtttttattgtttattttttgagacagactcttactctgtcacccaagctggagtgcagtggcacaacctgggctcactgcaacctccacctcccgggttcaagtgagcctcggcctctcaattagctgggactacagtggactacagacatgcaccaccacgcccagctaatttttgtatttttagcagagacagggttttaacatgttggccaggctggtctccaacttttggcctcatgtgatctgcccaccccagcctcccaaagtgctgggattacaagcatgagccaccatgcccagcttcacctttaaatattctaaatgaaaacttttgcagcctggctttatgggggttagaatttggggcataattactcctgtgggtagagacaactccaggttgtgtttggaggaaactgttggccccattcacaggtatatgcccagccaaccactggcaaaggaagacgacttcatcaacctgttttgctttctctgaagtcattcttacttgtctcttggccggatggtctgcccaatagctacccttctaagggacaataacctagacctcctggttcctagattcacatcaaaccctccactgagaacactattgatggaaaactgaccgaaggaccaacagcccgttagtcttctagggattctaaacccatctagaccagcccctttcagtcctcttcatccacttatttgactagtcctttgggggttatatctatgttaagctatattatcagaaacaatgctttgatacttgtgtttattattggtaaaactgttaagtttgccatgttgtagtgttctctttatgggaactagagggaaaggttccttagatctccagattaggggtagctgcctcaggtttatcgcatggagtctgaacttgatcttgtttccttctttacactgacaactaggaagcaaaatctgttatttatccttaagtgtataagacctgctgtaatgcagtttgtgtggataagattattttcctggcctcaacttttattttcctttagcccaatttccctacttaaaatcgtgtaatttttgtatttttgtaagttgtccttaaacttttttggggagaattttaaaaatagaagaaaaactactctctggtgttagacttcagaatagaggatatccttgtggggacagtgactggaacgagacacaggggtggcgtgggttctggggtgccagtcatgctggacgcgtcatacaggtatgttcactctgtgatgtcagtgagctaaatacttatgatttgtgcacttttctgtatgtatgttaagcttctatgttcaaaaaatgaggactgagggaaatgatactcacgtgccatatatatgtacttcctttaatcctctgaacacttttaagttagtagttatccccattataaaaacgaggaatgtgaggttcaaacaggttaaggaatgaggccaaaattccaaatgacttctgataacaaaagcacaggcttatcctactacactacactgctccttgctctttttttttttttttttcaattggacacggggtctcgctctgcacccatgctgtagtgcagtggtgtgataatggctcactccatcgctacagcctccaactcctgggctcatgggatccttcaacctcagtctcccaagtaggtgggactacaggcatataccaccatacctggctaattttcttatttttttcatagagatggggtcttgctacatcacccaggatcccactttcctactttaaatggcctgtctttatccagcttagccaataaaatccaagaaacattggtcagacctagtagagacacaggtgaaaggacttctacggagggggcagtgggcagcatctgaggctgaagctggctgtgggattcatttggcggagggggctttgggagacagcactggactgaaagtgcggagcttgaggctgcttctggacagggctggattctcactgtgagaaggcccatgaagccccctaaaggtccaccatctctacaagttccatcagcccctcccaagaagttgaggacagatggcagaatcacaacacccagcacgcacagtgtgagccctgctgcctgcccctcttctcttcaggagccaggatttattctgattgtacagaaccactatgactattatccaaccccttcacactgggacccctcctccagatgtagttggagttgaagggcccaggcctgctgcatgtgcagtccagtcatgtactcaagacagggttctcacaaacagctttctgcagaaaggcaaacagaaaggcttacaggctcaactcgtgagcagaacaaaataacctggattttacttcataaaggaaaagtcattaaaaggcaatgattgggaaagaggtcagcagaccaatttagggatttccccatattctgcaacactagctacgtgattttggactcatcatttaccccttgctactgcttcctcatttcccaatagggagttggaatgtccattctaaagcccctctcaactctgaaattctaactctaaactagacaccagtcatcttctccgagaaacagcactggacaaatggggcagaggggaggacaggtgatggccattccctctctcccccccagggcaaacaatgtggcaaggaactggcccagtgataaggggtctcaacaatcagatatggagccatggagggttcttgagcacagacagagcaaaagtggtatttgtggaacactggttttgaagaaatacataactgaactaaaggggagaccaatgggcaaatatgacactcgaaaaagaagaaaacagaacactcctttaggctagaaatatatatgagtgtcttattttagtctacttggcctcatttttccccatggttgtctgacatgttgcctgggggaacacttacagtcacatgagtaatgacaagaatctctttacgtgctacagggtccttaggcttttctttgtggaattttacagtgaacaatatggctaaattatgttattctataaaactttgactacttttcaggccttgaaattttatttacatgtctctaacacacacacatacacttcctattttttaatacaaaaagtacatagtagccccccgtatctgcgggtggtatgtttcaagacccccagtggttgcctgaaaccaagatggtaccaaactctaaaaaaaaaagaacaactttaacaatataccgtaataaaagttatgtgaatgtgatctttcaaattttttttgttttttttgagacagacttttgctctgtcgcccaggctggagtgcagtagcgtgatctcgacttactgcaacctccaccttccaggctcaagctaacctcccaccccagctgggactacaggcacatgccaccacatttggctaatttttgtattttctgtagagacagagtttcaccatgttgcccacactggtcttgaactcctgggctcaagggatctgctggccttggcctctcaaagtgctggggttataggcatgagcctataaccctcaaaatatcttaagaaaagtaactgactgcagttgaaaacaggtaattgaaattgtggtaagtgaaaccatggataaagcgggactactgtacatgctcattaaaaaaaattaagggccaggcatggtggcttacacctgtagtcctagctactcaggaggctgaggcaggaagactgcttgagcccaggggaggtcgaggctacaatgagctgtgatcacacaccactgcactccagcctgcgtaccacaagatcctgtctcaaaaaatatataaagtaaaaagagtgattttatttatttatgaaacagggtctcactctgtcgcccaggctggagtgcaatggcatgatcttggctcactgcagtctccgcctcttgggttcaagcgattctcttgcctcagcctcctgagtagctgggattacaggcactcgccactatgcccagctaatttttttgtatttttagtagagatggggtctcaccatgttggccaggctggtctcaaactcctgacctcagatgatcccccaacctcggcctcccgaagtgctgggattacaggcatgagccaccgcacccagacgaaagagtgattttaaattttcctcttcaagggaaggtataaatgccaacctcatgaaaggtcaggacttaggatccaggcccaggaccacaggagatgggttcttaggaggctttagaaatttgctctgaaggaaaactcttggcacacacaggccttcttttttattcaccgtctctcgaaacacatactcgtttaccacttcttcataacctgtgtccataaagagctgagccaggaagtcttgtaaatgttttgtaagacaaggtgcatcttatcaggatgaacagctgacagcacaaatatcaacataacaacatccacagactctggcggtacatgatccagaagatcatctttagtcagatcacactggaataccttgcatctttctgtatcatataaaggattttgcttaacatattcaatggctcttggagaaaaatcacaggcataggcaaagatattcggatcttcttctaaaagtgggaataaacagtttccaaccccacagccagcttcaagcattgttaacttttgatcttcaaactctctacatgatcttagctcctcaaactctctggtggtccagtgtctgtctttgaagaaattagtgctatttcttttgtaaaaaagatcccaatttttctgagcctcttgttccaatttctgctgtttaaaatcagacaccaaagtttggtctcttttcagtttctcctcttcttcagaggtgagaatccttgcctgcagccctttcctttgcaaagaagccatctctgaaactgacggtaacacttaacacagctgaagattctccatcaccaaataatatgaatccacgctaatggatcagatacatttcctgaggtgagtttcacgcctcaaacagcacagggggcccacagccagccccactgggcctcggaggcagaatacgggaagaaccgcgaaacaaccctaaaccaattctgaggaccacgaattcggattatccgggagttcttttgccatggcaccgcc

SEQ ID NO: 13262 - RNA, 1934 nt, Homo sapiens
  source 1..1934: mol_type = other RNA
gctgggattacaggcatgagccaccacgaccggccagctactgtcttttctttgaccctttccagtttctgaagataaagcaggaaataatcttctctgaagatacttgataaaaatttccaaaacaaaacacatgcttccacttcactgataaaaaatttaccgcagtttggcacctaagagtatgacaacagcaataaaaagtaatttcaaagagttaagatttcttcagcaaaatagatgattcacatcttcaagtcctttttgaaatcagttattaatattattctttcctcatttccatctgaatgactgcagcaatagtttttttttttttttttccgagatggagtctcgctctgtcgcccagctggagtgcactggtgcaatcttggctcactgcaatctctgcctcctgggttcaagcgattttcctgccttagcctctcgagtagctgggactacaggcacgcgccaccacacccagctcatttttgtatttttagtagagacagggtttcaccatgttggccaggatggtctcaatctcctgacctcatggtctgcccgccttggcctcccaaagtgctgggattacaggcgtgagccaccgcgcccggccagcaatacagtttttagttactcgacatctttaagcctataactcttaggctatgcatagccccatgtcctaatcaggcattcactgatcccagcaggtctccatctatttgtaccagcctcctctattcctcccaatctcaaggttactcttaaatactagtaaatgcaaaaagaacttgtaaagtggcaaggcatggcctatcaaaagtcagcccaagggcagttttcagccctgcctcacctgggtctagttcagctgacggatgagctgattgatgcgttcaccccgatagccaggtgtgcccatctccttgaggaagcccactctatttttggtagcatgacgggccactgagaggtggaaagggcacaagaaccatgagatctcctggaaatgcttccctgggaaggcaatttcatgaatgaggtcttccaagcaaatgacgccaaacttccccaggtgctcctcaatcactgtattgtctgtcagagggatggtcttattcttgaccttggcttgtccacgtttcaaaatgagttctcggacagacttcagatttggaaatccccaggtcacataaggttccactatacgcagcatttttagattctggggggtgacttttacaaagacaccactaaaaattttctttaggcgaagtcttgcaatggttctctgcaccagtaaactcacgccgtcaatcctttcgatgcgtacaacaaaggccaaggaatgtttatctggcaattccaaggcatgaggtttcacttctagtcgtctgagacgcaccttgtcacgtttctgccgccaggaatcatgtaggaatgattccagtcgcttaaacctgagcccttttcctttcttctgctccttctttgccaaaagtgcctgctttgcctgggtggctttgagggcttgataagccttcctctttttcaggagattttctggaaccaaagggatttttctttgctcttgctccgccatctttctagtggtgcagctactgatcatgcgcaaccccaccacatggggaagacagcacacgctctgtttacttgaccatagagacgtctgttctagctcacgctggaggaccagtcagcgttcacttagccgcagtgagcccttgaggtcccgctaaccccgattcctgccaaaagttgcaccgcttcttagggtttttagagcctgtgttattttcaaaacccagcccttttcttgtaagttacagtttcatcacaagcggcctggctgtggacagcaaagtgcttcccacaatgcacctatggcgtccgctcctagctac

SEQ ID NO: 13263 - RNA, 1245 nt, Homo sapiens
  source 1..1245: mol_type = other RNA
gctgggattacaggcatgagccaccacgaccggccagctactgtcttttctttgaccctttccagtttctgaagataaagcaggaaataatcttctctgaagatacttgataaaaatttccaaaacaaaacacatgcttccacttcactgataaaaaatttaccgcagtttggcacctgggtctagttcagctgacggatgagctgattgatgcgttcaccccgatagccaggtgtgcccatctccttgaggaagcccactctatttttggtagcatgacgggccactgagaggtggaaagggcacaagaaccatgagatctcctggaaatgcttccctgggaaggcaatttcatgaatgaggtcttccaagcaaatgacgccaaacttccccaggtgctcctcaatcactgtattgtctgtcagagggatggtcttattcttgaccttggcttgtccacgtttcaaaatgagttctcggacagacttcagatttggaaatccccaggtcacataaggttccactatacgcagcatttttagattctggggggtgacttttacaaagacaccactaaaaattttctttaggcgaagtcttgcaatggttctctgcaccagtaaactcacgccgtcaatcctttcgatgcgtacaacaaaggccaaggaatgtttatctggcaattccaaggcatgaggtttcacttctagtcgtctgagacgcaccttgtcacgtttctgccgccaggaatcatgtaggaatgattccagtcgcttaaacctgagcccttttcctttcttctgctccttctttgccaaaagtgcctgctttgcctgggtggctttgagggcttgataagccttcctctttttcaggagattttctggaaccaaagggatttttctttgctcttgctccgccatctttctagtggtgcagctactgatcatgcgcaaccccaccacatggggaagacagcacacgctctgtttacttgaccatagagacgtctgttctagctcacgctggaggaccagtcagcgttcacttagccgcagtgagcccttgaggtcccgctaaccccgattcctgccaaaagttgcaccgcttcttagggtttttagagcctgtgttattttcaaaacccagcccttttcttgtaagttacagtttcatcacaagcggcctggctgtggacagcaaagtgcttcccacaatgcacctatggcgtccgctcctagctac

SEQ ID NO: 13264 - RNA, 1361 nt, Homo sapiens
  source 1..1361: mol_type = other RNA
gctgggattacaggcatgagccaccacgaccggccagctactgtcttttctttgaccctttccagtttctgaagataaagcaggaaataatcttctctgaagatacttgataaaaatttccaaaacaaaacacatgcttccacttcactgataaaaaatttaccgcagtttggcacctgggtctagttcagctgacggatgagctgattgatgcgttcaccccgatagccaggtgtgcccatctccttgaggaagcccactctatttttggtagcatgacgggccactgagaggtggaaagggcacaagaaccatgagatctcctggaaatgcttccctgggaaggcaatttcatgaatgaggtcttccaagcaaatgacgccaaacttccccaggtgctcctcaatcactgtattgtctgtcagagggatggtcttattcttgaccttggcttgtccacgtttcaaaatgagttctcggacagacttcagatttggaaatccccaggtcacataaggttccactatacgcagcatttttagattctggggggtgacttttacaaagacaccactaaaaattttctttaggcgaagtcttgcaatggttctctgcaccagtaaactcacgccgtcaatcctttcgatgcgtacaacaaaggccaaggaatgtttatctggcaattccaaggcatgaggtttcacttctagtcgtctgagacgcaccttgtcacgtttctgccgccaggaatcatgtaggaatgattccagtcgcttaaacctgagcccttttcctttcttctgctggtctgtcaaaccgttggggggagctcgtcaataccaaatgtagtccaacacatgcgggataaaactcaccaaataaaaattctaattactttctcttggttccccaccattacctccttctttgccaaaagtgcctgctttgcctgggtggctttgagggcttgataagccttcctctttttcaggagattttctggaaccaaagggatttttctttgctcttgctccgccatctttctagtggtgcagctactgatcatgcgcaaccccaccacatggggaagacagcacacgctctgtttacttgaccatagagacgtctgttctagctcacgctggaggaccagtcagcgttcacttagccgcagtgagcccttgaggtcccgctaaccccgattcctgccaaaagttgcaccgcttcttagggtttttagagcctgtgttattttcaaaacccagcccttttcttgtaagttacagtttcatcacaagcggcctggctgtggacagcaaagtgcttcccacaatgcacctatggcgtccgctcctagctac

SEQ ID NO: 13265 - RNA, 1139 nt, Homo sapiens
  source 1..1139: mol_type = other RNA
gctgggattacaggcatgagccaccacgaccggccagctactgtcttttctttgaccctttccagtttctgaagataaagcaggaaataatcttctctgaagatacttgataaaaatttccaaaacaaaacacatgcttccacttcactgataaaaaatttaccgcagtttggcacctgggtctagttcagctgacggatgagctgattgatgcgttcaccccgatagccaggtgtgcccatctccttgaggaagcccactctatttttggtagcatgacgggccactgagaggtggaaagggcacaagaaccatgagatctcctggaaatgcttccctgggaaggcaatttcatgaatgaggtcttccaagcaaatgacgccaaacttccccaggtgctcctcaatcactgtattgtctgtcagagggatggtcttattcttgaccttggcttgtccacgtttcaaaatgagttctcggacagacttcagatttggaaatccccaggtcacataaggttccactatacgcagcatttttagattctggggggtgacttttacaaagacaccactaaaaattttctttaggcgaagtcttgcaatggttctctgcaccagtaaactcacgccgtcaatcctttcgatgcgtacaacaaaggccaaggaatgtttatctggcaattccaaggcatgaggtttcacttctagtcgtctgagacgcaccttgtcacgtttctgccgccaggaatcatgtaggaatgattccagtcgcttaaacctgagcccttttcctttcttctgtcttgctccgccatctttctagtggtgcagctactgatcatgcgcaaccccaccacatggggaagacagcacacgctctgtttacttgaccatagagacgtctgttctagctcacgctggaggaccagtcagcgttcacttagccgcagtgagcccttgaggtcccgctaaccccgattcctgccaaaagttgcaccgcttcttagggtttttagagcctgtgttattttcaaaacccagcccttttcttgtaagttacagtttcatcacaagcggcctggctgtggacagcaaagtgcttcccacaatgcacctatggcgtccgctcctagctac

SEQ ID NO: 13266 - RNA, 3047 nt, Homo sapiens
  source 1..3047: mol_type = other RNA
gctgggattacaggcatgagccaccacgactggcctgaaggggcttcttcatcttggggagttggtggaccctgtctctgccccttacaaggagtgttgctgaggaaaccagagcaccgagcaaaggcacagggggaaaaggccaagcaatcgtattgacatcattccacacctggagaactgtattagcgagtgcgtggaccacccaatcccctagcaaagcgctgaataggctggtctagccagcaggaacctggctgtcataagaggaggggctttcaccaagttcctcaaattgaataaagagtaattcttttaattcctgaattctacttttcctatctccagtagaagggccctggatctaagcagaaggtattttaaggctagagagtagtagaagtcgatgtttagaaaaggccgcttgttcaaaatctgaaaggcatactcagaggctttctctaaacacctctgttcccatcaaaaaacaagacccaagtctgagaagctgggtaggtttacatggtatcaaaatttaacatctgcagccaaaagccacacctgagctactcagaagccaagaaagtatgtgtatgtaacacagcaccaatcgcatggtccttttctcatttaaagctttctcaggtaagctttaagagctggaggatacatactgaaaaaaaatctcagtatgaaagaaagaaaaccccagtgttaaaatacatgaatacttcctgtgccatctgaatctctggctcaggatcagatcttatgaccacatctctggtgggcataaaatatttacaaccttgttaaaggcacagtggcatttaaaactaaagccttgggaatgtacagtaaaagattaattgtaatcattaacctggcttccattggtagaattcactcttgccggataacatgtgagggagatggtgattcggagcctgctggctggttatcaggcaaggcaagtccttgacccctggagcaggtgaaagtgaagtcacagaaacgtctcggtgttttttttctgctgatttacatctttcctgcttttttgccaacctgagtcgggatgcggaggatattgggggtttcttccatgaccctgacaagcaggttgtcaatgtagtcttccagctcgcggacctggaactccttcttgcttatcgtttccttctgtttgaggaccagctgaatcagctcatcgtgggtcagctgcgcatatgcaaatgcagggtccgaggggctgtatttcttcatcatgacctcattgttcaagttctcactgatgatggtggcagttcccaagctgcagttagcaaccttggtggccattgcattcattggcttcacaggatgaagtcggggcttgacagctctggtctggggagccctcggagaggaaattggaggtctcggttcagacttggactctggctcagcttctggttctgtgatctgcacatcttcaaagaggttcagggagctgccctgtctggagacaacagctgcagtatctttctcagatcttctcacaaggtcttcagcaggccccgatgcgtcctcccccggcttaacccccatcagcatgccttccttctccctccctgggaccgtgagagggttttcaccttcactgcccttagccacatccttcttccccgtcatcagagacagcaaagaggacctcctgctctctggcttcttgctctccttagcttcttttgtggcctctgagtttgcgggggccatgttttccctgaggtccccactgaccagtggggcaggtcggtaggacggcagggtcatagacttcaaggagtccttggtggaagattcggagagctgcctgtcagaagacagcccacctccttcagcaggctccttccaagacccagccgccaggttctctgtagaagagaacaaatgcttctttctgaagcccttgggggatggggaggaggacgggctgctatccttgatctcacccttggcttctggctgctccaggtaaacatggttcccattgatgcagacattagagcgggaaaggacatcattcttagaccgaaggccaccaagaaaggaaagtccttccttcttgggaagggtaaagttgacctggttcagttgcttaagatccgtactcgctgttctcttgtgagacatgacatccgaggccgaggaggactcatcctcattgtcatcttcatcccactgggactgaaagtctccgggacgaagcagcactttttctggctttgaagtcggcaggacagacatggactgggaaagaggcgtcttctgcaaatttgacttggaaagtaaggtcttgatctttgatttctttttcttgtctttaaccacagactcatcatcactgtcgaccgaaggtgtcgtgctagggatgatggcggaggcggtgtctgacccactgtccttattcttccccttgatcttgtccttcagctttccaaatggattccgagacttgtctttcatagaaaggtcaaacatgctggcagtcatgttgtttctcataaactggatgtcaacctcaatttctcctcgctccttgtccttctttcctggtttggatttcaacttataccactgcgtcttcctgcggccctggtcgcggtgcagatcccgcaggtccacctcggcgcggcccaggaacttgtcgaggccgagcagcgcgcggtgcagcacggtgagctgcagggtggcggcggccgcgggtccggaggacagcagcgatggcagctcgaaggtggcctcctcgcgccacacgggcgcgcccaggctgcgctccgacacggaggtggcgtacttctccttgcccacctggatcaccgcgtacgcgtcgctcgtgcccccggggcccttggcccgcaggccccgcgcctgcagcaccgtcacctgcacgtgggttggggaccacacggcccccaggccccggccagccgagaccattagggacatggtgacgataacactccagaagcgaggagaagatcgccgcgactggcggcctccac

SEQ ID NO: 13267 - RNA, 4949 nt, Homo sapiens
  source 1..4949: mol_type = other RNA
gctgggattacaggcatgagccaccacgactggcctgaaggggcttcttcatcttggggagttggtggaccctgtctctgccccttacaaggagtgttgctgaggaaaccagagcaccgagcaaaggcacagggggaaaaggccaagcaatcgtattgacatcattccacacctggagaactgtattagcgagtgcgtggaccacccaatcccctagcaaagcgctgaataggctggtctagccagcaggaacctggctgtcataagaggaggggctttcaccaagttcctcaaattgaataaagagtaattcttttaattcctgaattctacttttcctatctccagtagaagggccctggatctaagcagaaggtattttaaggctagagagtagtagaagtcgatgtttagaaaaggccgcttgttcaaaatctgaaaggcatactcagaggctttctctaaacacctctgttcccatcaaaaaacaagacccaagtctgagaagctgggtaggtttacatggtatcaaaatttaacatctgcagccaaaagccacacctgagctactcagaagccaagaaagtatgtgtatgtaacacagcaccaatcgcatggtccttttctcatttaaagctttctcaggtaagctttaagagctggaggatacatactgaaaaaaaatctcagtatgaaagaaagaaaaccccagtgttaaaatacatgaatacttcctgtgccatctgaatctctggctcaggatcagatcttatgaccacatctctggtgggcataaaatatttacaaccttgttaaaggcacagtggcatttaaaactaaagccttgggaatgtacagtaaaagattaattgtaatcattaacctggcttccattggtagaattcactcttgccggataacatgtgagggagatggtgattcggagcctgctggctggttatcaggcaaggcaagtccttgacccctggagcaggtgaaagtgaagtcacagaaacgtctcggtgttttttttctgctgatttacatctttcctgcttttttgccaacctgagtcgggatgcggaggatattgggggtttcttccatgaccctgacaagcaggttgtcaatgtagtcttccagctcgcggacctggaactccttcttgcttatcgtttccttctgtttgaggaccagctgaatcagctcatcgtgggtcagctgcgcatatgcaaatgcagggtccgaggggctgtatttcttcatcatgacctcattgttcaagttctcactgatgatggtggcagttcccaagctgcagttagcaaccttggtggccattgcattcattggcttcacaggatgaagtctgtgcttggctgacccagttccagcgcctggctgagctgagactggatgtgtctccgagggtgagacccaggcctggaggagtggcttcctcttgccaaaattttcaactctaccagcggagccctctgctgtggcttttttttgagattctgctgtgctggtgtggtgagtgtcagaatgtgcagagctggggaaagagtgtgtgacaggaaagatctcagaaggggaggggctgggtacaggattgtccagggatgtgccaggaggcgggcttggactcccatttcccatcggtttttcttcctcaccaccactggggcctggcagctgtttatccaagcttgagctcttgccaagatgtggtttgtgaattccgaactctgtggtctgctctgaaggagctgtcacagatgcctggggtgcttgcagcctgaaatcacacaggccctcccccagtaccaacctatctgcctcgccactgggcccctttcccctctcaggacaggggactaccaagcccaaggacaaagctcctatgtccagagttgacgactttgctgtctctccatcatcttcaacctgatctccgtcatcttcaacctgatctattctttcatcatccgatgcgacttcaggaatggaaggaaggcttaagttcagatcggccatgattggagatttaaaatctgagaccaactgaaggtcactcaaggggtcagacaataaaccttcgtggtcactggctttgctctgatactgagtcacaagggcatcctctccctccatcctaaagagtggagtgtctttcgctgagcttgcttcactcatggggacttcggagaaactctcctcctgggaggggaggaggaggtgatccgctggggaggctggcgcaccacacgtcgctggcccaggtgtggtcaccgattccctttctgagtcctctgcgtggggagactcaggaggctctccgtcagacgcgtttccagcaacagaccatgcagggttcagctcctggggacaactgctgtgtccttccaccagcaaggcagcccccgccactgcctcttccgtgaagagctgctcagaaaatgacacacgcttcttggttttcttctggtccttgcggaggttcagacccatctcttccagcttccgcatcatggaatcaatggaagggactgatgctcccatgggaagagggggcgccacttcttcagctgcatccctggctttgctctccacaagagacccagcctgactctccaagtctctgtctcctcctgctgcaagctccccaacagggctcacagctccatcactgctgagtgaaagggcaaacggtacttcctgggcttctccagatgatgggctgtagtcttgttttttgcaggggaatctcggaagttcttcctcttgtcgccctgtttcaggctgctctgggagagactcctccaactcaaggctgctggtgttcttctctgtgcctgtctcacgggtcctgcccatcagagaatcttctgtccctttatttgctggaaaggatggctgtttgaaaagtgatcccagggcagaagaaccagaatttggaaccggtgttaaactctcagtttgcaactctgccttagggagcaagggtggtccttcagacttggcctggcccctgtctacgagaggccagctttcaattggagtggatgtggaaatgggagctgctatgggagatgagagagaggagaagacagaaggactctcagaggactgtgtgtctgcaccatgtcccaattcagaggggacagatgcctggccagagctagaaggaagaggaggaagagaggaaggggagtcagtaggggaaggaagcctggctgtgggttgcgcctctggagacacttccagtcggggcttgacagctctggtctggggagccctcggagaggaaattggaggtctcggttcagacttggactctggctcagcttctggttctgtgatctgcacatcttcaaagaggttcagggagctgccctgtctggagacaacagctgcagtatctttctcagatcttctcacaaggtcttcagcaggccccgatgcgtcctcccccggcttaacccccatcagcatgccttccttctccctccctgggaccgtgagagggttttcaccttcactgcccttagccacatccttcttccccgtcatcagagacagcaaagaggacctcctgctctctggcttcttgctctccttagcttcttttgtggcctctgagtttgcgggggccatgttttccctgaggtccccactgaccagtggggcaggtcggtaggacggcagggtcatagacttcaaggagtccttggtggaagattcggagagctgcctgtcagaagacagcccacctccttcagcaggctccttccaagacccagccgccaggttctctgtagaagagaacaaatgcttctttctgaagcccttgggggatggggaggaggacgggctgctatccttgatctcacccttggcttctggctgctccaggtaaacatggttcccattgatgcagacattagagcgggaaaggacatcattcttagaccgaaggccaccaagaaaggaaagtccttccttcttgggaagggtaaagttgacctggttcagttgcttaagatccgtactcgctgttctcttgtgagacatgacatccgaggccgaggaggactcatcctcattgtcatcttcatcccactgggactgaaagtctccgggacgaagcagcactttttctggctttgaagtcggcaggacagacatggactgggaaagaggcgtcttctgcaaatttgacttggaaagtaaggtcttgatctttgatttctttttcttgtctttaaccacagactcatcatcactgtcgaccgaaggtgtcgtgctagggatgatggcggaggcggtgtctgacccactgtccttattcttccccttgatcttgtccttcagctttccaaatggattccgagacttgtctttcatagaaaggtcaaacatgctggcagtcatgttgtttctcataaactggatgtcaacctcaatttctcctcgctccttgtccttctttcctggtttggatttcaacttataccactgcgtcttcctgcggccctggtcgcggtgcagatcccgcaggtccacctcggcgcggcccaggaacttgtcgaggccgagcagcgcgcggtgcagcacggtgagctgcagggtggcggcggccgcgggtccggaggacagcagcgatggcagctcgaaggtggcctcctcgcgccacacgggcgcgcccaggctgcgctccgacacggaggtggcgtacttctccttgcccacctggatcaccgcgtacgcgtcgctcgtgcccccggggcccttggcccgcaggccccgcgcctgcagcaccgtcacctgcacgtgggttggggaccacacggcccccaggccccggccagccgagaccattagggacatggtgacgataacactccagaagcgaggagaagatcgccgcgactggcggcctccac

SEQ ID NO: 13268 - RNA, 1329 nt, Homo sapiens
  source 1..1329: mol_type = other RNA
gctgggattacaggcatgagccaccacgccaggccactgttcactgagatttctgttacttgcagcccaacgcatcttcacagaagagagatgggtcctgctcatggaaccatgtgcttctcatgcccgggcactcatcttgagggaggcagagaaggagaaaaggtctcaaagaatgggccagcattagtgcttgagtaagggggacaggtctgcggcaatccctgtccactccggcaggaaggctgcctctggcttaaagattttgaggaaaggggagtcggggagggtgtaattggccaggtagatggtgtctccgcccgtgaggtatgcggcccagatcccgaacgtcccaatggtcatgatggtgtggttacactgtgtgagtagagcaaaatctttggcaggtgagccctcaatgccatcgccagcaaacaccacatcaccgtgggaggtgtcaatgttctcccgacaccaggccatgccattactggtgaccacgaagatgagggagctgtagcgagctcggaaccagtccagggcctgctgtaggtatcgccggtcggccaccacccccttccacacttttggcatgacatggacatagtcccctcggcgaacatggacccctacaaaggtgcccggccggctcccgttcacctgcaggccccgcaggaacttctgggcctcctcccgcacgtggtcgtgcagggtgaactcctggaggatctcctggcggaggtggtggtagaaggtccaggagcaggggtagccggtgaagcggacgtactcccccgggatgtggcggtattcctcctccatccagtcgttcaggtggtagttctgccaggggatcctgctggccgtggcgctgtgcagcaccggcagggtgattctgaagatgggggccagggtgctgtgcatctgggccgggatgaaggcgggccgcccgttcatcttggccagggcgtacagtgtggcgtactcgcccatctggttccccaggcggcctattgcattgatcgtccacatccccctgagctggctgggtcccagtgcctttgatgttgaggctagcactggtatctgcaccggtaactcccacatggcttgaatcttcgctagccgctgctgaacgtgaaatatagtggaaaccgtaaagacaaagaggatgaagtgggccatgggaaaggagaaaggcatctgaacgaccagcatggctggtcctgctgaaggaaaccgggacagagtggttgggcaggcacctcagtgttccctctgggtctctcttcactcagggccaaagaaacccttccagcatcggtgact

SEQ ID NO: 13269 - RNA, 1339 nt, Homo sapiens
  source 1..1339: mol_type = other RNA
gctgggattacaggcatgagccaccacgccaggccactgttcactgagatttctgttacttgcagcccaacgcatcttcacagaagagagatgggtcctgctcatggaaccatgtgcttctcatgcccgggcactcatcttgagggaggcagagaaggagaaaaggtctcaaagaatgggccagcattagtgcttgagtaagggggacaggtctgcggcaatccctgtccactccggcaggaaggctgcctctggcttaaagattttgaggaaaggggagtcggggagggtgtaattggccaggtagatggtgtctccgcccgtgaggtatgcggcccagatcccgaacgtcccaatggtcatgatggtgtggttacactgtgtgagtagagcaaaatctttggcaggtgagccctcaatgccatcgccagcaaacaccacatcaccgtgggaggtgtcaatgttctcccgacaccaggccatgccattactggtgaccacgaagatgagggagctgtagcgagctcggaaccagtccagggcctgctgtaggtatcgccggtcggccaccacccccttccacacttttggcatgacatggacatagtcccctcggcgaacatggacccctacaaaggtgcccggccggctcccgttcacctgcaggccccgcaggaacttctgggcctcctcccgcacgtggtcgtgcagggtgaactcctggaggatctcctggcggaggtggtggtagaaggtccaggagcaggggtagccggtgaagcggacgtactcccccgggatgtggcggtattcctcctccatccagtcgttcaggtggtagttctgccaggggatcctgctggccgtggcgctgtgcagcaccggcagggtgattctgaagatgggggccagggtgctgtgcatctgggccgggatgaaggcgggccgcccgttcatcttggccagggcgtacagtgtggcgtactcgcccatctggttccccaggcggcctattgcattgatcgtccacatccccctgagctggctgggtcccagtgcctttgatgttgaggctagcactggtatctgcaccggtaactcccacatggcttgaatcttcgctagccgctgctgaacgtgaaatatagtggaaaccgtaaagacaaagaggatgaagtgggccatgggaaaggagaaaggcatctgaacgaccagcatggcttctctcacctggtcctgctgaaggaaaccgggacagagtggttgggcaggcacctcagtgttccctctgggtctctcttcactcagggccaaagaaacccttccagcatcggtgact

SEQ ID NO: 13270 - RNA, 3430 nt, Homo sapiens
  source 1..3430: mol_type = other RNA
gctgggattacaggcatgagccaccacgccaggcctgccttctttattcttaatttctttctaatgacagttatgccttttcaaataactttccactgtgatttttctcaatgatttccacaatgacaaaacgtgctaagtaaactattcttaattttttgtggcagaagtatataccttgggagtattactattgttaaaaaataattgatagttttttctacttacaaaccagggttgagttggtgacagtttttaaagaaattgacttttcacatagtacaagttttcttaaggtgagttacctgataaacacacttggcctttgtgatttccctttgaagaaaaatatagtcagatcaacacacacacacacaaatatacagataatactaatattgattatttccatttgtttaaaatgtatctccatattgcaatagaattaataagataattttgtgtctcttctcttgcaacttgtacaaaatcctgaaaaagaaactaaaaactgattctgaacaagtcccatatgcttgaaaattttgagttttgcttatttaacagtagataacttttagcaaatcaattcaaatatgcaaagaaaacaaaggattgctttaaacaagttattaacaaaggtataagtataaaggcaagttgctcctccttgaataaatgtatcttggctttggtaagtctctgtgtcacgtccacagcagatagaagtatcagaatgtcagttctgtttgttaatggcaagattccaattttagaattttgacctcgtctgtactcctttatacctaattttaaagaaatatgccattattatctggccccagactacatattttttaaatttaagtttttattgatgtatttcttgcaatatacttgggaaggatgccaaaatgttaacattgacatcaataaaaaataatataaatgctttaaatgaaagagtgaaagaaaagaagaaagataaaccatttcatgtctgtagccatattattgtcatcattaaagtagagatacagtaaaagtaagaagagataaaagaatggcacacacatgtatccaatcatatttatctcaaaaatatgccaaatttccatttaaaatgtcatggcatttattatttttaaaccattcaaaatttcttcttactgaggttcttgaagtgggctcctataatttgagtagttgaagacattatttgcctaatatgaagttttcagttattagtgtagttagaatgtaatttctcttaatttgcactaaaacttataaagtttgatacttttttgcaacctaaaactaggctttatgtttattgtgatgtttgggatccttaaataatttcttattactaaaatatctttatacattgggaatcatttaaatatgtattaggctaaaattggtactatgaaatcagtgtcatactttttacaggacacattataactgaatagagtttcaaagaaaggagtaaatagttattagaactttactgcatattcctgccaataatattgcaaagaaatgttcttgtgggaattgaacaagatggacttttctgttcagctactcccccattccaatttctgaaaaaaaaaacaaaaaagatgttccttaattatattaacctttcatctgagacagggtgtggtggcccacacctgtaatcccagcactttgggaagctgaggcgagcagatcacttgaggtcaggagtttgagaccagcctggccaacatggtgaaaccctttctctactaaaaatacaaaaattcaccaggcctggtggtgtgctgtggtcccagctactcgggaggctgaggcaggagaatcgcttgaacccgggaggtagaggttgcagtgagccaagatggcaccactacactctggcctgggcaacagagcaagactccatctaaaaaaaaaacaaaaaaaaaaaattttcatctgagagcaggtaaaccattgcaaagtcatgccccaatcgttgtacaatatccatttcctacagttgacataacaaattccaaaaaacaggtcacctaaaacaacagaaatttactctctcacagtttcggggctaaaagtctgaaatcaaggtaccatcagtgctgtgtttttgctgacagctttggggagaatcctttcttgcctcttctagcttctggtgatacttgccagcaatccttggtatgtgtgttggtttgtagatgctccactccaaccacgtggtcaccttctctctgtgtgtcttcaggtagtcttcctctgtgcccctctcatgtccacatttctcccttcacttctggattgcgaggagtataggtcatattaaggcttaatgttccaattctatttttaaattatccgtttataaattaagccactttaagcctgatgctcatcctcgtagttctctttacagctctctctcctctttaagtaatcagtttcttctctttctcttttatgtcaaaagccttcctgagataatgaaggtcaattctttctccgttagggatatctcaaatctctccaagggcttcttcaaatctctccgagggcttcatttcctatgcagagtgtgctatccttaatcacttgaagaatcttttgacagagccttttgtaacgtttttgtagtttcctgctttacagaatttgcaggcttagtaaaagcatggatagaaccagagccactgcaagcagagccaaaggtggaaggatagtgaggcagatccttgacctcaatgctccctaaaaattataaacagcattctctttcattcctggtaagtttccacttccttttgcattttctcataaagaaatccatgtatccttacagtaaattttcttgtttagctttagctagtcatctagatttctggtttttgcagccaaacaacccctaagagatctatgtcttagtggggccaatttcaatcccatttaattcaattcaaccgatgtttattgaatacctattgtgtctcttatacccaataattggggttgagtcttgaatctggcctatgactggaatctatgaaagattcaaagggaaaaataggcataggttatgatgagctataaaaaaagaaacgagacagaacataatgtagagttcttagctctccccacccagatttatgttctgagttttctttaacattctgtccaatcgagtgcgagtgggctgagacgtgggtggcagagctgagacacggcccctctaactgtctcatgtacaaacttgaggggtaagaggaagtttgacacaggaaataacagccagcagccgggctctctgacgaacactacccagtgaagccttttaattaggcaagatcatttttgttaaatctgctcagaaaatactgccttaatctctgaagataataaa

SEQ ID NO: 13271 - RNA, 1190 nt, Homo sapiens
  source 1..1190: mol_type = other RNA
gctgggattacaggcatgagccaccacgcccagatagaagctccttgcaaatccatccacctggttggagagctgggcctttcatctgcactcttagtcactgcaccctcatcatcgtcaggcagcgtgatacagaaagccctgtctggtcttcagtagctgaagggaaggttctcagctactctccaagccctcgccaatcagggtctgcagtcccagctctgggcagcaggtaaacgtctttcccggagcagctctctggggcacccaggtcggacttgcagagccccagccaggctgggcctccgctaatattcttgggtcgcagcctgggattcctgcaggttccgacaataggctggaccatcctcttgtaggaggcggggttcaaagtaaccccaagcgcggggaggggagctctggcaggggcgtccatgtgtccaggactctaggcctgggggttgggggtgacatcggcacgcccccctccccaggcctgatgcaggaggaaggaggtgtgggacagggaaagaggaccgcgtttggagtgcacacggcacattacataattattctattttaatataacaagcctggatggtagctatgactaatctctagttaataggtgaggaaaccgaggccgggagaggttaaggagttaggggtgggtggagggccggtgaggggtggcggctgtgacgggcagagcgtgaggccaggccccttggaaactccccctcagcctccgtgtccacctaagctaccagtgcggggcctgcggctgcggcccgtgggctgtgcaggctcagagccccgggacccgcaggccccaggcctgcatgtgtgagcgcaggaggcggggaggcagacaccgcatttccacaggaccctgcgggatcagggcgcagaccgggcggcggggtccctcggggcctcccctggccccagcacctcccgcccgccgccgcggggttcttccagtccatgccaacctggctcgagcaggacaaggtgatcgaggctcagcggcccctggtcccccagccccacgcccggcccgtggccatggcaaccgctgcgctgtggctccctcgccgggcaacggagagaggggaagggaacgcgcccggccgcgccgccggctgcgaattcctcaggccttccatcagccccgccggccccgacgg

SEQ ID NO: 13272 - RNA, 2370 nt, Homo sapiens
  source 1..2370: mol_type = other RNA
gctgggattacaggcatgagccaccacgcccagccaactcacctgtttaaatggtcaacttcctcctctctgaggaaagaataaaaaccaggaaagagaaaccattggcgatgcttctttctcagccctttcctgttagtgactcagcacaggtatctccttcactatccccagctcctgaggtgcaacaagcagcccttagtgacaactgaatggttatcattgtcatcatcatcaatccatctcggttctgatatctgcaggctggtcattcagatcagatactcgctctcggcatccaaagcgctggtggcttcatccaggatgaggactggggggttccgcaccagagcccgggccatggccacccgctgcttctggccacctgacagctgggcgcccttctcccctgtctctgtgctgtagccgtcctggagttccatgatgaagccgtgggcattggccttctgtgcggcctccaccaccatctcgaaaggcacagtgggcaggccgtaggagatgttatccgtgatggagcgggcgaacagcacgggctcctggctcaccagggagatcacacggtgcaagtacttgtggtcgtaggcgctgatgggcttgccgtccagcagcacccggcccccctccagggggtagaagttctccaggatgttgacacaggagctcttcccactgcccgagggccccaccagggccgtcaccttgccgggggacaggctgaaggagacattctccatacaatctcccaggacaaactcgtagatgatgaaggcgatgaggttgccgctggtcatctggcctgagatgacaaggtggcccccgtagtagaggatgctgacctggaccaccagcagtgtgagcccgctgccccagacgtagtacatgtaggcagctgcctccttcctgttcagcttgtacacctgctgcagcttccgcaggtacacctctgcctcctcctcctcattggcgaagctccggacagtcttcatggcactgatggtctcctccgccgtgttgctcgctctggccagggcattctggacctctttggagagcctcttgtagtacttgccgtagatgttggacaccatcatgatgatggggaagcccatgaaggtgaccaaggagagctgccatgagaggctgaacatgaagaccaccacgcccgtgaccttgactgtgttccgcaggaagacattgatgttctgggagaccaggtcgctgaccatggtggtgtccgaggtcaggcgggagatgaggtcccctgtgcggttctcatcaaagaagcttgtctcctgggacaccagtgagcggaagagacagtttcgaaggcgaatgttcagtctggcaaatatgagggtaaaaatgccgccccgaatacctgccaatggccagcaggcacacgatgacgacagccgtgctgaactgatccatgcttttctggatgacgatgccatcaatggcgcggcccgtgtagtagggcaggaaggtctctcccagagctgccacgatgaggaagaaggaggcggccacgaggaaggccacgtcgggcttggtgtaggagagcagcttctgcagcgtggccccagacgcctgctcgggcggtggccggccgctcccagggaagccctcagcctcggtggccgcccctggctccagggcctgggtgcctggccgcacggtggacagcagccaccagagcaggaaggatgcgccgagtgaaatgtacgtccacacgaacagggcccaaaaccaggggtcccggatgggcctgcgcacctctgagaagagcagcagcttcaccatggcatagatgcccacgaagaggcacacgagggtgatgaccagccacgaggcccgcagccgccggggccccagcgcactgttcttggccacaccaatggtggctcccagcagcaggcagctgcggtacaggcaggctgcccagagatccagcaccgagtcaaagatgttgaagtggcggatgtcctccaggaggctgcggtccaggtggctgaagacatagatggccgtggtcacgcagatgtccacactcatgaaggccaaagtcaccaccaccgccttccacagccgcatcctgctggttggaggtgggcgggtgctgaaggccaggttgtagctcacgggggcaaggccatcatcatccacagggcgaggccaggcctgttacctggcaccaggtgagctctgggagggggcgcgcagcaggctcgggtctggggtgcagtttccgcgctgctcattgaagactgcgccggacgcggtcctcgctccgctcttcccgctgctcctccccgcctcccacccgcgctgcgccgctgcaaggtcgga

SEQ ID NO: 13273 - RNA, 2393 nt, Homo sapiens
  source 1..2393: mol_type = other RNA
gctgggattacaggcatgagccaccacgcccagccaactcacctgtttaaatggtcaacttcctcctctctgaggaaagaataaaaaccaggaaagagaaaccattggcgatgcttctttctcagccctttcctgttagtgactcagcacaggtatctccttcactatccccagctcctgaggtgcaacaagcagcccttagtgacaactgaatggttatcattgtcatcatcatcaatccatctcggttctgatatctgcaggctggtcattcagatcagatactcgctctcggcatccaaagcgctggtggcttcatccaggatgaggactggggggttccgcaccagagcccgggccatggccacccgctgcttctggccacctgacagctgggcgcccttctcccctgtctctgtgctgtagccgtcctggagttccatgatgaagccgtgggcattggccttctgtgcggcctccaccaccatctcgaaaggcacagtgggcaggccgtaggagatgttatccgtgatggagcgggcgaacagcacgggctcctggctcaccagggagatcacacggtgcaagtacttgtggtcgtaggcgctgatgggcttgccgtccagcagcacccggcccccctccagggggtagaagttctccaggatgttgacacaggagctcttcccactgcccgagggccccaccagggccgtcaccttgccgggggacaggctgaaggagacattctccatacaatctcccaggacaaactcgtagatgatgaaggcgatgaggttgccgctggtcatctggcctgagatgacaaggtggcccccgtagtagaggatgctgacctggaccaccagcagtgtgagcccgctgccccagacgtagtacatgtaggcagctgcctccttcctgttcagcttgtacacctgctgcagcttccgcaggtacacctctgcctcctcctcctcattggcgaagctccggacagtcttcatggcactgatggtctcctccgccgtgttgctcgctctggccagggcattctggacctctttggagagcctcttgtagtacttgccgtagatgttggacaccatcatgatgatggggaagcccatgaaggtgaccaaggagagctgccatgagaggctgaacatgaagaccaccacgcccgtgaccttgactgtgttccgcaggaagacattgatgttctgggagaccaggtcgctgaccatggtggtgtccgaggtcaggcgggagatgaggtcccctgtgcggttctcatcaaagaagcttgtctcctgggacaccagtgagcggaagagacagtttcgaaggcgaatgttcagtctggcaaatatgagggtaaaaatgccgccccgaatacctgcggcaaatgagctgccaatggccagcaggcacacgatgacgacagccgtgctgaactgatccatgcttttctggatgacgatgccatcaatggcgcggcccgtgtagtagggcaggaaggtctctcccagagctgccacgatgaggaagaaggaggcggccacgaggaaggccacgtcgggcttggtgtaggagagcagcttctgcagcgtggccccagacgcctgctcgggcggtggccggccgctcccagggaagccctcagcctcggtggccgcccctggctccagggcctgggtgcctggccgcacggtggacagcagccaccagagcaggaaggatgcgccgagtgaaatgtacgtccacacgaacagggcccaaaaccaggggtcccggatgggcctgcgcacctctgagaagagcagcagcttcaccatggcatagatgcccacgaagaggcacacgagggtgatgaccagccacgaggcccgcagccgccggggccccagcgcactgttcttggccacaccaatggtggctcccagcagcaggcagctgcggtacaggcaggctgcccagagatccagcaccgagtcaaagatgttgaagtggcggatgtcctccaggaggctgcggtccaggtggctgaagacatagatggccgtggtcacgcagatgtccacactcatgaaggccaaagtcaccaccaccgccttccacagccgcatcctgctggttggaggtgggcgggtgctgaaggccaggttgtagctcacgggggcaaggccatcatcatccacagggcgaggccaggcctgttacctggcaccaggtgagctctgggagggggcgcgcagcaggctcgggtctggggtgcagtttccgcgctgctcattgaagactgcgccggacgcggtcctcgctccgctcttcccgctgctcctccccgcctcccacccgcgctgcgccgctgcaaggtcggagctgagact

SEQ ID NO: 13274 - RNA, 2568 nt, Homo sapiens
  source 1..2568: mol_type = other RNA
gctgggattacaggcatgagccaccacgcccagccaactcacctgtttaaatggtcaacttcctcctctctgaggaaagaataaaaaccaggaaagagaaaccattggcgatgcttctttctcagccctttcctgttagtgactcagcacaggtatctccttcactatccccagctcctgaggtgcaacaagcagcccttagtgacaactgaatggttatcattgtcatcatcatcaatccatctcggttctgatatctgcaggctggtcattcagatcagatactcgctctcggcatccaaagcgctggtggcttcatccaggatgaggactggggggttccgcaccagagcccgggccatggccacccgctgcttctggccacctgacagctgggcgcccttctcccctgtctctgtgctgtagccgtcctggagttccatgatgaagccgtgggcattggccttctgtgcggcctccaccaccatctcgaaaggcacagtgggcaggccgtaggagatgttatccgtgatggagcgggcgaacagcacgggctcctggctcaccagggagatcacacggtgcaagtacttgtggtcgtaggcgctgatgggcttgccgtccagcagcacccggcccccctccagggggtagaagttctccaggatgttgacacaggagctcttcccactgcccgagggccccaccagggccgtcaccttgccgggggacaggctgaaggagacattctgcaggacctgggtgtggggccgagtgcggtaggtgaaggtcacattctcaaagtccacccggccctccaggtggtcgggggccaagctgccatcgtgcaccatggtcggctgccggtcgatgaactcgaacaccttctcagcagcccccactccctgcatcaggccactgtagacggagcccacggactccatacaatctcccaggacaaactcgtagatgatgaaggcgatgaggttgccgctggtcatctggcctgagatgacaaggtggcccccgtagtagaggatgctgacctggaccaccagcagtgtgagcccgctgccccagacgtagtacatgtaggcagctgcctccttcctgttcagcttgtacacctgctgcagcttccgcaggtacacctctgcctcctcctcctcattggcgaagctccggacagtcttcatggcactgatggtctcctccgccgtgttgctcgctctggccagggcattctggacctctttggagagcctcttgtagtacttgccgtagatgttggacaccatcatgatgatggggaagcccatgaaggtgaccaaggagagctgccatgagaggctgaacatgaagaccaccacgcccgtgaccttgactgtgttccgcaggaagacattgatgttctgggagaccaggtcgctgaccatggtggtgtccgaggtcaggcgggagatgaggtcccctgtgcggttctcatcaaagaagcttgtctcctgggacaccagtgagcggaagagacagtttcgaaggcgaatgttcagtctggcaaatatgagggtaaaaatgccgccccgaatacctgccaatggccagcaggcacacgatgacgacagccgtgctgaactgatccatgcttttctggatgacgatgccatcaatggcgcggcccgtgtagtagggcaggaaggtctctcccagagctgccacgatgaggaagaaggaggcggccacgaggaaggccacgtcgggcttggtgtaggagagcagcttctgcagcgtggccccagacgcctgctcgggcggtggccggccgctcccagggaagccctcagcctcggtggccgcccctggctccagggcctgggtgcctggccgcacggtggacagcagccaccagagcaggaaggatgcgccgagtgaaatgtacgtccacacgaacagggcccaaaaccaggggtcccggatgggcctgcgcacctctgagaagagcagcagcttcaccatggcatagatgcccacgaagaggcacacgagggtgatgaccagccacgaggcccgcagccgccggggccccagcgcactgttcttggccacaccaatggtggctcccagcagcaggcagctgcggtacaggcaggctgcccagagatccagcaccgagtcaaagatgttgaagtggcggatgtcctccaggaggctgcggtccaggtggctgaagacatagatggccgtggtcacgcagatgtccacactcatgaaggccaaagtcaccaccaccgccttccacagccgcatcctgctggttggaggtgggcgggtgctgaaggccaggttgtagctcacgggggcaaggccatcatcatccacagggcgaggccaggcctgttacctggcaccaggtgagctctgggagggggcgcgcagcaggctcgggtctggggtgcagtttccgcgctgctcattgaagactgcgccggacgcggtcctcgctccgctcttcccgctgctcctccccgcctcccacccgcgctgcgccgctgcaaggtcggagctgagact

SEQ ID NO: 13275 - RNA, 2582 nt, Homo sapiens
  source 1..2582: mol_type = other RNA
gctgggattacaggcatgagccaccacgcccagccaactcacctgtttaaatggtcaacttcctcctctctgaggaaagaataaaaaccaggaaagagaaaccattggcgatgcttctttctcagccctttcctgttagtgactcagcacaggtatctccttcactatccccagctcctgaggtgcaacaagcagcccttagtgacaactgaatggttatcattgtcatcatcatcaatccatctcggttctgatatctgcaggctggtcattcagatcagatactcgctctcggcatccaaagcgctggtggcttcatccaggatgaggactggggggttccgcaccagagcccgggccatggccacccgctgcttctggccacctgacagctgggcgcccttctcccctgtctctgtgctgtagccgtcctggagttccatgatgaagccgtgggcattggccttctgtgcggcctccaccaccatctcgaaaggcacagtgggcaggccgtaggagatgttatccgtgatggagcgggcgaacagcacgggctcctggctcaccagggagatcacacggtgcaagtacttgtggtcgtaggcgctgatgggcttgccgtccagcagcacccggcccccctccagggggtagaagttctccaggatgttgacacaggagctcttcccactgcccgagggccccaccagggccgtcaccttgccgggggacaggctgaaggagacattctgcaggacctgggtgtggggccgagtgcggtaggtgaaggtcacattctcaaagtccacccggccctccaggtggtcgggggccaagctgccatcgtgcaccatggtcggctgccggtcgatgaactcgaacaccttctcagcagcccccactccctgcatcaggccactgtagacggagcccacggactccatacaatctcccaggacaaactcgtagatgatgaaggcgatgaggttgccgctggtcatctggcctgagatgacaaggtggcccccgtagtagaggatgctgacctggaccaccagcagtgtgagcccgctgccccagacgtagtacatgtaggcagctgcctccttcctgttcagcttgtacacctgctgcagcttccgcaggtacacctctgcctcctcctcctcattggcgaagctccggacagtcttcatggcactgatggtctcctccgccgtgttgctcgctctggccagggcattctggacctctttggagagcctcttgtagtacttgccgtagatgttggacaccatcatgatgatggggaagcccatgaaggtgaccaaggagagctgccatgagaggctgaacatgaagaccaccacgcccgtgaccttgactgtgttccgcaggaagacattgatgttctgggagaccaggtcgctgaccatggtggtgtccgaggtcaggcgggagatgaggtcccctgtgcggttctcatcaaagaagcttgtctcctgggacaccagtgagcggaagagacagtttcgaaggcgaatgttcagtctggcaaatatgagggtaaaaatgccgccccgaatacctgcggcaaatgagctgccaatggccagcaggcacacgatgacgacagccgtgctgaactgatccatgcttttctggatgacgatgccatcaatggcgcggcccgtgtagtagggcaggaaggtctctcccagagctgccacgatgaggaagaaggaggcggccacgaggaaggccacgtcgggcttggtgtaggagagcagcttctgcagcgtggccccagacgcctgctcgggcggtggccggccgctcccagggaagccctcagcctcggtggccgcccctggctccagggcctgggtgcctggccgcacggtggacagcagccaccagagcaggaaggatgcgccgagtgaaatgtacgtccacacgaacagggcccaaaaccaggggtcccggatgggcctgcgcacctctgagaagagcagcagcttcaccatggcatagatgcccacgaagaggcacacgagggtgatgaccagccacgaggcccgcagccgccggggccccagcgcactgttcttggccacaccaatggtggctcccagcagcaggcagctgcggtacaggcaggctgcccagagatccagcaccgagtcaaagatgttgaagtggcggatgtcctccaggaggctgcggtccaggtggctgaagacatagatggccgtggtcacgcagatgtccacactcatgaaggccaaagtcaccaccaccgccttccacagccgcatcctgctggttggaggtgggcgggtgctgaaggccaggttgtagctcacgggggcaaggccatcatcatccacagggcgaggccaggcctgttacctggcaccaggtgagctctgggagggggcgcgcagcaggctcgggtctggggtgcagtttccgcgctgctcattgaagactgcgccggacgcggtcctcgctccgctcttcccgctgctcctccccgcctcccacccgcgctgcgccgctgcaaggtcggagctgagact

SEQ ID NO: 13276 - RNA, 2066 nt, Homo sapiens
  source 1..2066: mol_type = other RNA
gctgggattacaggcatgagccaccacgcccagccaactgccacccctttttatccctctgtatagacatcctagagttgccaatgtctgtgatgttgaaagaaagaatgcttcttattgtctcttcttttcagtgttggtatgatttgggtttcttgtttgtgtgttctgttcattatatggtcaaacgaacaaatataaatgatgtactgtataagcatcttggaacggtgagagttgacggagacatacttcaactttcttaaattcttccagcatagcgtccaacttggtgtcattgaaaacaaagtgcaaggggtggttataaaatttggtgatggttttcaggggggtacagtcatcgggatccacgaaggccaagtctttgacaaacagcaggtccacgatattggagcgctccccttcaaacactggaatgcgggtgtagccgctctccatgatctcagacatggtgttgaagtccaggatggcttcgccggtgatcatgaagcagtcccggagtggggtcatcacgtcctccaccgtcttggtgcggagctccagcgccccttggatgatgttcagctcctccttaacgaggtcgttgtagggatcggtgacccggagcatctccagcagtttttcccggttatagacggtgcctatctcctggcccaggacgcagtccagcagcttgctgaccgggtaggaagcggggaaggtcatcatcatgaaaaacttggtgaggaagatggtgttggcccccacagccaggccatgccgggagcagatggcctggggcacgatctctccgaagatgacgataccgatggtggagactaccacggccacgaggcccgagccggcgatgtcgtcgagcaggatggtgagcgtggtgttgaccagcacgttgcccagcagcagtgagcacagcaggtagttgccctgcctgcgcaccggctcgatgcgcttggcgtaattcttctccttctccgtgccgcagttctgcacgatgcgcagctccatcgggtccagggccatgagccccaggttgaggccgctgaacatgcccgacaggcacagcagcagcgaaatgaagatcacctgcagccagaagggcagcaggaacttcttctcttcgcctacgatcatcttggtgtcctcgccgtcgtggtaaatccaggtggtctcggcccacgggggcggcgggagcccggccacccccgagccacccttgcccccgacggcgccacccgtggaccccgagccgccggcgcccagggcgggcgtggagagcgacgtgcacaggtaataggacttgctcttctccatcttgcgtagcggtttgatctcgatctcgatgatgcccgaggtgcggcggttgagaatgatgtggggcaagatgatgatgtctgaggtgcggatgccgcatcgctgggggccgctgtccggctctggcggcgcggggccccccagcccgcgctcccccgggctgtggcgccgccgctcgtgctcggtgaaggcgatgcgggaccacgtctcgttattgatgttctgcccgtacacccgcagcttgacccgggtccgttcgctcacccgcagcgcccccccttccatgaacgacacgtcgttcgtgtcctccagtcgcagcccgatgatcaccgtctcctcattctcgcccaccgctgcgcagccgcccgcaccgcagcagcagctcagcaggagcagcggcagcagccgccccgcagccgcctgcaggatcccccggccgcgagcgctgaggctgcggcgcgccgccatcttccaagtgggcagtgcggcggctgcctgcccgcccgccatctttactttgggttcacaagcgccacagccaatcatagggtggctgctccagctgcggcttcatcctttcaacccggcggcgcgagcgcaggtaccggcccctgggcgagactgcaacggagcgtccgcggccagtgctcagcagttcgcctccctgactgacactgactccacctcagccagctgaggaaccccgaggctcgcgggagggaaagagggaggga

SEQ ID NO: 13277 - RNA, 1976 nt, Homo sapiens
  source 1..1976: mol_type = other RNA
gctgggattacaggcatgagccaccacgcccagccaactgccacccctttttatccctctgtatagacatcctagagttgccaatgtctgtgatgttgaaagaaagaatgcttcttattgtctcttcttttcagtgttggtatgatttgggtttcttgtttgtgtgttctttcttaaattcttccagcatagcgtccaacttggtgtcattgaaaacaaagtgcaaggggtggttataaaatttggtgatggttttcaggggggtacagtcatcgggatccacgaaggccaagtctttgacaaacagcaggtccacgatattggagcgctccccttcaaacactggaatgcgggtgtagccgctctccatgatctcagacatggtgttgaagtccaggatggcttcgccggtgatcatgaagcagtcccggagtggggtcatcacgtcctccaccgtcttggtgcggagctccagcgccccttggatgatgttcagctcctccttaacgaggtcgttgtagggatcggtgacccggagcatctccagcagtttttcccggttatagacggtgcctatctcctggcccaggacgcagtccagcagcttgctgaccgggtaggaagcggggaaggtcatcatcatgaaaaacttggtgaggaagatggtgttggcccccacagccaggccatgccgggagcagatggcctggggcacgatctctccgaagatgacgataccgatggtggagactaccacggccacgaggcccgagccggcgatgtcgtcgagcaggatggtgagcgtggtgttgaccagcacgttgcccagcagcagtgagcacagcaggtagttgccctgcctgcgcaccggctcgatgcgcttggcgtaattcttctccttctccgtgccgcagttctgcacgatgcgcagctccatcgggtccagggccatgagccccaggttgaggccgctgaacatgcccgacaggcacagcagcagcgaaatgaagatcacctgcagccagaagggcagcaggaacttcttctcttcgcctacgatcatcttggtgtcctcgccgtcgtggtaaatccaggtggtctcggcccacgggggcggcgggagcccggccacccccgagccacccttgcccccgacggcgccacccgtggaccccgagccgccggcgcccagggcgggcgtggagagcgacgtgcacaggtaataggacttgctcttctccatcttgcgtagcggtttgatctcgatctcgatgatgcccgaggtgcggcggttgagaatgatgtggggcaagatgatgatgtctgaggtgcggatgccgcatcgctgggggccgctgtccggctctggcggcgcggggccccccagcccgcgctcccccgggctgtggcgccgccgctcgtgctcggtgaaggcgatgcgggaccacgtctcgttattgatgttctgcccgtacacccgcagcttgacccgggtccgttcgctcacccgcagcgcccccccttccatgaacgacacgtcgttcgtgtcctccagtcgcagcccgatgatcaccgtctcctcattctcgcccaccgctgcgcagccgcccgcaccgcagcagcagctcagcaggagcagcggcagcagccgccccgcagccgcctgcaggatcccccggccgcgagcgctgaggctgcggcgcgccgccatcttccaagtgggcagtgcggcggctgcctgcccgcccgccatctttactttgggttcacaagcgccacagccaatcatagggtggctgctccagctgcggcttcatcctttcaacccggcggcgcgagcgcaggtaccggcccctgggcgagactgcaacggagcgtccgcggccagtgctcagcagttcgcctccctgactgacactgactccacctcagccagctgaggaaccccgaggctcgcgggagggaaagagggaggg

SEQ ID NO: 13278 - RNA, 2065 nt, Homo sapiens
  source 1..2065: mol_type = other RNA
gctgggattacaggcatgagccaccacgcccagccaactgccacccctttttatccctctgtatagacatcctagagttgccaatgtctgtgatgttgaaagaaagaatgcttcttattgtctcttcttttcagtgttggtatgatttgggtttcttgtttgtgtgtttatttgttttttcaatgatgctgctaccttcatctctgaataacttgggaccagaagaccagcctgctggagcaggaagaactccaatctttcttaaattcttccagcatagcgtccaacttggtgtcattgaaaacaaagtgcaaggggtggttataaaatttggtgatggttttcaggggggtacagtcatcgggatccacgaaggccaagtctttgacaaacagcaggtccacgatattggagcgctccccttcaaacactggaatgcgggtgtagccgctctccatgatctcagacatggtgttgaagtccaggatggcttcgccggtgatcatgaagcagtcccggagtggggtcatcacgtcctccaccgtcttggtgcggagctccagcgccccttggatgatgttcagctcctccttaacgaggtcgttgtagggatcggtgacccggagcatctccagcagtttttcccggttatagacggtgcctatctcctggcccaggacgcagtccagcagcttgctgaccgggtaggaagcggggaaggtcatcatcatgaaaaacttggtgaggaagatggtgttggcccccacagccaggccatgccgggagcagatggcctggggcacgatctctccgaagatgacgataccgatggtggagactaccacggccacgaggcccgagccggcgatgtcgtcgagcaggatggtgagcgtggtgttgaccagcacgttgcccagcagcagtgagcacagcaggtagttgccctgcctgcgcaccggctcgatgcgcttggcgtaattcttctccttctccgtgccgcagttctgcacgatgcgcagctccatcgggtccagggccatgagccccaggttgaggccgctgaacatgcccgacaggcacagcagcagcgaaatgaagatcacctgcagccagaagggcagcaggaacttcttctcttcgcctacgatcatcttggtgtcctcgccgtcgtggtaaatccaggtggtctcggcccacgggggcggcgggagcccggccacccccgagccacccttgcccccgacggcgccacccgtggaccccgagccgccggcgcccagggcgggcgtggagagcgacgtgcacaggtaataggacttgctcttctccatcttgcgtagcggtttgatctcgatctcgatgatgcccgaggtgcggcggttgagaatgatgtggggcaagatgatgatgtctgaggtgcggatgccgcatcgctgggggccgctgtccggctctggcggcgcggggccccccagcccgcgctcccccgggctgtggcgccgccgctcgtgctcggtgaaggcgatgcgggaccacgtctcgttattgatgttctgcccgtacacccgcagcttgacccgggtccgttcgctcacccgcagcgcccccccttccatgaacgacacgtcgttcgtgtcctccagtcgcagcccgatgatcaccgtctcctcattctcgcccaccgctgcgcagccgcccgcaccgcagcagcagctcagcaggagcagcggcagcagccgccccgcagccgcctgcaggatcccccggccgcgagcgctgaggctgcggcgcgccgccatcttccaagtgggcagtgcggcggctgcctgcccgcccgccatctttactttgggttcacaagcgccacagccaatcatagggtggctgctccagctgcggcttcatcctttcaacccggcggcgcgagcgcaggtaccggcccctgggcgagactgcaacggagcgtccgcggccagtgctcagcagttcgcctccctgactgacactgactccacctcagccagctgaggaaccccgaggctcgcgggagggaaagagggaggga

SEQ ID NO: 13279 - RNA, 692 nt, Homo sapiens
  source 1..692: mol_type = other RNA
gctgggattacaggcatgagccaccacgcccagccagattacaaaatactttgacatcttttctctacagccctcaaaaggaggcagggcaagcacaattaaatcccattacaaatggggtgactgaagctccattcatggcttgcccagggtcacacaaagaatgaatagcagagccctgagcctgtgtgcttccctctgtgccaggctgctttacccaggcatgggtgcaccttgtgcatgggacatttctcctttgttgtgtcctgagtaccttaagccactcagatattgctcaggtggagtgaggggaaaatgttttcaggttgtattagtcaaaacaaaataccacacactgggcgactttaaaatcatacatttatccctcacagttctggaggcttggaagtccaagttcaaggtggcagctggacgggttcccggtgagggctctcttcctggtttgcagacagccaccttctcttcgcatcctcactctggtaaggggaccacacgctgcagccagcgagacagtggcatgttcttgttacaactcgatctaactcccccagaagaggaggcagggaaggcggacaaaaccattgaacacgagctgcccaactccgccttgcttccccattcctggcgaccactgcttctgtctctgtgaattttgactattctaggcactt

SEQ ID NO: 13280 - RNA, 705 nt, Homo sapiens
  source 1..705: mol_type = other RNA
gctgggattacaggcatgagccaccacgcccagccagattacaaaatactttgacatcttttctctacagccctcaaaaggaggcagggcaagcacaattaaatcccattacaaatggggtgactgaagctccattcatggcttgcccagggtcacacaaagaatgaatagcagagccctgagcctgtgtgcttccctctgtgccaggctgctttacccaggcatgggtgcaccttgtgcatgggacatttctcctttgttgtgtcctgagtaccttaagccactcagatattgctcaggtggagtgaggggaaaatgttttcaggttgtattagtcaaaacaaaataccacacactgggcgactttaaaatcatacatttatccctcacagttctggaggcttggaagtccaagttcaaggtggcagctggacgggttcccggtgagggctctcttcctggtttgcagacagccaccttctcttcgcatcctcactctggtaaggggaccacccgctgcagccagcgagacagtggcatgttcttgttacaactcgatctaactcccccagaagaggaggcagggaaggcggacaaaaccattgaacacgagctgcccaactccgccttgcttccccattcctggcgaccactgcttctgtctctgtgaattttgactattctaggcacttcacaaaactggac

SEQ ID NO: 13281 - RNA, 713 nt, Homo sapiens
  source 1..713: mol_type = other RNA
gctgggattacaggcatgagccaccacgcccagccagattacaaaatactttgacatcttttctctacagccctcaaaaggaggcagggcaagcacaattaaatcccattacaaatggggtgactgaagctccattcatggcttgcccagggtcacacaaagaatgaatagcagagccctgagcctgtgtgcttccctctgtgccaggctgctttacccaggcatgggtgcaccttgtgcatgggacatttctcctttgttgtgtcctgagtaccttaagccactcagatattgctcaggtggagtgaggggaaaatgttttcaggttgtattagtcaaaacaaaataccacacactgggcgactttaaaatcatacatttatccctcacagttctggaggcttggaagtccaagttcaaggtggcagctggacgggttcccggtgagggctctcttcctggtttgcagacagccaccttctcttcgcatcctcactctggtaaggggaccacccgctgcagccagcgagacagtggcatgttcttgttacaactcgatctaactcccccagaagaggaggcagggaaggcggacaaaaccattgaacacgagctgcccaactccgccttgcttccccattcctggcgaccactgcttctgtctctgtgaattttgactattctaggcacttcacaaaactggactcatacga

SEQ ID NO: 13282 - RNA, 1292 nt, Homo sapiens
  source 1..1292: mol_type = other RNA
gctgggattacaggcatgagccaccacgcccagccattccttgtcatttctatcatttgatacatctatacttctgaataatcataactgatactcaaagagatgccctgacaccctccaaggttctacaaggtgaccaaatcagagaggtcacctcatgcctagtattattttggggttagcatacattttataataattattttaaaactggcaatccattttgggactcaatgacagctctctctattaatcatattgttttattaactgaaatagtccactcagtcagtaggattaatgatcagagattatgacacaactaaaaccaaagctggggcaatgggctctcagaatggaaccacccattatgaactatccatctgaccaactctttaactttcttcctaaatatgagatcaccaaggcgtttcaatgcagcctgcacaattcatggggcagggtcctcagattaaagactttacatttatgtagaattcagtatcatttttcactaagcaaactctatttgctcactctcttctacatgtaattgtccaactttggttgactgctgagtcctcatggaagaattcccattctgcccctgagcctctcctttagggacttggaaacggaaggtagtgcagttctttctggccatctgccaggcatggaaccccaggcttcttggggtaagttcgacgagcaagcttaaagaactcttctgcagcatcaagtgcaatgagacggtccacaacaaagagatatctctctgagagctcccaacttgttgggaaaatattggtttcttcagccagttttaacaacatctctcgagctttccttgtgtttttagaatcactgatggtgctgagtttagtcactgacaacaaagagtcagcttccttttgaaaacctaaatcttctaagatgcacttccatctgtttcttacttcccttcgaacctgccgcagggtatggatatcatagttgagcttctgccactcctctgagtctttggcctgctgattacgaatgactatcaaattgtacagggttctgtcgtcgtctgcctctgtgtgggacacatcatggggcatactccataaattcttctcatcatccctcaccagagttgctccaaatgaggaatatggattgttatcactatcttggagtggggaggagacctctgtaaggcaatgtgaatgctgatggcatcaggacttggcaaatcttaagactctgactcccaccaggcagaacgcaggactgcctctcactagact

SEQ ID NO: 13283 - RNA, 1489 nt, Homo sapiens
  source 1..1489: mol_type = other RNA
gctgggattacaggcatgagccaccacgcccagccattccttgtcatttctatcatttgatacatctatacttctgaataatcataactgatactcaaagagatgccctgacaccctccaaggttctacaaggtgaccaaatcagagaggtcacctcatgcctagtattattttggggttagcatacattttataataattattttaaaactggcaatccattttgggactcaatgacagctctctctattaatcatattgttttattaactgaaatagtccactcagtcagtaggattaatgatcagagattatgacacaactaaaaccaaagctggggcaatgggctctcagaatggaaccacccattatgaactatccatctgaccaactctttaactttcttcctaaatatgagatcaccaaggcgtttcaatgcagcctgcacaattcatggggcagggtcctcagattaaagactttacatttatgtagaattcagtatcatttttcactaagcaaactctatttgctcactctcttctacatgtaattgtccaactttggttgactgctgagtcctcatggaagaattcccattctgcccctgagcctctcctttagggacttggaaacggaaggtagtgcagttctttctggccatctgccaggcatggaaccccaggcttcttggggtaagttcgacgagcaagcttaaagaactcttctgcagcatcaagtgcaatgagacggtccacaacaaagagatatctctctgagagctcccaacttgttgggaaaatattggtttcttcagccagttttaacaacatctctcgagctttccttgtgtttttagaatcactgatggtgctgagtttagtcactgacaacaaagagtcagcttccttttgaaaacctaaatcttctaagatgcacttccatctgtttcttacttcccttcgaacctgccgcagggtatggatatcatagttgagcttctgccactcctctgagtctttggcctgctgattacgaatgactatcaaattgtacagggttctgtcgtcgtctgcctctgtgtgggacacatcatggggcatactccataaattcttctcatcatccctcaccagagttgctccaaatgaggaatatggattgttatcactgacgaggggctccttctcaggcagggcgcgctcctccaagcactcgcacccgcagcagcagcacacggttctcagccagtccctcagccccatggagagcgagggcccccaccggcgccggaagcctggggccgagtcgccgcggcgagcgatcgaggctggggcgcggccaccgcgccagcgtccaggtgcggggacagcggcagcccgggcgtcgcgggctggtccgcgcgcatcacgccgcggccggggacgcgggcgagggctgcaggccgcgcgccctcctctccttgcgttttgtttggggcgtgagtttt

SEQ ID NO: 13284 - RNA, 1305 nt, Homo sapiens
  source 1..1305: mol_type = other RNA
gctgggattacaggcatgagccaccacgcccagccattccttgtcatttctatcatttgatacatctatacttctgaataatcataactgatactcaaagagatgccctgacaccctccaaggttctacaaggtgaccaaatcagagaggtcacctcatgcctagtattattttggggttagcatacattttataataattattttaaaactggcaatccattttgggactcaatgacagctctctctattaatcatattgttttattaactgaaatagtccactcagtcagtaggattaatgatcagagattatgacacaactaaaaccaaagctggggcaatgggctctcagaatggaaccacccattatgaactatccatctgaccaactctttaactttcttcctaaatatgagatcaccaaggcgtttcaatgcagcctgcacaattcatggggcagggtcctcagattaaagactttacatttatgtagaattcagtatcatttttcactaagcaaactctatttgctcactctcttctacatgtaattgtccaactttggttgactgctgagtcctcatggaagaattcccattctgcccctgagcctctcctttagggacttggaaacggaaggtagtgcagttctttctggccatctgccaggcatggaaccccaggcttcttggggtaagttcgacgagcaagcttaaagaactcttctgcagcatcaagtgcaatgagacggtccacaacaaagagatatctctctgagagctcccaacttgttgggaaaatattggtttcttcagccagttttaacaacatctctcgagctttccttgtgtttttagaatcactgatggtgctgagtttagtcactgacaacaaagagtcagcttccttttgaaaacctaaatcttctaagatgcacttccatctgtttcttacttcccttcgaacctgccgcagggtatggatatcatagttgagcttctgccactcctctgagtctttggcctgctgattacgaatgactatcaaattgtacagggttctgtcgtcgtctgcctctgtgtgggacacatcatggggcatactccataaattcttctcatcatccctcaccagagttgctccaaatgaggaatatggattgttatcactttcctgaatatggtttagaatcttcccgctggttgatcttatttcaatagatggctcctttgctgaaatgaaatccttgtaaacaaggagtgcagaagaaataccaaaggaagaaactaaagctcaagttgaa

SEQ ID NO: 13285 - RNA, 1639 nt, Homo sapiens
  source 1..1639: mol_type = other RNA
gctgggattacaggcatgagccaccacgcccagccattccttgtcatttctatcatttgatacatctatacttctgaataatcataactgatactcaaagagatgccctgacaccctccaaggttctacaaggtgaccaaatcagagaggtcacctcatgcctagtattattttggggttagcatacattttataataattattttaaaactggcaatccattttgggactcaatgacagctctctctattaatcatattgttttattaactgaaatagtccactcagtcagtaggattaatgatcagagattatgacacaactaaaaccaaagctggggcaatgggctctcagaatggaaccacccattatgaactatccatctgaccaactctttaactttcttcctaaatatgagatcaccaaggcgtttcaatgcagcctgcacaattcatggggcagggtcctcagattaaagactttacatttatgtagaattcagtatcatttttcactaagcaaactctatttgctcactctcttctacatgtaattgtccaactttggttgactgctgagtcctcatggaagaattcccattctgcccctgagcctctcctttagggacttggaaacggaaggtagtgcagttctttctggccatctgccaggcatggaaccccaggcttcttggggtaagttcgacgagcaagcttaaagaactcttctgcagcatcaagtgcaatgagacggtccacaacaaagagatatctctctgagagctcccaacttgttgggaaaatattggtttcttcagccagttttaacaacatctctcgagctttccttgtgtttttagaatcactgatggtgctgagtttagtcactgacaacaaagagtcagcttccttttgaaaacctaaatcttctaagatgcacttccatctgtttcttacttcccttcgaacctgccgcagggtatggatatcatagttgagcttctgccactccttggagtagcggttggcagggggtggaggccaggagaggcctgtgcccagcggtctggcaccttcaagacttagaggggccgtcaataactcccaacaatggttggctttatgctttagcttggatgtctcaccactctggagcactccctctgagtctttggcctgctgattacgaatgactatcaaattgtacagggttctgtcgtcgtctgcctctgtgtgggacacatcatggggcatactccataaattcttctcatcatccctcaccagagttgctccaaatgaggaatatggattgttatcactgacgaggggctccttctcaggcagggcgcgctcctccaagcactcgcacccgcagcagcagcacacggttctcagccagtccctcagccccatggagagcgagggcccccaccggcgccggaagcctggggccgagtcgccgcggcgagcgatcgaggctggggcgcggccaccgcgccagcgtccaggtgcggggacagcggcagcccgggcgtcgcgggctggtccgcgcgcatcacgccgcggccggggacgcgggcgagggctgcaggccgcgcgccctcctctccttgcgttttgtttggggcgtgagtttt

SEQ ID NO: 13286 - RNA, 1945 nt, Homo sapiens
  source 1..1945: mol_type = other RNA
gctgggattacaggcatgagccaccacgcccagcccctgcaagcagtttctttaactctgttgggatgccattcgtgggcaaagctagatttgggacaagttgcccagctctgctaggaagagtcagtcctcagggggaagtttcttttcacctccgggatccccagggcttcctgggttgactcaggacttcatacgcagcctggatctccaggaagtgcctctgtgcctcctctgtctggtccaggttgtggtctgggtgccagaccttcactagctcctggtaactccgatgtatttcttcatttgttgccccttctgagaggcccaaaacctggtaagccagctgacgcttctcatcctgaaaactgtgaacaaactcatagagcttcgcccactcctgaaagcagctgctgttgaagccagtctcccccatcagtagcctccagatccggtaaggcagaaggaggacaaactccatgaggcggccaagaagggggaagaagctgaaccaattcaagaaggagccaaaggtttctgccacatagctgagggtggcagctgtgttgcagagggcactgtatgccagtgggcctgtgaaagcaaggtaagccaagcccagacgatagagccgcacactgagcggctctgatgccaccaaagctttgtagcggcgatgcctctgagctgtaatgctggcggccacgctaatgggcagtatggctatggggcggccatagaagataggtgaagtgagaaatgctgaccccagagtgttcttaaagtctgaggtctggttgccaacagcagccaccagcaagacccctaagccaactgccagtgggagggccacaatatagaagttgaccatggaagaaaggctaatcagtgccacaaggccaaaatagatgccaactatcacctgggcagcaaagcgaatgggactcagagggggtgtcacccctctggggctctgcctctgtccctgggctctgttggcctgagctacaaagcttgggagcttccagaactcccagagccagcccagcccacctccccccagggtcagcatccagagcagggcgtggctgtcccttcccaggtacaggtggtggagcccagcagggccccccacagcccagagggcataggtcaccaggagccccttggccatcctctagggcaaaggtctcagaacaagtccggttactcgcagcacagaagtctcggggtcctctgtgagactcatggctgtcatggccccagagttatccttagaccctcaagctgcacgctcctctcttcacgctccgttgaccttcaagactggatggttccacctccaattcccttaaggcagagacatccacggacaggctgcagtgagggacatccaacccaagctgtcctcaaccccccacagggcttgcttgcctcaccggcccacctccgagccttccagttaggggctctgcttctgcacctgagcctgagacctgaggagcctcccaatccagggctgctctgtcccgcgggctatgaaccagagggagaaacgggagcagagggttggagggcaggaggctcgaccaggagggcgaggccgcagcccgaggctcgtggtagtctgccttcctgcgcctctgcgctgcaacggagctgcaatgcaagacgccttcatttcaatgtcccgggctccaatcccgggttctactccgtgaacttggctaagtcatgcagcttcttgggcctcaatttccttctctggcaatctcgtggatctccgaggtcccccagtctggacttgcgggggcttcgggggacggtcggcctcgcgggtgtcacctcccggcagtaggcagagcgcttccctccaaacgccctcagccctcatctcggcctggagaggaaatgctgctctctatatgacctcttagggctcact

SEQ ID NO: 13287 - RNA, 2407 nt, Homo sapiens
  source 1..2407: mol_type = other RNA
gctgggattacaggcatgagccaccacgcccagcccctgcaagcagtttctttaactctgttgggatgccattcgtgggcaaagctagatttgggacaagttgcccagctctgctaggaagagtcagtcctcagggggaagtttcttttcacctccgggatccccagggcttcctgggttgactcaggacttcatacgcagcctggatctccaggaagtgcctctgtgcctcctctgtctggtccaggttgtggtctgggtgccagaccttcactagctcctggtaactccgatgtatttcttcatttgttgccccttctgagaggcccaaaacctggtaagccagctgacgcttctcatcctgaaaactgtgaacaaactcatagagcttcgcccactcctgaaagcagctgctgttgaagccagtctcccccatcagtagcctccagatccggtaaggcagaaggaggacaaactccatgaggcggccaagaagggggaagaagctgaaccaattcaagaaggagccaaaggtttctgccacatagctgagggtggcagctgtgttgcagagggcactgtatgccagtgggcctgtgaaagcaaggtaagccaagcccagacgatagagccgcacactgagcggctctgatgccaccaaagctttgtagcggcgatgcctctgagctgtaatgctggcggccacgctaatgggcagtatggctatggggcggccatagaagataggtgaagtgagaaatgctgaccccagagtgttcttaaagtctgaggtctggttgccaacagcagccaccagcaagacccctaagccaactgccagtgggagggccacaatatagaagttgaccatggaagaaaggctaatcagtgccacaaggccaaaatagatgccaactatcacctgggcagcaaagcgaatgggactcagagggggtgtcacccctctggggctctgcctctgtccctgggctctgttggcctgagctacaaagcttgggagcttccagaactcccagagccagcccagcccacctccccccagggtcagcatccagagcagggcgtggctgtcccttcccaggtacaggtggtggagcccagcagggccccccacagcccagagggcataggtcaccaggagccccttggccatcctctagggcaaaggtctcagaacaagtccggttactcgcagcacagaagtctcggggtcctctgtgagactcatggctgtcatggccccagagttatccttagaccctgggtgccccgctcccagaccgagtcagaccagtcatttcctttgaccacagagtgaaaatggcccgtctcgccctgctcccacttccatccaaatggactttgtcttttgtgtctgttgtgtcacggaagtccggcttccccaggccaggctcctccccagggccctccccggccccctggggatcacattcccgcctgggactcctcccgcccgccctcgcggggaaactcggtgcaaggctctgcagacgcctgcagctccggtgggctcagtgcccagcccgggcccagctcctcccacaccaccgcaccatggccgccaggtggcgctgccgccgatggaagggggggtccgggcggtccccagacaccttgtgcgggtaccgaggcacagcagcacaggactgcccctatggaggggctgcctggcaggagcaagggacgctcctatctgtagtgctcaagctgcacgctcctctcttcacgctccgttgaccttcaagactggatggttccacctccaattcccttaaggcagagacatccacggacaggctgcagtgagggacatccaacccaagctgtcctcaaccccccacagggcttgcttgcctcaccggcccacctccgagccttccagttaggggctctgcttctgcacctgagcctgagacctgaggagcctcccaatccagggctgctctgtcccgcgggctatgaaccagagggagaaacgggagcagagggttggagggcaggaggctcgaccaggagggcgaggccgcagcccgaggctcgtggtagtctgccttcctgcgcctctgcgctgcaacggagctgcaatgcaagacgccttcatttcaatgtcccgggctccaatcccgggttctactccgtgaacttggctaagtcatgcagcttcttgggcctcaatttccttctctggcaatctcgtggatctccgaggtcccccagtctggacttgcgggggcttcgggggacggtcggcctcgcgggtgtcacctcccggcagtaggcagagcgcttccctccaaacgccctcagccctcatctcggcctggagaggaaatgctgctctctatatgacctcttagggctcact

SEQ ID NO: 13288 - RNA, 1478 nt, Homo sapiens
  source 1..1478: mol_type = other RNA
gctgggattacaggcatgagccaccacgcccagccgcatgtttactttttaaaataaaatagaaatatggcaactagctttgtaagttaaaggaaactcagtttcacaataacttattagcttgagcacacatttgcaccaaagccagtcacaaccctaaaagttctataatgttggttgtattatatacaacatggactgttcttgctgtgaaaagataaaatactttgacttttgttacctgcagtatatgaaatgtgtttcctttattttgatttcttgggccgactgaagggtaaaatgtccaagctgaaatatcactgccaagcaagttcactaaacccagctacaacggatgcaaagggttttgactgacgtgcattcctctgatatcttccaccttgaagtctctgatgaggtagcaaggcaaaaaagttaaatctctctcccatcttctttggattcattaacatatcatatccttgaagtaactgctgcctcactgatggctcatttgatttatctaaaagaaccttcagccggacatcaatacccatattttttaaaaatgtgtgttgttttattgggcccagagaggctacttttccctgtgccattcttcgcaaataactgaagtccacatcagctgttagatctgctgttcctggggcaattaagacatcatgaagcttgtggtcgcaaaaccctctgaaggtatctgtctttgttccatcatgaccataatcagcaaccagtgcagcacctccagttaatgcaatgcgttgagaaagttcctcgatgataacaccagcatcaggacacacttcaacatgatcccttgtttcgtcatgttgtatgaaggcttctgctggggtggcagaaggtgccaaaacaaacctcagtttatcagaaacctgtggatcaatgtcaacaaatacttctcgccatccctgtggtgttttctctaccagatgtactgaaatgtcacaatttttcagcacagatccaagttgagtgaacaccctcaaaatatctcccacgagggttcccctacctgggcccagttccaccagctggaaagctgtgctttttccagtggccatccattcactaatgaaccatatacctagtagctccccaaagatttgacttatttcaggtgaagtaatgaaatctcctttttcgcctagcatgtcacggtacacataataacccttggctggattagtcaacacctccttcatgtactcggccacagtgatgggaccagtagactttattttgtacataagatgccgcagcatcggcgtcaccgggttttctgcaggctcattcccggagctgaagtatttccctctccaaataaaaggaatggctgcgcgcgccacggcacacaacggccccaaacctgacctcagcagtacactcatgctgaaattcgcaggctagctcgctccgccaggagctggggcttagac

SEQ ID NO: 13289 - RNA, 1485 nt, Homo sapiens
  source 1..1485: mol_type = other RNA
gctgggattacaggcatgagccaccacgcccagccgcatgtttactttttaaaataaaatagaaatatggcaactagctttgtaagttaaaggaaactcagtttcacaataacttattagcttgagcacacatttgcaccaaagccagtcacaaccctaaaagttctataatgttggttgtattatatacaacatggactgttcttgctgtgaaaagataaaatactttgacttttgttacctgcagtatatgaaatgtgtttcctttattttgatttcttgggccgactgaagggtaaaatgtccaagctgaaatatcactgccaagcaagttcactaaacccagctacaacggatgcaaagggttttgactgacgtgcattcctctgatatcttccaccttgaagtctctgatgaggtagcaaggcaaaaaagttaaatctctctcccatcttctttggattcattaacatatcatatccttgaagtaactgctgcctcactgatggctcatttgatttatctaaaagaaccttcagccggacatcaatacccatattttttaaaaatgtgtgttgttttattgggcccagagaggctacttttccctgtgccattcttcgcaaataactgaagtccacatcagctgttagatctgctgttcctggggcaattaagacatcatgaagcttgtggtcgcaaaaccctctgaaggtatctgtctttgttccatcatgaccataatcagcaaccagtgcagcacctccagttaatgcaatgcgttgagaaagttcctcgatgataacaccagcatcaggacacacttcaacatgatcccttgtttcgtcatgttgtatgaaggcttctgctggggtggcagaaggtgccaaaacaaacctcagtttatcagaaacctgtggatcaatgtcaacaaatacttctcgccatccctgtggtgttttctctaccagatgtactgaaatgtcacaatttttcagcacagatccaagttgagtgaacaccctcaaaatatctcccacgagggttcccctacctgggcccagttccaccagctggaaagctgtgctttttccagtggccatccattcactaatgaaccatatacctagtagctccccaaagatttgacttatttcaggtgaagtaatgaaatctcctttttcgcctagcatgtcacggtacacataataacccttggctggattagtcaacacctccttcatgtactcggccacagtgatgggaccagtagactttattttgtacataagatgccgcagcatcggcgtcaccgggttttctgcaggctcattcccggagctgaagtatttccctctccaaataaaaggaatggcttcaaggtggaagtgagcccccgagcccttgatcccccggtaccctcaactgaagagctgaggaaggcgccccacgcggcttccacggcaaccgggcttcgaggggact

SEQ ID NO: 13290 - RNA, 1397 nt, Homo sapiens
  source 1..1397: mol_type = other RNA
gctgggattacaggcatgagccaccacgcccagccgcatgtttactttttaaaataaaatagaaatatggcaactagctttgtaagttaaaggaaactcagtttcacaataacttattagcttgagcacacatttgcaccaaagccagtcacaaccctaaaagttctataatgttggttgtattatatacaacatggactgttcttgctgtgaaaagataaaatactttgacttttgttacctgcagtatatgaaatgtgtttcctttattttgatttcttgggccgactgaagggtaaaatgtccaagctgaaatatcactgccaagcaagttcactaaacccagctacaacggatgcaaagggttttgactgacgtgcattcctctgatatcttccaccttgaagtctctgatgaggtagcaaggcaaaaaagttaaatctctctcccatcttctttggattcattaacatatcatatccttgaagtaactgctgcctcactgatggctcatttgatttatctaaaagaaccttcagccggacatcaatacccatattttttaaaaatgtgtgttgttttattgggcccagagaggctacttttccctgtgccattcttcgcaaataactgaagtccacatcagctgttagatctgctgttcctggggcaattaagacatcatgaagcttgtggtcgcaaaaccctctgaaggtatctgtctttgttccatcatgaccataatcagcaaccagtgcagcacctccagttaatgcaatgcgttgagaaagttcctcgatgataacaccagcatcaggacacacttcaacatgatcccttgtttcgtcatgttgtatgaaggcttctgctggggtggcagaaggtgccaaaacaaacctcagtttatcagaaacctgtggatcaatgtcaacaaatacttctcgccatccctgtggtgttttctctaccagatgtactgaaatgtcacaatttttcagcacagatccaagttgagtgaacaccctcaaaatatctcccacgagggttcccctacctgggcccagttccaccagctggaaagctgtgctttttccagtggccatccattcactaatgaaccatatacctagtagcttggctggattagtcaacacctccttcatgtactcggccacagtgatgggaccagtagactttattttgtacataagatgccgcagcatcggcgtcaccgggttttctgcaggctcattcccggagctgaagtatttccctctccaaataaaaggaatggctgcgcgcgccacggcacacaacggccccaaacctgacctcagcagtacactcatgctgaaattcgcaggctagctcgctccgccaggagctggggcttagac

SEQ ID NO: 13291 - RNA, 1446 nt, Homo sapiens
  source 1..1446: mol_type = other RNA
gctgggattacaggcatgagccaccacgcccagccgcatgtttactttttaaaataaaatagaaatatggcaactagctttgtaagttaaaggaaactcagtttcacaataacttattagcttgagcacacatttgcaccaaagccagtcacaaccctaaaagttctataatgttggttgtattatatacaacatggactgttcttgctgtgaaaagataaaatactttgacttttgttacctgcagtatatgaaatgtgtttcctttattttgatttcttgggccgactgaagggtaaaatgtccaagctgaaatatcactgccaagcaagttcactaaacccagctacaacggatgcaaagggttttgactgacgtgcattcctctgatatcttccaccttgaagtctctgatgaggtagcaaggcaaaaaagttaaatctctctcccatcttctttggattcattaacatatcatatccttgaagtaactgctgcctcactgatggctcatttgatttatctaaaagaaccttcagccggacatcaatacccatattttttaaaaatgtgtgttgttttattgggcccagagaggctacttttccctgtgccattcttcgcaaataactgaagtccacatcagctgttagatctgctgttcctggggcaattaagacatcatgaagcttgtggtcgcaaaaccctctgaaggtatctgtctttgttccatcatgaccataatcagcaaccagtgcagcacctccagttaatgcaatgcgttgagaaagttcctcgatgataacaccagcatcaggacacacttcaacatgatcccttgtttcgtcatgttgtatgaaggcttctgctggggtggcagaaggtgccaaaacaaacctcagtttatcagaaacctgtggatcaatgtcaacaaatacttctcgccatccctgtggtgttttctctaccagatgtactgaaatgtcacaatttttcagcacagatccaagttgagtgaacacctgggcccagttccaccagctggaaagctgtgctttttccagtggccatccattcactaatgaaccatatacctagtagctccccaaagatttgacttatttcaggtgaagtaatgaaatctcctttttcgcctagcatgtcacggtacacataataacccttggctggattagtcaacacctccttcatgtactcggccacagtgatgggaccagtagactttattttgtacataagatgccgcagcatcggcgtcaccgggttttctgcaggctcattcccggagctgaagtatttccctctccaaataaaaggaatggctgcgcgcgccacggcacacaacggccccaaacctgacctcagcagtacactcatgctgaaattcgcaggctagctcgctccgccaggagctggggcttagac

SEQ ID NO: 13292 - RNA, 1537 nt, Homo sapiens
  source 1..1537: mol_type = other RNA
gctgggattacaggcatgagccaccacgcccagccgcatgtttactttttaaaataaaatagaaatatggcaactagctttgtaagttaaaggaaactcagtttcacaataacttattagcttgagcacacatttgcaccaaagccagtcacaaccctaaaagttctataatgttggttgtattatatacaacatggactgttcttgctgtgaaaagataaaatactttgacttttgttacctgcagtatatgaaatgtgtttcctttattttgatttcttgggccgactgaagggtaaaatgtccaagctgaaatatcactgccaagcaagttcactaaacccagctacaacggatgcaaagggttttgactgacgtgcattcctctgatatcttccaccttgaagtctctgatgaggtagcaaggcaaaaaagttaaatctctctcccatcttctttggattcattaacatatcatatccttgaagtaactgctgcctcactgatggctcatttgatttatctaaaagaaccttcagccggacatcaatacccatattttttaaaaatgtgtgttgttttattgggcccagagaggctacttttccctgtgccattcttcgcaaataactgaagtccacatcagctgttagatctgctgttcctggggcaattaagacatcatgaagcttgtggtcgcaaaaccctctgaaggtatctgtctttgttccatcatgaccataatcagcaaccagtgcagcacctccagttaatgcaatgcgttgagaaagttcctcgatgataacaccagcatcaggacacacttcaacatgatcccttgtttcgtcatgttgtatgaaggcttctgctggggtggcagaaggtgccaaaacaaacctcagtttatcagaaacctgtggatcaatgtcaacaaatacttctcgccatccctgtggtgttttctgaaatttatgcacaggaagaacatcaaaaaattcatgtgcaagataaaagctgtaccctctaccagatgtactgaaatgtcacaatttttcagcacagatccaagttgagtgaacaccctcaaaatatctcccacgagggttcccctacctgggcccagttccaccagctggaaagctgtgctttttccagtggccatccattcactaatgaaccatatacctagtagctccccaaagatttgacttatttcaggtgaagtaatgaaatctcctttttcgcctagcatgtcacggtacacataataacccttggctggattagtcaacacctccttcatgtactcggccacagtgatgggaccagtagactttattttgtacataagatgccgcagcatcggcgtcaccgggttttctgcaggctcattcccggagctgaagtatttccctctccaaataaaaggaatggctgcgcgcgccacggcacacaacggccccaaacctgacctcagcagtacactcatgctgaaattcgcaggctagctcgctccgccaggagctggggcttagac

SEQ ID NO: 13293 - RNA, 1456 nt, Homo sapiens
  source 1..1456: mol_type = other RNA
gctgggattacaggcatgagccaccacgcccagccgcatgtttactttttaaaataaaatagaaatatggcaactagctttgtaagttaaaggaaactcagtttcacaataacttattagcttgagcacacatttgcaccaaagccagtcacaaccctaaaagttctataatgttggttgtattatatacaacatggactgttcttgctgtgaaaagataaaatactttgacttttgttacctgcagtatatgaaatgtgtttcctttattttgatttcttgggccgactgaagggtaaaatgtccaagctgaaatatcactgccaagcaagttcactaaacccagctacaacggatgcaaagggttttgactgacgtgcattcctctgatatcttccaccttgaagtctctgatgaggtagcaaggcaaaaaagttaaatctctctcccatcttctttggattcattaacatatcatatccttgaagtaactgctgcctcactgatggctcatttgatttatctaaaagaaccttcagccggacatcaatacccatattttttaaaaatgtgtgttgttttattgggcccagagaggctacttttccctgtgccattcttcgcaaataactgaagtccacatcagctgttagatctgctgttcctggggcaattaagacatcatgaagcttgtggtcgcaaaaccctctgaaggtatctgtctttgttccatcatgaccataatcagcaaccagtgcagcacctccagttaatgcaatgcgttgagaaagttcctcgatgataacaccagcatcaggacacacttcaacatgatcccttgtttcgtcatgttgtatgaaggcttctgctggggtggcagaaggtgccaaaacaaacctcagtttatcagaaacctgtggatcaatgtcaacaaatacttctcgccatccctgtggtgttttctgaaatttatgcacaggaagaacatcaaaaaattcatgtgcaagataaaagctgtaccctctaccagatgtactgaaatgtcacaatttttcagcacagatccaagttgagtgaacaccctcaaaatatctcccacgagggttcccctacctgggcccagttccaccagctggaaagctgtgctttttccagtggccatccattcactaatgaaccatatacctagtagcttggctggattagtcaacacctccttcatgtactcggccacagtgatgggaccagtagactttattttgtacataagatgccgcagcatcggcgtcaccgggttttctgcaggctcattcccggagctgaagtatttccctctccaaataaaaggaatggctgcgcgcgccacggcacacaacggccccaaacctgacctcagcagtacactcatgctgaaattcgcaggctagctcgctccgccaggagctggggcttagac

SEQ ID NO: 13294 - RNA, 2324 nt, Homo sapiens
  source 1..2324: mol_type = other RNA
gctgggattacaggcatgagccaccacgcccagccgcatgtttactttttaaaataaaatagaaatatggcaactagctttgtaagttaaaggaaactcagtttcacaataacttattagcttgagcacacatttgcaccaaagccagtcacaaccctaaaagttctataatgttggttgtattatatacaacatggactgttcttgctgtgaaaagataaaatactttgacttttgttacctgcagtatatgaaatgtgtttcctttattttgatttcttgggccgactgaagggtaaaatgtccaagctgaaatatcactgccaagcaagttcactaaacccagctacaacggatgcaaagggttttgactgacgtgcattcctctgatatcttccaccttgaagtctctgatgaggtagcaaggcaaaaaagttaaatctctctcccatcttctttggattcattaacatatcatatccttgaagtaactgctgcctcactgatggctcatttgatttatctaaaagaaccttcagccggacatcaatacccatattttttaaaaatgtgtgttgttttattgggcccagagaggctacttttccctgtgccattcttcgcaaataactgaagtccacatcagctgttagatctgctgttcctggggcaattaagacatcatgaagcttgtggtcgcaaaaccctctgaaggtatctgtctttgttccatcatgaccataatcagcaaccagtgcagcacctccagttaatgcaatgcgttgagaaagttcctcgatgataacaccagcatcaggacacacttcaacatgatcccttgtttcgtcatgttgtatgaaggcttctgctggggtggcagaaggtgccaaaacaaacctcagtttatcagaaacctgtggatcaatgtcaacaaatacttctcgccatccctgtggtgttttctgaaatttatgcacaggaagaacatcaaaaaattcatgtgcaagataaaagctgtaccctgaaatagcagttaaagcttttattcatcacaaggcttgaaagaaattagaagtcagagttgttagctggaagggaatttgatttcataaaatcgggcttctcagcctgagaaggctgaggcaggaatggcttgagatcccttacccaagatcgtacccccactttggctttgagtcaagactcaaactagtcaatactagtcagtattcctgactagtacagggattttcccccacaccttgcttgtctttaggcaagtaaggattttttaaaagactctataactgaactaaacccacctactaacactgcttccatcagccccagctgccttgggctgctccgtcatcggtacaaccctagctatagggaaatactcaaaagtacaaaggagatttacattttgtttgggattttacaaagcttcatgaaataaactactacttaatgtcaggcaactttattttctattaagatgctcttttctagaaaaaagtaggctactctctatggataagggacttggcagcagtaactcaatctattatattgctgtaaaaagttacagtcccatcaatactgtgagggttgtgatcaaaattctttcattaatccacataaaggtaattaccttttggaacatcgtgcagatctcggtaccaggaaattggaatcccagacttagtgacacctttcatatacactggggatccagcatttcgctctaacgggaccttctctttagtcagtgtcaatgcttgaatctcacttaatttttggcttacctctaccagatgtactgaaatgtcacaatttttcagcacagatccaagttgagtgaacaccctcaaaatatctcccacgagggttcccctacctgggcccagttccaccagctggaaagctgtgctttttccagtggccatccattcactaatgaaccatatacctagtagctccccaaagatttgacttatttcaggtgaagtaatgaaatctcctttttcgcctagcatgtcacggtacacataataacccttggctggattagtcaacacctccttcatgtactcggccacagtgatgggaccagtagactttattttgtacataagatgccgcagcatcggcgtcaccgggttttctgcaggctcattcccggagctgaagtatttccctctccaaataaaaggaatggctgcgcgcgccacggcacacaacggccccaaacctgacctcagcagtacactcatgctgaaattcgcaggctagctcgctccgccaggagctggggcttagac

SEQ ID NO: 13295 - RNA, 1691 nt, Homo sapiens
  source 1..1691: mol_type = other RNA
gctgggattacaggcatgagccaccacgcccagccgcatgtttactttttaaaataaaatagaaatatggcaactagctttgtaagttaaaggaaactcagtttcacaataacttattagcttgagcacacatttgcaccaaagccagtcacaaccctaaaagttctataatgttggttgtattatatacaacatggactgttcttgctgtgaaaagataaaatactttgacttttgttacctgcagtatatgaaatgtgtttcctttattttgatttcttgggccgactgaagggtaaaatgtccaagctgaaatatcactgccaagcaagttcactaaacccagctacaacggatgcaaagggttttgactgacgtgcattcctctgatatcttccaccttgaagtctctgatgaggtagcaaggcaaaaaagttaaatctctctcccatcttctttggattcattaacatatcatatccttgaagtaactgctgcctcactgatggctcatttgatttatctaaaagaaccttcagccggacatcaatacccatattttttaaaaatgtgtgttgttttattgggcccagagaggctacttttccctgtgccattcttcgcaaataactgaagtccacatcagctgttagatctgctgttcctggggcaattaagacatcatgaagcttgtggtcgcaaaaccctctgaaggtatctgtctttgttccatcatgaccataatcagcaaccagtgcagcacctccagttaatgcaatgcgttgagaaagttcctcgatgataacaccagcatcaggacacacttcaacatgatcccttgtttcgtcatgttgtatgaaggcttctgctggggtggcagaaggtgccaaaacaaacctcagtttatcagaaacctgtggatcaatgtcaacaaatacttctcgccatccctgtggtgttttctgaaatttatgcacaggaagaacatcaaaaaattcatgtgcaagataaaagctgtacccttttggaacatcgtgcagatctcggtaccaggaaattggaatcccagacttagtgacacctttcatatacactggggatccagcatttcgctctaacgggaccttctctttagtcagtgtcaatgcttgaatctcacttaatttttggcttacctctaccagatgtactgaaatgtcacaatttttcagcacagatccaagttgagtgaacaccctcaaaatatctcccacgagggttcccctacctgggcccagttccaccagctggaaagctgtgctttttccagtggccatccattcactaatgaaccatatacctagtagctccccaaagatttgacttatttcaggtgaagtaatgaaatctcctttttcgcctagcatgtcacggtacacataataacccttggctggattagtcaacacctccttcatgtactcggccacagtgatgggaccagtagactttattttgtacataagatgccgcagcatcggcgtcaccgggttttctgcaggctcattcccggagctgaagtatttccctctccaaataaaaggaatggctgcgcgcgccacggcacacaacggccccaaacctgacctcagcagtacactcatgctgaaattcgcaggctagctcgctccgccaggagctggggcttagac

SEQ ID NO: 13296 - RNA, 1701 nt, Homo sapiens
  source 1..1701: mol_type = other RNA
gctgggattacaggcatgagccaccacgcccagccgcatgtttactttttaaaataaaatagaaatatggcaactagctttgtaagttaaaggaaactcagtttcacaataacttattagcttgagcacacatttgcaccaaagccagtcacaaccctaaaagttctataatgttggttgtattatatacaacatggactgttcttgctgtgaaaagataaaatactttgacttttgttacctgcagtatatgaaatgtgtttcctttattttgatttcttgggccgactgaagggtaaaatgtccaagctgaaatatcactgccaagcaagttcactaaacccagctacaacggatgcaaagggttttgactgacgtgcattcctctgatatcttccaccttgaagtctctgatgaggtagcaaggcaaaaaagttaaatctctctcccatcttctttggattcattaacatatcatatccttgaagtaactgctgcctcactgatggctcatttgatttatctaaaagaaccttcagccggacatcaatacccatattttttaaaaatgtgtgttgttttattgggcccagagaggctacttttccctgtgccattcttcgcaaataactgaagtccacatcagctgttagatctgctgttcctggggcaattaagacatcatgaagcttgtggtcgcaaaaccctctgaaggtatctgtctttgttccatcatgaccataatcagcaaccagtgcagcacctccagttaatgcaatgcgttgagaaagttcctcgatgataacaccagcatcaggacacacttcaacatgatcccttgtttcgtcatgttgtatgaaggcttctgctggggtggcagaaggtgccaaaacaaacctcagtttatcagaaacctgtggatcaatgtcaacaaatacttctcgccatccctgtggtgttttctgaaatttatgcacaggaagaacatcaaaaaattcatgtgcaagataaaagctgtacccttttggaacatcgtgcagatctcggtaccaggaaattggaatcccagacttagtgacacctttcatatacactggggatccagcatttcgctctaacgggaccttctctttagtcagtgtcaatgcttgaatctcacttaatttttggcttacctctaccagatgtactgaaatgtcacaatttttcagcacagatccaagttgagtgaacaccctcaaaatatctcccacgagggttcccctacctgggcccagttccaccagctggaaagctgtgctttttccagtggccatccattcactaatgaaccatatacctagtagctccccaaagatttgacttatttcaggtgaagtaatgaaatctcctttttcgcctagcatgtcacggtacacataataacccttggctggattagtcaacacctccttcatgtactcggccacagtgatgggaccagtagactttattttgtacataagatgccgcagcatcggcgtcaccgggttttctgcaggctcattcccggagctgaagtatttccctctccaaataaaaggaatggcttcaaggtggaagtgagcccccgagcccttgatcccccggtaccctcaactgaagagctgaggaaggcgccccacgcggcttccacggcaaccgggcttcgaggggactgac

SEQ ID NO: 13297 - RNA, 1654 nt, Homo sapiens
  source 1..1654: mol_type = other RNA
gctgggattacaggcatgagccaccacgcccagccgcatgtttactttttaaaataaaatagaaatatggcaactagctttgtaagttaaaggaaactcagtttcacaataacttattagcttgagcacacatttgcaccaaagccagtcacaaccctaaaagttctataatgttggttgtattatatacaacatggactgttcttgctgtgaaaagataaaatactttgacttttgttacctgcagtatatgaaatgtgtttcctttattttgatttcttgggccgactgaagggtaaaatgtccaagctgaaatatcactgccaagcaagttcactaaacccagctacaacggatgcaaagggttttgactgacgtgcattcctctgatatcttccaccttgaagtctctgatgaggtagcaaggcaaaaaagttaaatctctctcccatcttctttggattcattaacatatcatatccttgaagtaactgctgcctcactgatggctcatttgatttatctaaaagaaccttcagccggacatcaatacccatattttttaaaaatgtgtgttgttttattgggcccagagaggctacttttccctgtgccattcttcgcaaataactgaagtccacatcagctgttagatctgctgttcctggggcaattaagacatcatgaagcttgtggtcgcaaaaccctctgaaggtatctgtctttgttccatcatgaccataatcagcaaccagtgcagcacctccagttaatgcaatgcgttgagaaagttcctcgatgataacaccagcatcaggacacacttcaacatgatcccttgtttcgtcatgttgtatgaaggcttctgctggggtggcagaaggtgccaaaacaaacctcagtttatcagaaacctgtggatcaatgtcaacaaatacttctcgccatccctgtggtgttttctgaaatttatgcacaggaagaacatcaaaaaattcatgtgcaagataaaagctgtacccttttggaacatcgtgcagatctcggtaccaggaaattggaatcccagacttagtgacacctttcatatacactggggatccagcatttcgctctaacgggaccttctctttagtcagtgtcaatgcttgaatctcacttaatttttggcttacctctaccagatgtactgaaatgtcacaatttttcagcacagatccaagttgagtgaacacctgggcccagttccaccagctggaaagctgtgctttttccagtggccatccattcactaatgaaccatatacctagtagctccccaaagatttgacttatttcaggtgaagtaatgaaatctcctttttcgcctagcatgtcacggtacacataataacccttggctggattagtcaacacctccttcatgtactcggccacagtgatgggaccagtagactttattttgtacataagatgccgcagcatcggcgtcaccgggttttctgcaggctcattcccggagctgaagtatttccctctccaaataaaaggaatggctgcgcgcgccacggcacacaacggccccaaacctgacctcagcagtacactcatgctgaaattcgcaggctagctcgctccgccaggagctggggct

SEQ ID NO: 13298 - RNA, 1632 nt, Homo sapiens
  source 1..1632: mol_type = other RNA
gctgggattacaggcatgagccaccacgcccagccgcatgtttactttttaaaataaaatagaaatatggcaactagctttgtaagttaaaggaaactcagtttcacaataacttattagcttgagcacacatttgcaccaaagccagtcacaaccctaaaagttctataatgttggttgtattatatacaacatggactgttcttgctgtgaaaagataaaatactttgacttttgttacctgcagtatatgaaatgtgtttcctttattttgatttcttgggccgactgaagggtaaaatgtccaagctgaaatatcactgccaagcaagttcactaaacccagctacaacggatgcaaagggttttgactgacgtgcattcctctgatatcttccaccttgaagtctctgatgaggtagcaaggcaaaaaagttaaatctctctcccatcttctttggattcattaacatatcatatccttgaagtaactgctgcctcactgatggctcatttgatttatctaaaagaaccttcagccggacatcaatacccatattttttaaaaatgtgtgttgttttattgggcccagagaggctacttttccctgtgccattcttcgcaaataactgaagtccacatcagctgttagatctgctgttcctggggcaattaagacatcatgaagcttgtggtcgcaaaaccctctgaaggtatctgtctttgttccatcatgaccataatcagcaaccagtgcagcacctccagttaatgcaatgcgttgagaaagttcctcgatgataacaccagcatcaggacacacttcaacatgatcccttgtttcgtcatgttgtatgaaggcttctgctggggtggcagaaggtgccaaaacaaacctcagtttatcagaaacctgtggatcaatgtcaacaaatacttctcgccatccctgtggtgttttcttttggaacatcgtgcagatctcggtaccaggaaattggaatcccagacttagtgacacctttcatatacactggggatccagcatttcgctctaacgggaccttctctttagtcagtgtcaatgcttgaatctcacttaatttttggcttacctctaccagatgtactgaaatgtcacaatttttcagcacagatccaagttgagtgaacaccctcaaaatatctcccacgagggttcccctacctgggcccagttccaccagctggaaagctgtgctttttccagtggccatccattcactaatgaaccatatacctagtagctccccaaagatttgacttatttcaggtgaagtaatgaaatctcctttttcgcctagcatgtcacggtacacataataacccttggctggattagtcaacacctccttcatgtactcggccacagtgatgggaccagtagactttattttgtacataagatgccgcagcatcggcgtcaccgggttttctgcaggctcattcccggagctgaagtatttccctctccaaataaaaggaatggctgcgcgcgccacggcacacaacggccccaaacctgacctcagcagtacactcatgctgaaattcgcaggctagctcgctccgccaggagctggggcttagac

SEQ ID NO: 13299 - RNA, 1568 nt, Homo sapiens
  source 1..1568: mol_type = other RNA
gctgggattacaggcatgagccaccacgcccagccgcatgtttactttttaaaataaaatagaaatatggcaactagctttgtaagttaaaggaaactcagtttcacaataacttattagcttgagcacacatttgcaccaaagccagtcacaaccctaaaagttctataatgttggttgtattatatacaacatggactgttcttgctgtgaaaagataaaatactttgacttttgttacctgcagtatatgaaatgtgtttcctttattttgatttcttgggccgactgaagggtaaaatgtccaagctgaaatatcactgccaagcaagttcactaaacccagctacaacggatgcaaagggttttgactgacgtgcattcctctgatatcttccaccttgaagtctcttcagccggacatcaatacccatattttttaaaaatgtgtgttgttttattgggcccagagaggctacttttccctgtgccattcttcgcaaataactgaagtccacatcagctgttagatctgctgttcctggggcaattaagacatcatgaagcttgtggtcgcaaaaccctctgaaggtatctgtctttgttccatcatgaccataatcagcaaccagtgcagcacctccagttaatgcaatgcgttgagaaagttcctcgatgataacaccagcatcaggacacacttcaacatgatcccttgtttcgtcatgttgtatgaaggcttctgctggggtggcagaaggtgccaaaacaaacctcagtttatcagaaacctgtggatcaatgtcaacaaatacttctcgccatccctgtggtgttttctgaaatttatgcacaggaagaacatcaaaaaattcatgtgcaagataaaagctgtacccttttggaacatcgtgcagatctcggtaccaggaaattggaatcccagacttagtgacacctttcatatacactggggatccagcatttcgctctaacgggaccttctctttagtcagtgtcaatgcttgaatctcacttaatttttggcttacctctaccagatgtactgaaatgtcacaatttttcagcacagatccaagttgagtgaacaccctcaaaatatctcccacgagggttcccctacctgggcccagttccaccagctggaaagctgtgctttttccagtggccatccattcactaatgaaccatatacctagtagctccccaaagatttgacttatttcaggtgaagtaatgaaatctcctttttcgcctagcatgtcacggtacacataataacccttggctggattagtcaacacctccttcatgtactcggccacagtgatgggaccagtagactttattttgtacataagatgccgcagcatcggcgtcaccgggttttctgcaggctcattcccggagctgaagtatttccctctccaaataaaaggaatggctgcgcgcgccacggcacacaacggccccaaacctgacctcagcagtacactcatgctgaaattcgcaggctagctcgctccgccaggagctggggcttagac

SEQ ID NO: 13300 - RNA, 1487 nt, Homo sapiens
  source 1..1487: mol_type = other RNA
gctgggattacaggcatgagccaccacgcccagccgcatgtttactttttaaaataaaatagaaatatggcaactagctttgtaagttaaaggaaactcagtttcacaataacttattagcttgagcacacatttgcaccaaagccagtcacaaccctaaaagttctataatgttggttgtattatatacaacatggactgttcttgctgtgaaaagataaaatactttgacttttgttacctgcagtatatgaaatgtgtttcctttattttgatttcttgggccgactgaagggtaaaatgtccaagctgaaatatcactgccaagcaagttcactaaacccagctacaacggatgcaaagggttttgactgacgtgcattcctctgatatcttccaccttgaagtctcttcagccggacatcaatacccatattttttaaaaatgtgtgttgttttattgggcccagagaggctacttttccctgtgccattcttcgcaaataactgaagtccacatcagctgttagatctgctgttcctggggcaattaagacatcatgaagcttgtggtcgcaaaaccctctgaaggtatctgtctttgttccatcatgaccataatcagcaaccagtgcagcacctccagttaatgcaatgcgttgagaaagttcctcgatgataacaccagcatcaggacacacttcaacatgatcccttgtttcgtcatgttgtatgaaggcttctgctggggtggcagaaggtgccaaaacaaacctcagtttatcagaaacctgtggatcaatgtcaacaaatacttctcgccatccctgtggtgttttctgaaatttatgcacaggaagaacatcaaaaaattcatgtgcaagataaaagctgtacccttttggaacatcgtgcagatctcggtaccaggaaattggaatcccagacttagtgacacctttcatatacactggggatccagcatttcgctctaacgggaccttctctttagtcagtgtcaatgcttgaatctcacttaatttttggcttacctctaccagatgtactgaaatgtcacaatttttcagcacagatccaagttgagtgaacaccctcaaaatatctcccacgagggttcccctacctgggcccagttccaccagctggaaagctgtgctttttccagtggccatccattcactaatgaaccatatacctagtagcttggctggattagtcaacacctccttcatgtactcggccacagtgatgggaccagtagactttattttgtacataagatgccgcagcatcggcgtcaccgggttttctgcaggctcattcccggagctgaagtatttccctctccaaataaaaggaatggctgcgcgcgccacggcacacaacggccccaaacctgacctcagcagtacactcatgctgaaattcgcaggctagctcgctccgccaggagctggggcttagac

SEQ ID NO: 13301 - RNA, 2485 nt, Homo sapiens
  source 1..2485: mol_type = other RNA
gctgggattacaggcatgagccaccacgcccagcctatttttagttttttgaggaaactgtactgttctccatagtggctatactaatttacattcccaccaatagtatatggggattcctctttctccactttctcatcagcatttgtcattgcctgtcttttggataaaagccattgtaactggggtgagatgtcttgttcatggcctcgttattcccctagcctgtggccctttcctcttgccagcttacctgggacccaggcatgcctccctcctctccctaagccccaaggaccacaggagctaaggtgatcaacaaattcaccctgaggtgtaaatagggaagcacccctccaagtcagcctgcccgcgttagggcaaagggggtgaagttgccagtgcgtttggacttcgcacgccctgagaggctgcaggtcagagaggtcagagctgtagctgctttacgcacggactctccggccagacctcccctcaggtctcccggcttcagctcctgagacagtggttcccagataccttgagagaggggagcctggtttccatttcctaggggtcccagctcaaggcaatgcagggcagctgatggggcaagagttgggcagagggtgtgggacagtcacagtggagatcccagggggcatggggtaaaggccccaggcctctccctgccaccaagtttccaggatttgatgttcctctgaccacacgtttgcacagcccctgccccaggcttgctctctggaactctgtgttctccgtgacactgctgcaggggccacacttctccaagaactgactgcacgtccaaaggtcactctgcaaagagggttctgtcatgcccctcatgagaagatggctttgtactttccaaagccccttcatatccattatttcctcagatctttgtagtcctcccagccaggagggaagaatatgattgtccgtgttcaacagtaaatgaattgagacccagagaagtgaagagagtgtcccaggtccacacagcaagtcggtgacagaggaggacaagactgggcctccaggccctgtaaacagtttcctgtctgctttactatagcaggtgttctaggtaagaaagggcaagggaacatttctggaagtttcacgctcaagctaatgcgtgtactctctctctctctctctcacacacacacacacacacagacgtatgcacatttacgaaatgctggcaaaaatatcagggagctccgaaatggttgtccacataggaggccagatgagcctccttgagcagggtcttgaccttgagcaggggaggagccacccagctgggggctgccaaggtgcccgagaaccaggactggctgtgccagccaagcctcgcactggcctttgttctttacagtgctgaaatggatgttggtggctgagggactcctcacggtgagcacatggtggctggtgggctccgggggttcatctggctcaaattttcataattggactcctgggcctgggaccgtggtggggtgtccggggtgtccagatgctctgggcggcggcgggcagcgcgggcggccaggaccccgagcagcagcagcgccttgaagccgagagcgccgagcaggagggcgaccgtcgaggccccgctggcgccatggaagcggaacaggtagacgctggcctcggagcggcccaggctgttggcggccgtacacgtgtagcggccgtcatgggtcagtgcgggcagttcggcggtcactaggtggccgtgaccctcacgcgggctccgcacggctgccaagctgttgcccagggccgggccggaccaggcgagggcgggcggcggctccccttcggcagtgcagagcgcgcggaaggcgtgagccggactgggcagcaccgagatgttgacgatccgcggcgcggctgtcacgtgcagccggacgccgtggcggctctcgtagcggtcatggacgtcgccggcgaactcgacgcggcagaagtagcggcggtcgtcagccagggcgaggcgctcgacgcgcagcgagaggtcgttgcggcgcgggttgcccagcagccggaagcggccgtgcaggctcagcgccgtctggcagagctcgctgccccgcgccgcagcgcagcggaacacctgcgggcccgcatagggctcgcccgcgcgccagatggccgtcagcggcccgtcgtagtggcggtgcgggtgcgtgaaggtgcagggcagcactgccgcgtcgcctgcctccgcgctcacctcgggtggcacctgcatggaccagcgctgcgctggcgagctgtgcacctctgtgttgagcaagttctccgtagtatctattttagttctcacaaatgagcctgtcgggagaacccacgccaagcaggccagcagccagatggacttttccatgctgtgagcatctgaacaccccaggccagacccgctctcggccacctccccagt

SEQ ID NO: 13302 - RNA, 2343 nt, Homo sapiens
  source 1..2343: mol_type = other RNA
gctgggattacaggcatgagccaccacgcccagcctctgtatctcacttctaaccctttgcatattctgtgtcctctgcctagaacacccctcttcctttcctaatccacacttgtccttatctttccaggttagaatgcatctctgtcttcccacaagcattgcccaacccccaggctggcccagcagcctctctgaccatccacagtgctccgtgctgccctcctcacacctcatcacaccctgcctgtcacattctaggctctgtcccagctcctggcccatcctagactcccaaccaatgaaaccaaggctcagaaaggttacgtgacctgtacaaagctgcagagattagaaagccaggtttgtctgacttcaggtcattctggggctggatatgggtgagaacctggagccgtgtctccagccatgcacacgccgtggagcagcacgagatgccggtacgacacttggctcatcaagctcgctgcttccaggaatgactccatgcagttcttgtgcttggcatccatgaccttcagcagcacctctgtctttcgggcctccccatccaccacctcatggcgacagccccggtaaatcttggtgaaggacccatggcccaggttctcatgccactccaggctgtcagcagggatcttgtgaaatgtcatctgactcagctggtattgggattggggctgaaccaaggatgatgtgggtgggctgtgacctctctggaccacgatcaggttggacttttctttgggtctggggatacagcaggaagtgagggtcactgccaccccatctacgtgcagccccccatcccagcaggttgccaggagctctcgaagactgctgtggggtcggctgaggccaaccagaaggaaggttcctgtggggctgcgccggatgaggcagcccttataatcaggaccaagggggttctggacacagacagtgaggaggaagctgtcaaagtcctgggggctgcggcggagaacataggagccaggacgtgagcccccagtcttgagcttgttgatggcaaagtccagagtgatggggccgtggcactgctcggccacttcctccagcagcctcggcggtgccacctccttgcagaagaagtgctgggagtccgtggtcagccggaagtagccgtccacgagcgccacgaacgacagagcctcgggcagccctgggaactcggcctctaaaatctggttgtctgtcctggtaacagtgaccaggcggtgctctccggccgggccaacgcgcggggcctgcttgatgctaatgtctacgatttctggaaagtcgcagaagggctggaggacctcctgttctccctgggtccaggcgatgccgccgtcaccagccacgcggagcagccccagcccgtcgtggccaccaagggccccagggaggcccacgtggaaggtctcggcggccccggctggatccagccgctccaggtccatgatgtacttggccatgagcgagtgccggtctgcctggcaggcggccacgcggcgcagggctctgcgcaccgtcctccgaatacgcctccgcgtcacgaagctcaggccctggatcaggtcgcgcaggcttgggggtaggcaggccttgtagctgacagtcttcagcagctctcccggccgctgggcctgctctcgcgccatccgggccaggtccaacacggccaggctgagacactcaccctgctccttgagactgaggcccacggggaggcgcccactcaccaggtcactgcggtgctgggcaaagaggtgctccaggactggcaggtcaaggatagcactggccaaatccttgcgtagcccgaagcggtggcacttctccagcccaaaccaattggggaagtaaaagcgaatcctgtacagcaggacttgggtgctggcatcctccacggagaagatgtggctcggggggaaccagcaggacaggtcctccgtggccagagcaaagagggagtggtacacaggcaggatgccgctggccttggcagcctgcacgcacaggtcctcagccaagtggtccccaaaggagaaagataggcgctgggggggcccggggccccgagcgggcagcagcacatgcagggcaccagcctccgtggacaagaggctgcatgaacgctgagggatcaggggcgtctcttcacttggaggtgccatgagtgcaacttgcctagcgggcagggaccctggactttcgaagggcgggcagagccgggaggcagcgagaggaaagtcccactcggctccttcctgtgtgggccccttggtttcctgagccactgtcatttaccgaaag

SEQ ID NO: 13303 - RNA, 11068 nt, Homo sapiens
  source 1..11068: mol_type = other RNA
gctgggattacaggcatgagccaccacgcccagccttcagtctgtttttgttcaaactgtggagctgcagattaaagttattccattttagggaaaatgtccaccatacatcctacttgcaaagactatcctctctgtcaaacctgtgagccaattctgaccttctaacagaaaaagtctgattttatttttccattcaaatcaatgtggttaatatgtatcctgtgtcaaccatctcactttcagtttaaattcttctttatttctttttttagagttaaggtctcgctctgttgccaggctggagtgccataatgtgattatggctcactgtaacctcgaactccagagttcaagtgatcctcttgcttcagcctctggagtagctgggtctacaggcgcatatcaccatgcccagctaatttttatttttattttattatttatttatttattttgagatgtagtctcgctctgtcacccaggctggagtgcaatggcatgatcttggctcactgcaacctctgcctccagggttcaagcgattgtccttcctcagcctcctgagtagctgggactacaggcatgctccaccacgcccggctaatttttgtatttttagtagagacagggttttgccatgttggccaggctggtgttgaactcctgacctcagatgatctacctgcctcggcctcccagagtgctgggattacaggcgtgagccaccgcgcccggcccatgcccagctaatttttaaaattattttttgtagatacgggatcttgctatgttgcccaagctggtctcaaactcctggcctcaagccatcctcccacttcagcctttcaaaacactgggattataggcatgagccactgtgtctcacctgaagttgaattatttttaaaaatttttattattttttcctttttaatatatatttatatattttacaatataacatgtcaatgaatttgaattcttaaatgaagaaggcacagaactgagccacagggctgcccctgtgaactttctcaaagaagctctccaggctttgctctttcaaggacttcctcaagcagagcattctcaagtggcccttttatttgttttttacagcgcagagcaaggagccagagtaggattcagaatgagggaggggaggcaactgggaaagtggaagttgggaaggacagctgtcaggcctgtggcttcttaggcccaccaatataaggaggggaacatatggagaaggcggctctggaaactgattactttaaaactatctgtgtccacctaccttctagaaagtcttcatgtccttgtaggggagtgcaaaccctcgtgtgaaggcctctgacaccaagtgtgagaagccattgatggagccattactgcttccttcgttgtagcagaagggatggggagaggagcaggcaggagcgggggtaggtaagttgtggctttggtgccttgaaggtgaggaaatttctatttgaaggcttcagttttcttcatgaagaattttttttttttttttgtccactgaggggtgggggaaggtgagatatttgaggaaggtggagaaaatataaaagagtcaatacaaataatcaaaactagtagctagaatgaatactagctaggcagagctgagggtccagttaagataggtggtcatgaattcaaatctacatcaatctgctcagctgtgtgattttctttagcaatattaaagctcttgtttgtttgatggttgtggatttggtaaaatgctgatctttcccctatattgagaaaaatgtgagtaatcacaaagaggcccgataataattatgagaaatttatcaaggcccttccagtgttcctctgcataaggtggctttggatggccagacatttacatagcacatagtggctttcttttgtttctcatattcctggtgaattgaactacgatttcttctcctaagcataaatacctgcagaccttagttacagtcatccctgtgaacaagggtgtgggtagaaagggtgaggaatgtctgtctttcctatcaccaggtaaatgggatcttgatgcttggcatggggtcccaagagcttgccattacccatgtgtattatcaaaaaatgagatactgccaccgtcaaagaaaagatcagggccgggtgtagtggctcacacctgtaatcccagcactctgggaggccgaggtgggcggatcacaaggtcaggagatcgaaaccatcctggctaacacaatgaaaccccgtctttactaaaaatacaaaaaatttgccaggcgtggtggcaggtgcctgtagtcccaactgctcgggaggctggggcaggagaatggcgtgaacctgggaggcagagcttgcagtgagccaagatcgtgccactacactccagcctgggcgacagagcaagactccgtctcaaaaaaaaagaaaagatcagaaactctctggacgataggcaaaggttgtaaaccaatgtatcctctttcttaaaatctgatttaaagccttcttccctgtcctgacatgcactgggagaaggacagaatgagttggagggggctagggaaattttggcttataactctcttgagaaatgtctttttaaaaattgtctcggccaggcgcggtggctcatgcctgtaatcccagcactctgggaggccgaggcaggcggatcatgaggtcaggagatcgagaccatcctggctaacactaaaaatactctactgtctctactaaaaatacaaaaaattagtgcagtgagccgaaattgtgccactgcactccagcctgggcgacagagcaagactctgtctcaaaaaaaaaaaaaaaaaattgtctcaagctggaatattgcccgcatatcatggtatgggatatgctatatatcagtaaaatctaagattcagccaataaaatcagtctgtctaacactgtcactctaaaagtccccaaatcaccacagccatggaaggatggttttcccatggtaacagactatatcaagtttacatatatatatatatatattttttttttttaagatggagtctcgctctgttgcccaggctggagtgcagtggcgcaatctcggcttactgcaagctctgcctcctgggttcacatcattctcctgcctcagcctcccgagtagctgggactacaggcgcccgccaccacacccggctaatttttgtatttttagtagagacggggtttcaccatgttagccaggatggtttcgatctcctgacctcatgatccacctgccttggcctcccaaagtgctgggattacaggcgtgagccaccgtgcccgacttatttatttatttattttttgagacggtgtcttgctctgtcatccaggctggagtgcagtggcacgatctcggctcacttcaacctctgcatcccgggttcaaatgattttcctgcctcagcctcctgggtagctaggactacaggcatcccccaccacgcccaactaatttttgtatttttagtagaggcggggtttcaccatgttggccaggctggtctcaaactcctaacgtctagtgatccacctgcctcagcctcccaaagtgctgggattacaggcatgagccatcatgtccggcctcaagttatattttaatagcatacaggatacatactcgtactcagaatgtgagttcaaggatcagtggcacaaataggggaaatgacctcaagttccaaatgttaatgtagttctattagagtgtctgagtggggagaaatcatttcttgaattttgcagggcaagcataagtgctttgactcatttttgtacgcctcacagcgtgcttgtaagccatgtctccagggccatacactcattgtaagtgcccctaataataataaagcaaaggatctgctgcaactcaaaggaaataggaagtgctttaagttccacattccaaagtcagggctagagaggcaggctggatttcctgctgatgtggattgcctgctgttggtttgggccattctaggtataaggtaatgttttagattactgctgggttcttctgggcctggcaacataaagaacaaatctaatcaatgcatcagctgctatggctcattcaccttcctgaagtgttgtgtggccacagcctgcaagaatatgacctggaaatccccaggtagggccctcgggtgtgctcagatccctcatgcccacccatccacccctctgcattctaacatttcagtggttatgttcaggcaaagtgtcttctgctcatgcttgggaggaagagttcccttaacctccctgtggctcattgtccctgaggataccagggctctctcagcctggctgcatgatgacagagggacaccattatcagagaaaccagggctgatgagcagctctaggtcagagaggccgaatgctacctggacatgaagagagaggtcccagcagaccccctggggacaggttcaaattaggttccagcttccccttcctggtgtcaggagttactcatcttgatttacttatcttgcaaaggagccaaggtatcctgccgtacctgcctattgccttctgtctcttccacaactcccatgtctcttttcggtttctgctccacttctcatgggctacttggagtaggaagtaggtctcaataataaaaaactaaataaaacaaaaacatcatctgatttgcctccagctctgccacagactatttggccctagaacaatcccttccctttcctgatactcctctgtaaaatagcctggatcagtagctttcatattacattctgtgaagctgccaggagccggaggggttccccagatacccggagaggctgcagtggaaagacaggctaagctgactccacccccaacacccagcgcccaccagagtagctgccttttacctgttttatatattgtttttccacacagagcttctttgaagaaagagtcctgaggctacaaaatttgaaaactgctggaataaacgatcgccaaggccccttccagtctgagacgcttggtcttctgaagcccagctcaagtttttcctcctccagaaagcctttcttgttacccagtcctgggtacttgagctccaacaataatgatgatggcaggcatatggtgccgtccgtgagccatccgatgcctgcatgtgtgcataagctgtctccccagctagaaggtgagctctttgagggtggtgttcaatttttcttccacacctctgtccccttgtaataccatatgcaaagtaggtgttcaataaacatgttgatgccacctggtgtcatgagctctcacatgggataaaacttccctaccaggaagtttgggaaggaggaaccagcctttggtctgcttaacgctccacagagagacttgtccttaaaaagctggggaccctaacctgggaagcagcttcagactcatacacttcccaaagggcaggtctgagttcctgccttgattggatttggcttcacctcttctgcccctcagtacctcttctggtggggcctcttatacactgtggctgtagaagaggcacggtcctgaagcctgggaatcaggtcagctaggacgccccagggccagcagacatctcagccagattccagagggaggcacgggggagatggagaggaactcctgggtttttttggaatacagctctctcaggaagtggaggcccaaagagggtggctggattcagtcagagacaccagagaaagcagattggaggagggtgctagcggtgaaagaaggcaggtagccaaagggaaactggaggttgtagtggtggaatgaaaccgctctgccatttagtggctaagtgaccctgaggtcagttcatcttacttagtctcaatgtctttacctataaattgggtgtcaaaagaacctgaccaatgtcaggctaccctgtagtgaagtagtgagatagattccaaggagactaaaatgtgcagagatggaaaggattattactgtttattaacacaggaaagcacaggagcctgcttccaaagagggactgtcccgtaattgagagatgctccaaggctgaccatcctccttctcctgctgcacacccagcagccatctatggctggatttggagaatttctggtcaaaccggtgagtatgaggagagcagggcagttggggagagaggtcccagcccaattctgcccagagaagctcccaaaagagagggaagtgtcctgatgaagagcccatgaaaggggtgagacccaggaggctgtggagattgctgcgggctcctctggtcagtaaggaaccctgacaagatccctaggatgggggtcccttagtctcactgaagttcttgtaacttgggatgggggccaggtcagcctcctctgatacccgaagctacacatctggccttccccacttctagaggaggggtcttagatggtgctgtgggagcagacaagccctcagcaggtcgcaagcaggtcccctccaaaacccctcctgctggaatcctccagatgtgaggagtaggagcagacagatcaaggctgggacatctggcagggtttaacatccacagctggagggtgagacctctccctgtggatctggagaaataccttcgggctccagcctattgctgcccttgccttgtcatccatgacagggttccgcgccctgtccagcctccccgggtccccctcagctgctatagcctgacgtgtgagtgctgggcctgcgcagccaaacatctggcaggtctggctggctattgggcagcaccacagggctgccatcccctggcccccctcggcccttccaggacaagctgctgtgatgggaagcgggcaatgatgggtcatacactgtctccctcagcgccagccacagggtgtcccgcttcccattgagctggcctcgctcaaggactggctgcccagtgtcatccaggtcatctggggacacacccacggaatctggtacacgggcactgggctcagaggtgcttaggcaggtctcatcagagacgctgagcccctccagggtgctggctgaggaacagaagccatcaggaggatctgcagccttggccttaggagagtgggctggggcttctggtgaggctggcaggggctcagcctcctccccttgggagtcctgcctggcccgggttttggggctggggccagcctgcttatagggggaggaggtctgcagggcagggcactggctgaagactgcctggtggtccagcagcagctcccttggggaggcaggggctggtgggggccgggaacagcacggaccatcatggagctgcagatcctcagagagtactgagggccggtgggacagcttgctggtggctgtgctggtgtcaaagctggggctccgacgccgtgccaggggctgtagctcatattgctctgagcaggacccgggcatccctcccactgaccctggtcgtgggcggcctgccttctccccaccagggtccccagtaccagcatcccatggcaggtgggcacagggccagaggatctgcccacagttcttctctggcccgaagaaacagcagagagattggaagaagaagctggcaaagccacaactgacgcatttgaccatcatgaggatgatgcccagcttgcgatagagcagcactgtggcaggcagcatgagcacgcctgccgcaaacagggctgcagcccccacggctgtggcgcagctggtctggcgcagagagaaggccacacggctcaggcggtcagggtgtgggcacaggtgataggagatgcagtagttgacagtgaagtctactgagaggcccactgaggcagagagaaacagggcctcggcagtgttgagctgccactcgaggagaaccaggagtcctacagtgagcagcacggtgcctgccacagctgccacggagaataggctgaggggaacattccaggtgcccaggagcagtgtggcaaaggccagcgccaaagccaggcccagcaccacagcaggctcagtgctcaggctgtgctgcaggctatacagctctagacggctagtgaaccaaccacggcggaggcctggaggtgccatgcccagctccgctgccagccagtggctgacctcattgtagaagagctgggtctggttgtagtccggactgttccggaagttggtctggaattgtaggaccagggcggccaggctgccatgggcatcaaagcggagtcccaggtcctgggtgccatcggggccttgctccagagccatcattttcaggcagtgcaggaaaaactggggggcccaggggaagtccgagtggccgcagcagaggtcaggccccaggcgggcgcagctggggctctccatccagcgctggagggtctccacgaaacacagcgtgggccagccttcctgcagggtgtcgaagaagctctgattccgggcccggtgacagagtgccagcagccagcgctgggcctcagggccgctggccgagaaggcagggtccctcaccaggctgctgttgctacgagggtccagagggtcgccagtgtccacaggcaggacgccccacaccaaaaccacgggcatgtggccgccctcgccctgcggcagctgctcgaacaggaacagctggcgatactccgcgtcgaagcgctcgaaggggtggctgggccggaagacctggccgccgggcggcggcagcgtgggcagccgcaggcgggggctgactccggcgatgtaggcgccccctgccgccagtgctgcgaaccagcagatccagatgtagcggaacttgatgacgccgcagggcagcaggcgctggaagagcagacgcgaggtgccagccgccgccctccgcaggccgcggagccgccggtgcagcgccagcagtagccgccggggcgcgctgccctcccaccggccccgcgcccggcgcgcacagccgcgcgccaggtagcgctcgtggagcacggcggaggcgggcagccagaccagcgtgagcgccaggtgcaccagcacagccgtgcccatgaagagggcgaggcagcgaacggccggcaggcggctcaggtagctggcatagaaggccgcgctcgtggtgaggccggagaccagcagcaggtagccgaagtggtgcatggtgcggcccacgcgctgcgccagcccccccgacggcagctggctcttgctaaggcgccacaggtcgaagaagatgagcgtgtggttggcgcagacgctgctcagcaggaggagggctgccagattgacgaaggggaagtaggccatgcggaaggccacctggtaaaggaagaaggccaccagcagtgagcccagcacccccagcagcaccatgagcgtgaggaagagtgagcgcaggtacagggccatgccgaagaagatggcaaccagagccagcaaggggtacaccgtgtcctggaccaggaagtgcctcagcagctcctgcttgaggcccaggtccatgccagtgacagaggtgtagttgtcagcaagcccccagggggtggccagccggtccaggtagatgtccatgagggaagcaccctttggggtgggcaggaagagcaggctgtacttgagggaaggcacctggtagtcagtggtctggggactcagaaagtccctgtcaagcagaaagtgcaggagttggtagatggcactactctgggagcacttggtgggaacctgggcacagcgtggggacttgttctgcccaggtcccagacaagagggcaccaaggcgccactgtggtagtagagggcacaggtccgaagcagggccagtgtgcgggctgcgtcagcttgggtagtgtccaggcaggaggagcggttggagagcacagccagatagttgcccagggaccagctggggcagcactggttggctgctgtccgctggcacagagccccgaagctggtatgggagcggatctggtcctgttccatgcgacacatggaatggatggcatgcaggttccataggctgcccgaggaggtggacatgaacaccagctttgcatagctcttctcaggggggccacagaagaagttctcttgccttctgtcctccaggggctccaccattctccgaggccggacagcgctctcctgggcactgcctctgggtgcaggcctcagagtgttgtgggagctcgagctgttcagctcaaggtctggggaaaggaaaagcagcttcctggggcctgtgagggcttgtagtgctctccagaccactaacttgctcccaatgtctgtgtcccgtggctcaaagcccagcaaaggcttggagaagtcgggcagccgggcccccaacagtccagccagggtgcagaggaagatgacagccagacacagcatcagcacggccactggccactcagcaatcagctgggaatagctctttggcatctggaaggctcgttcctgcctgacgctgaccacatggtgctgcacagcgggtggcttccaggtcccatcgcgctgtgagggggctggagaagggctgaggctggagccgtgggagcagagagctgcccgatccccaagtcctggcagggaactgcccccctggtattcctgcagtgcccggggataggtgaagtgggcaggggccaaggggctggatggacccacaggctggagggtggaagttgttggtgggggtcctgaagagctggaagggtcctccagggggcagctgtggagggagcagcttctctctgggcttgcctcagggggcacagccttggtctgggtgctgtccggggagccgccgtctggggccaagggctccccctcgggccgttgctccccttccggacccgggccgggagccggaccgctgccgccgctgctgctgctgctgtcaccgtccatgcccgtgggcggcaccgctgtccgggcgctggtgctgaagccgcggcggcggcggcggcggcggcggtggcggcggcagcggcggcggggtgctcgtgcgcat

SEQ ID NO: 13304 - RNA, 2078 nt, Homo sapiens
  source 1..2078: mol_type = other RNA
gctgggattacaggcatgagccaccacgcccagccttctttatttttaagatggggtctcgctctactgtccaggctgcagctgagttttagctgaccaaactacttctctgttgtggcaaaggcctgtgcaaatggccatttaacactgttgttctgtcatcttccccatctcaacctgcttttgttgtttcctatcaagatacacttagcaaaacccccaaagacatccagagcttctgaggtacctctgtgtacctcagtttttctccctgtgctgtgagagccatgctgtctgccactctgtgggctcacaagtataacttactactgtaagtataagtagtactatgttccatacaatgagaagacttggaaataaatagaaaatgtgatcacggctcacacctagaaatttacataaagtgctcagacttcaacaagtggccctggggagggagaaggctgagaggtaggaagagatggtgttgggctgggctagagtctctgaaggtagggattttcattctgtcctttggcttcatctcttccactgaagcagcagcactggccgggggtaagggaatgagcttcgctgggctgagtcttcacatccaggcctcacagtgctcagcccggggcctgggtctcccccagtcccactctactgcttgttccccactccatcaaggtcccagaaagtctgtttgtcaatcagcaagggatcccagtcccaaagtgattttaagatcaaatctaagatcaaagtacccagttatccaagcagcagtgtgattacacctttcaatctgtgaaaaggggtcacgttgatcacttcttgataggagctcatgggtgcccttgggtagctcccaaatgaaaacttggctgaagtgactttacaaatggccagttgtgcctacaggctggacagatggtggggggcccctggggtgagcgacggtccaatgccttcaataaggttgttccattgattatagtcttctttcaggtcgaggtgcttctgcaggaaggccaacatggcccgtaccataacctcctgcccttcataggggtccaggctcccacgggtttcagtggagaagaatttaccaatcaagttgccagtcacaaaagcaaagtcagtttgactccgatgaacagaaccaagaacggttatgatcctagactgttcatgctgggcacatatcttcttcatcaaattgacactctccattgtctggaatttctcagtattgataaagaacacaggtcctcgggccttggggtaaaagtcacgttccagaggaaacatccaagcatccagagccaccgcacaccgaaattgggtctccttggccaaagccagaatagctgtggcccctccaaatgaatgtcccatcacagccacacggctcatgtcaatgttgcccttcaaagtcatcagatccaagccaccaggcaagatgttgaagacagtctgcccagcagtgacctcttgcaggatcttcaacacccgtaaacactcgcttacccgctgatgcacctggggattccgaacatgaaattccttctccccttcctcaactcgacggaaagggatccattcctcctgcagcgattcattggtgggctggttctcttctggggcctgcttgcagaaataggtggttgccgctgaccggtccctgtgctctggcacagcaaccacaaagccacgtgaggccagctccatgcagaaggctgaatacaaagtcccaccgccaggttgaacagcaagcccccgcagcgcttattaaactgcaggtactcggccaggccagtgcagtactcatagcggggaatccacaggggctgctccatggtctcctctgccttttggcaggggtagaagagtcgaaagaagctcccctggagattctgaccctccatcacatccccacagcctacgaggtggggtcctgtgacaggtggaaagcccacagactggttgacccccatttcatcaccgggtgaatcaaatgacttgccggagctgaacttgctggccagtcaagctgattcctcagaagcagcccc

SEQ ID NO: 13305 - RNA, 2302 nt, Homo sapiens
  source 1..2302: mol_type = other RNA
gctgggattacaggcatgagccaccacgcccagccttctttatttttaagatggggtctcgctctactgtccaggctgcagctgagttttagctgaccaaactacttctctgttgtggcaaaggcctgtgcaaatggccatttaacactgttgttctgtcatcttccccatctcaacctgcttttgttgtttcctatcaagatacacttagcaaaacccccaaagacatccagagcttctgaggtacctctgtgtacctcagtttttctccctgtgctgtgagagccatgctgtctgccactctgtgggctcacaagtataacttactactgtaagtataagtagtactatgttccatacaatgagaagacttggaaataaatagaaaatgtgatcacggctcacacctagaaatttacataaagtgctcagacttcaacaagtggccctggggagggagaaggctgagaggtaggaagagatggtgttgggctgggctagagtctctgaaggtagggattttcattctgtcctttggcttcatctcttccactgaagcagcagcactggccgggggtaagggaatgagcttcgctgggctgagtcttcacatccaggcctcacagtgctcagcccggggcctgggtctcccccagtcccactctactgcttgttccccactccatcaaggtcccagaaagtctgtttgtcaatcagcaagggatcccagtcccaaagtgattttaagatcaaatctaagatcaaagtacccagttatccaagcagcagtgtgattacacctttcaatctgtgaaaaggggtcacgttgatcacttcttgataggagctcatgggtgcccttgggtagctcccaaatgaaaacttggctgaagtgactttacaaatggccagttgtgcctacaggctggacagatggtggggggcccctggggtgagcgacggtccaatgccttcaataaggttgttccattgattatagtcttctttcaggtcgaggtgcttctgcaggaaggccaacatggcccgtaccataacctcctgcccttcataggggtccaggctcccacgggtttcagtggagaagaatttaccaatcaagttgccagtcacaaaagcaaagtcagtttgactccgatgaacagaaccaagaacggttatgatcctagactgttcatgctgggcacatatcttcttcatcaaattgacactctccattgtctggaatttctcagtattgataaagaacacaggtcctcgggccttggggtaaaagtcacgttccagaggaaacatccaagcatccagagccaccgcacaccgaaattgggtctccttggccaaagccagaatagctgtggcccctccaaatgaatgtcccatcacagccacacggctcatgtcaatgttgcccttcaaagtcatcagatccaagccaccaggcaagatgttgaagacagtctgcccagcagtgacctcttgcaggatcttcaacacccgtaaacactcgcttacccgctgatgcacctggggattccgaacatgaaattccttctccccttcctcaactcgacggaaagggatccattcctcctgcagcgattcattggtgggctggttctcttctggggcctgcttgcagaaataggtggttgccgctgaccggtccctgtgctctggcacagcaaccacaaagccacgtgaggccagctccatgcagaaggctgaatacaaagtcccaccgccaggttgaacagcaagcccccgcagcgcttattaaactgcaggtactcggccaggccagtgcagtactcatagcggggaatccacaggggctgctccatggtctcctctgccttttggcaggggtagaagagtcgaaagaagctcccctggagattctgaccctccatcacatccccacagcctacgaggtggggtcctgtgacaggtggaaagcccacagactggttgacccccatttcatcaccgggtgaatcaaatgacttgccggagctgaacttgctggctgagactgatggagcaacagtcatctccgttttagagaggaagaaactgagtcccagagttgtatgatttgcccaaggtcacagagggtgagaggcagagctggcctagaaccgggtctgctgacttcgagtccagggtaatcgcggatcggaaagaaggaatggggacccttccagtcaagctgattcctcagaagcagccccagacgtttaactcgacggaaatgagaaacgacccatgaacccgtggccct

SEQ ID NO: 13306 - RNA, 2183 nt, Homo sapiens
  source 1..2183: mol_type = other RNA
gctgggattacaggcatgagccaccacgcccagccttctttatttttaagatggggtctcgctctactgtccaggctgcagctgagttttagctgaccaaactacttctctgttgtggcaaaggcctgtgcaaatggccatttaacactgttgttctgtcatcttccccatctcaacctgcttttgttgtttcctatcaagatacacttagcaaaacccccaaagacatccagagcttctgaggtacctctgtgtacctcagtttttctccctgtgctgtgagagccatgctgtctgccactctgtgggctcacaagtataacttactactgtaagtataagtagtactatgttccatacaatgagaagacttggaaataaatagaaaatgtgatcacggctcacacctagaaatttacataaagtgctcagacttcaacaagtggccctggggagggagaaggctgagaggtaggaagagatggtgttgggctgggctagagtctctgaaggtagggattttcattctgtcctttggcttcatctcttccactgaagcagcagcactggccgggggtaagggaatgagcttcgctgggctgagtcttcacatccaggcctcacagtgctcagcccggggcctgggtctcccccagtcccactctactgcttgttccccactccatcaaggtcccagaaagtctgtttgtcaatcagcaagggatcccagtcccaaagtgattttaagatcaaatctaagatcaaagtacccagttatccaagcagcagtgtgattacacctttcaatctgtgaaaaggggtcacgttgatcacttcttgataggagctcatgggtgcccttgggtagctcccaaatgaaaacttggctgaagtgactttacaaatggccagttgtgcctacaggctggacagatggtggggggcccctggggtgagcgacggtccaatgccttcaataaggttgttccattgattatagtcttctttcaggtcgaggtgcttctgcaggaaggccaacatggcccgtaccataacctcctgcccttcataggggtccaggctcccacgggtttcagtggagaagaatttaccaatcaagttgccagtcacaaaagcaaagtcagtttgactccgatgaacagaaccaagaacggttatgatcctagactgttcatgctgggcacatatcttcttcatcaaattgacactctccattgtctggaatttctcagtattgataaagaacacaggtcctcgggccttggggtaaaagtcacgttccagaggaaacatccaagcatccagagccaccgcacaccgaaattgggtctccttggccaaagccagaatagctgtggcccctccaaatgaatgtcccatcacagccacacggctcatgtcaatgttgcccttcaaagtcatcagatccaagccaccaggcaagatgttgaagacagtctgcccagcagtgacctcttgcaggatcttcaacacccgtaaacactcgcttacccgctgatgcacctggggattccgaacatgaaattccttctccccttcctcaactcgacggaaagggatccattcctcctgcagcgattcattggtgggctggttctcttctggggcctgcttgcagaaataggtggttgccgctgaccggtccctgtgctctggcacagcaaccacaaagccacgtgaggccagctccatgcagaaggctgaatacaaagtcctgaaggctcctaggccatgggagaagatgatcaaggggtatccagagtcctttgtcttaaaggggccattccagctaacaggcaggcgacaagatcccaccgccaggttgaacagcaagcccccgcagcgcttattaaactgcaggtactcggccaggccagtgcagtactcatagcggggaatccacaggggctgctccatggtctcctctgccttttggcaggggtagaagagtcgaaagaagctcccctggagattctgaccctccatcacatccccacagcctacgaggtggggtcctgtgacaggtggaaagcccacagactggttgacccccatttcatcaccgggtgaatcaaatgacttgccggagctgaacttgctggccagtcaagctgattcctcagaagcagccccagacgttt

SEQ ID NO: 13307 - RNA, 2408 nt, Homo sapiens
  source 1..2408: mol_type = other RNA
gctgggattacaggcatgagccaccacgcccagccttctttatttttaagatggggtctcgctctactgtccaggctgcagctgagttttagctgaccaaactacttctctgttgtggcaaaggcctgtgcaaatggccatttaacactgttgttctgtcatcttccccatctcaacctgcttttgttgtttcctatcaagatacacttagcaaaacccccaaagacatccagagcttctgaggtacctctgtgtacctcagtttttctccctgtgctgtgagagccatgctgtctgccactctgtgggctcacaagtataacttactactgtaagtataagtagtactatgttccatacaatgagaagacttggaaataaatagaaaatgtgatcacggctcacacctagaaatttacataaagtgctcagacttcaacaagtggccctggggagggagaaggctgagaggtaggaagagatggtgttgggctgggctagagtctctgaaggtagggattttcattctgtcctttggcttcatctcttccactgaagcagcagcactggccgggggtaagggaatgagcttcgctgggctgagtcttcacatccaggcctcacagtgctcagcccggggcctgggtctcccccagtcccactctactgcttgttccccactccatcaaggtcccagaaagtctgtttgtcaatcagcaagggatcccagtcccaaagtgattttaagatcaaatctaagatcaaagtacccagttatccaagcagcagtgtgattacacctttcaatctgtgaaaaggggtcacgttgatcacttcttgataggagctcatgggtgcccttgggtagctcccaaatgaaaacttggctgaagtgactttacaaatggccagttgtgcctacaggctggacagatggtggggggcccctggggtgagcgacggtccaatgccttcaataaggttgttccattgattatagtcttctttcaggtcgaggtgcttctgcaggaaggccaacatggcccgtaccataacctcctgcccttcataggggtccaggctcccacgggtttcagtggagaagaatttaccaatcaagttgccagtcacaaaagcaaagtcagtttgactccgatgaacagaaccaagaacggttatgatcctagactgttcatgctgggcacatatcttcttcatcaaattgacactctccattgtctggaatttctcagtattgataaagaacacaggtcctcgggccttggggtaaaagtcacgttccagaggaaacatccaagcatccagagccaccgcacaccgaaattgggtctccttggccaaagccagaatagctgtggcccctccaaatgaatgtcccatcacagccacacggctcatgtcaatgttgcccttcaaagtcatcagatccaagccaccaggcaagatgttgaagacagtctgcccagcagtgacctcttgcaggatcttcaacacccgtaaacactcgcttacccgctgatgcacctggggattccgaacatgaaattccttctccccttcctcaactcgacggaaagggatccattcctcctgcagcgattcattggtgggctggttctcttctggggcctgcttgcagaaataggtggttgccgctgaccggtccctgtgctctggcacagcaaccacaaagccacgtgaggccagctccatgcagaaggctgaatacaaagtcctgaaggctcctaggccatgggagaagatgatcaaggggtatccagagtcctttgtcttaaaggggccattccagctaacaggcaggcgacaagatcccaccgccaggttgaacagcaagcccccgcagcgcttattaaactgcaggtactcggccaggccagtgcagtactcatagcggggaatccacaggggctgctccatggtctcctctgccttttggcaggggtagaagagtcgaaagaagctcccctggagattctgaccctccatcacatccccacagcctacgaggtggggtcctgtgacaggtggaaagcccacagactggttgacccccatttcatcaccgggtgaatcaaatgacttgccggagctgaacttgctggctgagactgatggagcaacagtcatctccgttttagagaggaagaaactgagtcccagagttgtatgatttgcccaaggtcacagagggtgagaggcagagctggcctagaaccgggtctgctgacttcgagtccagggtaatcgcggatcggaaagaaggaatggggacccttccagtcaagctgattcctcagaagcagccccagacgtttaactcgacggaaatgagaaacgacccatgaacccgtggccctttggtcgtc

SEQ ID NO: 13308 - RNA, 2342 nt, Homo sapiens
  source 1..2342: mol_type = other RNA
gctgggattacaggcatgagccaccacgcccagccttctttatttttaagatggggtctcgctctactgtccaggctgcagctgagttttagctgaccaaactacttctctgttgtggcaaaggcctgtgcaaatggccatttaacactgttgttctgtcatcttccccatctcaacctgcttttgttgtttcctatcaagatacacttagcaaaacccccaaagacatccagagcttctgaggtacctctgtgtacctcagtttttctccctgtgctgtgagagccatgctgtctgccactctgtgggctcacaagtataacttactactgtaagtataagtagtactatgttccatacaatgagaagacttggaaataaatagaaaatgtgatcacggctcacacctagaaatttacataaagtgctcagacttcaacaagtggccctggggagggagaaggctgagaggtaggaagagatggtgttgggctgggctagagtctctgaaggtagggattttcattctgtcctttggcttcatctcttccactgaagcagcagcactggccgggggtaagggaatgagcttcgctgggctgagtcttcacatccaggcctcacagtgctcagcccggggcctgggtctcccccagtcccactctactgcttgttccccactccatcaaggtcccagaaagtctgtttgtcaatcagcaagggatcccagtcccaaagtgattttaagatcaaatctaagatcaaagtacccagttatccaagcagcagtgtgattacacctttcaatctgtgaaaaggggtcacgttgatcacttcttgataggagctcatgggtgcccttgggtagctcccaaatgaaaacttggctgaagtgactttacaaatggccagttgtgcctacaggctggacagatggtggggggcccctggggtgagcgacggtccaatgccttcaataaggttgttccattgattatagtcttctttcaggtcgaggtgcttctgcaggaaggccaacatggcccgtaccataacctcctgcccttcataggggtccaggctcccacgggtttcagtggagaagaatttaccaatcaagttgccagtcacaaaagcaaagtcagtttgactccgatgaacagaaccaagaacggttatgatcctagactgttcatgctgggcacatatcttcttcatcaaattgacactctccattgtctggaatttctcagtattgataaagaacacaggtcctcgggccttggggtaaaagtcacgttccagaggaaacatccaagcatccagagccaccgcacaccgaaattgggtctccttggccaaagccagaatagctgtggcccctccaaatgaatgtcccatcacagccacacggctcatgtcaatgttgcccttcaaagtcatcagatccaagccaccaggcaagatgttgaagacagtctgcccagcagtgacctcttgcaggatcttcaacacccgtaaacactcgcttacccgctgatgcacctggggattccgaacatgaaattccttctccccttcctcaactcgacggaaagggatccattcctcctgcagcgattcattggtgggctggttctcttctggggcctgcttgcagaaataggtggttgccgctgaccggtccctgtgctctggcacagcaaccacaaagccacgtgaggccagctccatgcagaaggctgaatacaaagtcctgaaggctcctaggccatgggagaagatgatcaaggggtatccagagtcctttgtcttaaaggggccattccagctaacaggcaggcgacaagatcccaccgccaggttgaacagcaagcccccgcagcgcttattaaactgcaggtactcggccaggccagtgcagtactcatagcggggaatccacaggggctgctccatggtctcctctgccttttggcaggggtagaagagtcgaaagaagctcccctggagattctgaccctccatcacatccccacagcctacgaggtggggtcctgtgacaggtggaaagcccacagactggttgacccccatttcatcaccgggtgaatcaaatgacttgccggagctgaacttgctggctggatgggggaacacagaacagcagccgcttgctggtttcctctcggcttcctgttgccagtcaagctgattcctcagaagcagccccagacgtttaactcgacggaaatgagaaacgacccatgaacccgtggccctttggtcgtcgtagtttccaaggctcaaaatggacgcttggaagcacttctcgttcctca

SEQ ID NO: 13309 - RNA, 2030 nt, Homo sapiens
  source 1..2030: mol_type = other RNA
gctgggattacaggcatgagccaccacgcccagccttctttatttttaagatggggtctcgctctactgtccaggctgcagctgagttttagctgaccaaactacttctctgttgtggcaaaggcctgtgcaaatggccatttaacactgttgttctgtcatcttccccatctcaacctgcttttgttgtttcctatcaagatacacttagcaaaacccccaaagacatccagagcttctgaggtacctctgtgtacctcagtttttctccctgtgctgtgagagccatgctgtctgccactctgtgggctcacaagtataacttactactgtaagtataagtagtactatgttccatacaatgagaagacttggaaataaatagaaaatgtgatcacggctcacacctagaaatttacataaagtgctcagacttcaacaagtggccctggggagggagaaggctgagaggtaggaagagatggtgttgggctgggctagagtctctgaaggtagggattttcattctgtcctttggcttcatctcttccactgaagcagcagcactggccgggggtaagggaatgagcttcgctgggctgagtcttcacatccaggcctcacagtgctcagcccggggcctgggtctcccccagtcccactctactgcttgttccccactccatcaaggtcccagaaagtctgtttgtcaatcagcaagggatcccagtcccaaagtgattttaagatcaaatctaagatcaaagtacccagttatccaagcagcagtgtgattacacctttcaatctgtgaaaaggggtcacgttgatcacttcttgataggagctcatgggtgcccttgggtagctcccaaatgaaaacttggctgaagtgactttacaaatggccagttgtgcctacaggctggacagatggtggggggcccctggggtgagcgacggtccaatgccttcaataaggttgttccattgattatagtcttctttcaggtcgaggtgcttctgcaggaaggccaacatggcccgtaccataacctcctgcccttcataggggtccaggctcccacgggtttcagtggagaagaatttaccaatcaagttgccagtcacaaaagcaaagtcagtttgactccgatgaacagaaccaagaacggttatgatcctagactgttcatgctgggcacatatcttcttcatcaaattgacactctccattgtctggaatttctcagtattgataaagaacacaggtcctcgggccttggggtaaaagtcacgttccagaggaaacatccaagcatccagagccaccgcacaccgaaattgggtctccttggccaaagccagaatagctgtggcccctccaaatgaatgtcccatcacagccacacggctcatgtcaatgttgcccttcaaagtcatcagatccaagccaccaggcaagatgttgaagacagtctgcccagcagtgacctcttgcaggatcttcaacacccgtaaacactcgcttacccgctgatgcacctggggattccgaacatgaaattccttctccccttcctcaactcgacggaaagggatccattcctcctgcagcgattcattggtgggctggttctcttctggggcctgcttgcagaaataggtggttgccgctgaccggtccctgtgctctggcacagcaaccacaaagccacgtgaggccagctccatgcagaaggctgaatacaaagtcctggagattctgaccctccatcacatccccacagcctacgaggtggggtcctgtgacaggtggaaagcccacagactggttgacccccatttcatcaccgggtgaatcaaatgacttgccggagctgaacttgctggccagtcaagctgattcctcagaagcagccccagacgtttaactcgacggaaatgagaaacgacccatgaacccgtggccctttggtcgtcgtagtttccaaggctcaaaatggacgcttggaagcacttctcgttcc

SEQ ID NO: 13310 - RNA, 2148 nt, Homo sapiens
  source 1..2148: mol_type = other RNA
gctgggattacaggcatgagccaccacgcccagccttctttatttttaagatggggtctcgctctactgtccaggctgcagctgagttttagctgaccaaactacttctctgttgtggcaaaggcctgtgcaaatggccatttaacactgttgttctgtcatcttccccatctcaacctgcttttgttgtttcctatcaagatacacttagcaaaacccccaaagacatccagagcttctgaggtacctctgtgtacctcagtttttctccctgtgctgtgagagccatgctgtctgccactctgtgggctcacaagtataacttactactgtaagtataagtagtactatgttccatacaatgagaagacttggaaataaatagaaaatgtgatcacggctcacacctagaaatttacataaagtgctcagacttcaacaagtggccctggggagggagaaggctgagaggtaggaagagatggtgttgggctgggctagagtctctgaaggtagggattttcattctgtcctttggcttcatctcttccactgaagcagcagcactggccgggggtaagggaatgagcttcgctgggctgagtcttcacatccaggcctcacagtgctcagcccggggcctgggtctcccccagtcccactctactgcttgttccccactccatcaaggtcccagaaagtctgtttgtcaatcagcaagggatcccagtcccaaagtgattttaagatcaaatctaagatcaaagtacccagttatccaagcagcagtgtgattacacctttcaatctgtgaaaaggggtcacgttgatcacttcttgataggagctcatgggtgcccttgggtagctcccaaatgaaaacttggctgaagtgactttacaaatggccagttgtgcctacaggctggacagatggtggggggcccctggggtgagcgacggtccaatgccttcaataaggttgttccattgattatagtcttctttcaggtcgaggtgcttctgcaggaaggccaacatggcccgtaccataacctcctgcccttcataggggtccaggctcccacgggtttcagtggagaagaatttaccaatcaagttgccagtcacaaaagcaaagtcagtttgactccgatgaacagaaccaagaacggttatgatcctagactgttcatgctgggcacatatcttcttcatcaaattgacactctccattgtctggaatttctcagtattgataaagaacacaggtcctcgggccttggggtaaaagtcacgttccagaggaaacatccaagcatccagagccaccgcacaccgaaattgggtctccttggccaaagccagaatagctgtggcccctccaaatgaatgtcccatcacagccacacggctcatgtcaatgttgcccttcaaagtcatcagatccaagccaccaggcaagatgttgaagacagtctgcccagcagtgacctcttgcaggatcttcaacacccgtaaacactcgcttacccgctgatgcacctggggattccgaacatgaaattccttctccccttcctcaactcgacggaaagggatccattcctcctgcagcgattcattggtgggctggttctcttctggggcctgcttgcagaaataggtggttgccgctgaccggtccctgtgctctggcacagcaaccacaaagccacgtgaggccagctccatgcagaaggctgaatacaaagtcctggagattctgaccctccatcacatccccacagcctacgaggtggggtcctgtgacaggtggaaagcccacagactggttgacccccatttcatcaccgggtgaatcaaatgacttgccggagctgaacttgctggctgagactgatggagcaacagtcatctccgttttagagaggaagaaactgagtcccagagttgtatgatttgcccaaggtcacagagggtgagaggcagagctggcctagaaccgggtctgctgacttcgagtccagggtaatcgcggatcggaaagaaggaatggggacccttccagtcaagctgattcctcagaagcagccccagacgtttaactcgacggaaatgagaaacgacccatgaacccgtggccct

SEQ ID NO: 13311 - RNA, 2569 nt, Homo sapiens
  source 1..2569: mol_type = other RNA
gctgggattacaggcatgagccaccacgcccagccttctttatttttaagatggggtctcgctctactgtccaggctgcagctgagttttagctgaccaaactacttctctgttgtggcaaaggcctgtgcaaatggccatttaacactgttgttctgtcatcttccccatctcaacctgcttttgttgtttcctatcaagatacacttagcaaaacccccaaagacatccagagcttctgaggtacctctgtgtacctcagtttttctccctgtgctgtgagagccatgctgtctgccactctgtgggctcacaagtataacttactactgtaagtataagtagtactatgttccatacaatgagaagacttggaaataaatagaaaatgtgatcacggctcacacctagaaatttacataaagtgctcagacttcaacaagtggccctggggagggagaaggctgagaggtaggaagagatggtgttgggctgggctagagtctctgaaggtagggattttcattctgtcctttggcttcatctcttccactgaagcagcagcactggccgggggtaagggaatgagcttcgctgggctgagtcttcacatccaggcctcacagtgctcagcccggggcctgggtctcccccagtcccactctactgcttgttccccactccatcaaggtcccagaaagtctgtttgtcaatcagcaagggatcccagtcccaaagtgattttaagatcaaatctaagatcaaagtacccagttatccaagcagcagtgtgattacacctttcaatctgtgaaaaggggtcacgttgatcacttcttgataggagctcatgggtgcccttgggtagctcccaaatgaaaacttggctgaagtgactttacaaatggccagttgtgcctacaggctggacagatggtggggggcccctggggtgagcgacggtccaatgccttcaataaggttgttccattgattatagtcttctttcaggtcgaggtgcttctgcaggaaggccaacatggcccgtaccataacctcctgcccttcataggggtccaggctcccacgggtttcagtggagaagaatttaccaatcaagttgccagtcacaaaagcaaagtcagtttgactccgatgaacagaaccaagaacggttatgatcctagactgttcatgctgggcacatatcttcttcatcaaattgacactctccattgtctggaatttctcagtattgataaagaacacaggtcctcgggccttggggtaaaagtcacgttccagaggaaacatccaagcatccagagccaccgcacaccgaaattgggtctccttggccaaagccagaatagctgtggcccctccaaatgaatgtcccatcacagccacacggctcatgtcaatgttgcccttcaaagtcatcagatccaagccaccaggcaagatgttgaagacagtctgcccagcagtgacctcttgcaggatcttcaacacccgtaaacactcgcttacccgctgatgcacctggggattccgaacatgaaattccttctccccttcctcaactcgacggaaagggatccattcctcctgcagcgattcattggtgggctggttctcttctggggcctgcttgcagaaataggtggttgccgctgaccggtccctgtgctctggcacagcaaccacaaagccacgtgaggccagctccatgcagaaggctgaatacaaagtcctttctaacttcatctccatatttactctccacttcctgccatgggctacagttacaggagtctatgttcctgctcctctagcagatgcgatttcctcgatttgttaatcttggtatgtcccaccttcctctcatgccaaggggctggcacagagcaggtgctccacagatgtctgctgaatgaatgagaacctagcacagcacagcccttgtattcattcaataaatacttatggctaaacaactactttccaggcactgtcctagaagccagagcaatagaagacagatgtggtctctgccttcagaaggcttacaatctagtgaagaagacaggcattaaagaataattacacaagtaattaattcattacaattatgttaaatgctgagaagtatagattgtcttatgaaagcacattctggaaaaattaacctaatataatataggtgtcaagatgggtgtccctaggacaatgacatccaaactaagatcttaaaggtaatctggaattagcaggaaaagacggagaggggcaagaggaagagaagagcagaacggtgaatagtccaggcaaaaagatcagccacaaagcatagcacagatgaagacagcgagggaggaaataacccagtgcctttcagtaagtgaaagaaggccattttgtctggagagctacactggggcaaatagcaaggaacaggcctagaaactttgtcttggacctgcattgaggtaagaccatgaaaagaactgaattaggttcaaagagctattaaattttttttttctgagatgcagttttgttcttg

SEQ ID NO: 13312 - RNA, 2724 nt, Homo sapiens
  source 1..2724: mol_type = other RNA
gctgggattacaggcatgagccaccacgcccagctaaaagaagcttttctgatagtaactttgttttcccattctggagtttatggcagtatgaaaaagactgaatttataagcagaagatctgtttttgaaatccggggacctgtatttcacaatggctttgatgtgttttgattgtgcacctttagacaacttatcagtttcctcatttttatacagcaataaaatagtaacagctacccattaaattctgtacagaagctagggacagacgcaataacacttgcatatctataaaggctttgtaaatgtgggtattatatctaatgtttatgcacatgctgtttgattattttcatttggaattccactccattaaaggaaaagtaacatacgaattcagattcttgtaagtcttcaggcatgaggcctccattgactaagtacattgcctacataatttctcctaacccaaatgaatctccagttaaaccaagctggtggttatgtactgtctccagaggatgccaagcataaagtccttgagtatattcatcttggatcctctgattggacaactgcggtattgagacttcaagttcccccttgaaggccccagacggtacctgtaattttactcaagttttaaatgtatgctctttgttaagaaagagtgacaatgatttgatttattttccgtgactggggttagggatgggggagactctaggaatgtgacttaccagtgaggttctagttttataaatcataggacaagttttgataggcaaatgttggactatagggctgaggttgttttccaccacaacatatagacttctactagcccttgaaggaaaaaacacgagaaaatcagttgggtcagctgagtattcctttacgagtatggaacagacttacataacaattctgcaggtaatggctctggaaaggtcaaccacttagttttggacaactcttttctattctgtataaccactttttcaccaaaatgatactaaataaatatgctataggaagctatattttgacatgactgttttaggcaaagatacactcaccaacttactccacaagagtttctaatcagagaatatcatatggatctatttgaattgctcccatgcttggctgagcccaaaataatttactgtgcatatgtacaccaagtgagaaggttgaggaggtgtcacttgtacatctctttattcttttttttttgtatgtgtgtgttattttcatgtgttttgaaaggctctcttgcttagcttttattttgccattaaagatttttttctgtgctataactgtatttttaagtctggtttgagttcaagaaatccacaaattcacaaaagattaggaataatttgtgaacaaaatgatgcagaaataaaaaatgcattttccaaataactcccttgcagtccttctcgcccaactaccactttctattaagtttcttcttcctactctatgaagtgccatgagctttcaattcattgtattttaagtataagctatacttactaaccttcacgttattctttgctacttaaataagcttgctttcatagttcaattgacgtattgtttaactgatatttttaattggtatattttgatatatattgataattgatagatacataattcatttgagatattttgggtatggagggttggaaggaatcctttcataatttttctacttaaaagaaatcttttttcatttaacagcttttcccatggggatagagttttcatgaataaagcaaagtcattaaatgaggtatatggtacatcttttaagagtcacagaaagaagcaacaacaatttacccaggcagagggtataagtttagaccttggttgcctgatttgtgggacaagttctttaattttttttctttatattttgacttttttttggactctctcctccccttccaggctccaggtcaaatacttgacacctgaatgatgttcaattatttaaaagatggattggccagctcagctcctgtctcagacagactgtctttaaatgtattttcaacatgtcttcagacagttatttttcctctgttcaattttgttcatcttcttacttaaccgttcaagtgctcctatttcctttttaaatgtagtattgagaagtgcaaacattattggaaaagagagtctcactagcataattgtgcattatcttcctcttatatcgccggcctccctgcacccccatgcccacctcctcctcgcgcctccatgccgcctcccactgctccagctccttgcagctgcgagtccagtcactggtcacctttcgtatctcctcactcagagcctggttggccaaacctgcctggtccagctgttctcagagcatggcattcacctgggccaggctggcactcctgaatggggcacaggggatcagtaggcgctcgcccagggggccatgctgccagccctggccctccctgctgctcctcctccagccagatgagggcactctccaggtcttggctgtgctctgcgtccctcagctgctgctgctccagctctccggatctctccaacagctgctccagctccgagaacctcttcttgtactggagaatttccgatccgcggtcctgaacccgctcccagggcacgggaactccttcgtggcgaagcagcaagtggcgaagcagcagc

SEQ ID NO: 13313 - RNA, 5023 nt, Homo sapiens
  source 1..5023: mol_type = other RNA
gctgggattacaggcatgagccaccacgcccagctaattttgtatttttagtagagacggggtttctccatgttggtcaggctggtctcgacctcccgacctcaggtgatctgcccgcctcggcctcccaaagtgctgggattacaggcatgagccaccgcgcccagctgatttatatcttatctatgagaaacaccaaaaactatgagtaagcatcactgagttatcatgtaagaattttttctaagttttagcccaaatttccaggtcaagacaaacccacagagaggtaaaagggtattaggatgggagttcatatttacagcaggaactttacatacatggtctccttgagctcttgcaaccttgtaagataagtattattttcctttcacagatgaataaactgctaccctttttttaacaagtagatttgactaaaaagaactatgtcaaatattgcttcccattttcttatttcttttttttttttttttgagacagagtcttgctctgttgcccaggctggagtgcagtggcgagatctcggctcactgcaagctctgcctcccgggttcacaccattctcctgcctcagcctcccgagtagctgggactacaggcgcccgccaccacgcccggctaattttctgttttttagtagagacggggtttcaccgtgttagccaggatggtctcgatctcctgacctcgtgatccacctgcctcagcctcccaaagtgctgggattacaggcgtgagccactgagcccagccccattttatttcatttctctaacagcaatgatatatatacatcccatagtatatcctactgatatactagcccctttccccattcaacacctgtgtaatcaggaaataaaacaatgattcgggtttaaagggtatatcatgtgaaactaatgctggggcggtagtctccattcatagttcaaaatacaaattttatccactaaaatggaaacacaaaaaacaactactgaaatgtaaataatataacaacaaaaataacaaaatatcataatacacagggccaaatcacattatatacactcactacacccactctaccctaccttagcccgtaatcaaagggacaggggaaaaaaccaaatgtagcaggaaaggcaatataaagctattaattaattaactggaatttagtttgtaaatgctaaaaccagttctcaaaaattaagacaatgcttttgatcagcagactaaattattacaaataaagataagtacttattgcaaaactacttgaatctttgcatgactaaaatgtaaaataagtggtgacttgaaatcctagagtgaactttatacagaaaaggaatagtctacatgtagacactgagaactcttgggagggggaaaagatttggatatggctatagttttgactttgcaaatgatcaatttttgcggaattagatggaaaagatccggtgctttttatagttcaaacacagacaaatgctgttaagtctccaaaaatttgattagaagttggagtgctgagtgattttaagaacctgaagcaacagcatttctaaacaattcttaaaataaacttgttagccacatcagcgttgtgcattaaatttcacaactcatggagaggaagaaaaaaagtcttgcttaactctaaacatacaagttttagaagaattttaatgaagtgcggctcccagaacaggaaaagccttatgttaaaacaattcagtccttgagtccttggctaacaactagattgaactacctacctgacttggaagtgaagtgtcctggaaaacatattttaaaaattttaacacttttctccccttgtagaaaactttaaatttaaagtctagactatacagaccaaattcaagttaatgactatataaccaaactaagtggcagacagtgcaaaggtgaagaactgaggatttacatactaaaacagaaacagggcagtcattatttaatttttaaaactctcatttaaatttgcaatgttttagccgggcgtggtggctcaagcctgtaatcccagcactttgggagggcaaggcgagtggatctcttgaggtcaggagtttgataccagcctggccaacatggtgaaaccccgtctctactaaaaataaaaaaaaattagtcgggcatggtggcacctgcctgtaattccagctactcaggaagctgaggcacgagaatcgcttgaacccagaaggcggaggttgcagtgagcagagatcactccactgcactccagcctgggtgacaagcaagactccatctcaaaaagaaaattaaataaataaaataaatttgcaatgttttaaatgaatatcacttaaagtagtaatcaacagaagttaggagaacataacaatactctttctcttagaaagtacaacaaaaatataattttttacagttttactctcaaactttcctctgtagtaacatgccttactcacctctacaataggtttgttgtgagaatcttgtaatgtaaaccctggacgttctatgaagcatttttaaacttctagtttataccctactgattcttattcaagtgttttttaaaaaatatttaaacaactattcttcttttcttgccaatatttttataatttccaagaggttttaaggatcttgagagaacatttatttcagaagtatctactactattactagccaagaaaacaaatgtaggtagaggaaagacttaacattttgtcctatatacatcttaatcatcctaacggtaaaaactcacatgaaactttaagatacaagatgatatgagaatctcaacatggaaagctgtcactataactacaagcagtgtacaaacatgcttctacttttacctacataagctgacagatgtttaaaatactgagttaacaaagatcttttagtaaagtgacttaggcaggcttaaactagcaaggattaaggatgaatccttactaattaattggaagatctgagacatattttatatttcattttacaaaatcagaaatacttattttgaaacaagataagacatggtctacctgtcaaaaaactaccactcagaaatatttttcatccacaaagcaggaaaaacataaaatcatttacatttcacattggcaccaaaaaggttaactgccctgccttcttggattagaaaaactaaagctgagtgataagtagttttgcaggcgtttgaacatgcctaagcctttaaatcagcaaaatactttctaaaaattctgattacaaaagtaatacatacttataaaaaattcgaacagaacaaaatgaaaaaagtagaaagtgaaaaggcccctataaaacccctctggggcccctcccccaatccccccctccccgaagagaaaccacatttaacagtttggtgtatatctttccaaatcttttgttctatgcatattaaaaacatacatactttgatctggctcagactatacatagtgttttgccacttgcattttacacttaacatatctttgacatctttccatgtcagtacatgttggctcgatagtattctatcattaaatacgctttcaaaaatggcaaatcactttaaaaaaataattcgcacaagtacgtgtttataactttaaaagaaaatggacagaatcctaaaacacaacaaccaacctctaaaaacaatctctatctttccaccagcatggaacaatttattcctttttcacacaaaacaaattatgtgattggggagattaactctaatctccacatttatatacagaaagctccatttgttaagcctatctgaaaagaataaaaaatccagatgattaattcacttacacttagaaattaaatcagtatactatgaatacacattgtgttcagttatagtatgatgcttcttattcttagtctatggtttcaattaaataacagtaaaaaaaatggataatacagctaataccctgaaaaatcaagaaattcaaagattatattgccaactaaaacactgccatgtacattttttttcctacttggtagcaaatgctaatggaattcaatcctgattacttaaagtcagttcacatcacacattcaatcagggtaataagaacaacataacatgcctactatagagttagattaagacataaaaattttttgcttgaaagtaatgactgtgtagcacatgggacacttgtcaactgcttcagcacattgtttacaagtgactagatgtccacaaggaacaaaaacgatagcaatatttctatccatacagattttgcaaagcttctcctcttgcaggcgccttagctgctcttcagtactaatctctttctgtaatgaagtctgacttgactcatcttgcatactgtctttctgagcattcactagatctgcaaccagaacctcaagtgatttatagttgctcccagatatctgaattttttcctccattattttcttaatgtccttgaaactgaaccccattcgtatagcttcttgtaccataggattttggaagatggtatcatcaattcttctagttagtgatggtgttttctcagtagttcttaccagacactcctcaagtgaatgagttaaatgaatattgtttatatattcttgtcccttctgttctaacagatatttgcaccctggataccatttagcatgttgttcccaagggtcttcactgggcttccaatcagttagccctcctccacagtgaaagcactttactttatcaccttcaccgcgccaggacagccggcccgaactgccccgcggcgatcggctcggtccaaggggagggtcccggaggaggcgcggcccgagccccaatctggaaatgccaactccgctctgcggcttggccccagccacttgggccgggcgtccctcgatgagcgccacgccggctccgggcgccgccaaggtcccgccacctagcgcgcgcacatgcgcagtgagcacctc

SEQ ID NO: 13314 - RNA, 5041 nt, Homo sapiens
  source 1..5041: mol_type = other RNA
gctgggattacaggcatgagccaccacgcccagctaattttgtatttttagtagagacggggtttctccatgttggtcaggctggtctcgacctcccgacctcaggtgatctgcccgcctcggcctcccaaagtgctgggattacaggcatgagccaccgcgcccagctgatttatatcttatctatgagaaacaccaaaaactatgagtaagcatcactgagttatcatgtaagaattttttctaagttttagcccaaatttccaggtcaagacaaacccacagagaggtaaaagggtattaggatgggagttcatatttacagcaggaactttacatacatggtctccttgagctcttgcaaccttgtaagataagtattattttcctttcacagatgaataaactgctaccctttttttaacaagtagatttgactaaaaagaactatgtcaaatattgcttcccattttcttatttcttttttttttttttttgagacagagtcttgctctgttgcccaggctggagtgcagtggcgagatctcggctcactgcaagctctgcctcccgggttcacaccattctcctgcctcagcctcccgagtagctgggactacaggcgcccgccaccacgcccggctaattttctgttttttagtagagacggggtttcaccgtgttagccaggatggtctcgatctcctgacctcgtgatccacctgcctcagcctcccaaagtgctgggattacaggcgtgagccactgagcccagccccattttatttcatttctctaacagcaatgatatatatacatcccatagtatatcctactgatatactagcccctttccccattcaacacctgtgtaatcaggaaataaaacaatgattcgggtttaaagggtatatcatgtgaaactaatgctggggcggtagtctccattcatagttcaaaatacaaattttatccactaaaatggaaacacaaaaaacaactactgaaatgtaaataatataacaacaaaaataacaaaatatcataatacacagggccaaatcacattatatacactcactacacccactctaccctaccttagcccgtaatcaaagggacaggggaaaaaaccaaatgtagcaggaaaggcaatataaagctattaattaattaactggaatttagtttgtaaatgctaaaaccagttctcaaaaattaagacaatgcttttgatcagcagactaaattattacaaataaagataagtacttattgcaaaactacttgaatctttgcatgactaaaatgtaaaataagtggtgacttgaaatcctagagtgaactttatacagaaaaggaatagtctacatgtagacactgagaactcttgggagggggaaaagatttggatatggctatagttttgactttgcaaatgatcaatttttgcggaattagatggaaaagatccggtgctttttatagttcaaacacagacaaatgctgttaagtctccaaaaatttgattagaagttggagtgctgagtgattttaagaacctgaagcaacagcatttctaaacaattcttaaaataaacttgttagccacatcagcgttgtgcattaaatttcacaactcatggagaggaagaaaaaaagtcttgcttaactctaaacatacaagttttagaagaattttaatgaagtgcggctcccagaacaggaaaagccttatgttaaaacaattcagtccttgagtccttggctaacaactagattgaactacctacctgacttggaagtgaagtgtcctggaaaacatattttaaaaattttaacacttttctccccttgtagaaaactttaaatttaaagtctagactatacagaccaaattcaagttaatgactatataaccaaactaagtggcagacagtgcaaaggtgaagaactgaggatttacatactaaaacagaaacagggcagtcattatttaatttttaaaactctcatttaaatttgcaatgttttagccgggcgtggtggctcaagcctgtaatcccagcactttgggagggcaaggcgagtggatctcttgaggtcaggagtttgataccagcctggccaacatggtgaaaccccgtctctactaaaaataaaaaaaaattagtcgggcatggtggcacctgcctgtaattccagctactcaggaagctgaggcacgagaatcgcttgaacccagaaggcggaggttgcagtgagcagagatcactccactgcactccagcctgggtgacaagcaagactccatctcaaaaagaaaattaaataaataaaataaatttgcaatgttttaaatgaatatcacttaaagtagtaatcaacagaagttaggagaacataacaatactctttctcttagaaagtacaacaaaaatataattttttacagttttactctcaaactttcctctgtagtaacatgccttactcacctctacaataggtttgttgtgagaatcttgtaatgtaaaccctggacgttctatgaagcatttttaaacttctagtttataccctactgattcttattcaagtgttttttaaaaaatatttaaacaactattcttcttttcttgccaatatttttataatttccaagaggttttaaggatcttgagagaacatttatttcagaagtatctactactattactagccaagaaaacaaatgtaggtagaggaaagacttaacattttgtcctatatacatcttaatcatcctaacggtaaaaactcacatgaaactttaagatacaagatgatatgagaatctcaacatggaaagctgtcactataactacaagcagtgtacaaacatgcttctacttttacctacataagctgacagatgtttaaaatactgagttaacaaagatcttttagtaaagtgacttaggcaggcttaaactagcaaggattaaggatgaatccttactaattaattggaagatctgagacatattttatatttcattttacaaaatcagaaatacttattttgaaacaagataagacatggtctacctgtcaaaaaactaccactcagaaatatttttcatccacaaagcaggaaaaacataaaatcatttacatttcacattggcaccaaaaaggttaactgccctgccttcttggattagaaaaactaaagctgagtgataagtagttttgcaggcgtttgaacatgcctaagcctttaaatcagcaaaatactttctaaaaattctgattacaaaagtaatacatacttataaaaaattcgaacagaacaaaatgaaaaaagtagaaagtgaaaaggcccctataaaacccctctggggcccctcccccaatccccccctccccgaagagaaaccacatttaacagtttggtgtatatctttccaaatcttttgttctatgcatattaaaaacatacatactttgatctggctcagactatacatagtgttttgccacttgcattttacacttaacatatctttgacatctttccatgtcagtacatgttggctcgatagtattctatcattaaatacgctttcaaaaatggcaaatcactttaaaaaaataattcgcacaagtacgtgtttataactttaaaagaaaatggacagaatcctaaaacacaacaaccaacctctaaaaacaatctctatctttccaccagcatggaacaatttattcctttttcacacaaaacaaattatgtgattggggagattaactctaatctccacatttatatacagaaagctccatttgttaagcctatctgaaaagaataaaaaatccagatgattaattcacttacacttagaaattaaatcagtatactatgaatacacattgtgttcagttatagtatgatgcttcttattcttagtctatggtttcaattaaataacagtaaaaaaaatggataatacagctaataccctgaaaaatcaagaaattcaaagattatattgccaactaaaacactgccatgtacattttttttcctacttggtagcaaatgctaatggaattcaatcctgattacttaaagtcagttcacatcacacattcaatcagggtaataagaacaacataacatgcctactatagagttagattaagacataaaaattttttgcttgaaagtaatgactgtgtagcacatgggacacttgtcaactgcttcagcacattgtttacaagtgactagatgtccacaaggaacaaaaacgatagcaatatttctatccatacagattttgcaaagcttctcctcttgcaggcgccttagctgctcttcagtactaatctctttctgtaatgaagtctgacttgactcatcttgcatactgtctttctgagcattcactagatctgcaaccagaacctcaagtgatttatagttgctcccagatatctgaattttttcctccattattttcttaatgtccttgaaactgaaccccattcgtatagcttcttgtaccataggattttggaagatggtatcatcaattcttctagttagtgatggtgttttctcagtagttcttaccagacactcctcaagtgaatgagttaaatgaatattgtttatatattcttgtcccttctgttctaacagatatttgcaccctggataccatttagcatgttgttcccaagggtcttcactgggcttccaatcagttagccctcctccacagtgaaagcactttactttatcaccttcaccgcgccaggacagccggcccgaactgccccgcggcgatcggctcggtccaaggggagggtcccggaggaggcgcggcccgagccccaatctggaaatgccaactccgctctgcggcttggccccagcctaggtgaaggaaacggaagtcccttcgtctccctcacgcgcctctaccggccggcccatcccctggagaaacccggagtcgtgaaacccgaagtgtgtccacgtcagggcctc

SEQ ID NO: 13315 - RNA, 5801 nt, Homo sapiens
  source 1..5801: mol_type = other RNA
gctgggattacaggcatgagccaccacgcccagctaattttgtatttttagtagagacggggtttctccatgttggtcaggctggtctcgacctcccgacctcaggtgatctgcccgcctcggcctcccaaagtgctgggattacaggcatgagccaccgcgcccagctgatttatatcttatctatgagaaacaccaaaaactatgagtaagcatcactgagttatcatgtaagaattttttctaagttttagcccaaatttccaggtcaagacaaacccacagagaggtaaaagggtattaggatgggagttcatatttacagcaggaactttacatacatggtctccttgagctcttgcaaccttgtaagataagtattattttcctttcacagatgaataaactgctaccctttttttaacaagtagatttgactaaaaagaactatgtcaaatattgcttcccattttcttatttcttttttttttttttttgagacagagtcttgctctgttgcccaggctggagtgcagtggcgagatctcggctcactgcaagctctgcctcccgggttcacaccattctcctgcctcagcctcccgagtagctgggactacaggcgcccgccaccacgcccggctaattttctgttttttagtagagacggggtttcaccgtgttagccaggatggtctcgatctcctgacctcgtgatccacctgcctcagcctcccaaagtgctgggattacaggcgtgagccactgagcccagccccattttatttcatttctctaacagcaatgatatatatacatcccatagtatatcctactgatatactagcccctttccccattcaacacctgtgtaatcaggaaataaaacaatgattcgggtttaaagggtatatcatgtgaaactaatgctggggcggtagtctccattcatagttcaaaatacaaattttatccactaaaatggaaacacaaaaaacaactactgaaatgtaaataatataacaacaaaaataacaaaatatcataatacacagggccaaatcacattatatacactcactacacccactctaccctaccttagcccgtaatcaaagggacaggggaaaaaaccaaatgtagcaggaaaggcaatataaagctattaattaattaactggaatttagtttgtaaatgctaaaaccagttctcaaaaattaagacaatgcttttgatcagcagactaaattattacaaataaagataagtacttattgcaaaactacttgaatctttgcatgactaaaatgtaaaataagtggtgacttgaaatcctagagtgaactttatacagaaaaggaatagtctacatgtagacactgagaactcttgggagggggaaaagatttggatatggctatagttttgactttgcaaatgatcaatttttgcggaattagatggaaaagatccggtgctttttatagttcaaacacagacaaatgctgttaagtctccaaaaatttgattagaagttggagtgctgagtgattttaagaacctgaagcaacagcatttctaaacaattcttaaaataaacttgttagccacatcagcgttgtgcattaaatttcacaactcatggagaggaagaaaaaaagtcttgcttaactctaaacatacaagttttagaagaattttaatgaagtgcggctcccagaacaggaaaagccttatgttaaaacaattcagtccttgagtccttggctaacaactagattgaactacctacctgacttggaagtgaagtgtcctggaaaacatattttaaaaattttaacacttttctccccttgtagaaaactttaaatttaaagtctagactatacagaccaaattcaagttaatgactatataaccaaactaagtggcagacagtgcaaaggtgaagaactgaggatttacatactaaaacagaaacagggcagtcattatttaatttttaaaactctcatttaaatttgcaatgttttagccgggcgtggtggctcaagcctgtaatcccagcactttgggagggcaaggcgagtggatctcttgaggtcaggagtttgataccagcctggccaacatggtgaaaccccgtctctactaaaaataaaaaaaaattagtcgggcatggtggcacctgcctgtaattccagctactcaggaagctgaggcacgagaatcgcttgaacccagaaggcggaggttgcagtgagcagagatcactccactgcactccagcctgggtgacaagcaagactccatctcaaaaagaaaattaaataaataaaataaatttgcaatgttttaaatgaatatcacttaaagtagtaatcaacagaagttaggagaacataacaatactctttctcttagaaagtacaacaaaaatataattttttacagttttactctcaaactttcctctgtagtaacatgccttactcacctctacaataggtttgttgtgagaatcttgtaatgtaaaccctggacgttctatgaagcatttttaaacttctagtttataccctactgattcttattcaagtgttttttaaaaaatatttaaacaactattcttcttttcttgccaatatttttataatttccaagaggttttaaggatcttgagagaacatttatttcagaagtatctactactattactagccaagaaaacaaatgtaggtagaggaaagacttaacattttgtcctatatacatcttaatcatcctaacggtaaaaactcacatgaaactttaagatacaagatgatatgagaatctcaacatggaaagctgtcactataactacaagcagtgtacaaacatgcttctacttttacctacataagctgacagatgtttaaaatactgagttaacaaagatcttttagtaaagtgacttaggcaggcttaaactagcaaggattaaggatgaatccttactaattaattggaagatctgagacatattttatatttcattttacaaaatcagaaatacttattttgaaacaagataagacatggtctacctgtcaaaaaactaccactcagaaatatttttcatccacaaagcaggaaaaacataaaatcatttacatttcacattggcaccaaaaaggttaactgccctgccttcttggattagaaaaactaaagctgagtgataagtagttttgcaggcgtttgaacatgcctaagcctttaaatcagcaaaatactttctaaaaattctgattacaaaagtaatacatacttataaaaaattcgaacagaacaaaatgaaaaaagtagaaagtgaaaaggcccctataaaacccctctggggcccctcccccaatccccccctccccgaagagaaaccacatttaacagtttggtgtatatctttccaaatcttttgttctatgcatattaaaaacatacatactttgatctggctcagactatacatagtgttttgccacttgcattttacacttaacatatctttgacatctttccatgtcagtacatgttggctcgatagtattctatcattaaatacgctttcaaaaatggcaaatcactttaaaaaaataattcgcacaagtacgtgtttataactttaaaagaaaatggacagaatcctaaaacacaacaaccaacctctaaaaacaatctctatctttccaccagcatggaacaatttattcctttttcacacaaaacaaattatgtgattggggagattaactctaatctccacatttatatacagaaagctccatttgttaagcctatctgaaaagaataaaaaatccagatgattaattcacttacacttagaaattaaatcagtatactatgaatacacattgtgttcagttatagtatgatgcttcttattcttagtctatggtttcaattaaataacagtaaaaaaaatggataatacagctaataccctgaaaaatcaagaaattcaaagattatattgccaactaaaacactgccatgtacattttttttcctacttggtagcaaatgctaatggaattcaatcctgattacttaaagtcagttcacatcacacattcaatcagggtaataagaacaacataacatgcctactatagagttagattaagacataaaaattttttgcttgaaagtaatgactgtgtagcacatgggacacttgtcaactgcttcagcacattgtttacaagtgactagatgtccacaaggaacaaaaacgatagcaatatttctatccatacagattttgcaaagcttctcctcttgcaggcgccttagctgctcttcagtactaatctctttctgtaatgaagtctgacttgactcatcttgcatactgtctttctgagcattcactagatctgcaaccagaacctcaagtgatttatagttgctcccagatatctgaattttttcctccattattttcttaatgtccttgaaactgaaccccattcgtatagcttcttgtaccataggattttggaagatggtatcatcaattcttctagttagtgatggtgttttctcagtagttcttaccagacactcctcaagtgaatgagttaaatgaatattgtttatatattcttgtcccttctgttctaacagatatttgcaccctggataccatttagcatgttgttcccaagggtcttcactgggcttccaatcagttagccctcctccacagtgaaagcactttactttatcaccttcacctaaagcataaaatccagctcttgcaagctgctccttgttaactgagtatatccatgtcccaaaagtaaagatccgtgcttcataatctgccatggatggatttcttggaagatttgttgaatttgggaaattcctatcagaactcacagcatcagattcacttcgaatattaagattccggcccaaaacaaagaagcaattaggaaagtgtcgcctgtgttctgaccaggcacgatcacaaggttcccaatttttcagttttccaccacaacaaaagcactgcacttggtcaccaatacctgtgtagtagagtccagcacttgctaactctcttggggttaggtgagcatagtctggccagttctgaaaggactttaatctagcttcttcactatacatggcagggttcctcgggtatatggtgtctgatatatctacaacctgcccagttctcaaaagatagtctgcatgtgtctcagatggcctgtctaaggcaaaatgatctctgcttcccagatagttttcaactttgtactgaccattctggataccagaatttgtagactgcgtggcactattttcaagataaaagccgttgataaatctgcaatttggggatactttcctgtgtcttccaactgctgagtctccatattgccatctatctacagctgcatgacaactaaagcaccgcacggtatctccttcaccagtataaagaaaccctgctcgtgccagtgttgatgctgaaacaggactaccacttggaaaattagcaaaagtttttaatctattaaactcttctacaaattcttcttccttattgatgtctgcaggtacacaagttttagatccttcaaaactgttaaaagtcatcttctcttgaaaataggacttgtccaccttttcacttgggccgggcgtccctcgatgagcgccacgccggctccgggcgccgccaaggtcccgccacctccccgaaccggatgggggcagtaag

SEQ ID NO: 13316 - RNA, 5928 nt, Homo sapiens
  source 1..5928: mol_type = other RNA
gctgggattacaggcatgagccaccacgcccagctaattttgtatttttagtagagacggggtttctccatgttggtcaggctggtctcgacctcccgacctcaggtgatctgcccgcctcggcctcccaaagtgctgggattacaggcatgagccaccgcgcccagctgatttatatcttatctatgagaaacaccaaaaactatgagtaagcatcactgagttatcatgtaagaattttttctaagttttagcccaaatttccaggtcaagacaaacccacagagaggtaaaagggtattaggatgggagttcatatttacagcaggaactttacatacatggtctccttgagctcttgcaaccttgtaagataagtattattttcctttcacagatgaataaactgctaccctttttttaacaagtagatttgactaaaaagaactatgtcaaatattgcttcccattttcttatttcttttttttttttttttgagacagagtcttgctctgttgcccaggctggagtgcagtggcgagatctcggctcactgcaagctctgcctcccgggttcacaccattctcctgcctcagcctcccgagtagctgggactacaggcgcccgccaccacgcccggctaattttctgttttttagtagagacggggtttcaccgtgttagccaggatggtctcgatctcctgacctcgtgatccacctgcctcagcctcccaaagtgctgggattacaggcgtgagccactgagcccagccccattttatttcatttctctaacagcaatgatatatatacatcccatagtatatcctactgatatactagcccctttccccattcaacacctgtgtaatcaggaaataaaacaatgattcgggtttaaagggtatatcatgtgaaactaatgctggggcggtagtctccattcatagttcaaaatacaaattttatccactaaaatggaaacacaaaaaacaactactgaaatgtaaataatataacaacaaaaataacaaaatatcataatacacagggccaaatcacattatatacactcactacacccactctaccctaccttagcccgtaatcaaagggacaggggaaaaaaccaaatgtagcaggaaaggcaatataaagctattaattaattaactggaatttagtttgtaaatgctaaaaccagttctcaaaaattaagacaatgcttttgatcagcagactaaattattacaaataaagataagtacttattgcaaaactacttgaatctttgcatgactaaaatgtaaaataagtggtgacttgaaatcctagagtgaactttatacagaaaaggaatagtctacatgtagacactgagaactcttgggagggggaaaagatttggatatggctatagttttgactttgcaaatgatcaatttttgcggaattagatggaaaagatccggtgctttttatagttcaaacacagacaaatgctgttaagtctccaaaaatttgattagaagttggagtgctgagtgattttaagaacctgaagcaacagcatttctaaacaattcttaaaataaacttgttagccacatcagcgttgtgcattaaatttcacaactcatggagaggaagaaaaaaagtcttgcttaactctaaacatacaagttttagaagaattttaatgaagtgcggctcccagaacaggaaaagccttatgttaaaacaattcagtccttgagtccttggctaacaactagattgaactacctacctgacttggaagtgaagtgtcctggaaaacatattttaaaaattttaacacttttctccccttgtagaaaactttaaatttaaagtctagactatacagaccaaattcaagttaatgactatataaccaaactaagtggcagacagtgcaaaggtgaagaactgaggatttacatactaaaacagaaacagggcagtcattatttaatttttaaaactctcatttaaatttgcaatgttttagccgggcgtggtggctcaagcctgtaatcccagcactttgggagggcaaggcgagtggatctcttgaggtcaggagtttgataccagcctggccaacatggtgaaaccccgtctctactaaaaataaaaaaaaattagtcgggcatggtggcacctgcctgtaattccagctactcaggaagctgaggcacgagaatcgcttgaacccagaaggcggaggttgcagtgagcagagatcactccactgcactccagcctgggtgacaagcaagactccatctcaaaaagaaaattaaataaataaaataaatttgcaatgttttaaatgaatatcacttaaagtagtaatcaacagaagttaggagaacataacaatactctttctcttagaaagtacaacaaaaatataattttttacagttttactctcaaactttcctctgtagtaacatgccttactcacctctacaataggtttgttgtgagaatcttgtaatgtaaaccctggacgttctatgaagcatttttaaacttctagtttataccctactgattcttattcaagtgttttttaaaaaatatttaaacaactattcttcttttcttgccaatatttttataatttccaagaggttttaaggatcttgagagaacatttatttcagaagtatctactactattactagccaagaaaacaaatgtaggtagaggaaagacttaacattttgtcctatatacatcttaatcatcctaacggtaaaaactcacatgaaactttaagatacaagatgatatgagaatctcaacatggaaagctgtcactataactacaagcagtgtacaaacatgcttctacttttacctacataagctgacagatgtttaaaatactgagttaacaaagatcttttagtaaagtgacttaggcaggcttaaactagcaaggattaaggatgaatccttactaattaattggaagatctgagacatattttatatttcattttacaaaatcagaaatacttattttgaaacaagataagacatggtctacctgtcaaaaaactaccactcagaaatatttttcatccacaaagcaggaaaaacataaaatcatttacatttcacattggcaccaaaaaggttaactgccctgccttcttggattagaaaaactaaagctgagtgataagtagttttgcaggcgtttgaacatgcctaagcctttaaatcagcaaaatactttctaaaaattctgattacaaaagtaatacatacttataaaaaattcgaacagaacaaaatgaaaaaagtagaaagtgaaaaggcccctataaaacccctctggggcccctcccccaatccccccctccccgaagagaaaccacatttaacagtttggtgtatatctttccaaatcttttgttctatgcatattaaaaacatacatactttgatctggctcagactatacatagtgttttgccacttgcattttacacttaacatatctttgacatctttccatgtcagtacatgttggctcgatagtattctatcattaaatacgctttcaaaaatggcaaatcactttaaaaaaataattcgcacaagtacgtgtttataactttaaaagaaaatggacagaatcctaaaacacaacaaccaacctctaaaaacaatctctatctttccaccagcatggaacaatttattcctttttcacacaaaacaaattatgtgattggggagattaactctaatctccacatttatatacagaaagctccatttgttaagcctatctgaaaagaataaaaaatccagatgattaattcacttacacttagaaattaaatcagtatactatgaatacacattgtgttcagttatagtatgatgcttcttattcttagtctatggtttcaattaaataacagtaaaaaaaatggataatacagctaataccctgaaaaatcaagaaattcaaagattatattgccaactaaaacactgccatgtacattttttttcctacttggtagcaaatgctaatggaattcaatcctgattacttaaagtcagttcacatcacacattcaatcagggtaataagaacaacataacatgcctactatagagttagattaagacataaaaattttttgcttgaaagtaatgactgtgtagcacatgggacacttgtcaactgcttcagcacattgtttacaagtgactagatgtccacaaggaacaaaaacgatagcaatatttctatccatacagattttgcaaagcttctcctcttgcaggcgccttagctgctcttcagtactaatctctttctgtaatgaagtctgacttgactcatcttgcatactgtctttctgagcattcactagatctgcaaccagaacctcaagtgatttatagttgctcccagatatctgaattttttcctccattattttcttaatgtccttgaaactgaaccccattcgtatagcttcttgtaccataggattttggaagatggtatcatcaattcttctagttagtgatggtgttttctcagtagttcttaccagacactcctcaagtgaatgagttaaatgaatattgtttatatattcttgtcccttctgttctaacagatatttgcaccctggataccatttagcatgttgttcccaagggtcttcactgggcttccaatcagttagccctcctccacagtgaaagcactttactttatcaccttcacctaaagcataaaatccagctcttgcaagctgctccttgttaactgagtatatccatgtcccaaaagtaaagatccgtgcttcataatctgccatggatggatttcttggaagatttgttgaatttgggaaattcctatcagaactcacagcatcagattcacttcgaatattaagattccggcccaaaacaaagaagcaattaggaaagtgtcgcctgtgttctgaccaggcacgatcacaaggttcccaatttttcagttttccaccacaacaaaagcactgcacttggtcaccaatacctgtgtagtagagtccagcacttgctaactctcttggggttaggtgagcatagtctggccagttctgaaaggactttaatctagcttcttcactatacatggcagggttcctcgggtatatggtgtctgatatatctacaacctgcccagttctcaaaagatagtctgcatgtgtctcagatggcctgtctaaggcaaaatgatctctgcttcccagatagttttcaactttgtactgaccattctggataccagaatttgtagactgcgtggcactattttcaagataaaagccgttgataaatctgcaatttggggatactttcctgtgtcttccaactgctgagtctccatattgccatctatctacagctgcatgacaactaaagcaccgcacggtatctccttcaccagtataaagaaaccctgctcgtgccagtgttgatgctgaaacaggactaccacttggaaaattagcaaaagtttttaatctattaaactcttctacaaattcttcttccttattgatgtctgcaggtacacaagttttagatccttcaaaactgttaaaagtcatcttctcttgaaaataggacttgtccaccttttcgcgccaggacagccggcccgaactgccccgcggcgatcggctcggtccaaggggagggtcccggaggaggcgcggcccgagccccaatctggaaatgccaactccgctctgcggcttggccccagccacttgggccgggcgtccctcgatgagcgccacgccggctccgggcgccgccaaggtcccgccacctccccgaaccggatgggggcagtaag

SEQ ID NO: 13317 - RNA, 5950 nt, Homo sapiens
  source 1..5950: mol_type = other RNA
gctgggattacaggcatgagccaccacgcccagctaattttgtatttttagtagagacggggtttctccatgttggtcaggctggtctcgacctcccgacctcaggtgatctgcccgcctcggcctcccaaagtgctgggattacaggcatgagccaccgcgcccagctgatttatatcttatctatgagaaacaccaaaaactatgagtaagcatcactgagttatcatgtaagaattttttctaagttttagcccaaatttccaggtcaagacaaacccacagagaggtaaaagggtattaggatgggagttcatatttacagcaggaactttacatacatggtctccttgagctcttgcaaccttgtaagataagtattattttcctttcacagatgaataaactgctaccctttttttaacaagtagatttgactaaaaagaactatgtcaaatattgcttcccattttcttatttcttttttttttttttttgagacagagtcttgctctgttgcccaggctggagtgcagtggcgagatctcggctcactgcaagctctgcctcccgggttcacaccattctcctgcctcagcctcccgagtagctgggactacaggcgcccgccaccacgcccggctaattttctgttttttagtagagacggggtttcaccgtgttagccaggatggtctcgatctcctgacctcgtgatccacctgcctcagcctcccaaagtgctgggattacaggcgtgagccactgagcccagccccattttatttcatttctctaacagcaatgatatatatacatcccatagtatatcctactgatatactagcccctttccccattcaacacctgtgtaatcaggaaataaaacaatgattcgggtttaaagggtatatcatgtgaaactaatgctggggcggtagtctccattcatagttcaaaatacaaattttatccactaaaatggaaacacaaaaaacaactactgaaatgtaaataatataacaacaaaaataacaaaatatcataatacacagggccaaatcacattatatacactcactacacccactctaccctaccttagcccgtaatcaaagggacaggggaaaaaaccaaatgtagcaggaaaggcaatataaagctattaattaattaactggaatttagtttgtaaatgctaaaaccagttctcaaaaattaagacaatgcttttgatcagcagactaaattattacaaataaagataagtacttattgcaaaactacttgaatctttgcatgactaaaatgtaaaataagtggtgacttgaaatcctagagtgaactttatacagaaaaggaatagtctacatgtagacactgagaactcttgggagggggaaaagatttggatatggctatagttttgactttgcaaatgatcaatttttgcggaattagatggaaaagatccggtgctttttatagttcaaacacagacaaatgctgttaagtctccaaaaatttgattagaagttggagtgctgagtgattttaagaacctgaagcaacagcatttctaaacaattcttaaaataaacttgttagccacatcagcgttgtgcattaaatttcacaactcatggagaggaagaaaaaaagtcttgcttaactctaaacatacaagttttagaagaattttaatgaagtgcggctcccagaacaggaaaagccttatgttaaaacaattcagtccttgagtccttggctaacaactagattgaactacctacctgacttggaagtgaagtgtcctggaaaacatattttaaaaattttaacacttttctccccttgtagaaaactttaaatttaaagtctagactatacagaccaaattcaagttaatgactatataaccaaactaagtggcagacagtgcaaaggtgaagaactgaggatttacatactaaaacagaaacagggcagtcattatttaatttttaaaactctcatttaaatttgcaatgttttagccgggcgtggtggctcaagcctgtaatcccagcactttgggagggcaaggcgagtggatctcttgaggtcaggagtttgataccagcctggccaacatggtgaaaccccgtctctactaaaaataaaaaaaaattagtcgggcatggtggcacctgcctgtaattccagctactcaggaagctgaggcacgagaatcgcttgaacccagaaggcggaggttgcagtgagcagagatcactccactgcactccagcctgggtgacaagcaagactccatctcaaaaagaaaattaaataaataaaataaatttgcaatgttttaaatgaatatcacttaaagtagtaatcaacagaagttaggagaacataacaatactctttctcttagaaagtacaacaaaaatataattttttacagttttactctcaaactttcctctgtagtaacatgccttactcacctctacaataggtttgttgtgagaatcttgtaatgtaaaccctggacgttctatgaagcatttttaaacttctagtttataccctactgattcttattcaagtgttttttaaaaaatatttaaacaactattcttcttttcttgccaatatttttataatttccaagaggttttaaggatcttgagagaacatttatttcagaagtatctactactattactagccaagaaaacaaatgtaggtagaggaaagacttaacattttgtcctatatacatcttaatcatcctaacggtaaaaactcacatgaaactttaagatacaagatgatatgagaatctcaacatggaaagctgtcactataactacaagcagtgtacaaacatgcttctacttttacctacataagctgacagatgtttaaaatactgagttaacaaagatcttttagtaaagtgacttaggcaggcttaaactagcaaggattaaggatgaatccttactaattaattggaagatctgagacatattttatatttcattttacaaaatcagaaatacttattttgaaacaagataagacatggtctacctgtcaaaaaactaccactcagaaatatttttcatccacaaagcaggaaaaacataaaatcatttacatttcacattggcaccaaaaaggttaactgccctgccttcttggattagaaaaactaaagctgagtgataagtagttttgcaggcgtttgaacatgcctaagcctttaaatcagcaaaatactttctaaaaattctgattacaaaagtaatacatacttataaaaaattcgaacagaacaaaatgaaaaaagtagaaagtgaaaaggcccctataaaacccctctggggcccctcccccaatccccccctccccgaagagaaaccacatttaacagtttggtgtatatctttccaaatcttttgttctatgcatattaaaaacatacatactttgatctggctcagactatacatagtgttttgccacttgcattttacacttaacatatctttgacatctttccatgtcagtacatgttggctcgatagtattctatcattaaatacgctttcaaaaatggcaaatcactttaaaaaaataattcgcacaagtacgtgtttataactttaaaagaaaatggacagaatcctaaaacacaacaaccaacctctaaaaacaatctctatctttccaccagcatggaacaatttattcctttttcacacaaaacaaattatgtgattggggagattaactctaatctccacatttatatacagaaagctccatttgttaagcctatctgaaaagaataaaaaatccagatgattaattcacttacacttagaaattaaatcagtatactatgaatacacattgtgttcagttatagtatgatgcttcttattcttagtctatggtttcaattaaataacagtaaaaaaaatggataatacagctaataccctgaaaaatcaagaaattcaaagattatattgccaactaaaacactgccatgtacattttttttcctacttggtagcaaatgctaatggaattcaatcctgattacttaaagtcagttcacatcacacattcaatcagggtaataagaacaacataacatgcctactatagagttagattaagacataaaaattttttgcttgaaagtaatgactgtgtagcacatgggacacttgtcaactgcttcagcacattgtttacaagtgactagatgtccacaaggaacaaaaacgatagcaatatttctatccatacagattttgcaaagcttctcctcttgcaggcgccttagctgctcttcagtactaatctctttctgtaatgaagtctgacttgactcatcttgcatactgtctttctgagcattcactagatctgcaaccagaacctcaagtgatttatagttgctcccagatatctgaattttttcctccattattttcttaatgtccttgaaactgaaccccattcgtatagcttcttgtaccataggattttggaagatggtatcatcaattcttctagttagtgatggtgttttctcagtagttcttaccagacactcctcaagtgaatgagttaaatgaatattgtttatatattcttgtcccttctgttctaacagatatttgcaccctggataccatttagcatgttgttcccaagggtcttcactgggcttccaatcagttagccctcctccacagtgaaagcactttactttatcaccttcacctaaagcataaaatccagctcttgcaagctgctccttgttaactgagtatatccatgtcccaaaagtaaagatccgtgcttcataatctgccatggatggatttcttggaagatttgttgaatttgggaaattcctatcagaactcacagcatcagattcacttcgaatattaagattccggcccaaaacaaagaagcaattaggaaagtgtcgcctgtgttctgaccaggcacgatcacaaggttcccaatttttcagttttccaccacaacaaaagcactgcacttggtcaccaatacctgtgtagtagagtccagcacttgctaactctcttggggttaggtgagcatagtctggccagttctgaaaggactttaatctagcttcttcactatacatggcagggttcctcgggtatatggtgtctgatatatctacaacctgcccagttctcaaaagatagtctgcatgtgtctcagatggcctgtctaaggcaaaatgatctctgcttcccagatagttttcaactttgtactgaccattctggataccagaatttgtagactgcgtggcactattttcaagataaaagccgttgataaatctgcaatttggggatactttcctgtgtcttccaactgctgagtctccatattgccatctatctacagctgcatgacaactaaagcaccgcacggtatctccttcaccagtataaagaaaccctgctcgtgccagtgttgatgctgaaacaggactaccacttggaaaattagcaaaagtttttaatctattaaactcttctacaaattcttcttccttattgatgtctgcaggtacacaagttttagatccttcaaaactgttaaaagtcatcttctcttgaaaataggacttgtccaccttttcgcgccaggacagccggcccgaactgccccgcggcgatcggctcggtccaaggggagggtcccggaggaggcgcggcccgagccccaatctggaaatgccaactccgctctgcggcttggccccagcctaggtgaaggaaacggaagtcccttcgtctccctcacgcgcctctaccggccggcccatcccctggagaaacccggagtcgtgaaacccgaagtgtgtccacgtcagggcctc

SEQ ID NO: 13318 - RNA, 5740 nt, Homo sapiens
  source 1..5740: mol_type = other RNA
gctgggattacaggcatgagccaccacgcccagctaattttgtatttttagtagagacggggtttctccatgttggtcaggctggtctcgacctcccgacctcaggtgatctgcccgcctcggcctcccaaagtgctgggattacaggcatgagccaccgcgcccagctgatttatatcttatctatgagaaacaccaaaaactatgagtaagcatcactgagttatcatgtaagaattttttctaagttttagcccaaatttccaggtcaagacaaacccacagagaggtaaaagggtattaggatgggagttcatatttacagcaggaactttacatacatggtctccttgagctcttgcaaccttgtaagataagtattattttcctttcacagatgaataaactgctaccctttttttaacaagtagatttgactaaaaagaactatgtcaaatattgcttcccattttcttatttcttttttttttttttttgagacagagtcttgctctgttgcccaggctggagtgcagtggcgagatctcggctcactgcaagctctgcctcccgggttcacaccattctcctgcctcagcctcccgagtagctgggactacaggcgcccgccaccacgcccggctaattttctgttttttagtagagacggggtttcaccgtgttagccaggatggtctcgatctcctgacctcgtgatccacctgcctcagcctcccaaagtgctgggattacaggcgtgagccactgagcccagccccattttatttcatttctctaacagcaatgatatatatacatcccatagtatatcctactgatatactagcccctttccccattcaacacctgtgtaatcaggaaataaaacaatgattcgggtttaaagggtatatcatgtgaaactaatgctggggcggtagtctccattcatagttcaaaatacaaattttatccactaaaatggaaacacaaaaaacaactactgaaatgtaaataatataacaacaaaaataacaaaatatcataatacacagggccaaatcacattatatacactcactacacccactctaccctaccttagcccgtaatcaaagggacaggggaaaaaaccaaatgtagcaggaaaggcaatataaagctattaattaattaactggaatttagtttgtaaatgctaaaaccagttctcaaaaattaagacaatgcttttgatcagcagactaaattattacaaataaagataagtacttattgcaaaactacttgaatctttgcatgactaaaatgtaaaataagtggtgacttgaaatcctagagtgaactttatacagaaaaggaatagtctacatgtagacactgagaactcttgggagggggaaaagatttggatatggctatagttttgactttgcaaatgatcaatttttgcggaattagatggaaaagatccggtgctttttatagttcaaacacagacaaatgctgttaagtctccaaaaatttgattagaagttggagtgctgagtgattttaagaacctgaagcaacagcatttctaaacaattcttaaaataaacttgttagccacatcagcgttgtgcattaaatttcacaactcatggagaggaagaaaaaaagtcttgcttaactctaaacatacaagttttagaagaattttaatgaagtgcggctcccagaacaggaaaagccttatgttaaaacaattcagtccttgagtccttggctaacaactagattgaactacctacctgacttggaagtgaagtgtcctggaaaacatattttaaaaattttaacacttttctccccttgtagaaaactttaaatttaaagtctagactatacagaccaaattcaagttaatgactatataaccaaactaagtggcagacagtgcaaaggtgaagaactgaggatttacatactaaaacagaaacagggcagtcattatttaatttttaaaactctcatttaaatttgcaatgttttagccgggcgtggtggctcaagcctgtaatcccagcactttgggagggcaaggcgagtggatctcttgaggtcaggagtttgataccagcctggccaacatggtgaaaccccgtctctactaaaaataaaaaaaaattagtcgggcatggtggcacctgcctgtaattccagctactcaggaagctgaggcacgagaatcgcttgaacccagaaggcggaggttgcagtgagcagagatcactccactgcactccagcctgggtgacaagcaagactccatctcaaaaagaaaattaaataaataaaataaatttgcaatgttttaaatgaatatcacttaaagtagtaatcaacagaagttaggagaacataacaatactctttctcttagaaagtacaacaaaaatataattttttacagttttactctcaaactttcctctgtagtaacatgccttactcacctctacaataggtttgttgtgagaatcttgtaatgtaaaccctggacgttctatgaagcatttttaaacttctagtttataccctactgattcttattcaagtgttttttaaaaaatatttaaacaactattcttcttttcttgccaatatttttataatttccaagaggttttaaggatcttgagagaacatttatttcagaagtatctactactattactagccaagaaaacaaatgtaggtagaggaaagacttaacattttgtcctatatacatcttaatcatcctaacggtaaaaactcacatgaaactttaagatacaagatgatatgagaatctcaacatggaaagctgtcactataactacaagcagtgtacaaacatgcttctacttttacctacataagctgacagatgtttaaaatactgagttaacaaagatcttttagtaaagtgacttaggcaggcttaaactagcaaggattaaggatgaatccttactaattaattggaagatctgagacatattttatatttcattttacaaaatcagaaatacttattttgaaacaagataagacatggtctacctgtcaaaaaactaccactcagaaatatttttcatccacaaagcaggaaaaacataaaatcatttacatttcacattggcaccaaaaaggttaactgccctgccttcttggattagaaaaactaaagctgagtgataagtagttttgcaggcgtttgaacatgcctaagcctttaaatcagcaaaatactttctaaaaattctgattacaaaagtaatacatacttataaaaaattcgaacagaacaaaatgaaaaaagtagaaagtgaaaaggcccctataaaacccctctggggcccctcccccaatccccccctccccgaagagaaaccacatttaacagtttggtgtatatctttccaaatcttttgttctatgcatattaaaaacatacatactttgatctggctcagactatacatagtgttttgccacttgcattttacacttaacatatctttgacatctttccatgtcagtacatgttggctcgatagtattctatcattaaatacgctttcaaaaatggcaaatcactttaaaaaaataattcgcacaagtacgtgtttataactttaaaagaaaatggacagaatcctaaaacacaacaaccaacctctaaaaacaatctctatctttccaccagcatggaacaatttattcctttttcacacaaaacaaattatgtgattggggagattaactctaatctccacatttatatacagaaagctccatttgttaagcctatctgaaaagaataaaaaatccagatgattaattcacttacacttagaaattaaatcagtatactatgaatacacattgtgttcagttatagtatgatgcttcttattcttagtctatggtttcaattaaataacagtaaaaaaaatggataatacagctaataccctgaaaaatcaagaaattcaaagattatattgccaactaaaacactgccatgtacattttttttcctacttggtagcaaatgctaatggaattcaatcctgattacttaaagtcagttcacatcacacattcaatcagggtaataagaacaacataacatgcctactatagagttagattaagacataaaaattttttgcttgaaagtaatgactgtgtagcacatgggacacttgtcaactgcttcagcacattgtttacaagtgactagatgtccacaaggaacaaaaacgatagcaatatttctatccatacagattttgcaaagcttctcctcttgcaggcgccttagctgctcttcagtactaatctctttctgtaatgaagtctgacttgactcatcttgcatactgtctttctgagcattcactagatctgcaaccagaacctcaagtgatttatagttgctcccagatatctgaattttttcctccattattttcttaatgtccttgaaactgaaccccattcgtatagcttcttgtaccataggattttggaagatggtatcatcaattcttctagttagtgatggtgttttctcagtagttcttaccagacactcctcaagtgaatgagttaaatgaatattgtttatatattcttgtcccttctgttctaacagatatttgcaccctggataccatttagcatgttgttcccaagggtcttcactgggcttccaatcagttagccctcctccacagtgaaagcactttactttatcaccttcacctaaagcataaaatccagctcttgcaagctgctccttgttaactgagtatatccatgtcccaaaagtaaagatccgtgcttcataatctgccatggatggatttcttggaagatttgttgaatttgggaaattcctatcagaactcacagcatcagattcacttcgaatattaagattccggcccaaaacaaagaagcaattaggaaagtgtcgcctgtgttctgaccaggcacgatcacaaggttcccaatttttcagttttccaccacaacaaaagcactgcacttggtcaccaatacctgtgtagtagagtccagcacttgctaactctcttggggttaggtgagcatagtctggccagttctgaaaggactttaatctagcttcttcactatacatggcagggttcctcgggtatatggtgtctgatatatctacaacctgcccagttctcaaaagatagtctgcatgtgtctcagatggcctgtctaaggcaaaatgatctctgcttcccagatagttttcaactttgtactgaccattctggataccagaatttgtagactgcgtggcactattttcaagataaaagccgttgataaatctgcaatttggggatactttcctgtgtcttccaactgctgagtctccatattgccatctatctacagctgcatgacaactaaagcaccgcacggtatctccttcaccagtataaagaaaccctgctcgtgccagtgttgatgctgaaacaggactaccacttggaaaattagcaaaagtttttaatctattaaactcttctacaaattcttcttccttattgatgtctgcaggtacacaagttttagatccttcaaaactgttaaaagtcatcttctcttgaaaataggacttgtccaccttttctagcgcgcgcacatgcgcagtgagcacctc

SEQ ID NO: 13319 - RNA, 5805 nt, Homo sapiens
  source 1..5805: mol_type = other RNA
gctgggattacaggcatgagccaccacgcccagctaattttgtatttttagtagagacggggtttctccatgttggtcaggctggtctcgacctcccgacctcaggtgatctgcccgcctcggcctcccaaagtgctgggattacaggcatgagccaccgcgcccagctgatttatatcttatctatgagaaacaccaaaaactatgagtaagcatcactgagttatcatgtaagaattttttctaagttttagcccaaatttccaggtcaagacaaacccacagagaggtaaaagggtattaggatgggagttcatatttacagcaggaactttacatacatggtctccttgagctcttgcaaccttgtaagataagtattattttcctttcacagatgaataaactgctaccctttttttaacaagtagatttgactaaaaagaactatgtcaaatattgcttcccattttcttatttcttttttttttttttttgagacagagtcttgctctgttgcccaggctggagtgcagtggcgagatctcggctcactgcaagctctgcctcccgggttcacaccattctcctgcctcagcctcccgagtagctgggactacaggcgcccgccaccacgcccggctaattttctgttttttagtagagacggggtttcaccgtgttagccaggatggtctcgatctcctgacctcgtgatccacctgcctcagcctcccaaagtgctgggattacaggcgtgagccactgagcccagccccattttatttcatttctctaacagcaatgatatatatacatcccatagtatatcctactgatatactagcccctttccccattcaacacctgtgtaatcaggaaataaaacaatgattcgggtttaaagggtatatcatgtgaaactaatgctggggcggtagtctccattcatagttcaaaatacaaattttatccactaaaatggaaacacaaaaaacaactactgaaatgtaaataatataacaacaaaaataacaaaatatcataatacacagggccaaatcacattatatacactcactacacccactctaccctaccttagcccgtaatcaaagggacaggggaaaaaaccaaatgtagcaggaaaggcaatataaagctattaattaattaactggaatttagtttgtaaatgctaaaaccagttctcaaaaattaagacaatgcttttgatcagcagactaaattattacaaataaagataagtacttattgcaaaactacttgaatctttgcatgactaaaatgtaaaataagtggtgacttgaaatcctagagtgaactttatacagaaaaggaatagtctacatgtagacactgagaactcttgggagggggaaaagatttggatatggctatagttttgactttgcaaatgatcaatttttgcggaattagatggaaaagatccggtgctttttatagttcaaacacagacaaatgctgttaagtctccaaaaatttgattagaagttggagtgctgagtgattttaagaacctgaagcaacagcatttctaaacaattcttaaaataaacttgttagccacatcagcgttgtgcattaaatttcacaactcatggagaggaagaaaaaaagtcttgcttaactctaaacatacaagttttagaagaattttaatgaagtgcggctcccagaacaggaaaagccttatgttaaaacaattcagtccttgagtccttggctaacaactagattgaactacctacctgacttggaagtgaagtgtcctggaaaacatattttaaaaattttaacacttttctccccttgtagaaaactttaaatttaaagtctagactatacagaccaaattcaagttaatgactatataaccaaactaagtggcagacagtgcaaaggtgaagaactgaggatttacatactaaaacagaaacagggcagtcattatttaatttttaaaactctcatttaaatttgcaatgttttagccgggcgtggtggctcaagcctgtaatcccagcactttgggagggcaaggcgagtggatctcttgaggtcaggagtttgataccagcctggccaacatggtgaaaccccgtctctactaaaaataaaaaaaaattagtcgggcatggtggcacctgcctgtaattccagctactcaggaagctgaggcacgagaatcgcttgaacccagaaggcggaggttgcagtgagcagagatcactccactgcactccagcctgggtgacaagcaagactccatctcaaaaagaaaattaaataaataaaataaatttgcaatgttttaaatgaatatcacttaaagtagtaatcaacagaagttaggagaacataacaatactctttctcttagaaagtacaacaaaaatataattttttacagttttactctcaaactttcctctgtagtaacatgccttactcacctctacaataggtttgttgtgagaatcttgtaatgtaaaccctggacgttctatgaagcatttttaaacttctagtttataccctactgattcttattcaagtgttttttaaaaaatatttaaacaactattcttcttttcttgccaatatttttataatttccaagaggttttaaggatcttgagagaacatttatttcagaagtatctactactattactagccaagaaaacaaatgtaggtagaggaaagacttaacattttgtcctatatacatcttaatcatcctaacggtaaaaactcacatgaaactttaagatacaagatgatatgagaatctcaacatggaaagctgtcactataactacaagcagtgtacaaacatgcttctacttttacctacataagctgacagatgtttaaaatactgagttaacaaagatcttttagtaaagtgacttaggcaggcttaaactagcaaggattaaggatgaatccttactaattaattggaagatctgagacatattttatatttcattttacaaaatcagaaatacttattttgaaacaagataagacatggtctacctgtcaaaaaactaccactcagaaatatttttcatccacaaagcaggaaaaacataaaatcatttacatttcacattggcaccaaaaaggttaactgccctgccttcttggattagaaaaactaaagctgagtgataagtagttttgcaggcgtttgaacatgcctaagcctttaaatcagcaaaatactttctaaaaattctgattacaaaagtaatacatacttataaaaaattcgaacagaacaaaatgaaaaaagtagaaagtgaaaaggcccctataaaacccctctggggcccctcccccaatccccccctccccgaagagaaaccacatttaacagtttggtgtatatctttccaaatcttttgttctatgcatattaaaaacatacatactttgatctggctcagactatacatagtgttttgccacttgcattttacacttaacatatctttgacatctttccatgtcagtacatgttggctcgatagtattctatcattaaatacgctttcaaaaatggcaaatcactttaaaaaaataattcgcacaagtacgtgtttataactttaaaagaaaatggacagaatcctaaaacacaacaaccaacctctaaaaacaatctctatctttccaccagcatggaacaatttattcctttttcacacaaaacaaattatgtgattggggagattaactctaatctccacatttatatacagaaagctccatttgttaagcctatctgaaaagaataaaaaatccagatgattaattcacttacacttagaaattaaatcagtatactatgaatacacattgtgttcagttatagtatgatgcttcttattcttagtctatggtttcaattaaataacagtaaaaaaaatggataatacagctaataccctgaaaaatcaagaaattcaaagattatattgccaactaaaacactgccatgtacattttttttcctacttggtagcaaatgctaatggaattcaatcctgattacttaaagtcagttcacatcacacattcaatcagggtaataagaacaacataacatgcctactatagagttagattaagacataaaaattttttgcttgaaagtaatgactgtgtagcacatgggacacttgtcaactgcttcagcacattgtttacaagtgactagatgtccacaaggaacaaaaacgatagcaatatttctatccatacagattttgcaaagcttctcctcttgcaggcgccttagctgctcttcagtactaatctctttctgtaatgaagtctgacttgactcatcttgcatactgtctttctgagcattcactagatctgcaaccagaacctcaagtgatttatagttgctcccagatatctgaattttttcctccattattttcttaatgtccttgaaactgaaccccattcgtatagcttcttgtaccataggattttggaagatggtatcatcaattcttctagttagtgatggtgttttctcagtagttcttaccagacactcctcaagtgaatgagttaaatgaatattgtttatatattcttgtcccttctgttctaacagatatttgcaccctggataccatttagcatgttgttcccaagggtcttcactgggcttccaatcagttagccctcctccacagtgaaagcactttactttatcaccttcacctaaagcataaaatccagctcttgcaagctgctccttgttaactgagtatatccatgtcccaaaagtaaagatccgtgcttcataatctgccatggatggatttcttggaagatttgttgaatttgggaaattcctatcagaactcacagcatcagattcacttcgaatattaagattccggcccaaaacaaagaagcaattaggaaagtgtcgcctgtgttctgaccaggcacgatcacaaggttcccaatttttcagttttccaccacaacaaaagcactgcacttggtcaccaatacctgtgtagtagagtccagcacttgctaactctcttggggttaggtgagcatagtctggccagttctgaaaggactttaatctagcttcttcactatacatggcagggttcctcgggtatatggtgtctgatatatctacaacctgcccagttctcaaaagatagtctgcatgtgtctcagatggcctgtctaaggcaaaatgatctctgcttcccagatagttttcaactttgtactgaccattctggataccagaatttgtagactgcgtggcactattttcaagataaaagccgttgataaatctgcaatttggggatactttcctgtgtcttccaactgctgagtctccatattgccatctatctacagctgcatgacaactaaagcaccgcacggtatctccttcaccagtataaagaaaccctgctcgtgccagtgttgatgctgaaacaggactaccacttggaaaattagcaaaagtttttaatctattaaactcttctacaaattcttcttccttattgatgtctgcaggtacacaagttttagatccttcaaaactgttaaaagtcatcttctcttgaaaataggacttgtccaccttttcttaggtgtcacagggtttaggaaggcaatcctgcaggcctgaagtcacccacccacccacgcctgccgtcggcagtccgaggaacccgggcaagc

SEQ ID NO: 13320 - RNA, 138 nt, Homo sapiens
  source 1..138: mol_type = other RNA
gctgggattacaggcatgagccaccacgcccagctaattttgtatttttagtagagatggggtttctccatgttggtcaggctggtcttgaactcccagcctcaggtgatccacccatctcggcctcccaaagtgctg

SEQ ID NO: 13321 - RNA, 891 nt, Homo sapiens
  source 1..891: mol_type = other RNA
gctgggattacaggcatgagccaccacgcccagctaattttttgtacttttagtggagatggggttccgccatgttggccaggctggtctcgaactcctgacctcaggtgatccaccctccttggcctcccaaagtgttgggattacaggcgtgagccactgtgcccggcagacttttaatacagtgatattaattcatttgatggtctcctcctgtgtcttctaaatcaatatcaaaatctaaatcatcatcactttcttcatttcttctgcagcttcttctatggttggaacttagattattttcagtatgttctattttttctgtttctttattcaacggaataacaatgtcttctttctttccacattttgcgcaaacttcaagttcacaggcacatggcctgcacattatgtgataagaatccttcactgtcttttgtaaacatttaacacactttttaggttttgataatggtttgtatttgctgtattttacacgccactcaagaacttctttacagcgctgacatactccatcatgaagttttgcattaattttctgcagttcaactcctgctgtgtggcccagttcctgacaggccatggaccgatgcgggggtcgggggctggggacccctgctccacagggagacaaactcaaacatcatgactagagtttgcagataaagacttggtctgcacacttttatcgaacttgtcatttttgaagctaaacgtattctggtgcttctgaggtctggaacgagccacgttgcctttctgggagctcatcgccgaaatcaaagccacccctcgccgggagcaggcaaaaggatgaggggaaagaaaaccaacgaactactcccaggaattgacgcttctgtcaat

SEQ ID NO: 13322 - RNA, 760 nt, Homo sapiens
  source 1..760: mol_type = other RNA
gctgggattacaggcatgagccaccacgcccagctaattttttgtacttttagtggagatggggttccgccatgttggccaggctggtctcgaactcctgacctcaggtgatccaccctccttggcctcccaaagtgttgggattacaggcgtgagccactgtgcccggcagacttttaatacagtgatattaattcatttgatggtctcctcctgtgtcttctaaatcaatatcaaaatctaaatcatcatcactttcttcatttcttctgcagcttcttctatggttggaacttagattattttcagtatgttctattttttctgtttctttattcaacggaataacaatgtcttctttctttccacattttgcgcaaacttcaagttcacaggcacatggcctgcacattatgtgataagaatccttcactgtcttttgtaaacatttaacacactttttaggttttgataatggtttgtatttgctgtattttacacgccactcaagaacttctttacagcgctgacatactccatcatgaagttttgcattaattttcttggtctgcacacttttatcgaacttgtcatttttgaagctaaacgtattctggtgcttctgaggtctggaacgagccacgttgcctttctgggagctcatcgccgaaatcaaagccacccctcgccgggagcaggcaaaaggatgaggggaaagaaaaccaacgaactactcccaggaattgacgcttctgtcaat

SEQ ID NO: 13323 - RNA, 890 nt, Homo sapiens
  source 1..890: mol_type = other RNA
gctgggattacaggcatgagccaccacgcccagctaattttttgtacttttagtggagatggggttccgccatgttggccaggctggtctcgaactcctgacctcaggtgatccaccctccttggcctcccaaagtgttgggattacaggcgtgagccactgtgcccggcagacttttaatacagtgatattaattcatttgatggtctcctcctgtgtcttctaaatcaatatcaaaatctaaatcatcatcactttcttcatttcttctgcagcttcttctatggttggaacttagattattttcagtatgttctattttttctgtttctttattcaacggaataacaatgtcttctttctttccacattttgcgcaaacttcaagttcacaggcacatggcctgcacattatgtgataagaatccttcactgtcttttgtaaacatttaacacactttttaggttttgataatggtttgtatttgctgtattttacacgccactcaagaacttctttacagcgctgacatactccatcatgaagttttgcattaattttctttttgctttttgtgtgtatgggtacaggtaaaataacttatggatatcaagacacttcacttcttaatactcatcatatcctagcaataaagaccttctcgtgcttaaccacaatactgttaccacaccttggtctgcacacttttatcgaacttgtcatttttgaagctaaacgtattctggtgcttctgaggtctggaacgagccacgttgcctttctgggagctcatcgccgaaatcaaagccacccctcgccgggagcaggcaaaaggatgaggggaaagaaaaccaacgaactactcccaggaattgacgcttctgtcaat

SEQ ID NO: 13324 - RNA, 1138 nt, Homo sapiens
  source 1..1138: mol_type = other RNA
gctgggattacaggcatgagccaccacgcccagctggcatctgggaacttgactggtaaagagctcctatgtggatacaatactatccccaaataacaactgctcactcttttctatacaaatcatgtgatatttgctgaacacttgcttttcttctgagcctggcatttcggtgaccatattcagtcacgcaggcacaacgtacctacatgagcaacccccagtgaaaaccctggactcctgggctcaggcaggcttccctggtagagaacactttgcacatgtcacagctcgaggctggaggattcagcacattctgcgggaggggaccccaggggaggggactctgggggcttgtacctggtttcctccggccctcaccccaaatgcatcttcctgttactaattctgcgtcgcatcttttcaccgtagtaaatcccagccactagtatgatggtaggctaagtcctgtgagtccctcaagtgcagtcaccaagcctagtgtgtgatggggatgcctcatggcttctgtgtggcaggagtccggggaggggactgctgaacctctgctcagggtctcacaggctgcactcaaggtgtcagccagggctgggatctcaaccgaggcgcgaggtcccctcctgagcgcatgtcgttgtgtgcataatctttctcgcagctgtggagccgatggccatatgcttctttggcatcaggagggggcggctctgtggcttccagcctcttaaagggtgcacctgagctagccaggctcggccagatcaacctcccttctgatgaacgccaagtcacctgattagaaaccccggtcacacctgcagaaatcccgccactccttgttccgccttccaggaaccaggtcatggtcgtcctcacttgctgggaagggcgggactggctctgctcgcccccacaccagcccccagaccagctaaggctcttggtctctcaccttccaggggtcccgtgcccccccaccctactcaggccatgcaccactgaccgggcctggccctacctgtggacagcctccctccccagggtgcaggaaggggcctctctccatggaaagtgaagcctcaacctgagcaggaggaacaggaagaaagggcttggc

SEQ ID NO: 13325 - RNA, 8328 nt, Homo sapiens
  source 1..8328: mol_type = other RNA
gctgggattacaggcatgagccaccacgcccagcttctgtgactttaaaaaaatctttttagacagggtcttgctctgtcacttgggcttgagtactgtggcacaatcacacctcactgcagccttgacttcttgggctcaggcaattaattctcgtcctttggcctccccagtagctaggacacaggcgcacaccaccacactcagctaatctattttttgtagaggtgggttttcgccatgttgtccaggctggtctgggactcccggctcccaaagtgttccaaccacaggtgtgtgggccttccgtggtatcttaacctcatcacccagaggcaacaacagctagtattcttctagtttttaccacccccaccacctcaatcctgcccctgtagcctttccaagtgccacagcattgtttcagtttctatcttagaaagcccgggagtctgtgtcctatctccctgggggcattcaaaccctagtccatagcctgaggcccacctatacccagacccagtgtcttggaagcactgactttaatacccacttaggctgggcgcagtggctcacgcctgtaatcccaccactttgggaggcttgggcgggcggatcacctgaggtcgggagttcgagaccagcctgaccaacatggagaaaccccgtctctactaaaaatacaaaattagctgggcgtggtggtgcatgtaatcccatgcctgtctcaaaaacaaaacaaacaaacaaaacaaaacaaaacaaaaaaaccccagttacattcaggatgaattctgccttcctttttgccaccttgggatttccatttctttctctgaaataggcatttgcatttttcctaggattttttttttaaaacagttggaattatcccatatacacaattttttcacttttctaattaacatacatttccccatgggcttgtgtctcacctctcaatccccagtgtatagcaaagaccaggctcaggggcacttacaaatgtttgttgaaaccaaagacatcctatattacagaaatgaactttggaaagaccagtcagcgtgggtgggtgaggaatgccagagacgggagaacaaaatgaggtataccgtcaggtttgaagggttgagggttatggagggttcttcataggaagttcaccatggagttcttggaactgttcaacacacagaagcaaggtcctctccttctaggtatggctagaaatgtttatcaatagctgagactctgattcccagggtgggatcaggaagccagccccagctgctgcagcatttttttccctttttctcattacaggagccaagaaaactgtcaaagcagatgatgcaagagtgaagctgactcagaaatactcaatccccccaggaacttctctaagaaatggactgaccatcctgtaagcttccatctggaggtacctggggaagggcttctcacattgaggccaataagaatccctagtgggccaggtgtggtggctcatgcctctaatctcagcactttgggaggccaaggcgggtagactgttgagctcaggagttcaagaccagcctgggcaacacggcaaaacttcatctctaccaaaaaaaaaaaaaaaaaaattagccaagcatgatggctcgtgcctgtagtccctggaaggctgagttgggaggatcacctgagcctgggaggttgaggctgcagtgagctgtgatggcgctactgcactctagcctgggtaacagagcaagacccgtatcaaaaaacaaaacaaacaaaaaacttctagtgagtagagcgacagggagacaaatccagtttgtaatttgctacagtgcaaaatatctggctttccatagagggagtgggaacaaggcaatgctggccttcattcaatcagaaacttgacttgtacccgttgaaaacctgtcatgtttaatgcttggatattttttcttctagtaaagacactttactgccacctgctggaaaagagtcagaaattttccaaatgcaaacatctatggcctccctataatgtagcatccttttactgtacatagtctgcacaactgtacaatttagaagagaaaccaacatttggtgtaactctaccatataccaggcatctgtcatagaatctgaacaaccgctctatgaaatcagtacttataccccaatttaacagataggaaatattgggacctctggggaagggaggaagaagagggtatcaccaaaaaagggcaaaaagggggcttggtctgtattggcaatggaaattcaacttgggtggtaggattatggatgtgttacagctttctttataatttggtacatgcctaaaatgttttacaataacaatttaaatcacctgtgaagaaaagattcagagaggttaactgatcaaaaaaatcacactgccagacagaactctgttagaggtagaccacttgcagtaacattacattgcttctctaatggttaaatttagcacagaatcaaaggagagctataaagtctaggaagtacttatttacataggattgagtccagaacatcttgtgacaccatctacatatgttttacttggagaatagtctgaatttcgtattacacgttgagcatttctaatttgaaaatacaaaatcctcaaaaatctgaaattttttaagcatcaacatgatgcctaaagtaaatgctatttggaatatttcaaatttcagattaggaatattgaactggtatgtattccgcaaatattccaaaaatccaaaaaaattcaaaacacttctggtcccaaccattttggataggggatattcaacctatattacacacaggtaatacagcaggggaaaagcagggagactgcagcatctaagtctactaaattggccaggatcattccttagtcttcagatacctatttatcagggtctcattaaataaagttacttgtcatgttagttcagtctggcctgtggcttgtaattatagctgcaaactcaagggcaaagttcttaggattttgagatgctctttatgcaacaatacttccatttactttgtgtgtgtgtgtgtgtgtgtgtgggtgggtgggtgtgtgtgtgtagggagagaaagggggcaatggagtggagagtggaactacaatttattaagcacctattattacaagccaagtagggtgttaaatattttcctcgtgccattccattcaatactcttcgatcctgagggaaaacgaacccacttaaaaaaaaaaacaaaaggttttaatgaggattgcataagacatgcaaggtcaccagggagtttacatgcaagtggggagatacaaaataatacaacaaaagttcaggtgttctgaggaaaaagaagggcaagggtaagtgatgacagtgggggaagtcggattcaggataaaccaattttagactcattttttgaggaaggaactgagcatgaccttaccacacagcctttttagttaagtgtttctttaactaggaaaaggccctgggaagacaggctctctactatgcaaacccaattccagtcttgggagagaatttgctggtgggacaaaatcaggtttttcaagagatgcttaaatggtcaattctaattataaccatacttgtcaaaaggtgaagcaaagatgaaagttaaaaactaagaagaaattaaaattcccaaatctgtcaaccaatctctaattttctctgctactttaggactatagtaattagccataccctgaggatctactttacaagatatattcctctgacagtcccactctaacaatttaatctatcttatgtaagctggacaggcatttcaagtacaagaaacagaattcaaaacgtgaaaacggagccatctatcacacacggtgtcggttggagaagcatattgctcaggctgcagggacatttcatttatttaaatgtttttattaaaaaaaattaaagaccttcatggcacaacttcttcccagcacagttatggtttagtcataccaattacaatacaattacaaccaataaagcaaggtggggagggccttctggcttcaaacttaaaaaaaagcagaggaagaggggagggaccacttcaaacaaagtttaaaaatactttaaaaaatctttcagagtaattgccaacataacctttcatgttggccattccatttcctgccatctaagcaatgcagacacaggtagtgctgagaaatagtgtcccaatacaaggtatacagatgaggtaatttacaacaacacgtaagttgttactctgtaaacccttgcctcccccccaccccccacccaattgggtcttttttttttttctctctctccatgcttctgcagtgactcttaagtagcatttttaaaaacttctatttattttaaaaggctcttgggtggcacctcagagtcctctgcattcaccttcggtttattccaaggtctgatgggtgtaaggaggtccagctgtctgcagctctccgcatcagcctaagctacacctcaatttccgagctacaaggatagggtatgaagtcttgatttacaaccctctccccacctcaaaagaaagaactcattagttataagtgtcctgttcaaatcacaatccagtgcaaacataatcacaaattgcatctctggcacatctggtgcttttagcttctgcacaaattcaacatggtaaccctcacagcattctagggcataaaagggtcaagtacaataaatatccactgtaagtggtcataaggaagaaaatcaccctgccacacagtcagaatgttttcccttcagctctccctaccgttgagaagcgctataaaaggaggctttagcgtcctctaaagtttaccattatattcactaaagccaccaccttgataaagttactaaagccaagatgggttacaaagttagataagttcattaaattcaactccccaaacaattacgtttatctatgatgcctaggcgagaaaggcctgtgaatctataaggtaggagaatggggaactaagattttaggccttaaaatatgttggaagaatttttcctagttcccacaagcagctactgtaatgaaataacaggagaaaatacagagctgatggttttgctattgtgcttaaaaaactaggcttcctcagtgaagcacctgataaacttaggtggttggattacagtggaaagtccactttacacacacacacaaacacacaaaaactggcgactttttccatccccaatccctgcactgctgagacacaaaatgagttttatggcaaaggatccttaatccccagagacgctttggcttgtggtgctttttttttaaggcctctctgctctgcccggtaccatgggtcgaacgaggggtgtataaaatgggggccttgggaagcctccacggtacagggctgcaggcccctcagatgtgaacatgagacacccacccagcaagacctttacacagggaacttaaatctaaccttgataaataaaaccaaacgtttatttacaccaaagaattccaacactggatctttcacatatgaaggacaaagtattatatatatacacacagcaaggggtggcggggctgtaacaagagagtttatagttttcccacaattacaggtctaccatttcagcttcaatggagatagtggctctgctcctacctctcaagatacatttacaagactgaggagcaggtcttctcactggatggcatgtgagggaaggggacggtcggaggaaaagaaggtagaaagcttaaaatggaagtcagtgtggccacatctcccattagctctagcatgaaacctgtacagacaatgtttgtttcttttgtaaaaagcagtaagttatgcccagtaactaaatgaattcaaaatggccaagacaaagaaaactaagaaagattttgccttccctctcctaccagctatggagcacagcatgttgggagatgaacagggaaaagaccaaggtaaggagcctgggagggaaggtatcaacattttaaactgaactaaaaataaaagtataaatgagttggatttagggttagatcagtaagacatgattcttactgaacagaagtttttagtatctgtctgcattttgggtagattttcaacatcttgatgtaactaagacacacttccacaagagccactaggataaccccactgaagcgcttatggagtaaagtgatgtaagcgaccagcaagcagtccactgctcctatagattgggtcctcccttccttctttccttccttcctttcttcctgcctcccctgagaagctacatttttgtaatctctggagaagagcacgagataccaaccccctaaagtgtgggacggtggaggaacaatggtgggaatgggaagaagtctccacctaaatgcagcagccgggattgaggctggtttatctttgttcttttgtgatgaggaactaaatttgggaggggagaaaaaaaaatttgtccatgaaatattccacctgcaggtaatttttcagggaatcccctgagttatgaaaagttcgagttaaaaaaaaaaagaaaaaagaaaatcagcctattataattttttttttatgactgaactactataaatccacaagcaacggttcagacacggtgcttctgaagtgtttcacccctccccgccaggcgcaagctgcatcaaggagagggtggactcccccacctctgctcaggcatcaggagacagatagggccgttactgctgagcgccagcggcagctggaacaggcatcccaagggggttggcagcagcaatcactggtgagcctgccagaggtccaaggggtgaaggggttggcactgaagaaatccctgacatcatattggcgctgctgacgggcgtactgccccctggcatgctagatgaacccattcgagcctggtccttcacaacagtgtagaaataggggtgctccattgcctctcttgcagtaagccgtgactggtggtcatatcgcagcagtttgtccaggaaatccaaggcctcagggctgacaaggtgctgattttcactgtggacaaagcgttcccatcgctttcgagagtgtctgcccaagatatcattgaaacgtggatctaattcaatgttgtatttgtcaatatagtcatataaatcttctgtccccagaaccttggctatcctcaccaactgatcataattgtcatgtccatggaaaaatggctccttccgaaagatcatacttgccagcatacaacccaaactccacatatccaaactataatcgtacatctgatagtctacaagtagctcaggacctttgaagtatcgggaagcaactcggacattatattcttggccaggatgataaaactcagccaaaccccagtctattagtcgtagctttctgtgctcatgatcaatcatgacattatggggcttgacatctctgtgcataattcccatgctgtgacaataatccagggccttcagaatctcatacatgtaaaatcgaatatcatagtctgttaacgtctggtacaattgcttgaagtctgtgttgtttacgtgttcaaaaaccaaggcgggggttcgtgacacagggtcttttacaatgtctgccagtgtgatgatgttgggacctcctctcaaattctccaaaatctttatttcacgcttaattttcttcttttttactggcttgagaattttaacaacaactttttcattatttgtgatgttgatggcttcaaatacttcactgtatttacctcggcctaattttcgaaccagctggtagtcatcttgatttccccattccaccacatgtgactcgtaatcccagtattctcgaggtctgtgtgtattaacatctgtgtaaactctggccctgcttggcacgggtcccgacatgtcagacaggttggcggacaaagctggacttgatgtttggagatctggcagtcactgtgttcagaagcagctgggggtaagaccttgtttcagacctgttttcttcaaacaaagagatgtgaaactagtcagtatgggtgaatgatgtttcttggagattttatgaggttccacgctgcatgatttaccatgtgatgagcacactgcttgacaagccttgatagagctgtggtggaagcggcagcggcggcggccgctctcccctctgctcacacagacaatatggcggcgatggaggaggagacacacggctcggccgccagccgcagggaccagagcgaggct

SEQ ID NO: 13326 - RNA, 8211 nt, Homo sapiens
  source 1..8211: mol_type = other RNA
gctgggattacaggcatgagccaccacgcccagcttctgtgactttaaaaaaatctttttagacagggtcttgctctgtcacttgggcttgagtactgtggcacaatcacacctcactgcagccttgacttcttgggctcaggcaattaattctcgtcctttggcctccccagtagctaggacacaggcgcacaccaccacactcagctaatctattttttgtagaggtgggttttcgccatgttgtccaggctggtctgggactcccggctcccaaagtgttccaaccacaggtgtgtgggccttccgtggtatcttaacctcatcacccagaggcaacaacagctagtattcttctagtttttaccacccccaccacctcaatcctgcccctgtagcctttccaagtgccacagcattgtttcagtttctatcttagaaagcccgggagtctgtgtcctatctccctgggggcattcaaaccctagtccatagcctgaggcccacctatacccagacccagtgtcttggaagcactgactttaatacccacttaggctgggcgcagtggctcacgcctgtaatcccaccactttgggaggcttgggcgggcggatcacctgaggtcgggagttcgagaccagcctgaccaacatggagaaaccccgtctctactaaaaatacaaaattagctgggcgtggtggtgcatgtaatcccatgcctgtctcaaaaacaaaacaaacaaacaaaacaaaacaaaacaaaaaaaccccagttacattcaggatgaattctgccttcctttttgccaccttgggatttccatttctttctctgaaataggcatttgcatttttcctaggattttttttttaaaacagttggaattatcccatatacacaattttttcacttttctaattaacatacatttccccatgggcttgtgtctcacctctcaatccccagtgtatagcaaagaccaggctcaggggcacttacaaatgtttgttgaaaccaaagacatcctatattacagaaatgaactttggaaagaccagtcagcgtgggtgggtgaggaatgccagagacgggagaacaaaatgaggtataccgtcaggtttgaagggttgagggttatggagggttcttcataggaagttcaccatggagttcttggaactgttcaacacacagaagcaaggtcctctccttctaggtatggctagaaatgtttatcaatagctgagactctgattcccagggtgggatcaggaagccagccccagctgctgcagcatttttttccctttttctcattacaggagccaagaaaactgtcaaagcagatgatgcaagagtgaagctgactcagaaatactcaatccccccaggaacttctctaagaaatggactgaccatcctgtaagcttccatctggaggtacctggggaagggcttctcacattgaggccaataagaatccctagtgggccaggtgtggtggctcatgcctctaatctcagcactttgggaggccaaggcgggtagactgttgagctcaggagttcaagaccagcctgggcaacacggcaaaacttcatctctaccaaaaaaaaaaaaaaaaaaattagccaagcatgatggctcgtgcctgtagtccctggaaggctgagttgggaggatcacctgagcctgggaggttgaggctgcagtgagctgtgatggcgctactgcactctagcctgggtaacagagcaagacccgtatcaaaaaacaaaacaaacaaaaaacttctagtgagtagagcgacagggagacaaatccagtttgtaatttgctacagtgcaaaatatctggctttccatagagggagtgggaacaaggcaatgctggccttcattcaatcagaaacttgacttgtacccgttgaaaacctgtcatgtttaatgcttggatattttttcttctagtaaagacactttactgccacctgctggaaaagagtcagaaattttccaaatgcaaacatctatggcctccctataatgtagcatccttttactgtacatagtctgcacaactgtacaatttagaagagaaaccaacatttggtgtaactctaccatataccaggcatctgtcatagaatctgaacaaccgctctatgaaatcagtacttataccccaatttaacagataggaaatattgggacctctggggaagggaggaagaagagggtatcaccaaaaaagggcaaaaagggggcttggtctgtattggcaatggaaattcaacttgggtggtaggattatggatgtgttacagctttctttataatttggtacatgcctaaaatgttttacaataacaatttaaatcacctgtgaagaaaagattcagagaggttaactgatcaaaaaaatcacactgccagacagaactctgttagaggtagaccacttgcagtaacattacattgcttctctaatggttaaatttagcacagaatcaaaggagagctataaagtctaggaagtacttatttacataggattgagtccagaacatcttgtgacaccatctacatatgttttacttggagaatagtctgaatttcgtattacacgttgagcatttctaatttgaaaatacaaaatcctcaaaaatctgaaattttttaagcatcaacatgatgcctaaagtaaatgctatttggaatatttcaaatttcagattaggaatattgaactggtatgtattccgcaaatattccaaaaatccaaaaaaattcaaaacacttctggtcccaaccattttggataggggatattcaacctatattacacacaggtaatacagcaggggaaaagcagggagactgcagcatctaagtctactaaattggccaggatcattccttagtcttcagatacctatttatcagggtctcattaaataaagttacttgtcatgttagttcagtctggcctgtggcttgtaattatagctgcaaactcaagggcaaagttcttaggattttgagatgctctttatgcaacaatacttccatttactttgtgtgtgtgtgtgtgtgtgtgtgggtgggtgggtgtgtgtgtgtagggagagaaagggggcaatggagtggagagtggaactacaatttattaagcacctattattacaagccaagtagggtgttaaatattttcctcgtgccattccattcaatactcttcgatcctgagggaaaacgaacccacttaaaaaaaaaaacaaaaggttttaatgaggattgcataagacatgcaaggtcaccagggagtttacatgcaagtggggagatacaaaataatacaacaaaagttcaggtgttctgaggaaaaagaagggcaagggtaagtgatgacagtgggggaagtcggattcaggataaaccaattttagactcattttttgaggaaggaactgagcatgaccttaccacacagcctttttagttaagtgtttctttaactaggaaaaggccctgggaagacaggctctctactatgcaaacccaattccagtcttgggagagaatttgctggtgggacaaaatcaggtttttcaagagatgcttaaatggtcaattctaattataaccatacttgtcaaaaggtgaagcaaagatgaaagttaaaaactaagaagaaattaaaattcccaaatctgtcaaccaatctctaattttctctgctactttaggactatagtaattagccataccctgaggatctactttacaagatatattcctctgacagtcccactctaacaatttaatctatcttatgtaagctggacaggcatttcaagtacaagaaacagaattcaaaacgtgaaaacggagccatctatcacacacggtgtcggttggagaagcatattgctcaggctgcagggacatttcatttatttaaatgtttttattaaaaaaaattaaagaccttcatggcacaacttcttcccagcacagttatggtttagtcataccaattacaatacaattacaaccaataaagcaaggtggggagggccttctggcttcaaacttaaaaaaaagcagaggaagaggggagggaccacttcaaacaaagtttaaaaatactttaaaaaatctttcagagtaattgccaacataacctttcatgttggccattccatttcctgccatctaagcaatgcagacacaggtagtgctgagaaatagtgtcccaatacaaggtatacagatgaggtaatttacaacaacacgtaagttgttactctgtaaacccttgcctcccccccaccccccacccaattgggtcttttttttttttctctctctccatgcttctgcagtgactcttaagtagcatttttaaaaacttctatttattttaaaaggctcttgggtggcacctcagagtcctctgcattcaccttcggtttattccaaggtctgatgggtgtaaggaggtccagctgtctgcagctctccgcatcagcctaagctacacctcaatttccgagctacaaggatagggtatgaagtcttgatttacaaccctctccccacctcaaaagaaagaactcattagttataagtgtcctgttcaaatcacaatccagtgcaaacataatcacaaattgcatctctggcacatctggtgcttttagcttctgcacaaattcaacatggtaaccctcacagcattctagggcataaaagggtcaagtacaataaatatccactgtaagtggtcataaggaagaaaatcaccctgccacacagtcagaatgttttcccttcagctctccctaccgttgagaagcgctataaaaggaggctttagcgtcctctaaagtttaccattatattcactaaagccaccaccttgataaagttactaaagccaagatgggttacaaagttagataagttcattaaattcaactccccaaacaattacgtttatctatgatgcctaggcgagaaaggcctgtgaatctataaggtaggagaatggggaactaagattttaggccttaaaatatgttggaagaatttttcctagttcccacaagcagctactgtaatgaaataacaggagaaaatacagagctgatggttttgctattgtgcttaaaaaactaggcttcctcagtgaagcacctgataaacttaggtggttggattacagtggaaagtccactttacacacacacacaaacacacaaaaactggcgactttttccatccccaatccctgcactgctgagacacaaaatgagttttatggcaaaggatccttaatccccagagacgctttggcttgtggtgctttttttttaaggcctctctgctctgcccggtaccatgggtcgaacgaggggtgtataaaatgggggccttgggaagcctccacggtacagggctgcaggcccctcagatgtgaacatgagacacccacccagcaagacctttacacagggaacttaaatctaaccttgataaataaaaccaaacgtttatttacaccaaagaattccaacactggatctttcacatatgaaggacaaagtattatatatatacacacagcaaggggtggcggggctgtaacaagagagtttatagttttcccacaattacaggtctaccatttcagcttcaatggagatagtggctctgctcctacctctcaagatacatttacaagactgaggagcaggtcttctcactggatggcatgtgagggaaggggacggtcggaggaaaagaaggtagaaagcttaaaatggaagtcagtgtggccacatctcccattagctctagcatgaaacctgtacagacaatgtttgtttcttttgtaaaaagcagtaagttatgcccagtaactaaatgaattcaaaatggccaagacaaagaaaactaagaaagattttgccttccctctcctaccagctatggagcacagcatgttgggagatgaacagggaaaagaccaaggtaaggagcctgggagggaaggtatcaacattttaaactgaactaaaaataaaagtataaatgagttggatttagggttagatcagtaagacatgattcttactgaacagaagtttttagtatctgtctgcattttgggtagattttcaacatcttgatgtaactaagacacacttccacaagagccactaggataaccccactgaagcgcttatggagtaaagtgatgtaagcgaccagcaagcagtccactgctcctatagattgggtcctcccttccttctttccttccttcctttcttcctgcctcccctgagaagctacatttttgtaatctctggagaagagcacgagataccaaccccctaaagtgtgggacggtggaggaacaatggtgggaatgggaagaagtctccacctaaatgcagcagccgggattgaggctggtttatctttgttcttttgtgatgaggaactaaatttgggaggggagaaaaaaaaatttgtccatgaaatattccacctgcaggtaatttttcagggaatcccctgagttatgaaaagttcgagttaaaaaaaaaaagaaaaaagaaaatcagcctattataattttttttttatgactgaactactataaatccacaagcaacggttcagacacggtgcttctgaagtgtttcacccctccccgccaggcgcaagctgcatcaaggagagggtggactcccccacctctgctcaggcatcaggagacagatagggccgttactgctgagcgccagcggcagctggaacaggcatcccaagggggttggcagcagcaatcactggtgagcctgccagaggtccaaggggtgaaggggttggcactgaagaaatccctgacatcatattggcgctgctgacgggcgtactgccccctggcatgctagatgaacccattcgagcctggtccttcacaacagtgtagaaataggggtgctccattgcctctcttgcagtaagccgtgactggtggtcatatcgcagcagtttgtccaggaaatccaaggcctcagggctgacaaggtgctgattttcactgtggacaaagcgttcccatcgctttcgagagtgtctgcccaagatatcattgaaacgtggatctaattcaatgttgtatttgtcaatatagtcatataaatcttctgtccccagaaccttggctatcctcaccaactgatcataattgtcatgtccatggaaaaatggctccttccgaaagatcatacttgccagcatacaacccaaactccacatatccaaactataatcgtacatctgatagtctacaagtagctcaggacctttgaagtatcgggaagcaactcggacattatattcttggccaggatgataaaactcagccaaaccccagtctattagtcgtagctttctgtgctcatgatcaatcatgacattatggggcttgacatctctgtgcataattcccatgctgtgacaataatccagggccttcagaatctcatacatgtaaaatcgaatatcatagtctgttaacgtctggtacaattgcttgaagtctgtgttgtttacgtgttcaaaaaccaaggcgggggttcgtgacacagggtcttttacaatgtctgccagtgtgatgatgttgggacctcctctcaaattctccaaaatctttatttcacgcttaattttcttcttttttactggcttgagaattttaacaacaactttttcattatttgtgatgttgatggcttcaaatacttcactgtatttacctcggcctaattttcgaaccagctggtagtcatcttgatttccccattccaccacatgtgactcgtaatcccagtattctcgaggtctgtgtgtattaacatctgtgtaaactctggccctgcttggcacgggtcccgacatgtcagacaggttggcggacaaagctggacttgatgtttggagatctggcagtcactgtgttcagaagcagctgggggtaagaccttgtttcagacctgttttcttcaaactgtggtggaagcggcagcggcggcggccgctctcccctctgctcacacagacaatatggcggcgatggaggaggagacacacggctcggccgccagccgcagggaccagagcgaggct

SEQ ID NO: 13327 - RNA, 8001 nt, Homo sapiens
  source 1..8001: mol_type = other RNA
gctgggattacaggcatgagccaccacgcccagcttctgtgactttaaaaaaatctttttagacagggtcttgctctgtcacttgggcttgagtactgtggcacaatcacacctcactgcagccttgacttcttgggctcaggcaattaattctcgtcctttggcctccccagtagctaggacacaggcgcacaccaccacactcagctaatctattttttgtagaggtgggttttcgccatgttgtccaggctggtctgggactcccggctcccaaagtgttccaaccacaggtgtgtgggccttccgtggtatcttaacctcatcacccagaggcaacaacagctagtattcttctagtttttaccacccccaccacctcaatcctgcccctgtagcctttccaagtgccacagcattgtttcagtttctatcttagaaagcccgggagtctgtgtcctatctccctgggggcattcaaaccctagtccatagcctgaggcccacctatacccagacccagtgtcttggaagcactgactttaatacccacttaggctgggcgcagtggctcacgcctgtaatcccaccactttgggaggcttgggcgggcggatcacctgaggtcgggagttcgagaccagcctgaccaacatggagaaaccccgtctctactaaaaatacaaaattagctgggcgtggtggtgcatgtaatcccatgcctgtctcaaaaacaaaacaaacaaacaaaacaaaacaaaacaaaaaaaccccagttacattcaggatgaattctgccttcctttttgccaccttgggatttccatttctttctctgaaataggcatttgcatttttcctaggattttttttttaaaacagttggaattatcccatatacacaattttttcacttttctaattaacatacatttccccatgggcttgtgtctcacctctcaatccccagtgtatagcaaagaccaggctcaggggcacttacaaatgtttgttgaaaccaaagacatcctatattacagaaatgaactttggaaagaccagtcagcgtgggtgggtgaggaatgccagagacgggagaacaaaatgaggtataccgtcaggtttgaagggttgagggttatggagggttcttcataggaagttcaccatggagttcttggaactgttcaacacacagaagcaaggtcctctccttctaggtatggctagaaatgtttatcaatagctgagactctgattcccagggtgggatcaggaagccagccccagctgctgcagcatttttttccctttttctcattacaggagccaagaaaactgtcaaagcagatgatgcaagagtgaagctgactcagaaatactcaatccccccaggaacttctctaagaaatggactgaccatcctgtaagcttccatctggaggtacctggggaagggcttctcacattgaggccaataagaatccctagtgggccaggtgtggtggctcatgcctctaatctcagcactttgggaggccaaggcgggtagactgttgagctcaggagttcaagaccagcctgggcaacacggcaaaacttcatctctaccaaaaaaaaaaaaaaaaaaattagccaagcatgatggctcgtgcctgtagtccctggaaggctgagttgggaggatcacctgagcctgggaggttgaggctgcagtgagctgtgatggcgctactgcactctagcctgggtaacagagcaagacccgtatcaaaaaacaaaacaaacaaaaaacttctagtgagtagagcgacagggagacaaatccagtttgtaatttgctacagtgcaaaatatctggctttccatagagggagtgggaacaaggcaatgctggccttcattcaatcagaaacttgacttgtacccgttgaaaacctgtcatgtttaatgcttggatattttttcttctagtaaagacactttactgccacctgctggaaaagagtcagaaattttccaaatgcaaacatctatggcctccctataatgtagcatccttttactgtacatagtctgcacaactgtacaatttagaagagaaaccaacatttggtgtaactctaccatataccaggcatctgtcatagaatctgaacaaccgctctatgaaatcagtacttataccccaatttaacagataggaaatattgggacctctggggaagggaggaagaagagggtatcaccaaaaaagggcaaaaagggggcttggtctgtattggcaatggaaattcaacttgggtggtaggattatggatgtgttacagctttctttataatttggtacatgcctaaaatgttttacaataacaatttaaatcacctgtgaagaaaagattcagagaggttaactgatcaaaaaaatcacactgccagacagaactctgttagaggtagaccacttgcagtaacattacattgcttctctaatggttaaatttagcacagaatcaaaggagagctataaagtctaggaagtacttatttacataggattgagtccagaacatcttgtgacaccatctacatatgttttacttggagaatagtctgaatttcgtattacacgttgagcatttctaatttgaaaatacaaaatcctcaaaaatctgaaattttttaagcatcaacatgatgcctaaagtaaatgctatttggaatatttcaaatttcagattaggaatattgaactggtatgtattccgcaaatattccaaaaatccaaaaaaattcaaaacacttctggtcccaaccattttggataggggatattcaacctatattacacacaggtaatacagcaggggaaaagcagggagactgcagcatctaagtctactaaattggccaggatcattccttagtcttcagatacctatttatcagggtctcattaaataaagttacttgtcatgttagttcagtctggcctgtggcttgtaattatagctgcaaactcaagggcaaagttcttaggattttgagatgctctttatgcaacaatacttccatttactttgtgtgtgtgtgtgtgtgtgtgtgggtgggtgggtgtgtgtgtgtagggagagaaagggggcaatggagtggagagtggaactacaatttattaagcacctattattacaagccaagtagggtgttaaatattttcctcgtgccattccattcaatactcttcgatcctgagggaaaacgaacccacttaaaaaaaaaaacaaaaggttttaatgaggattgcataagacatgcaaggtcaccagggagtttacatgcaagtggggagatacaaaataatacaacaaaagttcaggtgttctgaggaaaaagaagggcaagggtaagtgatgacagtgggggaagtcggattcaggataaaccaattttagactcattttttgaggaaggaactgagcatgaccttaccacacagcctttttagttaagtgtttctttaactaggaaaaggccctgggaagacaggctctctactatgcaaacccaattccagtcttgggagagaatttgctggtgggacaaaatcaggtttttcaagagatgcttaaatggtcaattctaattataaccatacttgtcaaaaggtgaagcaaagatgaaagttaaaaactaagaagaaattaaaattcccaaatctgtcaaccaatctctaattttctctgctactttaggactatagtaattagccataccctgaggatctactttacaagatatattcctctgacagtcccactctaacaatttaatctatcttatgtaagctggacaggcatttcaagtacaagaaacagaattcaaaacgtgaaaacggagccatctatcacacacggtgtcggttggagaagcatattgctcaggctgcagggacatttcatttatttaaatgtttttattaaaaaaaattaaagaccttcatggcacaacttcttcccagcacagttatggtttagtcataccaattacaatacaattacaaccaataaagcaaggtggggagggccttctggcttcaaacttaaaaaaaagcagaggaagaggggagggaccacttcaaacaaagtttaaaaatactttaaaaaatctttcagagtaattgccaacataacctttcatgttggccattccatttcctgccatctaagcaatgcagacacaggtagtgctgagaaatagtgtcccaatacaaggtatacagatgaggtaatttacaacaacacgtaagttgttactctgtaaacccttgcctcccccccaccccccacccaattgggtcttttttttttttctctctctccatgcttctgcagtgactcttaagtagcatttttaaaaacttctatttattttaaaaggctcttgggtggcacctcagagtcctctgcattcaccttcggtttattccaaggtctgatgggtgtaaggaggtccagctgtctgcagctctccgcatcagcctaagctacacctcaatttccgagctacaaggatagggtatgaagtcttgatttacaaccctctccccacctcaaaagaaagaactcattagttataagtgtcctgttcaaatcacaatccagtgcaaacataatcacaaattgcatctctggcacatctggtgcttttagcttctgcacaaattcaacatggtaaccctcacagcattctagggcataaaagggtcaagtacaataaatatccactgtaagtggtcataaggaagaaaatcaccctgccacacagtcagaatgttttcccttcagctctccctaccgttgagaagcgctataaaaggaggctttagcgtcctctaaagtttaccattatattcactaaagccaccaccttgataaagttactaaagccaagatgggttacaaagttagataagttcattaaattcaactccccaaacaattacgtttatctatgatgcctaggcgagaaaggcctgtgaatctataaggtaggagaatggggaactaagattttaggccttaaaatatgttggaagaatttttcctagttcccacaagcagctactgtaatgaaataacaggagaaaatacagagctgatggttttgctattgtgcttaaaaaactaggcttcctcagtgaagcacctgataaacttaggtggttggattacagtggaaagtccactttacacacacacacaaacacacaaaaactggcgactttttccatccccaatccctgcactgctgagacacaaaatgagttttatggcaaaggatccttaatccccagagacgctttggcttgtggtgctttttttttaaggcctctctgctctgcccggtaccatgggtcgaacgaggggtgtataaaatgggggccttgggaagcctccacggtacagggctgcaggcccctcagatgtgaacatgagacacccacccagcaagacctttacacagggaacttaaatctaaccttgataaataaaaccaaacgtttatttacaccaaagaattccaacactggatctttcacatatgaaggacaaagtattatatatatacacacagcaaggggtggcggggctgtaacaagagagtttatagttttcccacaattacaggtctaccatttcagcttcaatggagatagtggctctgctcctacctctcaagatacatttacaagactgaggagcaggtcttctcactggatggcatgtgagggaaggggacggtcggaggaaaagaaggtagaaagcttaaaatggaagtcagtgtggccacatctcccattagctctagcatgaaacctgtacagacaatgtttgtttcttttgtaaaaagcagtaagttatgcccagtaactaaatgaattcaaaatggccaagacaaagaaaactaagaaagattttgccttccctctcctaccagctatggagcacagcatgttgggagatgaacagggaaaagaccaaggtaaggagcctgggagggaaggtatcaacattttaaactgaactaaaaataaaagtataaatgagttggatttagggttagatcagtaagacatgattcttactgaacagaagtttttagtatctgtctgcattttgggtagattttcaacatcttgatgtaactaagacacacttccacaagagccactaggataaccccactgaagcgcttatggagtaaagtgatgtaagcgaccagcaagcagtccactgctcctatagattgggtcctcccttccttctttccttccttcctttcttcctgcctcccctgagaagctacatttttgtaatctctggagaagagcacgagataccaaccccctaaagtgtgggacggtggaggaacaatggtgggaatgggaagaagtctccacctaaatgcagcagccgggattgaggctggtttatctttgttcttttgtgatgaggaactaaatttgggaggggagaaaaaaaaatttgtccatgaaatattccacctgcaggtaatttttcagggaatcccctgagttatgaaaagttcgagttaaaaaaaaaaagaaaaaagaaaatcagcctattataattttttttttatgactgaactactataaatccacaagcaacggttcagacacggtgcttctgaagtgtttcacccctccccgccaggcgcaagctgcatcaaggagagggtggactcccccacctctgctcaggcatcaggagacagatagggccgttactgctgagcgccagcggcagctggaacaggcatcccaagggggttggcagcagcaatcactggtgagcctgccagaggtccaaggggtgaaggggttggcactgaagaaatccctgacatcatattggcgctgctgacgggcgtactgccccctggcatgctagatgaacccattcgagcctggtccttcacaacagtgtagaaataggggtgctccattgcctctcttgcagtaagccgtgactggtggtcatatcgcagcagtttgtccaggaaatccaaggcctcagggctgacaaggtgctgattttcactgtggacaaagcgttcccatcgctttcgagagtgtctgcccaagatatcattgaaacgtggatctaattcaatgttgtatttgtcaatatagtcatataaatcttctgtccccagaaccttggctatcctcaccaactgatcataattgtcatgtccatggaaaaatggctccttccgaaagatcatacttgccagcatacaacccaaactccacatatccaaactataatcgtacatctgatagtctacaagtagctcaggacctttgaagtatcgggaagcaactcggacattatattcttggccaggatgataaaactcagccaaaccccagtctattagtcgtagctttctgtgctcatgatcaatcatgacattatggggcttgacatctctgtgcataattcccatgctgtgacaataatccagggccttcagaatctcatacatgtaaaatcgaatatcatagtctgttaacgtctggtacaattgcttgaagtctgtgttgtttacgtgttcaaaaaccaaggcgggggttcgtgacacagggtcttttacaatgtctgccagtgtgatgatgttgggacctcctctcaaattctccaaaatctttatttcacgcttaattttcttcttttttactggcttgagaattttaacaacaactttttcattatttgtgatgttgatggcttcaaatacttcactgtatttacctcggcctaattttcgaaccagctggtagtcatcttgatttctgtggtggaagcggcagcggcggcggccgctctcccctctgctcacacagacaatatggcggcgatggaggaggagacacacggctcggccgccagccgcagggaccagagcgaggct

SEQ ID NO: 13328 - RNA, 14799 nt, Homo sapiens
  source 1..14799: mol_type = other RNA
gctgggattacaggcatgagccaccacgcccagctttttttttttttgagacagggtcttgctctgtcacccaggctggagtgcagtggtgagatcacagctcactgcagcctcgacctcttgggcttgggtgatcctcccacctcagccctcaagtagctgggactacaggcatgcaccaccacacctgatttaatttcctgtagagacggggtctcactatgttgccgaggctggtctttaactcccagactcccaaagtgctgcgattaaaggtgtgaaccatggtgcccgggccccagggccttcagagccacagctggctgcatctgtgtctgtgaagggccccaaggtcttcattcatgagtgctgtggccgctcgggagcgagctcatgatgaaagcgaggtggggaggggcatggctgccgtgggctgccctccctgggcagcatggaaggcaaggctctgtgccctgggatgaaagcggagacagaagaggcggagccggctcatgcttagtgttttatttcctcaaaggagccacgccattggccttcccaaatacctcctggtatccttccaatttccaccactcccaaccgtcagattccattcagcttcctccaacctcagaccaaccactttcttttcacaagctcagaccttccaaatattttaaaaatgaataaatgttaaataccaactttcactattacagaaaggggcagctagaaaagtttactctgtgcacaagactgcgacaccccgctcgtagaagctgcgaggatcctcctttgtagcaatttcgaagtccacggtgaagatgaggtctgcacgggtgaagttcaggtagacaggtaaggttaccacactggccttcttctcggtgtttgtctgcttgacccagcgcagctgcgtcaggggaagggcggttgagatggcattggacagtgacagcttgttgttgttgcacgtggccccttgaagtttcaaacccgtgactccgaagctgcaagcgtcaagggtggcgccctgtgaggtggtgacgttgacttccaggcagagctcctccagggaccagctgttggcctgggccacatactgcctggtggcagtgatgtacgcctcaggcacgaacaggccacccaggcacacgtggatgttctttagctccttggcgccaccagatgcagctgccagtgagatgttctgcagctgtttgatcctctcgctgaagtcggacacccactggatgacggtcatgccggcaggcaccgtgtagtgggaccagctccgaggcaagatccctttcactagctcgttgatcagcgtgcgcaagtagttggtctgcttcttctttccttcgcacacctggacgacatctgcaaggtcctggcgaacgtcctgaagcagctttgcgcccatcttcacttctctctcaaagaacctgaacaaaggatccttgatattctccacggtgcgcttgaggtggctcagcgtctgggggatgaggtgcagccagttggacgcggtggtgtgcagtgtccgcatccaggcagggcgcccgtcggacgtggagtctgtcctcgtcttcttctcagtctctgcgtaggccaggtcgtcctcatcctccaacatctgcatcttcagcattttactgatcatgtccacaccctgtgtggtaaggaggactctctcggcgttgttgggcaggcccagccaggagggcgtctgggtgtcggggagcaactccacccactgcacaaactcctctcgcctgatgccatctggcatttgaatgtctttatgtccgtcgaccttgcatgccagcttaaactcactgtcgaaactcctggttgtgaacaggcgctccaggaaggtgttgagcagacgctggtcaaactcgttgtccacgcgcccgccataaatggactgggccattaaggtctttagtgcagaccacgggatcttatccggtgagatgttctgcctgcccttggccgtgtcatccagccacgtgtccaccgtatcgcaagctgaccgcaggtcagactctccaaattcatacttctttgaccaccccagtggtgcgtatcgtaagcgttcttggatgatcgcatgaaaccaggccagcaggaagtacaagcgggcacgctcgttgggagacttgcatatccgtgagacgggaatgctgctgaacgtcctcagcatgttggccttcacccctggcggtggctcgaacacaaagatgcggcccgcacggagcagattcacaggcaccttggggttgatctccatggtgaggaagagtcggaagcaggcatgcggctgcagggaatgcaacttcttctccagctgcatcagccaccctggggccagatgcacattcttcagcatcacccacctgcccgactttacagcggtgtttattgccttatctgcttggttaaagccttctgcagagccgattgcaattgaagtgatctgcgtgttctgctcggctgcaaggtcctcgacatgtccactggcatcataaccaggcacagagcacattaagacaggagtgttgggcttcacctctgtgcccacaatgtgggtcaggtcgagcggctgctccatgatggacatgaaagactccccaaggtttgttgaaacaaacatgtgggccatggccaacaggcgatcgggccggaaagcctggatcaggagcaggcggtggatggcctggccaatgggtgttgcaggtgtttcttcactccagaggtagggcacagtctgctccggggagctgctgtccagccagatgccaaattgctcgtctgcctgaacctttgcaatcaagtccttaaacgcgggaaggcagctcagcctcaccaccgcctccgcctgctccacagtcaggccctggatcctgggggtggagccagcactcaggacaatctcatttcctctcaagaagtgctggaattctgcatcgtaggtgggctcccccacggtgcccttcagtttgattcttgccagcagcatggcaaaggtaatgtggtcctgatgcagcatgcctcgagccactcggttaaacgccacctggaagaggtcctttgttataatggacaggcgctgtgtgtggtcggtgacacccttcaggttcgggttctcgtataggacgttgtgataaatgtccaggaaaaactggagggagtactggtacaagaagtgtatctgcttgagggactccatggtgaagtagatgctgctgcaggcggtggagagcgggaggtactgctgggacacggtctccacctcctgcatgacaatgtccgtctcctcaactttcctggtgacctctgcagcctctctcttcaggttctccagagtggttatgatcgtgtcgtcatccaaaatgcgccctttcacctcgttcagagcttgtagtagagatttttccagctgacgcaaacggagctgaaattccccttgaagtttaagaagatcagatcgtttctcgtccacatcaggtctttctgctttaagtacttcatttagacactggctttgtaaactgctacgggtaactgtgaagtttacaaaagtaacccgggaacagagatctggtgggaactcgacagttggatcccgggtggacaggaagatgacaaacgatggcgacaggtctatgtcctggtccccgagagtgatcagcactctcccccctgttcgccgcacttcacggttcagcaccgggttcaaaactggatcgtagctttccacatcctggaccagaagggggttaccgaatctcagtgcactctctaagttctttctgaaggcgtcatccaggaagctggtccgtgtgatcttacgatccttatattcattcataatgaattctgtggcctgtccagaggggtcaatgatcagcggatacctattgaatcgtttcagcatgatggcattttctgtgcaaaggtcatcagcaggcaaggagctggcctgccagcgaagacgctcatcagcattggaaaggtattccgtcctggcaatatctgtacggaactggatgttggcttgctgtaggtgatgggaccaggtagtgaacaagttctgacgcatctgctggtcaaagtaacccgcgtaggcaatgaacgcagctgacaagagacagtccccagcaatggtggacatctggtttttgaaagtttcacttgttttttcccatcgttcacgttcagcagacaagctcttcagaagagcagtgctccggtttacttttgcctcgacagctgccaggtctgccttgatggcctgggcctctgagatcaggacggcgtattcctccttgtagcgggcgatgctggcttccaggtctcggatcatctgctccacctcgttggccttctgctggttgtccttggcgtcatcttccagcttctgcagctcattgcgtaggggctccactctctttaacatgtctgcatagttaagctgtgcaattgcccatttcaccatagggccgcaagccagggaagcccgattcacaatttcataattgtaacttggattggacatgtaatttttcttcatcttctcccttatggcgtcactgatctcctctgcagagaagttgacgatggtggggatgaagttctcccgcatgatgatggagcggatctgcttccagtctgtggtgctttcccccagcagcaggcagatggactccagcgccagcttcacagcagcaggagggttggccatggacctcacctccaccaggtgctgcttcttgatcgacttcacagcattctgggcctcaatgacggcaggttccaccttatcaagatcttctttgacactcatctgtttgtctgcaattacctcctgctgcttatgcagctgttcctggatttcttggctcataaccttcttcttttcagcctcctgctggtctttcaccatctttttcagcttgtcattggctgctgcattcttcacctccagctcttggctctttatcctcaagtcacgacgcagttcttctacctggtcgactgtctctttgatcttcctgagccccacgttcaagtgcatctgctgctcctccagctcgctccgcttctcgtggaacaggttggcatagtgattgatgaagtccaggtagtggcgaggggtgatggccatcgttctgccgcctcgctttgctagccgagcattcgcctggtgaagagtctgatgaacaaacacacagctgttcacaatggcttcccgatgggatggtggctgcggcagcttatcatacacaactggcatgtaatcaggcacgatgtaatttggcttctccagatccatcttacttgtgaattctttgccaacctgatacagtgcttcggtggaccagtctccaaaccaattcaacacacacctgttgaaaagtgctggtgatgtagctgcccggtccttgagtccctccgaggacgggttcatggtgaacacgacgtggaggttgcggataacctggctagtgaaccacttgtagagctcctcgtgcgagtccagcatcaggccttccttctgtgccccctctttgcactgcgtcatcaaggtggcatactcgtctccttcaaagagaccaggcacctctccattggccagaagggtattcattcgctccaggaatccagaatctaacacattagattcatccattataaatgctatcttttcatttttacagccagaacgtctcaacactgtccgtagatcttcatcaaagtcttcccctgtgtacttcctatggaccttaatctggtacacactcaaaccgttcatccaggcgacgaaacgagacagggtagtttttcctgctccactaacaccaatcagaagcaagtggccttgaggttgacggaatattctgtcaatcctcagcacgtggtctaggacttcattaaacagcaccagcggaacatcaagttcttcttcataaaagaccttcagcctagctttgacataatctcttaactcttcttggtctactgggatgtaatcctttgacagccagttgctgtacaagatgggtcggctcattgccttctctctgtcgatgttagggaagtgcttcagagcaaccgtgtcgatgttctcatcagtccaacgcctctcctcatcctctacgagtctatcttggaagagacgcagagcttcatgtgcccaaatccgaatgaggccttcaacaggcagggtctccagaggtctcagcgcttcaaagatgcctctcacccacctagtcatttcacggggtgaatagatatagtgaggttgtgtatcctgggtgaatctctcctgagacatggtgtagaactccaccatggcagcagtgagcggctctgcatacgtccgcagggatggaatgagcctcagcatggcgcggttgaaggtgccgtagatctgtgtgagggaggcggggcccgggtaatccacatacacgacaggcacgtggcgcaggaacctgtgtgagaggggctttcttccagggtctgtggggggattacaagccccaacaaactggattctctccagcttcacccatgtttgatctgaggtacggtaaaagcctccgtgctccaccatctgtctgatgaaggatatgaccctctgggtcccatatttatccatatctggcaagttgatttcatcacagaacaacaccagccactttccaagttgaacaggagccaaaaccaccccattaggtgtgcgcctgtactcgcagtagtgatcaaaagtcttcagaagcagctctggagtagtagcactggagaagttgagacccaccacctccatgtcaggcaaggcccggagggcgctgaagagtgtcatggtcttgccagacccaggagggccacacaagaccaggggcttgtgttcggccagccaagtgtacaagagggcttcgtggcggactgtgtccagcgttggcacgacgacatcaggggctgccaccttgtgcgtctccacttcaatctgaggcaccttggcctgccacggagaccattctccgctgatggacacctcataatcgataatgggtatgttgggcgcagtgggcagaggcacggtcgtgattcttctgatgtattcacccagctctgctctcatttttagccggctgtctccagacagggaccagagtatggcataaaccagatatcgctgaatgtagcgctccagctgctcgatctgcatggggaagtcgggatggttggcgttatactgcgccacgttgcggcaggcctggtgcagcatggagaagagcgagcccaggcagcgcaggcgtgttaggtccatgatgtgctccagctggaaggcgtgctctagcgccttggtgaccaggccgttggacgtgaagtacggttgcatgatcgtagctgcatctctttggatctgcagcatgggggaagcggcctcctccccctcatcctctttgcccttacgccgccgctgtgcctcatcctccccttcatccagcgggatgctgcgcagcctggccaggaagttgttgaagatcatgtcggtgctcagcacatcctcactgaaccagaccatgccgcagcgcgacactgtggccaaggtcgcgtatttcaagtcctgtacctcaaacattattctcacattgggtggaagactgaggcgctctccattgggcaaagttaggagcttattgtcatccagcactgagttcaagttctcaacccactctggatccacatcgccatcgaagacgatccactggcgcttctgcagctcgcctctcacgctgtcgatgatctttctcagcacgtgtgtgaagagcccatctgtccattccctggtgttggggtccagggttccgtagaggtggtctttgctgatggccttggggtcgatgatatgggccacaccttccacaccctcgagtctctccaatgccttcagcaggacacgccaggccatgctcttcccacttcccgagggccccaccatcatcaggccatgattgatctgggtgatctgatagagctggagaaccttttcaacccacattccaccaacttcttctccatctccatatgtcaaatacatctcctgacacactttcttcagctcctctcgaagggcagtcatctcacccctgtgatactggactccagggaacacgtccgacaggaggctgaagagcagcgggatgtcctctgccaccagctttggcaccatcgtctcacagacgctctgtatcagaatctcttgttcagggagattttcagcaatttctccttcatcaactgcttcccctcgttcctctttctccctctttatcttctggattctctctctcttcacattgcctgcactcaccagcacactcttcaaagcccgaagaccgaagtcataatggctttgggaagagagctgctcatcgcatagtttaaaaaacgggacgattttgttggcaagcacttcagcagtgcggaaaccctgtgagtacagcatgacctgggcgattaactgccggtcgggcttggtcatggccaagctccggaacagcttcttcaagttgtcaggaaggttagaccggcccgcgtagccagggttcatggtgatgaagatggccatgtccgggctcaccttgacttgtttgttcagcagctcacaagtaatgggggcagaggtcttgtcgtagttggggttggaatgttcacgcagtgcttcctgtatgcactgcacctgctgggacacagccgagagcatccgctcctccaggcggttgaactcgtcaaagcagccccaggcacccacctggcaaaggcccacaaagatccggcccattgcctggaaatcaaaggtttcatcacagttgaaaactaaaacaaaccgtccaagctgatggccaagagctttgacagactctgttttcccagttccagcaggtccaaatggggaaccccccagcctggcctccaaggcttgtgtcattgtcaaatagcagcggtcagtgaggggggtctggaccagtttgtcctgaacacccaggtactcaaagccatagttaaatttggcatttgccatttgaattgacaactgctgtaacacatcagtttgcttagggtcaaagtaaaatcgcatctggctgagccattcaaaagatttggcgttgtcaatcttgcttttgatcaaggaccttgtaacatctctctggtgaaccaactctgtaatcaagtgttctagcttccgccttcggagtgggggctgctccatgaggacagagtctgctaacacattgagggtgacctccacattgctcagcacagagtgcaagggcgcggcatctccacctccgcccatgctgctcagtgcggtctccacgttctcagaccaggctatctgggctgacaaaaccacaagctgggcctggtatttatcaatccaagtgatgtaggtatttgggtcaattgaagttgctttaccaaaaatctcaacttccgtaacagactcagcaagcagtttggccagggtgactctcatctccttttctaccaatgtgagccactcattgattttgggatgttcagtaattgacacaggagttttaaacataacctcctctccttcccgagatgaaatacccaaaacaacagagttatcctcgttcaggatgatgctcgaaactccagcaaacatcttcttgaagtgtttctgtaatttagcgacattcttgctgtttccaatgatttcaagcaaatcttcatcacccacaaaatagaacctggggaaagatgaccgctctctttccagatattctcccaatgctttctggatctttcctagcaggtctgccaatctttccagagacctctgtactccctggatgttcagaacatccataacaaggggagacttggacacttttttcattagagccaaaaactcagtgctgatgctctgaaaccgctgggtttccactggcagcaggtgcttgatatctgcactgcctgtgaagataccttccaggtagacccaccgcctctgcacatcaatccacacatcaaagagagccatgatcctgttcagcttatcttcccagctgagagcatcctcttcaaaaaccttgtaatacggagagagcttcatggccgagacgctgttgatgtgttctttgaccttgttgaagaggtcatcccagccacggatcaagcggcacttgttctgataattaaccaagtctagttcataagtattccacacttctcttatctgcttcaaaaattcttccaaagccatctccccttgtgccacaagcagtacatccttgacaatcgcttcatttttctgcaagtcaacatcccagatttggccaagggttagctcagaaacaacccaattaacgtgaagccttttcatgagctgtttccaatggcggtctttaagtgcttcggatttcagttcaatcaccagcatatttatcttcatgtaacctttcagaagcctctgaacaaactcataggacgcatactgtcgcaaccgggcagggaagcttttcagctggttcaggagggcatccaaattttgtcgaagctttcgaggctgtactgaaacccagggttgctccttcatctgatcgatttgctcccaaaccttagaaagttctgaccaaacgcctttgaggtcctgtaattcttctaaggccacctgcacgcgctcttcactgccactgagaagcccagtatctgtcaattccagcgcctccttggcctttgcacacttctctctgtcgtccttcagcctaccaaacttcccctcatatatggtgagagcctgaagtgcctcttctgggcgaaggttgcccgtgacaggcttggtcttctcccagtcagtcagcaggtcggtggtgcggctttccacggcccgatcctcctggacaatcttcatttgcaggtttgccacctgctgctgaatggcagagtcctttcgccgcatgatgtcattgaaggctccccactctccctcgatgttgtcaatataaagccaggaaggtgggaactggaacctttgcttttccagtaagcgctggccattgcggtagagctcaacttgcttctcaaactgcttgatcttccgtttcaaagactgcacataggtgatgaaggtcactgcatcggaggtgctggccgtgtctactgagtgctgctccaactcttggcgggactttgagatctgggaatggaattccgtcatgtttgatcctagcatctgcccaaatttgctaagaacctccttatgccaagagtcatatttcaagttcaccttagattgtaccttgccataatctataactactggtccaaactctttcttggtttctgcattgtcaaaggttcctctggccttccttatttggaccaggagagcctgccatttgttgagatcttctccaagtctgttatagatgttttcagcttgcatatcccataaacactgatactgaagccaaaccttgacatactgttcaacttcagatacaatgcccatgacagcagaatacgactcttccagggcaacagggccatcaggcatccgtgttaaagcattccgatagaatttctcttcctcagtcaattcgtaatgtacacccacctggtacctctgactctggatcctggggagagacagtacaaccatcttccaggcaaacatttcctgatacagcttgtatctgcactcttcaattggtggattcaagtagattacctgattggttattcttagctcatgaacgacatttttgatctttggctctccaccaggcttgtgactaacttgtggagcatctgtgtccatgtcaacttctgctttatcttcagcttgtccaagaagaacctgcgtccaagctctcaggccagcttgcagacggacgcccaatattctttcaatctccatgtcaagcttgttgacccagatgggcaaattggaataggagtgcagatttaagtcatccactgctttctggactctgttcaagatttccgagaatgtcttatggtcatacatacaagtttccaaggaacggacttctaggtctattttttcttcaatgatcagcagatcatccaccttttcttggaagttgaagacagtctctgctaagcgctgtacatatgggtcaagtttgtaggactcccacaccaacgcaatgccttctgcgatcagggcctgcacttcctttttcaagccagccaccaaaagggaaatggtgttccgctcctccaccttctcgcaggtccgttcataggtacgaacgctctcgatcagtgagatggcaaacgggtaaagctggtttgcttgatgggctttgttcacaatcgccagtgggacgcggaaaccaagccatttgaggttccggacttctttggatagtgtgataatctcaggaagaaagttaactttcagcttaagcacatttccagttcggccccgaacccgagtactttcgatggtgaaaatgcgccccgagacaccgaggttgcgctgctgcaccttccttgcccagtcatcaaagatctcctgcgtgttgagcttcatgcggaagctgtctccatcctgcttcagcttctgcccctccacgtgattctcccagcccttgccaaggacatcttccacccgcttcatgtaggccgtcagctgcctgtcgatctgtttagcccagatgatagaccctgacacagggggcaagtcacgaacgtgactcatcttacaagcctgactctgtgggtactggaccttgaacttgtcgtgaagagactcaatgtcatctttcacgcgctggatcagctgggtctggtattcgcgaatggccccacggatgtgaggcctgacaaacagtgcattaaacctggagaaaatcctaaacatctcgttggcattcttggctgtgccaagctgatcccgaaggcgagcggtgatccgggtctccactctgtcgatcctctcatcgtacctcttcatagcagcctcccaggcttccgtgccctctttggaaacatccagtccatccacttccttgacgttctcataagcaaggtttacttcctcaatggcatttgcatctgcagcatcaaagagaacctcagccactttcatatcttggggttcagggacctctccttgattctgttgtgcaactgccgtgacctgtggcctcaggaccctgacgataacagctcttagctgttcatgctggcgtctaaattttctcatctggtcaaggcgggcctgcagcttcctgtgggcagggttgatacgccacaccatcttcagattttcttccctttttcttttgacgatgtctctcaacaatacctgaagtttctcatactcatcatcccaagtctgaaaaacttcaaagcatgctaccataactttttcaaattcttcataagcaacatgcatcaatttcctagtgcccaatactttgagtaattgagaactcaagtctcttgaaattgcctccaccaaacgcagtgccctctgaataggatattttgtgtttcggatctttctcaaatgtgtgaaaatggcaacaagcgcctgtcttattttgtccagctccgtggcagacagcaaatcattcagagggaaatctttcatcagaggattgtagtcattcacagtttccaaagcctgttttagacctgtgtcagtgtcaaaactgacggtggcatggaagcgcttgccatgtttcaagatatccagagtcaggagaacttccgggctctcccgtttctcctggatgcggtataacgcacgttccaagtttagccaaaaactaatttcctgtaaggcagttcctgatgcaggatctcgatccagtttggtcactttttgaatttctcggatccagcggttaactccagattgtaactgattaagaaatgttgggtcttcaaccttatcaccaaagtctgtaacttttggcttttctccacgctcataacactgttttgcaacatttgtgatcattggatgaatcggcaggctgatctccggaatttcaatattttgctgcaagtgaaggagtcccatttcgagttctgcaatcttcttttcaactgaaggagccattttatcaccatccctgtctgccttgccagactctctaatgtaggacttaaaaaaaggagccactgcattgctaatgaaagaatgcaaagtttcgtagggcgagtcttcactgagtgtaaggacccggagctgagaagacacgggtttatctgcatcaatcacgggagtacgtttaatgaatgccaagctattggatttaaccccataatgaatgtctatgttgatgttataggaaatgaattctttttcttcttctccttcatcaccgacgtcctctttgagcgtggagcgctccaccagcaccgtgtggacctgcgggtccgaaaggaacttgcgcatctgctccagggcgctcttctcctccagcgccgcctccagcgcggccggcgcctcgccgccgtcctccagcagcagcggcaccagcttgcgcaggtgcttctgcagcaccgacacgtccgccacattctgcacggccgacacttccaatccggccgagccgtcctcgccgccgccgcccccgggctccgacatggtgtcgcgctcgggaccttccaggagcgatgagaaggcggccgcgactcagcgagacagccagcaagagacagaaacggccgccggaagccggaccgtccgctagcccaccgcagact

SEQ ID NO: 13329 - RNA, 922 nt, Homo sapiens
  source 1..922: mol_type = other RNA
gctgggattacaggcatgagccaccacgcccggcaggagatccagcttcttaagcctcaaactcaaattcgaagtactgtgggtcgaagtaatggatacggacgtaaccatcttcgccgccgctgctgtagctcttgccatcaggatggaaggcaacactgttgataggtccaaagtgacccttgactcttccaaactcttcttcaaaggccaaatggaagaacctggcctcaaacttgccaatcctggtggaggttgtggttacatccatggcttcctgaccaccgcccaggaccacatggtcatagttgggggagagggcagctgagttgacaggacgttctgtccggaaagtcttctgatgttcaagagttgtggagtcaaaaagcttggctgtgttgtccttggacgcggtcacaaacatggtcatgtccctggataactggatgtcgttgatctgccgggagtgctccttaacattcaccaacacctctccagactgtttcacagtcccagagacgacagctgttgtcagctgagccagtgaggacatgcttggtgtcccagtcagcgtccacacaccacacagctccggtatggcccatgtaggtgcccagcctctcaccattcacagagtaccatacattgacgatagggtccttggccacagtaaagaggaggtctccttcgcggttatacttaatctgcgtaatggaccgctcatggccctgcagtaggatcggcttcatcccggctgtgacgcgaggaaggccgcaacgtgagtaagaccggaaaaggtttcgaggtcacttccggattatgggtctccgccctcgtctgcattcagggcaggtgttggctctggtgctggtggccgctctgtggggtggcacgcagccgctgctgaagcgggcctccgccg

SEQ ID NO: 13330 - RNA, 1560 nt, Homo sapiens
  source 1..1560: mol_type = other RNA
gctgggattacaggcatgagccaccacgcccggcaggagatccagcttcttaagcctcaaactcaaattcgaagtactgtgggtcgaagtaatggatacggacgtaaccatcttcgccgccgctgctgtagctcttgccatcaggatggaaggcaacactgttgataggtccaaagtgacccttgactcttccaaactcttcttcaaaggccaaatggaagaacctggcctcaaacttgccaatcctggtggaggttgtggttacatccatggcttcctgaccaccgcccaggaccacatggtcatagttgggggagagggcagctgagttgacaggacgttctgtccggaaagtcttctgatgttcaagagttgtggagtcaaaaagcttggctgtgttgtccttggacgcggtcacaaacatggtcatgtccctggataactggatgtcgttgatctgccgggagtgctccttaacattcaccaacacctctccagacttggcactatactggttgagctctccactctcatggccagcgatgatgcactcccccaggggtccccaaacagcactggtgattttagagtcattgcaagggatcttcatgtagggctcattgttgtcaatctggctcggatcccgcaggtcaaaaaagctcacaaagcactggtagcccatctgcttgtccgtggagaacatgatgatgttgcccccaaagtcaaaaccgcaggtccggacagccgaattggtcttgagaagggccagctgctttcctgtttcacagtcccagagacgacagctgttgtcagctgagccagtgaggacatgcttggtgtcccagtcagcgtccacacaccacacagctccggtatggcccatgtaggtgcccagcctctcaccattcacagagtaccatacattgacgatagggtccttggccacagtaaagaggaggtctccttcgcggttatacttaatctgcgtaatggaccgctcatggccctgcagtaggatcggcttcatcccggctgtgacgcgaggaaggccgcaacgtgagtaagaccggaaaaggtttcgaggtcacttccggattatgggtctccgccctcgtctgcattcagggcaggtgttggctctggtgctggtggccgctctgtggggtggcacgcagccgctgctgaagcgggcctccgccggcctgcagcgggttcatgagccgacctgggcccagcagttgctacaggagatgaagaccctcttcttgaatactgaggtgcgtctctgtgaaaggcccctctctcggtggagttgccgccaagaatttggtctttggagtcaaacaggtctgggtcagccccaccacttactcactagaaattctcggaaaagtcagttgtccttgagcctcagtttcatcatctgtaaatggcgattataataataaccatctgataggtcagttgcaggaattaggtgagatacgtagagcacttagcattaggcctagaacatagtaagtgctcaatctatggctgccattattcacattttattgt

SEQ ID NO: 13331 - RNA, 3817 nt, Homo sapiens
  source 1..3817: mol_type = other RNA
gctgggattacaggcatgagccaccacgcccggccaaaaacatttaaaaaatgactgtccctgctcaaatactgcagtaggaaatgtaatttgacatatatcacttccagaaaaaaactttaaatctttctataaaatgaatttgatacatcatcagcatgaagtgaagttaaaatctcttacaaagtaaattcaggtatatcaacaatgagatccaaaagtatcggttcaagatcaaagactcatatgaggtaaaggcaaataaagcccctcatgctttcagacatttacttgttatccttaaaatgattattgttctaaggtgcaaatcttatcattcagtgacctatttgctatttggctgtttatctcctttaaataaaataccatacaggttataatgtacattttaaaatcaaatatgaaagtacacatatgtgaacaagacattaatttaaatatcaattatattcataatacagaagtctaagaatgctatttggtcatttcaattagatgctgatatatttggtcaagaaaacccacattcctatcagcctaaggcaaatagtaaatgcctctatttttattaagtggactataaacagtagacattattgtttgatactactggaatgctctcaattagaacgtacactgataacaaatatgtctttctaatctgggtgataacctcaatgattacatggaaatctacaagtaacagtctataacttaaagcagtagagcacctggtaattgtcatacagtgcctctctatgaatttagaacattctacttacattggcagtggagagaaaagaccccttcacactgagacttcctgtgcaccgcgcctgccgcctgcctcagcttaggacatggtacagtcttctttgcttttgcccttctcattccctcctctggtatcttctctgctttctggattgaagtgccctggctctcttcctggtgccgacaagtcatcgttctctaggctattgctgtctaaagctttcctgacggtctgacttggatgttctgacatctcacacctctctgtactttctgcttcacaggcatcactaatgtcctgtgagggactttcatgttcgggcagggtgcagcgatctgcgtcttcgctctttggttctgcaggactgctttgagtggcaccatctattttagcattatcttttgcaacaccttcatctaattcttcaccaccagccctcgggcctgatgattgaacggtgtcatcctcaaaatctaatgtgtctccatcagctagtacctcctcagctgctgtttgtacatcatcaccttcttggtcaagttttccatccaacttaattttaggattctccggacaatcaacattttcactgctttctgctgcaattttctgttttggattttcagtcacctcgttttgggcttccactgctgactttctgtcagtagactttacctgctcttcttccttaatttcacttaaatctgtgttctgatacgttaactcttttttaacatctttaagggtttctacgggtactggggattttttcttcttgtttttctttttcttgttctttgtcttcttctgcgatgagtccaatgcctctccctgttggtcactcttttcttcatcgggctctttcatatctaagggttcattttgagtgtctactgtacttggacctgtcgcttcctgacagttgccctcagttcctgctggagaaccaggaacttctgtcttgattggtttctcgtcccttaatcctgtttcttcaccctcttcttcgttgtgatccctacctacttctgtactgtgcgctggaacctccttgggctcagctgcttcctggttggtgaattctttctctaaactatgccctgtgcttgtctctaactcttgggggacctctaccatacatttgtcatcatgataaactgtgtcatcactatgccctaaaggacacgaggccactgtgcctgcctgctcttcaacctgagtcactgctgcctctcccacattctctgtgtggttcccaccatctaagtcactccaacagttggatggctcaaggggagttctggtcctgtcatctggtgcacccatgacctcatttgactcaacctgtactgtgttttcagggagagaactgctctcaagaatttggctttgaacctgttcctcataggtagcacctgctaaggttcctaggaatggggcagtgtcttcagaggatttctggtcctcggtattctcaccagcagggaatacctctatgtccacacagtccttcactgtgtcctctgtgtgttgttctttctcagtattgtgcaagatttctcttttccccacattcgccacgatttcatttttcacctccacttcactggctcttcctagggtcccatcccctgtcgacttgagggcatttaactcttcttttgtcatcttggtaggaccttggtatccaacattattgagggtgtcggaagtctctccattggtagctatttctgaatttaggattattccatgtttctcgagcatttcctctctttgcttcagggcctccttgacttcagcaaactgaaattgcagtatactgtgggcgtgtttttccctttcaaattctttgtttttctcttcgtactgccgcctagattcagccagctgttcttcaagctccagcaacatatcttttagggtatcaacctggtacatgaagtttgtcttttcattgtctagctgagcattggaaaccatagccttcttatatttctcttcaacttctgctagagagtccttcatctctttcaatccctgcatgtatttgccttctacatcctgaatctggtcctttaactcattgagttccttgatttccctgatggatgcctcggtgtcgatggagatggaggtgtctccgctgcctctccgagaggaagtcccacccagagaggccagcgtggctgcagacaggcccggcatgttacgagaccccttctcagtaaaatctttttctggtctctcttctaccacagggctggcccgggccgagctggccctggaggaggcgcgggagctggagttgaggtggccgctgtactccgagggagcacgggagccggaggtgctgccccgtcgggtcccaccgaagctgccttcatccaacacagacgcccggtaactccccgaaggccgggcagcgctgtacagacaggagggcaacttctcctccctggatgatgacaaagtagagaatctgctgtcaccgctgtagctggaattcctgccagatcttctattcagggactgtgatccatacaattctccatcataaccatttgtccaggcgtaaggacccccatactccaagtcaggctgcgacctcaggcttccacgactacccactgacatgcgctcgtcttcatcagaagccgatgtgtttcttctggatctacgagagtagcgctcactgtcttccatccactgctcgatgtcaccccattttgtatccagcccataatatttcttttggacctgatagatctccttctgctgccgctccagctccttcatgcggatctcgcgagcctccgcgcgggccgcccgttttgcagcgagccgggcttccgcctcccgcgcgatctggttgagcgcgtcgtcctccgccgtgagccgctcccggttggggagccgcttgcgccccgatccctgggtgcccatgtccatcgaccgcgtcgcccgcagctgccgcggggcccgttgctccagccgctcgcgccgccccggcccggcccc

SEQ ID NO: 13332 - RNA, 3395 nt, Homo sapiens
  source 1..3395: mol_type = other RNA
gctgggattacaggcatgagccaccacgcccggccaaaaacatttaaaaaatgactgtccctgctcaaatactgcagtaggaaatgtaatttgacatatatcacttccagaaaaaaactttaaatctttctataaaatgaatttgatacatcatcagcatgaagtgaagttaaaatctcttacaaagtaaattcaggtatatcaacaatgagatccaaaagtatcggttcaagatcaaagactcatatgaggtaaaggcaaataaagcccctcatgctttcagacatttacttgttatccttaaaatgattattgttctaaggtgcaaatcttatcattcagtgacctatttgctatttggctgtttatctcctttaaataaaataccatacaggttataatgtacattttaaaatcaaatatgaaagtacacatatgtgaacaagacattaatttaaatatcaattatattcataatacagaagtctaagaatgctatttggtcatttcaattagatgctgatatatttggtcaagaaaacccacattcctatcagcctaaggcaaatagtaaatgcctctatttttattaagtggactataaacagtagacattattgtttgatactactggaatgctctcaattagaacgtacactgataacaaatatgtctttctaatctgggtgataacctcaatgattacatggaaatctacaagtaacagtctataacttaaagcagtagagcacctggtaattgtcatacagtgcctctctatgaatttagaacattctacttacattggcagtggagagaaaagaccccttcacactgagacttcctgtgcaccgcgcctgccgcctgcctcagcttaggacatggtacagtcttctttgcttttgcccttctcattccctcctctggtatcttctctgctttctggattgaagtgccctggctctcttcctggtgccgacaagtcatcgttctctaggctattgctgtctaaagctttcctgacggtctgacttggatgttctgacatctcacacctctctgtactttctgcttcacaggcatcactaatgtcctgtgagggactttcatgttcgggcagggtgcagcgatctgcgtcttcgctctttggttctgcaggactgctttgagtggcaccatctattttagcattatcttttgcaacaccttcatctaattcttcaccaccagccctcgggcctgatgattgaacggtgtcatcctcaaaatctaatgtgtctccatcagctagtacctcctcagctgctgtttgtacatcatcaccttcttggtcaagttttccatccaacttaattttaggattctccggacaatcaacattttcactgctttctgctgcaattttctgttttggattttcagtcacctcgttttgggcttccactgctgactttctgtcagtagactttacctgctcttcttccttaatttcacttaaatctgtgttctgatacgttaactcttttttaacatctttaagggtttctacgggtactggggattttttcttcttgtttttctttttcttgttctttgtcttcttctgcgatgagtccaatgcctctccctgttggtcactcttttcttcatcgggctctttcatatctaagggttcattttgagtgtctactgtacttggacctgtcgcttcctgacagttgccctcagttcctgctggagaaccaggaacttctgtcttgattggtttctcgtcccttaatcctgtttcttcaccctcttcttcgttgtgatccctacctacttctgtactgtgcgctggaacctccttgggctcagctgcttcctggttggtgaattctttctctaaactatgccctgtgcttgtctctaactcttgggggacctctaccatacatttgtcatcatgataaactgtgtcatcactatgccctaaaggacacgaggccactgtgcctgcctgctcttcaacctgagtcactgctgcctctcccacattctctgtgtggttcccaccatctaagtcactccaacagttggatggctcaaggggagttctggtcctgtcatctggtgcacccatgacctcatttgactcaacctgtactgtgttttcagggagagaactgctctcaagaatttggctttgaacctgttcctcataggtagcacctgctaaggttcctaggaatggggcagtgtcttcagaggatttctggtcctcggtattctcaccagcagggaatacctctatgtccacacagtccttcactgtgtcctctgtgtgttgttctttctcagtattgtgcaagatttctcttttccccacattcgccacgatttcatttttcacctccacttcactggctcttcctagggtcccatcccctgtcgacttgagggcatttaactcttcttttgtcatcttggtaggaccttggtatccaacattattgagggtgtcggaagtctctccattggtagctatttctgaatttaggattattccatgtttctcgagcatttcctctctttgcttcagggcctccttgacttcagcaaactgaaattgcagtatactgtgggcgtgtttttccctttcaaattctttgtttttctcttcgtactgccgcctagattcagccagctgttcttcaagctccagcaacatatcttttagggtatcaacctggtacatgaagtttgtcttttcattgtctagctgagcattggaaaccatagccttcttatatttctcttcaacttctgctagagagtccttcatctctttcaatccctgcatgtatttgccttctacatcctgaatctggtcctttaactcattgagttccttgatttccctgatggatgcctcggtgtcgatggagatggaggtgtctccgctgcctctccgagaggaagtcccacccagagaggccagcgtggctgcagacaggcccggcatgttacgagaccccttctcagtaaaatctttttctggtctctcttctaccctcaggcttccacgactacccactgacatgcgctcgtcttcatcagaagccgatgtgtttcttctggatctacgagagtagcgctcactgtcttcctccttctgctgccgctccagctccttcatgcggatctcgcgagcctccgcgcgggccgcccgttttgcagcgagccgggcttccgccagcttctgcgcttccgggctcaaacagtcgatctcccggctttgagcggccgcggggctggtcatcctgccgggctcggcccgctccacccggcgggaaatgctcggggaccgcgccgggagcccctcgcgggccgggccagggggcgcgcgctctgtc

SEQ ID NO: 13333 - RNA, 3552 nt, Homo sapiens
  source 1..3552: mol_type = other RNA
gctgggattacaggcatgagccaccacgcccggccaaaaacatttaaaaaatgactgtccctgctcaaatactgcagtaggaaatgtaatttgacatatatcacttccagaaaaaaactttaaatctttctataaaatgaatttgatacatcatcagcatgaagtgaagttaaaatctcttacaaagtaaattcaggtatatcaacaatgagatccaaaagtatcggttcaagatcaaagactcatatgaggtaaaggcaaataaagcccctcatgctttcagacatttacttgttatccttaaaatgattattgttctaaggtgcaaatcttatcattcagtgacctatttgctatttggctgtttatctcctttaaataaaataccatacaggttataatgtacattttaaaatcaaatatgaaagtacacatatgtgaacaagacattaatttaaatatcaattatattcataatacagaagtctaagaatgctatttggtcatttcaattagatgctgatatatttggtcaagaaaacccacattcctatcagcctaaggcaaatagtaaatgcctctatttttattaagtggactataaacagtagacattattgtttgatactactggaatgctctcaattagaacgtacactgataacaaatatgtctttctaatctgggtgataacctcaatgattacatggaaatctacaagtaacagtctataacttaaagcagtagagcacctggtaattgtcatacagtgcctctctatgaatttagaacattctacttacattggcagtggagagaaaagaccccttcacactgagacttcctgtgcaccgcgcctgccgcctgcctcagcttaggacatggtacagtcttctttgcttttgcccttctcattccctcctctggtatcttctctgctttctggattgaagtgccctggctctcttcctggtgccgacaagtcatcgttctctaggctattgctgtctaaagctttcctgacggtctgacttggatgttctgacatctcacacctctctgtactttctgcttcacaggcatcactaatgtcctgtgagggactttcatgttcgggcagggtgcagcgatctgcgtcttcgctctttggttctgcaggactgctttgagtggcaccatctattttagcattatcttttgcaacaccttcatctaattcttcaccaccagccctcgggcctgatgattgaacggtgtcatcctcaaaatctaatgtgtctccatcagctagtacctcctcagctgctgtttgtacatcatcaccttcttggtcaagttttccatccaacttaattttaggattctccggacaatcaacattttcactgctttctgctgcaattttctgttttggattttcagtcacctcgttttgggcttccactgctgactttctgtcagtagactttacctgctcttcttccttaatttcacttaaatctgtgttctgatacgttaactcttttttaacatctttaagggtttctacgggtactggggattttttcttcttgtttttctttttcttgttctttgtcttcttctgcgatgagtccaatgcctctccctgttggtcactcttttcttcatcgggctctttcatatctaagggttcattttgagtgtctactgtacttggacctgtcgcttcctgacagttgccctcagttcctgctggagaaccaggaacttctgtcttgattggtttctcgtcccttaatcctgtttcttcaccctcttcttcgttgtgatccctacctacttctgtactgtgcgctggaacctccttgggctcagctgcttcctggttggtgaattctttctctaaactatgccctgtgcttgtctctaactcttgggggacctctaccatacatttgtcatcatgataaactgtgtcatcactatgccctaaaggacacgaggccactgtgcctgcctgctcttcaacctgagtcactgctgcctctcccacattctctgtgtggttcccaccatctaagtcactccaacagttggatggctcaaggggagttctggtcctgtcatctggtgcacccatgacctcatttgactcaacctgtactgtgttttcagggagagaactgctctcaagaatttggctttgaacctgttcctcataggtagcacctgctaaggttcctaggaatggggcagtgtcttcagaggatttctggtcctcggtattctcaccagcagggaatacctctatgtccacacagtccttcactgtgtcctctgtgtgttgttctttctcagtattgtgcaagatttctcttttccccacattcgccacgatttcatttttcacctccacttcactggctcttcctagggtcccatcccctgtcgacttgagggcatttaactcttcttttgtcatcttggtaggaccttggtatccaacattattgagggtgtcggaagtctctccattggtagctatttctgaatttaggattattccatgtttctcgagcatttcctctctttgcttcagggcctccttgacttcagcaaactgaaattgcagtatactgtgggcgtgtttttccctttcaaattctttgtttttctcttcgtactgccgcctagattcagccagctgttcttcaagctccagcaacatatcttttagggtatcaacctggtacatgaagtttgtcttttcattgtctagctgagcattggaaaccatagccttcttatatttctcttcaacttctgctagagagtccttcatctctttcaatccctgcatgtatttgccttctacatcctgaatctggtcctttaactcattgagttccttgatttccctgatggatgcctcggtgtcgatggagatggaggtgtctccgctgcctctccgagaggaagtcccacccagagaggccagcgtggctgcagacaggcccggcatgttacgagaccccttctcagtaaaatctttttctggtctctcttctaccctcaggcttccacgactacccactgacatgcgctcgtcttcatcagaagccgatgtgtttcttctggatctacgagagtagcgctcactgtcttcctccttctgctgccgctccagctccttcatgcggatctcgcgagcctccgcgcgggccgcccgttttgcagcgagccgggcttccgccagcttctgcgcttccgggctcaaacagtcgatctcccggctttgagcggccgcggggctggtcatcctgccgggctcggcccgctccacccggcgggaaatgctcggggaccgcgccgggagcccctcgcgggccgggccagggggcgcgcgctctgtccgcggagacggagccactcgccgctaagtgaacgctcgcgcttccggggccaggagccagcccgccggggagcggctcgcggcgctgggctcgggcgcggccgacaggggcggggcgcaggtggccgcgggctgagtcgggctcggggtggaagggc

SEQ ID NO: 13334 - RNA, 3565 nt, Homo sapiens
  source 1..3565: mol_type = other RNA
gctgggattacaggcatgagccaccacgcccggccaaaaacatttaaaaaatgactgtccctgctcaaatactgcagtaggaaatgtaatttgacatatatcacttccagaaaaaaactttaaatctttctataaaatgaatttgatacatcatcagcatgaagtgaagttaaaatctcttacaaagtaaattcaggtatatcaacaatgagatccaaaagtatcggttcaagatcaaagactcatatgaggtaaaggcaaataaagcccctcatgctttcagacatttacttgttatccttaaaatgattattgttctaaggtgcaaatcttatcattcagtgacctatttgctatttggctgtttatctcctttaaataaaataccatacaggttataatgtacattttaaaatcaaatatgaaagtacacatatgtgaacaagacattaatttaaatatcaattatattcataatacagaagtctaagaatgctatttggtcatttcaattagatgctgatatatttggtcaagaaaacccacattcctatcagcctaaggcaaatagtaaatgcctctatttttattaagtggactataaacagtagacattattgtttgatactactggaatgctctcaattagaacgtacactgataacaaatatgtctttctaatctgggtgataacctcaatgattacatggaaatctacaagtaacagtctataacttaaagcagtagagcacctggtaattgtcatacagtgcctctctatgaatttagaacattctacttacattggcagtggagagaaaagaccccttcacactgagacttcctgtgcaccgcgcctgccgcctgcctcagcttaggacatggtacagtcttctttgcttttgcccttctcattccctcctctggtatcttctctgctttctggattgaagtgccctggctctcttcctggtgccgacaagtcatcgttctctaggctattgctgtctaaagctttcctgacggtctgacttggatgttctgacatctcacacctctctgtactttctgcttcacaggcatcactaatgtcctgtgagggactttcatgttcgggcagggtgcagcgatctgcgtcttcgctctttggttctgcaggactgctttgagtggcaccatctattttagcattatcttttgcaacaccttcatctaattcttcaccaccagccctcgggcctgatgattgaacggtgtcatcctcaaaatctaatgtgtctccatcagctagtacctcctcagctgctgtttgtacatcatcaccttcttggtcaagttttccatccaacttaattttaggattctccggacaatcaacattttcactgctttctgctgcaattttctgttttggattttcagtcacctcgttttgggcttccactgctgactttctgtcagtagactttacctgctcttcttccttaatttcacttaaatctgtgttctgatacgttaactcttttttaacatctttaagggtttctacgggtactggggattttttcttcttgtttttctttttcttgttctttgtcttcttctgcgatgagtccaatgcctctccctgttggtcactcttttcttcatcgggctctttcatatctaagggttcattttgagtgtctactgtacttggacctgtcgcttcctgacagttgccctcagttcctgctggagaaccaggaacttctgtcttgattggtttctcgtcccttaatcctgtttcttcaccctcttcttcgttgtgatccctacctacttctgtactgtgcgctggaacctccttgggctcagctgcttcctggttggtgaattctttctctaaactatgccctgtgcttgtctctaactcttgggggacctctaccatacatttgtcatcatgataaactgtgtcatcactatgccctaaaggacacgaggccactgtgcctgcctgctcttcaacctgagtcactgctgcctctcccacattctctgtgtggttcccaccatctaagtcactccaacagttggatggctcaaggggagttctggtcctgtcatctggtgcacccatgacctcatttgactcaacctgtactgtgttttcagggagagaactgctctcaagaatttggctttgaacctgttcctcataggtagcacctgctaaggttcctaggaatggggcagtgtcttcagaggatttctggtcctcggtattctcaccagcagggaatacctctatgtccacacagtccttcactgtgtcctctgtgtgttgttctttctcagtattgtgcaagatttctcttttccccacattcgccacgatttcatttttcacctccacttcactggctcttcctagggtcccatcccctgtcgacttgagggcatttaactcttcttttgtcatcttggtaggaccttggtatccaacattattgagggtgtcggaagtctctccattggtagctatttctgaatttaggattattccatgtttctcgagcatttcctctctttgcttcagggcctccttgacttcagcaaactgaaattgcagtatactgtgggcgtgtttttccctttcaaattctttgtttttctcttcgtactgccgcctagattcagccagctgttcttcaagctccagcaacatatcttttagggtatcaacctggtacatgaagtttgtcttttcattgtctagctgagcattggaaaccatagccttcttatatttctcttcaacttctgctagagagtccttcatctctttcaatccctgcatgtatttgccttctacatcctgaatctggtcctttaactcattgagttccttgatttccctgatggatgcctcggtgtcgatggagatggaggtgtctccgctgcctctccgagaggaagtcccacccagagaggccagcgtggctgcagacaggcccggcatgttacgagaccccttctcagtaaaatctttttctggtctctcttctaccctgccagatcttctattcagggactgtgatccatacaattctccatcataaccatttgtccaggcgtaaggacccccatactccaagtcaggctgcgacctcaggcttccacgactacccactgacatgcgctcgtcttcatcagaagccgatgtgtttcttctggatctacgagagtagcgctcactgtcttccatccactgctcgatgtcaccccattttgtatccagcccataatatttcttttggacctgatagatctccttctgctgccgctccagctccttcatgcggatctcgcgagcctccgcgcgggccgcccgttttgcagcgagccgggcttccgcctcccgcgcgatctggttgagcgcgtcgtcctccgccgtgagccgctcccggttggggagccgcttgcgccccgatccctgggtgcccatgtccatcgaccgcgtcgcccgcagctgccgcggggcccgttgctccagccgctcgcgccgccccggcccggcccc

SEQ ID NO: 13335 - RNA, 3500 nt, Homo sapiens
  source 1..3500: mol_type = other RNA
gctgggattacaggcatgagccaccacgcccggccaaaaacatttaaaaaatgactgtccctgctcaaatactgcagtaggaaatgtaatttgacatatatcacttccagaaaaaaactttaaatctttctataaaatgaatttgatacatcatcagcatgaagtgaagttaaaatctcttacaaagtaaattcaggtatatcaacaatgagatccaaaagtatcggttcaagatcaaagactcatatgaggtaaaggcaaataaagcccctcatgctttcagacatttacttgttatccttaaaatgattattgttctaaggtgcaaatcttatcattcagtgacctatttgctatttggctgtttatctcctttaaataaaataccatacaggttataatgtacattttaaaatcaaatatgaaagtacacatatgtgaacaagacattaatttaaatatcaattatattcataatacagaagtctaagaatgctatttggtcatttcaattagatgctgatatatttggtcaagaaaacccacattcctatcagcctaaggcaaatagtaaatgcctctatttttattaagtggactataaacagtagacattattgtttgatactactggaatgctctcaattagaacgtacactgataacaaatatgtctttctaatctgggtgataacctcaatgattacatggaaatctacaagtaacagtctataacttaaagcagtagagcacctggtaattgtcatacagtgcctctctatgaatttagaacattctacttacattggcagtggagagaaaagaccccttcacactgagacttcctgtgcaccgcgcctgccgcctgcctcagcttaggacatggtacagtcttctttgcttttgcccttctcattccctcctctggtatcttctctgctttctggattgaagtgccctggctctcttcctggtgccgacaagtcatcgttctctaggctattgctgtctaaagctttcctgacggtctgacttggatgttctgacatctcacacctctctgtactttctgcttcacaggcatcactaatgtcctgtgagggactttcatgttcgggcagggtgcagcgatctgcgtcttcgctctttggttctgcaggactgctttgagtggcaccatctattttagcattatcttttgcaacaccttcatctaattcttcaccaccagccctcgggcctgatgattgaacggtgtcatcctcaaaatctaatgtgtctccatcagctagtacctcctcagctgctgtttgtacatcatcaccttcttggtcaagttttccatccaacttaattttaggattctccggacaatcaacattttcactgctttctgctgcaattttctgttttggattttcagtcacctcgttttgggcttccactgctgactttctgtcagtagactttacctgctcttcttccttaatttcacttaaatctgtgttctgatacgttaactcttttttaacatctttaagggtttctacgggtactggggattttttcttcttgtttttctttttcttgttctttgtcttcttctgcgatgagtccaatgcctctccctgttggtcactcttttcttcatcgggctctttcatatctaagggttcattttgagtgtctactgtacttggacctgtcgcttcctgacagttgccctcagttcctgctggagaaccaggaacttctgtcttgattggtttctcgtcccttaatcctgtttcttcaccctcttcttcgttgtgatccctacctacttctgtactgtgcgctggaacctccttgggctcagctgcttcctggttggtgaattctttctctaaactatgccctgtgcttgtctctaactcttgggggacctctaccatacatttgtcatcatgataaactgtgtcatcactatgccctaaaggacacgaggccactgtgcctgcctgctcttcaacctgagtcactgctgcctctcccacattctctgtgtggttcccaccatctaagtcactccaacagttggatggctcaaggggagttctggtcctgtcatctggtgcacccatgacctcatttgactcaacctgtactgtgttttcagggagagaactgctctcaagaatttggctttgaacctgttcctcataggtagcacctgctaaggttcctaggaatggggcagtgtcttcagaggatttctggtcctcggtattctcaccagcagggaatacctctatgtccacacagtccttcactgtgtcctctgtgtgttgttctttctcagtattgtgcaagatttctcttttccccacattcgccacgatttcatttttcacctccacttcactggctcttcctagggtcccatcccctgtcgacttgagggcatttaactcttcttttgtcatcttggtaggaccttggtatccaacattattgagggtgtcggaagtctctccattggtagctatttctgaatttaggattattccatgtttctcgagcatttcctctctttgcttcagggcctccttgacttcagcaaactgaaattgcagtatactgtgggcgtgtttttccctttcaaattctttgtttttctcttcgtactgccgcctagattcagccagctgttcttcaagctccagcaacatatcttttagggtatcaacctggtacatgaagtttgtcttttcattgtctagctgagcattggaaaccatagccttcttatatttctcttcaacttctgctagagagtccttcatctctttcaatccctgcatgtatttgccttctacatcctgaatctggtcctttaactcattgagttccttgatttccctgatggatgcctcggtgtcgatggagatggaggtgtctccgctgcctctccgagaggaagtcccacccagagaggccagcgtggctgcagacaggcccggcatgttacgagaccccttctcagtaaaatctttttctggtctctcttctacctccttctgctgccgctccagctccttcatgcggatctcgcgagcctccgcgcgggccgcccgttttgcagcgagccgggcttccgccagcttctgcgcttccgggctcaaacagtcgatctcccggctttgagcggccgcggggctggtcatcctgccgggctcggcccgctccacccggcgggaaatgctcggggaccgcgccgggagcccctcgcgggccgggccagggggcgcgcgctctgtccgcggagacggagccactcgccgctaagtgaacgctcgcgcttccggggccaggagccagcccgccggggagcggctcgcggcgctgggctcgggcgcggccgacaggggcggggcgcaggtggccgcgggctgagtcgggctcggggtggaagggcgccggggaagcgggactcgggcgcctccgcccgtcccacggccc

SEQ ID NO: 13336 - RNA, 3394 nt, Homo sapiens
  source 1..3394: mol_type = other RNA
gctgggattacaggcatgagccaccacgcccggccaaaaacatttaaaaaatgactgtccctgctcaaatactgcagtaggaaatgtaatttgacatatatcacttccagaaaaaaactttaaatctttctataaaatgaatttgatacatcatcagcatgaagtgaagttaaaatctcttacaaagtaaattcaggtatatcaacaatgagatccaaaagtatcggttcaagatcaaagactcatatgaggtaaaggcaaataaagcccctcatgctttcagacatttacttgttatccttaaaatgattattgttctaaggtgcaaatcttatcattcagtgacctatttgctatttggctgtttatctcctttaaataaaataccatacaggttataatgtacattttaaaatcaaatatgaaagtacacatatgtgaacaagacattaatttaaatatcaattatattcataatacagaagtctaagaatgctatttggtcatttcaattagatgctgatatatttggtcaagaaaacccacattcctatcagcctaaggcaaatagtaaatgcctctatttttattaagtggactataaacagtagacattattgtttgatactactggaatgctctcaattagaacgtacactgataacaaatatgtctttctaatctgggtgataacctcaatgattacatggaaatctacaagtaacagtctataacttaaagcagtagagcacctggtaattgtcatacagtgcctctctatgaatttagaacattctacttacattggcagtggagagaaaagaccccttcacactgagacttcctgtgcaccgcgcctgccgcctgcctcagcttaggacatggtacagtcttctttgcttttgcccttctcattccctcctctggtatcttctctgctttctggattgaagtgccctggctctcttcctggtgccgacaagtcatcgttctctaggctattgctgtctaaagctttcctgacggtctgacttggatgttctgacatctcacacctctctgtactttctgcttcacaggcatcactaatgtcctgtgagggactttcatgttcgggcagggtgcagcgatctgcgtcttcgctctttggttctgcaggactgctttgagtggcaccatctattttagcattatcttttgcaacaccttcatctaattcttcaccaccagccctcgggcctgatgattgaacggtgtcatcctcaaaatctaatgtgtctccatcagctagtacctcctcagctgctgtttgtacatcatcaccttcttggtcaagttttccatccaacttaattttaggattctccggacaatcaacattttcactgctttctgctgcaattttctgttttggattttcagtcacctcgttttgggcttccactgctgactttctgtcagtagactttacctgctcttcttccttaatttcacttaaatctgtgttctgatacgttaactcttttttaacatctttaagggtttctacgggtactggggattttttcttcttgtttttctttttcttgttctttgtcttcttctgcgatgagtccaatgcctctccctgttggtcactcttttcttcatcgggctctttcatatctaagggttcattttgagtgtctactgtacttggacctgtcgcttcctgacagttgccctcagttcctgctggagaaccaggaacttctgtcttgattggtttctcgtcccttaatcctgtttcttcaccctcttcttcgttgtgatccctacctacttctgtactgtgcgctggaacctccttgggctcagctgcttcctggttggtgaattctttctctaaactatgccctgtgcttgtctctaactcttgggggacctctaccatacatttgtcatcatgataaactgtgtcatcactatgccctaaaggacacgaggccactgtgcctgcctgctcttcaacctgagtcactgctgcctctcccacattctctgtgtggttcccaccatctaagtcactccaacagttggatggctcaaggggagttctggtcctgtcatctggtgcacccatgacctcatttgactcaacctgtactgtgttttcagggagagaactgctctcaagaatttggctttgaacctgttcctcataggtagcacctgctaaggttcctaggaatggggcagtgtcttcagaggatttctggtcctcggtattctcaccagcagggaatacctctatgtccacacagtccttcactgtgtcctctgtgtgttgttctttctcagtattgtgcaagatttctcttttccccacattcgccacgatttcatttttcacctccacttcactggctcttcctagggtcccatcccctgtcgacttgagggcatttaactcttcttttgtcatcttggtaggaccttggtatccaacattattgagggtgtcggaagtctctccattggtagctatttctgaatttaggattattccatgtttctcgagcatttcctctctttgcttcagggcctccttgacttcagcaaactgaaattgcagtatactgtgggcgtgtttttccctttcaaattctttgtttttctcttcgtactgccgcctagattcagccagctgttcttcaagctccagcaacatatcttttagggtatcaacctggtacatgaagtttgtcttttcattgtctagctgagcattggaaaccatagccttcttatatttctcttcaacttctgctagagagtccttgatttccctgatggatgcctcggtgtcgatggagatggaggtgtctccgctgcctctccgagaggaagtcccacccagagaggccagcgtggctgcagacaggcccggcatgttacgagaccccttctcagtaaaatctttttctggtctctcttctaccctcaggcttccacgactacccactgacatgcgctcgtcttcatcagaagccgatgtgtttcttctggatctacgagagtagcgctcactgtcttccatccactgctcgatgtcaccccattttgtatccagcccataatatttcttttggacctgatagatctccttctgctgccgctccagctccttcatgcggatctcgcgagcctccgcgcgggccgcccgttttgcagcgagccgggcttccgcctcccgcgcgatctggttgagcgcgtcgtcctccgccgtgagccgctcccggttggggagccgcttgcgccccgatccctgggtgcccatgtccatcgaccgcgtcgcccgcagctgccgcggggcccgttgctccagccgctcgcgccgccccggcccggcccc

SEQ ID NO: 13337 - RNA, 3323 nt, Homo sapiens
  source 1..3323: mol_type = other RNA
gctgggattacaggcatgagccaccacgcccggccaaaaacatttaaaaaatgactgtccctgctcaaatactgcagtaggaaatgtaatttgacatatatcacttccagaaaaaaactttaaatctttctataaaatgaatttgatacatcatcagcatgaagtgaagttaaaatctcttacaaagtaaattcaggtatatcaacaatgagatccaaaagtatcggttcaagatcaaagactcatatgaggtaaaggcaaataaagcccctcatgctttcagacatttacttgttatccttaaaatgattattgttctaaggtgcaaatcttatcattcagtgacctatttgctatttggctgtttatctcctttaaataaaataccatacaggttataatgtacattttaaaatcaaatatgaaagtacacatatgtgaacaagacattaatttaaatatcaattatattcataatacagaagtctaagaatgctatttggtcatttcaattagatgctgatatatttggtcaagaaaacccacattcctatcagcctaaggcaaatagtaaatgcctctatttttattaagtggactataaacagtagacattattgtttgatactactggaatgctctcaattagaacgtacactgataacaaatatgtctttctaatctgggtgataacctcaatgattacatggaaatctacaagtaacagtctataacttaaagcagtagagcacctggtaattgtcatacagtgcctctctatgaatttagaacattctacttacattggcagtggagagaaaagaccccttcacactgagacttcctgtgcaccgcgcctgccgcctgcctcagcttaggacatggtacagtcttctttgcttttgcccttctcattccctcctctggtatcttctctgctttctggattgaagtgccctggctctcttcctggtgccgacaagtcatcgttctctaggctattgctgtctaaagctttcctgacggtctgacttggatgttctgacatctcacacctctctgtactttctgcttcacaggcatcactaatgtcctgtgagggactttcatgttcgggcagggtgcagcgatctgcgtcttcgctctttggttctgcaggactgctttgagtggcaccatctattttagcattatcttttgcaacaccttcatctaattcttcaccaccagccctcgggcctgatgattgaacggtgtcatcctcaaaatctaatgtgtctccatcagctagtacctcctcagctgctgtttgtacatcatcaccttcttggtcaagttttccatccaacttaattttaggattctccggacaatcaacattttcactgctttctgctgcaattttctgttttggattttcagtcacctcgttttgggcttccactgctgactttctgtcagtagactttacctgctcttcttccttaatttcacttaaatctgtgttctgatacgttaactcttttttaacatctttaagggtttctacgggtactggggattttttcttcttgtttttctttttcttgttctttgtcttcttctgcgatgagtccaatgcctctccctgttggtcactcttttcttcatcgggctctttcatatctaagggttcattttgagtgtctactgtacttggacctgtcgcttcctgacagttgccctcagttcctgctggagaaccaggaacttctgtcttgattggtttctcgtcccttaatcctgtttcttcaccctcttcttcgttgtgatccctacctacttctgtactgtgcgctggaacctccttgggctcagctgcttcctggttggtgaattctttctctaaactatgccctgtgcttgtctctaactcttgggggacctctaccatacatttgtcatcatgataaactgtgtcatcactatgccctaaaggacacgaggccactgtgcctgcctgctcttcaacctgagtcactgctgcctctcccacattctctgtgtggttcccaccatctaagtcactccaacagttggatggctcaaggggagttctggtcctgtcatctggtgcacccatgacctcatttgactcaacctgtactgtgttttcagggagagaactgctctcaagaatttggctttgaacctgttcctcataggtagcacctgctaaggttcctaggaatggggcagtgtcttcagaggatttctggtcctcggtattctcaccagcagggaatacctctatgtccacacagtccttcactgtgtcctctgtgtgttgttctttctcagtattgtgcaagatttctcttttccccacattcgccacgatttcatttttcacctccacttcactggctcttcctagggtcccatcccctgtcgacttgagggcatttaactcttcttttgtcatcttggtaggaccttggtatccaacattattgagggtgtcggaagtctctccattggtagctatttctgaatttaggattattccatgtttctcgagcatttcctctctttgcttcagggcctccttgacttcagcaaactgaaattgcagtatactgtgggcgtgtttttccctttcaaattctttgtttttctcttcgtactgccgcctagattcagccagctgttcttcaagctccagcaacatatcttttagggtatcaacctggtacatgaagtttgtcttttcattgtctagctgagcattggaaaccatagccttcttatatttctcttcaacttctgctagagagtccttgatttccctgatggatgcctcggtgtcgatggagatggaggtgtctccgctgcctctccgagaggaagtcccacccagagaggccagcgtggctgcagacaggcccggcatgttacgagaccccttctcagtaaaatctttttctggtctctcttctaccctcaggcttccacgactacccactgacatgcgctcgtcttcatcagaagccgatgtgtttcttctggatctacgagagtagcgctcactgtcttcctccttctgctgccgctccagctccttcatgcggatctcgcgagcctccgcgcgggccgcccgttttgcagcgagccgggcttccgccagcttctgcgcttccgggctcaaacagtcgatctcccggctttgagcggccgcggggctggtcatcctgccgggctcggcccgctccacccggcgggaaatgctcggggaccgcgccgggagcccctcgcgggccgggccagggggcgcgcgctctgtc

SEQ ID NO: 13338 - RNA, 3480 nt, Homo sapiens
  source 1..3480: mol_type = other RNA
gctgggattacaggcatgagccaccacgcccggccaaaaacatttaaaaaatgactgtccctgctcaaatactgcagtaggaaatgtaatttgacatatatcacttccagaaaaaaactttaaatctttctataaaatgaatttgatacatcatcagcatgaagtgaagttaaaatctcttacaaagtaaattcaggtatatcaacaatgagatccaaaagtatcggttcaagatcaaagactcatatgaggtaaaggcaaataaagcccctcatgctttcagacatttacttgttatccttaaaatgattattgttctaaggtgcaaatcttatcattcagtgacctatttgctatttggctgtttatctcctttaaataaaataccatacaggttataatgtacattttaaaatcaaatatgaaagtacacatatgtgaacaagacattaatttaaatatcaattatattcataatacagaagtctaagaatgctatttggtcatttcaattagatgctgatatatttggtcaagaaaacccacattcctatcagcctaaggcaaatagtaaatgcctctatttttattaagtggactataaacagtagacattattgtttgatactactggaatgctctcaattagaacgtacactgataacaaatatgtctttctaatctgggtgataacctcaatgattacatggaaatctacaagtaacagtctataacttaaagcagtagagcacctggtaattgtcatacagtgcctctctatgaatttagaacattctacttacattggcagtggagagaaaagaccccttcacactgagacttcctgtgcaccgcgcctgccgcctgcctcagcttaggacatggtacagtcttctttgcttttgcccttctcattccctcctctggtatcttctctgctttctggattgaagtgccctggctctcttcctggtgccgacaagtcatcgttctctaggctattgctgtctaaagctttcctgacggtctgacttggatgttctgacatctcacacctctctgtactttctgcttcacaggcatcactaatgtcctgtgagggactttcatgttcgggcagggtgcagcgatctgcgtcttcgctctttggttctgcaggactgctttgagtggcaccatctattttagcattatcttttgcaacaccttcatctaattcttcaccaccagccctcgggcctgatgattgaacggtgtcatcctcaaaatctaatgtgtctccatcagctagtacctcctcagctgctgtttgtacatcatcaccttcttggtcaagttttccatccaacttaattttaggattctccggacaatcaacattttcactgctttctgctgcaattttctgttttggattttcagtcacctcgttttgggcttccactgctgactttctgtcagtagactttacctgctcttcttccttaatttcacttaaatctgtgttctgatacgttaactcttttttaacatctttaagggtttctacgggtactggggattttttcttcttgtttttctttttcttgttctttgtcttcttctgcgatgagtccaatgcctctccctgttggtcactcttttcttcatcgggctctttcatatctaagggttcattttgagtgtctactgtacttggacctgtcgcttcctgacagttgccctcagttcctgctggagaaccaggaacttctgtcttgattggtttctcgtcccttaatcctgtttcttcaccctcttcttcgttgtgatccctacctacttctgtactgtgcgctggaacctccttgggctcagctgcttcctggttggtgaattctttctctaaactatgccctgtgcttgtctctaactcttgggggacctctaccatacatttgtcatcatgataaactgtgtcatcactatgccctaaaggacacgaggccactgtgcctgcctgctcttcaacctgagtcactgctgcctctcccacattctctgtgtggttcccaccatctaagtcactccaacagttggatggctcaaggggagttctggtcctgtcatctggtgcacccatgacctcatttgactcaacctgtactgtgttttcagggagagaactgctctcaagaatttggctttgaacctgttcctcataggtagcacctgctaaggttcctaggaatggggcagtgtcttcagaggatttctggtcctcggtattctcaccagcagggaatacctctatgtccacacagtccttcactgtgtcctctgtgtgttgttctttctcagtattgtgcaagatttctcttttccccacattcgccacgatttcatttttcacctccacttcactggctcttcctagggtcccatcccctgtcgacttgagggcatttaactcttcttttgtcatcttggtaggaccttggtatccaacattattgagggtgtcggaagtctctccattggtagctatttctgaatttaggattattccatgtttctcgagcatttcctctctttgcttcagggcctccttgacttcagcaaactgaaattgcagtatactgtgggcgtgtttttccctttcaaattctttgtttttctcttcgtactgccgcctagattcagccagctgttcttcaagctccagcaacatatcttttagggtatcaacctggtacatgaagtttgtcttttcattgtctagctgagcattggaaaccatagccttcttatatttctcttcaacttctgctagagagtccttgatttccctgatggatgcctcggtgtcgatggagatggaggtgtctccgctgcctctccgagaggaagtcccacccagagaggccagcgtggctgcagacaggcccggcatgttacgagaccccttctcagtaaaatctttttctggtctctcttctaccctcaggcttccacgactacccactgacatgcgctcgtcttcatcagaagccgatgtgtttcttctggatctacgagagtagcgctcactgtcttcctccttctgctgccgctccagctccttcatgcggatctcgcgagcctccgcgcgggccgcccgttttgcagcgagccgggcttccgccagcttctgcgcttccgggctcaaacagtcgatctcccggctttgagcggccgcggggctggtcatcctgccgggctcggcccgctccacccggcgggaaatgctcggggaccgcgccgggagcccctcgcgggccgggccagggggcgcgcgctctgtccgcggagacggagccactcgccgctaagtgaacgctcgcgcttccggggccaggagccagcccgccggggagcggctcgcggcgctgggctcgggcgcggccgacaggggcggggcgcaggtggccgcgggctgagtcgggctcggggtggaagggc

SEQ ID NO: 13339 - RNA, 3302 nt, Homo sapiens
  source 1..3302: mol_type = other RNA
gctgggattacaggcatgagccaccacgcccggccaaaaacatttaaaaaatgactgtccctgctcaaatactgcagtaggaaatgtaatttgacatatatcacttccagaaaaaaactttaaatctttctataaaatgaatttgatacatcatcagcatgaagtgaagttaaaatctcttacaaagtaaattcaggtatatcaacaatgagatccaaaagtatcggttcaagatcaaagactcatatgaggtaaaggcaaataaagcccctcatgctttcagacatttacttgttatccttaaaatgattattgttctaaggtgcaaatcttatcattcagtgacctatttgctatttggctgtttatctcctttaaataaaataccatacaggttataatgtacattttaaaatcaaatatgaaagtacacatatgtgaacaagacattaatttaaatatcaattatattcataatacagaagtctaagaatgctatttggtcatttcaattagatgctgatatatttggtcaagaaaacccacattcctatcagcctaaggcaaatagtaaatgcctctatttttattaagtggactataaacagtagacattattgtttgatactactggaatgctctcaattagaacgtacactgataacaaatatgtctttctaatctgggtgataacctcaatgattacatggaaatctacaagtaacagtctataacttaaagcagtagagcacctggtaattgtcatacagtgcctctctatgaatttagaacattctacttacattggcagtggagagaaaagaccccttcacactgagacttcctgtgcaccgcgcctgccgcctgcctcagcttaggacatggtacagtcttctttgcttttgcccttctcattccctcctctggtatcttctctgctttctggattgaagtgccctggctctcttcctggtgccgacaagtcatcgttctctaggctattgctgtctaaagctttcctgacggtctgacttggatgttctgacatctcacacctctctgtactttctgcttcacaggcatcactaatgtcctgtgagggactttcatgttcgggcagggtgcagcgatctgcgtcttcgctctttggttctgcaggactgctttgagtggcaccatctattttagcattatcttttgcaacaccttcatctaattcttcaccaccagccctcgggcctgatgattgaacggtgtcatcctcaaaatctaatgtgtctccatcagctagtacctcctcagctgctgtttgtacatcatcaccttcttggtcaagttttccatccaacttaattttaggattctccggacaatcaacattttcactgctttctgctgcaattttctgttttggattttcagtcacctcgttttgggcttccactgctgactttctgtcagtagactttacctgctcttcttccttaatttcacttaaatctgtgttctgatacgttaactcttttttaacatctttaagggtttctacgggtactggggattttttcttcttgtttttctttttcttgttctttgtcttcttctgcgatgagtccaatgcctctccctgttggtcactcttttcttcatcgggctctttcatatctaagggttcattttgagtgtctactgtacttggacctgtcgcttcctgacagttgccctcagttcctgctggagaaccaggaacttctgtcttgattggtttctcgtcccttaatcctgtttcttcaccctcttcttcgttgtgatccctacctacttctgtactgtgcgctggaacctccttgggctcagctgcttcctggttggtgaattctttctctaaactatgccctgtgcttgtctctaactcttgggggacctctaccatacatttgtcatcatgataaactgtgtcatcactatgccctaaaggacacgaggccactgtgcctgcctgctcttcaacctgagtcactgctgcctctcccacattctctgtgtggttcccaccatctaagtcactccaacagttggatggctcaaggggagttctggtcctgtcatctggtgcacccatgacctcatttgactcaacctgtactgtgttttcagggagagaactgctctcaagaatttggctttgaacctgttcctcataggtagcacctgctaaggttcctaggaatggggcagtgtcttcagaggatttctggtcctcggtattctcaccagcagggaatacctctatgtccacacagtccttcactgtgtcctctgtgtgttgttctttctcagtattgtgcaagatttctcttttccccacattcgccacgatttcatttttcacctccacttcactggctcttcctagggtcccatcccctgtcgacttgagggcatttaactcttcttttgtcatcttggtaggaccttggtatccaacattattgagggtgtcggaagtctctccattggtagctatttctgaatttaggattattccatgtttctcgagcatttcctctctttgcttcagggcctccttgacttcagcaaactgaaattgcagtatactgtgggcgtgtttttccctttcaaattctttgtttttctcttcgtactgccgcctagattcagccagctgttcttcaagctccagcaacatatcttttagggtatcaacctggtacatgaagtttgtcttttcattgtctagctgagcattggaaaccatagccttcttatatttctcttcaacttctgctagagagtccttgatttccctgatggatgcctcggtgtcgatggagatggaggtgtctccgctgcctctccgagaggaagtcccacccagagaggccagcgtggctgcagacaggcccggcatgttacgagaccccttctcagtaaaatctttttctggtctctcttctaccctcaggcttccacgactacccactgacatgcgctcgtcttcatcagaagccgatgtgtttcttctggatctacgagagtagcgctcactgtcttcctccttctgctgccgctccagctccttcatgcggatctcgcgagcctccgcgcgggccgcccgttttgcagcgagccgggcttccgcctcccgcgcgatctggttgagcgcgtcgtcctccgccgtgagccgctcccggttggggagccgcttgcgccccgatccctgggtgcccatgtccatcgaccgcgtcgcccgcagctgccgcggggcccgttgctccagc

SEQ ID NO: 13340 - RNA, 3493 nt, Homo sapiens
  source 1..3493: mol_type = other RNA
gctgggattacaggcatgagccaccacgcccggccaaaaacatttaaaaaatgactgtccctgctcaaatactgcagtaggaaatgtaatttgacatatatcacttccagaaaaaaactttaaatctttctataaaatgaatttgatacatcatcagcatgaagtgaagttaaaatctcttacaaagtaaattcaggtatatcaacaatgagatccaaaagtatcggttcaagatcaaagactcatatgaggtaaaggcaaataaagcccctcatgctttcagacatttacttgttatccttaaaatgattattgttctaaggtgcaaatcttatcattcagtgacctatttgctatttggctgtttatctcctttaaataaaataccatacaggttataatgtacattttaaaatcaaatatgaaagtacacatatgtgaacaagacattaatttaaatatcaattatattcataatacagaagtctaagaatgctatttggtcatttcaattagatgctgatatatttggtcaagaaaacccacattcctatcagcctaaggcaaatagtaaatgcctctatttttattaagtggactataaacagtagacattattgtttgatactactggaatgctctcaattagaacgtacactgataacaaatatgtctttctaatctgggtgataacctcaatgattacatggaaatctacaagtaacagtctataacttaaagcagtagagcacctggtaattgtcatacagtgcctctctatgaatttagaacattctacttacattggcagtggagagaaaagaccccttcacactgagacttcctgtgcaccgcgcctgccgcctgcctcagcttaggacatggtacagtcttctttgcttttgcccttctcattccctcctctggtatcttctctgctttctggattgaagtgccctggctctcttcctggtgccgacaagtcatcgttctctaggctattgctgtctaaagctttcctgacggtctgacttggatgttctgacatctcacacctctctgtactttctgcttcacaggcatcactaatgtcctgtgagggactttcatgttcgggcagggtgcagcgatctgcgtcttcgctctttggttctgcaggactgctttgagtggcaccatctattttagcattatcttttgcaacaccttcatctaattcttcaccaccagccctcgggcctgatgattgaacggtgtcatcctcaaaatctaatgtgtctccatcagctagtacctcctcagctgctgtttgtacatcatcaccttcttggtcaagttttccatccaacttaattttaggattctccggacaatcaacattttcactgctttctgctgcaattttctgttttggattttcagtcacctcgttttgggcttccactgctgactttctgtcagtagactttacctgctcttcttccttaatttcacttaaatctgtgttctgatacgttaactcttttttaacatctttaagggtttctacgggtactggggattttttcttcttgtttttctttttcttgttctttgtcttcttctgcgatgagtccaatgcctctccctgttggtcactcttttcttcatcgggctctttcatatctaagggttcattttgagtgtctactgtacttggacctgtcgcttcctgacagttgccctcagttcctgctggagaaccaggaacttctgtcttgattggtttctcgtcccttaatcctgtttcttcaccctcttcttcgttgtgatccctacctacttctgtactgtgcgctggaacctccttgggctcagctgcttcctggttggtgaattctttctctaaactatgccctgtgcttgtctctaactcttgggggacctctaccatacatttgtcatcatgataaactgtgtcatcactatgccctaaaggacacgaggccactgtgcctgcctgctcttcaacctgagtcactgctgcctctcccacattctctgtgtggttcccaccatctaagtcactccaacagttggatggctcaaggggagttctggtcctgtcatctggtgcacccatgacctcatttgactcaacctgtactgtgttttcagggagagaactgctctcaagaatttggctttgaacctgttcctcataggtagcacctgctaaggttcctaggaatggggcagtgtcttcagaggatttctggtcctcggtattctcaccagcagggaatacctctatgtccacacagtccttcactgtgtcctctgtgtgttgttctttctcagtattgtgcaagatttctcttttccccacattcgccacgatttcatttttcacctccacttcactggctcttcctagggtcccatcccctgtcgacttgagggcatttaactcttcttttgtcatcttggtaggaccttggtatccaacattattgagggtgtcggaagtctctccattggtagctatttctgaatttaggattattccatgtttctcgagcatttcctctctttgcttcagggcctccttgacttcagcaaactgaaattgcagtatactgtgggcgtgtttttccctttcaaattctttgtttttctcttcgtactgccgcctagattcagccagctgttcttcaagctccagcaacatatcttttagggtatcaacctggtacatgaagtttgtcttttcattgtctagctgagcattggaaaccatagccttcttatatttctcttcaacttctgctagagagtccttgatttccctgatggatgcctcggtgtcgatggagatggaggtgtctccgctgcctctccgagaggaagtcccacccagagaggccagcgtggctgcagacaggcccggcatgttacgagaccccttctcagtaaaatctttttctggtctctcttctaccctgccagatcttctattcagggactgtgatccatacaattctccatcataaccatttgtccaggcgtaaggacccccatactccaagtcaggctgcgacctcaggcttccacgactacccactgacatgcgctcgtcttcatcagaagccgatgtgtttcttctggatctacgagagtagcgctcactgtcttccatccactgctcgatgtcaccccattttgtatccagcccataatatttcttttggacctgatagatctccttctgctgccgctccagctccttcatgcggatctcgcgagcctccgcgcgggccgcccgttttgcagcgagccgggcttccgcctcccgcgcgatctggttgagcgcgtcgtcctccgccgtgagccgctcccggttggggagccgcttgcgccccgatccctgggtgcccatgtccatcgaccgcgtcgcccgcagctgccgcggggcccgttgctccagccgctcgcgccgccccggcccggcccc

SEQ ID NO: 13341 - RNA, 3384 nt, Homo sapiens
  source 1..3384: mol_type = other RNA
gctgggattacaggcatgagccaccacgcccggccaaaaacatttaaaaaatgactgtccctgctcaaatactgcagtaggaaatgtaatttgacatatatcacttccagaaaaaaactttaaatctttctataaaatgaatttgatacatcatcagcatgaagtgaagttaaaatctcttacaaagtaaattcaggtatatcaacaatgagatccaaaagtatcggttcaagatcaaagactcatatgaggtaaaggcaaataaagcccctcatgctttcagacatttacttgttatccttaaaatgattattgttctaaggtgcaaatcttatcattcagtgacctatttgctatttggctgtttatctcctttaaataaaataccatacaggttataatgtacattttaaaatcaaatatgaaagtacacatatgtgaacaagacattaatttaaatatcaattatattcataatacagaagtctaagaatgctatttggtcatttcaattagatgctgatatatttggtcaagaaaacccacattcctatcagcctaaggcaaatagtaaatgcctctatttttattaagtggactataaacagtagacattattgtttgatactactggaatgctctcaattagaacgtacactgataacaaatatgtctttctaatctgggtgataacctcaatgattacatggaaatctacaagtaacagtctataacttaaagcagtagagcacctggtaattgtcatacagtgcctctctatgaatttagaacattctacttacattggcagtggagagaaaagaccccttcacactgagacttcctgtgcaccgcgcctgccgcctgcctcagcttaggacatggtacagtcttctttgcttttgcccttctcattccctcctctggtatcttctctgctttctggattgaagtgccctggctctcttcctggtgccgacaagtcatcgttctctaggctattgctgtctaaagctttcctgacggtctgacttggatgttctgacatctcacacctctctgtactttctgcttcacaggcatcactaatgtcctgtgagggactttcatgttcgggcagggtgcagcgatctgcgtcttcgctctttggttctgcaggactgctttgagtggcaccatctattttagcattatcttttgcaacaccttcatctaattcttcaccaccagccctcgggcctgatgattgaacggtgtcatcctcaaaatctaatgtgtctccatcagctagtacctcctcagctgctgtttgtacatcatcaccttcttggtcaagttttccatccaacttaattttaggattctccggacaatcaacattttcactgctttctgctgcaattttctgttttggattttcagtcacctcgttttgggcttccactgctgactttctgtcagtagactttacctgctcttcttccttaatttcacttaaatctgtgttctgatacgttaactcttttttaacatctttaagggtttctacgggtactggggattttttcttcttgtttttctttttcttgttctttgtcttcttctgcgatgagtccaatgcctctccctgttggtcactcttttcttcatcgggctctttcatatctaagggttcattttgagtgtctactgtacttggacctgtcgcttcctgacagttgccctcagttcctgctggagaaccaggaacttctgtcttgattggtttctcgtcccttaatcctgtttcttcaccctcttcttcgttgtgatccctacctacttctgtactgtgcgctggaacctccttgggctcagctgcttcctggttggtgaattctttctctaaactatgccctgtgcttgtctctaactcttgggggacctctaccatacatttgtcatcatgataaactgtgtcatcactatgccctaaaggacacgaggccactgtgcctgcctgctcttcaacctgagtcactgctgcctctcccacattctctgtgtggttcccaccatctaagtcactccaacagttggatggctcaaggggagttctggtcctgtcatctggtgcacccatgacctcatttgactcaacctgtactgtgttttcagggagagaactgctctcaagaatttggctttgaacctgttcctcataggtagcacctgctaaggttcctaggaatggggcagtgtcttcagaggatttctggtcctcggtattctcaccagcagggaatacctctatgtccacacagtccttcactgtgtcctctgtgtgttgttctttctcagtattgtgcaagatttctcttttccccacattcgccacgatttcatttttcacctccacttcactggctcttcctagggtcccatcccctgtcgacttgagggcatttaactcttcttttgtcatcttggtaggaccttggtatccaacattattgagggtgtcggaagtctctccattggtagctatttctgaatttaggattattccatgtttctcgagcatttcctctctttgcttcagggcctccttgacttcagcaaactgaaattgcagtatactgtgggcgtgtttttccctttcaaattctttgtttttctcttcgtactgccgcctagattcagccagctgttcttcaagctccagcaacatatcttttagggtatcaacctggtacatgaagtttgtcttttcattgtctagctgagcattggaaaccatagccttcttatatttctcttcaacttctgctagagagtccttgatttccctgatggatgcctcggtgtcgatggagatggaggtgtctccgctgcctctccgagaggaagtcccacccagagaggccagcgtggctgcagacaggcccggcatgttacgagaccccttctcagtaaaatctttttctggtctctcttctacctccttctgctgccgctccagctccttcatgcggatctcgcgagcctccgcgcgggccgcccgttttgcagcgagccgggcttccgccagcttctgcgcttccgggctcaaacagtcgatctcccggctttgagcggccgcggggctggtcatcctgccgggctcggcccgctccacccggcgggaaatgctcggggaccgcgccgggagcccctcgcgggccgggccagggggcgcgcgctctgtccgcggagacggagccactcgccgctaagtgaacgctcgcgcttccggggccaggagccagcccgccggggagcggctcgcggcgctgggctcgggcgcggccgacaggggcggggcgcaggtggccgcgggctgagtcgggctcggggtggaagggc

SEQ ID NO: 13342 - RNA, 3468 nt, Homo sapiens
  source 1..3468: mol_type = other RNA
gctgggattacaggcatgagccaccacgcccggccaaaaacatttaaaaaatgactgtccctgctcaaatactgcagtaggaaatgtaatttgacatatatcacttccagaaaaaaactttaaatctttctataaaatgaatttgatacatcatcagcatgaagtgaagttaaaatctcttacaaagtaaattcaggtatatcaacaatgagatccaaaagtatcggttcaagatcaaagactcatatgaggtaaaggcaaataaagcccctcatgctttcagacatttacttgttatccttaaaatgattattgttctaaggtgcaaatcttatcattcagtgacctatttgctatttggctgtttatctcctttaaataaaataccatacaggttataatgtacattttaaaatcaaatatgaaagtacacatatgtgaacaagacattaatttaaatatcaattatattcataatacagaagtctaagaatgctatttggtcatttcaattagatgctgatatatttggtcaagaaaacccacattcctatcagcctaaggcaaatagtaaatgcctctatttttattaagtggactataaacagtagacattattgtttgatactactggaatgctctcaattagaacgtacactgataacaaatatgtctttctaatctgggtgataacctcaatgattacatggaaatctacaagtaacagtctataacttaaagcagtagagcacctggtaattgtcatacagtgcctctctatgaatttagaacattctacttacattggcagtggagagaaaagaccccttcacactgagacttcctgtgcaccgcgcctgccgcctgcctcagcttaggacatggtacagtcttctttgcttttgcccttctcattccctcctctggtatcttctctgctttctggattgaagtgccctggctctcttcctggtgccgacaagtcatcgttctctaggctattgctgtctaaagctttcctgacggtctgacttggatgttctgacatctcacacctctctgtactttctgcttcacaggcatcactaatgtcctgtgagggactttcatgttcgggcagggtgcagcgatctgcgtcttcgctctttggttctgcaggactgctttgagtggcaccatctattttagcattatcttttgcaacaccttcatctaattcttcaccaccagccctcgggcctgatgattgaacggtgtcatcctcaaaatctaatgtgtctccatcagctagtacctcctcagctgctgtttgtacatcatcaccttcttggtcaagttttccatccaacttaattttaggattctccggacaatcaacattttcactgctttctgctgcaattttctgttttggattttcagtcacctcgttttgggcttccactgctgactttctgtcagtagactttacctgctcttcttccttaatttcacttaaatctgtgttctgatacgttaactcttttttaacatctttaagggtttctacgggtactggggattttttcttcttgtttttctttttcttgttctttgtcttcttctgcgatgagtccaatgcctctccctgttggtcactcttttcttcatcgggctctttcatatctaagggttcattttgagtgtctactgtacttggacctgtcgcttcctgacagttgccctcagttcctgctggagaaccaggaacttctgtcttgattggtttctcgtcccttaatcctgtttcttcaccctcttcttcgttgtgatccctacctacttctgtactgtgcgctggaacctccttgggctcagctgcttcctggttggtgaattctttctctaaactatgccctgtgcttgtctctaactcttgggggacctctaccatacatttgtcatcatgataaactgtgtcatcactatgccctaaaggacacgaggccactgtgcctgcctgctcttcaacctgagtcactgctgcctctcccacattctctgtgtggttcccaccatctaagtcactccaacagttggatggctcaaggggagttctggtcctgtcatctggtgcacccatgacctcatttgactcaacctgtactgtgttttcagggagagaactgctctcaagaatttggctttgaacctgttcctcataggtagcacctgctaaggttcctaggaatggggcagtgtcttcagaggatttctggtcctcggtattctcaccagcagggaatacctctatgtccacacagtccttcactgtgtcctctgtgtgttgttctttctcagtattgtgcaagatttctcttttccccacattcgccacgatttcatttttcacctccacttcactggctcttcctagggtcccatcccctgtcgacttgagggcatttaactcttcttttgtcatcttggtaggaccttggtatccaacattattgagggtgtcggaagtctctccattggtagctatttctgaatttaggattattccatgtttctcgagcatttcctctctttgcttcagggcctccttgacttcagcaaactgaaattgcagtatactgtgggcgtgtttttccctttcaaattctttgtttttctcttcgtactgccgcctagattcagccagctgttcttcaagctccagcaacatatcttttagggtatcaacctggtacatgaagtttgtcttttcattgtctagctgagcattggaaaccatagccttcttatatttctcttcaacttctgctagagagtccttgatttccctgatggatgcctcggtgtcgatggagatggaggtgtctccgctgcctctccgagaggaagtcccacccagagaggccagcgtggctgcagacaggcccggcatgttacgagaccccttctcagtaaaatctttttctggtctctcttctacctccttctgctgccgctccagctccttcatgcggatctcgcgagcctccgcgcgggccgcccgttttgcagcgagccgggcttccgccagcttctgcgcttccgggctcaaacagtcgatctcccggctttgagcggccgcggggctggtcatcctgccgggctcggcccgctccacccggcgggaaatgctcggggaccgcgccgggagcccctcgcgggccgggccagggggcgcgcgctctgtccgcggagacggagccactcgccgctaagtgaacgctcgcgcttccggggccaggagccagcccgccggggagcggctcgcggcgctgggctcgggcgcggccgacaggggcggggcgcaggtggccgcgggctgagtcgggctcggggtggaagggcgccggggaagcgggactcgggcgcctccgcccgtcccacggcccgccccgccccccacgcagttccgcctcggaggggccctcc

SEQ ID NO: 13343 - RNA, 3222 nt, Homo sapiens
  source 1..3222: mol_type = other RNA
gctgggattacaggcatgagccaccacgcccggccaaaaacatttaaaaaatgactgtccctgctcaaatactgcagtaggaaatgtaatttgacatatatcacttccagaaaaaaactttaaatctttctataaaatgaatttgatacatcatcagcatgaagtgaagttaaaatctcttacaaagtaaattcaggtatatcaacaatgagatccaaaagtatcggttcaagatcaaagactcatatgaggtaaaggcaaataaagcccctcatgctttcagacatttacttgttatccttaaaatgattattgttctaaggtgcaaatcttatcattcagtgacctatttgctatttggctgtttatctcctttaaataaaataccatacaggttataatgtacattttaaaatcaaatatgaaagtacacatatgtgaacaagacattaatttaaatatcaattatattcataatacagaagtctaagaatgctatttggtcatttcaattagatgctgatatatttggtcaagaaaacccacattcctatcagcctaaggcaaatagtaaatgcctctatttttattaagtggactataaacagtagacattattgtttgatactactggaatgctctcaattagaacgtacactgataacaaatatgtctttctaatctgggtgataacctcaatgattacatggaaatctacaagtaacagtctataacttaaagcagtagagcacctggtaattgtcatacagtgcctctctatgaatttagaacattctacttacattggcagtggagagaaaagaccccttcacactgagacttcctgtgcaccgcgcctgccgcctgcctcagcttaggacatggtacagtcttctttgcttttgcccttctcattccctcctctggtatcttctctgctttctggattgaagtgccctggctctcttcctggtgccgacaagtcatcgttctctaggctattgctgtctaaagctttcctgacggtctgacttggatgttctgacatctcacacctctctgtactttctgcttcacaggcatcactaatgtcctgtgagggactttcatgttcgggcagggtgcagcgatctgcgtcttcgctctttggttctgcaggactgctttgagtggcaccatctattttagcattatcttttgcaacaccttcatctaattcttcaccaccagccctcgggcctgatgattgaacggtgtcatcctcaaaatctaatgtgtctccatcagctagtacctcctcagctgctgtttgtacatcatcaccttcttggtcaagttttccatccaacttaattttaggattctccggacaatcaacattttcactgctttctgctgcaattttctgttttggattttcagtcacctcgttttgggcttccactgctgactttctgtcagtagactttacctgctcttcttccttaatttcacttaaatctgtgttctgatacgttaactcttttttaacatctttaagggtttctacgggtactggggattttttcttcttgtttttctttttcttgttctttgtcttcttctgcgatgagtccaatgcctctccctgttggtcactcttttcttcatcgggctctttcatatctaagggttcattttgagtgtctactgtacttggacctgtcgcttcctgacagttgccctcagttcctgctggagaaccaggaacttctgtcttgattggtttctcgtcccttaatcctgtttcttcaccctcttcttcgttgtgatccctacctacttctgtactgtgcgctggaacctccttgggctcagctgcttcctggttggtgaattctttctctaaactatgccctgtgcttgtctctaactcttgggggacctctaccatacatttgtcatcatgataaactgtgtcatcactatgccctaaaggacacgaggccactgtgcctgcctgctcttcaacctgagtcactgctgcctctcccacattctctgtgtggttcccaccatctaagtcactccaacagttggatggctcaaggggagttctggtcctgtcatctggtgcacccatgacctcatttgactcaacctgtactgtgttttcagggagagaactgctctcaagaatttggctttgaacctgttcctcataggtagcacctgctaaggttcctaggaatggggcagtgtcttcagaggatttctggtcctcggtattctcaccagcagggaatacctctatgtccacacagtccttcactgtgtcctctgtgtgttgttctttctcagtattgtgcaagatttctcttttccccacattcgccacgatttcatttttcacctccacttcactggctcttcctagggtcccatcccctgtcgacttgagggcatttaactcttcttttgtcatcttggtaggaccttggtatccaacattattgagggtgtcggaagtctctccattggtagctatttctgaatttaggattattccatgtttctcgagcatttcctctctttgcttcagggcctccttgacttcagcaaactgaaattgcagtatactgtgggcgtgtttttccctttcaaattctttgtttttctcttcgtactgccgcctagattcagccagctgttcttcaagctccagcaacatatcttttagggtatcaacctggtacatgaagtttgtcttttcattgtctagctgagcattggaaaccatagccttcttatatttctcttcaacttctgctagagagtccttgatttccctgatggatgcctcggtgtcgatggagatggaggtgtctccgctgcctctccgagaggaagtcccacccagagaggccagcgtggctgcagacaggcccggcatgttacgagaccccttctcagtaaaatctttttctggtctctcttctacctccttctgctgccgctccagctccttcatgcggatctcgcgagcctccgcgcgggccgcccgttttgcagcgagccgggcttccgcctcccgcgcgatctggttgagcgcgtcgtcctccgccgtgagccgctcccggttggggagccgcttgcgccccgatccctgggtgcccatgtccatcgaccgcgtcgcccgcagctgccgcggggcccgttgctccagccgctcgcgccgccccg

SEQ ID NO: 13344 - RNA, 4168 nt, Homo sapiens
  source 1..4168: mol_type = other RNA
gctgggattacaggcatgagccaccacgcccggccaaaaacatttaaaaaatgactgtccctgctcaaatactgcagtaggaaatgtaatttgacatatatcacttccagaaaaaaactttaaatctttctataaaatgaatttgatacatcatcagcatgaagtgaagttaaaatctcttacaaagtaaattcaggtatatcaacaatgagatccaaaagtatcggttcaagatcaaagactcatatgaggtaaaggcaaataaagcccctcatgctttcagacatttacttgttatccttaaaatgattattgttctaaggtgcaaatcttatcattcagtgacctatttgctatttggctgtttatctcctttaaataaaataccatacaggttataatgtacattttaaaatcaaatatgaaagtacacatatgtgaacaagacattaatttaaatatcaattatattcataatacagaagtctaagaatgctatttggtcatttcaattagatgctgatatatttggtcaagaaaacccacattcctatcagcctaaggcaaatagtaaatgcctctatttttattaagtggactataaacagtagacattattgtttgatactactggaatgctctcaattagaacgtacactgataacaaatatgtctttctaatctgggtgataacctcaatgattacatggaaatctacaagtaacagtctataacttaaagcagtagagcacctggtaattgtcatacagtgcctctctatgaatttagaacattctacttacattggcagtggagagaaaagaccccttcacactgagacttcctgtgcaccgcgcctgccgcctgcctcagcttaggacatggtacagtcttctttgcttttgcccttctcattccctcctctggtatcttctctgctttctggattgaagtgccctggctctcttcctggtgccgacaagtcatcgttctctaggctattgctgtctaaagctttcctgacggtctgacttggatgttctgacatctcacacctctctgtactttctgcttcacaggcatcactaatgtcctgtgagggactttcatgttcgggcagggtgcagcgatctgcgtcttcgctctttggttctgcaggactgctttgagtggcaccatctattttagcattatcttttgcaacaccttcatctaattcttcaccaccagccctcgggcctgatgattgaacggtgtcatcctcaaaatctaatgtgtctccatcagctagtacctcctcagctgctgtttgtacatcatcaccttcttggtcaagttttccatccaacttaattttaggattctccggacaatcaacattttcactgctttctgctgcaattttctgttttggattttcagtcacctcgttttgggcttccactgctgactttctgtcagtagactttacctgctcttcttccttaatttcacttaaatctgtgttctgatacgttaactcttttttaacatctttaagggtttctacgggtactggggattttttcttcttgtttttctttttcttgttctttgtcttcttctgcgatgagtccaatgcctctccctgttggtcactcttttcttcatcgggctctttcatatctaagggttcattttgagtgtctactgtacttggacctgtcgcttcctgacagttgccctcagttcctgctggagaaccaggaacttctgtcttgattggtttctcgtcccttaatcctgtttcttcaccctcttcttcgttgtgatccctacctacttctgtactgtgcgctggaacctccttgggctcagctgcttcctggttggtgaattctttctctaaactatgccctgtgcttgtctctaactcttgggggacctctaccatacatttgtcatcatgataaactgtgtcatcactatgccctaaaggacacgaggccactgtgcctgcctgctcttcaacctgagtcactgctgcctctcccacattctctgtgtggttcccaccatctaagtcactccaacagttggatggctcaaggggagttctggtcctgtcatctggtgcacccatgacctcatttgactcaacctgtactgtgttttcagggagagaactgctctcaagaatttggctttgaacctgttcctcataggtagcacctgctaaggttcctaggaatggggcagtgtcttcagaggatttctggtcctcggtattctcaccagcagggaatacctctatgtccacacagtccttcactgtgtcctctgtgtgttgttctttctcagtattgtgcaagatttctcttttccccacattcgccacgatttcatttttcacctccacttcactggctcttcctagggtcccatcccctgtcgacttgagggcatttaactcttcttttgtcatcttggtaggaccttggtatccaacattattgagggtgtcggaagtctctccattggtagctatttctgaatttaggattattccatgtttctttaattcctctttcagcatgactacttcttctctaagatcatcccgttcactccttacggaatcaaagaactctttctgcctctctaatgcccctatctttttgtctttccactctattgtttcctgaagatcagaaatctccctgatagaactcgcctgtttctgctgtagctgtcggatttcctcgagcatttcctctctttgcttcagggcctccttgacttcagcaaactgaaattgcagtatactgtgggcgtgtttttccctttcaaattctttgtttttctcttcgtactgccgcctagattcagccagctgttcttcaagctccagcaacatatcttttagggtatcaacctggtacatgaagtttgtcttttcattgtctagctgagcattggaaaccatagccttcttatatttctcttcaacttctgctagagagtccttcatctctttcaatccctgcatgtatttgccttctacatcctgaatctggtcctttaactcattgagttccttgatttccctgatggatgcctcggtgtcgatggagatggaggtgtctccgctgcctctccgagaggaagtcccacccagagaggccagcgtggctgcagacaggcccggcatgttacgagaccccttctcagtaaaatctttttctggtctctcttctaccacagggctggcccgggccgagctggccctggaggaggcgcgggagctggagttgaggtggccgctgtactccgagggagcacgggagccggaggtgctgccccgtcgggtcccaccgaagctgccttcatccaacacagacgcccggtaactccccgaaggccgggcagcgctgtacagacaggagggcaacttctcctccctggatgatgacaaagtagagaatctgctgtcaccgctgtagctggaattcctgccagatcttctattcagggactgtgatccatacaattctccatcataaccatttgtccaggcgtaaggacccccatactccaagtcaggctgcgacctcaggcttccacgactacccactgacatgcgctcgtcttcatcagaagccgatgtgtttcttctggatctacgagagtagcgctcactgtcttccatccactgctcgatgtcaccccattttgtatccagcccataatatttcttttggacctgatagatctccttctgctgccgctccagctccttcatgcggatctcgcgagcctccgcgcgggccgcccgttttgcagcgagccgggcttccgccagcttctgcgcttccgggctcaaacagtcgatctcccggctttgagcggccgcggggctggtcatcctgccgggctcggcccgctccacccggcgggaaatgctcggggaccgcgccgggagcccctcgcgggccgggccagggggcgcgcgctctgtccgcggagacggagccactcgccgctaagtgaacgctcgcgcttccggggccaggagccagcccgccggggagcggctcgcggcgctgggctcgggcgcggccgacaggggcggggcgcaggtggccgcgggctgagtcgggctcggggtggaagggcgccggggaagcgg

SEQ ID NO: 13345 - RNA, 4003 nt, Homo sapiens
  source 1..4003: mol_type = other RNA
gctgggattacaggcatgagccaccacgcccggccaaaaacatttaaaaaatgactgtccctgctcaaatactgcagtaggaaatgtaatttgacatatatcacttccagaaaaaaactttaaatctttctataaaatgaatttgatacatcatcagcatgaagtgaagttaaaatctcttacaaagtaaattcaggtatatcaacaatgagatccaaaagtatcggttcaagatcaaagactcatatgaggtaaaggcaaataaagcccctcatgctttcagacatttacttgttatccttaaaatgattattgttctaaggtgcaaatcttatcattcagtgacctatttgctatttggctgtttatctcctttaaataaaataccatacaggttataatgtacattttaaaatcaaatatgaaagtacacatatgtgaacaagacattaatttaaatatcaattatattcataatacagaagtctaagaatgctatttggtcatttcaattagatgctgatatatttggtcaagaaaacccacattcctatcagcctaaggcaaatagtaaatgcctctatttttattaagtggactataaacagtagacattattgtttgatactactggaatgctctcaattagaacgtacactgataacaaatatgtctttctaatctgggtgataacctcaatgattacatggaaatctacaagtaacagtctataacttaaagcagtagagcacctggtaattgtcatacagtgcctctctatgaatttagaacattctacttacattggcagtggagagaaaagaccccttcacactgagacttcctgtgcaccgcgcctgccgcctgcctcagcttaggacatggtacagtcttctttgcttttgcccttctcattccctcctctggtatcttctctgctttctggattgaagtgccctggctctcttcctggtgccgacaagtcatcgttctctaggctattgctgtctaaagctttcctgacggtctgacttggatgttctgacatctcacacctctctgtactttctgcttcacaggcatcactaatgtcctgtgagggactttcatgttcgggcagggtgcagcgatctgcgtcttcgctctttggttctgcaggactgctttgagtggcaccatctattttagcattatcttttgcaacaccttcatctaattcttcaccaccagccctcgggcctgatgattgaacggtgtcatcctcaaaatctaatgtgtctccatcagctagtacctcctcagctgctgtttgtacatcatcaccttcttggtcaagttttccatccaacttaattttaggattctccggacaatcaacattttcactgctttctgctgcaattttctgttttggattttcagtcacctcgttttgggcttccactgctgactttctgtcagtagactttacctgctcttcttccttaatttcacttaaatctgtgttctgatacgttaactcttttttaacatctttaagggtttctacgggtactggggattttttcttcttgtttttctttttcttgttctttgtcttcttctgcgatgagtccaatgcctctccctgttggtcactcttttcttcatcgggctctttcatatctaagggttcattttgagtgtctactgtacttggacctgtcgcttcctgacagttgccctcagttcctgctggagaaccaggaacttctgtcttgattggtttctcgtcccttaatcctgtttcttcaccctcttcttcgttgtgatccctacctacttctgtactgtgcgctggaacctccttgggctcagctgcttcctggttggtgaattctttctctaaactatgccctgtgcttgtctctaactcttgggggacctctaccatacatttgtcatcatgataaactgtgtcatcactatgccctaaaggacacgaggccactgtgcctgcctgctcttcaacctgagtcactgctgcctctcccacattctctgtgtggttcccaccatctaagtcactccaacagttggatggctcaaggggagttctggtcctgtcatctggtgcacccatgacctcatttgactcaacctgtactgtgttttcagggagagaactgctctcaagaatttggctttgaacctgttcctcataggtagcacctgctaaggttcctaggaatggggcagtgtcttcagaggatttctggtcctcggtattctcaccagcagggaatacctctatgtccacacagtccttcactgtgtcctctgtgtgttgttctttctcagtattgtgcaagatttctcttttccccacattcgccacgatttcatttttcacctccacttcactggctcttcctagggtcccatcccctgtcgacttgagggcatttaactcttcttttgtcatcttggtaggaccttggtatccaacattattgagggtgtcggaagtctctccattggtagctatttctgaatttaggattattccatgtttctttaattcctctttcagcatgactacttcttctctaagatcatcccgttcactccttacggaatcaaagaactctttctgcctctctaatgcccctatctttttgtctttccactctattgtttcctgaagatcagaaatctccctgatagaactcgcctgtttctgctgtagctgtcggatttcctcgagcatttcctctctttgcttcagggcctccttgacttcagcaaactgaaattgcagtatactgtgggcgtgtttttccctttcaaattctttgtttttctcttcgtactgccgcctagattcagccagctgttcttcaagctccagcaacatatcttttagggtatcaacctggtacatgaagtttgtcttttcattgtctagctgagcattggaaaccatagccttcttatatttctcttcaacttctgctagagagtccttcatctctttcaatccctgcatgtatttgccttctacatcctgaatctggtcctttaactcattgagttccttgatttccctgatggatgcctcggtgtcgatggagatggaggtgtctccgctgcctctccgagaggaagtcccacccagagaggccagcgtggctgcagacaggcccggcatgttacgagaccccttctcagtaaaatctttttctggtctctcttctaccacagggctggcccgggccgagctggccctggaggaggcgcgggagctggagttgaggtggccgctgtactccgagggagcacgggagccggaggtgctgccccgtcgggtcccaccgaagctgccttcatccaacacagacgcccggtaactccccgaaggccgggcagcgctgtacagacaggagggcaacttctcctccctggatgatgacaaagtagagaatctgctgtcaccgctgtagctggaattcctgccagatcttctattcagggactgtgatccatacaattctccatcataaccatttgtccaggcgtaaggacccccatactccaagtcaggctgcgacctcaggcttccacgactacccactgacatgcgctcgtcttcatcagaagccgatgtgtttcttctggatctacgagagtagcgctcactgtcttccatccactgctcgatgtcaccccattttgtatccagcccataatatttcttttggacctgatagatctccttctgctgccgctccagctccttcatgcggatctcgcgagcctccgcgcgggccgcccgttttgcagcgagccgggcttccgcctcccgcgcgatctggttgagcgcgtcgtcctccgccgtgagccgctcccggttggggagccgcttgcgccccgatccctgggtgcccatgtccatcgaccgcgtcgcccgcagctgccgcggggcccgttgctccagccgctcgcgccgccccggcccggcccc

SEQ ID NO: 13346 - RNA, 4248 nt, Homo sapiens
  source 1..4248: mol_type = other RNA
gctgggattacaggcatgagccaccacgcccggccaaaaacatttaaaaaatgactgtccctgctcaaatactgcagtaggaaatgtaatttgacatatatcacttccagaaaaaaactttaaatctttctataaaatgaatttgatacatcatcagcatgaagtgaagttaaaatctcttacaaagtaaattcaggtatatcaacaatgagatccaaaagtatcggttcaagatcaaagactcatatgaggtaaaggcaaataaagcccctcatgctttcagacatttacttgttatccttaaaatgattattgttctaaggtgcaaatcttatcattcagtgacctatttgctatttggctgtttatctcctttaaataaaataccatacaggttataatgtacattttaaaatcaaatatgaaagtacacatatgtgaacaagacattaatttaaatatcaattatattcataatacagaagtctaagaatgctatttggtcatttcaattagatgctgatatatttggtcaagaaaacccacattcctatcagcctaaggcaaatagtaaatgcctctatttttattaagtggactataaacagtagacattattgtttgatactactggaatgctctcaattagaacgtacactgataacaaatatgtctttctaatctgggtgataacctcaatgattacatggaaatctacaagtaacagtctataacttaaagcagtagagcacctggtaattgtcatacagtgcctctctatgaatttagaacattctacttacattggcagtggagagaaaagaccccttcacactgagacttcctgtgcaccgcgcctgccgcctgcctcagcttaggacatggtacagtcttctttgcttttgcccttctcattccctcctctggtatcttctctgctttctggattgaagtgccctggctctcttcctggtgccgacaagtcatcgttctctaggctattgctgtctaaagctttcctgacggtctgacttggatgttctgacatctcacacctctctgtactttctgcttcacaggcatcactaatgtcctgtgagggactttcatgttcgggcagggtgcagcgatctgcgtcttcgctctttggttctgcaggactgctttgagtggcaccatctattttagcattatcttttgcaacaccttcatctaattcttcaccaccagccctcgggcctgatgattgaacggtgtcatcctcaaaatctaatgtgtctccatcagctagtacctcctcagctgctgtttgtacatcatcaccttcttggtcaagttttccatccaacttaattttaggattctccggacaatcaacattttcactgctttctgctgcaattttctgttttggattttcagtcacctcgttttgggcttccactgctgactttctgtcagtagactttacctgctcttcttccttaatttcacttaaatctgtgttctgatacgttaactcttttttaacatctttaagggtttctacgggtactggggattttttcttcttgtttttctttttcttgttctttgtcttcttctgcgatgagtccaatgcctctccctgttggtcactcttttcttcatcgggctctttcatatctaagggttcattttgagtgtctactgtacttggacctgtcgcttcctgacagttgccctcagttcctgctggagaaccaggaacttctgtcttgattggtttctcgtcccttaatcctgtttcttcaccctcttcttcgttgtgatccctacctacttctgtactgtgcgctggaacctccttgggctcagctgcttcctggttggtgaattctttctctaaactatgccctgtgcttgtctctaactcttgggggacctctaccatacatttgtcatcatgataaactgtgtcatcactatgccctaaaggacacgaggccactgtgcctgcctgctcttcaacctgagtcactgctgcctctcccacattctctgtgtggttcccaccatctaagtcactccaacagttggatggctcaaggggagttctggtcctgtcatctggtgcacccatgacctcatttgactcaacctgtactgtgttttcagggagagaactgctctcaagaatttggctttgaacctgttcctcataggtagcacctgctaaggttcctaggaatggggcagtgtcttcagaggatttctggtcctcggtattctcaccagcagggaatacctctatgtccacacagtccttcactgtgtcctctgtgtgttgttctttctcagtattgtgcaagatttctcttttccccacattcgccacgatttcatttttcacctccacttcactggctcttcctagggtcccatcccctgtcgacttgagggcatttaactcttcttttgtcatcttggtaggaccttggtatccaacattattgagggtgtcggaagtctctccattggtagctatttctgaatttaggattattccatgtttctttaattcctctttcagcatgactacttcttctctaagatcatcccgttcactccttacggaatcaaagaactctttctgcctctctaatgcccctatctttttgtctttccactctattgtttcctgaagatcagaaatctccctgatagaactcgcctgtttctgctgtagctgtcggatttcctcgagcatttcctctctttgcttcagggcctccttgacttcagcaaactgaaattgcagtatactgtgggcgtgtttttccctttcaaattctttgtttttctcttcgtactgccgcctagattcagccagctgttcttcaagctccagcaacatatcttttagggtatcaacctggtacatgaagtttgtcttttcattgtctagctgagcattggaaaccatagccttcttatatttctcttcaacttctgctagagagtccttcatctctttcaatccctgcatgtatttgccttctacatcctgaatctggtcctttaactcattgagttccttgatttccctgatggatgcctcggtgtcgatggagatggaggtgtctccgctgcctctccgagaggaagtcccacccagagaggccagcgtggctgcagacaggcccggcatgttacgagaccccttctcagtaaaatctttttctggtctctcttctaccacagggctggcccgggccgagctggccctggaggaggcgcgggagctggagttgaggtggccgctgtactccgagggagcacgggagccggaggtgctgccccgtcgggtcccaccgaagctgccttcatccaacacagacgcccggtaactccccgaaggccgggcagcgctgtacagacaggagggcaacttctcctccctggatgatgacaaagtagagaatctgctgtcaccgctgtagctggaattcctgccagatcttctattcagggactgtgatccatacaattctccatcataaccatttgtccaggcgtaaggacccccatactccaagtcaggctgcgacctcaggcttccacgactacccactgacatgcgctcgtcttcatcagaagccgatgtgtttcttctggatctacgagagtagcgctcactgtcttccatccactgctcgatgtcaccccattttgtatccagcccataatatttcttttggacctgatagatctccttctgctgccgctccagctccttcatgcggatctcgcgagcctccgcgcgggccgcccgttttgcagcgagccgggcttccgcctttgaagaatgaagatcttagatgaacttcagggggagtgtgaggaacgccagagagcagccatttggagagacatgcttggcacgagagtggaaattctggaataactggagatcaaatagccactcctgaccacgtcacctttataccctgtacctcactgggcagctgccttggcatgatgagagggcgtggtcccctaaacgcactggaggctttccaaatgcttctctgacctgaccgtcggcttgattttagttgctgagattccactgaagccctcgccccttgtctccaccccgttggtggcatctgtatcaaatgtgctgtcgggctttttgggaaaccctaggattgataaagagcagggtcccctgacgtttggggttgcacagttccttgtcgtggg

SEQ ID NO: 13347 - RNA, 3916 nt, Homo sapiens
  source 1..3916: mol_type = other RNA
gctgggattacaggcatgagccaccacgcccggccaaaaacatttaaaaaatgactgtccctgctcaaatactgcagtaggaaatgtaatttgacatatatcacttccagaaaaaaactttaaatctttctataaaatgaatttgatacatcatcagcatgaagtgaagttaaaatctcttacaaagtaaattcaggtatatcaacaatgagatccaaaagtatcggttcaagatcaaagactcatatgaggtaaaggcaaataaagcccctcatgctttcagacatttacttgttatccttaaaatgattattgttctaaggtgcaaatcttatcattcagtgacctatttgctatttggctgtttatctcctttaaataaaataccatacaggttataatgtacattttaaaatcaaatatgaaagtacacatatgtgaacaagacattaatttaaatatcaattatattcataatacagaagtctaagaatgctatttggtcatttcaattagatgctgatatatttggtcaagaaaacccacattcctatcagcctaaggcaaatagtaaatgcctctatttttattaagtggactataaacagtagacattattgtttgatactactggaatgctctcaattagaacgtacactgataacaaatatgtctttctaatctgggtgataacctcaatgattacatggaaatctacaagtaacagtctataacttaaagcagtagagcacctggtaattgtcatacagtgcctctctatgaatttagaacattctacttacattggcagtggagagaaaagaccccttcacactgagacttcctgtgcaccgcgcctgccgcctgcctcagcttaggacatggtacagtcttctttgcttttgcccttctcattccctcctctggtatcttctctgctttctggattgaagtgccctggctctcttcctggtgccgacaagtcatcgttctctaggctattgctgtctaaagctttcctgacggtctgacttggatgttctgacatctcacacctctctgtactttctgcttcacaggcatcactaatgtcctgtgagggactttcatgttcgggcagggtgcagcgatctgcgtcttcgctctttggttctgcaggactgctttgagtggcaccatctattttagcattatcttttgcaacaccttcatctaattcttcaccaccagccctcgggcctgatgattgaacggtgtcatcctcaaaatctaatgtgtctccatcagctagtacctcctcagctgctgtttgtacatcatcaccttcttggtcaagttttccatccaacttaattttaggattctccggacaatcaacattttcactgctttctgctgcaattttctgttttggattttcagtcacctcgttttgggcttccactgctgactttctgtcagtagactttacctgctcttcttccttaatttcacttaaatctgtgttctgatacgttaactcttttttaacatctttaagggtttctacgggtactggggattttttcttcttgtttttctttttcttgttctttgtcttcttctgcgatgagtccaatgcctctccctgttggtcactcttttcttcatcgggctctttcatatctaagggttcattttgagtgtctactgtacttggacctgtcgcttcctgacagttgccctcagttcctgctggagaaccaggaacttctgtcttgattggtttctcgtcccttaatcctgtttcttcaccctcttcttcgttgtgatccctacctacttctgtactgtgcgctggaacctccttgggctcagctgcttcctggttggtgaattctttctctaaactatgccctgtgcttgtctctaactcttgggggacctctaccatacatttgtcatcatgataaactgtgtcatcactatgccctaaaggacacgaggccactgtgcctgcctgctcttcaacctgagtcactgctgcctctcccacattctctgtgtggttcccaccatctaagtcactccaacagttggatggctcaaggggagttctggtcctgtcatctggtgcacccatgacctcatttgactcaacctgtactgtgttttcagggagagaactgctctcaagaatttggctttgaacctgttcctcataggtagcacctgctaaggttcctaggaatggggcagtgtcttcagaggatttctggtcctcggtattctcaccagcagggaatacctctatgtccacacagtccttcactgtgtcctctgtgtgttgttctttctcagtattgtgcaagatttctcttttccccacattcgccacgatttcatttttcacctccacttcactggctcttcctagggtcccatcccctgtcgacttgagggcatttaactcttcttttgtcatcttggtaggaccttggtatccaacattattgagggtgtcggaagtctctccattggtagctatttctgaatttaggattattccatgtttctttaattcctctttcagcatgactacttcttctctaagatcatcccgttcactccttacggaatcaaagaactctttctgcctctctaatgcccctatctttttgtctttccactctattgtttcctgaagatcagaaatctccctgatagaactcgcctgtttctgctgtagctgtcggatttcctcgagcatttcctctctttgcttcagggcctccttgacttcagcaaactgaaattgcagtatactgtgggcgtgtttttccctttcaaattctttgtttttctcttcgtactgccgcctagattcagccagctgttcttcaagctccagcaacatatcttttagggtatcaacctggtacatgaagtttgtcttttcattgtctagctgagcattggaaaccatagccttcttatatttctcttcaacttctgctagagagtccttcatctctttcaatccctgcatgtatttgccttctacatcctgaatctggtcctttaactcattgagttccttgatttccctgatggatgcctcggtgtcgatggagatggaggtgtctccgctgcctctccgagaggaagtcccacccagagaggccagcgtggctgcagacaggcccggcatgttacgagaccccttctcagtaaaatctttttctggtctctcttctaccacagggctggcccgggccgagctggccctggaggaggcgcgggagctggagttgaggtggccgctgtactccgagggagcacgggagccggaggtgctgccccgtcgggtcccaccgaagctgccttcatccaacacagacgcccggtaactccccgaaggccgggcagcgctgtacagacaggagggcaacttctcctccctggatgatgacaaagtagagaatctgctgtcaccgctgtagctggaattcctgccagatcttctattcagggactgtgatccatacaattctccatcataaccatttgtccaggcgtaaggacccccatactccaagtcaggctgcgacctcaggcttccacgactacccactgacatgcgctcgtcttcatcagaagccgatgtgtttcttctggatctacgagagtagcgctcactgtcttcctccttctgctgccgctccagctccttcatgcggatctcgcgagcctccgcgcgggccgcccgttttgcagcgagccgggcttccgcctcccgcgcgatctggttgagcgcgtcgtcctccgccgtgagccgctcccggttggggagccgcttgcgccccgatccctgggtgcccatgtccatcgaccgcgtcgcccgcagctgccgcggggcccgttgctccagccgctc

SEQ ID NO: 13348 - RNA, 3964 nt, Homo sapiens
  source 1..3964: mol_type = other RNA
gctgggattacaggcatgagccaccacgcccggccaaaaacatttaaaaaatgactgtccctgctcaaatactgcagtaggaaatgtaatttgacatatatcacttccagaaaaaaactttaaatctttctataaaatgaatttgatacatcatcagcatgaagtgaagttaaaatctcttacaaagtaaattcaggtatatcaacaatgagatccaaaagtatcggttcaagatcaaagactcatatgaggtaaaggcaaataaagcccctcatgctttcagacatttacttgttatccttaaaatgattattgttctaaggtgcaaatcttatcattcagtgacctatttgctatttggctgtttatctcctttaaataaaataccatacaggttataatgtacattttaaaatcaaatatgaaagtacacatatgtgaacaagacattaatttaaatatcaattatattcataatacagaagtctaagaatgctatttggtcatttcaattagatgctgatatatttggtcaagaaaacccacattcctatcagcctaaggcaaatagtaaatgcctctatttttattaagtggactataaacagtagacattattgtttgatactactggaatgctctcaattagaacgtacactgataacaaatatgtctttctaatctgggtgataacctcaatgattacatggaaatctacaagtaacagtctataacttaaagcagtagagcacctggtaattgtcatacagtgcctctctatgaatttagaacattctacttacattggcagtggagagaaaagaccccttcacactgagacttcctgtgcaccgcgcctgccgcctgcctcagcttaggacatggtacagtcttctttgcttttgcccttctcattccctcctctggtatcttctctgctttctggattgaagtgccctggctctcttcctggtgccgacaagtcatcgttctctaggctattgctgtctaaagctttcctgacggtctgacttggatgttctgacatctcacacctctctgtactttctgcttcacaggcatcactaatgtcctgtgagggactttcatgttcgggcagggtgcagcgatctgcgtcttcgctctttggttctgcaggactgctttgagtggcaccatctattttagcattatcttttgcaacaccttcatctaattcttcaccaccagccctcgggcctgatgattgaacggtgtcatcctcaaaatctaatgtgtctccatcagctagtacctcctcagctgctgtttgtacatcatcaccttcttggtcaagttttccatccaacttaattttaggattctccggacaatcaacattttcactgctttctgctgcaattttctgttttggattttcagtcacctcgttttgggcttccactgctgactttctgtcagtagactttacctgctcttcttccttaatttcacttaaatctgtgttctgatacgttaactcttttttaacatctttaagggtttctacgggtactggggattttttcttcttgtttttctttttcttgttctttgtcttcttctgcgatgagtccaatgcctctccctgttggtcactcttttcttcatcgggctctttcatatctaagggttcattttgagtgtctactgtacttggacctgtcgcttcctgacagttgccctcagttcctgctggagaaccaggaacttctgtcttgattggtttctcgtcccttaatcctgtttcttcaccctcttcttcgttgtgatccctacctacttctgtactgtgcgctggaacctccttgggctcagctgcttcctggttggtgaattctttctctaaactatgccctgtgcttgtctctaactcttgggggacctctaccatacatttgtcatcatgataaactgtgtcatcactatgccctaaaggacacgaggccactgtgcctgcctgctcttcaacctgagtcactgctgcctctcccacattctctgtgtggttcccaccatctaagtcactccaacagttggatggctcaaggggagttctggtcctgtcatctggtgcacccatgacctcatttgactcaacctgtactgtgttttcagggagagaactgctctcaagaatttggctttgaacctgttcctcataggtagcacctgctaaggttcctaggaatggggcagtgtcttcagaggatttctggtcctcggtattctcaccagcagggaatacctctatgtccacacagtccttcactgtgtcctctgtgtgttgttctttctcagtattgtgcaagatttctcttttccccacattcgccacgatttcatttttcacctccacttcactggctcttcctagggtcccatcccctgtcgacttgagggcatttaactcttcttttgtcatcttggtaggaccttggtatccaacattattgagggtgtcggaagtctctccattggtagctatttctgaatttaggattattccatgtttctttaattcctctttcagcatgactacttcttctctaagatcatcccgttcactccttacggaatcaaagaactctttctgcctctctaatgcccctatctttttgtctttccactctattgtttcctgaagatcagaaatctccctgatagaactcgcctgtttctgctgtagctgtcggatttcctcgagcatttcctctctttgcttcagggcctccttgacttcagcaaactgaaattgcagtatactgtgggcgtgtttttccctttcaaattctttgtttttctcttcgtactgccgcctagattcagccagctgttcttcaagctccagcaacatatcttttagggtatcaacctggtacatgaagtttgtcttttcattgtctagctgagcattggaaaccatagccttcttatatttctcttcaacttctgctagagagtccttcatctctttcaatccctgcatgtatttgccttctacatcctgaatctggtcctttaactcattgagttccttgatttccctgatggatgcctcggtgtcgatggagatggaggtgtctccgctgcctctccgagaggaagtcccacccagagaggccagcgtggctgcagacaggcccggcatgttacgagaccccttctcagtaaaatctttttctggtctctcttctaccacagggctggcccgggccgagctggccctggaggaggcgcgggagctggagttgaggtggccgctgtactccgagggagcacgggagccggaggtgctgccccgtcgggtcccaccgaagctgccttcatccaacacagacgcccggtaactccccgaaggccgggcagcgctgtacagacaggagggcaacttctcctccctggatgatgacaaagtagagaatctgctgtcaccgctgtagctggaattcctgccagatcttctattcagggactgtgatccatacaattctccatcataaccatttgtcctcaggcttccacgactacccactgacatgcgctcgtcttcatcagaagccgatgtgtttcttctggatctacgagagtagcgctcactgtcttccatccactgctcgatgtcaccccattttgtatccagcccataatatttcttttggacctgatagatctccttctgctgccgctccagctccttcatgcggatctcgcgagcctccgcgcgggccgcccgttttgcagcgagccgggcttccgcctcccgcgcgatctggttgagcgcgtcgtcctccgccgtgagccgctcccggttggggagccgcttgcgccccgatccctgggtgcccatgtccatcgaccgcgtcgcccgcagctgccgcggggcccgttgctccagccgctcgcgccgccccggcccggcccc

SEQ ID NO: 13349 - RNA, 4006 nt, Homo sapiens
  source 1..4006: mol_type = other RNA
gctgggattacaggcatgagccaccacgcccggccaaaaacatttaaaaaatgactgtccctgctcaaatactgcagtaggaaatgtaatttgacatatatcacttccagaaaaaaactttaaatctttctataaaatgaatttgatacatcatcagcatgaagtgaagttaaaatctcttacaaagtaaattcaggtatatcaacaatgagatccaaaagtatcggttcaagatcaaagactcatatgaggtaaaggcaaataaagcccctcatgctttcagacatttacttgttatccttaaaatgattattgttctaaggtgcaaatcttatcattcagtgacctatttgctatttggctgtttatctcctttaaataaaataccatacaggttataatgtacattttaaaatcaaatatgaaagtacacatatgtgaacaagacattaatttaaatatcaattatattcataatacagaagtctaagaatgctatttggtcatttcaattagatgctgatatatttggtcaagaaaacccacattcctatcagcctaaggcaaatagtaaatgcctctatttttattaagtggactataaacagtagacattattgtttgatactactggaatgctctcaattagaacgtacactgataacaaatatgtctttctaatctgggtgataacctcaatgattacatggaaatctacaagtaacagtctataacttaaagcagtagagcacctggtaattgtcatacagtgcctctctatgaatttagaacattctacttacattggcagtggagagaaaagaccccttcacactgagacttcctgtgcaccgcgcctgccgcctgcctcagcttaggacatggtacagtcttctttgcttttgcccttctcattccctcctctggtatcttctctgctttctggattgaagtgccctggctctcttcctggtgccgacaagtcatcgttctctaggctattgctgtctaaagctttcctgacggtctgacttggatgttctgacatctcacacctctctgtactttctgcttcacaggcatcactaatgtcctgtgagggactttcatgttcgggcagggtgcagcgatctgcgtcttcgctctttggttctgcaggactgctttgagtggcaccatctattttagcattatcttttgcaacaccttcatctaattcttcaccaccagccctcgggcctgatgattgaacggtgtcatcctcaaaatctaatgtgtctccatcagctagtacctcctcagctgctgtttgtacatcatcaccttcttggtcaagttttccatccaacttaattttaggattctccggacaatcaacattttcactgctttctgctgcaattttctgttttggattttcagtcacctcgttttgggcttccactgctgactttctgtcagtagactttacctgctcttcttccttaatttcacttaaatctgtgttctgatacgttaactcttttttaacatctttaagggtttctacgggtactggggattttttcttcttgtttttctttttcttgttctttgtcttcttctgcgatgagtccaatgcctctccctgttggtcactcttttcttcatcgggctctttcatatctaagggttcattttgagtgtctactgtacttggacctgtcgcttcctgacagttgccctcagttcctgctggagaaccaggaacttctgtcttgattggtttctcgtcccttaatcctgtttcttcaccctcttcttcgttgtgatccctacctacttctgtactgtgcgctggaacctccttgggctcagctgcttcctggttggtgaattctttctctaaactatgccctgtgcttgtctctaactcttgggggacctctaccatacatttgtcatcatgataaactgtgtcatcactatgccctaaaggacacgaggccactgtgcctgcctgctcttcaacctgagtcactgctgcctctcccacattctctgtgtggttcccaccatctaagtcactccaacagttggatggctcaaggggagttctggtcctgtcatctggtgcacccatgacctcatttgactcaacctgtactgtgttttcagggagagaactgctctcaagaatttggctttgaacctgttcctcataggtagcacctgctaaggttcctaggaatggggcagtgtcttcagaggatttctggtcctcggtattctcaccagcagggaatacctctatgtccacacagtccttcactgtgtcctctgtgtgttgttctttctcagtattgtgcaagatttctcttttccccacattcgccacgatttcatttttcacctccacttcactggctcttcctagggtcccatcccctgtcgacttgagggcatttaactcttcttttgtcatcttggtaggaccttggtatccaacattattgagggtgtcggaagtctctccattggtagctatttctgaatttaggattattccatgtttctttaattcctctttcagcatgactacttcttctctaagatcatcccgttcactccttacggaatcaaagaactctttctgcctctctaatgcccctatctttttgtctttccactctattgtttcctgaagatcagaaatctccctgatagaactcgcctgtttctgctgtagctgtcggatttcctcgagcatttcctctctttgcttcagggcctccttgacttcagcaaactgaaattgcagtatactgtgggcgtgtttttccctttcaaattctttgtttttctcttcgtactgccgcctagattcagccagctgttcttcaagctccagcaacatatcttttagggtatcaacctggtacatgaagtttgtcttttcattgtctagctgagcattggaaaccatagccttcttatatttctcttcaacttctgctagagagtccttcatctctttcaatccctgcatgtatttgccttctacatcctgaatctggtcctttaactcattgagttccttgatttccctgatggatgcctcggtgtcgatggagatggaggtgtctccgctgcctctccgagaggaagtcccacccagagaggccagcgtggctgcagacaggcccggcatgttacgagaccccttctcagtaaaatctttttctggtctctcttctaccacagggctggcccgggccgagctggccctggaggaggcgcgggagctggagttgaggtggccgctgtactccgagggagcacgggagccggaggtgctgccccgtcgggtcccaccgaagctgccttcatccaacacagacgcccggtaactccccgaaggccgggcagcgctgtacagacaggagggcctcaggcttccacgactacccactgacatgcgctcgtcttcatcagaagccgatgtgtttcttctggatctacgagagtagcgctcactgtcttccatccactgctcgatgtcaccccattttgtatccagcccataatatttcttttggacctgatagatctccttctgctgccgctccagctccttcatgcggatctcgcgagcctccgcgcgggccgcccgttttgcagcgagccgggcttccgccagcttctgcgcttccgggctcaaacagtcgatctcccggctttgagcggccgcggggctggtcatcctgccgggctcggcccgctccacccggcgggaaatgctcggggaccgcgccgggagcccctcgcgggccgggccagggggcgcgcgctctgtccgcggagacggagccactcgccgctaagtgaacgctcgcgcttccggggccaggagccagcccgccggggagcggctcgcggcgctgggctcgggcgcggccgacaggggcggggcgcaggtggccgcgggctgagtcgggctcggggtggaagggcgccggggaagcgg

SEQ ID NO: 13350 - RNA, 3940 nt, Homo sapiens
  source 1..3940: mol_type = other RNA
gctgggattacaggcatgagccaccacgcccggccaaaaacatttaaaaaatgactgtccctgctcaaatactgcagtaggaaatgtaatttgacatatatcacttccagaaaaaaactttaaatctttctataaaatgaatttgatacatcatcagcatgaagtgaagttaaaatctcttacaaagtaaattcaggtatatcaacaatgagatccaaaagtatcggttcaagatcaaagactcatatgaggtaaaggcaaataaagcccctcatgctttcagacatttacttgttatccttaaaatgattattgttctaaggtgcaaatcttatcattcagtgacctatttgctatttggctgtttatctcctttaaataaaataccatacaggttataatgtacattttaaaatcaaatatgaaagtacacatatgtgaacaagacattaatttaaatatcaattatattcataatacagaagtctaagaatgctatttggtcatttcaattagatgctgatatatttggtcaagaaaacccacattcctatcagcctaaggcaaatagtaaatgcctctatttttattaagtggactataaacagtagacattattgtttgatactactggaatgctctcaattagaacgtacactgataacaaatatgtctttctaatctgggtgataacctcaatgattacatggaaatctacaagtaacagtctataacttaaagcagtagagcacctggtaattgtcatacagtgcctctctatgaatttagaacattctacttacattggcagtggagagaaaagaccccttcacactgagacttcctgtgcaccgcgcctgccgcctgcctcagcttaggacatggtacagtcttctttgcttttgcccttctcattccctcctctggtatcttctctgctttctggattgaagtgccctggctctcttcctggtgccgacaagtcatcgttctctaggctattgctgtctaaagctttcctgacggtctgacttggatgttctgacatctcacacctctctgtactttctgcttcacaggcatcactaatgtcctgtgagggactttcatgttcgggcagggtgcagcgatctgcgtcttcgctctttggttctgcaggactgctttgagtggcaccatctattttagcattatcttttgcaacaccttcatctaattcttcaccaccagccctcgggcctgatgattgaacggtgtcatcctcaaaatctaatgtgtctccatcagctagtacctcctcagctgctgtttgtacatcatcaccttcttggtcaagttttccatccaacttaattttaggattctccggacaatcaacattttcactgctttctgctgcaattttctgttttggattttcagtcacctcgttttgggcttccactgctgactttctgtcagtagactttacctgctcttcttccttaatttcacttaaatctgtgttctgatacgttaactcttttttaacatctttaagggtttctacgggtactggggattttttcttcttgtttttctttttcttgttctttgtcttcttctgcgatgagtccaatgcctctccctgttggtcactcttttcttcatcgggctctttcatatctaagggttcattttgagtgtctactgtacttggacctgtcgcttcctgacagttgccctcagttcctgctggagaaccaggaacttctgtcttgattggtttctcgtcccttaatcctgtttcttcaccctcttcttcgttgtgatccctacctacttctgtactgtgcgctggaacctccttgggctcagctgcttcctggttggtgaattctttctctaaactatgccctgtgcttgtctctaactcttgggggacctctaccatacatttgtcatcatgataaactgtgtcatcactatgccctaaaggacacgaggccactgtgcctgcctgctcttcaacctgagtcactgctgcctctcccacattctctgtgtggttcccaccatctaagtcactccaacagttggatggctcaaggggagttctggtcctgtcatctggtgcacccatgacctcatttgactcaacctgtactgtgttttcagggagagaactgctctcaagaatttggctttgaacctgttcctcataggtagcacctgctaaggttcctaggaatggggcagtgtcttcagaggatttctggtcctcggtattctcaccagcagggaatacctctatgtccacacagtccttcactgtgtcctctgtgtgttgttctttctcagtattgtgcaagatttctcttttccccacattcgccacgatttcatttttcacctccacttcactggctcttcctagggtcccatcccctgtcgacttgagggcatttaactcttcttttgtcatcttggtaggaccttggtatccaacattattgagggtgtcggaagtctctccattggtagctatttctgaatttaggattattccatgtttctttaattcctctttcagcatgactacttcttctctaagatcatcccgttcactccttacggaatcaaagaactctttctgcctctctaatgcccctatctttttgtctttccactctattgtttcctgaagatcagaaatctccctgatagaactcgcctgtttctgctgtagctgtcggatttcctcgagcatttcctctctttgcttcagggcctccttgacttcagcaaactgaaattgcagtatactgtgggcgtgtttttccctttcaaattctttgtttttctcttcgtactgccgcctagattcagccagctgttcttcaagctccagcaacatatcttttagggtatcaacctggtacatgaagtttgtcttttcattgtctagctgagcattggaaaccatagccttcttatatttctcttcaacttctgctagagagtccttcatctctttcaatccctgcatgtatttgccttctacatcctgaatctggtcctttaactcattgagttccttgatttccctgatggatgcctcggtgtcgatggagatggaggtgtctccgctgcctctccgagaggaagtcccacccagagaggccagcgtggctgcagacaggcccggcatgttacgagaccccttctcagtaaaatctttttctggtctctcttctaccacagggctggcccgggccgagctggccctggaggaggcgcgggagctggagttgaggtggccgctgtactccgagggagcacgggagccggaggtgctgccccgtcgggtcccaccgaagctgccttcatccaacacagacgcccggtaactccccgaaggccgggcagcgctgtacagacaggagggcctgccagatcttctattcagggactgtgatccatacaattctccatcataaccatttgtccaggcgtaaggacccccatactccaagtcaggctgcgacctcaggcttccacgactacccactgacatgcgctcgtcttcatcagaagccgatgtgtttcttctggatctacgagagtagcgctcactgtcttccatccactgctcgatgtcaccccattttgtatccagcccataatatttcttttggacctgatagatctccttctgctgccgctccagctccttcatgcggatctcgcgagcctccgcgcgggccgcccgttttgcagcgagccgggcttccgcctcccgcgcgatctggttgagcgcgtcgtcctccgccgtgagccgctcccggttggggagccgcttgcgccccgatccctgggtgcccatgtccatcgaccgcgtcgcccgcagctgccgcggggcccgttgctccagccgctcgcgccgccccggcccggcccc

SEQ ID NO: 13351 - RNA, 3901 nt, Homo sapiens
  source 1..3901: mol_type = other RNA
gctgggattacaggcatgagccaccacgcccggccaaaaacatttaaaaaatgactgtccctgctcaaatactgcagtaggaaatgtaatttgacatatatcacttccagaaaaaaactttaaatctttctataaaatgaatttgatacatcatcagcatgaagtgaagttaaaatctcttacaaagtaaattcaggtatatcaacaatgagatccaaaagtatcggttcaagatcaaagactcatatgaggtaaaggcaaataaagcccctcatgctttcagacatttacttgttatccttaaaatgattattgttctaaggtgcaaatcttatcattcagtgacctatttgctatttggctgtttatctcctttaaataaaataccatacaggttataatgtacattttaaaatcaaatatgaaagtacacatatgtgaacaagacattaatttaaatatcaattatattcataatacagaagtctaagaatgctatttggtcatttcaattagatgctgatatatttggtcaagaaaacccacattcctatcagcctaaggcaaatagtaaatgcctctatttttattaagtggactataaacagtagacattattgtttgatactactggaatgctctcaattagaacgtacactgataacaaatatgtctttctaatctgggtgataacctcaatgattacatggaaatctacaagtaacagtctataacttaaagcagtagagcacctggtaattgtcatacagtgcctctctatgaatttagaacattctacttacattggcagtggagagaaaagaccccttcacactgagacttcctgtgcaccgcgcctgccgcctgcctcagcttaggacatggtacagtcttctttgcttttgcccttctcattccctcctctggtatcttctctgctttctggattgaagtgccctggctctcttcctggtgccgacaagtcatcgttctctaggctattgctgtctaaagctttcctgacggtctgacttggatgttctgacatctcacacctctctgtactttctgcttcacaggcatcactaatgtcctgtgagggactttcatgttcgggcagggtgcagcgatctgcgtcttcgctctttggttctgcaggactgctttgagtggcaccatctattttagcattatcttttgcaacaccttcatctaattcttcaccaccagccctcgggcctgatgattgaacggtgtcatcctcaaaatctaatgtgtctccatcagctagtacctcctcagctgctgtttgtacatcatcaccttcttggtcaagttttccatccaacttaattttaggattctccggacaatcaacattttcactgctttctgctgcaattttctgttttggattttcagtcacctcgttttgggcttccactgctgactttctgtcagtagactttacctgctcttcttccttaatttcacttaaatctgtgttctgatacgttaactcttttttaacatctttaagggtttctacgggtactggggattttttcttcttgtttttctttttcttgttctttgtcttcttctgcgatgagtccaatgcctctccctgttggtcactcttttcttcatcgggctctttcatatctaagggttcattttgagtgtctactgtacttggacctgtcgcttcctgacagttgccctcagttcctgctggagaaccaggaacttctgtcttgattggtttctcgtcccttaatcctgtttcttcaccctcttcttcgttgtgatccctacctacttctgtactgtgcgctggaacctccttgggctcagctgcttcctggttggtgaattctttctctaaactatgccctgtgcttgtctctaactcttgggggacctctaccatacatttgtcatcatgataaactgtgtcatcactatgccctaaaggacacgaggccactgtgcctgcctgctcttcaacctgagtcactgctgcctctcccacattctctgtgtggttcccaccatctaagtcactccaacagttggatggctcaaggggagttctggtcctgtcatctggtgcacccatgacctcatttgactcaacctgtactgtgttttcagggagagaactgctctcaagaatttggctttgaacctgttcctcataggtagcacctgctaaggttcctaggaatggggcagtgtcttcagaggatttctggtcctcggtattctcaccagcagggaatacctctatgtccacacagtccttcactgtgtcctctgtgtgttgttctttctcagtattgtgcaagatttctcttttccccacattcgccacgatttcatttttcacctccacttcactggctcttcctagggtcccatcccctgtcgacttgagggcatttaactcttcttttgtcatcttggtaggaccttggtatccaacattattgagggtgtcggaagtctctccattggtagctatttctgaatttaggattattccatgtttctttaattcctctttcagcatgactacttcttctctaagatcatcccgttcactccttacggaatcaaagaactctttctgcctctctaatgcccctatctttttgtctttccactctattgtttcctgaagatcagaaatctccctgatagaactcgcctgtttctgctgtagctgtcggatttcctcgagcatttcctctctttgcttcagggcctccttgacttcagcaaactgaaattgcagtatactgtgggcgtgtttttccctttcaaattctttgtttttctcttcgtactgccgcctagattcagccagctgttcttcaagctccagcaacatatcttttagggtatcaacctggtacatgaagtttgtcttttcattgtctagctgagcattggaaaccatagccttcttatatttctcttcaacttctgctagagagtccttcatctctttcaatccctgcatgtatttgccttctacatcctgaatctggtcctttaactcattgagttccttgatttccctgatggatgcctcggtgtcgatggagatggaggtgtctccgctgcctctccgagaggaagtcccacccagagaggccagcgtggctgcagacaggcccggcatgttacgagaccccttctcagtaaaatctttttctggtctctcttctaccacagggctggcccgggccgagctggccctggaggaggcgcgggagctggagttgaggtggccgctgtactccgagggagcacgggagccggaggtgctgccccgtcgggtcccaccgaagctgccttcatccaacacagacgcccggtaactccccgaaggccgggcagcgctgtacagacaggagggcctgccagatcttctattcagggactgtgatccatacaattctccatcataaccatttgtcctcaggcttccacgactacccactgacatgcgctcgtcttcatcagaagccgatgtgtttcttctggatctacgagagtagcgctcactgtcttccatccactgctcgatgtcaccccattttgtatccagcccataatatttcttttggacctgatagatctccttctgctgccgctccagctccttcatgcggatctcgcgagcctccgcgcgggccgcccgttttgcagcgagccgggcttccgcctcccgcgcgatctggttgagcgcgtcgtcctccgccgtgagccgctcccggttggggagccgcttgcgccccgatccctgggtgcccatgtccatcgaccgcgtcgcccgcagctgccgcggggcccgttgctccagccgctcgcgccgccccggcccggcccc

SEQ ID NO: 13352 - RNA, 3598 nt, Homo sapiens
  source 1..3598: mol_type = other RNA
gctgggattacaggcatgagccaccacgcccggccaaaaacatttaaaaaatgactgtccctgctcaaatactgcagtaggaaatgtaatttgacatatatcacttccagaaaaaaactttaaatctttctataaaatgaatttgatacatcatcagcatgaagtgaagttaaaatctcttacaaagtaaattcaggtatatcaacaatgagatccaaaagtatcggttcaagatcaaagactcatatgaggtaaaggcaaataaagcccctcatgctttcagacatttacttgttatccttaaaatgattattgttctaaggtgcaaatcttatcattcagtgacctatttgctatttggctgtttatctcctttaaataaaataccatacaggttataatgtacattttaaaatcaaatatgaaagtacacatatgtgaacaagacattaatttaaatatcaattatattcataatacagaagtctaagaatgctatttggtcatttcaattagatgctgatatatttggtcaagaaaacccacattcctatcagcctaaggcaaatagtaaatgcctctatttttattaagtggactataaacagtagacattattgtttgatactactggaatgctctcaattagaacgtacactgataacaaatatgtctttctaatctgggtgataacctcaatgattacatggaaatctacaagtaacagtctataacttaaagcagtagagcacctggtaattgtcatacagtgcctctctatgaatttagaacattctacttacattggcagtggagagaaaagaccccttcacactgagacttcctgtgcaccgcgcctgccgcctgcctcagcttaggacatggtacagtcttctttgcttttgcccttctcattccctcctctggtatcttctctgctttctggattgaagtgccctggctctcttcctggtgccgacaagtcatcgttctctaggctattgctgtctaaagctttcctgacggtctgacttggatgttctgacatctcacacctctctgtactttctgcttcacaggcatcactaatgtcctgtgagggactttcatgttcgggcagggtgcagcgatctgcgtcttcgctctttggttctgcaggactgctttgagtggcaccatctattttagcattatcttttgcaacaccttcatctaattcttcaccaccagccctcgggcctgatgattgaacggtgtcatcctcaaaatctaatgtgtctccatcagctagtacctcctcagctgctgtttgtacatcatcaccttcttggtcaagttttccatccaacttaattttaggattctccggacaatcaacattttcactgctttctgctgcaattttctgttttggattttcagtcacctcgttttgggcttccactgctgactttctgtcagtagactttacctgctcttcttccttaatttcacttaaatctgtgttctgatacgttaactcttttttaacatctttaagggtttctacgggtactggggattttttcttcttgtttttctttttcttgttctttgtcttcttctgcgatgagtccaatgcctctccctgttggtcactcttttcttcatcgggctctttcatatctaagggttcattttgagtgtctactgtacttggacctgtcgcttcctgacagttgccctcagttcctgctggagaaccaggaacttctgtcttgattggtttctcgtcccttaatcctgtttcttcaccctcttcttcgttgtgatccctacctacttctgtactgtgcgctggaacctccttgggctcagctgcttcctggttggtgaattctttctctaaactatgccctgtgcttgtctctaactcttgggggacctctaccatacatttgtcatcatgataaactgtgtcatcactatgccctaaaggacacgaggccactgtgcctgcctgctcttcaacctgagtcactgctgcctctcccacattctctgtgtggttcccaccatctaagtcactccaacagttggatggctcaaggggagttctggtcctgtcatctggtgcacccatgacctcatttgactcaacctgtactgtgttttcagggagagaactgctctcaagaatttggctttgaacctgttcctcataggtagcacctgctaaggttcctaggaatggggcagtgtcttcagaggatttctggtcctcggtattctcaccagcagggaatacctctatgtccacacagtccttcactgtgtcctctgtgtgttgttctttctcagtattgtgcaagatttctcttttccccacattcgccacgatttcatttttcacctccacttcactggctcttcctagggtcccatcccctgtcgacttgagggcatttaactcttcttttgtcatcttggtaggaccttggtatccaacattattgagggtgtcggaagtctctccattggtagctatttctgaatttaggattattccatgtttctttaattcctctttcagcatgactacttcttctctaagatcatcccgttcactccttacggaatcaaagaactctttctgcctctctaatgcccctatctttttgtctttccactctattgtttcctgaagatcagaaatctccctgatagaactcgcctgtttctgctgtagctgtcggatttcctcgagcatttcctctctttgcttcagggcctccttgacttcagcaaactgaaattgcagtatactgtgggcgtgtttttccctttcaaattctttgtttttctcttcgtactgccgcctagattcagccagctgttcttcaagctccagcaacatatcttttagggtatcaacctggtacatgaagtttgtcttttcattgtctagctgagcattggaaaccatagccttcttatatttctcttcaacttctgctagagagtccttcatctctttcaatccctgcatgtatttgccttctacatcctgaatctggtcctttaactcattgagttccttgatttccctgatggatgcctcggtgtcgatggagatggaggtgtctccgctgcctctccgagaggaagtcccacccagagaggccagcgtggctgcagacaggcccggcatgttacgagaccccttctcagtaaaatctttttctggtctctcttctaccagcttctgcgcttccgggctcaaacagtcgatctcccggctttgagcggccgcggggctggtcatcctgccgggctcggcccgctccacccggcgggaaatgctcggggaccgcgccgggagcccctcgcgggccgggccagggggcgcgcgctctgtccgcggagacggagccactcgccgctaagtgaacgctcgcgcttccggggccaggagccagcccgccggggagcggctcgcggcgctgggctcgggcgcggccgacaggggcggggcgcaggtggccgcgggctgagtcgggctcggggtggaagggcgccggggaagcgggactcgggcgcctccgcccgtcccacggcc

SEQ ID NO: 13353 - RNA, 3652 nt, Homo sapiens
  source 1..3652: mol_type = other RNA
gctgggattacaggcatgagccaccacgcccggccaaaaacatttaaaaaatgactgtccctgctcaaatactgcagtaggaaatgtaatttgacatatatcacttccagaaaaaaactttaaatctttctataaaatgaatttgatacatcatcagcatgaagtgaagttaaaatctcttacaaagtaaattcaggtatatcaacaatgagatccaaaagtatcggttcaagatcaaagactcatatgaggtaaaggcaaataaagcccctcatgctttcagacatttacttgttatccttaaaatgattattgttctaaggtgcaaatcttatcattcagtgacctatttgctatttggctgtttatctcctttaaataaaataccatacaggttataatgtacattttaaaatcaaatatgaaagtacacatatgtgaacaagacattaatttaaatatcaattatattcataatacagaagtctaagaatgctatttggtcatttcaattagatgctgatatatttggtcaagaaaacccacattcctatcagcctaaggcaaatagtaaatgcctctatttttattaagtggactataaacagtagacattattgtttgatactactggaatgctctcaattagaacgtacactgataacaaatatgtctttctaatctgggtgataacctcaatgattacatggaaatctacaagtaacagtctataacttaaagcagtagagcacctggtaattgtcatacagtgcctctctatgaatttagaacattctacttacattggcagtggagagaaaagaccccttcacactgagacttcctgtgcaccgcgcctgccgcctgcctcagcttaggacatggtacagtcttctttgcttttgcccttctcattccctcctctggtatcttctctgctttctggattgaagtgccctggctctcttcctggtgccgacaagtcatcgttctctaggctattgctgtctaaagctttcctgacggtctgacttggatgttctgacatctcacacctctctgtactttctgcttcacaggcatcactaatgtcctgtgagggactttcatgttcgggcagggtgcagcgatctgcgtcttcgctctttggttctgcaggactgctttgagtggcaccatctattttagcattatcttttgcaacaccttcatctaattcttcaccaccagccctcgggcctgatgattgaacggtgtcatcctcaaaatctaatgtgtctccatcagctagtacctcctcagctgctgtttgtacatcatcaccttcttggtcaagttttccatccaacttaattttaggattctccggacaatcaacattttcactgctttctgctgcaattttctgttttggattttcagtcacctcgttttgggcttccactgctgactttctgtcagtagactttacctgctcttcttccttaatttcacttaaatctgtgttctgatacgttaactcttttttaacatctttaagggtttctacgggtactggggattttttcttcttgtttttctttttcttgttctttgtcttcttctgcgatgagtccaatgcctctccctgttggtcactcttttcttcatcgggctctttcatatctaagggttcattttgagtgtctactgtacttggacctgtcgcttcctgacagttgccctcagttcctgctggagaaccaggaacttctgtcttgattggtttctcgtcccttaatcctgtttcttcaccctcttcttcgttgtgatccctacctacttctgtactgtgcgctggaacctccttgggctcagctgcttcctggttggtgaattctttctctaaactatgccctgtgcttgtctctaactcttgggggacctctaccatacatttgtcatcatgataaactgtgtcatcactatgccctaaaggacacgaggccactgtgcctgcctgctcttcaacctgagtcactgctgcctctcccacattctctgtgtggttcccaccatctaagtcactccaacagttggatggctcaaggggagttctggtcctgtcatctggtgcacccatgacctcatttgactcaacctgtactgtgttttcagggagagaactgctctcaagaatttggctttgaacctgttcctcataggtagcacctgctaaggttcctaggaatggggcagtgtcttcagaggatttctggtcctcggtattctcaccagcagggaatacctctatgtccacacagtccttcactgtgtcctctgtgtgttgttctttctcagtattgtgcaagatttctcttttccccacattcgccacgatttcatttttcacctccacttcactggctcttcctagggtcccatcccctgtcgacttgagggcatttaactcttcttttgtcatcttggtaggaccttggtatccaacattattgagggtgtcggaagtctctccattggtagctatttctgaatttaggattattccatgtttctttaattcctctttcagcatgactacttcttctctaagatcatcccgttcactccttacggaatcaaagaactctttctgcctctctaatgcccctatctttttgtctttccactctattgtttcctgaagatcagaaatctccctgatagaactcgcctgtttctgctgtagctgtcggatttcctcgagcatttcctctctttgcttcagggcctccttgacttcagcaaactgaaattgcagtatactgtgggcgtgtttttccctttcaaattctttgtttttctcttcgtactgccgcctagattcagccagctgttcttcaagctccagcaacatatcttttagggtatcaacctggtacatgaagtttgtcttttcattgtctagctgagcattggaaaccatagccttcttatatttctcttcaacttctgctagagagtccttcatctctttcaatccctgcatgtatttgccttctacatcctgaatctggtcctttaactcattgagttccttgatttccctgatggatgcctcggtgtcgatggagatggaggtgtctccgctgcctctccgagaggaagtcccacccagagaggccagcgtggctgcagacaggcccggcatgttacgagaccccttctcagtaaaatctttttctggtctctcttctaccctcaggcttccacgactacccactgacatgcgctcgtcttcatcagaagccgatgtgtttcttctggatctacgagagtagcgctcactgtcttccatccactgctcgatgtcaccccattttgtatccagcccataatatttcttttggacctgatagatctccttctgctgccgctccagctccttcatgcggatctcgcgagcctccgcgcgggccgcccgttttgcagcgagccgggcttccgcctcccgcgcgatctggttgagcgcgtcgtcctccgccgtgagccgctcccggttggggagccgcttgcgccccgatccctgggtgcccatgtccatcgaccgcgtcgcccgcagctgccgcggggcccgttgctccagccgctcgcgccgccccggcccggcccc

SEQ ID NO: 13354 - RNA, 3581 nt, Homo sapiens
  source 1..3581: mol_type = other RNA
gctgggattacaggcatgagccaccacgcccggccaaaaacatttaaaaaatgactgtccctgctcaaatactgcagtaggaaatgtaatttgacatatatcacttccagaaaaaaactttaaatctttctataaaatgaatttgatacatcatcagcatgaagtgaagttaaaatctcttacaaagtaaattcaggtatatcaacaatgagatccaaaagtatcggttcaagatcaaagactcatatgaggtaaaggcaaataaagcccctcatgctttcagacatttacttgttatccttaaaatgattattgttctaaggtgcaaatcttatcattcagtgacctatttgctatttggctgtttatctcctttaaataaaataccatacaggttataatgtacattttaaaatcaaatatgaaagtacacatatgtgaacaagacattaatttaaatatcaattatattcataatacagaagtctaagaatgctatttggtcatttcaattagatgctgatatatttggtcaagaaaacccacattcctatcagcctaaggcaaatagtaaatgcctctatttttattaagtggactataaacagtagacattattgtttgatactactggaatgctctcaattagaacgtacactgataacaaatatgtctttctaatctgggtgataacctcaatgattacatggaaatctacaagtaacagtctataacttaaagcagtagagcacctggtaattgtcatacagtgcctctctatgaatttagaacattctacttacattggcagtggagagaaaagaccccttcacactgagacttcctgtgcaccgcgcctgccgcctgcctcagcttaggacatggtacagtcttctttgcttttgcccttctcattccctcctctggtatcttctctgctttctggattgaagtgccctggctctcttcctggtgccgacaagtcatcgttctctaggctattgctgtctaaagctttcctgacggtctgacttggatgttctgacatctcacacctctctgtactttctgcttcacaggcatcactaatgtcctgtgagggactttcatgttcgggcagggtgcagcgatctgcgtcttcgctctttggttctgcaggactgctttgagtggcaccatctattttagcattatcttttgcaacaccttcatctaattcttcaccaccagccctcgggcctgatgattgaacggtgtcatcctcaaaatctaatgtgtctccatcagctagtacctcctcagctgctgtttgtacatcatcaccttcttggtcaagttttccatccaacttaattttaggattctccggacaatcaacattttcactgctttctgctgcaattttctgttttggattttcagtcacctcgttttgggcttccactgctgactttctgtcagtagactttacctgctcttcttccttaatttcacttaaatctgtgttctgatacgttaactcttttttaacatctttaagggtttctacgggtactggggattttttcttcttgtttttctttttcttgttctttgtcttcttctgcgatgagtccaatgcctctccctgttggtcactcttttcttcatcgggctctttcatatctaagggttcattttgagtgtctactgtacttggacctgtcgcttcctgacagttgccctcagttcctgctggagaaccaggaacttctgtcttgattggtttctcgtcccttaatcctgtttcttcaccctcttcttcgttgtgatccctacctacttctgtactgtgcgctggaacctccttgggctcagctgcttcctggttggtgaattctttctctaaactatgccctgtgcttgtctctaactcttgggggacctctaccatacatttgtcatcatgataaactgtgtcatcactatgccctaaaggacacgaggccactgtgcctgcctgctcttcaacctgagtcactgctgcctctcccacattctctgtgtggttcccaccatctaagtcactccaacagttggatggctcaaggggagttctggtcctgtcatctggtgcacccatgacctcatttgactcaacctgtactgtgttttcagggagagaactgctctcaagaatttggctttgaacctgttcctcataggtagcacctgctaaggttcctaggaatggggcagtgtcttcagaggatttctggtcctcggtattctcaccagcagggaatacctctatgtccacacagtccttcactgtgtcctctgtgtgttgttctttctcagtattgtgcaagatttctcttttccccacattcgccacgatttcatttttcacctccacttcactggctcttcctagggtcccatcccctgtcgacttgagggcatttaactcttcttttgtcatcttggtaggaccttggtatccaacattattgagggtgtcggaagtctctccattggtagctatttctgaatttaggattattccatgtttctttaattcctctttcagcatgactacttcttctctaagatcatcccgttcactccttacggaatcaaagaactctttctgcctctctaatgcccctatctttttgtctttccactctattgtttcctgaagatcagaaatctccctgatagaactcgcctgtttctgctgtagctgtcggatttcctcgagcatttcctctctttgcttcagggcctccttgacttcagcaaactgaaattgcagtatactgtgggcgtgtttttccctttcaaattctttgtttttctcttcgtactgccgcctagattcagccagctgttcttcaagctccagcaacatatcttttagggtatcaacctggtacatgaagtttgtcttttcattgtctagctgagcattggaaaccatagccttcttatatttctcttcaacttctgctagagagtccttcatctctttcaatccctgcatgtatttgccttctacatcctgaatctggtcctttaactcattgagttccttgatttccctgatggatgcctcggtgtcgatggagatggaggtgtctccgctgcctctccgagaggaagtcccacccagagaggccagcgtggctgcagacaggcccggcatgttacgagaccccttctcagtaaaatctttttctggtctctcttctaccctcaggcttccacgactacccactgacatgcgctcgtcttcatcagaagccgatgtgtttcttctggatctacgagagtagcgctcactgtcttcctccttctgctgccgctccagctccttcatgcggatctcgcgagcctccgcgcgggccgcccgttttgcagcgagccgggcttccgccagcttctgcgcttccgggctcaaacagtcgatctcccggctttgagcggccgcggggctggtcatcctgccgggctcggcccgctccacccggcgggaaatgctcggggaccgcgccgggagcccctcgcgggccgggccagggggcgcgcgctctgtc

SEQ ID NO: 13355 - RNA, 3563 nt, Homo sapiens
  source 1..3563: mol_type = other RNA
gctgggattacaggcatgagccaccacgcccggccaaaaacatttaaaaaatgactgtccctgctcaaatactgcagtaggaaatgtaatttgacatatatcacttccagaaaaaaactttaaatctttctataaaatgaatttgatacatcatcagcatgaagtgaagttaaaatctcttacaaagtaaattcaggtatatcaacaatgagatccaaaagtatcggttcaagatcaaagactcatatgaggtaaaggcaaataaagcccctcatgctttcagacatttacttgttatccttaaaatgattattgttctaaggtgcaaatcttatcattcagtgacctatttgctatttggctgtttatctcctttaaataaaataccatacaggttataatgtacattttaaaatcaaatatgaaagtacacatatgtgaacaagacattaatttaaatatcaattatattcataatacagaagtctaagaatgctatttggtcatttcaattagatgctgatatatttggtcaagaaaacccacattcctatcagcctaaggcaaatagtaaatgcctctatttttattaagtggactataaacagtagacattattgtttgatactactggaatgctctcaattagaacgtacactgataacaaatatgtctttctaatctgggtgataacctcaatgattacatggaaatctacaagtaacagtctataacttaaagcagtagagcacctggtaattgtcatacagtgcctctctatgaatttagaacattctacttacattggcagtggagagaaaagaccccttcacactgagacttcctgtgcaccgcgcctgccgcctgcctcagcttaggacatggtacagtcttctttgcttttgcccttctcattccctcctctggtatcttctctgctttctggattgaagtgccctggctctcttcctggtgccgacaagtcatcgttctctaggctattgctgtctaaagctttcctgacggtctgacttggatgttctgacatctcacacctctctgtactttctgcttcacaggcatcactaatgtcctgtgagggactttcatgttcgggcagggtgcagcgatctgcgtcttcgctctttggttctgcaggactgctttgagtggcaccatctattttagcattatcttttgcaacaccttcatctaattcttcaccaccagccctcgggcctgatgattgaacggtgtcatcctcaaaatctaatgtgtctccatcagctagtacctcctcagctgctgtttgtacatcatcaccttcttggtcaagttttccatccaacttaattttaggattctccggacaatcaacattttcactgctttctgctgcaattttctgttttggattttcagtcacctcgttttgggcttccactgctgactttctgtcagtagactttacctgctcttcttccttaatttcacttaaatctgtgttctgatacgttaactcttttttaacatctttaagggtttctacgggtactggggattttttcttcttgtttttctttttcttgttctttgtcttcttctgcgatgagtccaatgcctctccctgttggtcactcttttcttcatcgggctctttcatatctaagggttcattttgagtgtctactgtacttggacctgtcgcttcctgacagttgccctcagttcctgctggagaaccaggaacttctgtcttgattggtttctcgtcccttaatcctgtttcttcaccctcttcttcgttgtgatccctacctacttctgtactgtgcgctggaacctccttgggctcagctgcttcctggttggtgaattctttctctaaactatgccctgtgcttgtctctaactcttgggggacctctaccatacatttgtcatcatgataaactgtgtcatcactatgccctaaaggacacgaggccactgtgcctgcctgctcttcaacctgagtcactgctgcctctcccacattctctgtgtggttcccaccatctaagtcactccaacagttggatggctcaaggggagttctggtcctgtcatctggtgcacccatgacctcatttgactcaacctgtactgtgttttcagggagagaactgctctcaagaatttggctttgaacctgttcctcataggtagcacctgctaaggttcctaggaatggggcagtgtcttcagaggatttctggtcctcggtattctcaccagcagggaatacctctatgtccacacagtccttcactgtgtcctctgtgtgttgttctttctcagtattgtgcaagatttctcttttccccacattcgccacgatttcatttttcacctccacttcactggctcttcctagggtcccatcccctgtcgacttgagggcatttaactcttcttttgtcatcttggtaggaccttggtatccaacattattgagggtgtcggaagtctctccattggtagctatttctgaatttaggattattccatgtttctttaattcctctttcagcatgactacttcttctctaagatcatcccgttcactccttacggaatcaaagaactctttctgcctctctaatgcccctatctttttgtctttccactctattgtttcctgaagatcagaaatctccctgatagaactcgcctgtttctgctgtagctgtcggatttcctcgagcatttcctctctttgcttcagggcctccttgacttcagcaaactgaaattgcagtatactgtgggcgtgtttttccctttcaaattctttgtttttctcttcgtactgccgcctagattcagccagctgttcttcaagctccagcaacatatcttttagggtatcaacctggtacatgaagtttgtcttttcattgtctagctgagcattggaaaccatagccttcttatatttctcttcaacttctgctagagagtccttcatctctttcaatccctgcatgtatttgccttctacatcctgaatctggtcctttaactcattgagttccttgatttccctgatggatgcctcggtgtcgatggagatggaggtgtctccgctgcctctccgagaggaagtcccacccagagaggccagcgtggctgcagacaggcccggcatgttacgagaccccttctcagtaaaatctttttctggtctctcttctaccctcaggcttccacgactacccactgacatgcgctcgtcttcatcagaagccgatgtgtttcttctggatctacgagagtagcgctcactgtcttcctccttctgctgccgctccagctccttcatgcggatctcgcgagcctccgcgcgggccgcccgttttgcagcgagccgggcttccgcctcccgcgcgatctggttgagcgcgtcgtcctccgccgtgagccgctcccggttggggagccgcttgcgccccgatccctgggtgcccatgtccatcgaccgcgtcgcccgcagctgccgcggggcccgttgctccagccgc

SEQ ID NO: 13356 - RNA, 3751 nt, Homo sapiens
  source 1..3751: mol_type = other RNA
gctgggattacaggcatgagccaccacgcccggccaaaaacatttaaaaaatgactgtccctgctcaaatactgcagtaggaaatgtaatttgacatatatcacttccagaaaaaaactttaaatctttctataaaatgaatttgatacatcatcagcatgaagtgaagttaaaatctcttacaaagtaaattcaggtatatcaacaatgagatccaaaagtatcggttcaagatcaaagactcatatgaggtaaaggcaaataaagcccctcatgctttcagacatttacttgttatccttaaaatgattattgttctaaggtgcaaatcttatcattcagtgacctatttgctatttggctgtttatctcctttaaataaaataccatacaggttataatgtacattttaaaatcaaatatgaaagtacacatatgtgaacaagacattaatttaaatatcaattatattcataatacagaagtctaagaatgctatttggtcatttcaattagatgctgatatatttggtcaagaaaacccacattcctatcagcctaaggcaaatagtaaatgcctctatttttattaagtggactataaacagtagacattattgtttgatactactggaatgctctcaattagaacgtacactgataacaaatatgtctttctaatctgggtgataacctcaatgattacatggaaatctacaagtaacagtctataacttaaagcagtagagcacctggtaattgtcatacagtgcctctctatgaatttagaacattctacttacattggcagtggagagaaaagaccccttcacactgagacttcctgtgcaccgcgcctgccgcctgcctcagcttaggacatggtacagtcttctttgcttttgcccttctcattccctcctctggtatcttctctgctttctggattgaagtgccctggctctcttcctggtgccgacaagtcatcgttctctaggctattgctgtctaaagctttcctgacggtctgacttggatgttctgacatctcacacctctctgtactttctgcttcacaggcatcactaatgtcctgtgagggactttcatgttcgggcagggtgcagcgatctgcgtcttcgctctttggttctgcaggactgctttgagtggcaccatctattttagcattatcttttgcaacaccttcatctaattcttcaccaccagccctcgggcctgatgattgaacggtgtcatcctcaaaatctaatgtgtctccatcagctagtacctcctcagctgctgtttgtacatcatcaccttcttggtcaagttttccatccaacttaattttaggattctccggacaatcaacattttcactgctttctgctgcaattttctgttttggattttcagtcacctcgttttgggcttccactgctgactttctgtcagtagactttacctgctcttcttccttaatttcacttaaatctgtgttctgatacgttaactcttttttaacatctttaagggtttctacgggtactggggattttttcttcttgtttttctttttcttgttctttgtcttcttctgcgatgagtccaatgcctctccctgttggtcactcttttcttcatcgggctctttcatatctaagggttcattttgagtgtctactgtacttggacctgtcgcttcctgacagttgccctcagttcctgctggagaaccaggaacttctgtcttgattggtttctcgtcccttaatcctgtttcttcaccctcttcttcgttgtgatccctacctacttctgtactgtgcgctggaacctccttgggctcagctgcttcctggttggtgaattctttctctaaactatgccctgtgcttgtctctaactcttgggggacctctaccatacatttgtcatcatgataaactgtgtcatcactatgccctaaaggacacgaggccactgtgcctgcctgctcttcaacctgagtcactgctgcctctcccacattctctgtgtggttcccaccatctaagtcactccaacagttggatggctcaaggggagttctggtcctgtcatctggtgcacccatgacctcatttgactcaacctgtactgtgttttcagggagagaactgctctcaagaatttggctttgaacctgttcctcataggtagcacctgctaaggttcctaggaatggggcagtgtcttcagaggatttctggtcctcggtattctcaccagcagggaatacctctatgtccacacagtccttcactgtgtcctctgtgtgttgttctttctcagtattgtgcaagatttctcttttccccacattcgccacgatttcatttttcacctccacttcactggctcttcctagggtcccatcccctgtcgacttgagggcatttaactcttcttttgtcatcttggtaggaccttggtatccaacattattgagggtgtcggaagtctctccattggtagctatttctgaatttaggattattccatgtttctttaattcctctttcagcatgactacttcttctctaagatcatcccgttcactccttacggaatcaaagaactctttctgcctctctaatgcccctatctttttgtctttccactctattgtttcctgaagatcagaaatctccctgatagaactcgcctgtttctgctgtagctgtcggatttcctcgagcatttcctctctttgcttcagggcctccttgacttcagcaaactgaaattgcagtatactgtgggcgtgtttttccctttcaaattctttgtttttctcttcgtactgccgcctagattcagccagctgttcttcaagctccagcaacatatcttttagggtatcaacctggtacatgaagtttgtcttttcattgtctagctgagcattggaaaccatagccttcttatatttctcttcaacttctgctagagagtccttcatctctttcaatccctgcatgtatttgccttctacatcctgaatctggtcctttaactcattgagttccttgatttccctgatggatgcctcggtgtcgatggagatggaggtgtctccgctgcctctccgagaggaagtcccacccagagaggccagcgtggctgcagacaggcccggcatgttacgagaccccttctcagtaaaatctttttctggtctctcttctaccctgccagatcttctattcagggactgtgatccatacaattctccatcataaccatttgtccaggcgtaaggacccccatactccaagtcaggctgcgacctcaggcttccacgactacccactgacatgcgctcgtcttcatcagaagccgatgtgtttcttctggatctacgagagtagcgctcactgtcttccatccactgctcgatgtcaccccattttgtatccagcccataatatttcttttggacctgatagatctccttctgctgccgctccagctccttcatgcggatctcgcgagcctccgcgcgggccgcccgttttgcagcgagccgggcttccgcctcccgcgcgatctggttgagcgcgtcgtcctccgccgtgagccgctcccggttggggagccgcttgcgccccgatccctgggtgcccatgtccatcgaccgcgtcgcccgcagctgccgcggggcccgttgctccagccgctcgcgccgccccggcccggcccc

SEQ ID NO: 13357 - RNA, 3712 nt, Homo sapiens
  source 1..3712: mol_type = other RNA
gctgggattacaggcatgagccaccacgcccggccaaaaacatttaaaaaatgactgtccctgctcaaatactgcagtaggaaatgtaatttgacatatatcacttccagaaaaaaactttaaatctttctataaaatgaatttgatacatcatcagcatgaagtgaagttaaaatctcttacaaagtaaattcaggtatatcaacaatgagatccaaaagtatcggttcaagatcaaagactcatatgaggtaaaggcaaataaagcccctcatgctttcagacatttacttgttatccttaaaatgattattgttctaaggtgcaaatcttatcattcagtgacctatttgctatttggctgtttatctcctttaaataaaataccatacaggttataatgtacattttaaaatcaaatatgaaagtacacatatgtgaacaagacattaatttaaatatcaattatattcataatacagaagtctaagaatgctatttggtcatttcaattagatgctgatatatttggtcaagaaaacccacattcctatcagcctaaggcaaatagtaaatgcctctatttttattaagtggactataaacagtagacattattgtttgatactactggaatgctctcaattagaacgtacactgataacaaatatgtctttctaatctgggtgataacctcaatgattacatggaaatctacaagtaacagtctataacttaaagcagtagagcacctggtaattgtcatacagtgcctctctatgaatttagaacattctacttacattggcagtggagagaaaagaccccttcacactgagacttcctgtgcaccgcgcctgccgcctgcctcagcttaggacatggtacagtcttctttgcttttgcccttctcattccctcctctggtatcttctctgctttctggattgaagtgccctggctctcttcctggtgccgacaagtcatcgttctctaggctattgctgtctaaagctttcctgacggtctgacttggatgttctgacatctcacacctctctgtactttctgcttcacaggcatcactaatgtcctgtgagggactttcatgttcgggcagggtgcagcgatctgcgtcttcgctctttggttctgcaggactgctttgagtggcaccatctattttagcattatcttttgcaacaccttcatctaattcttcaccaccagccctcgggcctgatgattgaacggtgtcatcctcaaaatctaatgtgtctccatcagctagtacctcctcagctgctgtttgtacatcatcaccttcttggtcaagttttccatccaacttaattttaggattctccggacaatcaacattttcactgctttctgctgcaattttctgttttggattttcagtcacctcgttttgggcttccactgctgactttctgtcagtagactttacctgctcttcttccttaatttcacttaaatctgtgttctgatacgttaactcttttttaacatctttaagggtttctacgggtactggggattttttcttcttgtttttctttttcttgttctttgtcttcttctgcgatgagtccaatgcctctccctgttggtcactcttttcttcatcgggctctttcatatctaagggttcattttgagtgtctactgtacttggacctgtcgcttcctgacagttgccctcagttcctgctggagaaccaggaacttctgtcttgattggtttctcgtcccttaatcctgtttcttcaccctcttcttcgttgtgatccctacctacttctgtactgtgcgctggaacctccttgggctcagctgcttcctggttggtgaattctttctctaaactatgccctgtgcttgtctctaactcttgggggacctctaccatacatttgtcatcatgataaactgtgtcatcactatgccctaaaggacacgaggccactgtgcctgcctgctcttcaacctgagtcactgctgcctctcccacattctctgtgtggttcccaccatctaagtcactccaacagttggatggctcaaggggagttctggtcctgtcatctggtgcacccatgacctcatttgactcaacctgtactgtgttttcagggagagaactgctctcaagaatttggctttgaacctgttcctcataggtagcacctgctaaggttcctaggaatggggcagtgtcttcagaggatttctggtcctcggtattctcaccagcagggaatacctctatgtccacacagtccttcactgtgtcctctgtgtgttgttctttctcagtattgtgcaagatttctcttttccccacattcgccacgatttcatttttcacctccacttcactggctcttcctagggtcccatcccctgtcgacttgagggcatttaactcttcttttgtcatcttggtaggaccttggtatccaacattattgagggtgtcggaagtctctccattggtagctatttctgaatttaggattattccatgtttctttaattcctctttcagcatgactacttcttctctaagatcatcccgttcactccttacggaatcaaagaactctttctgcctctctaatgcccctatctttttgtctttccactctattgtttcctgaagatcagaaatctccctgatagaactcgcctgtttctgctgtagctgtcggatttcctcgagcatttcctctctttgcttcagggcctccttgacttcagcaaactgaaattgcagtatactgtgggcgtgtttttccctttcaaattctttgtttttctcttcgtactgccgcctagattcagccagctgttcttcaagctccagcaacatatcttttagggtatcaacctggtacatgaagtttgtcttttcattgtctagctgagcattggaaaccatagccttcttatatttctcttcaacttctgctagagagtccttcatctctttcaatccctgcatgtatttgccttctacatcctgaatctggtcctttaactcattgagttccttgatttccctgatggatgcctcggtgtcgatggagatggaggtgtctccgctgcctctccgagaggaagtcccacccagagaggccagcgtggctgcagacaggcccggcatgttacgagaccccttctcagtaaaatctttttctggtctctcttctaccctgccagatcttctattcagggactgtgatccatacaattctccatcataaccatttgtcctcaggcttccacgactacccactgacatgcgctcgtcttcatcagaagccgatgtgtttcttctggatctacgagagtagcgctcactgtcttccatccactgctcgatgtcaccccattttgtatccagcccataatatttcttttggacctgatagatctccttctgctgccgctccagctccttcatgcggatctcgcgagcctccgcgcgggccgcccgttttgcagcgagccgggcttccgcctcccgcgcgatctggttgagcgcgtcgtcctccgccgtgagccgctcccggttggggagccgcttgcgccccgatccctgggtgcccatgtccatcgaccgcgtcgcccgcagctgccgcggggcccgttgctccagccgctcgcgccgccccggcccggcccc

SEQ ID NO: 13358 - RNA, 3641 nt, Homo sapiens
  source 1..3641: mol_type = other RNA
gctgggattacaggcatgagccaccacgcccggccaaaaacatttaaaaaatgactgtccctgctcaaatactgcagtaggaaatgtaatttgacatatatcacttccagaaaaaaactttaaatctttctataaaatgaatttgatacatcatcagcatgaagtgaagttaaaatctcttacaaagtaaattcaggtatatcaacaatgagatccaaaagtatcggttcaagatcaaagactcatatgaggtaaaggcaaataaagcccctcatgctttcagacatttacttgttatccttaaaatgattattgttctaaggtgcaaatcttatcattcagtgacctatttgctatttggctgtttatctcctttaaataaaataccatacaggttataatgtacattttaaaatcaaatatgaaagtacacatatgtgaacaagacattaatttaaatatcaattatattcataatacagaagtctaagaatgctatttggtcatttcaattagatgctgatatatttggtcaagaaaacccacattcctatcagcctaaggcaaatagtaaatgcctctatttttattaagtggactataaacagtagacattattgtttgatactactggaatgctctcaattagaacgtacactgataacaaatatgtctttctaatctgggtgataacctcaatgattacatggaaatctacaagtaacagtctataacttaaagcagtagagcacctggtaattgtcatacagtgcctctctatgaatttagaacattctacttacattggcagtggagagaaaagaccccttcacactgagacttcctgtgcaccgcgcctgccgcctgcctcagcttaggacatggtacagtcttctttgcttttgcccttctcattccctcctctggtatcttctctgctttctggattgaagtgccctggctctcttcctggtgccgacaagtcatcgttctctaggctattgctgtctaaagctttcctgacggtctgacttggatgttctgacatctcacacctctctgtactttctgcttcacaggcatcactaatgtcctgtgagggactttcatgttcgggcagggtgcagcgatctgcgtcttcgctctttggttctgcaggactgctttgagtggcaccatctattttagcattatcttttgcaacaccttcatctaattcttcaccaccagccctcgggcctgatgattgaacggtgtcatcctcaaaatctaatgtgtctccatcagctagtacctcctcagctgctgtttgtacatcatcaccttcttggtcaagttttccatccaacttaattttaggattctccggacaatcaacattttcactgctttctgctgcaattttctgttttggattttcagtcacctcgttttgggcttccactgctgactttctgtcagtagactttacctgctcttcttccttaatttcacttaaatctgtgttctgatacgttaactcttttttaacatctttaagggtttctacgggtactggggattttttcttcttgtttttctttttcttgttctttgtcttcttctgcgatgagtccaatgcctctccctgttggtcactcttttcttcatcgggctctttcatatctaagggttcattttgagtgtctactgtacttggacctgtcgcttcctgacagttgccctcagttcctgctggagaaccaggaacttctgtcttgattggtttctcgtcccttaatcctgtttcttcaccctcttcttcgttgtgatccctacctacttctgtactgtgcgctggaacctccttgggctcagctgcttcctggttggtgaattctttctctaaactatgccctgtgcttgtctctaactcttgggggacctctaccatacatttgtcatcatgataaactgtgtcatcactatgccctaaaggacacgaggccactgtgcctgcctgctcttcaacctgagtcactgctgcctctcccacattctctgtgtggttcccaccatctaagtcactccaacagttggatggctcaaggggagttctggtcctgtcatctggtgcacccatgacctcatttgactcaacctgtactgtgttttcagggagagaactgctctcaagaatttggctttgaacctgttcctcataggtagcacctgctaaggttcctaggaatggggcagtgtcttcagaggatttctggtcctcggtattctcaccagcagggaatacctctatgtccacacagtccttcactgtgtcctctgtgtgttgttctttctcagtattgtgcaagatttctcttttccccacattcgccacgatttcatttttcacctccacttcactggctcttcctagggtcccatcccctgtcgacttgagggcatttaactcttcttttgtcatcttggtaggaccttggtatccaacattattgagggtgtcggaagtctctccattggtagctatttctgaatttaggattattccatgtttctttaattcctctttcagcatgactacttcttctctaagatcatcccgttcactccttacggaatcaaagaactctttctgcctctctaatgcccctatctttttgtctttccactctattgtttcctgaagatcagaaatctccctgatagaactcgcctgtttctgctgtagctgtcggatttcctcgagcatttcctctctttgcttcagggcctccttgacttcagcaaactgaaattgcagtatactgtgggcgtgtttttccctttcaaattctttgtttttctcttcgtactgccgcctagattcagccagctgttcttcaagctccagcaacatatcttttagggtatcaacctggtacatgaagtttgtcttttcattgtctagctgagcattggaaaccatagccttcttatatttctcttcaacttctgctagagagtccttcatctctttcaatccctgcatgtatttgccttctacatcctgaatctggtcctttaactcattgagttccttgatttccctgatggatgcctcggtgtcgatggagatggaggtgtctccgctgcctctccgagaggaagtcccacccagagaggccagcgtggctgcagacaggcccggcatgttacgagaccccttctcagtaaaatctttttctggtctctcttctaccctgccagatcttctattcagggactgtgatccatacaattctccatcataaccatttgtcctcaggcttccacgactacccactgacatgcgctcgtcttcatcagaagccgatgtgtttcttctggatctacgagagtagcgctcactgtcttcctccttctgctgccgctccagctccttcatgcggatctcgcgagcctccgcgcgggccgcccgttttgcagcgagccgggcttccgccagcttctgcgcttccgggctcaaacagtcgatctcccggctttgagcggccgcggggctggtcatcctgccgggctcggcccgctccacccggcgggaaatgctcggggaccgcgccgggagcccctcgcgggccgggccagggggcgcgcgctctgtc

SEQ ID NO: 13359 - RNA, 3686 nt, Homo sapiens
  source 1..3686: mol_type = other RNA
gctgggattacaggcatgagccaccacgcccggccaaaaacatttaaaaaatgactgtccctgctcaaatactgcagtaggaaatgtaatttgacatatatcacttccagaaaaaaactttaaatctttctataaaatgaatttgatacatcatcagcatgaagtgaagttaaaatctcttacaaagtaaattcaggtatatcaacaatgagatccaaaagtatcggttcaagatcaaagactcatatgaggtaaaggcaaataaagcccctcatgctttcagacatttacttgttatccttaaaatgattattgttctaaggtgcaaatcttatcattcagtgacctatttgctatttggctgtttatctcctttaaataaaataccatacaggttataatgtacattttaaaatcaaatatgaaagtacacatatgtgaacaagacattaatttaaatatcaattatattcataatacagaagtctaagaatgctatttggtcatttcaattagatgctgatatatttggtcaagaaaacccacattcctatcagcctaaggcaaatagtaaatgcctctatttttattaagtggactataaacagtagacattattgtttgatactactggaatgctctcaattagaacgtacactgataacaaatatgtctttctaatctgggtgataacctcaatgattacatggaaatctacaagtaacagtctataacttaaagcagtagagcacctggtaattgtcatacagtgcctctctatgaatttagaacattctacttacattggcagtggagagaaaagaccccttcacactgagacttcctgtgcaccgcgcctgccgcctgcctcagcttaggacatggtacagtcttctttgcttttgcccttctcattccctcctctggtatcttctctgctttctggattgaagtgccctggctctcttcctggtgccgacaagtcatcgttctctaggctattgctgtctaaagctttcctgacggtctgacttggatgttctgacatctcacacctctctgtactttctgcttcacaggcatcactaatgtcctgtgagggactttcatgttcgggcagggtgcagcgatctgcgtcttcgctctttggttctgcaggactgctttgagtggcaccatctattttagcattatcttttgcaacaccttcatctaattcttcaccaccagccctcgggcctgatgattgaacggtgtcatcctcaaaatctaatgtgtctccatcagctagtacctcctcagctgctgtttgtacatcatcaccttcttggtcaagttttccatccaacttaattttaggattctccggacaatcaacattttcactgctttctgctgcaattttctgttttggattttcagtcacctcgttttgggcttccactgctgactttctgtcagtagactttacctgctcttcttccttaatttcacttaaatctgtgttctgatacgttaactcttttttaacatctttaagggtttctacgggtactggggattttttcttcttgtttttctttttcttgttctttgtcttcttctgcgatgagtccaatgcctctccctgttggtcactcttttcttcatcgggctctttcatatctaagggttcattttgagtgtctactgtacttggacctgtcgcttcctgacagttgccctcagttcctgctggagaaccaggaacttctgtcttgattggtttctcgtcccttaatcctgtttcttcaccctcttcttcgttgtgatccctacctacttctgtactgtgcgctggaacctccttgggctcagctgcttcctggttggtgaattctttctctaaactatgccctgtgcttgtctctaactcttgggggacctctaccatacatttgtcatcatgataaactgtgtcatcactatgccctaaaggacacgaggccactgtgcctgcctgctcttcaacctgagtcactgctgcctctcccacattctctgtgtggttcccaccatctaagtcactccaacagttggatggctcaaggggagttctggtcctgtcatctggtgcacccatgacctcatttgactcaacctgtactgtgttttcagggagagaactgctctcaagaatttggctttgaacctgttcctcataggtagcacctgctaaggttcctaggaatggggcagtgtcttcagaggatttctggtcctcggtattctcaccagcagggaatacctctatgtccacacagtccttcactgtgtcctctgtgtgttgttctttctcagtattgtgcaagatttctcttttccccacattcgccacgatttcatttttcacctccacttcactggctcttcctagggtcccatcccctgtcgacttgagggcatttaactcttcttttgtcatcttggtaggaccttggtatccaacattattgagggtgtcggaagtctctccattggtagctatttctgaatttaggattattccatgtttctttaattcctctttcagcatgactacttcttctctaagatcatcccgttcactccttacggaatcaaagaactctttctgcctctctaatgcccctatctttttgtctttccactctattgtttcctgaagatcagaaatctccctgatagaactcgcctgtttctgctgtagctgtcggatttcctcgagcatttcctctctttgcttcagggcctccttgacttcagcaaactgaaattgcagtatactgtgggcgtgtttttccctttcaaattctttgtttttctcttcgtactgccgcctagattcagccagctgttcttcaagctccagcaacatatcttttagggtatcaacctggtacatgaagtttgtcttttcattgtctagctgagcattggaaaccatagccttcttatatttctcttcaacttctgctagagagtccttcatctctttcaatccctgcatgtatttgccttctacatcctgaatctggtcctttaactcattgagttccttgatttccctgatggatgcctcggtgtcgatggagatggaggtgtctccgctgcctctccgagaggaagtcccacccagagaggccagcgtggctgcagacaggcccggcatgttacgagaccccttctcagtaaaatctttttctggtctctcttctacctccttctgctgccgctccagctccttcatgcggatctcgcgagcctccgcgcgggccgcccgttttgcagcgagccgggcttccgccagcttctgcgcttccgggctcaaacagtcgatctcccggctttgagcggccgcggggctggtcatcctgccgggctcggcccgctccacccggcgggaaatgctcggggaccgcgccgggagcccctcgcgggccgggccagggggcgcgcgctctgtccgcggagacggagccactcgccgctaagtgaacgctcgcgcttccggggccaggagccagcccgccggggagcggctcgcggcgctgggctcgggcgcggccgacaggggcggggcgcaggtggccgcgggctgagtcgggctcggggtggaagggcgccggggaagcgggactcgggcgcctccgcccgtcccacggccc

SEQ ID NO: 13360 - RNA, 3467 nt, Homo sapiens
  source 1..3467: mol_type = other RNA
gctgggattacaggcatgagccaccacgcccggccaaaaacatttaaaaaatgactgtccctgctcaaatactgcagtaggaaatgtaatttgacatatatcacttccagaaaaaaactttaaatctttctataaaatgaatttgatacatcatcagcatgaagtgaagttaaaatctcttacaaagtaaattcaggtatatcaacaatgagatccaaaagtatcggttcaagatcaaagactcatatgaggtaaaggcaaataaagcccctcatgctttcagacatttacttgttatccttaaaatgattattgttctaaggtgcaaatcttatcattcagtgacctatttgctatttggctgtttatctcctttaaataaaataccatacaggttataatgtacattttaaaatcaaatatgaaagtacacatatgtgaacaagacattaatttaaatatcaattatattcataatacagaagtctaagaatgctatttggtcatttcaattagatgctgatatatttggtcaagaaaacccacattcctatcagcctaaggcaaatagtaaatgcctctatttttattaagtggactataaacagtagacattattgtttgatactactggaatgctctcaattagaacgtacactgataacaaatatgtctttctaatctgggtgataacctcaatgattacatggaaatctacaagtaacagtctataacttaaagcagtagagcacctggtaattgtcatacagtgcctctctatgaatttagaacattctacttacattggcagtggagagaaaagaccccttcacactgagacttcctgtgcaccgcgcctgccgcctgcctcagcttaggacatggtacagtcttctttgcttttgcccttctcattccctcctctggtatcttctctgctttctggattgaagtgccctggctctcttcctggtgccgacaagtcatcgttctctaggctattgctgtctaaagctttcctgacggtctgacttggatgttctgacatctcacacctctctgtactttctgcttcacaggcatcactaatgtcctgtgagggactttcatgttcgggcagggtgcagcgatctgcgtcttcgctctttggttctgcaggactgctttgagtggcaccatctattttagcattatcttttgcaacaccttcatctaattcttcaccaccagccctcgggcctgatgattgaacggtgtcatcctcaaaatctaatgtgtctccatcagctagtacctcctcagctgctgtttgtacatcatcaccttcttggtcaagttttccatccaacttaattttaggattctccggacaatcaacattttcactgctttctgctgcaattttctgttttggattttcagtcacctcgttttgggcttccactgctgactttctgtcagtagactttacctgctcttcttccttaatttcacttaaatctgtgttctgatacgttaactcttttttaacatctttaagggtttctacgggtactggggattttttcttcttgtttttctttttcttgttctttgtcttcttctgcgatgagtccaatgcctctccctgttggtcactcttttcttcatcgggctctttcatatctaagggttcattttgagtgtctactgtacttggacctgtcgcttcctgacagttgccctcagttcctgctggagaaccaggaacttctgtcttgattggtttctcgtcccttaatcctgtttcttcaccctcttcttcgttgtgatccctacctacttctgtactgtgcgctggaacctccttgggctcagctgcttcctggttggtgaattctttctctaaactatgccctgtgcttgtctctaactcttgggggacctctaccatacatttgtcatcatgataaactgtgtcatcactatgccctaaaggacacgaggccactgtgcctgcctgctcttcaacctgagtcactgctgcctctcccacattctctgtgtggttcccaccatctaagtcactccaacagttggatggctcaaggggagttctggtcctgtcatctggtgcacccatgacctcatttgactcaacctgtactgtgttttcagggagagaactgctctcaagaatttggctttgaacctgttcctcataggtagcacctgctaaggttcctaggaatggggcagtgtcttcagaggatttctggtcctcggtattctcaccagcagggaatacctctatgtccacacagtccttcactgtgtcctctgtgtgttgttctttctcagtattgtgcaagatttctcttttccccacattcgccacgatttcatttttcacctccacttcactggctcttcctagggtcccatcccctgtcgacttgagggcatttaactcttcttttgtcatcttggtaggaccttggtatccaacattattgagggtgtcggaagtctctccattggtagctatttctgaatttaggattattccatgtttctttaattcctctttcagcatgactacttcttctctaagatcatcccgttcactccttacggaatcaaagaactctttctgcctctctaatgcccctatctttttgtctttccactctattgtttcctgaagatcagaaatctccctgatagaactcgcctgtttctgctgtagctgtcggatttcctcgagcatttcctctctttgcttcagggcctccttgacttcagcaaactgaaattgcagtatactgtgggcgtgtttttccctttcaaattctttgtttttctcttcgtactgccgcctagattcagccagctgttcttcaagctccagcaacatatcttttagggtatcaacctggtacatgaagtttgtcttttcattgtctagctgagcattggaaaccatagccttcttatatttctcttcaacttctgctagagagtccttcatctctttcaatccctgcatgtatttgccttctacatcctgaatctggtcctttaactcattgagttccttgatttccctgatggatgcctcggtgtcgatggagatggaggtgtctccgctgcctctccgagaggaagtcccacccagagaggccagcgtggctgcagacaggcccggcatgttacgagaccccttctcagtaaaatctttttctggtctctcttctacctccttctgctgccgctccagctccttcatgcggatctcgcgagcctccgcgcgggccgcccgttttgcagcgagccgggcttccgcctcccgcgcgatctggttgagcgcgtcgtcctccgccgtgagccgctcccggttggggagccgcttgcgccccgatccctgggtgcccatgtccatcgaccgcgtcgcccgcagctgccgcggggcccgttgctccagccgc

SEQ ID NO: 13361 - RNA, 3931 nt, Homo sapiens
  source 1..3931: mol_type = other RNA
gctgggattacaggcatgagccaccacgcccggccaaaaacatttaaaaaatgactgtccctgctcaaatactgcagtaggaaatgtaatttgacatatatcacttccagaaaaaaactttaaatctttctataaaatgaatttgatacatcatcagcatgaagtgaagttaaaatctcttacaaagtaaattcaggtatatcaacaatgagatccaaaagtatcggttcaagatcaaagactcatatgaggtaaaggcaaataaagcccctcatgctttcagacatttacttgttatccttaaaatgattattgttctaaggtgcaaatcttatcattcagtgacctatttgctatttggctgtttatctcctttaaataaaataccatacaggttataatgtacattttaaaatcaaatatgaaagtacacatatgtgaacaagacattaatttaaatatcaattatattcataatacagaagtctaagaatgctatttggtcatttcaattagatgctgatatatttggtcaagaaaacccacattcctatcagcctaaggcaaatagtaaatgcctctatttttattaagtggactataaacagtagacattattgtttgatactactggaatgctctcaattagaacgtacactgataacaaatatgtctttctaatctgggtgataacctcaatgattacatggaaatctacaagtaacagtctataacttaaagcagtagagcacctggtaattgtcatacagtgcctctctatgaatttagaacattctacttacattggcagtggagagaaaagaccccttcacactgagacttcctgtgcaccgcgcctgccgcctgcctcagcttaggacatggtacagtcttctttgcttttgcccttctcattccctcctctggtatcttctctgctttctggattgaagtgccctggctctcttcctggtgccgacaagtcatcgttctctaggctattgctgtctaaagctttcctgacggtctgacttggatgttctgacatctcacacctctctgtactttctgcttcacaggcatcactaatgtcctgtgagggactttcatgttcgggcagggtgcagcgatctgcgtcttcgctctttggttctgcaggactgctttgagtggcaccatctattttagcattatcttttgcaacaccttcatctaattcttcaccaccagccctcgggcctgatgattgaacggtgtcatcctcaaaatctaatgtgtctccatcagctagtacctcctcagctgctgtttgtacatcatcaccttcttggtcaagttttccatccaacttaattttaggattctccggacaatcaacattttcactgctttctgctgcaattttctgttttggattttcagtcacctcgttttgggcttccactgctgactttctgtcagtagactttacctgctcttcttccttaatttcacttaaatctgtgttctgatacgttaactcttttttaacatctttaagggtttctacgggtactggggattttttcttcttgtttttctttttcttgttctttgtcttcttctgcgatgagtccaatgcctctccctgttggtcactcttttcttcatcgggctctttcatatctaagggttcattttgagtgtctactgtacttggacctgtcgcttcctgacagttgccctcagttcctgctggagaaccaggaacttctgtcttgattggtttctcgtcccttaatcctgtttcttcaccctcttcttcgttgtgatccctacctacttctgtactgtgcgctggaacctccttgggctcagctgcttcctggttggtgaattctttctctaaactatgccctgtgcttgtctctaactcttgggggacctctaccatacatttgtcatcatgataaactgtgtcatcactatgccctaaaggacacgaggccactgtgcctgcctgctcttcaacctgagtcactgctgcctctcccacattctctgtgtggttcccaccatctaagtcactccaacagttggatggctcaaggggagttctggtcctgtcatctggtgcacccatgacctcatttgactcaacctgtactgtgttttcagggagagaactgctctcaagaatttggctttgaacctgttcctcataggtagcacctgctaaggttcctaggaatggggcagtgtcttcagaggatttctggtcctcggtattctcaccagcagggaatacctctatgtccacacagtccttcactgtgtcctctgtgtgttgttctttctcagtattgtgcaagatttctcttttccccacattcgccacgatttcatttttcacctccacttcactggctcttcctagggtcccatcccctgtcgacttgagggcatttaactcttcttttgtcatcttggtaggaccttggtatccaacattattgagggtgtcggaagtctctccattggtagctatttctgaatttaggattattccatgtttctttaattcctctttcagcatgactacttcttctctaagatcatcccgttcactccttacggaatcaaagaactctttctgcctctctaatgcccctatctttttgtctttccactctattgtttcctgaagatcagaaatctccctgatagaactcgcctgtttctgctgtagctgtcggatttcctcgagcatttcctctctttgcttcagggcctccttgacttcagcaaactgaaattgcagtatactgtgggcgtgtttttccctttcaaattctttgtttttctcttcgtactgccgcctagattcagccagctgttcttcaagctccagcaacatatcttttagggtatcaacctggtacatgaagtttgtcttttcattgtctagctgagcattggaaaccatagccttcttatatttctcttcaacttctgctagagagtccttgatttccctgatggatgcctcggtgtcgatggagatggaggtgtctccgctgcctctccgagaggaagtcccacccagagaggccagcgtggctgcagacaggcccggcatgttacgagaccccttctcagtaaaatctttttctggtctctcttctaccacagggctggcccgggccgagctggccctggaggaggcgcgggagctggagttgaggtggccgctgtactccgagggagcacgggagccggaggtgctgccccgtcgggtcccaccgaagctgccttcatccaacacagacgcccggtaactccccgaaggccgggcagcgctgtacagacaggagggcaacttctcctccctggatgatgacaaagtagagaatctgctgtcaccgctgtagctggaattcctgccagatcttctattcagggactgtgatccatacaattctccatcataaccatttgtccaggcgtaaggacccccatactccaagtcaggctgcgacctcaggcttccacgactacccactgacatgcgctcgtcttcatcagaagccgatgtgtttcttctggatctacgagagtagcgctcactgtcttccatccactgctcgatgtcaccccattttgtatccagcccataatatttcttttggacctgatagatctccttctgctgccgctccagctccttcatgcggatctcgcgagcctccgcgcgggccgcccgttttgcagcgagccgggcttccgcctcccgcgcgatctggttgagcgcgtcgtcctccgccgtgagccgctcccggttggggagccgcttgcgccccgatccctgggtgcccatgtccatcgaccgcgtcgcccgcagctgccgcggggcccgttgctccagccgctcgcgccgccccggcccggcccc

SEQ ID NO: 13362 - RNA, 3760 nt, Homo sapiens
  source 1..3760: mol_type = other RNA
gctgggattacaggcatgagccaccacgcccggccaaaaacatttaaaaaatgactgtccctgctcaaatactgcagtaggaaatgtaatttgacatatatcacttccagaaaaaaactttaaatctttctataaaatgaatttgatacatcatcagcatgaagtgaagttaaaatctcttacaaagtaaattcaggtatatcaacaatgagatccaaaagtatcggttcaagatcaaagactcatatgaggtaaaggcaaataaagcccctcatgctttcagacatttacttgttatccttaaaatgattattgttctaaggtgcaaatcttatcattcagtgacctatttgctatttggctgtttatctcctttaaataaaataccatacaggttataatgtacattttaaaatcaaatatgaaagtacacatatgtgaacaagacattaatttaaatatcaattatattcataatacagaagtctaagaatgctatttggtcatttcaattagatgctgatatatttggtcaagaaaacccacattcctatcagcctaaggcaaatagtaaatgcctctatttttattaagtggactataaacagtagacattattgtttgatactactggaatgctctcaattagaacgtacactgataacaaatatgtctttctaatctgggtgataacctcaatgattacatggaaatctacaagtaacagtctataacttaaagcagtagagcacctggtaattgtcatacagtgcctctctatgaatttagaacattctacttacattggcagtggagagaaaagaccccttcacactgagacttcctgtgcaccgcgcctgccgcctgcctcagcttaggacatggtacagtcttctttgcttttgcccttctcattccctcctctggtatcttctctgctttctggattgaagtgccctggctctcttcctggtgccgacaagtcatcgttctctaggctattgctgtctaaagctttcctgacggtctgacttggatgttctgacatctcacacctctctgtactttctgcttcacaggcatcactaatgtcctgtgagggactttcatgttcgggcagggtgcagcgatctgcgtcttcgctctttggttctgcaggactgctttgagtggcaccatctattttagcattatcttttgcaacaccttcatctaattcttcaccaccagccctcgggcctgatgattgaacggtgtcatcctcaaaatctaatgtgtctccatcagctagtacctcctcagctgctgtttgtacatcatcaccttcttggtcaagttttccatccaacttaattttaggattctccggacaatcaacattttcactgctttctgctgcaattttctgttttggattttcagtcacctcgttttgggcttccactgctgactttctgtcagtagactttacctgctcttcttccttaatttcacttaaatctgtgttctgatacgttaactcttttttaacatctttaagggtttctacgggtactggggattttttcttcttgtttttctttttcttgttctttgtcttcttctgcgatgagtccaatgcctctccctgttggtcactcttttcttcatcgggctctttcatatctaagggttcattttgagtgtctactgtacttggacctgtcgcttcctgacagttgccctcagttcctgctggagaaccaggaacttctgtcttgattggtttctcgtcccttaatcctgtttcttcaccctcttcttcgttgtgatccctacctacttctgtactgtgcgctggaacctccttgggctcagctgcttcctggttggtgaattctttctctaaactatgccctgtgcttgtctctaactcttgggggacctctaccatacatttgtcatcatgataaactgtgtcatcactatgccctaaaggacacgaggccactgtgcctgcctgctcttcaacctgagtcactgctgcctctcccacattctctgtgtggttcccaccatctaagtcactccaacagttggatggctcaaggggagttctggtcctgtcatctggtgcacccatgacctcatttgactcaacctgtactgtgttttcagggagagaactgctctcaagaatttggctttgaacctgttcctcataggtagcacctgctaaggttcctaggaatggggcagtgtcttcagaggatttctggtcctcggtattctcaccagcagggaatacctctatgtccacacagtccttcactgtgtcctctgtgtgttgttctttctcagtattgtgcaagatttctcttttccccacattcgccacgatttcatttttcacctccacttcactggctcttcctagggtcccatcccctgtcgacttgagggcatttaactcttcttttgtcatcttggtaggaccttggtatccaacattattgagggtgtcggaagtctctccattggtagctatttctgaatttaggattattccatgtttctttaattcctctttcagcatgactacttcttctctaagatcatcccgttcactccttacggaatcaaagaactctttctgcctctctaatgcccctatctttttgtctttccactctattgtttcctgaagatcagaaatctccctgatagaactcgcctgtttctgctgtagctgtcggatttcctcgagcatttcctctctttgcttcagggcctccttgacttcagcaaactgaaattgcagtatactgtgggcgtgtttttccctttcaaattctttgtttttctcttcgtactgccgcctagattcagccagctgttcttcaagctccagcaacatatcttttagggtatcaacctggtacatgaagtttgtcttttcattgtctagctgagcattggaaaccatagccttcttatatttctcttcaacttctgctagagagtccttgatttccctgatggatgcctcggtgtcgatggagatggaggtgtctccgctgcctctccgagaggaagtcccacccagagaggccagcgtggctgcagacaggcccggcatgttacgagaccccttctcagtaaaatctttttctggtctctcttctaccctcaggcttccacgactacccactgacatgcgctcgtcttcatcagaagccgatgtgtttcttctggatctacgagagtagcgctcactgtcttccatccactgctcgatgtcaccccattttgtatccagcccataatatttcttttggacctgatagatctccttctgctgccgctccagctccttcatgcggatctcgcgagcctccgcgcgggccgcccgttttgcagcgagccgggcttccgccagcttctgcgcttccgggctcaaacagtcgatctcccggctttgagcggccgcggggctggtcatcctgccgggctcggcccgctccacccggcgggaaatgctcggggaccgcgccgggagcccctcgcgggccgggccagggggcgcgcgctctgtccgcggagacggagccactcgccgctaagtgaacgctcgcgcttccggggccaggagccagcccgccggggagcggctcgcggcgctgggctcgggcgcggccgacaggggcggggcgcaggtggccgcgggctgagtcgggctcggggtggaagggcgccggggaagcgggactcgggcgcctcc

SEQ ID NO: 13363 - RNA, 3580 nt, Homo sapiens
  source 1..3580: mol_type = other RNA
gctgggattacaggcatgagccaccacgcccggccaaaaacatttaaaaaatgactgtccctgctcaaatactgcagtaggaaatgtaatttgacatatatcacttccagaaaaaaactttaaatctttctataaaatgaatttgatacatcatcagcatgaagtgaagttaaaatctcttacaaagtaaattcaggtatatcaacaatgagatccaaaagtatcggttcaagatcaaagactcatatgaggtaaaggcaaataaagcccctcatgctttcagacatttacttgttatccttaaaatgattattgttctaaggtgcaaatcttatcattcagtgacctatttgctatttggctgtttatctcctttaaataaaataccatacaggttataatgtacattttaaaatcaaatatgaaagtacacatatgtgaacaagacattaatttaaatatcaattatattcataatacagaagtctaagaatgctatttggtcatttcaattagatgctgatatatttggtcaagaaaacccacattcctatcagcctaaggcaaatagtaaatgcctctatttttattaagtggactataaacagtagacattattgtttgatactactggaatgctctcaattagaacgtacactgataacaaatatgtctttctaatctgggtgataacctcaatgattacatggaaatctacaagtaacagtctataacttaaagcagtagagcacctggtaattgtcatacagtgcctctctatgaatttagaacattctacttacattggcagtggagagaaaagaccccttcacactgagacttcctgtgcaccgcgcctgccgcctgcctcagcttaggacatggtacagtcttctttgcttttgcccttctcattccctcctctggtatcttctctgctttctggattgaagtgccctggctctcttcctggtgccgacaagtcatcgttctctaggctattgctgtctaaagctttcctgacggtctgacttggatgttctgacatctcacacctctctgtactttctgcttcacaggcatcactaatgtcctgtgagggactttcatgttcgggcagggtgcagcgatctgcgtcttcgctctttggttctgcaggactgctttgagtggcaccatctattttagcattatcttttgcaacaccttcatctaattcttcaccaccagccctcgggcctgatgattgaacggtgtcatcctcaaaatctaatgtgtctccatcagctagtacctcctcagctgctgtttgtacatcatcaccttcttggtcaagttttccatccaacttaattttaggattctccggacaatcaacattttcactgctttctgctgcaattttctgttttggattttcagtcacctcgttttgggcttccactgctgactttctgtcagtagactttacctgctcttcttccttaatttcacttaaatctgtgttctgatacgttaactcttttttaacatctttaagggtttctacgggtactggggattttttcttcttgtttttctttttcttgttctttgtcttcttctgcgatgagtccaatgcctctccctgttggtcactcttttcttcatcgggctctttcatatctaagggttcattttgagtgtctactgtacttggacctgtcgcttcctgacagttgccctcagttcctgctggagaaccaggaacttctgtcttgattggtttctcgtcccttaatcctgtttcttcaccctcttcttcgttgtgatccctacctacttctgtactgtgcgctggaacctccttgggctcagctgcttcctggttggtgaattctttctctaaactatgccctgtgcttgtctctaactcttgggggacctctaccatacatttgtcatcatgataaactgtgtcatcactatgccctaaaggacacgaggccactgtgcctgcctgctcttcaacctgagtcactgctgcctctcccacattctctgtgtggttcccaccatctaagtcactccaacagttggatggctcaaggggagttctggtcctgtcatctggtgcacccatgacctcatttgactcaacctgtactgtgttttcagggagagaactgctctcaagaatttggctttgaacctgttcctcataggtagcacctgctaaggttcctaggaatggggcagtgtcttcagaggatttctggtcctcggtattctcaccagcagggaatacctctatgtccacacagtccttcactgtgtcctctgtgtgttgttctttctcagtattgtgcaagatttctcttttccccacattcgccacgatttcatttttcacctccacttcactggctcttcctagggtcccatcccctgtcgacttgagggcatttaactcttcttttgtcatcttggtaggaccttggtatccaacattattgagggtgtcggaagtctctccattggtagctatttctgaatttaggattattccatgtttctttaattcctctttcagcatgactacttcttctctaagatcatcccgttcactccttacggaatcaaagaactctttctgcctctctaatgcccctatctttttgtctttccactctattgtttcctgaagatcagaaatctccctgatagaactcgcctgtttctgctgtagctgtcggatttcctcgagcatttcctctctttgcttcagggcctccttgacttcagcaaactgaaattgcagtatactgtgggcgtgtttttccctttcaaattctttgtttttctcttcgtactgccgcctagattcagccagctgttcttcaagctccagcaacatatcttttagggtatcaacctggtacatgaagtttgtcttttcattgtctagctgagcattggaaaccatagccttcttatatttctcttcaacttctgctagagagtccttgatttccctgatggatgcctcggtgtcgatggagatggaggtgtctccgctgcctctccgagaggaagtcccacccagagaggccagcgtggctgcagacaggcccggcatgttacgagaccccttctcagtaaaatctttttctggtctctcttctaccctcaggcttccacgactacccactgacatgcgctcgtcttcatcagaagccgatgtgtttcttctggatctacgagagtagcgctcactgtcttccatccactgctcgatgtcaccccattttgtatccagcccataatatttcttttggacctgatagatctccttctgctgccgctccagctccttcatgcggatctcgcgagcctccgcgcgggccgcccgttttgcagcgagccgggcttccgcctcccgcgcgatctggttgagcgcgtcgtcctccgccgtgagccgctcccggttggggagccgcttgcgccccgatccctgggtgcccatgtccatcgaccgcgtcgcccgcagctgccgcggggcccgttgctccagccgctcgcgccgccccggcccggcccc

SEQ ID NO: 13364 - RNA, 3509 nt, Homo sapiens
  source 1..3509: mol_type = other RNA
gctgggattacaggcatgagccaccacgcccggccaaaaacatttaaaaaatgactgtccctgctcaaatactgcagtaggaaatgtaatttgacatatatcacttccagaaaaaaactttaaatctttctataaaatgaatttgatacatcatcagcatgaagtgaagttaaaatctcttacaaagtaaattcaggtatatcaacaatgagatccaaaagtatcggttcaagatcaaagactcatatgaggtaaaggcaaataaagcccctcatgctttcagacatttacttgttatccttaaaatgattattgttctaaggtgcaaatcttatcattcagtgacctatttgctatttggctgtttatctcctttaaataaaataccatacaggttataatgtacattttaaaatcaaatatgaaagtacacatatgtgaacaagacattaatttaaatatcaattatattcataatacagaagtctaagaatgctatttggtcatttcaattagatgctgatatatttggtcaagaaaacccacattcctatcagcctaaggcaaatagtaaatgcctctatttttattaagtggactataaacagtagacattattgtttgatactactggaatgctctcaattagaacgtacactgataacaaatatgtctttctaatctgggtgataacctcaatgattacatggaaatctacaagtaacagtctataacttaaagcagtagagcacctggtaattgtcatacagtgcctctctatgaatttagaacattctacttacattggcagtggagagaaaagaccccttcacactgagacttcctgtgcaccgcgcctgccgcctgcctcagcttaggacatggtacagtcttctttgcttttgcccttctcattccctcctctggtatcttctctgctttctggattgaagtgccctggctctcttcctggtgccgacaagtcatcgttctctaggctattgctgtctaaagctttcctgacggtctgacttggatgttctgacatctcacacctctctgtactttctgcttcacaggcatcactaatgtcctgtgagggactttcatgttcgggcagggtgcagcgatctgcgtcttcgctctttggttctgcaggactgctttgagtggcaccatctattttagcattatcttttgcaacaccttcatctaattcttcaccaccagccctcgggcctgatgattgaacggtgtcatcctcaaaatctaatgtgtctccatcagctagtacctcctcagctgctgtttgtacatcatcaccttcttggtcaagttttccatccaacttaattttaggattctccggacaatcaacattttcactgctttctgctgcaattttctgttttggattttcagtcacctcgttttgggcttccactgctgactttctgtcagtagactttacctgctcttcttccttaatttcacttaaatctgtgttctgatacgttaactcttttttaacatctttaagggtttctacgggtactggggattttttcttcttgtttttctttttcttgttctttgtcttcttctgcgatgagtccaatgcctctccctgttggtcactcttttcttcatcgggctctttcatatctaagggttcattttgagtgtctactgtacttggacctgtcgcttcctgacagttgccctcagttcctgctggagaaccaggaacttctgtcttgattggtttctcgtcccttaatcctgtttcttcaccctcttcttcgttgtgatccctacctacttctgtactgtgcgctggaacctccttgggctcagctgcttcctggttggtgaattctttctctaaactatgccctgtgcttgtctctaactcttgggggacctctaccatacatttgtcatcatgataaactgtgtcatcactatgccctaaaggacacgaggccactgtgcctgcctgctcttcaacctgagtcactgctgcctctcccacattctctgtgtggttcccaccatctaagtcactccaacagttggatggctcaaggggagttctggtcctgtcatctggtgcacccatgacctcatttgactcaacctgtactgtgttttcagggagagaactgctctcaagaatttggctttgaacctgttcctcataggtagcacctgctaaggttcctaggaatggggcagtgtcttcagaggatttctggtcctcggtattctcaccagcagggaatacctctatgtccacacagtccttcactgtgtcctctgtgtgttgttctttctcagtattgtgcaagatttctcttttccccacattcgccacgatttcatttttcacctccacttcactggctcttcctagggtcccatcccctgtcgacttgagggcatttaactcttcttttgtcatcttggtaggaccttggtatccaacattattgagggtgtcggaagtctctccattggtagctatttctgaatttaggattattccatgtttctttaattcctctttcagcatgactacttcttctctaagatcatcccgttcactccttacggaatcaaagaactctttctgcctctctaatgcccctatctttttgtctttccactctattgtttcctgaagatcagaaatctccctgatagaactcgcctgtttctgctgtagctgtcggatttcctcgagcatttcctctctttgcttcagggcctccttgacttcagcaaactgaaattgcagtatactgtgggcgtgtttttccctttcaaattctttgtttttctcttcgtactgccgcctagattcagccagctgttcttcaagctccagcaacatatcttttagggtatcaacctggtacatgaagtttgtcttttcattgtctagctgagcattggaaaccatagccttcttatatttctcttcaacttctgctagagagtccttgatttccctgatggatgcctcggtgtcgatggagatggaggtgtctccgctgcctctccgagaggaagtcccacccagagaggccagcgtggctgcagacaggcccggcatgttacgagaccccttctcagtaaaatctttttctggtctctcttctaccctcaggcttccacgactacccactgacatgcgctcgtcttcatcagaagccgatgtgtttcttctggatctacgagagtagcgctcactgtcttcctccttctgctgccgctccagctccttcatgcggatctcgcgagcctccgcgcgggccgcccgttttgcagcgagccgggcttccgccagcttctgcgcttccgggctcaaacagtcgatctcccggctttgagcggccgcggggctggtcatcctgccgggctcggcccgctccacccggcgggaaatgctcggggaccgcgccgggagcccctcgcgggccgggccagggggcgcgcgctctgtc

SEQ ID NO: 13365 - RNA, 3679 nt, Homo sapiens
  source 1..3679: mol_type = other RNA
gctgggattacaggcatgagccaccacgcccggccaaaaacatttaaaaaatgactgtccctgctcaaatactgcagtaggaaatgtaatttgacatatatcacttccagaaaaaaactttaaatctttctataaaatgaatttgatacatcatcagcatgaagtgaagttaaaatctcttacaaagtaaattcaggtatatcaacaatgagatccaaaagtatcggttcaagatcaaagactcatatgaggtaaaggcaaataaagcccctcatgctttcagacatttacttgttatccttaaaatgattattgttctaaggtgcaaatcttatcattcagtgacctatttgctatttggctgtttatctcctttaaataaaataccatacaggttataatgtacattttaaaatcaaatatgaaagtacacatatgtgaacaagacattaatttaaatatcaattatattcataatacagaagtctaagaatgctatttggtcatttcaattagatgctgatatatttggtcaagaaaacccacattcctatcagcctaaggcaaatagtaaatgcctctatttttattaagtggactataaacagtagacattattgtttgatactactggaatgctctcaattagaacgtacactgataacaaatatgtctttctaatctgggtgataacctcaatgattacatggaaatctacaagtaacagtctataacttaaagcagtagagcacctggtaattgtcatacagtgcctctctatgaatttagaacattctacttacattggcagtggagagaaaagaccccttcacactgagacttcctgtgcaccgcgcctgccgcctgcctcagcttaggacatggtacagtcttctttgcttttgcccttctcattccctcctctggtatcttctctgctttctggattgaagtgccctggctctcttcctggtgccgacaagtcatcgttctctaggctattgctgtctaaagctttcctgacggtctgacttggatgttctgacatctcacacctctctgtactttctgcttcacaggcatcactaatgtcctgtgagggactttcatgttcgggcagggtgcagcgatctgcgtcttcgctctttggttctgcaggactgctttgagtggcaccatctattttagcattatcttttgcaacaccttcatctaattcttcaccaccagccctcgggcctgatgattgaacggtgtcatcctcaaaatctaatgtgtctccatcagctagtacctcctcagctgctgtttgtacatcatcaccttcttggtcaagttttccatccaacttaattttaggattctccggacaatcaacattttcactgctttctgctgcaattttctgttttggattttcagtcacctcgttttgggcttccactgctgactttctgtcagtagactttacctgctcttcttccttaatttcacttaaatctgtgttctgatacgttaactcttttttaacatctttaagggtttctacgggtactggggattttttcttcttgtttttctttttcttgttctttgtcttcttctgcgatgagtccaatgcctctccctgttggtcactcttttcttcatcgggctctttcatatctaagggttcattttgagtgtctactgtacttggacctgtcgcttcctgacagttgccctcagttcctgctggagaaccaggaacttctgtcttgattggtttctcgtcccttaatcctgtttcttcaccctcttcttcgttgtgatccctacctacttctgtactgtgcgctggaacctccttgggctcagctgcttcctggttggtgaattctttctctaaactatgccctgtgcttgtctctaactcttgggggacctctaccatacatttgtcatcatgataaactgtgtcatcactatgccctaaaggacacgaggccactgtgcctgcctgctcttcaacctgagtcactgctgcctctcccacattctctgtgtggttcccaccatctaagtcactccaacagttggatggctcaaggggagttctggtcctgtcatctggtgcacccatgacctcatttgactcaacctgtactgtgttttcagggagagaactgctctcaagaatttggctttgaacctgttcctcataggtagcacctgctaaggttcctaggaatggggcagtgtcttcagaggatttctggtcctcggtattctcaccagcagggaatacctctatgtccacacagtccttcactgtgtcctctgtgtgttgttctttctcagtattgtgcaagatttctcttttccccacattcgccacgatttcatttttcacctccacttcactggctcttcctagggtcccatcccctgtcgacttgagggcatttaactcttcttttgtcatcttggtaggaccttggtatccaacattattgagggtgtcggaagtctctccattggtagctatttctgaatttaggattattccatgtttctttaattcctctttcagcatgactacttcttctctaagatcatcccgttcactccttacggaatcaaagaactctttctgcctctctaatgcccctatctttttgtctttccactctattgtttcctgaagatcagaaatctccctgatagaactcgcctgtttctgctgtagctgtcggatttcctcgagcatttcctctctttgcttcagggcctccttgacttcagcaaactgaaattgcagtatactgtgggcgtgtttttccctttcaaattctttgtttttctcttcgtactgccgcctagattcagccagctgttcttcaagctccagcaacatatcttttagggtatcaacctggtacatgaagtttgtcttttcattgtctagctgagcattggaaaccatagccttcttatatttctcttcaacttctgctagagagtccttgatttccctgatggatgcctcggtgtcgatggagatggaggtgtctccgctgcctctccgagaggaagtcccacccagagaggccagcgtggctgcagacaggcccggcatgttacgagaccccttctcagtaaaatctttttctggtctctcttctaccctgccagatcttctattcagggactgtgatccatacaattctccatcataaccatttgtccaggcgtaaggacccccatactccaagtcaggctgcgacctcaggcttccacgactacccactgacatgcgctcgtcttcatcagaagccgatgtgtttcttctggatctacgagagtagcgctcactgtcttccatccactgctcgatgtcaccccattttgtatccagcccataatatttcttttggacctgatagatctccttctgctgccgctccagctccttcatgcggatctcgcgagcctccgcgcgggccgcccgttttgcagcgagccgggcttccgcctcccgcgcgatctggttgagcgcgtcgtcctccgccgtgagccgctcccggttggggagccgcttgcgccccgatccctgggtgcccatgtccatcgaccgcgtcgcccgcagctgccgcggggcccgttgctccagccgctcgcgccgccccggcccggcccc

SEQ ID NO: 13366 - RNA, 3654 nt, Homo sapiens
  source 1..3654: mol_type = other RNA
gctgggattacaggcatgagccaccacgcccggccaaaaacatttaaaaaatgactgtccctgctcaaatactgcagtaggaaatgtaatttgacatatatcacttccagaaaaaaactttaaatctttctataaaatgaatttgatacatcatcagcatgaagtgaagttaaaatctcttacaaagtaaattcaggtatatcaacaatgagatccaaaagtatcggttcaagatcaaagactcatatgaggtaaaggcaaataaagcccctcatgctttcagacatttacttgttatccttaaaatgattattgttctaaggtgcaaatcttatcattcagtgacctatttgctatttggctgtttatctcctttaaataaaataccatacaggttataatgtacattttaaaatcaaatatgaaagtacacatatgtgaacaagacattaatttaaatatcaattatattcataatacagaagtctaagaatgctatttggtcatttcaattagatgctgatatatttggtcaagaaaacccacattcctatcagcctaaggcaaatagtaaatgcctctatttttattaagtggactataaacagtagacattattgtttgatactactggaatgctctcaattagaacgtacactgataacaaatatgtctttctaatctgggtgataacctcaatgattacatggaaatctacaagtaacagtctataacttaaagcagtagagcacctggtaattgtcatacagtgcctctctatgaatttagaacattctacttacattggcagtggagagaaaagaccccttcacactgagacttcctgtgcaccgcgcctgccgcctgcctcagcttaggacatggtacagtcttctttgcttttgcccttctcattccctcctctggtatcttctctgctttctggattgaagtgccctggctctcttcctggtgccgacaagtcatcgttctctaggctattgctgtctaaagctttcctgacggtctgacttggatgttctgacatctcacacctctctgtactttctgcttcacaggcatcactaatgtcctgtgagggactttcatgttcgggcagggtgcagcgatctgcgtcttcgctctttggttctgcaggactgctttgagtggcaccatctattttagcattatcttttgcaacaccttcatctaattcttcaccaccagccctcgggcctgatgattgaacggtgtcatcctcaaaatctaatgtgtctccatcagctagtacctcctcagctgctgtttgtacatcatcaccttcttggtcaagttttccatccaacttaattttaggattctccggacaatcaacattttcactgctttctgctgcaattttctgttttggattttcagtcacctcgttttgggcttccactgctgactttctgtcagtagactttacctgctcttcttccttaatttcacttaaatctgtgttctgatacgttaactcttttttaacatctttaagggtttctacgggtactggggattttttcttcttgtttttctttttcttgttctttgtcttcttctgcgatgagtccaatgcctctccctgttggtcactcttttcttcatcgggctctttcatatctaagggttcattttgagtgtctactgtacttggacctgtcgcttcctgacagttgccctcagttcctgctggagaaccaggaacttctgtcttgattggtttctcgtcccttaatcctgtttcttcaccctcttcttcgttgtgatccctacctacttctgtactgtgcgctggaacctccttgggctcagctgcttcctggttggtgaattctttctctaaactatgccctgtgcttgtctctaactcttgggggacctctaccatacatttgtcatcatgataaactgtgtcatcactatgccctaaaggacacgaggccactgtgcctgcctgctcttcaacctgagtcactgctgcctctcccacattctctgtgtggttcccaccatctaagtcactccaacagttggatggctcaaggggagttctggtcctgtcatctggtgcacccatgacctcatttgactcaacctgtactgtgttttcagggagagaactgctctcaagaatttggctttgaacctgttcctcataggtagcacctgctaaggttcctaggaatggggcagtgtcttcagaggatttctggtcctcggtattctcaccagcagggaatacctctatgtccacacagtccttcactgtgtcctctgtgtgttgttctttctcagtattgtgcaagatttctcttttccccacattcgccacgatttcatttttcacctccacttcactggctcttcctagggtcccatcccctgtcgacttgagggcatttaactcttcttttgtcatcttggtaggaccttggtatccaacattattgagggtgtcggaagtctctccattggtagctatttctgaatttaggattattccatgtttctttaattcctctttcagcatgactacttcttctctaagatcatcccgttcactccttacggaatcaaagaactctttctgcctctctaatgcccctatctttttgtctttccactctattgtttcctgaagatcagaaatctccctgatagaactcgcctgtttctgctgtagctgtcggatttcctcgagcatttcctctctttgcttcagggcctccttgacttcagcaaactgaaattgcagtatactgtgggcgtgtttttccctttcaaattctttgtttttctcttcgtactgccgcctagattcagccagctgttcttcaagctccagcaacatatcttttagggtatcaacctggtacatgaagtttgtcttttcattgtctagctgagcattggaaaccatagccttcttatatttctcttcaacttctgctagagagtccttgatttccctgatggatgcctcggtgtcgatggagatggaggtgtctccgctgcctctccgagaggaagtcccacccagagaggccagcgtggctgcagacaggcccggcatgttacgagaccccttctcagtaaaatctttttctggtctctcttctacctccttctgctgccgctccagctccttcatgcggatctcgcgagcctccgcgcgggccgcccgttttgcagcgagccgggcttccgccagcttctgcgcttccgggctcaaacagtcgatctcccggctttgagcggccgcggggctggtcatcctgccgggctcggcccgctccacccggcgggaaatgctcggggaccgcgccgggagcccctcgcgggccgggccagggggcgcgcgctctgtccgcggagacggagccactcgccgctaagtgaacgctcgcgcttccggggccaggagccagcccgccggggagcggctcgcggcgctgggctcgggcgcggccgacaggggcggggcgcaggtggccgcgggctgagtcgggctcggggtggaagggcgccggggaagcgggactcgggcgcctccgcccgtcccacggcccgccccgccccccacgcagttccgcctcggaggggccctcc

SEQ ID NO: 13367 - RNA, 3393 nt, Homo sapiens
  source 1..3393: mol_type = other RNA
gctgggattacaggcatgagccaccacgcccggccaaaaacatttaaaaaatgactgtccctgctcaaatactgcagtaggaaatgtaatttgacatatatcacttccagaaaaaaactttaaatctttctataaaatgaatttgatacatcatcagcatgaagtgaagttaaaatctcttacaaagtaaattcaggtatatcaacaatgagatccaaaagtatcggttcaagatcaaagactcatatgaggtaaaggcaaataaagcccctcatgctttcagacatttacttgttatccttaaaatgattattgttctaaggtgcaaatcttatcattcagtgacctatttgctatttggctgtttatctcctttaaataaaataccatacaggttataatgtacattttaaaatcaaatatgaaagtacacatatgtgaacaagacattaatttaaatatcaattatattcataatacagaagtctaagaatgctatttggtcatttcaattagatgctgatatatttggtcaagaaaacccacattcctatcagcctaaggcaaatagtaaatgcctctatttttattaagtggactataaacagtagacattattgtttgatactactggaatgctctcaattagaacgtacactgataacaaatatgtctttctaatctgggtgataacctcaatgattacatggaaatctacaagtaacagtctataacttaaagcagtagagcacctggtaattgtcatacagtgcctctctatgaatttagaacattctacttacattggcagtggagagaaaagaccccttcacactgagacttcctgtgcaccgcgcctgccgcctgcctcagcttaggacatggtacagtcttctttgcttttgcccttctcattccctcctctggtatcttctctgctttctggattgaagtgccctggctctcttcctggtgccgacaagtcatcgttctctaggctattgctgtctaaagctttcctgacggtctgacttggatgttctgacatctcacacctctctgtactttctgcttcacaggcatcactaatgtcctgtgagggactttcatgttcgggcagggtgcagcgatctgcgtcttcgctctttggttctgcaggactgctttgagtggcaccatctattttagcattatcttttgcaacaccttcatctaattcttcaccaccagccctcgggcctgatgattgaacggtgtcatcctcaaaatctaatgtgtctccatcagctagtacctcctcagctgctgtttgtacatcatcaccttcttggtcaagttttccatccaacttaattttaggattctccggacaatcaacattttcactgctttctgctgcaattttctgttttggattttcagtcacctcgttttgggcttccactgctgactttctgtcagtagactttacctgctcttcttccttaatttcacttaaatctgtgttctgatacgttaactcttttttaacatctttaagggtttctacgggtactggggattttttcttcttgtttttctttttcttgttctttgtcttcttctgcgatgagtccaatgcctctccctgttggtcactcttttcttcatcgggctctttcatatctaagggttcattttgagtgtctactgtacttggacctgtcgcttcctgacagttgccctcagttcctgctggagaaccaggaacttctgtcttgattggtttctcgtcccttaatcctgtttcttcaccctcttcttcgttgtgatccctacctacttctgtactgtgcgctggaacctccttgggctcagctgcttcctggttggtgaattctttctctaaactatgccctgtgcttgtctctaactcttgggggacctctaccatacatttgtcatcatgataaactgtgtcatcactatgccctaaaggacacgaggccactgtgcctgcctgctcttcaacctgagtcactgctgcctctcccacattctctgtgtggttcccaccatctaagtcactccaacagttggatggctcaaggggagttctggtcctgtcatctggtgcacccatgacctcatttgactcaacctgtactgtgttttcagggagagaactgctctcaagaatttggctttgaacctgttcctcataggtagcacctgctaaggttcctaggaatggggcagtgtcttcagaggatttctggtcctcggtattctcaccagcagggaatacctctatgtccacacagtccttcactgtgtcctctgtgtgttgttctttctcagtattgtgcaagatttctcttttccccacattcgccacgatttcatttttcacctccacttcactggctcttcctagggtcccatcccctgtcgacttgagggcatttaactcttcttttgtcatcttggtaggaccttggtatccaacattattgagggtgtcggaagtctctccattggtagctatttctgaatttaggattattccatgtttctttaattcctctttcagcatgactacttcttctctaagatcatcccgttcactccttacggaatcaaagaactctttctgcctctctaatgcccctatctttttgtctttccactctattgtttcctgaagatcagaaatctccctgatagaactcgcctgtttctgctgtagctgtcggatttcctcgagcatttcctctctttgcttcagggcctccttgacttcagcaaactgaaattgcagtatactgtgggcgtgtttttccctttcaaattctttgtttttctcttcgtactgccgcctagattcagccagctgttcttcaagctccagcaacatatcttttagggtatcaacctggtacatgaagtttgtcttttcattgtctagctgagcattggaaaccatagccttcttatatttctcttcaacttctgctagagagtccttgatttccctgatggatgcctcggtgtcgatggagatggaggtgtctccgctgcctctccgagaggaagtcccacccagagaggccagcgtggctgcagacaggcccggcatgttacgagaccccttctcagtaaaatctttttctggtctctcttctacctccttctgctgccgctccagctccttcatgcggatctcgcgagcctccgcgcgggccgcccgttttgcagcgagccgggcttccgcctcccgcgcgatctggttgagcgcgtcgtcctccgccgtgagccgctcccggttggggagccgcttgcgccccgatccctgggtgcccatgtccatcgaccgcgtcgcccgcagctgccgcggggcccgttgctccagcc

SEQ ID NO: 13368 - RNA, 3364 nt, Homo sapiens
  source 1..3364: mol_type = other RNA
gctgggattacaggcatgagccaccacgcccggccaaaaacatttaaaaaatgactgtccctgctcaaatactgcagtaggaaatgtaatttgacatatatcacttccagaaaaaaactttaaatctttctataaaatgaatttgatacatcatcagcatgaagtgaagttaaaatctcttacaaagtaaattcaggtatatcaacaatgagatccaaaagtatcggttcaagatcaaagactcatatgaggtaaaggcaaataaagcccctcatgctttcagacatttacttgttatccttaaaatgattattgttctaaggtgcaaatcttatcattcagtgacctatttgctatttggctgtttatctcctttaaataaaataccatacaggttataatgtacattttaaaatcaaatatgaaagtacacatatgtgaacaagacattaatttaaatatcaattatattcataatacagaagtctaagaatgctatttggtcatttcaattagatgctgatatatttggtcaagaaaacccacattcctatcagcctaaggcaaatagtaaatgcctctatttttattaagtggactataaacagtagacattattgtttgatactactggaatgctctcaattagaacgtacactgataacaaatatgtctttctaatctgggtgataacctcaatgattacatggaaatctacaagtaacagtctataacttaaagcagtagagcacctggtaattgtcatacagtgcctctctatgaatttagaacattctacttacattggcagtggagagaaaagaccccttcacactgagacttcctgtgcaccgcgcctgccgcctgcctcagcttaggacatggtacagtcttctttgcttttgcccttctcattccctcctctggtatcttctctgctttctggattgaagtgccctggctctcttcctggtgccgacaagtcatcgttctctaggctattgctgtctaaagctttcctgacggtctgacttggatgttctgacatctcacacctctctgtactttctgcttcacaggcatcactaatgtcctgtgagggactttcatgttcgggcagggtgcagcgatctgcgtcttcgctctttggttctgcaggactgctttgagtggcaccatctattttagcattatcttttgcaacaccttcatctaattcttcaccaccagccctcgggcctgatgattgaacggtgtcatcctcaaaatctaatgtgtctccatcagctagtacctcctcagctgctgtttgtacatcatcaccttcttggtcaagttttccatccaacttaattttaggattctccggacaatcaacattttcactgctttctgctgcaattttctgttttggattttcagtcacctcgttttgggcttccactgctgactttctgtcagtagactttacctgctcttcttccttaatttcacttaaatctgtgttctgatacgttaactcttttttaacatctttaagggtttctacgggtactggggattttttcttcttgtttttctttttcttgttctttgtcttcttctgcgatgagtccaatgcctctccctgttggtcactcttttcttcatcgggctctttcatatctaagggttcattttgagtgtctactgtacttggacctgtcgcttcctgacagttgccctcagttcctgctggagaaccaggaacttctgtcttgattggtttctcgtcccttaatcctgtttcttcaccctcttcttcgttgtgatccctacctacttctgtactgtgcgctggaacctccttgggctcagctgcttcctggttggtgaattctttctctaaactatgccctgtgcttgtctctaactcttgggggacctctaccatacatttgtcatcatgataaactgtgtcatcactatgccctaaaggacacgaggccactgtgcctgcctgctcttcaacctgagtcactgctgcctctcccacattctctgtgtggttcccaccatctaagtcactccaacagttggatggctcaaggggagttctggtcctgtcatctggtgcacccatgacctcatttgactcaacctgtactgtgttttcagggagagaactgctctcaagaatttggctttgaacctgttcctcataggtagcacctgctaaggttcctaggaatggggcagtgtcttcagaggatttctggtcctcggtattctcaccagcagggaatacctctatgtccacacagtccttcactgtgtcctctgtgtgttgttctttctcagtattgtgcaagatttctcttttccccacattcgccacgatttcatttttcacctccacttcactggctcttcctagggtcccatcccctgtcgacttgagggcatttaactcttcttttgtcatcttggtaggaccttggtatccaacattattgagggtgtcggaagtctctccattggtagctatttctgaatttaggattattccatgtttctttaattcctctttcagcatgactacttcttctctaagatcatcccgttcactccttacggaatcaaagaactctttctgcctctctaatgcccctatctttttgtctttccactctattgtttcctgaagatcagaaatctccctgatagaactcgcctgtttctgctgtagctgtcggatttcctcgagcatttcctctctttgcttcagggcctccttgacttcagcaaactgaaattgcagtatactgtgggcgtgtttttccctttcaaattctttgtttttctcttcgtactgccgcctagattcagccagctgttcttcaagctccagcaacatatcttttagggtatcaacctggtacatgaagtttgtcttttcattgtctagctgagcattggaaaccatagccttcttatatttctcttcaacttctgctagagagtccttgatttccctgatggatgcctcggtgtcgatggagatggaggtgtctccgctgcctctccgagaggaagtcccacccagagaggccagcgtggctgcagacaggcccggcatgttacgagaccccttctcagtaaaatctttttctggtctctcttctacctccttctgctgccgctccagctccttcatgcggatctcgcgagcctccgcgcgggccgcccgttttgcagcgagccgggcttccgcctttgaagaatgaagatcttagatgaacttcagggggagtgtgaggaacgccagagagcagccatttggagagacatgcttggcacgagagtggaaattctggaataactg

SEQ ID NO: 13369 - RNA, 1781 nt, Homo sapiens
  source 1..1781: mol_type = other RNA
gctgggattacaggcatgagccaccacgcccggccaacatctgtatttttaatgcaggtcctctctattgagttccaaacccaaatagccagtgagtggtaggatgtcactggatgttttttgaactcctcaaattcactgtgtcccaaatggaattgattgtccctctcaaacctgtttctcattgttcgctttacctcagtgactacaacttccatccaagacacacacctgagccatcctaggctggttcatcacctggcccaagtcaccaagccatgggatgtctatttcttcggtgtctctggaatgtgtcccctcttctcactgccttagcctcagttataaaattcagttaaagaatgcaaatgcattatccagagtcacacgttctcaagcccagcagggactagaccgtaacctcatgctcagctccagattcagctcagctcctgtgctttgaagacatgtaccttccacttcctgtgaatgtggttgttagaaccagatttcagcatgctggagcagctaacggcagggaagttaggagtcagaatatctgtgtttgaagctcacatccatcacttgaagtgaatgtggtgatgttggttaatttctctgtgcttcagtctcctcatcgtgttagccaggatggtctcgatctcctgatctcgtgatctgcccacctcagcctcccaaagtgctgggattacaggcatgagccaccgcgccgggccggaattattgttctttgctctcaattctgtatgacatctaagctcctgtgccctgagctcagaacttcagggggatgaccggccagtacttgggctgctttcggtcacagtgcttgtcaaagctcagctgcaccgcggcctccatggcttggatcttggcagcactgtccccgtacaaacgcttcatctcggcctggcgccgctcaccaggcctctcagttggggcttctaccgaccggcgggtgttgcagtacaggtcgtggtcagcgttcacatagctgtccaggcgctctgcatccagctgctgctgccgccgtcgttcttctctatgcctctcggtctctgcaaagtactggcggagctcttcagtgatttccatattgctcaggtcacattctacctctgcatctgactcagtctccatctcttcctctttggacaaagcttggtcttcttttgtggatgcctggatcctactgctgtaacgtggatgctgcccagatcttctgaaatgtgaagaactgcaggggtagtcctgccaggccacatgatggtcatagaaggactgaggatacgcagcctcattatcgtaagagctttggggaagaagcgcagaaggtaagtaccatggaagattgaaacaggattccacggccttcctgtaggcattgtgatggctttgcatccaagccattgcttgatgataatgttgccagtatcttgcatataccggatgagaataccaaggcctggtagctttcgatgttgatgcctttaccgctgccatctctgattgtgaaagtccaaatgggtgctgaaactccctgggaatgtctcccactcttttatggcacaagccttcagggactgaacagtaacttttctccaatgggctggtggagctcgtgggcgcgcagcttgcggatcctgggcgttggccgcgcaggggcctagttttccttggagagacagagggggagtgggggacgcgagggaggcggctgttgccggggcgactggaagcgcgcttccggtgcggaacac

SEQ ID NO: 13370 - RNA, 5335 nt, Homo sapiens
  source 1..5335: mol_type = other RNA
gctgggattacaggcatgagccaccacgcccggccaacatctgtatttttaatgcaggtcctctctattgagttccaaacccaaatagccagtgagtggtaggatgtcactggatgttttttgaactcctcaaattcactgtgtcccaaatggaattgattgtccctctcaaacctgtttctcattgttcgctttacctcagtgactacaacttccatccaagacacacacctgagccatcctaggctggttcatcacctggcccaagtcaccaagccatgggatgtctatttcttcggtgtctctggaatgtgtcccctcttctcactgccttagcctcagttataaaattcagttaaagaatgcaaatgcattatccagagtcacacgttctcaagcccagcagggactagaccgtaacctcatgctcagctccagattcagctcagctcctgtgctttgaagacatgtaccttccacttcctgtgaatgtggttgttagaaccagatttcagcatgctggagcagctaacggcagggaagttaggagtcagaatatctgtgtttgaagctcacatccatcacttgaagtgaatgtggtgatgttggttaatttctctgtgcttcagtctcctcatcgtgttagccaggatggtctcgatctcctgatctcgtgatctgcccacctcagcctcccaaagtgctgggattacaggcatgagccaccgcgccgggccggaattattgttctttgctctcaattctgtatgacatctaagctcctgtgccctgagctcagaacttcagggggatgaccggccagtacttgggctgctttcggtcacagtgcttgtcaaagctcagctgcaccgcggcctccatggcttggatcttggcagcactgtccccgtacaaacgcttcatctcggcctggcgccgctcaccaggcctctcagttggggcttctaccgaccggcgggtgttgcagtacaggtcgtggtcagcgttcacatagctgtccaggcgctctgcatccagctgctgctgccgccgtcgttcttctctatgcctctcggtctctgcaaagtactggcggagctcttcagtgatttccatattgctcaggtcacattctacctctgcatctgactcagtctccatctcttcctctttggacaaagcttggtcttcttttgtggatgcctggatcctactgctgtaacgtggatgctgcccagatcttctgaaatgtgaagaactgcaggggtagtcctgccaggccacatgatggtcatagaaggactgaggatacgcagcctcattatcgtaagagctttggggaagaagcgcagaaggtaagtaccatggaagattgaaacaggattccacggccttcctgtaggcattgtgatggctttgcatccaagccattgcttgatgataatgttgccagtatcttgcatataccggatgagaataccaaggcctggtagctttcgatgttgatgcctttaccgctgccatctctgattgtgaaagtccaaatgggtgctgaaactccctgggaatgtctcccactcttttatggcacaagccttcagggactgaacagtaacttttctccaatgggctggtggagctgaaagaaaagagattggcaatgtcagggaaggccgggatccgcagctctacaaacccggcagccctctccagtgagcacaatggcataatggccaccacccagctgagcccaggcgagtacagagaccattcattgtctgtcctcaaccaccaaagaaggaaggaaaaaaacagggttgaggtcattcactaaacactgacgaggcctataggcaaggcagagactgagtcttgaatgatatatttttccatatagcctctcttaaaaaacggatttacacttcagtacatctgctcatcctgcaggatctatttttaatgcataaatatacacaaagaacaatagataagagctttgtagttttcaatggataaaatgtgactatttccatcaagttaccaaaaaatttcacaaataagtggctttgttgacaggtagtgccatcaaatatattcttttaattacatatttatgttcttataaatatagaatataggacaaatcgtagcaaccaaaaaagtaaaataaaaacacaaattcccctaaaaactagaatgtatacttgaactagattttcctatcttccttttctactagaattctaaaaatacatgaaaattcacctgctttgatctttgcacagaaacacattaaaagccaatcattaaataagttactctggctaaagccctgaaagtcaaaccttccctacaaagctccagtgatttggttctctgaaccaaccaggtaatttggaggatttagttaggtcttcagtacacactgtttcaaggagatctgctggacactgcagcaaaataagtgaaggtatggtgagaaatctgagtgagatagattgagtcatatgcggttccaaggaatctctctgtacatgcaataataaccctatcacagaagatgtcttccaataatacacacaacagtaagaacttcctcactaagacaaagaatataatagggttttgttgagggctgggcttcctgccccacctacttgggcagccctgcccccatccctggctggttgctgaggctggcaagctcatctggcttgatgccctcatggcctccctcctgtgtctttgcatggtccctgcttagtgatttggacatcaaagatggctcaagtccaaatggccttcttccacctgcagacatccaagctccatcttgggcaggacacaggcctactcaagtgcacatgccactgtgttcagaaagcctgcatctccccgtctataatagctacagttaaaactgataggcaagggagccaaaaaactgagttttattttcttttcattccctcaatccccaaccccaatttaccctcttctggatgttgtaataagtactgtcacaaagaaggcatagcatggggaaggagtaaggctgaaaggatgcagttaacaattctttttttcatacaaatgacattccacccacagaagggcattgtttaatttgtcagcaagtgtgatgaatttgtgaatgggtttatttgcaagttctctgaatccccttgtgactaatatcagaatcaaaagtgaaatatgaggccaggaacaaagttaccctctgactcaggaacacaacaagcaatgggatgactgagaatgacataatgataacatagttcaaaagaggaaacagataagtttgtttcacagcaagcatgtccttcataagcaaaacctagtgtgaccataaggtaataagggttgaataggcaggttctgcaaattaagagcataacagcaaaaaccatggctagtttaaagtagttaagatcgctagtacatttcaggcgtcttatttcaaatttacttttttctataaacatattcacggtaattccatgttaatctctcttttctgaatttataggcactcactatgcctcatttacttgggcacttactcagttacctgtaggcatggattctacaatctactccttttaagtttcctattttccttccagcataaaaataatagctaatatttcatgctcttagatgctgctgaaattgttgagcttgtctgttgtttcctgataacgttctctcctcctgcatctactccccaaaatctctgaggacctagtaactcaaaaaactgactataaagcaccaaatcttttcaggaagcaaatatttaaatacattatgttttcaaagatcttttcaattcatctgatatttgatcaactacattcttttttcacttgtccagctgttccgtggctgaatttcctcttgtagagaagttgttcaaaaaaagttctgtacctactttgcaaactctccaatttacactctagccttaactgttcaaaactttcccccgtcattctcatctcaccctatcctttaaaaaaaaacccaaaatgattaatcaccatctatagaacagtttcagaatgaacatttctctctggaactttagtttgtatacttccccagcacagcaatgaacacacagaggggatttatacacctgtgaacttgctttcagttatgcttattccaagttactaaccagcagtctttaaaaatatatggtttctgttcacattgaaattacaaagagactgttattccgataaattatgctagcaaaaatagtatttttaaagggtagctctcatcctacaattcatgggggctgtgagcataaataatcctagaagtgttgcgttactaatctttagtctagattttttaagtaatattgttctgatttgagatgaagaacagctgaatacacagcctagcctgtcaaacgagtttaaaaacatcattcctgaaaaaaataaaattgttcagaaccatctgatctgtactaagggaacatcaagatttcagagctaaaatgcacttcgttggccactggttcaattacagctcattactgataagtgggcagagacacaaggcccataaactgtaggcgccagatgtctcaagataactcccaccaaaagctgacctcctgcagaggttaaagtgcaagagaaaagaaagaaacccgaatttttgagcagagagggcaatatcctagacatccttcaagtatgtggctgtcctgggcgatcttctattcagatactggactggatgggcaaaatccgaattcacctacagaccttaacacggtggttctcggcaccccagaatcacctgggcagctttaaaaactaccgatgccagggccccactattagagattctgatttcattggtccgggatgggggcccggggatcagaattcttaaagagtcgtccagtgattcggaagcactgcagagctgagagcctctgggactggtcccctctcacaattaacctgcaatgatttaggaatctcatgggcctccggccccaccttttgtcgcgggattaagataattatgagagcaacgtgacgtccaagacctcggctctctgcgcatcagaagaagccagggcccggggcgtctaagctcctccctcactccccaaaggaaacccagccgtccccgaagtcacctcgtgggcgcgcagcttgcggatcctgggcgttggccgcgcaggggcctagttttccttggagagacagagggggagtgggggacgcgagggaggcggctgttgccggggcgactggaagcgcgcttccggtgcggaaca

SEQ ID NO: 13371 - RNA, 3574 nt, Homo sapiens
  source 1..3574: mol_type = other RNA
gctgggattacaggcatgagccaccacgcccggccaagctattgtaacttttctaatgcattatttgtgttcgcctctaggtggtgatgatgggccttttcatctactaaagtgtcgctaaggattagaataaatttaaatttttcatagcctctggcctagaggtctaggcttcctttcttatatgatatctaaaatctcctttaactcatttcttcttcttcctgcaggaggaaaaaacatgggcctttaccaaaaacattttcagtataccatctcagtcttcacaaccccttaactaggatcatcatctccattttggctaagtgaaaacagactcagagtaaactgcccaaatctcacagctgtagtaagtggaacccagataagaaatataggtttagccataaactactgcccctccaacagacttctttgattttatcaaagaagtgaattgttctctcgaggcttcaagagaattccaagttttgagttgataatttgcgtttcagagatctccaggctgtctgcctctttttccaacaagttctctttttcacacaagtacacgcccccttcagggaacattcttccagaaatccaaagtccactaacagcatttcctgtcctaggtgcagggaaatgtgtgaagtctggctgcagtgcccaagagataagaatcttctaagctggctgttgtccagacttgccatcctcattgtagtaaaacactggccaggaagacaaaagtgcataagtgtgcttctcagaacaggagcattcattccacttcatactctggcttctccaccttctggcttcaagacagtttgtccctcggctagggcagagaggttcatatgggcacttgggctcggtgcaccttgggctctgggggtcgaggggcaggctgcagtatgggagcggggggagccacactcatctgaggtgatgtctggcacatcgtctgactgtgcatcagaactctctaggtcactgcggatgctttcaggctgggccaggctgatgtcccaaggtttgctggccaggcagtctttctgttcacagctttggtgtctgcaggggggatcctcttcactgcctccgccaccactaccttcttcttcattctctgccatctgagcatgaacatggagcgagtcctccgtgctgcttccactcaccagctgatagtggcttggtttggcttcaatgtccacttggatttccatattgttgcattctctgtcctgtgggttgtaggaactgattatggaaccggccatagcacgagtgcttgcgttgtcactaattgcaccaagactggctgtgtctttggggaaaatttccttttggacatcggcttgaacttctaacctgctatattttcccttgccactggagagaatgccgccactcagcgtgccccctgagagggctgcaaagctggccgtttcgctgtaaggaccttgcataacactaagtccatctgtagggcttccactagtgctcaatacactagtcaggccttcaatgctgctttccccaatgctgggattcttgagggctctccaggcatctgccactgtgattggaccatcatcttcatcaaattcaattttcactccttttccgttggctgtgctaactccacagccgcctccacgacaaagagaaatgggcacaaccccataaacatatgccagcataatggggacaccaataccaacactaactgcagcaataactggggatgcaatgaccgacaaagtcactcctccagtgatagccaaattcctcttgtgtttggaggttttccttccctcatacctgctgtgaatcttccttccaacataaacaggaatgccaatgaccatggcaggaatggcaatgccagcaatgagagaaatccccactggagcaccaatcaacgtgcccagctgccaaagaattttcttcttacggctccatggcttcttgccccagaatgtacagccagaggggctgaggtaatgcaagtctgagatctctttcatacaaagccaacagaattcacagccacacactgcacaggtcatgtgattacagcttccatcattcatcttgataatgtatgcactgcatcgtgggcatggcttgatgtcatctgctggtccagattcttgcccataactgagacctgaagtgtgtttggtccgaactcgtaaagtctgggccctctgttgacgggccatatcgcatgtctgatttggatgccatatctgcttgcagtggtagcagaactcagtctggcaaccttccctctcacaagttagcttcgggcagctggcacagccataggcaataacagcataaccgcagtccggggccgggcaccagcggcagtcggggtccgaggctaggtagcggcgcagcatgaactcctcgtacttgtgcataagcggcgggtcggcgagcagcaagcggatgtcgtgcgggttgagtcgctcgctgcactcggggcagctgatgggcaccctgctctcgcttatctccaggcgcaggtagtggcggaggcagtcccggcacgagcggtgcggacagctgaggaggcgcggggcccgctcaggcggcagccgcaccaggcacagcggacactccacctcctccgcgcccgggccaccgccctccgccgcctcctcatcgtcgaacccaggctccgccgccgccgccgcggcctccgcctcggcctcggcggccggctcggcgggcagcgcctcgggcggcgggccctgggccgcggcaggggccggggcgggcggcggctgcgcagccgggggcggcggctcggcctgcggcttggcccgggcgcggcggccgcgggccgaggcagagaagacgctgtgcaaggtgaggcgccggcgccggccgccgctgcggcacttagggtcgggtgcggccgcatgtagcgatgtggagcgcggcgactcggagtccttctcggagcccatggccggcagaggccgaggagccaggggcgcccagcgccgccacagctcccgcctcagcgcccctcagccagcgcccggccgccgccgacgccgccaccaccgcctcaaccgccctcccggcgatagaagccgagcggcaacgacgaagtgattataaagcctccgccccgcgcgccgctgccctgcgcaggcgcttcgctcaaacacctcacaacccttgcgccccggtctaggagtgcgctgggcagggccgagcggggtggggccgagcgagctggggcggagctccgcctcctgccggtcaggtggttccagggccgccatgttgcggagactctcagagatcctagcccgctgctctccctggtctccgcctccaattccatcaccatgacacccaaggtggactttttggtttgccgttcctcacaggttgattgccacttccagtaaatgatggttcagttacattatttataaaaagcaggcaggggttgatcagatggtgactcccaactggttcaccttccaacatttctgtttattaagcagacggcataaattaataaagaatatattca

SEQ ID NO: 13372 - RNA, 2223 nt, Homo sapiens
  source 1..2223: mol_type = other RNA
gctgggattacaggcatgagccaccacgcccggccacagtattttttaaatgccagttaggttttataagatgtagaattctataactccaacacaagaatgacaggtgatgcttgcatgactttggcaactaacttccaggaagccctaggatttacaagatgctttgagtgacattagtcacaagagattgttgcaactaaacagaacacaggatgataaagaatgaatgaggaagaatgaagaccactggtgagatggcacttctgaccaggggcctactcctggaggtcaagtccttgagtcccattggaggaggagtaacccctcccttccccacatagagttttagtgcctgaaacctcacagggaaccaagaagatctaatctcacctctctggactacagaggactgccggtagccctgggaagtaccaagctcttgaaagcttcacacagtgatggtggcagcagaggcaggaagtgagcagtgccattaactggagtgaaggattcagtgaggttctgagactcccttacaaccccgcagtttgtatttagtctaatacattctcctcccctagctcaaagttccaagatttagataagcacaatttaagacaggttccctgaataccctattagggaatgttgggacgtagttgaaatggcaacttttattaatgatgaatggcaatgacttttaagtttgatcacagagtgtttgcatattttcttactatttttggtatgatttaaaaattattggttcattaaccatttaaaagaggaataattcagtagaggcactaggaggttgaacaggatcattcttcagtaatattctgcccactcctccaaatgggaaagagttgagcgtgaagtgcataatgacgtcattgcctgtgacacctccactggatgtctcatcaatcatccgtttgatgagcttatggttatgcgaaaatacataaagagccagaggcttttcacgttcatttatgaaatttatggcctcatctacatttttcacaggcactattggaagaattggtccaaaaatttcttcttgcatcaccttggttttaggatcaacatcggtaagtactgttggggctatgtagcgtgtggcctcatcagtctccccaccaaaagctatcttttgtccttcaagcaaacttagtatcctcttaaaatgacgaagattgatgatcctttcataatcaggagactcttttatattttctccataaaattccttcactgtttccttaatcttccatacaatttgattttggagggatgcttcacagagaatatagtcgggtgcaatgcaggtttggccacaattcatgtattttccccaggttatgcgtctgcaaacaatgtccaggtcacaatctttatcaatataacatggacttttccctcccagttcaagagtcacaggggtcagatgcttggcagcagcttccatgacaattttgccaaccgcagtgtttcccgtatagaaaatgtggtcaaatcgctgcttcaggagctccgtggtttcctcaacaccaccattaataacaatatagagatcctggtctaaatactgagggagaagctttgccaagatcttggctgtattttcactcagttcagaaggctttataatcacagcatttcctgcagcgatggctcctatcagtggctgaatggtgagaacgaaggggtaattccaagctccgattatcagcaccactcccagaggctgtggctgaatataggcctcatccagcatggtgagcacgttcttcttaactggtttagcagtaacccattcaggaagattctcaagcataaaatcaatttccccaaggacagtaatgacttcctgactgtacacattgaattcactcttgcacaggtcggcggcgatggccgtcaggatatccttctcgcgctcctgcaccatcctccgcagggcctccagctgctgcagccgaaaccgcagaggtcgcgaccggccggacaggaacgcctgtcggacccgccggacttcgagctccatggcctggtcctgcagagaactgcacggtccgggggcgcgtcccagttccctggagagctagtccctgagggcgggaagccggggttcgtctcccgcggagccgggacagcggtcatttccttcttgcacaagcatcatcctcgcacgtccgttactcagagcttctc

SEQ ID NO: 13373 - RNA, 2547 nt, Homo sapiens
  source 1..2547: mol_type = other RNA
gctgggattacaggcatgagccaccacgcccggccacagtattttttaaatgccagttaggttttataagatgtagaattctataactccaacacaagaatgacaggtgatgcttgcatgactttggcaactaacttccaggaagccctaggatttacaagatgctttgagtgacattagtcacaagagattgttgcaactaaacagaacacaggatgataaagaatgaatgaggaagaatgaagaccactggtgagatggcacttctgaccaggggcctactcctggaggtcaagtccttgagtcccattggaggaggagtaacccctcccttccccacatagagttttagtgcctgaaacctcacagggaaccaagaagatctaatctcacctctctggactacagaggactgccggtagccctgggaagtaccaagctcttgaaagcttcacacagtgatggtggcagcagaggcaggaagtgagcagtgccattaactggagtgaaggattcagtgaggttctgagactcccttacaaccccgcagtttgtatttagtctaatacattctcctcccctagctcaaagttccaagatttagataagcacaatttaagacaggttccctgaataccctattagggaatgttgggacgtagttgaaatggcaacttttattaatgatgaatggcaatgacttttaagtttgatcacagagtgtttgcatattttcttactatttttggtatgatttaaaaattattggttcattaaccatttaaaagaggaataattcagtagaggcactaggaggttgaacaggatcattcttcagtaatattctgcctcactcttaacagacagggctgggttttgaaatctggtgttcatctctgcttactggaccaacgcagtctgtgaactaccagaaaaatcaacagggcctttctcctcagcacagcttggtatttcttgacaagcacagcggctacaatacccaggaaagtgagcaacaggagaccgagtttttctttgttgaaccgtttcaagagaaaaaattttccccaatccacctttgactggctgttgggaggatatctgagtttgttagcaccttctctctttaaactttttaataaacagggacgctgatgagaaaaagtatcaaaactatgttttccgtgataagctcccatcccactggaacccactcctccaaatgggaaagagttgagcgtgaagtgcataatgacgtcattgcctgtgacacctccactggatgtctcatcaatcatccgtttgatgagcttatggttatgcgaaaatacataaagagccagaggcttttcacgttcatttatgaaatttatggcctcatctacatttttcacaggcactattggaagaattggtccaaaaatttcttcttgcatcaccttggttttaggatcaacatcggtaagtactgttggggctatgtagcgtgtggcctcatcagtctccccaccaaaagctatcttttgtccttcaagcaaacttagtatcctcttaaaatgacgaagattgatgatcctttcataatcaggagactcttttatattttctccataaaattccttcactgtttccttaatcttccatacaatttgattttggagggatgcttcacagagaatatagtcgggtgcaatgcaggtttggccacaattcatgtattttccccaggttatgcgtctgcaaacaatgtccaggtcacaatctttatcaatataacatggacttttccctcccagttcaagagtcacaggggtcagatgcttggcagcagcttccatgacaattttgccaaccgcagtgtttcccgtatagaaaatgtggtcaaatcgctgcttcaggagctccgtggtttcctcaacaccaccattaataacaatatagagatcctggtctaaatactgagggagaagctttgccaagatcttggctgtattttcactcagttcagaaggctttataatcacagcatttcctgcagcgatggctcctatcagtggctgaatggtgagaacgaaggggtaattccaagctccgattatcagcaccactcccagaggctgtggctgaatataggcctcatccagcatggtgagcacgttcttcttaactggtttagcagtaacccattcaggaagattctcaagcataaaatcaatttccccaaggacagtaatgacttcctgactgtacacattgaattcactcttgcacaggtcggcggcgatggccgtcaggatatccttctcgcgctcctgcaccatcctccgcagggcctccagctgctgcagccgaaaccgcagaggtcgcgaccggccggacaggaacgcctgtcggacccgccggacttcgagctccatggcctggtcctgcagagaactgcacggtccgggggcgagccacaattcactcgcccagggctcgctcgctcagccgcgacctccacgcccgctgagtcccactgccagtcggaggcgccgggggaggact

SEQ ID NO: 13374 - RNA, 2584 nt, Homo sapiens
  source 1..2584: mol_type = other RNA
gctgggattacaggcatgagccaccacgcccggccacagtattttttaaatgccagttaggttttataagatgtagaattctataactccaacacaagaatgacaggtgatgcttgcatgactttggcaactaacttccaggaagccctaggatttacaagatgctttgagtgacattagtcacaagagattgttgcaactaaacagaacacaggatgataaagaatgaatgaggaagaatgaagaccactggtgagatggcacttctgaccaggggcctactcctggaggtcaagtccttgagtcccattggaggaggagtaacccctcccttccccacatagagttttagtgcctgaaacctcacagggaaccaagaagatctaatctcacctctctggactacagaggactgccggtagccctgggaagtaccaagctcttgaaagcttcacacagtgatggtggcagcagaggcaggaagtgagcagtgccattaactggagtgaaggattcagtgaggttctgagactcccttacaaccccgcagtttgtatttagtctaatacattctcctcccctagctcaaagttccaagatttagataagcacaatttaagacaggttccctgaataccctattagggaatgttgggacgtagttgaaatggcaacttttattaatgatgaatggcaatgacttttaagtttgatcacagagtgtttgcatattttcttactatttttggtatgatttaaaaattattggttcattaaccatttaaaagaggaataattcagtagaggcactaggaggttgaacaggatcattcttcagtaatattctgcctcactcttaacagacagggctgggttttgaaatctggtgttcatctctgcttactggaccaacgcagtctgtgaactaccagaaaaatcaacagggcctttctcctcagcacagcttggtatttcttgacaagcacagcggctacaatacccaggaaagtgagcaacaggagaccgagtttttctttgttgaaccgtttcaagagaaaaaattttccccaatccacctttgactggctgttgggaggatatctgagtttgttagcaccttctctctttaaactttttaataaacagggacgctgatgagaaaaagtatcaaaactatgttttccgtgataagctcccatcccactggaacccactcctccaaatgggaaagagttgagcgtgaagtgcataatgacgtcattgcctgtgacacctccactggatgtctcatcaatcatccgtttgatgagcttatggttatgcgaaaatacataaagagccagaggcttttcacgttcatttatgaaatttatggcctcatctacatttttcacaggcactattggaagaattggtccaaaaatttcttcttgcatcaccttggttttaggatcaacatcggtaagtactgttggggctatgtagcgtgtggcctcatcagtctccccaccaaaagctatcttttgtccttcaagcaaacttagtatcctcttaaaatgacgaagattgatgatcctttcataatcaggagactcttttatattttctccataaaattccttcactgtttccttaatcttccatacaatttgattttggagggatgcttcacagagaatatagtcgggtgcaatgcaggtttggccacaattcatgtattttccccaggttatgcgtctgcaaacaatgtccaggtcacaatctttatcaatataacatggacttttccctcccagttcaagagtcacaggggtcagatgcttggcagcagcttccatgacaattttgccaaccgcagtgtttcccgtatagaaaatgtggtcaaatcgctgcttcaggagctccgtggtttcctcaacaccaccattaataacaatatagagatcctggtctaaatactgagggagaagctttgccaagatcttggctgtattttcactcagttcagaaggctttataatcacagcatttcctgcagcgatggctcctatcagtggctgaatggtgagaacgaaggggtaattccaagctccgattatcagcaccactcccagaggctgtggctgaatataggcctcatccagcatggtgagcacgttcttcttaactggtttagcagtaacccattcaggaagattctcaagcataaaatcaatttccccaaggacagtaatgacttcctgactgtacacattgaattcactcttgcacaggtcggcggcgatggccgtcaggatatccttctcgcgctcctgcaccatcctccgcagggcctccagctgctgcagccgaaaccgcagaggtcgcgaccggccggacaggaacgcctgtcggacccgccggacttcgagctccatggcctggtcctgcagagaactgcacggtccgggggcgcgtcccagttccctggagagctagtccctgagggcgggaagccggggttcgtctcccgcggagccgggacagcggtcatttccttcttgcacaagcatcatcctcgcacgtccgttactcagagcttctc

SEQ ID NO: 13375 - RNA, 2638 nt, Homo sapiens
  source 1..2638: mol_type = other RNA
gctgggattacaggcatgagccaccacgcccggccacagtattttttaaatgccagttaggttttataagatgtagaattctataactccaacacaagaatgacaggtgatgcttgcatgactttggcaactaacttccaggaagccctaggatttacaagatgctttgagtgacattagtcacaagagattgttgcaactaaacagaacacaggatgataaagaatgaatgaggaagaatgaagaccactggtgagatggcacttctgaccaggggcctactcctggaggtcaagtccttgagtcccattggaggaggagtaacccctcccttccccacatagagttttagtgcctgaaacctcacagggaaccaagaagatctaatctcacctctctggactacagaggactgccggtagccctgggaagtaccaagctcttgaaagcttcacacagtgatggtggcagcagaggcaggaagtgagcagtgccattaactggagtgaaggattcagtgaggttctgagactcccttacaaccccgcagtttgtatttagtctaatacattctcctcccctagctcaaagttccaagatttagataagcacaatttaagacaggttccctgaataccctattagggaatgttgggacgtagttgaaatggcaacttttattaatgatgaatggcaatgacttttaagtttgatcacagagtgtttgcatattttcttactatttttggtatgatttaaaaattattggttcattaaccatttaaaagaggaataattcagtagaggcactaggaggttgaacaggatcattcttcagtaatattctgcctcactcttaacagacagggctgggttttgaaatctggtgttcatctctgcttactggaccaacgcagtctgtgaactaccagaaaaatcaacagggcctttctcctcagcacagcttggtatttcttgacaagcacagcggctacaatacccaggaaagtgagcaacaggagaccgagtttttctttgttgaaccgtttcaagagaaaaaattttccccaatccacctttgactggctgttgggaggatatctgagtttgttagcaccttctctctttaaactttttaataaacagggacgctgatgagaaaaagtatcaaaactatgttttccgtgataagctcccatcccactggaacccactcctccaaatgggaaagagttgagcgtgaagtgcataatgacgtcattgcctgtgacacctccactggatgtctcatcaatcatccgtttgatgagcttatggttatgcgaaaatacataaagagccagaggcttttcacgttcatttatgaaatttatggcctcatctacatttttcacaggcactattggaagaattggtccaaaaatttcttcttgcatcaccttggttttaggatcaacatcggtaagtactgttggggctatgtagcgtgtggcctcatcagtctccccaccaaaagctatcttttgtccttcaagcaaacttagtatcctcttaaaatgacgaagattgatgatcctttcataatcaggagactcttttatattttctccataaaattccttcactgtttccttaatcttccatacaatttgattttggagggatgcttcacagagaatatagtcgggtgcaatgcaggtttggccacaattcatgtattttccccaggttatgcgtctgcaaacaatgtccaggtcacaatctttatcaatataacatggacttttccctcccagttcaagagtcacaggggtcagatgcttggcagcagcttccatgacaattttgccaaccgcagtgtttcccgtatagaaaatgtggtcaaatcgctgcttcaggagctccgtggtttcctcaacaccaccattaataacaatatagagatcctggtctaaatactgagggagaagctttgccaagatcttggctgtattttcactcagttcagaaggctttataatcacagcatttcctgcagcgatggctcctatcagtggctgaatggtgagaacgaaggggtaattccaagctccgattatcagcaccactcccagaggctgtggctgaatataggcctcatccagcatggtgagcacgttcttcttaactggtttagcagtaacccattcaggaagattctcaagcataaaatcaatttccccaaggacagtaatgacttcctgactgtacacattgaattcactcttgcacaggtcggcggcgatggccgtcaggatatccttctcgcgctcctgcaccatcctccgcagggcctccagctgctgcagccgaaaccgcagaggtcgcgaccggccggacaggaacgcctgtcggacccgccggacttcgagctccatggcctggtcctgcagagaactgcacggtccgggggcgctggggagtgggaggcgggaagcatgcaggtgcaggcctcgcctcccttccctccgcctccctccggggggtgtctccaccgtcaacccacagccacaattcactcgcccagggctcgctcgctcagccgcgacctccacgcccgctgagtcccactgccagtcggaggcgccgggggaggact

SEQ ID NO: 13376 - RNA, 2317 nt, Homo sapiens
  source 1..2317: mol_type = other RNA
gctgggattacaggcatgagccaccacgcccggccacagtattttttaaatgccagttaggttttataagatgtagaattctataactccaacacaagaatgacaggtgatgcttgcatgactttggcaactaacttccaggaagccctaggatttacaagatgctttgagtgacattagtcacaagagattgttgcaactaaacagaacacaggatgataaagaatgaatgaggaagaatgaagaccactggtgagatggcacttctgaccaggggcctactcctggaggtcaagtccttgagtcccattggaggaggagtaacccctcccttccccacatagagttttagtgcctgaaacctcacagggaaccaagaagatctaatctcacctctctggactacagaggactgccggtagccctgggaagtaccaagctcttgaaagcttcacacagtgatggtggcagcagaggcaggaagtgagcagtgccattaactggagtgaaggattcagtgaggttctgagactcccttacaaccccgcagtttgtatttagtctaatacattctcctcccctagctcaaagttccaagatttagataagcacaatttaagacaggttccctgaataccctattagggaatgttgggacgtagttgaaatggcaacttttattaatgatgaatggcaatgacttttaagtttgatcacagagtgtttgcatattttcttactatttttggtatgatttaaaaattattggttcattaaccatttaaaagaggaataattcagtagaggcactaggaggttgaacaggatcattcttcagtaatattctgcctcactcttaacagacagggctgggttttgaaatctggtgttcatctctgcttactggaccaacgcagtctgtgaactaccagaaaaatcaacagggcctttctcctcagcacagcttggtatttcttgacaagcacagcggctacaatacccaggaaagtgagcaacaggagaccgagtttttctttgttgaaccgtttcaagagaaaaaattttccccaatccacctttgactggctgttgggaggatatctgagtttgttagcaccttctctctttaaactttttaataaacagggacgctgatgagaaaaagtatcaaaactatgttttccgtgataagctcccatcccactggaacccactcctccaaatgggaaagagttgagcgtgaagtgcataatgacgtcattgcctgtgacacctccactggatgtctcatcaatcatccgtttgatgagcttatggttatgcgaaaatacataaagagccagaggcttttcacgttcatttatgaaatttatggcctcatctacatttttcacaggcactattggaagaattggtccaaaaatttcttcttgcatcaccttggttttaggatcaacatcggtaagtactgttggggctatgtagcgtgtggcctcatcagtctccccaccaaaagctatcttttgtccttcaagcaaacttagtatcctcttaaaatgacgaagattgatgatcctttcataatcaggagactcttttatattttctccataaaattccttcactgtttccttaatcttccatacaatttgattttggagggatgcttcacagagaatatagtcgggtgcaatgcaggtttggccacaattcatgtattttccccaggttatgcgtctgcaaacaatgtccaggtcacaatctttatcaatataacatggacttttccctcccagttcaagagtcacaggggtcagatgcttggcagcagcttccatgacaattttgccaaccgcagtgtttcccgtatagaaaatgtggtcaaatcgctgcttcaggagctccgtggtttcctcaacaccaccattaataacaatatagagatccttcaacctctatcttctggttctacgtcctattcaatccttgacatctcactgtcttccatttcatctttcttgattggatcatcacagctattagaacaaaatggctctggtctaaatactgagggagaagctttgccaagatcttggctgtattttcactcagttcagaaggctttataatcacagcatttcctgcagcgatggctcctatcagtggctgaatggtgagaacgaaggggtaattccaagctccgattatcagcaccactcccagaggctgtggctgaatataggcctcatccagcatggtgagcacgttcttcttaactggtttagcagtaacccattcaggaagattctcaagcata

SEQ ID NO: 13377 - RNA, 2422 nt, Homo sapiens
  source 1..2422: mol_type = other RNA
gctgggattacaggcatgagccaccacgcccggccacagtattttttaaatgccagttaggttttataagatgtagaattctataactccaacacaagaatgacaggtgatgcttgcatgactttggcaactaacttccaggaagccctaggatttacaagatgctttgagtgacattagtcacaagagattgttgcaactaaacagaacacaggatgataaagaatgaatgaggaagaatgaagaccactggtgagatggcacttctgaccaggggcctactcctggaggtcaagtccttgagtcccattggaggaggagtaacccctcccttccccacatagagttttagtgcctgaaacctcacagggaaccaagaagatctaatctcacctctctggactacagaggactgccggtagccctgggaagtaccaagctcttgaaagcttcacacagtgatggtggcagcagaggcaggaagtgagcagtgccattaactggagtgaaggattcagtgaggttctgagactcccttacaaccccgcagtttgtatttagtctaatacattctcctcccctagctcaaagttccaagatttagataagcacaatttaagacaggttccctgaataccctattagggaatgttgggacgtagttgaaatggcaacttttattaatgatgaatggcaatgacttttaagtttgatcacagagtgtttgcatattttcttactatttttggtatgatttaaaaattattggttcattaaccatttaaaagaggaataattcagtagaggcactaggaggttgaacaggatcattcttcagtaatattctgccttgacaagcacagcggctacaatacccaggaaagtgagcaacaggagaccgagtttttctttgttgaaccgtttcaagagaaaaaattttccccaatccacctttgactggctgttgggaggatatctgagtttgttagcaccttctctctttaaactttttaataaacagggacgctgatgagaaaaagtatcaaaactatgttttccgtgataagctcccatcccactggaacccactcctccaaatgggaaagagttgagcgtgaagtgcataatgacgtcattgcctgtgacacctccactggatgtctcatcaatcatccgtttgatgagcttatggttatgcgaaaatacataaagagccagaggcttttcacgttcatttatgaaatttatggcctcatctacatttttcacaggcactattggaagaattggtccaaaaatttcttcttgcatcaccttggttttaggatcaacatcggtaagtactgttggggctatgtagcgtgtggcctcatcagtctccccaccaaaagctatcttttgtccttcaagcaaacttagtatcctcttaaaatgacgaagattgatgatcctttcataatcaggagactcttttatattttctccataaaattccttcactgtttccttaatcttccatacaatttgattttggagggatgcttcacagagaatatagtcgggtgcaatgcaggtttggccacaattcatgtattttccccaggttatgcgtctgcaaacaatgtccaggtcacaatctttatcaatataacatggacttttccctcccagttcaagagtcacaggggtcagatgcttggcagcagcttccatgacaattttgccaaccgcagtgtttcccgtatagaaaatgtggtcaaatcgctgcttcaggagctccgtggtttcctcaacaccaccattaataacaatatagagatcctggtctaaatactgagggagaagctttgccaagatcttggctgtattttcactcagttcagaaggctttataatcacagcatttcctgcagcgatggctcctatcagtggctgaatggtgagaacgaaggggtaattccaagctccgattatcagcaccactcccagaggctgtggctgaatataggcctcatccagcatggtgagcacgttcttcttaactggtttagcagtaacccattcaggaagattctcaagcataaaatcaatttccccaaggacagtaatgacttcctgactgtacacattgaattcactcttgcacaggtcggcggcgatggccgtcaggatatccttctcgcgctcctgcaccatcctccgcagggcctccagctgctgcagccgaaaccgcagaggtcgcgaccggccggacaggaacgcctgtcggacccgccggacttcgagctccatggcctggtcctgcagagaactgcacggtccgggggcgagccacaattcactcgcccagggctcgctcgctcagccgcgacctccacgcccgctgagtcccactgccagtcggaggcgccgggggaggact

SEQ ID NO: 13378 - RNA, 2459 nt, Homo sapiens
  source 1..2459: mol_type = other RNA
gctgggattacaggcatgagccaccacgcccggccacagtattttttaaatgccagttaggttttataagatgtagaattctataactccaacacaagaatgacaggtgatgcttgcatgactttggcaactaacttccaggaagccctaggatttacaagatgctttgagtgacattagtcacaagagattgttgcaactaaacagaacacaggatgataaagaatgaatgaggaagaatgaagaccactggtgagatggcacttctgaccaggggcctactcctggaggtcaagtccttgagtcccattggaggaggagtaacccctcccttccccacatagagttttagtgcctgaaacctcacagggaaccaagaagatctaatctcacctctctggactacagaggactgccggtagccctgggaagtaccaagctcttgaaagcttcacacagtgatggtggcagcagaggcaggaagtgagcagtgccattaactggagtgaaggattcagtgaggttctgagactcccttacaaccccgcagtttgtatttagtctaatacattctcctcccctagctcaaagttccaagatttagataagcacaatttaagacaggttccctgaataccctattagggaatgttgggacgtagttgaaatggcaacttttattaatgatgaatggcaatgacttttaagtttgatcacagagtgtttgcatattttcttactatttttggtatgatttaaaaattattggttcattaaccatttaaaagaggaataattcagtagaggcactaggaggttgaacaggatcattcttcagtaatattctgccttgacaagcacagcggctacaatacccaggaaagtgagcaacaggagaccgagtttttctttgttgaaccgtttcaagagaaaaaattttccccaatccacctttgactggctgttgggaggatatctgagtttgttagcaccttctctctttaaactttttaataaacagggacgctgatgagaaaaagtatcaaaactatgttttccgtgataagctcccatcccactggaacccactcctccaaatgggaaagagttgagcgtgaagtgcataatgacgtcattgcctgtgacacctccactggatgtctcatcaatcatccgtttgatgagcttatggttatgcgaaaatacataaagagccagaggcttttcacgttcatttatgaaatttatggcctcatctacatttttcacaggcactattggaagaattggtccaaaaatttcttcttgcatcaccttggttttaggatcaacatcggtaagtactgttggggctatgtagcgtgtggcctcatcagtctccccaccaaaagctatcttttgtccttcaagcaaacttagtatcctcttaaaatgacgaagattgatgatcctttcataatcaggagactcttttatattttctccataaaattccttcactgtttccttaatcttccatacaatttgattttggagggatgcttcacagagaatatagtcgggtgcaatgcaggtttggccacaattcatgtattttccccaggttatgcgtctgcaaacaatgtccaggtcacaatctttatcaatataacatggacttttccctcccagttcaagagtcacaggggtcagatgcttggcagcagcttccatgacaattttgccaaccgcagtgtttcccgtatagaaaatgtggtcaaatcgctgcttcaggagctccgtggtttcctcaacaccaccattaataacaatatagagatcctggtctaaatactgagggagaagctttgccaagatcttggctgtattttcactcagttcagaaggctttataatcacagcatttcctgcagcgatggctcctatcagtggctgaatggtgagaacgaaggggtaattccaagctccgattatcagcaccactcccagaggctgtggctgaatataggcctcatccagcatggtgagcacgttcttcttaactggtttagcagtaacccattcaggaagattctcaagcataaaatcaatttccccaaggacagtaatgacttcctgactgtacacattgaattcactcttgcacaggtcggcggcgatggccgtcaggatatccttctcgcgctcctgcaccatcctccgcagggcctccagctgctgcagccgaaaccgcagaggtcgcgaccggccggacaggaacgcctgtcggacccgccggacttcgagctccatggcctggtcctgcagagaactgcacggtccgggggcgcgtcccagttccctggagagctagtccctgagggcgggaagccggggttcgtctcccgcggagccgggacagcggtcatttccttcttgcacaagcatcatcctcgcacgtccgttactcagagcttctc

SEQ ID NO: 13379 - RNA, 2513 nt, Homo sapiens
  source 1..2513: mol_type = other RNA
gctgggattacaggcatgagccaccacgcccggccacagtattttttaaatgccagttaggttttataagatgtagaattctataactccaacacaagaatgacaggtgatgcttgcatgactttggcaactaacttccaggaagccctaggatttacaagatgctttgagtgacattagtcacaagagattgttgcaactaaacagaacacaggatgataaagaatgaatgaggaagaatgaagaccactggtgagatggcacttctgaccaggggcctactcctggaggtcaagtccttgagtcccattggaggaggagtaacccctcccttccccacatagagttttagtgcctgaaacctcacagggaaccaagaagatctaatctcacctctctggactacagaggactgccggtagccctgggaagtaccaagctcttgaaagcttcacacagtgatggtggcagcagaggcaggaagtgagcagtgccattaactggagtgaaggattcagtgaggttctgagactcccttacaaccccgcagtttgtatttagtctaatacattctcctcccctagctcaaagttccaagatttagataagcacaatttaagacaggttccctgaataccctattagggaatgttgggacgtagttgaaatggcaacttttattaatgatgaatggcaatgacttttaagtttgatcacagagtgtttgcatattttcttactatttttggtatgatttaaaaattattggttcattaaccatttaaaagaggaataattcagtagaggcactaggaggttgaacaggatcattcttcagtaatattctgccttgacaagcacagcggctacaatacccaggaaagtgagcaacaggagaccgagtttttctttgttgaaccgtttcaagagaaaaaattttccccaatccacctttgactggctgttgggaggatatctgagtttgttagcaccttctctctttaaactttttaataaacagggacgctgatgagaaaaagtatcaaaactatgttttccgtgataagctcccatcccactggaacccactcctccaaatgggaaagagttgagcgtgaagtgcataatgacgtcattgcctgtgacacctccactggatgtctcatcaatcatccgtttgatgagcttatggttatgcgaaaatacataaagagccagaggcttttcacgttcatttatgaaatttatggcctcatctacatttttcacaggcactattggaagaattggtccaaaaatttcttcttgcatcaccttggttttaggatcaacatcggtaagtactgttggggctatgtagcgtgtggcctcatcagtctccccaccaaaagctatcttttgtccttcaagcaaacttagtatcctcttaaaatgacgaagattgatgatcctttcataatcaggagactcttttatattttctccataaaattccttcactgtttccttaatcttccatacaatttgattttggagggatgcttcacagagaatatagtcgggtgcaatgcaggtttggccacaattcatgtattttccccaggttatgcgtctgcaaacaatgtccaggtcacaatctttatcaatataacatggacttttccctcccagttcaagagtcacaggggtcagatgcttggcagcagcttccatgacaattttgccaaccgcagtgtttcccgtatagaaaatgtggtcaaatcgctgcttcaggagctccgtggtttcctcaacaccaccattaataacaatatagagatcctggtctaaatactgagggagaagctttgccaagatcttggctgtattttcactcagttcagaaggctttataatcacagcatttcctgcagcgatggctcctatcagtggctgaatggtgagaacgaaggggtaattccaagctccgattatcagcaccactcccagaggctgtggctgaatataggcctcatccagcatggtgagcacgttcttcttaactggtttagcagtaacccattcaggaagattctcaagcataaaatcaatttccccaaggacagtaatgacttcctgactgtacacattgaattcactcttgcacaggtcggcggcgatggccgtcaggatatccttctcgcgctcctgcaccatcctccgcagggcctccagctgctgcagccgaaaccgcagaggtcgcgaccggccggacaggaacgcctgtcggacccgccggacttcgagctccatggcctggtcctgcagagaactgcacggtccgggggcgctggggagtgggaggcgggaagcatgcaggtgcaggcctcgcctcccttccctccgcctccctccggggggtgtctccaccgtcaacccacagccacaattcactcgcccagggctcgctcgctcagccgcgacctccacgcccgctgagtcccactgccagtcggaggcgccgggggaggact

SEQ ID NO: 13380 - RNA, 2568 nt, Homo sapiens
  source 1..2568: mol_type = other RNA
gctgggattacaggcatgagccaccacgcccggccacagtattttttaaatgccagttaggttttataagatgtagaattctataactccaacacaagaatgacaggtgatgcttgcatgactttggcaactaacttccaggaagccctaggatttacaagatgctttgagtgacattagtcacaagagattgttgcaactaaacagaacacaggatgataaagaatgaatgaggaagaatgaagaccactggtgagatggcacttctgaccaggggcctactcctggaggtcaagtccttgagtcccattggaggaggagtaacccctcccttccccacatagagttttagtgcctgaaacctcacagggaaccaagaagatctaatctcacctctctggactacagaggactgccggtagccctgggaagtaccaagctcttgaaagcttcacacagtgatggtggcagcagaggcaggaagtgagcagtgccattaactggagtgaaggattcagtgaggttctgagactcccttacaaccccgcagtttgtatttagtctaatacattctcctcccctagctcaaagttccaagatttagataagcacaatttaagacaggttccctgaataccctattagggaatgttgggacgtagttgaaatggcaacttttattaatgatgaatggcaatgacttttaagtttgatcacagagtgtttgcatattttcttactatttttggtatgatttaaaaattattggttcattaaccatttaaaagaggaataattcagtagaggcactaggaggttgaacaggatcattcttcagtaatattctgccttgacaagcacagcggctacaatacccaggaaagtgagcaacaggagaccgagtttttctttgttgaaccgtttcaagagaaaaaattttccccaatccacctttgactggctgttgggaggatatctgagtttgttagcaccttctctctttaaactttttaataaacagggacgctgatgagaaaaagtatcaaaactatgttttccgtgataagctcccatcccactggaacccactcctccaaatgggaaagagttgagcgtgaagtgcataatgacgtcattgcctgtgacacctccactggatgtctcatcaatcatccgtttgatgagcttatggttatgcgaaaatacataaagagccagaggcttttcacgttcatttatgaaatttatggcctcatctacatttttcacaggcactattggaagaattggtccaaaaatttcttcttgcatcaccttggttttaggatcaacatcggtaagtactgttggggctatgtagcgtgtggcctcatcagtctccccaccaaaagctatcttttgtccttcaagcaaacttagtatcctcttaaaatgacgaagattgatgatcctttcataatcaggagactcttttatattttctccataaaattccttcactgtttccttaatcttccatacaatttgattttggagggatgcttcacagagaatatagtcgggtgcaatgcaggtttggccacaattcatgtattttccccaggttatgcgtctgcaaacaatgtccaggtcacaatctttatcaatataacatggacttttccctcccagttcaagagtcacaggggtcagatgcttggcagcagcttccatgacaattttgccaaccgcagtgtttcccgtatagaaaatgtggtcaaatcgctgcttcaggagctccgtggtttcctcaacaccaccattaataacaatatagagatccttcaacctctatcttctggttctacgtcctattcaatccttgacatctcactgtcttccatttcatctttcttgattggatcatcacagctattagaacaaaatggctctggtctaaatactgagggagaagctttgccaagatcttggctgtattttcactcagttcagaaggctttataatcacagcatttcctgcagcgatggctcctatcagtggctgaatggtgagaacgaaggggtaattccaagctccgattatcagcaccactcccagaggctgtggctgaatataggcctcatccagcatggtgagcacgttcttcttaactggtttagcagtaacccattcaggaagattctcaagcataaaatcaatttccccaaggacagtaatgacttcctgactgtacacattgaattcactcttgcacaggtcggcggcgatggccgtcaggatatccttctcgcgctcctgcaccatcctccgcagggcctccagctgctgcagccgaaaccgcagaggtcgcgaccggccggacaggaacgcctgtcggacccgccggacttcgagctccatggcctggtcctgcagagaactgcacggtccgggggcgcgtcccagttccctggagagctagtccctgagggcgggaagccggggttcgtctcccgcggagccgggacagcggtcatttccttcttgcacaagcatcatcctcgcacgtccgttactcagagcttctc

SEQ ID NO: 13381 - RNA, 10702 nt, Homo sapiens
  source 1..10702: mol_type = other RNA
gctgggattacaggcatgagccaccacgcccggccacatgtgctttttaacatttttattatttcatttttggagtcattattatttttgttacaccacacaaattgcaataacattaagagattgagatgatgatggtatgagggtggtgttggtgatgacagtgatgatgacagcaatgttgctgatgttccatagtggtaatggtgaagatgatggtgatactggggagatatgatggtggtggtgatggaagtgatgcttacattacaagtccactctacacacacatgttctttacaaatgtggatgaaccctatctcctgcatggagtgggcagcacagattgtggaggaagctgttttccttccctggcatcttctgttcttggaaatcaatgaatgtccttcattattttccccatagttcctaagaggatactttcctgcttctgaaacattcactatttctataaagtcagtttgtcttcattctgtaagctcctcagcaaccctcactatttgccatgatgctggtcaccgggcctacaagacatagatcttgtctttgaaaagcctgtgttcctagggagagaaacatctgaaaagtgaaagaacatgagagcaaaatagcatgcatactgcattagaaggtgcaccctcattccgcacgggtgtgtcagggactggcagggtcggggatggcttccctgggaaggtgcctttcaagctggccagtgactaaggggtcactcatcctccagggaatgggtggatagagagcactctaggccacaaacaaagcagagaatatacactgctgtagggtatgatctgagggatatgggagatttcaggggaaagagcttactttaagttttttgaagtgataaaatatttgaattttatcttggaagaactatggatccgttaaaggtctctcagcgtaggaatgaaatgagctgaatctgcatgttacgatgtttcctctgtagagcctaaccccctccacttgtgttcccaagagccccagcatcactcaggagcttataagaaatgcagagtcccaggccccattgctaaacctcttgaataagaatctgcacttttcaaaagtttcattttctaaattactatacagtaaatttaattttttatttttggtgtaaagttctacgaatgttagtatatgtgtcaatttgtatagccaccaccataatcaagatacagaacaactctgccccaaaaactatcttgcattatcctttatgatcacacctatcacccctacccactaataaccactaatctgtcctctgtcactacagttttacctatccaaggaagtaacataaatgaaattgatataatatgtaacctattaacgctggcttttttaattgagcaaaatgttgttgagattcatccaagttgttgcttttatcaatagttcattcttttttgctactgcatgtattcatggtaaggatgtatcacagttgttttagccattcacccactgagattcttcctagttttgggtaattatgaatagagatgctacaaacatgtatatgaatgttttttctgtaaacttaagttttcatttccctagggtaaatatctagacattgaatttctggtaatatgctaagtatatgcttaattttataagaaaacttctaaactgttttcctgaatagcaacattgttttgcattcccattagtaatgtctgagagttccagttgccccccatcctcatcactacttggtattgttggtatttttatttcagccattataataggtgtgttcacatctcatcattgcttacacttgcatttccctaatggctaaagatgctgatgttctttttctgagcttatttgccatccaaatatcctctttgatcatgtgtctattcaagtcttttgcccattttccagttgggtagcttgttctcttcctgttgaattttgagagttctttatatatcctggctataaagccttctgtaatatatgtgatttttaagtattctctcccattatgtagcttatcttttcattctcataatagtatctttcacagaataatagtttctaattttgacgtgtctaagtgatccatttttcttttgtgaatcatctttttggggtcatgtctaacttacctaagttcagatcagaaagattttctcctatgtgtttttatcaaagctttatagttttacacttatatctgtgatccactttgagtcaatttttgtataagacatgaagtttaggttgagctttttgttttgttttgtttcatttgcccttggatgtccaattgttccaagaccattgtagaaaagactccttctccattgaattgtctttgtacctctatcaaagcaattgaccatatttgttgtaggtctatttttggactctagtctactccattgatctatgtgtctatccctttgccaatatgacactgtcttgattactatagctttatagcaagtgttaaaatcaggtagggcgattggtgatttcttcaaatatacacttctttttcaaaattattttacctattctagttgctttgccttttcacataaattttagaaattggtttgtttatatctgcaaacagtcctgcttagattttggttggagttacattaaatctgtagagaaatctgggggtgagctggcaccattactaggatgagtcttccagtccatgaacatggtatgtcttgccatttctctaggtcctcagaatctgcatcttaacaagaatcccaggtaatttccctgtacattagagtctgggaagcacagctctagagtggaaatgacagtgaagtcatctgggaggatttacaaaatatggaagcctagacctcactcagaccaactgaataagaatctctgaagggggacctaggtgctggaattttttctatgtcttgtaggtgattctaactggcagccatgtgtgaacctctactctaaacccagtctgggctcttgtggctctggccctatgctcattaaatcaatctgattaaggccatcagttcattccttttcaaccctagatgtatattggaatcctttgaggatagaggttacttcaatgagaattttcaagaaaaaattctagttgacagattcaccaaacttcctctgaggccccacctatatttgaggattacctttccctgcccaaccccaggagctagaacaacattccagaagttttaactctcaactctaaaaacctgctctctttttggaagtctctctacaagttactgaggcaggaggagacagaggagagagggaacatgtgtgcacacaagagaaatgtccaattgaatgagtctgatcaataagatctatgactcaaaaatacttgcttcatggcaagggaacatcttttgctttcatatccatctcacatacctgctgagtcaaggaaacagctccatatttaggagaaaaatcctcttctaatctctaaatgcaatcgaaggttttctatgtctttttctgtggctccttggaaatgttaaaggcatgtctcagctacagcaaggtggggcatgacatattgccccccaaaatatgaaccaattgaatgtcgtctgaagtcagctctgtttctgttatcttttaatggattttaggtaaagaagtgttgatgtagataaaatagatataaaaccaaattcttctgctttggatgtgcaccaaccccagcaggctaaaaatagattcaactgcatcaataatatttctctttaaagttgcaggtcctttgggggtttggaaacattcagagaggataaaaggggagaaagatatgaaaacagcagaagctgcagtctaagcctccaggtgggggccttggggacagccatgctggaatgcctgatttttacatgtccaagtacctatttcctaccaaaaaaaaagcccttccacatatgataagaacacatcttttcttgcagggctgtcaagttcattctaaacacccctgccgctgcctgtttgagattgatgcctctccaatctctagctctttgtttgaaattaaacatccaaagacctttagaataaaaaaagtcaacatacaaatgaaatgcatttcaacatgcatctcaactgcagaaccacagcatgttgagactggaccaagcaaaccctgaagaagtttcccctcttgctcctctgtggtagatgacctatccaagttcacacaacaggtaacatggagcatgtggagagactcagcataggccagtgcagtagcggggtctactggaaaagacttggcctttgaagtctcattccaatcccagccttgcattgaccaactctgtgaccttgaccttgaaaaagtagagtcacagtgccctctacttcacagggttgtttggagaattactgaaaatgtgcacaaaatacctgatacacagtggggcactcagctaacaccagtcattcctgtaatccaggtctcccaacttctagtccagtgctctttgcacaacaacaccatatgaagactctgagctatccaaataagtgcacttgaaccacaggttaaatccccttcctctcatcagaaatacaggctagcaccgcccagcgttctttaaagacagccaggaaaacaaaccaaattcatactacttacccaacactgaacgagacacgctggctccctttcctttattttgtttcccttctatttgtcctgggtttgtggttctcgggcaaggtgaactctgctcagtatgatatgtgacccctggccacagttgcatatggccctgcctcagttgctgcctgctccttacttgattctccaggtccacactcctttcctgtgccatcttcccctgtggcacctgtgtgtaggaatcttcaacagctgcaccgccaacagagaagccacaagctggagccccacaagtttccccccaggccccatgcatgggtcagcagtcttgacccctgggctgattttaatattttaattaaattgacaacatgtaaaaaatctggagatttcacaacaatgcagatttctgacttcttttgacaaattacaaactggccaaatgtccacagctggccagagctgtgaggcagctgctcccttcatctggaaagactcttgctccactggtcaaagtccccaccggtcccctcattgcaacctcaccattccctatcaacctctgagttttccacccctgttatgatatgcacttccagttctccagctggacactcaagatgtgtcaccacatggcccactgcacttattcaatctcttctcctgggaaccctggaaaatctctctgcttctaggctctgctgggagcaattcccctcctacaatgtcctccttgctcttttatttatccaacccaatcaagagtatctctgcttaaaaaattcttgctgaccacccaagccacaaagagctctcctttccttaaagcatggagtcaacagttatcttacctaccttcacatagttggttcttcctgtttgcacatcctgtttccctagctaaattgtaaacttcttgagttcacatttgtttgccttccccagaaggcagccacagactttccaaagggaaagttctgaacaaagattaattgtttggtcaggagctatcaaccatatcatcactcagtgcaagaccagtctctccagcctcttttgcctccactccacttcccttgttcccctctcaaatccacccaaacccccatcctcctggaatcactccaaaaggactagaatttgtttcctgttttgcccacgattgttcccatcgctgccactccccagggctaaacacagaacctgccacataacaaaagctcagcatatgcacattaaatggaaagtgccttactttttagtccctatatcttaacatctgcagttcaccaggctgaccatgcccttctcccttttcaccaacagatctacgggtcttggaaatcccagttcagtgttcctctctcaatctttttctcttcctttactcagccaagtcactcctctctctaggcgccgcagtcctttgctcttgcctgccacagccattgccaaatgttggtgcaattgtttgcccacacctgtttttcccttggatgccaaggtcttccggatccaggattgtgtgatcttcttccatgcgcttgcctggttccccaagtcataactggacataattagtctggtggagaaggcaagtattatggccctcatttttccaatgagaaaatggaagcaaggcaccaggctccctgcatgcagcagagagatggaagaggaagagaggagcagcttgggtgagaagacttggttctattagcaggggtcaagcaatggaatggaaatgtgtcatgtcctttcaaggtcatctgtggagcaatgtttaacagcctgcccaagaaatatttaattacctagaggaaagtaagtacctttgttgacttgatatttgctaccaactaaatagccagattatgtgaagttacacattaatgtgtaggattttgcctagtagaaatacaaatgttttctgttcaggagaaaagataatctcaaagtttattaattgactcccgtgtaggacattaaccagttttgtttctaatttagcaatctcattccaacactcttcctccagtgcctatgtaaactcatgctgccatcttgttggtttcctcattaatgagctaaatgcatttttgacatgtccacattctagatttgtatgagtcacaattttaactttttgaaaattatactttgccacccaggtgccaccaactctgggagtgtgagcaagtccctccctcccctcttctggactcagtttcttcaacagtaacatgagggcgtaggtctgcatgggaaattacaagccccaggaatatttgattttaagcctgaatcttaaaaagaataatttcctcatagggttgaacatcttacggagttattttccaaaataacaacaataatgggacagtgcttcatacctggggctaagtattttaattctcacataatgagatggggctattgttcctagctctattacaggtgaggttaggaaagctgaaacagtattttttttaacgaggagacactatgtttgtccttccactcatgtttccttccattcttcttttcacctgtctggtcatccatgtttccagtcatccatcccactgatgcaaaaagaaggtggtttccattttcactctggatctatctaattgactatttaattgatgtggactttagtagaggcagtgattgcttccagttggtgggcccaggaagactgtgaaaaaggtaccactttcagcttgaccctgaaggttcaagcagaattatttagggataggttgaagaagcatctttgcctgaaggaaccatggcagggacaccagaagacaaaggagggagacatgcacagtgaccagtgggtggttatggctgtgggaagggtggataatgggagatgagatgaaaaagattgattggtcttggcatatgtcaatggctgattgagaatcttaagtttccttgatctgaagccctgtccacaatcacccagactctgagtacttcatgtggtagtaagaggcagagacaaacccttccccaggtgccctgatctggccaagcctgggcgctctgactaccagagtcctgaactcttagaagggagagctgcaaacaaccatggcgggaatctactccagcctcccttcccgaacatgtgggcctgagctaatttaagctagtctgagctcactttgcaagcagttgtcacaaggtgctacatcaaaagactcccaaggcccaaatatttaacaaccagaacactccctccatccatcagtttggtaattctatccacacaaaaaaactattggggtttcatttctggcctgctcatttcttataaacatgccagggccatttacagctcacaactcactgctctctaaacatttacacatttctccctcttaacacatccttggctatttgattaagtagtagatcacaggggatggaaggcaaggccttggcatctttgggttttctccaaacctatcttgacatgggttcaatgccagcctccccttccagtaaacacaaggattattgcactcctgggcacagacttgctgatgccttggtcttttctatcccttctcttgcagtttctttaggtaggagggaatacaaaccccaaaaacaaacagacatgagtccattttaccagctgggtttaatgggaaagctggtagggttccccatgacccctaggactgaatgagtgcccacatttcacaacaccctgattccagacaggaagcttggagaagtatctatatttgggggaaggaagctgccccagacacagcttcctggactgttagcaaaggaatctcacacaaggcctaaaccagtttccatacaacttccttgccttttgggaaggtgcaatctcacaggactggtgggacttacccaatgcagtcatccaaaaacagttatggccaacacctaagtgctgagaaaagtcaagaggaagaggaagccccaagggcagagaaagtggtgaaggtcacagaaaaggcatggagctgtggcaccattggcgggggacagctagagtccaggcacagagctaaaactgggtatgagcaagggtaggagaggggacactgctgaacacccacaatggtcctgctcctgttggctctgccttcaatctcaaaggcaattatgaataaaggaaagcacactgccttcagagtccgacctaagtttgaatcctggcatctttcccagctggccgtattacccctaggagctactcaacacttcagaacctcactttcttcttcagcaaaacagaggtgcaggtatatatctcctaggagtgacaagggaattcacgcggctgttaatgacctggtgcctgcctggggctaccaagcagccaccacaagagtcctccataatagcatccaccgcactgcagtcagggcaacagcactgcaagcacttcatggacagagaccaagcctttccaacttgatctgccatgtttcaacacagtgcctcagccattgagaaaatcctgtgacaggcacagacccccttcaagaaggacttgctgctcagctcgtgagagggttgtcagcagcttcttcagggcttgctcagttgcagagagctacctggccagaggtcatgcccttcaggggcagcccacctcctctgagtgatgggagtgatggaataaaggcccatgtcagcccatcccagcactcattccagcacaatgctggcaggccatcttggtgctcttggggctggctgtggctgcatccagcctgcatcacgactcaacctctgcacagtcctgctgccttcccctcctcccgtgggtatgagcctccagcacactcaacttcgtgtcagagcttaccttccaagaaccctacctgcaatgaacttggtatttgttgatgagtaaatgtctgaaacaagatccccaatcttctaaatccagagttaaaactcagacaggccacggtccttggtcattctaggtccaagaggctcttgctgcaggactctgccagtcagtgtctgggcggatatcatcacccccgcccagtccttcacggaggtcatccagccgacctcggcggccactgcctcctctttttcatccactggtttgagagtgccatccgcctggcttgagccattgttaatcttctgggcctcctctaatgtggttccagttgagtcaccatatttcttgtgaacctccaaagcactggaagacttctgggcctcgcgtggctgcaggtgaaacatacagccaatcactccaccctggagtcttggtttcctccccttcgtcttgcccccgcagtggcagcacacggtccacaggtacttgagcgtccgccagagcaagatgatgaagaggcccccgaagaaagtcaccatggaggaggccaggaaagcccaccacatgcgttggccccggctgtcgcacggcacctccatggtcaccgggatgatgagcgcatccatcttgggctcgtggaccgaggacgaggaggaagaggaggaggaagaagaagaagaggaagaggaggaggaggaggaggaggacgcgtctaggctgagatggttcgcgtggatattgctactcattctaagactgctgcctccgccgccgccgccgccgccgctgctgccgccgccgccgccgccaccatttgccatagctagcaacgggcagccggcgcaggggctcgggggagctcctcccgccgccagcgccaccccaaacacccatcaacagccatattgctgctactgctgccgccgccgccgccgccgcggagcgcgggaggggggcggggaggcgcctgggctcggggcgctgtgcgcgacctggcggggtgcgccgagatatatacagcgagccgccgccgcccgcccgggggggagggggatggagtgcgcgggcagctccccctccccggcccgcgccccgctcgccccgggctgcgctggccccgagcgccgagagccagggggcgccgcggg

SEQ ID NO: 13382 - RNA, 6501 nt, Homo sapiens
  source 1..6501: mol_type = other RNA
gctgggattacaggcatgagccaccacgcccggccagaagtgattcttaattaggttccttagaatctaaggttctacccctgtctccttatcctattctcaggaaggtggccattggcttttcttgtataaaagttatctgattttaagttatatgcctagtattcctggccacagttaactgaaccaacggactgacagccgggcataagacctctatctagtaggaatactgcacacaggctggttactagctgacttaactagagcctctatgggaagtctaaacatcaaatagaaaggagcagaaacagagatagcaggagaaaaagcagaaaaagaatagtaaggttataaaaatggcagtcgcaaaccctatggtattgaattaaaaccgtatctaaactcatgatttttatttatttttaaaaatatgaaacggagtcttgctctgtcactcaggctgcagtgcagtggtacaatcacagttcactacagcctcaaccttctgaactcaagcgatcctcctgcctcagcctcctacgtagctaggattacaggaatgcaccaccatgcctggctaattttttattttttaaacgtttggaggatgaggtcttgctatgatgcgcaggctggtcttgaactcctgggctcaagtgatcctcccactttggcctcccaaagtcctgggatacaggcacgagccaccatacctggctcacggtttttaataacatacagatggatagaataataaattcaggtgcttgtatttgcatgttttaacatatatacatatatgttttctagctctgtctgctgagcaggcctacaagcaatgacactccgccaatgatactctagccaggagtatatattctgtccagatcttggtttccagtggcatcaagaaacaacttggtttctaagttccttttttctggaataaaaggaactgggagcttcttagagaatgactgatgccagggctgagatagggaaaatgtgaggaagcctgaaacatcttgtggtgccagaaaatgcttaaaaagtgacaggggcaatgtcgaaacaacacagtgccaacttcaatgagttctcactggccaaatctgagccaatttgagcaaccaaataaactgttagcattagattgtagcctgtagaataaaacagatatccactcattcatactgatataaattatcaaataaataaatggggaaaagggacagctcttccttatagtagaataccaattaataaatacaggtaaaataatgaaacaaagtcaccattaggcaagcataacattaatacctgttataagcaagaatcattgatgatggaaatgaaaatcagtaggcaaaattttaagaataagacattcacatagcttcaaagtggaagattcttgttaatttcaaagggaaaattcctaattttacagtggagaaacctggcacacaccaccttagccatgtgatcaaagttaccaccacctagtctaggtgtggtggctcatgcctgtaatctcagcactttgggaggccgaggtgggtggatcacctgaggtcaggagttcaagaccagcctggccaacatggcgaaaacctgtctctactaaaaatacaaaaattagctgggtgtggtggtgggcacctgcaatcccagctactcaggaggctgaggcaggagaatcactttgaacccaggaggcagaggttgcagtgagccgagattgcgccactgcactccatcctgggtgacagagcgggactccgtctcaaaaaaaaaaaaaaaaccaaaacaaaaagttaccaccaccctccgctaggaggcactaagaatagcacagtatcacttctgtggttgtcttggcaaaaatgcagatcctcaatcatatcatgtaaaaacattaaacaaactaaaactggggaatattctataaaataactggcctggactcttccaaagtgtcaaggtcatgaaagataaagaccaagaaactgtcacaggctgacagagatgaaggaaacaccacaacaaaatgcaatatgggaccctggaccagacaaaggacatcatcgggaaaactggcaaaatttgaatgtccgtagattagttagtagtagtttatcaatgttaacttcctggttttctttttttgagacggagtctcactctgtcgcccaggctggagtgcagtggcgtgatttcagctcactgcaacctccgcctcctgggctcaagtgattctcctgcctcagcctcccaagtagctgggattacaggtgggcaccagcgggcctggctaatttttgtatttttagtacagacagggtttcaccatgttggccaggctggtctcgaactcctgacctcaggtaatctgcctgcctcagcctcccaaagtgctggaattacaggcatgagccaccacacccggcaatttcctggttttgataaactacagtatggctttgtaggatgtaatcattgggagatgctagatgaaagatacatgggaattttctactatttctgcaactttctctaagtctaaaattatttcaaaacaaaaagtaaaaaacaatgaaaagcaggccgggtccagtggctcatgcctgtaatcccagcactttgggaggccgaggcaggcagatcacaaggtcaggagattgagaccatcctggctaacatggtgaaaccctgtctctactaaaaatacaaaaaggtagccgggcgtggtggtgggcacctgtagtcccagctactcgggaggctgaggcaggagaatggcgtgaacctgggaggcagggcttgcagtgagccgagatcgcgccactgcactccagcttgggggacagagtgagactctgtctcaaaaaaaaaaaaaaaaaaaaaaaggcagtcagtgaggtagggagcagcagcccctgaggggtagacagtgatccaagcatctgctggagctcacaccctggattctgactgcctcatacccaccatactgttaggacatgcttccattacccaagggactttgattcctggccccattctctgcttcctgaaagactagctaacactacgcgagggttccatgaagggcctgtgggggaaggtgggtggactgcttatcagcagtggctactgtagatggtgcccaaggatgcaccaggccttactgtgcctggctaaggtgggcttgaaacattggctggtctgtgaaatgcccttgggggacggtgtccagaccctctgctttgtgactaacatgcagactgaataaactgcatgtttattccaggctcgtttagctggacgagcagtacagacagggctgaggctgactccatggccatgtgggcagaggtcaaacccatgatctctcttcctacagcttcctaatgtctgcgatgttggtcttttgaaggaggcccccacagagctgagcttgcttggttatctgggactgctgctcagtctgagtaggggagggtaatgaaccagtcaggcctcctcctggaggtgcccaacactggcctagtccccaaggctgacgaaacatggtctggcctgaccccaggacgtggggtgaggaggaacactgggcataatatagtagcggaaacaggcaagcctctatgggtcccttccccttagaattttagggtagggaacgaggaggctacagactaaattgcagaactatctgcacctgggcctctgagctcttcctccactcccagtggagccattctggggactgagttgcatgaggactagcagagggtggcagttcagtctggtccctgtcttcttccagccagctgtgttcttagctgccatacttctgagcttcctgggaacatgagaaagtctggcgactatgggggatggggatcattctgaaggaaataagggacctccatccctccttgccttgaagggggtggaaaggcagctcctctcctgaaggcttgttagcaggttatgggcccacaacaaaggggccagagtagggcgaaattcctccttcaggttttggggctgagaaggggtcttcatgggctgtgaggaggtaagcaggcctgagactgggtagagatgggagcggcatgaggggaaggtaagtcagttgccatgccacagccaaggggcctttattggatggtgagggcacataggagcaggcaggtggctgctagatggtgttgcacaccttctcagggtgcagtggtgcccggatgtccagtctgcgagtcttgctgtccttgtcgatgatctccagacgcagcttggggaggcgcttctcagcctggggtgagggcagttctgggcttttgagtagctgcttgtctgagtcctccaccgtgatgcgcaaagtacagccccctggcagcaggtcctgctcataggctgctgccagctggttcaccacacggcgttctacctcatgtttgatggagcgggcgccatagtgcacattgtagccgtcgaccagcacatctgccacctcgcggtcccagagcagcgtgatgttgtgcctttgcttggctctcttggcccagaagtttagttccttgttgacgagttggatgagctccgagtggcagaaggggaggaagtagacgatctcattgatccgtcccagaaactcatccctccggaagtgagctttcaggatagggcgaatcacattctccttgaagttctttgagatggtgatcttgtcacttatctggacatcccccaggttttcggcaatacggttacggctcatctccaaagcttcctgcctcagctgcagcgcgtgctgtgcgatctcgtcgctggccacattggaggtcatgatgaagatggcgtccttgcaatcaatggtcttcccttttccatctgtcagccggccctcatcaaacagctgcagcatgatggtgagcacatctggatgggccttgtctacttcatcaaagagcaccacagcattggggcactgcttcaacttcttggtcagctggccaccctcctcatggccaacgtagcctggtggagacccaataaacttggccacctcgtgtcgctcctggaactcggacatgtccagcctgatgaagccctttttagcatctttgtgcatatatttggctgtctgcttggccagctctgtttttcctattccagatgatcccaagaagaggaagaccagagggtgttcttcatcgtaccagccattctccttcctccggatcgcagcacccactgtggcgatggcgctctcctggccaatgatgtgctcctttagtcgctgctccagggggaagcggcgccgctcctcagcctcacgcttccgctgcttctcttggtacttggcttcagaagtcctcagaagcttcatcacttccccttctcgggcataatccaagggtgtgtgtcccatttcattcctctgcagggggttggctcctccatcaagcagctccttgacagtgcggtagtcatcagcaagaacagcatagtgcaaggccgtgcagcccttgaaactggcgcggttgttcagcctgttgttgaagtcatcctctcgggtgatcaggacgccagcggggagtcctagccatctcctgaactccagggcacttgtccactggtttgtgatgtgccggcttgcaccgtcctgtcccccatcttccaaagaatggattccctgttccttggcagtcttgtaaacactgctgaaatcatctccaaggtttggatcagccccagcagcaagcaggacctgtaccacactgttgtttcggttgatggctgccaccatgagtgctgtccagccaagtctgtgctttgcattgacatctgcaccttctgacaacagcctgaggggccattcagaggaggaaatcttggtgttcttcagtgagactccagcattcagccctgcccagcttcttgactgagcatcattctttgcagtctcttggggctgctgacttcttgcatattgttggcacgggcagcttccaacagggctgcatccttgttggacggactcttgctgtagcaatgaaccaccagcgctgcggccagggcgcacatgcccagtccggccctgctggggaccccgttccagctgtcctgtcctgggagtgtttcttcgggaccaggaaggcgtccccaagtggcagccgcgaggcatttggtatcgaagcgtcctccctggcgccccccggtggctgccccacgtccggagaacaaggccggcgatgttccagggcgccccccggtggctaccctcagccactgcggctccccgagactcccagtagtcacattccggccggaagcacctccatggccccggagcgttggggacctgagcagccggaggagtagccgtggcgccagtgcttttctcctcaacaccagggaccccagcatcttgacagctgcttcgataaccccgtggtgccggcccctgtgctgaccacgtccaac

SEQ ID NO: 13383 - RNA, 6394 nt, Homo sapiens
  source 1..6394: mol_type = other RNA
gctgggattacaggcatgagccaccacgcccggccagaagtgattcttaattaggttccttagaatctaaggttctacccctgtctccttatcctattctcaggaaggtggccattggcttttcttgtataaaagttatctgattttaagttatatgcctagtattcctggccacagttaactgaaccaacggactgacagccgggcataagacctctatctagtaggaatactgcacacaggctggttactagctgacttaactagagcctctatgggaagtctaaacatcaaatagaaaggagcagaaacagagatagcaggagaaaaagcagaaaaagaatagtaaggttataaaaatggcagtcgcaaaccctatggtattgaattaaaaccgtatctaaactcatgatttttatttatttttaaaaatatgaaacggagtcttgctctgtcactcaggctgcagtgcagtggtacaatcacagttcactacagcctcaaccttctgaactcaagcgatcctcctgcctcagcctcctacgtagctaggattacaggaatgcaccaccatgcctggctaattttttattttttaaacgtttggaggatgaggtcttgctatgatgcgcaggctggtcttgaactcctgggctcaagtgatcctcccactttggcctcccaaagtcctgggatacaggcacgagccaccatacctggctcacggtttttaataacatacagatggatagaataataaattcaggtgcttgtatttgcatgttttaacatatatacatatatgttttctagctctgtctgctgagcaggcctacaagcaatgacactccgccaatgatactctagccaggagtatatattctgtccagatcttggtttccagtggcatcaagaaacaacttggtttctaagttccttttttctggaataaaaggaactgggagcttcttagagaatgactgatgccagggctgagatagggaaaatgtgaggaagcctgaaacatcttgtggtgccagaaaatgcttaaaaagtgacaggggcaatgtcgaaacaacacagtgccaacttcaatgagttctcactggccaaatctgagccaatttgagcaaccaaataaactgttagcattagattgtagcctgtagaataaaacagatatccactcattcatactgatataaattatcaaataaataaatggggaaaagggacagctcttccttatagtagaataccaattaataaatacaggtaaaataatgaaacaaagtcaccattaggcaagcataacattaatacctgttataagcaagaatcattgatgatggaaatgaaaatcagtaggcaaaattttaagaataagacattcacatagcttcaaagtggaagattcttgttaatttcaaagggaaaattcctaattttacagtggagaaacctggcacacaccaccttagccatgtgatcaaagttaccaccacctagtctaggtgtggtggctcatgcctgtaatctcagcactttgggaggccgaggtgggtggatcacctgaggtcaggagttcaagaccagcctggccaacatggcgaaaacctgtctctactaaaaatacaaaaattagctgggtgtggtggtgggcacctgcaatcccagctactcaggaggctgaggcaggagaatcactttgaacccaggaggcagaggttgcagtgagccgagattgcgccactgcactccatcctgggtgacagagcgggactccgtctcaaaaaaaaaaaaaaaaccaaaacaaaaagttaccaccaccctccgctaggaggcactaagaatagcacagtatcacttctgtggttgtcttggcaaaaatgcagatcctcaatcatatcatgtaaaaacattaaacaaactaaaactggggaatattctataaaataactggcctggactcttccaaagtgtcaaggtcatgaaagataaagaccaagaaactgtcacaggctgacagagatgaaggaaacaccacaacaaaatgcaatatgggaccctggaccagacaaaggacatcatcgggaaaactggcaaaatttgaatgtccgtagattagttagtagtagtttatcaatgttaacttcctggttttctttttttgagacggagtctcactctgtcgcccaggctggagtgcagtggcgtgatttcagctcactgcaacctccgcctcctgggctcaagtgattctcctgcctcagcctcccaagtagctgggattacaggtgggcaccagcgggcctggctaatttttgtatttttagtacagacagggtttcaccatgttggccaggctggtctcgaactcctgacctcaggtaatctgcctgcctcagcctcccaaagtgctggaattacaggcatgagccaccacacccggcaatttcctggttttgataaactacagtatggctttgtaggatgtaatcattgggagatgctagatgaaagatacatgggaattttctactatttctgcaactttctctaagtctaaaattatttcaaaacaaaaagtaaaaaacaatgaaaagcaggccgggtccagtggctcatgcctgtaatcccagcactttgggaggccgaggcaggcagatcacaaggtcaggagattgagaccatcctggctaacatggtgaaaccctgtctctactaaaaatacaaaaaggtagccgggcgtggtggtgggcacctgtagtcccagctactcgggaggctgaggcaggagaatggcgtgaacctgggaggcagggcttgcagtgagccgagatcgcgccactgcactccagcttgggggacagagtgagactctgtctcaaaaaaaaaaaaaaaaaaaaaaaggcagtcagtgaggtagggagcagcagcccctgaggggtagacagtgatccaagcatctgctggagctcacaccctggattctgactgcctcatacccaccatactgttaggacatgcttccattacccaagggactttgattcctggccccattctctgcttcctgaaagactagctaacactacgcgagggttccatgaagggcctgtgggggaaggtgggtggactgcttatcagcagtggctactgtagatggtgcccaaggatgcaccaggccttactgtgcctggctaaggtgggcttgaaacattggctggtctgtgaaatgcccttgggggacggtgtccagaccctctgctttgtgactaacatgcagactgaataaactgcatgtttattccaggctcgtttagctggacgagcagtacagacagggctgaggctgactccatggccatgtgggcagaggtcaaacccatgatctctcttcctacagcttcctaatgtctgcgatgttggtcttttgaaggaggcccccacagagctgagcttgcttggttatctgggactgctgctcagtctgagtaggggagggtaatgaaccagtcaggcctcctcctggaggtgcccaacactggcctagtccccaaggctgacgaaacatggtctggcctgaccccaggacgtggggtgaggaggaacactgggcataatatagtagcggaaacaggcaagcctctatgggtcccttccccttagaattttagggtagggaacgaggaggctacagactaaattgcagaactatctgcacctgggcctctgagctcttcctccactcccagtggagccattctggggactgagttgcatgaggactagcagagggtggcagttcagtctggtccctgtcttcttccagccagctgtgttcttagctgccatacttctgagcttcctgggaacatgagaaagtctggcgactatgggggatggggatcattctgaaggaaataagggacctccatccctccttgccttgaagggggtggaaaggcagctcctctcctgaaggcttgttagcaggttatgggcccacaacaaaggggccagagtagggcgaaattcctccttcaggttttggggctgagaaggggtcttcatgggctgtgaggaggtaagcaggcctgagactgggtagagatgggagcggcatgaggggaaggtaagtcagttgccatgccacagccaaggggcctttattggatggtgagggcacataggagcaggcaggtggctgctagatggtgttgcacaccttctcagggtgcagtggtgcccggatgtccagtctgcgagtcttgctgtccttgtcgatgatctccagacgcagcttggggaggcgcttctcagcctggggtgagggcagttctgggcttttgagtagctgcttgtctgagtcctccaccgtgatgcgcaaagtacagccccctggcagcaggtcctgctcataggctgctgccagctggttcaccacacggcgttctacctcatgtttgatggagcgggcgccatagtgcacattgtagccgtcgaccagcacatctgccacctcgcggtcccagagcagcgtgatgttgtgcctttgcttggctctcttggcccagaagtttagttccttgttgacgagttggatgagctccgagtggcagaaggggaggaagtagacgatctcattgatccgtcccagaaactcatccctccggaagtgagctttcaggatagggcgaatcacattctccttgaagttctttgagatggtgatcttgtcacttatctggacatcccccaggttttcggcaatacggttacggctcatctccaaagcttcctgcctcagctgcagcgcgtgctgtgcgatctcgtcgctggccacattggaggtcatgatgaagatggcgtccttgcaatcaatggtcttcccttttccatctgtcagccggccctcatcaaacagctgcagcatgatggtgagcacatctggatgggccttgtctacttcatcaaagagcaccacagcattggggcactgcttcaacttcttggtcagctggccaccctcctcatggccaacgtagcctggtggagacccaataaacttggccacctcgtgtcgctcctggaactcggacatgtccagcctgatgaagccctttttagcatctttgtgcatatatttggctgtctgcttggccagctctgtttttcctattccagatgatcccaagaagaggaagaccagagggtgttcttcatcgtaccagccattctccttcctccggatcgcagcacccactgtggcgatggcgctctcctggccaatgatgtgctcctttagtcgctgctccagggggaagcggcgccgctcctcagcctcacgcttccgctgcttctcttggtacttggcttcagaagtcctcagaagcttcatcacttccccttctcgggcataatccaagggtgtgtgtcccatttcattcctctgcagggggttggctcctccatcaagcagctccttgacagtgcggtagtcatcagcaagaacagcatagtgcaaggccgtgcagcccttgaaactggcgcggttgttcagcctgttgttgaagtcatcctctcgggtgatcaggacgccagcggggagtcctagccatctcctgaactccagggcacttgtccactggtttgtgatgtgccggcttgcaccgtcctgtcccccatcttccaaagaatggattccctgttccttggcagtcttgtaaacactgctgaaatcatctccaaggtttggatcagccccagcagcaagcaggacctgtaccacactgttgtttcggttgatggctgccaccatgagtgctgtccagccaagtctgtgctttgcattgacatctgcaccttctgacaacagcctgctgacttcttgcatattgttggcacgggcagcttccaacagggctgcatccttgttggacggactcttgctgtagcaatgaaccaccagcgctgcggccagggcgcacatgcccagtccggccctgctggggaccccgttccagctgtcctgtcctgggagtgtttcttcgggaccaggaaggcgtccccaagtggcagccgcgaggcatttggtatcgaagcgtcctccctggcgccccccggtggctgccccacgtccggagaacaaggccggcgatgttccagggcgccccccggtggctaccctcagccactgcggctccccgagactcccagtagtcacattccggccggaagcacctccatggccccggagcgttggggacctgagcagccggaggagtagccgtggcgccagtgcttttctcctcaacaccagggaccccagcatcttgacagctgcttcgataaccccgtggtgccggcccctgtgctgaccacgtccaac

SEQ ID NO: 13384 - RNA, 6217 nt, Homo sapiens
  source 1..6217: mol_type = other RNA
gctgggattacaggcatgagccaccacgcccggccagaagtgattcttaattaggttccttagaatctaaggttctacccctgtctccttatcctattctcaggaaggtggccattggcttttcttgtataaaagttatctgattttaagttatatgcctagtattcctggccacagttaactgaaccaacggactgacagccgggcataagacctctatctagtaggaatactgcacacaggctggttactagctgacttaactagagcctctatgggaagtctaaacatcaaatagaaaggagcagaaacagagatagcaggagaaaaagcagaaaaagaatagtaaggttataaaaatggcagtcgcaaaccctatggtattgaattaaaaccgtatctaaactcatgatttttatttatttttaaaaatatgaaacggagtcttgctctgtcactcaggctgcagtgcagtggtacaatcacagttcactacagcctcaaccttctgaactcaagcgatcctcctgcctcagcctcctacgtagctaggattacaggaatgcaccaccatgcctggctaattttttattttttaaacgtttggaggatgaggtcttgctatgatgcgcaggctggtcttgaactcctgggctcaagtgatcctcccactttggcctcccaaagtcctgggatacaggcacgagccaccatacctggctcacggtttttaataacatacagatggatagaataataaattcaggtgcttgtatttgcatgttttaacatatatacatatatgttttctagctctgtctgctgagcaggcctacaagcaatgacactccgccaatgatactctagccaggagtatatattctgtccagatcttggtttccagtggcatcaagaaacaacttggtttctaagttccttttttctggaataaaaggaactgggagcttcttagagaatgactgatgccagggctgagatagggaaaatgtgaggaagcctgaaacatcttgtggtgccagaaaatgcttaaaaagtgacaggggcaatgtcgaaacaacacagtgccaacttcaatgagttctcactggccaaatctgagccaatttgagcaaccaaataaactgttagcattagattgtagcctgtagaataaaacagatatccactcattcatactgatataaattatcaaataaataaatggggaaaagggacagctcttccttatagtagaataccaattaataaatacaggtaaaataatgaaacaaagtcaccattaggcaagcataacattaatacctgttataagcaagaatcattgatgatggaaatgaaaatcagtaggcaaaattttaagaataagacattcacatagcttcaaagtggaagattcttgttaatttcaaagggaaaattcctaattttacagtggagaaacctggcacacaccaccttagccatgtgatcaaagttaccaccacctagtctaggtgtggtggctcatgcctgtaatctcagcactttgggaggccgaggtgggtggatcacctgaggtcaggagttcaagaccagcctggccaacatggcgaaaacctgtctctactaaaaatacaaaaattagctgggtgtggtggtgggcacctgcaatcccagctactcaggaggctgaggcaggagaatcactttgaacccaggaggcagaggttgcagtgagccgagattgcgccactgcactccatcctgggtgacagagcgggactccgtctcaaaaaaaaaaaaaaaaccaaaacaaaaagttaccaccaccctccgctaggaggcactaagaatagcacagtatcacttctgtggttgtcttggcaaaaatgcagatcctcaatcatatcatgtaaaaacattaaacaaactaaaactggggaatattctataaaataactggcctggactcttccaaagtgtcaaggtcatgaaagataaagaccaagaaactgtcacaggctgacagagatgaaggaaacaccacaacaaaatgcaatatgggaccctggaccagacaaaggacatcatcgggaaaactggcaaaatttgaatgtccgtagattagttagtagtagtttatcaatgttaacttcctggttttctttttttgagacggagtctcactctgtcgcccaggctggagtgcagtggcgtgatttcagctcactgcaacctccgcctcctgggctcaagtgattctcctgcctcagcctcccaagtagctgggattacaggtgggcaccagcgggcctggctaatttttgtatttttagtacagacagggtttcaccatgttggccaggctggtctcgaactcctgacctcaggtaatctgcctgcctcagcctcccaaagtgctggaattacaggcatgagccaccacacccggcaatttcctggttttgataaactacagtatggctttgtaggatgtaatcattgggagatgctagatgaaagatacatgggaattttctactatttctgcaactttctctaagtctaaaattatttcaaaacaaaaagtaaaaaacaatgaaaagcaggccgggtccagtggctcatgcctgtaatcccagcactttgggaggccgaggcaggcagatcacaaggtcaggagattgagaccatcctggctaacatggtgaaaccctgtctctactaaaaatacaaaaaggtagccgggcgtggtggtgggcacctgtagtcccagctactcgggaggctgaggcaggagaatggcgtgaacctgggaggcagggcttgcagtgagccgagatcgcgccactgcactccagcttgggggacagagtgagactctgtctcaaaaaaaaaaaaaaaaaaaaaaaggcagtcagtgaggtagggagcagcagcccctgaggggtagacagtgatccaagcatctgctggagctcacaccctggattctgactgcctcatacccaccatactgttaggacatgcttccattacccaagggactttgattcctggccccattctctgcttcctgaaagactagctaacactacgcgagggttccatgaagggcctgtgggggaaggtgggtggactgcttatcagcagtggctactgtagatggtgcccaaggatgcaccaggccttactgtgcctggctaaggtgggcttgaaacattggctggtctgtgaaatgcccttgggggacggtgtccagaccctctgctttgtgactaacatgcagactgaataaactgcatgtttattccaggctcgtttagctggacgagcagtacagacagggctgaggctgactccatggccatgtgggcagaggtcaaacccatgatctctcttcctacagcttcctaatgtctgcgatgttggtcttttgaaggaggcccccacagagctgagcttgcttggttatctgggactgctgctcagtctgagtaggggagggtaatgaaccagtcaggcctcctcctggaggtgcccaacactggcctagtccccaaggctgacgaaacatggtctggcctgaccccaggacgtggggtgaggaggaacactgggcataatatagtagcggaaacaggcaagcctctatgggtcccttccccttagaattttagggtagggaacgaggaggctacagactaaattgcagaactatctgcacctgggcctctgagctcttcctccactcccagtggagccattctggggactgagttgcatgaggactagcagagggtggcagttcagtctggtccctgtcttcttccagccagctgtgttcttagctgccatacttctgagcttcctgggaacatgagaaagtctggcgactatgggggatggggatcattctgaaggaaataagggacctccatccctccttgccttgaagggggtggaaaggcagctcctctcctgaaggcttgttagcaggttatgggcccacaacaaaggggccagagtagggcgaaattcctccttcaggttttggggctgagaaggggtcttcatgggctgtgaggaggtaagcaggcctgagactgggtagagatgggagcggcatgaggggaaggtaagtcagttgccatgccacagccaaggggcctttattggatggtgagggcacataggagcaggcaggtggctgctagatggtgttgcacaccttctcagggtgcagtggtgcccggatgtccagtctgcgagtcttgctgtccttgtcgatgatctccagacgcagcttggggaggcgcttctcagcctggggtgagggcagttctgggcttttgagtagctgcttgtctgagtcctccaccgtgatgcgcaaagtacagccccctggcagcaggtcctgctcataggctgctgccagctggttcaccacacggcgttctacctcatgtttgatggagcgggcgccatagtgcacattgtagccgtcgaccagcacatctgccacctcgcggtcccagagcagcgtgatgttgtgcctttgcttggctctcttggcccagaagtttagttccttgttgacgagttggatgagctccgagtggcagaaggggaggaagtagacgatctcattgatccgtcccagaaactcatccctccggaagtgagctttcaggatagggcgaatcacattctccttgaagttctttgagatggtgatcttgtcacttatctggacatcccccaggttttcggcaatacggttacggctcatctccaaagcttcctgcctcagctgcagcgcgtgctgtgcgatctcgtcgctggccacattggaggtcatgatgaagatggcgtccttgcaatcaatggtcttcccttttccatctgtcagccggccctcatcaaacagctgcagcatgatggtgagcacatctggatgggccttgtctacttcatcaaagagcaccacagcattggggcactgcttcaacttcttggtcagctggccaccctcctcatggccaacgtagcctggtggagacccaataaacttggccacctcgtgtcgctcctggaactcggacatgtccagcctgatgaagccctttttagcatctttgtgcatatatttggctgtctgcttggccagctctgtttttcctattccagatgatcccaagaagaggaagaccagagggtgttcttcatcgtaccagccattctccttcctccggatcgcagcacccactgtggcgatggcgctctcctggccaatgatgtgctcctttagtcgctgctccagggggaagcggcgccgctcctcagcctcacgcttccgctgcttctcttggtacttggcttcagaagtcctcagaagcttcatcacttccccttctcgggcataatccaagggtgtgtgtcccatttcattcctctgcagggggttggctcctccatcaagcagctccttgacagtgcggtagtcatcagcaagaacagcatagtgcaaggccgtgcagcccttgaaactggcgcggttgttcagcctgttgttgaagtcatcctctcgggtgatcaggacttccaaagaatggattccctgttccttggcagtcttgtaaacactgctgaaatcatctccaaggtttggatcagccccagcagcaagcaggacctgtaccacactgctgacttcttgcatattgttggcacgggcagcttccaacagggctgcatccttgttggacggactcttgctgtagcaatgaaccaccagcgctgcggccagggcgcacatgcccagtccggccctgctggggaccccgttccagctgtcctgtcctgggagtgtttcttcgggaccaggaaggcgtccccaagtggcagccgcgaggcatttggtatcgaagcgtcctccctggcgccccccggtggctgccccacgtccggagaacaaggccggcgatgttccagggcgccccccggtggctaccctcagccactgcggctccccgagactcccagtagtcacattccggccggaagcacctccatggccccggagcgttggggacctgagcagccggaggagtagccgtggcgccagtgcttttctcctcaacaccagggaccccagcatcttgacagctgcttcgataaccccgtggtgccggcccctgtgctgaccacgtccaac

SEQ ID NO: 13385 - RNA, 6304 nt, Homo sapiens
  source 1..6304: mol_type = other RNA
gctgggattacaggcatgagccaccacgcccggccagaagtgattcttaattaggttccttagaatctaaggttctacccctgtctccttatcctattctcaggaaggtggccattggcttttcttgtataaaagttatctgattttaagttatatgcctagtattcctggccacagttaactgaaccaacggactgacagccgggcataagacctctatctagtaggaatactgcacacaggctggttactagctgacttaactagagcctctatgggaagtctaaacatcaaatagaaaggagcagaaacagagatagcaggagaaaaagcagaaaaagaatagtaaggttataaaaatggcagtcgcaaaccctatggtattgaattaaaaccgtatctaaactcatgatttttatttatttttaaaaatatgaaacggagtcttgctctgtcactcaggctgcagtgcagtggtacaatcacagttcactacagcctcaaccttctgaactcaagcgatcctcctgcctcagcctcctacgtagctaggattacaggaatgcaccaccatgcctggctaattttttattttttaaacgtttggaggatgaggtcttgctatgatgcgcaggctggtcttgaactcctgggctcaagtgatcctcccactttggcctcccaaagtcctgggatacaggcacgagccaccatacctggctcacggtttttaataacatacagatggatagaataataaattcaggtgcttgtatttgcatgttttaacatatatacatatatgttttctagctctgtctgctgagcaggcctacaagcaatgacactccgccaatgatactctagccaggagtatatattctgtccagatcttggtttccagtggcatcaagaaacaacttggtttctaagttccttttttctggaataaaaggaactgggagcttcttagagaatgactgatgccagggctgagatagggaaaatgtgaggaagcctgaaacatcttgtggtgccagaaaatgcttaaaaagtgacaggggcaatgtcgaaacaacacagtgccaacttcaatgagttctcactggccaaatctgagccaatttgagcaaccaaataaactgttagcattagattgtagcctgtagaataaaacagatatccactcattcatactgatataaattatcaaataaataaatggggaaaagggacagctcttccttatagtagaataccaattaataaatacaggtaaaataatgaaacaaagtcaccattaggcaagcataacattaatacctgttataagcaagaatcattgatgatggaaatgaaaatcagtaggcaaaattttaagaataagacattcacatagcttcaaagtggaagattcttgttaatttcaaagggaaaattcctaattttacagtggagaaacctggcacacaccaccttagccatgtgatcaaagttaccaccacctagtctaggtgtggtggctcatgcctgtaatctcagcactttgggaggccgaggtgggtggatcacctgaggtcaggagttcaagaccagcctggccaacatggcgaaaacctgtctctactaaaaatacaaaaattagctgggtgtggtggtgggcacctgcaatcccagctactcaggaggctgaggcaggagaatcactttgaacccaggaggcagaggttgcagtgagccgagattgcgccactgcactccatcctgggtgacagagcgggactccgtctcaaaaaaaaaaaaaaaaccaaaacaaaaagttaccaccaccctccgctaggaggcactaagaatagcacagtatcacttctgtggttgtcttggcaaaaatgcagatcctcaatcatatcatgtaaaaacattaaacaaactaaaactggggaatattctataaaataactggcctggactcttccaaagtgtcaaggtcatgaaagataaagaccaagaaactgtcacaggctgacagagatgaaggaaacaccacaacaaaatgcaatatgggaccctggaccagacaaaggacatcatcgggaaaactggcaaaatttgaatgtccgtagattagttagtagtagtttatcaatgttaacttcctggttttctttttttgagacggagtctcactctgtcgcccaggctggagtgcagtggcgtgatttcagctcactgcaacctccgcctcctgggctcaagtgattctcctgcctcagcctcccaagtagctgggattacaggtgggcaccagcgggcctggctaatttttgtatttttagtacagacagggtttcaccatgttggccaggctggtctcgaactcctgacctcaggtaatctgcctgcctcagcctcccaaagtgctggaattacaggcatgagccaccacacccggcaatttcctggttttgataaactacagtatggctttgtaggatgtaatcattgggagatgctagatgaaagatacatgggaattttctactatttctgcaactttctctaagtctaaaattatttcaaaacaaaaagtaaaaaacaatgaaaagcaggccgggtccagtggctcatgcctgtaatcccagcactttgggaggccgaggcaggcagatcacaaggtcaggagattgagaccatcctggctaacatggtgaaaccctgtctctactaaaaatacaaaaaggtagccgggcgtggtggtgggcacctgtagtcccagctactcgggaggctgaggcaggagaatggcgtgaacctgggaggcagggcttgcagtgagccgagatcgcgccactgcactccagcttgggggacagagtgagactctgtctcaaaaaaaaaaaaaaaaaaaaaaaggcagtcagtgaggtagggagcagcagcccctgaggggtagacagtgatccaagcatctgctggagctcacaccctggattctgactgcctcatacccaccatactgttaggacatgcttccattacccaagggactttgattcctggccccattctctgcttcctgaaagactagctaacactacgcgagggttccatgaagggcctgtgggggaaggtgggtggactgcttatcagcagtggctactgtagatggtgcccaaggatgcaccaggccttactgtgcctggctaaggtgggcttgaaacattggctggtctgtgaaatgcccttgggggacggtgtccagaccctctgctttgtgactaacatgcagactgaataaactgcatgtttattccaggctcgtttagctggacgagcagtacagacagggctgaggctgactccatggccatgtgggcagaggtcaaacccatgatctctcttcctacagcttcctaatgtctgcgatgttggtcttttgaaggaggcccccacagagctgagcttgcttggttatctgggactgctgctcagtctgagtaggggagggtaatgaaccagtcaggcctcctcctggaggtgcccaacactggcctagtccccaaggctgacgaaacatggtctggcctgaccccaggacgtggggtgaggaggaacactgggcataatatagtagcggaaacaggcaagcctctatgggtcccttccccttagaattttagggtagggaacgaggaggctacagactaaattgcagaactatctgcacctgggcctctgagctcttcctccactcccagtggagccattctggggactgagttgcatgaggactagcagagggtggcagttcagtctggtccctgtcttcttccagccagctgtgttcttagctgccatacttctgagcttcctgggaacatgagaaagtctggcgactatgggggatggggatcattctgaaggaaataagggacctccatccctccttgccttgaagggggtggaaaggcagctcctctcctgaaggcttgttagcaggttatgggcccacaacaaaggggccagagtagggcgaaattcctccttcaggttttggggctgagaaggggtcttcatgggctgtgaggaggtaagcaggcctgagactgggtagagatgggagcggcatgaggggaaggtaagtcagttgccatgccacagccaaggggcctttattggatggtgagggcacataggagcaggcaggtggctgctagatggtgttgcacaccttctcagggtgcagtggtgcccggatgtccagtctgcgagtcttgctgtccttgtcgatgatctccagacgcagcttggggaggcgcttctcagcctggggtgagggcagttctgggcttttgagtagctgcttgtctgagtcctccaccgtgatgcgcaaagtacagccccctggcagcaggtcctgctcataggctgctgccagctggttcaccacacggcgttctacctcatgtttgatggagcgggcgccatagtgcacattgtagccgtcgaccagcacatctgccacctcgcggtcccagagcagcgtgatgttgtgcctttgcttggctctcttggcccagaagtttagttccttgttgacgagttggatgagctccgagtggcagaaggggaggaagtagacgatctcattgatccgtcccagaaactcatccctccggaagtgagctttcaggatagggcgaatcacattctccttgaagttctttgagatggtgatcttgtcacttatctggacatcccccaggttttcggcaatacggttacggctcatctccaaagcttcctgcctcagctgcagcgcgtgctgtgcgatctcgtcgctggccacattggaggtcatgatgaagatggcgtccttgcaatcaatggtcttcccttttccatctgtcagccggccctcatcaaacagctgcagcatgatggtgagcacatctggatgggccttgtctacttcatcaaagagcaccacagcattggggcactgcttcaacttcttggtcagctggccaccctcctcatggccaacgtagcctggtggagacccaataaacttggccacctcgtgtcgctcctggaactcggacatgtccagcctgatgaagccctttttagcatctttgtgcatatatttggctgtctgcttggccagctctgtttttcctattccagatgatcccaagaagaggaagaccagagggtgttcttcatcgtaccagccattctccttcctccggatcgcagcacccactgtggcgatggcgctctcctggccaatgatgtgctcctttagtcgctgctccagggggaagcggcgccgctcctcagcctcacgcttccgctgcttctcttggtacttggcttcagaagtcctcagaagcttcatcacttccccttctcgggcataatccaagggtgtgtgtcccatttcattcctctgcagggggttggctcctccatcaagcagctccttgacagtgcggtagtcatcagcaagaacagcatagtgcaaggccgtgcagcccttgaaactggcgcggttgttcagcctgttgttgaagtcatcctctcgggtgatcaggacttccaaagaatggattccctgttccttggcagtcttgtaaacactgctgaaatcatctccaaggtttggatcagccccagcagcaagcaggacctgtaccacactgttgtttcggttgatggctgccaccatgagtgctgtccagccaagtctgtgctttgcattgacatctgcaccttctgacaacagcctgctgacttcttgcatattgttggcacgggcagcttccaacagggctgcatccttgttggacggactcttgctgtagcaatgaaccaccagcgctgcggccagggcgcacatgcccagtccggccctgctggggaccccgttccagctgtcctgtcctgggagtgtttcttcgggaccaggaaggcgtccccaagtggcagccgcgaggcatttggtatcgaagcgtcctccctggcgccccccggtggctgccccacgtccggagaacaaggccggcgatgttccagggcgccccccggtggctaccctcagccactgcggctccccgagactcccagtagtcacattccggccggaagcacctccatggccccggagcgttggggacctgagcagccggaggagtagccgtggcgccagtgcttttctcctcaacaccagggaccccagcatcttgacagctgcttcgataaccccgtggtgccggcccctgtgctgaccacgtccaac

SEQ ID NO: 13386 - RNA, 775 nt, Homo sapiens
  source 1..775: mol_type = other RNA
gctgggattacaggcatgagccaccacgcccggccagattcaatttttaaatatcaaaacaataagaatccccaggcttctgtgcagtggaaagtacaagtttgtcttgaaatggtttatggcattctgcatcagtcagaggaggataatactgccgatagcagacataggcaaatgtcattccaatcatggatccaactagtacatcttgccagtgatgcttgtagtcacatgtgcgggacagtgcaatcacagctgcaaaaagtagaggtgacagaaaggcacagaacctccaagatttcccacggccttgtggtgtgaagcagtgtaacttccctgccaggtagaaggacgcaaaggccagaccagcaaatgcaaaggaagaatgtccactggggaagctctttcggccctcattcaccacgtccttatcccctgtacacatcaagtcagaatgggctagcccatcagggaagcagcggtagaagaaatctgggcgtggcctccctacgatcagttttattgtgttggtaaagacgccattcagagccagggcaaggctggcagaaacatcggcttggtggggaaatactccgcctccacgtaggggttccggtagagccacatctcctccggctggatgagtctctggaacggggggagcagctccgtcaccaggaaggccgcgaacagcgcgagccgcacgcccacttcggccccaaaggccaccgccgccgccgccttccccatccggccgcgagctccgagcgacgct

SEQ ID NO: 13387 - RNA, 820 nt, Homo sapiens
  source 1..820: mol_type = other RNA
gctgggattacaggcatgagccaccacgcccggccagattcaatttttaaatatcaaaacaataagaatccccaggcttctgtgcagtggaaagtacaagtttgtcttgaaatggtttatggcattctgcatcagtcagaggaggataatactgccgatagcagacataggcaaatgtcattccaatcatggatccaactagtacatcttgccagtgatgcttgtagtcacatgtgcgggacagtgcaatcacagctgcaaaaagtagaggtgacagaaaggcacagaacctccaagatttcccacggccttgtggtgtgaagcagtgtaacttccctgccaggtagaaggacgcaaaggccagaccagcaaatgcaaaggaagaatgtccactggggaagctctttcggccctcattcaccacgtccttatcccctgtacacatcaagtcagaatgggctagcccatcagggaagcagcggtagaagaaatctgggcgtggcctccctacgatcagttttattgtgttggtaaagacgccattcagagccagggcaaggctggcagaaacatcggcttggtggggaaatactccgcctccacgtaggggttccggtagagccacatctcctccggctggatgagtctctggaacggggggagcagctccgtcaccctgggaagcggggccgcccgggcccggccgtggatctttcttacaggaaggccgcgaacagcgcgagccgcacgcccacttcggccccaaaggccaccgccgccgccgccttccccatccggccgcgagctccgagcgacgctg

SEQ ID NO: 13388 - RNA, 812 nt, Homo sapiens
  source 1..812: mol_type = other RNA
gctgggattacaggcatgagccaccacgcccggccagattcaatttttaaatatcaaaacaataagaatccccaggcttctgtgcagtggaaagtacaagtttgtcttgaaatggtttatggcattctgcatcagtcagaggaggataatactgccgatagcagacataggcaaatgtcattccaatcatggatccaactagtacatcttgccagtgatgcttgtagtcacatgtgcgggacagtgcaatcacagctgcaaaaagtagaggtgacagaaaggcacagaacctccaagatttcccacggccttgtggtgtgaagcagtgtaacttccctgccaggtagaaggacgcaaaggccagaccagcaaatgcaaaggaagaatgtccactggggaagctctttcggccctcattcaccacgtccttatcccctgtacacatcaagtcagaatgggctagcccatcagggaagcagcggtagaagaaatctgggcgtggcctccctacgatcagttttattgtgttggtaaagacgccattcagagccagggcaaggctggcagccaggcaggcttgtctgctgtctcttgtgtctgccttaaacatcggcttggtggggaaatactccgcctccacgtaggggttccggtagagccacatctcctccggctggatgagtctctggaacggggggagcagctccgtcaccaggaaggccgcgaacagcgcgagccgcacgcccacttcggccccaaaggccaccgccgccgccgccttccccatccggccgcgagctccgagcgacgct

SEQ ID NO: 13389 - RNA, 866 nt, Homo sapiens
  source 1..866: mol_type = other RNA
gctgggattacaggcatgagccaccacgcccggccagattcaatttttaaatatcaaaacaataagaatccccaggcttctgtgcagtggaaagtacaagtttgtcttgaaatggtttatggcattctgcatcagtcagaggaggataatactgccgatagcagacataggcaaatgtcattccaatcatggatccaactagtacatcttgccagtgatgcttgtagtcacatgtgcgggacagtgcaatcacagctgcaaaaagtagaggtgacagaaaggcacagaacctccaagatttcccacggccttgtggtgtgaagcagtgtaacttccctgccaggtagaaggacgcaaaggccagaccagcaaatgcaaaggaagaatgtccactggggaagctctttcggccctcattcaccacgtccttatcccctgtacacatcaagtcagaatgggctagcccatcagggaagcagcggtagaagaaatctgggcgtggcctccctacgatcagttttattgtgttggtaaagacgccattcagagccagggcaaggctggcagccaggcaggcttgtctgctgtctcttgtgtctgccttcttgagaaatttggccaggaagatcagagacagtggagagagaaatgcaataacaaacatcggcttggtggggaaatactccgcctccacgtaggggttccggtagagccacatctcctccggctggatgagtctctggaacggggggagcagctccgtcaccaggaaggccgcgaacagcgcgagccgcacgcccacttcggccccaaaggccaccgccgccgccgccttccccatccggccgcgagctccgagcgacgct

SEQ ID NO: 13390 - RNA, 846 nt, Homo sapiens
  source 1..846: mol_type = other RNA
gctgggattacaggcatgagccaccacgcccggccagattcaatttttaaatatcaaaacaataagaatccccaggcttctgtgcagtggaaagtacaagtttgtcttgaaatggtttatggcattctgcatcagtcagaggaggataatactgccgatagcagacataggcaaatgtcattccaatcatggatccaactagtacatcttgccagtgatgcttgtagtcacatgtgcgggacagtgcaatcacagctgcaaaaagtagaggtgacagaaaggcacagaacctccaagatttcccacggccttgtggtgtgaagcagtgtaacttccctgccaggtagaaggacgcaaaggccagaccagcaaatgcaaaggaagaatgtccactggggaagctctttcggccctcattcaccacgtccttatcccctgtacacatcaagtcagaatgggctagcccatcagggaagcagcggtagaagaaatctgggcgtggcctccctacgatcagttttattgtgttggtaaagacgccattcagagccagggcaaggctggcagccaggcaggcttgtctgctgtctcttgtgtctgccttcttgagaaatttggccaggaagatcagagacagtggagagagaaatgcaataacaaacatcggcttggtggggaaatactccgcctccacgtaggggttccggtagagccacatctcctccggctggatgagtctctggaacggggggagcagctccgtcaccctgggaagcggggccgcccgggcccggccgtggatctttcttacaggaaggccgcgaacagcgcgagccgcacgcccac

SEQ ID NO: 13391 - RNA, 1149 nt, Homo sapiens
  source 1..1149: mol_type = other RNA
gctgggattacaggcatgagccaccacgcccggccagattcaatttttaaatatcaaaacaataagaatccccaggcttctgtgcagtggaaagtacaagtttgtcttgaaatggtttatggcattctgcatcagtcagaggaggataatactgccgatagcagacataggcaaatgtcattccaatcatggatccaactagtacatcttgccagtgatgcttgtagtcacatgtgcgggacagtgcaatcacagctgcaaaaagtagaggtgacagaaaggcacagaacctccaagatttcccacggccttgtggtgtgaagcagtgtaacttccctgccaggtagaaggacgcaaaggccagaccagcaaatgcaaaggaagaatgtccactggggaagctctttcggccctcattcaccacgtccttatcccctgtacacatcaagtcagaatgggctagcccatcagggaagcagcggtagaagaaatctgggcgtggcctccctacgatcagttttattgtgttggtaaagacgccattcagagccagggcaaggctggcagccaggcaggcttgtctgctgtctcttgtgtctgccttcttgagaaatttggccaggaagatcagagacagtggagagagaaatgcaataacaaaggccgtctcggggtggaaaacgcacaggtgcccgcgggaagccgggtcatggggagggaggaaagacgatctttctccacgcacaaacatcggcttggtggggaaatactccgcctccacgtaggggttccggtagagccacatctcctccggctggatgagtctctggaacggggggagcagctccgtcaccaggaaggccgcgaacagcgcgagccgcacgcccacttcggccccaaaggccaccgccgccgccgccttccccatccggccgcgagctccgagcgacgctgcgctgacgtggccacctccgcggggagggccgggccgggaactgggcaccgccccctctcccagttgcccgcgctccggcggctccccaggaagacggcctggcggctgtgccgagggcatcgtctggcaaagggtacgcaaagccagcggagctgccctctggtgcgttcagcagggagccagcgccccagttc

SEQ ID NO: 13392 - RNA, 925 nt, Homo sapiens
  source 1..925: mol_type = other RNA
gctgggattacaggcatgagccaccacgcccggccagattcaatttttaaatatcaaaacaataagaatccccaggcttctgtgcagtggaaagtacaagtttgtcttgaaatggtttatggcattctgcatcagtcagaggaggataatactgccgatagcagacataggcaaatgtcattccaatcatggatccaactagtacatcttgccagtgatgcttgtagtcacatgtgcgggacagtgcaatcacagctgcaaaaagtagaggtgacagaaaggcacagaacctccaagatttcccacggccttgtggtgtgaagcagtgtaacttccctgccaggtagaaggacgcaaaggccagaccagcaaatgcaaaggaagaatgtccactggggaagctctttcggccctcattcaccacgtccttatcccctgtacacatcaagtcagaatgggctagcccatcagggaagcagcggtagaagaaatctgggcgtggcctccctacgatcagttttattgtgttggtaaagacgccattcagagccagggcaaggctggcagccaggcaggcttgtctgctgtctcttgtgtctgccttcttgagaaatttggccaggaagatcagagacagtggagagagaaatgcaataacaggtgcccgcgggaagccgggtcatggggagggaggaaagacgatctttctccacgcacaaacatcggcttggtggggaaatactccgcctccacgtaggggttccggtagagccacatctcctccggctggatgagtctctggaacggggggagcagctccgtcaccaggaaggccgcgaacagcgcgagccgcacgcccacttcggccccaaaggccaccgccgccgccgccttccccatccggccgcgagctccgagcgacgct

SEQ ID NO: 13393 - RNA, 1202 nt, Homo sapiens
  source 1..1202: mol_type = other RNA
gctgggattacaggcatgagccaccacgcccggccagattcaatttttaaatatcaaaacaataagaatccccaggcttctgtgcagtggaaagtacaagtttgtcttgaaatggtttatggcattctgcatcagtcagaggaggataatactgccgatagcagacataggcaaatgtcattccaatcatggatccaactagtacatcttgccagtgatgcttgtagtcacatgtgcgggacagtgcaatcacagctgcaaaaagtagaggtgacagaaaggcacagaacctccaagatttcccacggccttgtggtgtgaagcagtgtaacttccctgccaggtagaaggacgcaaaggccagaccagcaaatgcaaaggaagaatgtccactggggaagctctttcggccctcattcaccacgtccttatcccctgtacacatcaagtcagaatgggctagcccatcagggaagcagcggtagaagaaatctgggcgtggcctccctacgatcagttttattgtgttggtaaagacgccattcagagccagggcaaggctggcagccaggcaggcttgtctgctgtctcttgtgtctgccttcttgagaaatttggccaggaagatcagagacagtggagagagaaatgcaataactggagctaacataaggtctctgagtgcgcgtaaccgggcgccaggcagcgccaccagtgaacagcagcgcccgtgcggctcgggccccggtacctcaggctgaggcacagagcgcccgggaaaacgttgtctcagcccaaagaggctcggacaccctcctctctcaatcaggatcttaaacactcgagccctaggaggcggaacccagcgcacagcagcggagtgggcagtgggtccctacaaaggccgtctcggggtggaaaacgcacaggtgcccgcgggaagccgggtcatggggagggaggaaagacgatctttctccacgcacaaacatcggcttggtggggaaatactccgcctccacgtaggggttccggtagagccacatctcctccggctggatgagtctctggaacggggggagcagctccgtcaccaggaaggccgcgaacagcgcgagccgcacgcccacttcggccccaaaggccaccgccgccgccgccttccccatccggccgcgagctccgagcgacgctgcgctgac

SEQ ID NO: 13394 - RNA, 1179 nt, Homo sapiens
  source 1..1179: mol_type = other RNA
gctgggattacaggcatgagccaccacgcccggccagattcaatttttaaatatcaaaacaataagaatccccaggcttctgtgcagtggaaagtacaagtttgtcttgaaatggtttatggcattctgcatcagtcagaggaggataatactgccgatagcagacataggcaaatgtcattccaatcatggatccaactagtacatcttgccagtgatgcttgtagtcacatgtgcgggacagtgcaatcacagctgcaaaaagtagaggtgacagaaaggcacagaacctccaagatttcccacggccttgtggtgtgaagcagtgtaacttccctgccaggtagaaggacgcaaaggccagaccagcaaatgcaaaggaagaatgtccactggggaagctctttcggccctcattcaccacgtccttatcccctgtacacatcaagtcagaatgggctagcccatcagggaagcagcggtagaagaaatctgggcgtggcctccctacgatcagttttattgtgttggtaaagacgccattcagagccagggcaaggctggcagctgcaaagcaaagccattagttgaaaggatctgtctaggaggaaaggtatggtcatggcctcgttatgagagcagccgtgctgtttctgagatggatagaatccaaccaggcccaggcaggcttgtctgctgtctcttgtgtctgccttcttgagaaatttggccaggaagatcagagacagtggagagagaaatgcaataacaaacatcggcttggtggggaaatactccgcctccacgtaggggttccggtagagccacatctcctccggctggatgagtctctggaacggggggagcagctccgtcaccaggaaggccgcgaacagcgcgagccgcacgcccacttcggccccaaaggccaccgccgccgccgccttccccatccggccgcgagctccgagcgacgctgcgctgacgtggccacctccgcggggagggccgggccgggaactgggcaccgccccctctcccagttgcccgcgctccggcggctccccaggaagacggcctggcggctgtgccgagggcatcgtctggcaaagggtacgcaaagccagcggagctgccctctggtgcgttcagcagggagccagcgccccagttccagcc

SEQ ID NO: 13395 - RNA, 1275 nt, Homo sapiens
  source 1..1275: mol_type = other RNA
gctgggattacaggcatgagccaccacgcccggccagattcaatttttaaatatcaaaacaataagaatccccaggcttctgtgcagtggaaagtacaagtttgtcttgaaatggtttatggcattctgcatcagtcagaggaggataatactgccgatagcagacataggcaaatgtcattccaatcatggatccaactagtacatcttgccagtgatgcttgtagtcacatgtgcgggacagtgcaatcacagctgcaaaaagtagaggtgacagaaaggcacagaacctccaagatttcccacggccttgtggtgtgaagcagtgtaacttccctgccaggtagaaggacgcaaaggccagaccagcaaatgcaaaggaagaatgtccactggggaagctctttcggccctcattcaccacgtccttatcccctgtacacatcaagtcagaatgggctagcccatcagggaagcagcggtagaagaaatctgggcgtggctttttagggcaaacagcaaatgacactgcagcttcaggaggtgctcaagaggacactgaccgactgctgtggccgttggtgggaaatgctccctacgatcagttttattgtgttggtaaagacgccattcagagccagggcaaggctggcagctgcaaagcaaagccattagttgaaaggatctgtctaggaggaaaggtatggtcatggcctcgttatgagagcagccgtgctgtttctgagatggatagaatccaaccaggcccaggcaggcttgtctgctgtctcttgtgtctgccttcttgagaaatttggccaggaagatcagagacagtggagagagaaatgcaataacaaacatcggcttggtggggaaatactccgcctccacgtaggggttccggtagagccacatctcctccggctggatgagtctctggaacggggggagcagctccgtcaccaggaaggccgcgaacagcgcgagccgcacgcccacttcggccccaaaggccaccgccgccgccgccttccccatccggccgcgagctccgagcgacgctgcgctgacgtggccacctccgcggggagggccgggccgggaactgggcaccgccccctctcccagttgcccgcgctccggcggctccccaggaagacggcctggcggctgtgccgagggcatcgtctggcaaagggtacgcaaagccagcggagctgccctctggtgcgttcagcagggagccagcgccccagttccagccgagtaggt

SEQ ID NO: 13396 - RNA, 1733 nt, Homo sapiens
  source 1..1733: mol_type = other RNA
gctgggattacaggcatgagccaccacgcccggccagattcaatttttaaatatcaaaacaataagaatccccaggcttctgtgcagtggaaagtacaagtttgtcttgaaatggtttatggcattctgcatcagtcagaggaggataatactgccgatagcagacataggcaaatgtcattccaatcatggatccaactagtacatcttgccagtgatgcttgtagtcacatgtgcgggacagtgcaatcacagctgcaaaaagtagaggtgacagaaaggcacagaacctccaagatttcccacggccttgtggtgtgaagcagtgtaacttccctgccaggtagaaggacgcaaaggccagaccagcaaatgcaaaggaagaatgtccactggggaagctctttcggccctcattcaccacgtccttatcccctgtacacatcaagtcagaatgggctagcccatcagggaagcagcggtagaagaaatctgggcgtggctttttagggcaaacagcaaatgacactgcagcttcaggaggtgctcaagaggacactgaccgactgctgtggccgttggtgggaaatgctccctacgatcagttttattgtgttggtaaagacgccattcagagccagggcaaggctggcagctgcaaagcaaagccattagttgaaaggatctgtctaggaggaaaggtatggtcatggcctcgttatgagagcagccgtgctgtttctgagatggatagaatccaaccaggcctgggcacaaaaataattagggtcctcagtgatcactcttttgtagccgagaacttttgtactaggccaaagacatttctgaggtacaaataacccagtgcatttaggcacagggctgcctgccgtgtagcctgcgtaaccaagtccctgcagtgctattttcctctcccgcggggatagagttcctttaggaatgcagaactcagtggcctccacacaggctcaccgtggctgaatcccacaacgacctcctaggttcccagcacgaagaaaccggcccgaaagggctagcgctcacccaggcaggcttgtctgctgtctcttgtgtctgccttcttgagaaatttggccaggaagatcagagacagtggagagagaaatgcaataacctgaatcagaatgtcagaggttaaaaacaatccaaaaaaaagccacactcgtgctcctacaggaaagagggatgtgacacagcaggactcactggagctaacataaggtctctgagtgcgcgtaaccgggcgccaggcagcgccaccagtgaacagcagcgcccgtgcggctcgggccccggtacctcaggctgaggcacagagcgcccgggaaaacgttgtctcagcccaaagaggctcggacaccctcctctctcaatcaggatcttaaacactcgagccctaggaggcggaacccagcgcacagcagcggagtgggcagtgggtccctacaaaggccgtctcggggtggaaaacgcacaggtgcccgcgggaagccgggtcatggggagggaggaaagacgatctttctccacgcacaaacatcggcttggtggggaaatactccgcctccacgtaggggttccggtagagccacatctcctccggctggatgagtctctggaacggggggagcagctccgtcaccaggaaggccgcgaacagcgcgagccgcacgcccacttcggccccaaag

SEQ ID NO: 13397 - RNA, 993 nt, Homo sapiens
  source 1..993: mol_type = other RNA
gctgggattacaggcatgagccaccacgcccggccagattcaatttttaaatatcaaaacaataagaatccccaggcttctgtgcagtggaaagtacaagtttgtcttgaaatggtttatggcattctgcatcagtcagaggaggataatactgccgatagcagacataggcaaatgtcattccaatcatggatccaactagtacatcttgccagtgatgcttgtagtcacatgtgcgggacagtgcaatcacagctgcaaaaagtagaggtgacagaaaggcacagaacctccaagatttcccacggccttgtggtgtgaagcagtgtaacttccctgccaggtagaaggacgcaaaggccagaccagcaaatgcaaaggaagaatgtccactggggaagctctttcggccctcattcaccacgtccttatcccctgtacacatcaagtcagaatgggctagcccatcagggaagcagcggtagaagaaatctgggcgtggctttttagggcaaacagcaaatgacactgcagcttcaggaggtgctcaagaggacactgaccgactgctgtggccgttggtgggaaatgctgttcaggcagaaaagagcccaggtgtcacctggaggactccctacgatcagttttattgtgttggtaaagacgccattcagagccagggcaaggctggcagccaggcaggcttgtctgctgtctcttgtgtctgccttcttgagaaatttggccaggaagatcagagacagtggagagagaaatgcaataacaaacatcggcttggtggggaaatactccgcctccacgtaggggttccggtagagccacatctcctccggctggatgagtctctggaacggggggagcagctccgtcaccaggaaggccgcgaacagcgcgagccgcacgcccacttcggccccaaaggccaccgccgccgccgccttccccatccggccgcgagctccgagcgacgct

SEQ ID NO: 13398 - RNA, 2084 nt, Homo sapiens
  source 1..2084: mol_type = other RNA
gctgggattacaggcatgagccaccacgcccggccatctagattagttctttacattgaaagtaacatccagggtcactgatattctgagaaaattagaaccacctttgagttaagacttctagaaagacacatacgttgttatattttaattggaatcagacatttaatggcataaaaacattgcatatatggctttgctgttccgaatgtcatgaacttaaaatccaaatatgacataagcagttttaagacttattttggccagcctccccaatcccaaaggagatttaaaagtaataatgtaaaaaagttaaggtcaaggtgttttaaaatcaacatctcagctaatgactaaccctttgtttcctggggacttctgctctactgtgaaaactgctgagcttaacccgctgttgaacaactggttagttattagttccctgggtgattgtccctgaagttaagccatgctctggggacacatgaggcactttaattggggtagttactttttccaggttgggtacaatgtttggctctcaaaagcaaggtaaacagtttacagtcaaaaggaatgctctgtgattgtgtgcctttgggatcaagggttgagatcttagagtattctcataaacatctgtaccaggtgctcaaagatgtttgagggttgtcaagcaagctgttcaacttctgcattttctgtggatatgggcacaatgacccactcagatttttctcctagtgtcctgaatgacagctcatctacacagagtgaaactccagatatgtgacaagcagcatgggacagatgctgacaatcagaacagatgctggatgtaaacaactggtaaggctgcactggtgcatgctggcagaatcacctgctatgcatccagggagcaaatgcatctgcatgctcagcatgacaccagcttacctccctgtgcaaatcccctcccctaatcagtctcatccaaatcttctcctgcagtagcagcttctaaagctgcaagggcctccgccaccgctgcatcctcgtccacaatctccccatccccatctccatcggagccatgggtatcctcctgcctgtttcctgagtcaaccacaggcatggcatgaacaggacccttctcattaaagcagatgcttagaacttctgtttccacatcctcattcaatgaatcccagcttctcctcacagagaagggcgtattcaaaccatgctcccccactgggggctgaattccctctagggattcatcctcagtatggttcttgaaaacacagtccttttcattatgatcaacgttgtctccagctgggccccaatgctgaaggtaatctggggctggtatctggaagacatggtcttgtacttccaaggcaaaactttctgcctcagaaggagctctggagtctccatttctcatgacttgggtcccttctgaggccagcagcacacagtcctgtttcctggtgccccctccttccaggaagggttgagttgggggaacagtatttgcagtactggcccaggagcccctgtcatcctgggtggggctggaattcccagtgggctgtggagtggcagcagggccgatgccgttgacaccgcaggcatggtgttcccctccagcgtccccctgtgggagcggcccttggtgaggccagcagggctcccatggatcagctgtcctgctgctgctctcagtcttctttgagccctgcctctgagggtcatttttctgcaccaagacttcactgctccatttgccttttaatttatcagtgtcgtcttcatctagcttgcagctgttgacttcattgacatagccaggagagggcacttgaactggatcaaagagatagctttgtattattttacagcacctgcaccccatctggattgttttctgttaccacctgagggtcatgcttccgcgcctctccggagcttggcggggacagcctcttcctggttagaggttctgtcctctctcacctcgccctgagttttccttccccagcaacattccttctctagatcagacggacaggctctaatgtccaaggttgtgt

SEQ ID NO: 13399 - RNA, 2153 nt, Homo sapiens
  source 1..2153: mol_type = other RNA
gctgggattacaggcatgagccaccacgcccggccatctagattagttctttacattgaaagtaacatccagggtcactgatattctgagaaaattagaaccacctttgagttaagacttctagaaagacacatacgttgttatattttaattggaatcagacatttaatggcataaaaacattgcatatatggctttgctgttccgaatgtcatgaacttaaaatccaaatatgacataagcagttttaagacttattttggccagcctccccaatcccaaaggagatttaaaagtaataatgtaaaaaagttaaggtcaaggtgttttaaaatcaacatctcagctaatgactaaccctttgtttcctggggacttctgctctactgtgaaaactgctgagcttaacccgctgttgaacaactggttagttattagttccctgggtgattgtccctgaagttaagccatgctctggggacacatgaggcactttaattggggtagttactttttccaggttgggtacaatgtttggctctcaaaagcaaggtaaacagtttacagtcaaaaggaatgctctgtgattgtgtgcctttgggatcaagggttgagatcttagagtattctcataaacatctgtaccaggtgctcaaagatgtttgagggttgtcaagcaagctgttcaacttctgcattttctgtggatatgggcacaatgacccactcagatttttctcctagtgtcctgaatgacagctcatctacacagagtgaaactccagatatgtgacaagcagcatgggacagatgctgacaatcagaacagatgctggatgtaaacaactggtaaggctgcactggtgcatgctggcagaatcacctgctatgcatccagggagcaaatgcatctgcatgctcagcatgacaccagcttacctccctgtgcaaatcccctcccctaatcagtctcatccaaatcttctcctgcagtagcagcttctaaagctgcaagggcctccgccaccgctgcatcctcgtccacaatctccccatccccatctccatcggagccatgggtatcctcctgcctgtttcctgagtcaaccacaggcatggcatgaacaggacccttctcattaaagcagatgcttagaacttctgtttccacatcctcattcaatgaatcccagcttctcctcacagagaagggcgtattcaaaccatgctcccccactgggggctgaattccctctagggattcatcctcagtatggttcttgaaaacacagtccttttcattatgatcaacgttgtctccagctgggccccaatgctgaaggtaatctggggctggtatctggaagacatggtcttgtacttccaaggcaaaactttctgcctcagaaggagctctggagtctccatttctcatgacttgggtcccttctgaggccagcagcacacagtcctgtttcctggtgccccctccttccaggaagggttgagttgggggaacagtatttgcagtactggcccaggagcccctgtcatcctgggtggggctggaattcccagtgggctgtggagtggcagcagggccgatgccgttgacaccgcaggcatggtgttcccctccagcgtccccctgtgggagcggcccttggtgaggccagcagggctcccatggatcagctgtcctgctgctgctctcagtcttctttgagccctgcctctgagggtcatttttctgcaccaagacttcactgctccatttgccttttaatttatcagtgtcgtcttcatctagcttgcagctgttgacttcattgacatagccaggagagggcacttgaactggatcaaagagatagctttgtattattttacagcacctgcaccccatctggattgttttctgttaccacctgttgtggatattgtctgttaggtttctctagaagtttaacttctcttcagttaatgcaatgcatattgaagtgctggggtgaaatgaactgatgtttgcaacttgctctggggccagacggcggcggcggcggcggcggcggggtcccggcgcccatggcttcgccggcctcgggcagccgcgccgggagacgctagcggctccgcgctgccctgagcccgcc

SEQ ID NO: 13400 - RNA, 2355 nt, Homo sapiens
  source 1..2355: mol_type = other RNA
gctgggattacaggcatgagccaccacgcccggccatctagattagttctttacattgaaagtaacatccagggtcactgatattctgagaaaattagaaccacctttgagttaagacttctagaaagacacatacgttgttatattttaattggaatcagacatttaatggcataaaaacattgcatatatggctttgctgttccgaatgtcatgaacttaaaatccaaatatgacataagcagttttaagacttattttggccagcctccccaatcccaaaggagatttaaaagtaataatgtaaaaaagttaaggtcaaggtgttttaaaatcaacatctcagctaatgactaaccctttgtttcctggggacttctgctctactgtgaaaactgctgagcttaacccgctgttgaacaactggttagttattagttccctgggtgattgtccctgaagttaagccatgctctggggacacatgaggcactttaattggggtagttactttttccaggttgggtacaatgtttggctctcaaaagcaaggtaaacagtttacagtcaaaaggaatgctctgtgattgtgtgcctttgggatcaagggttgagatcttagagtattctcataaacatctgtaccaggtgctcaaagatgtttgagggttgtcaagcaagctgttcaacttctgcattttctgtggatatgggcacaatgacccactcagatttttctcctagtgtcctgaatgacagctcatctacacagagtgaaactccagatatgtgacaagcagcatgggacagatgctgacaatcagaacagatgctggatgtaaacaactggtaaggctgcactggtgcatgctggcagaatcacctgctatgcatccagggagcaaatgcatctgcatgctcagcatgacaccagcttacctccctgtgcaaatcccctcccctaatcagtctcatccaaatcttctcctgcagtagcagcttctaaagctgcaagggcctccgccaccgctgcatcctcgtccacaatctccccatccccatctccatcggagccatgggtatcctcctgcctgtttcctgagtcaaccacaggcatggcatgaacaggacccttctcattaaagcagatgcttagaacttctgtttccacatcctcattcaatgaatcccagcttctcctcacagagaagggcgtattcaaaccatgctcccccactgggggctgaattccctctagggattcatcctcagtatggttcttgaaaacacagtccttttcattatgatcaacgttgtctccagctgggccccaatgctgaaggtaatctggggctggtatctggaagacatggtcttgtacttccaaggcaaaactttctgcctcagaaggagctctggagtctccatttctcatgacttgggtcccttctgaggccagcagcacacagtcctgtttcctggtgccccctccttccaggaagggttgagttgggggaacagtatttgcagtactggcccaggagcccctgtcatcctgggtggggctggaattcccagtgggctgtggagtggcagcagggccgatgccgttgacaccgcaggcatggtgttcccctccagcgtccccctgtgggagcggcccttggtgaggccagcagggctcccatggatcagctgtcctgctgctgctctcagtcttctttgagccctgcctctgagggtcatttttctgcaccaagacttcactgctccatttgccttttaatttatcagtgtcgtcttcatctagcttgcagctgttgacttcattgacatagccaggagagggcacttgaactggatcaaagagatagctttgtattattttacagcacctgcaccccatctggattgttttctgttaccacctgttgtggatattgtctgttaggtttctctagaagtttaacttctcttcctgcacgccccgaggatgcggcggggctagggctcgaaaccctggagtacgatgtccgacatccccggggccggggtggcagtcccgggcgcactgaagcagaaaatccacgcgcttgttggcctctgagcacaaacgaccgcgccaaccgcctgccatcacgggaaactccggggtgcttactccaatgttgcgctggagagaagggagcttcctatgatcaagggactggagtacggggatacacaaaacaaatgcacccgctggcaaatagttgtgtactcccaaaccccgagaacttggcatttttcagtttcctccttatttctggcattcgccgcctagacctgctgtgagttccatggccagccctgtat

SEQ ID NO: 13401 - RNA, 2094 nt, Homo sapiens
  source 1..2094: mol_type = other RNA
gctgggattacaggcatgagccaccacgcccggccatctagattagttctttacattgaaagtaacatccagggtcactgatattctgagaaaattagaaccacctttgagttaagacttctagaaagacacatacgttgttatattttaattggaatcagacatttaatggcataaaaacattgcatatatggctttgctgttccgaatgtcatgaacttaaaatccaaatatgacataagcagttttaagacttattttggccagcctccccaatcccaaaggagatttaaaagtaataatgtaaaaaagttaaggtcaaggtgttttaaaatcaacatctcagctaatgactaaccctttgtttcctggggacttctgctctactgtgaaaactgctgagcttaacccgctgttgaacaactggttagttattagttccctgggtgattgtccctgaagttaagccatgctctggggacacatgaggcactttaattggggtagttactttttccaggttgggtacaatgtttggctctcaaaagcaaggtaaacagtttacagtcaaaaggaatgctctgtgattgtgtgcctttgggatcaagggttgagatcttagagtattctcataaacatctgtaccaggtgctcaaagatgtttgagggttgtcaagcaagctgttcaacttctgcattttctgtggatatgggcacaatgacccactcagatttttctcctagtgtcctgaatgacagctcatctacacagagtgaaactccagatatgtgacaagcagcatgggacagatgctgacaatcagaacagatgctggatgtaaacaactggtaaggctgcactggtgcatgctggcagaatcacctgctatgcatccagggagcaaatgcatctgcatgctcagcatgacaccagcttacctccctgtgcaaatcccctcccctaatcagtctcatccaaatcttctcctgcagtagcagcttctaaagctgcaagggcctccgccaccgctgcatcctcgtccacaatctccccatccccatctccatcggagccatgggtatcctcctgcctgtttcctgagtcaaccacaggcatggcatgaacaggacccttctcattaaagcagatgcttagaacttctgtttccacatcctcattcaatgaatcccagcttctcctcacagagaagggcgtattcaaaccatgctcccccactgggggctgaattccctctagggattcatcctcagtatggttcttgaaaacacagtccttttcattatgatcaacgttgtctccagctgggccccaatgctgaaggtaatctggggctggtatctggaagacatggtcttgtacttccaaggcaaaactttctgcctcagaaggagctctggagtctccatttctcatgacttgggtcccttctgaggccagcagcacacagtcctgtttcctggtgccccctccttccaggaagggttgagttgggggaacagtatttgcagtactggcccaggagcccctgtcatcctgggtggggctggaattcccagtgggctgtggagtggcagcagggccgatgccgttgacaccgcaggcatggtgttcccctccagcgtccccctgtgggagcggcccttggtgaggccagcagggctcccatggatcagctgtcctgctgctgctctcagtcttctttgagccctgcctctgagggtcatttttctgcaccaagacttcactgctccatttgccttttaatttatcagtgtcgtcttcatctagcttgcagctgttgacttcattgacatagccaggagagggcacttgaactggatcaaagagatagctttgtattattttacagcacctgcaccccatctggattgttttctgttaccacctgttgtggatattgtctgttaggtttctctagaagtttaacttctcttcctggggccagacggcggcggcggcggcggcggcggggtcccggcgcccatggcttcgccggcctcgggcagccgcgccgggagacgctagcggctccgcgctgccctgagcccgcc

SEQ ID NO: 13402 - RNA, 654 nt, Homo sapiens
  source 1..654: mol_type = other RNA
gctgggattacaggcatgagccaccacgcccggccatcttcttgccagcaactcttagaccaggaagcctcggatggcagctatgaagtcctgtgggcggtcagcgtggatccagtggccagcgttcggcaccgtctgcatctgggcccgagggaagagccgcataatctcagggtggtggctgggacctctgtagtgccagcagcatggctgtctttcctcccatgctgtggccaacgacgacgcagggcaccaggcccagctggggcagaaggtcctgcaggtcctggctcatgatctcgtagctcatgtctgggctgtgggggctgtcaccgtggttacgagcatccaccgtcagcaccctacggcctgtctgctgggccaagatcttggcgatggagttgaagttagttttgctgccgaagagcccgtgcaaaaagacgacggccgggagggctgcctccccgtccagaagcctgtaggaaagcggaagcggcctcggctcggcgccccctcggccgccgctgctgctgctgggtgcgacaggcaccctcgcgaagctagggccgtgggggccgagtccctcacgcgggagcctccaggctcgggtccagcggagcatgcttgcaagctgttggccggctcgcatctcac

SEQ ID NO: 13403 - RNA, 1070 nt, Homo sapiens
  source 1..1070: mol_type = other RNA
gctgggattacaggcatgagccaccacgcccggccatcttcttgccagcaactcttagaccaggaagcctcggatggcagctatgaagtcctgtgggcggtcagcgtggatccagtggccagcgttcggcaccgtctgcatctgggcccgagggaagagccgcataatctcagggtggtggctgggacctctgtagtgccagcagcatggctgtctttcctcccatgctgtggccaacgacgacgcagggcaccaggcccagctggggcagaaggtcctgcaggtcctggctcatgatctcgtagctcatgtctgggctgtgggggctgtcaccgtggttacgagcatccaccgtcagcacctggggccactctgccagagaagagcaggccccagggttgtgaccacgtctctgaagggctggcctggctgggtggcaatctcggagaatgccaggaaggagactccaggaatttccaacagtaggagcacagaagaatgggctgccataagaggtggtgagctcccggtcatcccctacggcctgtctgctgggccaagatcttggcgatggagttgaagttagttttgctgccgaagagcccgtgcaaaaagacgacggccgggagggctgcctccccgtccagaagcctgtaggaaagcggaagcggcctggcaggggaaggatcgaggtcagagtctgagccggcggagacggggaaaggggtagggggaaagagctttgggggagaggcctgggaggtgacaggcccaaagggaggagatggggccgtcggggcccggcaggaaaaggaggacagaggatggcctcccgcccggtgcccttgactgacctcggctcggcgccccctcggccgccgctgctgctgctgggtgcgacaggcaccctcgcgaagctagggccgtgggggccgagtccctcacgcgggagcctccaggctcgggtccagcggagcatgcttgcaagctgttggccggctcgcatctcacaaggtacgtcctccccgcgctccttctcccgccctagctcgcagccccgcccatttccg

SEQ ID NO: 13404 - RNA, 836 nt, Homo sapiens
  source 1..836: mol_type = other RNA
gctgggattacaggcatgagccaccacgcccggccatcttcttgccagcaactcttagaccaggaagcctcggatggcagctatgaagtcctgtgggcggtcagcgtggatccagtggccagcgttcggcaccgtctgcatctgggcccgagggaagagccgcataatctcagggtggtggctgggatgcacgaactgggagtttccaccaaggagaaagagtgttggcccgaggtaggactcctgcctctgtgggaaagccaagatcttgtctaggtgctgggtcagggcatccaagttcaccctccacacgaagcgcccgtctacctctaccaggttagtgagcaggtgctgccgcacggccatgtccctctgtagtgccagcagcatggctgtctttcctcccatgctgtggccaacgacgacgcagggcaccaggcccagctggggcagaaggtcctgcaggtcctggctcatgatctcgtagctcatgtctgggctgtgggggctgtcaccgtggttacgagcatccaccgtcagcaccctacggcctgtctgctgggccaagatcttggcgatggagttgaagttagttttgctgccgaagagcccgtgcaaaaagacgacggccgggagggctgcctccccgtccagaagcctgtaggaaagcggaagcggcctcggctcggcgccccctcggccgccgctgctgctgctgggtgcgacaggcaccctcgcgaagctagggccgtgggggccgagtccctcacgcgggagcctccaggctcgggtccagcggagcatgcttgcaagctgttggccggctcgcatctcac

SEQ ID NO: 13405 - RNA, 1238 nt, Homo sapiens
  source 1..1238: mol_type = other RNA
gctgggattacaggcatgagccaccacgcccggccatcttcttgccagcaactcttagaccaggaagcctcggatggcagctatgaagtcctgtgggcggtcagcgtggatccagtggccagcgttcggcaccgtctgcatctgggcccgagggaagagccgcataatctcagggtggtggctgggatgcacgaactgggagtttccaccaaggagaaagagtgttggcccgaggtaggactcctgcctctgtgggaaagccaagatcttgtctaggtgctgggtcagggcatccaagttcaccctccacacgaagcgcccgtctacctctaccaggttagtgagcaggtgctgccgcacggccatgtccctctgtagtgccagcagcatggctgtctttcctcccatgctgtggccaacgacgacgcagggcaccaggcccagctggggcagaaggtcctgcaggtcctggctcatgatctcgtagctcatgtctgggctgtgggggctgtcaccgtggttacgagcatccaccgtcagcacctggggccactctgccagagaagagcaggccccagggttgtgaccacgtctctgaagggctggcctggctgggtggcaatctcggagaatgccaggaaggagactccaggaatttccaacagtaggagcacagaagaatgggctgccataagaggtggtgagctcccggtcatcccctacggcctgtctgctgggccaagatcttggcgatggagttgaagttagttttgctgccgaagagcccgtgcaaaaagacgacggccgggagggctgcctccccgtccagaagcctgtaggaaagcggaagcggcctggcaggggaaggatcgaggtcagagtctgagccggcggagacggggaaaggggtagggggaaagagctttgggggagaggcctgggaggtgacaggcccaaagggaggagatggggccgtcggggcccggcaggaaaaggaggacagaggatggcctcccgcccggtgcccttgactgacctcggctcggcgccccctcggccgccgctgctgctgctgggtgcgacaggcaccctcgcgaagctagggccgtgggggccgagtccctcacgcgggagcctccaggctcgggtccagcggagcatgcttgcaagctgttggccggctcgcatctcacaaggtacgtcctccccgcgctccttctcccgccctagctcgcagc

SEQ ID NO: 13406 - RNA, 986 nt, Homo sapiens
  source 1..986: mol_type = other RNA
gctgggattacaggcatgagccaccacgcccggccatcttcttgccagcaactcttagaccaggaagcctcggatggcagctatgaagtcctgtgggcggtcagcgtggatccagtggccagcgttcggcaccgtctgcatctgggcccgagggaagagccgcataatctcagggtggtggctgggatgcacgaactgggagtttccaccaaggagaaagagtgttggcccgaggtaggactcctgcctctgtgggaaagccaagatcttgtctaggtgctgggtcagggcatccaagttcaccctccacacgaagcgcccgtctacctctaccaggttagtgagcaggtgctgccgcacggccatgtcctggatgacagaactgagctgttcatccgccagttttcgggcacgggagcggggcagctcatctgcgatgttgatggccctcatggctgccacataggttgcaaagtgggagacacctgtgctttccactgggctgatatctacagcaatgagacgttccaccagctctggcctctgtagtgccagcagcatggctgtctttcctcccatgctgtggccaacgacgacgcagggcaccaggcccagctggggcagaaggtcctgcaggtcctggctcatgatctcgtagctcatgtctgggctgtgggggctgtcaccgtggttacgagcatccaccgtcagcaccctacggcctgtctgctgggccaagatcttggcgatggagttgaagttagttttgctgccgaagagcccgtgcaaaaagacgacggccgggagggctgcctccccgtccagaagcctcggctcggcgccccctcggccgccgctgctgctgctgggtgcgacaggcaccctcgcgaagctagggccgtgggggccgagtccctcacgcgggagcctccaggctcgggtccagcggagcatgcttgcaagctgttggccggctcgcatctcac

SEQ ID NO: 13407 - RNA, 1007 nt, Homo sapiens
  source 1..1007: mol_type = other RNA
gctgggattacaggcatgagccaccacgcccggccatcttcttgccagcaactcttagaccaggaagcctcggatggcagctatgaagtcctgtgggcggtcagcgtggatccagtggccagcgttcggcaccgtctgcatctgggcccgagggaagagccgcataatctcagggtggtggctgggatgcacgaactgggagtttccaccaaggagaaagagtgttggcccgaggtaggactcctgcctctgtgggaaagccaagatcttgtctaggtgctgggtcagggcatccaagttcaccctccacacgaagcgcccgtctacctctaccaggttagtgagcaggtgctgccgcacggccatgtcctggatgacagaactgagctgttcatccgccagttttcgggcacgggagcggggcagctcatctgcgatgttgatggccctcatggctgccacataggttgcaaagtgggagacacctgtgctttccactgggctgatatctacagcaatgagacgttccaccagctctggcctctgtagtgccagcagcatggctgtctttcctcccatgctgtggccaacgacgacgcagggcaccaggcccagctggggcagaaggtcctgcaggtcctggctcatgatctcgtagctcatgtctgggctgtgggggctgtcaccgtggttacgagcatccaccgtcagcaccctacggcctgtctgctgggccaagatcttggcgatggagttgaagttagttttgctgccgaagagcccgtgcaaaaagacgacggccgggagggctgcctccccgtccagaagcctgtaggaaagcggaagcggcctcggctcggcgccccctcggccgccgctgctgctgctgggtgcgacaggcaccctcgcgaagctagggccgtgggggccgagtccctcacgcgggagcctccaggctcgggtccagcggagcatgcttgcaagctgttggccggctcgcatctcac

SEQ ID NO: 13408 - RNA, 1169 nt, Homo sapiens
  source 1..1169: mol_type = other RNA
gctgggattacaggcatgagccaccacgcccggccatcttcttgccagcaactcttagaccaggaagcctcggatggcagctatgaagtcctgtgggcggtcagcgtggatccagtggccagcgttcggcaccgtctgcatctgggcccgagggaagagccgcataatctcagggtggtggctgggatgcacgaactgggagtttccaccaaggagaaagagtgttggcccgaggtaggactcctgcctctgtgggaaagccaagatcttgtctaggtgctgggtcagggcatccaagttcaccctccacacgaagcgcccgtctacctctaccaggttagtgagcaggtgctgccgcacggccatgtcctggatgacagaactgagctgttcatccgccagttttcgggcacgggagcggggcagctcatctgcgatgttgatggccctcatggctgccacataggttgcaaagtgggagacacctgtgctttccactgggctgatatctacagcaatgagacgttccaccagctctggcctctgtagtgccagcagcatggctgtctttcctcccatgctgtggccaacgacgacgcagggcaccaggcccagctggggcagaaggtcctgcaggtcctggctcatgatctcgtagctcatgtctgggctgtgggggctgtcaccgtggttacgagcatccaccgtcagcacctaggaggcccagatgaagaacctggggccactctgccagagaagagcaggccccagggttgtgaccacgtctctgaagggctggcctggctgggtggcaatctcggagaatgccaggaaggagactccaggaatttccaacagtaggagcacagaagaatgggctgccataagaggtggtgagctcccggtcatcccctacggcctgtctgctgggccaagatcttggcgatggagttgaagttagttttgctgccgaagagcccgtgcaaaaagacgacggccgggagggctgcctccccgtccagaagcctgtaggaaagcggaagcggcctcggctcggcgccccctcggccgccgctgctgctgctgggtgcgacaggcaccctcgcgaagctagggccgtgggggccgagtccctcacgcgggagcctccaggctcgggtccagcggag

SEQ ID NO: 13409 - RNA, 1037 nt, Homo sapiens
  source 1..1037: mol_type = other RNA
gctgggattacaggcatgagccaccacgcccggccatcttcttgccagcaactcttagaccaggaagcctcggatggcagctatgaagtcctgtgggcggtcagcgtggatccagtggccagcgttcggcaccgtctgcatctgggcccgagggaagagccgcataatctcagggtggtggctgggatgcacgaactgggagtttccaccaaggagaaagagtgttggcccgaggtaggactcctgcctctgtgggaaagccaagatcttgtctaggtgctgggtcagggcatccaagttcaccctccacacgaagcgcccgtctacctctaccaggttagtgagcaggtgctgccgcacggccatgtcctggatgacagaactgagctgttcatccgccagttttcgggcacgggagcggggcagctcatctgcgatgttgatggccctcatggctgccacataggttgcaaagtgggagacacctgtgctttccactgggctgatatctacagcaatgagacgttccaccagctctggcctctgtagtgccagcagcatggctgtctttcctcccatgctgtggccaacgacgacgcagggcaccaggcccagctggggcagaaggtcctgcaggtcctggctcatgatctcgtagctcatgtctgggctgtgggggctgtcaccgtggttacgagcatccaccgtcagcacctaggaggcccagatgaagaacctggggccactctgccagagaagagcaggccccagggttgtgaccacgtctctgaagggctggcctggctgggtggcaatctcggagaatgccaggaaggagactccaggaatttccaacagtaggagcacagaagaatgggctgccataagaggtggtgagctcccggtcatccctagtgaacaagcaggccccttcatggaaagggtgcaggcgcctaggcatgggccagccccgatggagatcctacggcctgtctgctgggccaagatcttggcgatggagttgaagttagttttgc

SEQ ID NO: 13410 - RNA, 1447 nt, Homo sapiens
  source 1..1447: mol_type = other RNA
gctgggattacaggcatgagccaccacgcccggccatcttcttgccagcaactcttagaccaggaagcctcggatggcagctatgaagtcctgtgggcggtcagcgtggatccagtggccagcgttcggcaccgtctgcatctgggcccgagggaagagccgcataatctcagggtggtggctgggatgcacgaactgggagtttccaccaaggagaaagagtgttggcccgaggtaggactcctgcctctgtgggaaagccaagatcttgtctaggtgctgggtcagggcatccaagttcaccctccacacgaagcgcccgtctacctctaccaggttagtgagcaggtgctgccgcacggccatgtcctggatgacagaactgagctgttcatccgccagttttcgggcacgggagcggggcagctcatctgcgatgttgatggccctcatggctgccacataggttgcaaagtgggagacacctgtgctttccactgggctgatatctacagcaatgagacgttccaccagctctggcctctgtagtgccagcagcatggctgtctttcctcccatgctgtggccaacgacgacgcagggcaccaggcccagctggggcagaaggtcctgcaggtcctggctcatgatctcgtagctcatgtctgggctgtgggggctgtcaccgtggttacgagcatccaccgtcagcacctggggagtggggtgagacggggctgcgttgatatccccattctgggggtagacagccaaaggcttgtagggacagcaggtcaaaggtgtggagagcctggggatacaccctgtggaggggaagggcccagtttccagacctaggaggcccagatgaagaacctggggccactctgccagagaagagcaggccccagggttgtgaccacgtctctgaagggctggcctggctgggtggcaatctcggagaatgccaggaaggagactccaggaatttccaacagtaggagcacagaagaatgggctgccataagaggtggtgagctcccggtcatccctagtgaacaagcaggccccttcatggaaagggtgcaggcgcctaggcatgggccagccccgatggagatcctacggcctgtctgctgggccaagatcttggcgatggagttgaagttagttttgctgccgaagagcccgtgcaaaaagacgacggccgggagggctgcctccccgtccagaagcctgtaggaaagcggaagcggcctcggctcggcgccccctcggccgccgctgctgctgctgggtgcgacaggcaccctcgcgaagctagggccgtgggggccgagtccctcacgcgggagcctccaggctcgggtccagcggagcatgcttgcaagctgttggccggctcgcatctcacaaggtacgtcctccccgcgctccttctcccgcc

SEQ ID NO: 13411 - RNA, 1412 nt, Homo sapiens
  source 1..1412: mol_type = other RNA
gctgggattacaggcatgagccaccacgcccggccatcttcttgccagcaactcttagaccaggaagcctcggatggcagctatgaagtcctgtgggcggtcagcgtggatccagtggccagcgttcggcaccgtctgcatctgggcccgagggaagagccgcataatctcagggtggtggctgggatgcacgaactgggagtttccaccaaggagaaagagtgttggcccgaggtaggactcctgcctctgtgggaaagccaagatcttgtctaggtgctgggtcagggcatccaagttcaccctccacacgaagcgcccgtctacctctaccaggttagtgagcaggtgctgccgcacggccatgtcctggatgacagaactgagctgttcatccgccagttttcgggcacgggagcggggcagctcatctgcgatgttgatggccctcatggctgccacataggttgcaaagtgggagacacctgtgctttccactgggctgatatctacagcaatgagacgttccaccagctctggcctctgtagtgccagcagcatggctgtctttcctcccatgctgtggccaacgacgacgcagggcaccaggcccagctggggcagaaggtcctgcaggtcctggctcatgatctcgtagctcatgtctgggctgtgggggctgtcaccgtggttacgagcatccaccgtcagcacctggggccactctgccagagaagagcaggccccagggttgtgaccacgtctctgaagggctggcctggctgggtggcaatctcggagaatgccaggaaggagactccaggaatttccaacagtaggagcacagaagaatgggctgccataagaggtggtgagctcccggtcatcccctacggcctgtctgctgggccaagatcttggcgatggagttgaagttagttttgctgccgaagagcccgtgcaaaaagacgacggccgggagggctgcctccccgtccagaagcctgtaggaaagcggaagcggcctggcaggggaaggatcgaggtcagagtctgagccggcggagacggggaaaggggtagggggaaagagctttgggggagaggcctgggaggtgacaggcccaaagggaggagatggggccgtcggggcccggcaggaaaaggaggacagaggatggcctcccgcccggtgcccttgactgacctcggctcggcgccccctcggccgccgctgctgctgctgggtgcgacaggcaccctcgcgaagctagggccgtgggggccgagtccctcacgcgggagcctccaggctcgggtccagcggagcatgcttgcaagctgttggccggctcgcatctcacaaggtacgtcctccccgcgctccttctcccgccctagctcgcagcccc

SEQ ID NO: 13412 - RNA, 1002 nt, Homo sapiens
  source 1..1002: mol_type = other RNA
gctgggattacaggcatgagccaccacgcccggccatcttcttgccagcaactcttagaccaggaagcctcggatggcagctatgaagtcctgtgggcggtcagcgtggatccagtggccagcgttcggcaccgtctgcatctgggcccgagggaagagccgcataatctcagggtggtggctgggatgcacgaactgggagtttccaccaaggagaaagagtgttggcccgaggtaggactcctgcctctgtgggaaagccaagatcttgtctaggtgctgggtcagggcatccaagttcaccctccacacgaagcgcccgtctacctctaccaggttagtgagcaggtgctgccgcacggccatgtcctggatgacagaactgagctgttcatccgccagttttcgggcacgggagcggggcagctcatctgcgatgttgatggccctcatggctgccacataggttgcaaagtgggagacacctgtgctttccactgggctgatatctacagcaatgagacgttccaccagctctggcctctgtagtgccagcagcatggctgtctttcctcccatgctgtggccaacgacgacgcagggcaccaggcccagctggggcagaaggtcctgcaggtcctggctcatgatctcgtagctcatgtctgggctgtgggggctgtcaccgtggttacgagcatccaccgtcagcacggcctgtctgctgggccaagatcttggcgatggagttgaagttagttttgctgccgaagagcccgtgcaaaaagacgacggccgggagggctgcctccccgtccagaagcctgtaggaaagcggaagcggcctcggctcggcgccccctcggccgccgctgctgctgctgggtgcgacaggcaccctcgcgaagctagggccgtgggggccgagtccctcacgcgggagcctccaggctcgggtccagcggagcatgcttgcaagctgttggccggctcgcatctcac

SEQ ID NO: 13413 - RNA, 946 nt, Homo sapiens
  source 1..946: mol_type = other RNA
gctgggattacaggcatgagccaccacgcccggccatcttcttgccagcaactcttagaccaggaagcctcggatggcagctatgaagtcctgtgggcggtcagcgtggatccagtggccagcgttcggcaccgtctgcatctgggcccgagggaagagccgcataatctcagggtggtggctgggatgcacgaactgggagtttccaccaaggagaaagagtgttggcccgaggtaggactcctgcctctgtgggaaagccaagatcttgtctaggtgctgggtcagggcatccaagttcaccctccacacgaagcgcccgtctacctctaccaggttagtgagcaggtgctgccgcacggccatgtcctgtgggggtgcagcagttgggggaggttccttgtgcggtctgggggtgccactcttcccttgacaggtcctggtctacaataccatccggggcaccttgggtgtatcaccctctgtagtgccagcagcatggctgtctttcctcccatgctgtggccaacgacgacgcagggcaccaggcccagctggggcagaaggtcctgcaggtcctggctcatgatctcgtagctcatgtctgggctgtgggggctgtcaccgtggttacgagcatccaccgtcagcaccctacggcctgtctgctgggccaagatcttggcgatggagttgaagttagttttgctgccgaagagcccgtgcaaaaagacgacggccgggagggctgcctccccgtccagaagcctgtaggaaagcggaagcggcctcggctcggcgccccctcggccgccgctgctgctgctgggtgcgacaggcaccctcgcgaagctagggccgtgggggccgagtccctcacgcgggagcctccaggctcgggtccagcggagcatgcttgcaagctgttggccggctcgcatctcac

SEQ ID NO: 13414 - RNA, 1367 nt, Homo sapiens
  source 1..1367: mol_type = other RNA
gctgggattacaggcatgagccaccacgcccggccatcttcttgccagcaactcttagaccaggaagcctcggatggcagctatgaagtcctgtgggcggtcagcgtggatccagtggccagcgttcggcaccgtctgcatctgggcccgagggaagagccgcataatctcagggtggtggctgggatgcacgaactgggagtttccaccaaggagaaagagtgttggcccgaggtaggactcctgcctctgtgggaaagccaagatcttgtctaggtgctgggtcagggcatccaagttcaccctccacacgaagcgcccgtctacctctaccaggttagtgagcaggtgctgccgcacggccatgtcctgtgggggtgcagcagttgggggaggttccttgtgcggtctgggggtgccactcttcccttgacaggtcctggtctacaataccatccggggcaccttgggtgtatcaccctctgtagtgccagcagcatggctgtctttcctcccatgctgtggccaacgacgacgcagggcaccaggcccagctggggcagaaggtcctgcaggtcctggctcatgatctcgtagctcatgtctgggctgtgggggctgtcaccgtggttacgagcatccaccgtcagcacctggggccactctgccagagaagagcaggccccagggttgtgaccacgtctctgaagggctggcctggctgggtggcaatctcggagaatgccaggaaggagactccaggaatttccaacagtaggagcacagaagaatgggctgccataagaggtggtgagctcccggtcatcccctacggcctgtctgctgggccaagatcttggcgatggagttgaagttagttttgctgccgaagagcccgtgcaaaaagacgacggccgggagggctgcctccccgtccagaagcctgtaggaaagcggaagcggcctggcaggggaaggatcgaggtcagagtctgagccggcggagacggggaaaggggtagggggaaagagctttgggggagaggcctgggaggtgacaggcccaaagggaggagatggggccgtcggggcccggcaggaaaaggaggacagaggatggcctcccgcccggtgcccttgactgacctcggctcggcgccccctcggccgccgctgctgctgctgggtgcgacaggcaccctcgcgaagctagggccgtgggggccgagtccctcacgcgggagcctccaggctcgggtccagcggagcatgcttgcaagctgttggccggctcgcatctcacaaggtacgtcctccccgcgctccttctcccgccctagctcgcagccccgcccatttccgtcttc

SEQ ID NO: 13415 - RNA, 3922 nt, Homo sapiens
  source 1..3922: mol_type = other RNA
gctgggattacaggcatgagccaccacgcccggcccacttacactttttaaacttcttcctcttctcctatacctaagggctccaatgatactacttatcagggaagaaagtactgtatctagataaactacccttaagtattacaggcttagcaagttgaatttctagaaaatactcattcataatttatttatttattttttttgagacagagtcttgctctgttgcccaggctggagtgcagtggcgtgatcttggctcactgcaagctctgcctcccgggttcccaccattctcctgcctcagcctcccgagtagctgggactgcaggtgcccgccaccacgcccggctaatttttttgtagtagagatggggtttcagtggtagccaggatggtcttgatctcctgacctcgtgatccacctgcctcgacctcccaaagtgctgggattacaggtgtgaggcaccgtgcctgtccactaattcatattttaaaagaggactgagcaaagacagcaatggaacctctggctgcaggagatgcctgggtatgcctgatatgtaaacaaacacaagcagtcgagttcaggccatgcatcttcaaagtgacgaagaatatatgtaaatgcttgtttttctcctccatatttctcgtgtagaggtatatgagaatttagcatcaagacgctatactgcaaaccctgttctgtgttgcctatattcatagcataatatttaataaatactcccaaggttgtcattgctggtcacatattagctgacaaaggcacactgaagggactttgattcttactgtaaaatgcaaagattgttttaaactactcaacatatacaatcttaaactatgtgatgattattctcgatcatttatgataatttcaattctaaaagattactaaaaaaaattggttgtagggtatctgaaaacaaaaatagaatgtactccataaagtacatgcacagaatttttaaaaatgcaggcatacaaatatttaatggcagagtggtaataacctgagactttttaaaaatggcaaaacaatatttcagcaatttttggaaaaaaaacccaaatattttccctaagaagtctctcttggcaactttctttttaagcaacaaagcagcagcaacatttttaaatgttcataaagctcgctttccattaacaagtttattaaggaagagtggtcctgaaacttcaggataaaacttttgataaaaatagaatcactaattttgacctaaaacagacactaaaacacccctccttccaatttaagagtgtcatttatacctcctacttacagtaaataaatcaaattaattataagatttcaaatggaaaatctgaaacacatatcaacatcattttcttctaataagataacagaaattaacttcaatggatttccccaaaaagagaatagtttctaaaaacttaattacagctgtggtaaatgaatctgggtttaccaatctcagatctcaatgcacttagttttagttggtattctgtgagatggctagaattcctgatttaagtatgtagtatgtatgtttttaaggcaaggcaagtttgagtatgtataaagcatagatattagcatggttataaaggcaatatgaccgacatacacattcagttttctgaagcaatatattccaagctacatacaatttaatttcatgtcctattctaagactacatgcttaacattaagcttagaaacataattgctgtaatacattaaaaatacttcattttccaatattgtaaagtatatttccaaatacctggtataaatttttttttgcacaaaaatttaaaggacatcctacagctagctattactactgcgttaagtaatcatttgaaggaagaattcacaaggagagcaggttataaaactaagcataataattattgcatttaactaaaaaaaatcaagtagttctgaattacacttgttttttgtcttagtaatgtgcatattcactttctagctactagtttgataaatatactaagattgtataagatttgtttttcttgtttttgtttttcttgggtggttatttttcttttctgtgtccttccccaacagcagttggaattttcttttgaacacaaagtaaattaatgtttatactgttttttcacctgagtcatgtaaaaggtgactcctttcattttaaaaagttatatttaatttttgggggccttaattaaaatttaacatttaaccatgtgttttttttttgtaaacagtctacatgtcaacaaatggataagggttaacaaaggcaaatactgacttcatttgtgttttaaacacgattatatgaatttttcttttttaattaaaaaaatgacataaaaccattcatataggtcctcttctctcaactgctttgagatatagctttaaatatgggtagatcaagacaagtaatgttggtaatctcttatcttgcatagaaaagaaaaaataaaggaacttatttccttcctaaggtctcagctagtttcttaagtcttttcttcagctccaatggaaatttctcatagcacttcttacagactggcttcatgtcaaactccacaaacttattccaaaggagaaagcagtgaaaatgatgacacagggatagaaaagtttacaaacagactggctttttctttttctgcttgtccttatcctttgcttctctctcccgtttggcaagtcgcctcttaaattcttctggcattttctcataacagtgtttgcagactggctttaggtcaatttcaacaaacttatccttgagtgttaatttagtgttgcaggtagaacaggcaaagcagttcacgcaccaggccttattaagagcagagaccacatcaccttctataacacgattgcagtggaagcaaacatcaccaaatagctggttatagtgagtttcacaatatgccaggcctttcctctcataatggcgatgtccaagaaagggtttctcacacttggcacaaacaaaatgctccacatgccactgcttgcccatagcgttcaccacgcgcccttcgatgggccgtcggcaagcaccacagatggggacccccattttatcatggcatgggaggcagtatagctcccctttcagctcccgtgcatcggcagtcagctccttcccgcagttggcgcagttgaaatggtctggatggtaggggtcgttcttgaatatcagaggctgctcatcgatgatagcatggcatttctggcagatgtatttcccaaggcctctggctttctcacgattatgacaggggcgacacaggtgtctcccagcattcttgacaaacccgatatctgccagaacttcctggcagaggtcacagcggaagcactccggatgccagctgttattcatggctttgataactcggccaatgatgaattcaccacactgatgacagcaaggggcaaagagcatctgaaagtcatgttcacagtactttcttccttcaaactcatagaagagtccttctgggaactgctggaagcactgagcgcacacgaaacactgctcatggtacagctccccattactgttcacgatcttctcagcgggcgcaaagccgcccttgcagcgctcgcaagtggcgctggccagggcgttggccatgttgaatttcgcataaaagtcacagaactccttgtagactttcacgtcactgtgcctgcgctgcagtttggaaacagccctctcgtcctcggtcccattggcctcgtggacagtgttaagggctgctcgggggatttcttcgttctctgggataatgcaggggcgcgctcggcctgagaaggccatcgtgggtgcttgagagctctgagcacagggacgagaatggc

SEQ ID NO: 13416 - RNA, 3824 nt, Homo sapiens
  source 1..3824: mol_type = other RNA
gctgggattacaggcatgagccaccacgcccggcccacttacactttttaaacttcttcctcttctcctatacctaagggctccaatgatactacttatcagggaagaaagtactgtatctagataaactacccttaagtattacaggcttagcaagttgaatttctagaaaatactcattcataatttatttatttattttttttgagacagagtcttgctctgttgcccaggctggagtgcagtggcgtgatcttggctcactgcaagctctgcctcccgggttcccaccattctcctgcctcagcctcccgagtagctgggactgcaggtgcccgccaccacgcccggctaatttttttgtagtagagatggggtttcagtggtagccaggatggtcttgatctcctgacctcgtgatccacctgcctcgacctcccaaagtgctgggattacaggtgtgaggcaccgtgcctgtccactaattcatattttaaaagaggactgagcaaagacagcaatggaacctctggctgcaggagatgcctgggtatgcctgatatgtaaacaaacacaagcagtcgagttcaggccatgcatcttcaaagtgacgaagaatatatgtaaatgcttgtttttctcctccatatttctcgtgtagaggtatatgagaatttagcatcaagacgctatactgcaaaccctgttctgtgttgcctatattcatagcataatatttaataaatactcccaaggttgtcattgctggtcacatattagctgacaaaggcacactgaagggactttgattcttactgtaaaatgcaaagattgttttaaactactcaacatatacaatcttaaactatgtgatgattattctcgatcatttatgataatttcaattctaaaagattactaaaaaaaattggttgtagggtatctgaaaacaaaaatagaatgtactccataaagtacatgcacagaatttttaaaaatgcaggcatacaaatatttaatggcagagtggtaataacctgagactttttaaaaatggcaaaacaatatttcagcaatttttggaaaaaaaacccaaatattttccctaagaagtctctcttggcaactttctttttaagcaacaaagcagcagcaacatttttaaatgttcataaagctcgctttccattaacaagtttattaaggaagagtggtcctgaaacttcaggataaaacttttgataaaaatagaatcactaattttgacctaaaacagacactaaaacacccctccttccaatttaagagtgtcatttatacctcctacttacagtaaataaatcaaattaattataagatttcaaatggaaaatctgaaacacatatcaacatcattttcttctaataagataacagaaattaacttcaatggatttccccaaaaagagaatagtttctaaaaacttaattacagctgtggtaaatgaatctgggtttaccaatctcagatctcaatgcacttagttttagttggtattctgtgagatggctagaattcctgatttaagtatgtagtatgtatgtttttaaggcaaggcaagtttgagtatgtataaagcatagatattagcatggttataaaggcaatatgaccgacatacacattcagttttctgaagcaatatattccaagctacatacaatttaatttcatgtcctattctaagactacatgcttaacattaagcttagaaacataattgctgtaatacattaaaaatacttcattttccaatattgtaaagtatatttccaaatacctggtataaatttttttttgcacaaaaatttaaaggacatcctacagctagctattactactgcgttaagtaatcatttgaaggaagaattcacaaggagagcaggttataaaactaagcataataattattgcatttaactaaaaaaaatcaagtagttctgaattacacttgttttttgtcttagtaatgtgcatattcactttctagctactagtttgataaatatactaagattgtataagatttgtttttcttgtttttgtttttcttgggtggttatttttcttttctgtgtccttccccaacagcagttggaattttcttttgaacacaaagtaaattaatgtttatactgttttttcacctgagtcatgtaaaaggtgactcctttcattttaaaaagttatatttaatttttgggggccttaattaaaatttaacatttaaccatgtgttttttttttgtaaacagtctacatgtcaacaaatggataagggttaacaaaggcaaatactgacttcatttgtgttttaaacacgattatatgaatttttcttttttaattaaaaaaatgacataaaaccattcatataggtcctcttctctcaactgctttgagatatagctttaaatatgggtagatcaagacaagtaatgttggtaatctcttatcttgcatagaaaagaaaaaataaaggaacttatttccttcctaaggtctcagctagtttcttaagtcttttcttcagctccaatggaaatttctcatagcacttcttacagactggcttcatgtcaaactccacaaacttattccaaaggagaaagcagtgaaaatgatgacacagggatagaaaagtttacaaacagactggctttttctttttctgcttgtccttatcctttgcttctctctcccgtttggcaagtcgcctcttaaattcttctggcattttctcataacagtgtttgcagactggctttaggtcaatttcaacaaacttatccttgagtgttaatttagtgttgcaggtagaacaggcaaagcagttcacgcaccaggccttattaagagcagagaccacatcaccttctataacacgattgcagtggaagcaaacatcaccaaatagctggttatagtgagtttcacaatatgccaggcctttcctctcataatggcgatgtccaagaaagggtttctcacacttggcacaaacaaaatgctccacatgccactgcttgcccatagcgttcaccacgcgcccttcgatgggccgtcggcaagcaccacagatggggacccccattttatcatggcatgggaggcagtatagctcccctttcagctcccgtgcatcggcagtcagctccttcccgcagttggcgcagttgaaatggtctggatggtaggggtcgttcttgaatatcagaggctgctcatcgatgatagcatggcatttctggcagatgtatttcccaaggcctctggctttctcacgattatgacaggggcgacacaggtgtctcccagcattcttgacaaacccgatatctgccagaacttcctggcagaggtcacagcggaagcactccggatgccagctgttattcatggctttgataactcggccaatgatgaattcaccacactgatgacagcaaggggcaaagagcatctgaaagtcatgttcacagtactttcttccttcaaactcatagaagagtccttctgggaactgctggaagcactgagcgcacacgaaacactgctcatggtacagctccccattactgttcacgatcttctcagcgggcgcaaagccgcccttgcagcgctcgcaagtggcgctggccagggcgttggccatgttgctgtgggtcatcccggccgccacgcccagcatctctccgctttcggccgccgccgtctctcagcccctcgtctcccggcgccgctccagccgcgtcctagtccctcgccgccgcggccggctact

SEQ ID NO: 13417 - RNA, 3730 nt, Homo sapiens
  source 1..3730: mol_type = other RNA
gctgggattacaggcatgagccaccacgcccggcccacttacactttttaaacttcttcctcttctcctatacctaagggctccaatgatactacttatcagggaagaaagtactgtatctagataaactacccttaagtattacaggcttagcaagttgaatttctagaaaatactcattcataatttatttatttattttttttgagacagagtcttgctctgttgcccaggctggagtgcagtggcgtgatcttggctcactgcaagctctgcctcccgggttcccaccattctcctgcctcagcctcccgagtagctgggactgcaggtgcccgccaccacgcccggctaatttttttgtagtagagatggggtttcagtggtagccaggatggtcttgatctcctgacctcgtgatccacctgcctcgacctcccaaagtgctgggattacaggtgtgaggcaccgtgcctgtccactaattcatattttaaaagaggactgagcaaagacagcaatggaacctctggctgcaggagatgcctgggtatgcctgatatgtaaacaaacacaagcagtcgagttcaggccatgcatcttcaaagtgacgaagaatatatgtaaatgcttgtttttctcctccatatttctcgtgtagaggtatatgagaatttagcatcaagacgctatactgcaaaccctgttctgtgttgcctatattcatagcataatatttaataaatactcccaaggttgtcattgctggtcacatattagctgacaaaggcacactgaagggactttgattcttactgtaaaatgcaaagattgttttaaactactcaacatatacaatcttaaactatgtgatgattattctcgatcatttatgataatttcaattctaaaagattactaaaaaaaattggttgtagggtatctgaaaacaaaaatagaatgtactccataaagtacatgcacagaatttttaaaaatgcaggcatacaaatatttaatggcagagtggtaataacctgagactttttaaaaatggcaaaacaatatttcagcaatttttggaaaaaaaacccaaatattttccctaagaagtctctcttggcaactttctttttaagcaacaaagcagcagcaacatttttaaatgttcataaagctcgctttccattaacaagtttattaaggaagagtggtcctgaaacttcaggataaaacttttgataaaaatagaatcactaattttgacctaaaacagacactaaaacacccctccttccaatttaagagtgtcatttatacctcctacttacagtaaataaatcaaattaattataagatttcaaatggaaaatctgaaacacatatcaacatcattttcttctaataagataacagaaattaacttcaatggatttccccaaaaagagaatagtttctaaaaacttaattacagctgtggtaaatgaatctgggtttaccaatctcagatctcaatgcacttagttttagttggtattctgtgagatggctagaattcctgatttaagtatgtagtatgtatgtttttaaggcaaggcaagtttgagtatgtataaagcatagatattagcatggttataaaggcaatatgaccgacatacacattcagttttctgaagcaatatattccaagctacatacaatttaatttcatgtcctattctaagactacatgcttaacattaagcttagaaacataattgctgtaatacattaaaaatacttcattttccaatattgtaaagtatatttccaaatacctggtataaatttttttttgcacaaaaatttaaaggacatcctacagctagctattactactgcgttaagtaatcatttgaaggaagaattcacaaggagagcaggttataaaactaagcataataattattgcatttaactaaaaaaaatcaagtagttctgaattacacttgttttttgtcttagtaatgtgcatattcactttctagctactagtttgataaatatactaagattgtataagatttgtttttcttgtttttgtttttcttgggtggttatttttcttttctgtgtccttccccaacagcagttggaattttcttttgaacacaaagtaaattaatgtttatactgttttttcacctgagtcatgtaaaaggtgactcctttcattttaaaaagttatatttaatttttgggggccttaattaaaatttaacatttaaccatgtgttttttttttgtaaacagtctacatgtcaacaaatggataagggttaacaaaggcaaatactgacttcatttgtgttttaaacacgattatatgaatttttcttttttaattaaaaaaatgacataaaaccattcatataggtcctcttctctcaactgctttgagatatagctttaaatatgggtagatcaagacaagtaatgttggtaatctcttatcttgcatagaaaagaaaaaataaaggaacttatttccttcctaaggtctcagctagtttcttaagtcttttcttcagctccaatggaaatttctcatagcacttcttacagactggcttcatgtcaaactccacaaacttattcttgagtgttaatttagtgttgcaggtagaacaggcaaagcagttcacgcaccaggccttattaagagcagagaccacatcaccttctataacacgattgcagtggaagcaaacatcaccaaatagctggttatagtgagtttcacaatatgccaggcctttcctctcataatggcgatgtccaagaaagggtttctcacacttggcacaaacaaaatgctccacatgccactgcttgcccatagcgttcaccacgcgcccttcgatgggccgtcggcaagcaccacagatggggacccccattttatcatggcatgggaggcagtatagctcccctttcagctcccgtgcatcggcagtcagctccttcccgcagttggcgcagttgaaatggtctggatggtaggggtcgttcttgaatatcagaggctgctcatcgatgatagcatggcatttctggcagatgtatttcccaaggcctctggctttctcacgattatgacaggggcgacacaggtgtctcccagcattcttgacaaacccgatatctgccagaacttcctggcagaggtcacagcggaagcactccggatgccagctgttattcatggctttgataactcggccaatgatgaattcaccacactgatgacagcaaggggcaaagagcatctgaaagtcatgttcacagtactttcttccttcaaactcatagaagagtccttctgggaactgctggaagcactgagcgcacacgaaacactgctcatggtacagctccccattactgttcacgatcttctcagcgggcgcaaagccgcccttgcagcgctcgcaagtggcgctggccagggcgttggccatgttgaatttcgcataaaagtcacagaactccttgtagactttcacgtcactgtgcctgcgctgcagtttggaaacagccctctcgtcctcggtcccattggcctcgtggacagtgttaagggctgctcgggggatttcttcgttctctgggataatgcaggggcgcgctcggcctgagaaggccatcgtgggtgcttgagagctctgagcacagggacgagaatggc

SEQ ID NO: 13418 - RNA, 3616 nt, Homo sapiens
  source 1..3616: mol_type = other RNA
gctgggattacaggcatgagccaccacgcccggcccacttacactttttaaacttcttcctcttctcctatacctaagggctccaatgatactacttatcagggaagaaagtactgtatctagataaactacccttaagtattacaggcttagcaagttgaatttctagaaaatactcattcataatttatttatttattttttttgagacagagtcttgctctgttgcccaggctggagtgcagtggcgtgatcttggctcactgcaagctctgcctcccgggttcccaccattctcctgcctcagcctcccgagtagctgggactgcaggtgcccgccaccacgcccggctaatttttttgtagtagagatggggtttcagtggtagccaggatggtcttgatctcctgacctcgtgatccacctgcctcgacctcccaaagtgctgggattacaggtgtgaggcaccgtgcctgtccactaattcatattttaaaagaggactgagcaaagacagcaatggaacctctggctgcaggagatgcctgggtatgcctgatatgtaaacaaacacaagcagtcgagttcaggccatgcatcttcaaagtgacgaagaatatatgtaaatgcttgtttttctcctccatatttctcgtgtagaggtatatgagaatttagcatcaagacgctatactgcaaaccctgttctgtgttgcctatattcatagcataatatttaataaatactcccaaggttgtcattgctggtcacatattagctgacaaaggcacactgaagggactttgattcttactgtaaaatgcaaagattgttttaaactactcaacatatacaatcttaaactatgtgatgattattctcgatcatttatgataatttcaattctaaaagattactaaaaaaaattggttgtagggtatctgaaaacaaaaatagaatgtactccataaagtacatgcacagaatttttaaaaatgcaggcatacaaatatttaatggcagagtggtaataacctgagactttttaaaaatggcaaaacaatatttcagcaatttttggaaaaaaaacccaaatattttccctaagaagtctctcttggcaactttctttttaagcaacaaagcagcagcaacatttttaaatgttcataaagctcgctttccattaacaagtttattaaggaagagtggtcctgaaacttcaggataaaacttttgataaaaatagaatcactaattttgacctaaaacagacactaaaacacccctccttccaatttaagagtgtcatttatacctcctacttacagtaaataaatcaaattaattataagatttcaaatggaaaatctgaaacacatatcaacatcattttcttctaataagataacagaaattaacttcaatggatttccccaaaaagagaatagtttctaaaaacttaattacagctgtggtaaatgaatctgggtttaccaatctcagatctcaatgcacttagttttagttggtattctgtgagatggctagaattcctgatttaagtatgtagtatgtatgtttttaaggcaaggcaagtttgagtatgtataaagcatagatattagcatggttataaaggcaatatgaccgacatacacattcagttttctgaagcaatatattccaagctacatacaatttaatttcatgtcctattctaagactacatgcttaacattaagcttagaaacataattgctgtaatacattaaaaatacttcattttccaatattgtaaagtatatttccaaatacctggtataaatttttttttgcacaaaaatttaaaggacatcctacagctagctattactactgcgttaagtaatcatttgaaggaagaattcacaaggagagcaggttataaaactaagcataataattattgcatttaactaaaaaaaatcaagtagttctgaattacacttgttttttgtcttagtaatgtgcatattcactttctagctactagtttgataaatatactaagattgtataagatttgtttttcttgtttttgtttttcttgggtggttatttttcttttctgtgtccttccccaacagcagttggaattttcttttgaacacaaagtaaattaatgtttatactgttttttcacctgagtcatgtaaaaggtgactcctttcattttaaaaagttatatttaatttttgggggccttaattaaaatttaacatttaaccatgtgttttttttttgtaaacagtctacatgtcaacaaatggataagggttaacaaaggcaaatactgacttcatttgtgttttaaacacgattatatgaatttttcttttttaattaaaaaaatgacataaaaccattcatataggtcctcttctctcaactgctttgagatatagctttaaatatgggtagatcaagacaagtaatgttggtaatctcttatcttgcatagaaaagaaaaaataaaggaacttatttccttcctaaggtctcagctagtttcttaagtcttttcttcagctccaatggaaatttctcatagcacttcttacagactggcttcatgtcaaactccacaaacttattcttgagtgttaatttagtgttgcaggtagaacaggcaaagcagttcacgcaccaggccttattaagagcagagaccacatcaccttctataacacgattgcagtggaagcaaacatcaccaaatagctggttatagtgagtttcacaatatgccaggcctttcctctcataatggcgatgtccaagaaagggtttctcacacttggcacaaacaaaatgctccacatgccactgcttgcccatagcgttcaccacgcgcccttcgatgggccgtcggcaagcaccacagatggggacccccattttatcatggcatgggaggcagtatagctcccctttcagctcccgtgcatcggcagtcagctccttcccgcagttggcgcagttgaaatggtctggatggtaggggtcgttcttgaatatcagaggctgctcatcgatgatagcatggcatttctggcagatgtatttcccaaggcctctggctttctcacgattatgacaggggcgacacaggtgtctcccagcattcttgacaaacccgatatctgccagaacttcctggcagaggtcacagcggaagcactccggatgccagctgttattcatggctttgataactcggccaatgatgaattcaccacactgatgacagcaaggggcaaagagcatctgaaagtcatgttcacagtactttcttccttcaaactcatagaagagtccttctgggaactgctggaagcactgagcgcacacgaaacactgctcatggtacagctccccattactgttcacgatcttctcagcgggcgcaaagccgcccttgcagcgctcgcaagtggcgctggccagggcgttggccatgttgcatgtcatgtatcttgattcgatgtgtccctcatcagctggctgtccaagctaagctctccatgctcatagatggcaccctctcactgtgtcctcacatgcaggaaggg

SEQ ID NO: 13419 - RNA, 3830 nt, Homo sapiens
  source 1..3830: mol_type = other RNA
gctgggattacaggcatgagccaccacgcccggcccacttacactttttaaacttcttcctcttctcctatacctaagggctccaatgatactacttatcagggaagaaagtactgtatctagataaactacccttaagtattacaggcttagcaagttgaatttctagaaaatactcattcataatttatttatttattttttttgagacagagtcttgctctgttgcccaggctggagtgcagtggcgtgatcttggctcactgcaagctctgcctcccgggttcccaccattctcctgcctcagcctcccgagtagctgggactgcaggtgcccgccaccacgcccggctaatttttttgtagtagagatggggtttcagtggtagccaggatggtcttgatctcctgacctcgtgatccacctgcctcgacctcccaaagtgctgggattacaggtgtgaggcaccgtgcctgtccactaattcatattttaaaagaggactgagcaaagacagcaatggaacctctggctgcaggagatgcctgggtatgcctgatatgtaaacaaacacaagcagtcgagttcaggccatgcatcttcaaagtgacgaagaatatatgtaaatgcttgtttttctcctccatatttctcgtgtagaggtatatgagaatttagcatcaagacgctatactgcaaaccctgttctgtgttgcctatattcatagcataatatttaataaatactcccaaggttgtcattgctggtcacatattagctgacaaaggcacactgaagggactttgattcttactgtaaaatgcaaagattgttttaaactactcaacatatacaatcttaaactatgtgatgattattctcgatcatttatgataatttcaattctaaaagattactaaaaaaaattggttgtagggtatctgaaaacaaaaatagaatgtactccataaagtacatgcacagaatttttaaaaatgcaggcatacaaatatttaatggcagagtggtaataacctgagactttttaaaaatggcaaaacaatatttcagcaatttttggaaaaaaaacccaaatattttccctaagaagtctctcttggcaactttctttttaagcaacaaagcagcagcaacatttttaaatgttcataaagctcgctttccattaacaagtttattaaggaagagtggtcctgaaacttcaggataaaacttttgataaaaatagaatcactaattttgacctaaaacagacactaaaacacccctccttccaatttaagagtgtcatttatacctcctacttacagtaaataaatcaaattaattataagatttcaaatggaaaatctgaaacacatatcaacatcattttcttctaataagataacagaaattaacttcaatggatttccccaaaaagagaatagtttctaaaaacttaattacagctgtggtaaatgaatctgggtttaccaatctcagatctcaatgcacttagttttagttggtattctgtgagatggctagaattcctgatttaagtatgtagtatgtatgtttttaaggcaaggcaagtttgagtatgtataaagcatagatattagcatggttataaaggcaatatgaccgacatacacattcagttttctgaagcaatatattccaagctacatacaatttaatttcatgtcctattctaagactacatgcttaacattaagcttagaaacataattgctgtaatacattaaaaatacttcattttccaatattgtaaagtatatttccaaatacctggtataaatttttttttgcacaaaaatttaaaggacatcctacagctagctattactactgcgttaagtaatcatttgaaggaagaattcacaaggagagcaggttataaaactaagcataataattattgcatttaactaaaaaaaatcaagtagttctgaattacacttgttttttgtcttagtaatgtgcatattcactttctagctactagtttgataaatatactaagattgtataagatttgtttttcttgtttttgtttttcttgggtggttatttttcttttctgtgtccttccccaacagcagttggaattttcttttgaacacaaagtaaattaatgtttatactgttttttcacctgagtcatgtaaaaggtgactcctttcattttaaaaagttatatttaatttttgggggccttaattaaaatttaacatttaaccatgtgttttttttttgtaaacagtctacatgtcaacaaatggataagggttaacaaaggcaaatactgacttcatttgtgttttaaacacgattatatgaatttttcttttttaattaaaaaaatgacataaaaccattcatataggtcctcttctctcaactgctttgagatatagctttaaatatgggtagatcaagacaagtaatgttggtaatctcttatcttgcatagaaaagaaaaaataaaggaacttatttccttcctaaggtctcagctagtttcttaagtcttttcttcagctccaatggaaatttctcatagcacttcttacagactggcttcatgtcaaactccacaaacttattcttgagtgttaatttagtgttgcaggtagaacaggcaaagcagttcacgcaccaggccttattaagagcagagaccacatcaccttctataacacgattgcagtggaagcaaacatcaccaaatagctggttatagtgagtttcacaatatgccaggcctttcctctcataatggcgatgtccaagaaagggtttctcacacttggcacaaacaaaatgctccacatgccactgcttgcccatagcgttcaccacgcgcccttcgatgggccgtcggcaagcaccacagatggggacccccattttatcatggcatgggaggcagtatagctcccctttcagctcccgtgcatcggcagtcagctccttcccgcagttggcgcagttgaaatggtctggatggtaggggtcgttcttgaatatcagaggctgctcatcgatgatagcatggcatttctggcagatgtatttcccaaggcctctggctttctcacgattatgacaggggcgacacaggtgtctcccagcattcttgacaaacccgatatctgccagaacttcctggcagaggtcacagcggaagcactccggatgccagctgttattcatggctttgataactcggccaatgatgaattcaccacactgatgacagcaaggggcaaagagcatctgaaagtcatgttcacagtactttcttccttcaaactcatagaagagtccttctgggaactgctggaagcactgagcgcacacgaaacactgctcatggtacagctccccattactgttcacgatcttctcagcgggcgcaaagccgcccttgcagcgctcgcaagtggcgctggccagggcgttggccatgttgcctgtgtttggctgatttaggcaatcatgtccatttcttctcttaaacttctctcaaacttccactcctttgccttagtcactttacacacacaggcccagttctgcaaacctacgcactctacctgagccacctccagctccccttctcttaattcaagagtaaagaacctccctcctggctcctactcttatttaacttacttatcagggcttgggaggccagtttcacatcactgcgaattatctttgaaagcctctatttcctaaactgtacagaacttcctcatcttagctttgtctctgttgtcttgaactatattt

SEQ ID NO: 13420 - RNA, 3632 nt, Homo sapiens
  source 1..3632: mol_type = other RNA
gctgggattacaggcatgagccaccacgcccggcccacttacactttttaaacttcttcctcttctcctatacctaagggctccaatgatactacttatcagggaagaaagtactgtatctagataaactacccttaagtattacaggcttagcaagttgaatttctagaaaatactcattcataatttatttatttattttttttgagacagagtcttgctctgttgcccaggctggagtgcagtggcgtgatcttggctcactgcaagctctgcctcccgggttcccaccattctcctgcctcagcctcccgagtagctgggactgcaggtgcccgccaccacgcccggctaatttttttgtagtagagatggggtttcagtggtagccaggatggtcttgatctcctgacctcgtgatccacctgcctcgacctcccaaagtgctgggattacaggtgtgaggcaccgtgcctgtccactaattcatattttaaaagaggactgagcaaagacagcaatggaacctctggctgcaggagatgcctgggtatgcctgatatgtaaacaaacacaagcagtcgagttcaggccatgcatcttcaaagtgacgaagaatatatgtaaatgcttgtttttctcctccatatttctcgtgtagaggtatatgagaatttagcatcaagacgctatactgcaaaccctgttctgtgttgcctatattcatagcataatatttaataaatactcccaaggttgtcattgctggtcacatattagctgacaaaggcacactgaagggactttgattcttactgtaaaatgcaaagattgttttaaactactcaacatatacaatcttaaactatgtgatgattattctcgatcatttatgataatttcaattctaaaagattactaaaaaaaattggttgtagggtatctgaaaacaaaaatagaatgtactccataaagtacatgcacagaatttttaaaaatgcaggcatacaaatatttaatggcagagtggtaataacctgagactttttaaaaatggcaaaacaatatttcagcaatttttggaaaaaaaacccaaatattttccctaagaagtctctcttggcaactttctttttaagcaacaaagcagcagcaacatttttaaatgttcataaagctcgctttccattaacaagtttattaaggaagagtggtcctgaaacttcaggataaaacttttgataaaaatagaatcactaattttgacctaaaacagacactaaaacacccctccttccaatttaagagtgtcatttatacctcctacttacagtaaataaatcaaattaattataagatttcaaatggaaaatctgaaacacatatcaacatcattttcttctaataagataacagaaattaacttcaatggatttccccaaaaagagaatagtttctaaaaacttaattacagctgtggtaaatgaatctgggtttaccaatctcagatctcaatgcacttagttttagttggtattctgtgagatggctagaattcctgatttaagtatgtagtatgtatgtttttaaggcaaggcaagtttgagtatgtataaagcatagatattagcatggttataaaggcaatatgaccgacatacacattcagttttctgaagcaatatattccaagctacatacaatttaatttcatgtcctattctaagactacatgcttaacattaagcttagaaacataattgctgtaatacattaaaaatacttcattttccaatattgtaaagtatatttccaaatacctggtataaatttttttttgcacaaaaatttaaaggacatcctacagctagctattactactgcgttaagtaatcatttgaaggaagaattcacaaggagagcaggttataaaactaagcataataattattgcatttaactaaaaaaaatcaagtagttctgaattacacttgttttttgtcttagtaatgtgcatattcactttctagctactagtttgataaatatactaagattgtataagatttgtttttcttgtttttgtttttcttgggtggttatttttcttttctgtgtccttccccaacagcagttggaattttcttttgaacacaaagtaaattaatgtttatactgttttttcacctgagtcatgtaaaaggtgactcctttcattttaaaaagttatatttaatttttgggggccttaattaaaatttaacatttaaccatgtgttttttttttgtaaacagtctacatgtcaacaaatggataagggttaacaaaggcaaatactgacttcatttgtgttttaaacacgattatatgaatttttcttttttaattaaaaaaatgacataaaaccattcatataggtcctcttctctcaactgctttgagatatagctttaaatatgggtagatcaagacaagtaatgttggtaatctcttatcttgcatagaaaagaaaaaataaaggaacttatttccttcctaaggtctcagctagtttcttaagtcttttcttcagctccaatggaaatttctcatagcacttcttacagactggcttcatgtcaaactccacaaacttattcttgagtgttaatttagtgttgcaggtagaacaggcaaagcagttcacgcaccaggccttattaagagcagagaccacatcaccttctataacacgattgcagtggaagcaaacatcaccaaatagctggttatagtgagtttcacaatatgccaggcctttcctctcataatggcgatgtccaagaaagggtttctcacacttggcacaaacaaaatgctccacatgccactgcttgcccatagcgttcaccacgcgcccttcgatgggccgtcggcaagcaccacagatggggacccccattttatcatggcatgggaggcagtatagctcccctttcagctcccgtgcatcggcagtcagctccttcccgcagttggcgcagttgaaatggtctggatggtaggggtcgttcttgaatatcagaggctgctcatcgatgatagcatggcatttctggcagatgtatttcccaaggcctctggctttctcacgattatgacaggggcgacacaggtgtctcccagcattcttgacaaacccgatatctgccagaacttcctggcagaggtcacagcggaagcactccggatgccagctgttattcatggctttgataactcggccaatgatgaattcaccacactgatgacagcaaggggcaaagagcatctgaaagtcatgttcacagtactttcttccttcaaactcatagaagagtccttctgggaactgctggaagcactgagcgcacacgaaacactgctcatggtacagctccccattactgttcacgatcttctcagcgggcgcaaagccgcccttgcagcgctcgcaagtggcgctggccagggcgttggccatgttgctgtgggtcatcccggccgccacgcccagcatctctccgctttcggccgccgccgtctctcagcccctcgtctcccggcgccgctccagccgcgtcctagtccctcgccgccgcggccggctact

SEQ ID NO: 13421 - RNA, 3718 nt, Homo sapiens
  source 1..3718: mol_type = other RNA
gctgggattacaggcatgagccaccacgcccggcccacttacactttttaaacttcttcctcttctcctatacctaagggctccaatgatactacttatcagggaagaaagtactgtatctagataaactacccttaagtattacaggcttagcaagttgaatttctagaaaatactcattcataatttatttatttattttttttgagacagagtcttgctctgttgcccaggctggagtgcagtggcgtgatcttggctcactgcaagctctgcctcccgggttcccaccattctcctgcctcagcctcccgagtagctgggactgcaggtgcccgccaccacgcccggctaatttttttgtagtagagatggggtttcagtggtagccaggatggtcttgatctcctgacctcgtgatccacctgcctcgacctcccaaagtgctgggattacaggtgtgaggcaccgtgcctgtccactaattcatattttaaaagaggactgagcaaagacagcaatggaacctctggctgcaggagatgcctgggtatgcctgatatgtaaacaaacacaagcagtcgagttcaggccatgcatcttcaaagtgacgaagaatatatgtaaatgcttgtttttctcctccatatttctcgtgtagaggtatatgagaatttagcatcaagacgctatactgcaaaccctgttctgtgttgcctatattcatagcataatatttaataaatactcccaaggttgtcattgctggtcacatattagctgacaaaggcacactgaagggactttgattcttactgtaaaatgcaaagattgttttaaactactcaacatatacaatcttaaactatgtgatgattattctcgatcatttatgataatttcaattctaaaagattactaaaaaaaattggttgtagggtatctgaaaacaaaaatagaatgtactccataaagtacatgcacagaatttttaaaaatgcaggcatacaaatatttaatggcagagtggtaataacctgagactttttaaaaatggcaaaacaatatttcagcaatttttggaaaaaaaacccaaatattttccctaagaagtctctcttggcaactttctttttaagcaacaaagcagcagcaacatttttaaatgttcataaagctcgctttccattaacaagtttattaaggaagagtggtcctgaaacttcaggataaaacttttgataaaaatagaatcactaattttgacctaaaacagacactaaaacacccctccttccaatttaagagtgtcatttatacctcctacttacagtaaataaatcaaattaattataagatttcaaatggaaaatctgaaacacatatcaacatcattttcttctaataagataacagaaattaacttcaatggatttccccaaaaagagaatagtttctaaaaacttaattacagctgtggtaaatgaatctgggtttaccaatctcagatctcaatgcacttagttttagttggtattctgtgagatggctagaattcctgatttaagtatgtagtatgtatgtttttaaggcaaggcaagtttgagtatgtataaagcatagatattagcatggttataaaggcaatatgaccgacatacacattcagttttctgaagcaatatattccaagctacatacaatttaatttcatgtcctattctaagactacatgcttaacattaagcttagaaacataattgctgtaatacattaaaaatacttcattttccaatattgtaaagtatatttccaaatacctggtataaatttttttttgcacaaaaatttaaaggacatcctacagctagctattactactgcgttaagtaatcatttgaaggaagaattcacaaggagagcaggttataaaactaagcataataattattgcatttaactaaaaaaaatcaagtagttctgaattacacttgttttttgtcttagtaatgtgcatattcactttctagctactagtttgataaatatactaagattgtataagatttgtttttcttgtttttgtttttcttgggtggttatttttcttttctgtgtccttccccaacagcagttggaattttcttttgaacacaaagtaaattaatgtttatactgttttttcacctgagtcatgtaaaaggtgactcctttcattttaaaaagttatatttaatttttgggggccttaattaaaatttaacatttaaccatgtgttttttttttgtaaacagtctacatgtcaacaaatggataagggttaacaaaggcaaatactgacttcatttgtgttttaaacacgattatatgaatttttcttttttaattaaaaaaatgacataaaaccattcatataggtcctcttctctcaactgctttgagatatagctttaaatatgggtagatcaagacaagtaatgttggtaatctcttatcttgcatagaaaagaaaaaataaaggaacttatttccttcctaaggtctcagctagtttcttaagtcttttcttcagctccaatggaaatttctcatagcacttcttacagactggcttcatgtcaaactccacaaacttattcttgagtgttaatttagtgttgcaggtagaacaggcaaagcagttcacgcaccaggccttattaagagcagagaccacatcaccttctataacacgattgcagtggaagcaaacatcaccaaatagctggttatagtgagtttcacaatatgccaggcctttcctctcataatggcgatgtccaagaaagggtttctcacacttggcacaaacaaaatgctccacatgccactgcttgcccatagcgttcaccacgcgcccttcgatgggccgtcggcaagcaccacagatggggacccccattttatcatggcatgggaggcagtatagctcccctttcagctcccgtgcatcggcagtcagctccttcccgcagttggcgcagttgaaatggtctggatggtaggggtcgttcttgaatatcagaggctgctcatcgatgatagcatggcatttctggcagatgtatttcccaaggcctctggctttctcacgattatgacaggggcgacacaggtgtctcccagcattcttgacaaacccgatatctgccagaacttcctggcagaggtcacagcggaagcactccggatgccagctgttattcatggctttgataactcggccaatgatgaattcaccacactgatgacagcaaggggcaaagagcatctgaaagtcatgttcacagtactttcttccttcaaactcatagaagagtccttctgggaactgctggaagcactgagcgcacacgaaacactgctcatggtacagctccccattactgttcacgatcttctcagcgggcgcaaagccgcccttgcagcgctcgcaagtggcgctggccagggcgttggccatgttgcttagctcttcctctggtaacccatttactctcaaactatcggggcgatctcgtcttctcctgtagagacctgaatgtgaaagctctttaagctgtaatgcagtcatacttctctccacacatcaattgctgacactttaaagcatttatgctcagcagtgtggctgccaggggaaagcagcgtcccttgccgagggacctcagcacacct

SEQ ID NO: 13422 - RNA, 3603 nt, Homo sapiens
  source 1..3603: mol_type = other RNA
gctgggattacaggcatgagccaccacgcccggcccacttacactttttaaacttcttcctcttctcctatacctaagggctccaatgatactacttatcagggaagaaagtactgtatctagataaactacccttaagtattacaggcttagcaagttgaatttctagaaaatactcattcataatttatttatttattttttttgagacagagtcttgctctgttgcccaggctggagtgcagtggcgtgatcttggctcactgcaagctctgcctcccgggttcccaccattctcctgcctcagcctcccgagtagctgggactgcaggtgcccgccaccacgcccggctaatttttttgtagtagagatggggtttcagtggtagccaggatggtcttgatctcctgacctcgtgatccacctgcctcgacctcccaaagtgctgggattacaggtgtgaggcaccgtgcctgtccactaattcatattttaaaagaggactgagcaaagacagcaatggaacctctggctgcaggagatgcctgggtatgcctgatatgtaaacaaacacaagcagtcgagttcaggccatgcatcttcaaagtgacgaagaatatatgtaaatgcttgtttttctcctccatatttctcgtgtagaggtatatgagaatttagcatcaagacgctatactgcaaaccctgttctgtgttgcctatattcatagcataatatttaataaatactcccaaggttgtcattgctggtcacatattagctgacaaaggcacactgaagggactttgattcttactgtaaaatgcaaagattgttttaaactactcaacatatacaatcttaaactatgtgatgattattctcgatcatttatgataatttcaattctaaaagattactaaaaaaaattggttgtagggtatctgaaaacaaaaatagaatgtactccataaagtacatgcacagaatttttaaaaatgcaggcatacaaatatttaatggcagagtggtaataacctgagactttttaaaaatggcaaaacaatatttcagcaatttttggaaaaaaaacccaaatattttccctaagaagtctctcttggcaactttctttttaagcaacaaagcagcagcaacatttttaaatgttcataaagctcgctttccattaacaagtttattaaggaagagtggtcctgaaacttcaggataaaacttttgataaaaatagaatcactaattttgacctaaaacagacactaaaacacccctccttccaatttaagagtgtcatttatacctcctacttacagtaaataaatcaaattaattataagatttcaaatggaaaatctgaaacacatatcaacatcattttcttctaataagataacagaaattaacttcaatggatttccccaaaaagagaatagtttctaaaaacttaattacagctgtggtaaatgaatctgggtttaccaatctcagatctcaatgcacttagttttagttggtattctgtgagatggctagaattcctgatttaagtatgtagtatgtatgtttttaaggcaaggcaagtttgagtatgtataaagcatagatattagcatggttataaaggcaatatgaccgacatacacattcagttttctgaagcaatatattccaagctacatacaatttaatttcatgtcctattctaagactacatgcttaacattaagcttagaaacataattgctgtaatacattaaaaatacttcattttccaatattgtaaagtatatttccaaatacctggtataaatttttttttgcacaaaaatttaaaggacatcctacagctagctattactactgcgttaagtaatcatttgaaggaagaattcacaaggagagcaggttataaaactaagcataataattattgcatttaactaaaaaaaatcaagtagttctgaattacacttgttttttgtcttagtaatgtgcatattcactttctagctactagtttgataaatatactaagattgtataagatttgtttttcttgtttttgtttttcttgggtggttatttttcttttctgtgtccttccccaacagcagttggaattttcttttgaacacaaagtaaattaatgtttatactgttttttcacctgagtcatgtaaaaggtgactcctttcattttaaaaagttatatttaatttttgggggccttaattaaaatttaacatttaaccatgtgttttttttttgtaaacagtctacatgtcaacaaatggataagggttaacaaaggcaaatactgacttcatttgtgttttaaacacgattatatgaatttttcttttttaattaaaaaaatgacataaaaccattcatataggtcctcttctctcaactgctttgagatatagctttaaatatgggtagatcaagacaagtaatgttggtaatctcttatcttgcatagaaaagaaaaaataaaggaacttatttccttcctaaggtctcagctagtttcttaagtcttttcttcagctccaatggaaatttctcatagcacttcttacagactggcttcatgtcaaactccacaaacttattcttgagtgttaatttagtgttgcaggtagaacaggcaaagcagttcacgcaccaggccttattaagagcagagaccacatcaccttctataacacgattgcagtggaagcaaacatcaccaaatagctggttatagtgagtttcacaatatgccaggcctttcctctcataatggcgatgtccaagaaagggtttctcacacttggcacaaacaaaatgctccacatgccactgcttgcccatagcgttcaccacgcgcccttcgatgggccgtcggcaagcaccacagatggggacccccattttatcatggcatgggaggcagtatagctcccctttcagctcccgtgcatcggcagtcagctccttcccgcagttggcgcagttgaaatggtctggatggtaggggtcgttcttgaatatcagaggctgctcatcgatgatagcatggcatttctggcagatgtatttcccaaggcctctggctttctcacgattatgacaggggcgacacaggtgtctcccagcattcttgacaaacccgatatctgccagaacttcctggcagaggtcacagcggaagcactccggatgccagctgttattcatggctttgataactcggccaatgatgaattcaccacactgatgacagcaaggggcaaagagcatctgaaagtcatgttcacagtactttcttccttcaaactcatagaagagtccttctgggaactgctggaagcactgagcgcacacgaaacactgctcatggtacagctccccattactgttcacgatcttctcagcgggcgcaaagccgcccttgcagcgctcgcaagtggcgctggccagggcgttggccatgttgcttcagtctggtcttcctcaaggtcgctgctcacaaccactctcagcactgcggacctccagggctctcccttgctaactcctcccgctcttctcc

SEQ ID NO: 13423 - RNA, 3724 nt, Homo sapiens
  source 1..3724: mol_type = other RNA
gctgggattacaggcatgagccaccacgcccggcccacttacactttttaaacttcttcctcttctcctatacctaagggctccaatgatactacttatcagggaagaaagtactgtatctagataaactacccttaagtattacaggcttagcaagttgaatttctagaaaatactcattcataatttatttatttattttttttgagacagagtcttgctctgttgcccaggctggagtgcagtggcgtgatcttggctcactgcaagctctgcctcccgggttcccaccattctcctgcctcagcctcccgagtagctgggactgcaggtgcccgccaccacgcccggctaatttttttgtagtagagatggggtttcagtggtagccaggatggtcttgatctcctgacctcgtgatccacctgcctcgacctcccaaagtgctgggattacaggtgtgaggcaccgtgcctgtccactaattcatattttaaaagaggactgagcaaagacagcaatggaacctctggctgcaggagatgcctgggtatgcctgatatgtaaacaaacacaagcagtcgagttcaggccatgcatcttcaaagtgacgaagaatatatgtaaatgcttgtttttctcctccatatttctcgtgtagaggtatatgagaatttagcatcaagacgctatactgcaaaccctgttctgtgttgcctatattcatagcataatatttaataaatactcccaaggttgtcattgctggtcacatattagctgacaaaggcacactgaagggactttgattcttactgtaaaatgcaaagattgttttaaactactcaacatatacaatcttaaactatgtgatgattattctcgatcatttatgataatttcaattctaaaagattactaaaaaaaattggttgtagggtatctgaaaacaaaaatagaatgtactccataaagtacatgcacagaatttttaaaaatgcaggcatacaaatatttaatggcagagtggtaataacctgagactttttaaaaatggcaaaacaatatttcagcaatttttggaaaaaaaacccaaatattttccctaagaagtctctcttggcaactttctttttaagcaacaaagcagcagcaacatttttaaatgttcataaagctcgctttccattaacaagtttattaaggaagagtggtcctgaaacttcaggataaaacttttgataaaaatagaatcactaattttgacctaaaacagacactaaaacacccctccttccaatttaagagtgtcatttatacctcctacttacagtaaataaatcaaattaattataagatttcaaatggaaaatctgaaacacatatcaacatcattttcttctaataagataacagaaattaacttcaatggatttccccaaaaagagaatagtttctaaaaacttaattacagctgtggtaaatgaatctgggtttaccaatctcagatctcaatgcacttagttttagttggtattctgtgagatggctagaattcctgatttaagtatgtagtatgtatgtttttaaggcaaggcaagtttgagtatgtataaagcatagatattagcatggttataaaggcaatatgaccgacatacacattcagttttctgaagcaatatattccaagctacatacaatttaatttcatgtcctattctaagactacatgcttaacattaagcttagaaacataattgctgtaatacattaaaaatacttcattttccaatattgtaaagtatatttccaaatacctggtataaatttttttttgcacaaaaatttaaaggacatcctacagctagctattactactgcgttaagtaatcatttgaaggaagaattcacaaggagagcaggttataaaactaagcataataattattgcatttaactaaaaaaaatcaagtagttctgaattacacttgttttttgtcttagtaatgtgcatattcactttctagctactagtttgataaatatactaagattgtataagatttgtttttcttgtttttgtttttcttgggtggttatttttcttttctgtgtccttccccaacagcagttggaattttcttttgaacacaaagtaaattaatgtttatactgttttttcacctgagtcatgtaaaaggtgactcctttcattttaaaaagttatatttaatttttgggggccttaattaaaatttaacatttaaccatgtgttttttttttgtaaacagtctacatgtcaacaaatggataagggttaacaaaggcaaatactgacttcatttgtgttttaaacacgattatatgaatttttcttttttaattaaaaaaatgacataaaaccattcatataggtcctcttctctcaactgctttgagatatagctttaaatatgggtagatcaagacaagtaatgttggtaatctcttatcttgcatagaaaagaaaaaataaaggaacttatttccttcctaaggtctcagctagtttcttaagtcttttcttcagctccaatggaaatttctcatagcacttcttacagactggcttcatgtcaaactccacaaacttattcttgagtgttaatttagtgttgcaggtagaacaggcaaagcagttcacgcaccaggccttattaagagcagagaccacatcaccttctataacacgattgcagtggaagcaaacatcaccaaatagctggttatagtgagtttcacaatatgccaggcctttcctctcataatggcgatgtccaagaaagggtttctcacacttggcacaaacaaaatgctccacatgccactgcttgcccatagcgttcaccacgcgcccttcgatgggccgtcggcaagcaccacagatggggacccccattttatcatggcatgggaggcagtatagctcccctttcagctcccgtgcatcggcagtcagctccttcccgcagttggcgcagttgaaatggtctggatggtaggggtcgttcttgaatatcagaggctgctcatcgatgatagcatggcatttctggcagatgtatttcccaaggcctctggctttctcacgattatgacaggggcgacacaggtgtctcccagcattcttgacaaacccgatatctgccagaacttcctggcagaggtcacagcggaagcactccggatgccagctgttattcatggctttgataactcggccaatgatgaattcaccacactgatgacagcaaggggcaaagagcatctgaaagtcatgttcacagtactttcttccttcaaactcatagaagagtccttctgggaactgctggaagcactgagcgcacacgaaacactgctcatggtacagctccccattactgttcacgatcttctcagcgggcgcaaagccgcccttgcagcgctcgcaagtggcgctggccagggcgttggccatgttgcttgattgactaggcatggtgcttcttcctatcctctggccacaatgactggtcctggtccatttggactatggacttgaactaagttaatcagatactatttctcaaagactagaaatctgagtagagactaacaccctgcagttagaggaagtcaactcagagcactgctctatagagacatcccacaagttctgcagagacaccgggaaagccc

SEQ ID NO: 13424 - RNA, 3645 nt, Homo sapiens
  source 1..3645: mol_type = other RNA
gctgggattacaggcatgagccaccacgcccggcccacttacactttttaaacttcttcctcttctcctatacctaagggctccaatgatactacttatcagggaagaaagtactgtatctagataaactacccttaagtattacaggcttagcaagttgaatttctagaaaatactcattcataatttatttatttattttttttgagacagagtcttgctctgttgcccaggctggagtgcagtggcgtgatcttggctcactgcaagctctgcctcccgggttcccaccattctcctgcctcagcctcccgagtagctgggactgcaggtgcccgccaccacgcccggctaatttttttgtagtagagatggggtttcagtggtagccaggatggtcttgatctcctgacctcgtgatccacctgcctcgacctcccaaagtgctgggattacaggtgtgaggcaccgtgcctgtccactaattcatattttaaaagaggactgagcaaagacagcaatggaacctctggctgcaggagatgcctgggtatgcctgatatgtaaacaaacacaagcagtcgagttcaggccatgcatcttcaaagtgacgaagaatatatgtaaatgcttgtttttctcctccatatttctcgtgtagaggtatatgagaatttagcatcaagacgctatactgcaaaccctgttctgtgttgcctatattcatagcataatatttaataaatactcccaaggttgtcattgctggtcacatattagctgacaaaggcacactgaagggactttgattcttactgtaaaatgcaaagattgttttaaactactcaacatatacaatcttaaactatgtgatgattattctcgatcatttatgataatttcaattctaaaagattactaaaaaaaattggttgtagggtatctgaaaacaaaaatagaatgtactccataaagtacatgcacagaatttttaaaaatgcaggcatacaaatatttaatggcagagtggtaataacctgagactttttaaaaatggcaaaacaatatttcagcaatttttggaaaaaaaacccaaatattttccctaagaagtctctcttggcaactttctttttaagcaacaaagcagcagcaacatttttaaatgttcataaagctcgctttccattaacaagtttattaaggaagagtggtcctgaaacttcaggataaaacttttgataaaaatagaatcactaattttgacctaaaacagacactaaaacacccctccttccaatttaagagtgtcatttatacctcctacttacagtaaataaatcaaattaattataagatttcaaatggaaaatctgaaacacatatcaacatcattttcttctaataagataacagaaattaacttcaatggatttccccaaaaagagaatagtttctaaaaacttaattacagctgtggtaaatgaatctgggtttaccaatctcagatctcaatgcacttagttttagttggtattctgtgagatggctagaattcctgatttaagtatgtagtatgtatgtttttaaggcaaggcaagtttgagtatgtataaagcatagatattagcatggttataaaggcaatatgaccgacatacacattcagttttctgaagcaatatattccaagctacatacaatttaatttcatgtcctattctaagactacatgcttaacattaagcttagaaacataattgctgtaatacattaaaaatacttcattttccaatattgtaaagtatatttccaaatacctggtataaatttttttttgcacaaaaatttaaaggacatcctacagctagctattactactgcgttaagtaatcatttgaaggaagaattcacaaggagagcaggttataaaactaagcataataattattgcatttaactaaaaaaaatcaagtagttctgaattacacttgttttttgtcttagtaatgtgcatattcactttctagctactagtttgataaatatactaagattgtataagatttgtttttcttgtttttgtttttcttgggtggttatttttcttttctgtgtccttccccaacagcagttggaattttcttttgaacacaaagtaaattaatgtttatactgttttttcacctgagtcatgtaaaaggtgactcctttcattttaaaaagttatatttaatttttgggggccttaattaaaatttaacatttaaccatgtgttttttttttgtaaacagtctacatgtcaacaaatggataagggttaacaaaggcaaatactgacttcatttgtgttttaaacacgattatatgaatttttcttttttaattaaaaaaatgacataaaaccattcatataggtcctcttctctcaactgctttgagatatagctttaaatatgggtagatcaagacaagtaatgttggtaatctcttatcttgcatagaaaagaaaaaataaaggaacttatttccttcctaaggtctcagctagtttcttaagtcttttcttcagctccaatggaaatttctcatagcacttcttacagactggcttcatgtcaaactccacaaacttattcttgagtgttaatttagtgttgcaggtagaacaggcaaagcagttcacgcaccaggccttattaagagcagagaccacatcaccttctataacacgattgcagtggaagcaaacatcaccaaatagctggttatagtgagtttcacaatatgccaggcctttcctctcataatggcgatgtccaagaaagggtttctcacacttggcacaaacaaaatgctccacatgccactgcttgcccatagcgttcaccacgcgcccttcgatgggccgtcggcaagcaccacagatggggacccccattttatcatggcatgggaggcagtatagctcccctttcagctcccgtgcatcggcagtcagctccttcccgcagttggcgcagttgaaatggtctggatggtaggggtcgttcttgaatatcagaggctgctcatcgatgatagcatggcatttctggcagatgtatttcccaaggcctctggctttctcacgattatgacaggggcgacacaggtgtctcccagcattcttgacaaacccgatatctgccagaacttcctggcagaggtcacagcggaagcactccggatgccagctgttattcatggctttgataactcggccaatgatgaattcaccacactgatgacagcaaggggcaaagagcatctgaaagtcatgttcacagtactttcttccttcaaactcatagaagagtccttctgggaactgctggaagcactgagcgcacacgaaacactgctcatggtacagctccccattactgttcacgatcttctcagcgggcgcaaagccgcccttgcagcgctcgcaagtggcgctggccagggcgttggccatgttgctttcttggagagtttccagtcttgcctctgcatcctgttcttccttgctagctctcattttcttcacccattccgtctatcaaaacctgaaattttggggccggcgcagtggctcacgcctgtaatcccagcacttt

SEQ ID NO: 13425 - RNA, 3627 nt, Homo sapiens
  source 1..3627: mol_type = other RNA
gctgggattacaggcatgagccaccacgcccggcccacttacactttttaaacttcttcctcttctcctatacctaagggctccaatgatactacttatcagggaagaaagtactgtatctagataaactacccttaagtattacaggcttagcaagttgaatttctagaaaatactcattcataatttatttatttattttttttgagacagagtcttgctctgttgcccaggctggagtgcagtggcgtgatcttggctcactgcaagctctgcctcccgggttcccaccattctcctgcctcagcctcccgagtagctgggactgcaggtgcccgccaccacgcccggctaatttttttgtagtagagatggggtttcagtggtagccaggatggtcttgatctcctgacctcgtgatccacctgcctcgacctcccaaagtgctgggattacaggtgtgaggcaccgtgcctgtccactaattcatattttaaaagaggactgagcaaagacagcaatggaacctctggctgcaggagatgcctgggtatgcctgatatgtaaacaaacacaagcagtcgagttcaggccatgcatcttcaaagtgacgaagaatatatgtaaatgcttgtttttctcctccatatttctcgtgtagaggtatatgagaatttagcatcaagacgctatactgcaaaccctgttctgtgttgcctatattcatagcataatatttaataaatactcccaaggttgtcattgctggtcacatattagctgacaaaggcacactgaagggactttgattcttactgtaaaatgcaaagattgttttaaactactcaacatatacaatcttaaactatgtgatgattattctcgatcatttatgataatttcaattctaaaagattactaaaaaaaattggttgtagggtatctgaaaacaaaaatagaatgtactccataaagtacatgcacagaatttttaaaaatgcaggcatacaaatatttaatggcagagtggtaataacctgagactttttaaaaatggcaaaacaatatttcagcaatttttggaaaaaaaacccaaatattttccctaagaagtctctcttggcaactttctttttaagcaacaaagcagcagcaacatttttaaatgttcataaagctcgctttccattaacaagtttattaaggaagagtggtcctgaaacttcaggataaaacttttgataaaaatagaatcactaattttgacctaaaacagacactaaaacacccctccttccaatttaagagtgtcatttatacctcctacttacagtaaataaatcaaattaattataagatttcaaatggaaaatctgaaacacatatcaacatcattttcttctaataagataacagaaattaacttcaatggatttccccaaaaagagaatagtttctaaaaacttaattacagctgtggtaaatgaatctgggtttaccaatctcagatctcaatgcacttagttttagttggtattctgtgagatggctagaattcctgatttaagtatgtagtatgtatgtttttaaggcaaggcaagtttgagtatgtataaagcatagatattagcatggttataaaggcaatatgaccgacatacacattcagttttctgaagcaatatattccaagctacatacaatttaatttcatgtcctattctaagactacatgcttaacattaagcttagaaacataattgctgtaatacattaaaaatacttcattttccaatattgtaaagtatatttccaaatacctggtataaatttttttttgcacaaaaatttaaaggacatcctacagctagctattactactgcgttaagtaatcatttgaaggaagaattcacaaggagagcaggttataaaactaagcataataattattgcatttaactaaaaaaaatcaagtagttctgaattacacttgttttttgtcttagtaatgtgcatattcactttctagctactagtttgataaatatactaagattgtataagatttgtttttcttgtttttgtttttcttgggtggttatttttcttttctgtgtccttccccaacagcagttggaattttcttttgaacacaaagtaaattaatgtttatactgttttttcacctgagtcatgtaaaaggtgactcctttcattttaaaaagttatatttaatttttgggggccttaattaaaatttaacatttaaccatgtgttttttttttgtaaacagtctacatgtcaacaaatggataagggttaacaaaggcaaatactgacttcatttgtgttttaaacacgattatatgaatttttcttttttaattaaaaaaatgacataaaaccattcatataggtcctcttctctcaactgctttgagatatagctttaaatatgggtagatcaagacaagtaatgttggtaatctcttatcttgcatagaaaagaaaaaataaaggaacttatttccttcctaaggtctcagctagtttcttaagtcttttcttcagctccaatggaaatttctcatagcacttcttacagactggcttcatgtcaaactccacaaacttattcttgagtgttaatttagtgttgcaggtagaacaggcaaagcagttcacgcaccaggccttattaagagcagagaccacatcaccttctataacacgattgcagtggaagcaaacatcaccaaatagctggttatagtgagtttcacaatatgccaggcctttcctctcataatggcgatgtccaagaaagggtttctcacacttggcacaaacaaaatgctccacatgccactgcttgcccatagcgttcaccacgcgcccttcgatgggccgtcggcaagcaccacagatggggacccccattttatcatggcatgggaggcagtatagctcccctttcagctcccgtgcatcggcagtcagctccttcccgcagttggcgcagttgaaatggtctggatggtaggggtcgttcttgaatatcagaggctgctcatcgatgatagcatggcatttctggcagatgtatttcccaaggcctctggctttctcacgattatgacaggggcgacacaggtgtctcccagcattcttgacaaacccgatatctgccagaacttcctggcagaggtcacagcggaagcactccggatgccagctgttattcatggctttgataactcggccaatgatgaattcaccacactgatgacagcaaggggcaaagagcatctgaaagtcatgttcacagtactttcttccttcaaactcatagaagagtccttctgggaactgctggaagcactgagcgcacacgaaacactgctcatggtacagctccccattactgttcacgatcttctcagcgggcgcaaagccgcccttgcagcgctcgcaagtggcgctggccagggcgttggccatgttgttatcagggcttgggaggccagtttcacatcactgcgaattatctttgaaagcctctatttcctaaactgtacagaacttcctcatcttagctttgtctctgttgtcttgaactatattt

SEQ ID NO: 13426 - RNA, 7034 nt, Homo sapiens
  source 1..7034: mol_type = other RNA
gctgggattacaggcatgagccaccacgcccggcccgggtcccagatctctgagtccaccagagtggggctcagagtcctctatccaccaaccacatgcagccatccaacacgctgtctctcttctggcctcagcctcattgtccttggagtgccagtctcttgtttaagcatggcagagccttaatactggaccatccactacatgctagaaggggaagaactcctcacaatgtaacaatttttgtatttaacttatggatatgctcattctttctaaacaattcttataaggaaattttaagtatattaaaaaattagaatagtatgaccaccccaacactgcccagcttcattaataatccacacatctaaaacccatctagtccttgacacacacacaatcattatgaaacaacccaagacataaattgatttcatccataaatactgaaattatgattcaagagaactttttttttttttttcttaaaccaaggctgaggtgggagaactgcttgagcccaggagttcaagaccagcttaggtaacactgcaaaacccagtctctagagaaaaaaaaaacaaaaccaatcataaccatagccccactgtcatatgtttaaatgttgtttccttaatatcatcaaatatccagccagagttcaaatttgctttgtcccttaagcacatttttacaagattgattggctagttcagatcaagaggcaaacaaggttcatacattgcactggattcacacgtctcaagtatctttcaatctccaggcttcccttcccttcccttttcctcttgtaatgtatttgttgaagaatctaggtccctctgtagtcactcctctccccattcccagcccctggtaaccacttacctgttttctgaccctataattttgtagggcccactttgtactgatgtacttctgactaggtgtgtttatgttcaagcatcagagccaaggcccaaacctctaccctggccctccttctgctgtggcccaactgtacccagagctgggctctcccgtctccctgcctgttaatcctagaagtgggtgccgaggagggagaaacaggaaggagggagttggggagggcagcttgttacatggacatcagggctgttcccactagcagcaacagctttgtgttagcttggctccaatttgaatgaaatattccaaggccattttccccaacacgttgttaccaaaaaaactcccagcatgcagaaaagttgaaagaattgtacagtgaacaccccttaaggagtttctaccattaacattttatttaaaggctttgggactctgaagtataatgtttgtgaaatgctatgagccagaccctccacactgaaaattcccagtgtaaattaatttgttaaatgctcttagaattcctgcaataaagaacacctatctaaccttagttatccctgtgtttcccaaatatatcttactttggagcactttttttttagtaccgatttacatcctgggaaatggtgtttaccatgctttaaaaaaaactgtggtaaaataaagataagatttaccatcttaaccattttagagtgtacagttgagttggcatacagcattcacataacttaactgtgcaaccaatccacaggactttttatcttgcaaaactgaaacactatacccattaaacaactcctcatttcctcctcccccagtccttggcaactaccattctacttgtttctatgcatttgactgctctagatacttcacataaatggaagcatagagtatttgtcttccagtgactggcttacttcacttagcatcatgtcctcaagattcatccatgttgcagcacatgtcagcgtatcttccttttagaggctgaataatattccactgtatgaatataccacattttgttgatcattcacccactgatgggcacatattgcttccatctcttagctactgtgaataatggtgccgtgagtatgggcatacaaaaactaccactaatattttacagtgcttgcttcatatctgtccatgtgtccgtcactccacccatcatattttttatgtatttcataagttacagaccacagtaacttccctcaaacatgtcagtatacatatcaatgaccagcgttcattgtttttttccaagtcattttgaactgccgtagcaatgagtaatatagcctcaaacgcacacatacacacacaacacgtgcgtcactacagaaaacttttcctggcagacaggaaagggcccattgttggtgatgtcattttaattaagataaaaccaccaccaccatttagtaatagcctggggtaacaagggctgcgtcacggactgccacttttgccatcctgctcagagcagggccatgcctaacccgtatctggggattgcttcagatattatgaatcgcttcaatattatgaattactacaattcataataattgcttcagatattatgaattacaatatggttcaaaggtgctttagcagatgaagacacaaatgtgtaaacacatatgaattacaatgcagactgcccagatgtgtagcaagtcctctgaatgtttactaaacagtaaggtgattccagaggaagatgcttgaggacaatttgggaaaactgacaacttgaaaactcagtctctctaggcaaggcctacttgcagataaccttgggagttctgtgctgggaggaaagctaaaggactaagttaggcctctgaatctgctctggaagcctgcatgcacttgggtcagaacaagcccatgtgtcaatgtgggtaaagattcctcagctgataagcaggaaaatgggcagggcattttggtctttgaggttcaaagctcagatgctcactgccttggtatacacgcacacacaccccaccccccagctgacggcacaagagtatacagatgcaatagtctaaagtacattgtccaaatatggatggccatgagccacatgtggctatgaagcacttaaatgtggctagtctgaactgagatgggccctataaaatatttcagtaacaggtttttatactgattataggttgacataataatattttggatataccgtattaaaggaaatatgtcattaaatttcacctgtttcctttattatgtggctacttgaaaattttaaaattacatatgtagctcacactataaaacacagattagaaatattgtatagcactgacctagaaacctccatttaggtaaaacatcttaacccctttggaagcaaaatatgttaaataacagcataaactcccaccaagaaaatcctcaccttcctcctttcaacacatttattatatacagctgtcactgcattgtcaatctgccaaatggctctatgttccaacagggctggagtagtcccctgctcacaccagccttcacaatacttcccatgtcttccctgttaacctctctccacccagcacccaggctcccaactctcctggctgcctccagccctcagctggcaccactgacatgctgtttccagtacccttttcttctttctgcatcctccctgggggacatatatccctcatctcgtgacttcagctgtcacataaattcaaatgtttcagaactctattttttacctcctacatctgtcagtttaaatgtcaggatattttactttcagtaaagccctaaaaagacaaatctatgtacttttaaagaataaaagaaatgactggctgcagctcaaacctacaactgcttgcgaaactctacaatgtctggcagatgctagaaagaaggggatcaagacagagcacacttggcgtggtatgctatctatagaaaatgttaaaataaaattaagtaatctaggtttcctctctttattttctacatctactctctgaagagggcaataaataaggaaatgtcccaaagagggacaaattaagtcccaaaataacacaaaattgggcaaatccagtcatgaagaaagaacagaggttcttaaattgggacacacagaggcaggtctgcaggtctaggaatctctgaacatatgtgcaaaattctgggtatgtgtgcatatgttatataacaaagcgaagggtccatatagctttcatcgcatttcaaagggtctagcactgaaataaggactactgctatgtgacttaaaaaatgaaactcaggctgggcgcagtggctcacgcctgtaatcccagcactttgggaggccgaggcaagcagatcacctgagacgaggagtttgagacccgcctggccaacggtgaaacccagtctctactaaaaatacaaaaattagccggaattggtggtgtgcctctagtcccagctactcaggaggctgaagaaagagaatcgcttgaacctgggaggtggaggttgtgacaaagcaagactccatctcaaaaaaaaaaaaaacccagaaactcaattcagttatgaaggtaaagatgacctgtttacatgataatattttaagataccagtgactgcaagcatgtagttattaagtccattacagtgcacatttattgactctgtgtatcttcacagtgtgatcttcaccacagcttgcaaagtgtaaccactcagcaccttctgcttccttctgttcagtttttccactgcaattcttccagcataattttctgatagccagtgtatgactttggctttgacttgtttctacacagtgggtccagtcatttatttctggaacttgatcagtctttttccaggtatataagcaaatctttccacactccaatcctactgcaaccacgtatcgttgagaagggtggagcactgggcagacgctgacagctgtcacagccccacccacgtccaggactgaggagcaggggccaatgttgtgctcaatacagtcatcagtggagtcgcactcaccccagacaaccacctttttgtctcgactcccagtgaagaaatacttgctgtcaggactccaatcacaagaccaaataattcgaactcaggtgagattgtatcctgctttttccacaatgaccaggttcgatctctggaaacagctagtaagaacttctcattaggtgagaaggccatctgcgtgactgtcaaactgtggaaaactaaattctgcacctgtttccaagatgtagtgttccaaagaatgatagctgcatgctctttcttagctgccttacaagctgaggcaagcagagtctttgaactgttacaagtaacacaaaatatttcataaccgtgcccatatagtttttgaacttcaggccacaaagtattctgcagaagatgatcctcagtgggaggctcagtaagtatggagggctgaaaggccacctgctgatactcaaaaccagtactagttaacagctcctcttcatcagaaggctgagaagctatatctccctgaaagacagctttatttgataatcccaatgcagggacagtggctccttctggaagatcactatcttgattacagagcacatgattcagtgattgtcctgtaatggcacaaaaattttccacaaaattccgaggtgcagaaaaaacccgaagaactttttcatctgctccagatacaaactgaaaccgattaatcattgccaaacatttcaggtcatacccatgtatctgaggccttgcaatttcatgccaagtcacctgtgattggtcttttctcttccatggagcaaaaagtctagttgtctgatcagtaccaacagtgataataaattctccttctggatcccagactaggtcttggacaccatcaaagtgtcctgaaatgacaatctctggagtccactctcttgggttaactgtattctgtttccaaaggtgcaacgctccgtggaaagcatgagcaatgatcatggagccatcttcattgaactggcaatcataaaatcccaaagtattcccacctacttcacctactcgaacctgttctagccaaactcctgactcttcatctggagcccagagaatcatggttttatccatggaagcagataataatctcactggctgctgtaggacaccatctttgtaaaacacaggttgccagtgaactgcatttacccagttttcatgaccggctagcactgtctccagagtaacagcaaatgctattttaacactttcattttctatggtaaaagtattttctttcagtcttatgttatcgtcatcctgagtttctaaagatgttgactttatatacagcttccatattcttatcaggcaatcttgtgaacagcttgctaggaaaagatctctaccaaaggctgcccattccactcctctaatccaatcctcatgtccacagagagaaagcactttctgaaactgatcattttgttgagcaaatatgtgaattctgcaatcatcattgccacatgctaatattggtacatcagtatttggcaaaaaagataagcagagagccaaagcaaatccatttccaaagtttaaagtctgaaggcacattacttctggaccctttttagaccagagtcgaacagcagaatctgcagctgcagaaacgatcagtgtacataatgcaggatctgatgtcctcctctggtaaacagcatgcaccgcataaacaggtccttcatggccttgaagatgcactgcttttaaaagctgattatcctctatttcccagtgaatcacttgattatcagatcctccagaaactaattcagtagaaggggagccatcctgtttacaaatccactgtatgcaattgactcgggcggtgtgaccattcaagttggtaacaacaacccttttcagggggtcatagagcaccacggagcaggacgtgccaaaggccagaagtcctctgggcccagagctccagttcaggactccccgcacccggtttgggcagcaaaacacgtgagaagtctccagcacgggtgccaccatgtcgccaactggtcagccgcacaaacaagagacgc

SEQ ID NO: 13427 - RNA, 7037 nt, Homo sapiens
  source 1..7037: mol_type = other RNA
gctgggattacaggcatgagccaccacgcccggcccgggtcccagatctctgagtccaccagagtggggctcagagtcctctatccaccaaccacatgcagccatccaacacgctgtctctcttctggcctcagcctcattgtccttggagtgccagtctcttgtttaagcatggcagagccttaatactggaccatccactacatgctagaaggggaagaactcctcacaatgtaacaatttttgtatttaacttatggatatgctcattctttctaaacaattcttataaggaaattttaagtatattaaaaaattagaatagtatgaccaccccaacactgcccagcttcattaataatccacacatctaaaacccatctagtccttgacacacacacaatcattatgaaacaacccaagacataaattgatttcatccataaatactgaaattatgattcaagagaactttttttttttttttcttaaaccaaggctgaggtgggagaactgcttgagcccaggagttcaagaccagcttaggtaacactgcaaaacccagtctctagagaaaaaaaaaacaaaaccaatcataaccatagccccactgtcatatgtttaaatgttgtttccttaatatcatcaaatatccagccagagttcaaatttgctttgtcccttaagcacatttttacaagattgattggctagttcagatcaagaggcaaacaaggttcatacattgcactggattcacacgtctcaagtatctttcaatctccaggcttcccttcccttcccttttcctcttgtaatgtatttgttgaagaatctaggtccctctgtagtcactcctctccccattcccagcccctggtaaccacttacctgttttctgaccctataattttgtagggcccactttgtactgatgtacttctgactaggtgtgtttatgttcaagcatcagagccaaggcccaaacctctaccctggccctccttctgctgtggcccaactgtacccagagctgggctctcccgtctccctgcctgttaatcctagaagtgggtgccgaggagggagaaacaggaaggagggagttggggagggcagcttgttacatggacatcagggctgttcccactagcagcaacagctttgtgttagcttggctccaatttgaatgaaatattccaaggccattttccccaacacgttgttaccaaaaaaactcccagcatgcagaaaagttgaaagaattgtacagtgaacaccccttaaggagtttctaccattaacattttatttaaaggctttgggactctgaagtataatgtttgtgaaatgctatgagccagaccctccacactgaaaattcccagtgtaaattaatttgttaaatgctcttagaattcctgcaataaagaacacctatctaaccttagttatccctgtgtttcccaaatatatcttactttggagcactttttttttagtaccgatttacatcctgggaaatggtgtttaccatgctttaaaaaaaactgtggtaaaataaagataagatttaccatcttaaccattttagagtgtacagttgagttggcatacagcattcacataacttaactgtgcaaccaatccacaggactttttatcttgcaaaactgaaacactatacccattaaacaactcctcatttcctcctcccccagtccttggcaactaccattctacttgtttctatgcatttgactgctctagatacttcacataaatggaagcatagagtatttgtcttccagtgactggcttacttcacttagcatcatgtcctcaagattcatccatgttgcagcacatgtcagcgtatcttccttttagaggctgaataatattccactgtatgaatataccacattttgttgatcattcacccactgatgggcacatattgcttccatctcttagctactgtgaataatggtgccgtgagtatgggcatacaaaaactaccactaatattttacagtgcttgcttcatatctgtccatgtgtccgtcactccacccatcatattttttatgtatttcataagttacagaccacagtaacttccctcaaacatgtcagtatacatatcaatgaccagcgttcattgtttttttccaagtcattttgaactgccgtagcaatgagtaatatagcctcaaacgcacacatacacacacaacacgtgcgtcactacagaaaacttttcctggcagacaggaaagggcccattgttggtgatgtcattttaattaagataaaaccaccaccaccatttagtaatagcctggggtaacaagggctgcgtcacggactgccacttttgccatcctgctcagagcagggccatgcctaacccgtatctggggattgcttcagatattatgaatcgcttcaatattatgaattactacaattcataataattgcttcagatattatgaattacaatatggttcaaaggtgctttagcagatgaagacacaaatgtgtaaacacatatgaattacaatgcagactgcccagatgtgtagcaagtcctctgaatgtttactaaacagtaaggtgattccagaggaagatgcttgaggacaatttgggaaaactgacaacttgaaaactcagtctctctaggcaaggcctacttgcagataaccttgggagttctgtgctgggaggaaagctaaaggactaagttaggcctctgaatctgctctggaagcctgcatgcacttgggtcagaacaagcccatgtgtcaatgtgggtaaagattcctcagctgataagcaggaaaatgggcagggcattttggtctttgaggttcaaagctcagatgctcactgccttggtatacacgcacacacaccccaccccccagctgacggcacaagagtatacagatgcaatagtctaaagtacattgtccaaatatggatggccatgagccacatgtggctatgaagcacttaaatgtggctagtctgaactgagatgggccctataaaatatttcagtaacaggtttttatactgattataggttgacataataatattttggatataccgtattaaaggaaatatgtcattaaatttcacctgtttcctttattatgtggctacttgaaaattttaaaattacatatgtagctcacactataaaacacagattagaaatattgtatagcactgacctagaaacctccatttaggtaaaacatcttaacccctttggaagcaaaatatgttaaataacagcataaactcccaccaagaaaatcctcaccttcctcctttcaacacatttattatatacagctgtcactgcattgtcaatctgccaaatggctctatgttccaacagggctggagtagtcccctgctcacaccagccttcacaatacttcccatgtcttccctgttaacctctctccacccagcacccaggctcccaactctcctggctgcctccagccctcagctggcaccactgacatgctgtttccagtacccttttcttctttctgcatcctccctgggggacatatatccctcatctcgtgacttcagctgtcacataaattcaaatgtttcagaactctattttttacctcctacatctgtcagtttaaatgtcaggatattttactttcagtaaagccctaaaaagacaaatctatgtacttttaaagaataaaagaaatgactggctgcagctcaaacctacaactgcttgcgaaactctacaatgtctggcagatgctagaaagaaggggatcaagacagagcacacttggcgtggtatgctatctatagaaaatgttaaaataaaattaagtaatctaggtttcctctctttattttctacatctactctctgaagagggcaataaataaggaaatgtcccaaagagggacaaattaagtcccaaaataacacaaaattgggcaaatccagtcatgaagaaagaacagaggttcttaaattgggacacacagaggcaggtctgcaggtctaggaatctctgaacatatgtgcaaaattctgggtatgtgtgcatatgttatataacaaagcgaagggtccatatagctttcatcgcatttcaaagggtctagcactgaaataaggactactgctatgtgacttaaaaaatgaaactcaggctgggcgcagtggctcacgcctgtaatcccagcactttgggaggccgaggcaagcagatcacctgagacgaggagtttgagacccgcctggccaacggtgaaacccagtctctactaaaaatacaaaaattagccggaattggtggtgtgcctctagtcccagctactcaggaggctgaagaaagagaatcgcttgaacctgggaggtggaggttgtgacaaagcaagactccatctcaaaaaaaaaaaaaacccagaaactcaattcagttatgaaggtaaagatgacctgtttacatgataatattttaagataccagtgactgcaagcatgtagttattaagtccattacagtgcacatttattgactctgtgtatcttcacagtgtgatcttcaccacagcttgcaaagtgtaaccactcagcaccttctgcttccttctgttcagtttttccactgcaattcttccagcataattttctgatagccagtgtatgactttggctttgacttgtttctacacagtgggtccagtcatttatttctggaacttgatcagtctttttccaggtatataagcaaatctttccacactccaatcctactgcaaccacgtatcgttgagaagggtggagcactgggcagacgctgacagctgtcacagccccacccacgtccaggactgaggagcaggggccaatgttgtgctcaatacagtcatcagtggagtcgcactcaccccagacaaccacctttttgtctcgactcccagtgaagaaatacttgctgtcaggactccaatcacaagaccaaataattctacgaactcaggtgagattgtatcctgctttttccacaatgaccaggttcgatctctggaaacagctagtaagaacttctcattaggtgagaaggccatctgcgtgactgtcaaactgtggaaaactaaattctgcacctgtttccaagatgtagtgttccaaagaatgatagctgcatgctctttcttagctgccttacaagctgaggcaagcagagtctttgaactgttacaagtaacacaaaatatttcataaccgtgcccatatagtttttgaacttcaggccacaaagtattctgcagaagatgatcctcagtgggaggctcagtaagtatggagggctgaaaggccacctgctgatactcaaaaccagtactagttaacagctcctcttcatcagaaggctgagaagctatatctccctgaaagacagctttatttgataatcccaatgcagggacagtggctccttctggaagatcactatcttgattacagagcacatgattcagtgattgtcctgtaatggcacaaaaattttccacaaaattccgaggtgcagaaaaaacccgaagaactttttcatctgctccagatacaaactgaaaccgattaatcattgccaaacatttcaggtcatacccatgtatctgaggccttgcaatttcatgccaagtcacctgtgattggtcttttctcttccatggagcaaaaagtctagttgtctgatcagtaccaacagtgataataaattctccttctggatcccagactaggtcttggacaccatcaaagtgtcctgaaatgacaatctctggagtccactctcttgggttaactgtattctgtttccaaaggtgcaacgctccgtggaaagcatgagcaatgatcatggagccatcttcattgaactggcaatcataaaatcccaaagtattcccacctacttcacctactcgaacctgttctagccaaactcctgactcttcatctggagcccagagaatcatggttttatccatggaagcagataataatctcactggctgctgtaggacaccatctttgtaaaacacaggttgccagtgaactgcatttacccagttttcatgaccggctagcactgtctccagagtaacagcaaatgctattttaacactttcattttctatggtaaaagtattttctttcagtcttatgttatcgtcatcctgagtttctaaagatgttgactttatatacagcttccatattcttatcaggcaatcttgtgaacagcttgctaggaaaagatctctaccaaaggctgcccattccactcctctaatccaatcctcatgtccacagagagaaagcactttctgaaactgatcattttgttgagcaaatatgtgaattctgcaatcatcattgccacatgctaatattggtacatcagtatttggcaaaaaagataagcagagagccaaagcaaatccatttccaaagtttaaagtctgaaggcacattacttctggaccctttttagaccagagtcgaacagcagaatctgcagctgcagaaacgatcagtgtacataatgcaggatctgatgtcctcctctggtaaacagcatgcaccgcataaacaggtccttcatggccttgaagatgcactgcttttaaaagctgattatcctctatttcccagtgaatcacttgattatcagatcctccagaaactaattcagtagaaggggagccatcctgtttacaaatccactgtatgcaattgactcgggcggtgtgaccattcaagttggtaacaacaacccttttcagggggtcatagagcaccacggagcaggacgtgccaaaggccagaagtcctctgggcccagagctccagttcaggactccccgcacccggtttgggcagcaaaacacgtgagaagtctccagcacgggtgccaccatgtcgccaactggtcagccgcacaaacaagagacgc

SEQ ID NO: 13428 - RNA, 6970 nt, Homo sapiens
  source 1..6970: mol_type = other RNA
gctgggattacaggcatgagccaccacgcccggcccgggtcccagatctctgagtccaccagagtggggctcagagtcctctatccaccaaccacatgcagccatccaacacgctgtctctcttctggcctcagcctcattgtccttggagtgccagtctcttgtttaagcatggcagagccttaatactggaccatccactacatgctagaaggggaagaactcctcacaatgtaacaatttttgtatttaacttatggatatgctcattctttctaaacaattcttataaggaaattttaagtatattaaaaaattagaatagtatgaccaccccaacactgcccagcttcattaataatccacacatctaaaacccatctagtccttgacacacacacaatcattatgaaacaacccaagacataaattgatttcatccataaatactgaaattatgattcaagagaactttttttttttttttcttaaaccaaggctgaggtgggagaactgcttgagcccaggagttcaagaccagcttaggtaacactgcaaaacccagtctctagagaaaaaaaaaacaaaaccaatcataaccatagccccactgtcatatgtttaaatgttgtttccttaatatcatcaaatatccagccagagttcaaatttgctttgtcccttaagcacatttttacaagattgattggctagttcagatcaagaggcaaacaaggttcatacattgcactggattcacacgtctcaagtatctttcaatctccaggcttcccttcccttcccttttcctcttgtaatgtatttgttgaagaatctaggtccctctgtagtcactcctctccccattcccagcccctggtaaccacttacctgttttctgaccctataattttgtagggcccactttgtactgatgtacttctgactaggtgtgtttatgttcaagcatcagagccaaggcccaaacctctaccctggccctccttctgctgtggcccaactgtacccagagctgggctctcccgtctccctgcctgttaatcctagaagtgggtgccgaggagggagaaacaggaaggagggagttggggagggcagcttgttacatggacatcagggctgttcccactagcagcaacagctttgtgttagcttggctccaatttgaatgaaatattccaaggccattttccccaacacgttgttaccaaaaaaactcccagcatgcagaaaagttgaaagaattgtacagtgaacaccccttaaggagtttctaccattaacattttatttaaaggctttgggactctgaagtataatgtttgtgaaatgctatgagccagaccctccacactgaaaattcccagtgtaaattaatttgttaaatgctcttagaattcctgcaataaagaacacctatctaaccttagttatccctgtgtttcccaaatatatcttactttggagcactttttttttagtaccgatttacatcctgggaaatggtgtttaccatgctttaaaaaaaactgtggtaaaataaagataagatttaccatcttaaccattttagagtgtacagttgagttggcatacagcattcacataacttaactgtgcaaccaatccacaggactttttatcttgcaaaactgaaacactatacccattaaacaactcctcatttcctcctcccccagtccttggcaactaccattctacttgtttctatgcatttgactgctctagatacttcacataaatggaagcatagagtatttgtcttccagtgactggcttacttcacttagcatcatgtcctcaagattcatccatgttgcagcacatgtcagcgtatcttccttttagaggctgaataatattccactgtatgaatataccacattttgttgatcattcacccactgatgggcacatattgcttccatctcttagctactgtgaataatggtgccgtgagtatgggcatacaaaaactaccactaatattttacagtgcttgcttcatatctgtccatgtgtccgtcactccacccatcatattttttatgtatttcataagttacagaccacagtaacttccctcaaacatgtcagtatacatatcaatgaccagcgttcattgtttttttccaagtcattttgaactgccgtagcaatgagtaatatagcctcaaacgcacacatacacacacaacacgtgcgtcactacagaaaacttttcctggcagacaggaaagggcccattgttggtgatgtcattttaattaagataaaaccaccaccaccatttagtaatagcctggggtaacaagggctgcgtcacggactgccacttttgccatcctgctcagagcagggccatgcctaacccgtatctggggattgcttcagatattatgaatcgcttcaatattatgaattactacaattcataataattgcttcagatattatgaattacaatatggttcaaaggtgctttagcagatgaagacacaaatgtgtaaacacatatgaattacaatgcagactgcccagatgtgtagcaagtcctctgaatgtttactaaacagtaaggtgattccagaggaagatgcttgaggacaatttgggaaaactgacaacttgaaaactcagtctctctaggcaaggcctacttgcagataaccttgggagttctgtgctgggaggaaagctaaaggactaagttaggcctctgaatctgctctggaagcctgcatgcacttgggtcagaacaagcccatgtgtcaatgtgggtaaagattcctcagctgataagcaggaaaatgggcagggcattttggtctttgaggttcaaagctcagatgctcactgccttggtatacacgcacacacaccccaccccccagctgacggcacaagagtatacagatgcaatagtctaaagtacattgtccaaatatggatggccatgagccacatgtggctatgaagcacttaaatgtggctagtctgaactgagatgggccctataaaatatttcagtaacaggtttttatactgattataggttgacataataatattttggatataccgtattaaaggaaatatgtcattaaatttcacctgtttcctttattatgtggctacttgaaaattttaaaattacatatgtagctcacactataaaacacagattagaaatattgtatagcactgacctagaaacctccatttaggtaaaacatcttaacccctttggaagcaaaatatgttaaataacagcataaactcccaccaagaaaatcctcaccttcctcctttcaacacatttattatatacagctgtcactgcattgtcaatctgccaaatggctctatgttccaacagggctggagtagtcccctgctcacaccagccttcacaatacttcccatgtcttccctgttaacctctctccacccagcacccaggctcccaactctcctggctgcctccagccctcagctggcaccactgacatgctgtttccagtacccttttcttctttctgcatcctccctgggggacatatatccctcatctcgtgacttcagctgtcacataaattcaaatgtttcagaactctattttttacctcctacatctgtcagtttaaatgtcaggatattttactttcagtaaagccctaaaaagacaaatctatgtacttttaaagaataaaagaaatgactggctgcagctcaaacctacaactgcttgcgaaactctacaatgtctggcagatgctagaaagaaggggatcaagacagagcacacttggcgtggtatgctatctatagaaaatgttaaaataaaattaagtaatctaggtttcctctctttattttctacatctactctctgaagagggcaataaataaggaaatgtcccaaagagggacaaattaagtcccaaaataacacaaaattgggcaaatccagtcatgaagaaagaacagaggttcttaaattgggacacacagaggcaggtctgcaggtctaggaatctctgaacatatgtgcaaaattctgggtatgtgtgcatatgttatataacaaagcgaagggtccatatagctttcatcgcatttcaaagggtctagcactgaaataaggactactgctatgtgacttaaaaaatgaaactcaggctgggcgcagtggctcacgcctgtaatcccagcactttgggaggccgaggcaagcagatcacctgagacgaggagtttgagacccgcctggccaacggtgaaacccagtctctactaaaaatacaaaaattagccggaattggtggtgtgcctctagtcccagctactcaggaggctgaagaaagagaatcgcttgaacctgggaggtggaggttgtgacaaagcaagactccatctcaaaaaaaaaaaaaacccagaaactcaattcagttatgaaggtaaagatgacctgtttacatgataatattttaagataccagtgactgcaagcatgtagttattaagtccattacagtgcacatttattgactctgtgtatcttcacagtgtgatcttcaccacagcttgcaaagtgtaaccactcagcaccttctgcttccttctgttcagtttttccactgcaattcttccagcataattttctgatagccagtgtatgactttggctttgacttgtttctacacagtgggtccagtcatttatttctggaacttgatcagtctttttccaggtatataagcaaatctttccacactccaatcctactgcaaccacgtatcgttgagaagggtggagcactgggcagacgctgacagctgtcacagccccacccacgtccaggactgaggagcaggggccaatgttgtgctcaatacagtcatcagtggagtcgcactcaccccagacaaccacctttttgtctcgactcccagtgaagaaatacttgctgtcaggactccaatcacaagaccaaataattctacgaactcaggtgagattgtatcctgctttttccacaatgaccaggttcgatctctggaaacagctagtaagaacttctcattaggtgagaaggccatctgcgtgactgtcaaactgtggaaaactaaattctgcacctgtttccaagatgtagtgttccaaagaatgatagctgcatgctctttcttagctgccttacaagctgaggcaagcagagtctttgaactgttacaagtaacacaaaatatttcataaccgtgcccatatagtttttgaacttcaggccacaaagtattctgcagaagatgatcctcagtgggaggctcagtaagtatggagggctgaaaggccacctgctgatactcaaaaccagtactagttaacagctcctcttcatcagaaggctgagaagctatatctccctgaaagacagctttatttgataatcccaatgcagggacagtggctccttctggaagatcactatcttgattacagagcacatgattcagtgattgtcctgtaatggcacaaaaattttccacaaaattccgaggtgcagaaaaaacccgaagaactttttcatctgctccagatacaaactgaaaccgattaatcattgccaaacatttcaggtcatacccatgtatctgaggccttgcaatttcatgccaagtcacctgtgattggtcttttctcttccatggagcaaaaagtctagttgtctgatcagtaccaacagtgataataaattctccttctggatcccagactaggtcttggacaccatcaaagtgtcctgaaatgacaatctctggagtccactctcttgggttaactgtattctgtttccaaaggtgcaacgctccgtggaaagcatgagcaatgatcatggagccatcttcattgaactggcaatcataaaatcccaaagtattcccacctacttcacctactcgaacctgttctagccaaactcctgactcttcatctggagcccagagaatcatggttttatccatggaagcagataataatctcactggctgctgtaggacaccatctttgtaaaacacaggttgccagtgaactgcatttacccagttttcatgaccggctagcactgtctccagagtaacagcaaatgctattttaacactttcattttctatggtaaaagtattttctttcagtcttatgttatcgtcatcctgagtttctaaagatgttgactttatatacagcttccatattcttatcaggcaatcttgtgaacagcttgctaggaaaagatctctacctgatcattttgttgagcaaatatgtgaattctgcaatcatcattgccacatgctaatattggtacatcagtatttggcaaaaaagataagcagagagccaaagcaaatccatttccaaagtttaaagtctgaaggcacattacttctggaccctttttagaccagagtcgaacagcagaatctgcagctgcagaaacgatcagtgtacataatgcaggatctgatgtcctcctctggtaaacagcatgcaccgcataaacaggtccttcatggccttgaagatgcactgcttttaaaagctgattatcctctatttcccagtgaatcacttgattatcagatcctccagaaactaattcagtagaaggggagccatcctgtttacaaatccactgtatgcaattgactcgggcggtgtgaccattcaagttggtaacaacaacccttttcagggggtcatagagcaccacggagcaggacgtgccaaaggccagaagtcctctgggcccagagctccagttcaggactccccgcacccggtttgggcagcaaaacacgtgagaagtctccagcacgggtgccaccatgtcgccaactggtcagccgcacaaacaagagacgc

SEQ ID NO: 13429 - RNA, 6957 nt, Homo sapiens
  source 1..6957: mol_type = other RNA
gctgggattacaggcatgagccaccacgcccggcccgggtcccagatctctgagtccaccagagtggggctcagagtcctctatccaccaaccacatgcagccatccaacacgctgtctctcttctggcctcagcctcattgtccttggagtgccagtctcttgtttaagcatggcagagccttaatactggaccatccactacatgctagaaggggaagaactcctcacaatgtaacaatttttgtatttaacttatggatatgctcattctttctaaacaattcttataaggaaattttaagtatattaaaaaattagaatagtatgaccaccccaacactgcccagcttcattaataatccacacatctaaaacccatctagtccttgacacacacacaatcattatgaaacaacccaagacataaattgatttcatccataaatactgaaattatgattcaagagaactttttttttttttttcttaaaccaaggctgaggtgggagaactgcttgagcccaggagttcaagaccagcttaggtaacactgcaaaacccagtctctagagaaaaaaaaaacaaaaccaatcataaccatagccccactgtcatatgtttaaatgttgtttccttaatatcatcaaatatccagccagagttcaaatttgctttgtcccttaagcacatttttacaagattgattggctagttcagatcaagaggcaaacaaggttcatacattgcactggattcacacgtctcaagtatctttcaatctccaggcttcccttcccttcccttttcctcttgtaatgtatttgttgaagaatctaggtccctctgtagtcactcctctccccattcccagcccctggtaaccacttacctgttttctgaccctataattttgtagggcccactttgtactgatgtacttctgactaggtgtgtttatgttcaagcatcagagccaaggcccaaacctctaccctggccctccttctgctgtggcccaactgtacccagagctgggctctcccgtctccctgcctgttaatcctagaagtgggtgccgaggagggagaaacaggaaggagggagttggggagggcagcttgttacatggacatcagggctgttcccactagcagcaacagctttgtgttagcttggctccaatttgaatgaaatattccaaggccattttccccaacacgttgttaccaaaaaaactcccagcatgcagaaaagttgaaagaattgtacagtgaacaccccttaaggagtttctaccattaacattttatttaaaggctttgggactctgaagtataatgtttgtgaaatgctatgagccagaccctccacactgaaaattcccagtgtaaattaatttgttaaatgctcttagaattcctgcaataaagaacacctatctaaccttagttatccctgtgtttcccaaatatatcttactttggagcactttttttttagtaccgatttacatcctgggaaatggtgtttaccatgctttaaaaaaaactgtggtaaaataaagataagatttaccatcttaaccattttagagtgtacagttgagttggcatacagcattcacataacttaactgtgcaaccaatccacaggactttttatcttgcaaaactgaaacactatacccattaaacaactcctcatttcctcctcccccagtccttggcaactaccattctacttgtttctatgcatttgactgctctagatacttcacataaatggaagcatagagtatttgtcttccagtgactggcttacttcacttagcatcatgtcctcaagattcatccatgttgcagcacatgtcagcgtatcttccttttagaggctgaataatattccactgtatgaatataccacattttgttgatcattcacccactgatgggcacatattgcttccatctcttagctactgtgaataatggtgccgtgagtatgggcatacaaaaactaccactaatattttacagtgcttgcttcatatctgtccatgtgtccgtcactccacccatcatattttttatgtatttcataagttacagaccacagtaacttccctcaaacatgtcagtatacatatcaatgaccagcgttcattgtttttttccaagtcattttgaactgccgtagcaatgagtaatatagcctcaaacgcacacatacacacacaacacgtgcgtcactacagaaaacttttcctggcagacaggaaagggcccattgttggtgatgtcattttaattaagataaaaccaccaccaccatttagtaatagcctggggtaacaagggctgcgtcacggactgccacttttgccatcctgctcagagcagggccatgcctaacccgtatctggggattgcttcagatattatgaatcgcttcaatattatgaattactacaattcataataattgcttcagatattatgaattacaatatggttcaaaggtgctttagcagatgaagacacaaatgtgtaaacacatatgaattacaatgcagactgcccagatgtgtagcaagtcctctgaatgtttactaaacagtaaggtgattccagaggaagatgcttgaggacaatttgggaaaactgacaacttgaaaactcagtctctctaggcaaggcctacttgcagataaccttgggagttctgtgctgggaggaaagctaaaggactaagttaggcctctgaatctgctctggaagcctgcatgcacttgggtcagaacaagcccatgtgtcaatgtgggtaaagattcctcagctgataagcaggaaaatgggcagggcattttggtctttgaggttcaaagctcagatgctcactgccttggtatacacgcacacacaccccaccccccagctgacggcacaagagtatacagatgcaatagtctaaagtacattgtccaaatatggatggccatgagccacatgtggctatgaagcacttaaatgtggctagtctgaactgagatgggccctataaaatatttcagtaacaggtttttatactgattataggttgacataataatattttggatataccgtattaaaggaaatatgtcattaaatttcacctgtttcctttattatgtggctacttgaaaattttaaaattacatatgtagctcacactataaaacacagattagaaatattgtatagcactgacctagaaacctccatttaggtaaaacatcttaacccctttggaagcaaaatatgttaaataacagcataaactcccaccaagaaaatcctcaccttcctcctttcaacacatttattatatacagctgtcactgcattgtcaatctgccaaatggctctatgttccaacagggctggagtagtcccctgctcacaccagccttcacaatacttcccatgtcttccctgttaacctctctccacccagcacccaggctcccaactctcctggctgcctccagccctcagctggcaccactgacatgctgtttccagtacccttttcttctttctgcatcctccctgggggacatatatccctcatctcgtgacttcagctgtcacataaattcaaatgtttcagaactctattttttacctcctacatctgtcagtttaaatgtcaggatattttactttcagtaaagccctaaaaagacaaatctatgtacttttaaagaataaaagaaatgactggctgcagctcaaacctacaactgcttgcgaaactctacaatgtctggcagatgctagaaagaaggggatcaagacagagcacacttggcgtggtatgctatctatagaaaatgttaaaataaaattaagtaatctaggtttcctctctttattttctacatctactctctgaagagggcaataaataaggaaatgtcccaaagagggacaaattaagtcccaaaataacacaaaattgggcaaatccagtcatgaagaaagaacagaggttcttaaattgggacacacagaggcaggtctgcaggtctaggaatctctgaacatatgtgcaaaattctgggtatgtgtgcatatgttatataacaaagcgaagggtccatatagctttcatcgcatttcaaagggtctagcactgaaataaggactactgctatgtgacttaaaaaatgaaactcaggctgggcgcagtggctcacgcctgtaatcccagcactttgggaggccgaggcaagcagatcacctgagacgaggagtttgagacccgcctggccaacggtgaaacccagtctctactaaaaatacaaaaattagccggaattggtggtgtgcctctagtcccagctactcaggaggctgaagaaagagaatcgcttgaacctgggaggtggaggttgtgacaaagcaagactccatctcaaaaaaaaaaaaaacccagaaactcaattcagttatgaaggtaaagatgacctgtttacatgataatattttaagataccagtgactgcaagcatgtagttattaagtccattacagtgcacatttattgactctgtgtatcttcacagtgtgatcttcaccacagcttgcaaagtgtaaccactcagcaccttctgcttccttctgttcagtttttccactgcaattcttccagcataattttctgatagccagtgtatgactttggctttgacttgtttctacacagtgggtccagtcatttatttctggaacttgatcagtctttttccaggtatataagcaaatctttccacactccaatcctactgcaaccacgtatcgttgagaagggtggagcactgggcagacgctgacagctgtcacagccccacccacgtccaggactgaggagcaggggccaatgttgtgctcaatacagtcatcagtggagtcgcactcaccccagacaaccacctttttgtctcgactcccagtgaagaaatacttgctgtcaggactccaatcacaagaccaaataattctactgtgcacagaagtaattttgttggtgaaggcaaaaagactaaaaactggctcgaactcaggtgagattgtatcctgctttttccacaatgaccaggttcgatctctggaaacagctagtaagaacttctcattaggtgagaaggccatctgcgtgactgtcaaactgtggaaaactaaattctgcacctgtttccaagatgtagtgttccaaagaatgatagctgcatgctctttcttagctgccttacaagctgaggcaagcagagtctttgaactgttacaagtaacacaaaatatttcataaccgtgcccatatagtttttgaacttcaggccacaaagtattctgcagaagatgatcctcagtgggaggctcagtaagtatggagggctgaaaggccacctgctgatactcaaaaccagtactagttaacagctcctcttcatcagaaggctgagaagctatatctccctgaaagacagctttatttgataatcccaatgcagggacagtggctccttctggaagatcactatcttgattacagagcacatgattcagtgattgtcctgtaatggcacaaaaattttccacaaaattccgaggtgcagaaaaaacccgaagaactttttcatctgctccagatacaaactgaaaccgattaatcattgccaaacatttcaggtcatacccatgtatctgaggccttgcaatttcatgccaagtcacctgtgattggtcttttctcttccatggagcaaaaagtctagttgtctgatcagtaccaacagtgataataaattctccttctggatcccagactaggtcttggacaccatcaaagtgtcctgaaatgacaatctctggagtccactctctctgttctagccaaactcctgactcttcatctggagcccagagaatcatggttttatccatggaagcagataataatctcactggctgctgtaggacaccatctttgtaaaacacaggttgccagtgaactgcatttacccagttttcatgaccggctagcactgtctccagagtaacagcaaatgctattttaacactttcattttctatggtaaaagtattttctttcagtcttatgttatcgtcatcctgagtttctaaagatgttgactttatatacagcttccatattcttatcaggcaatcttgtgaacagcttgctaggaaaagatctctaccaaaggctgcccattccactcctctaatccaatcctcatgtccacagagagaaagcactttctgaaactgatcattttgttgagcaaatatgtgaattctgcaatcatcattgccacatgctaatattggtacatcagtatttggcaaaaaagataagcagagagccaaagcaaatccatttccaaagtttaaagtctgaaggcacattacttctggaccctttttagaccagagtcgaacagcagaatctgcagctgcagaaacgatcagtgtacataatgcaggatctgatgtcctcctctggtaaacagcatgcaccgcataaacaggtccttcatggccttgaagatgcactgcttttaaaagctgattatcctctatttcccagtgaatcacttgattatcagatcctccagaaactaattcagtagaaggggagccatcctgtttacaaatccactgtatgcaattgactcgggcggtgtgaccattcaagttggtaacaacaacccttttcagggggtcatagagcaccacggagcaggacgtgccaaaggccagaagtcctctgggcccagagctccagttcaggactccccgcacccggtttgggcagcaaaacacgtgagaagtctccagcacgggtgccaccatgtcgccaactggtcagccgcacaaacaagagacgc

SEQ ID NO: 13430 - RNA, 6879 nt, Homo sapiens
  source 1..6879: mol_type = other RNA
gctgggattacaggcatgagccaccacgcccggcccgggtcccagatctctgagtccaccagagtggggctcagagtcctctatccaccaaccacatgcagccatccaacacgctgtctctcttctggcctcagcctcattgtccttggagtgccagtctcttgtttaagcatggcagagccttaatactggaccatccactacatgctagaaggggaagaactcctcacaatgtaacaatttttgtatttaacttatggatatgctcattctttctaaacaattcttataaggaaattttaagtatattaaaaaattagaatagtatgaccaccccaacactgcccagcttcattaataatccacacatctaaaacccatctagtccttgacacacacacaatcattatgaaacaacccaagacataaattgatttcatccataaatactgaaattatgattcaagagaactttttttttttttttcttaaaccaaggctgaggtgggagaactgcttgagcccaggagttcaagaccagcttaggtaacactgcaaaacccagtctctagagaaaaaaaaaacaaaaccaatcataaccatagccccactgtcatatgtttaaatgttgtttccttaatatcatcaaatatccagccagagttcaaatttgctttgtcccttaagcacatttttacaagattgattggctagttcagatcaagaggcaaacaaggttcatacattgcactggattcacacgtctcaagtatctttcaatctccaggcttcccttcccttcccttttcctcttgtaatgtatttgttgaagaatctaggtccctctgtagtcactcctctccccattcccagcccctggtaaccacttacctgttttctgaccctataattttgtagggcccactttgtactgatgtacttctgactaggtgtgtttatgttcaagcatcagagccaaggcccaaacctctaccctggccctccttctgctgtggcccaactgtacccagagctgggctctcccgtctccctgcctgttaatcctagaagtgggtgccgaggagggagaaacaggaaggagggagttggggagggcagcttgttacatggacatcagggctgttcccactagcagcaacagctttgtgttagcttggctccaatttgaatgaaatattccaaggccattttccccaacacgttgttaccaaaaaaactcccagcatgcagaaaagttgaaagaattgtacagtgaacaccccttaaggagtttctaccattaacattttatttaaaggctttgggactctgaagtataatgtttgtgaaatgctatgagccagaccctccacactgaaaattcccagtgtaaattaatttgttaaatgctcttagaattcctgcaataaagaacacctatctaaccttagttatccctgtgtttcccaaatatatcttactttggagcactttttttttagtaccgatttacatcctgggaaatggtgtttaccatgctttaaaaaaaactgtggtaaaataaagataagatttaccatcttaaccattttagagtgtacagttgagttggcatacagcattcacataacttaactgtgcaaccaatccacaggactttttatcttgcaaaactgaaacactatacccattaaacaactcctcatttcctcctcccccagtccttggcaactaccattctacttgtttctatgcatttgactgctctagatacttcacataaatggaagcatagagtatttgtcttccagtgactggcttacttcacttagcatcatgtcctcaagattcatccatgttgcagcacatgtcagcgtatcttccttttagaggctgaataatattccactgtatgaatataccacattttgttgatcattcacccactgatgggcacatattgcttccatctcttagctactgtgaataatggtgccgtgagtatgggcatacaaaaactaccactaatattttacagtgcttgcttcatatctgtccatgtgtccgtcactccacccatcatattttttatgtatttcataagttacagaccacagtaacttccctcaaacatgtcagtatacatatcaatgaccagcgttcattgtttttttccaagtcattttgaactgccgtagcaatgagtaatatagcctcaaacgcacacatacacacacaacacgtgcgtcactacagaaaacttttcctggcagacaggaaagggcccattgttggtgatgtcattttaattaagataaaaccaccaccaccatttagtaatagcctggggtaacaagggctgcgtcacggactgccacttttgccatcctgctcagagcagggccatgcctaacccgtatctggggattgcttcagatattatgaatcgcttcaatattatgaattactacaattcataataattgcttcagatattatgaattacaatatggttcaaaggtgctttagcagatgaagacacaaatgtgtaaacacatatgaattacaatgcagactgcccagatgtgtagcaagtcctctgaatgtttactaaacagtaaggtgattccagaggaagatgcttgaggacaatttgggaaaactgacaacttgaaaactcagtctctctaggcaaggcctacttgcagataaccttgggagttctgtgctgggaggaaagctaaaggactaagttaggcctctgaatctgctctggaagcctgcatgcacttgggtcagaacaagcccatgtgtcaatgtgggtaaagattcctcagctgataagcaggaaaatgggcagggcattttggtctttgaggttcaaagctcagatgctcactgccttggtatacacgcacacacaccccaccccccagctgacggcacaagagtatacagatgcaatagtctaaagtacattgtccaaatatggatggccatgagccacatgtggctatgaagcacttaaatgtggctagtctgaactgagatgggccctataaaatatttcagtaacaggtttttatactgattataggttgacataataatattttggatataccgtattaaaggaaatatgtcattaaatttcacctgtttcctttattatgtggctacttgaaaattttaaaattacatatgtagctcacactataaaacacagattagaaatattgtatagcactgacctagaaacctccatttaggtaaaacatcttaacccctttggaagcaaaatatgttaaataacagcataaactcccaccaagaaaatcctcaccttcctcctttcaacacatttattatatacagctgtcactgcattgtcaatctgccaaatggctctatgttccaacagggctggagtagtcccctgctcacaccagccttcacaatacttcccatgtcttccctgttaacctctctccacccagcacccaggctcccaactctcctggctgcctccagccctcagctggcaccactgacatgctgtttccagtacccttttcttctttctgcatcctccctgggggacatatatccctcatctcgtgacttcagctgtcacataaattcaaatgtttcagaactctattttttacctcctacatctgtcagtttaaatgtcaggatattttactttcagtaaagccctaaaaagacaaatctatgtacttttaaagaataaaagaaatgactggctgcagctcaaacctacaactgcttgcgaaactctacaatgtctggcagatgctagaaagaaggggatcaagacagagcacacttggcgtggtatgctatctatagaaaatgttaaaataaaattaagtaatctaggtttcctctctttattttctacatctactctctgaagagggcaataaataaggaaatgtcccaaagagggacaaattaagtcccaaaataacacaaaattgggcaaatccagtcatgaagaaagaacagaggttcttaaattgggacacacagaggcaggtctgcaggtctaggaatctctgaacatatgtgcaaaattctgggtatgtgtgcatatgttatataacaaagcgaagggtccatatagctttcatcgcatttcaaagggtctagcactgaaataaggactactgctatgtgacttaaaaaatgaaactcaggctgggcgcagtggctcacgcctgtaatcccagcactttgggaggccgaggcaagcagatcacctgagacgaggagtttgagacccgcctggccaacggtgaaacccagtctctactaaaaatacaaaaattagccggaattggtggtgtgcctctagtcccagctactcaggaggctgaagaaagagaatcgcttgaacctgggaggtggaggttgtgacaaagcaagactccatctcaaaaaaaaaaaaaacccagaaactcaattcagttatgaaggtaaagatgacctgtttacatgataatattttaagataccagtgactgcaagcatgtagttattaagtccattacagtgcacatttattgactctgtgtatcttcacagtgtgatcttcaccacagcttgcaaagtgtaaccactcagcaccttctgcttccttctgttcagtttttccactgcaattcttccagcataattttctgatagccagtgtatgactttggctttgacttgtttctacacagtgggtccagtcatttatttctggaacttgatcagtctttttccaggtatataagcaaatctttccacactccaatcctactgcaaccacgtatcgttgagaagggtggagcactgggcagacgctgacagctgtcacagccccacccacgtccaggactgaggagcaggggccaatgttgtgctcaatacagtcatcagtggagtcgcactcaccccagacaaccacctttttgtctcgactcccagtgaagaaatacttgctgtcaggactccaatcacaagaccaaataattctactgtgcacagaagtaattttgttggtgaaggcaaaaagactaaaaactggctcgaactcaggtgagattgtatcctgctttttccacaatgaccaggttcgatctctggaaacagctagtaagaacttctcattaggtgagaaggccatctgcgtgactgtcaaactgtggaaaactaaattctgcacctgtttccaagatgtagtgttccaaagaatgatagctgcatgctctttcttagctgccttacaagctgaggcaagcagagtctttgaactgttacaagtaacacaaaatatttcataaccgtgcccatatagtttttgaacttcaggccacaaagtattctgcagaagatgatcctcagtgggaggctcagtaagtatggagggctgaaaggccacctgctgatactcaaaaccagtactagttaacagctcctcttcatcagaaggctgagaagctatatctccctgaaagacagctttatttgataatcccaatgcagggacagtggctccttctggaagatcactatcttgattacagagcacatgattcagtgattgtcctgtaatggcacaaaaattttccacaaaattccgaggtgcagaaaaaacccgaagaactttttcatctgctccagatacaaactgaaaccgattaatcattgccaaacatttcaggtcatacccatgtatctgaggccttgcaatttcatgccaagtcacctgtgattggtcttttctcttccatggagcaaaaagtctagttgtctgatcagtaccaacagtgataataaattctccttctggatcccagactaggtcttggacaccatcaaagtgtcctgaaatgacaatctctggagtccactctctctgttctagccaaactcctgactcttcatctggagcccagagaatcatggttttatccatggaagcagataataatctcactggctgctgtaggacaccatctttgtaaaacacaggttgccagtgaactgcatttacccagttttcatgaccggctagcactgtctccagagtaacagcaaatgctattttaacactttcattttctatggtaaaagtattttctttcagtcttatgttatcgtcatcctgagtttctaaagatgttgactttatatacagcttccatattcttatcaggcaatcttgtgaacagcttgctaggaaaagatctctaccaaaggctgcccattccactcctctaatccaatcctcatgtccacagagagaaagcactttctgaaactgatcattttgttgagcaaatatgtgaattctgcaatcatcattgccacatgctaatattggtacttctggaccctttttagaccagagtcgaacagcagaatctgcagctgcagaaacgatcagtgtacataatgcaggatctgatgtcctcctctggtaaacagcatgcaccgcataaacaggtccttcatggccttgaagatgcactgcttttaaaagctgattatcctctatttcccagtgaatcacttgattatcagatcctccagaaactaattcagtagaaggggagccatcctgtttacaaatccactgtatgcaattgactcgggcggtgtgaccattcaagttggtaacaacaacccttttcagggggtcatagagcaccacggagcaggacgtgccaaaggccagaagtcctctgggcccagagctccagttcaggactccccgcacccggtttgggcagcaaaacacgtgagaagtctccagcacgggtgccaccatgtcgccaactggtcagccgcacaaacaagagacgc

SEQ ID NO: 13431 - RNA, 7074 nt, Homo sapiens
  source 1..7074: mol_type = other RNA
gctgggattacaggcatgagccaccacgcccggcccgggtcccagatctctgagtccaccagagtggggctcagagtcctctatccaccaaccacatgcagccatccaacacgctgtctctcttctggcctcagcctcattgtccttggagtgccagtctcttgtttaagcatggcagagccttaatactggaccatccactacatgctagaaggggaagaactcctcacaatgtaacaatttttgtatttaacttatggatatgctcattctttctaaacaattcttataaggaaattttaagtatattaaaaaattagaatagtatgaccaccccaacactgcccagcttcattaataatccacacatctaaaacccatctagtccttgacacacacacaatcattatgaaacaacccaagacataaattgatttcatccataaatactgaaattatgattcaagagaactttttttttttttttcttaaaccaaggctgaggtgggagaactgcttgagcccaggagttcaagaccagcttaggtaacactgcaaaacccagtctctagagaaaaaaaaaacaaaaccaatcataaccatagccccactgtcatatgtttaaatgttgtttccttaatatcatcaaatatccagccagagttcaaatttgctttgtcccttaagcacatttttacaagattgattggctagttcagatcaagaggcaaacaaggttcatacattgcactggattcacacgtctcaagtatctttcaatctccaggcttcccttcccttcccttttcctcttgtaatgtatttgttgaagaatctaggtccctctgtagtcactcctctccccattcccagcccctggtaaccacttacctgttttctgaccctataattttgtagggcccactttgtactgatgtacttctgactaggtgtgtttatgttcaagcatcagagccaaggcccaaacctctaccctggccctccttctgctgtggcccaactgtacccagagctgggctctcccgtctccctgcctgttaatcctagaagtgggtgccgaggagggagaaacaggaaggagggagttggggagggcagcttgttacatggacatcagggctgttcccactagcagcaacagctttgtgttagcttggctccaatttgaatgaaatattccaaggccattttccccaacacgttgttaccaaaaaaactcccagcatgcagaaaagttgaaagaattgtacagtgaacaccccttaaggagtttctaccattaacattttatttaaaggctttgggactctgaagtataatgtttgtgaaatgctatgagccagaccctccacactgaaaattcccagtgtaaattaatttgttaaatgctcttagaattcctgcaataaagaacacctatctaaccttagttatccctgtgtttcccaaatatatcttactttggagcactttttttttagtaccgatttacatcctgggaaatggtgtttaccatgctttaaaaaaaactgtggtaaaataaagataagatttaccatcttaaccattttagagtgtacagttgagttggcatacagcattcacataacttaactgtgcaaccaatccacaggactttttatcttgcaaaactgaaacactatacccattaaacaactcctcatttcctcctcccccagtccttggcaactaccattctacttgtttctatgcatttgactgctctagatacttcacataaatggaagcatagagtatttgtcttccagtgactggcttacttcacttagcatcatgtcctcaagattcatccatgttgcagcacatgtcagcgtatcttccttttagaggctgaataatattccactgtatgaatataccacattttgttgatcattcacccactgatgggcacatattgcttccatctcttagctactgtgaataatggtgccgtgagtatgggcatacaaaaactaccactaatattttacagtgcttgcttcatatctgtccatgtgtccgtcactccacccatcatattttttatgtatttcataagttacagaccacagtaacttccctcaaacatgtcagtatacatatcaatgaccagcgttcattgtttttttccaagtcattttgaactgccgtagcaatgagtaatatagcctcaaacgcacacatacacacacaacacgtgcgtcactacagaaaacttttcctggcagacaggaaagggcccattgttggtgatgtcattttaattaagataaaaccaccaccaccatttagtaatagcctggggtaacaagggctgcgtcacggactgccacttttgccatcctgctcagagcagggccatgcctaacccgtatctggggattgcttcagatattatgaatcgcttcaatattatgaattactacaattcataataattgcttcagatattatgaattacaatatggttcaaaggtgctttagcagatgaagacacaaatgtgtaaacacatatgaattacaatgcagactgcccagatgtgtagcaagtcctctgaatgtttactaaacagtaaggtgattccagaggaagatgcttgaggacaatttgggaaaactgacaacttgaaaactcagtctctctaggcaaggcctacttgcagataaccttgggagttctgtgctgggaggaaagctaaaggactaagttaggcctctgaatctgctctggaagcctgcatgcacttgggtcagaacaagcccatgtgtcaatgtgggtaaagattcctcagctgataagcaggaaaatgggcagggcattttggtctttgaggttcaaagctcagatgctcactgccttggtatacacgcacacacaccccaccccccagctgacggcacaagagtatacagatgcaatagtctaaagtacattgtccaaatatggatggccatgagccacatgtggctatgaagcacttaaatgtggctagtctgaactgagatgggccctataaaatatttcagtaacaggtttttatactgattataggttgacataataatattttggatataccgtattaaaggaaatatgtcattaaatttcacctgtttcctttattatgtggctacttgaaaattttaaaattacatatgtagctcacactataaaacacagattagaaatattgtatagcactgacctagaaacctccatttaggtaaaacatcttaacccctttggaagcaaaatatgttaaataacagcataaactcccaccaagaaaatcctcaccttcctcctttcaacacatttattatatacagctgtcactgcattgtcaatctgccaaatggctctatgttccaacagggctggagtagtcccctgctcacaccagccttcacaatacttcccatgtcttccctgttaacctctctccacccagcacccaggctcccaactctcctggctgcctccagccctcagctggcaccactgacatgctgtttccagtacccttttcttctttctgcatcctccctgggggacatatatccctcatctcgtgacttcagctgtcacataaattcaaatgtttcagaactctattttttacctcctacatctgtcagtttaaatgtcaggatattttactttcagtaaagccctaaaaagacaaatctatgtacttttaaagaataaaagaaatgactggctgcagctcaaacctacaactgcttgcgaaactctacaatgtctggcagatgctagaaagaaggggatcaagacagagcacacttggcgtggtatgctatctatagaaaatgttaaaataaaattaagtaatctaggtttcctctctttattttctacatctactctctgaagagggcaataaataaggaaatgtcccaaagagggacaaattaagtcccaaaataacacaaaattgggcaaatccagtcatgaagaaagaacagaggttcttaaattgggacacacagaggcaggtctgcaggtctaggaatctctgaacatatgtgcaaaattctgggtatgtgtgcatatgttatataacaaagcgaagggtccatatagctttcatcgcatttcaaagggtctagcactgaaataaggactactgctatgtgacttaaaaaatgaaactcaggctgggcgcagtggctcacgcctgtaatcccagcactttgggaggccgaggcaagcagatcacctgagacgaggagtttgagacccgcctggccaacggtgaaacccagtctctactaaaaatacaaaaattagccggaattggtggtgtgcctctagtcccagctactcaggaggctgaagaaagagaatcgcttgaacctgggaggtggaggttgtgacaaagcaagactccatctcaaaaaaaaaaaaaacccagaaactcaattcagttatgaaggtaaagatgacctgtttacatgataatattttaagataccagtgactgcaagcatgtagttattaagtccattacagtgcacatttattgactctgtgtatcttcacagtgtgatcttcaccacagcttgcaaagtgtaaccactcagcaccttctgcttccttctgttcagtttttccactgcaattcttccagcataattttctgatagccagtgtatgactttggctttgacttgtttctacacagtgggtccagtcatttatttctggaacttgatcagtctttttccaggtatataagcaaatctttccacactccaatcctactgcaaccacgtatcgttgagaagggtggagcactgggcagacgctgacagctgtcacagccccacccacgtccaggactgaggagcaggggccaatgttgtgctcaatacagtcatcagtggagtcgcactcaccccagacaaccacctttttgtctcgactcccagtgaagaaatacttgctgtcaggactccaatcacaagaccaaataattctactgtgcacagaagtaattttgttggtgaaggcaaaaagactaaaaactggctcgaactcaggtgagattgtatcctgctttttccacaatgaccaggttcgatctctggaaacagctagtaagaacttctcattaggtgagaaggccatctgcgtgactgtcaaactgtggaaaactaaattctgcacctgtttccaagatgtagtgttccaaagaatgatagctgcatgctctttcttagctgccttacaagctgaggcaagcagagtctttgaactgttacaagtaacacaaaatatttcataaccgtgcccatatagtttttgaacttcaggccacaaagtattctgcagaagatgatcctcagtgggaggctcagtaagtatggagggctgaaaggccacctgctgatactcaaaaccagtactagttaacagctcctcttcatcagaaggctgagaagctatatctccctgaaagacagctttatttgataatcccaatgcagggacagtggctccttctggaagatcactatcttgattacagagcacatgattcagtgattgtcctgtaatggcacaaaaattttccacaaaattccgaggtgcagaaaaaacccgaagaactttttcatctgctccagatacaaactgaaaccgattaatcattgccaaacatttcaggtcatacccatgtatctgaggccttgcaatttcatgccaagtcacctgtgattggtcttttctcttccatggagcaaaaagtctagttgtctgatcagtaccaacagtgataataaattctccttctggatcccagactaggtcttggacaccatcaaagtgtcctgaaatgacaatctctggagtccactctctctgttctagccaaactcctgactcttcatctggagcccagagaatcatggttttatccatggaagcagataataatctcactggctgctgtaggacaccatctttgtaaaacacaggttgccagtgaactgcatttacccagttttcatgaccggctagcactgtctccagagtaacagcaaatgctattttaacactttcattttctatggtaaaagtattttctttcagtcttatgttatcgtcatcctgagtttctaaagatgttgactttatatacagcttccatattcttatcaggcaatcttgtgaacagcttgctaggaaaagatctctaccaaaggctgcccattccactcctctaatccaatcctcatgtccacagagagaaagcactttctgaaactgatcattttgttgagcaaatatgtgaattctgcaatcatcattgccacatgctaatattggtattggcctgaatgcagatggaagaaatgaaattctgttatgatgccagaatgtgtgcagcttctccttccacagagccttgcacagaatggaagcgtaacatgaaaccatagagtcgcagctcctgctacagagggcgagagaggctggtggcttccaggccctgcctcgttccacctggccagtcttccaggtaacttctggaccctttttagaccagagtcgaacagcagaatctgcagctgcagaaacgatcagtgtacataatgcaggatctgatgtcctcctctggtaaacagcatgcaccgcataaacaggtccttcatggccttgaagatgcactgcttttaaaagctgattatcctctatttcccagtgaatcacttgattatcagatcctccagaaactaattcagtagaaggggagccatcctgtttacaaatccactgtatgcaattgactcgggcggtgtgaccattcaagttggtaacaacaacccttttcagggggtcatagagcaccacggagcaggacgtgccaaaggccagaagtcctctgggcccagagctccagttcaggactccccgcacccggtttgggcagcaaaacacgtgagaagtctccagcacgggtgccaccatgtcgccaactggtcagccgcacaaacaagagacgc

SEQ ID NO: 13432 - RNA, 7089 nt, Homo sapiens
  source 1..7089: mol_type = other RNA
gctgggattacaggcatgagccaccacgcccggcccgggtcccagatctctgagtccaccagagtggggctcagagtcctctatccaccaaccacatgcagccatccaacacgctgtctctcttctggcctcagcctcattgtccttggagtgccagtctcttgtttaagcatggcagagccttaatactggaccatccactacatgctagaaggggaagaactcctcacaatgtaacaatttttgtatttaacttatggatatgctcattctttctaaacaattcttataaggaaattttaagtatattaaaaaattagaatagtatgaccaccccaacactgcccagcttcattaataatccacacatctaaaacccatctagtccttgacacacacacaatcattatgaaacaacccaagacataaattgatttcatccataaatactgaaattatgattcaagagaactttttttttttttttcttaaaccaaggctgaggtgggagaactgcttgagcccaggagttcaagaccagcttaggtaacactgcaaaacccagtctctagagaaaaaaaaaacaaaaccaatcataaccatagccccactgtcatatgtttaaatgttgtttccttaatatcatcaaatatccagccagagttcaaatttgctttgtcccttaagcacatttttacaagattgattggctagttcagatcaagaggcaaacaaggttcatacattgcactggattcacacgtctcaagtatctttcaatctccaggcttcccttcccttcccttttcctcttgtaatgtatttgttgaagaatctaggtccctctgtagtcactcctctccccattcccagcccctggtaaccacttacctgttttctgaccctataattttgtagggcccactttgtactgatgtacttctgactaggtgtgtttatgttcaagcatcagagccaaggcccaaacctctaccctggccctccttctgctgtggcccaactgtacccagagctgggctctcccgtctccctgcctgttaatcctagaagtgggtgccgaggagggagaaacaggaaggagggagttggggagggcagcttgttacatggacatcagggctgttcccactagcagcaacagctttgtgttagcttggctccaatttgaatgaaatattccaaggccattttccccaacacgttgttaccaaaaaaactcccagcatgcagaaaagttgaaagaattgtacagtgaacaccccttaaggagtttctaccattaacattttatttaaaggctttgggactctgaagtataatgtttgtgaaatgctatgagccagaccctccacactgaaaattcccagtgtaaattaatttgttaaatgctcttagaattcctgcaataaagaacacctatctaaccttagttatccctgtgtttcccaaatatatcttactttggagcactttttttttagtaccgatttacatcctgggaaatggtgtttaccatgctttaaaaaaaactgtggtaaaataaagataagatttaccatcttaaccattttagagtgtacagttgagttggcatacagcattcacataacttaactgtgcaaccaatccacaggactttttatcttgcaaaactgaaacactatacccattaaacaactcctcatttcctcctcccccagtccttggcaactaccattctacttgtttctatgcatttgactgctctagatacttcacataaatggaagcatagagtatttgtcttccagtgactggcttacttcacttagcatcatgtcctcaagattcatccatgttgcagcacatgtcagcgtatcttccttttagaggctgaataatattccactgtatgaatataccacattttgttgatcattcacccactgatgggcacatattgcttccatctcttagctactgtgaataatggtgccgtgagtatgggcatacaaaaactaccactaatattttacagtgcttgcttcatatctgtccatgtgtccgtcactccacccatcatattttttatgtatttcataagttacagaccacagtaacttccctcaaacatgtcagtatacatatcaatgaccagcgttcattgtttttttccaagtcattttgaactgccgtagcaatgagtaatatagcctcaaacgcacacatacacacacaacacgtgcgtcactacagaaaacttttcctggcagacaggaaagggcccattgttggtgatgtcattttaattaagataaaaccaccaccaccatttagtaatagcctggggtaacaagggctgcgtcacggactgccacttttgccatcctgctcagagcagggccatgcctaacccgtatctggggattgcttcagatattatgaatcgcttcaatattatgaattactacaattcataataattgcttcagatattatgaattacaatatggttcaaaggtgctttagcagatgaagacacaaatgtgtaaacacatatgaattacaatgcagactgcccagatgtgtagcaagtcctctgaatgtttactaaacagtaaggtgattccagaggaagatgcttgaggacaatttgggaaaactgacaacttgaaaactcagtctctctaggcaaggcctacttgcagataaccttgggagttctgtgctgggaggaaagctaaaggactaagttaggcctctgaatctgctctggaagcctgcatgcacttgggtcagaacaagcccatgtgtcaatgtgggtaaagattcctcagctgataagcaggaaaatgggcagggcattttggtctttgaggttcaaagctcagatgctcactgccttggtatacacgcacacacaccccaccccccagctgacggcacaagagtatacagatgcaatagtctaaagtacattgtccaaatatggatggccatgagccacatgtggctatgaagcacttaaatgtggctagtctgaactgagatgggccctataaaatatttcagtaacaggtttttatactgattataggttgacataataatattttggatataccgtattaaaggaaatatgtcattaaatttcacctgtttcctttattatgtggctacttgaaaattttaaaattacatatgtagctcacactataaaacacagattagaaatattgtatagcactgacctagaaacctccatttaggtaaaacatcttaacccctttggaagcaaaatatgttaaataacagcataaactcccaccaagaaaatcctcaccttcctcctttcaacacatttattatatacagctgtcactgcattgtcaatctgccaaatggctctatgttccaacagggctggagtagtcccctgctcacaccagccttcacaatacttcccatgtcttccctgttaacctctctccacccagcacccaggctcccaactctcctggctgcctccagccctcagctggcaccactgacatgctgtttccagtacccttttcttctttctgcatcctccctgggggacatatatccctcatctcgtgacttcagctgtcacataaattcaaatgtttcagaactctattttttacctcctacatctgtcagtttaaatgtcaggatattttactttcagtaaagccctaaaaagacaaatctatgtacttttaaagaataaaagaaatgactggctgcagctcaaacctacaactgcttgcgaaactctacaatgtctggcagatgctagaaagaaggggatcaagacagagcacacttggcgtggtatgctatctatagaaaatgttaaaataaaattaagtaatctaggtttcctctctttattttctacatctactctctgaagagggcaataaataaggaaatgtcccaaagagggacaaattaagtcccaaaataacacaaaattgggcaaatccagtcatgaagaaagaacagaggttcttaaattgggacacacagaggcaggtctgcaggtctaggaatctctgaacatatgtgcaaaattctgggtatgtgtgcatatgttatataacaaagcgaagggtccatatagctttcatcgcatttcaaagggtctagcactgaaataaggactactgctatgtgacttaaaaaatgaaactcaggctgggcgcagtggctcacgcctgtaatcccagcactttgggaggccgaggcaagcagatcacctgagacgaggagtttgagacccgcctggccaacggtgaaacccagtctctactaaaaatacaaaaattagccggaattggtggtgtgcctctagtcccagctactcaggaggctgaagaaagagaatcgcttgaacctgggaggtggaggttgtgacaaagcaagactccatctcaaaaaaaaaaaaaacccagaaactcaattcagttatgaaggtaaagatgacctgtttacatgataatattttaagataccagtgactgcaagcatgtagttattaagtccattacagtgcacatttattgactctgtgtatcttcacagtgtgatcttcaccacagcttgcaaagtgtaaccactcagcaccttctgcttccttctgttcagtttttccactgcaattcttccagcataattttctgatagccagtgtatgactttggctttgacttgtttctacacagtgggtccagtcatttatttctggaacttgatcagtctttttccaggtatataagcaaatctttccacactccaatcctactgcaaccacgtatcgttgagaagggtggagcactgggcagacgctgacagctgtcacagccccacccacgtccaggactgaggagcaggggccaatgttgtgctcaatacagtcatcagtggagtcgcactcaccccagacaaccacctttttgtctcgactcccagtgaagaaatacttgctgtcaggactccaatcacaagaccaaataattctactgtgcacagaagtaattttgttggtgaaggcaaaaagactaaaaactggctcgaactcaggtgagattgtatcctgctttttccacaatgaccaggttcgatctctggaaacagctagtaagaacttctcattaggtgagaaggccatctgcgtgactgtcaaactgtggaaaactaaattctgcacctgtttccaagatgtagtgttccaaagaatgatagctgcatgctctttcttagctgccttacaagctgaggcaagcagagtctttgaactgttacaagtaacacaaaatatttcataaccgtgcccatatagtttttgaacttcaggccacaaagtattctgcagaagatgatcctcagtgggaggctcagtaagtatggagggctgaaaggccacctgctgatactcaaaaccagtactagttaacagctcctcttcatcagaaggctgagaagctatatctccctgaaagacagctttatttgataatcccaatgcagggacagtggctccttctggaagatcactatcttgattacagagcacatgattcagtgattgtcctgtaatggcacaaaaattttccacaaaattccgaggtgcagaaaaaacccgaagaactttttcatctgctccagatacaaactgaaaccgattaatcattgccaaacatttcaggtcatacccatgtatctgaggccttgcaatttcatgccaagtcacctgtgattggtcttttctcttccatggagcaaaaagtctagttgtctgatcagtaccaacagtgataataaattctccttctggatcccagactaggtcttggacaccatcaaagtgtcctgaaatgacaatctctggagtccactctcttgggttaactgtattctgtttccaaaggtgcaacgctccgtggaaagcatgagcaatgatcatggagccatcttcattgaactggcaatcataaaatcccaaagtattcccacctacttcacctactcgaacctgttctagccaaactcctgactcttcatctggagcccagagaatcatggttttatccatggaagcagataataatctcactggctgctgtaggacaccatctttgtaaaacacaggttgccagtgaactgcatttacccagttttcatgaccggctagcactgtctccagagtaacagcaaatgctattttaacactttcattttctatggtaaaagtattttctttcagtcttatgttatcgtcatcctgagtttctaaagatgttgactttatatacagcttccatattcttatcaggcaatcttgtgaacagcttgctaggaaaagatctctaccaaaggctgcccattccactcctctaatccaatcctcatgtccacagagagaaagcactttctgaaactgatcattttgttgagcaaatatgtgaattctgcaatcatcattgccacatgctaatattggtacatcagtatttggcaaaaaagataagcagagagccaaagcaaatccatttccaaagtttaaagtctgaaggcacattacttctggaccctttttagaccagagtcgaacagcagaatctgcagctgcagaaacgatcagtgtacataatgcaggatctgatgtcctcctctggtaaacagcatgcaccgcataaacaggtccttcatggccttgaagatgcactgcttttaaaagctgattatcctctatttcccagtgaatcacttgattatcagatcctccagaaactaattcagtagaaggggagccatcctgtttacaaatccactgtatgcaattgactcgggcggtgtgaccattcaagttggtaacaacaacccttttcagggggtcatagagcaccacggagcaggacgtgccaaaggccagaagtcctctgggcccagagctccagttcaggactccccgcacccggtttgggcagcaaaacacgtgagaagtctccagcacgggtgccaccatgtcgccaactggtcagccgcacaaacaagagacgc

SEQ ID NO: 13433 - RNA, 7010 nt, Homo sapiens
  source 1..7010: mol_type = other RNA
gctgggattacaggcatgagccaccacgcccggcccgggtcccagatctctgagtccaccagagtggggctcagagtcctctatccaccaaccacatgcagccatccaacacgctgtctctcttctggcctcagcctcattgtccttggagtgccagtctcttgtttaagcatggcagagccttaatactggaccatccactacatgctagaaggggaagaactcctcacaatgtaacaatttttgtatttaacttatggatatgctcattctttctaaacaattcttataaggaaattttaagtatattaaaaaattagaatagtatgaccaccccaacactgcccagcttcattaataatccacacatctaaaacccatctagtccttgacacacacacaatcattatgaaacaacccaagacataaattgatttcatccataaatactgaaattatgattcaagagaactttttttttttttttcttaaaccaaggctgaggtgggagaactgcttgagcccaggagttcaagaccagcttaggtaacactgcaaaacccagtctctagagaaaaaaaaaacaaaaccaatcataaccatagccccactgtcatatgtttaaatgttgtttccttaatatcatcaaatatccagccagagttcaaatttgctttgtcccttaagcacatttttacaagattgattggctagttcagatcaagaggcaaacaaggttcatacattgcactggattcacacgtctcaagtatctttcaatctccaggcttcccttcccttcccttttcctcttgtaatgtatttgttgaagaatctaggtccctctgtagtcactcctctccccattcccagcccctggtaaccacttacctgttttctgaccctataattttgtagggcccactttgtactgatgtacttctgactaggtgtgtttatgttcaagcatcagagccaaggcccaaacctctaccctggccctccttctgctgtggcccaactgtacccagagctgggctctcccgtctccctgcctgttaatcctagaagtgggtgccgaggagggagaaacaggaaggagggagttggggagggcagcttgttacatggacatcagggctgttcccactagcagcaacagctttgtgttagcttggctccaatttgaatgaaatattccaaggccattttccccaacacgttgttaccaaaaaaactcccagcatgcagaaaagttgaaagaattgtacagtgaacaccccttaaggagtttctaccattaacattttatttaaaggctttgggactctgaagtataatgtttgtgaaatgctatgagccagaccctccacactgaaaattcccagtgtaaattaatttgttaaatgctcttagaattcctgcaataaagaacacctatctaaccttagttatccctgtgtttcccaaatatatcttactttggagcactttttttttagtaccgatttacatcctgggaaatggtgtttaccatgctttaaaaaaaactgtggtaaaataaagataagatttaccatcttaaccattttagagtgtacagttgagttggcatacagcattcacataacttaactgtgcaaccaatccacaggactttttatcttgcaaaactgaaacactatacccattaaacaactcctcatttcctcctcccccagtccttggcaactaccattctacttgtttctatgcatttgactgctctagatacttcacataaatggaagcatagagtatttgtcttccagtgactggcttacttcacttagcatcatgtcctcaagattcatccatgttgcagcacatgtcagcgtatcttccttttagaggctgaataatattccactgtatgaatataccacattttgttgatcattcacccactgatgggcacatattgcttccatctcttagctactgtgaataatggtgccgtgagtatgggcatacaaaaactaccactaatattttacagtgcttgcttcatatctgtccatgtgtccgtcactccacccatcatattttttatgtatttcataagttacagaccacagtaacttccctcaaacatgtcagtatacatatcaatgaccagcgttcattgtttttttccaagtcattttgaactgccgtagcaatgagtaatatagcctcaaacgcacacatacacacacaacacgtgcgtcactacagaaaacttttcctggcagacaggaaagggcccattgttggtgatgtcattttaattaagataaaaccaccaccaccatttagtaatagcctggggtaacaagggctgcgtcacggactgccacttttgccatcctgctcagagcagggccatgcctaacccgtatctggggattgcttcagatattatgaatcgcttcaatattatgaattactacaattcataataattgcttcagatattatgaattacaatatggttcaaaggtgctttagcagatgaagacacaaatgtgtaaacacatatgaattacaatgcagactgcccagatgtgtagcaagtcctctgaatgtttactaaacagtaaggtgattccagaggaagatgcttgaggacaatttgggaaaactgacaacttgaaaactcagtctctctaggcaaggcctacttgcagataaccttgggagttctgtgctgggaggaaagctaaaggactaagttaggcctctgaatctgctctggaagcctgcatgcacttgggtcagaacaagcccatgtgtcaatgtgggtaaagattcctcagctgataagcaggaaaatgggcagggcattttggtctttgaggttcaaagctcagatgctcactgccttggtatacacgcacacacaccccaccccccagctgacggcacaagagtatacagatgcaatagtctaaagtacattgtccaaatatggatggccatgagccacatgtggctatgaagcacttaaatgtggctagtctgaactgagatgggccctataaaatatttcagtaacaggtttttatactgattataggttgacataataatattttggatataccgtattaaaggaaatatgtcattaaatttcacctgtttcctttattatgtggctacttgaaaattttaaaattacatatgtagctcacactataaaacacagattagaaatattgtatagcactgacctagaaacctccatttaggtaaaacatcttaacccctttggaagcaaaatatgttaaataacagcataaactcccaccaagaaaatcctcaccttcctcctttcaacacatttattatatacagctgtcactgcattgtcaatctgccaaatggctctatgttccaacagggctggagtagtcccctgctcacaccagccttcacaatacttcccatgtcttccctgttaacctctctccacccagcacccaggctcccaactctcctggctgcctccagccctcagctggcaccactgacatgctgtttccagtacccttttcttctttctgcatcctccctgggggacatatatccctcatctcgtgacttcagctgtcacataaattcaaatgtttcagaactctattttttacctcctacatctgtcagtttaaatgtcaggatattttactttcagtaaagccctaaaaagacaaatctatgtacttttaaagaataaaagaaatgactggctgcagctcaaacctacaactgcttgcgaaactctacaatgtctggcagatgctagaaagaaggggatcaagacagagcacacttggcgtggtatgctatctatagaaaatgttaaaataaaattaagtaatctaggtttcctctctttattttctacatctactctctgaagagggcaataaataaggaaatgtcccaaagagggacaaattaagtcccaaaataacacaaaattgggcaaatccagtcatgaagaaagaacagaggttcttaaattgggacacacagaggcaggtctgcaggtctaggaatctctgaacatatgtgcaaaattctgggtatgtgtgcatatgttatataacaaagcgaagggtccatatagctttcatcgcatttcaaagggtctagcactgaaataaggactactgctatgtgacttaaaaaatgaaactcaggctgggcgcagtggctcacgcctgtaatcccagcactttgggaggccgaggcaagcagatcacctgagacgaggagtttgagacccgcctggccaacggtgaaacccagtctctactaaaaatacaaaaattagccggaattggtggtgtgcctctagtcccagctactcaggaggctgaagaaagagaatcgcttgaacctgggaggtggaggttgtgacaaagcaagactccatctcaaaaaaaaaaaaaacccagaaactcaattcagttatgaaggtaaagatgacctgtttacatgataatattttaagataccagtgactgcaagcatgtagttattaagtccattacagtgcacatttattgactctgtgtatcttcacagtgtgatcttcaccacagcttgcaaagtgtaaccactcagcaccttctgcttccttctgttcagtttttccactgcaattcttccagcataattttctgatagccagtgtatgactttggctttgacttgtttctacacagtgggtccagtcatttatttctggaacttgatcagtctttttccaggtatataagcaaatctttccacactccaatcctactgcaaccacgtatcgttgagaagggtggagcactgggcagacgctgacagctgtcacagccccacccacgtccaggactgaggagcaggggccaatgttgtgctcaatacagtcatcagtggagtcgcactcaccccagacaaccacctttttgtctcgactcccagtgaagaaatacttgctgtcaggactccaatcacaagaccaaataattctactgtgcacagaagtaattttgttggtgaaggcaaaaagactaaaaactggctcgaactcaggtgagattgtatcctgctttttccacaatgaccaggttcgatctctggaaacagctagtaagaacttctcattaggtgagaaggccatctgcgtgactgtcaaactgtggaaaactaaattctgcacctgtttccaagatgtagtgttccaaagaatgatagctgcatgctctttcttagctgccttacaagctgaggcaagcagagtctttgaactgttacaagtaacacaaaatatttcataaccgtgcccatatagtttttgaacttcaggccacaaagtattctgcagaagatgatcctcagtgggaggctcagtaagtatggagggctgaaaggccacctgctgatactcaaaaccagtactagttaacagctcctcttcatcagaaggctgagaagctatatctccctgaaagacagctttatttgataatcccaatgcagggacagtggctccttctggaagatcactatcttgattacagagcacatgattcagtgattgtcctgtaatggcacaaaaattttccacaaaattccgaggtgcagaaaaaacccgaagaactttttcatctgctccagatacaaactgaaaccgattaatcattgccaaacatttcaggtcatacccatgtatctgaggccttgcaatttcatgccaagtcacctgtgattggtcttttctcttccatggagcaaaaagtctagttgtctgatcagtaccaacagtgataataaattctccttctggatcccagactaggtcttggacaccatcaaagtgtcctgaaatgacaatctctggagtccactctcttgggttaactgtattctgtttccaaaggtgcaacgctccgtggaaagcatgagcaatgatcatggagccatcttcattgaactggcaatcataaaatcccaaagtattcccacctacttcacctactcgaacctgttctagccaaactcctgactcttcatctggagcccagagaatcatggttttatccatggaagcagataataatctcactggctgctgtaggacaccatctttgtaaaacacaggttgccagtgaactgcatttacccagttttcatgaccggctagcactgtctccagagtaacagcaaatgctattttaacactttcattttctatggtaaaagtattttctttcagtcttatgttatcgtcatcctgagtttctaaagatgttgactttatatacagcttccatattcttatcaggcaatcttgtgaacagcttgctaggaaaagatctctaccaaaggctgcccattccactcctctaatccaatcctcatgtccacagagagaaagcactttctgaaactgatcattttgttgagcaaatatgtgaattctgcaatcatcattgccacatgctaatattggtacatcagtatttggcaaaaaagataagcagagagccaaagcaaatccatttccaaagtttaaagtctgaaggcacattacttctggaccctttttagaccagagtcgaacagcagaatctgcagctgcagaaacgatcagtgtacataatgcaggatctgatgtcctcctctggtaaacagcatgcaccgcataaacaggtccttcatggccttgaagatgcactgcttttaaaagctgattatcctctatttcccagtgaatcacttgattatcagatcctccagaaactaattcagtagaaggggcagggggtcatagagcaccacggagcaggacgtgccaaaggccagaagtcctctgggcccagagctccagttcaggactccccgcacccggtttgggcagcaaaacacgtgagaagtctccagcacgggtgccaccatgtcgccaactggtcagccgcacaaacaagagacgc

SEQ ID NO: 13434 - RNA, 7011 nt, Homo sapiens
  source 1..7011: mol_type = other RNA
gctgggattacaggcatgagccaccacgcccggcccgggtcccagatctctgagtccaccagagtggggctcagagtcctctatccaccaaccacatgcagccatccaacacgctgtctctcttctggcctcagcctcattgtccttggagtgccagtctcttgtttaagcatggcagagccttaatactggaccatccactacatgctagaaggggaagaactcctcacaatgtaacaatttttgtatttaacttatggatatgctcattctttctaaacaattcttataaggaaattttaagtatattaaaaaattagaatagtatgaccaccccaacactgcccagcttcattaataatccacacatctaaaacccatctagtccttgacacacacacaatcattatgaaacaacccaagacataaattgatttcatccataaatactgaaattatgattcaagagaactttttttttttttttcttaaaccaaggctgaggtgggagaactgcttgagcccaggagttcaagaccagcttaggtaacactgcaaaacccagtctctagagaaaaaaaaaacaaaaccaatcataaccatagccccactgtcatatgtttaaatgttgtttccttaatatcatcaaatatccagccagagttcaaatttgctttgtcccttaagcacatttttacaagattgattggctagttcagatcaagaggcaaacaaggttcatacattgcactggattcacacgtctcaagtatctttcaatctccaggcttcccttcccttcccttttcctcttgtaatgtatttgttgaagaatctaggtccctctgtagtcactcctctccccattcccagcccctggtaaccacttacctgttttctgaccctataattttgtagggcccactttgtactgatgtacttctgactaggtgtgtttatgttcaagcatcagagccaaggcccaaacctctaccctggccctccttctgctgtggcccaactgtacccagagctgggctctcccgtctccctgcctgttaatcctagaagtgggtgccgaggagggagaaacaggaaggagggagttggggagggcagcttgttacatggacatcagggctgttcccactagcagcaacagctttgtgttagcttggctccaatttgaatgaaatattccaaggccattttccccaacacgttgttaccaaaaaaactcccagcatgcagaaaagttgaaagaattgtacagtgaacaccccttaaggagtttctaccattaacattttatttaaaggctttgggactctgaagtataatgtttgtgaaatgctatgagccagaccctccacactgaaaattcccagtgtaaattaatttgttaaatgctcttagaattcctgcaataaagaacacctatctaaccttagttatccctgtgtttcccaaatatatcttactttggagcactttttttttagtaccgatttacatcctgggaaatggtgtttaccatgctttaaaaaaaactgtggtaaaataaagataagatttaccatcttaaccattttagagtgtacagttgagttggcatacagcattcacataacttaactgtgcaaccaatccacaggactttttatcttgcaaaactgaaacactatacccattaaacaactcctcatttcctcctcccccagtccttggcaactaccattctacttgtttctatgcatttgactgctctagatacttcacataaatggaagcatagagtatttgtcttccagtgactggcttacttcacttagcatcatgtcctcaagattcatccatgttgcagcacatgtcagcgtatcttccttttagaggctgaataatattccactgtatgaatataccacattttgttgatcattcacccactgatgggcacatattgcttccatctcttagctactgtgaataatggtgccgtgagtatgggcatacaaaaactaccactaatattttacagtgcttgcttcatatctgtccatgtgtccgtcactccacccatcatattttttatgtatttcataagttacagaccacagtaacttccctcaaacatgtcagtatacatatcaatgaccagcgttcattgtttttttccaagtcattttgaactgccgtagcaatgagtaatatagcctcaaacgcacacatacacacacaacacgtgcgtcactacagaaaacttttcctggcagacaggaaagggcccattgttggtgatgtcattttaattaagataaaaccaccaccaccatttagtaatagcctggggtaacaagggctgcgtcacggactgccacttttgccatcctgctcagagcagggccatgcctaacccgtatctggggattgcttcagatattatgaatcgcttcaatattatgaattactacaattcataataattgcttcagatattatgaattacaatatggttcaaaggtgctttagcagatgaagacacaaatgtgtaaacacatatgaattacaatgcagactgcccagatgtgtagcaagtcctctgaatgtttactaaacagtaaggtgattccagaggaagatgcttgaggacaatttgggaaaactgacaacttgaaaactcagtctctctaggcaaggcctacttgcagataaccttgggagttctgtgctgggaggaaagctaaaggactaagttaggcctctgaatctgctctggaagcctgcatgcacttgggtcagaacaagcccatgtgtcaatgtgggtaaagattcctcagctgataagcaggaaaatgggcagggcattttggtctttgaggttcaaagctcagatgctcactgccttggtatacacgcacacacaccccaccccccagctgacggcacaagagtatacagatgcaatagtctaaagtacattgtccaaatatggatggccatgagccacatgtggctatgaagcacttaaatgtggctagtctgaactgagatgggccctataaaatatttcagtaacaggtttttatactgattataggttgacataataatattttggatataccgtattaaaggaaatatgtcattaaatttcacctgtttcctttattatgtggctacttgaaaattttaaaattacatatgtagctcacactataaaacacagattagaaatattgtatagcactgacctagaaacctccatttaggtaaaacatcttaacccctttggaagcaaaatatgttaaataacagcataaactcccaccaagaaaatcctcaccttcctcctttcaacacatttattatatacagctgtcactgcattgtcaatctgccaaatggctctatgttccaacagggctggagtagtcccctgctcacaccagccttcacaatacttcccatgtcttccctgttaacctctctccacccagcacccaggctcccaactctcctggctgcctccagccctcagctggcaccactgacatgctgtttccagtacccttttcttctttctgcatcctccctgggggacatatatccctcatctcgtgacttcagctgtcacataaattcaaatgtttcagaactctattttttacctcctacatctgtcagtttaaatgtcaggatattttactttcagtaaagccctaaaaagacaaatctatgtacttttaaagaataaaagaaatgactggctgcagctcaaacctacaactgcttgcgaaactctacaatgtctggcagatgctagaaagaaggggatcaagacagagcacacttggcgtggtatgctatctatagaaaatgttaaaataaaattaagtaatctaggtttcctctctttattttctacatctactctctgaagagggcaataaataaggaaatgtcccaaagagggacaaattaagtcccaaaataacacaaaattgggcaaatccagtcatgaagaaagaacagaggttcttaaattgggacacacagaggcaggtctgcaggtctaggaatctctgaacatatgtgcaaaattctgggtatgtgtgcatatgttatataacaaagcgaagggtccatatagctttcatcgcatttcaaagggtctagcactgaaataaggactactgctatgtgacttaaaaaatgaaactcaggctgggcgcagtggctcacgcctgtaatcccagcactttgggaggccgaggcaagcagatcacctgagacgaggagtttgagacccgcctggccaacggtgaaacccagtctctactaaaaatacaaaaattagccggaattggtggtgtgcctctagtcccagctactcaggaggctgaagaaagagaatcgcttgaacctgggaggtggaggttgtgacaaagcaagactccatctcaaaaaaaaaaaaaacccagaaactcaattcagttatgaaggtaaagatgacctgtttacatgataatattttaagataccagtgactgcaagcatgtagttattaagtccattacagtgcacatttattgactctgtgtatcttcacagtgtgatcttcaccacagcttgcaaagtgtaaccactcagcaccttctgcttccttctgttcagtttttccactgcaattcttccagcataattttctgatagccagtgtatgactttggctttgacttgtttctacacagtgggtccagtcatttatttctggaacttgatcagtctttttccaggtatataagcaaatctttccacactccaatcctactgcaaccacgtatcgttgagaagggtggagcactgggcagacgctgacagctgtcacagccccacccacgtccaggactgaggagcaggggccaatgttgtgctcaatacagtcatcagtggagtcgcactcaccccagacaaccacctttttgtctcgactcccagtgaagaaatacttgctgtcaggactccaatcacaagaccaaataattctactgtgcacagaagtaattttgttggtgaaggcaaaaagactaaaaactggctcgaactcaggtgagattgtatcctgctttttccacaatgaccaggttcgatctctggaaacagctagtaagaacttctcattaggtgagaaggccatctgcgtgactgtcaaactgtggaaaactaaattctgcacctgtttccaagatgtagtgttccaaagaatgatagctgcatgctctttcttagctgccttacaagctgaggcaagcagagtctttgaactgttacaagtaacacaaaatatttcataaccgtgcccatatagtttttgaacttcaggccacaaagtattctgcagaagatgatcctcagtgggaggctcagtaagtatggagggctgaaaggccacctgctgatactcaaaaccagtactagttaacagctcctcttcatcagaaggctgagaagctatatctccctgaaagacagctttatttgataatcccaatgcagggacagtggctccttctggaagatcactatcttgattacagagcacatgattcagtgattgtcctgtaatggcacaaaaattttccacaaaattccgaggtgcagaaaaaacccgaagaactttttcatctgctccagatacaaactgaaaccgattaatcattgccaaacatttcaggtcatacccatgtatctgaggccttgcaatttcatgccaagtcacctgtgattggtcttttctcttccatggagcaaaaagtctagttgtctgatcagtaccaacagtgataataaattctccttctggatcccagactaggtcttggacaccatcaaagtgtcctgaaatgacaatctctggagtccactctcttgggttaactgtattctgtttccaaaggtgcaacgctccgtggaaagcatgagcaatgatcatggagccatcttcattgaactggcaatcataaaatcccaaagtattcccacctacttcacctactcgaacctgttctagccaaactcctgactcttcatctggagcccagagaatcatggttttatccatggaagcagataataatctcactggctgctgtaggacaccatctttgtaaaacacaggttgccagtgaactgcatttacccagttttcatgaccggctagcactgtctccagagtaacagcaaatgctattttaacactttcattttctatggtaaaagtattttctttcagtcttatgttatcgtcatcctgagtttctaaagatgttgactttatatacagcttccatattcttatcaggcaatcttgtgaacagcttgctaggaaaagatctctaccaaaggctgcccattccactcctctaatccaatcctcatgtccacagagagaaagcactttctgaaactgatcattttgttgagcaaatatgtgaattctgcaatcatcattgccacatgctaatattggtacttctggaccctttttagaccagagtcgaacagcagaatctgcagctgcagaaacgatcagtgtacataatgcaggatctgatgtcctcctctggtaaacagcatgcaccgcataaacaggtccttcatggccttgaagatgcactgcttttaaaagctgattatcctctatttcccagtgaatcacttgattatcagatcctccagaaactaattcagtagaaggggagccatcctgtttacaaatccactgtatgcaattgactcgggcggtgtgaccattcaagttggtaacaacaacccttttcagggggtcatagagcaccacggagcaggacgtgccaaaggccagaagtcctctgggcccagagctccagttcaggactccccgcacccggtttgggcagcaaaacacgtgagaagtctccagcacgggtgccaccatgtcgccaactggtcagccgcacaaacaagagacgc

SEQ ID NO: 13435 - RNA, 7284 nt, Homo sapiens
  source 1..7284: mol_type = other RNA
gctgggattacaggcatgagccaccacgcccggcccgggtcccagatctctgagtccaccagagtggggctcagagtcctctatccaccaaccacatgcagccatccaacacgctgtctctcttctggcctcagcctcattgtccttggagtgccagtctcttgtttaagcatggcagagccttaatactggaccatccactacatgctagaaggggaagaactcctcacaatgtaacaatttttgtatttaacttatggatatgctcattctttctaaacaattcttataaggaaattttaagtatattaaaaaattagaatagtatgaccaccccaacactgcccagcttcattaataatccacacatctaaaacccatctagtccttgacacacacacaatcattatgaaacaacccaagacataaattgatttcatccataaatactgaaattatgattcaagagaactttttttttttttttcttaaaccaaggctgaggtgggagaactgcttgagcccaggagttcaagaccagcttaggtaacactgcaaaacccagtctctagagaaaaaaaaaacaaaaccaatcataaccatagccccactgtcatatgtttaaatgttgtttccttaatatcatcaaatatccagccagagttcaaatttgctttgtcccttaagcacatttttacaagattgattggctagttcagatcaagaggcaaacaaggttcatacattgcactggattcacacgtctcaagtatctttcaatctccaggcttcccttcccttcccttttcctcttgtaatgtatttgttgaagaatctaggtccctctgtagtcactcctctccccattcccagcccctggtaaccacttacctgttttctgaccctataattttgtagggcccactttgtactgatgtacttctgactaggtgtgtttatgttcaagcatcagagccaaggcccaaacctctaccctggccctccttctgctgtggcccaactgtacccagagctgggctctcccgtctccctgcctgttaatcctagaagtgggtgccgaggagggagaaacaggaaggagggagttggggagggcagcttgttacatggacatcagggctgttcccactagcagcaacagctttgtgttagcttggctccaatttgaatgaaatattccaaggccattttccccaacacgttgttaccaaaaaaactcccagcatgcagaaaagttgaaagaattgtacagtgaacaccccttaaggagtttctaccattaacattttatttaaaggctttgggactctgaagtataatgtttgtgaaatgctatgagccagaccctccacactgaaaattcccagtgtaaattaatttgttaaatgctcttagaattcctgcaataaagaacacctatctaaccttagttatccctgtgtttcccaaatatatcttactttggagcactttttttttagtaccgatttacatcctgggaaatggtgtttaccatgctttaaaaaaaactgtggtaaaataaagataagatttaccatcttaaccattttagagtgtacagttgagttggcatacagcattcacataacttaactgtgcaaccaatccacaggactttttatcttgcaaaactgaaacactatacccattaaacaactcctcatttcctcctcccccagtccttggcaactaccattctacttgtttctatgcatttgactgctctagatacttcacataaatggaagcatagagtatttgtcttccagtgactggcttacttcacttagcatcatgtcctcaagattcatccatgttgcagcacatgtcagcgtatcttccttttagaggctgaataatattccactgtatgaatataccacattttgttgatcattcacccactgatgggcacatattgcttccatctcttagctactgtgaataatggtgccgtgagtatgggcatacaaaaactaccactaatattttacagtgcttgcttcatatctgtccatgtgtccgtcactccacccatcatattttttatgtatttcataagttacagaccacagtaacttccctcaaacatgtcagtatacatatcaatgaccagcgttcattgtttttttccaagtcattttgaactgccgtagcaatgagtaatatagcctcaaacgcacacatacacacacaacacgtgcgtcactacagaaaacttttcctggcagacaggaaagggcccattgttggtgatgtcattttaattaagataaaaccaccaccaccatttagtaatagcctggggtaacaagggctgcgtcacggactgccacttttgccatcctgctcagagcagggccatgcctaacccgtatctggggattgcttcagatattatgaatcgcttcaatattatgaattactacaattcataataattgcttcagatattatgaattacaatatggttcaaaggtgctttagcagatgaagacacaaatgtgtaaacacatatgaattacaatgcagactgcccagatgtgtagcaagtcctctgaatgtttactaaacagtaaggtgattccagaggaagatgcttgaggacaatttgggaaaactgacaacttgaaaactcagtctctctaggcaaggcctacttgcagataaccttgggagttctgtgctgggaggaaagctaaaggactaagttaggcctctgaatctgctctggaagcctgcatgcacttgggtcagaacaagcccatgtgtcaatgtgggtaaagattcctcagctgataagcaggaaaatgggcagggcattttggtctttgaggttcaaagctcagatgctcactgccttggtatacacgcacacacaccccaccccccagctgacggcacaagagtatacagatgcaatagtctaaagtacattgtccaaatatggatggccatgagccacatgtggctatgaagcacttaaatgtggctagtctgaactgagatgggccctataaaatatttcagtaacaggtttttatactgattataggttgacataataatattttggatataccgtattaaaggaaatatgtcattaaatttcacctgtttcctttattatgtggctacttgaaaattttaaaattacatatgtagctcacactataaaacacagattagaaatattgtatagcactgacctagaaacctccatttaggtaaaacatcttaacccctttggaagcaaaatatgttaaataacagcataaactcccaccaagaaaatcctcaccttcctcctttcaacacatttattatatacagctgtcactgcattgtcaatctgccaaatggctctatgttccaacagggctggagtagtcccctgctcacaccagccttcacaatacttcccatgtcttccctgttaacctctctccacccagcacccaggctcccaactctcctggctgcctccagccctcagctggcaccactgacatgctgtttccagtacccttttcttctttctgcatcctccctgggggacatatatccctcatctcgtgacttcagctgtcacataaattcaaatgtttcagaactctattttttacctcctacatctgtcagtttaaatgtcaggatattttactttcagtaaagccctaaaaagacaaatctatgtacttttaaagaataaaagaaatgactggctgcagctcaaacctacaactgcttgcgaaactctacaatgtctggcagatgctagaaagaaggggatcaagacagagcacacttggcgtggtatgctatctatagaaaatgttaaaataaaattaagtaatctaggtttcctctctttattttctacatctactctctgaagagggcaataaataaggaaatgtcccaaagagggacaaattaagtcccaaaataacacaaaattgggcaaatccagtcatgaagaaagaacagaggttcttaaattgggacacacagaggcaggtctgcaggtctaggaatctctgaacatatgtgcaaaattctgggtatgtgtgcatatgttatataacaaagcgaagggtccatatagctttcatcgcatttcaaagggtctagcactgaaataaggactactgctatgtgacttaaaaaatgaaactcaggctgggcgcagtggctcacgcctgtaatcccagcactttgggaggccgaggcaagcagatcacctgagacgaggagtttgagacccgcctggccaacggtgaaacccagtctctactaaaaatacaaaaattagccggaattggtggtgtgcctctagtcccagctactcaggaggctgaagaaagagaatcgcttgaacctgggaggtggaggttgtgacaaagcaagactccatctcaaaaaaaaaaaaaacccagaaactcaattcagttatgaaggtaaagatgacctgtttacatgataatattttaagataccagtgactgcaagcatgtagttattaagtccattacagtgcacatttattgactctgtgtatcttcacagtgtgatcttcaccacagcttgcaaagtgtaaccactcagcaccttctgcttccttctgttcagtttttccactgcaattcttccagcataattttctgatagccagtgtatgactttggctttgacttgtttctacacagtgggtccagtcatttatttctggaacttgatcagtctttttccaggtatataagcaaatctttccacactccaatcctactgcaaccacgtatcgttgagaagggtggagcactgggcagacgctgacagctgtcacagccccacccacgtccaggactgaggagcaggggccaatgttgtgctcaatacagtcatcagtggagtcgcactcaccccagacaaccacctttttgtctcgactcccagtgaagaaatacttgctgtcaggactccaatcacaagaccaaataattctactgtgcacagaagtaattttgttggtgaaggcaaaaagactaaaaactggctcgaactcaggtgagattgtatcctgctttttccacaatgaccaggttcgatctctggaaacagctagtaagaacttctcattaggtgagaaggccatctgcgtgactgtcaaactgtggaaaactaaattctgcacctgtttccaagatgtagtgttccaaagaatgatagctgcatgctctttcttagctgccttacaagctgaggcaagcagagtctttgaactgttacaagtaacacaaaatatttcataaccgtgcccatatagtttttgaacttcaggccacaaagtattctgcagaagatgatcctcagtgggaggctcagtaagtatggagggctgaaaggccacctgctgatactcaaaaccagtactagttaacagctcctcttcatcagaaggctgagaagctatatctccctgaaagacagctttatttgataatcccaatgcagggacagtggctccttctggaagatcactatcttgattacagagcacatgattcagtgattgtcctgtaatggcacaaaaattttccacaaaattccgaggtgcagaaaaaacccgaagaactttttcatctgctccagatacaaactgaaaccgattaatcattgccaaacatttcaggtcatacccatgtatctgaggccttgcaatttcatgccaagtcacctgtgattggtcttttctcttccatggagcaaaaagtctagttgtctgatcagtaccaacagtgataataaattctccttctggatcccagactaggtcttggacaccatcaaagtgtcctgaaatgacaatctctggagtccactctcttgggttaactgtattctgtttccaaaggtgcaacgctccgtggaaagcatgagcaatgatcatggagccatcttcattgaactggcaatcataaaatcccaaagtattcccacctacttcacctactcgaacctgttctagccaaactcctgactcttcatctggagcccagagaatcatggttttatccatggaagcagataataatctcactggctgctgtaggacaccatctttgtaaaacacaggttgccagtgaactgcatttacccagttttcatgaccggctagcactgtctccagagtaacagcaaatgctattttaacactttcattttctatggtaaaagtattttctttcagtcttatgttatcgtcatcctgagtttctaaagatgttgactttatatacagcttccatattcttatcaggcaatcttgtgaacagcttgctaggaaaagatctctaccaaaggctgcccattccactcctctaatccaatcctcatgtccacagagagaaagcactttctgaaactgatcattttgttgagcaaatatgtgaattctgcaatcatcattgccacatgctaatattggtattggcctgaatgcagatggaagaaatgaaattctgttatgatgccagaatgtgtgcagcttctccttccacagagccttgcacagaatggaagcgtaacatgaaaccatagagtcgcagctcctgctacagagggcgagagaggctggtggcttccaggccctgcctcgttccacctggccagtcttccaggtaacatcagtatttggcaaaaaagataagcagagagccaaagcaaatccatttccaaagtttaaagtctgaaggcacattacttctggaccctttttagaccagagtcgaacagcagaatctgcagctgcagaaacgatcagtgtacataatgcaggatctgatgtcctcctctggtaaacagcatgcaccgcataaacaggtccttcatggccttgaagatgcactgcttttaaaagctgattatcctctatttcccagtgaatcacttgattatcagatcctccagaaactaattcagtagaaggggagccatcctgtttacaaatccactgtatgcaattgactcgggcggtgtgaccattcaagttggtaacaacaacccttttcagggggtcatagagcaccacggagcaggacgtgccaaaggccagaagtcctctgggcccagagctccagttcaggactccccgcacccggtttgggcagcaaaacacgtgagaagtctccagcacgggtgccaccatgtcgccaactggtcagccgcacaaacaagagacgc

SEQ ID NO: 13436 - RNA, 7206 nt, Homo sapiens
  source 1..7206: mol_type = other RNA
gctgggattacaggcatgagccaccacgcccggcccgggtcccagatctctgagtccaccagagtggggctcagagtcctctatccaccaaccacatgcagccatccaacacgctgtctctcttctggcctcagcctcattgtccttggagtgccagtctcttgtttaagcatggcagagccttaatactggaccatccactacatgctagaaggggaagaactcctcacaatgtaacaatttttgtatttaacttatggatatgctcattctttctaaacaattcttataaggaaattttaagtatattaaaaaattagaatagtatgaccaccccaacactgcccagcttcattaataatccacacatctaaaacccatctagtccttgacacacacacaatcattatgaaacaacccaagacataaattgatttcatccataaatactgaaattatgattcaagagaactttttttttttttttcttaaaccaaggctgaggtgggagaactgcttgagcccaggagttcaagaccagcttaggtaacactgcaaaacccagtctctagagaaaaaaaaaacaaaaccaatcataaccatagccccactgtcatatgtttaaatgttgtttccttaatatcatcaaatatccagccagagttcaaatttgctttgtcccttaagcacatttttacaagattgattggctagttcagatcaagaggcaaacaaggttcatacattgcactggattcacacgtctcaagtatctttcaatctccaggcttcccttcccttcccttttcctcttgtaatgtatttgttgaagaatctaggtccctctgtagtcactcctctccccattcccagcccctggtaaccacttacctgttttctgaccctataattttgtagggcccactttgtactgatgtacttctgactaggtgtgtttatgttcaagcatcagagccaaggcccaaacctctaccctggccctccttctgctgtggcccaactgtacccagagctgggctctcccgtctccctgcctgttaatcctagaagtgggtgccgaggagggagaaacaggaaggagggagttggggagggcagcttgttacatggacatcagggctgttcccactagcagcaacagctttgtgttagcttggctccaatttgaatgaaatattccaaggccattttccccaacacgttgttaccaaaaaaactcccagcatgcagaaaagttgaaagaattgtacagtgaacaccccttaaggagtttctaccattaacattttatttaaaggctttgggactctgaagtataatgtttgtgaaatgctatgagccagaccctccacactgaaaattcccagtgtaaattaatttgttaaatgctcttagaattcctgcaataaagaacacctatctaaccttagttatccctgtgtttcccaaatatatcttactttggagcactttttttttagtaccgatttacatcctgggaaatggtgtttaccatgctttaaaaaaaactgtggtaaaataaagataagatttaccatcttaaccattttagagtgtacagttgagttggcatacagcattcacataacttaactgtgcaaccaatccacaggactttttatcttgcaaaactgaaacactatacccattaaacaactcctcatttcctcctcccccagtccttggcaactaccattctacttgtttctatgcatttgactgctctagatacttcacataaatggaagcatagagtatttgtcttccagtgactggcttacttcacttagcatcatgtcctcaagattcatccatgttgcagcacatgtcagcgtatcttccttttagaggctgaataatattccactgtatgaatataccacattttgttgatcattcacccactgatgggcacatattgcttccatctcttagctactgtgaataatggtgccgtgagtatgggcatacaaaaactaccactaatattttacagtgcttgcttcatatctgtccatgtgtccgtcactccacccatcatattttttatgtatttcataagttacagaccacagtaacttccctcaaacatgtcagtatacatatcaatgaccagcgttcattgtttttttccaagtcattttgaactgccgtagcaatgagtaatatagcctcaaacgcacacatacacacacaacacgtgcgtcactacagaaaacttttcctggcagacaggaaagggcccattgttggtgatgtcattttaattaagataaaaccaccaccaccatttagtaatagcctggggtaacaagggctgcgtcacggactgccacttttgccatcctgctcagagcagggccatgcctaacccgtatctggggattgcttcagatattatgaatcgcttcaatattatgaattactacaattcataataattgcttcagatattatgaattacaatatggttcaaaggtgctttagcagatgaagacacaaatgtgtaaacacatatgaattacaatgcagactgcccagatgtgtagcaagtcctctgaatgtttactaaacagtaaggtgattccagaggaagatgcttgaggacaatttgggaaaactgacaacttgaaaactcagtctctctaggcaaggcctacttgcagataaccttgggagttctgtgctgggaggaaagctaaaggactaagttaggcctctgaatctgctctggaagcctgcatgcacttgggtcagaacaagcccatgtgtcaatgtgggtaaagattcctcagctgataagcaggaaaatgggcagggcattttggtctttgaggttcaaagctcagatgctcactgccttggtatacacgcacacacaccccaccccccagctgacggcacaagagtatacagatgcaatagtctaaagtacattgtccaaatatggatggccatgagccacatgtggctatgaagcacttaaatgtggctagtctgaactgagatgggccctataaaatatttcagtaacaggtttttatactgattataggttgacataataatattttggatataccgtattaaaggaaatatgtcattaaatttcacctgtttcctttattatgtggctacttgaaaattttaaaattacatatgtagctcacactataaaacacagattagaaatattgtatagcactgacctagaaacctccatttaggtaaaacatcttaacccctttggaagcaaaatatgttaaataacagcataaactcccaccaagaaaatcctcaccttcctcctttcaacacatttattatatacagctgtcactgcattgtcaatctgccaaatggctctatgttccaacagggctggagtagtcccctgctcacaccagccttcacaatacttcccatgtcttccctgttaacctctctccacccagcacccaggctcccaactctcctggctgcctccagccctcagctggcaccactgacatgctgtttccagtacccttttcttctttctgcatcctccctgggggacatatatccctcatctcgtgacttcagctgtcacataaattcaaatgtttcagaactctattttttacctcctacatctgtcagtttaaatgtcaggatattttactttcagtaaagccctaaaaagacaaatctatgtacttttaaagaataaaagaaatgactggctgcagctcaaacctacaactgcttgcgaaactctacaatgtctggcagatgctagaaagaaggggatcaagacagagcacacttggcgtggtatgctatctatagaaaatgttaaaataaaattaagtaatctaggtttcctctctttattttctacatctactctctgaagagggcaataaataaggaaatgtcccaaagagggacaaattaagtcccaaaataacacaaaattgggcaaatccagtcatgaagaaagaacagaggttcttaaattgggacacacagaggcaggtctgcaggtctaggaatctctgaacatatgtgcaaaattctgggtatgtgtgcatatgttatataacaaagcgaagggtccatatagctttcatcgcatttcaaagggtctagcactgaaataaggactactgctatgtgacttaaaaaatgaaactcaggctgggcgcagtggctcacgcctgtaatcccagcactttgggaggccgaggcaagcagatcacctgagacgaggagtttgagacccgcctggccaacggtgaaacccagtctctactaaaaatacaaaaattagccggaattggtggtgtgcctctagtcccagctactcaggaggctgaagaaagagaatcgcttgaacctgggaggtggaggttgtgacaaagcaagactccatctcaaaaaaaaaaaaaacccagaaactcaattcagttatgaaggtaaagatgacctgtttacatgataatattttaagataccagtgactgcaagcatgtagttattaagtccattacagtgcacatttattgactctgtgtatcttcacagtgtgatcttcaccacagcttgcaaagtgtaaccactcagcaccttctgcttccttctgttcagtttttccactgcaattcttccagcataattttctgatagccagtgtatgactttggctttgacttgtttctacacagtgggtccagtcatttatttctggaacttgatcagtctttttccaggtatataagcaaatctttccacactccaatcctactgcaaccacgtatcgttgagaagggtggagcactgggcagacgctgacagctgtcacagccccacccacgtccaggactgaggagcaggggccaatgttgtgctcaatacagtcatcagtggagtcgcactcaccccagacaaccacctttttgtctcgactcccagtgaagaaatacttgctgtcaggactccaatcacaagaccaaataattctactgtgcacagaagtaattttgttggtgaaggcaaaaagactaaaaactggctcgaactcaggtgagattgtatcctgctttttccacaatgaccaggttcgatctctggaaacagctagtaagaacttctcattaggtgagaaggccatctgcgtgactgtcaaactgtggaaaactaaattctgcacctgtttccaagatgtagtgttccaaagaatgatagctgcatgctctttcttagctgccttacaagctgaggcaagcagagtctttgaactgttacaagtaacacaaaatatttcataaccgtgcccatatagtttttgaacttcaggccacaaagtattctgcagaagatgatcctcagtgggaggctcagtaagtatggagggctgaaaggccacctgctgatactcaaaaccagtactagttaacagctcctcttcatcagaaggctgagaagctatatctccctgaaagacagctttatttgataatcccaatgcagggacagtggctccttctggaagatcactatcttgattacagagcacatgattcagtgattgtcctgtaatggcacaaaaattttccacaaaattccgaggtgcagaaaaaacccgaagaactttttcatctgctccagatacaaactgaaaccgattaatcattgccaaacatttcaggtcatacccatgtatctgaggccttgcaatttcatgccaagtcacctgtgattggtcttttctcttccatggagcaaaaagtctagttgtctgatcagtaccaacagtgataataaattctccttctggatcccagactaggtcttggacaccatcaaagtgtcctgaaatgacaatctctggagtccactctcttgggttaactgtattctgtttccaaaggtgcaacgctccgtggaaagcatgagcaatgatcatggagccatcttcattgaactggcaatcataaaatcccaaagtattcccacctacttcacctactcgaacctgttctagccaaactcctgactcttcatctggagcccagagaatcatggttttatccatggaagcagataataatctcactggctgctgtaggacaccatctttgtaaaacacaggttgccagtgaactgcatttacccagttttcatgaccggctagcactgtctccagagtaacagcaaatgctattttaacactttcattttctatggtaaaagtattttctttcagtcttatgttatcgtcatcctgagtttctaaagatgttgactttatatacagcttccatattcttatcaggcaatcttgtgaacagcttgctaggaaaagatctctaccaaaggctgcccattccactcctctaatccaatcctcatgtccacagagagaaagcactttctgaaactgatcattttgttgagcaaatatgtgaattctgcaatcatcattgccacatgctaatattggtattggcctgaatgcagatggaagaaatgaaattctgttatgatgccagaatgtgtgcagcttctccttccacagagccttgcacagaatggaagcgtaacatgaaaccatagagtcgcagctcctgctacagagggcgagagaggctggtggcttccaggccctgcctcgttccacctggccagtcttccaggtaacttctggaccctttttagaccagagtcgaacagcagaatctgcagctgcagaaacgatcagtgtacataatgcaggatctgatgtcctcctctggtaaacagcatgcaccgcataaacaggtccttcatggccttgaagatgcactgcttttaaaagctgattatcctctatttcccagtgaatcacttgattatcagatcctccagaaactaattcagtagaaggggagccatcctgtttacaaatccactgtatgcaattgactcgggcggtgtgaccattcaagttggtaacaacaacccttttcagggggtcatagagcaccacggagcaggacgtgccaaaggccagaagtcctctgggcccagagctccagttcaggactccccgcacccggtttgggcagcaaaacacgtgagaagtctccagcacgggtgccaccatgtcgccaactggtcagccgcacaaacaagagacgc

SEQ ID NO: 13437 - RNA, 6879 nt, Homo sapiens
  source 1..6879: mol_type = other RNA
gctgggattacaggcatgagccaccacgcccggcccgggtcccagatctctgagtccaccagagtggggctcagagtcctctatccaccaaccacatgcagccatccaacacgctgtctctcttctggcctcagcctcattgtccttggagtgccagtctcttgtttaagcatggcagagccttaatactggaccatccactacatgctagaaggggaagaactcctcacaatgtaacaatttttgtatttaacttatggatatgctcattctttctaaacaattcttataaggaaattttaagtatattaaaaaattagaatagtatgaccaccccaacactgcccagcttcattaataatccacacatctaaaacccatctagtccttgacacacacacaatcattatgaaacaacccaagacataaattgatttcatccataaatactgaaattatgattcaagagaactttttttttttttttcttaaaccaaggctgaggtgggagaactgcttgagcccaggagttcaagaccagcttaggtaacactgcaaaacccagtctctagagaaaaaaaaaacaaaaccaatcataaccatagccccactgtcatatgtttaaatgttgtttccttaatatcatcaaatatccagccagagttcaaatttgctttgtcccttaagcacatttttacaagattgattggctagttcagatcaagaggcaaacaaggttcatacattgcactggattcacacgtctcaagtatctttcaatctccaggcttcccttcccttcccttttcctcttgtaatgtatttgttgaagaatctaggtccctctgtagtcactcctctccccattcccagcccctggtaaccacttacctgttttctgaccctataattttgtagggcccactttgtactgatgtacttctgactaggtgtgtttatgttcaagcatcagagccaaggcccaaacctctaccctggccctccttctgctgtggcccaactgtacccagagctgggctctcccgtctccctgcctgttaatcctagaagtgggtgccgaggagggagaaacaggaaggagggagttggggagggcagcttgttacatggacatcagggctgttcccactagcagcaacagctttgtgttagcttggctccaatttgaatgaaatattccaaggccattttccccaacacgttgttaccaaaaaaactcccagcatgcagaaaagttgaaagaattgtacagtgaacaccccttaaggagtttctaccattaacattttatttaaaggctttgggactctgaagtataatgtttgtgaaatgctatgagccagaccctccacactgaaaattcccagtgtaaattaatttgttaaatgctcttagaattcctgcaataaagaacacctatctaaccttagttatccctgtgtttcccaaatatatcttactttggagcactttttttttagtaccgatttacatcctgggaaatggtgtttaccatgctttaaaaaaaactgtggtaaaataaagataagatttaccatcttaaccattttagagtgtacagttgagttggcatacagcattcacataacttaactgtgcaaccaatccacaggactttttatcttgcaaaactgaaacactatacccattaaacaactcctcatttcctcctcccccagtccttggcaactaccattctacttgtttctatgcatttgactgctctagatacttcacataaatggaagcatagagtatttgtcttccagtgactggcttacttcacttagcatcatgtcctcaagattcatccatgttgcagcacatgtcagcgtatcttccttttagaggctgaataatattccactgtatgaatataccacattttgttgatcattcacccactgatgggcacatattgcttccatctcttagctactgtgaataatggtgccgtgagtatgggcatacaaaaactaccactaatattttacagtgcttgcttcatatctgtccatgtgtccgtcactccacccatcatattttttatgtatttcataagttacagaccacagtaacttccctcaaacatgtcagtatacatatcaatgaccagcgttcattgtttttttccaagtcattttgaactgccgtagcaatgagtaatatagcctcaaacgcacacatacacacacaacacgtgcgtcactacagaaaacttttcctggcagacaggaaagggcccattgttggtgatgtcattttaattaagataaaaccaccaccaccatttagtaatagcctggggtaacaagggctgcgtcacggactgccacttttgccatcctgctcagagcagggccatgcctaacccgtatctggggattgcttcagatattatgaatcgcttcaatattatgaattactacaattcataataattgcttcagatattatgaattacaatatggttcaaaggtgctttagcagatgaagacacaaatgtgtaaacacatatgaattacaatgcagactgcccagatgtgtagcaagtcctctgaatgtttactaaacagtaaggtgattccagaggaagatgcttgaggacaatttgggaaaactgacaacttgaaaactcagtctctctaggcaaggcctacttgcagataaccttgggagttctgtgctgggaggaaagctaaaggactaagttaggcctctgaatctgctctggaagcctgcatgcacttgggtcagaacaagcccatgtgtcaatgtgggtaaagattcctcagctgataagcaggaaaatgggcagggcattttggtctttgaggttcaaagctcagatgctcactgccttggtatacacgcacacacaccccaccccccagctgacggcacaagagtatacagatgcaatagtctaaagtacattgtccaaatatggatggccatgagccacatgtggctatgaagcacttaaatgtggctagtctgaactgagatgggccctataaaatatttcagtaacaggtttttatactgattataggttgacataataatattttggatataccgtattaaaggaaatatgtcattaaatttcacctgtttcctttattatgtggctacttgaaaattttaaaattacatatgtagctcacactataaaacacagattagaaatattgtatagcactgacctagaaacctccatttaggtaaaacatcttaacccctttggaagcaaaatatgttaaataacagcataaactcccaccaagaaaatcctcaccttcctcctttcaacacatttattatatacagctgtcactgcattgtcaatctgccaaatggctctatgttccaacagggctggagtagtcccctgctcacaccagccttcacaatacttcccatgtcttccctgttaacctctctccacccagcacccaggctcccaactctcctggctgcctccagccctcagctggcaccactgacatgctgtttccagtacccttttcttctttctgcatcctccctgggggacatatatccctcatctcgtgacttcagctgtcacataaattcaaatgtttcagaactctattttttacctcctacatctgtcagtttaaatgtcaggatattttactttcagtaaagccctaaaaagacaaatctatgtacttttaaagaataaaagaaatgactggctgcagctcaaacctacaactgcttgcgaaactctacaatgtctggcagatgctagaaagaaggggatcaagacagagcacacttggcgtggtatgctatctatagaaaatgttaaaataaaattaagtaatctaggtttcctctctttattttctacatctactctctgaagagggcaataaataaggaaatgtcccaaagagggacaaattaagtcccaaaataacacaaaattgggcaaatccagtcatgaagaaagaacagaggttcttaaattgggacacacagaggcaggtctgcaggtctaggaatctctgaacatatgtgcaaaattctgggtatgtgtgcatatgttatataacaaagcgaagggtccatatagctttcatcgcatttcaaagggtctagcactgaaataaggactactgctatgtgacttaaaaaatgaaactcaggctgggcgcagtggctcacgcctgtaatcccagcactttgggaggccgaggcaagcagatcacctgagacgaggagtttgagacccgcctggccaacggtgaaacccagtctctactaaaaatacaaaaattagccggaattggtggtgtgcctctagtcccagctactcaggaggctgaagaaagagaatcgcttgaacctgggaggtggaggttgtgacaaagcaagactccatctcaaaaaaaaaaaaaacccagaaactcaattcagttatgaaggtaaagatgacctgtttacatgataatattttaagataccagtgactgcaagcatgtagttattaagtccattacagtgcacatttattgactctgtgtatcttcacagtgtgatcttcaccacagcttgcaaagtgtaaccactcagcaccttctgcttccttctgttcagtttttccactgcaattcttccagcataattttctgatagccagtgtatgactttggctttgacttgtttctacacagtgggtccagtcatttatttctggaacttgatcagtctttttccaggtatataagcaaatctttccacactccaatcctactgcaaccacgtatcgttgagaagggtggagcactgggcagacgctgacagctgtcacagccccacccacgtccaggactgaggagcaggggccaatgttgtgctcaatacagtcatcagtggagtcgcactcaccccagacaaccacctttttgtctcgactcccagtgaagaaatacttgctgtcaggactccaatcacaagaccaaataattctactgtgcacagaagtaattttgttggtgaaggcaaaaagactaaaaactggctcgaactcaggtgagattgtatcctgctttttccacaatgaccaggttcgatctctggaaacagctagtaagaacttctcattaggtgagaaggccatctgcgtgactgtcaaactgtggaaaactaaattctgcacctgtttccaagatgtagtgttccaaagaatgatagctgcatgctctttcttagctgccttacaagctgaggcaagcagagtctttgaactgttacaagtaacacaaaatatttcataaccgtgcccatatagtttttgaacttcaggccacaaagtattctgcagaagatgatcctcagtgggaggctcagtaagtatggagggctgaaaggccacctgctgatactcaaaaccagtactagttaacagctcctcttcatcagaaggctgagaagctatatctccctgaaagacagctttatttgataatcccaatgcagggacagtggctccttctggaagatcactatcttgattacagagcacatgattcagtgattgtcctgtaatggcacaaaaattttccacaaaattccgaggtgcagaaaaaacccgaagaactttttcatctgctccagatacaaactgaaaccgattaatcattgccaaacatttcaggtcatacccatgtatctgaggccttgcaatttcatgccaagtcacctgtgattggtcttttctcttccatggagcaaaaagtctagttgtctgatcagtaccaacagtgataataaattctccttctggatcccagactaggtcttggacaccatcaaagtgtcctgaaatgacaatctctggagtccactctcttgggttaactgtattctgtttccaaaggtgcaacgctccgtggaaagcatgagcaatgatcatggagccatcttcattgaactggcaatcataaaatcccaaagtattcccacctacttcacctactcgaacctgttctagccaaactcctgactcttcatctggagcccagagaatcatggttttatccatggaagcagataataatctcactggctgctgtaggacaccatctttgtaaaacacaggttgccagtgaactgcatttacccagttttcatgaccggctagcactgtctccagagtaacagcaaatgctattttaacactttcattttctatggtaaaagtattttctttcagtcttatgttatcgtcatcctgagtttctaaagatgttgactttatatacagcttccatattcttatcaggcaatcttgtgaacagcttgctaggaaaagatctctaccttctggaccctttttagaccagagtcgaacagcagaatctgcagctgcagaaacgatcagtgtacataatgcaggatctgatgtcctcctctggtaaacagcatgcaccgcataaacaggtccttcatggccttgaagatgcactgcttttaaaagctgattatcctctatttcccagtgaatcacttgattatcagatcctccagaaactaattcagtagaaggggagccatcctgtttacaaatccactgtatgcaattgactcgggcggtgtgaccattcaagttggtaacaacaacccttttcagggggtcatagagcaccacggagcaggacgtgccaaaggccagaagtcctctgggcccagagctccagttcaggactccccgcacccggtttgggcagcaaaacacgtgagaagtctccagcacgggtgccaccatgtcgccaactggtcagccgcacaaacaagagacgc

SEQ ID NO: 13438 - RNA, 6939 nt, Homo sapiens
  source 1..6939: mol_type = other RNA
gctgggattacaggcatgagccaccacgcccggcccgggtcccagatctctgagtccaccagagtggggctcagagtcctctatccaccaaccacatgcagccatccaacacgctgtctctcttctggcctcagcctcattgtccttggagtgccagtctcttgtttaagcatggcagagccttaatactggaccatccactacatgctagaaggggaagaactcctcacaatgtaacaatttttgtatttaacttatggatatgctcattctttctaaacaattcttataaggaaattttaagtatattaaaaaattagaatagtatgaccaccccaacactgcccagcttcattaataatccacacatctaaaacccatctagtccttgacacacacacaatcattatgaaacaacccaagacataaattgatttcatccataaatactgaaattatgattcaagagaactttttttttttttttcttaaaccaaggctgaggtgggagaactgcttgagcccaggagttcaagaccagcttaggtaacactgcaaaacccagtctctagagaaaaaaaaaacaaaaccaatcataaccatagccccactgtcatatgtttaaatgttgtttccttaatatcatcaaatatccagccagagttcaaatttgctttgtcccttaagcacatttttacaagattgattggctagttcagatcaagaggcaaacaaggttcatacattgcactggattcacacgtctcaagtatctttcaatctccaggcttcccttcccttcccttttcctcttgtaatgtatttgttgaagaatctaggtccctctgtagtcactcctctccccattcccagcccctggtaaccacttacctgttttctgaccctataattttgtagggcccactttgtactgatgtacttctgactaggtgtgtttatgttcaagcatcagagccaaggcccaaacctctaccctggccctccttctgctgtggcccaactgtacccagagctgggctctcccgtctccctgcctgttaatcctagaagtgggtgccgaggagggagaaacaggaaggagggagttggggagggcagcttgttacatggacatcagggctgttcccactagcagcaacagctttgtgttagcttggctccaatttgaatgaaatattccaaggccattttccccaacacgttgttaccaaaaaaactcccagcatgcagaaaagttgaaagaattgtacagtgaacaccccttaaggagtttctaccattaacattttatttaaaggctttgggactctgaagtataatgtttgtgaaatgctatgagccagaccctccacactgaaaattcccagtgtaaattaatttgttaaatgctcttagaattcctgcaataaagaacacctatctaaccttagttatccctgtgtttcccaaatatatcttactttggagcactttttttttagtaccgatttacatcctgggaaatggtgtttaccatgctttaaaaaaaactgtggtaaaataaagataagatttaccatcttaaccattttagagtgtacagttgagttggcatacagcattcacataacttaactgtgcaaccaatccacaggactttttatcttgcaaaactgaaacactatacccattaaacaactcctcatttcctcctcccccagtccttggcaactaccattctacttgtttctatgcatttgactgctctagatacttcacataaatggaagcatagagtatttgtcttccagtgactggcttacttcacttagcatcatgtcctcaagattcatccatgttgcagcacatgtcagcgtatcttccttttagaggctgaataatattccactgtatgaatataccacattttgttgatcattcacccactgatgggcacatattgcttccatctcttagctactgtgaataatggtgccgtgagtatgggcatacaaaaactaccactaatattttacagtgcttgcttcatatctgtccatgtgtccgtcactccacccatcatattttttatgtatttcataagttacagaccacagtaacttccctcaaacatgtcagtatacatatcaatgaccagcgttcattgtttttttccaagtcattttgaactgccgtagcaatgagtaatatagcctcaaacgcacacatacacacacaacacgtgcgtcactacagaaaacttttcctggcagacaggaaagggcccattgttggtgatgtcattttaattaagataaaaccaccaccaccatttagtaatagcctggggtaacaagggctgcgtcacggactgccacttttgccatcctgctcagagcagggccatgcctaacccgtatctggggattgcttcagatattatgaatcgcttcaatattatgaattactacaattcataataattgcttcagatattatgaattacaatatggttcaaaggtgctttagcagatgaagacacaaatgtgtaaacacatatgaattacaatgcagactgcccagatgtgtagcaagtcctctgaatgtttactaaacagtaaggtgattccagaggaagatgcttgaggacaatttgggaaaactgacaacttgaaaactcagtctctctaggcaaggcctacttgcagataaccttgggagttctgtgctgggaggaaagctaaaggactaagttaggcctctgaatctgctctggaagcctgcatgcacttgggtcagaacaagcccatgtgtcaatgtgggtaaagattcctcagctgataagcaggaaaatgggcagggcattttggtctttgaggttcaaagctcagatgctcactgccttggtatacacgcacacacaccccaccccccagctgacggcacaagagtatacagatgcaatagtctaaagtacattgtccaaatatggatggccatgagccacatgtggctatgaagcacttaaatgtggctagtctgaactgagatgggccctataaaatatttcagtaacaggtttttatactgattataggttgacataataatattttggatataccgtattaaaggaaatatgtcattaaatttcacctgtttcctttattatgtggctacttgaaaattttaaaattacatatgtagctcacactataaaacacagattagaaatattgtatagcactgacctagaaacctccatttaggtaaaacatcttaacccctttggaagcaaaatatgttaaataacagcataaactcccaccaagaaaatcctcaccttcctcctttcaacacatttattatatacagctgtcactgcattgtcaatctgccaaatggctctatgttccaacagggctggagtagtcccctgctcacaccagccttcacaatacttcccatgtcttccctgttaacctctctccacccagcacccaggctcccaactctcctggctgcctccagccctcagctggcaccactgacatgctgtttccagtacccttttcttctttctgcatcctccctgggggacatatatccctcatctcgtgacttcagctgtcacataaattcaaatgtttcagaactctattttttacctcctacatctgtcagtttaaatgtcaggatattttactttcagtaaagccctaaaaagacaaatctatgtacttttaaagaataaaagaaatgactggctgcagctcaaacctacaactgcttgcgaaactctacaatgtctggcagatgctagaaagaaggggatcaagacagagcacacttggcgtggtatgctatctatagaaaatgttaaaataaaattaagtaatctaggtttcctctctttattttctacatctactctctgaagagggcaataaataaggaaatgtcccaaagagggacaaattaagtcccaaaataacacaaaattgggcaaatccagtcatgaagaaagaacagaggttcttaaattgggacacacagaggcaggtctgcaggtctaggaatctctgaacatatgtgcaaaattctgggtatgtgtgcatatgttatataacaaagcgaagggtccatatagctttcatcgcatttcaaagggtctagcactgaaataaggactactgctatgtgacttaaaaaatgaaactcaggctgggcgcagtggctcacgcctgtaatcccagcactttgggaggccgaggcaagcagatcacctgagacgaggagtttgagacccgcctggccaacggtgaaacccagtctctactaaaaatacaaaaattagccggaattggtggtgtgcctctagtcccagctactcaggaggctgaagaaagagaatcgcttgaacctgggaggtggaggttgtgacaaagcaagactccatctcaaaaaaaaaaaaaacccagaaactcaattcagttatgaaggtaaagatgacctgtttacatgataatattttaagataccagtgactgcaagcatgtagttattaagtccattacagtgcacatttattgactctgtgtatcttcacagtgtgatcttcaccacagcttgcaaagtgtaaccactcagcaccttctgcttccttctgttcagtttttccactgcaattcttccagcataattttctgatagccagtgtatgactttggctttgacttgtttctacacagtgggtccagtcatttatttctggaacttgatcagtctttttccaggtatataagcaaatctttccacactccaatcctactgcaaccacgtatcgttgagaagggtggagcactgggcagacgctgacagctgtcacagccccacccacgtccaggactgaggagcaggggccaatgttgtgctcaatacagtcatcagtggagtcgcactcaccccagacaaccacctttttgtctcgactcccagtgaagaaatacttgctgtcaggactccaatcacaagaccaaataattctactgtgcacagaagtaattttgttggtgaaggcaaaaagactaaaaactggctcgaactcaggtgagattgtatcctgctttttccacaatgaccaggttcgatctctggaaacagctagtaagaacttctcattaggtgagaaggccatctgcgtgactgtcaaactgtggaaaactaaattctgcacctgtttccaagatgtagtgttccaaagaatgatagctgcatgctctttcttagctgccttacaagctgaggcaagcagagtctttgaactgttacaagtaacacaaaatatttcataaccgtgcccatatagtttttgaacttcaggccacaaagtattctgcagaagatgatcctcagtgggaggctcagtaagtatggagggctgaaaggccacctgctgatactcaaaaccagtactagttaacagctcctcttcatcagaaggctgagaagctatatctccctgaaagacagctttatttgataatcccaatgcagggacagtggctccttctggaagatcactatcttgattacagagcacatgattcagtgattgtcctgtaatggcacaaaaattttccacaaaattccgaggtgcagaaaaaacccgaagaactttttcatctgctccagatacaaactgaaaccgattaatcattgccaaacatttcaggtcatacccatgtatctgaggccttgcaatttcatgccaagtcactgggttaactgtattctgtttccaaaggtgcaacgctccgtggaaagcatgagcaatgatcatggagccatcttcattgaactggcaatcataaaatcccaaagtattcccacctacttcacctactcgaacctgttctagccaaactcctgactcttcatctggagcccagagaatcatggttttatccatggaagcagataataatctcactggctgctgtaggacaccatctttgtaaaacacaggttgccagtgaactgcatttacccagttttcatgaccggctagcactgtctccagagtaacagcaaatgctattttaacactttcattttctatggtaaaagtattttctttcagtcttatgttatcgtcatcctgagtttctaaagatgttgactttatatacagcttccatattcttatcaggcaatcttgtgaacagcttgctaggaaaagatctctaccaaaggctgcccattccactcctctaatccaatcctcatgtccacagagagaaagcactttctgaaactgatcattttgttgagcaaatatgtgaattctgcaatcatcattgccacatgctaatattggtacatcagtatttggcaaaaaagataagcagagagccaaagcaaatccatttccaaagtttaaagtctgaaggcacattacttctggaccctttttagaccagagtcgaacagcagaatctgcagctgcagaaacgatcagtgtacataatgcaggatctgatgtcctcctctggtaaacagcatgcaccgcataaacaggtccttcatggccttgaagatgcactgcttttaaaagctgattatcctctatttcccagtgaatcacttgattatcagatcctccagaaactaattcagtagaaggggagccatcctgtttacaaatccactgtatgcaattgactcgggcggtgtgaccattcaagttggtaacaacaacccttttcagggggtcatagagcaccacggagcaggacgtgccaaaggccagaagtcctctgggcccagagctccagttcaggactccccgcacccggtttgggcagcaaaacacgtgagaagtctccagcacgggtgccaccatgtcgccaactggtcagccgcacaaacaagagacgc

SEQ ID NO: 13439 - RNA, 6955 nt, Homo sapiens
  source 1..6955: mol_type = other RNA
gctgggattacaggcatgagccaccacgcccggcccgggtcccagatctctgagtccaccagagtggggctcagagtcctctatccaccaaccacatgcagccatccaacacgctgtctctcttctggcctcagcctcattgtccttggagtgccagtctcttgtttaagcatggcagagccttaatactggaccatccactacatgctagaaggggaagaactcctcacaatgtaacaatttttgtatttaacttatggatatgctcattctttctaaacaattcttataaggaaattttaagtatattaaaaaattagaatagtatgaccaccccaacactgcccagcttcattaataatccacacatctaaaacccatctagtccttgacacacacacaatcattatgaaacaacccaagacataaattgatttcatccataaatactgaaattatgattcaagagaactttttttttttttttcttaaaccaaggctgaggtgggagaactgcttgagcccaggagttcaagaccagcttaggtaacactgcaaaacccagtctctagagaaaaaaaaaacaaaaccaatcataaccatagccccactgtcatatgtttaaatgttgtttccttaatatcatcaaatatccagccagagttcaaatttgctttgtcccttaagcacatttttacaagattgattggctagttcagatcaagaggcaaacaaggttcatacattgcactggattcacacgtctcaagtatctttcaatctccaggcttcccttcccttcccttttcctcttgtaatgtatttgttgaagaatctaggtccctctgtagtcactcctctccccattcccagcccctggtaaccacttacctgttttctgaccctataattttgtagggcccactttgtactgatgtacttctgactaggtgtgtttatgttcaagcatcagagccaaggcccaaacctctaccctggccctccttctgctgtggcccaactgtacccagagctgggctctcccgtctccctgcctgttaatcctagaagtgggtgccgaggagggagaaacaggaaggagggagttggggagggcagcttgttacatggacatcagggctgttcccactagcagcaacagctttgtgttagcttggctccaatttgaatgaaatattccaaggccattttccccaacacgttgttaccaaaaaaactcccagcatgcagaaaagttgaaagaattgtacagtgaacaccccttaaggagtttctaccattaacattttatttaaaggctttgggactctgaagtataatgtttgtgaaatgctatgagccagaccctccacactgaaaattcccagtgtaaattaatttgttaaatgctcttagaattcctgcaataaagaacacctatctaaccttagttatccctgtgtttcccaaatatatcttactttggagcactttttttttagtaccgatttacatcctgggaaatggtgtttaccatgctttaaaaaaaactgtggtaaaataaagataagatttaccatcttaaccattttagagtgtacagttgagttggcatacagcattcacataacttaactgtgcaaccaatccacaggactttttatcttgcaaaactgaaacactatacccattaaacaactcctcatttcctcctcccccagtccttggcaactaccattctacttgtttctatgcatttgactgctctagatacttcacataaatggaagcatagagtatttgtcttccagtgactggcttacttcacttagcatcatgtcctcaagattcatccatgttgcagcacatgtcagcgtatcttccttttagaggctgaataatattccactgtatgaatataccacattttgttgatcattcacccactgatgggcacatattgcttccatctcttagctactgtgaataatggtgccgtgagtatgggcatacaaaaactaccactaatattttacagtgcttgcttcatatctgtccatgtgtccgtcactccacccatcatattttttatgtatttcataagttacagaccacagtaacttccctcaaacatgtcagtatacatatcaatgaccagcgttcattgtttttttccaagtcattttgaactgccgtagcaatgagtaatatagcctcaaacgcacacatacacacacaacacgtgcgtcactacagaaaacttttcctggcagacaggaaagggcccattgttggtgatgtcattttaattaagataaaaccaccaccaccatttagtaatagcctggggtaacaagggctgcgtcacggactgccacttttgccatcctgctcagagcagggccatgcctaacccgtatctggggattgcttcagatattatgaatcgcttcaatattatgaattactacaattcataataattgcttcagatattatgaattacaatatggttcaaaggtgctttagcagatgaagacacaaatgtgtaaacacatatgaattacaatgcagactgcccagatgtgtagcaagtcctctgaatgtttactaaacagtaaggtgattccagaggaagatgcttgaggacaatttgggaaaactgacaacttgaaaactcagtctctctaggcaaggcctacttgcagataaccttgggagttctgtgctgggaggaaagctaaaggactaagttaggcctctgaatctgctctggaagcctgcatgcacttgggtcagaacaagcccatgtgtcaatgtgggtaaagattcctcagctgataagcaggaaaatgggcagggcattttggtctttgaggttcaaagctcagatgctcactgccttggtatacacgcacacacaccccaccccccagctgacggcacaagagtatacagatgcaatagtctaaagtacattgtccaaatatggatggccatgagccacatgtggctatgaagcacttaaatgtggctagtctgaactgagatgggccctataaaatatttcagtaacaggtttttatactgattataggttgacataataatattttggatataccgtattaaaggaaatatgtcattaaatttcacctgtttcctttattatgtggctacttgaaaattttaaaattacatatgtagctcacactataaaacacagattagaaatattgtatagcactgacctagaaacctccatttaggtaaaacatcttaacccctttggaagcaaaatatgttaaataacagcataaactcccaccaagaaaatcctcaccttcctcctttcaacacatttattatatacagctgtcactgcattgtcaatctgccaaatggctctatgttccaacagggctggagtagtcccctgctcacaccagccttcacaatacttcccatgtcttccctgttaacctctctccacccagcacccaggctcccaactctcctggctgcctccagccctcagctggcaccactgacatgctgtttccagtacccttttcttctttctgcatcctccctgggggacatatatccctcatctcgtgacttcagctgtcacataaattcaaatgtttcagaactctattttttacctcctacatctgtcagtttaaatgtcaggatattttactttcagtaaagccctaaaaagacaaatctatgtacttttaaagaataaaagaaatgactggctgcagctcaaacctacaactgcttgcgaaactctacaatgtctggcagatgctagaaagaaggggatcaagacagagcacacttggcgtggtatgctatctatagaaaatgttaaaataaaattaagtaatctaggtttcctctctttattttctacatctactctctgaagagggcaataaataaggaaatgtcccaaagagggacaaattaagtcccaaaataacacaaaattgggcaaatccagtcatgaagaaagaacagaggttcttaaattgggacacacagaggcaggtctgcaggtctaggaatctctgaacatatgtgcaaaattctgggtatgtgtgcatatgttatataacaaagcgaagggtccatatagctttcatcgcatttcaaagggtctagcactgaaataaggactactgctatgtgacttaaaaaatgaaactcaggctgggcgcagtggctcacgcctgtaatcccagcactttgggaggccgaggcaagcagatcacctgagacgaggagtttgagacccgcctggccaacggtgaaacccagtctctactaaaaatacaaaaattagccggaattggtggtgtgcctctagtcccagctactcaggaggctgaagaaagagaatcgcttgaacctgggaggtggaggttgtgacaaagcaagactccatctcaaaaaaaaaaaaaacccagaaactcaattcagttatgaaggtaaagatgacctgtttacatgataatattttaagataccagtgactgcaagcatgtagttattaagtccattacagtgcacatttattgactctgtgtatcttcacagtgtgatcttcaccacagcttgcaaagtgtaaccactcagcaccttctgcttccttctgttcagtttttccactgcaattcttccagcataattttctgatagccagtgtatgactttggctttgacttgtttctacacagtgggtccagtcatttatttctggaacttgatcagtctttttccaggtatataagcaaatctttccacactccaatcctactgcaaccacgtatctttttgtctcgactcccagtgaagaaatacttgctgtcaggactccaatcacaagaccaaataattctactgtgcacagaagtaattttgttggtgaaggcaaaaagactaaaaactggctcgaactcaggtgagattgtatcctgctttttccacaatgaccaggttcgatctctggaaacagctagtaagaacttctcattaggtgagaaggccatctgcgtgactgtcaaactgtggaaaactaaattctgcacctgtttccaagatgtagtgttccaaagaatgatagctgcatgctctttcttagctgccttacaagctgaggcaagcagagtctttgaactgttacaagtaacacaaaatatttcataaccgtgcccatatagtttttgaacttcaggccacaaagtattctgcagaagatgatcctcagtgggaggctcagtaagtatggagggctgaaaggccacctgctgatactcaaaaccagtactagttaacagctcctcttcatcagaaggctgagaagctatatctccctgaaagacagctttatttgataatcccaatgcagggacagtggctccttctggaagatcactatcttgattacagagcacatgattcagtgattgtcctgtaatggcacaaaaattttccacaaaattccgaggtgcagaaaaaacccgaagaactttttcatctgctccagatacaaactgaaaccgattaatcattgccaaacatttcaggtcatacccatgtatctgaggccttgcaatttcatgccaagtcacctgtgattggtcttttctcttccatggagcaaaaagtctagttgtctgatcagtaccaacagtgataataaattctccttctggatcccagactaggtcttggacaccatcaaagtgtcctgaaatgacaatctctggagtccactctcttgggttaactgtattctgtttccaaaggtgcaacgctccgtggaaagcatgagcaatgatcatggagccatcttcattgaactggcaatcataaaatcccaaagtattcccacctacttcacctactcgaacctgttctagccaaactcctgactcttcatctggagcccagagaatcatggttttatccatggaagcagataataatctcactggctgctgtaggacaccatctttgtaaaacacaggttgccagtgaactgcatttacccagttttcatgaccggctagcactgtctccagagtaacagcaaatgctattttaacactttcattttctatggtaaaagtattttctttcagtcttatgttatcgtcatcctgagtttctaaagatgttgactttatatacagcttccatattcttatcaggcaatcttgtgaacagcttgctaggaaaagatctctaccaaaggctgcccattccactcctctaatccaatcctcatgtccacagagagaaagcactttctgaaactgatcattttgttgagcaaatatgtgaattctgcaatcatcattgccacatgctaatattggtacatcagtatttggcaaaaaagataagcagagagccaaagcaaatccatttccaaagtttaaagtctgaaggcacattacttctggaccctttttagaccagagtcgaacagcagaatctgcagctgcagaaacgatcagtgtacataatgcaggatctgatgtcctcctctggtaaacagcatgcaccgcataaacaggtccttcatggccttgaagatgcactgcttttaaaagctgattatcctctatttcccagtgaatcacttgattatcagatcctccagaaactaattcagtagaaggggagccatcctgtttacaaatccactgtatgcaattgactcgggcggtgtgaccattcaagttggtaacaacaacccttttcagggggtcatagagcaccacggagcaggacgtgccaaaggccagaagtcctctgggcccagagctccagttcaggactccccgcacccggtttgggcagcaaaacacgtgagaagtctccagcacgggtgccaccatgtcgccaactggtcagccgcacaaacaagagacgc

SEQ ID NO: 13440 - RNA, 4463 nt, Homo sapiens
  source 1..4463: mol_type = other RNA
gctgggattacaggcatgagccaccacgcccggccctgtggtggagttttcttaccagaacttgaccagactaggcctagcaaaatcctttaattgatggaaacatacctcatttataggctgtatttgccagacagacctctgacctacctaggagggctccctgcagaccgtggctctctggcacactttgcggagtgcggacatcctagacaggacttgagttttgcaatcaggattgactcaggcctgaaaatcagttaattcttgggactcttctgtgaggtttctacaatccagaaagaccagaagagggaaaagctgagggaagacaattgggttcacctgataatcacactagccacaaattccctaggttcagcattgaagagtcaaggattcagcaactctgaaaacctagggcagagtttctctaatccttgatgcaaatacaagttgcagggagatttagcttaatacgtagtagagctgcatttgaactcaaggcacaaaacccaggctccttttaagagaagagctgcctcccttttaaagggagaccttgttaaaatgcaaattctgacttagtaggcctgatgtggggcctgagattttgcatttctaacaagcttctaagtgcggtcagtgctgctggcctggaaagcacactttgaataggaagaacacagggaagggcaatgcaaaaccatgaggaattgatttcatattccccttaaactcctgatagacggacaaacaagagagaaaggaggagccactgttttcagcctgccctgctcacctcctcctagccagagtgtatccccaacactcgagatttatttttaactcccagcagctttgattagcttgtctctgccgcttcagacacctgctggcaggataaattgggggaaaggagtggctgacccagatctgacaaatccaaggcaggaagaaaagctctcaggaattcactgcttcccctttgctgaggctggtgaaaaaccccgtcgccggcagagtgctaaacatgctaatgacctcacaccactaatgaccctgggcatgttcagccttagcaccagtgaactgccgaactgaatccatgcccttttatcacaggacgagttgtcacttccatgctcctgtggcagccggggctctatctatggagaagctctgctctgggcagatgcctggactagagctttaggcattgcagcagttttcctggggggataagtctccgccacccctagctaagattgctagtgttctgcttctggaaaagcagaagccgagctaggcgcggtgactcacgcctataatcccagcactttgggaagcctaggagggcagatcgcctgaggtcgggagttcgagaccaacctgaccaacatgtagaaacctggtctctactaaaaatataaaattagctgggtgtggtgctgcatgcctgtaatcccagctactcgggaggctgaggcaggagaatcacttgaacgtgggaggcggagtttgcggcgagctgagatagcgccattgtactccagcctgagcaacaagagtcaaactccgtctgaaaaaaaaaaagcagaggcccaggaagggaggcagggcactgggagtgccttctgtgtcccctagatggattctgtggccttctgtggagctgctgatgtgataaagtatggctttctctgtggcatgcttagttcaagcagacactaaactcctgggaatcaatggaagtctcactggataagaaacctaaatgccagcctgactctaccacttcctacacag[450 bp omitted]tacaggaaacaagttgcagtcccctacgttgggaaagctcagcagagctgacttcccgcaggccctgagcctccaggtccccgtggacagcctggggagggtctccagggccagcctggccatcccaccaggagatctgcagctgtgtggctcctccatgaggcccactttctatctgctaattgcacactctcacccccgtctcacccactctgaccagctcctttctgcagcccctggtgcagctcccttgcatgtggctgagcagcaaaaactgaggttgcagagggtctccttctgcctatgctgtatgcagccccactgtgtcccatgatcccaccacgacccacaacaggacatgcgcccggtccctaaacacagcactggctgccacaggccacaggccggcgtgcaaagaatgctatacagcccgtctctggagtctggagcagagggctaatggacatcacactccaaagcacatgaagaatattaattaaatgaaggttttatttcaaaattagtcttaagagtataagctgtttttgagggctgtagccagactacataatgagcggtgaaagcggctgccttcccctctcctgacaccagcaagggggaggcaccatcaccggccctgccccatcatgcatccaatgattactagcactagaagccaacggcaaaggaccccgcgcgcttgctcgtgtttaatccaggttaagctatacacgtttaaatacatgtcggaggttacatggtctcatgcagtccctgtgatggaatgactcttgctcagtgacctcctgcagcgaggctgctccaaagggcaaggttaggtagggcagagcacttttaaaatgtagtccgttagcaaagtaggcaccttctcattatcctccttcatggcaaagagaatgtttgtcagcatctgcaggtcttccactgagggaggagaggctttcttctcgtaaggaatgactgtgttcagatactgtttgtcagttcctgaggagccaaaggtctggcggatgccactctgcagaatgttggagatgccttccatgctgaagcgcttgagaggcatctggtttcccttctctatccggctgctctgcaggctcagccctttctctttccgcctctttttcatcagttctcgctgctccttctgcttgttctgaacctcaataagcaccgtgataaaggagttcttcacttccttctcaaactccagctcgtcccggcgggccagctgctgcaccagctcctccgagaagtcacggatggcaccctccacctggtccagcagctcggtcagctcagacccagacatgtgcctcagcccttcataggaccagttgttgttgaaggtctgtgtcaatgcctgcatctcctgcaggaggaccgagtctgcctgggaggaagtttctcctccatcctcttcttccagaacctcctcttcttcctcagggtctggggagttctgcatcatttcctcaatctcctcaattacctgatctgctgtgagcagaggctcctcgttgataccggaatcattttcactcttctcattgaactcttcctcttctttctcatggatctcagtgtcagagcagttgccattcagagcctcgatgtttggatccctccagtcttctgagagtgaagggatgtaattgtctgtcagagcatcccaaacctcctcgtcctgaagggtctcctcctcctcttggatctgtaactggttcttcacgggagctaggttctcggtcttggcgttgtagttccgaaagcagacattgagcttctcatcaaattcatttacgaggtcctccatggacttgaagctgattatttcggaagaaaaattctcaagctcggagagggaggggtcctcgagatggtggggagatgaaccatagaaacactggggcttctcctccgggtcctccgagcaggagggtcgaaggtcctcaaactcttcatccagactcaccagtggggcctccattcttgctcagcaggagaacaacagcgactttcaggatgagtttatctgtgcgggtcctggcggagggaggcggatcccggggctcagccggacacccccatccacgggccgcgggagcggccggagcgcagcgcagcgcagcggagagccagccagccagccagccagcgagcgctccccgcgcagctcc

SEQ ID NO: 13441 - RNA, 4111 nt, Homo sapiens
  source 1..4111: mol_type = other RNA
gctgggattacaggcatgagccaccacgcccggccgggtccctgtgttttaacaagtctatcagatgattctgatgtagactaaagtttgagaattactgctctaaggtgaagaactattgtaaaattatcctttagataattgagttgacttcctcaattagggtttcaactagaagccagaggtgaatgatgtcttcaagaaaatggagacattttgagaataaatgatctgacatctttataaggcctttaataatgtctgacaaatcctactgaatgtagaatacttatcactctgttttctattgccaggattatgcaggcagcttacctcaaaatataatcaagtctcttaagtacaactttttaaggggttccaaaatacaaccctattttgtaccacaacaaagcatttcttgatgtggaactatctttgctggatcacctatctccccatcatctgaggttcatcttcctctgatatgtcaaagagaaagttacagaggaatcttcttcagacatatatatattaagttacattaattttcaattaattccttagattaaaattttcaacatcatttctctcttttttgatgagggctatttagcttatatttacattctttactttttattttgataacaaatgcaagttatagagcctcctactgagctatgtgttttaacattagatctagttgctgaagaaaatcatttaacaaataagggaactaagatatagaaaggttatgtaatctatccaggtccacatagccactaagtcatggaaagtattacttgggctaatttagtttttcaaatttgacataactgtgatgaaatccaaagcctcagacatatgaagcatatgctgtctcctgagctgtattcctgaaattccagtgacacaattgtgaagccctgtgtggaatctaattgttagcctaggtttttttttaaaaactgtacagttcacattctacatggcattgctccctgaatttctcaagacttctgcattgatagttttaaataattcctactaaatttaaagaaatcttcttagtaactcactttgaaagcatctatagagcaatgcctattaagctactgtctttctaagaatattttcagtatactagaaaacttgaaagaagagagtctatttttaataagagcagcaaaggcatgtacagacatgatttctagttaatcagtggatgatttctcagggagtttccctcaaaatagaatttattatactcaatgtactcttgcatgcttcttgtactttttttatcccagcttgaatgtgattcatctattcttagcaataatttaaggatcaacgtattttttctataaaatcaactttctttcctctttattttctcagaaaaatgtgatttattaagtttaacagtgtaaattatggttcaccacaggtcaactacccttctgtgagttatataatgataaattggcataattatcaatacttaaaagtccaacaatgtatttatacatggaaattaatatggatgatttgataatgcttatttaaacatatgagctttagtttttaaatttgccatatttaatatttttaaatgttcccacaagctatatattgctatgaagatactctttgaaagagtggccccatagcatttcaacaaataaggctcattcaacaaataatgtttattggcacagtatttattggaactcaaagcttatttctctggaaaaaccatgctcttttttaaggagtatgttgtggcaatacttctacaaaattatcacaaaaatgtctcactcctattatagcagttatatcataattttccattctcttatttgtctccctggaattaagaagcagtataatctatgagttgcccagatctcttcaaatggaggccagaagcctatgataatctatttaacccataatataatagattgggttagaacagaggacaatgtaataaaataaaggaaaagaaagtttgtctccatttattgtgcatgcctgaccctaggcacttttcacctatatcctgtcgctttttccccaggcttctagtcttttaggcacccattcacagatctcaaagatgtattggggaaagcaatttgattaaactagtttacgttaaaatatgaatgacaacacagagcttcattttttaaaaagcccttataaatacaacataaactgaaattggtggacttataagcagtattaatagaaaatatttcagatagttaaagtatgtttggtcaattaaaatgccactgttatctaaactgtttgtttcatttgattagcacttatgcgcttctcaacactgagaagacatattcagtgctaaccttaagtattttacattgactttcaaggcacaggcaatgaggggagaaaagttgaggcttgttacaagtggtcatatatgagctcttcaaaaatttaatgtaagtcaggaatactttaagtctcaaatatcatcagaatgtggcagcagtgggtgagtagtgtattagaaagggcacagcctggggtcaagtggactctgcctgggtggcttggggtaggtttaacctcacagcttttttaatctattaaacaaggttttggtatctattttatagggtagtgatgaggattaaacgagatgatgtatataaattgtttagcacctagtaaatgctcaataaataatgcagctaatattagttattattttatagtaacaacagcaaatataataatagacaccagatatgaatctgacaagaccaaaaagaaatgataaagaaatgactaagataaggaaaatgattttattgattttagtgtggctcagatatctttgaatgttccctttactctcaaataaggagattcaagtagcacaaatctaaaaggaaaaatgaaatttagaggaaaaaaatttatgaatcttaaggggatatgaagattttttttaattaaaggagactggaacataatatgtgatgaaaaatcacaaaccaaattactgaaattaagaaattatgctatcatggttgacattaaaggtgactggtccttgatgaagtgattaatagacatgcatatgggtgtgggtgttttcaaagaaatactcattaatagtgatgacataaatggacctgacaactaagaccacgtttataaaaggcaagttttaaaatgtagattagatagccttatatatattatcaagaagaaacatgacaatacatgaatttagatataatgtagacatgaagaaataagagttatgttttaattttacagcagtgatagaaacaaaatacttggggaaaagtatttttcttagggagaaaaattgagctgctgttagtatgtaactcagcccagtaacatgatgaggtggatagagccaggctttgtgcctgctacaggaagagctgctgcagcgtcagttctcaagctaccaagaaaacctagtattcatgtaaaacagacgtcattatgcatgtgtaagatggaatcctctgataaatagaacaagaggattctaataggcatgatcttgtgaacgcagtctcagggagtacaataagatgttttaaatagaaagtaatgaatgaagcattcttctttggaataagcaatctactgtttcatgaacagaagttgggttcagattttcaaaaaaatgcctgctaggcatagtctaacagatatccagcagaatggttttctatttttgaattagaattaagatcacttactcatgattttcaactcgagccaagtcaagtaatcttatcttgtactgatgaagatgtcagagactatgccagtggctgtacctggatttcttcaatgaaacacatcacttctataaacgcttattttactttttcatattttcctattattttatttatttcttcatgcctcagcaagcagataacttcaggtcctatagcagaatcccaagagaaatatctggaaatcagtgaacctgcaaagcccttgggggttccagtgtatatttgttgtcatcaggaatctgggtgtggtggctggtgcctgtaatcccagctag

SEQ ID NO: 13442 - RNA, 3140 nt, Homo sapiens
  source 1..3140: mol_type = other RNA
gctgggattacaggcatgagccaccacgcccggcctcaattgtatttctatatactaataatgagcaattggaaaaaaaatctacaatagccacccccccgccaagtgaaatatagtttgagacccattcatggatctcaaatccaaaaatgtgaaatgctcaaaatctaaaactttttgagagctgaaatgactatcaaaggaaatactcatttaagcattctggattttagagttgggatgctcaagtaatatttgcttcaggtaaagcaaatattaacctgaaaataatccaaaatatttctggtcccaagcatttctttttttcttttctttttctttttttttttttttctttttgagatggagtctcactcttgttgcccaggctggagtgcaatggtgcaagctcggctcactgcaacctccgcctcctgggttcaagcaattctcctgcctcagcctcccaagtaactgggattacaggcacccagctgttaaaagaaaaagcatttggcttctactggaatctggagccacagtttggtgtcaaacagagcagctgtgcttttgtttcaaatgctgtttgctgaaaacctctggatcagaagagctggtcttcagccaggtccttggcaccaagaggatgtgaacaatcctgaattccagggcctactgatggagtccactagttagtccctttgacacggcccccttatggatcccagtagtcagccggggtgcaggttttcatagtgattctaaacaaggctgcagtcactgtttagaagtgattgggggaagctggaactgtgctccttgtttcaggacctctagattgcacctagattaaacaagacggaagctctcaaaaggctctaagtctaggcctcctgtgaggtagggtctgaaaggacttaaaccatttttttttttttttttttttacacacagggtaactttttggaagagtactttgtaacaataaagtgctgtgcacagaaaggagaaatgccattatggggatgtgtgtgccgacctgggaccagcagggtgaaagagtctatcattcatgatgagagctgccatttgcgctaagcacacaccatgtgccaggcactatgccaagaaattgttgaatcttcacaataactctgtgagaaaagggctgtcattggacagatgaggacactgatgctcccaggggtccacatcacatgaagaggaggtgacagggctgggccttggtccgaagctccagccttccaagccaaggcctgtgagaggaaccgctgagacctgatgttaggcctgtttttctcatgtgccctggagaaggggactaacaccatcttttgccaaagtttggtgagggatggccaagagctctttgaaactttgccatgtacaatagcactcacaattttttttaaattttttatacagtggtatcggggtacagtggctcatcaacactttgggaggctgaggcgtgaggattgcttgaggccaggagtttgagaccagtctgggcgacatagtaaaatctcatctctataaaaaaagaaaaaaaatgaggcgggcatggtggcaaacatctgtagtcccagccacgcaggaggctaaggtaagaggatcacttgagcctgagaggttgtggctacagtgagccatgatcacactactgcactctaggatgggtgacagagcaggacagtttcaaaaaaagacaaaaaaaaatttacacagtggaatgctttctttaaaaactatcttatgcataagtacaatctagaaaaccagaactgggccacttatagtgaaggtggaagcagaggtggcctgggaccccccaggattcctggagcactgcctgaaggccatttatctagtagattggcactcactgtaagaagcgcaagaggtaccatgatgcttaaggctctggctctgggtgtgaaagaatgaggtggaattgtagcagattcattcctgggtcaatctgtttttggggagggctgcaggattccaggcctgccatgtgcaatgggtgctgccctctttcttctgggcaccatctgcctcaacctatcccctggccagtgtcactcacagggcagaaaatttatcttcaccatctcacaattagtttaatctctgactccaatgcaggggctcgtgggatggctcacagtggaatcatcaaacggacttccttctcatagatgtcagggatcattcccactggggaactgaccatgtgcacagtgttcttgccaaacaattggaactcatagtggatgagctgctcccaaaagccgctgttgggtcggatgatgggccggcatgacttggtccacgtgtgggcgtccagcagggacatggcgtggtacttcatgaggtaggcgaggcacagggcagctgagcggctcacaccagcagcacagtgcagcaaagtacggccctgcttcatctccacgctccactgagacattgatgaccatggtgatctggttgctagacagcatgagcttgttgttggcggccacaccattgctgatatacaggcttttggttatctgcgagaggccgctgactgagggctgccggaactgaactgggaaggcacacgagggtgctgtcatcaaggcggtgggtcagtggtcagcagtcagcgaagcacgaaggctgcgtctttctgctaggctgtgtccatggaaaactctctccttcaggcgggtgggcgggttcgctcaggaagtagccgcttggggaagccttaggcaaggttcttcgggagagagacccgtcatgatcccgcagcctcaatccccgctggcctaacgctttggtttccatagcaatgggctcgtcgcagaaaggaatagcctgtgccgggtcttcagagaaatcctggcctcggctccacgcccctgagcagccccaccctggctcaacctgttacccgccctgccggcaagccggggtcactgcagtccccgtggcgaagcagggtcagctcagctcaccgcaccccactccatccagccctgcccatctctacggcaacgggccgggtcgcaccagggctgcagccgagagacagtctcaccgcttccgtagccgcccgggctctgtgc

SEQ ID NO: 13443 - RNA, 3256 nt, Homo sapiens
  source 1..3256: mol_type = other RNA
gctgggattacaggcatgagccaccacgcccggcctcaattgtatttctatatactaataatgagcaattggaaaaaaaatctacaatagccacccccccgccaagtgaaatatagtttgagacccattcatggatctcaaatccaaaaatgtgaaatgctcaaaatctaaaactttttgagagctgaaatgactatcaaaggaaatactcatttaagcattctggattttagagttgggatgctcaagtaatatttgcttcaggtaaagcaaatattaacctgaaaataatccaaaatatttctggtcccaagcatttctttttttcttttctttttctttttttttttttttctttttgagatggagtctcactcttgttgcccaggctggagtgcaatggtgcaagctcggctcactgcaacctccgcctcctgggttcaagcaattctcctgcctcagcctcccaagtaactgggattacaggcacccagctgttaaaagaaaaagcatttggcttctactggaatctggagccacagtttggtgtcaaacagagcagctgtgcttttgtttcaaatgctgtttgctgaaaacctctggatcagaagagctggtcttcagccaggtccttggcaccaagaggatgtgaacaatcctgaattccagggcctactgatggagtccactagttagtccctttgacacggcccccttatggatcccagtagtcagccggggtgcaggttttcatagtgattctaaacaaggctgcagtcactgtttagaagtgattgggggaagctggaactgtgctccttgtttcaggacctctagattgcacctagattaaacaagacggaagctctcaaaaggctctaagtctaggcctcctgtgaggtagggtctgaaaggacttaaaccatttttttttttttttttttttacacacagggtaactttttggaagagtactttgtaacaataaagtgctgtgcacagaaaggagaaatgccattatggggatgtgtgtgccgacctgggaccagcagggtgaaagagtctatcattcatgatgagagctgccatttgcgctaagcacacaccatgtgccaggcactatgccaagaaattgttgaatcttcacaataactctgtgagaaaagggctgtcattggacagatgaggacactgatgctcccaggggtccacatcacatgaagaggaggtgacagggctgggccttggtccgaagctccagccttccaagccaaggcctgtgagaggaaccgctgagacctgatgttaggcctgtttttctcatgtgccctggagaaggggactaacaccatcttttgccaaagtttggtgagggatggccaagagctctttgaaactttgccatgtacaatagcactcacaattttttttaaattttttatacagtggtatcggggtacagtggctcatcaacactttgggaggctgaggcgtgaggattgcttgaggccaggagtttgagaccagtctgggcgacatagtaaaatctcatctctataaaaaaagaaaaaaaatgaggcgggcatggtggcaaacatctgtagtcccagccacgcaggaggctaaggtaagaggatcacttgagcctgagaggttgtggctacagtgagccatgatcacactactgcactctaggatgggtgacagagcaggacagtttcaaaaaaagacaaaaaaaaatttacacagtggaatgctttctttaaaaactatcttatgcataagtacaatctagaaaaccagaactgggccacttatagtgaaggtggaagcagaggtggcctgggaccccccaggattcctggagcactgcctgaaggccatttatctagtagattggcactcactgtaagaagcgcaagaggtaccatgatgcttaaggctctggctctgggtgtgaaagaatgaggtggaattgtagcagattcattcctgggtcaatctgtttttggggagggctgcaggattccaggcctgccatgtgcaatgggtgctgccctctttcttctgggcaccatctgcctcaacctatcccctggccagtgtcactcacagggcagaaaatttatcttcaccatctcacaattagtttaatctctgactccaatgcaggggctcgtgggatggctcacagtggaatcatcaaacggacttccttctcatagatgtcagggatcattcccactggggaactgaccatgtgcacagtgttcttgccaaacaattggaactcatagtggatgagctgctcccaaaagccgctgttgggtcggatgatgggccggcatgacttggtccacgtgtgggcgtccagcagggacatggcgtggtacttcatgaggtaggcgaggcacagggcagctgagcggctcacaccagcagcacagtgcagcaaagtacggccctgcttcatctccacgctgtggatatggtcagcaatagggtcaaagaagtcacagagacgtgagttaggggagtcagccacaggtacctgcatgtactggatatcctcatacaaggtgttcactacctccactgagacattgatgaccatggtgatctggttgctagacagcatgagcttgttgttggcggccacaccattgctgatatacaggcttttggttatctgcgagaggccgctgactgagggctgccggaactgaactgggaaggcacacgagggtgctgtcatcaaggcggtgggtcagtggtcagcagtcagcgaagcacgaaggctgcgtctttctgctaggctgtgtccatggaaaactctctccttcaggcgggtgggcgggttcgctcaggaagtagccgcttggggaagccttaggcaaggttcttcgggagagagacccgtcatgatcccgcagcctcaatccccgctggcctaacgctttggtttccatagcaatgggctcgtcgcagaaaggaatagcctgtgccgggtcttcagagaaatcctggcctcggctccacgcccctgagcagccccaccctggctcaacctgttacccgccctgccggcaagccggggtcactgcagtccccgtggcgaagcagggtcagctcagctcaccgcaccccactccatccagccctgcccatctctacggcaacgggccgggtcgcaccagggctgcagccgagagacagtctcaccgcttccgtagccgcccgggctctgtgcgcatgt

SEQ ID NO: 13444 - RNA, 3390 nt, Homo sapiens
  source 1..3390: mol_type = other RNA
gctgggattacaggcatgagccaccacgcccggcctcaattgtatttctatatactaataatgagcaattggaaaaaaaatctacaatagccacccccccgccaagtgaaatatagtttgagacccattcatggatctcaaatccaaaaatgtgaaatgctcaaaatctaaaactttttgagagctgaaatgactatcaaaggaaatactcatttaagcattctggattttagagttgggatgctcaagtaatatttgcttcaggtaaagcaaatattaacctgaaaataatccaaaatatttctggtcccaagcatttctttttttcttttctttttctttttttttttttttctttttgagatggagtctcactcttgttgcccaggctggagtgcaatggtgcaagctcggctcactgcaacctccgcctcctgggttcaagcaattctcctgcctcagcctcccaagtaactgggattacaggcacccagctgttaaaagaaaaagcatttggcttctactggaatctggagccacagtttggtgtcaaacagagcagctgtgcttttgtttcaaatgctgtttgctgaaaacctctggatcagaagagctggtcttcagccaggtccttggcaccaagaggatgtgaacaatcctgaattccagggcctactgatggagtccactagttagtccctttgacacggcccccttatggatcccagtagtcagccggggtgcaggttttcatagtgattctaaacaaggctgcagtcactgtttagaagtgattgggggaagctggaactgtgctccttgtttcaggacctctagattgcacctagattaaacaagacggaagctctcaaaaggctctaagtctaggcctcctgtgaggtagggtctgaaaggacttaaaccatttttttttttttttttttttacacacagggtaactttttggaagagtactttgtaacaataaagtgctgtgcacagaaaggagaaatgccattatggggatgtgtgtgccgacctgggaccagcagggtgaaagagtctatcattcatgatgagagctgccatttgcgctaagcacacaccatgtgccaggcactatgccaagaaattgttgaatcttcacaataactctgtgagaaaagggctgtcattggacagatgaggacactgatgctcccaggggtccacatcacatgaagaggaggtgacagggctgggccttggtccgaagctccagccttccaagccaaggcctgtgagaggaaccgctgagacctgatgttaggcctgtttttctcatgtgccctggagaaggggactaacaccatcttttgccaaagtttggtgagggatggccaagagctctttgaaactttgccatgtacaatagcactcacaattttttttaaattttttatacagtggtatcggggtacagtggctcatcaacactttgggaggctgaggcgtgaggattgcttgaggccaggagtttgagaccagtctgggcgacatagtaaaatctcatctctataaaaaaagaaaaaaaatgaggcgggcatggtggcaaacatctgtagtcccagccacgcaggaggctaaggtaagaggatcacttgagcctgagaggttgtggctacagtgagccatgatcacactactgcactctaggatgggtgacagagcaggacagtttcaaaaaaagacaaaaaaaaatttacacagtggaatgctttctttaaaaactatcttatgcataagtacaatctagaaaaccagaactgggccacttatagtgaaggtggaagcagaggtggcctgggaccccccaggattcctggagcactgcctgaaggccatttatctagtagattggcactcactgtaagaagcgcaagaggtaccatgatgcttaaggctctggctctgggtgtgaaagaatgaggtggaattgtagcagattcattcctgggtcaatctgtttttggggagggctgcaggattccaggcctgccatgtgcaatgggtgctgccctctttcttctgggcaccatctgcctcaacctatcccctggccagtgtcactcacagggcagaaaatttatcttcaccatctcacaattagtttaatctctgactccaatgcaggggctcgtgggatggctcacagtggaatcatcaaacggacttccttctcatagatgtcagggatcattcccactggggaactgaccatgtgcacagtgttcttgccaaacaattggaactcatagtggatgagctgctcccaaaagccgctgttgggtcggatgatgggccggcatgacttggtccacgtgtgggcgtccagcagggacatggcgtggtacttcatgaggtaggcgaggcacagggcagctgagcggctcacaccagcagcacagtgcagcaaagtacggccctgcttcatctccacgctgtggatatggtcagcaatagggtcaaagaagtcacagagacgtgagttaggggagtcagccacaggtacctgcatgtactggatatcctcatacaaggtgttcactacctccactgagacattgatgaccatggtgatctggttgctagacagcatgagcttgttgttggcggccacaccattgctgatatacaggcttttggttatctgcgagaggccgctgactgagggctgccggaactgaactgggaaggcacacgagggtgctgtcatcaaggcggtgggtcagtggtcagcagtcagcgaagcacgaaggctgcgtctttctgctaggctgtgtccatggaaaacttaaaaggatgttgtgaaattaaacgagataatccacgtaaagagttttctcagggcttggcatagagtaagccctctcaaaatgataactatttttctcgcttctgatagggaagttaaaatgcagggctctctctccttcaggcgggtgggcgggttcgctcaggaagtagccgcttggggaagccttaggcaaggttcttcgggagagagacccgtcatgatcccgcagcctcaatccccgctggcctaacgctttggtttccatagcaatgggctcgtcgcagaaaggaatagcctgtgccgggtcttcagagaaatcctggcctcggctccacgcccctgagcagccccaccctggctcaacctgttacccgccctgccggcaagccggggtcactgcagtccccgtggcgaagcagggtcagctcagctcaccgcaccccactccatccagccctgcccatctctacggcaacgggccgggtcgcaccagggctgcagccgagagacagtctcaccgcttccgtagccgcccgggctctgtgcgcatgtgc

SEQ ID NO: 13445 - RNA, 9170 nt, Homo sapiens
  source 1..9170: mol_type = other RNA
gctgggattacaggcatgagccaccacgcccggcctcccctgcacttttcttactttattcttccaggattccaattacactcagctcttagatgctctgttctgctttattcactctttctctctttgtgttttagtttaggaattccttaatgacatcttcaagtctaccaaatctttcctttgatatgtcaagtctactgataagatgaaggtttcttcatcactgctactatgttttccattcctagatttctacttgatttttaccatctatctattgaaattagcctgctgatgatgcatattgtctgtgttttccagtagagcttcaatatatgaattagagttatttcaaattctctatgtgatagttccaatacctatgtcatatctgattctggttctgttgattgctttgtctcttggtagtttccttccccccactgttttctcatatgcttaataactttttgctgaagctcgacattttgtccaaaagagtggagactaaatagtttctaaacctaagaataggcatgtttttacttctgataggtcgttagtgtggaagtttgagcaatgtagtcagtagttgtgctgggtttgggtttgttatgcttgcactctaccactggcttccacttcctttggttatacttgtgtttagagtgaggactggtttgccagagagtagtctgtttcactcccatctttagggtaatctcttcacactgcaactctctgttagtccatttgcattgcattcctatgtaaaaggaaatcctgaggctgtgcaatttataaagaaaagaagcctattttggctcgtggttctgcaggctgtacaagaagcacggtgccaacatcttctggtgagagtctcaggacacttccactcataggggaaggcaaaatgggagcaggagcatcacatggcaaaagagggagcaagaatgacagggggaaggtatcaggctcgttttaaacaaccaaatcttgcataaactcattgagtgagaacttactcattaccacaaggacagcacaagccattcatgagggatctgccctcaggacccaaactattcccactaggcccacttccaacactaaaggttatatttcagcatgagatttggagatgacaaaacatccaaactatatcaatctcggagtctctacccacacacttttgtaactctcaaagctcttaatcactgttagatgtcactggaggcttttcagcccgggagcgtggtggtaagaggagcattgctgttctaattaagccttggttttaggcgaattatgtccttaggtttcagaaaggtggctgcctccgtgttccagtgtttcccacagctgtaattctgggaagggagtagagttttatttttaatgcttcttatctctagctgcaatggctgttccctagttccctaagacacttcctcctgcagtttaaagcttttctcccaaggagaattaggggagggtgggatacaagcaggacttcttgtctttcctgcagtggctgctgttctcctccccatgttttgtacaatgaggattctaccacagtcatttttttgtgtgtgcatgagcttctggtggggcccaaggaaagagcctattctgggtgcaaatttccctgttatcttgccccaaggttttctacagtgagaatctacaagccagttaaaatttgttttatgcctgcagccaactgaaccacattccttctttactaatttgttaccaggtgagcaaatgctagcttaccctctctccccataggcacatatctttttttaggttttaagttagttggtattcctgcaatcacagctctctgactagttcaagaaaagttatgaatttgcaatttgtccaattcttttttaatgctgagagtgggcataatacttttttattccagctttgttcatcccaagcaaaagttggaggtctctgaaacttaatttcaaatagttcagcaaaaaaaatgaaaagaaagagaaagagtaaatgaaagagaaggagaaagagagagagagacagtgagagaaagatacataaagaaagagcacaaatgtggcaacatatcaagaattaatgaatcaagatgaagtggggatgggtattcataatactttccatttctgtgttgacacacaggcagtgctcaattaattaccttgaatgtaattaagacataatttgctgaatgacagtattattcttgttattagttcccaccaaaatagatgaatcaatttttttccctttctagtttgacattgttaccctaagatactaatcctgctgactctatttttaaaatccaggtttactaaatattttatctacttatctgtcagcaatgtttcaactagaatagaaatgcttttgcataaattcatcactcattgagggatcagctaattggaaagagcattagatatggaattttgaaaaacaggcttaaatgcaagcttattcatttcaccaatatttatggagatcttacagtgttctattgattgtatgagaggtttgggagtgaatagtagctctgctgcctctcagtcccttgcacctgcacacatttatatggtttgagccttggtctccacctctgtgaagtatggataacaacgcctccctcatttgtgagagttaaaatccctgttatatgataaagtgctttgtgaatcataaacaaatgatccaaaagcatattattctaattctcttttagtttcttcctcacttgttcttattttttttacttttttttctttgcatttttgtaatgtccttggccttggtttcttactttattttattatgactgcttacactgttgtagtcatttacaacttcatgttaatcaaaattgtgaatttcggcaaaggcaacagtccctgcctagtgtatgaccttttttcccctttgatcttggcatctgaaagctttttatacattctaattctcttccattttaatagctctgtgaagcagtactattttctttgactgataagatcattgaaggtgacctgattttctctagagatgcacaatgaataaaacacattctccactacacaactcacttactcacatcccatgaagggggaaaaatcctgaggttgctctctctctataaaggtcacagaaaaaggagatgacttctcagatattgtgattatgcatgtatcatcaaattatgcaagctgcttattattccaaatcttaggggtttttttgttatttcatcctgttttacataaaactgagtagcaaaagtggcaaaacaaatatagcatttgtctttgtttgtgtatttttaatgagccgaataacacaaacaccttaattttgagggtgcatcttgttgagacacaatattatagatacctgtttgtacttgtgtgtatgtgtgtctccaggtattacatttatgcagttttcagttggaaaggtgacctctttctacggagtatgtgccctgcacatagggtttatcccttgtgactggtttgtgtgttaaggattcatggcttaaacagctaggttattcatgggtgtggaaaattgatatttgagagcattttattctgctcagtcaggctgattctttataaggaatcaaaacagtgataacatttaccaaaaactactgaatagaatattcaatgtgtatctatgccacacattgtttctttccatacactccatcataaaatacctcctctgcctatcatcgctctgacaacgtcactgccaaacccctatcctcatacactcatcacagaacatctcttcattttgttcagaaactgtgcttttttttcttaatcgttctgcttttcaaagctttattctttctaggcattcaatatatattgaataatttcaaggtatttttatattcattcattctactaatattttcttaactattttcagctactcttctaaacatcttgttcaggaattgtggaagaatctactcactgttttgtcccaatatccaagggagaaaaataaaactagctcaacatccctgtgcatgaacttttagtaactttatttccccactagaactggaatctgatgatgagcatctttgttctccagatttcaaggaggtactccaggtagctgactttccacagagcctgaaaagcactggcataattccgcaggcatggcctcttttcttcttatcttcatgtgtgtgctaatgttgtgatctttttaaaatgccaagatgaactgtacagggcatcatgttctcagactcctcacttcagaatctgattcttagctctgtggacttgggagactgggttttcttagcattctcagagtggatcagatctttatggagaaaaacttgcaaagaaaatttagaaaacatttacatataaatcagaaaaatgatatatttacttacattaatatattaatatgctaataatgtattattgtaatctgctgttttcttttttcatttaccatatacttacatctcttatctaggattccctgttctcaacctttagttcattatcaccctcctctcctcacaaaggagacttttgagaccactgccaatgaaattttgatactgcatttgtattgtttatctgtatatatctgtttatgtatttctgtgccttatacatggaaagtaacattttctttcatttctcccaataccccagagccaattttcacctccttgggggtgatgtcaactccattgagaacatgtatcttattccttttttcctgctacctggcagcatgagatgttatattaatcctgtctttttattttctgtacttttgatgctttgacatctagggacttgctgactctggaaagactgccctttccaaagttaggcaattcttagagattaaaaaaaaagactccccttccagcatccttttcatatgcctttaataggcaaatcaaacaatctactacccacatcccaaccatctcctttactgatcctttacactccacgccaggttcagcttgtcctaattattccggggccaggttccagacaactaaagacagcctctgcaccccagaatctgaagagatgatccaactagccatttctaagccttcttacattgtattcttttccatggaaacctctatacaggctcttgcctatgtttttctccactttctctgcctctaaactgagcctggtgattcctctgaaaccctgcatggtgggtcctgccccctcctcttgggacctgtgaataataaaccatcttttcaatggtaatcttctcctgatttcttgggttcatgatacctgaatagtaataaaacctaaatttaaaaatacctatgtatcagggagttggttggccagtatggaatatgaataatcttgagagatatttgttagagttttgatgaagacttgtaaattccccctgttccttagaaagagtgctgtgaaaacactaccaaactcttgttctttttacttttacttttcttttctgggtctatacagacatctttatagttaattgactttttagtaaagagtaactgattaaactcatagcctttgtttaggctccacctgattctgccttcttagtttaccttttgaatgaaactgagtgtctccaaacattttcaggcatatatttatagtcaactcttgtggctattttgacaggtggttgacctcattcattatgtattgaatcttactattctcacctttagtataatcttatttctacatttttgggacacatcactgaaaccttctgtgttccatacgagacctgtaccagatatctctgcagccaaagagaagttttttttttatttttattttttcatgagctaacacaaggcttgcacaaaactcagcagcaagtaattcctttcttgtccagtatgaaaaagtgctgtctttgtcataaagcaaaaagagacaatgaaaggttaggttcttattgccccatctcattattgttaatgcaaaactagactaatttgcttgtggttatggaaatacctcctttaaccttggtgactgaatcagaaagaatttgttttggagatgggcattgcttaacagcatttggcatttgctcaggctgagcattcatcgtgagagtaagagccttctttccttctttagtgtagtaatctctgcagaaatatcacatgaaatatggtgcagaaaaccttcagcatagtggctgggatagaggcagtgtgctttgagtaaggctcttcagttggggcctgcattttctctggagccaagatacttctgacctcagcaaatggcttaactgctctgataaaaagtggatgataatgataacacttccttcttttcagatccataagaagaagagatttttttgtttttgtttttgtttttgtttcatctcctgctgtatgcttggtctctaaaagtgactggcagagggaagacaataaatatttgttgttgaatgaatgaagtgttatgatgagggttaactgacattataatgcaaagctcttggaccaagacctgacttatcataggccctcgaaagatattccttccaaaaacaatgacagcaaaaacaaaataaatgcttcatactcaataaagtgtctggtgatgggtttataggaaatttagtaattttaatattaaaaactaccatttacatcatctgattatttattcgccaaatatgtatcaagcaatcactaaataccatgcattattgcaggtcttggagatttagaggtaaacaaaaatagccacaagtaaaagctgtccacctataaaactttctgcccagcctagcgcaggttagagttcccatatgtctatcagtgatcaatagctgtgggagaagaaacctgtagaacactgaaaaaaataaagcattcagatcattaacttttttattaatcttttgccatttgtggatctgtcagcttctctaaaactcttgagatacaaaagcattatctctgagacaagagataattcccaagctctcctcttgattgcccacgtttgcctgagagaatttctcaaccagttgtttcaggttatagacataattggctattagtcattgcagtgccattgttcattgacatacctctcagcatcatctctcacccatctgcaaagcaaggtcctggtttctgattaatctttggctggtcattgaggatactgaagcagctcctggttaattagaccattttgtctctaacctcatccattctctggatgtaataatagggatagaggtggcagcaattgtaagcacagccctgaaaacttgctaatcggcctttgtgatttgccaggggtgccattgtttaaattgttaaagccaaattgttgtgagaggcagtaagtgggcatttttatctccaagtcaattacacacatttagtgaaacctaaggagctcataaattaaaagtaaataagtaaataggaaagcagcatctacaacacttagtgatgtaagtcacacacatacacaccacatacagggtgataaaatagcaaaatgtgcacttatgtggagaggaagcccacgtagtgataaggggtgagggctcctgagtttaccagctgtgtgaacttgggcaagtaaccgctctctgaaccttcttatctgttaaatggaagtaatattaaagcctacagggacatcaaaaggattaaattacattaatattttatgttatttcattaaataagattttataaactatctcaaagtctgctctattacgtgtgctaattatctggtagttactattattctagaaaagcatcctatcccccctaactcatgcaaagaaacaatgaacgtttccaatacttcacattaaaaaaattactttgacagtatccacaggaaatcaggtaaaaagcaaagacagacaagcttagctctttccactggactttgtgagatgtgtctagttgtactagagttcaggcgagcattctaagagatgctggagggcagaaaatgaagtgaacttcattctatgaagcacttgagacttgtctttcccagtatttccccatcatctctcaaagaactgcctattaataaaaaacaaacaaaaaaaacttattccttggtatgctaccaaaaaaaatattcttcattcaagtaagtttggaaaccactgagtattacatttccctgtgaagaatcataatcattattttggtgttaaaaggcctgagaaatcaggaaaagctctaataaaaggaataaaaagaatagctttgaatcctttaacctaatttttcaaaaataccccacacaacatgtgttaccacacaaattgcattttgaaaaaatgctggccaggcacagtggctcatgcctgtaatctcagggctttgggtggccaaggcaggtggatcacctgaggttagggattcgagaccaacctgaccaacatggtgaaacccgatctctactaaaaatacaaaattagccagtcatgggggtgcatgcttgtaatccctgctattcaggaggctgaggcaggagaattgcttgagcccgggagatggagtttgcagtgagccaaggttgcaacattgcactccagcctgggcaacaagaacgaaactgtctcaaacaaaaaaaaaaaagaaagaaagaaaagaaaaaatgctgagctacaacatagtaggttgaagagtgtcctccaaagcatccgcacccactcagaaactaagagtgcgatcttatttagaaacagagtcttcgcatatgtaatttgttaaaaatcttgtaatttgttaaaacctggattttgactgggccttaaattcagtggctgatgtctctatgagaaaagaataggacacacagattcagagaagatggtgacgtgaagatggagacagagattgaaatcatgcatctacaagtcaaacaatgccaaggattgctggcaaccaccaaaagaaaccagaacgtcatgggatggtttttccttcagagcctccagaaggaaccaaccctgctgacacctcggtttcaggctgtagacttctagactcctgaaccatgagagacaatatatgctttttttttttt

SEQ ID NO: 13446 - RNA, 6363 nt, Homo sapiens
  source 1..6363: mol_type = other RNA
gctgggattacaggcatgagccaccacgcccggcctctcttttctattttattcatttattcactccatcactagagaacactggcttagagctgatgtgcctcagacacaggtgcactcatggagcacagaagcgagttggacaaagtccgggcctttgtagtgtgacgtggccattagggcccacagatccttccctgcagttgctgtctccctttcttcaggttccgaggaagccttccctggccgccttcataactctgacctcctccctccctccaacctaccagcatcaaatgcaccagctatgctcctcttttcccttgccgtctgttgccctgcactttgggaggctgaggcaggtggatcacccgaggtcgggagtttgagaccagcgtgaccaacatggagaaaacccatctctactaaaaatacaaaattagccgggcatggtggcatatgccaccactcttggagtgggcccaagaggaaaagatccctgcttatggccatgtcccagtgcctagaagagaggcggctcataggaagggttgaaaaaagtgtggaatgaatcaataaacagctcttgatttagtggcaggagaagtacaggcctcacctccaccgcgcaggcctcatctacgccatccagccctcacccacagtgtccagacctcacttctcccacccaggcctctacccagtcatctaggcattctccctgccgtctagcccaaaaccggaacagcacagccctcacctctgctgcccaggcctcatctacgccatccagccctcactcctgccgcccagccctcactcctgccgcccagccctcacctctgctgtccaggcatcacccttgctgtccagccgacacctacgatgcgcagtccatgtctccgctgcccaggcctcatctatgccacttagccctcacccatgccatctagccctcactcaagccacccagctctcacttcctccatccaggcatcattcctgccacccaggcctcatctacactgcctagccctcacctcccctgtccagcccgtcctcacctacactgcacagccctcacctctgccacccaggcctcatctatactgcccagccctcacctcccctgtccagccctcacctccccggtccagcccttgcctcccccgtccagccctcacctccatcatgcagccactgtctctgctgtccagtcctcacctatgccacattgtccgcatctacactgtacggccctcccctgtgccatccagctggcatcttctatgtaacacaacaagagctggaagagaagaggccctggtccctgggcgtggaggcgcagagccacccaggactgcaaaagaactcttaacggccaaccatggaactgggtgttgatatcccatggaacttgctaaactaggtgagcagaagagcactccaggccacccaaactgcgcggagaatccaggcacaaggaagtgctaagcagagccctcatgggctgtggggagtgggtggaggcactgccaacagggcaggagggattgagggaatgtccctgagccgccatactggggaggtgtgatctgggagcagagagccatggttggttacggagagtggcacaaacacggtgccagcgtccagcactgacagtcaggtggcgtggcagtcaatgcatggcccagatgggagactgaggcttgaactaagtcagtaatgagaaggataagctgaatataattcagaatactttcacaatttaggcaaaatttttttaaaaagtttccagttcactttgaggtttctacctggaataagcggatggtgatgtcattcaccgagatggaggcaaaagtttcggtggaaagataagatacctgggccaggcgcggtggctcacacctataatcctagcactctgggaggctgaggcaggcagatcacctgaggtcaggagttccagaccagcctggccaacacagtgaaaccccaactctactaaaaatacaaaaaatagccgggcatggtggcgtgcctagtcccagctactcgggaggctgaggcagaagaattgcttgaacccaggagacagaggttgcagtgagccgagatcgcaccactgcactccagcctgggcgacagagtgagactcagtctcaaaaaaaaaaaaaaagaaaagaaaagaaaagatatctagttctgaatatgatacaattgctactgttagttattcaagcgcataatgatctcccactactagcttggagagagggattgctttccaggtgacaaagcattgtcccctcccaggccaagagaaatgctcttgggtacagcaatagccctgctgagaaggggctggtctgaaggagtttcatgggaacctggttttcttgtctcgcttttacctatggtgtctttttccaccataagttccactcatccctgtggcctagtccacgggtcctcttttccatggtgccgcagagatgctccaggcagacgcctgctctggctgagacccgggccagctgcccctcctggctgctctccatcctgagatgcgcctgctcctttgtccccctgggagacacttgtacccccagctctgatcccagagcctggcctgctcctccttccacacatacgagcctgagaccccgctcacatgggaggcatttctcagtcacctccgcccagttacagcgagaaccgtgtggtcagagttgcatcttcctgagttgaatctggaaaatgcacgacctacttgtttaatgatgtaaaaacatgtgcttggatctgatctccatcactgaaccttaaacgcagagtcttccccttctgtctcctgcggctcataagtgccttatacttacatgatctgaggcaggttatcaaacgctcatgttctacctgctcctgagctctaggccaaaataggaatattaagagagccaagcatttgcttgtgctcatgttttgaaccatccagcccctcaccagtgccttcttccatttagctgacgtgacaatggcaggaaaccagcactccgcagcccatgcctcccaccaggatgctaccttgttggcgtccccatccgctctcaaatgctcacactcatataataaatacacgctacttaaaaaaaagaatggcttctttaaaaaccgcaaaggccagccgactgcagacagcctctgaagagctgctttccttgaccccccaaggctataaaataaatgcaatttgaataggaagtctgttcaaattcaccagctcctctgggaataatgaagataaaacccaagccttgatccctgtgttcgcaaaatgactcaaaaaaaaaaaaaaaaaaaaaaagaattgacatcatttaaaggactctgaggcttaagagtccaactctaaagtacacccactccctgaggacgcagagcaaatgcaggaaatcacgcccttccaggtgcaaaacaaatcagatcttgtccctctcacaggcatcaaaacacaaatcatcagttcccgacagaaacaaatcctgccctgccaagccaacagaaaaacactggagacagaaatgagctcagagaagggccgagggacaatgacaaggtggggaccctggacccttgggctccgctagccttccccacagcttgcagaagagggctcagctcctccattacagaagagacaaaatacagggactgcttccatcaaatcccccatcatctcactctgtctgtctgcagaagctgtcaggcctggctgggtgctgcctgtctcaggctcttactgcagagcttgtttccagagggccagaggccgtcctgtgtctcctttaatgcctgcgggggacgcagaggccactgagtctaggatcaggactgcgacacctactttctcaccgtcccatctgcctggtaaacctttgtctctctctgaacattctgcatttcagactgtcttgtagacaccatgaagtgaggttttggtttgagccaatttgaaaatctcttctttaaatgggcgagtaaagccgaatattcacaggcattgatacagctgttttttttttttttgtaaattatgctgacaatatggttattctaaggattaaatatttcacgtgttgaacacaatgcctggcacatagtaagttctattttaaatgtatattgaataaaacataaataggacgttaatgtgattaagacaaacagagaaaaggatttaaagagagaagaggccaggagacgcgggagaagacaatgctaacaggttgtcttaacaacacatggaaagctcctcactgcacagcccccagatgcctcactccacgagtgaaatccctgcacggcaggccgagagcgtgggtgcagcagtctgcctgacgtgagagccatgtcatcacatatctagaaggtaagggtacctccggttctggaacacacaatgtaggcacatttcgctgggggctccatgtacatttctaaatagataccagtgcagggacctggctaccctctgataagaaggaagtgaggcctgacagaaactgaccttccagtaacctggaagagactgctctgacggagacaggagatggctgctctgtgaatacacccaaatctcctagggcaggaggggcaaagtcaccgttctaggacacacctgtgaccacaccaggcctccaacaacggagcagctggctaaggaacgatgtcctggggctctggtcacatggaacagacccagtctgagctagagacaccccccaggcccaccaggcatcagcgtgggctcctgccatgcgtggagctcttcgtcttgacagggtccctgcgccaagaaggcaacaggctccgaggggaaaactcgagcaagagagtcccctgaatcggtgccatctgtctaaattccaagtatgcctgcctgatctaccagggcactgaagagtttaatagagaaaaaaaaaaacaatctgtgagctttatcccaagcacaaaacagccactcaggcgtgggagagctcctttctccccgtgtacgccacatgcactcactctacagggaccacaacatccaattcacaggcatggaggggaaacagcaaaataaacagacttcactttggagttgttttttagaaagctgcagtttgtgaatttctcttgctttttaaaacagaatatttccaaaacttgggcatcaatgcttggtctttttaggtgggggatagaagactgggccatcttcacagactctcagaccccggctctcggcggccccatttgccagccagacttcctgcttgggggacggctgctcccccggctcggtgcagttttgcagctgctggtcttgcttagtgaggcacagttctatctgaccaattgtctgtacttcctcatcctggcttggtggaaggcactggattttgggtatcactccatatactctggcaagggcatctttaaaatctgcaacttggtagtaattgatggatggttttatccccaattttagaagcacactgttgaggtccagctccctgtagagttccaggcttctgccaaagtacttcttctgggagttgagcgcatccacctgggcggcgcaggtcccatgcttttcccactcatgcttccagaagcggctgcgattgggaaacgagtgaattacgtcaggccagtatgccctcatttctggcaaaagatccttaatctcttctaaattgaagggccacgatctattacatccttcacttttatcgggccatagtccatgtattgtccagtaatccggagggtctctacagtcgttttgaattttctcgcatactgtctcaggccagtgctgaaccataattagttttttccactcatggttgtcacgcaggcgcttgtccgcaccgcccaggcaaagcaacgccaggcagaggcagcccagcagggccccgcgcagggctgcagggcgcatggtgccgacctgcggagagaacgctgccagctgccgctccggctcccacttcccacctgctgcccgaggaagacttccgggagaaacgctgtctccgagcccccgcgccgccgcgctccctccgctgcagcagcggccaccgggtgcgcccggagccctgggacggcctaaaccagtatctcgcgggccccgcgccgggctccgggaatggccgcagcagccctggcgacccgggcccctcggagctccccttcaggatcgtgcaccaagcgcgcacgtcccgggctctgcttcgcgacccacagcgaccccagctcctccacgctgcagccgccgtccgcccacgaccacggtcagtcgcgttgctc

SEQ ID NO: 13447 - RNA, 5219 nt, Homo sapiens
  source 1..5219: mol_type = other RNA
gctgggattacaggcatgagccaccacgcccggcctggtctgtattaactatatgaccataagctatcattcagaataattttattcagagtaaaaaagtatcatcttgtgagaaagccacattttaaaagattagaactactattacttaacctaaatctgttaagaagaataaaatctgatgcttttcaataagaagccaaaatgcaatacttacatatccagttaaaaggagccagtcaagttgttcccttggttttgcaatgaaacaagcaaatcaatcttttcgatgttctggttggtgtttatagaggatgccagtggagaattctctggcatttgctgagaaagaagtgttgtcacaggtggctggccctcgttttgtggttggcctggctgacttatggccatcaactgatcaggcaatgtagctggtccagaggttaaaagctgactacagttattttgaatgccaaataagaacattcctgatgtctgctgagatgagccaggagaattctgcagttggttcattgtgcctcctgctgtgttgtgaaataaagtagcctgtggttgaggcgaagatgtggctccttgaattccaggcatgttgttctgaggggaataaagaggagactgttgcatatcttgttgatttatactggtctgcaaggcagacatggatgctggagataagaagagagttacttgctgctcttgagaactaggtgacccttgtaccaactgaatctgaggagagctatggaacaagggggtctgtgatgattccgactgggtaggacctgggttctgaagtgaggaaactgtggactgactctgaaattgcatgggctgttgctcttgattcattggggccatgttactttgttggtgaaaaattgactggttctgttgctcctgattagccattggattttgatttgggttgaatatcatgtttggtggtggttgctttggagacgccattgtagccatggtattctgattactgaataaaatgctctgttgttgttgctgctgctgttgctgctgctgttgctgctgctgctgctgttcctgggatggagagttactctgcatggcaactattgagtgctgtgactggaacatggttccttgttggctttgaggcattggattaggtggaagggagcccagggccacctgaggctgaaataaaccctgctgcgggggttgtgcctgttcttgggaaagcataggagtctggatgtgtgatattggagcttgctgttggaaagcagcttgttgttcactgtttgatgttgactgaagtggagaaattgagttcggtgctgcaaaaaatgcttcttgggctactgtgttagtctgaagattattcatgggactctgggaaagaaatatgttggttgactgctggtcttgaggaactgaagagccctgtaacacagcaatggtactttgagagtgaaacattggaggctgcatttgttcagaggaggttgtagaagtctgactgtggacaataggatttggactatgaaagagagaaccttgagtttcctgggaaaggttctgagcatcggcaataggattttgaggatgaaaaagttgggcctgtgaatgagaagactgctgcaaaaaatttccagattgaagtgacatcatctcattcccttgctggaataaaccattaccttgttgttgggtaccactattctgaacactcatcatactttttgtggatgaaaaaaggttaacttgaggttgattgtccccactatgttgcatttggaccatggtctgaaagacactgttctgaatctgttttgcttgtgttccagtttcttctccatctcctgaacttgatgtctgaaacatggtagtgccaggggttgcaacctgctgtgtggtagttgtagaagtttcatttccagaaactgcaggaggagaagaaaacaattcacactgcatttgcatatcctcattggtagacaatgcactcatcatgtgagaagtctgctggtaaactggcgattgctgaaggtttccatttgctgaagcagttgaagggaataactctgactgaatctgggcagctgcctggcagatactctgttgcatctccatcaccattgcggctgaagattccatcacttgctgttgctgctgctgctgctgctgttgattagataacgtgttttcagactgtggatgaacactttcagctcttccaggtaataaattatctggtctggtatggactgttggctctgttgaggaaaacattccagggcttacaccactctgaatttgactgacttgttgaaaaatatctgcactaagctgctcttgaacattctcattaccatctggagcagaaaataaaactgaagataactgctgctgtgcctctaaaacttgttggaccaagtcaacacttccactgctgccactagcagtactgcctgtgaaactccctgcttgcagctgctgaatagtattctgaagctgactcacactatttggtgatggaaaaatatttgatgaaatctgctgctgtaaagtctgtgcttgttcttgtagtggtgactgctgctgttgttgtgatgcctcagtcagttgtgacaaattaaccactgtaccatctgactgtaatatctctctagactgagtttctcttgtctgaaactgtgtagcctgctgcaatagtgcatcgctgttgggcagctgactagaagcagaaactgctggaaaagtaccaggctgtgagatgtcctgggtttgaatagttgtcagggtctctgggttgtatgccttgggctgaatctgctgctgtttttcattttcagaaggtaggtgggaagatgatggtgatgaaaaagagccatttcctgctatgtttgagatgttttctaatgtttgctgagttgatccaacagactttgtagtcttaaaaatagtggaagatcttttttctgctgttacttccattggagtaacatcttcactcttaatcatactgcttggtatgagtggagtcatcagggcattagggataatatttaccttatctaaattacatccagtagttttcattgctttcatggcctcttcaaaagagcaaggtcttgctggactagatatttccttcttcacatttacattcaaagcaccagctgctgctgggtctggagtgtaagtgaatggttgaacatcatgagatcttccagcatttgtcactacatatattcccactgacacaggcaaagttatatgttggtcatgatagggaggaaccttcacaataagatgattctgatgaaatagttccatatcaatttcagcttctgacttccaagagttttcatcagaaacattttcttggaaaataactttagttcctttcagaaagttcttgccgattaaaaacacttcttcttctcctttcactgaacagctatgcaagcttttctttaagatttctggcactcctgctggctgagtacacaaaattggagaagagggtgtttgcagtgtcaaagtggagccatctttcctcatgatattaactcgaaaaaccaatctggcacgagtgcttttcttcttggaaccagcaattcctattctggcttcgacatcagcattcctcaatttcaatatccctacgcagtccaccgccagtgtcatgttgttgctaggatcaaggccgacttctataacagtagtgccttcaatgtccacttctttgcaaggagttgtatttcgtccagttactctgcaggcctgataaaatccatgtggtttcactcgtccagagtcgttgcccacaaacacttgcaacactacaggttcattatggccttccagctttactgtaggaaagccttgctgtgttctatctttcactgagccacggctgccctcagtcaggtaccgagctcggtgctgtgtctcaggttgtacaactatcttcagctcctttccctcacttttaacaggatattgtccacacaacatagggctcttctttactccagttcctttttggttttccaatgttccatttcccgcttttgagttgcctttgttgtccgtggtaagctgagaaagcacatagtgaggtgctttggcactgtcggcatcaaatatatccatattagattcttcacaatctcgtcgtttgacccccggcctctgctttggatttcgttttcgtgatttacgaggtacctcagtgttatcattgtaggaactggtgctcatgttactgaagttggagggggaatcctccatccacatactgcagctctgctcagattccaatccacacccctcatcctggcaggacatccgactgttatccagcaagtcctcaggtggtggtgagatgtacaagactgtgtgcctcttcggtgttgatggatgctgctgaactgtgttactggttaactgcttttcacttacccctctgttacttacccccacggctgaggagcagctctccacttgcatagccttgctgtcggtgactgaggtagaataaatggtagggctggaagaggtggtaaaggagctgcaagcaccgcccatggaggaagaggagggagctgaagaagcatctatgaagcagagaactacaggtcatttttaatgcagacactccctgcttcagaggcaaatccagcagcaacaacagctggaggaggcgagcctgcctcaccaccgcttgtctgactcattgatgctacagatgtttctctagatggaggtaactgtaactcctttgggagaagatcatagacagattctcgcgagtagagggacttgggcgattccaggtctaggtccgcgctgagcaatgagatgaagtccgagggcatcgcagctcgacccagcccggcccgagggcagcgggagggggggagcggcggtggcggcggcacctcctctccgggaccgcgggcaccgaaccgggggcggcgacgcgagggcggctgccgctgcctcctcctcgagggtagtgacttccactgggccgaggaccgaggaaacgatggcgaggtggagggggaactccacggggactgattctcggtgaccaggagaggggttcaggacggggaaggggaagggggagagccaaagggtccgtttcgtgtttctcctcagcgaaaactgacggtcgccgccaccgccgccgccgctgacaggaatct

SEQ ID NO: 13448 - RNA, 2272 nt, Homo sapiens
  source 1..2272: mol_type = other RNA
gctgggattacaggcatgagccaccacgcccggccttttgtattttcaaacgtccagcagcaccactggttgcgcacctcatctggagggaagggagggcctggaggacagatttacgttgattaggcctaactcacaggcaggagatggctctgtggactggggaggggagctaaggaactgcttgaaagggcaggggctaagacatttgtaatccatgaaaatgctggaagcattccctgcagaggaggggctcaaaaccagggaggccttcggtggacggacacatcatggccttgccacgcctctgcagtcctttgcacaaagtggctgaggccacaggcatggtggccacacaggctccgtagcctattcacccccaccagacccttccagcagcatggacagctgggcgcccatctttccaacagcgaggatggtgtctgagccctgatgtggcaccaccccctgtggggagggcagccagcctccaggaagcaggcagagcacacggcgtgccttttgtcgagagccagtccttgcagggatggatcctcaaagggacgggtcctcgcaggcttctcccgccagcatgccatccttggcctccttcgctgccttgggattccacaaatgacacttgtaatccagggccttgtttcagaggaaaaccagtgtggcgataagcttgtgtccatcagttccactggtctcactccacgcccttcacctagaagcaggaggcctaacagactggtggaatggttgcagcggggagactgcaccccttaacactgagatgcaggcctgtggggggcagaacaggcttctaacctgggaccgacctaggaggccgtttccccaccgccagaatgccgaactggaggtggccatgcctgtgagagggcttctgtggacggacgccagtcacggccttgccacgcctctgcagtccttacacagagtggccgtgacagctaatcggctatggagggatttttctttcccactctggtaaggtggggtcgcaggagtggcagtcctggctcccggtcctctggggaacgtgggtctgcttcccaaacacaggagcagagatgccctctggccatgtggggccgctcactgccgagctgaccgctggagaagggagctccgcgggccagagatctctgcagaggaatctcttcggagagatccctgcaggagggtgggaatgctgcctcaggtgaggaggaagcactgtgtcaaaacccagggattctggggcactgctcgatattcccatgtcacctaataaaggtccgtggaaaactagggcagctcccacagacagagctgtgaggctcagagccggcctgagtgaggactcgggtcgaggtgcctggtagagaccccagcctaagcgtggcagagggagaagcacatcggatgtgtggggagacagaagctgttacgggtcgaattgtgtcccctcgaattcatatgttgaaggcctaacccccagggcctcagaatgtgaccttgtttggaaatagggtctttgcagatgtgatccatcaagttagggtgagtcatcccgggagtgtgggcccctgatcctgtgtgactgtgtccttataaagacgggaaatttggacacagctcgcagggagaataccatgtgaagattcgggcagagattgaggcgctgcctccaccagccaaggaacagcaaagatggcctgcaaaccccacgagagtggaggagaggccaggttccccacaactgcctcagacccaaccagccctgtggacagctggagcctccagaactgggaccacacgctgctgctgttcacgccccgttggaggcacctccttacagtggccctagcacaccaacgctggagctgtactcaccagtgcgggcccccgacccgctcctgcgttgcaggccggcaatgccccgacccaggagctctgtcctgaggtccatgctgcagagttccttgctgtgccctcctccagctcaagggacatggcccctcagcacctagccccttccgtctaggttgctgcccacacaggcctgagcctgcttcccagacggcaggcctcttcctggggtctgcctcctgggtggacgccgccgctgcgtgcacacatctaggctcaagtggtggctgttggtggtgggcagtggacagagcttggtcgtcaggctggggttttgacatgcctctgggagagcctccatggtgcagggatgaggagtgggccagccgcagca

SEQ ID NO: 13449 - RNA, 225 nt, Homo sapiens
  source 1..225: mol_type = other RNA
gctgggattacaggcatgagccaccacgcccggctaatttttgtatttttcgtagagacgggggtttcaccatcttggccagacttgtctcgaactcttgaccttagatgatgcacccgcctcggcctcccaaactgctgggattacaggggtgagccaccgcgcccggccgcttcccagggacttttaaggacacgcacagccgttgagaatatgcgagatggc

SEQ ID NO: 13450 - RNA, 6075 nt, Homo sapiens
  source 1..6075: mol_type = other RNA
gctgggattacaggcatgagccaccacgcccggctaattttttgtatttttagtagagacagggtttctccatgttggtcaggctggtctcaaatccccgacctcaggtgatccacccgccttggcctcacagaatgctgagattacaggcgtgagccaccatgcctggccagtcttatttttttaaataagtttattctggagggaggtctattaagattttacacctccagttaattctgatgtcgtcaacttattaaaaatcacagactttttccagattttcagatatattataaaaatgtctataataccaacttttaagtttgttgttttaatttttttttttttctgtagagatgaggggagggggatctcattatgttacctagactggtcttgaactcctggcctcaagccattctcctacctcagcctcccaaagtgctggaattacaggcatgagccactgcaaccagccttaagtttttaaattgagatcaaattcacacagcataatattcacccttttaaagtgtatagttgagtgacctgtagtatataaacaaaattgtacaacctttacccatgccacattttcattaccccaaatgacacagttcttttaagtttacatatatagccatttcaatttctcatatacaatattgtttatttgtcatccttatttcacctctggaatcactaaactttgtctcattttttttctcttccatcaaatatcaattttggattcagatccagtttttttctttcaattatttctgccttttaaaataatactacctccttcctcccacaattcatttcagcttgttttagttccttgggttctatattttttcttcctagtattacaatatatgcacaaatattaggttataaaacttccaatacaacttttactgccactcacaggtttttcaattgttttcattttcatgtacatttaaataatgtatatattagggatttattccttaacccatgttaattaagagggaatattgaattaataatcagatatttgatggttatcctattgtactgcttcttctggtcaaataatgttgccagtatgttttctgcattttggggggaaatattagaaaaaattttataatctcttcctgcttttttgacagctgtgctttctactactcatcatattttcagggtttcagattggtaaccgtttattttttattttgtaagacagagtctcgctctgtcacccagtctggagtgtgcagtggtgcaatctcagctcactataacctccaactcccaggttcaagcaatcctcccacctcagcctcttgagtagctaggattacaggcatgcaacaccatgcctggctatttgtttttgtttttgttttttttgtatttttagtagagacggggtttcaccatgttggccaggctggtctcgagctcctgacctcaagtgatccacccaccttggcctcccaaagtgctaggattacaggtgtgagccaccgcgcccagcctcagactggtattctttatgtagcataaaagataaagtctgaacaaagactatgcacacatactttttctcttccttttaaaattccacactgaataataatgatagggaaaggcttcgttatactcattacaagtgtttctctttttccaccatgaattacaaatttgccaaaggtaaacaacatggttaaaatcctttccataaatcctaatgaagatacttatgataatgagtatatcactgataatagtggaaaacttttactaaacctgtattatgtgataacagtttgaggtactttgcatttattaattcattgactcttcacagcaatccaatacatacagccttattatagatgcctagacataattttttaaaataccactaacagccaggggcggtggctcacacctataatcccagcactttgggaagccaaggcaggaggatcacgaggtcaggagtttgagagcagcctggccaatatggtgaaaccccatctctactaataatacaaaaattagctaggcatggtggcgcgcgcctgtagtcccagctactcgggaggctgaggcggaagactcacttgaactcgggaggcagaggttgcagtgagccgagattgcaccactgccctccagcctgggcaacagagcgagactgtgtctcaaaaaacaaaaacaccactaatagctataagaaaaaataattgaccgggcacagtggctcacacctgtaatccccgaactttgggaggccgaggtgggtggatcacaaggtcaagagttcaagaccagcctggccaacatagtgaaaccctgtctctactaaaaatacaaaaattagccaggcatggtgtcgtgcgcctgtagtctcagatactaggaaggctgaggcaggagaatcgcttgaacccgggaggcagcagttgtggtgaactgagattgtgccactgcacttcagcctgggcaacagagtgaactccatctcaaaaaaaaaaaaaaacaaacaaacaaaaaattaatatctggattgataaataacactttcataacagtgttactttctagtatggcattgggattaggattgatgtaagggaacaaaacagctcacaaggagaaaatgtagataattttagcaattaaaataaatgttttaaaagtaaaaataagcatccaatgaggtcagcagtttttgtgtttttttgagacggaatctcactctgtcccccaggctggagtgcagtggcaccatctcagctcactgcaacctccgcctcccaggttcaagcaattctcctgtctcagcctcccgagtagctgggattacaggtacatgccaccacgcccagctaagtagagacggggtttcactgttagccaggatggccttaatcttcagaccttgtgatccgcccacctcggcctcccaaagtgctgggattacaggcatgagccactgtgcccagccgaggtcagcttttatagctgcaaaaatttagtggcaaccataatgggaatagtcattttaaagtcattaaatatgtcatgaaaataataaaaatctatatttactgaaatggcactcatgaaatctttggcatgataaaagcagttaagggtacagcatgcatatcataattacactttcttaaaaaagcaaagtatagcacgattttctctaccaaattgagagcagccatctataagtatgattacaattaattttggctttttagtttgtaattttttgctttgtgattttggcttaacaattaaaaatgtacatttgtaaaataaaaagaccggccgcagtggctcacgcctgtaatcccagcactttcggaggccgaggcgggtggatcacctgaagtcgggagattgagaccatcctggctaacatggtgaaaccccgtctctactaaaaatacaaaaaattagccgggtgttgtggcacatgcctgtaatcccaactactcaaaaggctgaggcagaagaaccacttgaacctgggaggcgaaggttgtgacgagccgagattgcaccattgcactccagcctaggcaacaagagcgaaactccgtctcaacaaaaaataaagccaggtgcaatcgctcatgcctgtaatcccagcactttgggaggctgaggcaggtggatcacctgaggtcaggagttcaagactatcctgaccaacatggagaaaccctgtctctactaaaaatagaaaattagcagggtgtggtggcacacgcctgtgatcccagctactcaggagtctgaggcaggagaattgcttgaagccgggaggtggaggttgcagcgagccgagattgcgccactgcactccagcctgggcaacagagtgaaactccgtctcaaaaaacatataataataataataaaataaaacaaaaagactaacactaacttcaaaaacaaagttaaacctccacaaggaatttaaaaatattaaaggtcacacaattcaaacagtgtgatactggtgcaaacacaaatacacagatcagaaaagatagctctaaaaacacaagcaaatataaacatgagtataatgtgtcaccaagaaagtagaacaaaacaatgaatgaaagaattatagaacagctggcatcggtatatgactgggggagagagggaatgtcactttagactccgaatttataacctggaatgaaatacatttggatacaaaatttaaatacaaagttttaaaaaaaactacggaagagggtaactattagacatgatttttggtttaaaatatgaggaaggtgacaggggctttaatttttattatttattagtatgaattccctgatgacgaatgagatccgagccactactaaaagccttcccacattccttacagttatagggcttttcaccagtgtgaattctcagatgtcgagtaaggtttgagcatttattaaaggcctttccacattcattacattcatatggtttttcatctgtatgaattctctgatgctggaaaagttgtgagttctgagtaaaggccttcccacattcaagacattcaaagggtttctcaccagcgtgaattctctgatgttgacgaagctgtgagctctgagtaaaagcctttccacattccttacaatcatagggtttctcaccagtgtgaattctctgatgattagtaagtgctgagccactactaaaggctttgccacattccttgcactcatagggtttctcaccagtatgaattctctgatgttgaacaagctttgagctctgggtaaaggctttgccacattccttacattcatagggtttctcacctgtatgaattcgtgcatgctgaaaaagttgtgagctcttagtaaaggctttcccacatactttacattcataaggtttttcaccagtgtgaattcgctgatggtcaataagatttgagcaataactaaaggccttcccacattccttacattcatagggtttcttaccggtatggattctctgatgttgagaaaggtatgagctacaactgaaggcctttccacattccttacattcaaagggtttttcgccagtatgaattttcagatgccgagtaacatgtgaaccacaactaaagaatttcccacactctttacattcataagatttttcaccaatatgaattctctgatgttgaataaattgtgagttctgactaaaggcctttccacatttcttacattcatagggtctgtcttcattattaattatttgatggagagtaaggaatgtctgttgaataaatgtgggcatgtattcaggagtgaatatttcttgactaaaatgcccatttggatatcccagttgttttgcaaggtggcttctatattccaaaacatctccaaaactggagtactcaaggccatgctttgtaagtcccattatctccctctggcataattctatttcataaacttccttctttagagataataacttggtttcacacatcgattccagatctgaacacaggcctcttgtaagctctctgccaaccatccagggctctttcccttgttccaataaggagatcacttgaggcttaggagtgtaaagtcccattgaaaccagattgccgtagttctccaacatcacatctctgtataagtccctctgaacagggtccaggcagtcccactcctcctgagagaagtctatggacacatcactgaacatcactgatccctcagccatggcttctagtattgcagatggttagtcttccttgaggccgttctcagaggtatctaaggtagtcaaactcatagaaacagaaagtagaacagtggctgccaggggctgtaatcccagctactcaggaggctgaggcaagagaatcgcttgaacccggaaagcagaggctgcagtgagctgagatcatgccactgcactccagcttgggcaacagagtgagactccgtctgcgggccccagccgagcctgcaagacccaggccgctcaccgcgcacttcccctaccctt

SEQ ID NO: 13451 - RNA, 6045 nt, Homo sapiens
  source 1..6045: mol_type = other RNA
gctgggattacaggcatgagccaccacgcccggctaattttttgtatttttagtagagacagggtttctccatgttggtcaggctggtctcaaatccccgacctcaggtgatccacccgccttggcctcacagaatgctgagattacaggcgtgagccaccatgcctggccagtcttatttttttaaataagtttattctggagggaggtctattaagattttacacctccagttaattctgatgtcgtcaacttattaaaaatcacagactttttccagattttcagatatattataaaaatgtctataataccaacttttaagtttgttgttttaatttttttttttttctgtagagatgaggggagggggatctcattatgttacctagactggtcttgaactcctggcctcaagccattctcctacctcagcctcccaaagtgctggaattacaggcatgagccactgcaaccagccttaagtttttaaattgagatcaaattcacacagcataatattcacccttttaaagtgtatagttgagtgacctgtagtatataaacaaaattgtacaacctttacccatgccacattttcattaccccaaatgacacagttcttttaagtttacatatatagccatttcaatttctcatatacaatattgtttatttgtcatccttatttcacctctggaatcactaaactttgtctcattttttttctcttccatcaaatatcaattttggattcagatccagtttttttctttcaattatttctgccttttaaaataatactacctccttcctcccacaattcatttcagcttgttttagttccttgggttctatattttttcttcctagtattacaatatatgcacaaatattaggttataaaacttccaatacaacttttactgccactcacaggtttttcaattgttttcattttcatgtacatttaaataatgtatatattagggatttattccttaacccatgttaattaagagggaatattgaattaataatcagatatttgatggttatcctattgtactgcttcttctggtcaaataatgttgccagtatgttttctgcattttggggggaaatattagaaaaaattttataatctcttcctgcttttttgacagctgtgctttctactactcatcatattttcagggtttcagattggtaaccgtttattttttattttgtaagacagagtctcgctctgtcacccagtctggagtgtgcagtggtgcaatctcagctcactataacctccaactcccaggttcaagcaatcctcccacctcagcctcttgagtagctaggattacaggcatgcaacaccatgcctggctatttgtttttgtttttgttttttttgtatttttagtagagacggggtttcaccatgttggccaggctggtctcgagctcctgacctcaagtgatccacccaccttggcctcccaaagtgctaggattacaggtgtgagccaccgcgcccagcctcagactggtattctttatgtagcataaaagataaagtctgaacaaagactatgcacacatactttttctcttccttttaaaattccacactgaataataatgatagggaaaggcttcgttatactcattacaagtgtttctctttttccaccatgaattacaaatttgccaaaggtaaacaacatggttaaaatcctttccataaatcctaatgaagatacttatgataatgagtatatcactgataatagtggaaaacttttactaaacctgtattatgtgataacagtttgaggtactttgcatttattaattcattgactcttcacagcaatccaatacatacagccttattatagatgcctagacataattttttaaaataccactaacagccaggggcggtggctcacacctataatcccagcactttgggaagccaaggcaggaggatcacgaggtcaggagtttgagagcagcctggccaatatggtgaaaccccatctctactaataatacaaaaattagctaggcatggtggcgcgcgcctgtagtcccagctactcgggaggctgaggcggaagactcacttgaactcgggaggcagaggttgcagtgagccgagattgcaccactgccctccagcctgggcaacagagcgagactgtgtctcaaaaaacaaaaacaccactaatagctataagaaaaaataattgaccgggcacagtggctcacacctgtaatccccgaactttgggaggccgaggtgggtggatcacaaggtcaagagttcaagaccagcctggccaacatagtgaaaccctgtctctactaaaaatacaaaaattagccaggcatggtgtcgtgcgcctgtagtctcagatactaggaaggctgaggcaggagaatcgcttgaacccgggaggcagcagttgtggtgaactgagattgtgccactgcacttcagcctgggcaacagagtgaactccatctcaaaaaaaaaaaaaaacaaacaaacaaaaaattaatatctggattgataaataacactttcataacagtgttactttctagtatggcattgggattaggattgatgtaagggaacaaaacagctcacaaggagaaaatgtagataattttagcaattaaaataaatgttttaaaagtaaaaataagcatccaatgaggtcagcagtttttgtgtttttttgagacggaatctcactctgtcccccaggctggagtgcagtggcaccatctcagctcactgcaacctccgcctcccaggttcaagcaattctcctgtctcagcctcccgagtagctgggattacaggtacatgccaccacgcccagctaagtagagacggggtttcactgttagccaggatggccttaatcttcagaccttgtgatccgcccacctcggcctcccaaagtgctgggattacaggcatgagccactgtgcccagccgaggtcagcttttatagctgcaaaaatttagtggcaaccataatgggaatagtcattttaaagtcattaaatatgtcatgaaaataataaaaatctatatttactgaaatggcactcatgaaatctttggcatgataaaagcagttaagggtacagcatgcatatcataattacactttcttaaaaaagcaaagtatagcacgattttctctaccaaattgagagcagccatctataagtatgattacaattaattttggctttttagtttgtaattttttgctttgtgattttggcttaacaattaaaaatgtacatttgtaaaataaaaagaccggccgcagtggctcacgcctgtaatcccagcactttcggaggccgaggcgggtggatcacctgaagtcgggagattgagaccatcctggctaacatggtgaaaccccgtctctactaaaaatacaaaaaattagccgggtgttgtggcacatgcctgtaatcccaactactcaaaaggctgaggcagaagaaccacttgaacctgggaggcgaaggttgtgacgagccgagattgcaccattgcactccagcctaggcaacaagagcgaaactccgtctcaacaaaaaataaagccaggtgcaatcgctcatgcctgtaatcccagcactttgggaggctgaggcaggtggatcacctgaggtcaggagttcaagactatcctgaccaacatggagaaaccctgtctctactaaaaatagaaaattagcagggtgtggtggcacacgcctgtgatcccagctactcaggagtctgaggcaggagaattgcttgaagccgggaggtggaggttgcagcgagccgagattgcgccactgcactccagcctgggcaacagagtgaaactccgtctcaaaaaacatataataataataataaaataaaacaaaaagactaacactaacttcaaaaacaaagttaaacctccacaaggaatttaaaaatattaaaggtcacacaattcaaacagtgtgatactggtgcaaacacaaatacacagatcagaaaagatagctctaaaaacacaagcaaatataaacatgagtataatgtgtcaccaagaaagtagaacaaaacaatgaatgaaagaattatagaacagctggcatcggtatatgactgggggagagagggaatgtcactttagactccgaatttataacctggaatgaaatacatttggatacaaaatttaaatacaaagttttaaaaaaaactacggaagagggtaactattagacatgatttttggtttaaaatatgaggaaggtgacaggggctttaatttttattatttattagtatgaattccctgatgacgaatgagatccgagccactactaaaagccttcccacattccttacagttatagggcttttcaccagtgtgaattctcagatgtcgagtaaggtttgagcatttattaaaggcctttccacattcattacattcatatggtttttcatctgtatgaattctctgatgctggaaaagttgtgagttctgagtaaaggccttcccacattcaagacattcaaagggtttctcaccagcgtgaattctctgatgttgacgaagctgtgagctctgagtaaaagcctttccacattccttacaatcatagggtttctcaccagtgtgaattctctgatgattagtaagtgctgagccactactaaaggctttgccacattccttgcactcatagggtttctcaccagtatgaattctctgatgttgaacaagctttgagctctgggtaaaggctttgccacattccttacattcatagggtttctcacctgtatgaattcgtgcatgctgaaaaagttgtgagctcttagtaaaggctttcccacatactttacattcataaggtttttcaccagtgtgaattcgctgatggtcaataagatttgagcaataactaaaggccttcccacattccttacattcatagggtttcttaccggtatggattctctgatgttgagaaaggtatgagctacaactgaaggcctttccacattccttacattcaaagggtttttcgccagtatgaattttcagatgccgagtaacatgtgaaccacaactaaagaatttcccacactctttacattcataagatttttcaccaatatgaattctctgatgttgaataaattgtgagttctgactaaaggcctttccacatttcttacattcatagggtctgtcttcattattaattatttgatggagagtaaggaatgtctgttgaataaatgtgggcatgtattcaggagtgaatatttcttgactaaaatgcccatttggatatcccagttgttttgcaaggtggcttctatattccaaaacatctccaaaactggagtactcaaggccatgctttgtaagtcccattatctccctctggcataattctatttcataaacttccttctttagagataataacttggtttcacacatcgattccagatctgaacacaggcctcttgtaagctctctgccaaccatccagggctctttcccttgttccaataaggagatcacttgaggcttaggagtgtaaagtcccattgaaaccagattgccgtagttctccaacatcacatctctgtataagtccctctgaacagggtccaggcagtcccactcctcctgagagaagtctatggacacatcactgaacatcactgatccctcagccatggcttctagtattgcagatggttagtcttccttgaggccgttctcatgtctgttgaagtataaaaagggactcagtctcatgatcaacagcttaggaaacttaaatgcacattgctaagtgaaagaagccaattcaaaaagactacatactgtatgattacaacattctggaaaaggcaaaactatggagacaataaaaagattaggagttgacagggagggaggatcagtcagggcacagaggccttttagagcaat

SEQ ID NO: 13452 - RNA, 6245 nt, Homo sapiens
  source 1..6245: mol_type = other RNA
gctgggattacaggcatgagccaccacgcccggctaattttttgtatttttagtagagacagggtttctccatgttggtcaggctggtctcaaatccccgacctcaggtgatccacccgccttggcctcacagaatgctgagattacaggcgtgagccaccatgcctggccagtcttatttttttaaataagtttattctggagggaggtctattaagattttacacctccagttaattctgatgtcgtcaacttattaaaaatcacagactttttccagattttcagatatattataaaaatgtctataataccaacttttaagtttgttgttttaatttttttttttttctgtagagatgaggggagggggatctcattatgttacctagactggtcttgaactcctggcctcaagccattctcctacctcagcctcccaaagtgctggaattacaggcatgagccactgcaaccagccttaagtttttaaattgagatcaaattcacacagcataatattcacccttttaaagtgtatagttgagtgacctgtagtatataaacaaaattgtacaacctttacccatgccacattttcattaccccaaatgacacagttcttttaagtttacatatatagccatttcaatttctcatatacaatattgtttatttgtcatccttatttcacctctggaatcactaaactttgtctcattttttttctcttccatcaaatatcaattttggattcagatccagtttttttctttcaattatttctgccttttaaaataatactacctccttcctcccacaattcatttcagcttgttttagttccttgggttctatattttttcttcctagtattacaatatatgcacaaatattaggttataaaacttccaatacaacttttactgccactcacaggtttttcaattgttttcattttcatgtacatttaaataatgtatatattagggatttattccttaacccatgttaattaagagggaatattgaattaataatcagatatttgatggttatcctattgtactgcttcttctggtcaaataatgttgccagtatgttttctgcattttggggggaaatattagaaaaaattttataatctcttcctgcttttttgacagctgtgctttctactactcatcatattttcagggtttcagattggtaaccgtttattttttattttgtaagacagagtctcgctctgtcacccagtctggagtgtgcagtggtgcaatctcagctcactataacctccaactcccaggttcaagcaatcctcccacctcagcctcttgagtagctaggattacaggcatgcaacaccatgcctggctatttgtttttgtttttgttttttttgtatttttagtagagacggggtttcaccatgttggccaggctggtctcgagctcctgacctcaagtgatccacccaccttggcctcccaaagtgctaggattacaggtgtgagccaccgcgcccagcctcagactggtattctttatgtagcataaaagataaagtctgaacaaagactatgcacacatactttttctcttccttttaaaattccacactgaataataatgatagggaaaggcttcgttatactcattacaagtgtttctctttttccaccatgaattacaaatttgccaaaggtaaacaacatggttaaaatcctttccataaatcctaatgaagatacttatgataatgagtatatcactgataatagtggaaaacttttactaaacctgtattatgtgataacagtttgaggtactttgcatttattaattcattgactcttcacagcaatccaatacatacagccttattatagatgcctagacataattttttaaaataccactaacagccaggggcggtggctcacacctataatcccagcactttgggaagccaaggcaggaggatcacgaggtcaggagtttgagagcagcctggccaatatggtgaaaccccatctctactaataatacaaaaattagctaggcatggtggcgcgcgcctgtagtcccagctactcgggaggctgaggcggaagactcacttgaactcgggaggcagaggttgcagtgagccgagattgcaccactgccctccagcctgggcaacagagcgagactgtgtctcaaaaaacaaaaacaccactaatagctataagaaaaaataattgaccgggcacagtggctcacacctgtaatccccgaactttgggaggccgaggtgggtggatcacaaggtcaagagttcaagaccagcctggccaacatagtgaaaccctgtctctactaaaaatacaaaaattagccaggcatggtgtcgtgcgcctgtagtctcagatactaggaaggctgaggcaggagaatcgcttgaacccgggaggcagcagttgtggtgaactgagattgtgccactgcacttcagcctgggcaacagagtgaactccatctcaaaaaaaaaaaaaaacaaacaaacaaaaaattaatatctggattgataaataacactttcataacagtgttactttctagtatggcattgggattaggattgatgtaagggaacaaaacagctcacaaggagaaaatgtagataattttagcaattaaaataaatgttttaaaagtaaaaataagcatccaatgaggtcagcagtttttgtgtttttttgagacggaatctcactctgtcccccaggctggagtgcagtggcaccatctcagctcactgcaacctccgcctcccaggttcaagcaattctcctgtctcagcctcccgagtagctgggattacaggtacatgccaccacgcccagctaagtagagacggggtttcactgttagccaggatggccttaatcttcagaccttgtgatccgcccacctcggcctcccaaagtgctgggattacaggcatgagccactgtgcccagccgaggtcagcttttatagctgcaaaaatttagtggcaaccataatgggaatagtcattttaaagtcattaaatatgtcatgaaaataataaaaatctatatttactgaaatggcactcatgaaatctttggcatgataaaagcagttaagggtacagcatgcatatcataattacactttcttaaaaaagcaaagtatagcacgattttctctaccaaattgagagcagccatctataagtatgattacaattaattttggctttttagtttgtaattttttgctttgtgattttggcttaacaattaaaaatgtacatttgtaaaataaaaagaccggccgcagtggctcacgcctgtaatcccagcactttcggaggccgaggcgggtggatcacctgaagtcgggagattgagaccatcctggctaacatggtgaaaccccgtctctactaaaaatacaaaaaattagccgggtgttgtggcacatgcctgtaatcccaactactcaaaaggctgaggcagaagaaccacttgaacctgggaggcgaaggttgtgacgagccgagattgcaccattgcactccagcctaggcaacaagagcgaaactccgtctcaacaaaaaataaagccaggtgcaatcgctcatgcctgtaatcccagcactttgggaggctgaggcaggtggatcacctgaggtcaggagttcaagactatcctgaccaacatggagaaaccctgtctctactaaaaatagaaaattagcagggtgtggtggcacacgcctgtgatcccagctactcaggagtctgaggcaggagaattgcttgaagccgggaggtggaggttgcagcgagccgagattgcgccactgcactccagcctgggcaacagagtgaaactccgtctcaaaaaacatataataataataataaaataaaacaaaaagactaacactaacttcaaaaacaaagttaaacctccacaaggaatttaaaaatattaaaggtcacacaattcaaacagtgtgatactggtgcaaacacaaatacacagatcagaaaagatagctctaaaaacacaagcaaatataaacatgagtataatgtgtcaccaagaaagtagaacaaaacaatgaatgaaagaattatagaacagctggcatcggtatatgactgggggagagagggaatgtcactttagactccgaatttataacctggaatgaaatacatttggatacaaaatttaaatacaaagttttaaaaaaaactacggaagagggtaactattagacatgatttttggtttaaaatatgaggaaggtgacaggggctttaatttttattatttattagtatgaattccctgatgacgaatgagatccgagccactactaaaagccttcccacattccttacagttatagggcttttcaccagtgtgaattctcagatgtcgagtaaggtttgagcatttattaaaggcctttccacattcattacattcatatggtttttcatctgtatgaattctctgatgctggaaaagttgtgagttctgagtaaaggccttcccacattcaagacattcaaagggtttctcaccagcgtgaattctctgatgttgacgaagctgtgagctctgagtaaaagcctttccacattccttacaatcatagggtttctcaccagtgtgaattctctgatgattagtaagtgctgagccactactaaaggctttgccacattccttgcactcatagggtttctcaccagtatgaattctctgatgttgaacaagctttgagctctgggtaaaggctttgccacattccttacattcatagggtttctcacctgtatgaattcgtgcatgctgaaaaagttgtgagctcttagtaaaggctttcccacatactttacattcataaggtttttcaccagtgtgaattcgctgatggtcaataagatttgagcaataactaaaggccttcccacattccttacattcatagggtttcttaccggtatggattctctgatgttgagaaaggtatgagctacaactgaaggcctttccacattccttacattcaaagggtttttcgccagtatgaattttcagatgccgagtaacatgtgaaccacaactaaagaatttcccacactctttacattcataagatttttcaccaatatgaattctctgatgttgaataaattgtgagttctgactaaaggcctttccacatttcttacattcatagggtctgtcttcattattaattatttgatggagagtaaggaatgtctgttgaataaatgtgggcatgtattcaggagtgaatatttcttgactaaaatgcccatttggatatcccagttgttttgcaaggtggcttctatattccaaaacatctccaaaactggagtactcaaggccatgctttgtaagtcccattatctccctctggcataattctatttcataaacttccttctttagagataataacttggtttcacacatcgattccagatctgaacacaggcctcttgtaagctctctgccaaccatccagggctctttcccttgttccaataaggagatcacttgaggcttaggagtgtaaagtcccattgaaaccagattgccgtagttctccaacatcacatctctgtataagtccctctgaacagggtccaggcagtcccactcctcctgagagaagtctatggacacatcactgaacatcactgatccctcagccatggcttctagtattgcagatggttagtcttccttgaggccgttctccgatcactggagatgactctcactccataccctgcccctttgccttatacacaataaataacagcgcgaccaggcattcggggccaataccggtctctgtgtcttggtgatagtggtccctcaggcccagctgtcttttcttctatctctgtcttgggtctttatttctacaatctctcgtctccacacacaaagagaaaatcccacaggccctgcagggctggtatcgcctgtaatcccagctactcaggaggctgaggcaagagaatcgcttgaacccggaaagcagaggctgcagtgagctgagatcatgccactgcactccagcttgggcaacagagtgagactccgtctgcgggccccagccgagcctgcaagacccaggccgctcaccgcgcacttcccctaccctt

SEQ ID NO: 13453 - RNA, 6033 nt, Homo sapiens
  source 1..6033: mol_type = other RNA
gctgggattacaggcatgagccaccacgcccggctaattttttgtatttttagtagagacagggtttctccatgttggtcaggctggtctcaaatccccgacctcaggtgatccacccgccttggcctcacagaatgctgagattacaggcgtgagccaccatgcctggccagtcttatttttttaaataagtttattctggagggaggtctattaagattttacacctccagttaattctgatgtcgtcaacttattaaaaatcacagactttttccagattttcagatatattataaaaatgtctataataccaacttttaagtttgttgttttaatttttttttttttctgtagagatgaggggagggggatctcattatgttacctagactggtcttgaactcctggcctcaagccattctcctacctcagcctcccaaagtgctggaattacaggcatgagccactgcaaccagccttaagtttttaaattgagatcaaattcacacagcataatattcacccttttaaagtgtatagttgagtgacctgtagtatataaacaaaattgtacaacctttacccatgccacattttcattaccccaaatgacacagttcttttaagtttacatatatagccatttcaatttctcatatacaatattgtttatttgtcatccttatttcacctctggaatcactaaactttgtctcattttttttctcttccatcaaatatcaattttggattcagatccagtttttttctttcaattatttctgccttttaaaataatactacctccttcctcccacaattcatttcagcttgttttagttccttgggttctatattttttcttcctagtattacaatatatgcacaaatattaggttataaaacttccaatacaacttttactgccactcacaggtttttcaattgttttcattttcatgtacatttaaataatgtatatattagggatttattccttaacccatgttaattaagagggaatattgaattaataatcagatatttgatggttatcctattgtactgcttcttctggtcaaataatgttgccagtatgttttctgcattttggggggaaatattagaaaaaattttataatctcttcctgcttttttgacagctgtgctttctactactcatcatattttcagggtttcagattggtaaccgtttattttttattttgtaagacagagtctcgctctgtcacccagtctggagtgtgcagtggtgcaatctcagctcactataacctccaactcccaggttcaagcaatcctcccacctcagcctcttgagtagctaggattacaggcatgcaacaccatgcctggctatttgtttttgtttttgttttttttgtatttttagtagagacggggtttcaccatgttggccaggctggtctcgagctcctgacctcaagtgatccacccaccttggcctcccaaagtgctaggattacaggtgtgagccaccgcgcccagcctcagactggtattctttatgtagcataaaagataaagtctgaacaaagactatgcacacatactttttctcttccttttaaaattccacactgaataataatgatagggaaaggcttcgttatactcattacaagtgtttctctttttccaccatgaattacaaatttgccaaaggtaaacaacatggttaaaatcctttccataaatcctaatgaagatacttatgataatgagtatatcactgataatagtggaaaacttttactaaacctgtattatgtgataacagtttgaggtactttgcatttattaattcattgactcttcacagcaatccaatacatacagccttattatagatgcctagacataattttttaaaataccactaacagccaggggcggtggctcacacctataatcccagcactttgggaagccaaggcaggaggatcacgaggtcaggagtttgagagcagcctggccaatatggtgaaaccccatctctactaataatacaaaaattagctaggcatggtggcgcgcgcctgtagtcccagctactcgggaggctgaggcggaagactcacttgaactcgggaggcagaggttgcagtgagccgagattgcaccactgccctccagcctgggcaacagagcgagactgtgtctcaaaaaacaaaaacaccactaatagctataagaaaaaataattgaccgggcacagtggctcacacctgtaatccccgaactttgggaggccgaggtgggtggatcacaaggtcaagagttcaagaccagcctggccaacatagtgaaaccctgtctctactaaaaatacaaaaattagccaggcatggtgtcgtgcgcctgtagtctcagatactaggaaggctgaggcaggagaatcgcttgaacccgggaggcagcagttgtggtgaactgagattgtgccactgcacttcagcctgggcaacagagtgaactccatctcaaaaaaaaaaaaaaacaaacaaacaaaaaattaatatctggattgataaataacactttcataacagtgttactttctagtatggcattgggattaggattgatgtaagggaacaaaacagctcacaaggagaaaatgtagataattttagcaattaaaataaatgttttaaaagtaaaaataagcatccaatgaggtcagcagtttttgtgtttttttgagacggaatctcactctgtcccccaggctggagtgcagtggcaccatctcagctcactgcaacctccgcctcccaggttcaagcaattctcctgtctcagcctcccgagtagctgggattacaggtacatgccaccacgcccagctaagtagagacggggtttcactgttagccaggatggccttaatcttcagaccttgtgatccgcccacctcggcctcccaaagtgctgggattacaggcatgagccactgtgcccagccgaggtcagcttttatagctgcaaaaatttagtggcaaccataatgggaatagtcattttaaagtcattaaatatgtcatgaaaataataaaaatctatatttactgaaatggcactcatgaaatctttggcatgataaaagcagttaagggtacagcatgcatatcataattacactttcttaaaaaagcaaagtatagcacgattttctctaccaaattgagagcagccatctataagtatgattacaattaattttggctttttagtttgtaattttttgctttgtgattttggcttaacaattaaaaatgtacatttgtaaaataaaaagaccggccgcagtggctcacgcctgtaatcccagcactttcggaggccgaggcgggtggatcacctgaagtcgggagattgagaccatcctggctaacatggtgaaaccccgtctctactaaaaatacaaaaaattagccgggtgttgtggcacatgcctgtaatcccaactactcaaaaggctgaggcagaagaaccacttgaacctgggaggcgaaggttgtgacgagccgagattgcaccattgcactccagcctaggcaacaagagcgaaactccgtctcaacaaaaaataaagccaggtgcaatcgctcatgcctgtaatcccagcactttgggaggctgaggcaggtggatcacctgaggtcaggagttcaagactatcctgaccaacatggagaaaccctgtctctactaaaaatagaaaattagcagggtgtggtggcacacgcctgtgatcccagctactcaggagtctgaggcaggagaattgcttgaagccgggaggtggaggttgcagcgagccgagattgcgccactgcactccagcctgggcaacagagtgaaactccgtctcaaaaaacatataataataataataaaataaaacaaaaagactaacactaacttcaaaaacaaagttaaacctccacaaggaatttaaaaatattaaaggtcacacaattcaaacagtgtgatactggtgcaaacacaaatacacagatcagaaaagatagctctaaaaacacaagcaaatataaacatgagtataatgtgtcaccaagaaagtagaacaaaacaatgaatgaaagaattatagaacagctggcatcggtatatgactgggggagagagggaatgtcactttagactccgaatttataacctggaatgaaatacatttggatacaaaatttaaatacaaagttttaaaaaaaactacggaagagggtaactattagacatgatttttggtttaaaatatgaggaaggtgacaggggctttaatttttattatttattagtatgaattccctgatgacgaatgagatccgagccactactaaaagccttcccacattccttacagttatagggcttttcaccagtgtgaattctcagatgtcgagtaaggtttgagcatttattaaaggcctttccacattcattacattcatatggtttttcatctgtatgaattctctgatgctggaaaagttgtgagttctgagtaaaggccttcccacattcaagacattcaaagggtttctcaccagcgtgaattctctgatgttgacgaagctgtgagctctgagtaaaagcctttccacattccttacaatcatagggtttctcaccagtgtgaattctctgatgattagtaagtgctgagccactactaaaggctttgccacattccttgcactcatagggtttctcaccagtatgaattctctgatgttgaacaagctttgagctctgggtaaaggctttgccacattccttacattcatagggtttctcacctgtatgaattcgtgcatgctgaaaaagttgtgagctcttagtaaaggctttcccacatactttacattcataaggtttttcaccagtgtgaattcgctgatggtcaataagatttgagcaataactaaaggccttcccacattccttacattcatagggtttcttaccggtatggattctctgatgttgagaaaggtatgagctacaactgaaggcctttccacattccttacattcaaagggtttttcgccagtatgaattttcagatgccgagtaacatgtgaaccacaactaaagaatttcccacactctttacattcataagatttttcaccaatatgaattctctgatgttgaataaattgtgagttctgactaaaggcctttccacatttcttacattcatagggtctgtcttcattattaattatttgatggagagtaaggaatgtctgttgaataaatgtgggcatgtattcaggagtgaatatttcttgactaaaatgcccatttggatatcccagttgttttgcaaggtggcttctatattccaaaacatctccaaaactggagtactcaaggccatgctttgtaagtcccattatctccctctggcataattctatttcataaacttccttctttagagataataacttggtttcacacatcgattccagatctgaacacaggcctcttgtaagctctctgccaaccatccagggctctttcccttgttccaataaggagatcacttgaggcttaggagtgtaaagtcccattgaaaccagattgccgtagttctccaacatcacatctctgtataagtccctctgaacagggtccaggcagtcccactcctcctgagagaagtctatggacacatcactgaacatcactgatccctcagccatggcttctagtattgcagatggttagtcttccttgaggccgttctcctgaaaaaggacagtgttctgtaatcccagctactcaggaggctgaggcaagagaatcgcttgaacccggaaagcagaggctgcagtgagctgagatcatgccactgcactccagcttgggcaacagagtgagactccgtctgcgggccccagccgagcctgcaagacccaggccgctcaccgcgcacttcccctaccctt

SEQ ID NO: 13454 - RNA, 5893 nt, Homo sapiens
  source 1..5893: mol_type = other RNA
gctgggattacaggcatgagccaccacgcccggctaattttttgtatttttagtagagacagggtttctccatgttggtcaggctggtctcaaatccccgacctcaggtgatccacccgccttggcctcacagaatgctgagattacaggcgtgagccaccatgcctggccagtcttatttttttaaataagtttattctggagggaggtctattaagattttacacctccagttaattctgatgtcgtcaacttattaaaaatcacagactttttccagattttcagatatattataaaaatgtctataataccaacttttaagtttgttgttttaatttttttttttttctgtagagatgaggggagggggatctcattatgttacctagactggtcttgaactcctggcctcaagccattctcctacctcagcctcccaaagtgctggaattacaggcatgagccactgcaaccagccttaagtttttaaattgagatcaaattcacacagcataatattcacccttttaaagtgtatagttgagtgacctgtagtatataaacaaaattgtacaacctttacccatgccacattttcattaccccaaatgacacagttcttttaagtttacatatatagccatttcaatttctcatatacaatattgtttatttgtcatccttatttcacctctggaatcactaaactttgtctcattttttttctcttccatcaaatatcaattttggattcagatccagtttttttctttcaattatttctgccttttaaaataatactacctccttcctcccacaattcatttcagcttgttttagttccttgggttctatattttttcttcctagtattacaatatatgcacaaatattaggttataaaacttccaatacaacttttactgccactcacaggtttttcaattgttttcattttcatgtacatttaaataatgtatatattagggatttattccttaacccatgttaattaagagggaatattgaattaataatcagatatttgatggttatcctattgtactgcttcttctggtcaaataatgttgccagtatgttttctgcattttggggggaaatattagaaaaaattttataatctcttcctgcttttttgacagctgtgctttctactactcatcatattttcagggtttcagattggtaaccgtttattttttattttgtaagacagagtctcgctctgtcacccagtctggagtgtgcagtggtgcaatctcagctcactataacctccaactcccaggttcaagcaatcctcccacctcagcctcttgagtagctaggattacaggcatgcaacaccatgcctggctatttgtttttgtttttgttttttttgtatttttagtagagacggggtttcaccatgttggccaggctggtctcgagctcctgacctcaagtgatccacccaccttggcctcccaaagtgctaggattacaggtgtgagccaccgcgcccagcctcagactggtattctttatgtagcataaaagataaagtctgaacaaagactatgcacacatactttttctcttccttttaaaattccacactgaataataatgatagggaaaggcttcgttatactcattacaagtgtttctctttttccaccatgaattacaaatttgccaaaggtaaacaacatggttaaaatcctttccataaatcctaatgaagatacttatgataatgagtatatcactgataatagtggaaaacttttactaaacctgtattatgtgataacagtttgaggtactttgcatttattaattcattgactcttcacagcaatccaatacatacagccttattatagatgcctagacataattttttaaaataccactaacagccaggggcggtggctcacacctataatcccagcactttgggaagccaaggcaggaggatcacgaggtcaggagtttgagagcagcctggccaatatggtgaaaccccatctctactaataatacaaaaattagctaggcatggtggcgcgcgcctgtagtcccagctactcgggaggctgaggcggaagactcacttgaactcgggaggcagaggttgcagtgagccgagattgcaccactgccctccagcctgggcaacagagcgagactgtgtctcaaaaaacaaaaacaccactaatagctataagaaaaaataattgaccgggcacagtggctcacacctgtaatccccgaactttgggaggccgaggtgggtggatcacaaggtcaagagttcaagaccagcctggccaacatagtgaaaccctgtctctactaaaaatacaaaaattagccaggcatggtgtcgtgcgcctgtagtctcagatactaggaaggctgaggcaggagaatcgcttgaacccgggaggcagcagttgtggtgaactgagattgtgccactgcacttcagcctgggcaacagagtgaactccatctcaaaaaaaaaaaaaaacaaacaaacaaaaaattaatatctggattgataaataacactttcataacagtgttactttctagtatggcattgggattaggattgatgtaagggaacaaaacagctcacaaggagaaaatgtagataattttagcaattaaaataaatgttttaaaagtaaaaataagcatccaatgaggtcagcagtttttgtgtttttttgagacggaatctcactctgtcccccaggctggagtgcagtggcaccatctcagctcactgcaacctccgcctcccaggttcaagcaattctcctgtctcagcctcccgagtagctgggattacaggtacatgccaccacgcccagctaagtagagacggggtttcactgttagccaggatggccttaatcttcagaccttgtgatccgcccacctcggcctcccaaagtgctgggattacaggcatgagccactgtgcccagccgaggtcagcttttatagctgcaaaaatttagtggcaaccataatgggaatagtcattttaaagtcattaaatatgtcatgaaaataataaaaatctatatttactgaaatggcactcatgaaatctttggcatgataaaagcagttaagggtacagcatgcatatcataattacactttcttaaaaaagcaaagtatagcacgattttctctaccaaattgagagcagccatctataagtatgattacaattaattttggctttttagtttgtaattttttgctttgtgattttggcttaacaattaaaaatgtacatttgtaaaataaaaagaccggccgcagtggctcacgcctgtaatcccagcactttcggaggccgaggcgggtggatcacctgaagtcgggagattgagaccatcctggctaacatggtgaaaccccgtctctactaaaaatacaaaaaattagccgggtgttgtggcacatgcctgtaatcccaactactcaaaaggctgaggcagaagaaccacttgaacctgggaggcgaaggttgtgacgagccgagattgcaccattgcactccagcctaggcaacaagagcgaaactccgtctcaacaaaaaataaagccaggtgcaatcgctcatgcctgtaatcccagcactttgggaggctgaggcaggtggatcacctgaggtcaggagttcaagactatcctgaccaacatggagaaaccctgtctctactaaaaatagaaaattagcagggtgtggtggcacacgcctgtgatcccagctactcaggagtctgaggcaggagaattgcttgaagccgggaggtggaggttgcagcgagccgagattgcgccactgcactccagcctgggcaacagagtgaaactccgtctcaaaaaacatataataataataataaaataaaacaaaaagactaacactaacttcaaaaacaaagttaaacctccacaaggaatttaaaaatattaaaggtcacacaattcaaacagtgtgatactggtgcaaacacaaatacacagatcagaaaagatagctctaaaaacacaagcaaatataaacatgagtataatgtgtcaccaagaaagtagaacaaaacaatgaatgaaagaattatagaacagctggcatcggtatatgactgggggagagagggaatgtcactttagactccgaatttataacctggaatgaaatacatttggatacaaaatttaaatacaaagttttaaaaaaaactacggaagagggtaactattagacatgatttttggtttaaaatatgaggaaggtgacaggggctttaatttttattatttattagtatgaattccctgatgacgaatgagatccgagccactactaaaagccttcccacattccttacagttatagggcttttcaccagtgtgaattctcagatgtcgagtaaggtttgagcatttattaaaggcctttccacattcattacattcatatggtttttcatctgtatgaattctctgatgctggaaaagttgtgagttctgagtaaaggccttcccacattcaagacattcaaagggtttctcaccagcgtgaattctctgatgttgacgaagctgtgagctctgagtaaaagcctttccacattccttacaatcatagggtttctcaccagtgtgaattctctgatgattagtaagtgctgagccactactaaaggctttgccacattccttgcactcatagggtttctcaccagtatgaattctctgatgttgaacaagctttgagctctgggtaaaggctttgccacattccttacattcatagggtttctcacctgtatgaattcgtgcatgctgaaaaagttgtgagctcttagtaaaggctttcccacatactttacattcataaggtttttcaccagtgtgaattcgctgatggtcaataagatttgagcaataactaaaggccttcccacattccttacattcatagggtttcttaccggtatggattctctgatgttgagaaaggtatgagctacaactgaaggcctttccacattccttacattcaaagggtttttcgccagtatgaattttcagatgccgagtaacatgtgaaccacaactaaagaatttcccacactctttacattcataagatttttcaccaatatgaattctctgatgttgaataaattgtgagttctgactaaaggcctttccacatttcttacattcatagggtctgtcttcattattaattatttgatggagagtaaggaatgtctgttgaataaatgtgggcatgtattcaggagtgaatatttcttgactaaaatgcccatttggatatcccagttgttttgcaaggtggcttctatattccaaaacatctccaaaactggagtactcaaggccatgctttgtaagtcccattatctccctctggcataattctatttcataaacttccttctttagagataataacttggtttcacacatcgattccagatctgaacacaggcctcttgtaagctctctgccaaccatccagggctctttcccttgttccaataaggagatcacttgaggcttaggagtgtaaagtcccattgaaaccagattgccgtagttctccaacatcacatctctgtataagtccctctgaacagggtccaggcagtcccactcctcctgagagaagtctatggacacatcactgaacatcactgatccctcagccatggcttctagtattgcagatggttagtcttccttgaggccgttctcctgcgggccccagccgagcctgcaagacccaggccgctcaccgcgcacttcccctaccctt

SEQ ID NO: 13455 - RNA, 6015 nt, Homo sapiens
  source 1..6015: mol_type = other RNA
gctgggattacaggcatgagccaccacgcccggctaattttttgtatttttagtagagacagggtttctccatgttggtcaggctggtctcaaatccccgacctcaggtgatccacccgccttggcctcacagaatgctgagattacaggcgtgagccaccatgcctggccagtcttatttttttaaataagtttattctggagggaggtctattaagattttacacctccagttaattctgatgtcgtcaacttattaaaaatcacagactttttccagattttcagatatattataaaaatgtctataataccaacttttaagtttgttgttttaatttttttttttttctgtagagatgaggggagggggatctcattatgttacctagactggtcttgaactcctggcctcaagccattctcctacctcagcctcccaaagtgctggaattacaggcatgagccactgcaaccagccttaagtttttaaattgagatcaaattcacacagcataatattcacccttttaaagtgtatagttgagtgacctgtagtatataaacaaaattgtacaacctttacccatgccacattttcattaccccaaatgacacagttcttttaagtttacatatatagccatttcaatttctcatatacaatattgtttatttgtcatccttatttcacctctggaatcactaaactttgtctcattttttttctcttccatcaaatatcaattttggattcagatccagtttttttctttcaattatttctgccttttaaaataatactacctccttcctcccacaattcatttcagcttgttttagttccttgggttctatattttttcttcctagtattacaatatatgcacaaatattaggttataaaacttccaatacaacttttactgccactcacaggtttttcaattgttttcattttcatgtacatttaaataatgtatatattagggatttattccttaacccatgttaattaagagggaatattgaattaataatcagatatttgatggttatcctattgtactgcttcttctggtcaaataatgttgccagtatgttttctgcattttggggggaaatattagaaaaaattttataatctcttcctgcttttttgacagctgtgctttctactactcatcatattttcagggtttcagattggtaaccgtttattttttattttgtaagacagagtctcgctctgtcacccagtctggagtgtgcagtggtgcaatctcagctcactataacctccaactcccaggttcaagcaatcctcccacctcagcctcttgagtagctaggattacaggcatgcaacaccatgcctggctatttgtttttgtttttgttttttttgtatttttagtagagacggggtttcaccatgttggccaggctggtctcgagctcctgacctcaagtgatccacccaccttggcctcccaaagtgctaggattacaggtgtgagccaccgcgcccagcctcagactggtattctttatgtagcataaaagataaagtctgaacaaagactatgcacacatactttttctcttccttttaaaattccacactgaataataatgatagggaaaggcttcgttatactcattacaagtgtttctctttttccaccatgaattacaaatttgccaaaggtaaacaacatggttaaaatcctttccataaatcctaatgaagatacttatgataatgagtatatcactgataatagtggaaaacttttactaaacctgtattatgtgataacagtttgaggtactttgcatttattaattcattgactcttcacagcaatccaatacatacagccttattatagatgcctagacataattttttaaaataccactaacagccaggggcggtggctcacacctataatcccagcactttgggaagccaaggcaggaggatcacgaggtcaggagtttgagagcagcctggccaatatggtgaaaccccatctctactaataatacaaaaattagctaggcatggtggcgcgcgcctgtagtcccagctactcgggaggctgaggcggaagactcacttgaactcgggaggcagaggttgcagtgagccgagattgcaccactgccctccagcctgggcaacagagcgagactgtgtctcaaaaaacaaaaacaccactaatagctataagaaaaaataattgaccgggcacagtggctcacacctgtaatccccgaactttgggaggccgaggtgggtggatcacaaggtcaagagttcaagaccagcctggccaacatagtgaaaccctgtctctactaaaaatacaaaaattagccaggcatggtgtcgtgcgcctgtagtctcagatactaggaaggctgaggcaggagaatcgcttgaacccgggaggcagcagttgtggtgaactgagattgtgccactgcacttcagcctgggcaacagagtgaactccatctcaaaaaaaaaaaaaaacaaacaaacaaaaaattaatatctggattgataaataacactttcataacagtgttactttctagtatggcattgggattaggattgatgtaagggaacaaaacagctcacaaggagaaaatgtagataattttagcaattaaaataaatgttttaaaagtaaaaataagcatccaatgaggtcagcagtttttgtgtttttttgagacggaatctcactctgtcccccaggctggagtgcagtggcaccatctcagctcactgcaacctccgcctcccaggttcaagcaattctcctgtctcagcctcccgagtagctgggattacaggtacatgccaccacgcccagctaagtagagacggggtttcactgttagccaggatggccttaatcttcagaccttgtgatccgcccacctcggcctcccaaagtgctgggattacaggcatgagccactgtgcccagccgaggtcagcttttatagctgcaaaaatttagtggcaaccataatgggaatagtcattttaaagtcattaaatatgtcatgaaaataataaaaatctatatttactgaaatggcactcatgaaatctttggcatgataaaagcagttaagggtacagcatgcatatcataattacactttcttaaaaaagcaaagtatagcacgattttctctaccaaattgagagcagccatctataagtatgattacaattaattttggctttttagtttgtaattttttgctttgtgattttggcttaacaattaaaaatgtacatttgtaaaataaaaagaccggccgcagtggctcacgcctgtaatcccagcactttcggaggccgaggcgggtggatcacctgaagtcgggagattgagaccatcctggctaacatggtgaaaccccgtctctactaaaaatacaaaaaattagccgggtgttgtggcacatgcctgtaatcccaactactcaaaaggctgaggcagaagaaccacttgaacctgggaggcgaaggttgtgacgagccgagattgcaccattgcactccagcctaggcaacaagagcgaaactccgtctcaacaaaaaataaagccaggtgcaatcgctcatgcctgtaatcccagcactttgggaggctgaggcaggtggatcacctgaggtcaggagttcaagactatcctgaccaacatggagaaaccctgtctctactaaaaatagaaaattagcagggtgtggtggcacacgcctgtgatcccagctactcaggagtctgaggcaggagaattgcttgaagccgggaggtggaggttgcagcgagccgagattgcgccactgcactccagcctgggcaacagagtgaaactccgtctcaaaaaacatataataataataataaaataaaacaaaaagactaacactaacttcaaaaacaaagttaaacctccacaaggaatttaaaaatattaaaggtcacacaattcaaacagtgtgatactggtgcaaacacaaatacacagatcagaaaagatagctctaaaaacacaagcaaatataaacatgagtataatgtgtcaccaagaaagtagaacaaaacaatgaatgaaagaattatagaacagctggcatcggtatatgactgggggagagagggaatgtcactttagactccgaatttataacctggaatgaaatacatttggatacaaaatttaaatacaaagttttaaaaaaaactacggaagagggtaactattagacatgatttttggtttaaaatatgaggaaggtgacaggggctttaatttttattatttattagtatgaattccctgatgacgaatgagatccgagccactactaaaagccttcccacattccttacagttatagggcttttcaccagtgtgaattctcagatgtcgagtaaggtttgagcatttattaaaggcctttccacattcattacattcatatggtttttcatctgtatgaattctctgatgctggaaaagttgtgagttctgagtaaaggccttcccacattcaagacattcaaagggtttctcaccagcgtgaattctctgatgttgacgaagctgtgagctctgagtaaaagcctttccacattccttacaatcatagggtttctcaccagtgtgaattctctgatgattagtaagtgctgagccactactaaaggctttgccacattccttgcactcatagggtttctcaccagtatgaattctctgatgttgaacaagctttgagctctgggtaaaggctttgccacattccttacattcatagggtttctcacctgtatgaattcgtgcatgctgaaaaagttgtgagctcttagtaaaggctttcccacatactttacattcataaggtttttcaccagtgtgaattcgctgatggtcaataagatttgagcaataactaaaggccttcccacattccttacattcatagggtttcttaccggtatggattctctgatgttgagaaaggtatgagctacaactgaaggcctttccacattccttacattcaaagggtttttcgccagtatgaattttcagatgccgagtaacatgtgaaccacaactaaagaatttcccacactctttacattcataagatttttcaccaatatgaattctctgatgttgaataaattgtgagttctgactaaaggcctttccacatttcttacattcatagggtctgtcttcattattaattatttgatggagagtaaggaatgtctgttgaataaatgtgggcatgtattcaggagtgaatatttcttgactaaaatgcccatttggatatcccagttgttttgcaaggtggcttctatattccaaaacatctccaaaactggagtactcaaggccatgctttgtaagtcccattatctccctctggcataattctatttcataaacttccttctttagagataataacttggtttcacacatcgattccagatctgaacacaggcctcttgtaagctctctgccaaccatccagggctctttcccttgttccaataaggagatcacttgaggcttaggagtgtaaagtcccattgaaaccagattgccgtagttctccaacatcacatctctgtataagtccctctgaacagggtccaggcagtcccactcctcctgagagaagtctatggacacatcactgaacatcactgatccctcagccatggcttctagtattgcagatggttagtcttccttgaggccgttctcctgtaatcccagctactcaggaggctgaggcaagagaatcgcttgaacccggaaagcagaggctgcagtgagctgagatcatgccactgcactccagcttgggcaacagagtgagactccgtctgcgggccccagccgagcctgcaagacccaggccgctcaccgcgcacttcccctaccctt

SEQ ID NO: 13456 - RNA, 6240 nt, Homo sapiens
  source 1..6240: mol_type = other RNA
gctgggattacaggcatgagccaccacgcccggctaattttttgtatttttagtagagacagggtttctccatgttggtcaggctggtctcaaatccccgacctcaggtgatccacccgccttggcctcacagaatgctgagattacaggcgtgagccaccatgcctggccagtcttatttttttaaataagtttattctggagggaggtctattaagattttacacctccagttaattctgatgtcgtcaacttattaaaaatcacagactttttccagattttcagatatattataaaaatgtctataataccaacttttaagtttgttgttttaatttttttttttttctgtagagatgaggggagggggatctcattatgttacctagactggtcttgaactcctggcctcaagccattctcctacctcagcctcccaaagtgctggaattacaggcatgagccactgcaaccagccttaagtttttaaattgagatcaaattcacacagcataatattcacccttttaaagtgtatagttgagtgacctgtagtatataaacaaaattgtacaacctttacccatgccacattttcattaccccaaatgacacagttcttttaagtttacatatatagccatttcaatttctcatatacaatattgtttatttgtcatccttatttcacctctggaatcactaaactttgtctcattttttttctcttccatcaaatatcaattttggattcagatccagtttttttctttcaattatttctgccttttaaaataatactacctccttcctcccacaattcatttcagcttgttttagttccttgggttctatattttttcttcctagtattacaatatatgcacaaatattaggttataaaacttccaatacaacttttactgccactcacaggtttttcaattgttttcattttcatgtacatttaaataatgtatatattagggatttattccttaacccatgttaattaagagggaatattgaattaataatcagatatttgatggttatcctattgtactgcttcttctggtcaaataatgttgccagtatgttttctgcattttggggggaaatattagaaaaaattttataatctcttcctgcttttttgacagctgtgctttctactactcatcatattttcagggtttcagattggtaaccgtttattttttattttgtaagacagagtctcgctctgtcacccagtctggagtgtgcagtggtgcaatctcagctcactataacctccaactcccaggttcaagcaatcctcccacctcagcctcttgagtagctaggattacaggcatgcaacaccatgcctggctatttgtttttgtttttgttttttttgtatttttagtagagacggggtttcaccatgttggccaggctggtctcgagctcctgacctcaagtgatccacccaccttggcctcccaaagtgctaggattacaggtgtgagccaccgcgcccagcctcagactggtattctttatgtagcataaaagataaagtctgaacaaagactatgcacacatactttttctcttccttttaaaattccacactgaataataatgatagggaaaggcttcgttatactcattacaagtgtttctctttttccaccatgaattacaaatttgccaaaggtaaacaacatggttaaaatcctttccataaatcctaatgaagatacttatgataatgagtatatcactgataatagtggaaaacttttactaaacctgtattatgtgataacagtttgaggtactttgcatttattaattcattgactcttcacagcaatccaatacatacagccttattatagatgcctagacataattttttaaaataccactaacagccaggggcggtggctcacacctataatcccagcactttgggaagccaaggcaggaggatcacgaggtcaggagtttgagagcagcctggccaatatggtgaaaccccatctctactaataatacaaaaattagctaggcatggtggcgcgcgcctgtagtcccagctactcgggaggctgaggcggaagactcacttgaactcgggaggcagaggttgcagtgagccgagattgcaccactgccctccagcctgggcaacagagcgagactgtgtctcaaaaaacaaaaacaccactaatagctataagaaaaaataattgaccgggcacagtggctcacacctgtaatccccgaactttgggaggccgaggtgggtggatcacaaggtcaagagttcaagaccagcctggccaacatagtgaaaccctgtctctactaaaaatacaaaaattagccaggcatggtgtcgtgcgcctgtagtctcagatactaggaaggctgaggcaggagaatcgcttgaacccgggaggcagcagttgtggtgaactgagattgtgccactgcacttcagcctgggcaacagagtgaactccatctcaaaaaaaaaaaaaaacaaacaaacaaaaaattaatatctggattgataaataacactttcataacagtgttactttctagtatggcattgggattaggattgatgtaagggaacaaaacagctcacaaggagaaaatgtagataattttagcaattaaaataaatgttttaaaagtaaaaataagcatccaatgaggtcagcagtttttgtgtttttttgagacggaatctcactctgtcccccaggctggagtgcagtggcaccatctcagctcactgcaacctccgcctcccaggttcaagcaattctcctgtctcagcctcccgagtagctgggattacaggtacatgccaccacgcccagctaagtagagacggggtttcactgttagccaggatggccttaatcttcagaccttgtgatccgcccacctcggcctcccaaagtgctgggattacaggcatgagccactgtgcccagccgaggtcagcttttatagctgcaaaaatttagtggcaaccataatgggaatagtcattttaaagtcattaaatatgtcatgaaaataataaaaatctatatttactgaaatggcactcatgaaatctttggcatgataaaagcagttaagggtacagcatgcatatcataattacactttcttaaaaaagcaaagtatagcacgattttctctaccaaattgagagcagccatctataagtatgattacaattaattttggctttttagtttgtaattttttgctttgtgattttggcttaacaattaaaaatgtacatttgtaaaataaaaagaccggccgcagtggctcacgcctgtaatcccagcactttcggaggccgaggcgggtggatcacctgaagtcgggagattgagaccatcctggctaacatggtgaaaccccgtctctactaaaaatacaaaaaattagccgggtgttgtggcacatgcctgtaatcccaactactcaaaaggctgaggcagaagaaccacttgaacctgggaggcgaaggttgtgacgagccgagattgcaccattgcactccagcctaggcaacaagagcgaaactccgtctcaacaaaaaataaagccaggtgcaatcgctcatgcctgtaatcccagcactttgggaggctgaggcaggtggatcacctgaggtcaggagttcaagactatcctgaccaacatggagaaaccctgtctctactaaaaatagaaaattagcagggtgtggtggcacacgcctgtgatcccagctactcaggagtctgaggcaggagaattgcttgaagccgggaggtggaggttgcagcgagccgagattgcgccactgcactccagcctgggcaacagagtgaaactccgtctcaaaaaacatataataataataataaaataaaacaaaaagactaacactaacttcaaaaacaaagttaaacctccacaaggaatttaaaaatattaaaggtcacacaattcaaacagtgtgatactggtgcaaacacaaatacacagatcagaaaagatagctctaaaaacacaagcaaatataaacatgagtataatgtgtcaccaagaaagtagaacaaaacaatgaatgaaagaattatagaacagctggcatcggtatatgactgggggagagagggaatgtcactttagactccgaatttataacctggaatgaaatacatttggatacaaaatttaaatacaaagttttaaaaaaaactacggaagagggtaactattagacatgatttttggtttaaaatatgaggaaggtgacaggggctttaatttttattatttattagtatgaattccctgatgacgaatgagatccgagccactactaaaagccttcccacattccttacagttatagggcttttcaccagtgtgaattctcagatgtcgagtaaggtttgagcatttattaaaggcctttccacattcattacattcatatggtttttcatctgtatgaattctctgatgctggaaaagttgtgagttctgagtaaaggccttcccacattcaagacattcaaagggtttctcaccagcgtgaattctctgatgttgacgaagctgtgagctctgagtaaaagcctttccacattccttacaatcatagggtttctcaccagtgtgaattctctgatgattagtaagtgctgagccactactaaaggctttgccacattccttgcactcatagggtttctcaccagtatgaattctctgatgttgaacaagctttgagctctgggtaaaggctttgccacattccttacattcatagggtttctcacctgtatgaattcgtgcatgctgaaaaagttgtgagctcttagtaaaggctttcccacatactttacattcataaggtttttcaccagtgtgaattcgctgatggtcaataagatttgagcaataactaaaggccttcccacattccttacattcatagggtttcttaccggtatggattctctgatgttgagaaaggtatgagctacaactgaaggcctttccacattccttacattcaaagggtttttcgccagtatgaattttcagatgccgagtaacatgtgaaccacaactaaagaatttcccacactctttacattcataagatttttcaccaatatgaattctctgatgttgaataaattgtgagttctgactaaaggcctttccacatttcttacattcatagggtctgtcttcattattaattatttgatggagagtaaggaatgtctgttgaataaatgtgggcatgtattcaggagtgaatatttcttgactaaaatgcccatttggatatcccagttgttttgcaaggtggcttctatattccaaaacatctccaaaactggagtactcaaggccatgctttgtaagtcccattatctccctctggcataattctatttcataaacttccttctttagagataataacttggtttcacacatcgattccagatctgaacacaggcctcttgtaagctctctgccaaccatccagggctctttcccttgttccaataaggagatcacttgaggcttaggagtgtaaagtcccattgaaaccagattgccgtagttctccaacatcacatctctgtataagtccctctgaacagggtccaggcagtcccactcctcctgagagaagtctatggacacatcactgaacatcactgatccctcagccatggcttctagtattgcagatggttagtcttccttgaggccgttctcctgtaatcccagctactcaggaggctgaggcaagagaatcgcttgaacccggaaagcagaggctgcagtgagctgagatcatgccactgcactccagcttgggcaacagagtgagactccgtcttgtatttggtttggtcaacagccattcttcctctgggtaactctcttgacgagagcagagctgaagaagaaaggaatgatgagatgccaggcctttcttgtggcccagactgagcagatcagaggtcattttggatctacagctactatatgcccgacacactcatacatgcccaacactccagaccagcctggtcagtcccttcaaactcccatgcacgtacctgcgggccccagccgagcctgcaagacccaggccgctcaccgcgcacttcccctaccctt

SEQ ID NO: 13457 - RNA, 6436 nt, Homo sapiens
  source 1..6436: mol_type = other RNA
gctgggattacaggcatgagccaccacgcccggctaattttttgtatttttagtagagacagggtttctccatgttggtcaggctggtctcaaatccccgacctcaggtgatccacccgccttggcctcacagaatgctgagattacaggcgtgagccaccatgcctggccagtcttatttttttaaataagtttattctggagggaggtctattaagattttacacctccagttaattctgatgtcgtcaacttattaaaaatcacagactttttccagattttcagatatattataaaaatgtctataataccaacttttaagtttgttgttttaatttttttttttttctgtagagatgaggggagggggatctcattatgttacctagactggtcttgaactcctggcctcaagccattctcctacctcagcctcccaaagtgctggaattacaggcatgagccactgcaaccagccttaagtttttaaattgagatcaaattcacacagcataatattcacccttttaaagtgtatagttgagtgacctgtagtatataaacaaaattgtacaacctttacccatgccacattttcattaccccaaatgacacagttcttttaagtttacatatatagccatttcaatttctcatatacaatattgtttatttgtcatccttatttcacctctggaatcactaaactttgtctcattttttttctcttccatcaaatatcaattttggattcagatccagtttttttctttcaattatttctgccttttaaaataatactacctccttcctcccacaattcatttcagcttgttttagttccttgggttctatattttttcttcctagtattacaatatatgcacaaatattaggttataaaacttccaatacaacttttactgccactcacaggtttttcaattgttttcattttcatgtacatttaaataatgtatatattagggatttattccttaacccatgttaattaagagggaatattgaattaataatcagatatttgatggttatcctattgtactgcttcttctggtcaaataatgttgccagtatgttttctgcattttggggggaaatattagaaaaaattttataatctcttcctgcttttttgacagctgtgctttctactactcatcatattttcagggtttcagattggtaaccgtttattttttattttgtaagacagagtctcgctctgtcacccagtctggagtgtgcagtggtgcaatctcagctcactataacctccaactcccaggttcaagcaatcctcccacctcagcctcttgagtagctaggattacaggcatgcaacaccatgcctggctatttgtttttgtttttgttttttttgtatttttagtagagacggggtttcaccatgttggccaggctggtctcgagctcctgacctcaagtgatccacccaccttggcctcccaaagtgctaggattacaggtgtgagccaccgcgcccagcctcagactggtattctttatgtagcataaaagataaagtctgaacaaagactatgcacacatactttttctcttccttttaaaattccacactgaataataatgatagggaaaggcttcgttatactcattacaagtgtttctctttttccaccatgaattacaaatttgccaaaggtaaacaacatggttaaaatcctttccataaatcctaatgaagatacttatgataatgagtatatcactgataatagtggaaaacttttactaaacctgtattatgtgataacagtttgaggtactttgcatttattaattcattgactcttcacagcaatccaatacatacagccttattatagatgcctagacataattttttaaaataccactaacagccaggggcggtggctcacacctataatcccagcactttgggaagccaaggcaggaggatcacgaggtcaggagtttgagagcagcctggccaatatggtgaaaccccatctctactaataatacaaaaattagctaggcatggtggcgcgcgcctgtagtcccagctactcgggaggctgaggcggaagactcacttgaactcgggaggcagaggttgcagtgagccgagattgcaccactgccctccagcctgggcaacagagcgagactgtgtctcaaaaaacaaaaacaccactaatagctataagaaaaaataattgaccgggcacagtggctcacacctgtaatccccgaactttgggaggccgaggtgggtggatcacaaggtcaagagttcaagaccagcctggccaacatagtgaaaccctgtctctactaaaaatacaaaaattagccaggcatggtgtcgtgcgcctgtagtctcagatactaggaaggctgaggcaggagaatcgcttgaacccgggaggcagcagttgtggtgaactgagattgtgccactgcacttcagcctgggcaacagagtgaactccatctcaaaaaaaaaaaaaaacaaacaaacaaaaaattaatatctggattgataaataacactttcataacagtgttactttctagtatggcattgggattaggattgatgtaagggaacaaaacagctcacaaggagaaaatgtagataattttagcaattaaaataaatgttttaaaagtaaaaataagcatccaatgaggtcagcagtttttgtgtttttttgagacggaatctcactctgtcccccaggctggagtgcagtggcaccatctcagctcactgcaacctccgcctcccaggttcaagcaattctcctgtctcagcctcccgagtagctgggattacaggtacatgccaccacgcccagctaagtagagacggggtttcactgttagccaggatggccttaatcttcagaccttgtgatccgcccacctcggcctcccaaagtgctgggattacaggcatgagccactgtgcccagccgaggtcagcttttatagctgcaaaaatttagtggcaaccataatgggaatagtcattttaaagtcattaaatatgtcatgaaaataataaaaatctatatttactgaaatggcactcatgaaatctttggcatgataaaagcagttaagggtacagcatgcatatcataattacactttcttaaaaaagcaaagtatagcacgattttctctaccaaattgagagcagccatctataagtatgattacaattaattttggctttttagtttgtaattttttgctttgtgattttggcttaacaattaaaaatgtacatttgtaaaataaaaagaccggccgcagtggctcacgcctgtaatcccagcactttcggaggccgaggcgggtggatcacctgaagtcgggagattgagaccatcctggctaacatggtgaaaccccgtctctactaaaaatacaaaaaattagccgggtgttgtggcacatgcctgtaatcccaactactcaaaaggctgaggcagaagaaccacttgaacctgggaggcgaaggttgtgacgagccgagattgcaccattgcactccagcctaggcaacaagagcgaaactccgtctcaacaaaaaataaagccaggtgcaatcgctcatgcctgtaatcccagcactttgggaggctgaggcaggtggatcacctgaggtcaggagttcaagactatcctgaccaacatggagaaaccctgtctctactaaaaatagaaaattagcagggtgtggtggcacacgcctgtgatcccagctactcaggagtctgaggcaggagaattgcttgaagccgggaggtggaggttgcagcgagccgagattgcgccactgcactccagcctgggcaacagagtgaaactccgtctcaaaaaacatataataataataataaaataaaacaaaaagactaacactaacttcaaaaacaaagttaaacctccacaaggaatttaaaaatattaaaggtcacacaattcaaacagtgtgatactggtgcaaacacaaatacacagatcagaaaagatagctctaaaaacacaagcaaatataaacatgagtataatgtgtcaccaagaaagtagaacaaaacaatgaatgaaagaattatagaacagctggcatcggtatatgactgggggagagagggaatgtcactttagactccgaatttataacctggaatgaaatacatttggatacaaaatttaaatacaaagttttaaaaaaaactacggaagagggtaactattagacatgatttttggtttaaaatatgaggaaggtgacaggggctttaatttttattatttattagtatgaattccctgatgacgaatgagatccgagccactactaaaagccttcccacattccttacagttatagggcttttcaccagtgtgaattctcagatgtcgagtaaggtttgagcatttattaaaggcctttccacattcattacattcatatggtttttcatctgtatgaattctctgatgctggaaaagttgtgagttctgagtaaaggccttcccacattcaagacattcaaagggtttctcaccagcgtgaattctctgatgttgacgaagctgtgagctctgagtaaaagcctttccacattccttacaatcatagggtttctcaccagtgtgaattctctgatgattagtaagtgctgagccactactaaaggctttgccacattccttgcactcatagggtttctcaccagtatgaattctctgatgttgaacaagctttgagctctgggtaaaggctttgccacattccttacattcatagggtttctcacctgtatgaattcgtgcatgctgaaaaagttgtgagctcttagtaaaggctttcccacatactttacattcataaggtttttcaccagtgtgaattcgctgatggtcaataagatttgagcaataactaaaggccttcccacattccttacattcatagggtttcttaccggtatggattctctgatgttgagaaaggtatgagctacaactgaaggcctttccacattccttacattcaaagggtttttcgccagtatgaattttcagatgccgagtaacatgtgaaccacaactaaagaatttcccacactctttacattcataagatttttcaccaatatgaattctctgatgttgaataaattgtgagttctgactaaaggcctttccacatttcttacattcatagggtctgtcttcattattaattatttgatggagagtaaggaatgtctgttgaataaatgtgggcatgtattcaggagtgaatatttcttgactaaaatgcccatttggatatcccagttgttttgcaaggtggcttctatattccaaaacatctccaaaactggagtactcaaggccatgctttgtaagtcccattatctccctctggcataattctatttcataaacttccttctttagagataataacttggtttcacacatcgattccagatctgaacacaggcctcttgtaagctctctgccaaccatccagggctctttcccttgttccaataaggagatcacttgaggcttaggagtgtaaagtcccattgaaaccagattgccgtagttctccaacatcacatctctgtataagtccctctgaacagggtccaggcagtcccactcctcctgagagaagtctatggacacatcactgaacatcactgatccctcagccatggcttctagtattgcagatggttagtcttccttgaggccgttctcctgtaatcccagctactcaggaggctgaggcaagagaatcgcttgaacccggaaagcagaggctgcagtgagctgagatcatgccactgcactccagcttgggcaacagagtgagactccgtcttgtatttggtttggtcaacagccattcttcctctgggtaactctcttgacgagagcagagctgaagaagaaaggaatgatgagatgccaggcctttcttgtggcccagactgagcagatcagaggtcattttggatctacagctactatctgaggtggggaggtcgagaccagcctgaccaacacggagaaaccccgtctctactgaaaatacaaaattagcagggcgtggtgacacacgcctgtaatcccagctactaggaaggctgaggcaggagaattgcttgaaccggggaggcggaggttgcggtgagccgagattgcgccattgcactccagcctgggcaacaacagcgaaactccgcatgcccaacactccagaccagcctggtcagtcccttcaaactcccatgcacgtacctgcgggccccagccgagcctgcaagacccaggccgctcaccgcgcacttcccctaccctt

SEQ ID NO: 13458 - RNA, 6432 nt, Homo sapiens
  source 1..6432: mol_type = other RNA
gctgggattacaggcatgagccaccacgcccggctaattttttgtatttttagtagagacagggtttctccatgttggtcaggctggtctcaaatccccgacctcaggtgatccacccgccttggcctcacagaatgctgagattacaggcgtgagccaccatgcctggccagtcttatttttttaaataagtttattctggagggaggtctattaagattttacacctccagttaattctgatgtcgtcaacttattaaaaatcacagactttttccagattttcagatatattataaaaatgtctataataccaacttttaagtttgttgttttaatttttttttttttctgtagagatgaggggagggggatctcattatgttacctagactggtcttgaactcctggcctcaagccattctcctacctcagcctcccaaagtgctggaattacaggcatgagccactgcaaccagccttaagtttttaaattgagatcaaattcacacagcataatattcacccttttaaagtgtatagttgagtgacctgtagtatataaacaaaattgtacaacctttacccatgccacattttcattaccccaaatgacacagttcttttaagtttacatatatagccatttcaatttctcatatacaatattgtttatttgtcatccttatttcacctctggaatcactaaactttgtctcattttttttctcttccatcaaatatcaattttggattcagatccagtttttttctttcaattatttctgccttttaaaataatactacctccttcctcccacaattcatttcagcttgttttagttccttgggttctatattttttcttcctagtattacaatatatgcacaaatattaggttataaaacttccaatacaacttttactgccactcacaggtttttcaattgttttcattttcatgtacatttaaataatgtatatattagggatttattccttaacccatgttaattaagagggaatattgaattaataatcagatatttgatggttatcctattgtactgcttcttctggtcaaataatgttgccagtatgttttctgcattttggggggaaatattagaaaaaattttataatctcttcctgcttttttgacagctgtgctttctactactcatcatattttcagggtttcagattggtaaccgtttattttttattttgtaagacagagtctcgctctgtcacccagtctggagtgtgcagtggtgcaatctcagctcactataacctccaactcccaggttcaagcaatcctcccacctcagcctcttgagtagctaggattacaggcatgcaacaccatgcctggctatttgtttttgtttttgttttttttgtatttttagtagagacggggtttcaccatgttggccaggctggtctcgagctcctgacctcaagtgatccacccaccttggcctcccaaagtgctaggattacaggtgtgagccaccgcgcccagcctcagactggtattctttatgtagcataaaagataaagtctgaacaaagactatgcacacatactttttctcttccttttaaaattccacactgaataataatgatagggaaaggcttcgttatactcattacaagtgtttctctttttccaccatgaattacaaatttgccaaaggtaaacaacatggttaaaatcctttccataaatcctaatgaagatacttatgataatgagtatatcactgataatagtggaaaacttttactaaacctgtattatgtgataacagtttgaggtactttgcatttattaattcattgactcttcacagcaatccaatacatacagccttattatagatgcctagacataattttttaaaataccactaacagccaggggcggtggctcacacctataatcccagcactttgggaagccaaggcaggaggatcacgaggtcaggagtttgagagcagcctggccaatatggtgaaaccccatctctactaataatacaaaaattagctaggcatggtggcgcgcgcctgtagtcccagctactcgggaggctgaggcggaagactcacttgaactcgggaggcagaggttgcagtgagccgagattgcaccactgccctccagcctgggcaacagagcgagactgtgtctcaaaaaacaaaaacaccactaatagctataagaaaaaataattgaccgggcacagtggctcacacctgtaatccccgaactttgggaggccgaggtgggtggatcacaaggtcaagagttcaagaccagcctggccaacatagtgaaaccctgtctctactaaaaatacaaaaattagccaggcatggtgtcgtgcgcctgtagtctcagatactaggaaggctgaggcaggagaatcgcttgaacccgggaggcagcagttgtggtgaactgagattgtgccactgcacttcagcctgggcaacagagtgaactccatctcaaaaaaaaaaaaaaacaaacaaacaaaaaattaatatctggattgataaataacactttcataacagtgttactttctagtatggcattgggattaggattgatgtaagggaacaaaacagctcacaaggagaaaatgtagataattttagcaattaaaataaatgttttaaaagtaaaaataagcatccaatgaggtcagcagtttttgtgtttttttgagacggaatctcactctgtcccccaggctggagtgcagtggcaccatctcagctcactgcaacctccgcctcccaggttcaagcaattctcctgtctcagcctcccgagtagctgggattacaggtacatgccaccacgcccagctaagtagagacggggtttcactgttagccaggatggccttaatcttcagaccttgtgatccgcccacctcggcctcccaaagtgctgggattacaggcatgagccactgtgcccagccgaggtcagcttttatagctgcaaaaatttagtggcaaccataatgggaatagtcattttaaagtcattaaatatgtcatgaaaataataaaaatctatatttactgaaatggcactcatgaaatctttggcatgataaaagcagttaagggtacagcatgcatatcataattacactttcttaaaaaagcaaagtatagcacgattttctctaccaaattgagagcagccatctataagtatgattacaattaattttggctttttagtttgtaattttttgctttgtgattttggcttaacaattaaaaatgtacatttgtaaaataaaaagaccggccgcagtggctcacgcctgtaatcccagcactttcggaggccgaggcgggtggatcacctgaagtcgggagattgagaccatcctggctaacatggtgaaaccccgtctctactaaaaatacaaaaaattagccgggtgttgtggcacatgcctgtaatcccaactactcaaaaggctgaggcagaagaaccacttgaacctgggaggcgaaggttgtgacgagccgagattgcaccattgcactccagcctaggcaacaagagcgaaactccgtctcaacaaaaaataaagccaggtgcaatcgctcatgcctgtaatcccagcactttgggaggctgaggcaggtggatcacctgaggtcaggagttcaagactatcctgaccaacatggagaaaccctgtctctactaaaaatagaaaattagcagggtgtggtggcacacgcctgtgatcccagctactcaggagtctgaggcaggagaattgcttgaagccgggaggtggaggttgcagcgagccgagattgcgccactgcactccagcctgggcaacagagtgaaactccgtctcaaaaaacatataataataataataaaataaaacaaaaagactaacactaacttcaaaaacaaagttaaacctccacaaggaatttaaaaatattaaaggtcacacaattcaaacagtgtgatactggtgcaaacacaaatacacagatcagaaaagatagctctaaaaacacaagcaaatataaacatgagtataatgtgtcaccaagaaagtagaacaaaacaatgaatgaaagaattatagaacagctggcatcggtatatgactgggggagagagggaatgtcactttagactccgaatttataacctggaatgaaatacatttggatacaaaatttaaatacaaagttttaaaaaaaactacggaagagggtaactattagacatgatttttggtttaaaatatgaggaaggtgacaggggctttaatttttattatttattagtatgaattccctgatgacgaatgagatccgagccactactaaaagccttcccacattccttacagttatagggcttttcaccagtgtgaattctcagatgtcgagtaaggtttgagcatttattaaaggcctttccacattcattacattcatatggtttttcatctgtatgaattctctgatgctggaaaagttgtgagttctgagtaaaggccttcccacattcaagacattcaaagggtttctcaccagcgtgaattctctgatgttgacgaagctgtgagctctgagtaaaagcctttccacattccttacaatcatagggtttctcaccagtgtgaattctctgatgattagtaagtgctgagccactactaaaggctttgccacattccttgcactcatagggtttctcaccagtatgaattctctgatgttgaacaagctttgagctctgggtaaaggctttgccacattccttacattcatagggtttctcacctgtatgaattcgtgcatgctgaaaaagttgtgagctcttagtaaaggctttcccacatactttacattcataaggtttttcaccagtgtgaattcgctgatggtcaataagatttgagcaataactaaaggccttcccacattccttacattcatagggtttcttaccggtatggattctctgatgttgagaaaggtatgagctacaactgaaggcctttccacattccttacattcaaagggtttttcgccagtatgaattttcagatgccgagtaacatgtgaaccacaactaaagaatttcccacactctttacattcataagatttttcaccaatatgaattctctgatgttgaataaattgtgagttctgactaaaggcctttccacatttcttacattcatagggtctgtcttcattattaattatttgatggagagtaaggaatgtctgttgaataaatgtgggcatgtattcaggagtgaatatttcttgactaaaatgcccatttggatatcccagttgttttgcaaggtggcttctatattccaaaacatctccaaaactggagtactcaaggccatgctttgtaagtcccattatctccctctggcataattctatttcataaacttccttctttagagataataacttggtttcacacatcgattccagatctgaacacaggcctcttgtaagctctctgccaaccatccagggctctttcccttgttccaataaggagatcacttgaggcttaggagtgtaaagtcccattgaaaccagattgccgtagttctccaacatcacatctctgtataagtccctctgaacagggtccaggcagtcccactcctcctgagagaagtctatggacacatcactgaacatcactgatccctcagccatggcttctagtattgcagatggttagtcttccttgaggccgttctcctgtaatcccagctactcaggaggctgaggcaagagaatcgcttgaacccggaaagcagaggctgcagtgagctgagatcatgccactgcactccagcttgggcaacagagtgagactccgtcttgtatttggtttggtcaacagccattcttcctctgggtaactctcttgacgagagcagagctgaagaagaaaggaatgatgagatgccaggcctttcttgtggcccagactgagcagatcagaggtcattttggatctacagctactatctgaggtggggaggtcgagaccagcctgaccaacacggagaaaccccgtctctactgaaaatacaaaattagcagggcgtggtgacacacgcctgtaatcccagctactaggaaggctgaggcaggagaattgcttgaaccggggaggcggaggttgcggtgagccgagattgcgccattgcactccagcctgggcaacaacagcgaaactccgcccaacactccagaccagcctggtcagtcccttcaaactcccatgcacgtacctgcgggccccagccgagcctgcaagacccaggccgctcaccgcgcacttcccctaccctt

SEQ ID NO: 13459 - RNA, 7382 nt, Homo sapiens
  source 1..7382: mol_type = other RNA
gctgggattacaggcatgagccaccacgcccggctaattttttgtatttttagtagagacagggtttctccatgttggtcaggctggtctcaaatccccgacctcaggtgatccacccgccttggcctcacagaatgctgagattacaggcgtgagccaccatgcctggccagtcttatttttttaaataagtttattctggagggaggtctattaagattttacacctccagttaattctgatgtcgtcaacttattaaaaatcacagactttttccagattttcagatatattataaaaatgtctataataccaacttttaagtttgttgttttaatttttttttttttctgtagagatgaggggagggggatctcattatgttacctagactggtcttgaactcctggcctcaagccattctcctacctcagcctcccaaagtgctggaattacaggcatgagccactgcaaccagccttaagtttttaaattgagatcaaattcacacagcataatattcacccttttaaagtgtatagttgagtgacctgtagtatataaacaaaattgtacaacctttacccatgccacattttcattaccccaaatgacacagttcttttaagtttacatatatagccatttcaatttctcatatacaatattgtttatttgtcatccttatttcacctctggaatcactaaactttgtctcattttttttctcttccatcaaatatcaattttggattcagatccagtttttttctttcaattatttctgccttttaaaataatactacctccttcctcccacaattcatttcagcttgttttagttccttgggttctatattttttcttcctagtattacaatatatgcacaaatattaggttataaaacttccaatacaacttttactgccactcacaggtttttcaattgttttcattttcatgtacatttaaataatgtatatattagggatttattccttaacccatgttaattaagagggaatattgaattaataatcagatatttgatggttatcctattgtactgcttcttctggtcaaataatgttgccagtatgttttctgcattttggggggaaatattagaaaaaattttataatctcttcctgcttttttgacagctgtgctttctactactcatcatattttcagggtttcagattggtaaccgtttattttttattttgtaagacagagtctcgctctgtcacccagtctggagtgtgcagtggtgcaatctcagctcactataacctccaactcccaggttcaagcaatcctcccacctcagcctcttgagtagctaggattacaggcatgcaacaccatgcctggctatttgtttttgtttttgttttttttgtatttttagtagagacggggtttcaccatgttggccaggctggtctcgagctcctgacctcaagtgatccacccaccttggcctcccaaagtgctaggattacaggtgtgagccaccgcgcccagcctcagactggtattctttatgtagcataaaagataaagtctgaacaaagactatgcacacatactttttctcttccttttaaaattccacactgaataataatgatagggaaaggcttcgttatactcattacaagtgtttctctttttccaccatgaattacaaatttgccaaaggtaaacaacatggttaaaatcctttccataaatcctaatgaagatacttatgataatgagtatatcactgataatagtggaaaacttttactaaacctgtattatgtgataacagtttgaggtactttgcatttattaattcattgactcttcacagcaatccaatacatacagccttattatagatgcctagacataattttttaaaataccactaacagccaggggcggtggctcacacctataatcccagcactttgggaagccaaggcaggaggatcacgaggtcaggagtttgagagcagcctggccaatatggtgaaaccccatctctactaataatacaaaaattagctaggcatggtggcgcgcgcctgtagtcccagctactcgggaggctgaggcggaagactcacttgaactcgggaggcagaggttgcagtgagccgagattgcaccactgccctccagcctgggcaacagagcgagactgtgtctcaaaaaacaaaaacaccactaatagctataagaaaaaataattgaccgggcacagtggctcacacctgtaatccccgaactttgggaggccgaggtgggtggatcacaaggtcaagagttcaagaccagcctggccaacatagtgaaaccctgtctctactaaaaatacaaaaattagccaggcatggtgtcgtgcgcctgtagtctcagatactaggaaggctgaggcaggagaatcgcttgaacccgggaggcagcagttgtggtgaactgagattgtgccactgcacttcagcctgggcaacagagtgaactccatctcaaaaaaaaaaaaaaacaaacaaacaaaaaattaatatctggattgataaataacactttcataacagtgttactttctagtatggcattgggattaggattgatgtaagggaacaaaacagctcacaaggagaaaatgtagataattttagcaattaaaataaatgttttaaaagtaaaaataagcatccaatgaggtcagcagtttttgtgtttttttgagacggaatctcactctgtcccccaggctggagtgcagtggcaccatctcagctcactgcaacctccgcctcccaggttcaagcaattctcctgtctcagcctcccgagtagctgggattacaggtacatgccaccacgcccagctaagtagagacggggtttcactgttagccaggatggccttaatcttcagaccttgtgatccgcccacctcggcctcccaaagtgctgggattacaggcatgagccactgtgcccagccgaggtcagcttttatagctgcaaaaatttagtggcaaccataatgggaatagtcattttaaagtcattaaatatgtcatgaaaataataaaaatctatatttactgaaatggcactcatgaaatctttggcatgataaaagcagttaagggtacagcatgcatatcataattacactttcttaaaaaagcaaagtatagcacgattttctctaccaaattgagagcagccatctataagtatgattacaattaattttggctttttagtttgtaattttttgctttgtgattttggcttaacaattaaaaatgtacatttgtaaaataaaaagaccggccgcagtggctcacgcctgtaatcccagcactttcggaggccgaggcgggtggatcacctgaagtcgggagattgagaccatcctggctaacatggtgaaaccccgtctctactaaaaatacaaaaaattagccgggtgttgtggcacatgcctgtaatcccaactactcaaaaggctgaggcagaagaaccacttgaacctgggaggcgaaggttgtgacgagccgagattgcaccattgcactccagcctaggcaacaagagcgaaactccgtctcaacaaaaaataaagccaggtgcaatcgctcatgcctgtaatcccagcactttgggaggctgaggcaggtggatcacctgaggtcaggagttcaagactatcctgaccaacatggagaaaccctgtctctactaaaaatagaaaattagcagggtgtggtggcacacgcctgtgatcccagctactcaggagtctgaggcaggagaattgcttgaagccgggaggtggaggttgcagcgagccgagattgcgccactgcactccagcctgggcaacagagtgaaactccgtctcaaaaaacatataataataataataaaataaaacaaaaagactaacactaacttcaaaaacaaagttaaacctccacaaggaatttaaaaatattaaaggtcacacaattcaaacagtgtgatactggtgcaaacacaaatacacagatcagaaaagatagctctaaaaacacaagcaaatataaacatgagtataatgtgtcaccaagaaagtagaacaaaacaatgaatgaaagaattatagaacagctggcatcggtatatgactgggggagagagggaatgtcactttagactccgaatttataacctggaatgaaatacatttggatacaaaatttaaatacaaagttttaaaaaaaactacggaagagggtaactattagacatgatttttggtttaaaatatgaggaaggtgacaggggctttaatttttattatttattagtatgaattccctgatgacgaatgagatccgagccactactaaaagccttcccacattccttacagttatagggcttttcaccagtgtgaattctcagatgtcgagtaaggtttgagcatttattaaaggcctttccacattcattacattcatatggtttttcatctgtatgaattctctgatgctggaaaagttgtgagttctgagtaaaggccttcccacattcaagacattcaaagggtttctcaccagcgtgaattctctgatgttgacgaagctgtgagctctgagtaaaagcctttccacattccttacaatcatagggtttctcaccagtgtgaattctctgatgattagtaagtgctgagccactactaaaggctttgccacattccttgcactcatagggtttctcaccagtatgaattctctgatgttgaacaagctttgagctctgggtaaaggctttgccacattccttacattcatagggtttctcacctgtatgaattcgtgcatgctgaaaaagttgtgagctcttagtaaaggctttcccacatactttacattcataaggtttttcaccagtgtgaattcgctgatggtcaataagatttgagcaataactaaaggccttcccacattccttacattcatagggtttcttaccggtatggattctctgatgttgagaaaggtatgagctacaactgaaggcctttccacattccttacattcaaagggtttttcgccagtatgaattttcagatgccgagtaacatgtgaaccacaactaaagaatttcccacactctttacattcataagatttttcaccaatatgaattctctgatgttgaataaattgtgagttctgactaaaggcctttccacatttcttacattcatagggtctgtcttcattattaattatttgatggagagtaaggaatgtctgttgaataaatgtgggcatgtattcaggagtgaatatttcttgactaaaatgcccatttggatatcccagttgttttgcaaggtggcttctatattccaaaacatctccaaaactggagtactcaaggccatgctttgtaagtcccattatctccctctggcataattctatttcataaacttccttctttagagataataacttggtttcacacatcgattccagatctgaacacaggcctcttgtaagctctctgccaaccatccagggctctttcccttgttccaataaggagatcacttgaggcttaggagtgtaaagtcccattgaaaccagattgccgtagttctccaacatcacatctctgtataagtccctctgaacagggtccaggcagtcccactcctcctgagagaagtctatggacacatcactgaacatcactgatccctcagccatggcttctagtattgcagatggttagtcttccttgaggccgttctcctgtaatcccagctactcaggaggctgaggcaagagaatcgcttgaacccggaaagcagaggctgcagtgagctgagatcatgccactgcactccagcttgggcaacagagtgagactccgtcttgtatttggtttggtcaacagccattcttcctctgggtaactctcttgacgagagcagagctgaagaagaaaggaatgatgagatgccaggcctttcttgtggcccagactgagcagatcagaggtcattttggatctacagctactatctgaggtggggaggtcgagaccagcctgaccaacacggagaaaccccgtctctactgaaaatacaaaattagcagggcgtggtgacacacgcctgtaatcccagctactaggaaggctgaggcaggagaattgcttgaaccggggaggcggaggttgcggtgagccgagattgcgccattgcactccagcctgggcaacaacagcgaaactccgccttaaaacaaaacaaaacaaaaacagagaagtgtaggctgtcatgagcattcttggtatcagaggggtgaggtctctcctctcgagaatctgtcctgacctcacagggagagctggagtcacaaagacagtcacaagcaccccctacccaatgctgcagtcacccagccaccatggggacccacatagacctccacaggcacgcctcacccaaacaataacactatatatggtcacacaatcattgtcccacatctaccttgaggataagttacactagcatatttacagacccctcaaacatagcaccattcagaaccagagtgctacagatagtcacaataccacacgcactactgagccacacaaagttacagttcccccctccccaggacccctattgagcactacacacaatcacacattcaaaataacacaatgaccactaggacacacatatcaccccggcacgattacacgcactttccaaccgcagacacagtgctacataaagttacatggtcacactctcacattctcacgttactgggttatttctgggtagtagatttactcagtaaggcatccagtacacttaagtgctgctaacagtcatacaaacacaattacacacacccctcagactaacacacagtcacagcctcatcagattctctccacacaaacaccctccacaaatgtcacgcaaagttacacagccacacacaatcacagtcccaacacgggacacagtcatacctacacatacagccttacattgttacaattacacaactacaacgaggatatacaatcacacccgcgcacacagagaggcacagtcacataaggtcacactcacacacggaagcccacgcctcgcgcccgcctccccaccaccccctctatcagcccgaccaactcatacatgcccgacacactcatacatgcccaacactccagaccagcctggtcagtcccttcaaactcccatgcacgtacctgcgggccccagccgagcctgcaagacccaggccgctcaccgcgcacttcccctaccctt

SEQ ID NO: 13460 - RNA, 6166 nt, Homo sapiens
  source 1..6166: mol_type = other RNA
gctgggattacaggcatgagccaccacgcccggctaattttttgtatttttagtagagacagggtttctccatgttggtcaggctggtctcaaatccccgacctcaggtgatccacccgccttggcctcacagaatgctgagattacaggcgtgagccaccatgcctggccagtcttatttttttaaataagtttattctggagggaggtctattaagattttacacctccagttaattctgatgtcgtcaacttattaaaaatcacagactttttccagattttcagatatattataaaaatgtctataataccaacttttaagtttgttgttttaatttttttttttttctgtagagatgaggggagggggatctcattatgttacctagactggtcttgaactcctggcctcaagccattctcctacctcagcctcccaaagtgctggaattacaggcatgagccactgcaaccagccttaagtttttaaattgagatcaaattcacacagcataatattcacccttttaaagtgtatagttgagtgacctgtagtatataaacaaaattgtacaacctttacccatgccacattttcattaccccaaatgacacagttcttttaagtttacatatatagccatttcaatttctcatatacaatattgtttatttgtcatccttatttcacctctggaatcactaaactttgtctcattttttttctcttccatcaaatatcaattttggattcagatccagtttttttctttcaattatttctgccttttaaaataatactacctccttcctcccacaattcatttcagcttgttttagttccttgggttctatattttttcttcctagtattacaatatatgcacaaatattaggttataaaacttccaatacaacttttactgccactcacaggtttttcaattgttttcattttcatgtacatttaaataatgtatatattagggatttattccttaacccatgttaattaagagggaatattgaattaataatcagatatttgatggttatcctattgtactgcttcttctggtcaaataatgttgccagtatgttttctgcattttggggggaaatattagaaaaaattttataatctcttcctgcttttttgacagctgtgctttctactactcatcatattttcagggtttcagattggtaaccgtttattttttattttgtaagacagagtctcgctctgtcacccagtctggagtgtgcagtggtgcaatctcagctcactataacctccaactcccaggttcaagcaatcctcccacctcagcctcttgagtagctaggattacaggcatgcaacaccatgcctggctatttgtttttgtttttgttttttttgtatttttagtagagacggggtttcaccatgttggccaggctggtctcgagctcctgacctcaagtgatccacccaccttggcctcccaaagtgctaggattacaggtgtgagccaccgcgcccagcctcagactggtattctttatgtagcataaaagataaagtctgaacaaagactatgcacacatactttttctcttccttttaaaattccacactgaataataatgatagggaaaggcttcgttatactcattacaagtgtttctctttttccaccatgaattacaaatttgccaaaggtaaacaacatggttaaaatcctttccataaatcctaatgaagatacttatgataatgagtatatcactgataatagtggaaaacttttactaaacctgtattatgtgataacagtttgaggtactttgcatttattaattcattgactcttcacagcaatccaatacatacagccttattatagatgcctagacataattttttaaaataccactaacagccaggggcggtggctcacacctataatcccagcactttgggaagccaaggcaggaggatcacgaggtcaggagtttgagagcagcctggccaatatggtgaaaccccatctctactaataatacaaaaattagctaggcatggtggcgcgcgcctgtagtcccagctactcgggaggctgaggcggaagactcacttgaactcgggaggcagaggttgcagtgagccgagattgcaccactgccctccagcctgggcaacagagcgagactgtgtctcaaaaaacaaaaacaccactaatagctataagaaaaaataattgaccgggcacagtggctcacacctgtaatccccgaactttgggaggccgaggtgggtggatcacaaggtcaagagttcaagaccagcctggccaacatagtgaaaccctgtctctactaaaaatacaaaaattagccaggcatggtgtcgtgcgcctgtagtctcagatactaggaaggctgaggcaggagaatcgcttgaacccgggaggcagcagttgtggtgaactgagattgtgccactgcacttcagcctgggcaacagagtgaactccatctcaaaaaaaaaaaaaaacaaacaaacaaaaaattaatatctggattgataaataacactttcataacagtgttactttctagtatggcattgggattaggattgatgtaagggaacaaaacagctcacaaggagaaaatgtagataattttagcaattaaaataaatgttttaaaagtaaaaataagcatccaatgaggtcagcagtttttgtgtttttttgagacggaatctcactctgtcccccaggctggagtgcagtggcaccatctcagctcactgcaacctccgcctcccaggttcaagcaattctcctgtctcagcctcccgagtagctgggattacaggtacatgccaccacgcccagctaagtagagacggggtttcactgttagccaggatggccttaatcttcagaccttgtgatccgcccacctcggcctcccaaagtgctgggattacaggcatgagccactgtgcccagccgaggtcagcttttatagctgcaaaaatttagtggcaaccataatgggaatagtcattttaaagtcattaaatatgtcatgaaaataataaaaatctatatttactgaaatggcactcatgaaatctttggcatgataaaagcagttaagggtacagcatgcatatcataattacactttcttaaaaaagcaaagtatagcacgattttctctaccaaattgagagcagccatctataagtatgattacaattaattttggctttttagtttgtaattttttgctttgtgattttggcttaacaattaaaaatgtacatttgtaaaataaaaagaccggccgcagtggctcacgcctgtaatcccagcactttcggaggccgaggcgggtggatcacctgaagtcgggagattgagaccatcctggctaacatggtgaaaccccgtctctactaaaaatacaaaaaattagccgggtgttgtggcacatgcctgtaatcccaactactcaaaaggctgaggcagaagaaccacttgaacctgggaggcgaaggttgtgacgagccgagattgcaccattgcactccagcctaggcaacaagagcgaaactccgtctcaacaaaaaataaagccaggtgcaatcgctcatgcctgtaatcccagcactttgggaggctgaggcaggtggatcacctgaggtcaggagttcaagactatcctgaccaacatggagaaaccctgtctctactaaaaatagaaaattagcagggtgtggtggcacacgcctgtgatcccagctactcaggagtctgaggcaggagaattgcttgaagccgggaggtggaggttgcagcgagccgagattgcgccactgcactccagcctgggcaacagagtgaaactccgtctcaaaaaacatataataataataataaaataaaacaaaaagactaacactaacttcaaaaacaaagttaaacctccacaaggaatttaaaaatattaaaggtcacacaattcaaacagtgtgatactggtgcaaacacaaatacacagatcagaaaagatagctctaaaaacacaagcaaatataaacatgagtataatgtgtcaccaagaaagtagaacaaaacaatgaatgaaagaattatagaacagctggcatcggtatatgactgggggagagagggaatgtcactttagactccgaatttataacctggaatgaaatacatttggatacaaaatttaaatacaaagttttaaaaaaaactacggaagagggtaactattagacatgatttttggtttaaaatatgaggaaggtgacaggggctttaatttttattatttattagtatgaattccctgatgacgaatgagatccgagccactactaaaagccttcccacattccttacagttatagggcttttcaccagtgtgaattctcagatgtcgagtaaggtttgagcatttattaaaggcctttccacattcattacattcatatggtttttcatctgtatgaattctctgatgctggaaaagttgtgagttctgagtaaaggccttcccacattcaagacattcaaagggtttctcaccagcgtgaattctctgatgttgacgaagctgtgagctctgagtaaaagcctttccacattccttacaatcatagggtttctcaccagtgtgaattctctgatgattagtaagtgctgagccactactaaaggctttgccacattccttgcactcatagggtttctcaccagtatgaattctctgatgttgaacaagctttgagctctgggtaaaggctttgccacattccttacattcatagggtttctcacctgtatgaattcgtgcatgctgaaaaagttgtgagctcttagtaaaggctttcccacatactttacattcataaggtttttcaccagtgtgaattcgctgatggtcaataagatttgagcaataactaaaggccttcccacattccttacattcatagggtttcttaccggtatggattctctgatgttgagaaaggtatgagctacaactgaaggcctttccacattccttacattcaaagggtttttcgccagtatgaattttcagatgccgagtaacatgtgaaccacaactaaagaatttcccacactctttacattcataagatttttcaccaatatgaattctctgatgttgaataaattgtgagttctgactaaaggcctttccacatttcttacattcatagggtctgtcttcattattaattatttgatggagagtaaggaatgtctgttgaataaatgtgggcatgtattcaggagtgaatatttcttgactaaaatgcccatttggatatcccagttgttttgcaaggtggcttctatattccaaaacatctccaaaactggagtactcaaggccatgctttgtaagtcccattatctccctctggcataattctatttcataaacttccttctttagagataataacttggtttcacacatcgattccagatctgaacacaggcctcttgtaagctctctgccaaccatccagggctctttcccttgttccaataaggagatcacttgaggcttaggagtgtaaagtcccattgaaaccagattgccgtagttctccaacatcacatctctgtataagtccctctgaacagggtccaggcagtcccactcctcctgagagaagtctatggacacatcactgaacatcactgatccctcagccatggcttctagtattgcagatggttagtcttccttgaggccgttctcctgtaatcccagctactcaggaggctgaggcaagagaatcgcttgaacccggaaagcagaggctgcagtgagctgagatcatgccactgcactccagcttgggcaacagagtgagactccgtcttgtatttggtttggtcaacagccattcttcctctgggtaactctcttgacgagagcagagctgaagaagaaaggaatgatgagatgccaggcctttcttgtggcccagactgagcagatcagaggtcattttggatctacagctactatctgcgggccccagccgagcctgcaagacccaggccgctcaccgcgcacttcccctaccctt

SEQ ID NO: 13461 - RNA, 6077 nt, Homo sapiens
  source 1..6077: mol_type = other RNA
gctgggattacaggcatgagccaccacgcccggctaattttttgtatttttagtagagacagggtttctccatgttggtcaggctggtctcaaatccccgacctcaggtgatccacccgccttggcctcacagaatgctgagattacaggcgtgagccaccatgcctggccagtcttatttttttaaataagtttattctggagggaggtctattaagattttacacctccagttaattctgatgtcgtcaacttattaaaaatcacagactttttccagattttcagatatattataaaaatgtctataataccaacttttaagtttgttgttttaatttttttttttttctgtagagatgaggggagggggatctcattatgttacctagactggtcttgaactcctggcctcaagccattctcctacctcagcctcccaaagtgctggaattacaggcatgagccactgcaaccagccttaagtttttaaattgagatcaaattcacacagcataatattcacccttttaaagtgtatagttgagtgacctgtagtatataaacaaaattgtacaacctttacccatgccacattttcattaccccaaatgacacagttcttttaagtttacatatatagccatttcaatttctcatatacaatattgtttatttgtcatccttatttcacctctggaatcactaaactttgtctcattttttttctcttccatcaaatatcaattttggattcagatccagtttttttctttcaattatttctgccttttaaaataatactacctccttcctcccacaattcatttcagcttgttttagttccttgggttctatattttttcttcctagtattacaatatatgcacaaatattaggttataaaacttccaatacaacttttactgccactcacaggtttttcaattgttttcattttcatgtacatttaaataatgtatatattagggatttattccttaacccatgttaattaagagggaatattgaattaataatcagatatttgatggttatcctattgtactgcttcttctggtcaaataatgttgccagtatgttttctgcattttggggggaaatattagaaaaaattttataatctcttcctgcttttttgacagctgtgctttctactactcatcatattttcagggtttcagattggtaaccgtttattttttattttgtaagacagagtctcgctctgtcacccagtctggagtgtgcagtggtgcaatctcagctcactataacctccaactcccaggttcaagcaatcctcccacctcagcctcttgagtagctaggattacaggcatgcaacaccatgcctggctatttgtttttgtttttgttttttttgtatttttagtagagacggggtttcaccatgttggccaggctggtctcgagctcctgacctcaagtgatccacccaccttggcctcccaaagtgctaggattacaggtgtgagccaccgcgcccagcctcagactggtattctttatgtagcataaaagataaagtctgaacaaagactatgcacacatactttttctcttccttttaaaattccacactgaataataatgatagggaaaggcttcgttatactcattacaagtgtttctctttttccaccatgaattacaaatttgccaaaggtaaacaacatggttaaaatcctttccataaatcctaatgaagatacttatgataatgagtatatcactgataatagtggaaaacttttactaaacctgtattatgtgataacagtttgaggtactttgcatttattaattcattgactcttcacagcaatccaatacatacagccttattatagatgcctagacataattttttaaaataccactaacagccaggggcggtggctcacacctataatcccagcactttgggaagccaaggcaggaggatcacgaggtcaggagtttgagagcagcctggccaatatggtgaaaccccatctctactaataatacaaaaattagctaggcatggtggcgcgcgcctgtagtcccagctactcgggaggctgaggcggaagactcacttgaactcgggaggcagaggttgcagtgagccgagattgcaccactgccctccagcctgggcaacagagcgagactgtgtctcaaaaaacaaaaacaccactaatagctataagaaaaaataattgaccgggcacagtggctcacacctgtaatccccgaactttgggaggccgaggtgggtggatcacaaggtcaagagttcaagaccagcctggccaacatagtgaaaccctgtctctactaaaaatacaaaaattagccaggcatggtgtcgtgcgcctgtagtctcagatactaggaaggctgaggcaggagaatcgcttgaacccgggaggcagcagttgtggtgaactgagattgtgccactgcacttcagcctgggcaacagagtgaactccatctcaaaaaaaaaaaaaaacaaacaaacaaaaaattaatatctggattgataaataacactttcataacagtgttactttctagtatggcattgggattaggattgatgtaagggaacaaaacagctcacaaggagaaaatgtagataattttagcaattaaaataaatgttttaaaagtaaaaataagcatccaatgaggtcagcagtttttgtgtttttttgagacggaatctcactctgtcccccaggctggagtgcagtggcaccatctcagctcactgcaacctccgcctcccaggttcaagcaattctcctgtctcagcctcccgagtagctgggattacaggtacatgccaccacgcccagctaagtagagacggggtttcactgttagccaggatggccttaatcttcagaccttgtgatccgcccacctcggcctcccaaagtgctgggattacaggcatgagccactgtgcccagccgaggtcagcttttatagctgcaaaaatttagtggcaaccataatgggaatagtcattttaaagtcattaaatatgtcatgaaaataataaaaatctatatttactgaaatggcactcatgaaatctttggcatgataaaagcagttaagggtacagcatgcatatcataattacactttcttaaaaaagcaaagtatagcacgattttctctaccaaattgagagcagccatctataagtatgattacaattaattttggctttttagtttgtaattttttgctttgtgattttggcttaacaattaaaaatgtacatttgtaaaataaaaagaccggccgcagtggctcacgcctgtaatcccagcactttcggaggccgaggcgggtggatcacctgaagtcgggagattgagaccatcctggctaacatggtgaaaccccgtctctactaaaaatacaaaaaattagccgggtgttgtggcacatgcctgtaatcccaactactcaaaaggctgaggcagaagaaccacttgaacctgggaggcgaaggttgtgacgagccgagattgcaccattgcactccagcctaggcaacaagagcgaaactccgtctcaacaaaaaataaagccaggtgcaatcgctcatgcctgtaatcccagcactttgggaggctgaggcaggtggatcacctgaggtcaggagttcaagactatcctgaccaacatggagaaaccctgtctctactaaaaatagaaaattagcagggtgtggtggcacacgcctgtgatcccagctactcaggagtctgaggcaggagaattgcttgaagccgggaggtggaggttgcagcgagccgagattgcgccactgcactccagcctgggcaacagagtgaaactccgtctcaaaaaacatataataataataataaaataaaacaaaaagactaacactaacttcaaaaacaaagttaaacctccacaaggaatttaaaaatattaaaggtcacacaattcaaacagtgtgatactggtgcaaacacaaatacacagatcagaaaagatagctctaaaaacacaagcaaatataaacatgagtataatgtgtcaccaagaaagtagaacaaaacaatgaatgaaagaattatagaacagctggcatcggtatatgactgggggagagagggaatgtcactttagactccgaatttataacctggaatgaaatacatttggatacaaaatttaaatacaaagttttaaaaaaaactacggaagagggtaactattagacatgatttttggtttaaaatatgaggaaggtgacaggggctttaatttttattatttattagtatgaattccctgatgacgaatgagatccgagccactactaaaagccttcccacattccttacagttatagggcttttcaccagtgtgaattctcagatgtcgagtaaggtttgagcatttattaaaggcctttccacattcattacattcatatggtttttcatctgtatgaattctctgatgctggaaaagttgtgagttctgagtaaaggccttcccacattcaagacattcaaagggtttctcaccagcgtgaattctctgatgttgacgaagctgtgagctctgagtaaaagcctttccacattccttacaatcatagggtttctcaccagtgtgaattctctgatgattagtaagtgctgagccactactaaaggctttgccacattccttgcactcatagggtttctcaccagtatgaattctctgatgttgaacaagctttgagctctgggtaaaggctttgccacattccttacattcatagggtttctcacctgtatgaattcgtgcatgctgaaaaagttgtgagctcttagtaaaggctttcccacatactttacattcataaggtttttcaccagtgtgaattcgctgatggtcaataagatttgagcaataactaaaggccttcccacattccttacattcatagggtttcttaccggtatggattctctgatgttgagaaaggtatgagctacaactgaaggcctttccacattccttacattcaaagggtttttcgccagtatgaattttcagatgccgagtaacatgtgaaccacaactaaagaatttcccacactctttacattcataagatttttcaccaatatgaattctctgatgttgaataaattgtgagttctgactaaaggcctttccacatttcttacattcatagggtctgtcttcattattaattatttgatggagagtaaggaatgtctgttgaataaatgtgggcatgtattcaggagtgaatatttcttgactaaaatgcccatttggatatcccagttgttttgcaaggtggcttctatattccaaaacatctccaaaactggagtactcaaggccatgctttgtaagtcccattatctccctctggcataattctatttcataaacttccttctttagagataataacttggtttcacacatcgattccagatctgaacacaggcctcttgtaagctctctgccaaccatccagggctctttcccttgttccaataaggagatcacttgaggcttaggagtgtaaagtcccattgaaaccagattgccgtagttctccaacatcacatctctgtataagtccctctgaacagggtccaggcagtcccactcctcctgagagaagtctatggacacatcactgaacatcactgatccctcagccatggcttctagtattgcagatggttagtcttccttgaggccgttctcctgtaatcccagctactcaggaggctgaggcaagagaatcgcttgaacccggaaagcagaggctgcagtgagctgagatcatgccactgcactccagcttgggcaacagagtgagactccgtcttgtatttggtttggtcaacagccattcttcctctgggtaactctcttgacgagagcagagctgcgggccccagccgagcctgcaagacccaggccgctcaccgcgcacttcccctaccctt

SEQ ID NO: 13462 - RNA, 7260 nt, Homo sapiens
  source 1..7260: mol_type = other RNA
gctgggattacaggcatgagccaccacgcccggctaattttttgtatttttagtagagacagggtttctccatgttggtcaggctggtctcaaatccccgacctcaggtgatccacccgccttggcctcacagaatgctgagattacaggcgtgagccaccatgcctggccagtcttatttttttaaataagtttattctggagggaggtctattaagattttacacctccagttaattctgatgtcgtcaacttattaaaaatcacagactttttccagattttcagatatattataaaaatgtctataataccaacttttaagtttgttgttttaatttttttttttttctgtagagatgaggggagggggatctcattatgttacctagactggtcttgaactcctggcctcaagccattctcctacctcagcctcccaaagtgctggaattacaggcatgagccactgcaaccagccttaagtttttaaattgagatcaaattcacacagcataatattcacccttttaaagtgtatagttgagtgacctgtagtatataaacaaaattgtacaacctttacccatgccacattttcattaccccaaatgacacagttcttttaagtttacatatatagccatttcaatttctcatatacaatattgtttatttgtcatccttatttcacctctggaatcactaaactttgtctcattttttttctcttccatcaaatatcaattttggattcagatccagtttttttctttcaattatttctgccttttaaaataatactacctccttcctcccacaattcatttcagcttgttttagttccttgggttctatattttttcttcctagtattacaatatatgcacaaatattaggttataaaacttccaatacaacttttactgccactcacaggtttttcaattgttttcattttcatgtacatttaaataatgtatatattagggatttattccttaacccatgttaattaagagggaatattgaattaataatcagatatttgatggttatcctattgtactgcttcttctggtcaaataatgttgccagtatgttttctgcattttggggggaaatattagaaaaaattttataatctcttcctgcttttttgacagctgtgctttctactactcatcatattttcagggtttcagattggtaaccgtttattttttattttgtaagacagagtctcgctctgtcacccagtctggagtgtgcagtggtgcaatctcagctcactataacctccaactcccaggttcaagcaatcctcccacctcagcctcttgagtagctaggattacaggcatgcaacaccatgcctggctatttgtttttgtttttgttttttttgtatttttagtagagacggggtttcaccatgttggccaggctggtctcgagctcctgacctcaagtgatccacccaccttggcctcccaaagtgctaggattacaggtgtgagccaccgcgcccagcctcagactggtattctttatgtagcataaaagataaagtctgaacaaagactatgcacacatactttttctcttccttttaaaattccacactgaataataatgatagggaaaggcttcgttatactcattacaagtgtttctctttttccaccatgaattacaaatttgccaaaggtaaacaacatggttaaaatcctttccataaatcctaatgaagatacttatgataatgagtatatcactgataatagtggaaaacttttactaaacctgtattatgtgataacagtttgaggtactttgcatttattaattcattgactcttcacagcaatccaatacatacagccttattatagatgcctagacataattttttaaaataccactaacagccaggggcggtggctcacacctataatcccagcactttgggaagccaaggcaggaggatcacgaggtcaggagtttgagagcagcctggccaatatggtgaaaccccatctctactaataatacaaaaattagctaggcatggtggcgcgcgcctgtagtcccagctactcgggaggctgaggcggaagactcacttgaactcgggaggcagaggttgcagtgagccgagattgcaccactgccctccagcctgggcaacagagcgagactgtgtctcaaaaaacaaaaacaccactaatagctataagaaaaaataattgaccgggcacagtggctcacacctgtaatccccgaactttgggaggccgaggtgggtggatcacaaggtcaagagttcaagaccagcctggccaacatagtgaaaccctgtctctactaaaaatacaaaaattagccaggcatggtgtcgtgcgcctgtagtctcagatactaggaaggctgaggcaggagaatcgcttgaacccgggaggcagcagttgtggtgaactgagattgtgccactgcacttcagcctgggcaacagagtgaactccatctcaaaaaaaaaaaaaaacaaacaaacaaaaaattaatatctggattgataaataacactttcataacagtgttactttctagtatggcattgggattaggattgatgtaagggaacaaaacagctcacaaggagaaaatgtagataattttagcaattaaaataaatgttttaaaagtaaaaataagcatccaatgaggtcagcagtttttgtgtttttttgagacggaatctcactctgtcccccaggctggagtgcagtggcaccatctcagctcactgcaacctccgcctcccaggttcaagcaattctcctgtctcagcctcccgagtagctgggattacaggtacatgccaccacgcccagctaagtagagacggggtttcactgttagccaggatggccttaatcttcagaccttgtgatccgcccacctcggcctcccaaagtgctgggattacaggcatgagccactgtgcccagccgaggtcagcttttatagctgcaaaaatttagtggcaaccataatgggaatagtcattttaaagtcattaaatatgtcatgaaaataataaaaatctatatttactgaaatggcactcatgaaatctttggcatgataaaagcagttaagggtacagcatgcatatcataattacactttcttaaaaaagcaaagtatagcacgattttctctaccaaattgagagcagccatctataagtatgattacaattaattttggctttttagtttgtaattttttgctttgtgattttggcttaacaattaaaaatgtacatttgtaaaataaaaagaccggccgcagtggctcacgcctgtaatcccagcactttcggaggccgaggcgggtggatcacctgaagtcgggagattgagaccatcctggctaacatggtgaaaccccgtctctactaaaaatacaaaaaattagccgggtgttgtggcacatgcctgtaatcccaactactcaaaaggctgaggcagaagaaccacttgaacctgggaggcgaaggttgtgacgagccgagattgcaccattgcactccagcctaggcaacaagagcgaaactccgtctcaacaaaaaataaagccaggtgcaatcgctcatgcctgtaatcccagcactttgggaggctgaggcaggtggatcacctgaggtcaggagttcaagactatcctgaccaacatggagaaaccctgtctctactaaaaatagaaaattagcagggtgtggtggcacacgcctgtgatcccagctactcaggagtctgaggcaggagaattgcttgaagccgggaggtggaggttgcagcgagccgagattgcgccactgcactccagcctgggcaacagagtgaaactccgtctcaaaaaacatataataataataataaaataaaacaaaaagactaacactaacttcaaaaacaaagttaaacctccacaaggaatttaaaaatattaaaggtcacacaattcaaacagtgtgatactggtgcaaacacaaatacacagatcagaaaagatagctctaaaaacacaagcaaatataaacatgagtataatgtgtcaccaagaaagtagaacaaaacaatgaatgaaagaattatagaacagctggcatcggtatatgactgggggagagagggaatgtcactttagactccgaatttataacctggaatgaaatacatttggatacaaaatttaaatacaaagttttaaaaaaaactacggaagagggtaactattagacatgatttttggtttaaaatatgaggaaggtgacaggggctttaatttttattatttattagtatgaattccctgatgacgaatgagatccgagccactactaaaagccttcccacattccttacagttatagggcttttcaccagtgtgaattctcagatgtcgagtaaggtttgagcatttattaaaggcctttccacattcattacattcatatggtttttcatctgtatgaattctctgatgctggaaaagttgtgagttctgagtaaaggccttcccacattcaagacattcaaagggtttctcaccagcgtgaattctctgatgttgacgaagctgtgagctctgagtaaaagcctttccacattccttacaatcatagggtttctcaccagtgtgaattctctgatgattagtaagtgctgagccactactaaaggctttgccacattccttgcactcatagggtttctcaccagtatgaattctctgatgttgaacaagctttgagctctgggtaaaggctttgccacattccttacattcatagggtttctcacctgtatgaattcgtgcatgctgaaaaagttgtgagctcttagtaaaggctttcccacatactttacattcataaggtttttcaccagtgtgaattcgctgatggtcaataagatttgagcaataactaaaggccttcccacattccttacattcatagggtttcttaccggtatggattctctgatgttgagaaaggtatgagctacaactgaaggcctttccacattccttacattcaaagggtttttcgccagtatgaattttcagatgccgagtaacatgtgaaccacaactaaagaatttcccacactctttacattcataagatttttcaccaatatgaattctctgatgttgaataaattgtgagttctgactaaaggcctttccacatttcttacattcatagggtctgtcttcattattaattatttgatggagagtaaggaatgtctgttgaataaatgtgggcatgtattcaggagtgaatatttcttgactaaaatgcccatttggatatcccagttgttttgcaaggtggcttctatattccaaaacatctccaaaactggagtactcaaggccatgctttgtaagtcccattatctccctctggcataattctatttcataaacttccttctttagagataataacttggtttcacacatcgattccagatctgaacacaggcctcttgtaagctctctgccaaccatccagggctctttcccttgttccaataaggagatcacttgaggcttaggagtgtaaagtcccattgaaaccagattgccgtagttctccaacatcacatctctgtataagtccctctgaacagggtccaggcagtcccactcctcctgagagaagtctatggacacatcactgaacatcactgatccctcagccatggcttctagtattgcagatggttagtcttccttgaggccgttctccttgtatttggtttggtcaacagccattcttcctctgggtaactctcttgacgagagcagagctgaagaagaaaggaatgatgagatgccaggcctttcttgtggcccagactgagcagatcagaggtcattttggatctacagctactatctgaggtggggaggtcgagaccagcctgaccaacacggagaaaccccgtctctactgaaaatacaaaattagcagggcgtggtgacacacgcctgtaatcccagctactaggaaggctgaggcaggagaattgcttgaaccggggaggcggaggttgcggtgagccgagattgcgccattgcactccagcctgggcaacaacagcgaaactccgccttaaaacaaaacaaaacaaaaacagagaagtgtaggctgtcatgagcattcttggtatcagaggggtgaggtctctcctctcgagaatctgtcctgacctcacagggagagctggagtcacaaagacagtcacaagcaccccctacccaatgctgcagtcacccagccaccatggggacccacatagacctccacaggcacgcctcacccaaacaataacactatatatggtcacacaatcattgtcccacatctaccttgaggataagttacactagcatatttacagacccctcaaacatagcaccattcagaaccagagtgctacagatagtcacaataccacacgcactactgagccacacaaagttacagttcccccctccccaggacccctattgagcactacacacaatcacacattcaaaataacacaatgaccactaggacacacatatcaccccggcacgattacacgcactttccaaccgcagacacagtgctacataaagttacatggtcacactctcacattctcacgttactgggttatttctgggtagtagatttactcagtaaggcatccagtacacttaagtgctgctaacagtcatacaaacacaattacacacacccctcagactaacacacagtcacagcctcatcagattctctccacacaaacaccctccacaaatgtcacgcaaagttacacagccacacacaatcacagtcccaacacgggacacagtcatacctacacatacagccttacattgttacaattacacaactacaacgaggatatacaatcacacccgcgcacacagagaggcacagtcacataaggtcacactcacacacggaagcccacgcctcgcgcccgcctccccaccaccccctctatcagcccgaccaactcatacatgcccgacacactcatacatgcccaacactccagaccagcctggtcagtcccttcaaactcccatgcacgtacctgcgggccccagccgagcctgcaagacccaggccgctcaccgcgcacttcccctaccctt

SEQ ID NO: 13463 - RNA, 5955 nt, Homo sapiens
  source 1..5955: mol_type = other RNA
gctgggattacaggcatgagccaccacgcccggctaattttttgtatttttagtagagacagggtttctccatgttggtcaggctggtctcaaatccccgacctcaggtgatccacccgccttggcctcacagaatgctgagattacaggcgtgagccaccatgcctggccagtcttatttttttaaataagtttattctggagggaggtctattaagattttacacctccagttaattctgatgtcgtcaacttattaaaaatcacagactttttccagattttcagatatattataaaaatgtctataataccaacttttaagtttgttgttttaatttttttttttttctgtagagatgaggggagggggatctcattatgttacctagactggtcttgaactcctggcctcaagccattctcctacctcagcctcccaaagtgctggaattacaggcatgagccactgcaaccagccttaagtttttaaattgagatcaaattcacacagcataatattcacccttttaaagtgtatagttgagtgacctgtagtatataaacaaaattgtacaacctttacccatgccacattttcattaccccaaatgacacagttcttttaagtttacatatatagccatttcaatttctcatatacaatattgtttatttgtcatccttatttcacctctggaatcactaaactttgtctcattttttttctcttccatcaaatatcaattttggattcagatccagtttttttctttcaattatttctgccttttaaaataatactacctccttcctcccacaattcatttcagcttgttttagttccttgggttctatattttttcttcctagtattacaatatatgcacaaatattaggttataaaacttccaatacaacttttactgccactcacaggtttttcaattgttttcattttcatgtacatttaaataatgtatatattagggatttattccttaacccatgttaattaagagggaatattgaattaataatcagatatttgatggttatcctattgtactgcttcttctggtcaaataatgttgccagtatgttttctgcattttggggggaaatattagaaaaaattttataatctcttcctgcttttttgacagctgtgctttctactactcatcatattttcagggtttcagattggtaaccgtttattttttattttgtaagacagagtctcgctctgtcacccagtctggagtgtgcagtggtgcaatctcagctcactataacctccaactcccaggttcaagcaatcctcccacctcagcctcttgagtagctaggattacaggcatgcaacaccatgcctggctatttgtttttgtttttgttttttttgtatttttagtagagacggggtttcaccatgttggccaggctggtctcgagctcctgacctcaagtgatccacccaccttggcctcccaaagtgctaggattacaggtgtgagccaccgcgcccagcctcagactggtattctttatgtagcataaaagataaagtctgaacaaagactatgcacacatactttttctcttccttttaaaattccacactgaataataatgatagggaaaggcttcgttatactcattacaagtgtttctctttttccaccatgaattacaaatttgccaaaggtaaacaacatggttaaaatcctttccataaatcctaatgaagatacttatgataatgagtatatcactgataatagtggaaaacttttactaaacctgtattatgtgataacagtttgaggtactttgcatttattaattcattgactcttcacagcaatccaatacatacagccttattatagatgcctagacataattttttaaaataccactaacagccaggggcggtggctcacacctataatcccagcactttgggaagccaaggcaggaggatcacgaggtcaggagtttgagagcagcctggccaatatggtgaaaccccatctctactaataatacaaaaattagctaggcatggtggcgcgcgcctgtagtcccagctactcgggaggctgaggcggaagactcacttgaactcgggaggcagaggttgcagtgagccgagattgcaccactgccctccagcctgggcaacagagcgagactgtgtctcaaaaaacaaaaacaccactaatagctataagaaaaaataattgaccgggcacagtggctcacacctgtaatccccgaactttgggaggccgaggtgggtggatcacaaggtcaagagttcaagaccagcctggccaacatagtgaaaccctgtctctactaaaaatacaaaaattagccaggcatggtgtcgtgcgcctgtagtctcagatactaggaaggctgaggcaggagaatcgcttgaacccgggaggcagcagttgtggtgaactgagattgtgccactgcacttcagcctgggcaacagagtgaactccatctcaaaaaaaaaaaaaaacaaacaaacaaaaaattaatatctggattgataaataacactttcataacagtgttactttctagtatggcattgggattaggattgatgtaagggaacaaaacagctcacaaggagaaaatgtagataattttagcaattaaaataaatgttttaaaagtaaaaataagcatccaatgaggtcagcagtttttgtgtttttttgagacggaatctcactctgtcccccaggctggagtgcagtggcaccatctcagctcactgcaacctccgcctcccaggttcaagcaattctcctgtctcagcctcccgagtagctgggattacaggtacatgccaccacgcccagctaagtagagacggggtttcactgttagccaggatggccttaatcttcagaccttgtgatccgcccacctcggcctcccaaagtgctgggattacaggcatgagccactgtgcccagccgaggtcagcttttatagctgcaaaaatttagtggcaaccataatgggaatagtcattttaaagtcattaaatatgtcatgaaaataataaaaatctatatttactgaaatggcactcatgaaatctttggcatgataaaagcagttaagggtacagcatgcatatcataattacactttcttaaaaaagcaaagtatagcacgattttctctaccaaattgagagcagccatctataagtatgattacaattaattttggctttttagtttgtaattttttgctttgtgattttggcttaacaattaaaaatgtacatttgtaaaataaaaagaccggccgcagtggctcacgcctgtaatcccagcactttcggaggccgaggcgggtggatcacctgaagtcgggagattgagaccatcctggctaacatggtgaaaccccgtctctactaaaaatacaaaaaattagccgggtgttgtggcacatgcctgtaatcccaactactcaaaaggctgaggcagaagaaccacttgaacctgggaggcgaaggttgtgacgagccgagattgcaccattgcactccagcctaggcaacaagagcgaaactccgtctcaacaaaaaataaagccaggtgcaatcgctcatgcctgtaatcccagcactttgggaggctgaggcaggtggatcacctgaggtcaggagttcaagactatcctgaccaacatggagaaaccctgtctctactaaaaatagaaaattagcagggtgtggtggcacacgcctgtgatcccagctactcaggagtctgaggcaggagaattgcttgaagccgggaggtggaggttgcagcgagccgagattgcgccactgcactccagcctgggcaacagagtgaaactccgtctcaaaaaacatataataataataataaaataaaacaaaaagactaacactaacttcaaaaacaaagttaaacctccacaaggaatttaaaaatattaaaggtcacacaattcaaacagtgtgatactggtgcaaacacaaatacacagatcagaaaagatagctctaaaaacacaagcaaatataaacatgagtataatgtgtcaccaagaaagtagaacaaaacaatgaatgaaagaattatagaacagctggcatcggtatatgactgggggagagagggaatgtcactttagactccgaatttataacctggaatgaaatacatttggatacaaaatttaaatacaaagttttaaaaaaaactacggaagagggtaactattagacatgatttttggtttaaaatatgaggaaggtgacaggggctttaatttttattatttattagtatgaattccctgatgacgaatgagatccgagccactactaaaagccttcccacattccttacagttatagggcttttcaccagtgtgaattctcagatgtcgagtaaggtttgagcatttattaaaggcctttccacattcattacattcatatggtttttcatctgtatgaattctctgatgctggaaaagttgtgagttctgagtaaaggccttcccacattcaagacattcaaagggtttctcaccagcgtgaattctctgatgttgacgaagctgtgagctctgagtaaaagcctttccacattccttacaatcatagggtttctcaccagtgtgaattctctgatgattagtaagtgctgagccactactaaaggctttgccacattccttgcactcatagggtttctcaccagtatgaattctctgatgttgaacaagctttgagctctgggtaaaggctttgccacattccttacattcatagggtttctcacctgtatgaattcgtgcatgctgaaaaagttgtgagctcttagtaaaggctttcccacatactttacattcataaggtttttcaccagtgtgaattcgctgatggtcaataagatttgagcaataactaaaggccttcccacattccttacattcatagggtttcttaccggtatggattctctgatgttgagaaaggtatgagctacaactgaaggcctttccacattccttacattcaaagggtttttcgccagtatgaattttcagatgccgagtaacatgtgaaccacaactaaagaatttcccacactctttacattcataagatttttcaccaatatgaattctctgatgttgaataaattgtgagttctgactaaaggcctttccacatttcttacattcatagggtctgtcttcattattaattatttgatggagagtaaggaatgtctgttgaataaatgtgggcatgtattcaggagtgaatatttcttgactaaaatgcccatttggatatcccagttgttttgcaaggtggcttctatattccaaaacatctccaaaactggagtactcaaggccatgctttgtaagtcccattatctccctctggcataattctatttcataaacttccttctttagagataataacttggtttcacacatcgattccagatctgaacacaggcctcttgtaagctctctgccaaccatccagggctctttcccttgttccaataaggagatcacttgaggcttaggagtgtaaagtcccattgaaaccagattgccgtagttctccaacatcacatctctgtataagtccctctgaacagggtccaggcagtcccactcctcctgagagaagtctatggacacatcactgaacatcactgatccctcagccatggcttctagtattgcagatggttagtcttccttgaggccgttctccttgtatttggtttggtcaacagccattcttcctctgggtaactctcttgacgagagcagagctgcgggccccagccgagcctgcaagacccaggccgctcaccgcgcacttcccctaccctt

SEQ ID NO: 13464 - RNA, 3407 nt, Homo sapiens
  source 1..3407: mol_type = other RNA
gctgggattacaggcatgagccaccacgcccggctcttctcagtttaaactcaaacctttggtgttctcatccacacttagggagttaaatacggtccctttgcagacaattcccaaatttgtatttcaagcccaaacctctctccccgaatccagactcttatatcgaactggctactcagcaactccacttgaatgcaacggacatctcaattacacctgcgtcttctccatcttgattgaaggcaactaacttcatcttcctctttttctcccacgcctgatccgccttcacaattcagaatccttccacttctcacagctgtactggatccctccaggtgggggcgactctcacctgactattactatagcctcctaagtggtttccctacttgcaaccttgcctgtataatatctatcctccacacagcaggcagggcgatcctttaagaatagaagttagatcatgaaaatgctctgctctgatccctgcaaaagctcgccacctccttacagtcaccgctgaactcgtagcagaggttcaggaggccttgctatggttccctgcggctgctctcatctcacttcccctgctcattaggccccagccacactggcctgcctgctcttcagagtttccaggtgtatgctgttgccttgctcttccctcttcttctgctcttcctccaggggtccctgggcctagctccatgtctccttccagtctctgctgacctgtcaccttttcaatgaggcccaccctcatgtgcagatgactccactgcccccgtgctccaattcccttcaccctgcccccagactttctctttccatccttcttctgtgttttggctgttgtttattatccatctctccttcctagaatattggttccctgaggtcagagatctgtgagtaaacattggcatgtcccacgtgcctggcctgcacatggcaggtgctcaataaacatttgttgactgactaagtcctagaatcagtaaaaatcagagctgaaagaaaccttaaagagatctgatccatcagcccagtggtagctacagctgctcatctcaaatgttaaaaaaaaatgatctatagttatatttactatgtatttattttaaaagttcctgcagtattaggaacagtttgtcttctgtgtcaattgtgtagctttatgaatgtaaatgctgcctatctgagaaatgtatctagttattaggaaaatcagatttctatataagcttatatttaatcagagtgaaataattacctatgagatattggcatttcatcctaattttaaaaacacagacccggaaaaaaaaaaaactgtatgattcaaatgatgccctctgccgtttctaaagcaacagaacatttgaaaagatttcgaagttatttgttaatataactttataatatatgctttcaaaacactaaatttgaatgaaactgctttgtcaccatgaaagagaaataatttcaagcagctgttttttaaaattggaaactatattgttcttactttttaaataattactaaagtgataataaaaacataatttgagtatagaaaaattatttgtcatggtaattttaaagtgctaataaaatttactttgaaaaaaatgcctggaacaagccatgctgattccctggatggaatcatggcagtaagaaaactgtcacacataccccgatactttgataagcccatattttgaaatactagactcatttgcgagtactttgcaacagacaaaatagcaggtgatgaaactgaaggctttcacttccatatacaaacccagttgtctttccttcccactaagaaacttccttggttctccagccttcatagcaaccttaacaaaactcatccggatagtacacatcttggtcagttcatacacgacttcaaagccgtggtgaactgactgggccaggagctgagcgaagagctggttgttgaagaccttgaggctgcagccgctggggatcttgcagacggtagctgggtggaagccgtgttgatagttgcagttccggctctgcacaaagatgctgctgtcactcacgcactcggcatacacctctcccccgacgtagtacaagtgcacaccctttcctatatgtctcctggtattttctatcgttgagtttctgtttacattagaaagaagtccaagacagaatctgttcctgttatttgaagggtcggtgaacccatctatgagcacacttcgggaggaagcctggaatgtctccccaactcggttgttcagttcatagtaggcgaccgagcaccagtgctggggctcctcgtaacaaactggtcgaaagtctccatttggtatcgatagcactacatgtctatcagctgtggcatctacaggttggccactctgggtctcagaggcttctgtggcatgataaggcaggggtggtgtgtcaactgagtgttgatagggactctctggctcagaaggacttcctggggagtgagggtagctggccgtgcacggggactgggagaacgcgtggctgggtgagggagggagtgcagagcacggaggctgctggaaagagtcaggataggtggcgttgtgtggcatgagtggctcactgtgcagggaggcgctgcggaacttggccaggaggctgagctgggggttatattcactgtgtcttggcacgagcacaggaggcagtactggagtctccacccggcggtagtggtaagggttaatgcacacttctttctgcttggagccaaatgggaactcacagcactccagcggcttcagctcgtggtgggactgcagatccggccagcgccacacgcgacagtaaatcacatggggcaggcccttgcggtgggacacctgcagccgcccgtccagggagcggggaatcgtgacgcatttgctgggctgccccgggcagctgagagccctctccagctcgtccatggctcccttcttcttctttaacttcttcactagagagtccactgccttctctgcccacttttcctcttcatctccttgcttccagcctagcagtctcttcactgcggggctggtgaaggagaagagggagctgatgggggtggtggagtgcataagaggccacagcaggctccggcgcgcacgggaaccgcacagcccttcacggcaaagtgggcggcgagtagctctccaggggtggcatagggaccaacccgcccgttcttctgggagcagctgggaccaattcaagttgcgaagtgtgttgactttctcctaagcccttgaacagggtggccaactctctgagatttcttgccagcacctggagcccgaaaccagaagagttgtcagcccaacaagaatataggatcaccggcccatcagtct

SEQ ID NO: 13465 - RNA, 3180 nt, Homo sapiens
  source 1..3180: mol_type = other RNA
gctgggattacaggcatgagccaccacgcccggctcttctcagtttaaactcaaacctttggtgttctcatccacacttagggagttaaatacggtccctttgcagacaattcccaaatttgtatttcaagcccaaacctctctccccgaatccagactcttatatcgaactggctactcagcaactccacttgaatgcaacggacatctcaattacacctgcgtcttctccatcttgattgaaggcaactaacttcatcttcctctttttctcccacgcctgatccgccttcacaattcagaatccttccacttctcacagctgtactggatccctccaggtgggggcgactctcacctgactattactatagcctcctaagtggtttccctacttgcaaccttgcctgtataatatctatcctccacacagcaggcagggcgatcctttaagaatagaagttagatcatgaaaatgctctgctctgatccctgcaaaagctcgccacctccttacagtcaccgctgaactcgtagcagaggttcaggaggccttgctatggttccctgcggctgctctcatctcacttcccctgctcattaggccccagccacactggcctgcctgctcttcagagtttccaggtgtatgctgttgccttgctcttccctcttcttctgctcttcctccaggggtccctgggcctagctccatgtctccttccagtctctgctgacctgtcaccttttcaatgaggcccaccctcatgtgcagatgactccactgcccccgtgctccaattcccttcaccctgcccccagactttctctttccatccttcttctgtgttttggctgttgtttattatccatctctccttcctagaatattggttccctgaggtcagagatctgtgagtaaacattggcatgtcccacgtgcctggcctgcacatggcaggtgctcaataaacatttgttgactgactaagtcctagaatcagtaaaaatcagagctgaaagaaaccttaaagagatctgatccatcagcccagtggtagctacagctgctcatctcaaatgttaaaaaaaaatgatctatagttatatttactatgtatttattttaaaagttcctgcagtattaggaacagtttgtcttctgtgtcaattgtgtagctttatgaatgtaaatgctgcctatctgagaaatgtatctagttattaggaaaatcagatttctatataagcttatatttaatcagagtgaaataattacctatgagatattggcatttcatcctaattttaaaaacacagacccggaaaaaaaaaaaactgtatgattcaaatgatgccctctgccgtttctaaagcaacagaacatttgaaaagatttcgaagttatttgttaatataactttataatatatgctttcaaaacactaaatttgaatgaaactgctttgtcaccatgaaagagaaataatttcaagcagctgttttttaaaattggaaactatattgttcttactttttaaataattactaaagtgataataaaaacataatttgagtatagaaaaattatttgtcatggtaattttaaagtgctaataaaatttactttgaaaaaaatgcctggaacaagccatgctgattccctggatggaatcatggcagtaagaaaactgtcacacataccccgatactttgataagcccatattttgaaatactagactcatttgcgagtactttgcaacagacaaaatagcaggtgatgaaactgaaggctttcacttccatatacaaacccagttgtctttccttcccactaagaaacttccttggttctccagccttcatagcaaccttaacaaaactcatccggatagtacacatcttggtcagttcatacacgacttcaaagccgtggtgaactgactgggccaggagctgagcgaagagctggttgttgaagaccttgaggctgcagccgctggggatcttgcagacggtagctgggtggaagccgtgttgatagttgcagttccggctctgcacaaagatgctgctgtcactcacgcactcggcatacacctctcccccgacgtagtacaagtgcacaccctttcctatatgtctcctggtattttctatcgttgagtttctgtttacattagaaagaagtccaagacagaatctgttcctgttatttgaagggtcggtgaacccatctatgagcacacttcgggaggaagcctggaatgtctccccaactcggttgttcagttcatagtaggcgaccgagcaccagtgctggggctcctcgtaacaaactggtcgaaagtctccatttggtatcgatagcactacatgtctatcagctgtggcatctacaggttggccactctgggtctcagaggcttctgtggcatgataaggcaggggtggtgtgtcaactggagtctccacccggcggtagtggtaagggttaatgcacacttctttctgcttggagccaaatgggaactcacagcactccagcggcttcagctcgtggtgggactgcagatccggccagcgccacacgcgacagtaaatcacatggggcaggcccttgcggtgggacacctgcagccgcccgtccagggagcggggaatcgtgacgcatttgctgggctgccccgggcagctgagagccctctccagctcgtccatggctcccttcttcttctttaacttcttcactagagagtccactgccttctctgcccacttttcctcttcatctccttgcttccagcctagcagtctcttcactgcggggctggtgaaggagaagagggagctgatgggggtggtggagtgcataagaggccacagcaggctccggcgcgcacgggaaccgcacagcccttcacggcaaagtgggcggcgagtagctctccaggggtggcatagggaccaacccgcccgttcttctgggagcagctgggaccaattcaagttgcgaagtgtgttgactttctcctaagcccttgaacagggtggccaacttgcctggctgcgcgcgcccagcgcctgcagggcccggcggcggcggcggggaccgagacagcggctgcagcagcggcggcggcggcggcggcggcggcggccccagccggcgtcagtc

SEQ ID NO: 13466 - RNA, 3075 nt, Homo sapiens
  source 1..3075: mol_type = other RNA
gctgggattacaggcatgagccaccacgcccggctcttctcagtttaaactcaaacctttggtgttctcatccacacttagggagttaaatacggtccctttgcagacaattcccaaatttgtatttcaagcccaaacctctctccccgaatccagactcttatatcgaactggctactcagcaactccacttgaatgcaacggacatctcaattacacctgcgtcttctccatcttgattgaaggcaactaacttcatcttcctctttttctcccacgcctgatccgccttcacaattcagaatccttccacttctcacagctgtactggatccctccaggtgggggcgactctcacctgactattactatagcctcctaagtggtttccctacttgcaaccttgcctgtataatatctatcctccacacagcaggcagggcgatcctttaagaatagaagttagatcatgaaaatgctctgctctgatccctgcaaaagctcgccacctccttacagtcaccgctgaactcgtagcagaggttcaggaggccttgctatggttccctgcggctgctctcatctcacttcccctgctcattaggccccagccacactggcctgcctgctcttcagagtttccaggtgtatgctgttgccttgctcttccctcttcttctgctcttcctccaggggtccctgggcctagctccatgtctccttccagtctctgctgacctgtcaccttttcaatgaggcccaccctcatgtgcagatgactccactgcccccgtgctccaattcccttcaccctgcccccagactttctctttccatccttcttctgtgttttggctgttgtttattatccatctctccttcctagaatattggttccctgaggtcagagatctgtgagtaaacattggcatgtcccacgtgcctggcctgcacatggcaggtgctcaataaacatttgttgactgactaagtcctagaatcagtaaaaatcagagctgaaagaaaccttaaagagatctgatccatcagcccagtggtagctacagctgctcatctcaaatgttaaaaaaaaatgatctatagttatatttactatgtatttattttaaaagttcctgcagtattaggaacagtttgtcttctgtgtcaattgtgtagctttatgaatgtaaatgctgcctatctgagaaatgtatctagttattaggaaaatcagatttctatataagcttatatttaatcagagtgaaataattacctatgagatattggcatttcatcctaattttaaaaacacagacccggaaaaaaaaaaaactgtatgattcaaatgatgccctctgccgtttctaaagcaacagaacatttgaaaagatttcgaagttatttgttaatataactttataatatatgctttcaaaacactaaatttgaatgaaactgctttgtcaccatgaaagagaaataatttcaagcagctgttttttaaaattggaaactatattgttcttactttttaaataattactaaagtgataataaaaacataatttgagtatagaaaaattatttgtcatggtaattttaaagtgctaataaaatttactttgaaaaaaatgcctggaacaagccatgctgattccctggatggaatcatggcagtaagaaaactgtcacacataccccgatactttgataagcccatattttgaaatactagactcatttgcgagtactttgcaacagacaaaatagcaggtgatgaaactgaaggctttcacttccatatacaaacccagttgtctttccttcccactaagaaacttccttggttctccagccttcatagcaaccttaacaaaactcatccggatagtacacatcttggtcagttcatacacgacttcaaagccgtggtgaactgactgggccaggagctgagcgaagagctggttgttgaagaccttgaggctgcagccgctggggatcttgcagacggtagctgggtggaagccgtgttgatagttgcagttccggctctgcacaaagatgctgctgtcactcacgcactcggcatacacctctcccccgacgtagtacaagtgcacaccctttcctatatgtctcctggtattttctatcgttgagtttctgtttacattagaaagaagtccaagacagaatctgttcctgttatttgaagggtcggtgaacccatctatgagcacacttcgggaggaagcctggaatgtctccccaactcggttgttcagttcatagtaggcgaccgagcaccagtgctggggctcctcgtaacaaactggtcgaaagtctgagtgttgatagggactctctggctcagaaggacttcctggggagtgagggtagctggccgtgcacggggactgggagaacgcgtggctgggtgagggagggagtgcagagcacggaggctgctggaaagagtcaggataggtggcgttgtgtggcatgagtggctcactgtgcagggaggcgctgcggaacttggccaggaggctgagctgggggttatattcactgtgtcttggcacgagcacaggaggcagtactggagtctccacccggcggtagtggtaagggttaatgcacacttctttctgcttggagccaaatgggaactcacagcactccagcggcttcagctcgtggtgggactgcagatccggccagcgccacacgcgacagtaaatcacatggggcaggcccttgcggtgggacacctgcagccgcccgtccagggagcggggaatcgtgacgcatttgctgggctgccccgggcagctgagagccctctccagctcgtccatggctcccttcttcttctttaacttcttcactagagagtccactgccttctctgcccacttttcctcttcatctccttgcttccagcctagcagtctcttcactgcggggctggtgaaggagaagagggagctgatgggggtggtggagtgcataagaggccacagcaggctccggcgcgcacgggaaccgcacagcccttcacgg

SEQ ID NO: 13467 - RNA, 3069 nt, Homo sapiens
  source 1..3069: mol_type = other RNA
gctgggattacaggcatgagccaccacgcccggctcttctcagtttaaactcaaacctttggtgttctcatccacacttagggagttaaatacggtccctttgcagacaattcccaaatttgtatttcaagcccaaacctctctccccgaatccagactcttatatcgaactggctactcagcaactccacttgaatgcaacggacatctcaattacacctgcgtcttctccatcttgattgaaggcaactaacttcatcttcctctttttctcccacgcctgatccgccttcacaattcagaatccttccacttctcacagctgtactggatccctccaggtgggggcgactctcacctgactattactatagcctcctaagtggtttccctacttgcaaccttgcctgtataatatctatcctccacacagcaggcagggcgatcctttaagaatagaagttagatcatgaaaatgctctgctctgatccctgcaaaagctcgccacctccttacagtcaccgctgaactcgtagcagaggttcaggaggccttgctatggttccctgcggctgctctcatctcacttcccctgctcattaggccccagccacactggcctgcctgctcttcagagtttccaggtgtatgctgttgccttgctcttccctcttcttctgctcttcctccaggggtccctgggcctagctccatgtctccttccagtctctgctgacctgtcaccttttcaatgaggcccaccctcatgtgcagatgactccactgcccccgtgctccaattcccttcaccctgcccccagactttctctttccatccttcttctgtgttttggctgttgtttattatccatctctccttcctagaatattggttccctgaggtcagagatctgtgagtaaacattggcatgtcccacgtgcctggcctgcacatggcaggtgctcaataaacatttgttgactgactaagtcctagaatcagtaaaaatcagagctgaaagaaaccttaaagagatctgatccatcagcccagtggtagctacagctgctcatctcaaatgttaaaaaaaaatgatctatagttatatttactatgtatttattttaaaagttcctgcagtattaggaacagtttgtcttctgtgtcaattgtgtagctttatgaatgtaaatgctgcctatctgagaaatgtatctagttattaggaaaatcagatttctatataagcttatatttaatcagagtgaaataattacctatgagatattggcatttcatcctaattttaaaaacacagacccggaaaaaaaaaaaactgtatgattcaaatgatgccctctgccgtttctaaagcaacagaacatttgaaaagatttcgaagttatttgttaatataactttataatatatgctttcaaaacactaaatttgaatgaaactgctttgtcaccatgaaagagaaataatttcaagcagctgttttttaaaattggaaactatattgttcttactttttaaataattactaaagtgataataaaaacataatttgagtatagaaaaattatttgtcatggtaattttaaagtgctaataaaatttactttgaaaaaaatgcctggaacaagccatgctgattccctggatggaatcatggcagtaagaaaactgtcacacataccccgatactttgataagcccatattttgaaatactagactcatttgcgagtactttgcaacagacaaaatagcaggtgatgaaactgaaggctttcacttccatatacaaacccagttgtctttccttcccactaagaaacttccttggttctccagccttcatagcaaccttaacaaaactcatccggatagtacacatcttggtcagttcatacacgacttcaaagccgtggtgaactgactgggccaggagctgagcgaagagctggttgttgaagaccttgaggctgcagccgctggggatcttgcagacggtagctgggtggaagccgtgttgatagttgcagttccggctctgcacaaagatgctgctgtcactcacgcactcggcatacacctctcccccgacgtagtacaagtgcacaccctttcctatatgtctcctggtattttctatcgttgagtttctgtttacattagaaagaagtccaagacagaatctgttcctgttatttgaagggtcggtgaacccatctatgagcacacttcgggaggaagcctggaatgtctccccaactcggttgttcagttcatagtaggcgaccgagcaccagtgctggggctcctcgtaacaaactggtcgaaagtctggagtctccacccggcggtagtggtaagggttaatgcacacttctttctgcttggagccaaatgggaactcacagcactccagcggcttcagctcgtggtgggactgcagatccggccagcgccacacgcgacagtaaatcacatggggcaggcccttgcggtgggacacctgcagccgcccgtccagggagcggggaatcgtgacgcatttgctgggctgccccgggcagctgagagccctctccagctcgtccatggctcccttcttcttctttaacttcttcactagagagtccactgccttctctgcccacttttcctcttcatctccttgcttccagcctagcagtctcttcactgcggggctggtgaaggagaagagggagctgatgggggtggtggagtgcataagaggccacagcaggctccggcgcgcacgggaaccgcacagcccttcacggcaaagtgggcggcgagtagctctccaggggtggcatagggaccaacccgcccgttcttctgggagcagctgggaccaattcaagttgcgaagtgtgttgactttctcctaagcccttgaacagggtggccaacttgcctggctgcgcgcgcccagcgcctgcagggcccggcggcggcggcggggaccgagacagcggctgcagcagcggcggcggcggcggcggcggcggcggccccagccggcgtcagtc

SEQ ID NO: 13468 - RNA, 4302 nt, Homo sapiens
  source 1..4302: mol_type = other RNA
gctgggattacaggcatgagccaccacgcctagctaattttgcactttttgcgtgtttttagtagagacagggtttcactatgttggtcaggctggtctcaaactcctgacctcaggtgattcacccaccttggcctcccaaagtgctgggattataggtgtgagccaccatacccggccataccaaataccttcatttttttaaaaaaggctgagcacagtcactcatgtctggttggctgaggtgggaggatcgcttgaggccatgagtttgagaccagcctgggcaacatagcaatacctatctctaaaagacagaacatctaaattctaccctggaggattgagaaagggaacatgacactggaattggacttgtaggatgggtagaagttagaatgtagagcaggataagatggaagaacattctaagaggacacactagcacaggcagagaaagaggcaataatgagcaaagcatgttcaagaaacaaatggtatgtcataaagacaatataatacacattagcagtagggtgggtaaggagagggaagataggattagaaggtaagctggaatcagatatgaagggccttgtatatcagactaaggagttttgattctgcaggcaatgatgagccactaaagatttcagaaagacagctattcattatagttgtcaagacaactatatcataatagacaaatgggttagaagaatagggtagtagatactgtatgttagctttaattcagcacctgttcccaaccccttaccccttgccttcctcaccacaggggaaaagaaacatgatttccctattccctatcttccttgagctaagtgtgtggctatatgacaagtactggttgagatatacacagaggtcttctgaggagattctaagaaagcatttacttttctggtaaaagggagtcagacgcatcttgtgtacatttttatctgctatttcctactttgaatgtgtatctgctccctggaggtacagcagacatcttgtgaccatgaggtgacaaaccagcatgctgtagaggacagagtggaaagagaaaaagtctacgtccttgatagcaccaatgagccactgtcccaaccctatactgcctaattctaggctataaataggataggcctttttttttttttttgcttaagctaatattaaatatttgtttaactagtttactgtcacctgcaagcagaacatattctgaaatgagagacagcaagattgacagtgagcaaattagcctgaaggctattacagtaacccagaaaagtgatgatgatgacttgagggagagtaattataggattagagaagacagaatagatttgaaggagcgggaggtagagacaattttgttttaggcacattgacattggcatatctatgggatgttaggtgaatataactagtaagtagaaataaaggtctacagcactagagagatatgggggttgaaaatatgaataataaaacaaatggtgcctgaagccagtgaagtctgttaaatgaaaaatgagtgtgcatatagaatgagaaaataggactagggatgaaacttgagcagcctcagcatttaagggattcagagcaagagaagaaaaatgaagaataacaaaagcaggaaaaatagagagcaaagggataagtgagtctcaaggagagagtggtgaagagtcaataatgacataaaaattcaagtaggggctgggtgcggtggctcacgcctgtaatcccaacactgtggtaggctgagtcggacagatgcttgagctcaggagttcgagaccagcctggacaacatggtgaaaccctgtcactaccaaaaatacaaaaaattaggcatggtggcgggtgcctatagtcccagctacttgggagggtgagatgggaggattgcttgatcctgggaggtggaggttgcagtgagctgtgtttgtgccactgcactccagcctgggcaacagagcaagaccccatctcaaaaaaaattaagcaggtatggaggccagaatgtcacaagacagagaggacttgaaagtagggaaaaaagggacaatatttacttttgtcaaaaagtaacaattactttttaaagaagtataacaattataggaaggagagagaaaaaatagttcaagggaagaggccaagttaaggaaaggtttttgtcttgttttgttattgttgatttaagacagagaagacctgcagctatgtagaggtggaggaaagaaactacagtatctactaccctattcttctaacctattcttctaatttgctcactgtaaaaagagaaaccgaagactagaaattaaacagggtggaatatggtcttagatgggaaggaatgaggtcaagaacacaaagagaagcatgtcttagaaaagggggatgcatggctgaaaagaggtaagtcttgaaggtagatgggaagaagttttgggaatggtcatatctaataatttagttttttctctatgaaataggaggcacagtcaactttgacagttctaagaggcttgagaagaataaaacgtttgtaatacctcttccagggaacacaatagtaaaccacttaggaaccagtagaaggattgctaagcagtattaggaagcctgtgtagcatatggccctctcaaataggtagagatgtttttagatatttaagaggaattaacattaacaaaaccaagggacaaagccaagctcaagtcccataaaacatggatattttattccagctctaggaaatgggaaaaaaaaaaaaaaaaaaaaaaaaaaaaacagagggaaacacacctttccatacaccattctaatttaactagcattaatctgggaaagctagagcagaaatatatgtttatatgtataaatatgtatgtatttatacatatatatgtataaatatgtatgtatttatacatatatgtataaatatgtatgtatttatacatatatgtataaatatgtatgtatttatacatatatgtataaatatgtatatgtatttatacatatatgtatatgtatttatacatatatgtataaatacgtatttatacatgtataaatatgtatgtatttatacatacatatatatatatgtatttttagattttaatctcactagaattcatgtcttcatttttttttaagtgcccttaaaggtcatcaaatgcaagctaatacttctacctaagtctcctcatcaatcatttaatattgtttacactgcattcacagtttgtgtgttaaccacttatgtaatttatcaaatggcatatttggaaatgtaagggagaaacttggtttaggtaatactctatgtatcagttacccattacatgatttattttcatcattatttgcaacgccacacatcttgtagttttctgtgtagtctctgcatgcagtctacttcagcttctagtgctgtacatatctatatcttctgggtgggactgcccgtgatccatgagcttggggtcaggcataaactgggttgcacctgaagtggattctgatttggtctttgcttcagagctgagttctgttggcaagggcactgagtgtttcaagacgtgagttgtttttgcaggtacttctatttcggaagaggatcctagcttagttttttctttaggtttagggagtgactcttctttgctgctttttgtccacaatgatttaactgctccaaaaatttgctggcttgtagcatataccttttttgctgttaccttagcaattattacggactgaactgggtagcaaacagttgctcctaaagtggccagtcccagaggataagtaattttcttaaacttggaaccttttctcgctgaaaccaagcccgccaatcctgaaactgtaataactcccattttcggaagaaaatctcgaggaggattcttcagatagacataagcatcttttccaaattgtactgtatccattatcccatttttcacaaagacataaacacccttgcaccagccaatgtaacaaccagttgcagtgcggatggaagcaaagcccatttgtaaatgaccaggctgctcttcaacatatttagactggagcggtggtgcagtatatatggggagctgctctggtttcactagctgctttttggattcctcttgtttggctgcatgtacacttacagatgcatatatcagacctgcaggcatggttgtcagttttcccatcctgatggccgccatgtctacaaccctttcggccaaggttttcagacggag

SEQ ID NO: 13469 - RNA, 2786 nt, Homo sapiens
  source 1..2786: mol_type = other RNA
gctgggattacaggcatgagccaccacgcctgacctactgtacgctttttacaagcagcgtgcttttctttttcttttttttaaagacagggtctcactctgtcacccaggctggagtgcagtggcatgatcacggctcattgcagcctcaacttcctggtctcaagtgattctcctgcctcagcctcctgaatagctgagaccacaggcatgcccctccacacctggctaattttttaattttttgtagagatggagtctcacttagttgtccaggctagtctaaaactcctgggctcaagtgatcctcccaccttggcctcctgagtagctggacccaagggcgcttgccaccactcccagctaagtacttttcatattaaaaaaaaagaagaagaaaaaagaaaaaaaccaactccacttctaatttcacaacagaaaaattcttctagtgctattactctacttaattcaatcctgtgttgttgtttttttaaatcagaaacatgaatctgtaccaacactttttcttaattggctccttcccctacagaaacacttaggtagcgagctgcaggaaacctgcctttgtccctgtgttgtgcactatgtcttgccacactttagacaaaacaaagctcctttagagaaaccctggctggagggaagaaaagtgtcccggctgtcattgccatgggagtctggagtttctgagagggcagcccaggtcaccagagtttccagatttagtaccaaccgtggaaacatgaaggtggctgtaatccaaggtgaactggactgccagaggaatgtcagcttcggacagaaaatggaggattcctcatctggagcctgtctctattgcctgattttcaaagaaaccaagttttcatttaactttagctaaccttctttcagaaaagtttagttattaaaatacatttaatgcttggtattgtgaacatgcagacgaaagaaaataagattacaaaatgaaataagagctagaattaaaagccgatgtataggaaatgttctcaactgtgcaagtgattaacagccagatgttcccctacgattccaaacatgagtccccagtgccaagttccagccccaactctgctggagtctcagagaaaatgtatagtaacaaaagcagccaagacttgtgtggcgtcagctcttatttcttcttgagtttttgtcccgtggatgtgaatcactaagaacacatgcattcctcaagttttagaagataaataaggtggaaaaaaataaatcttagggatttgcttcaattcttatttaagcttcatggaatgcaaacataggaggctaaagcagaaataagtattgcttcagtgatcatgagtccagccagcttagtaaacaaaacaggggttaccttcctaaccttctaagttcccatttacctacaagtctgagggttttaatctgccagggtcccttggcaaaagggtcagaagtcattgtcactctcatccaggggttcagatttccggacccttcgattgggcttggttggtgagagagaaatgctctcgtcttccaaatcgtcatcctcgtcatcatcatcttccatgtcaatttcactctcctccgagtcctcattgtcatcggagtctccaccttgcatcgtgcccacaatgcgtttgccaggtcttccttgcatgagcatctccatggctgtctgtggcttgggcagccgcctttcttccaactcactgtcggattcatcgtcctcctggatgtctatgtccgagtcatcgttacttccactcttgagcaggcgcttctcttcctccttgagcttgttctgtatcaggcagagagtgtttttagcttcctcaaacctttcttgctccatcctatgatggtcttcaagctgttgttccagataagtcagattttgaaatttctccagataagtgtcatactgcttttgtaattcttcctcagtcttctcatactcatccataaaacatggcctgacactctgcagagtctctagtcgcttccgatttctttccagttctaattttctcttttcgattttggcttctaaattagcttcatcagaggccacattattgagcaggtctttagtcttctgaacctgtgtcaaaatctcttttattgcaattctcatcactttttcagtctcgtttatttccagaggtctggcaatggcttctgttctcatttccctcaactctacttccatgccgagcaagtcatacagagatgctcctttggaggtgatttcagacgcaagctgcctggctgccttcaaatctgcaatctttgagccaagatcaaacttgaacttgttgacatcttcctctactatttcagagccctccatccccttggtcttcatagcattataaaggacagatgtgatcttcagcagctcttttaccgcatacccatctgcttgataaagcttcttagtgttgagttttatatgtgccttggtggccatgaactgggcaattgccttaatgaagaaaactcggtcctgttcagtatccacgtcaggcgggatgtcagtctggggctcatatcttttcacaagccagagaagcacttcagatacaagtccaaaattgggtgtacggaaattttccatagaaatatgtcgagggtatcccagggctctcatcatctctgtgaaattgcggaggtcgcggaaagacataacgctcaggtccccaggagcccagggtcgcaactgctcgcccctcagcgatcacaggcccagc

SEQ ID NO: 13470 - RNA, 2303 nt, Homo sapiens
  source 1..2303: mol_type = other RNA
gctgggattacaggcatgagccaccacgcctgacctactgtacgctttttacaagcagcgtgcttttctttttcttttttttaaagacagggtctcactctgtcacccaggctggagtgcagtggcatgatcacggctcattgcagcctcaacttcctggtctcaagtgattctcctgcctcagcctcctgaatagctgagaccacaggcatgcccctccacacctggctaattttttaattttttgtagagatggagtctcacttagttgtccaggctagtctaaaactcctgggctcaagtgatcctcccaccttggcctcctgagtagctggacccaagggcgcttgccaccactcccagctaagtacttttcatattaaaaaaaaagaagaagaaaaaagaaaaaaaccaactccacttctaatttcacaacagaaaaattcttctagtgctattactctacttaattcaatcctgtgttgttgtttttttaaatcagaaacatgaatctgtaccaacactttttcttaattggctccttcccctacagaaacacttaggtagcgagctgcaggaaacctgcctttgtccctgtgttgtgcactatgtcttgccacactttagacaaaacaaagctcctttagagaaaccctggctggagggaagaaaagtgtcccggctgtcattgccatgggagtctggagtttctgagagggcagcccaggtcaccagagtttccagatttagtaccaaccgtggaaacatgaaggtggctgtaatccaaggtgaactggactgccagaggaatgtcagcttcggacagaaaatggaggattcctcatctggagcctgtctctattgcctgattttcaaagaaaccaagttttcatttaactttagctaaccttctttcagaaaagtttagttattaaaatacatttaatgcttggtattgtgaacatgcagacgaaagaaaataagattacaaaatgaaataagagctagaattaaaagccgatgtataggaaatgttctcaactgtgcaagtgattaacagccagatgttcccctacgattccaaacatgagtccccagtgccaagttccagccccaactctgctggagtctcagagaaaatgtatagtaacaaaagcagccaagacttgtgtggcgtcagctcttatttcttcttgagtttttgtcccgtggatgtgaatcactaagaacacatgcattcctcaagttttagaagataaataaggtggaaaaaaataaatcttagggatttgcttcaattcttatttaagcttcatggaatgcaaacataggaggctaaagcagaaataagtattgcttcagtgatcatgagtccagccagcttagtaaacaaaacaggggttaccttcctaaccttctaagttcccatttacctacaagtctgagggttttaatctgccagggtcccttggcaaaagggtcagaagtcattgtcactctcatccaggggttcagatttccggacccttcgattgggcttggttggtgagagagaaatgctctcgtcttccaaatcgtcatcctcgtcatcatcatcttccatgtcaatttcactctcctccgagtcctcattgtcatcggagtctccaccttgcatcgtgcccacaatgcgtttgccaggtcttccttgcatgagcatctccatggctgtctgtggcttgggcagccgcctttcttccaactcactgtcggattcatcgtcctcctggatgtctatgtccgagtcatcgttacttccactcttgagcaggcgcttctcttcctccttgagcttgttctgtatcaggcagagagtgtttttagcttcctcaaacctttcttgctccatcctatgatggtcttcaagctgttgttccagataagtcagattttgaaatttctccagataagtgtcatactgcttttgtaattcttcctcagtcttctcatactcatccataaaacatggcctgacactctgcagagtctctagtcgcttccgatttctttccagttctaattttctcttttcgattttggcttctaaattagcttcatcagaggccacattattgagcaggtctttagtcttctgaacctgtgtcaaaatctcttttattgcaattctcatcactttttcagtctcgtttatttccagaggtctggcaatggcttctgttctcatttcctgtaatcccagctacttaggaggctgaggcagaagaatctcttgaacctgggaggcagaggcgcagcgagccaag

SEQ ID NO: 13471 - RNA, 2843 nt, Homo sapiens
  source 1..2843: mol_type = other RNA
gctgggattacaggcatgagccaccacgcctgacctactgtacgctttttacaagcagcgtgcttttctttttcttttttttaaagacagggtctcactctgtcacccaggctggagtgcagtggcatgatcacggctcattgcagcctcaacttcctggtctcaagtgattctcctgcctcagcctcctgaatagctgagaccacaggcatgcccctccacacctggctaattttttaattttttgtagagatggagtctcacttagttgtccaggctagtctaaaactcctgggctcaagtgatcctcccaccttggcctcctgagtagctggacccaagggcgcttgccaccactcccagctaagtacttttcatattaaaaaaaaagaagaagaaaaaagaaaaaaaccaactccacttctaatttcacaacagaaaaattcttctagtgctattactctacttaattcaatcctgtgttgttgtttttttaaatcagaaacatgaatctgtaccaacactttttcttaattggctccttcccctacagaaacacttaggtagcgagctgcaggaaacctgcctttgtccctgtgttgtgcactatgtcttgccacactttagacaaaacaaagctcctttagagaaaccctggctggagggaagaaaagtgtcccggctgtcattgccatgggagtctggagtttctgagagggcagcccaggtcaccagagtttccagatttagtaccaaccgtggaaacatgaaggtggctgtaatccaaggtgaactggactgccagaggaatgtcagcttcggacagaaaatggaggattcctcatctggagcctgtctctattgcctgattttcaaagaaaccaagttttcatttaactttagctaaccttctttcagaaaagtttagttattaaaatacatttaatgcttggtattgtgaacatgcagacgaaagaaaataagattacaaaatgaaataagagctagaattaaaagccgatgtataggaaatgttctcaactgtgcaagtgattaacagccagatgttcccctacgattccaaacatgagtccccagtgccaagttccagccccaactctgctggagtctcagagaaaatgtatagtaacaaaagcagccaagacttgtgtggcgtcagctcttatttcttcttgagtttttgtcccgtggatgtgaatcactaagaacacatgcattcctcaagttttagaagataaataaggtggaaaaaaataaatcttagggatttgcttcaattcttatttaagcttcatggaatgcaaacataggaggctaaagcagaaataagtattgcttcagtgatcatgagtccagccagcttagtaaacaaaacaggggttaccttcctaaccttctaagttcccatttacctacaagtctgagggttttaatctgccagggtcccttggcaaaagggtcagaagtcattgtcactctcatccaggggttcagatttccggacccttcgattgggcttggttggtgagagagaaatgctctcgtcttccaaatcgtcatcctcgtcatcatcatcttccatgtcaatttcactctcctccgagtcctcctgcttcttggagctggaagtcttgcatttacctaagagagctggtgctgcttccatattgtcatcggagtctccaccttgcatcgtgcccacaatgcgtttgccaggtcttccttgcatgagcatctccatggctgtctgtggcttgggcagccgcctttcttccaactcactgtcggattcatcgtcctcctggatgtctatgtccgagtcatcgttacttccactcttgagcaggcgcttctcttcctccttgagcttgttctgtatcaggcagagagtgtttttagcttcctcaaacctttcttgctccatcctatgatggtcttcaagctgttgttccagataagtcagattttgaaatttctccagataagtgtcatactgcttttgtaattcttcctcagtcttctcatactcatccataaaacatggcctgacactctgcagagtctctagtcgcttccgatttctttccagttctaattttctcttttcgattttggcttctaaattagcttcatcagaggccacattattgagcaggtctttagtcttctgaacctgtgtcaaaatctcttttattgcaattctcatcactttttcagtctcgtttatttccagaggtctggcaatggcttctgttctcatttccctcaactctacttccatgccgagcaagtcatacagagatgctcctttggaggtgatttcagacgcaagctgcctggctgccttcaaatctgcaatctttgagccaagatcaaacttgaacttgttgacatcttcctctactatttcagagccctccatccccttggtcttcatagcattataaaggacagatgtgatcttcagcagctcttttaccgcatacccatctgcttgataaagcttcttagtgttgagttttatatgtgccttggtggccatgaactgggcaattgccttaatgaagaaaactcggtcctgttcagtatccacgtcaggcgggatgtcagtctggggctcatatcttttcacaagccagagaagcacttcagatacaagtccaaaattgggtgtacggaaattttccatagaaatatgtcgagggtatcccagggctctcatcatctctgtgaaattgcggaggtcgcggaaagacataacgctcaggtccccaggagcccagggtcgcaactgctcgcccctcagcgatcacaggcccagc

SEQ ID NO: 13472 - RNA, 1387 nt, Homo sapiens
  source 1..1387: mol_type = other RNA
gctgggattacaggcatgagccaccacgcctgccctgccgtgtcttctttctcctcctaagcaactgtcttagtctcctgaattttgatattctacttaacactctcatgttcttacgcatgttgccatgctggaggcgtccttctctttgggaagcctgacccaccaacagtgcctcaggagatagacatggaagctttgccggtgggggccgctcgtctctatcacacctcagttgcaggggaggggtcggttgcagctgcagcggtggccccgacagttttcttttgtgggacctgtggccggcagctctgggtggagaagacctacttgatccaagagctgcaggatccttgggctgcatgtcctcccccaccatcagcaagcctggagagctgggcaggtggtcttcacccagcaccttcaaggccgccttctctggccacagggagcagcccggaactggggcagggagcactgttggaagtgggtcaggcttcccaaagggaaggatgcctccagcagggctgtgtgaactggcgactccatggcccttggagtagaaactcactgcatgcacctgggccttgtcagtctgattcttttctgtcaagctcttgaggtggacatttccctccaagggcctgggattgtaccaggaagaagtgaggtttccctgagtctccaggggcctagaggtggaggctgcttccccattgctacaggggccccttttattgtcctcctgcccctgggtctctacctggtctttcacctctgttgcttctttgggctcttctgcgctcacctccgtcttcgggagcctggctgggatcacctgatcatctaatgaaggaagttgaaggttaaacttgcctctgagacaagggatccttacggggctgaggtgtccaaacattatggagttgtgaggagacagcacgggtttcttccttgagggggggctccagaccacaggacgcaggaccctctgtggggtgcccgtgttccgagggataagacacagcctcataggggcgccgtcccacctgactggaaaagaaggcccaagatgtcgctgacggttgaagaggagtgggaaacggcccacaattccccgggcaggcacaggtgcaggagctgcagggtgagcccggccagctgggaaggcctcacggacaagacgagcaggttgccgatggcatggccaggacctgtattgatgcaaaaagcctcctgtaattggtcttcctgttttttcctgttgacttaacttcagtccattcttaatatagcaggtaaagtagttatatttaaatataagccatattatgtcactcttttgatgaaaatcctccattgacttttcatctcaaccagaataaaa

SEQ ID NO: 13473 - RNA, 34 nt, Homo sapiens
  source 1..34: mol_type = other RNA
gctgggattacaggcatgagccaccacgcctggc

SEQ ID NO: 13474 - RNA, 847 nt, Homo sapiens
  source 1..847: mol_type = other RNA
gctgggattacaggcatgagccaccacgcctggccaaaatgttttgtccattgttgtagtcagggtccctgtcacatagcttgtgagatggagatttgagtgccgggggtggattggtgagcaccctgggatccgaccaaggaacttcccagaggatcatcagctgccaacgttcccagtcctgaagagaagatgtggatggcaccagtgagggtcctcgccaatcatatattctagaacattcctgggcttttcgacagttctgaagactgggaaatccaatatcaaggggctcacatctggcaagggcctttgtgctgtgtcatccccacacaaacgtagcttgcatctgcctttataggagagagggcggctgtcaaggagcggtccatactgggaggggctgagactgatttctgggccaccaatgtgaagctgaccaggatccccagagaggagagaaaagctcgttgttgttttcctctgaagcactaacatcctacaacctccctttctccacactgacctggtcttcaccctttgtcctccccctccttaaagttagttgcatcgtcagccttttctacctgaccctcattccacctgccaaactgtaattctcctttggagaaatctggaaacacaaaagtcctcaggatacagcctcttgccactaagcatgggcaactgttctgtgactgcgattagatcctttagtttgtagcacctcaacttttgttttcaaggcttttgagtatattcacagaggcgcgcaaccatcaccgtaatctaactttgagcattttcatcaccccaaaaagaaattctgagccgggcacagtggctc

SEQ ID NO: 13475 - RNA, 5109 nt, Homo sapiens
  source 1..5109: mol_type = other RNA
gctgggattacaggcatgagccaccacgcctggccaaggcggcactcttgtaaataaaaatagacagggtacccagtgttgcctggctatctacatgcccaggttctataaaagttttagctctgagtgcattttggcttggtaataggagtttgtttccaggtcattatttatgactccagttttaatatgcatatcaaataaaaacttgggcaattgtcatgaaaggaacatgcaggatattttaatgaacacttctgcatttaaggaggtctgggagaagggtggtgagaatggtaatgagtcatacatctatgttgcgccactacccttagccattgcttttcggagaccctaggcctaattaaataatagctagactccatcatatgacaaatgattgactagctatgagcatggggcatcctcatttctcagcccagtctcatgttcatcatgtgctattagtcataagtctctagcatttatagaaaataaacacagttgctcagttcccacccccaaatgaggaaattagtatggaatggagccctggaatctgcattttgtaaggcttctttggtgatcctgatgcacatccatggtggagagctctgaaggggttgtgagaagagagacgggaaagcgaaggaagctacagaaacccagagaggcccgcagaggtctgaggaggggctgggggcacggaggcagcagtgcctggaaaaccagtcccgccccaagttcacatgcaggaacagagtgggcggcacagcgggctgcacacagggcacgtcttcgattcagagctggagtggaagaagcagccgccgcagccccggtggaaactccgtgactcttttctagcagccatcatggctgcaagggccgggctgtgaccaaaggaggggtctgaggcagggagggtggcatgtgcccttacagagaaggtcccacagagcagagccacccagaggcacagcctcaaaggactgacctgttacaagatcccagagccctaggctccccaggaacactgtcactggagagatcctctctgggcccagacccaaccatcacccaactccaatcctctcccttgagcccaagaccctggaccttccctgggcgggaccacagcagagccagcactgaccctcaggttttggcaaaatgtctagtgagggaacatcttcatttatggtccaaccaattcagtacaaagcctctgccttctcgctctgtgaggtaaggggaaggggtcatgttttagagacagtaatctcccccttctctggacagccagacatgtggtgcccgttgccacagggaaggtgacatagcagaagcgagccttggctttggaattttaaaagcttgattctgaaggtgggtggcaagaactcaggacacttacagtgcatttggaagaatatatgatgggttaaagaataaaagcctcctctctcccccactggtcaagattccataggttggcagggcttggggagcaaggcgaatgttgacatttctggaattcttgagaaaaggaccctgagaaggaggttgcggctaaagagggggaaagtatgacaaatactccatataggtttggaggtgataagtgtaggcaagcactgggtagaagaacccacacgcttcctgggtagagcctgggaaaacagcaagccacagagcggaacaagggactgggctgtctatcttagcagttggcctggaacagaattactgagcttcctgaagccagagggtgtgcagggccaggagctagaatcttccacatgctccaagccacaggtccccaaataggctttgtggaagtgaaggagcccctggcagaccttgcatgaccaactgatgaccagatggggaggggatgtccaggcaggtgcgagcatggacggatgatgatagccgaggaacagagtcttacatgacttaaagccacacccccacccgaccgagcttaaccccaggaaaaggtcagggggagactttgaattgactgagattaatttctaccacctgctgaaacggggttcctaatagaaattacattctgtgttagaaaaataaagttatgcttcttgcagattagagtttgtaggctgagttgtacctactatataagtaatgaattaattttttctttatgattttgtaaagaaaagagaagaaagaaatttcagtagaatagcgctacattgcaagagaaacggcacttgtgatttttatccattttccttctagtctttgaatttagaaagcacaagtctcttgccacaagttcaggtcaaatgactgcagcattttgagtgaaaccaataaaatctaagttcatggattgttccttttgttttgttttctcaattgctcattctcaggggtccatatacaaggccatccatccctggagactaagaacatggctcactgcgagagctaaggagttttctggacaagaatggagggaggactccccacctccaacaggcagttctataaataacggctgctccatggtggcccctgaaatgcagcatttcagcagccttgaaatgacaaagcctggagagtaggagggcagtggcgacgttgctgggaacaacagctgggactcccaggagctgaaggctgaagccataggtagcccagaaaccgaggaatccagaagccctgactaaacccactggggccatccgacccagtcaggcggcaaggggatgggcgggcatggagcacagatggccctggggtaatcctagtgcctctggttcagggacctccaagcttgactcagctgttctccttaatttcatcatcccatggtgcactgggcatgcccgagggcttctgggagcacaggtagggcaagggcaatttgggagggctgaagaagcctgtggggaaaagaaaagggaagatggtgaccacataggagggacagcggcctttccaacaggggacccttgccagccatggtgagtagatggaatctgtgcccatcctctgcaagcccctagcaaacgtgtgaccaggaaagagtctgagatcatgtcacatttcctgagatgagcacgtaggtagaagctccttcctttaagctttagttcttactggggatggaaattccatccaacaaatgttgatatagcttgcttccttctaaggggatttccagcaggtggaaattgaattgtgagggaacaagtaaatcttcccagagtgtctgaagtcacatcgcagccttagcttttagccggggctttgtccctcccttctaggacagtctccatgacctcagctgaaaatgggacaaagtggggacctgtgagtccttacacttgcagttttcacagggctgctcagctttgagcttggccactcccatcctcagggtgtcccaatctgagatccaggaaatcaggaagactaagaggctggtgtcatggcccagggcagagcctacctgaatcatagctgaaccagcaaatgggggtgggggaagatgaaggctgagttctccagttcccttcattggcttccaggtgtgcaggtggcttgggattgaggactcagatcttctcaggccccgagggcatcgatgccagcagggctgagcaccagtgcctgaaggatgtcggagagggagaccacgcccaagagatgctgggtctcgtccactagcaccagcctgtgtacctgctcccgagcaatcctgtcgatcacttcccccaagctctcgtggggctggcaggaaaggactccctccagacatagtgtcctctgcctcagggcttctcccacactcatgtccaggtggttgtaggtttgctgggcagccaggtgaatcacatcaaagcgggaatagaggcccacgacctgaccacattcgttgaccacaggcagtgcagacacacgccggtccacaaagatgtccagtgcagtcaggatgggtgctgtctccagcaccacagccaagtctcggaatgtgccgatgcccaaatcttggatagtgcggtagaggaaggagggccggggcagcagggaaccaaagatgtgcaggaacttgagcaggcgtttgtgtgtgaggatgtggagtacgttgcctgacaccgggtcaagaacaggcaggcgatggatccggttcttgatgagggtgtagacagcttcaaacaggctatcattaggagagatggagaccagaggcttgaagcagccttgcaggtagatctccctccaggtctcaatcttatgttgttcaatctcatagatctggaccaggggggacctgtagtagcgatgcagcaccaggatgaagtcagtgatggtcagcatccccacaaagctctgcttcttgctgtcccatagaggggctgcccgcacaccgttggccaccagagcaaagaaggccttcttgatctccagcatggtgtcgaagatgactagcttggagctagttgccatggcatcgtagcaggtgtgctcctgcatgaagcgcatgtagatctgggcgccgggtttccgcagttcgtcatcccagcccagcttgggaaatggggcctgcggggacaggcacagggcaggcctctcttccagcaggccttctagctcacactcccaggcctctgtggctgggaactccgtggccagctccacatcatctgtgctggagcctgcagctgaggctgtacagtcagaggggaggcagtcccaccctgttggtggagtgcccaccccggcaggatcagcttgagccaagggtgtggtcttggggaatgtggcctccagcccggtggactcagcagctggcctggaccggggaccttccccctgacctggtggctccccttcctccaccgacttctgccttgtccatctcaaggctttggccctccgtttcccacggattctttctgagctgctggtcacagctggtgatggccatgagctgctgttttcttgctctaggaagctcatctcttgatgctcagaacccccaaggctgctccaggaaggggtcctgcgcagtgcgtgctccagcccgggctccatgtggccagccccagaccaactgagagcaagtgt

SEQ ID NO: 13476 - RNA, 854 nt, Homo sapiens
  source 1..854: mol_type = other RNA
gctgggattacaggcatgagccaccacgcctggccaatacatttgtctggtttttaatgccacaaaatttttccaagtacctgagctccaattgcactcgttaacttaaagatatacaaaactatgtctaaaaatggcttactaagatttgaatacagatcgactacactgttacaaaatttttctacatcttgtgtaagcagctggtctggattagctattctgttgtccagattccccattttataatatgtgaaagcttgaagatactcctcatagaggtatttagtgagccttactcggaagcacagtttaagctcatttaacccatacttcaagaagttattaaccagagagataagaggcatggcagcgatgaagttgagtaagtatctcttgaaatctttcctgctacgaccaatgataccactttcaattagtgtcccattttgaatcatccaaacatcacaatatgttcgagacaccagcataacagcaataagtaccaagtaacctgtctctttacaaaatgttctagggaccatgattttcagaatctgtatgagccttgagaaaaacaccttgtccaccacagctcgctcctttttcccctctttctcattgttctgtaatggtggttttccacttttcttaccgtgcaggccgagggcgcggcgccgcttgtggagcaggcagagcagcaggaacgcggcaccagccagcgaggagtttcgcgccgtcaagtacttgctgaaggccgccatggcactgccggtaccagcgagccggcgaggggacgcggcggcggcggcggcggcggctaccttactgcacgcagcgcgggggagactggg

SEQ ID NO: 13477 - RNA, 1926 nt, Homo sapiens
  source 1..1926: mol_type = other RNA
gctgggattacaggcatgagccaccacgcctggccaatttaatttattgaattgtaaaaaggtatgttttaaccctatataaatgtatgactatatggagataattattattcacctgaataaaaaacagcaatataaagacacaaataggtaacagtacaatattaaatactataacatctaatccaatattaaaattatatatatacacatagatacaggtagggctgccaacaaatggtcttcatgtctaaaattgtggtaattgttgcagagacttctgtgactatattggaaaccttggaactgtacactgtgtgggggtgaaatttacggcattttaattatatctcaaagttctgttaaaaagtgagtggcttaatattctgtgaagtaaggaatggttttatttaaaacataaattaataatttccagtggattcccttaaaaagattacagcagggatttccagatcacacccacccccacctctagagtttttggctgttttctaaagtcttgaattcaatgaggtgaaggaggaagaaagtgtttaggaagtcagtgggttccagaagagctggtgctgggtggggcagagtggggagagatgctcctttcaaatggaaggctctggaacccgccaaaagggagtgcaagctggggcaatcttcctggacagccaccagagaaaggcttcagaccccacgctcccgctgacatccacagacagggacatctcactggcttttaaaatcatcaactctttttatatcgacacaaagaaataatgaaaaggggaattctggtttacagtcatttcattaaattatccaaaacaacttttgaaacaaaagttataaaagtgaaactcaaaattattctctgcttaataaatactctcagtggctcagatatagttcaggcaaactagccatggatgcagccaaagccagggggtggagggggtcccggcgtgctccaggaggcctctccggtgagtccggcagctgttccctcggcgctgcagccctctctttgctcagctgggggcctctattttgtaaacctcagaataagtcataagccccgtgaagacatccaagatattccttagggttatacctgtatcaggaacaggtttggatgcaggggaaattccaaggatgacgggtatggatcggaaaagacagtgatgtccaagtacaggcggtgcactccacaggtcatctcggacagtcactggaagctaggcaaagtctgtggtctcatggccacaagcccaatgatttgacctcagagggtatccttccacctctaaggagttctcttgtgctcttttactccagtgttggctccaggaccttgggtagagggtgctggtgatatgaggtggtccaggagcaggcccgtaatgctccttcccaaaggaacccagaatcaggtttccgtacactagatccagcaagtttgttcctcaggaagtgagccatttcagggtaaatactcccctctgaggttgatggcatattgccagcatcttcttttttgcagatgtctcctacagcaccctcaggaggagctaggagaacacagagtaagggtcagtgccctggtggtggcaactgtgtcacccagagagctttgcttggtgtggtgcatggaggtagctgatcacagcatgcgccaacctgatgctgggccatgctccaggtggaaggaggagggcaacagagagagcaggagggaactgagacaaggaggcctaggccttgtccttgtcctaaggcatcatgaagcagcacaaaggagtaaacccaaaatggacctaaaatgcacaccaaggttcaacagaagggtcccttcatcactcacatgatttgaaactcttctacacaaacaagactttcttaacgtattcaaga

SEQ ID NO: 13478 - RNA, 2111 nt, Homo sapiens
  source 1..2111: mol_type = other RNA
gctgggattacaggcatgagccaccacgcctggccacagaatcttttaatcgggtcatttttgtattaggaattgtcagaaatttaacatattttgaatggcaagaagcagcttttctatattcatttttttttagcatagattatctgatgcttaggaaacagtgagtgaggcaaaaagaattcccacatttatttaattttctttgggtgtgagttttctgatgttctatgatggaagtgacaggtgttttctgacattaattacactacattaaaaattacctagtactgagccagatgtgaactccacataaaggcttatctttatcccttacactcaaggctttctaaccagtatgaattctgtagtgttcaatgagttgtgagccaagaataaatgcctgcccacactctctacattcgtaaggtttgataccaggatgaattctctgatgttcggtaagttgtgaactacgaataaaggccattccacactccctgcattcatagggtttctcacaagtgtgaattcgctgatgatgagtcagttgtgaaacacgaataaaggccttcccacattccttacattcgtagggtttgtcacctgtatgaattctttgatgttgaatgaggtatgagctacgactaaatgccttcccgcagtccttacattcatagggtctgtcgccagtatggactctctgatgtcgtgtgagctgtgcgtgctgtctgaaggccttcccacattccttacactcatagggtttctccccagaatgaattctttgatgtcgagtaacttctgagctgtgaataaagccctttccgcattccttacactcgtagggtttctcaccagtgtggattcgctggtgtacagtcagctgtgagtgctgtctaaaggctttcccgcattctttacactcatagggtctggcccctgtgtggattctccgatgcacagtgagttgggagccacgaatgaaagccttgccacagtctttacatacgtagggtttctcgcctgtgtgagttctttgatgcagaatcagctgtgaatgctgcctaaaggtcttcccacattctttacattcataaggtttgacaccagtatgaagtctctgatgtagaataagttctgatgtacgaccaaaggccttcccacagtccttacagtcataaggtttctcacccgtgtgaattctctgatgctgaacaaggtgtgaggcacggctgaaggccttcccacattccttacatccaaagggtttttcaccagtgtgaattttctgatgttgaataaggtgtgagccacggctaaatgctttcccacattcatgacattccatcagtttctcaccagtctccctgctctgacgtacagtgtgagacgtgtgatgctggaacacgggcatatgtccataggtgacgttcacttgcttaaaatagcactcttcattgacttgtctctcaaactggccttcgcattcccagtcagctctaaaatcggagccctccaggtcactgcatttaaggctttccattatctcccagttgaatgccccgatttcaaaaatgtctttttgtagaaatttctcacacctggactccaagtctgggcaccatggtcctgtcacatcatttgcaatcatccagggctctttcccttgctccaataaggagacgacatcaggcttagaaatggagagtcctagtgaggccaagtgaccaaagttctccagagtcacctccctgtacaagtccctctgagcaggttccaggcacttccattcttccagagagaactctatggccacgtccctgaatgtcaccagtccctgggccatggcttttagaactatttgacctgctctgatttctctggattcttctcttggacaagtgcagagtcctcaagagctccatcgtcacagaaggaggcggccaagttcgcggggggaggggaggagacagagagtcgaccagtaaagcctcaagggaaatgtagtccaaggcctgagaagcgacgttgctggtaatagaaggtaattcagtaccagcctgggcctggccgcggtgaccgaggcgggccgcgtcgcggagacttct

SEQ ID NO: 13479 - RNA, 910 nt, Homo sapiens
  source 1..910: mol_type = other RNA
gctgggattacaggcatgagccaccacgcctggccaccaccgttttctttatctcacattctgtgggtcagaaacttggacagggctcagctgcgcaactcttctgttccatgtggtgttgactgagatgtccaactgacagctgggcaagtcgagggaatccacaacagctccgttcattgtctggcactttggcagagtcgcagagacaactagaaggctggacctgacggggaccacgtcccagagagcctgcatgtaatctctctaacttggccaatttagagtcatcagagttcttccatggtggctcaaagctaccagagtgagggtgttccaagagacccaggtagaagcagcaaggtttcttgtaagttagtctcagaagtcccagaatgttacttctacaaattctgttggctgagcaggtcactgagtccagcccagattcagagggtcatgaataagacagccccctgcagctgggctcatccttggagacctcgactgggcttcgccttcttcattccagtgaggtcacgcacctccaccctgctcctgcctctagagcagaaggctctgggggagattccaccgacaatggaggctccactccccagggcatagggcggaggtagagttggtggctaaccttctgttctgagggcaaagggagttcggatccttggtcctgccatccccatcctcttctaggcagctcctggctctccatgtgtggcagaaaatggctgcagtaactccaggcctcagatctccctataccttctggaggaagagcaagcctctttcctggtagcatctctggaagaggaggaagcttgtctttcccagaggcttcaaatggctcctgtgtcttcatggatctgaatgggttactgatttatctggg

SEQ ID NO: 13480 - RNA, 1034 nt, Homo sapiens
  source 1..1034: mol_type = other RNA
gctgggattacaggcatgagccaccacgcctggccaccaccgttttctttatctcacattctgtgggtcagaaacttggacagggctcagctgcgcaactcttctgttccatgtggtgttgactgagatgtccaactgacagctgggcaagtcgagggaatccacaacagctccgttcattgtctggcactttggcagagtcgcagagacaactagaaggctggacctgacggggaccacgtcccagagagcctgcatgtaatctctctaacttggccaatttagagtcatcagagttcttccatggtggctcaaagctaccagagtgagggtgttccaagagacccaggtagaagcagcaaggtttcttgtaagttagtctcagaagtcccagaatgttacttctacaaattctgttggctgagcaggtcactgagtccagcccagattcagagggtcatgaataagacagccccctgcagctgggctcatccttggagacctcgactgggcttcgccttcttcattccagtgaggtcacgcacctccaccctgctcctgcctctgcagcatggaacacatcaatttccttgtcagtaagttcttctagagaaggaattcttctttcccctacttcggtatcctcatgtctgatgatggatgaatgaattatgtgtggccctaagaactagagcagaaggctctgggggagattccaccgacaatggaggctccactccccagggcatagggcggaggtagagttggtggctaaccttctgttctgagggcaaagggagttcggatccttggtcctgccatccccatcctcttctaggcagctcctggctctccatgtgtggcagaaaatggctgcagtaactccaggcctcagatctccctataccttctggaggaagagcaagcctctttcctggtagcatctctggaagaggaggaagcttgtctttcccagaggcttcaaatggctcctgtgtcttcatggatctgaatgggttactgatttatctggg

SEQ ID NO: 13481 - RNA, 3570 nt, Homo sapiens
  source 1..3570: mol_type = other RNA
gctgggattacaggcatgagccaccacgcctggccacggcctttattttaaaatttggcataggagtcaaaagctgcccaaggagggcagctacctatggggtgtgcatacattcatgaccaatatttaagtccaatatagctttgataattgttctataaaatgtttacacctcactgaagaatctgtcgttttaaaagaaaatctttacatttattgtatccaattaactttgttagtaatctgccaagtaaaacaagtattcatagtaattagtgactctattgcattagaactgtaacttagtgccatttttgaagactgttttcccaacaaggaggcattatcatttatccaattactttattctctttgaatagcaagcatgatgtaggcctcagctcacaatttacttacctgattagcttccatttctctttaaggatattgactatgtgacacttctaagaaggctgactagtacgtaagattatgtaaaaatcctaccagagtatgtactaaaataaagttaacatgtctattttctagttgcttgtgatttatcttaattttcttcctatgtcactaagatatgggtaaagagccctaaactccaaacatttttacatgttaatataaatttaatggtggcatattattccatctactggctgggacatggtatatataattatttgcctattaatcggttctgaatatttgtattctgactcttggctaagctggcttctgtcttttctaactactgactgaactgaaccctttgatgaccagcaaggtctctgacttccaagtgcaatttgagcactatttatttttagaagttttaagtccaaactatttcctttaattgctcttgtccagaatacacaagctttttctatatagggccacataagaaatattttaggctttgcaagccaatctccctcacatattcctttcctttcccccattaacaactctttaaaacaaacaaacaaacaaacaacaaaacctgaaactggaagttttaagtttactgccacatgggtacaatcatatacttaggtcgataactttatagttttaaatgtaacatctcacatttcaagcatctcctaaaacttgccattgtaattctagttgctaacataatggacatcattatttttatgaaaatattcctatagaattaaaaataacacttgaaaaaaattaagattgtttttcaaatagcttacttggttaaagtctacttatggagcaagctacaagtccatataatctttgctgtttgccacctacctaaccaattcctcattttactcatgttttgttagacagaatcaacttaggatattgtcttccgtcctagggacccagaggaaaagagatgaccaaagatgcaataaactgccccaatatactgtgtctatttaaacagaaatcaatcagctgttaggcaagccaatgggtgcataagtagggagaggggtcagccaacactggacaccttagagcagtggttcccaacctttttggcaccagggacccgttttgtggaggacaatttttcaatggacagggcaaggggatggttttggcatgaaactcttccacctcagattatcaggcattagttagattctcataaggagagcacaacctagatccctcacacgtgcacttcacaattgggttctcacacctatgagaatctaatgcggccactgatctgacaggaggctgagctcagctatgatgttcactggcccatcactcacctcctgcaggtgcggccgatcaggggccgggattggggacctctatcttagagggttttaggcgaatcctaaatagtgtgtctccactaatatttgttaagtttatgcttaacatagcaagactgatatttgtgacagcccatagacacatctgctctcttaagatgtacaatgtttcacaggaattttaaggggtgttcttgtttatatatttggcagttgtgtaaactttggtcctaggaatagagagagatatgagtctccagggacagcaaaaacaatcaaatggtaaagaagagaggccatattttctttaacacccttaattccatccttatctctgctcttgggtgcttatacagcacattatttgtaactgtagtcactctaaattatcccttactgcctctttgatgaggaagaatgattaacacaatggaatgttggaaggtttaaagtctacacctcatctttcctggtatccttgaatttactagtcaggaggagttaaaatatagtcatctttaaaaaaatctctccccttttcacttcacagttctttattttatccatatactcttaagtgcaactgcattttcttttgccttaacagttaaagaatcccacagggaatgatcataggctactctggttttcaatttggggaaaccctatactttaacttgaataaaataacaaagtcctccaaactaatatgtgatttctgcccagagctctgaaagtcaaagtaaagaaattcaataaagtgagggtaacagggagtaaagatgactttcaaggtagccaaatgcctcaccatctaaataatgacgcccatcaatgaacaaacaagattcccactgtcccatctcctatccagtgaaacacagccaacttgataatttgtgcagggaaagactctgtttagcttataccttgaacctaagggaaattaaattgcacattttctgttcctggctaatcttctgaataatgtactgaacacagtaggagttaagaattaaaaatacctgtctgcagtttcagaaacaatcacacacaaaatatttgtttatttccagactgatgaaagactgaatttttggtctcatgtatttactgtattgtttcatatatttatctatatgctttggctgtattaacttgttgaaatagtttgtggttctttatatttagcttttataaataattgaaaatctaatgaatgcttacttaataaccaatctaaactggggacttcaaacatagggagtcaagtaatctggttgtgtaataaataagcaagttgttatctttcaggctgagggcatatcaaccaagctaaaagacgtgtgtgtattaaaaaaaaaaaaaagtctaccaaaccaccatatgatatccaaggttaactatataggaggtctaataacattcagaaggtgctagatgaatataccaaaaacatgcggaattaaatgatgaaaattatttactggcattaggacggaatttttaatgtcaaattttaaaaatggcccattaaagtcccagctcatgacatctaagtatctgaagacccactactattcctttttctttttctgagactgttactctgtcacccagggtggagtgcagtggcataatctcggcccactgcaacctctgcccctcgggttaaagcaattttcatgcctcagcctcctgagtagctacgattacaggtgtgtgccaccacacccagctaattcttacatttttagcagagacagggtttcaccat

SEQ ID NO: 13482 - RNA, 3190 nt, Homo sapiens
  source 1..3190: mol_type = other RNA
gctgggattacaggcatgagccaccacgcctggccagatcatgttcttgatttggctctcagctcggacattgtttgtgaatagaaatgctactgatttttgtacattgattttatatcctgaaactttgctgaaattgtgtagcagatctaggaacttttgggcagagactatggattttctaggtacataatcatattttctacaaacagagagagtttgacttactctcttcccgtttgcatgccttttatttctttctcttgcgtgactcctctggctaggacttccagtactatgttgaataggaatagtgaaagtgggtatccttgtcttgttctggttctcaaaggaaatacttcaagcttttgcccagtaagtatgatattggctgtgggtttgtcacagatggctcttattcttttgaggtatgttctttcaatgcctagtttgtagagggtttttaacgtgaagggatgttgaattttatcaaaagccttttctgtttctattgagatgaccaggtggttttgtttttggcttttttaaataaataaaataaaaataaaatcactttattgatttgcatatgttgaaccaaccttacattccagtgagaaaacctacttgattgtgttggattagcttttcaatatactactggatttggtttgataggattttgttgaaaagttctgcatctatgttcatcaatgatattggccagaagttttctttttttgttgtgtctctgccaggtttttatatcaggatgacaccgggcttgtagaatgagtgaaggaggagtccctcctcctcaattttttggaatagttgcagtggaatggtaccagttcttctttatacatctggtagaatttggctgtgcatccatctggtcctgggcttttcctggttggtggcctttttaatattgattcagtaagaactcattattggtctgtttaaggattcagtttcttcctggttcaatcttagaaggttgtatgtttccaggaatgtatacatttcttttagattttctagcttgtgtgcatagaggtgttcattgtagtctctgagggggttttgtatttatgtgagtttagtggcaatgtcccctttgtcatttctcattgtgtttatttggatcttctttatccttttatttattagtctagctagcagtctgttaatcttatttattatttcaaaaaaccagttcatggattcattgatcttttctgtggtttttcgcatcttgatttccttcggttcagctctgattttgcctcttccttgtcttccgctagctttggggttgatttgttcttgtttctttagtttctctaggtgtgatgttaggttgttaatttgagatctttctaatttttcgaggtagatgtctaatgctactgacttcccccttaatgcattagctgtgtcccagatattctggtatgttgtatctttgttctaatcagtttcaaataatttcttgatttctgccttaatttcattgtttacccaaaagtcattcaggagcaggttgtttaatttccatgtaattatatgagtttgagtaatgttcttagaattgatttctatttctatttttattgcactgtggtccaagagtgtgtttgatataatttcagttttttaaaaatttctgaggattgttctgtggccaattgtgtggctgattttagagtatgtgttatgtgcagatgagaagaatgtatattctgctgttttggtgtggagagttcggtagatatctattaggcctatttggtcaaatgtcaagttcaggtcccatatgcctttgtcaattttctccctcagtgatctgtctaataccatcagtggggtgttgaagtctcccactattattgcgtggtcatctaagtctcttcattggtctgtaaaaacttgcttcatcaatctgagtcttcctatgttgggtgcatatatttaggatagtcttcctgttgaattgaatcctttgccattgtctaatgcctctgtttgtctttgttgactgttgttggttgaaagtttgttttgtctgaaattagaattgtaactcctgatttttttctgttttccatttgctcgctagatttttctccatccctttactttgagcctatgggtgtcattgcaagtgagataggtctcttgtagacagcatatagttgggtcttgcttctttattcaacttgccactcagtgccttttaactggggcatttagtccatttactttaaagattaaatattaatatgtgcaggtttgatcctgtcatcatgttgttagctggttattatgcagacttgattgtgtggttgctttatgtcaatggtctatgtacttaagtcagttttcatggtggcaggtaacagtcttccctttccacatttagcattcccttaaggacctcttataaggcaggcctggtggtggcaaattcccctagcatttgcttgtctgaaaaggatgttatttgtcctttacttatgaagcttagtttggctggatatgaaattctcagctggaatttacgttttttaagaatgctgaatataggctcctaatctcttctggcttataaggtttctactgaaaggtttgctgttagcctgatgtggttccctttgtaggtgacctgacccttctctctagctgcctttaatattttttctttcattttgaccctggggaatctgatgactatgtgtcttggggatggtcattgatatcatttagatatttgtccctgctcaaatctcatgttaggatataatccccagtgttggaggtggggtctggtgggaggtatttggatcatgggggtggatcattttactcaccatgagtaaaagcttcctgagacctccctagaagcagatgccaatgttatgcttcctgtactacctaagagaggcttgcaagtgctgtcctcagtgcccttgcctgggtgtaaaatagcagagaccgaatccaggactgggtgtgaaaactgctgattggtcgcaaagcctgaaacaaatactgccttagaagtgagcggtactgtgattcttctgttaaaatgcccgttcatgctttacctatattctgtgcaaaaatgtgttcatagcagtgtaattacttcatgtaggagcctggaaatattcgtatcact

SEQ ID NO: 13483 - RNA, 22701 nt, Homo sapiens
  source 1..22701: mol_type = other RNA
gctgggattacaggcatgagccaccacgcctggccagtttttaaagtatttcatacagtgtaactaggcagtcagaaatacctgtatctcaaattcatttaacttttcaatgaatcaatcttcttattttctcagacatataaattatcataatactttacattgagtctctatggttgactatatgctgtgaaggaaggacataaatacatgtgaggaaacaattattgatatttttaaactaactagaaagcaccaagttatttgttaaataaacaaagttaattttatctacctgttcagtaagtgttggcaactatgaattaatctttgacaaattcacttacaactagcaattttaaagacttaaagtttaatttttattattaaaagggtatgattatttttactaaaattaataaaaagattaactgttactaaattaaagctccttcaaaaacataaatgtattctttagagagttaaaaaaagtagcaataaaatacatttttaatttagttaagcttacttaactaatgatcaaatagattaagttgtataaaattttacaaactttatatttttgcatacacttatcttcctggcatttttgaaataaaaaaaatacaagtgcatagggcagaggaggcgattcagttacttctgctatgttattaaatctctggtaaccactatacaatacaatacaatacaatacaatacaatacaatacaatacaatacaatacaatacaatacatgtagactcagcatccaaactttattttaccttcaagttctacctgataaagtggtggaataaagatggtattttccataactgtttaataataatcacatgttttatacccattgctttgaagaagaaaccttaagcaactagaaatgtcaatctaaaaggcagaaaagctggaaaaatctcatgaagactagaagatttacactcataagatcatgtaaatttatttggatatgctgaaaaaagagggggtataaaatctaaagtttggtaaatctttgctttacagggcttcaagttatagatttttcttttttccttttctcttcccctttctctctctttctcttttttatttttgccatttcttctcaggagcccctgcaatttcaaaccttggaattgaattggatttgaggaggaaaacccatattcagctttaattcaaatgaattttactactttagacaaaggtacaacactctattcaaaaaagttattgaaatcacatctttaaatctgacccagccacttgaataaataagttgtgttgtagtttctcagagcaaccgccgctcatctttcactcaccttaacaatttctcacttttttctgctttttttttttttttattttctgcttgctgaaatcgagatcaatattcattgttttcttctgggttaactcttttttatgttaactgaatcaattttggctttgtttctttatgaaattacttttagataaagtattgatattgtcatttatcaattttattatatgtcttttgcttattaaaggattaaaatccacctctaaacttatttagatcaaggtcagtttttttactcctctgtagaactgtgaagataatatcctattctccttttcttatggttttattgtgaagatctgtgcaaatagctatataaaatgcaattcggtattaaagaaaattgttgcacggactacattgattagagtctaatttttggaaagtatacttcgccttttcagtaattttatttttcggtctatggtgcccacattgtgtcaccagccagccgtatgcagacttacaaaggactacccactaagaataaaaacatgatacaacttgaagaaattttcatcaaacgtctttgtcttatccccttgttatacagacaaagatgacaagggccgaaaaggaagtgattttctcattgaataagagaatccgaactggcatcgaggatatctaattttgggatgaaaattgagagaagacagaatttcaagtctgaattatgacttcactactgtgtcgtcattggtagaataaggataacaatacttatcacacagatttgtggtctgaatcacatgagagacatagatgaaaaatgtaaaacaacaattagcatgtgacatgctctcagcaaatcaattaatccttcattctttttttctccccttactcctttgattttcagactaatttggatcatgattattggcctgtgtcccacccattattcacatatagaatgggttgcattatcctctccttggaaatatctttcaaagtgggtaatgagaaaactactttgaagactgtgctgaaggaaatgatggcatgaacaactctagataatttttgtttatttggatataacgtgaatgggcccataccataaactcctattaagctgaatcaccaaaaaaaaatttgatatgaaagtcatacattgaaaaaattcactcttaccactgatttgattgatactgagcctgtaaatatttatttatatgatgtttggcactttattttataaaactaccctttacttaaaataaatcattgtattcacataactttccagggcactatgcatttttaaacaagacagtcaacttactatttaaaaaacaaagtcagtcacctaaatgactttctgactataaatttgaaaacaatattctccttgtaatatatgtgccaccagggcaagaattacaaattgggagcaggtaagaaaattgttgttgactctcattagtattctaattctccttcagtcagatttataaagtatgacctatagcatccaactccatcattttccagtcattcttgagactgtcaactctatgggcattgtttagcagcctcgaaacactgaactttttacagtcttattggagagaaaaacacattaaatgatcaaataatcttttatgagctcagaaaaaaatgcctaacatgaacatttaagcatcttctgtttctgtgattcccatttttggagagtaaaaatttaagaaacaaagggaatgtgtctggggatggtactaataatattgagattttacaatttaggttataatcaagataattatgtatatatataaaattatatatggtatagtttcaacttctaatcttttatcatcctctaccacataattcctcctatattctctttttctgactgtggcctaatacctcaagaatattgtatatgcttgtcactatataaacttcaccctaaggaaatttccatgtcagatacaataagagcaacggaagaaaatgtatcaaaacacatctccaatttatttgaatttttctggcctaaccttgttggcatgagagttcccactttgtattataataggcaaattgatacacacttttcatttattctaaataatagattagcatagtcaggaggcttggattggcagctattaaatacaatttgaagccgtgggattttattaggattctaaggttattctgtgacgatggaacttaatgatgtaagagttaattacccattgtcaaaaatcattgcccatcaaagcagtgagactgtgtgctatgtccagttttattcatttcttttgtgtatctgaatggaacatgtggtaaacacaacagtagaatatacctacagtccccttagaaactcttaaatcttcaatttataaaagtcatcctaagacgttaaaaataacttacgaaaggatagattccaatgtcagtgggtgagatgtgctctagctagtgtgcacgaaagagaacatggagttagaataattattgtaggactgtagattgtcatctcaagatcagtgtcaaatacattcattcatgtagtattttcacatgcattctggtctaaatatcccaacatatctttcgttttgagatctgcagaacaaagtcaatgtctgaatttagagactaatttgaccattttgattcaaatgtctaaaggctaaaccagagcaatttacaacatccaatgaagtaaaattatataattaattatataattatataattatataaaattttataattaattataaaataaaatattaacaataattgaacattgtttacttttttatcctcacaacaattcaacatgatatgtatggttattactaaatgtataatacatttagtaatgtgatttgacaaatcacatttgtcaaataaggaatggctgaattaaatgattgaatgaaggagtgaaggatgtagattgtttaagtacattcaacttgtaatgaactgtaaacttcacccataacattattaatatatcagtgctatcaactacattttacataggatgaaaaaaatcattatttttattaatcccaagatattttatttcattatataaatgaaatattttatctgttataaagacctttatttttgttccactcattaaataacatggtaagactgttgtgtaattgactgaatagttaagtctaaatgggtaaatagctgtttatgttagtattgcagggtagctatttgataatgaaatatacttttcttacctacttgcaaaaaaaattacataaacaagtatttcctagagttcaaacactgatctttttaagtggcaaattgtccaaaagaatttaattaatataaacaataaattcacttaaacaactatttacatgcaaaagtaatatttttattgcccatttggaaaatagttttgctttctggtttataaggaacttttactagtttaattacttgggtgctttaaatgttttttggaggctattacaaaatcacatcctaaaattttaaaatggaaaaattataataattgaatttttaattcctcataaatattttaaaagtacacattgttccatggcttttgcctttagaataaatacaacatttttatgtagaaatatattcttgaaatgtaactagcacatagtcagtgtttcttaaccattttggggtcctgaaactttttgataatgatgaaagcacagagatgctatcaagaaaaatttacccacataggaacacacacacatacacacagacacacacagagtttgcttataagctcaggaagcttaaagatctgctaaagattatgcttgggtttgccatgaatcataaataccaagtcaaatacctttgaatttgattcttaacaaatctttgtggctgagaaaccatgagatttcattctggcatgtccccagaatgtaattatcaatgaacaatagccattgaaaaaatctgaacagatattattgaggctcaaggttgtttaatggcacagataatataattcaaatcatgaccccagggctgatgaagtcttgttgtaacgtgtaaatggggtgggtgatgggagagagaaaacaaaataattatttatgttaaatcatacataaacagtaaagccaacacaataagtaaaataagagaaagtagaatgcttgggaggtcatatgtttcaaatgtatgcatacacaaaagagtaagcaacaggatacttcaagagtaaaatgggaaaaaatcatattgggtaaatagtatcaccccaaagtgatagtcaaaagtacctatgtttgcctagttctcagattacaactatgatgataatttagataaacaagcagaaaacaaaactatagaaaaaagtcaaagtgacataaaacaattactggtgtttcaacagaaataaacccaacatcaggatttatcaaatatatgaaaaattatgaaagattataaaacaccaatgattagattatgttataaagacactatgaagagatactaaatgatattcttttcatctgtggttactgctaaaaaattctttcatagaaattcttggattttgaaattagtttaattccaaaatattttctttattttgcaaaaatgtaagacaaatgtataggatatttttctctgttgttatgcaaggatttattatcacattggccacagaacacatagaatgttagttttgtagaaaattttagagattttaataccaggatgaaataatagtatcattctatttcaggttcttaagcaacattcctaagactagaaccttatcttgaaaaattatgattttaaacttaagggaattcaggtaaaggaaattgactaggttaaggcaaatacatcatgtttactggtaaagataacattatttaaggaaggtaagatactcttatcctacatatacgccagaaaaattgcttctcctctgaaaactaccattatttttgccaaatattgtagcttagttttaagtttttctcggctgtttcctctgacagttctgtggtaaagaagaaacattataggaagcatttttttttcctacagagtctgccatatggagaagtagaatgagaggccacctaggtaatgtgatttattaaaagttctccatcccaaaatatatgtcccatctgtgggctaatgtctgaaagtcctatgattaaactcacttttatgtaagatagtgaggccccagagagccctcgagaaatgcaaataaactattactgacctcccttggattatgatgaaaaccgtggagtctttctattctctgtcaaatgtggaggtcatggatccttcttggcacctaagattaaaactcatagaatgtgctttaacttctgtaggcacatttcctttccaattagagtgaggtgttgaatatttatttatttgtttatttttattatactttaagttttagggtacatgtgcataacgtgcaggtttgttacatatgtatacatgtgccatgttggtgttctgcatcttaagagaagactatttataaaatttattgcttgtaagatttgttttttgttctcttactattatgaaaatcacgaacttgggaataaggacactctgggcccggcgcggtggctcacgcatgtaatcccagcactttgtgaggccgaggcgggaggatcacgaggtcaggagatcgagagcatcctggctaacaaggtgaaaccccgtctctactaaaaatacaaaaaattagccgggcgtggtggcgggcgcctgtactcccagctactcgggaggctgaggcaggagaatggcgtgaccccaggaggtggaacttgcagtgagcggagatagtgccactgcagtccggcctgggcaaaagagtgagactctgtctcaaaaaaaaaaaaaaaaaaaaaaaaggacactctgaacaattgaacaagactacgctgaaaggcagagaagaagtaattatgaacaaactgttcatgaagtgatcaattgaatttgaaacagaacttttcctagcttctaaatgattagaaatttcagctttggtttaacttaaaaacttagaattgtcaattctgtccaagtctctgagtcatgtacagaactcaaattattacatcatttttttacttatctgtattatttctccatttaaaagtggacaaatttttatactatatcctaataatgatacaaggtgacttgtaggactctggatagaaagagatggcccaggatacagagggcactccttaaatagctgccaaataaatgacattaaaaaatgtataaaaaggtatgttaagtaattaaaagtgtcaggcattattttcctattatgagacattttatattatggttatttactgtaattgcatccaaaataattcataaaacatttatttttgtactattaaaaatctaaacaataataaccagatggaggaaaatgataccatctgatttaattattaacttgaaggtcagtttctacaacttattctcatttatgtttatctgatttggccacagtttcttactttctcatattttgctaagcttgtggatgaagccgcatgtctcttttttttttaacctggcatataacactgtcactctatttaattattacccatcatctacctactttgaaactttggaggttttataaaaattatgagtatttaatcaaagttgtctctttatcatttgccagtgaaaatataaaacctggctgttttattctattgtgcactctaattacataaccaaaatctttttaaaaattcttagttcttttagaaataccatttgacccagccatcccattactgggtatatacccaaaggattataaatcatgcttctataaagacacatgcacacgtatgtttattgcggcactattcacaatagcaaagacttggaaccaatccaaatgtccaacaatgatagactggattaagaaaatgtggcacatatacaccatggaatactatgcagccataaaaaatgatgagttcatgtcctttgtagggacatggatgaagctggaaaccatcattctcagcaaactattgcaacgacaaaaaaaccaaacactgcatgttctcataggtgggaactgaacattgagaacacatagacacaggaaggggaacatcacacactgggcctgttgtggggtcaggggaggggggagggatagcattaggagatatacctaatgttaaatgacgagttaatgggtgcagcacaccaacatggcacaggtatacatatgtaacaaacctgcaagttgtgcacatgtaccctaaaacttaaagtataataataaaaaaattcttagttatttgaaaatagtttttttgaattcacaaacttgcaggatgaaaaaagttattagttcctgaagatataacattgatttgtctttttcttatttgatatcagctagcagtaaaattgtgaacaaatctggtaaatcttttggtgttgcaggttcataatcagttaattgagtgtattcactataaattgctttaattaagtgatgtttgcctaagaacaagtttcatttcatctcatgaaaaaaatgttactttttgtattaatcagtggaatgtttaaagaaaaaactggttatcttgaagctgtcaaataattataagaaatctctatacattacgttttaaaatacataaaacccataaattcaagcttattagttttcattttcagcaaggtttatacagagaaaataagtaatacaaattagttttccagaaaatctaattttatgcagataaaatctgaaaatcatataagtccaagatgaaactgatctcaaattattattttgaggtgtatccatttatttaaaaaagcctcattttagctagcaacactatgtagaaaaatattttaaataagacagagcattaaaataatgtattcattgatctcataaagaatagatgatcagattttttaaaagtgattttaattaaatggacatgtttctctttagccagaaatgactgagaaattttgagttggaattgatataggggaatccttggaactatgtgtgaatatgtgtgtgtgaattatctgtgtatatttacataatttacactattcacagtccttgtttttcttgactcaaatagctatctcaagtttcgtacactttttagatctctatgtaaatacattatttcatttgtggaaatatattgaggcctatatcaataacctcaaaccttttaaacacttagagcaagtcaatatgacttgttctgtttcagctatctgaaatttaaaaatttgacaaatttttaaagtacccagttcttggaaaaagaaaaacaaataaattggagatttggatcatatgggctatgactaaatgagacaaggcatacatgctgacatttgaaggatttatgaaaaaaagtccactgtggaaaactgatagtttttctccttctttcttgaatatgtttagttaattttgtggaaagaggaaggcagctcagtttacaaacagcagtgggttgaaggcaatgctgtttatattcttgaatttcaatatctacaaagatgtcatcattagattttatgtgttaaaaagtggatttatagtctctaattaataaggtgcatatgtcaagactcaggaaaacagatcacttacgtagttctccaaaaacgagagtcccagattcaataggaaggcatgcagagtgttctctataaacccagcaaaaccataaaaattgactggaacttttatttttcagtacaacaataatagtattgaaatacctaaaaagggcaggaaacaacacagaataatctacgcttgtcatcatgttttctaatctataatctttcaaactggataaatgggaagttttggaattttactgtggtacagtcttagttgctccgtggttgtcaaatctgtctgcacattaggatcacttaggaagaattttaaaagtatgctgatgcctggaaactccagaacaattatgataactctgagcatggagctcaggaatgggtgaaattcttccccagagatgttaatgaacagccagacttaaaaactagtaatttagacaagtgtgagcagaggttaataatgttgagatgaactgggcttaatatttcactaacaaggtcagagttttgatacatcacttaactcaaactttgagattcttcatcactgaagtagcaataataatagtcatttctgttttaatacttcatagacttgtaaggatgtaatgtagtgtttctaaaaggagtgaatggacaatctgcatcagtgttaactaaaatacattgaaagtgccaattcctagatctatcctagatttacagggaagaattcagtagtctgaaacacacattttcaatatattgaaaagatgattcttttgcatgatgacttgttataatcattactttcataggtaatggaagtaccgattaggagagtaccaaatacatattaaacactcagttcatgtaagctataggccaataaacacaactttggggtttactgatgttttccaacatccgaaataatagctgaaatttagaaacatagttaatcacacaaaaaatgttgcatacatactgtctaactaccagtttggtatgtttggggctggtgttatgaaagactattatatgattaatacaaagttataatttttggagtcttttagtgtacccagagcccatgagtttttattttctttttggaataacagaaattaggttgtggttcagtggaattacagaagcaagtgttttagatgttcaagtttaaaaaatgagaaaaaaatgttttacatgaagaaactaattatttaaattcatttttcaactatttaatgttattttaatatagtcatatcatccagaaaatcccatcttagacaaatgggttttcaataaattattattatagttaggaggcaatgtataatagtgataaggggcatagattttgaattacacaaacctgaaatccaatgctctctctttcatttattagttatgtgaccttggacaagttagtaaaaccctatttttcatatgctctttagcttttttaatacctcttaccttatatggttgtttaatctattaaatagacagtgaaatgcacatgaaatcttcacacagtgtctcatagttgcttggaacatatttatgtagtaagcattgttcttggctgagcttacattaagtgatctgtaaattagaagttatttgttatatttgtttcgtttccttattgccctagatgccttttctctggacctagataatttagtctcactctgtggcctttacccttcaataaatatggattattaatataatttagctacataattcctaaggaaatattaattcataaagattgttaaattgaactgaatatctttgctaagtcacaggcattgattaaattagataaaattgtcattttccattgattttgtttatataaataatattgaattatttatattcttatttagtctagtagattgacaggcagttttattaagaaatgaatcaaatggtaaattttgaatcatctggtaaaaatggacaaaatttagttttatcttgtggtctggaaatacaccctaaattattgggtcaagttagtgaaaactgttaaattgattatgaacgtaggcacattacttataaatccccttatgctaacttaaaacttgtgaatgtttagtgttatccagctataattcttctaaacatgtcttgtaatttttaagtttgcatgaaaataactccatcctgagtatactcatttcaataaattatttgtcctgagcatactgtaagaaatttagtaaagtactaattgaatttagtgattagactgtgattagactattacaaattcacagtgcttgtacaattcagatattattttgctttgaagtcaaatagaggaaccttaaataatttaaataaaaataattgtttttattaaagtttatacagcaagataataaattcactaatgtgaaatgttgatatagtatgtacaacttgtttcttaagttactaaaaatgtattttcctacctacataatgtcaatctctattgctcctaacacatgagtggctaaaattgcaaacttaatcacataaataatgagattaaagttaaaatgaaaaagtggtatgaggactattgtttgtgttaagtgaaattataccttgtaaaatttcatattatgagagcaatatgtaaatttcattgcaacaatggttattcaatttactgatgaaaatcagaagaatgttgaaaaattagtgcatttataataaatttaattattcataaaaaattaacattgatatatatattcataaggataaaagatatcaaaataattaaacaaatttcactttcttcttataaaagaaaataatttttatggtaactaattttagtagtgcatcagatcaacactattgggcacccagttatttggtggtacgctgagtgaaaatatgtagctttatctacattaccttggtttggacaactgaaaaatttgctaggaaacaaatattacaaaatatgttgttaacttttcaaagatgatcggtttagattgctttaacttgaaggacacttatattttgtatcacttttgtagcaaacacatgactcatcattgcccaaatcaattgcccaaatcaattcaaacatctcattgtagttcatcccatggcagaaaagtgtttatccacttagtaaaatggaaaacactagagcttcaggtttaatttgaaattttaacttcattaagaataaacttgacctgtttgttctagtaagtaaaaacactagatacgtaccaaaattgtcttttgaccctctcagggagtcaagttttgatttgcttgaatacaagcaagtcgagctatggtaatttgcaatgctgacaggaaagaagaacttgcttgaggcaaaatcatgaagtacaacttttcctctgcatccttttacctcatgtttgtaacatttcccctgttgttatttttacacatctggatgctcagaaaggcctccttaccacaataattgaaaggagtactttgtcaatagtcagaattgaatgagagataggttgttgggaatattcagggtgaatgtgtcttttctactttgactatatttaccattgactacagtaactcagcagaaagttagagggcagcatacatacattggtttatggatttaatgaaaatatccccaaccattacattacagacaattcatatatatgtcttgaaaatcttcttgacaatttgtgacaaattttctaaatgtttttccaaaaatagttggttcttgtaagtgattttgatatgactgattaccaaattatggtgggtaaagatgccacatgcaacagaaaatgtgtctaattatgtttgttttagagcttaagaaatgttaagaagagaagttacaactgcattaataggattttaatttttattcaaaatggacaacttatttattatgtacttctacacacagctaagcttatagatattttcatttaaagaaaaactatttgttcattttattagcagatatcaaatgcccttttgaaaattgagactgatttctaaaacaaaaaaaaagactttaggagttttaattatttttaatatattgcttctttattaaaaaaagatacaatccttcaatgtcattcaacagtattaattgttaaagtgtgggatatagtttacattaccgagtttattttctaagggtagtgaataactcctgacaactactgatatcgtcacatggtcctttagtgaccaaaaatgcacagttgtaagaatgcaagtgttacttgtattgaaaaccggattacattaaaggatggacaattatgataaaggatctgagataattggacaattatgataaaggatctgagataattattctaactttttggaactatactttcactcattgatgaagtaagttacaacgtggaataacaaagtttaagtgtggcagaaaatacatacatatgtttaaaagtagggaaaattttatcaattattaaagatggaaaaaataggactatgtcaaatagttaaacaaatgtggggtattttatggagaaaagaggcatgtactaccttaaacattttccaattggaacatactatagacaaaactgacagattattattcaatgagaaacctgactcagatgaagttacaaaaaaagtactttttaaatgtctagtttctaatagagttagagctttgttgattgagatatgtggaactgccacatatctctgtgccatacttttggtaccttcataataaacggtaaagtgagggaaagggtggaagagacaaatcctacgtctcttccagaacttcgagtgcactataaattaaatatttaaaatatttttgcaatagttagctttcaattatgaacactctcagcctctattgctttatatatgcatttattttggtaatttttatacatcaaaactataattacctgtatttgggcagaatgatttaggttatgccagctattgtggttaaagctgtagtaacttacagtacattgaaattatagactaaggttctgaatattggtaactcactgttgttgtgcacctttaaacaactcttaaataaagtaatgattctctttatattaaatttaatgtatgtgtgcctcatggaaatttgtattttatagaaaaatattgaatattttattattatgtctttggctcacctactttaaggagatggctacttagggtactttttaatccaatataatgtgaaaatttgatcatgctatattcttaatttaattgtacttctatggtcatatacaatttacctatcactttctcacataatcaatttaactttttggtaaatcttctaagagaccgtctagacagagtgaaatgaaagctgaaacaacagtcaaatcaaaaactgctttggtctcaaatccatgtttttcagaaaagatattcagatccagttatctggcaaatggtctcaaacatacatttcaatttcaatgttaaaaataggatattaaacatctcagaaaatattgggattattgaagcaaattctaccctggacttggagtaaatgtgatgaacagattaatgaggtggaagggactagaactttgggaaagtgcaaccttgttatcttaatatttttatagcttagaaagagaatgctatgcaactcatattttgatcttttaatgttaaagaattcaaataaaaaccataaacctgaaactctaaaagaaaaattctgttttgagagagatggcctcctctagtacacttttaataaatttaaagtatctaaaaggatgcacaaagatctctaatgtgctgtgattttcaaaggatgtcatgtataaaagatttgagtgagaacatgaaagcaaaagcaagttcagaagaggaacacaaccaggaggacagtgtgtcaggaaaatccaagaataagtggaggtgtaaaggctaaaaaataatgcaaatggtgcatatccttctgtctttctctcatacacacagacacacttacacaacacatatacaaatacatacatgtatatatgtatatatatacacaaatatacacacatattcacataatattcaagtatgtatacatatatacacatatgtacatacacatatgtatatatacatacacacagattgagagattaaccatatgtagatacacacatgcacatatgcaataatgaaatcatttcaaagcatgccaaaaagtaataaaagatatatcctctgtttgggataaataaaaaaaaagtttaaaagcaaacaaaaaataaatggcaataactaatcacattgaattttgttatggcctttttcttcctaaaaagaataaccccaatctgaacaaagaaattcaaagtaatggaaaactcaacaatgaaactcaaagtagactagcagataagatacctatttcaaacatcagtgccaaggtaatttataggtcagtgcattgataacttttgccaatgatagaaaagatgccagagaaccggatcctgacattaaaaaaaaaaagtaaaaagattctgaagactgcatttctgagcttaaggtagattctaaacaacatcttagaaactaggaaatgactttatgtttctttgtttttcaatgtaaatggatcaagatttcttaaaacagaaatgaatattattatttgtgatgagagcactaggggcaattttgatatttttgataaggtttctagagtaataaattagaatgacaggaatatatattgattttaggaaagtgtctgtataattccacatgatattctctggacaaaatatgaaaaggtaggctgaataacatttttaaagggcagtaaattttataattgttattgattacaatgaaggcctctggtaatgttttccagggtcatatcctgttacatatacgtgacatggataaaaaggaaacaaatatttattgtgtgcctagtttatgttatctcaattccagctctacaaggagctacaaggtaaaattgctacctttaaaaacatatgaggtaaaattattcctattcacagatgtagaaactgagtttcaagaaggttaagtaaatttcctcatattgggaggctggtaatgcagaactgggtgtcaaaatcaagtctgtatgaaccttctgttttgtctcccatgaagacaaaaggcatgcatataaaatttgttgaaacacaaagctgaggaggcataataagacgtggaatgacagaagcaagatctagaaagtttgggatcatgaatcaaaagaaacaggataaaattatcctaaaattaatattaaatcttacaagaaaccccccaaaatcagttgaatttgtacaaaacggtaaatcattttatcagtagatcccataataaatattataaagtttaagtgtgagctctattactcagtaatatgatgccattactgtgttgatggatgtattgtcaaggaaaaagaagagaattacacactgtttccttcaattgttagatggcactggatgtagtgttttcaatgttaatcctggtatcatgttctttgccataaacttgttgacaaattggcaaatactgacatgaaatatgccaatatttgagcatctaaaaatgtaggtactttccataccacatcatatattacaatttgaaaatgtttgtttcattttttatataattattatacagaacagtttttctatgatagcattataaaaattcccagagaatactggcccagtaagaaatggaatgttcacaactcatagtgtagctatatgaaagaaatagatctaaacgacaggttggtttccaaattatattttcatacctggaaaatatctactttataaatagcacaaagttatagttttcaatgaatatgaaaaagttcttgcattaacatattttatgtatcttttatattgacatttgtgattgccactaaaatgtgtattttctaaatttcattgtgcttttacaagatacttttttctttgatgtccataactgctgaaaaggctcccctaaggagaattttaagactaagtaaggtttttagtgagcttaaattatacaattctgaggcattatttaaggtgcatactgtattttttgcttgaaacctgtcagcattttatttgtatggcaattaaatgactcagccattcatgtctcatgccagtctttttcaattgttatttttaacaaagaaaattatatatatatgtatatatatattatatatatgtatatatgtattatatatgtatatatatataaacttacagcaaaaatgtttaaaaatagcaaatagtttgagtatagttaaacctaataactgtacttttgtttctatgcctctgagacaagattactagacccttattcaaagtttctaaatataggaaatagaacattgggccatgctaaaaaaattgttcagattttcttttgaaagagaatagttatttttcctcctgacctctaatgaagatgctttatttgtcaaggtgttttccttagaaaattgacccagtgtcaactgtaaagaaaacatagaggatccttggatgattgaccaacttatccaaacacaggtttagtaaagagaggatataaagataaaatgtgaaatgacctctctgagtcacatttgttttcataatttcctagcaaacatccaacttcactgctaccctcagcaatgtttcttgaaacatttttaagacattgatagacaccaatagctgatctttagaaagccattcccagaagaatatgtaaggggttacaactcatttcagggagtctgcctagctcttgatattacatgtctttggcatacaattgtgtaccttttatcattgacagtgaagaaaataatgccatttgtaacttctgagatatacacacaatactatcaactagccggttaataaaagataagaaaaataaagaaaatagaacatttttaggtgtctggcaagtatcctctaaatcaaggtaaagataataatttagtggcagtgttcatattttcctatgactgtaagatttaggtgcctcacaaaatattaatatttagcctcttatgaaaggttcgtttttcttctaacactttagtagctgaatacaaagaaaatacacaacagctgtttataaatgaaataaaaagtttccattttttatctgagtttctcatttatttgcagagaacgaataaaataaaaatatcctagtgttgtttgcaccacagcataccagtaaatcttaaggattgtgtttcagtatgaaaaggaagagcaggaagatttcctcattctgtcttaccagcaaaagtctagccttcacacacacacacacacacacacacacacacacacacacacacacacacacacagagtcatctatatgaacacgtacttgagtttcttaaacatatatgaagcaccttccatttccctttataataaatcccttagtttttgctgttcattaaaaaacaaaaaggaagagacaagctcaggacattctgaaaaccaatgtctttaggacacactaaggtgtcctgaattactttaacggacacattgtaaagacacactctccaatccctattaggaaaagtttagtcaagtttgcttactatttgggtgcttataccaaaaaagcatcatttaggacattatttaggataatattatttatgcaggaattgtaccacctatttccagatggtataacttattatctgacaggcatgtagcaaatagaacacaaagcataaatctgtcaggagaaatcatacgagaaaaagagcattgtctggttatcagaatatcagatctctcattctggccttgctaggaaatagatctttgattctagaaaagtcaactaatttctatggttcttacttttctcctttataatatacccatttaaattccaaaaaggtatatgataaatcacaataatttcaatcacatggattttaatacaaaatgtataaaatcaatttccaaaaattttctgcatatactgaaaatgtctgtacgaatgagctaactactataggccttccctaatttattctattaaatgtgggtactcaatgtaacctgaaaatattgagcttaactcttctttttttttttcaaaagggaaacttgaaaaagactgcttcccccagaaaatttatcaacaataggtgctcaattaaatgtttttaaacaatgaacaatatcccctttcatataaataatcaggggagagatatttttaagtcttttttttctttttccatagtgtcacctacacaaaaaattatgtaaagacaccacttctatgaggaggtattcattgtagatgtacagaagtcaacggaaacttaagtttacagaaaaaataaaccagattatcattccacccaactgtatattcccacagatgcttaataaaagctatctgatgatataatgaattatcagttcttgaggaagtatatacagttggtgactatttttcaaaaatcatcatccaacaaatttttttcatttaaaatctttcatattaccctttcgacaatcagttgaaattttaaaactaagaacatttaaaaatataaatgaaagtagcattagctatagactgatattcaacttcagacgttaaaataaatacaagtgtgtattaagagtaaaattatgtcaacaatgtataaatgaaaactgccaatgtaattaatgtttcttttaacatatcccatccattgctttccctccaaaagacaaaggtagcaaaagacgaagcaggaagaactgcttcagaaactgaacatactgatttaattggctaagaagtccaaatgctaatactcctaataattagccattccttttgtgttttggtgacatatatcctcatacaatgtatatcaaatggaattttttgatttacacctgacatttcaaagtttccatttttgaattctcctagtcttaagtaagtagaacattgtctcctttgtttgctaggcataacgttttccccaacatctagggctccatgatgcaaaatatcattttgccgatcttctgttccagtatttactttaattttttttattataattggattttcaaatacaatcacaaaaacatctcctgttgaaggtggtttcccccaaaagtactcatcaacactactgtaagccttgcttgcttcataattttcaaacacattcatgttggtgtacagacttgcaggggggttatcaggaatgtcaaatgactcctcttcaaaatcatcatccttcagcttattctccgtccctttgtatgatgaataatagcccatgtgctgaaagagagatggtttaaaacggatcacatttttctgagccaacagaccacggaaatgagtcaatagccaatcacaaggcatttcttgataaaacattaataaaaaatgggccaaacgtgggagatcatgagaatgatagagtttaccaatgtagccaagcttagagaattcaagagttacccagtaagttccttctagggatgcaatgactttcttgatggcagttaagaaattttttgaacatcgaacatcatcttcaagcattacataatagtctgaagtattggcacaaaaattaagcagaaaagcataatctacattttgcttggaacgaaatttgactctatcttctggatcattgtaatttcttttaaggccatctaggattgggtaatactcctctggagcatgtataaccattaatcttcctgcaataatatggtgcgcaaatttctgtgtaatatcctggaccatggcatcacgccaggaagaattaaagtctgctaggtgaaccaccactgaaatttccttcagctcttcatagctggattgctcaaaaattgacttaattgtctcaagtaaatagtttcctttttttcgctttactgaagaaagtccaattgtaagataccgctttctttgtaaaggtgtggcagctaggtagcgataggtgacatttatggctcctgagaaattagataaatccttgaaagtatgaacatagcgttctgaattcagttgatgtgtggatgtttcccttataagttgtttgtctccttccagaacatagctatcttcaatgtacaagttcataaaaaggagaaaaatgacaagaactcccaagaatgacactgtagaacgttttctcaggcatctcattttatcaagtatttcaaaaatatgtttcatttgatgaaatttaaacattctcttcgtctgtaatttcagcgctttgggaggctgaggtgggaggatcgcttgaggcccggagcttgacaccagcctgggcaacgtagtgagaacttgtctcttaagaaagacgctgtcataatctgtgctgtacagaaaccgttgatacccagagacagagaaaacaattcgttcagctagatccaacagtgctctgtgcagcctggaagcatgagtgatccttgggcctcacacaaaagcgagataattggctctcaatgaagagatgtaaacatccatcataatggcactgtgctgaaact

SEQ ID NO: 13484 - RNA, 22605 nt, Homo sapiens
  source 1..22605: mol_type = other RNA
gctgggattacaggcatgagccaccacgcctggccagtttttaaagtatttcatacagtgtaactaggcagtcagaaatacctgtatctcaaattcatttaacttttcaatgaatcaatcttcttattttctcagacatataaattatcataatactttacattgagtctctatggttgactatatgctgtgaaggaaggacataaatacatgtgaggaaacaattattgatatttttaaactaactagaaagcaccaagttatttgttaaataaacaaagttaattttatctacctgttcagtaagtgttggcaactatgaattaatctttgacaaattcacttacaactagcaattttaaagacttaaagtttaatttttattattaaaagggtatgattatttttactaaaattaataaaaagattaactgttactaaattaaagctccttcaaaaacataaatgtattctttagagagttaaaaaaagtagcaataaaatacatttttaatttagttaagcttacttaactaatgatcaaatagattaagttgtataaaattttacaaactttatatttttgcatacacttatcttcctggcatttttgaaataaaaaaaatacaagtgcatagggcagaggaggcgattcagttacttctgctatgttattaaatctctggtaaccactatacaatacaatacaatacaatacaatacaatacaatacaatacaatacaatacaatacaatacatgtagactcagcatccaaactttattttaccttcaagttctacctgataaagtggtggaataaagatggtattttccataactgtttaataataatcacatgttttatacccattgctttgaagaagaaaccttaagcaactagaaatgtcaatctaaaaggcagaaaagctggaaaaatctcatgaagactagaagatttacactcataagatcatgtaaatttatttggatatgctgaaaaaagagggggtataaaatctaaagtttggtaaatctttgctttacagggcttcaagttatagatttttcttttttccttttctcttcccctttctctctctttctcttttttatttttgccatttcttctcaggagcccctgcaatttcaaaccttggaattgaattggatttgaggaggaaaacccatattcagctttaattcaaatgaattttactactttagacaaaggtacaacactctattcaaaaaagttattgaaatcacatctttaaatctgacccagccacttgaataaataagttgtgttgtagtttctcagagcaaccgccgctcatctttcactcaccttaacaatttctcacttttttctgctttttttttttttttattttctgcttgctgaaatcgagatcaatattcattgttttcttctgggttaactcttttttatgttaactgaatcaattttggctttgtttctttatgaaattacttttagataaagtattgatattgtcatttatcaattttattatatgtcttttgcttattaaaggattaaaatccacctctaaacttatttagatcaaggtcagtttttttactcctctgtagaactgtgaagataatatcctattctccttttcttatggttttattgtgaagatctgtgcaaatagctatataaaatgcaattcggtattaaagaaaattgttgcacggactacattgattagagtctaatttttggaaagtatacttcgccttttcagtaattttatttttcggtctatggtgcccacattgtgtcaccagccagccgtatgcagacttacaaaggactacccactaagaataaaaacatgatacaacttgaagaaattttcatcaaacgtctttgtcttatccccttgttatacagacaaagatgacaagggccgaaaaggaagtgattttctcattgaataagagaatccgaactggcatcgaggatatctaattttgggatgaaaattgagagaagacagaatttcaagtctgaattatgacttcactactgtgtcgtcattggtagaataaggataacaatacttatcacacagatttgtggtctgaatcacatgagagacatagatgaaaaatgtaaaacaacaattagcatgtgacatgctctcagcaaatcaattaatccttcattctttttttctccccttactcctttgattttcagactaatttggatcatgattattggcctgtgtcccacccattattcacatatagaatgggttgcattatcctctccttggaaatatctttcaaagtgggtaatgagaaaactactttgaagactgtgctgaaggaaatgatggcatgaacaactctagataatttttgtttatttggatataacgtgaatgggcccataccataaactcctattaagctgaatcaccaaaaaaaaatttgatatgaaagtcatacattgaaaaaattcactcttaccactgatttgattgatactgagcctgtaaatatttatttatatgatgtttggcactttattttataaaactaccctttacttaaaataaatcattgtattcacataactttccagggcactatgcatttttaaacaagacagtcaacttactatttaaaaaacaaagtcagtcacctaaatgactttctgactataaatttgaaaacaatattctccttgtaatatatgtgccaccagggcaagaattacaaattgggagcaggtaagaaaattgttgttgactctcattagtattctaattctccttcagtcagatttataaagtatgacctatagcatccaactccatcattttccagtcattcttgagactgtcaactctatgggcattgtttagcagcctcgaaacactgaactttttacagtcttattggagagaaaaacacattaaatgatcaaataatcttttatgagctcagaaaaaaatgcctaacatgaacatttaagcatcttctgtttctgtgattcccatttttggagagtaaaaatttaagaaacaaagggaatgtgtctggggatggtactaataatattgagattttacaatttaggttataatcaagataattatgtatatatataaaattatatatggtatagtttcaacttctaatcttttatcatcctctaccacataattcctcctatattctctttttctgactgtggcctaatacctcaagaatattgtatatgcttgtcactatataaacttcaccctaaggaaatttccatgtcagatacaataagagcaacggaagaaaatgtatcaaaacacatctccaatttatttgaatttttctggcctaaccttgttggcatgagagttcccactttgtattataataggcaaattgatacacacttttcatttattctaaataatagattagcatagtcaggaggcttggattggcagctattaaatacaatttgaagccgtgggattttattaggattctaaggttattctgtgacgatggaacttaatgatgtaagagttaattacccattgtcaaaaatcattgcccatcaaagcagtgagactgtgtgctatgtccagttttattcatttcttttgtgtatctgaatggaacatgtggtaaacacaacagtagaatatacctacagtccccttagaaactcttaaatcttcaatttataaaagtcatcctaagacgttaaaaataacttacgaaaggatagattccaatgtcagtgggtgagatgtgctctagctagtgtgcacgaaagagaacatggagttagaataattattgtaggactgtagattgtcatctcaagatcagtgtcaaatacattcattcatgtagtattttcacatgcattctggtctaaatatcccaacatatctttcgttttgagatctgcagaacaaagtcaatgtctgaatttagagactaatttgaccattttgattcaaatgtctaaaggctaaaccagagcaatttacaacatccaatgaagtaaaattatataattaattatataattatataattatataaaattttataattaattataaaataaaatattaacaataattgaacattgtttacttttttatcctcacaacaattcaacatgatatgtatggttattactaaatgtataatacatttagtaatgtgatttgacaaatcacatttgtcaaataaggaatggctgaattaaatgattgaatgaaggagtgaaggatgtagattgtttaagtacattcaacttgtaatgaactgtaaacttcacccataacattattaatatatcagtgctatcaactacattttacataggatgaaaaaaatcattatttttattaatcccaagatattttatttcattatataaatgaaatattttatctgttataaagacctttatttttgttccactcattaaataacatggtaagactgttgtgtaattgactgaatagttaagtctaaatgggtaaatagctgtttatgttagtattgcagggtagctatttgataatgaaatatacttttcttacctacttgcaaaaaaaattacataaacaagtatttcctagagttcaaacactgatctttttaagtggcaaattgtccaaaagaatttaattaatataaacaataaattcacttaaacaactatttacatgcaaaagtaatatttttattgcccatttggaaaatagttttgctttctggtttataaggaacttttactagtttaattacttgggtgctttaaatgttttttggaggctattacaaaatcacatcctaaaattttaaaatggaaaaattataataattgaatttttaattcctcataaatattttaaaagtacacattgttccatggcttttgcctttagaataaatacaacatttttatgtagaaatatattcttgaaatgtaactagcacatagtcagtgtttcttaaccattttggggtcctgaaactttttgataatgatgaaagcacagagatgctatcaagaaaaatttacccacataggaacacacacacatacacacagacacacacagagtttgcttataagctcaggaagcttaaagatctgctaaagattatgcttgggtttgccatgaatcataaataccaagtcaaatacctttgaatttgattcttaacaaatctttgtggctgagaaaccatgagatttcattctggcatgtccccagaatgtaattatcaatgaacaatagccattgaaaaaatctgaacagatattattgaggctcaaggttgtttaatggcacagataatataattcaaatcatgaccccagggctgatgaagtcttgttgtaacgtgtaaatggggtgggtgatgggagagagaaaacaaaataattatttatgttaaatcatacataaacagtaaagccaacacaataagtaaaataagagaaagtagaatgcttgggaggtcatatgtttcaaatgtatgcatacacaaaagagtaagcaacaggatacttcaagagtaaaatgggaaaaaatcatattgggtaaatagtatcaccccaaagtgatagtcaaaagtacctatgtttgcctagttctcagattacaactatgatgataatttagataaacaagcagaaaacaaaactatagaaaaaagtcaaagtgacataaaacaattactggtgtttcaacagaaataaacccaacatcaggatttatcaaatatatgaaaaattatgaaagattataaaacaccaatgattagattatgttataaagacactatgaagagatactaaatgatattcttttcatctgtggttactgctaaaaaattctttcatagaaattcttggattttgaaattagtttaattccaaaatattttctttattttgcaaaaatgtaagacaaatgtataggatatttttctctgttgttatgcaaggatttattatcacattggccacagaacacatagaatgttagttttgtagaaaattttagagattttaataccaggatgaaataatagtatcattctatttcaggttcttaagcaacattcctaagactagaaccttatcttgaaaaattatgattttaaacttaagggaattcaggtaaaggaaattgactaggttaaggcaaatacatcatgtttactggtaaagataacattatttaaggaaggtaagatactcttatcctacatatacgccagaaaaattgcttctcctctgaaaactaccattatttttgccaaatattgtagcttagttttaagtttttctcggctgtttcctctgacagttctgtggtaaagaagaaacattataggaagcatttttttttcctacagagtctgccatatggagaagtagaatgagaggccacctaggtaatgtgatttattaaaagttctccatcccaaaatatatgtcccatctgtgggctaatgtctgaaagtcctatgattaaactcacttttatgtaagatagtgaggccccagagagccctcgagaaatgcaaataaactattactgacctcccttggattatgatgaaaaccgtggagtctttctattctctgtcaaatgtggaggtcatggatccttcttggcacctaagattaaaactcatagaatgtgctttaacttctgtaggcacatttcctttccaattagagtgaggtgttgaatatttatttatttgtttatttttattatactttaagttttagggtacatgtgcataacgtgcaggtttgttacatatgtatacatgtgccatgttggtgttctgcatcttaagagaagactatttataaaatttattgcttgtaagatttgttttttgttctcttactattatgaaaatcacgaacttgggaataaggacactctgggcccggcgcggtggctcacgcatgtaatcccagcactttgtgaggccgaggcgggaggatcacgaggtcaggagatcgagagcatcctggctaacaaggtgaaaccccgtctctactaaaaatacaaaaaattagccgggcgtggtggcgggcgcctgtactcccagctactcgggaggctgaggcaggagaatggcgtgaccccaggaggtggaacttgcagtgagcggagatagtgccactgcagtccggcctgggcaaaagagtgagactctgtctcaaaaaaaaaaaaaaaaaaaaaaaaggacactctgaacaattgaacaagactacgctgaaaggcagagaagaagtaattatgaacaaactgttcatgaagtgatcaattgaatttgaaacagaacttttcctagcttctaaatgattagaaatttcagctttggtttaacttaaaaacttagaattgtcaattctgtccaagtctctgagtcatgtacagaactcaaattattacatcatttttttacttatctgtattatttctccatttaaaagtggacaaatttttatactatatcctaataatgatacaaggtgacttgtaggactctggatagaaagagatggcccaggatacagagggcactccttaaatagctgccaaataaatgacattaaaaaatgtataaaaaggtatgttaagtaattaaaagtgtcaggcattattttcctattatgagacattttatattatggttatttactgtaattgcatccaaaataattcataaaacatttatttttgtactattaaaaatctaaacaataataaccagatggaggaaaatgataccatctgatttaattattaacttgaaggtcagtttctacaacttattctcatttatgtttatctgatttggccacagtttcttactttctcatattttgctaagcttgtggatgaagccgcatgtctcttttttttttaacctggcatataacactgtcactctatttaattattacccatcatctacctactttgaaactttggaggttttataaaaattatgagtatttaatcaaagttgtctctttatcatttgccagtgaaaatataaaacctggctgttttattctattgtgcactctaattacataaccaaaatctttttaaaaattcttagttcttttagaaataccatttgacccagccatcccattactgggtatatacccaaaggattataaatcatgcttctataaagacacatgcacacgtatgtttattgcggcactattcacaatagcaaagacttggaaccaatccaaatgtccaacaatgatagactggattaagaaaatgtggcacatatacaccatggaatactatgcagccataaaaaatgatgagttcatgtcctttgtagggacatggatgaagctggaaaccatcattctcagcaaactattgcaacgacaaaaaaaccaaacactgcatgttctcataggtgggaactgaacattgagaacacatagacacaggaaggggaacatcacacactgggcctgttgtggggtcaggggaggggggagggatagcattaggagatatacctaatgttaaatgacgagttaatgggtgcagcacaccaacatggcacaggtatacatatgtaacaaacctgcaagttgtgcacatgtaccctaaaacttaaagtataataataaaaaaattcttagttatttgaaaatagtttttttgaattcacaaacttgcaggatgaaaaaagttattagttcctgaagatataacattgatttgtctttttcttatttgatatcagctagcagtaaaattgtgaacaaatctggtaaatcttttggtgttgcaggttcataatcagttaattgagtgtattcactataaattgctttaattaagtgatgtttgcctaagaacaagtttcatttcatctcatgaaaaaaatgttactttttgtattaatcagtggaatgtttaaagaaaaaactggttatcttgaagctgtcaaataattataagaaatctctatacattacgttttaaaatacataaaacccataaattcaagcttattagttttcattttcagcaaggtttatacagagaaaataagtaatacaaattagttttccagaaaatctaattttatgcagataaaatctgaaaatcatataagtccaagatgaaactgatctcaaattattattttgaggtgtatccatttatttaaaaaagcctcattttagctagcaacactatgtagaaaaatattttaaataagacagagcattaaaataatgtattcattgatctcataaagaatagatgatcagattttttaaaagtgattttaattaaatggacatgtttctctttagccagaaatgactgagaaattttgagttggaattgatataggggaatccttggaactatgtgtgaatatgtgtgtgtgaattatctgtgtatatttacataatttacactattcacagtccttgtttttcttgactcaaatagctatctcaagtttcgtacactttttagatctctatgtaaatacattatttcatttgtggaaatatattgaggcctatatcaataacctcaaaccttttaaacacttagagcaagtcaatatgacttgttctgtttcagctatctgaaatttaaaaatttgacaaatttttaaagtacccagttcttggaaaaagaaaaacaaataaattggagatttggatcatatgggctatgactaaatgagacaaggcatacatgctgacatttgaaggatttatgaaaaaaagtccactgtggaaaactgatagtttttctccttctttcttgaatatgtttagttaattttgtggaaagaggaaggcagctcagtttacaaacagcagtgggttgaaggcaatgctgtttatattcttgaatttcaatatctacaaagatgtcatcattagattttatgtgttaaaaagtggatttatagtctctaattaataaggtgcatatgtcaagactcaggaaaacagatcacttacgtagttctccaaaaacgagagtcccagattcaataggaaggcatgcagagtgttctctataaacccagcaaaaccataaaaattgactggaacttttatttttcagtacaacaataatagtattgaaatacctaaaaagggcaggaaacaacacagaataatctacgcttgtcatcatgttttctaatctataatctttcaaactggataaatgggaagttttggaattttactgtggtacagtcttagttgctccgtggttgtcaaatctgtctgcacattaggatcacttaggaagaattttaaaagtatgctgatgcctggaaactccagaacaattatgataactctgagcatggagctcaggaatgggtgaaattcttccccagagatgttaatgaacagccagacttaaaaactagtaatttagacaagtgtgagcagaggttaataatgttgagatgaactgggcttaatatttcactaacaaggtcagagttttgatacatcacttaactcaaactttgagattcttcatcactgaagtagcaataataatagtcatttctgttttaatacttcatagacttgtaaggatgtaatgtagtgtttctaaaaggagtgaatggacaatctgcatcagtgttaactaaaatacattgaaagtgccaattcctagatctatcctagatttacagggaagaattcagtagtctgaaacacacattttcaatatattgaaaagatgattcttttgcatgatgacttgttataatcattactttcataggtaatggaagtaccgattaggagagtaccaaatacatattaaacactcagttcatgtaagctataggccaataaacacaactttggggtttactgatgttttccaacatccgaaataatagctgaaatttagaaacatagttaatcacacaaaaaatgttgcatacatactgtctaactaccagtttggtatgtttggggctggtgttatgaaagactattatatgattaatacaaagttataatttttggagtcttttagtgtacccagagcccatgagtttttattttctttttggaataacagaaattaggttgtggttcagtggaattacagaagcaagtgttttagatgttcaagtttaaaaaatgagaaaaaaatgttttacatgaagaaactaattatttaaattcatttttcaactatttaatgttattttaatatagtcatatcatccagaaaatcccatcttagacaaatgggttttcaataaattattattatagttaggaggcaatgtataatagtgataaggggcatagattttgaattacacaaacctgaaatccaatgctctctctttcatttattagttatgtgaccttggacaagttagtaaaaccctatttttcatatgctctttagcttttttaatacctcttaccttatatggttgtttaatctattaaatagacagtgaaatgcacatgaaatcttcacacagtgtctcatagttgcttggaacatatttatgtagtaagcattgttcttggctgagcttacattaagtgatctgtaaattagaagttatttgttatatttgtttcgtttccttattgccctagatgccttttctctggacctagataatttagtctcactctgtggcctttacccttcaataaatatggattattaatataatttagctacataattcctaaggaaatattaattcataaagattgttaaattgaactgaatatctttgctaagtcacaggcattgattaaattagataaaattgtcattttccattgattttgtttatataaataatattgaattatttatattcttatttagtctagtagattgacaggcagttttattaagaaatgaatcaaatggtaaattttgaatcatctggtaaaaatggacaaaatttagttttatcttgtggtctggaaatacaccctaaattattgggtcaagttagtgaaaactgttaaattgattatgaacgtaggcacattacttataaatccccttatgctaacttaaaacttgtgaatgtttagtgttatccagctataattcttctaaacatgtcttgtaatttttaagtttgcatgaaaataactccatcctgagtatactcatttcaataaattatttgtcctgagcatactgtaagaaatttagtaaagtactaattgaatttagtgattagactgtgattagactattacaaattcacagtgcttgtacaattcagatattattttgctttgaagtcaaatagaggaaccttaaataatttaaataaaaataattgtttttattaaagtttatacagcaagataataaattcactaatgtgaaatgttgatatagtatgtacaacttgtttcttaagttactaaaaatgtattttcctacctacataatgtcaatctctattgctcctaacacatgagtggctaaaattgcaaacttaatcacataaataatgagattaaagttaaaatgaaaaagtggtatgaggactattgtttgtgttaagtgaaattataccttgtaaaatttcatattatgagagcaatatgtaaatttcattgcaacaatggttattcaatttactgatgaaaatcagaagaatgttgaaaaattagtgcatttataataaatttaattattcataaaaaattaacattgatatatatattcataaggataaaagatatcaaaataattaaacaaatttcactttcttcttataaaagaaaataatttttatggtaactaattttagtagtgcatcagatcaacactattgggcacccagttatttggtggtacgctgagtgaaaatatgtagctttatctacattaccttggtttggacaactgaaaaatttgctaggaaacaaatattacaaaatatgttgttaacttttcaaagatgatcggtttagattgctttaacttgaaggacacttatattttgtatcacttttgtagcaaacacatgactcatcattgcccaaatcaattgcccaaatcaattcaaacatctcattgtagttcatcccatggcagaaaagtgtttatccacttagtaaaatggaaaacactagagcttcaggtttaatttgaaattttaacttcattaagaataaacttgacctgtttgttctagtaagtaaaaacactagatacgtaccaaaattgtcttttgaccctctcagggagtcaagttttgatttgcttgaatacaagcaagtcgagctatggtaatttgcaatgctgacaggaaagaagaacttgcttgaggcaaaatcatgaagtacaacttttcctctgcatccttttacctcatgtttgtaacatttcccctgttgttatttttacacatctggatgctcagaaaggcctccttaccacaataattgaaaggagtactttgtcaatagtcagaattgaatgagagataggttgttgggaatattcagggtgaatgtgtcttttctactttgactatatttaccattgactacagtaactcagcagaaagttagagggcagcatacatacattggtttatggatttaatgaaaatatccccaaccattacattacagacaattcatatatatgtcttgaaaatcttcttgacaatttgtgacaaattttctaaatgtttttccaaaaatagttggttcttgtaagtgattttgatatgactgattaccaaattatggtgggtaaagatgccacatgcaacagaaaatgtgtctaattatgtttgttttagagcttaagaaatgttaagaagagaagttacaactgcattaataggattttaatttttattcaaaatggacaacttatttattatgtacttctacacacagctaagcttatagatattttcatttaaagaaaaactatttgttcattttattagcagatatcaaatgcccttttgaaaattgagactgatttctaaaacaaaaaaaaagactttaggagttttaattatttttaatatattgcttctttattaaaaaaagatacaatccttcaatgtcattcaacagtattaattgttaaagtgtgggatatagtttacattaccgagtttattttctaagggtagtgaataactcctgacaactactgatatcgtcacatggtcctttagtgaccaaaaatgcacagttgtaagaatgcaagtgttacttgtattgaaaaccggattacattaaaggatggacaattatgataaaggatctgagataattggacaattatgataaaggatctgagataattattctaactttttggaactatactttcactcattgatgaagtaagttacaacgtggaataacaaagtttaagtgtggcagaaaatacatacatatgtttaaaagtagggaaaattttatcaattattaaagatggaaaaaataggactatgtcaaatagttaaacaaatgtggggtattttatggagaaaagaggcatgtactaccttaaacattttccaattggaacatactatagacaaaactgacagattattattcaatgagaaacctgactcagatgaagttacaaaaaaagtactttttaaatgtctagtttctaatagagttagagctttgttgattgagatatgtggaactgccacatatctctgtgccatacttttggtaccttcataataaacggtaaagtgagggaaagggtggaagagacaaatcctacgtctcttccagaacttcgagtgcactataaattaaatatttaaaatatttttgcaatagttagctttcaattatgaacactctcagcctctattgctttatatatgcatttattttggtaatttttatacatcaaaactataattacctgtatttgggcagaatgatttaggttatgccagctattgtggttaaagctgtagtaacttacagtacattgaaattatagactaaggttctgaatattggtaactcactgttgttgtgcacctttaaacaactcttaaataaagtaatgattctctttatattaaatttaatgtatgtgtgcctcatggaaatttgtattttatagaaaaatattgaatattttattattatgtctttggctcacctactttaaggagatggctacttagggtactttttaatccaatataatgtgaaaatttgatcatgctatattcttaatttaattgtacttctatggtcatatacaatttacctatcactttctcacataatcaatttaactttttggtaaatcttctaagagaccgtctagacagagtgaaatgaaagctgaaacaacagtcaaatcaaaaactgctttggtctcaaatccatgtttttcagaaaagatattcagatccagttatctggcaaatggtctcaaacatacatttcaatttcaatgttaaaaataggatattaaacatctcagaaaatattgggattattgaagcaaattctaccctggacttggagtaaatgtgatgaacagattaatgaggtggaagggactagaactttgggaaagtgcaaccttgttatcttaatatttttatagcttagaaagagaatgctatgcaactcatattttgatcttttaatgttaaagaattcaaataaaaaccataaacctgaaactctaaaagaaaaattctgttttgagagagatggcctcctctagtacacttttaataaatttaaagtatctaaaaggatgcacaaagatctctaatgtgctgtgattttcaaaggatgtcatgtataaaagatttgagtgagaacatgaaagcaaaagcaagttcagaagaggaacacaaccaggaggacagtgtgtcaggaaaatccaagaataagtggaggtgtaaaggctaaaaaataatgcaaatggtgcatatccttctgtctttctctcatacacacagacacacttacacaacacatatacaaatacatacatgtatatatgtatatatatacacaaatatacacacatattcacataatattcaagtatgtatacatatatacacatatgtacatacacatatgtatatatacatacacacagattgagagattaaccatatgtagatacacacatgcacatatgcaataatgaaatcatttcaaagcatgccaaaaagtaataaaagatatatcctctgtttgggataaataaaaaaaaagtttaaaagcaaacaaaaaataaatggcaataactaatcacattgaattttgttatggcctttttcttcctaaaaagaataaccccaatctgaacaaagaaattcaaagtaatggaaaactcaacaatgaaactcaaagtagactagcagataagatacctatttcaaacatcagtgccaaggtaatttataggtcagtgcattgataacttttgccaatgatagaaaagatgccagagaaccggatcctgacattaaaaaaaaaaagtaaaaagattctgaagactgcatttctgagcttaaggtagattctaaacaacatcttagaaactaggaaatgactttatgtttctttgtttttcaatgtaaatggatcaagatttcttaaaacagaaatgaatattattatttgtgatgagagcactaggggcaattttgatatttttgataaggtttctagagtaataaattagaatgacaggaatatatattgattttaggaaagtgtctgtataattccacatgatattctctggacaaaatatgaaaaggtaggctgaataacatttttaaagggcagtaaattttataattgttattgattacaatgaaggcctctggtaatgttttccagggtcatatcctgttacatatacgtgacatggataaaaaggaaacaaatatttattgtgtgcctagtttatgttatctcaattccagctctacaaggagctacaaggtaaaattgctacctttaaaaacatatgaggtaaaattattcctattcacagatgtagaaactgagtttcaagaaggttaagtaaatttcctcatattgggaggctggtaatgcagaactgggtgtcaaaatcaagtctgtatgaaccttctgttttgtctcccatgaagacaaaaggcatgcatataaaatttgttgaaacacaaagctgaggaggcataataagacgtggaatgacagaagcaagatctagaaagtttgggatcatgaatcaaaagaaacaggataaaattatcctaaaattaatattaaatcttacaagaaaccccccaaaatcagttgaatttgtacaaaacggtaaatcattttatcagtagatcccataataaatattataaagtttaagtgtgagctctattactcagtaatatgatgccattactgtgttgatggatgtattgtcaaggaaaaagaagagaattacacactgtttccttcaattgttagatggcactggatgtagtgttttcaatgttaatcctggtatcatgttctttgccataaacttgttgacaaattggcaaatactgacatgaaatatgccaatatttgagcatctaaaaatgtaggtactttccataccacatcatatattacaatttgaaaatgtttgtttcattttttatataattattatacagaacagtttttctatgatagcattataaaaattcccagagaatactggcccagtaagaaatggaatgttcacaactcatagtgtagctatatgaaagaaatagatctaaacgacaggttggtttccaaattatattttcatacctggaaaatatctactttataaatagcacaaagttatagttttcaatgaatatgaaaaagttcttgcattaacatattttatgtatcttttatattgacatttgtgattgccactaaaatgtgtattttctaaatttcattgtgcttttacaagatacttttttctttgatgtccataactgctgaaaaggctcccctaaggagaattttaagactaagtaaggtttttagtgagcttaaattatacaattctgaggcattatttaaggtgcatactgtattttttgcttgaaacctgtcagcattttatttgtatggcaattaaatgactcagccattcatgtctcatgccagtctttttcaattgttatttttaacaaagaaaattatatatatatgtatatatatattatatatatgtatatatgtattatatatgtatatatatataaacttacagcaaaaatgtttaaaaatagcaaatagtttgagtatagttaaacctaataactgtacttttgtttctatgcctctgagacaagattactagacccttattcaaagtttctaaatataggaaatagaacattgggccatgctaaaaaaattgttcagattttcttttgaaagagaatagttatttttcctcctgacctctaatgaagatgctttatttgtcaaggtgttttccttagaaaattgacccagtgtcaactgtaaagaaaacatagaggatccttggatgattgaccaacttatccaaacacaggtttagtaaagagaggatataaagataaaatgtgaaatgacctctctgagtcacatttgttttcataatttcctagcaaacatccaacttcactgctaccctcagcaatgtttcttgaaacatttttaagacattgatagacaccaatagctgatctttagaaagccattcccagaagaatatgtaaggggttacaactcatttcagggagtctgcctagctcttgatattacatgtctttggcatacaattgtgtaccttttatcattgacagtgaagaaaataatgccatttgtaacttctgagatatacacacaatactatcaactagccggttaataaaagataagaaaaataaagaaaatagaacatttttaggtgtctggcaagtatcctctaaatcaaggtaaagataataatttagtggcagtgttcatattttcctatgactgtaagatttaggtgcctcacaaaatattaatatttagcctcttatgaaaggttcgtttttcttctaacactttagtagctgaatacaaagaaaatacacaacagctgtttataaatgaaataaaaagtttccattttttatctgagtttctcatttatttgcagagaacgaataaaataaaaatatcctagtgttgtttgcaccacagcataccagtaaatcttaaggattgtgtttcagtatgaaaaggaagagcaggaagatttcctcattctgtcttaccagcaaaagtctagccttcacacacacacacacacacacacacacacacacacacacacacacacacacacagagtcatctatatgaacacgtacttgagtttcttaaacatatatgaagcaccttccatttccctttataataaatcccttagtttttgctgttcattaaaaaacaaaaaggaagagacaagctcaggacattctgaaaaccaatgtctttaggacacactaaggtgtcctgaattactttaacggacacattgtaaagacacactctccaatccctattaggaaaagtttagtcaagtttgcttactatttgggtgcttataccaaaaaagcatcatttaggacattatttaggataatattatttatgcaggaattgtaccacctatttccagatggtataacttattatctgacaggcatgtagcaaatagaacacaaagcataaatctgtcaggagaaatcatacgagaaaaagagcattgtctggttatcagaatatcagatctctcattctggccttgctaggaaatagatctttgattctagaaaagtcaactaatttctatggttcttacttttctcctttataatatacccatttaaattccaaaaaggtatatgataaatcacaataatttcaatcacatggattttaatacaaaatgtataaaatcaatttccaaaaattttctgcatatactgaaaatgtctgtacgaatgagctaactactataggccttccctaatttattctattaaatgtgggtactcaatgtaacctgaaaatattgagcttaactcttctttttttttttcaaaagggaaacttgaaaaagactgcttcccccagaaaatttatcaacaataggtgctcaattaaatgtttttaaacaatgaacaatatcccctttcatataaataatcaggggagagatatttttaagtcttttttttctttttccatagtgtcacctacacaaaaaattatgtaaagacaccacttctatgaggaggtattcattgtagatgtacagaagtcaacggaaacttaagtttacagaaaaaataaaccagattatcattccacccaactgtatattcccacagatgcttaataaaagctatctgatgatataatgaattatcagttcttgaggaagtatatacagttggtgactatttttcaaaaatcatcatccaacaaatttttttcatttaaaatctttcatattaccctttcgacaatcagttgaaattttaaaactaagaacatttaaaaatataaatgaaagtagcattagctatagactgatattcaacttcagacgttaaaataaatacaagtgtgtattaagagtaaaattatgtcaacaatgtataaatgaaaactgccaatgtaattaatgtttcttttaacatatcccatccattgctttccctccaaaagacaaaggtagcaaaagacgaagcaggaagaactgcttcagaaactgaacatactgatttaattggctaagaagtccaaatgctaatactcctaataattagccattccttttgtgttttggtgacatatatcctcatacaatgtatatcaaatggaattttttgatttacacctgacatttcaaagtttccatttttgaattctcctagtcttaagtaagtagaacattgtctcctttgtttgctaggcataacgttttccccaacatctagggctccatgatgcaaaatatcattttgccgatcttctgttccagtatttactttaattttttttattataattggattttcaaatacaatcacaaaaacatctcctgttgaaggtggtttcccccaaaagtactcatcaacactactgtaagccttgcttgcttcataattttcaaacacattcatgttggtgtacagacttgcaggggggttatcaggaatgtcaaatgactcctcttcaaaatcatcatccttcagcttattctccgtccctttgtatgatgaataatagcccatgtgctgaaagagagatggtttaaaacggatcacatttttctgagccaacagaccacggaaatgagtcaatagccaatcacaaggcatttcttgataaaacattaataaaaaatgggccaaacgtgggagatcatgagaatgatagagtttaccaatgtagccaagcttagagaattcaagagttacccagtaagttccttctagggatgcaatgactttcttgatggcagttaagaaattttttgaacatcgaacatcatcttcaagcattacataatagtctgaagtattggcacaaaaattaagcagaaaagcataatctacattttgcttggaacgaaatttgactctatcttctggatcattgtaatttcttttaaggccatctaggattgggtaatactcctctggagcatgtataaccattaatcttcctgcaataatatggtgcgcaaatttctgtgtaatatcctggaccatggcatcacgccaggaagaattaaagtctgctaggtgaaccaccactgaaatttccttcagctcttcatagctggattgctcaaaaattgacttaattgtctcaagtaaatagtttcctttttttcgctttactgaagaaagtccaattgtaagataccgctttctttgtaaaggtgtggcagctaggtagcgataggtgacatttatggctcctgagaaattagataaatccttgaaagtatgaacatagcgttctgaattcagttgatgtgtggatgtttcccttataagttgtttgtctccttccagaacatagctatcttcaatgtacaagttcataaaaaggagaaaaatgacaagaactcccaagaatgacactgtagaacgttttctcaggcatctcattttatcaagtatttcaaaaatatgtttcatttgatgaaatttaaacattctcttcttaagaaagacgctgtcataatctgtgctgtacagaaaccgttgatacccagagacagagaaaacaattcgttcagctagatccaacagtgctctgtgcagcctggaagcatgagtgatccttgggcctcacacaaaagcgagataattggctctcaatgaagagatgtaaacatccatcataatggcactgtgctgaaact

SEQ ID NO: 13485 - RNA, 22555 nt, Homo sapiens
  source 1..22555: mol_type = other RNA
gctgggattacaggcatgagccaccacgcctggccagtttttaaagtatttcatacagtgtaactaggcagtcagaaatacctgtatctcaaattcatttaacttttcaatgaatcaatcttcttattttctcagacatataaattatcataatactttacattgagtctctatggttgactatatgctgtgaaggaaggacataaatacatgtgaggaaacaattattgatatttttaaactaactagaaagcaccaagttatttgttaaataaacaaagttaattttatctacctgttcagtaagtgttggcaactatgaattaatctttgacaaattcacttacaactagcaattttaaagacttaaagtttaatttttattattaaaagggtatgattatttttactaaaattaataaaaagattaactgttactaaattaaagctccttcaaaaacataaatgtattctttagagagttaaaaaaagtagcaataaaatacatttttaatttagttaagcttacttaactaatgatcaaatagattaagttgtataaaattttacaaactttatatttttgcatacacttatcttcctggcatttttgaaataaaaaaaatacaagtgcatagggcagaggaggcgattcagttacttctgctatgttattaaatctctggtaaccactatacaatacaatacaatacaatacaatacaatacaatacaatacaatacaatacaatacaatacatgtagactcagcatccaaactttattttaccttcaagttctacctgataaagtggtggaataaagatggtattttccataactgtttaataataatcacatgttttatacccattgctttgaagaagaaaccttaagcaactagaaatgtcaatctaaaaggcagaaaagctggaaaaatctcatgaagactagaagatttacactcataagatcatgtaaatttatttggatatgctgaaaaaagagggggtataaaatctaaagtttggtaaatctttgctttacagggcttcaagttatagatttttcttttttccttttctcttcccctttctctctctttctcttttttatttttgccatttcttctcaggagcccctgcaatttcaaaccttggaattgaattggatttgaggaggaaaacccatattcagctttaattcaaatgaattttactactttagacaaaggtacaacactctattcaaaaaagttattgaaatcacatctttaaatctgacccagccacttgaataaataagttgtgttgtagtttctcagagcaaccgccgctcatctttcactcaccttaacaatttctcacttttttctgctttttttttttttttattttctgcttgctgaaatcgagatcaatattcattgttttcttctgggttaactcttttttatgttaactgaatcaattttggctttgtttctttatgaaattacttttagataaagtattgatattgtcatttatcaattttattatatgtcttttgcttattaaaggattaaaatccacctctaaacttatttagatcaaggtcagtttttttactcctctgtagaactgtgaagataatatcctattctccttttcttatggttttattgtgaagatctgtgcaaatagctatataaaatgcaattcggtattaaagaaaattgttgcacggactacattgattagagtctaatttttggaaagtatacttcgccttttcagtaattttatttttcggtctatggtgcccacattgtgtcaccagccagccgtatgcagacttacaaaggactacccactaagaataaaaacatgatacaacttgaagaaattttcatcaaacgtctttgtcttatccccttgttatacagacaaagatgacaagggccgaaaaggaagtgattttctcattgaataagagaatccgaactggcatcgaggatatctaattttgggatgaaaattgagagaagacagaatttcaagtctgaattatgacttcactactgtgtcgtcattggtagaataaggataacaatacttatcacacagatttgtggtctgaatcacatgagagacatagatgaaaaatgtaaaacaacaattagcatgtgacatgctctcagcaaatcaattaatccttcattctttttttctccccttactcctttgattttcagactaatttggatcatgattattggcctgtgtcccacccattattcacatatagaatgggttgcattatcctctccttggaaatatctttcaaagtgggtaatgagaaaactactttgaagactgtgctgaaggaaatgatggcatgaacaactctagataatttttgtttatttggatataacgtgaatgggcccataccataaactcctattaagctgaatcaccaaaaaaaaatttgatatgaaagtcatacattgaaaaaattcactcttaccactgatttgattgatactgagcctgtaaatatttatttatatgatgtttggcactttattttataaaactaccctttacttaaaataaatcattgtattcacataactttccagggcactatgcatttttaaacaagacagtcaacttactatttaaaaaacaaagtcagtcacctaaatgactttctgactataaatttgaaaacaatattctccttgtaatatatgtgccaccagggcaagaattacaaattgggagcaggtaagaaaattgttgttgactctcattagtattctaattctccttcagtcagatttataaagtatgacctatagcatccaactccatcattttccagtcattcttgagactgtcaactctatgggcattgtttagcagcctcgaaacactgaactttttacagtcttattggagagaaaaacacattaaatgatcaaataatcttttatgagctcagaaaaaaatgcctaacatgaacatttaagcatcttctgtttctgtgattcccatttttggagagtaaaaatttaagaaacaaagggaatgtgtctggggatggtactaataatattgagattttacaatttaggttataatcaagataattatgtatatatataaaattatatatggtatagtttcaacttctaatcttttatcatcctctaccacataattcctcctatattctctttttctgactgtggcctaatacctcaagaatattgtatatgcttgtcactatataaacttcaccctaaggaaatttccatgtcagatacaataagagcaacggaagaaaatgtatcaaaacacatctccaatttatttgaatttttctggcctaaccttgttggcatgagagttcccactttgtattataataggcaaattgatacacacttttcatttattctaaataatagattagcatagtcaggaggcttggattggcagctattaaatacaatttgaagccgtgggattttattaggattctaaggttattctgtgacgatggaacttaatgatgtaagagttaattacccattgtcaaaaatcattgcccatcaaagcagtgagactgtgtgctatgtccagttttattcatttcttttgtgtatctgaatggaacatgtggtaaacacaacagtagaatatacctacagtccccttagaaactcttaaatcttcaatttataaaagtcatcctaagacgttaaaaataacttacgaaaggatagattccaatgtcagtgggtgagatgtgctctagctagtgtgcacgaaagagaacatggagttagaataattattgtaggactgtagattgtcatctcaagatcagtgtcaaatacattcattcatgtagtattttcacatgcattctggtctaaatatcccaacatatctttcgttttgagatctgcagaacaaagtcaatgtctgaatttagagactaatttgaccattttgattcaaatgtctaaaggctaaaccagagcaatttacaacatccaatgaagtaaaattatataattaattatataattatataattatataaaattttataattaattataaaataaaatattaacaataattgaacattgtttacttttttatcctcacaacaattcaacatgatatgtatggttattactaaatgtataatacatttagtaatgtgatttgacaaatcacatttgtcaaataaggaatggctgaattaaatgattgaatgaaggagtgaaggatgtagattgtttaagtacattcaacttgtaatgaactgtaaacttcacccataacattattaatatatcagtgctatcaactacattttacataggatgaaaaaaatcattatttttattaatcccaagatattttatttcattatataaatgaaatattttatctgttataaagacctttatttttgttccactcattaaataacatggtaagactgttgtgtaattgactgaatagttaagtctaaatgggtaaatagctgtttatgttagtattgcagggtagctatttgataatgaaatatacttttcttacctacttgcaaaaaaaattacataaacaagtatttcctagagttcaaacactgatctttttaagtggcaaattgtccaaaagaatttaattaatataaacaataaattcacttaaacaactatttacatgcaaaagtaatatttttattgcccatttggaaaatagttttgctttctggtttataaggaacttttactagtttaattacttgggtgctttaaatgttttttggaggctattacaaaatcacatcctaaaattttaaaatggaaaaattataataattgaatttttaattcctcataaatattttaaaagtacacattgttccatggcttttgcctttagaataaatacaacatttttatgtagaaatatattcttgaaatgtaactagcacatagtcagtgtttcttaaccattttggggtcctgaaactttttgataatgatgaaagcacagagatgctatcaagaaaaatttacccacataggaacacacacacatacacacagacacacacagagtttgcttataagctcaggaagcttaaagatctgctaaagattatgcttgggtttgccatgaatcataaataccaagtcaaatacctttgaatttgattcttaacaaatctttgtggctgagaaaccatgagatttcattctggcatgtccccagaatgtaattatcaatgaacaatagccattgaaaaaatctgaacagatattattgaggctcaaggttgtttaatggcacagataatataattcaaatcatgaccccagggctgatgaagtcttgttgtaacgtgtaaatggggtgggtgatgggagagagaaaacaaaataattatttatgttaaatcatacataaacagtaaagccaacacaataagtaaaataagagaaagtagaatgcttgggaggtcatatgtttcaaatgtatgcatacacaaaagagtaagcaacaggatacttcaagagtaaaatgggaaaaaatcatattgggtaaatagtatcaccccaaagtgatagtcaaaagtacctatgtttgcctagttctcagattacaactatgatgataatttagataaacaagcagaaaacaaaactatagaaaaaagtcaaagtgacataaaacaattactggtgtttcaacagaaataaacccaacatcaggatttatcaaatatatgaaaaattatgaaagattataaaacaccaatgattagattatgttataaagacactatgaagagatactaaatgatattcttttcatctgtggttactgctaaaaaattctttcatagaaattcttggattttgaaattagtttaattccaaaatattttctttattttgcaaaaatgtaagacaaatgtataggatatttttctctgttgttatgcaaggatttattatcacattggccacagaacacatagaatgttagttttgtagaaaattttagagattttaataccaggatgaaataatagtatcattctatttcaggttcttaagcaacattcctaagactagaaccttatcttgaaaaattatgattttaaacttaagggaattcaggtaaaggaaattgactaggttaaggcaaatacatcatgtttactggtaaagataacattatttaaggaaggtaagatactcttatcctacatatacgccagaaaaattgcttctcctctgaaaactaccattatttttgccaaatattgtagcttagttttaagtttttctcggctgtttcctctgacagttctgtggtaaagaagaaacattataggaagcatttttttttcctacagagtctgccatatggagaagtagaatgagaggccacctaggtaatgtgatttattaaaagttctccatcccaaaatatatgtcccatctgtgggctaatgtctgaaagtcctatgattaaactcacttttatgtaagatagtgaggccccagagagccctcgagaaatgcaaataaactattactgacctcccttggattatgatgaaaaccgtggagtctttctattctctgtcaaatgtggaggtcatggatccttcttggcacctaagattaaaactcatagaatgtgctttaacttctgtaggcacatttcctttccaattagagtgaggtgttgaatatttatttatttgtttatttttattatactttaagttttagggtacatgtgcataacgtgcaggtttgttacatatgtatacatgtgccatgttggtgttctgcatcttaagagaagactatttataaaatttattgcttgtaagatttgttttttgttctcttactattatgaaaatcacgaacttgggaataaggacactctgggcccggcgcggtggctcacgcatgtaatcccagcactttgtgaggccgaggcgggaggatcacgaggtcaggagatcgagagcatcctggctaacaaggtgaaaccccgtctctactaaaaatacaaaaaattagccgggcgtggtggcgggcgcctgtactcccagctactcgggaggctgaggcaggagaatggcgtgaccccaggaggtggaacttgcagtgagcggagatagtgccactgcagtccggcctgggcaaaagagtgagactctgtctcaaaaaaaaaaaaaaaaaaaaaaaaggacactctgaacaattgaacaagactacgctgaaaggcagagaagaagtaattatgaacaaactgttcatgaagtgatcaattgaatttgaaacagaacttttcctagcttctaaatgattagaaatttcagctttggtttaacttaaaaacttagaattgtcaattctgtccaagtctctgagtcatgtacagaactcaaattattacatcatttttttacttatctgtattatttctccatttaaaagtggacaaatttttatactatatcctaataatgatacaaggtgacttgtaggactctggatagaaagagatggcccaggatacagagggcactccttaaatagctgccaaataaatgacattaaaaaatgtataaaaaggtatgttaagtaattaaaagtgtcaggcattattttcctattatgagacattttatattatggttatttactgtaattgcatccaaaataattcataaaacatttatttttgtactattaaaaatctaaacaataataaccagatggaggaaaatgataccatctgatttaattattaacttgaaggtcagtttctacaacttattctcatttatgtttatctgatttggccacagtttcttactttctcatattttgctaagcttgtggatgaagccgcatgtctcttttttttttaacctggcatataacactgtcactctatttaattattacccatcatctacctactttgaaactttggaggttttataaaaattatgagtatttaatcaaagttgtctctttatcatttgccagtgaaaatataaaacctggctgttttattctattgtgcactctaattacataaccaaaatctttttaaaaattcttagttcttttagaaataccatttgacccagccatcccattactgggtatatacccaaaggattataaatcatgcttctataaagacacatgcacacgtatgtttattgcggcactattcacaatagcaaagacttggaaccaatccaaatgtccaacaatgatagactggattaagaaaatgtggcacatatacaccatggaatactatgcagccataaaaaatgatgagttcatgtcctttgtagggacatggatgaagctggaaaccatcattctcagcaaactattgcaacgacaaaaaaaccaaacactgcatgttctcataggtgggaactgaacattgagaacacatagacacaggaaggggaacatcacacactgggcctgttgtggggtcaggggaggggggagggatagcattaggagatatacctaatgttaaatgacgagttaatgggtgcagcacaccaacatggcacaggtatacatatgtaacaaacctgcaagttgtgcacatgtaccctaaaacttaaagtataataataaaaaaattcttagttatttgaaaatagtttttttgaattcacaaacttgcaggatgaaaaaagttattagttcctgaagatataacattgatttgtctttttcttatttgatatcagctagcagtaaaattgtgaacaaatctggtaaatcttttggtgttgcaggttcataatcagttaattgagtgtattcactataaattgctttaattaagtgatgtttgcctaagaacaagtttcatttcatctcatgaaaaaaatgttactttttgtattaatcagtggaatgtttaaagaaaaaactggttatcttgaagctgtcaaataattataagaaatctctatacattacgttttaaaatacataaaacccataaattcaagcttattagttttcattttcagcaaggtttatacagagaaaataagtaatacaaattagttttccagaaaatctaattttatgcagataaaatctgaaaatcatataagtccaagatgaaactgatctcaaattattattttgaggtgtatccatttatttaaaaaagcctcattttagctagcaacactatgtagaaaaatattttaaataagacagagcattaaaataatgtattcattgatctcataaagaatagatgatcagattttttaaaagtgattttaattaaatggacatgtttctctttagccagaaatgactgagaaattttgagttggaattgatataggggaatccttggaactatgtgtgaatatgtgtgtgtgaattatctgtgtatatttacataatttacactattcacagtccttgtttttcttgactcaaatagctatctcaagtttcgtacactttttagatctctatgtaaatacattatttcatttgtggaaatatattgaggcctatatcaataacctcaaaccttttaaacacttagagcaagtcaatatgacttgttctgtttcagctatctgaaatttaaaaatttgacaaatttttaaagtacccagttcttggaaaaagaaaaacaaataaattggagatttggatcatatgggctatgactaaatgagacaaggcatacatgctgacatttgaaggatttatgaaaaaaagtccactgtggaaaactgatagtttttctccttctttcttgaatatgtttagttaattttgtggaaagaggaaggcagctcagtttacaaacagcagtgggttgaaggcaatgctgtttatattcttgaatttcaatatctacaaagatgtcatcattagattttatgtgttaaaaagtggatttatagtctctaattaataaggtgcatatgtcaagactcaggaaaacagatcacttacgtagttctccaaaaacgagagtcccagattcaataggaaggcatgcagagtgttctctataaacccagcaaaaccataaaaattgactggaacttttatttttcagtacaacaataatagtattgaaatacctaaaaagggcaggaaacaacacagaataatctacgcttgtcatcatgttttctaatctataatctttcaaactggataaatgggaagttttggaattttactgtggtacagtcttagttgctccgtggttgtcaaatctgtctgcacattaggatcacttaggaagaattttaaaagtatgctgatgcctggaaactccagaacaattatgataactctgagcatggagctcaggaatgggtgaaattcttccccagagatgttaatgaacagccagacttaaaaactagtaatttagacaagtgtgagcagaggttaataatgttgagatgaactgggcttaatatttcactaacaaggtcagagttttgatacatcacttaactcaaactttgagattcttcatcactgaagtagcaataataatagtcatttctgttttaatacttcatagacttgtaaggatgtaatgtagtgtttctaaaaggagtgaatggacaatctgcatcagtgttaactaaaatacattgaaagtgccaattcctagatctatcctagatttacagggaagaattcagtagtctgaaacacacattttcaatatattgaaaagatgattcttttgcatgatgacttgttataatcattactttcataggtaatggaagtaccgattaggagagtaccaaatacatattaaacactcagttcatgtaagctataggccaataaacacaactttggggtttactgatgttttccaacatccgaaataatagctgaaatttagaaacatagttaatcacacaaaaaatgttgcatacatactgtctaactaccagtttggtatgtttggggctggtgttatgaaagactattatatgattaatacaaagttataatttttggagtcttttagtgtacccagagcccatgagtttttattttctttttggaataacagaaattaggttgtggttcagtggaattacagaagcaagtgttttagatgttcaagtttaaaaaatgagaaaaaaatgttttacatgaagaaactaattatttaaattcatttttcaactatttaatgttattttaatatagtcatatcatccagaaaatcccatcttagacaaatgggttttcaataaattattattatagttaggaggcaatgtataatagtgataaggggcatagattttgaattacacaaacctgaaatccaatgctctctctttcatttattagttatgtgaccttggacaagttagtaaaaccctatttttcatatgctctttagcttttttaatacctcttaccttatatggttgtttaatctattaaatagacagtgaaatgcacatgaaatcttcacacagtgtctcatagttgcttggaacatatttatgtagtaagcattgttcttggctgagcttacattaagtgatctgtaaattagaagttatttgttatatttgtttcgtttccttattgccctagatgccttttctctggacctagataatttagtctcactctgtggcctttacccttcaataaatatggattattaatataatttagctacataattcctaaggaaatattaattcataaagattgttaaattgaactgaatatctttgctaagtcacaggcattgattaaattagataaaattgtcattttccattgattttgtttatataaataatattgaattatttatattcttatttagtctagtagattgacaggcagttttattaagaaatgaatcaaatggtaaattttgaatcatctggtaaaaatggacaaaatttagttttatcttgtggtctggaaatacaccctaaattattgggtcaagttagtgaaaactgttaaattgattatgaacgtaggcacattacttataaatccccttatgctaacttaaaacttgtgaatgtttagtgttatccagctataattcttctaaacatgtcttgtaatttttaagtttgcatgaaaataactccatcctgagtatactcatttcaataaattatttgtcctgagcatactgtaagaaatttagtaaagtactaattgaatttagtgattagactgtgattagactattacaaattcacagtgcttgtacaattcagatattattttgctttgaagtcaaatagaggaaccttaaataatttaaataaaaataattgtttttattaaagtttatacagcaagataataaattcactaatgtgaaatgttgatatagtatgtacaacttgtttcttaagttactaaaaatgtattttcctacctacataatgtcaatctctattgctcctaacacatgagtggctaaaattgcaaacttaatcacataaataatgagattaaagttaaaatgaaaaagtggtatgaggactattgtttgtgttaagtgaaattataccttgtaaaatttcatattatgagagcaatatgtaaatttcattgcaacaatggttattcaatttactgatgaaaatcagaagaatgttgaaaaattagtgcatttataataaatttaattattcataaaaaattaacattgatatatatattcataaggataaaagatatcaaaataattaaacaaatttcactttcttcttataaaagaaaataatttttatggtaactaattttagtagtgcatcagatcaacactattgggcacccagttatttggtggtacgctgagtgaaaatatgtagctttatctacattaccttggtttggacaactgaaaaatttgctaggaaacaaatattacaaaatatgttgttaacttttcaaagatgatcggtttagattgctttaacttgaaggacacttatattttgtatcacttttgtagcaaacacatgactcatcattgcccaaatcaattgcccaaatcaattcaaacatctcattgtagttcatcccatggcagaaaagtgtttatccacttagtaaaatggaaaacactagagcttcaggtttaatttgaaattttaacttcattaagaataaacttgacctgtttgttctagtaagtaaaaacactagatacgtaccaaaattgtcttttgaccctctcagggagtcaagttttgatttgcttgaatacaagcaagtcgagctatggtaatttgcaatgctgacaggaaagaagaacttgcttgaggcaaaatcatgaagtacaacttttcctctgcatccttttacctcatgtttgtaacatttcccctgttgttatttttacacatctggatgctcagaaaggcctccttaccacaataattgaaaggagtactttgtcaatagtcagaattgaatgagagataggttgttgggaatattcagggtgaatgtgtcttttctactttgactatatttaccattgactacagtaactcagcagaaagttagagggcagcatacatacattggtttatggatttaatgaaaatatccccaaccattacattacagacaattcatatatatgtcttgaaaatcttcttgacaatttgtgacaaattttctaaatgtttttccaaaaatagttggttcttgtaagtgattttgatatgactgattaccaaattatggtgggtaaagatgccacatgcaacagaaaatgtgtctaattatgtttgttttagagcttaagaaatgttaagaagagaagttacaactgcattaataggattttaatttttattcaaaatggacaacttatttattatgtacttctacacacagctaagcttatagatattttcatttaaagaaaaactatttgttcattttattagcagatatcaaatgcccttttgaaaattgagactgatttctaaaacaaaaaaaaagactttaggagttttaattatttttaatatattgcttctttattaaaaaaagatacaatccttcaatgtcattcaacagtattaattgttaaagtgtgggatatagtttacattaccgagtttattttctaagggtagtgaataactcctgacaactactgatatcgtcacatggtcctttagtgaccaaaaatgcacagttgtaagaatgcaagtgttacttgtattgaaaaccggattacattaaaggatggacaattatgataaaggatctgagataattggacaattatgataaaggatctgagataattattctaactttttggaactatactttcactcattgatgaagtaagttacaacgtggaataacaaagtttaagtgtggcagaaaatacatacatatgtttaaaagtagggaaaattttatcaattattaaagatggaaaaaataggactatgtcaaatagttaaacaaatgtggggtattttatggagaaaagaggcatgtactaccttaaacattttccaattggaacatactatagacaaaactgacagattattattcaatgagaaacctgactcagatgaagttacaaaaaaagtactttttaaatgtctagtttctaatagagttagagctttgttgattgagatatgtggaactgccacatatctctgtgccatacttttggtaccttcataataaacggtaaagtgagggaaagggtggaagagacaaatcctacgtctcttccagaacttcgagtgcactataaattaaatatttaaaatatttttgcaatagttagctttcaattatgaacactctcagcctctattgctttatatatgcatttattttggtaatttttatacatcaaaactataattacctgtatttgggcagaatgatttaggttatgccagctattgtggttaaagctgtagtaacttacagtacattgaaattatagactaaggttctgaatattggtaactcactgttgttgtgcacctttaaacaactcttaaataaagtaatgattctctttatattaaatttaatgtatgtgtgcctcatggaaatttgtattttatagaaaaatattgaatattttattattatgtctttggctcacctactttaaggagatggctacttagggtactttttaatccaatataatgtgaaaatttgatcatgctatattcttaatttaattgtacttctatggtcatatacaatttacctatcactttctcacataatcaatttaactttttggtaaatcttctaagagaccgtctagacagagtgaaatgaaagctgaaacaacagtcaaatcaaaaactgctttggtctcaaatccatgtttttcagaaaagatattcagatccagttatctggcaaatggtctcaaacatacatttcaatttcaatgttaaaaataggatattaaacatctcagaaaatattgggattattgaagcaaattctaccctggacttggagtaaatgtgatgaacagattaatgaggtggaagggactagaactttgggaaagtgcaaccttgttatcttaatatttttatagcttagaaagagaatgctatgcaactcatattttgatcttttaatgttaaagaattcaaataaaaaccataaacctgaaactctaaaagaaaaattctgttttgagagagatggcctcctctagtacacttttaataaatttaaagtatctaaaaggatgcacaaagatctctaatgtgctgtgattttcaaaggatgtcatgtataaaagatttgagtgagaacatgaaagcaaaagcaagttcagaagaggaacacaaccaggaggacagtgtgtcaggaaaatccaagaataagtggaggtgtaaaggctaaaaaataatgcaaatggtgcatatccttctgtctttctctcatacacacagacacacttacacaacacatatacaaatacatacatgtatatatgtatatatatacacaaatatacacacatattcacataatattcaagtatgtatacatatatacacatatgtacatacacatatgtatatatacatacacacagattgagagattaaccatatgtagatacacacatgcacatatgcaataatgaaatcatttcaaagcatgccaaaaagtaataaaagatatatcctctgtttgggataaataaaaaaaaagtttaaaagcaaacaaaaaataaatggcaataactaatcacattgaattttgttatggcctttttcttcctaaaaagaataaccccaatctgaacaaagaaattcaaagtaatggaaaactcaacaatgaaactcaaagtagactagcagataagatacctatttcaaacatcagtgccaaggtaatttataggtcagtgcattgataacttttgccaatgatagaaaagatgccagagaaccggatcctgacattaaaaaaaaaaagtaaaaagattctgaagactgcatttctgagcttaaggtagattctaaacaacatcttagaaactaggaaatgactttatgtttctttgtttttcaatgtaaatggatcaagatttcttaaaacagaaatgaatattattatttgtgatgagagcactaggggcaattttgatatttttgataaggtttctagagtaataaattagaatgacaggaatatatattgattttaggaaagtgtctgtataattccacatgatattctctggacaaaatatgaaaaggtaggctgaataacatttttaaagggcagtaaattttataattgttattgattacaatgaaggcctctggtaatgttttccagggtcatatcctgttacatatacgtgacatggataaaaaggaaacaaatatttattgtgtgcctagtttatgttatctcaattccagctctacaaggagctacaaggtaaaattgctacctttaaaaacatatgaggtaaaattattcctattcacagatgtagaaactgagtttcaagaaggttaagtaaatttcctcatattgggaggctggtaatgcagaactgggtgtcaaaatcaagtctgtatgaaccttctgttttgtctcccatgaagacaaaaggcatgcatataaaatttgttgaaacacaaagctgaggaggcataataagacgtggaatgacagaagcaagatctagaaagtttgggatcatgaatcaaaagaaacaggataaaattatcctaaaattaatattaaatcttacaagaaaccccccaaaatcagttgaatttgtacaaaacggtaaatcattttatcagtagatcccataataaatattataaagtttaagtgtgagctctattactcagtaatatgatgccattactgtgttgatggatgtattgtcaaggaaaaagaagagaattacacactgtttccttcaattgttagatggcactggatgtagtgttttcaatgttaatcctggtatcatgttctttgccataaacttgttgacaaattggcaaatactgacatgaaatatgccaatatttgagcatctaaaaatgtaggtactttccataccacatcatatattacaatttgaaaatgtttgtttcattttttatataattattatacagaacagtttttctatgatagcattataaaaattcccagagaatactggcccagtaagaaatggaatgttcacaactcatagtgtagctatatgaaagaaatagatctaaacgacaggttggtttccaaattatattttcatacctggaaaatatctactttataaatagcacaaagttatagttttcaatgaatatgaaaaagttcttgcattaacatattttatgtatcttttatattgacatttgtgattgccactaaaatgtgtattttctaaatttcattgtgcttttacaagatacttttttctttgatgtccataactgctgaaaaggctcccctaaggagaattttaagactaagtaaggtttttagtgagcttaaattatacaattctgaggcattatttaaggtgcatactgtattttttgcttgaaacctgtcagcattttatttgtatggcaattaaatgactcagccattcatgtctcatgccagtctttttcaattgttatttttaacaaagaaaattatatatatatgtatatatatattatatatatgtatatatgtattatatatgtatatatatataaacttacagcaaaaatgtttaaaaatagcaaatagtttgagtatagttaaacctaataactgtacttttgtttctatgcctctgagacaagattactagacccttattcaaagtttctaaatataggaaatagaacattgggccatgctaaaaaaattgttcagattttcttttgaaagagaatagttatttttcctcctgacctctaatgaagatgctttatttgtcaaggtgttttccttagaaaattgacccagtgtcaactgtaaagaaaacatagaggatccttggatgattgaccaacttatccaaacacaggtttagtaaagagaggatataaagataaaatgtgaaatgacctctctgagtcacatttgttttcataatttcctagcaaacatccaacttcactgctaccctcagcaatgtttcttgaaacatttttaagacattgatagacaccaatagctgatctttagaaagccattcccagaagaatatgtaaggggttacaactcatttcagggagtctgcctagctcttgatattacatgtctttggcatacaattgtgtaccttttatcattgacagtgaagaaaataatgccatttgtaacttctgagatatacacacaatactatcaactagccggttaataaaagataagaaaaataaagaaaatagaacatttttaggtgtctggcaagtatcctctaaatcaaggtaaagataataatttagtggcagtgttcatattttcctatgactgtaagatttaggtgcctcacaaaatattaatatttagcctcttatgaaaggttcgtttttcttctaacactttagtagctgaatacaaagaaaatacacaacagctgtttataaatgaaataaaaagtttccattttttatctgagtttctcatttatttgcagagaacgaataaaataaaaatatcctagtgttgtttgcaccacagcataccagtaaatcttaaggattgtgtttcagtatgaaaaggaagagcaggaagatttcctcattctgtcttaccagcaaaagtctagccttcacacacacacacacacacacacacacacacacacacacacacacacacacacagagtcatctatatgaacacgtacttgagtttcttaaacatatatgaagcaccttccatttccctttataataaatcccttagtttttgctgttcattaaaaaacaaaaaggaagagacaagctcaggacattctgaaaaccaatgtctttaggacacactaaggtgtcctgaattactttaacggacacattgtaaagacacactctccaatccctattaggaaaagtttagtcaagtttgcttactatttgggtgcttataccaaaaaagcatcatttaggacattatttaggataatattatttatgcaggaattgtaccacctatttccagatggtataacttattatctgacaggcatgtagcaaatagaacacaaagcataaatctgtcaggagaaatcatacgagaaaaagagcattgtctggttatcagaatatcagatctctcattctggccttgctaggaaatagatctttgattctagaaaagtcaactaatttctatggttcttacttttctcctttataatatacccatttaaattccaaaaaggtatatgataaatcacaataatttcaatcacatggattttaatacaaaatgtataaaatcaatttccaaaaattttctgcatatactgaaaatgtctgtacgaatgagctaactactataggccttccctaatttattctattaaatgtgggtactcaatgtaacctgaaaatattgagcttaactcttctttttttttttcaaaagggaaacttgaaaaagactgcttcccccagaaaatttatcaacaataggtgctcaattaaatgtttttaaacaatgaacaatatcccctttcatataaataatcaggggagagatatttttaagtcttttttttctttttccatagtgtcacctacacaaaaaattatgtaaagacaccacttctatgaggaggtattcattgtagatgtacagaagtcaacggaaacttaagtttacagaaaaaataaaccagattatcattccacccaactgtatattcccacagatgcttaataaaagctatctgatgatataatgaattatcagttcttgaggaagtatatacagttggtgactatttttcaaaaatcatcatccaacaaatttttttcatttaaaatctttcatattaccctttcgacaatcagttgaaattttaaaactaagaacatttaaaaatataaatgaaagtagcattagctatagactgatattcaacttcagacgttaaaataaatacaagtgtgtattaagagtaaaattatgtcaacaatgtataaatgaaaactgccaatgtaattaatgtttcttttaacatatcccatccattgctttccctccaaaagacaaaggtagcaaaagacgaagcaggaagaactgcttcagaaactgaacatactgatttaattggctaagaagtccaaatgctaatactcctaataattagccattccttttgtgttttggtgacatatatcctcatacaatgtatatcaaatggaattttttgatttacacctgacatttcaaagtttccatttttgaattctcctagtcttaagtaagtagaacattgtctcctttgtttgctaggcataacgttttccccaacatctagggctccatgatgcaaaatatcattttgccgatcttctgttccagtatttactttaattttttttattataattggattttcaaatacaatcacaaaaacatctcctgttgaaggtggtttcccccaaaagtactcatcaacactactgtaagccttgcttgcttcataattttcaaacacattcatgttggtgtacagacttgcaggggggttatcaggaatgtcaaatgactcctcttcaaaatcatcatccttcagcttattctccgtccctttgtatgatgaataatagcccatgtgctgaaagagagatggtttaaaacggatcacatttttctgagccaacagaccacggaaatgagtcaatagccaatcacaaggcatttcttgataaaacattaataaaaaatgggccaaacgtgggagatcatgagaatgatagagtttaccaatgtagccaagcttagagaattcaagagttacccagtaagttccttctagggatgcaatgactttcttgatggcagttaagaaattttttgaacatcgaacatcatcttcaagcattacataatagtctgaagtattggcacaaaaattaagcagaaaagcataatctacattttgcttggaacgaaatttgactctatcttctggatcattgtaatttcttttaaggccatctaggattgggtaatactcctctggagcatgtataaccattaatcttcctgcaataatatggtgcgcaaatttctgtgtaatatcctggaccatggcatcacgccaggaagaattaaagtctgctaggtgaaccaccactgaaatttccttcagctcttcatagctggattgctcaaaaattgacttaattgtctcaagtaaatagtttcctttttttcgctttactgaagaaagtccaattgtaagataccgctttctttgtaaaggtgtggcagctaggtagcgataggtgacatttatggctcctgagaaattagataaatccttgaaagtatgaacatagcgttctgaattcagttgatgtgtggatgtttcccttataagttgtttgtctccttccagaacatagctatcttcaatgtacaagttcataaaaaggagaaaaatgacaagaactcccaagaatgacactgtagaacgttttctcaggcatctcattttatcaagtatttcaaaaatatgtttcatttgatgaaatttaaacattctcttcttaagaaagacgctgtcataatctgtgctgtacagaaaccgttgatacccttctatcttgacaaaagccccagatttctccccaggcttaaatccagtgggagaggaggataatgggctaagctggttgcagcagcttgctgccagagggac

SEQ ID NO: 13486 - RNA, 22992 nt, Homo sapiens
  source 1..22992: mol_type = other RNA
gctgggattacaggcatgagccaccacgcctggccagtttttaaagtatttcatacagtgtaactaggcagtcagaaatacctgtatctcaaattcatttaacttttcaatgaatcaatcttcttattttctcagacatataaattatcataatactttacattgagtctctatggttgactatatgctgtgaaggaaggacataaatacatgtgaggaaacaattattgatatttttaaactaactagaaagcaccaagttatttgttaaataaacaaagttaattttatctacctgttcagtaagtgttggcaactatgaattaatctttgacaaattcacttacaactagcaattttaaagacttaaagtttaatttttattattaaaagggtatgattatttttactaaaattaataaaaagattaactgttactaaattaaagctccttcaaaaacataaatgtattctttagagagttaaaaaaagtagcaataaaatacatttttaatttagttaagcttacttaactaatgatcaaatagattaagttgtataaaattttacaaactttatatttttgcatacacttatcttcctggcatttttgaaataaaaaaaatacaagtgcatagggcagaggaggcgattcagttacttctgctatgttattaaatctctggtaaccactatacaatacaatacaatacaatacaatacaatacaatacaatacaatacaatacaatacaatacatgtagactcagcatccaaactttattttaccttcaagttctacctgataaagtggtggaataaagatggtattttccataactgtttaataataatcacatgttttatacccattgctttgaagaagaaaccttaagcaactagaaatgtcaatctaaaaggcagaaaagctggaaaaatctcatgaagactagaagatttacactcataagatcatgtaaatttatttggatatgctgaaaaaagagggggtataaaatctaaagtttggtaaatctttgctttacagggcttcaagttatagatttttcttttttccttttctcttcccctttctctctctttctcttttttatttttgccatttcttctcaggagcccctgcaatttcaaaccttggaattgaattggatttgaggaggaaaacccatattcagctttaattcaaatgaattttactactttagacaaaggtacaacactctattcaaaaaagttattgaaatcacatctttaaatctgacccagccacttgaataaataagttgtgttgtagtttctcagagcaaccgccgctcatctttcactcaccttaacaatttctcacttttttctgctttttttttttttttattttctgcttgctgaaatcgagatcaatattcattgttttcttctgggttaactcttttttatgttaactgaatcaattttggctttgtttctttatgaaattacttttagataaagtattgatattgtcatttatcaattttattatatgtcttttgcttattaaaggattaaaatccacctctaaacttatttagatcaaggtcagtttttttactcctctgtagaactgtgaagataatatcctattctccttttcttatggttttattgtgaagatctgtgcaaatagctatataaaatgcaattcggtattaaagaaaattgttgcacggactacattgattagagtctaatttttggaaagtatacttcgccttttcagtaattttatttttcggtctatggtgcccacattgtgtcaccagccagccgtatgcagacttacaaaggactacccactaagaataaaaacatgatacaacttgaagaaattttcatcaaacgtctttgtcttatccccttgttatacagacaaagatgacaagggccgaaaaggaagtgattttctcattgaataagagaatccgaactggcatcgaggatatctaattttgggatgaaaattgagagaagacagaatttcaagtctgaattatgacttcactactgtgtcgtcattggtagaataaggataacaatacttatcacacagatttgtggtctgaatcacatgagagacatagatgaaaaatgtaaaacaacaattagcatgtgacatgctctcagcaaatcaattaatccttcattctttttttctccccttactcctttgattttcagactaatttggatcatgattattggcctgtgtcccacccattattcacatatagaatgggttgcattatcctctccttggaaatatctttcaaagtgggtaatgagaaaactactttgaagactgtgctgaaggaaatgatggcatgaacaactctagataatttttgtttatttggatataacgtgaatgggcccataccataaactcctattaagctgaatcaccaaaaaaaaatttgatatgaaagtcatacattgaaaaaattcactcttaccactgatttgattgatactgagcctgtaaatatttatttatatgatgtttggcactttattttataaaactaccctttacttaaaataaatcattgtattcacataactttccagggcactatgcatttttaaacaagacagtcaacttactatttaaaaaacaaagtcagtcacctaaatgactttctgactataaatttgaaaacaatattctccttgtaatatatgtgccaccagggcaagaattacaaattgggagcaggtaagaaaattgttgttgactctcattagtattctaattctccttcagtcagatttataaagtatgacctatagcatccaactccatcattttccagtcattcttgagactgtcaactctatgggcattgtttagcagcctcgaaacactgaactttttacagtcttattggagagaaaaacacattaaatgatcaaataatcttttatgagctcagaaaaaaatgcctaacatgaacatttaagcatcttctgtttctgtgattcccatttttggagagtaaaaatttaagaaacaaagggaatgtgtctggggatggtactaataatattgagattttacaatttaggttataatcaagataattatgtatatatataaaattatatatggtatagtttcaacttctaatcttttatcatcctctaccacataattcctcctatattctctttttctgactgtggcctaatacctcaagaatattgtatatgcttgtcactatataaacttcaccctaaggaaatttccatgtcagatacaataagagcaacggaagaaaatgtatcaaaacacatctccaatttatttgaatttttctggcctaaccttgttggcatgagagttcccactttgtattataataggcaaattgatacacacttttcatttattctaaataatagattagcatagtcaggaggcttggattggcagctattaaatacaatttgaagccgtgggattttattaggattctaaggttattctgtgacgatggaacttaatgatgtaagagttaattacccattgtcaaaaatcattgcccatcaaagcagtgagactgtgtgctatgtccagttttattcatttcttttgtgtatctgaatggaacatgtggtaaacacaacagtagaatatacctacagtccccttagaaactcttaaatcttcaatttataaaagtcatcctaagacgttaaaaataacttacgaaaggatagattccaatgtcagtgggtgagatgtgctctagctagtgtgcacgaaagagaacatggagttagaataattattgtaggactgtagattgtcatctcaagatcagtgtcaaatacattcattcatgtagtattttcacatgcattctggtctaaatatcccaacatatctttcgttttgagatctgcagaacaaagtcaatgtctgaatttagagactaatttgaccattttgattcaaatgtctaaaggctaaaccagagcaatttacaacatccaatgaagtaaaattatataattaattatataattatataattatataaaattttataattaattataaaataaaatattaacaataattgaacattgtttacttttttatcctcacaacaattcaacatgatatgtatggttattactaaatgtataatacatttagtaatgtgatttgacaaatcacatttgtcaaataaggaatggctgaattaaatgattgaatgaaggagtgaaggatgtagattgtttaagtacattcaacttgtaatgaactgtaaacttcacccataacattattaatatatcagtgctatcaactacattttacataggatgaaaaaaatcattatttttattaatcccaagatattttatttcattatataaatgaaatattttatctgttataaagacctttatttttgttccactcattaaataacatggtaagactgttgtgtaattgactgaatagttaagtctaaatgggtaaatagctgtttatgttagtattgcagggtagctatttgataatgaaatatacttttcttacctacttgcaaaaaaaattacataaacaagtatttcctagagttcaaacactgatctttttaagtggcaaattgtccaaaagaatttaattaatataaacaataaattcacttaaacaactatttacatgcaaaagtaatatttttattgcccatttggaaaatagttttgctttctggtttataaggaacttttactagtttaattacttgggtgctttaaatgttttttggaggctattacaaaatcacatcctaaaattttaaaatggaaaaattataataattgaatttttaattcctcataaatattttaaaagtacacattgttccatggcttttgcctttagaataaatacaacatttttatgtagaaatatattcttgaaatgtaactagcacatagtcagtgtttcttaaccattttggggtcctgaaactttttgataatgatgaaagcacagagatgctatcaagaaaaatttacccacataggaacacacacacatacacacagacacacacagagtttgcttataagctcaggaagcttaaagatctgctaaagattatgcttgggtttgccatgaatcataaataccaagtcaaatacctttgaatttgattcttaacaaatctttgtggctgagaaaccatgagatttcattctggcatgtccccagaatgtaattatcaatgaacaatagccattgaaaaaatctgaacagatattattgaggctcaaggttgtttaatggcacagataatataattcaaatcatgaccccagggctgatgaagtcttgttgtaacgtgtaaatggggtgggtgatgggagagagaaaacaaaataattatttatgttaaatcatacataaacagtaaagccaacacaataagtaaaataagagaaagtagaatgcttgggaggtcatatgtttcaaatgtatgcatacacaaaagagtaagcaacaggatacttcaagagtaaaatgggaaaaaatcatattgggtaaatagtatcaccccaaagtgatagtcaaaagtacctatgtttgcctagttctcagattacaactatgatgataatttagataaacaagcagaaaacaaaactatagaaaaaagtcaaagtgacataaaacaattactggtgtttcaacagaaataaacccaacatcaggatttatcaaatatatgaaaaattatgaaagattataaaacaccaatgattagattatgttataaagacactatgaagagatactaaatgatattcttttcatctgtggttactgctaaaaaattctttcatagaaattcttggattttgaaattagtttaattccaaaatattttctttattttgcaaaaatgtaagacaaatgtataggatatttttctctgttgttatgcaaggatttattatcacattggccacagaacacatagaatgttagttttgtagaaaattttagagattttaataccaggatgaaataatagtatcattctatttcaggttcttaagcaacattcctaagactagaaccttatcttgaaaaattatgattttaaacttaagggaattcaggtaaaggaaattgactaggttaaggcaaatacatcatgtttactggtaaagataacattatttaaggaaggtaagatactcttatcctacatatacgccagaaaaattgcttctcctctgaaaactaccattatttttgccaaatattgtagcttagttttaagtttttctcggctgtttcctctgacagttctgtggtaaagaagaaacattataggaagcatttttttttcctacagagtctgccatatggagaagtagaatgagaggccacctaggtaatgtgatttattaaaagttctccatcccaaaatatatgtcccatctgtgggctaatgtctgaaagtcctatgattaaactcacttttatgtaagatagtgaggccccagagagccctcgagaaatgcaaataaactattactgacctcccttggattatgatgaaaaccgtggagtctttctattctctgtcaaatgtggaggtcatggatccttcttggcacctaagattaaaactcatagaatgtgctttaacttctgtaggcacatttcctttccaattagagtgaggtgttgaatatttatttatttgtttatttttattatactttaagttttagggtacatgtgcataacgtgcaggtttgttacatatgtatacatgtgccatgttggtgttctgcatcttaagagaagactatttataaaatttattgcttgtaagatttgttttttgttctcttactattatgaaaatcacgaacttgggaataaggacactctgggcccggcgcggtggctcacgcatgtaatcccagcactttgtgaggccgaggcgggaggatcacgaggtcaggagatcgagagcatcctggctaacaaggtgaaaccccgtctctactaaaaatacaaaaaattagccgggcgtggtggcgggcgcctgtactcccagctactcgggaggctgaggcaggagaatggcgtgaccccaggaggtggaacttgcagtgagcggagatagtgccactgcagtccggcctgggcaaaagagtgagactctgtctcaaaaaaaaaaaaaaaaaaaaaaaaggacactctgaacaattgaacaagactacgctgaaaggcagagaagaagtaattatgaacaaactgttcatgaagtgatcaattgaatttgaaacagaacttttcctagcttctaaatgattagaaatttcagctttggtttaacttaaaaacttagaattgtcaattctgtccaagtctctgagtcatgtacagaactcaaattattacatcatttttttacttatctgtattatttctccatttaaaagtggacaaatttttatactatatcctaataatgatacaaggtgacttgtaggactctggatagaaagagatggcccaggatacagagggcactccttaaatagctgccaaataaatgacattaaaaaatgtataaaaaggtatgttaagtaattaaaagtgtcaggcattattttcctattatgagacattttatattatggttatttactgtaattgcatccaaaataattcataaaacatttatttttgtactattaaaaatctaaacaataataaccagatggaggaaaatgataccatctgatttaattattaacttgaaggtcagtttctacaacttattctcatttatgtttatctgatttggccacagtttcttactttctcatattttgctaagcttgtggatgaagccgcatgtctcttttttttttaacctggcatataacactgtcactctatttaattattacccatcatctacctactttgaaactttggaggttttataaaaattatgagtatttaatcaaagttgtctctttatcatttgccagtgaaaatataaaacctggctgttttattctattgtgcactctaattacataaccaaaatctttttaaaaattcttagttcttttagaaataccatttgacccagccatcccattactgggtatatacccaaaggattataaatcatgcttctataaagacacatgcacacgtatgtttattgcggcactattcacaatagcaaagacttggaaccaatccaaatgtccaacaatgatagactggattaagaaaatgtggcacatatacaccatggaatactatgcagccataaaaaatgatgagttcatgtcctttgtagggacatggatgaagctggaaaccatcattctcagcaaactattgcaacgacaaaaaaaccaaacactgcatgttctcataggtgggaactgaacattgagaacacatagacacaggaaggggaacatcacacactgggcctgttgtggggtcaggggaggggggagggatagcattaggagatatacctaatgttaaatgacgagttaatgggtgcagcacaccaacatggcacaggtatacatatgtaacaaacctgcaagttgtgcacatgtaccctaaaacttaaagtataataataaaaaaattcttagttatttgaaaatagtttttttgaattcacaaacttgcaggatgaaaaaagttattagttcctgaagatataacattgatttgtctttttcttatttgatatcagctagcagtaaaattgtgaacaaatctggtaaatcttttggtgttgcaggttcataatcagttaattgagtgtattcactataaattgctttaattaagtgatgtttgcctaagaacaagtttcatttcatctcatgaaaaaaatgttactttttgtattaatcagtggaatgtttaaagaaaaaactggttatcttgaagctgtcaaataattataagaaatctctatacattacgttttaaaatacataaaacccataaattcaagcttattagttttcattttcagcaaggtttatacagagaaaataagtaatacaaattagttttccagaaaatctaattttatgcagataaaatctgaaaatcatataagtccaagatgaaactgatctcaaattattattttgaggtgtatccatttatttaaaaaagcctcattttagctagcaacactatgtagaaaaatattttaaataagacagagcattaaaataatgtattcattgatctcataaagaatagatgatcagattttttaaaagtgattttaattaaatggacatgtttctctttagccagaaatgactgagaaattttgagttggaattgatataggggaatccttggaactatgtgtgaatatgtgtgtgtgaattatctgtgtatatttacataatttacactattcacagtccttgtttttcttgactcaaatagctatctcaagtttcgtacactttttagatctctatgtaaatacattatttcatttgtggaaatatattgaggcctatatcaataacctcaaaccttttaaacacttagagcaagtcaatatgacttgttctgtttcagctatctgaaatttaaaaatttgacaaatttttaaagtacccagttcttggaaaaagaaaaacaaataaattggagatttggatcatatgggctatgactaaatgagacaaggcatacatgctgacatttgaaggatttatgaaaaaaagtccactgtggaaaactgatagtttttctccttctttcttgaatatgtttagttaattttgtggaaagaggaaggcagctcagtttacaaacagcagtgggttgaaggcaatgctgtttatattcttgaatttcaatatctacaaagatgtcatcattagattttatgtgttaaaaagtggatttatagtctctaattaataaggtgcatatgtcaagactcaggaaaacagatcacttacgtagttctccaaaaacgagagtcccagattcaataggaaggcatgcagagtgttctctataaacccagcaaaaccataaaaattgactggaacttttatttttcagtacaacaataatagtattgaaatacctaaaaagggcaggaaacaacacagaataatctacgcttgtcatcatgttttctaatctataatctttcaaactggataaatgggaagttttggaattttactgtggtacagtcttagttgctccgtggttgtcaaatctgtctgcacattaggatcacttaggaagaattttaaaagtatgctgatgcctggaaactccagaacaattatgataactctgagcatggagctcaggaatgggtgaaattcttccccagagatgttaatgaacagccagacttaaaaactagtaatttagacaagtgtgagcagaggttaataatgttgagatgaactgggcttaatatttcactaacaaggtcagagttttgatacatcacttaactcaaactttgagattcttcatcactgaagtagcaataataatagtcatttctgttttaatacttcatagacttgtaaggatgtaatgtagtgtttctaaaaggagtgaatggacaatctgcatcagtgttaactaaaatacattgaaagtgccaattcctagatctatcctagatttacagggaagaattcagtagtctgaaacacacattttcaatatattgaaaagatgattcttttgcatgatgacttgttataatcattactttcataggtaatggaagtaccgattaggagagtaccaaatacatattaaacactcagttcatgtaagctataggccaataaacacaactttggggtttactgatgttttccaacatccgaaataatagctgaaatttagaaacatagttaatcacacaaaaaatgttgcatacatactgtctaactaccagtttggtatgtttggggctggtgttatgaaagactattatatgattaatacaaagttataatttttggagtcttttagtgtacccagagcccatgagtttttattttctttttggaataacagaaattaggttgtggttcagtggaattacagaagcaagtgttttagatgttcaagtttaaaaaatgagaaaaaaatgttttacatgaagaaactaattatttaaattcatttttcaactatttaatgttattttaatatagtcatatcatccagaaaatcccatcttagacaaatgggttttcaataaattattattatagttaggaggcaatgtataatagtgataaggggcatagattttgaattacacaaacctgaaatccaatgctctctctttcatttattagttatgtgaccttggacaagttagtaaaaccctatttttcatatgctctttagcttttttaatacctcttaccttatatggttgtttaatctattaaatagacagtgaaatgcacatgaaatcttcacacagtgtctcatagttgcttggaacatatttatgtagtaagcattgttcttggctgagcttacattaagtgatctgtaaattagaagttatttgttatatttgtttcgtttccttattgccctagatgccttttctctggacctagataatttagtctcactctgtggcctttacccttcaataaatatggattattaatataatttagctacataattcctaaggaaatattaattcataaagattgttaaattgaactgaatatctttgctaagtcacaggcattgattaaattagataaaattgtcattttccattgattttgtttatataaataatattgaattatttatattcttatttagtctagtagattgacaggcagttttattaagaaatgaatcaaatggtaaattttgaatcatctggtaaaaatggacaaaatttagttttatcttgtggtctggaaatacaccctaaattattgggtcaagttagtgaaaactgttaaattgattatgaacgtaggcacattacttataaatccccttatgctaacttaaaacttgtgaatgtttagtgttatccagctataattcttctaaacatgtcttgtaatttttaagtttgcatgaaaataactccatcctgagtatactcatttcaataaattatttgtcctgagcatactgtaagaaatttagtaaagtactaattgaatttagtgattagactgtgattagactattacaaattcacagtgcttgtacaattcagatattattttgctttgaagtcaaatagaggaaccttaaataatttaaataaaaataattgtttttattaaagtttatacagcaagataataaattcactaatgtgaaatgttgatatagtatgtacaacttgtttcttaagttactaaaaatgtattttcctacctacataatgtcaatctctattgctcctaacacatgagtggctaaaattgcaaacttaatcacataaataatgagattaaagttaaaatgaaaaagtggtatgaggactattgtttgtgttaagtgaaattataccttgtaaaatttcatattatgagagcaatatgtaaatttcattgcaacaatggttattcaatttactgatgaaaatcagaagaatgttgaaaaattagtgcatttataataaatttaattattcataaaaaattaacattgatatatatattcataaggataaaagatatcaaaataattaaacaaatttcactttcttcttataaaagaaaataatttttatggtaactaattttagtagtgcatcagatcaacactattgggcacccagttatttggtggtacgctgagtgaaaatatgtagctttatctacattaccttggtttggacaactgaaaaatttgctaggaaacaaatattacaaaatatgttgttaacttttcaaagatgatcggtttagattgctttaacttgaaggacacttatattttgtatcacttttgtagcaaacacatgactcatcattgcccaaatcaattgcccaaatcaattcaaacatctcattgtagttcatcccatggcagaaaagtgtttatccacttagtaaaatggaaaacactagagcttcaggtttaatttgaaattttaacttcattaagaataaacttgacctgtttgttctagtaagtaaaaacactagatacgtaccaaaattgtcttttgaccctctcagggagtcaagttttgatttgcttgaatacaagcaagtcgagctatggtaatttgcaatgctgacaggaaagaagaacttgcttgaggcaaaatcatgaagtacaacttttcctctgcatccttttacctcatgtttgtaacatttcccctgttgttatttttacacatctggatgctcagaaaggcctccttaccacaataattgaaaggagtactttgtcaatagtcagaattgaatgagagataggttgttgggaatattcagggtgaatgtgtcttttctactttgactatatttaccattgactacagtaactcagcagaaagttagagggcagcatacatacattggtttatggatttaatgaaaatatccccaaccattacattacagacaattcatatatatgtcttgaaaatcttcttgacaatttgtgacaaattttctaaatgtttttccaaaaatagttggttcttgtaagtgattttgatatgactgattaccaaattatggtgggtaaagatgccacatgcaacagaaaatgtgtctaattatgtttgttttagagcttaagaaatgttaagaagagaagttacaactgcattaataggattttaatttttattcaaaatggacaacttatttattatgtacttctacacacagctaagcttatagatattttcatttaaagaaaaactatttgttcattttattagcagatatcaaatgcccttttgaaaattgagactgatttctaaaacaaaaaaaaagactttaggagttttaattatttttaatatattgcttctttattaaaaaaagatacaatccttcaatgtcattcaacagtattaattgttaaagtgtgggatatagtttacattaccgagtttattttctaagggtagtgaataactcctgacaactactgatatcgtcacatggtcctttagtgaccaaaaatgcacagttgtaagaatgcaagtgttacttgtattgaaaaccggattacattaaaggatggacaattatgataaaggatctgagataattggacaattatgataaaggatctgagataattattctaactttttggaactatactttcactcattgatgaagtaagttacaacgtggaataacaaagtttaagtgtggcagaaaatacatacatatgtttaaaagtagggaaaattttatcaattattaaagatggaaaaaataggactatgtcaaatagttaaacaaatgtggggtattttatggagaaaagaggcatgtactaccttaaacattttccaattggaacatactatagacaaaactgacagattattattcaatgagaaacctgactcagatgaagttacaaaaaaagtactttttaaatgtctagtttctaatagagttagagctttgttgattgagatatgtggaactgccacatatctctgtgccatacttttggtaccttcataataaacggtaaagtgagggaaagggtggaagagacaaatcctacgtctcttccagaacttcgagtgcactataaattaaatatttaaaatatttttgcaatagttagctttcaattatgaacactctcagcctctattgctttatatatgcatttattttggtaatttttatacatcaaaactataattacctgtatttgggcagaatgatttaggttatgccagctattgtggttaaagctgtagtaacttacagtacattgaaattatagactaaggttctgaatattggtaactcactgttgttgtgcacctttaaacaactcttaaataaagtaatgattctctttatattaaatttaatgtatgtgtgcctcatggaaatttgtattttatagaaaaatattgaatattttattattatgtctttggctcacctactttaaggagatggctacttagggtactttttaatccaatataatgtgaaaatttgatcatgctatattcttaatttaattgtacttctatggtcatatacaatttacctatcactttctcacataatcaatttaactttttggtaaatcttctaagagaccgtctagacagagtgaaatgaaagctgaaacaacagtcaaatcaaaaactgctttggtctcaaatccatgtttttcagaaaagatattcagatccagttatctggcaaatggtctcaaacatacatttcaatttcaatgttaaaaataggatattaaacatctcagaaaatattgggattattgaagcaaattctaccctggacttggagtaaatgtgatgaacagattaatgaggtggaagggactagaactttgggaaagtgcaaccttgttatcttaatatttttatagcttagaaagagaatgctatgcaactcatattttgatcttttaatgttaaagaattcaaataaaaaccataaacctgaaactctaaaagaaaaattctgttttgagagagatggcctcctctagtacacttttaataaatttaaagtatctaaaaggatgcacaaagatctctaatgtgctgtgattttcaaaggatgtcatgtataaaagatttgagtgagaacatgaaagcaaaagcaagttcagaagaggaacacaaccaggaggacagtgtgtcaggaaaatccaagaataagtggaggtgtaaaggctaaaaaataatgcaaatggtgcatatccttctgtctttctctcatacacacagacacacttacacaacacatatacaaatacatacatgtatatatgtatatatatacacaaatatacacacatattcacataatattcaagtatgtatacatatatacacatatgtacatacacatatgtatatatacatacacacagattgagagattaaccatatgtagatacacacatgcacatatgcaataatgaaatcatttcaaagcatgccaaaaagtaataaaagatatatcctctgtttgggataaataaaaaaaaagtttaaaagcaaacaaaaaataaatggcaataactaatcacattgaattttgttatggcctttttcttcctaaaaagaataaccccaatctgaacaaagaaattcaaagtaatggaaaactcaacaatgaaactcaaagtagactagcagataagatacctatttcaaacatcagtgccaaggtaatttataggtcagtgcattgataacttttgccaatgatagaaaagatgccagagaaccggatcctgacattaaaaaaaaaaagtaaaaagattctgaagactgcatttctgagcttaaggtagattctaaacaacatcttagaaactaggaaatgactttatgtttctttgtttttcaatgtaaatggatcaagatttcttaaaacagaaatgaatattattatttgtgatgagagcactaggggcaattttgatatttttgataaggtttctagagtaataaattagaatgacaggaatatatattgattttaggaaagtgtctgtataattccacatgatattctctggacaaaatatgaaaaggtaggctgaataacatttttaaagggcagtaaattttataattgttattgattacaatgaaggcctctggtaatgttttccagggtcatatcctgttacatatacgtgacatggataaaaaggaaacaaatatttattgtgtgcctagtttatgttatctcaattccagctctacaaggagctacaaggtaaaattgctacctttaaaaacatatgaggtaaaattattcctattcacagatgtagaaactgagtttcaagaaggttaagtaaatttcctcatattgggaggctggtaatgcagaactgggtgtcaaaatcaagtctgtatgaaccttctgttttgtctcccatgaagacaaaaggcatgcatataaaatttgttgaaacacaaagctgaggaggcataataagacgtggaatgacagaagcaagatctagaaagtttgggatcatgaatcaaaagaaacaggataaaattatcctaaaattaatattaaatcttacaagaaaccccccaaaatcagttgaatttgtacaaaacggtaaatcattttatcagtagatcccataataaatattataaagtttaagtgtgagctctattactcagtaatatgatgccattactgtgttgatggatgtattgtcaaggaaaaagaagagaattacacactgtttccttcaattgttagatggcactggatgtagtgttttcaatgttaatcctggtatcatgttctttgccataaacttgttgacaaattggcaaatactgacatgaaatatgccaatatttgagcatctaaaaatgtaggtactttccataccacatcatatattacaatttgaaaatgtttgtttcattttttatataattattatacagaacagtttttctatgatagcattataaaaattcccagagaatactggcccagtaagaaatggaatgttcacaactcatagtgtagctatatgaaagaaatagatctaaacgacaggttggtttccaaattatattttcatacctggaaaatatctactttataaatagcacaaagttatagttttcaatgaatatgaaaaagttcttgcattaacatattttatgtatcttttatattgacatttgtgattgccactaaaatgtgtattttctaaatttcattgtgcttttacaagatacttttttctttgatgtccataactgctgaaaaggctcccctaaggagaattttaagactaagtaaggtttttagtgagcttaaattatacaattctgaggcattatttaaggtgcatactgtattttttgcttgaaacctgtcagcattttatttgtatggcaattaaatgactcagccattcatgtctcatgccagtctttttcaattgttatttttaacaaagaaaattatatatatatgtatatatatattatatatatgtatatatgtattatatatgtatatatatataaacttacagcaaaaatgtttaaaaatagcaaatagtttgagtatagttaaacctaataactgtacttttgtttctatgcctctgagacaagattactagacccttattcaaagtttctaaatataggaaatagaacattgggccatgctaaaaaaattgttcagattttcttttgaaagagaatagttatttttcctcctgacctctaatgaagatgctttatttgtcaaggtgttttccttagaaaattgacccagtgtcaactgtaaagaaaacatagaggatccttggatgattgaccaacttatccaaacacaggtttagtaaagagaggatataaagataaaatgtgaaatgacctctctgagtcacatttgttttcataatttcctagcaaacatccaacttcactgctaccctcagcaatgtttcttgaaacatttttaagacattgatagacaccaatagctgatctttagaaagccattcccagaagaatatgtaaggggttacaactcatttcagggagtctgcctagctcttgatattacatgtctttggcatacaattgtgtaccttttatcattgacagtgaagaaaataatgccatttgtaacttctgagatatacacacaatactatcaactagccggttaataaaagataagaaaaataaagaaaatagaacatttttaggtgtctggcaagtatcctctaaatcaaggtaaagataataatttagtggcagtgttcatattttcctatgactgtaagatttaggtgcctcacaaaatattaatatttagcctcttatgaaaggttcgtttttcttctaacactttagtagctgaatacaaagaaaatacacaacagctgtttataaatgaaataaaaagtttccattttttatctgagtttctcatttatttgcagagaacgaataaaataaaaatatcctagtgttgtttgcaccacagcataccagtaaatcttaaggattgtgtttcagtatgaaaaggaagagcaggaagatttcctcattctgtcttaccagcaaaagtctagccttcacacacacacacacacacacacacacacacacacacacacacacacacacacagagtcatctatatgaacacgtacttgagtttcttaaacatatatgaagcaccttccatttccctttataataaatcccttagtttttgctgttcattaaaaaacaaaaaggaagagacaagctcaggacattctgaaaaccaatgtctttaggacacactaaggtgtcctgaattactttaacggacacattgtaaagacacactctccaatccctattaggaaaagtttagtcaagtttgcttactatttgggtgcttataccaaaaaagcatcatttaggacattatttaggataatattatttatgcaggaattgtaccacctatttccagatggtataacttattatctgacaggcatgtagcaaatagaacacaaagcataaatctgtcaggagaaatcatacgagaaaaagagcattgtctggttatcagaatatcagatctctcattctggccttgctaggaaatagatctttgattctagaaaagtcaactaatttctatggttcttacttttctcctttataatatacccatttaaattccaaaaaggtatatgataaatcacaataatttcaatcacatggattttaatacaaaatgtataaaatcaatttccaaaaattttctgcatatactgaaaatgtctgtacgaatgagctaactactataggccttccctaatttattctattaaatgtgggtactcaatgtaacctgaaaatattgagcttaactcttctttttttttttcaaaagggaaacttgaaaaagactgcttcccccagaaaatttatcaacaataggtgctcaattaaatgtttttaaacaatgaacaatatcccctttcatataaataatcaggggagagatatttttaagtcttttttttctttttccatagtgtcacctacacaaaaaattatgtaaagacaccacttctatgaggaggtattcattgtagatgtacagaagtcaacggaaacttaagtttacagaaaaaataaaccagattatcattccacccaactgtatattcccacagatgcttaataaaagctatctgatgatataatgaattatcagttcttgaggaagtatatacagttggtgactatttttcaaaaatcatcatccaacaaatttttttcatttaaaatctttcatattaccctttcgacaatcagttgaaattttaaaactaagaacatttaaaaatataaatgaaagtagcattagctatagactgatattcaacttcagacgttaaaataaatacaagtgtgtattaagagtaaaattatgtcaacaatgtataaatgaaaactgccaatgtaattaatgtttcttttaacatatcccatccattgctttccctccaaaagacaaaggtagcaaaagacgaagcaggaagaactgcttcagaaactgaacatactgatttaattggctaagaagtccaaatgctaatactcctaataattagccattccttttgtgttttggtgacatatatcctcatacaatgtatatcaaatggaattttttgatttacacctgacatttcaaagtttccatttttgaattctcctagtcttaagtaagtagaacattgtctcctttgtttgctaggcataacgttttccccaacatctagggctccatgatgcaaaatatcattttgccgatcttctgttccagtatttactttaattttttttattataattggattttcaaatacaatcacaaaaacatctcctgttgaaggtggtttcccccaaaagtactcatcaacactactgtaagccttgcttgcttcataattttcaaacacattcatgttggtgtacagacttgcaggggggttatcaggaatgtcaaatgactcctcttcaaaatcatcatccttcagcttattctccgtccctttgtatgatgaataatagcccatgtgctgaaagagagatggtttaaaacggatcacatttttctgagccaacagaccacggaaatgagtcaatagccaatcacaaggcatttcttgataaaacattaataaaaaatgggccaaacgtgggagatcatgagaatgatagagtttaccaatgtagccaagcttagagaattcaagagttacccagtaagttccttctagggatgcaatgactttcttgatggcagttaagaaattttttgaacatcgaacatcatcttcaagcattacataatagtctgaagtattggcacaaaaattaagcagaaaagcataatctacattttgcttggaacgaaatttgactctatcttctggatcattgtaatttcttttaaggccatctaggattgggtaatactcctctggagcatgtataaccattaatcttcctgcaataatatggtgcgcaaatttctgtgtaatatcctggaccatggcatcacgccaggaagaattaaagtctgctaggtgaaccaccactgaaatttccttcagctcttcatagctggattgctcaaaaattgacttaattgtctcaagtaaatagtttcctttttttcgctttactgaagaaagtccaattgtaagataccgctttctttgtaaaggtgtggcagctaggtagcgataggtgacatttatggctcctgagaaattagataaatccttgaaagtatgaacatagcgttctgaattcagttgatgtgtggatgtttcccttataagttgtttgtctccttccagaacatagctatcttcaatgtacaagttcataaaaaggagaaaaatgacaagaactcccaagaatgacactgtagaacgttttctcaggcatctcattttatcaagtatttcaaaaatatgtttcatttgatgaaatttaaacattctcttcttaagaaagacgctgtcataatctgtgctgtacagaaaccgttgataccgttttagtttctgtagagatagcctttctcacgcagaatcagggctgtgctttctgggtgagtcagagtggataaagcttcaaccttgctatagcgttttctgcagctcttgtttgaaagacagatccacagcagctttgtgcatacaagtgatctggctgatctccagttcccatccaagtagaatgtaacagcagctgagaagcttcagagaaaacctgcccgataacaataatccattagaaaactggcaatatcctctgatctattgcccgcaaagccatgacttgatggagagtttcattccctgggctcagttctccagaagaaaatcagcacaatttaaatatttcttggaatgtgacagctctctagatcccgggttgcattctgttccccagggatggcaatctggtgttcctgtgtgcatagagcagtgaagatgaattgaaaacgcttgagataaattaggaatggctaagttaaaattgtctctgctccagactctctcatctgcagtctgcaagcctgtttttctgt

SEQ ID NO: 13487 - RNA, 22959 nt, Homo sapiens
  source 1..22959: mol_type = other RNA
gctgggattacaggcatgagccaccacgcctggccagtttttaaagtatttcatacagtgtaactaggcagtcagaaatacctgtatctcaaattcatttaacttttcaatgaatcaatcttcttattttctcagacatataaattatcataatactttacattgagtctctatggttgactatatgctgtgaaggaaggacataaatacatgtgaggaaacaattattgatatttttaaactaactagaaagcaccaagttatttgttaaataaacaaagttaattttatctacctgttcagtaagtgttggcaactatgaattaatctttgacaaattcacttacaactagcaattttaaagacttaaagtttaatttttattattaaaagggtatgattatttttactaaaattaataaaaagattaactgttactaaattaaagctccttcaaaaacataaatgtattctttagagagttaaaaaaagtagcaataaaatacatttttaatttagttaagcttacttaactaatgatcaaatagattaagttgtataaaattttacaaactttatatttttgcatacacttatcttcctggcatttttgaaataaaaaaaatacaagtgcatagggcagaggaggcgattcagttacttctgctatgttattaaatctctggtaaccactatacaatacaatacaatacaatacaatacaatacaatacaatacaatacaatacaatacaatacatgtagactcagcatccaaactttattttaccttcaagttctacctgataaagtggtggaataaagatggtattttccataactgtttaataataatcacatgttttatacccattgctttgaagaagaaaccttaagcaactagaaatgtcaatctaaaaggcagaaaagctggaaaaatctcatgaagactagaagatttacactcataagatcatgtaaatttatttggatatgctgaaaaaagagggggtataaaatctaaagtttggtaaatctttgctttacagggcttcaagttatagatttttcttttttccttttctcttcccctttctctctctttctcttttttatttttgccatttcttctcaggagcccctgcaatttcaaaccttggaattgaattggatttgaggaggaaaacccatattcagctttaattcaaatgaattttactactttagacaaaggtacaacactctattcaaaaaagttattgaaatcacatctttaaatctgacccagccacttgaataaataagttgtgttgtagtttctcagagcaaccgccgctcatctttcactcaccttaacaatttctcacttttttctgctttttttttttttttattttctgcttgctgaaatcgagatcaatattcattgttttcttctgggttaactcttttttatgttaactgaatcaattttggctttgtttctttatgaaattacttttagataaagtattgatattgtcatttatcaattttattatatgtcttttgcttattaaaggattaaaatccacctctaaacttatttagatcaaggtcagtttttttactcctctgtagaactgtgaagataatatcctattctccttttcttatggttttattgtgaagatctgtgcaaatagctatataaaatgcaattcggtattaaagaaaattgttgcacggactacattgattagagtctaatttttggaaagtatacttcgccttttcagtaattttatttttcggtctatggtgcccacattgtgtcaccagccagccgtatgcagacttacaaaggactacccactaagaataaaaacatgatacaacttgaagaaattttcatcaaacgtctttgtcttatccccttgttatacagacaaagatgacaagggccgaaaaggaagtgattttctcattgaataagagaatccgaactggcatcgaggatatctaattttgggatgaaaattgagagaagacagaatttcaagtctgaattatgacttcactactgtgtcgtcattggtagaataaggataacaatacttatcacacagatttgtggtctgaatcacatgagagacatagatgaaaaatgtaaaacaacaattagcatgtgacatgctctcagcaaatcaattaatccttcattctttttttctccccttactcctttgattttcagactaatttggatcatgattattggcctgtgtcccacccattattcacatatagaatgggttgcattatcctctccttggaaatatctttcaaagtgggtaatgagaaaactactttgaagactgtgctgaaggaaatgatggcatgaacaactctagataatttttgtttatttggatataacgtgaatgggcccataccataaactcctattaagctgaatcaccaaaaaaaaatttgatatgaaagtcatacattgaaaaaattcactcttaccactgatttgattgatactgagcctgtaaatatttatttatatgatgtttggcactttattttataaaactaccctttacttaaaataaatcattgtattcacataactttccagggcactatgcatttttaaacaagacagtcaacttactatttaaaaaacaaagtcagtcacctaaatgactttctgactataaatttgaaaacaatattctccttgtaatatatgtgccaccagggcaagaattacaaattgggagcaggtaagaaaattgttgttgactctcattagtattctaattctccttcagtcagatttataaagtatgacctatagcatccaactccatcattttccagtcattcttgagactgtcaactctatgggcattgtttagcagcctcgaaacactgaactttttacagtcttattggagagaaaaacacattaaatgatcaaataatcttttatgagctcagaaaaaaatgcctaacatgaacatttaagcatcttctgtttctgtgattcccatttttggagagtaaaaatttaagaaacaaagggaatgtgtctggggatggtactaataatattgagattttacaatttaggttataatcaagataattatgtatatatataaaattatatatggtatagtttcaacttctaatcttttatcatcctctaccacataattcctcctatattctctttttctgactgtggcctaatacctcaagaatattgtatatgcttgtcactatataaacttcaccctaaggaaatttccatgtcagatacaataagagcaacggaagaaaatgtatcaaaacacatctccaatttatttgaatttttctggcctaaccttgttggcatgagagttcccactttgtattataataggcaaattgatacacacttttcatttattctaaataatagattagcatagtcaggaggcttggattggcagctattaaatacaatttgaagccgtgggattttattaggattctaaggttattctgtgacgatggaacttaatgatgtaagagttaattacccattgtcaaaaatcattgcccatcaaagcagtgagactgtgtgctatgtccagttttattcatttcttttgtgtatctgaatggaacatgtggtaaacacaacagtagaatatacctacagtccccttagaaactcttaaatcttcaatttataaaagtcatcctaagacgttaaaaataacttacgaaaggatagattccaatgtcagtgggtgagatgtgctctagctagtgtgcacgaaagagaacatggagttagaataattattgtaggactgtagattgtcatctcaagatcagtgtcaaatacattcattcatgtagtattttcacatgcattctggtctaaatatcccaacatatctttcgttttgagatctgcagaacaaagtcaatgtctgaatttagagactaatttgaccattttgattcaaatgtctaaaggctaaaccagagcaatttacaacatccaatgaagtaaaattatataattaattatataattatataattatataaaattttataattaattataaaataaaatattaacaataattgaacattgtttacttttttatcctcacaacaattcaacatgatatgtatggttattactaaatgtataatacatttagtaatgtgatttgacaaatcacatttgtcaaataaggaatggctgaattaaatgattgaatgaaggagtgaaggatgtagattgtttaagtacattcaacttgtaatgaactgtaaacttcacccataacattattaatatatcagtgctatcaactacattttacataggatgaaaaaaatcattatttttattaatcccaagatattttatttcattatataaatgaaatattttatctgttataaagacctttatttttgttccactcattaaataacatggtaagactgttgtgtaattgactgaatagttaagtctaaatgggtaaatagctgtttatgttagtattgcagggtagctatttgataatgaaatatacttttcttacctacttgcaaaaaaaattacataaacaagtatttcctagagttcaaacactgatctttttaagtggcaaattgtccaaaagaatttaattaatataaacaataaattcacttaaacaactatttacatgcaaaagtaatatttttattgcccatttggaaaatagttttgctttctggtttataaggaacttttactagtttaattacttgggtgctttaaatgttttttggaggctattacaaaatcacatcctaaaattttaaaatggaaaaattataataattgaatttttaattcctcataaatattttaaaagtacacattgttccatggcttttgcctttagaataaatacaacatttttatgtagaaatatattcttgaaatgtaactagcacatagtcagtgtttcttaaccattttggggtcctgaaactttttgataatgatgaaagcacagagatgctatcaagaaaaatttacccacataggaacacacacacatacacacagacacacacagagtttgcttataagctcaggaagcttaaagatctgctaaagattatgcttgggtttgccatgaatcataaataccaagtcaaatacctttgaatttgattcttaacaaatctttgtggctgagaaaccatgagatttcattctggcatgtccccagaatgtaattatcaatgaacaatagccattgaaaaaatctgaacagatattattgaggctcaaggttgtttaatggcacagataatataattcaaatcatgaccccagggctgatgaagtcttgttgtaacgtgtaaatggggtgggtgatgggagagagaaaacaaaataattatttatgttaaatcatacataaacagtaaagccaacacaataagtaaaataagagaaagtagaatgcttgggaggtcatatgtttcaaatgtatgcatacacaaaagagtaagcaacaggatacttcaagagtaaaatgggaaaaaatcatattgggtaaatagtatcaccccaaagtgatagtcaaaagtacctatgtttgcctagttctcagattacaactatgatgataatttagataaacaagcagaaaacaaaactatagaaaaaagtcaaagtgacataaaacaattactggtgtttcaacagaaataaacccaacatcaggatttatcaaatatatgaaaaattatgaaagattataaaacaccaatgattagattatgttataaagacactatgaagagatactaaatgatattcttttcatctgtggttactgctaaaaaattctttcatagaaattcttggattttgaaattagtttaattccaaaatattttctttattttgcaaaaatgtaagacaaatgtataggatatttttctctgttgttatgcaaggatttattatcacattggccacagaacacatagaatgttagttttgtagaaaattttagagattttaataccaggatgaaataatagtatcattctatttcaggttcttaagcaacattcctaagactagaaccttatcttgaaaaattatgattttaaacttaagggaattcaggtaaaggaaattgactaggttaaggcaaatacatcatgtttactggtaaagataacattatttaaggaaggtaagatactcttatcctacatatacgccagaaaaattgcttctcctctgaaaactaccattatttttgccaaatattgtagcttagttttaagtttttctcggctgtttcctctgacagttctgtggtaaagaagaaacattataggaagcatttttttttcctacagagtctgccatatggagaagtagaatgagaggccacctaggtaatgtgatttattaaaagttctccatcccaaaatatatgtcccatctgtgggctaatgtctgaaagtcctatgattaaactcacttttatgtaagatagtgaggccccagagagccctcgagaaatgcaaataaactattactgacctcccttggattatgatgaaaaccgtggagtctttctattctctgtcaaatgtggaggtcatggatccttcttggcacctaagattaaaactcatagaatgtgctttaacttctgtaggcacatttcctttccaattagagtgaggtgttgaatatttatttatttgtttatttttattatactttaagttttagggtacatgtgcataacgtgcaggtttgttacatatgtatacatgtgccatgttggtgttctgcatcttaagagaagactatttataaaatttattgcttgtaagatttgttttttgttctcttactattatgaaaatcacgaacttgggaataaggacactctgggcccggcgcggtggctcacgcatgtaatcccagcactttgtgaggccgaggcgggaggatcacgaggtcaggagatcgagagcatcctggctaacaaggtgaaaccccgtctctactaaaaatacaaaaaattagccgggcgtggtggcgggcgcctgtactcccagctactcgggaggctgaggcaggagaatggcgtgaccccaggaggtggaacttgcagtgagcggagatagtgccactgcagtccggcctgggcaaaagagtgagactctgtctcaaaaaaaaaaaaaaaaaaaaaaaaggacactctgaacaattgaacaagactacgctgaaaggcagagaagaagtaattatgaacaaactgttcatgaagtgatcaattgaatttgaaacagaacttttcctagcttctaaatgattagaaatttcagctttggtttaacttaaaaacttagaattgtcaattctgtccaagtctctgagtcatgtacagaactcaaattattacatcatttttttacttatctgtattatttctccatttaaaagtggacaaatttttatactatatcctaataatgatacaaggtgacttgtaggactctggatagaaagagatggcccaggatacagagggcactccttaaatagctgccaaataaatgacattaaaaaatgtataaaaaggtatgttaagtaattaaaagtgtcaggcattattttcctattatgagacattttatattatggttatttactgtaattgcatccaaaataattcataaaacatttatttttgtactattaaaaatctaaacaataataaccagatggaggaaaatgataccatctgatttaattattaacttgaaggtcagtttctacaacttattctcatttatgtttatctgatttggccacagtttcttactttctcatattttgctaagcttgtggatgaagccgcatgtctcttttttttttaacctggcatataacactgtcactctatttaattattacccatcatctacctactttgaaactttggaggttttataaaaattatgagtatttaatcaaagttgtctctttatcatttgccagtgaaaatataaaacctggctgttttattctattgtgcactctaattacataaccaaaatctttttaaaaattcttagttcttttagaaataccatttgacccagccatcccattactgggtatatacccaaaggattataaatcatgcttctataaagacacatgcacacgtatgtttattgcggcactattcacaatagcaaagacttggaaccaatccaaatgtccaacaatgatagactggattaagaaaatgtggcacatatacaccatggaatactatgcagccataaaaaatgatgagttcatgtcctttgtagggacatggatgaagctggaaaccatcattctcagcaaactattgcaacgacaaaaaaaccaaacactgcatgttctcataggtgggaactgaacattgagaacacatagacacaggaaggggaacatcacacactgggcctgttgtggggtcaggggaggggggagggatagcattaggagatatacctaatgttaaatgacgagttaatgggtgcagcacaccaacatggcacaggtatacatatgtaacaaacctgcaagttgtgcacatgtaccctaaaacttaaagtataataataaaaaaattcttagttatttgaaaatagtttttttgaattcacaaacttgcaggatgaaaaaagttattagttcctgaagatataacattgatttgtctttttcttatttgatatcagctagcagtaaaattgtgaacaaatctggtaaatcttttggtgttgcaggttcataatcagttaattgagtgtattcactataaattgctttaattaagtgatgtttgcctaagaacaagtttcatttcatctcatgaaaaaaatgttactttttgtattaatcagtggaatgtttaaagaaaaaactggttatcttgaagctgtcaaataattataagaaatctctatacattacgttttaaaatacataaaacccataaattcaagcttattagttttcattttcagcaaggtttatacagagaaaataagtaatacaaattagttttccagaaaatctaattttatgcagataaaatctgaaaatcatataagtccaagatgaaactgatctcaaattattattttgaggtgtatccatttatttaaaaaagcctcattttagctagcaacactatgtagaaaaatattttaaataagacagagcattaaaataatgtattcattgatctcataaagaatagatgatcagattttttaaaagtgattttaattaaatggacatgtttctctttagccagaaatgactgagaaattttgagttggaattgatataggggaatccttggaactatgtgtgaatatgtgtgtgtgaattatctgtgtatatttacataatttacactattcacagtccttgtttttcttgactcaaatagctatctcaagtttcgtacactttttagatctctatgtaaatacattatttcatttgtggaaatatattgaggcctatatcaataacctcaaaccttttaaacacttagagcaagtcaatatgacttgttctgtttcagctatctgaaatttaaaaatttgacaaatttttaaagtacccagttcttggaaaaagaaaaacaaataaattggagatttggatcatatgggctatgactaaatgagacaaggcatacatgctgacatttgaaggatttatgaaaaaaagtccactgtggaaaactgatagtttttctccttctttcttgaatatgtttagttaattttgtggaaagaggaaggcagctcagtttacaaacagcagtgggttgaaggcaatgctgtttatattcttgaatttcaatatctacaaagatgtcatcattagattttatgtgttaaaaagtggatttatagtctctaattaataaggtgcatatgtcaagactcaggaaaacagatcacttacgtagttctccaaaaacgagagtcccagattcaataggaaggcatgcagagtgttctctataaacccagcaaaaccataaaaattgactggaacttttatttttcagtacaacaataatagtattgaaatacctaaaaagggcaggaaacaacacagaataatctacgcttgtcatcatgttttctaatctataatctttcaaactggataaatgggaagttttggaattttactgtggtacagtcttagttgctccgtggttgtcaaatctgtctgcacattaggatcacttaggaagaattttaaaagtatgctgatgcctggaaactccagaacaattatgataactctgagcatggagctcaggaatgggtgaaattcttccccagagatgttaatgaacagccagacttaaaaactagtaatttagacaagtgtgagcagaggttaataatgttgagatgaactgggcttaatatttcactaacaaggtcagagttttgatacatcacttaactcaaactttgagattcttcatcactgaagtagcaataataatagtcatttctgttttaatacttcatagacttgtaaggatgtaatgtagtgtttctaaaaggagtgaatggacaatctgcatcagtgttaactaaaatacattgaaagtgccaattcctagatctatcctagatttacagggaagaattcagtagtctgaaacacacattttcaatatattgaaaagatgattcttttgcatgatgacttgttataatcattactttcataggtaatggaagtaccgattaggagagtaccaaatacatattaaacactcagttcatgtaagctataggccaataaacacaactttggggtttactgatgttttccaacatccgaaataatagctgaaatttagaaacatagttaatcacacaaaaaatgttgcatacatactgtctaactaccagtttggtatgtttggggctggtgttatgaaagactattatatgattaatacaaagttataatttttggagtcttttagtgtacccagagcccatgagtttttattttctttttggaataacagaaattaggttgtggttcagtggaattacagaagcaagtgttttagatgttcaagtttaaaaaatgagaaaaaaatgttttacatgaagaaactaattatttaaattcatttttcaactatttaatgttattttaatatagtcatatcatccagaaaatcccatcttagacaaatgggttttcaataaattattattatagttaggaggcaatgtataatagtgataaggggcatagattttgaattacacaaacctgaaatccaatgctctctctttcatttattagttatgtgaccttggacaagttagtaaaaccctatttttcatatgctctttagcttttttaatacctcttaccttatatggttgtttaatctattaaatagacagtgaaatgcacatgaaatcttcacacagtgtctcatagttgcttggaacatatttatgtagtaagcattgttcttggctgagcttacattaagtgatctgtaaattagaagttatttgttatatttgtttcgtttccttattgccctagatgccttttctctggacctagataatttagtctcactctgtggcctttacccttcaataaatatggattattaatataatttagctacataattcctaaggaaatattaattcataaagattgttaaattgaactgaatatctttgctaagtcacaggcattgattaaattagataaaattgtcattttccattgattttgtttatataaataatattgaattatttatattcttatttagtctagtagattgacaggcagttttattaagaaatgaatcaaatggtaaattttgaatcatctggtaaaaatggacaaaatttagttttatcttgtggtctggaaatacaccctaaattattgggtcaagttagtgaaaactgttaaattgattatgaacgtaggcacattacttataaatccccttatgctaacttaaaacttgtgaatgtttagtgttatccagctataattcttctaaacatgtcttgtaatttttaagtttgcatgaaaataactccatcctgagtatactcatttcaataaattatttgtcctgagcatactgtaagaaatttagtaaagtactaattgaatttagtgattagactgtgattagactattacaaattcacagtgcttgtacaattcagatattattttgctttgaagtcaaatagaggaaccttaaataatttaaataaaaataattgtttttattaaagtttatacagcaagataataaattcactaatgtgaaatgttgatatagtatgtacaacttgtttcttaagttactaaaaatgtattttcctacctacataatgtcaatctctattgctcctaacacatgagtggctaaaattgcaaacttaatcacataaataatgagattaaagttaaaatgaaaaagtggtatgaggactattgtttgtgttaagtgaaattataccttgtaaaatttcatattatgagagcaatatgtaaatttcattgcaacaatggttattcaatttactgatgaaaatcagaagaatgttgaaaaattagtgcatttataataaatttaattattcataaaaaattaacattgatatatatattcataaggataaaagatatcaaaataattaaacaaatttcactttcttcttataaaagaaaataatttttatggtaactaattttagtagtgcatcagatcaacactattgggcacccagttatttggtggtacgctgagtgaaaatatgtagctttatctacattaccttggtttggacaactgaaaaatttgctaggaaacaaatattacaaaatatgttgttaacttttcaaagatgatcggtttagattgctttaacttgaaggacacttatattttgtatcacttttgtagcaaacacatgactcatcattgcccaaatcaattgcccaaatcaattcaaacatctcattgtagttcatcccatggcagaaaagtgtttatccacttagtaaaatggaaaacactagagcttcaggtttaatttgaaattttaacttcattaagaataaacttgacctgtttgttctagtaagtaaaaacactagatacgtaccaaaattgtcttttgaccctctcagggagtcaagttttgatttgcttgaatacaagcaagtcgagctatggtaatttgcaatgctgacaggaaagaagaacttgcttgaggcaaaatcatgaagtacaacttttcctctgcatccttttacctcatgtttgtaacatttcccctgttgttatttttacacatctggatgctcagaaaggcctccttaccacaataattgaaaggagtactttgtcaatagtcagaattgaatgagagataggttgttgggaatattcagggtgaatgtgtcttttctactttgactatatttaccattgactacagtaactcagcagaaagttagagggcagcatacatacattggtttatggatttaatgaaaatatccccaaccattacattacagacaattcatatatatgtcttgaaaatcttcttgacaatttgtgacaaattttctaaatgtttttccaaaaatagttggttcttgtaagtgattttgatatgactgattaccaaattatggtgggtaaagatgccacatgcaacagaaaatgtgtctaattatgtttgttttagagcttaagaaatgttaagaagagaagttacaactgcattaataggattttaatttttattcaaaatggacaacttatttattatgtacttctacacacagctaagcttatagatattttcatttaaagaaaaactatttgttcattttattagcagatatcaaatgcccttttgaaaattgagactgatttctaaaacaaaaaaaaagactttaggagttttaattatttttaatatattgcttctttattaaaaaaagatacaatccttcaatgtcattcaacagtattaattgttaaagtgtgggatatagtttacattaccgagtttattttctaagggtagtgaataactcctgacaactactgatatcgtcacatggtcctttagtgaccaaaaatgcacagttgtaagaatgcaagtgttacttgtattgaaaaccggattacattaaaggatggacaattatgataaaggatctgagataattggacaattatgataaaggatctgagataattattctaactttttggaactatactttcactcattgatgaagtaagttacaacgtggaataacaaagtttaagtgtggcagaaaatacatacatatgtttaaaagtagggaaaattttatcaattattaaagatggaaaaaataggactatgtcaaatagttaaacaaatgtggggtattttatggagaaaagaggcatgtactaccttaaacattttccaattggaacatactatagacaaaactgacagattattattcaatgagaaacctgactcagatgaagttacaaaaaaagtactttttaaatgtctagtttctaatagagttagagctttgttgattgagatatgtggaactgccacatatctctgtgccatacttttggtaccttcataataaacggtaaagtgagggaaagggtggaagagacaaatcctacgtctcttccagaacttcgagtgcactataaattaaatatttaaaatatttttgcaatagttagctttcaattatgaacactctcagcctctattgctttatatatgcatttattttggtaatttttatacatcaaaactataattacctgtatttgggcagaatgatttaggttatgccagctattgtggttaaagctgtagtaacttacagtacattgaaattatagactaaggttctgaatattggtaactcactgttgttgtgcacctttaaacaactcttaaataaagtaatgattctctttatattaaatttaatgtatgtgtgcctcatggaaatttgtattttatagaaaaatattgaatattttattattatgtctttggctcacctactttaaggagatggctacttagggtactttttaatccaatataatgtgaaaatttgatcatgctatattcttaatttaattgtacttctatggtcatatacaatttacctatcactttctcacataatcaatttaactttttggtaaatcttctaagagaccgtctagacagagtgaaatgaaagctgaaacaacagtcaaatcaaaaactgctttggtctcaaatccatgtttttcagaaaagatattcagatccagttatctggcaaatggtctcaaacatacatttcaatttcaatgttaaaaataggatattaaacatctcagaaaatattgggattattgaagcaaattctaccctggacttggagtaaatgtgatgaacagattaatgaggtggaagggactagaactttgggaaagtgcaaccttgttatcttaatatttttatagcttagaaagagaatgctatgcaactcatattttgatcttttaatgttaaagaattcaaataaaaaccataaacctgaaactctaaaagaaaaattctgttttgagagagatggcctcctctagtacacttttaataaatttaaagtatctaaaaggatgcacaaagatctctaatgtgctgtgattttcaaaggatgtcatgtataaaagatttgagtgagaacatgaaagcaaaagcaagttcagaagaggaacacaaccaggaggacagtgtgtcaggaaaatccaagaataagtggaggtgtaaaggctaaaaaataatgcaaatggtgcatatccttctgtctttctctcatacacacagacacacttacacaacacatatacaaatacatacatgtatatatgtatatatatacacaaatatacacacatattcacataatattcaagtatgtatacatatatacacatatgtacatacacatatgtatatatacatacacacagattgagagattaaccatatgtagatacacacatgcacatatgcaataatgaaatcatttcaaagcatgccaaaaagtaataaaagatatatcctctgtttgggataaataaaaaaaaagtttaaaagcaaacaaaaaataaatggcaataactaatcacattgaattttgttatggcctttttcttcctaaaaagaataaccccaatctgaacaaagaaattcaaagtaatggaaaactcaacaatgaaactcaaagtagactagcagataagatacctatttcaaacatcagtgccaaggtaatttataggtcagtgcattgataacttttgccaatgatagaaaagatgccagagaaccggatcctgacattaaaaaaaaaaagtaaaaagattctgaagactgcatttctgagcttaaggtagattctaaacaacatcttagaaactaggaaatgactttatgtttctttgtttttcaatgtaaatggatcaagatttcttaaaacagaaatgaatattattatttgtgatgagagcactaggggcaattttgatatttttgataaggtttctagagtaataaattagaatgacaggaatatatattgattttaggaaagtgtctgtataattccacatgatattctctggacaaaatatgaaaaggtaggctgaataacatttttaaagggcagtaaattttataattgttattgattacaatgaaggcctctggtaatgttttccagggtcatatcctgttacatatacgtgacatggataaaaaggaaacaaatatttattgtgtgcctagtttatgttatctcaattccagctctacaaggagctacaaggtaaaattgctacctttaaaaacatatgaggtaaaattattcctattcacagatgtagaaactgagtttcaagaaggttaagtaaatttcctcatattgggaggctggtaatgcagaactgggtgtcaaaatcaagtctgtatgaaccttctgttttgtctcccatgaagacaaaaggcatgcatataaaatttgttgaaacacaaagctgaggaggcataataagacgtggaatgacagaagcaagatctagaaagtttgggatcatgaatcaaaagaaacaggataaaattatcctaaaattaatattaaatcttacaagaaaccccccaaaatcagttgaatttgtacaaaacggtaaatcattttatcagtagatcccataataaatattataaagtttaagtgtgagctctattactcagtaatatgatgccattactgtgttgatggatgtattgtcaaggaaaaagaagagaattacacactgtttccttcaattgttagatggcactggatgtagtgttttcaatgttaatcctggtatcatgttctttgccataaacttgttgacaaattggcaaatactgacatgaaatatgccaatatttgagcatctaaaaatgtaggtactttccataccacatcatatattacaatttgaaaatgtttgtttcattttttatataattattatacagaacagtttttctatgatagcattataaaaattcccagagaatactggcccagtaagaaatggaatgttcacaactcatagtgtagctatatgaaagaaatagatctaaacgacaggttggtttccaaattatattttcatacctggaaaatatctactttataaatagcacaaagttatagttttcaatgaatatgaaaaagttcttgcattaacatattttatgtatcttttatattgacatttgtgattgccactaaaatgtgtattttctaaatttcattgtgcttttacaagatacttttttctttgatgtccataactgctgaaaaggctcccctaaggagaattttaagactaagtaaggtttttagtgagcttaaattatacaattctgaggcattatttaaggtgcatactgtattttttgcttgaaacctgtcagcattttatttgtatggcaattaaatgactcagccattcatgtctcatgccagtctttttcaattgttatttttaacaaagaaaattatatatatatgtatatatatattatatatatgtatatatgtattatatatgtatatatatataaacttacagcaaaaatgtttaaaaatagcaaatagtttgagtatagttaaacctaataactgtacttttgtttctatgcctctgagacaagattactagacccttattcaaagtttctaaatataggaaatagaacattgggccatgctaaaaaaattgttcagattttcttttgaaagagaatagttatttttcctcctgacctctaatgaagatgctttatttgtcaaggtgttttccttagaaaattgacccagtgtcaactgtaaagaaaacatagaggatccttggatgattgaccaacttatccaaacacaggtttagtaaagagaggatataaagataaaatgtgaaatgacctctctgagtcacatttgttttcataatttcctagcaaacatccaacttcactgctaccctcagcaatgtttcttgaaacatttttaagacattgatagacaccaatagctgatctttagaaagccattcccagaagaatatgtaaggggttacaactcatttcagggagtctgcctagctcttgatattacatgtctttggcatacaattgtgtaccttttatcattgacagtgaagaaaataatgccatttgtaacttctgagatatacacacaatactatcaactagccggttaataaaagataagaaaaataaagaaaatagaacatttttaggtgtctggcaagtatcctctaaatcaaggtaaagataataatttagtggcagtgttcatattttcctatgactgtaagatttaggtgcctcacaaaatattaatatttagcctcttatgaaaggttcgtttttcttctaacactttagtagctgaatacaaagaaaatacacaacagctgtttataaatgaaataaaaagtttccattttttatctgagtttctcatttatttgcagagaacgaataaaataaaaatatcctagtgttgtttgcaccacagcataccagtaaatcttaaggattgtgtttcagtatgaaaaggaagagcaggaagatttcctcattctgtcttaccagcaaaagtctagccttcacacacacacacacacacacacacacacacacacacacacacacacacacacagagtcatctatatgaacacgtacttgagtttcttaaacatatatgaagcaccttccatttccctttataataaatcccttagtttttgctgttcattaaaaaacaaaaaggaagagacaagctcaggacattctgaaaaccaatgtctttaggacacactaaggtgtcctgaattactttaacggacacattgtaaagacacactctccaatccctattaggaaaagtttagtcaagtttgcttactatttgggtgcttataccaaaaaagcatcatttaggacattatttaggataatattatttatgcaggaattgtaccacctatttccagatggtataacttattatctgacaggcatgtagcaaatagaacacaaagcataaatctgtcaggagaaatcatacgagaaaaagagcattgtctggttatcagaatatcagatctctcattctggccttgctaggaaatagatctttgattctagaaaagtcaactaatttctatggttcttacttttctcctttataatatacccatttaaattccaaaaaggtatatgataaatcacaataatttcaatcacatggattttaatacaaaatgtataaaatcaatttccaaaaattttctgcatatactgaaaatgtctgtacgaatgagctaactactataggccttccctaatttattctattaaatgtgggtactcaatgtaacctgaaaatattgagcttaactcttctttttttttttcaaaagggaaacttgaaaaagactgcttcccccagaaaatttatcaacaataggtgctcaattaaatgtttttaaacaatgaacaatatcccctttcatataaataatcaggggagagatatttttaagtcttttttttctttttccatagtgtcacctacacaaaaaattatgtaaagacaccacttctatgaggaggtattcattgtagatgtacagaagtcaacggaaacttaagtttacagaaaaaataaaccagattatcattccacccaactgtatattcccacagatgcttaataaaagctatctgatgatataatgaattatcagttcttgaggaagtatatacagttggtgactatttttcaaaaatcatcatccaacaaatttttttcatttaaaatctttcatattaccctttcgacaatcagttgaaattttaaaactaagaacatttaaaaatataaatgaaagtagcattagctatagactgatattcaacttcagacgttaaaataaatacaagtgtgtattaagagtaaaattatgtcaacaatgtataaatgaaaactgccaatgtaattaatgtttcttttaacatatcccatccattgctttccctccaaaagacaaaggtagcaaaagacgaagcaggaagaactgcttcagaaactgaacatactgatttaattggctaagaagtccaaatgctaatactcctaataattagccattccttttgtgttttggtgacatatatcctcatacaatgtatatcaaatggaattttttgatttacacctgacatttcaaagtttccatttttgaattctcctagtcttaagtaagtagaacattgtctcctttgtttgctaggcataacgttttccccaacatctagggctccatgatgcaaaatatcattttgccgatcttctgttccagtatttactttaattttttttattataattggattttcaaatacaatcacaaaaacatctcctgttgaaggtggtttcccccaaaagtactcatcaacactactgtaagccttgcttgcttcataattttcaaacacattcatgttggtgtacagacttgcaggggggttatcaggaatgtcaaatgactcctcttcaaaatcatcatccttcagcttattctccgtccctttgtatgatgaataatagcccatgtgctgaaagagagatggtttaaaacggatcacatttttctgagccaacagaccacggaaatgagtcaatagccaatcacaaggcatttcttgataaaacattaataaaaaatgggccaaacgtgggagatcatgagaatgatagagtttaccaatgtagccaagcttagagaattcaagagttacccagtaagttccttctagggatgcaatgactttcttgatggcagttaagaaattttttgaacatcgaacatcatcttcaagcattacataatagtctgaagtattggcacaaaaattaagcagaaaagcataatctacattttgcttggaacgaaatttgactctatcttctggatcattgtaatttcttttaaggccatctaggattgggtaatactcctctggagcatgtataaccattaatcttcctgcaataatatggtgcgcaaatttctgtgtaatatcctggaccatggcatcacgccaggaagaattaaagtctgctaggtgaaccaccactgaaatttccttcagctcttcatagctggattgctcaaaaattgacttaattgtctcaagtaaatagtttcctttttttcgctttactgaagaaagtccaattgtaagataccgctttctttgtaaaggtgtggcagctaggtagcgataggtgacatttatggctcctgagaaattagataaatccttgaaagtatgaacatagcgttctgaattcagttgatgtgtggatgtttcccttataagttgtttgtctccttccagaacatagctatcttcaatgtacaagttcataaaaaggagaaaaatgacaagaactcccaagaatgacactgtagaacgttttctcaggcatctcattttatcaagtatttcaaaaatatgtttcatttgatgaaatttaaacattctcttcttaagaaagacgctgtcataatctgtgctgtacagaaaccgttgataccgttttagtttctgtagagatagcctttctcacgcagaatcagggctgtgctttctgggtgagtcagagtggataaagcttcaaccttgctatagcgttttctgcagctcttgtttgaaagacagatccacagcagctttgtgcatacaagtgatctggctgatctccagttccttcagagaaaacctgcccgataacaataatccattagaaaactggcaatatcctctgatctattgcccgcaaagccatgacttgatggagagtttcattccctgggctcagttctccagaagaaaatcagcacaatttaaatatttcttggaatgtgacagctctctagatcccgggttgcattctgttccccagggatggcaatctggtgttcctgtgtgcatagagcagtgaagatgaattgaaaacgcttgagataaattaggaatggctaagttaaaattgtctctgctccagactctctcatctgcagtctgcaagcctgtttttctgt

SEQ ID NO: 13488 - RNA, 23057 nt, Homo sapiens
  source 1..23057: mol_type = other RNA
gctgggattacaggcatgagccaccacgcctggccagtttttaaagtatttcatacagtgtaactaggcagtcagaaatacctgtatctcaaattcatttaacttttcaatgaatcaatcttcttattttctcagacatataaattatcataatactttacattgagtctctatggttgactatatgctgtgaaggaaggacataaatacatgtgaggaaacaattattgatatttttaaactaactagaaagcaccaagttatttgttaaataaacaaagttaattttatctacctgttcagtaagtgttggcaactatgaattaatctttgacaaattcacttacaactagcaattttaaagacttaaagtttaatttttattattaaaagggtatgattatttttactaaaattaataaaaagattaactgttactaaattaaagctccttcaaaaacataaatgtattctttagagagttaaaaaaagtagcaataaaatacatttttaatttagttaagcttacttaactaatgatcaaatagattaagttgtataaaattttacaaactttatatttttgcatacacttatcttcctggcatttttgaaataaaaaaaatacaagtgcatagggcagaggaggcgattcagttacttctgctatgttattaaatctctggtaaccactatacaatacaatacaatacaatacaatacaatacaatacaatacaatacaatacaatacaatacatgtagactcagcatccaaactttattttaccttcaagttctacctgataaagtggtggaataaagatggtattttccataactgtttaataataatcacatgttttatacccattgctttgaagaagaaaccttaagcaactagaaatgtcaatctaaaaggcagaaaagctggaaaaatctcatgaagactagaagatttacactcataagatcatgtaaatttatttggatatgctgaaaaaagagggggtataaaatctaaagtttggtaaatctttgctttacagggcttcaagttatagatttttcttttttccttttctcttcccctttctctctctttctcttttttatttttgccatttcttctcaggagcccctgcaatttcaaaccttggaattgaattggatttgaggaggaaaacccatattcagctttaattcaaatgaattttactactttagacaaaggtacaacactctattcaaaaaagttattgaaatcacatctttaaatctgacccagccacttgaataaataagttgtgttgtagtttctcagagcaaccgccgctcatctttcactcaccttaacaatttctcacttttttctgctttttttttttttttattttctgcttgctgaaatcgagatcaatattcattgttttcttctgggttaactcttttttatgttaactgaatcaattttggctttgtttctttatgaaattacttttagataaagtattgatattgtcatttatcaattttattatatgtcttttgcttattaaaggattaaaatccacctctaaacttatttagatcaaggtcagtttttttactcctctgtagaactgtgaagataatatcctattctccttttcttatggttttattgtgaagatctgtgcaaatagctatataaaatgcaattcggtattaaagaaaattgttgcacggactacattgattagagtctaatttttggaaagtatacttcgccttttcagtaattttatttttcggtctatggtgcccacattgtgtcaccagccagccgtatgcagacttacaaaggactacccactaagaataaaaacatgatacaacttgaagaaattttcatcaaacgtctttgtcttatccccttgttatacagacaaagatgacaagggccgaaaaggaagtgattttctcattgaataagagaatccgaactggcatcgaggatatctaattttgggatgaaaattgagagaagacagaatttcaagtctgaattatgacttcactactgtgtcgtcattggtagaataaggataacaatacttatcacacagatttgtggtctgaatcacatgagagacatagatgaaaaatgtaaaacaacaattagcatgtgacatgctctcagcaaatcaattaatccttcattctttttttctccccttactcctttgattttcagactaatttggatcatgattattggcctgtgtcccacccattattcacatatagaatgggttgcattatcctctccttggaaatatctttcaaagtgggtaatgagaaaactactttgaagactgtgctgaaggaaatgatggcatgaacaactctagataatttttgtttatttggatataacgtgaatgggcccataccataaactcctattaagctgaatcaccaaaaaaaaatttgatatgaaagtcatacattgaaaaaattcactcttaccactgatttgattgatactgagcctgtaaatatttatttatatgatgtttggcactttattttataaaactaccctttacttaaaataaatcattgtattcacataactttccagggcactatgcatttttaaacaagacagtcaacttactatttaaaaaacaaagtcagtcacctaaatgactttctgactataaatttgaaaacaatattctccttgtaatatatgtgccaccagggcaagaattacaaattgggagcaggtaagaaaattgttgttgactctcattagtattctaattctccttcagtcagatttataaagtatgacctatagcatccaactccatcattttccagtcattcttgagactgtcaactctatgggcattgtttagcagcctcgaaacactgaactttttacagtcttattggagagaaaaacacattaaatgatcaaataatcttttatgagctcagaaaaaaatgcctaacatgaacatttaagcatcttctgtttctgtgattcccatttttggagagtaaaaatttaagaaacaaagggaatgtgtctggggatggtactaataatattgagattttacaatttaggttataatcaagataattatgtatatatataaaattatatatggtatagtttcaacttctaatcttttatcatcctctaccacataattcctcctatattctctttttctgactgtggcctaatacctcaagaatattgtatatgcttgtcactatataaacttcaccctaaggaaatttccatgtcagatacaataagagcaacggaagaaaatgtatcaaaacacatctccaatttatttgaatttttctggcctaaccttgttggcatgagagttcccactttgtattataataggcaaattgatacacacttttcatttattctaaataatagattagcatagtcaggaggcttggattggcagctattaaatacaatttgaagccgtgggattttattaggattctaaggttattctgtgacgatggaacttaatgatgtaagagttaattacccattgtcaaaaatcattgcccatcaaagcagtgagactgtgtgctatgtccagttttattcatttcttttgtgtatctgaatggaacatgtggtaaacacaacagtagaatatacctacagtccccttagaaactcttaaatcttcaatttataaaagtcatcctaagacgttaaaaataacttacgaaaggatagattccaatgtcagtgggtgagatgtgctctagctagtgtgcacgaaagagaacatggagttagaataattattgtaggactgtagattgtcatctcaagatcagtgtcaaatacattcattcatgtagtattttcacatgcattctggtctaaatatcccaacatatctttcgttttgagatctgcagaacaaagtcaatgtctgaatttagagactaatttgaccattttgattcaaatgtctaaaggctaaaccagagcaatttacaacatccaatgaagtaaaattatataattaattatataattatataattatataaaattttataattaattataaaataaaatattaacaataattgaacattgtttacttttttatcctcacaacaattcaacatgatatgtatggttattactaaatgtataatacatttagtaatgtgatttgacaaatcacatttgtcaaataaggaatggctgaattaaatgattgaatgaaggagtgaaggatgtagattgtttaagtacattcaacttgtaatgaactgtaaacttcacccataacattattaatatatcagtgctatcaactacattttacataggatgaaaaaaatcattatttttattaatcccaagatattttatttcattatataaatgaaatattttatctgttataaagacctttatttttgttccactcattaaataacatggtaagactgttgtgtaattgactgaatagttaagtctaaatgggtaaatagctgtttatgttagtattgcagggtagctatttgataatgaaatatacttttcttacctacttgcaaaaaaaattacataaacaagtatttcctagagttcaaacactgatctttttaagtggcaaattgtccaaaagaatttaattaatataaacaataaattcacttaaacaactatttacatgcaaaagtaatatttttattgcccatttggaaaatagttttgctttctggtttataaggaacttttactagtttaattacttgggtgctttaaatgttttttggaggctattacaaaatcacatcctaaaattttaaaatggaaaaattataataattgaatttttaattcctcataaatattttaaaagtacacattgttccatggcttttgcctttagaataaatacaacatttttatgtagaaatatattcttgaaatgtaactagcacatagtcagtgtttcttaaccattttggggtcctgaaactttttgataatgatgaaagcacagagatgctatcaagaaaaatttacccacataggaacacacacacatacacacagacacacacagagtttgcttataagctcaggaagcttaaagatctgctaaagattatgcttgggtttgccatgaatcataaataccaagtcaaatacctttgaatttgattcttaacaaatctttgtggctgagaaaccatgagatttcattctggcatgtccccagaatgtaattatcaatgaacaatagccattgaaaaaatctgaacagatattattgaggctcaaggttgtttaatggcacagataatataattcaaatcatgaccccagggctgatgaagtcttgttgtaacgtgtaaatggggtgggtgatgggagagagaaaacaaaataattatttatgttaaatcatacataaacagtaaagccaacacaataagtaaaataagagaaagtagaatgcttgggaggtcatatgtttcaaatgtatgcatacacaaaagagtaagcaacaggatacttcaagagtaaaatgggaaaaaatcatattgggtaaatagtatcaccccaaagtgatagtcaaaagtacctatgtttgcctagttctcagattacaactatgatgataatttagataaacaagcagaaaacaaaactatagaaaaaagtcaaagtgacataaaacaattactggtgtttcaacagaaataaacccaacatcaggatttatcaaatatatgaaaaattatgaaagattataaaacaccaatgattagattatgttataaagacactatgaagagatactaaatgatattcttttcatctgtggttactgctaaaaaattctttcatagaaattcttggattttgaaattagtttaattccaaaatattttctttattttgcaaaaatgtaagacaaatgtataggatatttttctctgttgttatgcaaggatttattatcacattggccacagaacacatagaatgttagttttgtagaaaattttagagattttaataccaggatgaaataatagtatcattctatttcaggttcttaagcaacattcctaagactagaaccttatcttgaaaaattatgattttaaacttaagggaattcaggtaaaggaaattgactaggttaaggcaaatacatcatgtttactggtaaagataacattatttaaggaaggtaagatactcttatcctacatatacgccagaaaaattgcttctcctctgaaaactaccattatttttgccaaatattgtagcttagttttaagtttttctcggctgtttcctctgacagttctgtggtaaagaagaaacattataggaagcatttttttttcctacagagtctgccatatggagaagtagaatgagaggccacctaggtaatgtgatttattaaaagttctccatcccaaaatatatgtcccatctgtgggctaatgtctgaaagtcctatgattaaactcacttttatgtaagatagtgaggccccagagagccctcgagaaatgcaaataaactattactgacctcccttggattatgatgaaaaccgtggagtctttctattctctgtcaaatgtggaggtcatggatccttcttggcacctaagattaaaactcatagaatgtgctttaacttctgtaggcacatttcctttccaattagagtgaggtgttgaatatttatttatttgtttatttttattatactttaagttttagggtacatgtgcataacgtgcaggtttgttacatatgtatacatgtgccatgttggtgttctgcatcttaagagaagactatttataaaatttattgcttgtaagatttgttttttgttctcttactattatgaaaatcacgaacttgggaataaggacactctgggcccggcgcggtggctcacgcatgtaatcccagcactttgtgaggccgaggcgggaggatcacgaggtcaggagatcgagagcatcctggctaacaaggtgaaaccccgtctctactaaaaatacaaaaaattagccgggcgtggtggcgggcgcctgtactcccagctactcgggaggctgaggcaggagaatggcgtgaccccaggaggtggaacttgcagtgagcggagatagtgccactgcagtccggcctgggcaaaagagtgagactctgtctcaaaaaaaaaaaaaaaaaaaaaaaaggacactctgaacaattgaacaagactacgctgaaaggcagagaagaagtaattatgaacaaactgttcatgaagtgatcaattgaatttgaaacagaacttttcctagcttctaaatgattagaaatttcagctttggtttaacttaaaaacttagaattgtcaattctgtccaagtctctgagtcatgtacagaactcaaattattacatcatttttttacttatctgtattatttctccatttaaaagtggacaaatttttatactatatcctaataatgatacaaggtgacttgtaggactctggatagaaagagatggcccaggatacagagggcactccttaaatagctgccaaataaatgacattaaaaaatgtataaaaaggtatgttaagtaattaaaagtgtcaggcattattttcctattatgagacattttatattatggttatttactgtaattgcatccaaaataattcataaaacatttatttttgtactattaaaaatctaaacaataataaccagatggaggaaaatgataccatctgatttaattattaacttgaaggtcagtttctacaacttattctcatttatgtttatctgatttggccacagtttcttactttctcatattttgctaagcttgtggatgaagccgcatgtctcttttttttttaacctggcatataacactgtcactctatttaattattacccatcatctacctactttgaaactttggaggttttataaaaattatgagtatttaatcaaagttgtctctttatcatttgccagtgaaaatataaaacctggctgttttattctattgtgcactctaattacataaccaaaatctttttaaaaattcttagttcttttagaaataccatttgacccagccatcccattactgggtatatacccaaaggattataaatcatgcttctataaagacacatgcacacgtatgtttattgcggcactattcacaatagcaaagacttggaaccaatccaaatgtccaacaatgatagactggattaagaaaatgtggcacatatacaccatggaatactatgcagccataaaaaatgatgagttcatgtcctttgtagggacatggatgaagctggaaaccatcattctcagcaaactattgcaacgacaaaaaaaccaaacactgcatgttctcataggtgggaactgaacattgagaacacatagacacaggaaggggaacatcacacactgggcctgttgtggggtcaggggaggggggagggatagcattaggagatatacctaatgttaaatgacgagttaatgggtgcagcacaccaacatggcacaggtatacatatgtaacaaacctgcaagttgtgcacatgtaccctaaaacttaaagtataataataaaaaaattcttagttatttgaaaatagtttttttgaattcacaaacttgcaggatgaaaaaagttattagttcctgaagatataacattgatttgtctttttcttatttgatatcagctagcagtaaaattgtgaacaaatctggtaaatcttttggtgttgcaggttcataatcagttaattgagtgtattcactataaattgctttaattaagtgatgtttgcctaagaacaagtttcatttcatctcatgaaaaaaatgttactttttgtattaatcagtggaatgtttaaagaaaaaactggttatcttgaagctgtcaaataattataagaaatctctatacattacgttttaaaatacataaaacccataaattcaagcttattagttttcattttcagcaaggtttatacagagaaaataagtaatacaaattagttttccagaaaatctaattttatgcagataaaatctgaaaatcatataagtccaagatgaaactgatctcaaattattattttgaggtgtatccatttatttaaaaaagcctcattttagctagcaacactatgtagaaaaatattttaaataagacagagcattaaaataatgtattcattgatctcataaagaatagatgatcagattttttaaaagtgattttaattaaatggacatgtttctctttagccagaaatgactgagaaattttgagttggaattgatataggggaatccttggaactatgtgtgaatatgtgtgtgtgaattatctgtgtatatttacataatttacactattcacagtccttgtttttcttgactcaaatagctatctcaagtttcgtacactttttagatctctatgtaaatacattatttcatttgtggaaatatattgaggcctatatcaataacctcaaaccttttaaacacttagagcaagtcaatatgacttgttctgtttcagctatctgaaatttaaaaatttgacaaatttttaaagtacccagttcttggaaaaagaaaaacaaataaattggagatttggatcatatgggctatgactaaatgagacaaggcatacatgctgacatttgaaggatttatgaaaaaaagtccactgtggaaaactgatagtttttctccttctttcttgaatatgtttagttaattttgtggaaagaggaaggcagctcagtttacaaacagcagtgggttgaaggcaatgctgtttatattcttgaatttcaatatctacaaagatgtcatcattagattttatgtgttaaaaagtggatttatagtctctaattaataaggtgcatatgtcaagactcaggaaaacagatcacttacgtagttctccaaaaacgagagtcccagattcaataggaaggcatgcagagtgttctctataaacccagcaaaaccataaaaattgactggaacttttatttttcagtacaacaataatagtattgaaatacctaaaaagggcaggaaacaacacagaataatctacgcttgtcatcatgttttctaatctataatctttcaaactggataaatgggaagttttggaattttactgtggtacagtcttagttgctccgtggttgtcaaatctgtctgcacattaggatcacttaggaagaattttaaaagtatgctgatgcctggaaactccagaacaattatgataactctgagcatggagctcaggaatgggtgaaattcttccccagagatgttaatgaacagccagacttaaaaactagtaatttagacaagtgtgagcagaggttaataatgttgagatgaactgggcttaatatttcactaacaaggtcagagttttgatacatcacttaactcaaactttgagattcttcatcactgaagtagcaataataatagtcatttctgttttaatacttcatagacttgtaaggatgtaatgtagtgtttctaaaaggagtgaatggacaatctgcatcagtgttaactaaaatacattgaaagtgccaattcctagatctatcctagatttacagggaagaattcagtagtctgaaacacacattttcaatatattgaaaagatgattcttttgcatgatgacttgttataatcattactttcataggtaatggaagtaccgattaggagagtaccaaatacatattaaacactcagttcatgtaagctataggccaataaacacaactttggggtttactgatgttttccaacatccgaaataatagctgaaatttagaaacatagttaatcacacaaaaaatgttgcatacatactgtctaactaccagtttggtatgtttggggctggtgttatgaaagactattatatgattaatacaaagttataatttttggagtcttttagtgtacccagagcccatgagtttttattttctttttggaataacagaaattaggttgtggttcagtggaattacagaagcaagtgttttagatgttcaagtttaaaaaatgagaaaaaaatgttttacatgaagaaactaattatttaaattcatttttcaactatttaatgttattttaatatagtcatatcatccagaaaatcccatcttagacaaatgggttttcaataaattattattatagttaggaggcaatgtataatagtgataaggggcatagattttgaattacacaaacctgaaatccaatgctctctctttcatttattagttatgtgaccttggacaagttagtaaaaccctatttttcatatgctctttagcttttttaatacctcttaccttatatggttgtttaatctattaaatagacagtgaaatgcacatgaaatcttcacacagtgtctcatagttgcttggaacatatttatgtagtaagcattgttcttggctgagcttacattaagtgatctgtaaattagaagttatttgttatatttgtttcgtttccttattgccctagatgccttttctctggacctagataatttagtctcactctgtggcctttacccttcaataaatatggattattaatataatttagctacataattcctaaggaaatattaattcataaagattgttaaattgaactgaatatctttgctaagtcacaggcattgattaaattagataaaattgtcattttccattgattttgtttatataaataatattgaattatttatattcttatttagtctagtagattgacaggcagttttattaagaaatgaatcaaatggtaaattttgaatcatctggtaaaaatggacaaaatttagttttatcttgtggtctggaaatacaccctaaattattgggtcaagttagtgaaaactgttaaattgattatgaacgtaggcacattacttataaatccccttatgctaacttaaaacttgtgaatgtttagtgttatccagctataattcttctaaacatgtcttgtaatttttaagtttgcatgaaaataactccatcctgagtatactcatttcaataaattatttgtcctgagcatactgtaagaaatttagtaaagtactaattgaatttagtgattagactgtgattagactattacaaattcacagtgcttgtacaattcagatattattttgctttgaagtcaaatagaggaaccttaaataatttaaataaaaataattgtttttattaaagtttatacagcaagataataaattcactaatgtgaaatgttgatatagtatgtacaacttgtttcttaagttactaaaaatgtattttcctacctacataatgtcaatctctattgctcctaacacatgagtggctaaaattgcaaacttaatcacataaataatgagattaaagttaaaatgaaaaagtggtatgaggactattgtttgtgttaagtgaaattataccttgtaaaatttcatattatgagagcaatatgtaaatttcattgcaacaatggttattcaatttactgatgaaaatcagaagaatgttgaaaaattagtgcatttataataaatttaattattcataaaaaattaacattgatatatatattcataaggataaaagatatcaaaataattaaacaaatttcactttcttcttataaaagaaaataatttttatggtaactaattttagtagtgcatcagatcaacactattgggcacccagttatttggtggtacgctgagtgaaaatatgtagctttatctacattaccttggtttggacaactgaaaaatttgctaggaaacaaatattacaaaatatgttgttaacttttcaaagatgatcggtttagattgctttaacttgaaggacacttatattttgtatcacttttgtagcaaacacatgactcatcattgcccaaatcaattgcccaaatcaattcaaacatctcattgtagttcatcccatggcagaaaagtgtttatccacttagtaaaatggaaaacactagagcttcaggtttaatttgaaattttaacttcattaagaataaacttgacctgtttgttctagtaagtaaaaacactagatacgtaccaaaattgtcttttgaccctctcagggagtcaagttttgatttgcttgaatacaagcaagtcgagctatggtaatttgcaatgctgacaggaaagaagaacttgcttgaggcaaaatcatgaagtacaacttttcctctgcatccttttacctcatgtttgtaacatttcccctgttgttatttttacacatctggatgctcagaaaggcctccttaccacaataattgaaaggagtactttgtcaatagtcagaattgaatgagagataggttgttgggaatattcagggtgaatgtgtcttttctactttgactatatttaccattgactacagtaactcagcagaaagttagagggcagcatacatacattggtttatggatttaatgaaaatatccccaaccattacattacagacaattcatatatatgtcttgaaaatcttcttgacaatttgtgacaaattttctaaatgtttttccaaaaatagttggttcttgtaagtgattttgatatgactgattaccaaattatggtgggtaaagatgccacatgcaacagaaaatgtgtctaattatgtttgttttagagcttaagaaatgttaagaagagaagttacaactgcattaataggattttaatttttattcaaaatggacaacttatttattatgtacttctacacacagctaagcttatagatattttcatttaaagaaaaactatttgttcattttattagcagatatcaaatgcccttttgaaaattgagactgatttctaaaacaaaaaaaaagactttaggagttttaattatttttaatatattgcttctttattaaaaaaagatacaatccttcaatgtcattcaacagtattaattgttaaagtgtgggatatagtttacattaccgagtttattttctaagggtagtgaataactcctgacaactactgatatcgtcacatggtcctttagtgaccaaaaatgcacagttgtaagaatgcaagtgttacttgtattgaaaaccggattacattaaaggatggacaattatgataaaggatctgagataattggacaattatgataaaggatctgagataattattctaactttttggaactatactttcactcattgatgaagtaagttacaacgtggaataacaaagtttaagtgtggcagaaaatacatacatatgtttaaaagtagggaaaattttatcaattattaaagatggaaaaaataggactatgtcaaatagttaaacaaatgtggggtattttatggagaaaagaggcatgtactaccttaaacattttccaattggaacatactatagacaaaactgacagattattattcaatgagaaacctgactcagatgaagttacaaaaaaagtactttttaaatgtctagtttctaatagagttagagctttgttgattgagatatgtggaactgccacatatctctgtgccatacttttggtaccttcataataaacggtaaagtgagggaaagggtggaagagacaaatcctacgtctcttccagaacttcgagtgcactataaattaaatatttaaaatatttttgcaatagttagctttcaattatgaacactctcagcctctattgctttatatatgcatttattttggtaatttttatacatcaaaactataattacctgtatttgggcagaatgatttaggttatgccagctattgtggttaaagctgtagtaacttacagtacattgaaattatagactaaggttctgaatattggtaactcactgttgttgtgcacctttaaacaactcttaaataaagtaatgattctctttatattaaatttaatgtatgtgtgcctcatggaaatttgtattttatagaaaaatattgaatattttattattatgtctttggctcacctactttaaggagatggctacttagggtactttttaatccaatataatgtgaaaatttgatcatgctatattcttaatttaattgtacttctatggtcatatacaatttacctatcactttctcacataatcaatttaactttttggtaaatcttctaagagaccgtctagacagagtgaaatgaaagctgaaacaacagtcaaatcaaaaactgctttggtctcaaatccatgtttttcagaaaagatattcagatccagttatctggcaaatggtctcaaacatacatttcaatttcaatgttaaaaataggatattaaacatctcagaaaatattgggattattgaagcaaattctaccctggacttggagtaaatgtgatgaacagattaatgaggtggaagggactagaactttgggaaagtgcaaccttgttatcttaatatttttatagcttagaaagagaatgctatgcaactcatattttgatcttttaatgttaaagaattcaaataaaaaccataaacctgaaactctaaaagaaaaattctgttttgagagagatggcctcctctagtacacttttaataaatttaaagtatctaaaaggatgcacaaagatctctaatgtgctgtgattttcaaaggatgtcatgtataaaagatttgagtgagaacatgaaagcaaaagcaagttcagaagaggaacacaaccaggaggacagtgtgtcaggaaaatccaagaataagtggaggtgtaaaggctaaaaaataatgcaaatggtgcatatccttctgtctttctctcatacacacagacacacttacacaacacatatacaaatacatacatgtatatatgtatatatatacacaaatatacacacatattcacataatattcaagtatgtatacatatatacacatatgtacatacacatatgtatatatacatacacacagattgagagattaaccatatgtagatacacacatgcacatatgcaataatgaaatcatttcaaagcatgccaaaaagtaataaaagatatatcctctgtttgggataaataaaaaaaaagtttaaaagcaaacaaaaaataaatggcaataactaatcacattgaattttgttatggcctttttcttcctaaaaagaataaccccaatctgaacaaagaaattcaaagtaatggaaaactcaacaatgaaactcaaagtagactagcagataagatacctatttcaaacatcagtgccaaggtaatttataggtcagtgcattgataacttttgccaatgatagaaaagatgccagagaaccggatcctgacattaaaaaaaaaaagtaaaaagattctgaagactgcatttctgagcttaaggtagattctaaacaacatcttagaaactaggaaatgactttatgtttctttgtttttcaatgtaaatggatcaagatttcttaaaacagaaatgaatattattatttgtgatgagagcactaggggcaattttgatatttttgataaggtttctagagtaataaattagaatgacaggaatatatattgattttaggaaagtgtctgtataattccacatgatattctctggacaaaatatgaaaaggtaggctgaataacatttttaaagggcagtaaattttataattgttattgattacaatgaaggcctctggtaatgttttccagggtcatatcctgttacatatacgtgacatggataaaaaggaaacaaatatttattgtgtgcctagtttatgttatctcaattccagctctacaaggagctacaaggtaaaattgctacctttaaaaacatatgaggtaaaattattcctattcacagatgtagaaactgagtttcaagaaggttaagtaaatttcctcatattgggaggctggtaatgcagaactgggtgtcaaaatcaagtctgtatgaaccttctgttttgtctcccatgaagacaaaaggcatgcatataaaatttgttgaaacacaaagctgaggaggcataataagacgtggaatgacagaagcaagatctagaaagtttgggatcatgaatcaaaagaaacaggataaaattatcctaaaattaatattaaatcttacaagaaaccccccaaaatcagttgaatttgtacaaaacggtaaatcattttatcagtagatcccataataaatattataaagtttaagtgtgagctctattactcagtaatatgatgccattactgtgttgatggatgtattgtcaaggaaaaagaagagaattacacactgtttccttcaattgttagatggcactggatgtagtgttttcaatgttaatcctggtatcatgttctttgccataaacttgttgacaaattggcaaatactgacatgaaatatgccaatatttgagcatctaaaaatgtaggtactttccataccacatcatatattacaatttgaaaatgtttgtttcattttttatataattattatacagaacagtttttctatgatagcattataaaaattcccagagaatactggcccagtaagaaatggaatgttcacaactcatagtgtagctatatgaaagaaatagatctaaacgacaggttggtttccaaattatattttcatacctggaaaatatctactttataaatagcacaaagttatagttttcaatgaatatgaaaaagttcttgcattaacatattttatgtatcttttatattgacatttgtgattgccactaaaatgtgtattttctaaatttcattgtgcttttacaagatacttttttctttgatgtccataactgctgaaaaggctcccctaaggagaattttaagactaagtaaggtttttagtgagcttaaattatacaattctgaggcattatttaaggtgcatactgtattttttgcttgaaacctgtcagcattttatttgtatggcaattaaatgactcagccattcatgtctcatgccagtctttttcaattgttatttttaacaaagaaaattatatatatatgtatatatatattatatatatgtatatatgtattatatatgtatatatatataaacttacagcaaaaatgtttaaaaatagcaaatagtttgagtatagttaaacctaataactgtacttttgtttctatgcctctgagacaagattactagacccttattcaaagtttctaaatataggaaatagaacattgggccatgctaaaaaaattgttcagattttcttttgaaagagaatagttatttttcctcctgacctctaatgaagatgctttatttgtcaaggtgttttccttagaaaattgacccagtgtcaactgtaaagaaaacatagaggatccttggatgattgaccaacttatccaaacacaggtttagtaaagagaggatataaagataaaatgtgaaatgacctctctgagtcacatttgttttcataatttcctagcaaacatccaacttcactgctaccctcagcaatgtttcttgaaacatttttaagacattgatagacaccaatagctgatctttagaaagccattcccagaagaatatgtaaggggttacaactcatttcagggagtctgcctagctcttgatattacatgtctttggcatacaattgtgtaccttttatcattgacagtgaagaaaataatgccatttgtaacttctgagatatacacacaatactatcaactagccggttaataaaagataagaaaaataaagaaaatagaacatttttaggtgtctggcaagtatcctctaaatcaaggtaaagataataatttagtggcagtgttcatattttcctatgactgtaagatttaggtgcctcacaaaatattaatatttagcctcttatgaaaggttcgtttttcttctaacactttagtagctgaatacaaagaaaatacacaacagctgtttataaatgaaataaaaagtttccattttttatctgagtttctcatttatttgcagagaacgaataaaataaaaatatcctagtgttgtttgcaccacagcataccagtaaatcttaaggattgtgtttcagtatgaaaaggaagagcaggaagatttcctcattctgtcttaccagcaaaagtctagccttcacacacacacacacacacacacacacacacacacacacacacacacacacacagagtcatctatatgaacacgtacttgagtttcttaaacatatatgaagcaccttccatttccctttataataaatcccttagtttttgctgttcattaaaaaacaaaaaggaagagacaagctcaggacattctgaaaaccaatgtctttaggacacactaaggtgtcctgaattactttaacggacacattgtaaagacacactctccaatccctattaggaaaagtttagtcaagtttgcttactatttgggtgcttataccaaaaaagcatcatttaggacattatttaggataatattatttatgcaggaattgtaccacctatttccagatggtataacttattatctgacaggcatgtagcaaatagaacacaaagcataaatctgtcaggagaaatcatacgagaaaaagagcattgtctggttatcagaatatcagatctctcattctggccttgctaggaaatagatctttgattctagaaaagtcaactaatttctatggttcttacttttctcctttataatatacccatttaaattccaaaaaggtatatgataaatcacaataatttcaatcacatggattttaatacaaaatgtataaaatcaatttccaaaaattttctgcatatactgaaaatgtctgtacgaatgagctaactactataggccttccctaatttattctattaaatgtgggtactcaatgtaacctgaaaatattgagcttaactcttctttttttttttcaaaagggaaacttgaaaaagactgcttcccccagaaaatttatcaacaataggtgctcaattaaatgtttttaaacaatgaacaatatcccctttcatataaataatcaggggagagatatttttaagtcttttttttctttttccatagtgtcacctacacaaaaaattatgtaaagacaccacttctatgaggaggtattcattgtagatgtacagaagtcaacggaaacttaagtttacagaaaaaataaaccagattatcattccacccaactgtatattcccacagatgcttaataaaagctatctgatgatataatgaattatcagttcttgaggaagtatatacagttggtgactatttttcaaaaatcatcatccaacaaatttttttcatttaaaatctttcatattaccctttcgacaatcagttgaaattttaaaactaagaacatttaaaaatataaatgaaagtagcattagctatagactgatattcaacttcagacgttaaaataaatacaagtgtgtattaagagtaaaattatgtcaacaatgtataaatgaaaactgccaatgtaattaatgtttcttttaacatatcccatccattgctttccctccaaaagacaaaggtagcaaaagacgaagcaggaagaactgcttcagaaactgaacatactgatttaattggctaagaagtccaaatgctaatactcctaataattagccattccttttgtgttttggtgacatatatcctcatacaatgtatatcaaatggaattttttgatttacacctgacatttcaaagtttccatttttgaattctcctagtcttaagtaagtagaacattgtctcctttgtttgctaggcataacgttttccccaacatctagggctccatgatgcaaaatatcattttgccgatcttctgttccagtatttactttaattttttttattataattggattttcaaatacaatcacaaaaacatctcctgttgaaggtggtttcccccaaaagtactcatcaacactactgtaagccttgcttgcttcataattttcaaacacattcatgttggtgtacagacttgcaggggggttatcaggaatgtcaaatgactcctcttcaaaatcatcatccttcagcttattctccgtccctttgtatgatgaataatagcccatgtgctgaaagagagatggtttaaaacggatcacatttttctgagccaacagaccacggaaatgagtcaatagccaatcacaaggcatttcttgataaaacattaataaaaaatgggccaaacgtgggagatcatgagaatgatagagtttaccaatgtagccaagcttagagaattcaagagttacccagtaagttccttctagggatgcaatgactttcttgatggcagttaagaaattttttgaacatcgaacatcatcttcaagcattacataatagtctgaagtattggcacaaaaattaagcagaaaagcataatctacattttgcttggaacgaaatttgactctatcttctggatcattgtaatttcttttaaggccatctaggattgggtaatactcctctggagcatgtataaccattaatcttcctgcaataatatggtgcgcaaatttctgtgtaatatcctggaccatggcatcacgccaggaagaattaaagtctgctaggtgaaccaccactgaaatttccttcagctcttcatagctggattgctcaaaaattgacttaattgtctcaagtaaatagtttcctttttttcgctttactgaagaaagtccaattgtaagataccgctttctttgtaaaggtgtggcagctaggtagcgataggtgacatttatggctcctgagaaattagataaatccttgaaagtatgaacatagcgttctgaattcagttgatgtgtggatgtttcccttataagttgtttgtctccttccagaacatagctatcttcaatgtacaagttcataaaaaggagaaaaatgacaagaactcccaagaatgacactgtagaacgttttctcaggcatctcattttatcaagtatttcaaaaatatgtttcatttgatgaaatttaaacattctcttcttaagaaagacgctgtcataatctgtgctgtacagaaaccgttgataccgttttagtttctgtagagatagcctttctcacgcagaatcagggctgtgctttctgggtgagtcagagtggataaagcttcaaccttgctatagcgttttctgcagctcttgtttgaaagacagatccacagcagctttgtgcatacaagtgatctggctgatctccagttcttttgaaggcccccgtcatctgcatacgaatgcttattcgaggaaaaggaggaaagaaataggacccatccaagtagaatgtaacagcagctgagaagcttcagagaaaacctgcccgataacaataatccattagaaaactggcaatatcctctgatctattgcccgcaaagccatgacttgatggagagtttcattccctgggctcagttctccagaagaaaatcagcacaatttaaatatttcttggaatgtgacagctctctagatcccgggttgcattctgttccccagggatggcaatctggtgttcctgtgtgcatagagcagtgaagatgaattgaaaacgcttgagataaattaggaatggctaagttaaaattgtctctgctccagactctctcatctgcagtctgcaagcctgtttttctgt

SEQ ID NO: 13489 - RNA, 22709 nt, Homo sapiens
  source 1..22709: mol_type = other RNA
gctgggattacaggcatgagccaccacgcctggccagtttttaaagtatttcatacagtgtaactaggcagtcagaaatacctgtatctcaaattcatttaacttttcaatgaatcaatcttcttattttctcagacatataaattatcataatactttacattgagtctctatggttgactatatgctgtgaaggaaggacataaatacatgtgaggaaacaattattgatatttttaaactaactagaaagcaccaagttatttgttaaataaacaaagttaattttatctacctgttcagtaagtgttggcaactatgaattaatctttgacaaattcacttacaactagcaattttaaagacttaaagtttaatttttattattaaaagggtatgattatttttactaaaattaataaaaagattaactgttactaaattaaagctccttcaaaaacataaatgtattctttagagagttaaaaaaagtagcaataaaatacatttttaatttagttaagcttacttaactaatgatcaaatagattaagttgtataaaattttacaaactttatatttttgcatacacttatcttcctggcatttttgaaataaaaaaaatacaagtgcatagggcagaggaggcgattcagttacttctgctatgttattaaatctctggtaaccactatacaatacaatacaatacaatacaatacaatacaatacaatacaatacaatacaatacaatacatgtagactcagcatccaaactttattttaccttcaagttctacctgataaagtggtggaataaagatggtattttccataactgtttaataataatcacatgttttatacccattgctttgaagaagaaaccttaagcaactagaaatgtcaatctaaaaggcagaaaagctggaaaaatctcatgaagactagaagatttacactcataagatcatgtaaatttatttggatatgctgaaaaaagagggggtataaaatctaaagtttggtaaatctttgctttacagggcttcaagttatagatttttcttttttccttttctcttcccctttctctctctttctcttttttatttttgccatttcttctcaggagcccctgcaatttcaaaccttggaattgaattggatttgaggaggaaaacccatattcagctttaattcaaatgaattttactactttagacaaaggtacaacactctattcaaaaaagttattgaaatcacatctttaaatctgacccagccacttgaataaataagttgtgttgtagtttctcagagcaaccgccgctcatctttcactcaccttaacaatttctcacttttttctgctttttttttttttttattttctgcttgctgaaatcgagatcaatattcattgttttcttctgggttaactcttttttatgttaactgaatcaattttggctttgtttctttatgaaattacttttagataaagtattgatattgtcatttatcaattttattatatgtcttttgcttattaaaggattaaaatccacctctaaacttatttagatcaaggtcagtttttttactcctctgtagaactgtgaagataatatcctattctccttttcttatggttttattgtgaagatctgtgcaaatagctatataaaatgcaattcggtattaaagaaaattgttgcacggactacattgattagagtctaatttttggaaagtatacttcgccttttcagtaattttatttttcggtctatggtgcccacattgtgtcaccagccagccgtatgcagacttacaaaggactacccactaagaataaaaacatgatacaacttgaagaaattttcatcaaacgtctttgtcttatccccttgttatacagacaaagatgacaagggccgaaaaggaagtgattttctcattgaataagagaatccgaactggcatcgaggatatctaattttgggatgaaaattgagagaagacagaatttcaagtctgaattatgacttcactactgtgtcgtcattggtagaataaggataacaatacttatcacacagatttgtggtctgaatcacatgagagacatagatgaaaaatgtaaaacaacaattagcatgtgacatgctctcagcaaatcaattaatccttcattctttttttctccccttactcctttgattttcagactaatttggatcatgattattggcctgtgtcccacccattattcacatatagaatgggttgcattatcctctccttggaaatatctttcaaagtgggtaatgagaaaactactttgaagactgtgctgaaggaaatgatggcatgaacaactctagataatttttgtttatttggatataacgtgaatgggcccataccataaactcctattaagctgaatcaccaaaaaaaaatttgatatgaaagtcatacattgaaaaaattcactcttaccactgatttgattgatactgagcctgtaaatatttatttatatgatgtttggcactttattttataaaactaccctttacttaaaataaatcattgtattcacataactttccagggcactatgcatttttaaacaagacagtcaacttactatttaaaaaacaaagtcagtcacctaaatgactttctgactataaatttgaaaacaatattctccttgtaatatatgtgccaccagggcaagaattacaaattgggagcaggtaagaaaattgttgttgactctcattagtattctaattctccttcagtcagatttataaagtatgacctatagcatccaactccatcattttccagtcattcttgagactgtcaactctatgggcattgtttagcagcctcgaaacactgaactttttacagtcttattggagagaaaaacacattaaatgatcaaataatcttttatgagctcagaaaaaaatgcctaacatgaacatttaagcatcttctgtttctgtgattcccatttttggagagtaaaaatttaagaaacaaagggaatgtgtctggggatggtactaataatattgagattttacaatttaggttataatcaagataattatgtatatatataaaattatatatggtatagtttcaacttctaatcttttatcatcctctaccacataattcctcctatattctctttttctgactgtggcctaatacctcaagaatattgtatatgcttgtcactatataaacttcaccctaaggaaatttccatgtcagatacaataagagcaacggaagaaaatgtatcaaaacacatctccaatttatttgaatttttctggcctaaccttgttggcatgagagttcccactttgtattataataggcaaattgatacacacttttcatttattctaaataatagattagcatagtcaggaggcttggattggcagctattaaatacaatttgaagccgtgggattttattaggattctaaggttattctgtgacgatggaacttaatgatgtaagagttaattacccattgtcaaaaatcattgcccatcaaagcagtgagactgtgtgctatgtccagttttattcatttcttttgtgtatctgaatggaacatgtggtaaacacaacagtagaatatacctacagtccccttagaaactcttaaatcttcaatttataaaagtcatcctaagacgttaaaaataacttacgaaaggatagattccaatgtcagtgggtgagatgtgctctagctagtgtgcacgaaagagaacatggagttagaataattattgtaggactgtagattgtcatctcaagatcagtgtcaaatacattcattcatgtagtattttcacatgcattctggtctaaatatcccaacatatctttcgttttgagatctgcagaacaaagtcaatgtctgaatttagagactaatttgaccattttgattcaaatgtctaaaggctaaaccagagcaatttacaacatccaatgaagtaaaattatataattaattatataattatataattatataaaattttataattaattataaaataaaatattaacaataattgaacattgtttacttttttatcctcacaacaattcaacatgatatgtatggttattactaaatgtataatacatttagtaatgtgatttgacaaatcacatttgtcaaataaggaatggctgaattaaatgattgaatgaaggagtgaaggatgtagattgtttaagtacattcaacttgtaatgaactgtaaacttcacccataacattattaatatatcagtgctatcaactacattttacataggatgaaaaaaatcattatttttattaatcccaagatattttatttcattatataaatgaaatattttatctgttataaagacctttatttttgttccactcattaaataacatggtaagactgttgtgtaattgactgaatagttaagtctaaatgggtaaatagctgtttatgttagtattgcagggtagctatttgataatgaaatatacttttcttacctacttgcaaaaaaaattacataaacaagtatttcctagagttcaaacactgatctttttaagtggcaaattgtccaaaagaatttaattaatataaacaataaattcacttaaacaactatttacatgcaaaagtaatatttttattgcccatttggaaaatagttttgctttctggtttataaggaacttttactagtttaattacttgggtgctttaaatgttttttggaggctattacaaaatcacatcctaaaattttaaaatggaaaaattataataattgaatttttaattcctcataaatattttaaaagtacacattgttccatggcttttgcctttagaataaatacaacatttttatgtagaaatatattcttgaaatgtaactagcacatagtcagtgtttcttaaccattttggggtcctgaaactttttgataatgatgaaagcacagagatgctatcaagaaaaatttacccacataggaacacacacacatacacacagacacacacagagtttgcttataagctcaggaagcttaaagatctgctaaagattatgcttgggtttgccatgaatcataaataccaagtcaaatacctttgaatttgattcttaacaaatctttgtggctgagaaaccatgagatttcattctggcatgtccccagaatgtaattatcaatgaacaatagccattgaaaaaatctgaacagatattattgaggctcaaggttgtttaatggcacagataatataattcaaatcatgaccccagggctgatgaagtcttgttgtaacgtgtaaatggggtgggtgatgggagagagaaaacaaaataattatttatgttaaatcatacataaacagtaaagccaacacaataagtaaaataagagaaagtagaatgcttgggaggtcatatgtttcaaatgtatgcatacacaaaagagtaagcaacaggatacttcaagagtaaaatgggaaaaaatcatattgggtaaatagtatcaccccaaagtgatagtcaaaagtacctatgtttgcctagttctcagattacaactatgatgataatttagataaacaagcagaaaacaaaactatagaaaaaagtcaaagtgacataaaacaattactggtgtttcaacagaaataaacccaacatcaggatttatcaaatatatgaaaaattatgaaagattataaaacaccaatgattagattatgttataaagacactatgaagagatactaaatgatattcttttcatctgtggttactgctaaaaaattctttcatagaaattcttggattttgaaattagtttaattccaaaatattttctttattttgcaaaaatgtaagacaaatgtataggatatttttctctgttgttatgcaaggatttattatcacattggccacagaacacatagaatgttagttttgtagaaaattttagagattttaataccaggatgaaataatagtatcattctatttcaggttcttaagcaacattcctaagactagaaccttatcttgaaaaattatgattttaaacttaagggaattcaggtaaaggaaattgactaggttaaggcaaatacatcatgtttactggtaaagataacattatttaaggaaggtaagatactcttatcctacatatacgccagaaaaattgcttctcctctgaaaactaccattatttttgccaaatattgtagcttagttttaagtttttctcggctgtttcctctgacagttctgtggtaaagaagaaacattataggaagcatttttttttcctacagagtctgccatatggagaagtagaatgagaggccacctaggtaatgtgatttattaaaagttctccatcccaaaatatatgtcccatctgtgggctaatgtctgaaagtcctatgattaaactcacttttatgtaagatagtgaggccccagagagccctcgagaaatgcaaataaactattactgacctcccttggattatgatgaaaaccgtggagtctttctattctctgtcaaatgtggaggtcatggatccttcttggcacctaagattaaaactcatagaatgtgctttaacttctgtaggcacatttcctttccaattagagtgaggtgttgaatatttatttatttgtttatttttattatactttaagttttagggtacatgtgcataacgtgcaggtttgttacatatgtatacatgtgccatgttggtgttctgcatcttaagagaagactatttataaaatttattgcttgtaagatttgttttttgttctcttactattatgaaaatcacgaacttgggaataaggacactctgggcccggcgcggtggctcacgcatgtaatcccagcactttgtgaggccgaggcgggaggatcacgaggtcaggagatcgagagcatcctggctaacaaggtgaaaccccgtctctactaaaaatacaaaaaattagccgggcgtggtggcgggcgcctgtactcccagctactcgggaggctgaggcaggagaatggcgtgaccccaggaggtggaacttgcagtgagcggagatagtgccactgcagtccggcctgggcaaaagagtgagactctgtctcaaaaaaaaaaaaaaaaaaaaaaaaggacactctgaacaattgaacaagactacgctgaaaggcagagaagaagtaattatgaacaaactgttcatgaagtgatcaattgaatttgaaacagaacttttcctagcttctaaatgattagaaatttcagctttggtttaacttaaaaacttagaattgtcaattctgtccaagtctctgagtcatgtacagaactcaaattattacatcatttttttacttatctgtattatttctccatttaaaagtggacaaatttttatactatatcctaataatgatacaaggtgacttgtaggactctggatagaaagagatggcccaggatacagagggcactccttaaatagctgccaaataaatgacattaaaaaatgtataaaaaggtatgttaagtaattaaaagtgtcaggcattattttcctattatgagacattttatattatggttatttactgtaattgcatccaaaataattcataaaacatttatttttgtactattaaaaatctaaacaataataaccagatggaggaaaatgataccatctgatttaattattaacttgaaggtcagtttctacaacttattctcatttatgtttatctgatttggccacagtttcttactttctcatattttgctaagcttgtggatgaagccgcatgtctcttttttttttaacctggcatataacactgtcactctatttaattattacccatcatctacctactttgaaactttggaggttttataaaaattatgagtatttaatcaaagttgtctctttatcatttgccagtgaaaatataaaacctggctgttttattctattgtgcactctaattacataaccaaaatctttttaaaaattcttagttcttttagaaataccatttgacccagccatcccattactgggtatatacccaaaggattataaatcatgcttctataaagacacatgcacacgtatgtttattgcggcactattcacaatagcaaagacttggaaccaatccaaatgtccaacaatgatagactggattaagaaaatgtggcacatatacaccatggaatactatgcagccataaaaaatgatgagttcatgtcctttgtagggacatggatgaagctggaaaccatcattctcagcaaactattgcaacgacaaaaaaaccaaacactgcatgttctcataggtgggaactgaacattgagaacacatagacacaggaaggggaacatcacacactgggcctgttgtggggtcaggggaggggggagggatagcattaggagatatacctaatgttaaatgacgagttaatgggtgcagcacaccaacatggcacaggtatacatatgtaacaaacctgcaagttgtgcacatgtaccctaaaacttaaagtataataataaaaaaattcttagttatttgaaaatagtttttttgaattcacaaacttgcaggatgaaaaaagttattagttcctgaagatataacattgatttgtctttttcttatttgatatcagctagcagtaaaattgtgaacaaatctggtaaatcttttggtgttgcaggttcataatcagttaattgagtgtattcactataaattgctttaattaagtgatgtttgcctaagaacaagtttcatttcatctcatgaaaaaaatgttactttttgtattaatcagtggaatgtttaaagaaaaaactggttatcttgaagctgtcaaataattataagaaatctctatacattacgttttaaaatacataaaacccataaattcaagcttattagttttcattttcagcaaggtttatacagagaaaataagtaatacaaattagttttccagaaaatctaattttatgcagataaaatctgaaaatcatataagtccaagatgaaactgatctcaaattattattttgaggtgtatccatttatttaaaaaagcctcattttagctagcaacactatgtagaaaaatattttaaataagacagagcattaaaataatgtattcattgatctcataaagaatagatgatcagattttttaaaagtgattttaattaaatggacatgtttctctttagccagaaatgactgagaaattttgagttggaattgatataggggaatccttggaactatgtgtgaatatgtgtgtgtgaattatctgtgtatatttacataatttacactattcacagtccttgtttttcttgactcaaatagctatctcaagtttcgtacactttttagatctctatgtaaatacattatttcatttgtggaaatatattgaggcctatatcaataacctcaaaccttttaaacacttagagcaagtcaatatgacttgttctgtttcagctatctgaaatttaaaaatttgacaaatttttaaagtacccagttcttggaaaaagaaaaacaaataaattggagatttggatcatatgggctatgactaaatgagacaaggcatacatgctgacatttgaaggatttatgaaaaaaagtccactgtggaaaactgatagtttttctccttctttcttgaatatgtttagttaattttgtggaaagaggaaggcagctcagtttacaaacagcagtgggttgaaggcaatgctgtttatattcttgaatttcaatatctacaaagatgtcatcattagattttatgtgttaaaaagtggatttatagtctctaattaataaggtgcatatgtcaagactcaggaaaacagatcacttacgtagttctccaaaaacgagagtcccagattcaataggaaggcatgcagagtgttctctataaacccagcaaaaccataaaaattgactggaacttttatttttcagtacaacaataatagtattgaaatacctaaaaagggcaggaaacaacacagaataatctacgcttgtcatcatgttttctaatctataatctttcaaactggataaatgggaagttttggaattttactgtggtacagtcttagttgctccgtggttgtcaaatctgtctgcacattaggatcacttaggaagaattttaaaagtatgctgatgcctggaaactccagaacaattatgataactctgagcatggagctcaggaatgggtgaaattcttccccagagatgttaatgaacagccagacttaaaaactagtaatttagacaagtgtgagcagaggttaataatgttgagatgaactgggcttaatatttcactaacaaggtcagagttttgatacatcacttaactcaaactttgagattcttcatcactgaagtagcaataataatagtcatttctgttttaatacttcatagacttgtaaggatgtaatgtagtgtttctaaaaggagtgaatggacaatctgcatcagtgttaactaaaatacattgaaagtgccaattcctagatctatcctagatttacagggaagaattcagtagtctgaaacacacattttcaatatattgaaaagatgattcttttgcatgatgacttgttataatcattactttcataggtaatggaagtaccgattaggagagtaccaaatacatattaaacactcagttcatgtaagctataggccaataaacacaactttggggtttactgatgttttccaacatccgaaataatagctgaaatttagaaacatagttaatcacacaaaaaatgttgcatacatactgtctaactaccagtttggtatgtttggggctggtgttatgaaagactattatatgattaatacaaagttataatttttggagtcttttagtgtacccagagcccatgagtttttattttctttttggaataacagaaattaggttgtggttcagtggaattacagaagcaagtgttttagatgttcaagtttaaaaaatgagaaaaaaatgttttacatgaagaaactaattatttaaattcatttttcaactatttaatgttattttaatatagtcatatcatccagaaaatcccatcttagacaaatgggttttcaataaattattattatagttaggaggcaatgtataatagtgataaggggcatagattttgaattacacaaacctgaaatccaatgctctctctttcatttattagttatgtgaccttggacaagttagtaaaaccctatttttcatatgctctttagcttttttaatacctcttaccttatatggttgtttaatctattaaatagacagtgaaatgcacatgaaatcttcacacagtgtctcatagttgcttggaacatatttatgtagtaagcattgttcttggctgagcttacattaagtgatctgtaaattagaagttatttgttatatttgtttcgtttccttattgccctagatgccttttctctggacctagataatttagtctcactctgtggcctttacccttcaataaatatggattattaatataatttagctacataattcctaaggaaatattaattcataaagattgttaaattgaactgaatatctttgctaagtcacaggcattgattaaattagataaaattgtcattttccattgattttgtttatataaataatattgaattatttatattcttatttagtctagtagattgacaggcagttttattaagaaatgaatcaaatggtaaattttgaatcatctggtaaaaatggacaaaatttagttttatcttgtggtctggaaatacaccctaaattattgggtcaagttagtgaaaactgttaaattgattatgaacgtaggcacattacttataaatccccttatgctaacttaaaacttgtgaatgtttagtgttatccagctataattcttctaaacatgtcttgtaatttttaagtttgcatgaaaataactccatcctgagtatactcatttcaataaattatttgtcctgagcatactgtaagaaatttagtaaagtactaattgaatttagtgattagactgtgattagactattacaaattcacagtgcttgtacaattcagatattattttgctttgaagtcaaatagaggaaccttaaataatttaaataaaaataattgtttttattaaagtttatacagcaagataataaattcactaatgtgaaatgttgatatagtatgtacaacttgtttcttaagttactaaaaatgtattttcctacctacataatgtcaatctctattgctcctaacacatgagtggctaaaattgcaaacttaatcacataaataatgagattaaagttaaaatgaaaaagtggtatgaggactattgtttgtgttaagtgaaattataccttgtaaaatttcatattatgagagcaatatgtaaatttcattgcaacaatggttattcaatttactgatgaaaatcagaagaatgttgaaaaattagtgcatttataataaatttaattattcataaaaaattaacattgatatatatattcataaggataaaagatatcaaaataattaaacaaatttcactttcttcttataaaagaaaataatttttatggtaactaattttagtagtgcatcagatcaacactattgggcacccagttatttggtggtacgctgagtgaaaatatgtagctttatctacattaccttggtttggacaactgaaaaatttgctaggaaacaaatattacaaaatatgttgttaacttttcaaagatgatcggtttagattgctttaacttgaaggacacttatattttgtatcacttttgtagcaaacacatgactcatcattgcccaaatcaattgcccaaatcaattcaaacatctcattgtagttcatcccatggcagaaaagtgtttatccacttagtaaaatggaaaacactagagcttcaggtttaatttgaaattttaacttcattaagaataaacttgacctgtttgttctagtaagtaaaaacactagatacgtaccaaaattgtcttttgaccctctcagggagtcaagttttgatttgcttgaatacaagcaagtcgagctatggtaatttgcaatgctgacaggaaagaagaacttgcttgaggcaaaatcatgaagtacaacttttcctctgcatccttttacctcatgtttgtaacatttcccctgttgttatttttacacatctggatgctcagaaaggcctccttaccacaataattgaaaggagtactttgtcaatagtcagaattgaatgagagataggttgttgggaatattcagggtgaatgtgtcttttctactttgactatatttaccattgactacagtaactcagcagaaagttagagggcagcatacatacattggtttatggatttaatgaaaatatccccaaccattacattacagacaattcatatatatgtcttgaaaatcttcttgacaatttgtgacaaattttctaaatgtttttccaaaaatagttggttcttgtaagtgattttgatatgactgattaccaaattatggtgggtaaagatgccacatgcaacagaaaatgtgtctaattatgtttgttttagagcttaagaaatgttaagaagagaagttacaactgcattaataggattttaatttttattcaaaatggacaacttatttattatgtacttctacacacagctaagcttatagatattttcatttaaagaaaaactatttgttcattttattagcagatatcaaatgcccttttgaaaattgagactgatttctaaaacaaaaaaaaagactttaggagttttaattatttttaatatattgcttctttattaaaaaaagatacaatccttcaatgtcattcaacagtattaattgttaaagtgtgggatatagtttacattaccgagtttattttctaagggtagtgaataactcctgacaactactgatatcgtcacatggtcctttagtgaccaaaaatgcacagttgtaagaatgcaagtgttacttgtattgaaaaccggattacattaaaggatggacaattatgataaaggatctgagataattggacaattatgataaaggatctgagataattattctaactttttggaactatactttcactcattgatgaagtaagttacaacgtggaataacaaagtttaagtgtggcagaaaatacatacatatgtttaaaagtagggaaaattttatcaattattaaagatggaaaaaataggactatgtcaaatagttaaacaaatgtggggtattttatggagaaaagaggcatgtactaccttaaacattttccaattggaacatactatagacaaaactgacagattattattcaatgagaaacctgactcagatgaagttacaaaaaaagtactttttaaatgtctagtttctaatagagttagagctttgttgattgagatatgtggaactgccacatatctctgtgccatacttttggtaccttcataataaacggtaaagtgagggaaagggtggaagagacaaatcctacgtctcttccagaacttcgagtgcactataaattaaatatttaaaatatttttgcaatagttagctttcaattatgaacactctcagcctctattgctttatatatgcatttattttggtaatttttatacatcaaaactataattacctgtatttgggcagaatgatttaggttatgccagctattgtggttaaagctgtagtaacttacagtacattgaaattatagactaaggttctgaatattggtaactcactgttgttgtgcacctttaaacaactcttaaataaagtaatgattctctttatattaaatttaatgtatgtgtgcctcatggaaatttgtattttatagaaaaatattgaatattttattattatgtctttggctcacctactttaaggagatggctacttagggtactttttaatccaatataatgtgaaaatttgatcatgctatattcttaatttaattgtacttctatggtcatatacaatttacctatcactttctcacataatcaatttaactttttggtaaatcttctaagagaccgtctagacagagtgaaatgaaagctgaaacaacagtcaaatcaaaaactgctttggtctcaaatccatgtttttcagaaaagatattcagatccagttatctggcaaatggtctcaaacatacatttcaatttcaatgttaaaaataggatattaaacatctcagaaaatattgggattattgaagcaaattctaccctggacttggagtaaatgtgatgaacagattaatgaggtggaagggactagaactttgggaaagtgcaaccttgttatcttaatatttttatagcttagaaagagaatgctatgcaactcatattttgatcttttaatgttaaagaattcaaataaaaaccataaacctgaaactctaaaagaaaaattctgttttgagagagatggcctcctctagtacacttttaataaatttaaagtatctaaaaggatgcacaaagatctctaatgtgctgtgattttcaaaggatgtcatgtataaaagatttgagtgagaacatgaaagcaaaagcaagttcagaagaggaacacaaccaggaggacagtgtgtcaggaaaatccaagaataagtggaggtgtaaaggctaaaaaataatgcaaatggtgcatatccttctgtctttctctcatacacacagacacacttacacaacacatatacaaatacatacatgtatatatgtatatatatacacaaatatacacacatattcacataatattcaagtatgtatacatatatacacatatgtacatacacatatgtatatatacatacacacagattgagagattaaccatatgtagatacacacatgcacatatgcaataatgaaatcatttcaaagcatgccaaaaagtaataaaagatatatcctctgtttgggataaataaaaaaaaagtttaaaagcaaacaaaaaataaatggcaataactaatcacattgaattttgttatggcctttttcttcctaaaaagaataaccccaatctgaacaaagaaattcaaagtaatggaaaactcaacaatgaaactcaaagtagactagcagataagatacctatttcaaacatcagtgccaaggtaatttataggtcagtgcattgataacttttgccaatgatagaaaagatgccagagaaccggatcctgacattaaaaaaaaaaagtaaaaagattctgaagactgcatttctgagcttaaggtagattctaaacaacatcttagaaactaggaaatgactttatgtttctttgtttttcaatgtaaatggatcaagatttcttaaaacagaaatgaatattattatttgtgatgagagcactaggggcaattttgatatttttgataaggtttctagagtaataaattagaatgacaggaatatatattgattttaggaaagtgtctgtataattccacatgatattctctggacaaaatatgaaaaggtaggctgaataacatttttaaagggcagtaaattttataattgttattgattacaatgaaggcctctggtaatgttttccagggtcatatcctgttacatatacgtgacatggataaaaaggaaacaaatatttattgtgtgcctagtttatgttatctcaattccagctctacaaggagctacaaggtaaaattgctacctttaaaaacatatgaggtaaaattattcctattcacagatgtagaaactgagtttcaagaaggttaagtaaatttcctcatattgggaggctggtaatgcagaactgggtgtcaaaatcaagtctgtatgaaccttctgttttgtctcccatgaagacaaaaggcatgcatataaaatttgttgaaacacaaagctgaggaggcataataagacgtggaatgacagaagcaagatctagaaagtttgggatcatgaatcaaaagaaacaggataaaattatcctaaaattaatattaaatcttacaagaaaccccccaaaatcagttgaatttgtacaaaacggtaaatcattttatcagtagatcccataataaatattataaagtttaagtgtgagctctattactcagtaatatgatgccattactgtgttgatggatgtattgtcaaggaaaaagaagagaattacacactgtttccttcaattgttagatggcactggatgtagtgttttcaatgttaatcctggtatcatgttctttgccataaacttgttgacaaattggcaaatactgacatgaaatatgccaatatttgagcatctaaaaatgtaggtactttccataccacatcatatattacaatttgaaaatgtttgtttcattttttatataattattatacagaacagtttttctatgatagcattataaaaattcccagagaatactggcccagtaagaaatggaatgttcacaactcatagtgtagctatatgaaagaaatagatctaaacgacaggttggtttccaaattatattttcatacctggaaaatatctactttataaatagcacaaagttatagttttcaatgaatatgaaaaagttcttgcattaacatattttatgtatcttttatattgacatttgtgattgccactaaaatgtgtattttctaaatttcattgtgcttttacaagatacttttttctttgatgtccataactgctgaaaaggctcccctaaggagaattttaagactaagtaaggtttttagtgagcttaaattatacaattctgaggcattatttaaggtgcatactgtattttttgcttgaaacctgtcagcattttatttgtatggcaattaaatgactcagccattcatgtctcatgccagtctttttcaattgttatttttaacaaagaaaattatatatatatgtatatatatattatatatatgtatatatgtattatatatgtatatatatataaacttacagcaaaaatgtttaaaaatagcaaatagtttgagtatagttaaacctaataactgtacttttgtttctatgcctctgagacaagattactagacccttattcaaagtttctaaatataggaaatagaacattgggccatgctaaaaaaattgttcagattttcttttgaaagagaatagttatttttcctcctgacctctaatgaagatgctttatttgtcaaggtgttttccttagaaaattgacccagtgtcaactgtaaagaaaacatagaggatccttggatgattgaccaacttatccaaacacaggtttagtaaagagaggatataaagataaaatgtgaaatgacctctctgagtcacatttgttttcataatttcctagcaaacatccaacttcactgctaccctcagcaatgtttcttgaaacatttttaagacattgatagacaccaatagctgatctttagaaagccattcccagaagaatatgtaaggggttacaactcatttcagggagtctgcctagctcttgatattacatgtctttggcatacaattgtgtaccttttatcattgacagtgaagaaaataatgccatttgtaacttctgagatatacacacaatactatcaactagccggttaataaaagataagaaaaataaagaaaatagaacatttttaggtgtctggcaagtatcctctaaatcaaggtaaagataataatttagtggcagtgttcatattttcctatgactgtaagatttaggtgcctcacaaaatattaatatttagcctcttatgaaaggttcgtttttcttctaacactttagtagctgaatacaaagaaaatacacaacagctgtttataaatgaaataaaaagtttccattttttatctgagtttctcatttatttgcagagaacgaataaaataaaaatatcctagtgttgtttgcaccacagcataccagtaaatcttaaggattgtgtttcagtatgaaaaggaagagcaggaagatttcctcattctgtcttaccagcaaaagtctagccttcacacacacacacacacacacacacacacacacacacacacacacacacacacagagtcatctatatgaacacgtacttgagtttcttaaacatatatgaagcaccttccatttccctttataataaatcccttagtttttgctgttcattaaaaaacaaaaaggaagagacaagctcaggacattctgaaaaccaatgtctttaggacacactaaggtgtcctgaattactttaacggacacattgtaaagacacactctccaatccctattaggaaaagtttagtcaagtttgcttactatttgggtgcttataccaaaaaagcatcatttaggacattatttaggataatattatttatgcaggaattgtaccacctatttccagatggtataacttattatctgacaggcatgtagcaaatagaacacaaagcataaatctgtcaggagaaatcatacgagaaaaagagcattgtctggttatcagaatatcagatctctcattctggccttgctaggaaatagatctttgattctagaaaagtcaactaatttctatggttcttacttttctcctttataatatacccatttaaattccaaaaaggtatatgataaatcacaataatttcaatcacatggattttaatacaaaatgtataaaatcaatttccaaaaattttctgcatatactgaaaatgtctgtacgaatgagctaactactataggccttccctaatttattctattaaatgtgggtactcaatgtaacctgaaaatattgagcttaactcttctttttttttttcaaaagggaaacttgaaaaagactgcttcccccagaaaatttatcaacaataggtgctcaattaaatgtttttaaacaatgaacaatatcccctttcatataaataatcaggggagagatatttttaagtcttttttttctttttccatagtgtcacctacacaaaaaattatgtaaagacaccacttctatgaggaggtattcattgtagatgtacagaagtcaacggaaacttaagtttacagaaaaaataaaccagattatcattccacccaactgtatattcccacagatgcttaataaaagctatctgatgatataatgaattatcagttcttgaggaagtatatacagttggtgactatttttcaaaaatcatcatccaacaaatttttttcatttaaaatctttcatattaccctttcgacaatcagttgaaattttaaaactaagaacatttaaaaatataaatgaaagtagcattagctatagactgatattcaacttcagacgttaaaataaatacaagtgtgtattaagagtaaaattatgtcaacaatgtataaatgaaaactgccaatgtaattaatgtttcttttaacatatcccatccattgctttccctccaaaagacaaaggtagcaaaagacgaagcaggaagaactgcttcagaaactgaacatactgatttaattggctaagaagtccaaatgctaatactcctaataattagccattccttttgtgttttggtgacatatatcctcatacaatgtatatcaaatggaattttttgatttacacctgacatttcaaagtttccatttttgaattctcctagtcttaagtaagtagaacattgtctcctttgtttgctaggcataacgttttccccaacatctagggctccatgatgcaaaatatcattttgccgatcttctgttccagtatttactttaattttttttattataattggattttcaaatacaatcacaaaaacatctcctgttgaaggtggtttcccccaaaagtactcatcaacactactgtaagccttgcttgcttcataattttcaaacacattcatgttggtgtacagacttgcaggggggttatcaggaatgtcaaatgactcctcttcaaaatcatcatccttcagcttattctccgtccctttgtatgatgaataatagcccatgtgctgaaagagagatggtttaaaacggatcacatttttctgagccaacagaccacggaaatgagtcaatagccaatcacaaggcatttcttgataaaacattaataaaaaatgggccaaacgtgggagatcatgagaatgatagagtttaccaatgtagccaagcttagagaattcaagagttacccagtaagttccttctagggatgcaatgactttcttgatggcagttaagaaattttttgaacatcgaacatcatcttcaagcattacataatagtctgaagtattggcacaaaaattaagcagaaaagcataatctacattttgcttggaacgaaatttgactctatcttctggatcattgtaatttcttttaaggccatctaggattgggtaatactcctctggagcatgtataaccattaatcttcctgcaataatatggtgcgcaaatttctgtgtaatatcctggaccatggcatcacgccaggaagaattaaagtctgctaggtgaaccaccactgaaatttccttcagctcttcatagctggattgctcaaaaattgacttaattgtctcaagtaaatagtttcctttttttcgctttactgaagaaagtccaattgtaagataccgctttctttgtaaaggtgtggcagctaggtagcgataggtgacatttatggctcctgagaaattagataaatccttgaaagtatgaacatagcgttctgaattcagttgatgtgtggatgtttcccttataagttgtttgtctccttccagaacatagctatcttcaatgtacaagttcataaaaaggagaaaaatgacaagaactcccaagaatgacactgtagaacgttttctcaggcatctcattttatcaagtatttcaaaaatatgtttcatttgatgaaatttaaacattctcttcttgcatcttctggatccctttgccacactcctctgcacagtctttcttacaacaaatctgaccatgtccttcccaagcatgagacgttccaagattccatctgcttaagaaagacgctgtcataatctgtgctgtacagaaaccgttgatacccagagacagagaaaacaattcgttcagctagatccaacagtgctctgtgcagcctggaagcatgagtgatccttgggcctcacacaaaagcgagataattggctctcaatgaagagatgtaaacatccatcataatggcactgtgctgaaact

SEQ ID NO: 13490 - RNA, 22706 nt, Homo sapiens
  source 1..22706: mol_type = other RNA
gctgggattacaggcatgagccaccacgcctggccagtttttaaagtatttcatacagtgtaactaggcagtcagaaatacctgtatctcaaattcatttaacttttcaatgaatcaatcttcttattttctcagacatataaattatcataatactttacattgagtctctatggttgactatatgctgtgaaggaaggacataaatacatgtgaggaaacaattattgatatttttaaactaactagaaagcaccaagttatttgttaaataaacaaagttaattttatctacctgttcagtaagtgttggcaactatgaattaatctttgacaaattcacttacaactagcaattttaaagacttaaagtttaatttttattattaaaagggtatgattatttttactaaaattaataaaaagattaactgttactaaattaaagctccttcaaaaacataaatgtattctttagagagttaaaaaaagtagcaataaaatacatttttaatttagttaagcttacttaactaatgatcaaatagattaagttgtataaaattttacaaactttatatttttgcatacacttatcttcctggcatttttgaaataaaaaaaatacaagtgcatagggcagaggaggcgattcagttacttctgctatgttattaaatctctggtaaccactatacaatacaatacaatacaatacaatacaatacaatacaatacaatacaatacaatacaatacatgtagactcagcatccaaactttattttaccttcaagttctacctgataaagtggtggaataaagatggtattttccataactgtttaataataatcacatgttttatacccattgctttgaagaagaaaccttaagcaactagaaatgtcaatctaaaaggcagaaaagctggaaaaatctcatgaagactagaagatttacactcataagatcatgtaaatttatttggatatgctgaaaaaagagggggtataaaatctaaagtttggtaaatctttgctttacagggcttcaagttatagatttttcttttttccttttctcttcccctttctctctctttctcttttttatttttgccatttcttctcaggagcccctgcaatttcaaaccttggaattgaattggatttgaggaggaaaacccatattcagctttaattcaaatgaattttactactttagacaaaggtacaacactctattcaaaaaagttattgaaatcacatctttaaatctgacccagccacttgaataaataagttgtgttgtagtttctcagagcaaccgccgctcatctttcactcaccttaacaatttctcacttttttctgctttttttttttttttattttctgcttgctgaaatcgagatcaatattcattgttttcttctgggttaactcttttttatgttaactgaatcaattttggctttgtttctttatgaaattacttttagataaagtattgatattgtcatttatcaattttattatatgtcttttgcttattaaaggattaaaatccacctctaaacttatttagatcaaggtcagtttttttactcctctgtagaactgtgaagataatatcctattctccttttcttatggttttattgtgaagatctgtgcaaatagctatataaaatgcaattcggtattaaagaaaattgttgcacggactacattgattagagtctaatttttggaaagtatacttcgccttttcagtaattttatttttcggtctatggtgcccacattgtgtcaccagccagccgtatgcagacttacaaaggactacccactaagaataaaaacatgatacaacttgaagaaattttcatcaaacgtctttgtcttatccccttgttatacagacaaagatgacaagggccgaaaaggaagtgattttctcattgaataagagaatccgaactggcatcgaggatatctaattttgggatgaaaattgagagaagacagaatttcaagtctgaattatgacttcactactgtgtcgtcattggtagaataaggataacaatacttatcacacagatttgtggtctgaatcacatgagagacatagatgaaaaatgtaaaacaacaattagcatgtgacatgctctcagcaaatcaattaatccttcattctttttttctccccttactcctttgattttcagactaatttggatcatgattattggcctgtgtcccacccattattcacatatagaatgggttgcattatcctctccttggaaatatctttcaaagtgggtaatgagaaaactactttgaagactgtgctgaaggaaatgatggcatgaacaactctagataatttttgtttatttggatataacgtgaatgggcccataccataaactcctattaagctgaatcaccaaaaaaaaatttgatatgaaagtcatacattgaaaaaattcactcttaccactgatttgattgatactgagcctgtaaatatttatttatatgatgtttggcactttattttataaaactaccctttacttaaaataaatcattgtattcacataactttccagggcactatgcatttttaaacaagacagtcaacttactatttaaaaaacaaagtcagtcacctaaatgactttctgactataaatttgaaaacaatattctccttgtaatatatgtgccaccagggcaagaattacaaattgggagcaggtaagaaaattgttgttgactctcattagtattctaattctccttcagtcagatttataaagtatgacctatagcatccaactccatcattttccagtcattcttgagactgtcaactctatgggcattgtttagcagcctcgaaacactgaactttttacagtcttattggagagaaaaacacattaaatgatcaaataatcttttatgagctcagaaaaaaatgcctaacatgaacatttaagcatcttctgtttctgtgattcccatttttggagagtaaaaatttaagaaacaaagggaatgtgtctggggatggtactaataatattgagattttacaatttaggttataatcaagataattatgtatatatataaaattatatatggtatagtttcaacttctaatcttttatcatcctctaccacataattcctcctatattctctttttctgactgtggcctaatacctcaagaatattgtatatgcttgtcactatataaacttcaccctaaggaaatttccatgtcagatacaataagagcaacggaagaaaatgtatcaaaacacatctccaatttatttgaatttttctggcctaaccttgttggcatgagagttcccactttgtattataataggcaaattgatacacacttttcatttattctaaataatagattagcatagtcaggaggcttggattggcagctattaaatacaatttgaagccgtgggattttattaggattctaaggttattctgtgacgatggaacttaatgatgtaagagttaattacccattgtcaaaaatcattgcccatcaaagcagtgagactgtgtgctatgtccagttttattcatttcttttgtgtatctgaatggaacatgtggtaaacacaacagtagaatatacctacagtccccttagaaactcttaaatcttcaatttataaaagtcatcctaagacgttaaaaataacttacgaaaggatagattccaatgtcagtgggtgagatgtgctctagctagtgtgcacgaaagagaacatggagttagaataattattgtaggactgtagattgtcatctcaagatcagtgtcaaatacattcattcatgtagtattttcacatgcattctggtctaaatatcccaacatatctttcgttttgagatctgcagaacaaagtcaatgtctgaatttagagactaatttgaccattttgattcaaatgtctaaaggctaaaccagagcaatttacaacatccaatgaagtaaaattatataattaattatataattatataattatataaaattttataattaattataaaataaaatattaacaataattgaacattgtttacttttttatcctcacaacaattcaacatgatatgtatggttattactaaatgtataatacatttagtaatgtgatttgacaaatcacatttgtcaaataaggaatggctgaattaaatgattgaatgaaggagtgaaggatgtagattgtttaagtacattcaacttgtaatgaactgtaaacttcacccataacattattaatatatcagtgctatcaactacattttacataggatgaaaaaaatcattatttttattaatcccaagatattttatttcattatataaatgaaatattttatctgttataaagacctttatttttgttccactcattaaataacatggtaagactgttgtgtaattgactgaatagttaagtctaaatgggtaaatagctgtttatgttagtattgcagggtagctatttgataatgaaatatacttttcttacctacttgcaaaaaaaattacataaacaagtatttcctagagttcaaacactgatctttttaagtggcaaattgtccaaaagaatttaattaatataaacaataaattcacttaaacaactatttacatgcaaaagtaatatttttattgcccatttggaaaatagttttgctttctggtttataaggaacttttactagtttaattacttgggtgctttaaatgttttttggaggctattacaaaatcacatcctaaaattttaaaatggaaaaattataataattgaatttttaattcctcataaatattttaaaagtacacattgttccatggcttttgcctttagaataaatacaacatttttatgtagaaatatattcttgaaatgtaactagcacatagtcagtgtttcttaaccattttggggtcctgaaactttttgataatgatgaaagcacagagatgctatcaagaaaaatttacccacataggaacacacacacatacacacagacacacacagagtttgcttataagctcaggaagcttaaagatctgctaaagattatgcttgggtttgccatgaatcataaataccaagtcaaatacctttgaatttgattcttaacaaatctttgtggctgagaaaccatgagatttcattctggcatgtccccagaatgtaattatcaatgaacaatagccattgaaaaaatctgaacagatattattgaggctcaaggttgtttaatggcacagataatataattcaaatcatgaccccagggctgatgaagtcttgttgtaacgtgtaaatggggtgggtgatgggagagagaaaacaaaataattatttatgttaaatcatacataaacagtaaagccaacacaataagtaaaataagagaaagtagaatgcttgggaggtcatatgtttcaaatgtatgcatacacaaaagagtaagcaacaggatacttcaagagtaaaatgggaaaaaatcatattgggtaaatagtatcaccccaaagtgatagtcaaaagtacctatgtttgcctagttctcagattacaactatgatgataatttagataaacaagcagaaaacaaaactatagaaaaaagtcaaagtgacataaaacaattactggtgtttcaacagaaataaacccaacatcaggatttatcaaatatatgaaaaattatgaaagattataaaacaccaatgattagattatgttataaagacactatgaagagatactaaatgatattcttttcatctgtggttactgctaaaaaattctttcatagaaattcttggattttgaaattagtttaattccaaaatattttctttattttgcaaaaatgtaagacaaatgtataggatatttttctctgttgttatgcaaggatttattatcacattggccacagaacacatagaatgttagttttgtagaaaattttagagattttaataccaggatgaaataatagtatcattctatttcaggttcttaagcaacattcctaagactagaaccttatcttgaaaaattatgattttaaacttaagggaattcaggtaaaggaaattgactaggttaaggcaaatacatcatgtttactggtaaagataacattatttaaggaaggtaagatactcttatcctacatatacgccagaaaaattgcttctcctctgaaaactaccattatttttgccaaatattgtagcttagttttaagtttttctcggctgtttcctctgacagttctgtggtaaagaagaaacattataggaagcatttttttttcctacagagtctgccatatggagaagtagaatgagaggccacctaggtaatgtgatttattaaaagttctccatcccaaaatatatgtcccatctgtgggctaatgtctgaaagtcctatgattaaactcacttttatgtaagatagtgaggccccagagagccctcgagaaatgcaaataaactattactgacctcccttggattatgatgaaaaccgtggagtctttctattctctgtcaaatgtggaggtcatggatccttcttggcacctaagattaaaactcatagaatgtgctttaacttctgtaggcacatttcctttccaattagagtgaggtgttgaatatttatttatttgtttatttttattatactttaagttttagggtacatgtgcataacgtgcaggtttgttacatatgtatacatgtgccatgttggtgttctgcatcttaagagaagactatttataaaatttattgcttgtaagatttgttttttgttctcttactattatgaaaatcacgaacttgggaataaggacactctgggcccggcgcggtggctcacgcatgtaatcccagcactttgtgaggccgaggcgggaggatcacgaggtcaggagatcgagagcatcctggctaacaaggtgaaaccccgtctctactaaaaatacaaaaaattagccgggcgtggtggcgggcgcctgtactcccagctactcgggaggctgaggcaggagaatggcgtgaccccaggaggtggaacttgcagtgagcggagatagtgccactgcagtccggcctgggcaaaagagtgagactctgtctcaaaaaaaaaaaaaaaaaaaaaaaaggacactctgaacaattgaacaagactacgctgaaaggcagagaagaagtaattatgaacaaactgttcatgaagtgatcaattgaatttgaaacagaacttttcctagcttctaaatgattagaaatttcagctttggtttaacttaaaaacttagaattgtcaattctgtccaagtctctgagtcatgtacagaactcaaattattacatcatttttttacttatctgtattatttctccatttaaaagtggacaaatttttatactatatcctaataatgatacaaggtgacttgtaggactctggatagaaagagatggcccaggatacagagggcactccttaaatagctgccaaataaatgacattaaaaaatgtataaaaaggtatgttaagtaattaaaagtgtcaggcattattttcctattatgagacattttatattatggttatttactgtaattgcatccaaaataattcataaaacatttatttttgtactattaaaaatctaaacaataataaccagatggaggaaaatgataccatctgatttaattattaacttgaaggtcagtttctacaacttattctcatttatgtttatctgatttggccacagtttcttactttctcatattttgctaagcttgtggatgaagccgcatgtctcttttttttttaacctggcatataacactgtcactctatttaattattacccatcatctacctactttgaaactttggaggttttataaaaattatgagtatttaatcaaagttgtctctttatcatttgccagtgaaaatataaaacctggctgttttattctattgtgcactctaattacataaccaaaatctttttaaaaattcttagttcttttagaaataccatttgacccagccatcccattactgggtatatacccaaaggattataaatcatgcttctataaagacacatgcacacgtatgtttattgcggcactattcacaatagcaaagacttggaaccaatccaaatgtccaacaatgatagactggattaagaaaatgtggcacatatacaccatggaatactatgcagccataaaaaatgatgagttcatgtcctttgtagggacatggatgaagctggaaaccatcattctcagcaaactattgcaacgacaaaaaaaccaaacactgcatgttctcataggtgggaactgaacattgagaacacatagacacaggaaggggaacatcacacactgggcctgttgtggggtcaggggaggggggagggatagcattaggagatatacctaatgttaaatgacgagttaatgggtgcagcacaccaacatggcacaggtatacatatgtaacaaacctgcaagttgtgcacatgtaccctaaaacttaaagtataataataaaaaaattcttagttatttgaaaatagtttttttgaattcacaaacttgcaggatgaaaaaagttattagttcctgaagatataacattgatttgtctttttcttatttgatatcagctagcagtaaaattgtgaacaaatctggtaaatcttttggtgttgcaggttcataatcagttaattgagtgtattcactataaattgctttaattaagtgatgtttgcctaagaacaagtttcatttcatctcatgaaaaaaatgttactttttgtattaatcagtggaatgtttaaagaaaaaactggttatcttgaagctgtcaaataattataagaaatctctatacattacgttttaaaatacataaaacccataaattcaagcttattagttttcattttcagcaaggtttatacagagaaaataagtaatacaaattagttttccagaaaatctaattttatgcagataaaatctgaaaatcatataagtccaagatgaaactgatctcaaattattattttgaggtgtatccatttatttaaaaaagcctcattttagctagcaacactatgtagaaaaatattttaaataagacagagcattaaaataatgtattcattgatctcataaagaatagatgatcagattttttaaaagtgattttaattaaatggacatgtttctctttagccagaaatgactgagaaattttgagttggaattgatataggggaatccttggaactatgtgtgaatatgtgtgtgtgaattatctgtgtatatttacataatttacactattcacagtccttgtttttcttgactcaaatagctatctcaagtttcgtacactttttagatctctatgtaaatacattatttcatttgtggaaatatattgaggcctatatcaataacctcaaaccttttaaacacttagagcaagtcaatatgacttgttctgtttcagctatctgaaatttaaaaatttgacaaatttttaaagtacccagttcttggaaaaagaaaaacaaataaattggagatttggatcatatgggctatgactaaatgagacaaggcatacatgctgacatttgaaggatttatgaaaaaaagtccactgtggaaaactgatagtttttctccttctttcttgaatatgtttagttaattttgtggaaagaggaaggcagctcagtttacaaacagcagtgggttgaaggcaatgctgtttatattcttgaatttcaatatctacaaagatgtcatcattagattttatgtgttaaaaagtggatttatagtctctaattaataaggtgcatatgtcaagactcaggaaaacagatcacttacgtagttctccaaaaacgagagtcccagattcaataggaaggcatgcagagtgttctctataaacccagcaaaaccataaaaattgactggaacttttatttttcagtacaacaataatagtattgaaatacctaaaaagggcaggaaacaacacagaataatctacgcttgtcatcatgttttctaatctataatctttcaaactggataaatgggaagttttggaattttactgtggtacagtcttagttgctccgtggttgtcaaatctgtctgcacattaggatcacttaggaagaattttaaaagtatgctgatgcctggaaactccagaacaattatgataactctgagcatggagctcaggaatgggtgaaattcttccccagagatgttaatgaacagccagacttaaaaactagtaatttagacaagtgtgagcagaggttaataatgttgagatgaactgggcttaatatttcactaacaaggtcagagttttgatacatcacttaactcaaactttgagattcttcatcactgaagtagcaataataatagtcatttctgttttaatacttcatagacttgtaaggatgtaatgtagtgtttctaaaaggagtgaatggacaatctgcatcagtgttaactaaaatacattgaaagtgccaattcctagatctatcctagatttacagggaagaattcagtagtctgaaacacacattttcaatatattgaaaagatgattcttttgcatgatgacttgttataatcattactttcataggtaatggaagtaccgattaggagagtaccaaatacatattaaacactcagttcatgtaagctataggccaataaacacaactttggggtttactgatgttttccaacatccgaaataatagctgaaatttagaaacatagttaatcacacaaaaaatgttgcatacatactgtctaactaccagtttggtatgtttggggctggtgttatgaaagactattatatgattaatacaaagttataatttttggagtcttttagtgtacccagagcccatgagtttttattttctttttggaataacagaaattaggttgtggttcagtggaattacagaagcaagtgttttagatgttcaagtttaaaaaatgagaaaaaaatgttttacatgaagaaactaattatttaaattcatttttcaactatttaatgttattttaatatagtcatatcatccagaaaatcccatcttagacaaatgggttttcaataaattattattatagttaggaggcaatgtataatagtgataaggggcatagattttgaattacacaaacctgaaatccaatgctctctctttcatttattagttatgtgaccttggacaagttagtaaaaccctatttttcatatgctctttagcttttttaatacctcttaccttatatggttgtttaatctattaaatagacagtgaaatgcacatgaaatcttcacacagtgtctcatagttgcttggaacatatttatgtagtaagcattgttcttggctgagcttacattaagtgatctgtaaattagaagttatttgttatatttgtttcgtttccttattgccctagatgccttttctctggacctagataatttagtctcactctgtggcctttacccttcaataaatatggattattaatataatttagctacataattcctaaggaaatattaattcataaagattgttaaattgaactgaatatctttgctaagtcacaggcattgattaaattagataaaattgtcattttccattgattttgtttatataaataatattgaattatttatattcttatttagtctagtagattgacaggcagttttattaagaaatgaatcaaatggtaaattttgaatcatctggtaaaaatggacaaaatttagttttatcttgtggtctggaaatacaccctaaattattgggtcaagttagtgaaaactgttaaattgattatgaacgtaggcacattacttataaatccccttatgctaacttaaaacttgtgaatgtttagtgttatccagctataattcttctaaacatgtcttgtaatttttaagtttgcatgaaaataactccatcctgagtatactcatttcaataaattatttgtcctgagcatactgtaagaaatttagtaaagtactaattgaatttagtgattagactgtgattagactattacaaattcacagtgcttgtacaattcagatattattttgctttgaagtcaaatagaggaaccttaaataatttaaataaaaataattgtttttattaaagtttatacagcaagataataaattcactaatgtgaaatgttgatatagtatgtacaacttgtttcttaagttactaaaaatgtattttcctacctacataatgtcaatctctattgctcctaacacatgagtggctaaaattgcaaacttaatcacataaataatgagattaaagttaaaatgaaaaagtggtatgaggactattgtttgtgttaagtgaaattataccttgtaaaatttcatattatgagagcaatatgtaaatttcattgcaacaatggttattcaatttactgatgaaaatcagaagaatgttgaaaaattagtgcatttataataaatttaattattcataaaaaattaacattgatatatatattcataaggataaaagatatcaaaataattaaacaaatttcactttcttcttataaaagaaaataatttttatggtaactaattttagtagtgcatcagatcaacactattgggcacccagttatttggtggtacgctgagtgaaaatatgtagctttatctacattaccttggtttggacaactgaaaaatttgctaggaaacaaatattacaaaatatgttgttaacttttcaaagatgatcggtttagattgctttaacttgaaggacacttatattttgtatcacttttgtagcaaacacatgactcatcattgcccaaatcaattgcccaaatcaattcaaacatctcattgtagttcatcccatggcagaaaagtgtttatccacttagtaaaatggaaaacactagagcttcaggtttaatttgaaattttaacttcattaagaataaacttgacctgtttgttctagtaagtaaaaacactagatacgtaccaaaattgtcttttgaccctctcagggagtcaagttttgatttgcttgaatacaagcaagtcgagctatggtaatttgcaatgctgacaggaaagaagaacttgcttgaggcaaaatcatgaagtacaacttttcctctgcatccttttacctcatgtttgtaacatttcccctgttgttatttttacacatctggatgctcagaaaggcctccttaccacaataattgaaaggagtactttgtcaatagtcagaattgaatgagagataggttgttgggaatattcagggtgaatgtgtcttttctactttgactatatttaccattgactacagtaactcagcagaaagttagagggcagcatacatacattggtttatggatttaatgaaaatatccccaaccattacattacagacaattcatatatatgtcttgaaaatcttcttgacaatttgtgacaaattttctaaatgtttttccaaaaatagttggttcttgtaagtgattttgatatgactgattaccaaattatggtgggtaaagatgccacatgcaacagaaaatgtgtctaattatgtttgttttagagcttaagaaatgttaagaagagaagttacaactgcattaataggattttaatttttattcaaaatggacaacttatttattatgtacttctacacacagctaagcttatagatattttcatttaaagaaaaactatttgttcattttattagcagatatcaaatgcccttttgaaaattgagactgatttctaaaacaaaaaaaaagactttaggagttttaattatttttaatatattgcttctttattaaaaaaagatacaatccttcaatgtcattcaacagtattaattgttaaagtgtgggatatagtttacattaccgagtttattttctaagggtagtgaataactcctgacaactactgatatcgtcacatggtcctttagtgaccaaaaatgcacagttgtaagaatgcaagtgttacttgtattgaaaaccggattacattaaaggatggacaattatgataaaggatctgagataattggacaattatgataaaggatctgagataattattctaactttttggaactatactttcactcattgatgaagtaagttacaacgtggaataacaaagtttaagtgtggcagaaaatacatacatatgtttaaaagtagggaaaattttatcaattattaaagatggaaaaaataggactatgtcaaatagttaaacaaatgtggggtattttatggagaaaagaggcatgtactaccttaaacattttccaattggaacatactatagacaaaactgacagattattattcaatgagaaacctgactcagatgaagttacaaaaaaagtactttttaaatgtctagtttctaatagagttagagctttgttgattgagatatgtggaactgccacatatctctgtgccatacttttggtaccttcataataaacggtaaagtgagggaaagggtggaagagacaaatcctacgtctcttccagaacttcgagtgcactataaattaaatatttaaaatatttttgcaatagttagctttcaattatgaacactctcagcctctattgctttatatatgcatttattttggtaatttttatacatcaaaactataattacctgtatttgggcagaatgatttaggttatgccagctattgtggttaaagctgtagtaacttacagtacattgaaattatagactaaggttctgaatattggtaactcactgttgttgtgcacctttaaacaactcttaaataaagtaatgattctctttatattaaatttaatgtatgtgtgcctcatggaaatttgtattttatagaaaaatattgaatattttattattatgtctttggctcacctactttaaggagatggctacttagggtactttttaatccaatataatgtgaaaatttgatcatgctatattcttaatttaattgtacttctatggtcatatacaatttacctatcactttctcacataatcaatttaactttttggtaaatcttctaagagaccgtctagacagagtgaaatgaaagctgaaacaacagtcaaatcaaaaactgctttggtctcaaatccatgtttttcagaaaagatattcagatccagttatctggcaaatggtctcaaacatacatttcaatttcaatgttaaaaataggatattaaacatctcagaaaatattgggattattgaagcaaattctaccctggacttggagtaaatgtgatgaacagattaatgaggtggaagggactagaactttgggaaagtgcaaccttgttatcttaatatttttatagcttagaaagagaatgctatgcaactcatattttgatcttttaatgttaaagaattcaaataaaaaccataaacctgaaactctaaaagaaaaattctgttttgagagagatggcctcctctagtacacttttaataaatttaaagtatctaaaaggatgcacaaagatctctaatgtgctgtgattttcaaaggatgtcatgtataaaagatttgagtgagaacatgaaagcaaaagcaagttcagaagaggaacacaaccaggaggacagtgtgtcaggaaaatccaagaataagtggaggtgtaaaggctaaaaaataatgcaaatggtgcatatccttctgtctttctctcatacacacagacacacttacacaacacatatacaaatacatacatgtatatatgtatatatatacacaaatatacacacatattcacataatattcaagtatgtatacatatatacacatatgtacatacacatatgtatatatacatacacacagattgagagattaaccatatgtagatacacacatgcacatatgcaataatgaaatcatttcaaagcatgccaaaaagtaataaaagatatatcctctgtttgggataaataaaaaaaaagtttaaaagcaaacaaaaaataaatggcaataactaatcacattgaattttgttatggcctttttcttcctaaaaagaataaccccaatctgaacaaagaaattcaaagtaatggaaaactcaacaatgaaactcaaagtagactagcagataagatacctatttcaaacatcagtgccaaggtaatttataggtcagtgcattgataacttttgccaatgatagaaaagatgccagagaaccggatcctgacattaaaaaaaaaaagtaaaaagattctgaagactgcatttctgagcttaaggtagattctaaacaacatcttagaaactaggaaatgactttatgtttctttgtttttcaatgtaaatggatcaagatttcttaaaacagaaatgaatattattatttgtgatgagagcactaggggcaattttgatatttttgataaggtttctagagtaataaattagaatgacaggaatatatattgattttaggaaagtgtctgtataattccacatgatattctctggacaaaatatgaaaaggtaggctgaataacatttttaaagggcagtaaattttataattgttattgattacaatgaaggcctctggtaatgttttccagggtcatatcctgttacatatacgtgacatggataaaaaggaaacaaatatttattgtgtgcctagtttatgttatctcaattccagctctacaaggagctacaaggtaaaattgctacctttaaaaacatatgaggtaaaattattcctattcacagatgtagaaactgagtttcaagaaggttaagtaaatttcctcatattgggaggctggtaatgcagaactgggtgtcaaaatcaagtctgtatgaaccttctgttttgtctcccatgaagacaaaaggcatgcatataaaatttgttgaaacacaaagctgaggaggcataataagacgtggaatgacagaagcaagatctagaaagtttgggatcatgaatcaaaagaaacaggataaaattatcctaaaattaatattaaatcttacaagaaaccccccaaaatcagttgaatttgtacaaaacggtaaatcattttatcagtagatcccataataaatattataaagtttaagtgtgagctctattactcagtaatatgatgccattactgtgttgatggatgtattgtcaaggaaaaagaagagaattacacactgtttccttcaattgttagatggcactggatgtagtgttttcaatgttaatcctggtatcatgttctttgccataaacttgttgacaaattggcaaatactgacatgaaatatgccaatatttgagcatctaaaaatgtaggtactttccataccacatcatatattacaatttgaaaatgtttgtttcattttttatataattattatacagaacagtttttctatgatagcattataaaaattcccagagaatactggcccagtaagaaatggaatgttcacaactcatagtgtagctatatgaaagaaatagatctaaacgacaggttggtttccaaattatattttcatacctggaaaatatctactttataaatagcacaaagttatagttttcaatgaatatgaaaaagttcttgcattaacatattttatgtatcttttatattgacatttgtgattgccactaaaatgtgtattttctaaatttcattgtgcttttacaagatacttttttctttgatgtccataactgctgaaaaggctcccctaaggagaattttaagactaagtaaggtttttagtgagcttaaattatacaattctgaggcattatttaaggtgcatactgtattttttgcttgaaacctgtcagcattttatttgtatggcaattaaatgactcagccattcatgtctcatgccagtctttttcaattgttatttttaacaaagaaaattatatatatatgtatatatatattatatatatgtatatatgtattatatatgtatatatatataaacttacagcaaaaatgtttaaaaatagcaaatagtttgagtatagttaaacctaataactgtacttttgtttctatgcctctgagacaagattactagacccttattcaaagtttctaaatataggaaatagaacattgggccatgctaaaaaaattgttcagattttcttttgaaagagaatagttatttttcctcctgacctctaatgaagatgctttatttgtcaaggtgttttccttagaaaattgacccagtgtcaactgtaaagaaaacatagaggatccttggatgattgaccaacttatccaaacacaggtttagtaaagagaggatataaagataaaatgtgaaatgacctctctgagtcacatttgttttcataatttcctagcaaacatccaacttcactgctaccctcagcaatgtttcttgaaacatttttaagacattgatagacaccaatagctgatctttagaaagccattcccagaagaatatgtaaggggttacaactcatttcagggagtctgcctagctcttgatattacatgtctttggcatacaattgtgtaccttttatcattgacagtgaagaaaataatgccatttgtaacttctgagatatacacacaatactatcaactagccggttaataaaagataagaaaaataaagaaaatagaacatttttaggtgtctggcaagtatcctctaaatcaaggtaaagataataatttagtggcagtgttcatattttcctatgactgtaagatttaggtgcctcacaaaatattaatatttagcctcttatgaaaggttcgtttttcttctaacactttagtagctgaatacaaagaaaatacacaacagctgtttataaatgaaataaaaagtttccattttttatctgagtttctcatttatttgcagagaacgaataaaataaaaatatcctagtgttgtttgcaccacagcataccagtaaatcttaaggattgtgtttcagtatgaaaaggaagagcaggaagatttcctcattctgtcttaccagcaaaagtctagccttcacacacacacacacacacacacacacacacacacacacacacacacacacacagagtcatctatatgaacacgtacttgagtttcttaaacatatatgaagcaccttccatttccctttataataaatcccttagtttttgctgttcattaaaaaacaaaaaggaagagacaagctcaggacattctgaaaaccaatgtctttaggacacactaaggtgtcctgaattactttaacggacacattgtaaagacacactctccaatccctattaggaaaagtttagtcaagtttgcttactatttgggtgcttataccaaaaaagcatcatttaggacattatttaggataatattatttatgcaggaattgtaccacctatttccagatggtataacttattatctgacaggcatgtagcaaatagaacacaaagcataaatctgtcaggagaaatcatacgagaaaaagagcattgtctggttatcagaatatcagatctctcattctggccttgctaggaaatagatctttgattctagaaaagtcaactaatttctatggttcttacttttctcctttataatatacccatttaaattccaaaaaggtatatgataaatcacaataatttcaatcacatggattttaatacaaaatgtataaaatcaatttccaaaaattttctgcatatactgaaaatgtctgtacgaatgagctaactactataggccttccctaatttattctattaaatgtgggtactcaatgtaacctgaaaatattgagcttaactcttctttttttttttcaaaagggaaacttgaaaaagactgcttcccccagaaaatttatcaacaataggtgctcaattaaatgtttttaaacaatgaacaatatcccctttcatataaataatcaggggagagatatttttaagtcttttttttctttttccatagtgtcacctacacaaaaaattatgtaaagacaccacttctatgaggaggtattcattgtagatgtacagaagtcaacggaaacttaagtttacagaaaaaataaaccagattatcattccacccaactgtatattcccacagatgcttaataaaagctatctgatgatataatgaattatcagttcttgaggaagtatatacagttggtgactatttttcaaaaatcatcatccaacaaatttttttcatttaaaatctttcatattaccctttcgacaatcagttgaaattttaaaactaagaacatttaaaaatataaatgaaagtagcattagctatagactgatattcaacttcagacgttaaaataaatacaagtgtgtattaagagtaaaattatgtcaacaatgtataaatgaaaactgccaatgtaattaatgtttcttttaacatatcccatccattgctttccctccaaaagacaaaggtagcaaaagacgaagcaggaagaactgcttcagaaactgaacatactgatttaattggctaagaagtccaaatgctaatactcctaataattagccattccttttgtgttttggtgacatatatcctcatacaatgtatatcaaatggaattttttgatttacacctgacatttcaaagtttccatttttgaattctcctagtcttaagtaagtagaacattgtctcctttgtttgctaggcataacgttttccccaacatctagggctccatgatgcaaaatatcattttgccgatcttctgttccagtatttactttaattttttttattataattggattttcaaatacaatcacaaaaacatctcctgttgaaggtggtttcccccaaaagtactcatcaacactactgtaagccttgcttgcttcataattttcaaacacattcatgttggtgtacagacttgcaggggggttatcaggaatgtcaaatgactcctcttcaaaatcatcatccttcagcttattctccgtccctttgtatgatgaataatagcccatgtgctgaaagagagatggtttaaaacggatcacatttttctgagccaacagaccacggaaatgagtcaatagccaatcacaaggcatttcttgataaaacattaataaaaaatgggccaaacgtgggagatcatgagaatgatagagtttaccaatgtagccaagcttagagaattcaagagttacccagtaagttccttctagggatgcaatgactttcttgatggcagttaagaaattttttgaacatcgaacatcatcttcaagcattacataatagtctgaagtattggcacaaaaattaagcagaaaagcataatctacattttgcttggaacgaaatttgactctatcttctggatcattgtaatttcttttaaggccatctaggattgggtaatactcctctggagcatgtataaccattaatcttcctgcaataatatggtgcgcaaatttctgtgtaatatcctggaccatggcatcacgccaggaagaattaaagtctgctaggtgaaccaccactgaaatttccttcagctcttcatagctggattgctcaaaaattgacttaattgtctcaagtaaatagtttcctttttttcgctttactgaagaaagtccaattgtaagataccgctttctttgtaaaggtgtggcagctaggtagcgataggtgacatttatggctcctgagaaattagataaatccttgaaagtatgaacatagcgttctgaattcagttgatgtgtggatgtttcccttataagttgtttgtctccttccagaacatagctatcttcaatgtacaagttcataaaaaggagaaaaatgacaagaactcccaagaatgacactgtagaacgttttctcaggcatctcattttatcaagtatttcaaaaatatgtttcatttgatgaaatttaaacattctcttcttgcatcttctggatccctttgccacactcctctgcacagtctttcttacaacaaatctgaccatgtccttcccaagcatgagacgttccaagattccatcttaagaaagacgctgtcataatctgtgctgtacagaaaccgttgatacccagagacagagaaaacaattcgttcagctagatccaacagtgctctgtgcagcctggaagcatgagtgatccttgggcctcacacaaaagcgagataattggctctcaatgaagagatgtaaacatccatcataatggcactgtgctgaaact

SEQ ID NO: 13491 - RNA, 23725 nt, Homo sapiens
  source 1..23725: mol_type = other RNA
gctgggattacaggcatgagccaccacgcctggccagtttttaaagtatttcatacagtgtaactaggcagtcagaaatacctgtatctcaaattcatttaacttttcaatgaatcaatcttcttattttctcagacatataaattatcataatactttacattgagtctctatggttgactatatgctgtgaaggaaggacataaatacatgtgaggaaacaattattgatatttttaaactaactagaaagcaccaagttatttgttaaataaacaaagttaattttatctacctgttcagtaagtgttggcaactatgaattaatctttgacaaattcacttacaactagcaattttaaagacttaaagtttaatttttattattaaaagggtatgattatttttactaaaattaataaaaagattaactgttactaaattaaagctccttcaaaaacataaatgtattctttagagagttaaaaaaagtagcaataaaatacatttttaatttagttaagcttacttaactaatgatcaaatagattaagttgtataaaattttacaaactttatatttttgcatacacttatcttcctggcatttttgaaataaaaaaaatacaagtgcatagggcagaggaggcgattcagttacttctgctatgttattaaatctctggtaaccactatacaatacaatacaatacaatacaatacaatacaatacaatacaatacaatacaatacaatacatgtagactcagcatccaaactttattttaccttcaagttctacctgataaagtggtggaataaagatggtattttccataactgtttaataataatcacatgttttatacccattgctttgaagaagaaaccttaagcaactagaaatgtcaatctaaaaggcagaaaagctggaaaaatctcatgaagactagaagatttacactcataagatcatgtaaatttatttggatatgctgaaaaaagagggggtataaaatctaaagtttggtaaatctttgctttacagggcttcaagttatagatttttcttttttccttttctcttcccctttctctctctttctcttttttatttttgccatttcttctcaggagcccctgcaatttcaaaccttggaattgaattggatttgaggaggaaaacccatattcagctttaattcaaatgaattttactactttagacaaaggtacaacactctattcaaaaaagttattgaaatcacatctttaaatctgacccagccacttgaataaataagttgtgttgtagtttctcagagcaaccgccgctcatctttcactcaccttaacaatttctcacttttttctgctttttttttttttttattttctgcttgctgaaatcgagatcaatattcattgttttcttctgggttaactcttttttatgttaactgaatcaattttggctttgtttctttatgaaattacttttagataaagtattgatattgtcatttatcaattttattatatgtcttttgcttattaaaggattaaaatccacctctaaacttatttagatcaaggtcagtttttttactcctctgtagaactgtgaagataatatcctattctccttttcttatggttttattgtgaagatctgtgcaaatagctatataaaatgcaattcggtattaaagaaaattgttgcacggactacattgattagagtctaatttttggaaagtatacttcgccttttcagtaattttatttttcggtctatggtgcccacattgtgtcaccagccagccgtatgcagacttacaaaggactacccactaagaataaaaacatgatacaacttgaagaaattttcatcaaacgtctttgtcttatccccttgttatacagacaaagatgacaagggccgaaaaggaagtgattttctcattgaataagagaatccgaactggcatcgaggatatctaattttgggatgaaaattgagagaagacagaatttcaagtctgaattatgacttcactactgtgtcgtcattggtagaataaggataacaatacttatcacacagatttgtggtctgaatcacatgagagacatagatgaaaaatgtaaaacaacaattagcatgtgacatgctctcagcaaatcaattaatccttcattctttttttctccccttactcctttgattttcagactaatttggatcatgattattggcctgtgtcccacccattattcacatatagaatgggttgcattatcctctccttggaaatatctttcaaagtgggtaatgagaaaactactttgaagactgtgctgaaggaaatgatggcatgaacaactctagataatttttgtttatttggatataacgtgaatgggcccataccataaactcctattaagctgaatcaccaaaaaaaaatttgatatgaaagtcatacattgaaaaaattcactcttaccactgatttgattgatactgagcctgtaaatatttatttatatgatgtttggcactttattttataaaactaccctttacttaaaataaatcattgtattcacataactttccagggcactatgcatttttaaacaagacagtcaacttactatttaaaaaacaaagtcagtcacctaaatgactttctgactataaatttgaaaacaatattctccttgtaatatatgtgccaccagggcaagaattacaaattgggagcaggtaagaaaattgttgttgactctcattagtattctaattctccttcagtcagatttataaagtatgacctatagcatccaactccatcattttccagtcattcttgagactgtcaactctatgggcattgtttagcagcctcgaaacactgaactttttacagtcttattggagagaaaaacacattaaatgatcaaataatcttttatgagctcagaaaaaaatgcctaacatgaacatttaagcatcttctgtttctgtgattcccatttttggagagtaaaaatttaagaaacaaagggaatgtgtctggggatggtactaataatattgagattttacaatttaggttataatcaagataattatgtatatatataaaattatatatggtatagtttcaacttctaatcttttatcatcctctaccacataattcctcctatattctctttttctgactgtggcctaatacctcaagaatattgtatatgcttgtcactatataaacttcaccctaaggaaatttccatgtcagatacaataagagcaacggaagaaaatgtatcaaaacacatctccaatttatttgaatttttctggcctaaccttgttggcatgagagttcccactttgtattataataggcaaattgatacacacttttcatttattctaaataatagattagcatagtcaggaggcttggattggcagctattaaatacaatttgaagccgtgggattttattaggattctaaggttattctgtgacgatggaacttaatgatgtaagagttaattacccattgtcaaaaatcattgcccatcaaagcagtgagactgtgtgctatgtccagttttattcatttcttttgtgtatctgaatggaacatgtggtaaacacaacagtagaatatacctacagtccccttagaaactcttaaatcttcaatttataaaagtcatcctaagacgttaaaaataacttacgaaaggatagattccaatgtcagtgggtgagatgtgctctagctagtgtgcacgaaagagaacatggagttagaataattattgtaggactgtagattgtcatctcaagatcagtgtcaaatacattcattcatgtagtattttcacatgcattctggtctaaatatcccaacatatctttcgttttgagatctgcagaacaaagtcaatgtctgaatttagagactaatttgaccattttgattcaaatgtctaaaggctaaaccagagcaatttacaacatccaatgaagtaaaattatataattaattatataattatataattatataaaattttataattaattataaaataaaatattaacaataattgaacattgtttacttttttatcctcacaacaattcaacatgatatgtatggttattactaaatgtataatacatttagtaatgtgatttgacaaatcacatttgtcaaataaggaatggctgaattaaatgattgaatgaaggagtgaaggatgtagattgtttaagtacattcaacttgtaatgaactgtaaacttcacccataacattattaatatatcagtgctatcaactacattttacataggatgaaaaaaatcattatttttattaatcccaagatattttatttcattatataaatgaaatattttatctgttataaagacctttatttttgttccactcattaaataacatggtaagactgttgtgtaattgactgaatagttaagtctaaatgggtaaatagctgtttatgttagtattgcagggtagctatttgataatgaaatatacttttcttacctacttgcaaaaaaaattacataaacaagtatttcctagagttcaaacactgatctttttaagtggcaaattgtccaaaagaatttaattaatataaacaataaattcacttaaacaactatttacatgcaaaagtaatatttttattgcccatttggaaaatagttttgctttctggtttataaggaacttttactagtttaattacttgggtgctttaaatgttttttggaggctattacaaaatcacatcctaaaattttaaaatggaaaaattataataattgaatttttaattcctcataaatattttaaaagtacacattgttccatggcttttgcctttagaataaatacaacatttttatgtagaaatatattcttgaaatgtaactagcacatagtcagtgtttcttaaccattttggggtcctgaaactttttgataatgatgaaagcacagagatgctatcaagaaaaatttacccacataggaacacacacacatacacacagacacacacagagtttgcttataagctcaggaagcttaaagatctgctaaagattatgcttgggtttgccatgaatcataaataccaagtcaaatacctttgaatttgattcttaacaaatctttgtggctgagaaaccatgagatttcattctggcatgtccccagaatgtaattatcaatgaacaatagccattgaaaaaatctgaacagatattattgaggctcaaggttgtttaatggcacagataatataattcaaatcatgaccccagggctgatgaagtcttgttgtaacgtgtaaatggggtgggtgatgggagagagaaaacaaaataattatttatgttaaatcatacataaacagtaaagccaacacaataagtaaaataagagaaagtagaatgcttgggaggtcatatgtttcaaatgtatgcatacacaaaagagtaagcaacaggatacttcaagagtaaaatgggaaaaaatcatattgggtaaatagtatcaccccaaagtgatagtcaaaagtacctatgtttgcctagttctcagattacaactatgatgataatttagataaacaagcagaaaacaaaactatagaaaaaagtcaaagtgacataaaacaattactggtgtttcaacagaaataaacccaacatcaggatttatcaaatatatgaaaaattatgaaagattataaaacaccaatgattagattatgttataaagacactatgaagagatactaaatgatattcttttcatctgtggttactgctaaaaaattctttcatagaaattcttggattttgaaattagtttaattccaaaatattttctttattttgcaaaaatgtaagacaaatgtataggatatttttctctgttgttatgcaaggatttattatcacattggccacagaacacatagaatgttagttttgtagaaaattttagagattttaataccaggatgaaataatagtatcattctatttcaggttcttaagcaacattcctaagactagaaccttatcttgaaaaattatgattttaaacttaagggaattcaggtaaaggaaattgactaggttaaggcaaatacatcatgtttactggtaaagataacattatttaaggaaggtaagatactcttatcctacatatacgccagaaaaattgcttctcctctgaaaactaccattatttttgccaaatattgtagcttagttttaagtttttctcggctgtttcctctgacagttctgtggtaaagaagaaacattataggaagcatttttttttcctacagagtctgccatatggagaagtagaatgagaggccacctaggtaatgtgatttattaaaagttctccatcccaaaatatatgtcccatctgtgggctaatgtctgaaagtcctatgattaaactcacttttatgtaagatagtgaggccccagagagccctcgagaaatgcaaataaactattactgacctcccttggattatgatgaaaaccgtggagtctttctattctctgtcaaatgtggaggtcatggatccttcttggcacctaagattaaaactcatagaatgtgctttaacttctgtaggcacatttcctttccaattagagtgaggtgttgaatatttatttatttgtttatttttattatactttaagttttagggtacatgtgcataacgtgcaggtttgttacatatgtatacatgtgccatgttggtgttctgcatcttaagagaagactatttataaaatttattgcttgtaagatttgttttttgttctcttactattatgaaaatcacgaacttgggaataaggacactctgggcccggcgcggtggctcacgcatgtaatcccagcactttgtgaggccgaggcgggaggatcacgaggtcaggagatcgagagcatcctggctaacaaggtgaaaccccgtctctactaaaaatacaaaaaattagccgggcgtggtggcgggcgcctgtactcccagctactcgggaggctgaggcaggagaatggcgtgaccccaggaggtggaacttgcagtgagcggagatagtgccactgcagtccggcctgggcaaaagagtgagactctgtctcaaaaaaaaaaaaaaaaaaaaaaaaggacactctgaacaattgaacaagactacgctgaaaggcagagaagaagtaattatgaacaaactgttcatgaagtgatcaattgaatttgaaacagaacttttcctagcttctaaatgattagaaatttcagctttggtttaacttaaaaacttagaattgtcaattctgtccaagtctctgagtcatgtacagaactcaaattattacatcatttttttacttatctgtattatttctccatttaaaagtggacaaatttttatactatatcctaataatgatacaaggtgacttgtaggactctggatagaaagagatggcccaggatacagagggcactccttaaatagctgccaaataaatgacattaaaaaatgtataaaaaggtatgttaagtaattaaaagtgtcaggcattattttcctattatgagacattttatattatggttatttactgtaattgcatccaaaataattcataaaacatttatttttgtactattaaaaatctaaacaataataaccagatggaggaaaatgataccatctgatttaattattaacttgaaggtcagtttctacaacttattctcatttatgtttatctgatttggccacagtttcttactttctcatattttgctaagcttgtggatgaagccgcatgtctcttttttttttaacctggcatataacactgtcactctatttaattattacccatcatctacctactttgaaactttggaggttttataaaaattatgagtatttaatcaaagttgtctctttatcatttgccagtgaaaatataaaacctggctgttttattctattgtgcactctaattacataaccaaaatctttttaaaaattcttagttcttttagaaataccatttgacccagccatcccattactgggtatatacccaaaggattataaatcatgcttctataaagacacatgcacacgtatgtttattgcggcactattcacaatagcaaagacttggaaccaatccaaatgtccaacaatgatagactggattaagaaaatgtggcacatatacaccatggaatactatgcagccataaaaaatgatgagttcatgtcctttgtagggacatggatgaagctggaaaccatcattctcagcaaactattgcaacgacaaaaaaaccaaacactgcatgttctcataggtgggaactgaacattgagaacacatagacacaggaaggggaacatcacacactgggcctgttgtggggtcaggggaggggggagggatagcattaggagatatacctaatgttaaatgacgagttaatgggtgcagcacaccaacatggcacaggtatacatatgtaacaaacctgcaagttgtgcacatgtaccctaaaacttaaagtataataataaaaaaattcttagttatttgaaaatagtttttttgaattcacaaacttgcaggatgaaaaaagttattagttcctgaagatataacattgatttgtctttttcttatttgatatcagctagcagtaaaattgtgaacaaatctggtaaatcttttggtgttgcaggttcataatcagttaattgagtgtattcactataaattgctttaattaagtgatgtttgcctaagaacaagtttcatttcatctcatgaaaaaaatgttactttttgtattaatcagtggaatgtttaaagaaaaaactggttatcttgaagctgtcaaataattataagaaatctctatacattacgttttaaaatacataaaacccataaattcaagcttattagttttcattttcagcaaggtttatacagagaaaataagtaatacaaattagttttccagaaaatctaattttatgcagataaaatctgaaaatcatataagtccaagatgaaactgatctcaaattattattttgaggtgtatccatttatttaaaaaagcctcattttagctagcaacactatgtagaaaaatattttaaataagacagagcattaaaataatgtattcattgatctcataaagaatagatgatcagattttttaaaagtgattttaattaaatggacatgtttctctttagccagaaatgactgagaaattttgagttggaattgatataggggaatccttggaactatgtgtgaatatgtgtgtgtgaattatctgtgtatatttacataatttacactattcacagtccttgtttttcttgactcaaatagctatctcaagtttcgtacactttttagatctctatgtaaatacattatttcatttgtggaaatatattgaggcctatatcaataacctcaaaccttttaaacacttagagcaagtcaatatgacttgttctgtttcagctatctgaaatttaaaaatttgacaaatttttaaagtacccagttcttggaaaaagaaaaacaaataaattggagatttggatcatatgggctatgactaaatgagacaaggcatacatgctgacatttgaaggatttatgaaaaaaagtccactgtggaaaactgatagtttttctccttctttcttgaatatgtttagttaattttgtggaaagaggaaggcagctcagtttacaaacagcagtgggttgaaggcaatgctgtttatattcttgaatttcaatatctacaaagatgtcatcattagattttatgtgttaaaaagtggatttatagtctctaattaataaggtgcatatgtcaagactcaggaaaacagatcacttacgtagttctccaaaaacgagagtcccagattcaataggaaggcatgcagagtgttctctataaacccagcaaaaccataaaaattgactggaacttttatttttcagtacaacaataatagtattgaaatacctaaaaagggcaggaaacaacacagaataatctacgcttgtcatcatgttttctaatctataatctttcaaactggataaatgggaagttttggaattttactgtggtacagtcttagttgctccgtggttgtcaaatctgtctgcacattaggatcacttaggaagaattttaaaagtatgctgatgcctggaaactccagaacaattatgataactctgagcatggagctcaggaatgggtgaaattcttccccagagatgttaatgaacagccagacttaaaaactagtaatttagacaagtgtgagcagaggttaataatgttgagatgaactgggcttaatatttcactaacaaggtcagagttttgatacatcacttaactcaaactttgagattcttcatcactgaagtagcaataataatagtcatttctgttttaatacttcatagacttgtaaggatgtaatgtagtgtttctaaaaggagtgaatggacaatctgcatcagtgttaactaaaatacattgaaagtgccaattcctagatctatcctagatttacagggaagaattcagtagtctgaaacacacattttcaatatattgaaaagatgattcttttgcatgatgacttgttataatcattactttcataggtaatggaagtaccgattaggagagtaccaaatacatattaaacactcagttcatgtaagctataggccaataaacacaactttggggtttactgatgttttccaacatccgaaataatagctgaaatttagaaacatagttaatcacacaaaaaatgttgcatacatactgtctaactaccagtttggtatgtttggggctggtgttatgaaagactattatatgattaatacaaagttataatttttggagtcttttagtgtacccagagcccatgagtttttattttctttttggaataacagaaattaggttgtggttcagtggaattacagaagcaagtgttttagatgttcaagtttaaaaaatgagaaaaaaatgttttacatgaagaaactaattatttaaattcatttttcaactatttaatgttattttaatatagtcatatcatccagaaaatcccatcttagacaaatgggttttcaataaattattattatagttaggaggcaatgtataatagtgataaggggcatagattttgaattacacaaacctgaaatccaatgctctctctttcatttattagttatgtgaccttggacaagttagtaaaaccctatttttcatatgctctttagcttttttaatacctcttaccttatatggttgtttaatctattaaatagacagtgaaatgcacatgaaatcttcacacagtgtctcatagttgcttggaacatatttatgtagtaagcattgttcttggctgagcttacattaagtgatctgtaaattagaagttatttgttatatttgtttcgtttccttattgccctagatgccttttctctggacctagataatttagtctcactctgtggcctttacccttcaataaatatggattattaatataatttagctacataattcctaaggaaatattaattcataaagattgttaaattgaactgaatatctttgctaagtcacaggcattgattaaattagataaaattgtcattttccattgattttgtttatataaataatattgaattatttatattcttatttagtctagtagattgacaggcagttttattaagaaatgaatcaaatggtaaattttgaatcatctggtaaaaatggacaaaatttagttttatcttgtggtctggaaatacaccctaaattattgggtcaagttagtgaaaactgttaaattgattatgaacgtaggcacattacttataaatccccttatgctaacttaaaacttgtgaatgtttagtgttatccagctataattcttctaaacatgtcttgtaatttttaagtttgcatgaaaataactccatcctgagtatactcatttcaataaattatttgtcctgagcatactgtaagaaatttagtaaagtactaattgaatttagtgattagactgtgattagactattacaaattcacagtgcttgtacaattcagatattattttgctttgaagtcaaatagaggaaccttaaataatttaaataaaaataattgtttttattaaagtttatacagcaagataataaattcactaatgtgaaatgttgatatagtatgtacaacttgtttcttaagttactaaaaatgtattttcctacctacataatgtcaatctctattgctcctaacacatgagtggctaaaattgcaaacttaatcacataaataatgagattaaagttaaaatgaaaaagtggtatgaggactattgtttgtgttaagtgaaattataccttgtaaaatttcatattatgagagcaatatgtaaatttcattgcaacaatggttattcaatttactgatgaaaatcagaagaatgttgaaaaattagtgcatttataataaatttaattattcataaaaaattaacattgatatatatattcataaggataaaagatatcaaaataattaaacaaatttcactttcttcttataaaagaaaataatttttatggtaactaattttagtagtgcatcagatcaacactattgggcacccagttatttggtggtacgctgagtgaaaatatgtagctttatctacattaccttggtttggacaactgaaaaatttgctaggaaacaaatattacaaaatatgttgttaacttttcaaagatgatcggtttagattgctttaacttgaaggacacttatattttgtatcacttttgtagcaaacacatgactcatcattgcccaaatcaattgcccaaatcaattcaaacatctcattgtagttcatcccatggcagaaaagtgtttatccacttagtaaaatggaaaacactagagcttcaggtttaatttgaaattttaacttcattaagaataaacttgacctgtttgttctagtaagtaaaaacactagatacgtaccaaaattgtcttttgaccctctcagggagtcaagttttgatttgcttgaatacaagcaagtcgagctatggtaatttgcaatgctgacaggaaagaagaacttgcttgaggcaaaatcatgaagtacaacttttcctctgcatccttttacctcatgtttgtaacatttcccctgttgttatttttacacatctggatgctcagaaaggcctccttaccacaataattgaaaggagtactttgtcaatagtcagaattgaatgagagataggttgttgggaatattcagggtgaatgtgtcttttctactttgactatatttaccattgactacagtaactcagcagaaagttagagggcagcatacatacattggtttatggatttaatgaaaatatccccaaccattacattacagacaattcatatatatgtcttgaaaatcttcttgacaatttgtgacaaattttctaaatgtttttccaaaaatagttggttcttgtaagtgattttgatatgactgattaccaaattatggtgggtaaagatgccacatgcaacagaaaatgtgtctaattatgtttgttttagagcttaagaaatgttaagaagagaagttacaactgcattaataggattttaatttttattcaaaatggacaacttatttattatgtacttctacacacagctaagcttatagatattttcatttaaagaaaaactatttgttcattttattagcagatatcaaatgcccttttgaaaattgagactgatttctaaaacaaaaaaaaagactttaggagttttaattatttttaatatattgcttctttattaaaaaaagatacaatccttcaatgtcattcaacagtattaattgttaaagtgtgggatatagtttacattaccgagtttattttctaagggtagtgaataactcctgacaactactgatatcgtcacatggtcctttagtgaccaaaaatgcacagttgtaagaatgcaagtgttacttgtattgaaaaccggattacattaaaggatggacaattatgataaaggatctgagataattggacaattatgataaaggatctgagataattattctaactttttggaactatactttcactcattgatgaagtaagttacaacgtggaataacaaagtttaagtgtggcagaaaatacatacatatgtttaaaagtagggaaaattttatcaattattaaagatggaaaaaataggactatgtcaaatagttaaacaaatgtggggtattttatggagaaaagaggcatgtactaccttaaacattttccaattggaacatactatagacaaaactgacagattattattcaatgagaaacctgactcagatgaagttacaaaaaaagtactttttaaatgtctagtttctaatagagttagagctttgttgattgagatatgtggaactgccacatatctctgtgccatacttttggtaccttcataataaacggtaaagtgagggaaagggtggaagagacaaatcctacgtctcttccagaacttcgagtgcactataaattaaatatttaaaatatttttgcaatagttagctttcaattatgaacactctcagcctctattgctttatatatgcatttattttggtaatttttatacatcaaaactataattacctgtatttgggcagaatgatttaggttatgccagctattgtggttaaagctgtagtaacttacagtacattgaaattatagactaaggttctgaatattggtaactcactgttgttgtgcacctttaaacaactcttaaataaagtaatgattctctttatattaaatttaatgtatgtgtgcctcatggaaatttgtattttatagaaaaatattgaatattttattattatgtctttggctcacctactttaaggagatggctacttagggtactttttaatccaatataatgtgaaaatttgatcatgctatattcttaatttaattgtacttctatggtcatatacaatttacctatcactttctcacataatcaatttaactttttggtaaatcttctaagagaccgtctagacagagtgaaatgaaagctgaaacaacagtcaaatcaaaaactgctttggtctcaaatccatgtttttcagaaaagatattcagatccagttatctggcaaatggtctcaaacatacatttcaatttcaatgttaaaaataggatattaaacatctcagaaaatattgggattattgaagcaaattctaccctggacttggagtaaatgtgatgaacagattaatgaggtggaagggactagaactttgggaaagtgcaaccttgttatcttaatatttttatagcttagaaagagaatgctatgcaactcatattttgatcttttaatgttaaagaattcaaataaaaaccataaacctgaaactctaaaagaaaaattctgttttgagagagatggcctcctctagtacacttttaataaatttaaagtatctaaaaggatgcacaaagatctctaatgtgctgtgattttcaaaggatgtcatgtataaaagatttgagtgagaacatgaaagcaaaagcaagttcagaagaggaacacaaccaggaggacagtgtgtcaggaaaatccaagaataagtggaggtgtaaaggctaaaaaataatgcaaatggtgcatatccttctgtctttctctcatacacacagacacacttacacaacacatatacaaatacatacatgtatatatgtatatatatacacaaatatacacacatattcacataatattcaagtatgtatacatatatacacatatgtacatacacatatgtatatatacatacacacagattgagagattaaccatatgtagatacacacatgcacatatgcaataatgaaatcatttcaaagcatgccaaaaagtaataaaagatatatcctctgtttgggataaataaaaaaaaagtttaaaagcaaacaaaaaataaatggcaataactaatcacattgaattttgttatggcctttttcttcctaaaaagaataaccccaatctgaacaaagaaattcaaagtaatggaaaactcaacaatgaaactcaaagtagactagcagataagatacctatttcaaacatcagtgccaaggtaatttataggtcagtgcattgataacttttgccaatgatagaaaagatgccagagaaccggatcctgacattaaaaaaaaaaagtaaaaagattctgaagactgcatttctgagcttaaggtagattctaaacaacatcttagaaactaggaaatgactttatgtttctttgtttttcaatgtaaatggatcaagatttcttaaaacagaaatgaatattattatttgtgatgagagcactaggggcaattttgatatttttgataaggtttctagagtaataaattagaatgacaggaatatatattgattttaggaaagtgtctgtataattccacatgatattctctggacaaaatatgaaaaggtaggctgaataacatttttaaagggcagtaaattttataattgttattgattacaatgaaggcctctggtaatgttttccagggtcatatcctgttacatatacgtgacatggataaaaaggaaacaaatatttattgtgtgcctagtttatgttatctcaattccagctctacaaggagctacaaggtaaaattgctacctttaaaaacatatgaggtaaaattattcctattcacagatgtagaaactgagtttcaagaaggttaagtaaatttcctcatattgggaggctggtaatgcagaactgggtgtcaaaatcaagtctgtatgaaccttctgttttgtctcccatgaagacaaaaggcatgcatataaaatttgttgaaacacaaagctgaggaggcataataagacgtggaatgacagaagcaagatctagaaagtttgggatcatgaatcaaaagaaacaggataaaattatcctaaaattaatattaaatcttacaagaaaccccccaaaatcagttgaatttgtacaaaacggtaaatcattttatcagtagatcccataataaatattataaagtttaagtgtgagctctattactcagtaatatgatgccattactgtgttgatggatgtattgtcaaggaaaaagaagagaattacacactgtttccttcaattgttagatggcactggatgtagtgttttcaatgttaatcctggtatcatgttctttgccataaacttgttgacaaattggcaaatactgacatgaaatatgccaatatttgagcatctaaaaatgtaggtactttccataccacatcatatattacaatttgaaaatgtttgtttcattttttatataattattatacagaacagtttttctatgatagcattataaaaattcccagagaatactggcccagtaagaaatggaatgttcacaactcatagtgtagctatatgaaagaaatagatctaaacgacaggttggtttccaaattatattttcatacctggaaaatatctactttataaatagcacaaagttatagttttcaatgaatatgaaaaagttcttgcattaacatattttatgtatcttttatattgacatttgtgattgccactaaaatgtgtattttctaaatttcattgtgcttttacaagatacttttttctttgatgtccataactgctgaaaaggctcccctaaggagaattttaagactaagtaaggtttttagtgagcttaaattatacaattctgaggcattatttaaggtgcatactgtattttttgcttgaaacctgtcagcattttatttgtatggcaattaaatgactcagccattcatgtctcatgccagtctttttcaattgttatttttaacaaagaaaattatatatatatgtatatatatattatatatatgtatatatgtattatatatgtatatatatataaacttacagcaaaaatgtttaaaaatagcaaatagtttgagtatagttaaacctaataactgtacttttgtttctatgcctctgagacaagattactagacccttattcaaagtttctaaatataggaaatagaacattgggccatgctaaaaaaattgttcagattttcttttgaaagagaatagttatttttcctcctgacctctaatgaagatgctttatttgtcaaggtgttttccttagaaaattgacccagtgtcaactgtaaagaaaacatagaggatccttggatgattgaccaacttatccaaacacaggtttagtaaagagaggatataaagataaaatgtgaaatgacctctctgagtcacatttgttttcataatttcctagcaaacatccaacttcactgctaccctcagcaatgtttcttgaaacatttttaagacattgatagacaccaatagctgatctttagaaagccattcccagaagaatatgtaaggggttacaactcatttcagggagtctgcctagctcttgatattacatgtctttggcatacaattgtgtaccttttatcattgacagtgaagaaaataatgccatttgtaacttctgagatatacacacaatactatcaactagccggttaataaaagataagaaaaataaagaaaatagaacatttttaggtgtctggcaagtatcctctaaatcaaggtaaagataataatttagtggcagtgttcatattttcctatgactgtaagatttaggtgcctcacaaaatattaatatttagcctcttatgaaaggttcgtttttcttctaacactttagtagctgaatacaaagaaaatacacaacagctgtttataaatgaaataaaaagtttccattttttatctgagtttctcatttatttgcagagaacgaataaaataaaaatatcctagtgttgtttgcaccacagcataccagtaaatcttaaggattgtgtttcagtatgaaaaggaagagcaggaagatttcctcattctgtcttaccagcaaaagtctagccttcacacacacacacacacacacacacacacacacacacacacacacacacacacagagtcatctatatgaacacgtacttgagtttcttaaacatatatgaagcaccttccatttccctttataataaatcccttagtttttgctgttcattaaaaaacaaaaaggaagagacaagctcaggacattctgaaaaccaatgtctttaggacacactaaggtgtcctgaattactttaacggacacattgtaaagacacactctccaatccctattaggaaaagtttagtcaagtttgcttactatttgggtgcttataccaaaaaagcatcatttaggacattatttaggataatattatttatgcaggaattgtaccacctatttccagatggtataacttattatctgacaggcatgtagcaaatagaacacaaagcataaatctgtcaggagaaatcatacgagaaaaagagcattgtctggttatcagaatatcagatctctcattctggccttgctaggaaatagatctttgattctagaaaagtcaactaatttctatggttcttacttttctcctttataatatacccatttaaattccaaaaaggtatatgataaatcacaataatttcaatcacatggattttaatacaaaatgtataaaatcaatttccaaaaattttctgcatatactgaaaatgtctgtacgaatgagctaactactataggccttccctaatttattctattaaatgtgggtactcaatgtaacctgaaaatattgagcttaactcttctttttttttttcaaaagggaaacttgaaaaagactgcttcccccagaaaatttatcaacaataggtgctcaattaaatgtttttaaacaatgaacaatatcccctttcatataaataatcaggggagagatatttttaagtcttttttttctttttccatagtgtcacctacacaaaaaattatgtaaagacaccacttctatgaggaggtattcattgtagatgtacagaagtcaacggaaacttaagtttacagaaaaaataaaccagattatcattccacccaactgtatattcccacagatgcttaataaaagctatctgatgatataatgaattatcagttcttgaggaagtatatacagttggtgactatttttcaaaaatcatcatccaacaaatttttttcatttaaaatctttcatattaccctttcgacaatcagttgaaattttaaaactaagaacatttaaaaatataaatgaaagtagcattagctatagactgatattcaacttcagacgttaaaataaatacaagtgtgtattaagagtaaaattatgtcaacaatgtataaatgaaaactgccaatgtaattaatgtttcttttaacatatcccatccattgctttccctccaaaagacaaaggtagcaaaagacgaagcaggaagaactgcttcagaaactgaacatactgatttaattggctaagaagtccaaatgctaatactcctaataattagccattccttttgtgttttggtgacatatatcctcatacaatgtatatcaaatggaattttttgatttacacctgacatttcaaagtttccatttttgaattctcctagtcttaagtaagtagaacattgtctcctttgtttgctaggcataacgttttccccaacatctagggctccatgatgcaaaatatcattttgccgatcttctgttccagtatttactttaattttttttattataattggattttcaaatacaatcacaaaaacatctcctgttgaaggtggtttcccccaaaagtactcatcaacactactgtaagccttgcttgcttcataattttcaaacacattcatgttggtgtacagacttgcaggggggttatcaggaatgtcaaatgactcctcttcaaaatcatcatccttcagcttattctccgtccctttgtatgatgaataatagcccatgtgctgaaagagagatggtttaaaacggatcacatttttctgagccaacagaccacggaaatgagtcaatagccaatcacaaggcatttcttgataaaacattaataaaaaatgggccaaacgtgggagatcatgagaatgatagagtttaccaatgtagccaagcttagagaattcaagagttacccagtaagttccttctagggatgcaatgactttcttgatggcagttaagaaattttttgaacatcgaacatcatcttcaagcattacataatagtctgaagtattggcacaaaaattaagcagaaaagcataatctacattttgcttggaacgaaatttgactctatcttctggatcattgtaatttcttttaaggccatctaggattgggtaatactcctctggagcatgtataaccattaatcttcctgcaataatatggtgcgcaaatttctgtgtaatatcctggaccatggcatcacgccaggaagaattaaagtctgctaggtgaaccaccactgaaatttccttcagctcttcatagctggattgctcaaaaattgacttaattgtctcaagtaaatagtttcctttttttcgctttactgaagaaagtccaattgtaagataccgctttctttgtaaaggtgtggcagctaggtagcgataggtgacatttatggctcctgagaaattagataaatccttgaaagtatgaacatagcgttctgaattcagttgatgtgtggatgtttcccttataagttgtttgtctccttccagaacatagctatcttcaatgtacaagttcataaaaaggagaaaaatgacaagaactcccaagaatgacactgtagaacgttttctcaggcatctcattttatcaagtatttcaaaaatatgtttcatttgatgaaatttaaacattctcttctttgaagctttcgtcttcacttctggttgattgatggatgagccattggtgatttcgactcctgagccagtgctccaaatgataagtctgttgaagcacagtgagggctgagagagcctgagtacactatacagaggctgagttagtcctgtttctttttgtaagaagttggtatagtcacatgcttctctgttaggaaggtactggctgaattgtaaatcttacttcctgtttctgtctttgagtgggaatttacttcttgaatccctgagctgaaatattttccttggttctttgtgaggcaactctgttctatttgatcctatttctcccacggtaactttttagtcaacggaaacccccttcttaaactctcactgatcgtatactccacttcctttcttgtggtcatggttttgttaaggataatttgagacttcaggatctctttgggaaactgaagattttcccgaagtgagtcctctgagatctcttccttcccattgcttctgctcctccttcatccttttactaccttcaatcttcccttcagctttcttgaatcttttgatatgtgcctcttcagacctctttcctctgtctacctgtcctcccagacgtttttccttcctgcttcagcccttcagtcacctgaactttaggtctcctatttccatcataactttcaagggactctaggaccccaaaagcaattgtctgaggttgaaaaaggaaaaaaaaaggctgattgaaaaatagattggatattttatccagatgaggctttggagacatccagataggtgcttgatgttctttcagtttcttgcctaaaatgtggtcacagcctccataacattgcatgtatgggcaaaagaaaatcttaaatgtgtcttctccacaaatattggctaaaagctttagtcctcatattgagaaggtaaccttaacttgttccatctgtcagaaacacaatgaataaaacatcctttaccagctccaagtgttaaagtaaaactttggtctcaaatttgcaaccaggtgagcacaccctgataatataaacttccatgtcacatgctactgcggcttttctagtgtcagtcaggtccacagaatcttaagaaagacgctgtcataatctgtgctgtacagaaaccgttgatacccagagacagagaaaacaattcgttcagctagatccaacagtgctctgtgcagcctggaagcatgagtgatccttgggcctcacacaaaagcgagataattggctctcaatgaagagatgtaaacatccatcataatggcactgtgctgaaact

SEQ ID NO: 13492 - RNA, 22693 nt, Homo sapiens
  source 1..22693: mol_type = other RNA
gctgggattacaggcatgagccaccacgcctggccagtttttaaagtatttcatacagtgtaactaggcagtcagaaatacctgtatctcaaattcatttaacttttcaatgaatcaatcttcttattttctcagacatataaattatcataatactttacattgagtctctatggttgactatatgctgtgaaggaaggacataaatacatgtgaggaaacaattattgatatttttaaactaactagaaagcaccaagttatttgttaaataaacaaagttaattttatctacctgttcagtaagtgttggcaactatgaattaatctttgacaaattcacttacaactagcaattttaaagacttaaagtttaatttttattattaaaagggtatgattatttttactaaaattaataaaaagattaactgttactaaattaaagctccttcaaaaacataaatgtattctttagagagttaaaaaaagtagcaataaaatacatttttaatttagttaagcttacttaactaatgatcaaatagattaagttgtataaaattttacaaactttatatttttgcatacacttatcttcctggcatttttgaaataaaaaaaatacaagtgcatagggcagaggaggcgattcagttacttctgctatgttattaaatctctggtaaccactatacaatacaatacaatacaatacaatacaatacaatacaatacaatacaatacaatacaatacatgtagactcagcatccaaactttattttaccttcaagttctacctgataaagtggtggaataaagatggtattttccataactgtttaataataatcacatgttttatacccattgctttgaagaagaaaccttaagcaactagaaatgtcaatctaaaaggcagaaaagctggaaaaatctcatgaagactagaagatttacactcataagatcatgtaaatttatttggatatgctgaaaaaagagggggtataaaatctaaagtttggtaaatctttgctttacagggcttcaagttatagatttttcttttttccttttctcttcccctttctctctctttctcttttttatttttgccatttcttctcaggagcccctgcaatttcaaaccttggaattgaattggatttgaggaggaaaacccatattcagctttaattcaaatgaattttactactttagacaaaggtacaacactctattcaaaaaagttattgaaatcacatctttaaatctgacccagccacttgaataaataagttgtgttgtagtttctcagagcaaccgccgctcatctttcactcaccttaacaatttctcacttttttctgctttttttttttttttattttctgcttgctgaaatcgagatcaatattcattgttttcttctgggttaactcttttttatgttaactgaatcaattttggctttgtttctttatgaaattacttttagataaagtattgatattgtcatttatcaattttattatatgtcttttgcttattaaaggattaaaatccacctctaaacttatttagatcaaggtcagtttttttactcctctgtagaactgtgaagataatatcctattctccttttcttatggttttattgtgaagatctgtgcaaatagctatataaaatgcaattcggtattaaagaaaattgttgcacggactacattgattagagtctaatttttggaaagtatacttcgccttttcagtaattttatttttcggtctatggtgcccacattgtgtcaccagccagccgtatgcagacttacaaaggactacccactaagaataaaaacatgatacaacttgaagaaattttcatcaaacgtctttgtcttatccccttgttatacagacaaagatgacaagggccgaaaaggaagtgattttctcattgaataagagaatccgaactggcatcgaggatatctaattttgggatgaaaattgagagaagacagaatttcaagtctgaattatgacttcactactgtgtcgtcattggtagaataaggataacaatacttatcacacagatttgtggtctgaatcacatgagagacatagatgaaaaatgtaaaacaacaattagcatgtgacatgctctcagcaaatcaattaatccttcattctttttttctccccttactcctttgattttcagactaatttggatcatgattattggcctgtgtcccacccattattcacatatagaatgggttgcattatcctctccttggaaatatctttcaaagtgggtaatgagaaaactactttgaagactgtgctgaaggaaatgatggcatgaacaactctagataatttttgtttatttggatataacgtgaatgggcccataccataaactcctattaagctgaatcaccaaaaaaaaatttgatatgaaagtcatacattgaaaaaattcactcttaccactgatttgattgatactgagcctgtaaatatttatttatatgatgtttggcactttattttataaaactaccctttacttaaaataaatcattgtattcacataactttccagggcactatgcatttttaaacaagacagtcaacttactatttaaaaaacaaagtcagtcacctaaatgactttctgactataaatttgaaaacaatattctccttgtaatatatgtgccaccagggcaagaattacaaattgggagcaggtaagaaaattgttgttgactctcattagtattctaattctccttcagtcagatttataaagtatgacctatagcatccaactccatcattttccagtcattcttgagactgtcaactctatgggcattgtttagcagcctcgaaacactgaactttttacagtcttattggagagaaaaacacattaaatgatcaaataatcttttatgagctcagaaaaaaatgcctaacatgaacatttaagcatcttctgtttctgtgattcccatttttggagagtaaaaatttaagaaacaaagggaatgtgtctggggatggtactaataatattgagattttacaatttaggttataatcaagataattatgtatatatataaaattatatatggtatagtttcaacttctaatcttttatcatcctctaccacataattcctcctatattctctttttctgactgtggcctaatacctcaagaatattgtatatgcttgtcactatataaacttcaccctaaggaaatttccatgtcagatacaataagagcaacggaagaaaatgtatcaaaacacatctccaatttatttgaatttttctggcctaaccttgttggcatgagagttcccactttgtattataataggcaaattgatacacacttttcatttattctaaataatagattagcatagtcaggaggcttggattggcagctattaaatacaatttgaagccgtgggattttattaggattctaaggttattctgtgacgatggaacttaatgatgtaagagttaattacccattgtcaaaaatcattgcccatcaaagcagtgagactgtgtgctatgtccagttttattcatttcttttgtgtatctgaatggaacatgtggtaaacacaacagtagaatatacctacagtccccttagaaactcttaaatcttcaatttataaaagtcatcctaagacgttaaaaataacttacgaaaggatagattccaatgtcagtgggtgagatgtgctctagctagtgtgcacgaaagagaacatggagttagaataattattgtaggactgtagattgtcatctcaagatcagtgtcaaatacattcattcatgtagtattttcacatgcattctggtctaaatatcccaacatatctttcgttttgagatctgcagaacaaagtcaatgtctgaatttagagactaatttgaccattttgattcaaatgtctaaaggctaaaccagagcaatttacaacatccaatgaagtaaaattatataattaattatataattatataattatataaaattttataattaattataaaataaaatattaacaataattgaacattgtttacttttttatcctcacaacaattcaacatgatatgtatggttattactaaatgtataatacatttagtaatgtgatttgacaaatcacatttgtcaaataaggaatggctgaattaaatgattgaatgaaggagtgaaggatgtagattgtttaagtacattcaacttgtaatgaactgtaaacttcacccataacattattaatatatcagtgctatcaactacattttacataggatgaaaaaaatcattatttttattaatcccaagatattttatttcattatataaatgaaatattttatctgttataaagacctttatttttgttccactcattaaataacatggtaagactgttgtgtaattgactgaatagttaagtctaaatgggtaaatagctgtttatgttagtattgcagggtagctatttgataatgaaatatacttttcttacctacttgcaaaaaaaattacataaacaagtatttcctagagttcaaacactgatctttttaagtggcaaattgtccaaaagaatttaattaatataaacaataaattcacttaaacaactatttacatgcaaaagtaatatttttattgcccatttggaaaatagttttgctttctggtttataaggaacttttactagtttaattacttgggtgctttaaatgttttttggaggctattacaaaatcacatcctaaaattttaaaatggaaaaattataataattgaatttttaattcctcataaatattttaaaagtacacattgttccatggcttttgcctttagaataaatacaacatttttatgtagaaatatattcttgaaatgtaactagcacatagtcagtgtttcttaaccattttggggtcctgaaactttttgataatgatgaaagcacagagatgctatcaagaaaaatttacccacataggaacacacacacatacacacagacacacacagagtttgcttataagctcaggaagcttaaagatctgctaaagattatgcttgggtttgccatgaatcataaataccaagtcaaatacctttgaatttgattcttaacaaatctttgtggctgagaaaccatgagatttcattctggcatgtccccagaatgtaattatcaatgaacaatagccattgaaaaaatctgaacagatattattgaggctcaaggttgtttaatggcacagataatataattcaaatcatgaccccagggctgatgaagtcttgttgtaacgtgtaaatggggtgggtgatgggagagagaaaacaaaataattatttatgttaaatcatacataaacagtaaagccaacacaataagtaaaataagagaaagtagaatgcttgggaggtcatatgtttcaaatgtatgcatacacaaaagagtaagcaacaggatacttcaagagtaaaatgggaaaaaatcatattgggtaaatagtatcaccccaaagtgatagtcaaaagtacctatgtttgcctagttctcagattacaactatgatgataatttagataaacaagcagaaaacaaaactatagaaaaaagtcaaagtgacataaaacaattactggtgtttcaacagaaataaacccaacatcaggatttatcaaatatatgaaaaattatgaaagattataaaacaccaatgattagattatgttataaagacactatgaagagatactaaatgatattcttttcatctgtggttactgctaaaaaattctttcatagaaattcttggattttgaaattagtttaattccaaaatattttctttattttgcaaaaatgtaagacaaatgtataggatatttttctctgttgttatgcaaggatttattatcacattggccacagaacacatagaatgttagttttgtagaaaattttagagattttaataccaggatgaaataatagtatcattctatttcaggttcttaagcaacattcctaagactagaaccttatcttgaaaaattatgattttaaacttaagggaattcaggtaaaggaaattgactaggttaaggcaaatacatcatgtttactggtaaagataacattatttaaggaaggtaagatactcttatcctacatatacgccagaaaaattgcttctcctctgaaaactaccattatttttgccaaatattgtagcttagttttaagtttttctcggctgtttcctctgacagttctgtggtaaagaagaaacattataggaagcatttttttttcctacagagtctgccatatggagaagtagaatgagaggccacctaggtaatgtgatttattaaaagttctccatcccaaaatatatgtcccatctgtgggctaatgtctgaaagtcctatgattaaactcacttttatgtaagatagtgaggccccagagagccctcgagaaatgcaaataaactattactgacctcccttggattatgatgaaaaccgtggagtctttctattctctgtcaaatgtggaggtcatggatccttcttggcacctaagattaaaactcatagaatgtgctttaacttctgtaggcacatttcctttccaattagagtgaggtgttgaatatttatttatttgtttatttttattatactttaagttttagggtacatgtgcataacgtgcaggtttgttacatatgtatacatgtgccatgttggtgttctgcatcttaagagaagactatttataaaatttattgcttgtaagatttgttttttgttctcttactattatgaaaatcacgaacttgggaataaggacactctgggcccggcgcggtggctcacgcatgtaatcccagcactttgtgaggccgaggcgggaggatcacgaggtcaggagatcgagagcatcctggctaacaaggtgaaaccccgtctctactaaaaatacaaaaaattagccgggcgtggtggcgggcgcctgtactcccagctactcgggaggctgaggcaggagaatggcgtgaccccaggaggtggaacttgcagtgagcggagatagtgccactgcagtccggcctgggcaaaagagtgagactctgtctcaaaaaaaaaaaaaaaaaaaaaaaaggacactctgaacaattgaacaagactacgctgaaaggcagagaagaagtaattatgaacaaactgttcatgaagtgatcaattgaatttgaaacagaacttttcctagcttctaaatgattagaaatttcagctttggtttaacttaaaaacttagaattgtcaattctgtccaagtctctgagtcatgtacagaactcaaattattacatcatttttttacttatctgtattatttctccatttaaaagtggacaaatttttatactatatcctaataatgatacaaggtgacttgtaggactctggatagaaagagatggcccaggatacagagggcactccttaaatagctgccaaataaatgacattaaaaaatgtataaaaaggtatgttaagtaattaaaagtgtcaggcattattttcctattatgagacattttatattatggttatttactgtaattgcatccaaaataattcataaaacatttatttttgtactattaaaaatctaaacaataataaccagatggaggaaaatgataccatctgatttaattattaacttgaaggtcagtttctacaacttattctcatttatgtttatctgatttggccacagtttcttactttctcatattttgctaagcttgtggatgaagccgcatgtctcttttttttttaacctggcatataacactgtcactctatttaattattacccatcatctacctactttgaaactttggaggttttataaaaattatgagtatttaatcaaagttgtctctttatcatttgccagtgaaaatataaaacctggctgttttattctattgtgcactctaattacataaccaaaatctttttaaaaattcttagttcttttagaaataccatttgacccagccatcccattactgggtatatacccaaaggattataaatcatgcttctataaagacacatgcacacgtatgtttattgcggcactattcacaatagcaaagacttggaaccaatccaaatgtccaacaatgatagactggattaagaaaatgtggcacatatacaccatggaatactatgcagccataaaaaatgatgagttcatgtcctttgtagggacatggatgaagctggaaaccatcattctcagcaaactattgcaacgacaaaaaaaccaaacactgcatgttctcataggtgggaactgaacattgagaacacatagacacaggaaggggaacatcacacactgggcctgttgtggggtcaggggaggggggagggatagcattaggagatatacctaatgttaaatgacgagttaatgggtgcagcacaccaacatggcacaggtatacatatgtaacaaacctgcaagttgtgcacatgtaccctaaaacttaaagtataataataaaaaaattcttagttatttgaaaatagtttttttgaattcacaaacttgcaggatgaaaaaagttattagttcctgaagatataacattgatttgtctttttcttatttgatatcagctagcagtaaaattgtgaacaaatctggtaaatcttttggtgttgcaggttcataatcagttaattgagtgtattcactataaattgctttaattaagtgatgtttgcctaagaacaagtttcatttcatctcatgaaaaaaatgttactttttgtattaatcagtggaatgtttaaagaaaaaactggttatcttgaagctgtcaaataattataagaaatctctatacattacgttttaaaatacataaaacccataaattcaagcttattagttttcattttcagcaaggtttatacagagaaaataagtaatacaaattagttttccagaaaatctaattttatgcagataaaatctgaaaatcatataagtccaagatgaaactgatctcaaattattattttgaggtgtatccatttatttaaaaaagcctcattttagctagcaacactatgtagaaaaatattttaaataagacagagcattaaaataatgtattcattgatctcataaagaatagatgatcagattttttaaaagtgattttaattaaatggacatgtttctctttagccagaaatgactgagaaattttgagttggaattgatataggggaatccttggaactatgtgtgaatatgtgtgtgtgaattatctgtgtatatttacataatttacactattcacagtccttgtttttcttgactcaaatagctatctcaagtttcgtacactttttagatctctatgtaaatacattatttcatttgtggaaatatattgaggcctatatcaataacctcaaaccttttaaacacttagagcaagtcaatatgacttgttctgtttcagctatctgaaatttaaaaatttgacaaatttttaaagtacccagttcttggaaaaagaaaaacaaataaattggagatttggatcatatgggctatgactaaatgagacaaggcatacatgctgacatttgaaggatttatgaaaaaaagtccactgtggaaaactgatagtttttctccttctttcttgaatatgtttagttaattttgtggaaagaggaaggcagctcagtttacaaacagcagtgggttgaaggcaatgctgtttatattcttgaatttcaatatctacaaagatgtcatcattagattttatgtgttaaaaagtggatttatagtctctaattaataaggtgcatatgtcaagactcaggaaaacagatcacttacgtagttctccaaaaacgagagtcccagattcaataggaaggcatgcagagtgttctctataaacccagcaaaaccataaaaattgactggaacttttatttttcagtacaacaataatagtattgaaatacctaaaaagggcaggaaacaacacagaataatctacgcttgtcatcatgttttctaatctataatctttcaaactggataaatgggaagttttggaattttactgtggtacagtcttagttgctccgtggttgtcaaatctgtctgcacattaggatcacttaggaagaattttaaaagtatgctgatgcctggaaactccagaacaattatgataactctgagcatggagctcaggaatgggtgaaattcttccccagagatgttaatgaacagccagacttaaaaactagtaatttagacaagtgtgagcagaggttaataatgttgagatgaactgggcttaatatttcactaacaaggtcagagttttgatacatcacttaactcaaactttgagattcttcatcactgaagtagcaataataatagtcatttctgttttaatacttcatagacttgtaaggatgtaatgtagtgtttctaaaaggagtgaatggacaatctgcatcagtgttaactaaaatacattgaaagtgccaattcctagatctatcctagatttacagggaagaattcagtagtctgaaacacacattttcaatatattgaaaagatgattcttttgcatgatgacttgttataatcattactttcataggtaatggaagtaccgattaggagagtaccaaatacatattaaacactcagttcatgtaagctataggccaataaacacaactttggggtttactgatgttttccaacatccgaaataatagctgaaatttagaaacatagttaatcacacaaaaaatgttgcatacatactgtctaactaccagtttggtatgtttggggctggtgttatgaaagactattatatgattaatacaaagttataatttttggagtcttttagtgtacccagagcccatgagtttttattttctttttggaataacagaaattaggttgtggttcagtggaattacagaagcaagtgttttagatgttcaagtttaaaaaatgagaaaaaaatgttttacatgaagaaactaattatttaaattcatttttcaactatttaatgttattttaatatagtcatatcatccagaaaatcccatcttagacaaatgggttttcaataaattattattatagttaggaggcaatgtataatagtgataaggggcatagattttgaattacacaaacctgaaatccaatgctctctctttcatttattagttatgtgaccttggacaagttagtaaaaccctatttttcatatgctctttagcttttttaatacctcttaccttatatggttgtttaatctattaaatagacagtgaaatgcacatgaaatcttcacacagtgtctcatagttgcttggaacatatttatgtagtaagcattgttcttggctgagcttacattaagtgatctgtaaattagaagttatttgttatatttgtttcgtttccttattgccctagatgccttttctctggacctagataatttagtctcactctgtggcctttacccttcaataaatatggattattaatataatttagctacataattcctaaggaaatattaattcataaagattgttaaattgaactgaatatctttgctaagtcacaggcattgattaaattagataaaattgtcattttccattgattttgtttatataaataatattgaattatttatattcttatttagtctagtagattgacaggcagttttattaagaaatgaatcaaatggtaaattttgaatcatctggtaaaaatggacaaaatttagttttatcttgtggtctggaaatacaccctaaattattgggtcaagttagtgaaaactgttaaattgattatgaacgtaggcacattacttataaatccccttatgctaacttaaaacttgtgaatgtttagtgttatccagctataattcttctaaacatgtcttgtaatttttaagtttgcatgaaaataactccatcctgagtatactcatttcaataaattatttgtcctgagcatactgtaagaaatttagtaaagtactaattgaatttagtgattagactgtgattagactattacaaattcacagtgcttgtacaattcagatattattttgctttgaagtcaaatagaggaaccttaaataatttaaataaaaataattgtttttattaaagtttatacagcaagataataaattcactaatgtgaaatgttgatatagtatgtacaacttgtttcttaagttactaaaaatgtattttcctacctacataatgtcaatctctattgctcctaacacatgagtggctaaaattgcaaacttaatcacataaataatgagattaaagttaaaatgaaaaagtggtatgaggactattgtttgtgttaagtgaaattataccttgtaaaatttcatattatgagagcaatatgtaaatttcattgcaacaatggttattcaatttactgatgaaaatcagaagaatgttgaaaaattagtgcatttataataaatttaattattcataaaaaattaacattgatatatatattcataaggataaaagatatcaaaataattaaacaaatttcactttcttcttataaaagaaaataatttttatggtaactaattttagtagtgcatcagatcaacactattgggcacccagttatttggtggtacgctgagtgaaaatatgtagctttatctacattaccttggtttggacaactgaaaaatttgctaggaaacaaatattacaaaatatgttgttaacttttcaaagatgatcggtttagattgctttaacttgaaggacacttatattttgtatcacttttgtagcaaacacatgactcatcattgcccaaatcaattgcccaaatcaattcaaacatctcattgtagttcatcccatggcagaaaagtgtttatccacttagtaaaatggaaaacactagagcttcaggtttaatttgaaattttaacttcattaagaataaacttgacctgtttgttctagtaagtaaaaacactagatacgtaccaaaattgtcttttgaccctctcagggagtcaagttttgatttgcttgaatacaagcaagtcgagctatggtaatttgcaatgctgacaggaaagaagaacttgcttgaggcaaaatcatgaagtacaacttttcctctgcatccttttacctcatgtttgtaacatttcccctgttgttatttttacacatctggatgctcagaaaggcctccttaccacaataattgaaaggagtactttgtcaatagtcagaattgaatgagagataggttgttgggaatattcagggtgaatgtgtcttttctactttgactatatttaccattgactacagtaactcagcagaaagttagagggcagcatacatacattggtttatggatttaatgaaaatatccccaaccattacattacagacaattcatatatatgtcttgaaaatcttcttgacaatttgtgacaaattttctaaatgtttttccaaaaatagttggttcttgtaagtgattttgatatgactgattaccaaattatggtgggtaaagatgccacatgcaacagaaaatgtgtctaattatgtttgttttagagcttaagaaatgttaagaagagaagttacaactgcattaataggattttaatttttattcaaaatggacaacttatttattatgtacttctacacacagctaagcttatagatattttcatttaaagaaaaactatttgttcattttattagcagatatcaaatgcccttttgaaaattgagactgatttctaaaacaaaaaaaaagactttaggagttttaattatttttaatatattgcttctttattaaaaaaagatacaatccttcaatgtcattcaacagtattaattgttaaagtgtgggatatagtttacattaccgagtttattttctaagggtagtgaataactcctgacaactactgatatcgtcacatggtcctttagtgaccaaaaatgcacagttgtaagaatgcaagtgttacttgtattgaaaaccggattacattaaaggatggacaattatgataaaggatctgagataattggacaattatgataaaggatctgagataattattctaactttttggaactatactttcactcattgatgaagtaagttacaacgtggaataacaaagtttaagtgtggcagaaaatacatacatatgtttaaaagtagggaaaattttatcaattattaaagatggaaaaaataggactatgtcaaatagttaaacaaatgtggggtattttatggagaaaagaggcatgtactaccttaaacattttccaattggaacatactatagacaaaactgacagattattattcaatgagaaacctgactcagatgaagttacaaaaaaagtactttttaaatgtctagtttctaatagagttagagctttgttgattgagatatgtggaactgccacatatctctgtgccatacttttggtaccttcataataaacggtaaagtgagggaaagggtggaagagacaaatcctacgtctcttccagaacttcgagtgcactataaattaaatatttaaaatatttttgcaatagttagctttcaattatgaacactctcagcctctattgctttatatatgcatttattttggtaatttttatacatcaaaactataattacctgtatttgggcagaatgatttaggttatgccagctattgtggttaaagctgtagtaacttacagtacattgaaattatagactaaggttctgaatattggtaactcactgttgttgtgcacctttaaacaactcttaaataaagtaatgattctctttatattaaatttaatgtatgtgtgcctcatggaaatttgtattttatagaaaaatattgaatattttattattatgtctttggctcacctactttaaggagatggctacttagggtactttttaatccaatataatgtgaaaatttgatcatgctatattcttaatttaattgtacttctatggtcatatacaatttacctatcactttctcacataatcaatttaactttttggtaaatcttctaagagaccgtctagacagagtgaaatgaaagctgaaacaacagtcaaatcaaaaactgctttggtctcaaatccatgtttttcagaaaagatattcagatccagttatctggcaaatggtctcaaacatacatttcaatttcaatgttaaaaataggatattaaacatctcagaaaatattgggattattgaagcaaattctaccctggacttggagtaaatgtgatgaacagattaatgaggtggaagggactagaactttgggaaagtgcaaccttgttatcttaatatttttatagcttagaaagagaatgctatgcaactcatattttgatcttttaatgttaaagaattcaaataaaaaccataaacctgaaactctaaaagaaaaattctgttttgagagagatggcctcctctagtacacttttaataaatttaaagtatctaaaaggatgcacaaagatctctaatgtgctgtgattttcaaaggatgtcatgtataaaagatttgagtgagaacatgaaagcaaaagcaagttcagaagaggaacacaaccaggaggacagtgtgtcaggaaaatccaagaataagtggaggtgtaaaggctaaaaaataatgcaaatggtgcatatccttctgtctttctctcatacacacagacacacttacacaacacatatacaaatacatacatgtatatatgtatatatatacacaaatatacacacatattcacataatattcaagtatgtatacatatatacacatatgtacatacacatatgtatatatacatacacacagattgagagattaaccatatgtagatacacacatgcacatatgcaataatgaaatcatttcaaagcatgccaaaaagtaataaaagatatatcctctgtttgggataaataaaaaaaaagtttaaaagcaaacaaaaaataaatggcaataactaatcacattgaattttgttatggcctttttcttcctaaaaagaataaccccaatctgaacaaagaaattcaaagtaatggaaaactcaacaatgaaactcaaagtagactagcagataagatacctatttcaaacatcagtgccaaggtaatttataggtcagtgcattgataacttttgccaatgatagaaaagatgccagagaaccggatcctgacattaaaaaaaaaaagtaaaaagattctgaagactgcatttctgagcttaaggtagattctaaacaacatcttagaaactaggaaatgactttatgtttctttgtttttcaatgtaaatggatcaagatttcttaaaacagaaatgaatattattatttgtgatgagagcactaggggcaattttgatatttttgataaggtttctagagtaataaattagaatgacaggaatatatattgattttaggaaagtgtctgtataattccacatgatattctctggacaaaatatgaaaaggtaggctgaataacatttttaaagggcagtaaattttataattgttattgattacaatgaaggcctctggtaatgttttccagggtcatatcctgttacatatacgtgacatggataaaaaggaaacaaatatttattgtgtgcctagtttatgttatctcaattccagctctacaaggagctacaaggtaaaattgctacctttaaaaacatatgaggtaaaattattcctattcacagatgtagaaactgagtttcaagaaggttaagtaaatttcctcatattgggaggctggtaatgcagaactgggtgtcaaaatcaagtctgtatgaaccttctgttttgtctcccatgaagacaaaaggcatgcatataaaatttgttgaaacacaaagctgaggaggcataataagacgtggaatgacagaagcaagatctagaaagtttgggatcatgaatcaaaagaaacaggataaaattatcctaaaattaatattaaatcttacaagaaaccccccaaaatcagttgaatttgtacaaaacggtaaatcattttatcagtagatcccataataaatattataaagtttaagtgtgagctctattactcagtaatatgatgccattactgtgttgatggatgtattgtcaaggaaaaagaagagaattacacactgtttccttcaattgttagatggcactggatgtagtgttttcaatgttaatcctggtatcatgttctttgccataaacttgttgacaaattggcaaatactgacatgaaatatgccaatatttgagcatctaaaaatgtaggtactttccataccacatcatatattacaatttgaaaatgtttgtttcattttttatataattattatacagaacagtttttctatgatagcattataaaaattcccagagaatactggcccagtaagaaatggaatgttcacaactcatagtgtagctatatgaaagaaatagatctaaacgacaggttggtttccaaattatattttcatacctggaaaatatctactttataaatagcacaaagttatagttttcaatgaatatgaaaaagttcttgcattaacatattttatgtatcttttatattgacatttgtgattgccactaaaatgtgtattttctaaatttcattgtgcttttacaagatacttttttctttgatgtccataactgctgaaaaggctcccctaaggagaattttaagactaagtaaggtttttagtgagcttaaattatacaattctgaggcattatttaaggtgcatactgtattttttgcttgaaacctgtcagcattttatttgtatggcaattaaatgactcagccattcatgtctcatgccagtctttttcaattgttatttttaacaaagaaaattatatatatatgtatatatatattatatatatgtatatatgtattatatatgtatatatatataaacttacagcaaaaatgtttaaaaatagcaaatagtttgagtatagttaaacctaataactgtacttttgtttctatgcctctgagacaagattactagacccttattcaaagtttctaaatataggaaatagaacattgggccatgctaaaaaaattgttcagattttcttttgaaagagaatagttatttttcctcctgacctctaatgaagatgctttatttgtcaaggtgttttccttagaaaattgacccagtgtcaactgtaaagaaaacatagaggatccttggatgattgaccaacttatccaaacacaggtttagtaaagagaggatataaagataaaatgtgaaatgacctctctgagtcacatttgttttcataatttcctagcaaacatccaacttcactgctaccctcagcaatgtttcttgaaacatttttaagacattgatagacaccaatagctgatctttagaaagccattcccagaagaatatgtaaggggttacaactcatttcagggagtctgcctagctcttgatattacatgtctttggcatacaattgtgtaccttttatcattgacagtgaagaaaataatgccatttgtaacttctgagatatacacacaatactatcaactagccggttaataaaagataagaaaaataaagaaaatagaacatttttaggtgtctggcaagtatcctctaaatcaaggtaaagataataatttagtggcagtgttcatattttcctatgactgtaagatttaggtgcctcacaaaatattaatatttagcctcttatgaaaggttcgtttttcttctaacactttagtagctgaatacaaagaaaatacacaacagctgtttataaatgaaataaaaagtttccattttttatctgagtttctcatttatttgcagagaacgaataaaataaaaatatcctagtgttgtttgcaccacagcataccagtaaatcttaaggattgtgtttcagtatgaaaaggaagagcaggaagatttcctcattctgtcttaccagcaaaagtctagccttcacacacacacacacacacacacacacacacacacacacacacacacacacacagagtcatctatatgaacacgtacttgagtttcttaaacatatatgaagcaccttccatttccctttataataaatcccttagtttttgctgttcattaaaaaacaaaaaggaagagacaagctcaggacattctgaaaaccaatgtctttaggacacactaaggtgtcctgaattactttaacggacacattgtaaagacacactctccaatccctattaggaaaagtttagtcaagtttgcttactatttgggtgcttataccaaaaaagcatcatttaggacattatttaggataatattatttatgcaggaattgtaccacctatttccagatggtataacttattatctgacaggcatgtagcaaatagaacacaaagcataaatctgtcaggagaaatcatacgagaaaaagagcattgtctggttatcagaatatcagatctctcattctggccttgctaggaaatagatctttgattctagaaaagtcaactaatttctatggttcttacttttctcctttataatatacccatttaaattccaaaaaggtatatgataaatcacaataatttcaatcacatggattttaatacaaaatgtataaaatcaatttccaaaaattttctgcatatactgaaaatgtctgtacgaatgagctaactactataggccttccctaatttattctattaaatgtgggtactcaatgtaacctgaaaatattgagcttaactcttctttttttttttcaaaagggaaacttgaaaaagactgcttcccccagaaaatttatcaacaataggtgctcaattaaatgtttttaaacaatgaacaatatcccctttcatataaataatcaggggagagatatttttaagtcttttttttctttttccatagtgtcacctacacaaaaaattatgtaaagacaccacttctatgaggaggtattcattgtagatgtacagaagtcaacggaaacttaagtttacagaaaaaataaaccagattatcattccacccaactgtatattcccacagatgcttaataaaagctatctgatgatataatgaattatcagttcttgaggaagtatatacagttggtgactatttttcaaaaatcatcatccaacaaatttttttcatttaaaatctttcatattaccctttcgacaatcagttgaaattttaaaactaagaacatttaaaaatataaatgaaagtagcattagctatagactgatattcaacttcagacgttaaaataaatacaagtgtgtattaagagtaaaattatgtcaacaatgtataaatgaaaactgccaatgtaattaatgtttcttttaacatatcccatccattgctttccctccaaaagacaaaggtagcaaaagacgaagcaggaagaactgcttcagaaactgaacatactgatttaattggctaagaagtccaaatgctaatactcctaataattagccattccttttgtgttttggtgacatatatcctcatacaatgtatatcaaatggaattttttgatttacacctgacatttcaaagtttccatttttgaattctcctagtcttaagtaagtagaacattgtctcctttgtttgctaggcataacgttttccccaacatctagggctccatgatgcaaaatatcattttgccgatcttctgttccagtatttactttaattttttttattataattggattttcaaatacaatcacaaaaacatctcctgttgaaggtggtttcccccaaaagtactcatcaacactactgtaagccttgcttgcttcataattttcaaacacattcatgttggtgtacagacttgcaggggggttatcaggaatgtcaaatgactcctcttcaaaatcatcatccttcagcttattctccgtccctttgtatgatgaataatagcccatgtgctgaaagagagatggtttaaaacggatcacatttttctgagccaacagaccacggaaatgagtcaatagccaatcacaaggcatttcttgataaaacattaataaaaaatgggccaaacgtgggagatcatgagaatgatagagtttaccaatgtagccaagcttagagaattcaagagttacccagtaagttccttctagggatgcaatgactttcttgatggcagttaagaaattttttgaacatcgaacatcatcttcaagcattacataatagtctgaagtattggcacaaaaattaagcagaaaagcataatctacattttgcttggaacgaaatttgactctatcttctggatcattgtaatttcttttaaggccatctaggattgggtaatactcctctggagcatgtataaccattaatcttcctgcaataatatggtgcgcaaatttctgtgtaatatcctggaccatggcatcacgccaggaagaattaaagtctgctaggtgaaccaccactgaaatttccttcagctcttcatagctggattgctcaaaaattgacttaattgtctcaagtaaatagtttcctttttttcgctttactgaagaaagtccaattgtaagataccgctttctttgtaaaggtgtggcagctaggtagcgataggtgacatttatggctcctgagaaattagataaatccttgaaagtatgaacatagcgttctgaattcagttgatgtgtggatgtttcccttataagttgtttgtctccttccagaacatagctatcttcaatgtacaagttcataaaaaggagaaaaatgacaagaactcccaagaatgacactgtagaacgttttctcaggcatctcattttatcaagtatttcaaaaatatgtttcatttgatgaaatttaaacattctcttctttgaagctttcgtcttcacttctggttgattgatggatgagccattggtgatttcgactcctgagccagtgctccaaatgataagtcttaagaaagacgctgtcataatctgtgctgtacagaaaccgttgatacccagagacagagaaaacaattcgttcagctagatccaacagtgctctgtgcagcctggaagcatgagtgatccttgggcctcacacaaaagcgagataattggctctcaatgaagagatgtaaacatccatcataatggcactgtgctgaaact

SEQ ID NO: 13493 - RNA, 21967 nt, Homo sapiens
  source 1..21967: mol_type = other RNA
gctgggattacaggcatgagccaccacgcctggccagtttttaaagtatttcatacagtgtaactaggcagtcagaaatacctgtatctcaaattcatttaacttttcaatgaatcaatcttcttattttctcagacatataaattatcataatactttacattgagtctctatggttgactatatgctgtgaaggaaggacataaatacatgtgaggaaacaattattgatatttttaaactaactagaaagcaccaagttatttgttaaataaacaaagttaattttatctacctgttcagtaagtgttggcaactatgaattaatctttgacaaattcacttacaactagcaattttaaagacttaaagtttaatttttattattaaaagggtatgattatttttactaaaattaataaaaagattaactgttactaaattaaagctccttcaaaaacataaatgtattctttagagagttaaaaaaagtagcaataaaatacatttttaatttagttaagcttacttaactaatgatcaaatagattaagttgtataaaattttacaaactttatatttttgcatacacttatcttcctggcatttttgaaataaaaaaaatacaagtgcatagggcagaggaggcgattcagttacttctgctatgttattaaatctctggtaaccactatacaatacaatacaatacaatacaatacaatacaatacaatacaatacaatacaatacaatacatgtagactcagcatccaaactttattttaccttcaagttctacctgataaagtggtggaataaagatggtattttccataactgtttaataataatcacatgttttatacccattgctttgaagaagaaaccttaagcaactagaaatgtcaatctaaaaggcagaaaagctggaaaaatctcatgaagactagaagatttacactcataagatcatgtaaatttatttggatatgctgaaaaaagagggggtataaaatctaaagtttggtaaatctttgctttacagggcttcaagttatagatttttcttttttccttttctcttcccctttctctctctttctcttttttatttttgccatttcttctcaggagcccctgcaatttcaaaccttggaattgaattggatttgaggaggaaaacccatattcagctttaattcaaatgaattttactactttagacaaaggtacaacactctattcaaaaaagttattgaaatcacatctttaaatctgacccagccacttgaataaataagttgtgttgtagtttctcagagcaaccgccgctcatctttcactcaccttaacaatttctcacttttttctgctttttttttttttttattttctgcttgctgaaatcgagatcaatattcattgttttcttctgggttaactcttttttatgttaactgaatcaattttggctttgtttctttatgaaattacttttagataaagtattgatattgtcatttatcaattttattatatgtcttttgcttattaaaggattaaaatccacctctaaacttatttagatcaaggtcagtttttttactcctctgtagaactgtgaagataatatcctattctccttttcttatggttttattgtgaagatctgtgcaaatagctatataaaatgcaattcggtattaaagaaaattgttgcacggactacattgattagagtctaatttttggaaagtatacttcgccttttcagtaattttatttttcggtctatggtgcccacattgtgtcaccagccagccgtatgcagacttacaaaggactacccactaagaataaaaacatgatacaacttgaagaaattttcatcaaacgtctttgtcttatccccttgttatacagacaaagatgacaagggccgaaaaggaagtgattttctcattgaataagagaatccgaactggcatcgaggatatctaattttgggatgaaaattgagagaagacagaatttcaagtctgaattatgacttcactactgtgtcgtcattggtagaataaggataacaatacttatcacacagatttgtggtctgaatcacatgagagacatagatgaaaaatgtaaaacaacaattagcatgtgacatgctctcagcaaatcaattaatccttcattctttttttctccccttactcctttgattttcagactaatttggatcatgattattggcctgtgtcccacccattattcacatatagaatgggttgcattatcctctccttggaaatatctttcaaagtgggtaatgagaaaactactttgaagactgtgctgaaggaaatgatggcatgaacaactctagataatttttgtttatttggatataacgtgaatgggcccataccataaactcctattaagctgaatcaccaaaaaaaaatttgatatgaaagtcatacattgaaaaaattcactcttaccactgatttgattgatactgagcctgtaaatatttatttatatgatgtttggcactttattttataaaactaccctttacttaaaataaatcattgtattcacataactttccagggcactatgcatttttaaacaagacagtcaacttactatttaaaaaacaaagtcagtcacctaaatgactttctgactataaatttgaaaacaatattctccttgtaatatatgtgccaccagggcaagaattacaaattgggagcaggtaagaaaattgttgttgactctcattagtattctaattctccttcagtcagatttataaagtatgacctatagcatccaactccatcattttccagtcattcttgagactgtcaactctatgggcattgtttagcagcctcgaaacactgaactttttacagtcttattggagagaaaaacacattaaatgatcaaataatcttttatgagctcagaaaaaaatgcctaacatgaacatttaagcatcttctgtttctgtgattcccatttttggagagtaaaaatttaagaaacaaagggaatgtgtctggggatggtactaataatattgagattttacaatttaggttataatcaagataattatgtatatatataaaattatatatggtatagtttcaacttctaatcttttatcatcctctaccacataattcctcctatattctctttttctgactgtggcctaatacctcaagaatattgtatatgcttgtcactatataaacttcaccctaaggaaatttccatgtcagatacaataagagcaacggaagaaaatgtatcaaaacacatctccaatttatttgaatttttctggcctaaccttgttggcatgagagttcccactttgtattataataggcaaattgatacacacttttcatttattctaaataatagattagcatagtcaggaggcttggattggcagctattaaatacaatttgaagccgtgggattttattaggattctaaggttattctgtgacgatggaacttaatgatgtaagagttaattacccattgtcaaaaatcattgcccatcaaagcagtgagactgtgtgctatgtccagttttattcatttcttttgtgtatctgaatggaacatgtggtaaacacaacagtagaatatacctacagtccccttagaaactcttaaatcttcaatttataaaagtcatcctaagacgttaaaaataacttacgaaaggatagattccaatgtcagtgggtgagatgtgctctagctagtgtgcacgaaagagaacatggagttagaataattattgtaggactgtagattgtcatctcaagatcagtgtcaaatacattcattcatgtagtattttcacatgcattctggtctaaatatcccaacatatctttcgttttgagatctgcagaacaaagtcaatgtctgaatttagagactaatttgaccattttgattcaaatgtctaaaggctaaaccagagcaatttacaacatccaatgaagtaaaattatataattaattatataattatataattatataaaattttataattaattataaaataaaatattaacaataattgaacattgtttacttttttatcctcacaacaattcaacatgatatgtatggttattactaaatgtataatacatttagtaatgtgatttgacaaatcacatttgtcaaataaggaatggctgaattaaatgattgaatgaaggagtgaaggatgtagattgtttaagtacattcaacttgtaatgaactgtaaacttcacccataacattattaatatatcagtgctatcaactacattttacataggatgaaaaaaatcattatttttattaatcccaagatattttatttcattatataaatgaaatattttatctgttataaagacctttatttttgttccactcattaaataacatggtaagactgttgtgtaattgactgaatagttaagtctaaatgggtaaatagctgtttatgttagtattgcagggtagctatttgataatgaaatatacttttcttacctacttgcaaaaaaaattacataaacaagtatttcctagagttcaaacactgatctttttaagtggcaaattgtccaaaagaatttaattaatataaacaataaattcacttaaacaactatttacatgcaaaagtaatatttttattgcccatttggaaaatagttttgctttctggtttataaggaacttttactagtttaattacttgggtgctttaaatgttttttggaggctattacaaaatcacatcctaaaattttaaaatggaaaaattataataattgaatttttaattcctcataaatattttaaaagtacacattgttccatggcttttgcctttagaataaatacaacatttttatgtagaaatatattcttgaaatgtaactagcacatagtcagtgtttcttaaccattttggggtcctgaaactttttgataatgatgaaagcacagagatgctatcaagaaaaatttacccacataggaacacacacacatacacacagacacacacagagtttgcttataagctcaggaagcttaaagatctgctaaagattatgcttgggtttgccatgaatcataaataccaagtcaaatacctttgaatttgattcttaacaaatctttgtggctgagaaaccatgagatttcattctggcatgtccccagaatgtaattatcaatgaacaatagccattgaaaaaatctgaacagatattattgaggctcaaggttgtttaatggcacagataatataattcaaatcatgaccccagggctgatgaagtcttgttgtaacgtgtaaatggggtgggtgatgggagagagaaaacaaaataattatttatgttaaatcatacataaacagtaaagccaacacaataagtaaaataagagaaagtagaatgcttgggaggtcatatgtttcaaatgtatgcatacacaaaagagtaagcaacaggatacttcaagagtaaaatgggaaaaaatcatattgggtaaatagtatcaccccaaagtgatagtcaaaagtacctatgtttgcctagttctcagattacaactatgatgataatttagataaacaagcagaaaacaaaactatagaaaaaagtcaaagtgacataaaacaattactggtgtttcaacagaaataaacccaacatcaggatttatcaaatatatgaaaaattatgaaagattataaaacaccaatgattagattatgttataaagacactatgaagagatactaaatgatattcttttcatctgtggttactgctaaaaaattctttcatagaaattcttggattttgaaattagtttaattccaaaatattttctttattttgcaaaaatgtaagacaaatgtataggatatttttctctgttgttatgcaaggatttattatcacattggccacagaacacatagaatgttagttttgtagaaaattttagagattttaataccaggatgaaataatagtatcattctatttcaggttcttaagcaacattcctaagactagaaccttatcttgaaaaattatgattttaaacttaagggaattcaggtaaaggaaattgactaggttaaggcaaatacatcatgtttactggtaaagataacattatttaaggaaggtaagatactcttatcctacatatacgccagaaaaattgcttctcctctgaaaactaccattatttttgccaaatattgtagcttagttttaagtttttctcggctgtttcctctgacagttctgtggtaaagaagaaacattataggaagcatttttttttcctacagagtctgccatatggagaagtagaatgagaggccacctaggtaatgtgatttattaaaagttctccatcccaaaatatatgtcccatctgtgggctaatgtctgaaagtcctatgattaaactcacttttatgtaagatagtgaggccccagagagccctcgagaaatgcaaataaactattactgacctcccttggattatgatgaaaaccgtggagtctttctattctctgtcaaatgtggaggtcatggatccttcttggcacctaagattaaaactcatagaatgtgctttaacttctgtaggcacatttcctttccaattagagtgaggtgttgaatatttatttatttgtttatttttattatactttaagttttagggtacatgtgcataacgtgcaggtttgttacatatgtatacatgtgccatgttggtgttctgcatcttaagagaagactatttataaaatttattgcttgtaagatttgttttttgttctcttactattatgaaaatcacgaacttgggaataaggacactctgggcccggcgcggtggctcacgcatgtaatcccagcactttgtgaggccgaggcgggaggatcacgaggtcaggagatcgagagcatcctggctaacaaggtgaaaccccgtctctactaaaaatacaaaaaattagccgggcgtggtggcgggcgcctgtactcccagctactcgggaggctgaggcaggagaatggcgtgaccccaggaggtggaacttgcagtgagcggagatagtgccactgcagtccggcctgggcaaaagagtgagactctgtctcaaaaaaaaaaaaaaaaaaaaaaaaggacactctgaacaattgaacaagactacgctgaaaggcagagaagaagtaattatgaacaaactgttcatgaagtgatcaattgaatttgaaacagaacttttcctagcttctaaatgattagaaatttcagctttggtttaacttaaaaacttagaattgtcaattctgtccaagtctctgagtcatgtacagaactcaaattattacatcatttttttacttatctgtattatttctccatttaaaagtggacaaatttttatactatatcctaataatgatacaaggtgacttgtaggactctggatagaaagagatggcccaggatacagagggcactccttaaatagctgccaaataaatgacattaaaaaatgtataaaaaggtatgttaagtaattaaaagtgtcaggcattattttcctattatgagacattttatattatggttatttactgtaattgcatccaaaataattcataaaacatttatttttgtactattaaaaatctaaacaataataaccagatggaggaaaatgataccatctgatttaattattaacttgaaggtcagtttctacaacttattctcatttatgtttatctgatttggccacagtttcttactttctcatattttgctaagcttgtggatgaagccgcatgtctcttttttttttaacctggcatataacactgtcactctatttaattattacccatcatctacctactttgaaactttggaggttttataaaaattatgagtatttaatcaaagttgtctctttatcatttgccagtgaaaatataaaacctggctgttttattctattgtgcactctaattacataaccaaaatctttttaaaaattcttagttcttttagaaataccatttgacccagccatcccattactgggtatatacccaaaggattataaatcatgcttctataaagacacatgcacacgtatgtttattgcggcactattcacaatagcaaagacttggaaccaatccaaatgtccaacaatgatagactggattaagaaaatgtggcacatatacaccatggaatactatgcagccataaaaaatgatgagttcatgtcctttgtagggacatggatgaagctggaaaccatcattctcagcaaactattgcaacgacaaaaaaaccaaacactgcatgttctcataggtgggaactgaacattgagaacacatagacacaggaaggggaacatcacacactgggcctgttgtggggtcaggggaggggggagggatagcattaggagatatacctaatgttaaatgacgagttaatgggtgcagcacaccaacatggcacaggtatacatatgtaacaaacctgcaagttgtgcacatgtaccctaaaacttaaagtataataataaaaaaattcttagttatttgaaaatagtttttttgaattcacaaacttgcaggatgaaaaaagttattagttcctgaagatataacattgatttgtctttttcttatttgatatcagctagcagtaaaattgtgaacaaatctggtaaatcttttggtgttgcaggttcataatcagttaattgagtgtattcactataaattgctttaattaagtgatgtttgcctaagaacaagtttcatttcatctcatgaaaaaaatgttactttttgtattaatcagtggaatgtttaaagaaaaaactggttatcttgaagctgtcaaataattataagaaatctctatacattacgttttaaaatacataaaacccataaattcaagcttattagttttcattttcagcaaggtttatacagagaaaataagtaatacaaattagttttccagaaaatctaattttatgcagataaaatctgaaaatcatataagtccaagatgaaactgatctcaaattattattttgaggtgtatccatttatttaaaaaagcctcattttagctagcaacactatgtagaaaaatattttaaataagacagagcattaaaataatgtattcattgatctcataaagaatagatgatcagattttttaaaagtgattttaattaaatggacatgtttctctttagccagaaatgactgagaaattttgagttggaattgatataggggaatccttggaactatgtgtgaatatgtgtgtgtgaattatctgtgtatatttacataatttacactattcacagtccttgtttttcttgactcaaatagctatctcaagtttcgtacactttttagatctctatgtaaatacattatttcatttgtggaaatatattgaggcctatatcaataacctcaaaccttttaaacacttagagcaagtcaatatgacttgttctgtttcagctatctgaaatttaaaaatttgacaaatttttaaagtacccagttcttggaaaaagaaaaacaaataaattggagatttggatcatatgggctatgactaaatgagacaaggcatacatgctgacatttgaaggatttatgaaaaaaagtccactgtggaaaactgatagtttttctccttctttcttgaatatgtttagttaattttgtggaaagaggaaggcagctcagtttacaaacagcagtgggttgaaggcaatgctgtttatattcttgaatttcaatatctacaaagatgtcatcattagattttatgtgttaaaaagtggatttatagtctctaattaataaggtgcatatgtcaagactcaggaaaacagatcacttacgtagttctccaaaaacgagagtcccagattcaataggaaggcatgcagagtgttctctataaacccagcaaaaccataaaaattgactggaacttttatttttcagtacaacaataatagtattgaaatacctaaaaagggcaggaaacaacacagaataatctacgcttgtcatcatgttttctaatctataatctttcaaactggataaatgggaagttttggaattttactgtggtacagtcttagttgctccgtggttgtcaaatctgtctgcacattaggatcacttaggaagaattttaaaagtatgctgatgcctggaaactccagaacaattatgataactctgagcatggagctcaggaatgggtgaaattcttccccagagatgttaatgaacagccagacttaaaaactagtaatttagacaagtgtgagcagaggttaataatgttgagatgaactgggcttaatatttcactaacaaggtcagagttttgatacatcacttaactcaaactttgagattcttcatcactgaagtagcaataataatagtcatttctgttttaatacttcatagacttgtaaggatgtaatgtagtgtttctaaaaggagtgaatggacaatctgcatcagtgttaactaaaatacattgaaagtgccaattcctagatctatcctagatttacagggaagaattcagtagtctgaaacacacattttcaatatattgaaaagatgattcttttgcatgatgacttgttataatcattactttcataggtaatggaagtaccgattaggagagtaccaaatacatattaaacactcagttcatgtaagctataggccaataaacacaactttggggtttactgatgttttccaacatccgaaataatagctgaaatttagaaacatagttaatcacacaaaaaatgttgcatacatactgtctaactaccagtttggtatgtttggggctggtgttatgaaagactattatatgattaatacaaagttataatttttggagtcttttagtgtacccagagcccatgagtttttattttctttttggaataacagaaattaggttgtggttcagtggaattacagaagcaagtgttttagatgttcaagtttaaaaaatgagaaaaaaatgttttacatgaagaaactaattatttaaattcatttttcaactatttaatgttattttaatatagtcatatcatccagaaaatcccatcttagacaaatgggttttcaataaattattattatagttaggaggcaatgtataatagtgataaggggcatagattttgaattacacaaacctgaaatccaatgctctctctttcatttattagttatgtgaccttggacaagttagtaaaaccctatttttcatatgctctttagcttttttaatacctcttaccttatatggttgtttaatctattaaatagacagtgaaatgcacatgaaatcttcacacagtgtctcatagttgcttggaacatatttatgtagtaagcattgttcttggctgagcttacattaagtgatctgtaaattagaagttatttgttatatttgtttcgtttccttattgccctagatgccttttctctggacctagataatttagtctcactctgtggcctttacccttcaataaatatggattattaatataatttagctacataattcctaaggaaatattaattcataaagattgttaaattgaactgaatatctttgctaagtcacaggcattgattaaattagataaaattgtcattttccattgattttgtttatataaataatattgaattatttatattcttatttagtctagtagattgacaggcagttttattaagaaatgaatcaaatggtaaattttgaatcatctggtaaaaatggacaaaatttagttttatcttgtggtctggaaatacaccctaaattattgggtcaagttagtgaaaactgttaaattgattatgaacgtaggcacattacttataaatccccttatgctaacttaaaacttgtgaatgtttagtgttatccagctataattcttctaaacatgtcttgtaatttttaagtttgcatgaaaataactccatcctgagtatactcatttcaataaattatttgtcctgagcatactgtaagaaatttagtaaagtactaattgaatttagtgattagactgtgattagactattacaaattcacagtgcttgtacaattcagatattattttgctttgaagtcaaatagaggaaccttaaataatttaaataaaaataattgtttttattaaagtttatacagcaagataataaattcactaatgtgaaatgttgatatagtatgtacaacttgtttcttaagttactaaaaatgtattttcctacctacataatgtcaatctctattgctcctaacacatgagtggctaaaattgcaaacttaatcacataaataatgagattaaagttaaaatgaaaaagtggtatgaggactattgtttgtgttaagtgaaattataccttgtaaaatttcatattatgagagcaatatgtaaatttcattgcaacaatggttattcaatttactgatgaaaatcagaagaatgttgaaaaattagtgcatttataataaatttaattattcataaaaaattaacattgatatatatattcataaggataaaagatatcaaaataattaaacaaatttcactttcttcttataaaagaaaataatttttatggtaactaattttagtagtgcatcagatcaacactattgggcacccagttatttggtggtacgctgagtgaaaatatgtagctttatctacattaccttggtttggacaactgaaaaatttgctaggaaacaaatattacaaaatatgttgttaacttttcaaagatgatcggtttagattgctttaacttgaaggacacttatattttgtatcacttttgtagcaaacacatgactcatcattgcccaaatcaattgcccaaatcaattcaaacatctcattgtagttcatcccatggcagaaaagtgtttatccacttagtaaaatggaaaacactagagcttcaggtttaatttgaaattttaacttcattaagaataaacttgacctgtttgttctagtaagtaaaaacactagatacgtaccaaaattgtcttttgaccctctcagggagtcaagttttgatttgcttgaatacaagcaagtcgagctatggtaatttgcaatgctgacaggaaagaagaacttgcttgaggcaaaatcatgaagtacaacttttcctctgcatccttttacctcatgtttgtaacatttcccctgttgttatttttacacatctggatgctcagaaaggcctccttaccacaataattgaaaggagtactttgtcaatagtcagaattgaatgagagataggttgttgggaatattcagggtgaatgtgtcttttctactttgactatatttaccattgactacagtaactcagcagaaagttagagggcagcatacatacattggtttatggatttaatgaaaatatccccaaccattacattacagacaattcatatatatgtcttgaaaatcttcttgacaatttgtgacaaattttctaaatgtttttccaaaaatagttggttcttgtaagtgattttgatatgactgattaccaaattatggtgggtaaagatgccacatgcaacagaaaatgtgtctaattatgtttgttttagagcttaagaaatgttaagaagagaagttacaactgcattaataggattttaatttttattcaaaatggacaacttatttattatgtacttctacacacagctaagcttatagatattttcatttaaagaaaaactatttgttcattttattagcagatatcaaatgcccttttgaaaattgagactgatttctaaaacaaaaaaaaagactttaggagttttaattatttttaatatattgcttctttattaaaaaaagatacaatccttcaatgtcattcaacagtattaattgttaaagtgtgggatatagtttacattaccgagtttattttctaagggtagtgaataactcctgacaactactgatatcgtcacatggtcctttagtgaccaaaaatgcacagttgtaagaatgcaagtgttacttgtattgaaaaccggattacattaaaggatggacaattatgataaaggatctgagataattggacaattatgataaaggatctgagataattattctaactttttggaactatactttcactcattgatgaagtaagttacaacgtggaataacaaagtttaagtgtggcagaaaatacatacatatgtttaaaagtagggaaaattttatcaattattaaagatggaaaaaataggactatgtcaaatagttaaacaaatgtggggtattttatggagaaaagaggcatgtactaccttaaacattttccaattggaacatactatagacaaaactgacagattattattcaatgagaaacctgactcagatgaagttacaaaaaaagtactttttaaatgtctagtttctaatagagttagagctttgttgattgagatatgtggaactgccacatatctctgtgccatacttttggtaccttcataataaacggtaaagtgagggaaagggtggaagagacaaatcctacgtctcttccagaacttcgagtgcactataaattaaatatttaaaatatttttgcaatagttagctttcaattatgaacactctcagcctctattgctttatatatgcatttattttggtaatttttatacatcaaaactataattacctgtatttgggcagaatgatttaggttatgccagctattgtggttaaagctgtagtaacttacagtacattgaaattatagactaaggttctgaatattggtaactcactgttgttgtgcacctttaaacaactcttaaataaagtaatgattctctttatattaaatttaatgtatgtgtgcctcatggaaatttgtattttatagaaaaatattgaatattttattattatgtctttggctcacctactttaaggagatggctacttagggtactttttaatccaatataatgtgaaaatttgatcatgctatattcttaatttaattgtacttctatggtcatatacaatttacctatcactttctcacataatcaatttaactttttggtaaatcttctaagagaccgtctagacagagtgaaatgaaagctgaaacaacagtcaaatcaaaaactgctttggtctcaaatccatgtttttcagaaaagatattcagatccagttatctggcaaatggtctcaaacatacatttcaatttcaatgttaaaaataggatattaaacatctcagaaaatattgggattattgaagcaaattctaccctggacttggagtaaatgtgatgaacagattaatgaggtggaagggactagaactttgggaaagtgcaaccttgttatcttaatatttttatagcttagaaagagaatgctatgcaactcatattttgatcttttaatgttaaagaattcaaataaaaaccataaacctgaaactctaaaagaaaaattctgttttgagagagatggcctcctctagtacacttttaataaatttaaagtatctaaaaggatgcacaaagatctctaatgtgctgtgattttcaaaggatgtcatgtataaaagatttgagtgagaacatgaaagcaaaagcaagttcagaagaggaacacaaccaggaggacagtgtgtcaggaaaatccaagaataagtggaggtgtaaaggctaaaaaataatgcaaatggtgcatatccttctgtctttctctcatacacacagacacacttacacaacacatatacaaatacatacatgtatatatgtatatatatacacaaatatacacacatattcacataatattcaagtatgtatacatatatacacatatgtacatacacatatgtatatatacatacacacagattgagagattaaccatatgtagatacacacatgcacatatgcaataatgaaatcatttcaaagcatgccaaaaagtaataaaagatatatcctctgtttgggataaataaaaaaaaagtttaaaagcaaacaaaaaataaatggcaataactaatcacattgaattttgttatggcctttttcttcctaaaaagaataaccccaatctgaacaaagaaattcaaagtaatggaaaactcaacaatgaaactcaaagtagactagcagataagatacctatttcaaacatcagtgccaaggtaatttataggtcagtgcattgataacttttgccaatgatagaaaagatgccagagaaccggatcctgacattaaaaaaaaaaagtaaaaagattctgaagactgcatttctgagcttaaggtagattctaaacaacatcttagaaactaggaaatgactttatgtttctttgtttttcaatgtaaatggatcaagatttcttaaaacagaaatgaatattattatttgtgatgagagcactaggggcaattttgatatttttgataaggtttctagagtaataaattagaatgacaggaatatatattgattttaggaaagtgtctgtataattccacatgatattctctggacaaaatatgaaaaggtaggctgaataacatttttaaagggcagtaaattttataattgttattgattacaatgaaggcctctggtaatgttttccagggtcatatcctgttacatatacgtgacatggataaaaaggaaacaaatatttattgtgtgcctagtttatgttatctcaattccagctctacaaggagctacaaggtaaaattgctacctttaaaaacatatgaggtaaaattattcctattcacagatgtagaaactgagtttcaagaaggttaagtaaatttcctcatattgggaggctggtaatgcagaactgggtgtcaaaatcaagtctgtatgaaccttctgttttgtctcccatgaagacaaaaggcatgcatataaaatttgttgaaacacaaagctgaggaggcataataagacgtggaatgacagaagcaagatctagaaagtttgggatcatgaatcaaaagaaacaggataaaattatcctaaaattaatattaaatcttacaagaaaccccccaaaatcagttgaatttgtacaaaacggtaaatcattttatcagtagatcccataataaatattataaagtttaagtgtgagctctattactcagtaatatgatgccattactgtgttgatggatgtattgtcaaggaaaaagaagagaattacacactgtttccttcaattgttagatggcactggatgtagtgttttcaatgttaatcctggtatcatgttctttgccataaacttgttgacaaattggcaaatactgacatgaaatatgccaatatttgagcatctaaaaatgtaggtactttccataccacatcatatattacaatttgaaaatgtttgtttcattttttatataattattatacagaacagtttttctatgatagcattataaaaattcccagagaatactggcccagtaagaaatggaatgttcacaactcatagtgtagctatatgaaagaaatagatctaaacgacaggttggtttccaaattatattttcatacctggaaaatatctactttataaatagcacaaagttatagttttcaatgaatatgaaaaagttcttgcattaacatattttatgtatcttttatattgacatttgtgattgccactaaaatgtgtattttctaaatttcattgtgcttttacaagatacttttttctttgatgtccataactgctgaaaaggctcccctaaggagaattttaagactaagtaaggtttttagtgagcttaaattatacaattctgaggcattatttaaggtgcatactgtattttttgcttgaaacctgtcagcattttatttgtatggcaattaaatgactcagccattcatgtctcatgccagtctttttcaattgttatttttaacaaagaaaattatatatatatgtatatatatattatatatatgtatatatgtattatatatgtatatatatataaacttacagcaaaaatgtttaaaaatagcaaatagtttgagtatagttaaacctaataactgtacttttgtttctatgcctctgagacaagattactagacccttattcaaagtttctaaatataggaaatagaacattgggccatgctaaaaaaattgttcagattttcttttgaaagagaatagttatttttcctcctgacctctaatgaagatgctttatttgtcaaggtgttttccttagaaaattgacccagtgtcaactgtaaagaaaacatagaggatccttggatgattgaccaacttatccaaacacaggtttagtaaagagaggatataaagataaaatgtgaaatgacctctctgagtcacatttgttttcataatttcctagcaaacatccaacttcactgctaccctcagcaatgtttcttgaaacatttttaagacattgatagacaccaatagctgatctttagaaagccattcccagaagaatatgtaaggggttacaactcatttcagggagtctgcctagctcttgatattacatgtctttggcatacaattgtgtaccttttatcattgacagtgaagaaaataatgccatttgtaacttctgagatatacacacaatactatcaactagccggttaataaaagataagaaaaataaagaaaatagaacatttttaggtgtctggcaagtatcctctaaatcaaggtaaagataataatttagtggcagtgttcatattttcctatgactgtaagatttaggtgcctcacaaaatattaatatttagcctcttatgaaaggttcgtttttcttctaacactttagtagctgaatacaaagaaaatacacaacagctgtttataaatgaaataaaaagtttccattttttatctgagtttctcatttatttgcagagaacgaataaaataaaaatatcctagtgttgtttgcaccacagcataccagtaaatcttaaggattgtgtttcagtatgaaaaggaagagcaggaagatttcctcattctgtcttaccagcaaaagtctagccttcacacacacacacacacacacacacacacacacacacacacacacacacacacagagtcatctatatgaacacgtacttgagtttcttaaacatatatgaagcaccttccatttccctttataataaatcccttagtttttgctgttcattaaaaaacaaaaaggaagagacaagctcaggacattctgaaaaccaatgtctttaggacacactaaggtgtcctgaattactttaacggacacattgtaaagacacactctccaatccctattaggaaaagtttagtcaagtttgcttactatttgggtgcttataccaaaaaagcatcatttaggacattatttaggataatattatttatgcaggaattgtaccacctatttccagatggtataacttattatctgacaggcatgtagcaaatagaacacaaagcataaatctgtcaggagaaatcatacgagaaaaagagcattgtctggttatcagaatatcagatctctcattctggccttgctaggaaatagatctttgattctagaaaagtcaactaatttctatggttcttacttttctcctttataatatacccatttaaattccaaaaaggtatatgataaatcacaataatttcaatcacatggattttaatacaaaatgtataaaatcaatttccaaaaattttctgcatatactgaaaatgtctgtacgaatgagctaactactataggccttccctaatttattctattaaatgtgggtactcaatgtaacctgaaaatattgagcttaactcttctttttttttttcaaaagggaaacttgaaaaagactgcttcccccagaaaatttatcaacaataggtgctcaattaaatgtttttaaacaatgaacaatatcccctttcatataaataatcaggggagagatatttttaagtcttttttttctttttccatagtgtcacctacacaaaaaattatgtaaagacaccacttctatgaggaggtattcattgtagatgtacagaagtcaacggaaacttaagtttacagaaaaaataaaccagattatcattccacccaactgtatattcccacagatgcttaataaaagctatctgatgatataatgaattatcagttcttgaggaagtatatacagttggtgactatttttcaaaaatcatcatccaacaaatttttttcatttaaaatctttcatattaccctttcgacaatcagttgaaattttaaaactaagaacatttaaaaatataaatgaaagtagcattagctatagactgatattcaacttcagacgttaaaataaatacaagtgtgtattaagagtaaaattatgtcaacaatgtataaatgaaaactgccaatgtaattaatgtttcttttaacatatcccatccattgctttccctccaaaagacaaaggtagcaaaagacgaagcaggaagaactgcttcagaaactgaacatactgatttaattggctaagaagtccaaatgctaatactcctaataattagccattccttttgtgttttggtgacatatatcctcatacaatgtatatcaaatggaattttttgatttacacctgacatttcaaagtttccatttttgaattctcctagtcttaagtaagtagaacattgtctcctttgtttgctaggcataacgttttccccaacatctagggctccatgatgcaaaatatcattttgccgatcttctgttccagtatttactttaattttttttattataattggattttcaaatacaatcacaaaaacatctcctgttgaaggtggtttcccccaaaagtactcatcaacactactgtaagccttgcttgcttcataattttcaaacacattcatgttggtgtacagacttgcaggggggttatcaggaatgtcaaatgactcctcttcaaaatcatcatccttcagcttattctccgtccctttgtatgatgaataatagcccatgtggctttctttgtaaaggtgtggcagctaggtagcgataggtgacatttatggctcctgagaaattagataaatccttgaaagtatgaacatagcgttctgaattcagttgatgtgtggatgtttcccttataagttgtttgtctccttccagaacatagctatcttcaatgtacaagttcataaaaaggagaaaaatgacaagaactcccaagaatgacactgtagaacgttttctcaggcatctcattttatcaagtatttcaaaaatatgtttcatttgatgaaatttaaacattctcttaagaaagacgctgtcataatctgtgctgtacagaaaccgttgatacccagagacagagaaaacaattcgttcagctagatccaacagtgctctgtgcagcctggaagcatgagtgatccttgggcctcacacaaaagcgagataattggctctcaatgaagagatgtaaacatccatcataatggcactgtgctgaaact

SEQ ID NO: 13494 - RNA, 2411 nt, Homo sapiens
  source 1..2411: mol_type = other RNA
gctgggattacaggcatgagccaccacgcctggccagtttttttggttgttgttgttttttttttttttgagtgcagtggcaatcagggcagcctcgacttctccagactcaggcaatcctcccacctcagcctcctgagcagctgaactacagggcatgccgccatgcccagctaatcttttgcagagacgcggtttcaccattttacccaggctggtctggaactcctgtactcaagcgatctgcccacctcagcctcccaagtgctgggattacaggctgagccaacctcctgggcctttctcttttgttcagccgtatctgttctcaacgggacaccatgctgtgctcatctctgtggacgaaaaaaatgttaaaaaagactaagaaaaaggcaaaccaaggattgactaagcaaaatttgtacttgtttaataagaaaatcacttctttaaaaaaatagttctttacatgctgaggttcatctatgcaatgcaagagctgaaaacagattcgagaaaggctgttcctacaagggaaggtcctgaggttacaacgccggcatggccgggaaaacatggctgcagcgatcccagcttcttgctgcccacaggggtggcacatctgggcacacactgtgagctgctcagaggcactctggtgggcagctcccatcgcctcagtcagtgtctccgtccccttcactgccttccaggggactgggcaccttggcgcccgtgccacctgccgtgagagcggtggcactgaagttgtggatgggcaaggtgctcagccactgggccatggagcgttcgtcccgctcggtgccgatgatggtggggtagatgtgctcctccttgaaggctgcgacctttccttcctcctgcgcccagtccagcggctcatgcagcccatcgttgccaaagcgctggttgtacttctcgaagtgcaccctctccaggaccaggccgagtccgggcgccttgggcacgtccaccttctctgtgccccagctgcgctccagcacgctctcaggggcataacccttcacaatggccaccaccaggccgaccatcttccggatctgatgcatcatgaagctctggcccttcaccctgatcaccgcaaactccaggccctcccgcacaaagggttcctcgcagtacatctccaggatgtagcggcaggcactgggatcctgcggccccttctgcgaggtgaaattgtggaagttgtgcgtgcccttgtagcaggccaggagcctgttgacctgctgcagcgtctcggcgctcaggcggtaggtctcatcctgaacgtcccggtccttgtgcgcaaaggcaaacgtgggcagcaggtagcaataggtcctggcatcacatctgttcttggagttaaacccgcccgtgacccgcttcagtcccagaatccgaatgtgagagggaaggtggctgttgatcttttctagaatgtcgtcaatcagccacaccttcagggataccacctggccggctgcggacacacccttgtctgtccgggcgcagcgctggaaggacattttcctcatgtcctcaccatgattttcaggaatacagcctgaccggacgagggcggacaccaagtcatcttcaattgttttgaattgtgaggacccgacattcctctgcatgccgtggtagcccttgcccgaataggccatgagcagcacgatcttccgcttgggcggcttctcgcgccgctcctcgtcgccaccgctcttgagcttcttcgccggatgttctccgtcctcccagacgcggtcgcccccggcccggccgctgcaggacctccggtcctgggggcatgcggctccggcgggcggcggctccgcgttcccggccatgcgcggcgagcaggacggacgcggtcccaggcgcagggtccaccgtccgaaggctcccaacagcgcgcgaagctggaggcccatgcgcaggctaccagtgcacccgaccccgccctgatccccgacccctgacccccagtgccccagctccgcctctgccgacccctaacctctcggaccctgacgctgcagccctgttccttctgacccctgacctccgggaaaccggcgccccagcccctctccagctgacccctgacctctcggacctggacgccccagcctcactcctgctgacccctgacctctcaggccccgcgcccaagccccgtctctactgcccccagaccgccccgggaccctgacggatcaactccaacgtcccctgacgcccaggttaacctctgacttccccagcctcttcacctcccgccccgcccggtgggctttcctcaggagtcgaggagacccgggccacccgcgtcgggaccagagaggctcgctcctgccccattcgcgacgcggctgact

SEQ ID NO: 13495 - RNA, 1995 nt, Homo sapiens
  source 1..1995: mol_type = other RNA
gctgggattacaggcatgagccaccacgcctggccagtttttttggttgttgttgttttttttttttttgagtgcagtggcaatcagggcagcctcgacttctccagactcaggcaatcctcccacctcagcctcctgagcagctgaactacagggcatgccgccatgcccagctaatcttttgcagagacgcggtttcaccattttacccaggctggtctggaactcctgtactcaagcgatctgcccacctcagcctcccaagtgctgggattacaggctgagccaacctcctgggcctttctcttttgttcagccgtatctgttctcaacgggacaccatgctgtgctcatctctgtggacgaaaaaaatgttaaaaaagactaagaaaaaggcaaaccaaggattgactaagcaaaatttgtacttgtttaataagaaaatcacttctttaaaaaaatagttctttacatgctgaggttcatctatgcaatgcaagagctgaaaacagattcgagaaaggctgttcctacaagggaaggtcctgaggttacaacgccggcatggccgggaaaacatggctgcagcgatcccagcttcttgctgcccacaggggtggcacatctgggcacacactgtgagctgctcagaggcactctggtgggcagctcccatcgcctcagtcagtgtctccgtccccttcactgccttccaggggactgggcaccttggcgcccgtgccacctgccgtgagagcggtggcactgaagttgtggatgggcaaggtgctcagccactgggccatggagcgttcgtcccgctcggtgccgatgatggtggggtagatgtgctcctccttgaaggctgcgacctttccttcctcctgcgcccagtccagcggctcatgcagcccatcgttgccaaagcgctggttgtacttctcgaagtgcaccctctccaggaccaggccgagtccgggcgccttgggcacgtccaccttctctgtgccccagctgcgctccagcacgctctcaggggcataacccttcacaatggccaccaccaggccgaccatcttccggatctgatgcatcatgaagctctggcccttcaccctgatcaccgcaaactccaggccctcccgcacaaagggttcctcgcagtacatctccaggatgtagcggcaggcactgggatcctgcggccccttctgcgaggtgaaattgtggaagttgtgcgtgcccttgtagcaggccaggagcctgttgacctgctgcagcgtctcggcgctcaggcggtaggtctcatcctgaacgtcccggtccttgtgcgcaaaggcaaacgtgggcagcaggtagcaataggtcctggcatcacatctgttcttggagttaaacccgcccgtgacccgcttcagtcccagaatccgaatgtgagagggaaggtggctgttgatcttttctagaatgtcgtcaatcagccacaccttcagggataccacctggccggctgcggacacacccttgtctgtccgggcgcagcgctggaaggacattttcctcatgtcctcaccatgattttcaggaatacagcctgaccggacgagggcggacaccaagtcatcttcaattgttttgaattgtgaggacccgacattcctctgcatgccgtggtagcccttgcccgaataggccatgagcagcacgatcttccgcttgggcggcttctcgcgccgctcctcgtcgccaccgctcttgagcttcttcgccggatgttctccgtcctcccagacgcggtcgcccccggcccggccgctgcaggacctccggtcctgggggcatgcggctccggcgggcggcggctccgcgttcccggccatgcgcggcgagctcccgccccgcccggtgggctttcctcaggagtcgaggagacccgggccacccgcgtcgggaccagagaggctcgctcctgccccattcgcgacgcggctgact

SEQ ID NO: 13496 - RNA, 2019 nt, Homo sapiens
  source 1..2019: mol_type = other RNA
gctgggattacaggcatgagccaccacgcctggccagtttttttggttgttgttgttttttttttttttgagtgcagtggcaatcagggcagcctcgacttctccagactcaggcaatcctcccacctcagcctcctgagcagctgaactacagggcatgccgccatgcccagctaatcttttgcagagacgcggtttcaccattttacccaggctggtctggaactcctgtactcaagcgatctgcccacctcagcctcccaagtgctgggattacaggctgagccaacctcctgggcctttctcttttgttcagccgtatctgttctcaacgggacaccatgctgtgctcatctctgtggacgaaaaaaatgttaaaaaagactaagaaaaaggcaaaccaaggattgactaagcaaaatttgtacttgtttaataagaaaatcacttctttaaaaaaatagttctttacatgctgaggttcatctatgcaatgcaagagctgaaaacagattcgagaaaggctgttcctacaagggaaggtcctgaggttacaacgccggcatggccgggaaaacatggctgcagcgatcccagcttcttgctgcccacaggggtggcacatctgggcacacactgtgagctgctcagaggcactctggtgggcagctcccatcgcctcagtcagtgtctccgtccccttcactgccttccaggggactgggcaccttggcgcccgtgccacctgccgtgagagcggtggcactgaagttgtggatgggcaaggtgctcagccactgggccatggagcgttcgtcccgctcggtgccgatgatggtggggtagatgtgctcctccttgaaggctgcgacctttccttcctcctgcgcccagtccagcggctcatgcagcccatcgttgccaaagcgctggttgtacttctcgaagtgcaccctctccaggaccaggccgagtccgggcgccttgggcacgtccaccttctctgtgccccagctgcgctccagcacgctctcaggggcataacccttcacaatggccaccaccaggccgaccatcttccggatctgatgcatcatgaagctctggcccttcaccctgatcaccgcaaactccaggccctcccgcacaaagggttcctcgcagtacatctccaggatgtagcggcaggcactgggatcctgcggccccttctgcgaggtgaaattgtggaagttgtgcgtgcccttgtagcaggccaggagcctgttgacctgctgcagcgtctcggcgctcaggcggtaggtctcatcctgaacgtcccggtccttgtgcgcaaaggcaaacgtgggcagcaggtagcaataggtcctggcatcacatctgttcttggagttaaacccgcccgtgacccgcttcagtcccagaatccgaatgtgagagggaaggtggctgttgatcttttctagaatgtcgtcaatcagccacaccttcagggataccacctggccggctgcggacacacccttgtctgtccgggcgcagcgctggaaggacattttcctcatgtcctcaccatgattttcaggaatacagcctgaccggacgagggcggacaccaagtcatcttcaattgttttgaattgtgaggacccgacattcctctgcatgccgtggtagcccttgcccgaataggccatgagcagcacgatcttccgcttgggcggcttctcgcgccgctcctcgtcgccaccgctcttgagcttcttcgccggatgttctccgtcctcccagacgcggtcgcccccggcccggccgctgcaggacctccggtcctgggggcatgcggctccggcgggcggcggctccgcgttcccggccatgcgcggcgagctctgacttccccagcctcttcacctcccgccccgcccggtgggctttcctcaggagtcgaggagacccgggccacccgcgtcgggaccagagaggctcgctcctgccccattcgcgacgcggctgact

SEQ ID NO: 13497 - RNA, 5268 nt, Homo sapiens
  source 1..5268: mol_type = other RNA
gctgggattacaggcatgagccaccacgcctggcccaaacttgattttctactttaaaaaactttattatggaaaatttaaaatatatgtaaagatagtaagaacggcacaatgaaccctgtgtacctaatgatccagattaaacatttaccaacattttgctaatcttgtttcatctatccctcccaccttttgtttttaagtatttaaaagtaaatcacaggcataacatttcagccttaaatacctcagtatgaatctctaacacttaaggactcatacacatatacccataatgccatagtcatgcctaacatatgaacaataaattatttcgtatcatttagtaaccaatccatgtttacatttgtacaatatgtagagacattttattccttcaaatcttgtattgactatgttttctttattttctgtattcctgatgctctggccacttggggccttgatcctggataggctgcccctcccagggcaagctaatgcatagatgataaactccactgcaagcatgcctttcatatacaaaccaaccaatccagagcccatactcccaactatctcctttaccaaactctcatacaccaattcaatattcccctgccctaactagacaattacgaatcccccctagatcccagagaccaacaaaattactcaaactattcaatcctaagcttaccagtgtgcctacccctgccttgtccattccttcccatgaaaacccccaataaaagctctgggccatgctgtgctctcaccctctgcctcctgatacacccaggtgcttctttacgtgaccctgcatgccatgccatgcctcccgtttgtgggatctgcgtataaacttcttccttcatgacaataatttccatgtctgcctgtctcaccatgattgattaaaacaaatcccaagcgcattttaacacaaggatcctaaaatgctccatacactgtatttgaaggatacgtttcttagtctcctttaaagtgtaggattccatttttgtcttttttttttttttttttgacatgtattggttaaaaaactaggccattacttctgcagaatttcccaaattgtgcatttggttgtttgcttctttgtgttgttaatttgttcttttattccccatgtttcctgtaaactggtaattaggtttggagactaacttgtacttctcagttttgggggagccaagaaaacttcacaggtgtccactgtgtgtatccatttcatcacatcaagttcatctggctgatctcatttagagatgttaatatagattagtgtcctgtcattctgctccatgcattataagcttcctatccatttttcacctaatggtcttcgcatccattgctatcaccacgaaaatccatgattttgtaaaattaaagagcgtagttttcaaattctatcattcatttgatctttgttttgttttgttttttgttttttgtttgagacagagtctcggtctgtcacccaggctggagtgcagtggcgcgatctcggctcactgcaagctccgcctcccgggttcaagccattctcctgcctcagcctcctgagtagctgggactacaggcgcctgccaccacgcccggcgaattttttgtatttttagtagagatggggtttcaccgtgttagccaggatggtcttgatctcctgacctcacgatccacctgcctcggcctcccaaagtgctgggattacaggcttgagccaccgcgcctggcctcctttgaccttttaaccagttggaattctctaatcaacaactttccttcaccaacttttggttgtcttgaaatatagtttgtaaaggataggcaaggtaaatattccattcttttcctttatttgttaataatgctctagtatgctccataactaatcaatgcatttggttcaggaaaaaaaaaagctcaaaggttggagtggtcatgataaaaggacacaggagccaatttgaggggattgcctcaaaatgctaaattgacaatttagcatttttaaaaaacaatgaagtagtttaaaaaattaatggggcttcataatacaggtgacttttaatttccaaagtttcatgttatcctttgtcaatttttaatattgactggggccagagaatactgattgtagtttttttttttttttgagacagggtcttgcagtcactcaagctggagtgcagtggtacaatcacagctcactgaagcctcaactcttgggttcaaatgatcctcccacctcagcctcgagtagctaggactacaggcatgcaccattatgcccagctaatttttaaagttttttggtagagacagggtctcaccatgttgcccaggctggtctcgaacttctggcctcaagcaatcgtccttacttggcctcccaaagtgctggatttacaggcatgggccacctcacctggtctagggtatctgttttttaatgaacaaactggaaaggaattccttactttcaatattttaacgagaataagatatctcaagttcaatgaagattaaatgttggtggaaggcatttctatactcattatgcccacagcctttagtatgaattatgtaaaaataaatatttagtatgataataaaagaaagtttagtggcttaaaacaacaaccattttattatatctcatgtttttgtgggtcagaaatttgggccaggggctcagctggtcaattcttccattctacatggcatcagttcaggttaccaagtcgctcactggcatttagctggtggctggtctggtggatccaaaatttcactcaaatgtctggtatcttggtggatgtcaagaagacagggttcagcaggtgcctctccctctctacgtagtttcagggcctcttcatgtggtctcttcagcaaagtagccagactttgtaacaagacagttctgtcatttcatgagatgaagtaaccctaccagtaaagtctgagtcaagaaaccagcacagcagtacgtctaccatattctactgggcgaagcagtcacagagggatgtagattcctgtatacaacagagggatgtagattccacctcttgattgaaagtgtgtcaaactgctgcactcttatatgaccatgtcataaattaaaaaattatagcacagagcagttaagcgtcttgtccagtatgacacaaagtgatgggatagggatgacggtaaatgtctttttcattcttataacaggattagtttttagaacaaatatgctgaagtttcaggtttgagtgatgatggactacaatacattgtcacactcttttaatggtataaaacctctaatgccaacgcagttgcatgtatggagcaaaatagattaattactacattcatagaatgttctataacacagaagttgaaaagactttcttagatttttacattatgaattttcagatgatgagtaaggtgtgaatgttgcctaaaggccttcttacattccttacattcatagggtttctcaccagaatgaattctcagatgttgaataagggatgaattaagtctaaaggccttcctacattccttacactcaaagggtttttcgccagtatgaatgctctgatgtagagtaagtttttggcgcaatctaaaggccttgccacattccttacatttataaggtttctcaccaatatgaatactctgatgctgtgtgagttgtgaaagtagtctgaaggccttcccgcattccttacagtcatagggcttaacaccaatatgaatactctgatgtgaaataagttgtgagtagcgactaaaggctttccagcattccttacattcgtaaggtttttcaccagtatgaattctgtgatggagaataagatgataaccacggctaaaggtctttccacattccttacattcatagggtttctcaccagtatgaattctctgatggagtgttagttgttgtcgcactctaaaggccttcccgcattccttacattcatagggtttctcaccagtatgaagtttgtgatgtactctaagaccagagccacacaaaaaggccttcccacattctttgcattcatagagcctgtcagcactattaagcttctgatgccgagtcaggtgtgcgtactgtctaaaggcttttccacactctttacacacatagggtttctcaccagtatgaatcctctgatgcagagtaagttgtcctcgtaccctaaaagccttcccacattctttacattcatagggcttctcaccaatatgcattttctgatgtactctaagatctgcaccacatatgaaagcttccccacattccttacattcatagagtttttcaccagaatgaagtctctgatgtcgagtaaggtgtgcagtctgtctgaaggccatcccacattccttacattcatacggtttttcaccagtatgaattctgtgatgaaaagtaagctgttggcgcactctgaacgccttcccacattccttacattcatagggtttatcaacaaaatgaagtctctgatgtggagtaacagatgtgcgtttctggtaagaggacaccttttcagatggcattttcacactactgaagtatccttcttgaggtctctcctgtccttcaatttttcctgtggattcccaatcattttttaaaatgagacccttaaggccatggttttcaattctttccattatcttccactgggataaatttatttcataaatgtcattttctaaagataacttcttggtctcatacttggtctccaaatctggatattgtcttcttcctttcctcacaactttccaaggctcttttccttgctccaatgaggaaatcacatctggtttagaaatgaagcatcccagtgagaccaagttgctgtagttctccaacatgacatctctgtacaagtccttttgttccaagtccaggtattcccactcttctggagagaagtctatggatacatcactgaacatcactgatcgaagggccatggtatagaaattcaagaactggtcagtcctccttggggtttacttgccaggagaagcaccgagtccacagaggctgatctctctttaccccctgggccgcagcgcttttcctacagattaccaggaccgacgctccgggccaggactgctcactcggggcgcgaacccgaggcacagcgatgcccgaacggaggaagccgctgccgggtcacgccacaatccccggggcct

SEQ ID NO: 13498 - RNA, 5271 nt, Homo sapiens
  source 1..5271: mol_type = other RNA
gctgggattacaggcatgagccaccacgcctggcccaaacttgattttctactttaaaaaactttattatggaaaatttaaaatatatgtaaagatagtaagaacggcacaatgaaccctgtgtacctaatgatccagattaaacatttaccaacattttgctaatcttgtttcatctatccctcccaccttttgtttttaagtatttaaaagtaaatcacaggcataacatttcagccttaaatacctcagtatgaatctctaacacttaaggactcatacacatatacccataatgccatagtcatgcctaacatatgaacaataaattatttcgtatcatttagtaaccaatccatgtttacatttgtacaatatgtagagacattttattccttcaaatcttgtattgactatgttttctttattttctgtattcctgatgctctggccacttggggccttgatcctggataggctgcccctcccagggcaagctaatgcatagatgataaactccactgcaagcatgcctttcatatacaaaccaaccaatccagagcccatactcccaactatctcctttaccaaactctcatacaccaattcaatattcccctgccctaactagacaattacgaatcccccctagatcccagagaccaacaaaattactcaaactattcaatcctaagcttaccagtgtgcctacccctgccttgtccattccttcccatgaaaacccccaataaaagctctgggccatgctgtgctctcaccctctgcctcctgatacacccaggtgcttctttacgtgaccctgcatgccatgccatgcctcccgtttgtgggatctgcgtataaacttcttccttcatgacaataatttccatgtctgcctgtctcaccatgattgattaaaacaaatcccaagcgcattttaacacaaggatcctaaaatgctccatacactgtatttgaaggatacgtttcttagtctcctttaaagtgtaggattccatttttgtcttttttttttttttttttgacatgtattggttaaaaaactaggccattacttctgcagaatttcccaaattgtgcatttggttgtttgcttctttgtgttgttaatttgttcttttattccccatgtttcctgtaaactggtaattaggtttggagactaacttgtacttctcagttttgggggagccaagaaaacttcacaggtgtccactgtgtgtatccatttcatcacatcaagttcatctggctgatctcatttagagatgttaatatagattagtgtcctgtcattctgctccatgcattataagcttcctatccatttttcacctaatggtcttcgcatccattgctatcaccacgaaaatccatgattttgtaaaattaaagagcgtagttttcaaattctatcattcatttgatctttgttttgttttgttttttgttttttgtttgagacagagtctcggtctgtcacccaggctggagtgcagtggcgcgatctcggctcactgcaagctccgcctcccgggttcaagccattctcctgcctcagcctcctgagtagctgggactacaggcgcctgccaccacgcccggcgaattttttgtatttttagtagagatggggtttcaccgtgttagccaggatggtcttgatctcctgacctcacgatccacctgcctcggcctcccaaagtgctgggattacaggcttgagccaccgcgcctggcctcctttgaccttttaaccagttggaattctctaatcaacaactttccttcaccaacttttggttgtcttgaaatatagtttgtaaaggataggcaaggtaaatattccattcttttcctttatttgttaataatgctctagtatgctccataactaatcaatgcatttggttcaggaaaaaaaaaagctcaaaggttggagtggtcatgataaaaggacacaggagccaatttgaggggattgcctcaaaatgctaaattgacaatttagcatttttaaaaaacaatgaagtagtttaaaaaattaatggggcttcataatacaggtgacttttaatttccaaagtttcatgttatcctttgtcaatttttaatattgactggggccagagaatactgattgtagtttttttttttttttgagacagggtcttgcagtcactcaagctggagtgcagtggtacaatcacagctcactgaagcctcaactcttgggttcaaatgatcctcccacctcagcctcgagtagctaggactacaggcatgcaccattatgcccagctaatttttaaagttttttggtagagacagggtctcaccatgttgcccaggctggtctcgaacttctggcctcaagcaatcgtccttacttggcctcccaaagtgctggatttacaggcatgggccacctcacctggtctagggtatctgttttttaatgaacaaactggaaaggaattccttactttcaatattttaacgagaataagatatctcaagttcaatgaagattaaatgttggtggaaggcatttctatactcattatgcccacagcctttagtatgaattatgtaaaaataaatatttagtatgataataaaagaaagtttagtggcttaaaacaacaaccattttattatatctcatgtttttgtgggtcagaaatttgggccaggggctcagctggtcaattcttccattctacatggcatcagttcaggttaccaagtcgctcactggcatttagctggtggctggtctggtggatccaaaatttcactcaaatgtctggtatcttggtggatgtcaagaagacagggttcagcaggtgcctctccctctctacgtagtttcagggcctcttcatgtggtctcttcagcaaagtagccagactttgtaacaagacagttctgtcatttcatgagatgaagtaaccctaccagtaaagtctgagtcaagaaaccagcacagcagtacgtctaccatattctactgggcgaagcagtcacagagggatgtagattcctgtatacaacagagggatgtagattccacctcttgattgaaagtgtgtcaaactgctgcactcttatatgaccatgtcataaattaaaaaattatagcacagagcagttaagcgtcttgtccagtatgacacaaagtgatgggatagggatgacggtaaatgtctttttcattcttataacaggattagtttttagaacaaatatgctgaagtttcaggtttgagtgatgatggactacaatacattgtcacactcttttaatggtataaaacctctaatgccaacgcagttgcatgtatggagcaaaatagattaattactacattcatagaatgttctataacacagaagttgaaaagactttcttagatttttacattatgaattttcagatgatgagtaaggtgtgaatgttgcctaaaggccttcttacattccttacattcatagggtttctcaccagaatgaattctcagatgttgaataagggatgaattaagtctaaaggccttcctacattccttacactcaaagggtttttcgccagtatgaatgctctgatgtagagtaagtttttggcgcaatctaaaggccttgccacattccttacatttataaggtttctcaccaatatgaatactctgatgctgtgtgagttgtgaaagtagtctgaaggccttcccgcattccttacagtcatagggcttaacaccaatatgaatactctgatgtgaaataagttgtgagtagcgactaaaggctttccagcattccttacattcgtaaggtttttcaccagtatgaattctgtgatggagaataagatgataaccacggctaaaggtctttccacattccttacattcatagggtttctcaccagtatgaattctctgatggagtgttagttgttgtcgcactctaaaggccttcccgcattccttacattcatagggtttctcaccagtatgaagtttgtgatgtactctaagaccagagccacacaaaaaggccttcccacattctttgcattcatagagcctgtcagcactattaagcttctgatgccgagtcaggtgtgcgtactgtctaaaggcttttccacactctttacacacatagggtttctcaccagtatgaatcctctgatgcagagtaagttgtcctcgtaccctaaaagccttcccacattctttacattcatagggcttctcaccaatatgcattttctgatgtactctaagatctgcaccacatatgaaagcttccccacattccttacattcatagagtttttcaccagaatgaagtctctgatgtcgagtaaggtgtgcagtctgtctgaaggccatcccacattccttacattcatacggtttttcaccagtatgaattctgtgatgaaaagtaagctgttggcgcactctgaacgccttcccacattccttacattcatagggtttatcaacaaaatgaagtctctgatgtggagtaacagatgtgcgtttctggtaagaggacaccttttcagatggcattttcacactactgaagtatccttcttgaggtctctcctgtccttcaatttttcctgtggattcccaatcattttttaaaatgagacccttaaggccatggttttcaattctttccattatcttccactgggataaatttatttcataaatgtcattttctaaagataacttcttggtctcatacttggtctccaaatctggatattgtcttcttcctttcctcacaactttccaaggctcttttccttgctccaatgaggaaatcacatctggtttagaaatgaagcatcctgccagtgagaccaagttgctgtagttctccaacatgacatctctgtacaagtccttttgttccaagtccaggtattcccactcttctggagagaagtctatggatacatcactgaacatcactgatcgaagggccatggtatagaaattcaagaactggtcagtcctccttggggtttacttgccaggagaagcaccgagtccacagaggctgatctctctttaccccctgggccgcagcgcttttcctacagattaccaggaccgacgctccgggccaggactgctcactcggggcgcgaacccgaggcacagcgatgcccgaacggaggaagccgctgccgggtcacgccacaatccccggggcct

SEQ ID NO: 13499 - RNA, 2803 nt, Homo sapiens
  source 1..2803: mol_type = other RNA
gctgggattacaggcatgagccaccacgcctggcccaaatcctatttttcaatatttatttcctaattatgtcctactaggttaggttttattttcatttgttacatatttattgggttatttcctttatgctaggaactttattagtataaggatacagataaggtccattctctgttctcaagaatctgagtctacaggcagaagacaaaatgcagtacagaattatggaaatgtgaatggaaactgcattcagagaggggtattgcttgggaaaagccacattggcgtgccacagatgtatgccagcctggcaggcccatagtgtgattacttgagtttcaatatctgattcttttataggcttgaaattggtttatcaggtctggaagtgactggactctggagtactgagttacccaccacaaactgctaataaaatgctgtgtaaaagccattaatactaatgtattatttatgagaaacacaattatggggaagctaggatagttgagtttgctggtcattatcttccttgtattgaccaaattacaatgaaggctaaatccaaattataatcagaagattgcttggtaaatacagaacagaaacaatagaaatgtgtgtggtgcttttaatggctagtatttcaagcctgatgcagccctttccacttgagtcacattgtcttacattctttgacttggctagtgctaaaaatacattgccattttactttctccattttttttttttttttttttttgagacgacgtctggattgcaattggtgtgaggttggctcactacaacctctgcctcccgggttcaagcgattctcctgccccagcctcctgagtagctgggactacaggtgcacgccaccacgcccagctaatttttgtatttttagtagagacggggtttcaccatgttggccaggatggtctccatctcttgacctcgtgatccacctgcctcggcctcccaaagtgctgggattacaggcgtgagccaccacgcccagcccatcctttctcctcttaaattttctttgctgaccagtatctcttgatgtggaacgttctttcattagtggtaatactgtcaatcaggtctttggaagatattttgggttttgtttgctgaaccattatgcttattttacaaattaacttttctgaactttattgtggtagaatttacataacaatttaccattttgaccatttttaagttcaaaggaactaagtacattcacattgctatgcaactatgactaccatctagctccagaaccttttcatcttctcaaactgaaattctgtacccattaaacaataagctcccagccgggcacagtggctcgcgcctgtaatcccagcactttgggaggctgaggtgggcggattacctggagtcaggagttcgagaccagcctggccaacatgatggccatctctactaagaatacaaaaattagctggttgtggtgatgaatgcctgtaatcccagctacgtgggaggctgaggcatgagaatcacttgaacctgggaggcagacgttgcagtgagctgggattgcaccactgcactccagcctaggcaacagaaggagactcccgtctcaaaaaaaaaaaaacaaaacaaaaacaagaaccaataagctcccattccttctgccttccagcccttggcaaccaccattccactttaaatttgattattctaggagttcataaaagtggggtaacacagtatttgtcattttgtgactgacttatttcacctatcataaagtcttcaagattcatccaagatgtaatatatatcagaagtttcctcctttttaaggctgagtaatattccattgtgtgtatatgtcacatttcttttaaccattcatcccttgatggacacttggattgcttccaccttctggctattgtgaatgctgctgctgtgaacatagatgtacaaattatctgtccaagttcctgcttttacttcttttgggtatatacccggaagtggaattgctggatataattttaatttttgaggaatctccatactcagatgatcttatttccttatttttcaagtgtgtgggtctatgtgtggttttggcagggaagcgagtctctgttattcccacatactccccatgactgttaagtgctgtgttagaagcatatggtttgatgagaattctaggagagacaaatgtttcaaaggatctctgtattttcaccggcaataactaataaatcatctggcttcgctgttccccaccatgtagttgtggcattttgggaattagtacactcaggagagaagctgtgtttaggatgaagtgagttggatcatacttcgtatagaaacttgccagaaaatatagaattattggagaaattgtgaaaaacttccgtgaagatgtaaactgtactccatagtccagttgttcccaatgagttaggagccttgctttaccctggtcaggagtttcgaaaggtgttcctttcactgcatgcaaaaatacgtacatccccagattatgtataatatttgttaaagtccaagcaacaggaacactgaagaagggaatgctgagtaagacaatatgaagcaagccaactcccaatgcatatgtcagccacataccccggctgttcatgacacgggtatttggattcacttcactgtgggcaactccaacgttcatgtttgctccgccgccccactccgggccgccggctcgcagcaggaccagcccggctgctacggccgcggatacacgccc

SEQ ID NO: 13500 - RNA, 2697 nt, Homo sapiens
  source 1..2697: mol_type = other RNA
gctgggattacaggcatgagccaccacgcctggcccaaatcctatttttcaatatttatttcctaattatgtcctactaggttaggttttattttcatttgttacatatttattgggttatttcctttatgctaggaactttattagtataaggatacagataaggtccattctctgttctcaagaatctgagtctacaggcagaagacaaaatgcagtacagaattatggaaatgtgaatggaaactgcattcagagaggggtattgcttgggaaaagccacattggcgtgccacagatgtatgccagcctggcaggcccatagtgtgattacttgagtttcaatatctgattcttttataggcttgaaattggtttatcaggtctggaagtgactggactctggagtactgagttacccaccacaaactgctaataaaatgctgtgtaaaagccattaatactaatgtattatttatgagaaacacaattatggggaagctaggatagttgagtttgctggtcattatcttccttgtattgaccaaattacaatgaaggctaaatccaaattataatcagaagattgcttggtaaatacagaacagaaacaatagaaatgtgtgtggtgcttttaatggctagtatttcaagcctgatgcagccctttccacttgagtcacattgtcttacattctttgacttggctagtgctaaaaatacattgccattttactttctccattttttttttttttttttttttgagacgacgtctggattgcaattggtgtgaggttggctcactacaacctctgcctcccgggttcaagcgattctcctgccccagcctcctgagtagctgggactacaggtgcacgccaccacgcccagctaatttttgtatttttagtagagacggggtttcaccatgttggccaggatggtctccatctcttgacctcgtgatccacctgcctcggcctcccaaagtgctgggattacaggcgtgagccaccacgcccagcccatcctttctcctcttaaattttctttgctgaccagtatctcttgatgtggaacgttctttcattagtggtaatactgtcaatcaggtctttggaagatattttgggttttgtttgctgaaccattatgcttattttacaaattaacttttctgaactttattgtggtagaatttacataacaatttaccattttgaccatttttaagttcaaaggaactaagtacattcacattgctatgcaactatgactaccatctagctccagaaccttttcatcttctcaaactgaaattctgtacccattaaacaataagctcccagccgggcacagtggctcgcgcctgtaatcccagcactttgggaggctgaggtgggcggattacctggagtcaggagttcgagaccagcctggccaacatgatggccatctctactaagaatacaaaaattagctggttgtggtgatgaatgcctgtaatcccagctacgtgggaggctgaggcatgagaatcacttgaacctgggaggcagacgttgcagtgagctgggattgcaccactgcactccagcctaggcaacagaaggagactcccgtctcaaaaaaaaaaaaacaaaacaaaaacaagaaccaataagctcccattccttctgccttccagcccttggcaaccaccattccactttaaatttgattattctaggagttcataaaagtggggtaacacagtatttgtcattttgtgactgacttatttcacctatcataaagtcttcaagattcatccaagatgtaatatatatcagaagtttcctcctttttaaggctgagtaatattccattgtgtgtatatgtcacatttcttttaaccattcatcccttgatggacacttggattgcttccaccttctggctattgtgaatgctgctgctgtgaacatagatgtacaaattatctgtccaagttcctgcttttacttcttttgggtatatacccggaagtggaattgctggatataattttaatttttgaggaatctccatactcagatgatcttatttccttatttttcaagtgtgtgggtctatgtgtggttttggcagggaagcgagtctctgttattcccacatactccccatgactgttaagtgctgtgttagaagcatatggtttgatgagaattctaggagagacaaatgtttcaaaggatctctgtattttcaccggcaataactaataaatcatctggcttcgctgttccccagaattattggagaaattgtgaaaaacttccgtgaagatgtaaactgtactccatagtccagttgttcccaatgagttaggagccttgctttaccctggtcaggagtttcgaaaggtgttcctttcactgcatgcaaaaatacgtacatccccagattatgtataatatttgttaaagtccaagcaacaggaacactgaagaagggaatgctgagtaagacaatatgaagcaagccaactcccaatgcatatgtcagccacataccccggctgttcatgacacgggtatttggattcacttcactgtgggcaactccaacgttcatgtttgctccgccgccccactccgggccgccggctcgcagcaggaccagcccggctgctacggccgcggatacacgccc

SEQ ID NO: 13501 - RNA, 2741 nt, Homo sapiens
  source 1..2741: mol_type = other RNA
gctgggattacaggcatgagccaccacgcctggcccaaatcctatttttcaatatttatttcctaattatgtcctactaggttaggttttattttcatttgttacatatttattgggttatttcctttatgctaggaactttattagtataaggatacagataaggtccattctctgttctcaagaatctgagtctacaggcagaagacaaaatgcagtacagaattatggaaatgtgaatggaaactgcattcagagaggggtattgcttgggaaaagccacattggcgtgccacagatgtatgccagcctggcaggcccatagtgtgattacttgagtttcaatatctgattcttttataggcttgaaattggtttatcaggtctggaagtgactggactctggagtactgagttacccaccacaaactgctaataaaatgctgtgtaaaagccattaatactaatgtattatttatgagaaacacaattatggggaagctaggatagttgagtttgctggtcattatcttccttgtattgaccaaattacaatgaaggctaaatccaaattataatcagaagattgcttggtaaatacagaacagaaacaatagaaatgtgtgtggtgcttttaatggctagtatttcaagcctgatgcagccctttccacttgagtcacattgtcttacattctttgacttggctagtgctaaaaatacattgccattttactttctccattttttttttttttttttttttgagacgacgtctggattgcaattggtgtgaggttggctcactacaacctctgcctcccgggttcaagcgattctcctgccccagcctcctgagtagctgggactacaggtgcacgccaccacgcccagctaatttttgtatttttagtagagacggggtttcaccatgttggccaggatggtctccatctcttgacctcgtgatccacctgcctcggcctcccaaagtgctgggattacaggcgtgagccaccacgcccagcccatcctttctcctcttaaattttctttgctgaccagtatctcttgatgtggaacgttctttcattagtggtaatactgtcaatcaggtctttggaagatattttgggttttgtttgctgaaccattatgcttattttacaaattaacttttctgaactttattgtggtagaatttacataacaatttaccattttgaccatttttaagttcaaaggaactaagtacattcacattgctatgcaactatgactaccatctagctccagaaccttttcatcttctcaaactgaaattctgtacccattaaacaataagctcccagccgggcacagtggctcgcgcctgtaatcccagcactttgggaggctgaggtgggcggattacctggagtcaggagttcgagaccagcctggccaacatgatggccatctctactaagaatacaaaaattagctggttgtggtgatgaatgcctgtaatcccagctacgtgggaggctgaggcatgagaatcacttgaacctgggaggcagacgttgcagtgagctgggattgcaccactgcactccagcctaggcaacagaaggagactcccgtctcaaaaaaaaaaaaacaaaacaaaaacaagaaccaataagctcccattccttctgccttccagcccttggcaaccaccattccactttaaatttgattattctaggagttcataaaagtggggtaacacagtatttgtcattttgtgactgacttatttcacctatcataaagtcttcaagattcatccaagatgtaatatatatcagaagtttcctcctttttaaggctgagtaatattccattgtgtgtatatgtcacatttcttttaaccattcatcccttgatggacacttggattgcttccaccttctggctattgtgaatgctgctgctgtgaacatagatgtacaaattatctgtccaagttcctgcttttacttcttttgggtatatacccggaagtggaattgctggatataattttaatttttgaggaatctccatactcagatgatcttatttccttatttttcaagtgtgtgggtctatgtgtggttttggcagggaagcgagtctctgttattcccacatactccccatgactgttaagtgctgtgttagaagcatatggtttgatgagaattctaggagagacaaatgtttcaaaggatctctgtattttcaccggcaataactaataaatcatctggcttcgctgttccccagaattattggagaaattgtgaaaaacttccgtgaagatgtaaactgtactccatagtccagttgttcccaatgagttaggagccttgctttaccctggtcaggagtttcgaaaggtgttcctttcactgcatgcaaaaatacgtacatccccagattatgtataatatttgttaaagtccaagcaacaggaacactgaagaagggaatgctgagtaagacaatatgaagcaagccaactcccaatgcatatgtcagccacataccccggctgttcatgacacgggtatttggattcacttcactgtgggcaactccaacgttcatgtttgctcgtgaagaggctgttggctctgccctcgccggtgcctccgaagacggcgacccgcagcggcccctcaggggagtcccccctgctagaccgacagcccgagcgctctgggccagag

SEQ ID NO: 13502 - RNA, 2892 nt, Homo sapiens
  source 1..2892: mol_type = other RNA
gctgggattacaggcatgagccaccacgcctggcccaaatcctatttttcaatatttatttcctaattatgtcctactaggttaggttttattttcatttgttacatatttattgggttatttcctttatgctaggaactttattagtataaggatacagataaggtccattctctgttctcaagaatctgagtctacaggcagaagacaaaatgcagtacagaattatggaaatgtgaatggaaactgcattcagagaggggtattgcttgggaaaagccacattggcgtgccacagatgtatgccagcctggcaggcccatagtgtgattacttgagtttcaatatctgattcttttataggcttgaaattggtttatcaggtctggaagtgactggactctggagtactgagttacccaccacaaactgctaataaaatgctgtgtaaaagccattaatactaatgtattatttatgagaaacacaattatggggaagctaggatagttgagtttgctggtcattatcttccttgtattgaccaaattacaatgaaggctaaatccaaattataatcagaagattgcttggtaaatacagaacagaaacaatagaaatgtgtgtggtgcttttaatggctagtatttcaagcctgatgcagccctttccacttgagtcacattgtcttacattctttgacttggctagtgctaaaaatacattgccattttactttctccattttttttttttttttttttttgagacgacgtctggattgcaattggtgtgaggttggctcactacaacctctgcctcccgggttcaagcgattctcctgccccagcctcctgagtagctgggactacaggtgcacgccaccacgcccagctaatttttgtatttttagtagagacggggtttcaccatgttggccaggatggtctccatctcttgacctcgtgatccacctgcctcggcctcccaaagtgctgggattacaggcgtgagccaccacgcccagcccatcctttctcctcttaaattttctttgctgaccagtatctcttgatgtggaacgttctttcattagtggtaatactgtcaatcaggtctttggaagatattttgggttttgtttgctgaaccattatgcttattttacaaattaacttttctgaactttattgtggtagaatttacataacaatttaccattttgaccatttttaagttcaaaggaactaagtacattcacattgctatgcaactatgactaccatctagctccagaaccttttcatcttctcaaactgaaattctgtacccattaaacaataagctcccagccgggcacagtggctcgcgcctgtaatcccagcactttgggaggctgaggtgggcggattacctggagtcaggagttcgagaccagcctggccaacatgatggccatctctactaagaatacaaaaattagctggttgtggtgatgaatgcctgtaatcccagctacgtgggaggctgaggcatgagaatcacttgaacctgggaggcagacgttgcagtgagctgggattgcaccactgcactccagcctaggcaacagaaggagactcccgtctcaaaaaaaaaaaaacaaaacaaaaacaagaaccaataagctcccattccttctgccttccagcccttggcaaccaccattccactttaaatttgattattctaggagttcataaaagtggggtaacacagtatttgtcattttgtgactgacttatttcacctatcataaagtcttcaagattcatccaagatgtaatatatatcagaagtttcctcctttttaaggctgagtaatattccattgtgtgtatatgtcacatttcttttaaccattcatcccttgatggacacttggattgcttccaccttctggctattgtgaatgctgctgctgtgaacatagatgtacaaattatctgtccaagttcctgcttttacttcttttgggtatatacccggaagtggaattgctggatataattttaatttttgaggaatctccatactcagatgatcttatttccttatttttcaagtgtgtgggtctatgtgtggttttggcagggaagcgagtctctgttattcccacatactccccatgactgttaagtgctgtgttagaagcatatggtttgatgagaattctaggagagacaaatgtttcaaaggatctctgtattttcaccggcaataactaataaatcatctggcttcgctgttcccccactccttccttataagaaattcagtagctgtaaaattttttttcagtttcaaaacatttcaatacttattaattccaaagatccgaacaccatgtagttgtggcattttgggaattagtacactcaggagagaagctgtgtttaggatgaagtgagttggatcatacttcgtatagaaacttgccagaaaatatagaattattggagaaattgtgaaaaacttccgtgaagatgtaaactgtactccatagtccagttgttcccaatgagttaggagccttgctttaccctggtcaggagtttcgaaaggtgttcctttcactgcatgcaaaaatacgtacatccccagattatgtataatatttgttaaagtccaagcaacaggaacactgaagaagggaatgctgagtaagacaatatgaagcaagccaactcccaatgcatatgtcagccacataccccggctgttcatgacacgggtatttggattcacttcactgtgggcaactccaacgttcatgtttgctccgccgccccactccgggccgccggctcgcagcaggaccagcccggctgctacggccgcggatacacgccc

SEQ ID NO: 13503 - RNA, 2826 nt, Homo sapiens
  source 1..2826: mol_type = other RNA
gctgggattacaggcatgagccaccacgcctggcccaaatcctatttttcaatatttatttcctaattatgtcctactaggttaggttttattttcatttgttacatatttattgggttatttcctttatgctaggaactttattagtataaggatacagataaggtccattctctgttctcaagaatctgagtctacaggcagaagacaaaatgcagtacagaattatggaaatgtgaatggaaactgcattcagagaggggtattgcttgggaaaagccacattggcgtgccacagatgtatgccagcctggcaggcccatagtgtgattacttgagtttcaatatctgattcttttataggcttgaaattggtttatcaggtctggaagtgactggactctggagtactgagttacccaccacaaactgctaataaaatgctgtgtaaaagccattaatactaatgtattatttatgagaaacacaattatggggaagctaggatagttgagtttgctggtcattatcttccttgtattgaccaaattacaatgaaggctaaatccaaattataatcagaagattgcttggtaaatacagaacagaaacaatagaaatgtgtgtggtgcttttaatggctagtatttcaagcctgatgcagccctttccacttgagtcacattgtcttacattctttgacttggctagtgctaaaaatacattgccattttactttctccattttttttttttttttttttttgagacgacgtctggattgcaattggtgtgaggttggctcactacaacctctgcctcccgggttcaagcgattctcctgccccagcctcctgagtagctgggactacaggtgcacgccaccacgcccagctaatttttgtatttttagtagagacggggtttcaccatgttggccaggatggtctccatctcttgacctcgtgatccacctgcctcggcctcccaaagtgctgggattacaggcgtgagccaccacgcccagcccatcctttctcctcttaaattttctttgctgaccagtatctcttgatgtggaacgttctttcattagtggtaatactgtcaatcaggtctttggaagatattttgggttttgtttgctgaaccattatgcttattttacaaattaacttttctgaactttattgtggtagaatttacataacaatttaccattttgaccatttttaagttcaaaggaactaagtacattcacattgctatgcaactatgactaccatctagctccagaaccttttcatcttctcaaactgaaattctgtacccattaaacaataagctcccagccgggcacagtggctcgcgcctgtaatcccagcactttgggaggctgaggtgggcggattacctggagtcaggagttcgagaccagcctggccaacatgatggccatctctactaagaatacaaaaattagctggttgtggtgatgaatgcctgtaatcccagctacgtgggaggctgaggcatgagaatcacttgaacctgggaggcagacgttgcagtgagctgggattgcaccactgcactccagcctaggcaacagaaggagactcccgtctcaaaaaaaaaaaaacaaaacaaaaacaagaaccaataagctcccattccttctgccttccagcccttggcaaccaccattccactttaaatttgattattctaggagttcataaaagtggggtaacacagtatttgtcattttgtgactgacttatttcacctatcataaagtcttcaagattcatccaagatgtaatatatatcagaagtttcctcctttttaaggctgagtaatattccattgtgtgtatatgtcacatttcttttaaccattcatcccttgatggacacttggattgcttccaccttctggctattgtgaatgctgctgctgtgaacatagatgtacaaattatctgtccaagttcctgcttttacttcttttgggtatatacccggaagtggaattgctggatataattttaatttttgaggaatctccatactcagatgatcttatttccttatttttcaagtgtgtgggtctatgtgtggttttggcagggaagcgagtctctgttattcccacatactccccatgactgttaagtgctgtgttagaagcatatggtttgatgagaattctaggagagacaaatgtttcaaaggatctctgtattttcaccggcaataactaataaatcatctggcttcgctgttccccttattaattccaaagatccgaacaccatgtagttgtggcattttgggaattagtacactcaggagagaagctgtgtttaggatgaagtgagttggatcatacttcgtatagaaacttgccagaaaatatagaattattggagaaattgtgaaaaacttccgtgaagatgtaaactgtactccatagtccagttgttcccaatgagttaggagccttgctttaccctggtcaggagtttcgaaaggtgttcctttcactgcatgcaaaaatacgtacatccccagattatgtataatatttgttaaagtccaagcaacaggaacactgaagaagggaatgctgagtaagacaatatgaagcaagccaactcccaatgcatatgtcagccacataccccggctgttcatgacacgggtatttggattcacttcactgtgggcaactccaacgttcatgtttgctccgccgccccactccgggccgccggctcgcagcaggaccagcccggctgctacggccgcggatacacgccc

SEQ ID NO: 13504 - RNA, 2936 nt, Homo sapiens
  source 1..2936: mol_type = other RNA
gctgggattacaggcatgagccaccacgcctggcccaaatcctatttttcaatatttatttcctaattatgtcctactaggttaggttttattttcatttgttacatatttattgggttatttcctttatgctaggaactttattagtataaggatacagataaggtccattctctgttctcaagaatctgagtctacaggcagaagacaaaatgcagtacagaattatggaaatgtgaatggaaactgcattcagagaggggtattgcttgggaaaagccacattggcgtgccacagatgtatgccagcctggcaggcccatagtgtgattacttgagtttcaatatctgattcttttataggcttgaaattggtttatcaggtctggaagtgactggactctggagtactgagttacccaccacaaactgctaataaaatgctgtgtaaaagccattaatactaatgtattatttatgagaaacacaattatggggaagctaggatagttgagtttgctggtcattatcttccttgtattgaccaaattacaatgaaggctaaatccaaattataatcagaagattgcttggtaaatacagaacagaaacaatagaaatgtgtgtggtgcttttaatggctagtatttcaagcctgatgcagccctttccacttgagtcacattgtcttacattctttgacttggctagtgctaaaaatacattgccattttactttctccattttttttttttttttttttttgagacgacgtctggattgcaattggtgtgaggttggctcactacaacctctgcctcccgggttcaagcgattctcctgccccagcctcctgagtagctgggactacaggtgcacgccaccacgcccagctaatttttgtatttttagtagagacggggtttcaccatgttggccaggatggtctccatctcttgacctcgtgatccacctgcctcggcctcccaaagtgctgggattacaggcgtgagccaccacgcccagcccatcctttctcctcttaaattttctttgctgaccagtatctcttgatgtggaacgttctttcattagtggtaatactgtcaatcaggtctttggaagatattttgggttttgtttgctgaaccattatgcttattttacaaattaacttttctgaactttattgtggtagaatttacataacaatttaccattttgaccatttttaagttcaaaggaactaagtacattcacattgctatgcaactatgactaccatctagctccagaaccttttcatcttctcaaactgaaattctgtacccattaaacaataagctcccagccgggcacagtggctcgcgcctgtaatcccagcactttgggaggctgaggtgggcggattacctggagtcaggagttcgagaccagcctggccaacatgatggccatctctactaagaatacaaaaattagctggttgtggtgatgaatgcctgtaatcccagctacgtgggaggctgaggcatgagaatcacttgaacctgggaggcagacgttgcagtgagctgggattgcaccactgcactccagcctaggcaacagaaggagactcccgtctcaaaaaaaaaaaaacaaaacaaaaacaagaaccaataagctcccattccttctgccttccagcccttggcaaccaccattccactttaaatttgattattctaggagttcataaaagtggggtaacacagtatttgtcattttgtgactgacttatttcacctatcataaagtcttcaagattcatccaagatgtaatatatatcagaagtttcctcctttttaaggctgagtaatattccattgtgtgtatatgtcacatttcttttaaccattcatcccttgatggacacttggattgcttccaccttctggctattgtgaatgctgctgctgtgaacatagatgtacaaattatctgtccaagttcctgcttttacttcttttgggtatatacccggaagtggaattgctggatataattttaatttttgaggaatctccatactcagatgatcttatttccttatttttcaagtgtgtgggtctatgtgtggttttggcagggaagcgagtctctgttattcccacatactccccatgactgttaagtgctgtgttagaagcatatggtttgatgagaattctaggagagacaaatgtttcaaaggatctctgtattttcaccggcaataactaataaatcatctggcttcgctgttccccttattaattccaaagatccgaacaccatgtagttgtggcattttgggaattagtacactcaggagagaagctgtgtttaggatgaagtgagttggatcatacttcgtatagaaacttgccagaaaatatagaattattggagaaattgtgaaaaacttccgtgaagatgtaaactgtactccatagtccagttgttcccaatgagttaggagccttgctttaccctggtcaggagtttcgaaaggtgttcctttcactgcatgcaaaaatacgtacatccccagattatgtataatatttgttaaagtccaagcaacaggaacactgaagaagggaatgctgagtaagacaatatgaagcaagccaactcccaatgcatatgtcagccacataccccggctgttcatgacacgggtatttggattcacttcactgtgggcaactccaacgttcatgtttgctcgagccagtgtgtcaagtagtcagactcttatatttgacttaatgtatccataaagaatggtcagagttcagatcacttctttctgaatactcaatgtggaaggtacatgccgccgccccactccgggccgccggctcgcagcaggaccagcccggctgctacggccgcggatacacgccc

SEQ ID NO: 13505 - RNA, 1252 nt, Homo sapiens
  source 1..1252: mol_type = other RNA
gctgggattacaggcatgagccaccacgcctggcccaacatggctattattttttaaagtgctaaattatggccgggggctgtgactcacgcctgtaatcccagcactttgggaggccgaggcgggtgaatcacgaggtcaggagatggagaccagcctggccaacatggtgaaaccccatctctactaagaatacaaaaaattagctgggcgtggtggcaggcgcctgtaatcccatctactcaggaagctgaggctggagaatcgcttgaacccgggaggcggaggttgcagtgagcagagatcacgccactgcagtccagcctgggcaacagtgcgagactctgtctcaaaaaaaaaataaataaattacctgggtgtggcagcgcgtgcctgtaatcccagctacccaggaggctgaggcaagagaactgcttgaacccaggaggcagaggttgcatggagctgagatggcaccactgcactccagtctggtgacagagtgagactccatctcaaaaaaaaaaaaaaaaagtgctaagttacatctaagtttcctatttttgtttaaaaaactccttgtagtgggttgaatggtggaccccaaaatgatacatctgtccatctgatatgcgtgaatgtgacctatttgggaaaacagtttttgtagatgaaattaaggatttccaaatgagatcatcctaggttagaatggaacctaaatccaacagcaaaagtcctcataaaaagaagggaagaagacagaaaagaagaccacaaagacaaaggcagagataggagttatgctgccataagccaagtaatacctggagccaccagcagctggaagaggaaagcaaggattctcccttggagccttcagagggaggtgtggcccagctgacatcttgctctcagatttctggcctccagaactctgctttctctgagaggcagtcaagctatcctctttcctctttcccttgctaatttcctgggttttcttcatgtttttctggcgggcaagttctcgttgatttccacgggccatgccgaccaccaacggagcctggaagaagagcaactcggaaaagcaacggttctctggcactctgggataccgtcaccaccgctgaccgggaaggctgagccctcgtgggccctccgcccggctgcgcctcccctctgctccgccaacggccccgcccgctggaggcccgacaacagccgccggcatggccggcgcgtcact

SEQ ID NO: 13506 - RNA, 1252 nt, Homo sapiens
  source 1..1252: mol_type = other RNA
gctgggattacaggcatgagccaccacgcctggcccaacatggctattattttttaaagtgctaaattatggccgggggctgtgactcacgcctgtaatcccagcactttgggaggccgaggcgggtgaatcacgaggtcaggagatggagaccagcctggccaacatggtgaaaccccatctctactaagaatacaaaaaattagctgggcgtggtggcaggcgcctgtaatcccatctactcaggaagctgaggctggagaatcgcttgaacccgggaggcggaggttgcagtgagcagagatcacgccactgcagtccagcctgggcaacagtgcgagactctgtctcaaaaaaaaaataaataaattacctgggtgtggcagcgcgtgcctgtaatcccagctacccaggaggctgaggcaagagaactgcttgaacccaggaggcagaggttgcatggagctgagatggcgccactgcactccagtctggtgacagagtgagactccatctcaaaaaaaaaaaaaaaaagtgctaagttacatctaagtttcctatttttgtttaaaaaactccttgtagtgggttgaatggtggaccccaaaatgatacatctgtccatctgatatgcgtgaatgtgacctatttgggaaaacagtttttgtagatgaaattaaggatttccaaatgagatcatcctaggttagaatggaacctaaatccaacagcaaaagtcctcataaaaagaagggaagaagacagaaaagaagaccacaaagacaaaggcagagataggagttatgctgccataagccaagtaatacctggagccaccagcagctggaagaggaaagcaaggattctcccttggagccttcagagggaggtgtggcccagctgacatcttgctctcagatttctggcctccagaactctgctttctctgagaggcagtcaagctatcctctttcctctttcccttgctaatttcctgggttttcttcatgtttttctggcgggcaagttctcgttgatttccacgggccatgccgaccaccaacggagcctggaagaagagcaactcggaaaagcaacggttctctggcactctgggataccgtcaccaccgctgaccgggaaggctgagccctcgtgggccctccgcccggctgcgcctcccctctgctccgccaacggccccgcccgctggaggcccgacaacagccgccggcatggccggcgcgtcact

SEQ ID NO: 13507 - RNA, 2055 nt, Homo sapiens
  source 1..2055: mol_type = other RNA
gctgggattacaggcatgagccaccacgcctggcccagactcttctcagcttctcggcagcatttcttcctctaggggatgaggcagaacccaccctggaatgaggatcttctgacccacagtcagattagggtcttgagattcagcttcctgaggcctaaactgccccaacgtgataacaaaaggctataaccagggctgtgtgagttaggaggcaggagctggatttctctctggtcctccaagctgctgaacttgtcccctccgcagggcctccagcctggcatgctcttccctgggagcgccgcgtgctacttcttacaattttgggtcttgctcagatgataactccttggggcagccttccccgaccaccctccccaggcactccctgccacaaatgtccccactgcacttacgctgcggggagttctctatccgcttccttgttcaccctcactggtctccccaggaaagctccaggagggaggcgctggttctgtgtattcacctgtgctggggctggcactccaggcagagctgtggcggaaggaagtggcccgagacagcctgattccatcttttggtttctgtgtgtttcctcctcatagacccgcaccagcgaacagggaacctccagacaaacatcgctgccttcctgcagctccgttccaggcagggaggcacagatgagacgtggtgggcagatgaggttgtttcaggttgtgttagacagtgtggaggaaatcaacagaatgctgtggacagtgccccggcggtgatgggcagattagggactgcacgcaggagtcagtcacgggaggggaatggcaccactcttctcctggggatggtggagcctgaggcaccacgtccacgaggtcctcttggggtggaggcagacctctctctatatcaatatccatatccatattcatccattcccgtgcttatgtccacttccatatccacgcatgtcctgttactctgcttccctggggacccctggctgaaacaggaggcttctattgaactcactggatgtggcaaattaagaaaggtttctcttgttctggggtcttaggtgacccctgctggtcccctctgttggtgatttccttgaccctggggtgctgccctctctgcagcgtcagcctctactggttcttgaagagaagcagcaggccagccccatccctctggatttatatgtgggggcagatctctcggtcatgggtctctcaggtgctagcaccacagcatggagttatctgagttgtcatctcagagcaggaactcatcaccaaggagagagtgccaagccatgcatgaggaatccactgccatgatccaacacctcccatcaggccccacctccaacactggggaccacatttcaacatgagatttggaggggacacacatccaaaccacatcaccacacagttgtggtgataagatataaaatctatcatggcaaaggcaaaaaataaaaagaaatgaagttgagtttaacaatcagtggtaagtggcagttataaccactgtgtcttctgtctcatagtggaacaccgaggcatggggcagcttcccatcaccttacctttgatgatggtacctcttagctttcttcttggggcctccgtctctccatttgtaagcagaatattggatttgctagttcctgcggtcctcccagagtgacatgctaggctgctgactggaattgcggaggggccagagcagaccgcccctagaagggtccgcccaagtaggaaatgacagcctccctgccttgtcatctcctcctccagagtggacgtatggagacttcactgcacatgtggggattgtgcttgttgacctcgtagttccctctgaagagggcatttgggtctcaatagaggcccagttgctgcccagggaaataagaaattctataacatccacagcttatgtggccttaaaaactcaaagaagagctgggtgcggtggctcactcctgtaatcccagcactttgggaggccaagatgggcggatcacaaggtcaagag

SEQ ID NO: 13508 - RNA, 2093 nt, Homo sapiens
  source 1..2093: mol_type = other RNA
gctgggattacaggcatgagccaccacgcctggcccagactcttctcagcttctcggcagcatttcttcctctaggggatgaggcagaacccaccctggaatgaggatcttctgacccacagtcagattagggtcttgagattcagcttcctgaggcctaaactgccccaacgtgataacaaaaggctataaccagggctgtgtgagttaggaggcaggagctggatttctctctggtcctccaagctgctgaacttgtcccctccgcagggcctccagcctggcatgctcttccctgggagcgccgcgtgctacttcttacaattttgggtcttgctcagatgataactccttggggcagccttccccgaccaccctccccaggcactccctgccacaaatgtccccactgcacttacgctgcggggagttctctatccgcttccttgttcaccctcactggtctccccaggaaagctccaggagggaggcgctggttctgtgtattcacctgtgctggggctggcactccaggcagagctgtggcggaaggaagtggcccgagacagcctgattccatcttttggtttctgtgtgtttcctcctcatagacccgcaccagcgaacagggaacctccagacaaacatcgctgccttcctgcagctccgttccaggcagggaggcacagatgagacgtggtgggcagatgaggttgtttcaggttgtgttagacagtgtggaggaaatcaacagaatgctgtggacagtgccccggcggtgatgggcagattagggactgcacgcaggagtcagtcacgggaggggaatggcaccactgtcccaaaaacagcaaaaacgagtccaagcatggcactcttctcctggggatggtggagcctgaggcaccacgtccacgaggtcctcttggggtggaggcagacctctctctatatcaatatccatatccatattcatccattcccgtgcttatgtccacttccatatccacgcatgtcctgttactctgcttccctggggacccctggctgaaacaggaggcttctattgaactcactggatgtggcaaattaagaaaggtttctcttgttctggggtcttaggtgacccctgctggtcccctctgttggtgatttccttgaccctggggtgctgccctctctgcagcgtcagcctctactggttcttgaagagaagcagcaggccagccccatccctctggatttatatgtgggggcagatctctcggtcatgggtctctcaggtgctagcaccacagcatggagttatctgagttgtcatctcagagcaggaactcatcaccaaggagagagtgccaagccatgcatgaggaatccactgccatgatccaacacctcccatcaggccccacctccaacactggggaccacatttcaacatgagatttggaggggacacacatccaaaccacatcaccacacagttgtggtgataagatataaaatctatcatggcaaaggcaaaaaataaaaagaaatgaagttgagtttaacaatcagtggtaagtggcagttataaccactgtgtcttctgtctcatagtggaacaccgaggcatggggcagcttcccatcaccttacctttgatgatggtacctcttagctttcttcttggggcctccgtctctccatttgtaagcagaatattggatttgctagttcctgcggtcctcccagagtgacatgctaggctgctgactggaattgcggaggggccagagcagaccgcccctagaagggtccgcccaagtaggaaatgacagcctccctgccttgtcatctcctcctccagagtggacgtatggagacttcactgcacatgtggggattgtgcttgttgacctcgtagttccctctgaagagggcatttgggtctcaatagaggcccagttgctgcccagggaaataagaaattctataacatccacagcttatgtggccttaaaaactcaaagaagagctgggtgcggtggctcactcctgtaatcccagcactttgggaggccaagatgggcggatcacaaggtcaagag

SEQ ID NO: 13509 - RNA, 1499 nt, Homo sapiens
  source 1..1499: mol_type = other RNA
gctgggattacaggcatgagccaccacgcctggcccagactcttctcagcttctcggcagcatttcttcctctaggggatgaggcagaacccaccctggaatgaggatcttctgacccacagtcagattagggtcttgagattcagcttcctgaggcctaaactgccccaacgtgataacaaaaggctataaccagggctgtgtgagttaggaggcaggagctggatttctctctggtcctccaagctgctgaacttgtcccctccgcagggcctccagcctggcatgctcttccctgggagcgccgcgtgctacttcttacaattttgggtcttgctcagatgataactccttggggcagccttccccgaccaccctccccaggcactccctgccacaaatgtccccactgcacttacgctgcggggagttctctatccgcttccttgttcaccctcactggtctccccaggaaagctccaggagggaggcgctggttctgtgtattcacctgtgctggggctggcactccaggcagagctgtggcggaaggaagtggcccgagacagcctgattccatcttttggtttctgtgtgtttcctcctcatagacccgcaccagcgaacagggaacctccagacaaacatcgctgccttcctgcagctccgttccaggcagggaggcacagatgagacgtggtgggcagatgaggttgtttcaggttgtgttagacagtgtggaggaaatcaacagaatgctgtggacagtgccccggcggtgatgggcagattagggactgcacgcaggagtcagtcacgggaggggaatggcaccactgtcccaaaaacagcaaaaacgagtccaagcatggcactcttctcctggggatggtggagcctgaggcaccacgtccacgaggtcctcttggggtggaggcagacctctctctatatcaatatccatatccatattcatccattcccgtgcttatgtccacttccatatccacgcatgtcctgttactctgcttccctggggacccctggctttgatgatggtacctcttagctttcttcttggggcctccgtctctccatttgtaagcagaatattggatttgctagttcctgcggtcctcccagagtgacatgctaggctgctgactggaattgcggaggggccagagcagaccgcccctagaagggtccgcccaagtaggaaatgacagcctccctgccttgtcatctcctcctccagagtggacgtatggagacttcactgcacatgtggggattgtgcttgttgacctcgtagttccctctgaagagggcatttgggtctcaatagaggcccagttgctgcccagggaaataagaaattctataacatccacagcttatgtggccttaaaaactcaaagaagagctgggtgcggtggctcactcctgtaatcccagcactttgggaggccaagatgggcggatcacaaggtcaagag

SEQ ID NO: 13510 - RNA, 1394 nt, Homo sapiens
  source 1..1394: mol_type = other RNA
gctgggattacaggcatgagccaccacgcctggcccagactcttctcagcttctcggcagcatttcttcctctaggggatgaggcagaacccaccctggaatgaggatcttctgacccacagtcagattagggtcttgagattcagcttcctgaggcctaaactgccccaacgtgataacaaaaggctataaccagggctgtgtgagttaggaggcaggagctggatttctctctggtcctccaagctgctgaacttgtcccctccgcagggcctccagcctggcatgctcttccctgggagcgccgcgtgctacttcttacaattttgggtcttgctcagatgataactccttggggcagccttccccgaccaccctccccaggcactccctgccacaaatgtccccactgcacttacgctgcggggagttctctatccgcttccttgttcaccctcactggtctccccaggaaagctccaggagggaggcgctggttctgtgtattcacctgtgctggggctggcactccaggcagagctgtggcggaaggaagtggcccgagacagcctgattccatcttttggtttctgtgtgtttcctcctcatagacccgcaccagcgaacagggaacctccagacaaacatcgctgccttcctgcagctccgttccaggcagggaggcacagatgagacgtggtgggcagatgaggttgtttcaggttgtgttagacagtgtggaggaaatcaacagaatgctgtggacagtgccccggcggtgatgggcagattagggactgcacgcaggagtcagtcacgggaggggaatggcaccactgtcccaaaaacagcaaaaacgagtccaagcatggcactcttctcctggggatggtggagcctgaggcaccacgtccacgaggtcctcttggggtggaggcagacctttgatgatggtacctcttagctttcttcttggggcctccgtctctccatttgtaagcagaatattggatttgctagttcctgcggtcctcccagagtgacatgctaggctgctgactggaattgcggaggggccagagcagaccgcccctagaagggtccgcccaagtaggaaatgacagcctccctgccttgtcatctcctcctccagagtggacgtatggagacttcactgcacatgtggggattgtgcttgttgacctcgtagttccctctgaagagggcatttgggtctcaatagaggcccagttgctgcccagggaaataagaaattctataacatccacagcttatgtggccttaaaaactcaaagaagagctgggtgcggtggctcactcctgtaatcccagcactttgggaggccaagatgggcggatcacaaggtcaagag

SEQ ID NO: 13511 - RNA, 2113 nt, Homo sapiens
  source 1..2113: mol_type = other RNA
gctgggattacaggcatgagccaccacgcctggcccagactcttctcagcttctcggcagcatttcttcctctaggggatgaggcagaacccaccctggaatgaggatcttctgacccacagtcagattagggtcttgagattcagcttcctgaggcctaaactgccccaacgtgataacaaaaggctataaccagggctgtgtgagttaggaggcaggagctggatttctctctggtcctccaagctgctgaacttgtcccctccgcagggcctccagcctggcatgctcttccctgggagcgccgcgtgctacttcttacaattttgggtcttgctcagatgataactccttggggcagccttccccgaccaccctccccaggcactccctgccacaaatgtccccactgcacttacgctgcggggagttctctatccgcttccttgttcaccctcactggtctccccaggaaagctccaggagggaggcgctggttctgtgtattcacctgtgctggggctggcactccaggcagagctgtggcggaaggaagtggcccgagacagcctgattccatcttttggtttctgtgtgtttcctcctcatagacccgcaccagcgaacagggaacctgcaaccagggggtggacactccagacaaacatcgctgccttcctgcagctccgttccaggcagggaggcacagatgagacgtggtgggcagatgaggttgtttcaggttgtgttagacagtgtggaggaaatcaacagaatgctgtggacagtgccccggcggtgatgggcagattagggactgcacgcaggagtcagtcacgggaggggaatggcaccactgtcccaaaaacagcaaaaacgagtccaagcatggcactcttctcctggggatggtggagcctgaggcaccacgtccacgaggtcctcttggggtggaggcagacctctctctatatcaatatccatatccatattcatccattcccgtgcttatgtccacttccatatccacgcatgtcctgttactctgcttccctggggacccctggctgaaacaggaggcttctattgaactcactggatgtggcaaattaagaaaggtttctcttgttctggggtcttaggtgacccctgctggtcccctctgttggtgatttccttgaccctggggtgctgccctctctgcagcgtcagcctctactggttcttgaagagaagcagcaggccagccccatccctctggatttatatgtgggggcagatctctcggtcatgggtctctcaggtgctagcaccacagcatggagttatctgagttgtcatctcagagcaggaactcatcaccaaggagagagtgccaagccatgcatgaggaatccactgccatgatccaacacctcccatcaggccccacctccaacactggggaccacatttcaacatgagatttggaggggacacacatccaaaccacatcaccacacagttgtggtgataagatataaaatctatcatggcaaaggcaaaaaataaaaagaaatgaagttgagtttaacaatcagtggtaagtggcagttataaccactgtgtcttctgtctcatagtggaacaccgaggcatggggcagcttcccatcaccttacctttgatgatggtacctcttagctttcttcttggggcctccgtctctccatttgtaagcagaatattggatttgctagttcctgcggtcctcccagagtgacatgctaggctgctgactggaattgcggaggggccagagcagaccgcccctagaagggtccgcccaagtaggaaatgacagcctccctgccttgtcatctcctcctccagagtggacgtatggagacttcactgcacatgtggggattgtgcttgttgacctcgtagttccctctgaagagggcatttgggtctcaatagaggcccagttgctgcccagggaaataagaaattctataacatccacagcttatgtggccttaaaaactcaaagaagagctgggtgcggtggctcactcctgtaatcccagcactttgggaggccaagatgggcggatcacaaggtcaagag

SEQ ID NO: 13512 - RNA, 1991 nt, Homo sapiens
  source 1..1991: mol_type = other RNA
gctgggattacaggcatgagccaccacgcctggcccagactcttctcagcttctcggcagcatttcttcctctaggggatgaggcagaacccaccctggaatgaggatcttctgacccacagtcagattagggtcttgagattcagcttcctgaggcctaaactgccccaacgtgataacaaaaggctataaccagggctgtgtgagttaggaggcaggagctggatttctctctggtcctccaagctgctgaacttgtcccctccgcagggcctccagcctggcatgctcttccctgggagcgccgcgtgctacttgctgcggggagttctctatccgcttccttgttcaccctcactggtctccccaggaaagctccaggagggaggcgctggttctgtgtattcacctgtgctggggctggcactccaggcagagctgtggcggaaggaagtggcccgagacagcctgattccatcttttggtttctgtgtgtttcctcctcatagacccgcaccagcgaacagggaacctccagacaaacatcgctgccttcctgcagctccgttccaggcagggaggcacagatgagacgtggtgggcagatgaggttgtttcaggttgtgttagacagtgtggaggaaatcaacagaatgctgtggacagtgccccggcggtgatgggcagattagggactgcacgcaggagtcagtcacgggaggggaatggcaccactgtcccaaaaacagcaaaaacgagtccaagcatggcactcttctcctggggatggtggagcctgaggcaccacgtccacgaggtcctcttggggtggaggcagacctctctctatatcaatatccatatccatattcatccattcccgtgcttatgtccacttccatatccacgcatgtcctgttactctgcttccctggggacccctggctgaaacaggaggcttctattgaactcactggatgtggcaaattaagaaaggtttctcttgttctggggtcttaggtgacccctgctggtcccctctgttggtgatttccttgaccctggggtgctgccctctctgcagcgtcagcctctactggttcttgaagagaagcagcaggccagccccatccctctggatttatatgtgggggcagatctctcggtcatgggtctctcaggtgctagcaccacagcatggagttatctgagttgtcatctcagagcaggaactcatcaccaaggagagagtgccaagccatgcatgaggaatccactgccatgatccaacacctcccatcaggccccacctccaacactggggaccacatttcaacatgagatttggaggggacacacatccaaaccacatcaccacacagttgtggtgataagatataaaatctatcatggcaaaggcaaaaaataaaaagaaatgaagttgagtttaacaatcagtggtaagtggcagttataaccactgtgtcttctgtctcatagtggaacaccgaggcatggggcagcttcccatcaccttacctttgatgatggtacctcttagctttcttcttggggcctccgtctctccatttgtaagcagaatattggatttgctagttcctgcggtcctcccagagtgacatgctaggctgctgactggaattgcggaggggccagagcagaccgcccctagaagggtccgcccaagtaggaaatgacagcctccctgccttgtcatctcctcctccagagtggacgtatggagacttcactgcacatgtggggattgtgcttgttgacctcgtagttccctctgaagagggcatttgggtctcaatagaggcccagttgctgcccagggaaataagaaattctataacatccacagcttatgtggccttaaaaactcaaagaagagctgggtgcggtggctcactcctgtaatcccagcactttgggaggccaagatgggcggatcacaaggtcaagag

SEQ ID NO: 13513 - RNA, 1988 nt, Homo sapiens
  source 1..1988: mol_type = other RNA
gctgggattacaggcatgagccaccacgcctggcccagactcttctcagcttctcggcagcatttcttcctctaggggatgaggcagaacccaccctggaatgaggatcttctgacccacagtcagattagggtcttgagattcagcttcctgaggcctaaactgccccaacgtgataacaaaaggctataaccagggctgtgtgagttaggaggcaggagctggatttctctctggtcctccaagctgctgaacttgtcccctccgcagggcctccagcctggcatgctcttccctgggagcgccgcgtgctagctgcggggagttctctatccgcttccttgttcaccctcactggtctccccaggaaagctccaggagggaggcgctggttctgtgtattcacctgtgctggggctggcactccaggcagagctgtggcggaaggaagtggcccgagacagcctgattccatcttttggtttctgtgtgtttcctcctcatagacccgcaccagcgaacagggaacctccagacaaacatcgctgccttcctgcagctccgttccaggcagggaggcacagatgagacgtggtgggcagatgaggttgtttcaggttgtgttagacagtgtggaggaaatcaacagaatgctgtggacagtgccccggcggtgatgggcagattagggactgcacgcaggagtcagtcacgggaggggaatggcaccactgtcccaaaaacagcaaaaacgagtccaagcatggcactcttctcctggggatggtggagcctgaggcaccacgtccacgaggtcctcttggggtggaggcagacctctctctatatcaatatccatatccatattcatccattcccgtgcttatgtccacttccatatccacgcatgtcctgttactctgcttccctggggacccctggctgaaacaggaggcttctattgaactcactggatgtggcaaattaagaaaggtttctcttgttctggggtcttaggtgacccctgctggtcccctctgttggtgatttccttgaccctggggtgctgccctctctgcagcgtcagcctctactggttcttgaagagaagcagcaggccagccccatccctctggatttatatgtgggggcagatctctcggtcatgggtctctcaggtgctagcaccacagcatggagttatctgagttgtcatctcagagcaggaactcatcaccaaggagagagtgccaagccatgcatgaggaatccactgccatgatccaacacctcccatcaggccccacctccaacactggggaccacatttcaacatgagatttggaggggacacacatccaaaccacatcaccacacagttgtggtgataagatataaaatctatcatggcaaaggcaaaaaataaaaagaaatgaagttgagtttaacaatcagtggtaagtggcagttataaccactgtgtcttctgtctcatagtggaacaccgaggcatggggcagcttcccatcaccttacctttgatgatggtacctcttagctttcttcttggggcctccgtctctccatttgtaagcagaatattggatttgctagttcctgcggtcctcccagagtgacatgctaggctgctgactggaattgcggaggggccagagcagaccgcccctagaagggtccgcccaagtaggaaatgacagcctccctgccttgtcatctcctcctccagagtggacgtatggagacttcactgcacatgtggggattgtgcttgttgacctcgtagttccctctgaagagggcatttgggtctcaatagaggcccagttgctgcccagggaaataagaaattctataacatccacagcttatgtggccttaaaaactcaaagaagagctgggtgcggtggctcactcctgtaatcccagcactttgggaggccaagatgggcggatcacaaggtcaagag

SEQ ID NO: 13514 - RNA, 1895 nt, Homo sapiens
  source 1..1895: mol_type = other RNA
gctgggattacaggcatgagccaccacgcctggcccagactcttctcagcttctcggcagcatttcttcctctaggggatgaggcagaacccaccctggaatgaggatcttctgacccacagtcagattagggtcttgagattcagcttcctgaggcctaaactgccccaacgtgataacaaaaggctataaccagggctgtgtgagttaggaggcaggaggctgcggggagttctctatccgcttccttgttcaccctcactggtctccccaggaaagctccaggagggaggcgctggttctgtgtattcacctgtgctggggctggcactccaggcagagctgtggcggaaggaagtggcccgagacagcctgattccatcttttggtttctgtgtgtttcctcctcatagacccgcaccagcgaacagggaacctccagacaaacatcgctgccttcctgcagctccgttccaggcagggaggcacagatgagacgtggtgggcagatgaggttgtttcaggttgtgttagacagtgtggaggaaatcaacagaatgctgtggacagtgccccggcggtgatgggcagattagggactgcacgcaggagtcagtcacgggaggggaatggcaccactgtcccaaaaacagcaaaaacgagtccaagcatggcactcttctcctggggatggtggagcctgaggcaccacgtccacgaggtcctcttggggtggaggcagacctctctctatatcaatatccatatccatattcatccattcccgtgcttatgtccacttccatatccacgcatgtcctgttactctgcttccctggggacccctggctgaaacaggaggcttctattgaactcactggatgtggcaaattaagaaaggtttctcttgttctggggtcttaggtgacccctgctggtcccctctgttggtgatttccttgaccctggggtgctgccctctctgcagcgtcagcctctactggttcttgaagagaagcagcaggccagccccatccctctggatttatatgtgggggcagatctctcggtcatgggtctctcaggtgctagcaccacagcatggagttatctgagttgtcatctcagagcaggaactcatcaccaaggagagagtgccaagccatgcatgaggaatccactgccatgatccaacacctcccatcaggccccacctccaacactggggaccacatttcaacatgagatttggaggggacacacatccaaaccacatcaccacacagttgtggtgataagatataaaatctatcatggcaaaggcaaaaaataaaaagaaatgaagttgagtttaacaatcagtggtaagtggcagttataaccactgtgtcttctgtctcatagtggaacaccgaggcatggggcagcttcccatcaccttacctttgatgatggtacctcttagctttcttcttggggcctccgtctctccatttgtaagcagaatattggatttgctagttcctgcggtcctcccagagtgacatgctaggctgctgactggaattgcggaggggccagagcagaccgcccctagaagggtccgcccaagtaggaaatgacagcctccctgccttgtcatctcctcctccagagtggacgtatggagacttcactgcacatgtggggattgtgcttgttgacctcgtagttccctctgaagagggcatttgggtctcaatagaggcccagttgctgcccagggaaataagaaattctataacatccacagcttatgtggccttaaaaactcaaagaagagctgggtgcggtggctcactcctgtaatcccagcactttgggaggccaagatgggcggatcacaaggtcaagag

SEQ ID NO: 13515 - RNA, 1877 nt, Homo sapiens
  source 1..1877: mol_type = other RNA
gctgggattacaggcatgagccaccacgcctggcccagtttgtttactcactgatttaaccaatcctatagagtgccttctaggagctaggtgatattgcttcaggccctgggaataccctagggatgatctagactcagatccctgtcctcgtggaacttacattctagtggaaagagagacagtgaacagttacagacacaacataatgtcatgtagtggtaaatactaggaagaaaaataaagcagggtgagaggatatgaagtgatggcacgagacttctttttagacagtgtggtcaggaggacctctgtgaagaggggcatttgagcagaaaccttctccttctttgatagtataaatacaccaaccactgtgcaataaaaggccatatgatggcaaacgttagcacaccaggagacatctcgaagggccaccaagatggtctctgtgaggtgggctgaggagcagtctgcaatgttgatgttgatgattttgcctgcaaagcagtcagcgtttccagtttctgcagtctctgaaggacattctgcatgtcctcctgcagtctcatcagcacgagggcgatctgctcattgaggctgcctcgggaccctctgtcggagccccagcgctccccatcacctccacttcccacctgccggcccttggttccttcgctcaagtgttgcatcctatgtcctcttcctcttctaacattagagaattcgtcagtttctccgcctcgcttctcccggtgtggtgctccgctgttattcctgccatcttctcctccatgcttgacttcaccttttccttcaactgcaaccacctgcatattcccaatgttgccatttccaggaggtacttgaatatcttcacgaaatccagaattttccatgggttgactggaatgaccacccaagtaatactgaaatggtccattgttggacgtaaagctgtctaaagactcttcttgtccaaattgttccatagaatcacagtaaacttcactgtctgaatcgcttgtcaaatgctgaattcctgtaacatcttcaacatgatcatcatttatatcttggtgaatgcaaacagcagattttccagtttgccccaagttttcatcaatgggctttacttcttcagtgcttctgccattcagggaagaactggcatgaatgtcattctgtatatcctgaacaaagccatctttatcatagccattagtgacaatgacttccaaattcttatggtctgctgacttcttcatcattttcttatcattatcactttgttctgctcctttcacttcttcttgggcctcttcttcctcagactcggctccactgtcactgctttcagctttaccattaacggttttggcgtttggagtagaagtgagaacattaccaagatctgaggttatatcagaactcctgccactctttttgtcctcgacaatttcataaaatggacctatgacacgcagcaattcttcaactttctcagtcattggcatagtttcaataatctttttcatttcttcaacatatgcaatcatggcttcctctttggtcatatcacccagtgaactccaagcatcccattcttcggcaaactctggatcaccttcacggccgcctcaaacctagtctcgtgcacggatctcgtgtccgccatctccagctgccagtgttggccccggtcccaaggtctgtcggcgggaatcaggcagcagcagcaccagctttcccaagagccgagaggaagagcatgtctagcagaagacagagggggtccgggcatcggtggccgcggagccgctctcccaccctggggaccctggcggagcagccacaccccccattccgccggagtc

SEQ ID NO: 13516 - RNA, 1891 nt, Homo sapiens
  source 1..1891: mol_type = other RNA
gctgggattacaggcatgagccaccacgcctggcccagtttgtttactcactgatttaaccaatcctatagagtgccttctaggagctaggtgatattgcttcaggccctgggaataccctagggatgatctagactcagatccctgtcctcgtggaacttacattctagtggaaagagagacagtgaacagttacagacacaacataatgtcatgtagtggtaaatactaggaagaaaaataaagcagggtgagaggatatgaagtgatggcacgagacttctttttagacagtgtggtcaggaggacctctgtgaagaggggcatttgagcagaaaccttctccttctttgatagtataaatacaccaaccactgtgcaataaaaggccatatgatggcaaacgttagcacaccaggagacatctcgaagggccaccaagatggtctctgtgaggtgggctgaggagcagtctgcaatgttgatgttgatgattttgcctgcaaagcagtcagcgtttccagtttctgcagtctctgaaggacattctgcatgtcctcctgcagtctcatcagcacgagggcgatctgctcattgaggctgcctcgggaccctctgtcggagccccagcgctccccatcacctccacttcccacctgccggcccttggttccttcgctcaagtgttgcatcctatgtcctcttcctcttctaacattagagaattcgtcagtttctccgcctcgcttctcccggtgtggtgctccgctgttattcctgccatcttctcctccatgcttgacttcaccttttccttcaactgcaaccacctgcatattcccaatgttgccatttccaggaggtacttgaatatcttcacgaaatccagaattttccatgggttgactggaatgaccacccaagtaatactgaaatggtccattgttggacgtaaagctgtctaaagactcttcttgtccaaattgttccatagaatcacagtaaacttcactgtctgaatcgcttgtcaaatgctgaattcctgtaacatcttcaacatgatcatcatttatatcttggtgaatgcaaacagcagattttccagtttgccccaagttttcatcaatgggctttacttcttcagtgcttctgccattcagggaagaactggcatgaatgtcattctgtatatcctgaacaaagccatctttatcatagccattagtgacaatgacttccaaattcttatggtctgctgacttcttcatcattttcttatcattatcactttgttctgctcctttcacttcttcttgggcctcttcttcctcagactcggctccactgtcactgctttcagctttaccattaacggttttggcgtttggagtagaagtgagaacattaccaagatctgaggttatatcagaactcctgccactctttttgtcctcgacaatttcataaaatggacctatgacacgcagcaattcttcaactttctcagtcattggcatagtttcaataatctttttcatttcttcaacatatgcaatcatggcttcctctttggtcatatcacccagtgaactccaagcatcccattcttcggcaaactctggatcaccttcacggccgcctcaaacctagtctcgtgcacggatctcgtgtccgccatctccagctgccagtgttggccccggtcccaaggtctgtcggcgggaatcaggcagcagcagcaccagctttcccaagagcctgcatgaaacgagaggaagagcatgtctagcagaagacagagggggtccgggcatcggtggccgcggagccgctctcccaccctggggaccctggcggagcagccacaccccccattccgccggagtccgtc

SEQ ID NO: 13517 - RNA, 2025 nt, Homo sapiens
  source 1..2025: mol_type = other RNA
gctgggattacaggcatgagccaccacgcctggcccagtttgtttactcactgatttaaccaatcctatagagtgccttctaggagctaggtgatattgcttcaggccctgggaataccctagggatgatctagactcagatccctgtcctcgtggaacttacattctagtggaaagagagacagtgaacagttacagacacaacataatgtcatgtagtggtaaatactaggaagaaaaataaagcagggtgagaggatatgaagtgatggcacgagacttctttttagacagtgtggtcaggaggacctctgtgaagaggggcatttgagcagaaaccttctccttctttgatagtataaatacaccaaccactgtgcaataaaaggccatatgatggcaaacgttagcacaccaggagacatctcgaagggccaccaagatggtctctgtgaggtgggctgaggagcagtctgcaatgttgatgttgatgattttgcctgcaaagcagtcagcgtttccagtttctgcagtctctgaaggacattctgcatgtcctcctgcagtctcatcagcacgagggcgatctgctcattgaggctgcctcgggaccctctgtcggagccccagcgctccccatcacctccacttcccacctgccggcccttggttccttcgctcaagtgttgcatcctatgtcctcttcctcttctaacattagagaattcgtcagtttctccgcctcgcttctcccggtgtggtgctccgctgttattcctgccatcttctcctccatgcttgacttcaccttttccttcaactgcaaccacctgcatattcccaatgttgccatttccaggaggtacttgaatatcttcacgaaatccagaattttccatgggttgactggaatgaccacccaagtaatactgaaatggtccattgttggacgtaaagctgtctaaagactcttcttgtccaaattgttccatagaatcacagtaaacttcactgtctgaatcgcttgtcaaatgctgaattcctgtaacatcttcaacatgatcatcatttatatcttggtgaatgcaaacagcagattttccagtttgccccaagttttcatcaatgggctttacttcttcagtgcttctgccattcagggaagaactggcatgaatgtcattctgtatatcctgaacaaagccatctttatcatagccattagtgacaatgacttccaaattcttatggtctgctgacttcttcatcattttcttatcattatcactttgttctgctcctttcacttcttcttgggcctcttcttcctcagactcggctccactgtcactgctttcagctttaccattaacggttttggcgtttggagtagaagtgagaacattaccaagatctgaggttatatcagaactcctgccactctttttgtcctcgacaatttcataaaatggacctatgacacgcagcaattcttcaactttctcagtcattggcatagtttcaataatctttttcatttcttcaacatatgcaatcatggcttcctctttggtcatatcacccagtgaactccaagcatcccatttatatcttccaataggatcccaaaatccaggccttgaaagtttacagggtccttcagttgcctgcttatagaagctataaaatttaagcatcatttcatttgttggctggaatgaaccattcttcggcaaactctggatcaccttcacggccgcctcaaacctagtctcgtgcacggatctcgtgtccgccatctccagctgccagtgttggccccggtcccaaggtctgtcggcgggaatcaggcagcagcagcaccagctttcccaagagccgagaggaagagcatgtctagcagaagacagagggggtccgggcatcggtggccgcggagccgctctcccaccctggggaccctggcggagcagccacaccccccattccgccggagtccgtctgtcagtccgtgccctccccaca

SEQ ID NO: 13518 - RNA, 2095 nt, Homo sapiens
  source 1..2095: mol_type = other RNA
gctgggattacaggcatgagccaccacgcctggcccagtttgtttactcactgatttaaccaatcctatagagtgccttctaggagctaggtgatattgcttcaggccctgggaataccctagggatgatctagactcagatccctgtcctcgtggaacttacattctagtggaaagagagacagtgaacagttacagacacaacataatgtcatgtagtggtaaatactaggaagaaaaataaagcagggtgagaggatatgaagtgatggcacgagacttctttttagacagtgtggtcaggaggacctctgtgaagaggggcatttgagcagaaaccttctccttctttgatagtataaatacaccaaccactgtgcaataaaaggccatatgatggcaaacgttagcacaccaggagacatctcgaagggccaccaagatggtctctgtgaggtgggctgaggagcagtctgcaatgttgatgttgatgattttgcctgcaaagcagtcagcgtttccagtttctgcagtctctgaaggacattctgcatgtcctcctgcagtctcatcagcacgagggcgatctgctcattgaggctgcctcgggaccctctgtcggagccccagcgctccccatcacctccacttcccacctgccggcccttggttccttcgctcaagtgttgcatcctatgtcctcttcctcttctaacattagagaattcgtcagtttctccgcctcgcttctcccggtgtggtgctccgctgttattcctgccatcttctcctccatgcttgacttcaccttttccttcaactgcaaccacctgcatattcccaatgttgccatttccaggaggtacttgaatatcttcacgaaatccagaattttccatgggttgactggaatgaccacccaagtaatactgaaatggtccattgttggacgtaaagctgtctaaagactcttcttgtccaaattgttccatagaatcacagtaaacttcactgtctgaatcgcttgtcaaatgctgaattcctgtaacatcttcaacatgatcatcatttatatcttggtgaatgcaaacagcagattttccagtttgccccaagttttcatcaatgggctttacttcttcagtgcttctgccattcagggaagaactggcatgaatgtcattctgtatatcctgaacaaagccatctttatcatagccattagtgacaatgacttccaaattcttatggtctgctgacttcttcatcattttcttatcattatcactttgttctgctcctttcacttcttcttgggcctcttcttcctcagactcggctccactgtcactgctttcagctttaccattaacggttttggcgtttggagtagaagtgagaacattaccaagatctgaggttatatcagaactcctgccactctttttgtcctcgacaatttcataaaatggacctatgacacgcagcaattcttcaactttctcagtcattggcatagtttcaataatctttttcatttcttcaacatatgcaatcatggcttcctctttggtcatatcacccagtgaactccaagcatcccatttatatcttccaataggatcccaaaatccaggccttgaaagtttacagggtccttcagttgcctgcttatagaagctataaaatttaagcatcatttcatttgttggctggaatgaaccattcttcggcaaactctggatcaccttcacggccgcctcaaacctagtctcgtgcacggatctcgtgtccgccatctccagctgccagtgttggccccggtcccaaggtctgtcggcgggaatcaggcagcagcagcaccagctttcccaagagcctgcatgaaacgagaggaagagcatgtctagcagaagacagagggggtccgggcatcggtggccgcggagccgctctcccaccctggggaccctggcggagcagccacaccccccattccgccggagtccgtctgtcagtccgtgccctccccacagccccgccccagagtcaccggaggacccactggcgccgccgccgccgcagcagcagtgca

SEQ ID NO: 13519 - RNA, 1962 nt, Homo sapiens
  source 1..1962: mol_type = other RNA
gctgggattacaggcatgagccaccacgcctggcccagtttgtttactcactgatttaaccaatcctatagagtgccttctaggagctaggtgatattgcttcaggccctgggaataccctagggatgatctagactcagatccctgtcctcgtggaacttacattctagtggaaagagagacagtgaacagttacagacacaacataatgtcatgtagtggtaaatactaggaagaaaaataaagcagggtgagaggatatgaagtgatggcacgagacttctttttagacagtgtggtcaggaggacctctgtgaagaggggcatttgagcagaaaccttctccttctttgatagtataaatacaccaaccactgtgcaataaaaggccatatgatggcaaacgttagcacaccaggagacatctcgaagggccaccaagatggtctctgtgaggtgggctgaggagcagtctgcaatgttgatgttgatgattttgcctgcaaagcagtcagcgtttccagtttctgcagtctctgaaggacattctgcatgtcctcctgcagtctcatcagcacgagggcgatctgctcattgaggctgcctcgggaccctctgtcggagccccagcgctccccatcacctccacttcccacctgccggcccttggttccttcgctcaagtgttgcatcctatgtcctcttcctcttctaacattagagaattcgtcagtttctccgcctcgcttctcccggtgtggtgctccgctgttattcctgccatcttctcctccatgcttgacttcaccttttccttcaactgcaaccacctgcatattcccaatgttgccatttccaggaggtacttgaatatcttcacgaaatccagaattttccatgggttgactggaatgaccacccaagtaatactgaaatggtccattgttggacgtaaagctgtctaaagactcttcttgtccaaattgttccatagaatcacagtaaacttcactgtctgaatcgcttgtcaaatgctgaattcctgtaacatcttcaacatgatcatcatttatatcttggtgaatgcaaacagcagattttccagtttgccccaagttttcatcaatgggctttacttcttcagtgcttctgccattcagggaagaactggcatgaatgtcattctgtatatcctgaacaaagccatctttatcatagccattagtgacaatgacttccaaattcttatggtctgctgacttcttcatcattttcttatcattatcactttgttctgctcctttcacttcttcttgggcctcttcttcctcagactcggctccactgtcactgctttcagctttaccattaacggttttggcgtttggagtagaagtgagaacattaccaagatctgaggttatatcagaactcctgccactctttttgtcctcgacaatttcataaaatggacctatgacacgcagcaattcttcaactttctcagtcattggcatagtttcaataatctttttcatttcttcaacatatgcaatcatggcttcctctttggtcatatcacccagtgaactccaagcatcccatttatatcttccaataggatcccaaaatccaggccttgaaagtttacagggtccttcagttgcctgcttatagaagctataaaatttaagcatcatttcatttgttggctggaatgaaccattcttcggcaaactctggatcaccttcacggccgcctcaaacctagtctcgtgcacggatctcgtgtccgccatctccagctgccagtgttggccccggtcccaaggtctgtcggcgggaatcaggcagcagcagcaccagctttcccaagagcctgcatgaaacttggtattgccggacaaggcctgtccggtaatgtccccgacgcccgcccctcgccctgccccgcgggcttat

SEQ ID NO: 13520 - RNA, 3363 nt, Homo sapiens
  source 1..3363: mol_type = other RNA
gctgggattacaggcatgagccaccacgcctggcccagtttgtttactcactgatttaaccaatcctatagagtgccttctaggagctaggtgatattgcttcaggccctgggaataccctagggatgatctagactcagatccctgtcctcgtggaacttacattctagtggaaagagagacagtgaacagttacagacacaacataatgtcatgtagtggtaaatactaggaagaaaaataaagcagggtgagaggatatgaagtgatggcacgagacttctttttagacagtgtggtcaggaggacctctgtgaagaggggcatttgagcagaaaccttctccttctttgatagtataaatacaccaaccactgtgcaataaaaggccatatgatggcaaacgttagcacaccaggagacatctcgaagggccaccaagatggtctctgtgaggtgggctgaggagcagtctgcaatgttgatgttgatgattttgcctgcaaagcagtcagcgtttccagtttctgcagtctctgaaggacattctgcatgtcctcctgcagtctcatcagcacgagggcgatctgctcattgaggctgcctcgggaccctctgtcggagccccagcgctccccatcacctccacttcccacctgccggcccttggttccttcgctcaagtgttgcatcctatgtcctcttcctcttctaacattagagaattcgtcagtttctccgcctcgcttctcccggtgtggtgctccgctgttattcctgccatcttctcctccatgcttgacttcaccttttccttcaactgcaaccacctgcatattcccaatgttgccatttccaggaggtacttgaatatcttcacgaaatccagaattttccatgggttgactggaatgaccacccaagtaatactgaaatggtccattgttggacgtaaagctgtctaaagactcttcttgtccaaattgttccatagaatcacagtaaacttcactgtctgaatcgcttgtcaaatgctgaattcctgtaacatcttcaacatgatcatcatttatatcttggtgaatgcaaacagcagattttccagtttgccccaagttttcatcaatgggctttacttcttcagtgcttctgccattcagggaagaactggcatgaatgtcattctgtatatcctgaacaaagccatctttatcatagccattagtgacaatgacttccaaattcttatggtctgctgacttcttcatcattttcttatcattatcactttgttctgctcctttcacttcttcttgggcctcttcttcctcagactcggctccactgtcactgctttcagctttaccattaacggttttggcgtttggagtagaagtgagaacattaccaagatctgaggttatatcagaactcctgccactctttttgtcctcgacaatttcataaaatggacctatgacacgcagcaattcttcaactttctcagtcattggcatagtttcaataatctttttcatttcttcaacatatgcaatcatggcttcctctttggtcatatcacccagtgaactccaagcatcccatttatatcttccaataggatcccaaaatccaggccttgaaagtttacagggtccttcagttgcctgcttatagaagctataaaatttaagcatcatttcatttgttggctggaatgaaccattcttcggcaaactctggatcaccttcacggccgcctcaaacctagtctcgtgcacggatctcgtgtccgccatctccagctgccagtgttggccccggtcccaaggtctgtcggcgggaatcaggcagcagcagcaccagctttcccaagagccttggtattgccggacaaggcctgtccggtaatgtccccgacgcccgcccctcgccctgccccgcgggcttatgggaaatgtagtccgccgttccgccgcgcttccggacacgtcccagcggcgtccggcgttcctgctagctcttccggttaggcgtctctgtcccgcggacgccgcagccgtgcggcggaatccctccttcctagccggttgcatttcgtgcctctttgaaatgccacattcgcttccagcttaagtgtcttgagattgtcgcggtgtctgcagctgcggcttctccagcgccctccggaggctttgcttcgggtttgtctaatacaacacagggggaaatcatttgatcgtggacgtttcacgtttctttgtcttcaaaaatgaagaggacattttgtaaaattatcacacaaagatgagaaatagattagagaaccaactttgggttgtaaatactaaagaattccaaatggtaatgtatgaatggctaaaaagcagtgacacttatctaacgcgttattactttattccataaaaggaacaaacctaaattgaaggaatattcatttcccccttattggatttaatagaacccttttcatttttaatgggaaataatcaatgtgacctatagatgtttcaattttttttttaaataaataaacctctttagggtgatttctggtgggattgaggaaaatgaacgggtttagggttatcttggcccaaagtctatcttggatttgccgctagttcactgtgtgactgcgtcaggaaacaagctctgaaaaatttcgttttctccaataaagtatgtgaaattacctagcatgtagtagccttcaagatttttgtatttcctcttttttgatacttagctgagcaataaatattggacagcagcaccagggaagaatctgaatcaggcagggaggatgagcactgcccaggaggaaaaagcgaaaaggaaagtgtgctgagcaggtgccttggcgggggagagaggaaaaggaaatgacttcacacacacacacacacacacgcgcacacacacacagagagaatgaagtttctttctgtctcttaagtgatgtgtgagtggatggacagattgccctcagctttaagggcagttcaggatgatctgtcttaagatcgatgctctgtggaatgagaaaaatgcgctctgcagggcatgcccactgcatgtgctgggaggctctcctacatccaatgggcagatgcgcagtctccacggaggcctcaggcctcggtgtgagccagggctgcttcaaacatgtcggctatctaaagtaagtcccagcaggggtcatttatttaaggaccgtggtgctttccatggctgatttgctggtaaatgacaggtgtgagtgtagtgaacatgtcttgcctccacctacttcacccaccatcctgtgcatcatggaaacctgtctcgatgatcagcagc

SEQ ID NO: 13521 - RNA, 1892 nt, Homo sapiens
  source 1..1892: mol_type = other RNA
gctgggattacaggcatgagccaccacgcctggcccagtttgtttactcactgatttaaccaatcctatagagtgccttctaggagctaggtgatattgcttcaggccctgggaataccctagggatgatctagactcagatccctgtcctcgtggaacttacattctagtggaaagagagacagtgaacagttacagacacaacataatgtcatgtagtggtaaatactaggaagaaaaataaagcagggtgagaggatatgaagtgatggcacgagacttctttttagacagtgtggtcaggaggacctctgtgaagaggggcatttgagcagaaaccttctccttctttgatagtataaatacaccaaccactgtgcaataaaaggccatatgatggcaaacgttagcacaccaggagacatctcgaagggccaccaagatggtctctgtgaggtgggctgaggagcagtctgcaatgttgatgttgatgattttgcctgcaaagcagtcagcgtttccagtttctgcagtctctgaaggacattctgcatgtcctcctgcagtctcatcagcacgagggcgatctgctcattgaggctgcctcgggaccctctgtcggagccccagcgctccccatcacctccacttcccacctgccggcccttggttccttcgctcaagtgttgcatcctatgtcctcttcctcttctaacattagagaattcgtcagtttctccgcctcgcttctcccggtgtggtgctccgctgttattcctgccatcttctcctccatgcttgacttcaccttttccttcaactgcaaccacctgcatattcccaatgttgccatttccaggaggtacttgaatatcttcacgaaatccagaattttccatgggttgactggaatgaccacccaagtaatactgaaatggtccattgttggacgtaaagctgtctaaagactcttcttgtccaaattgttccatagaatcacagtaaacttcactgtctgaatcgcttgtcaaatgctgaattcctgtaacatcttcaacatgatcatcatttatatcttggtgaatgcaaacagcagattttccagtttgccccaagttttcatcaatgggctttacttcttcagtgcttctgccattcagggaagaactggcatgaatgtcattctgtatatcctgaacaaagccatctttatcatagccattagtgacaatgacttccaaattcttatggtctgctgacttcttcatcattttcttatcattatcactttgttctgctcctttcacttcttcttgggcctcttcttcctcagactcggctccactgtcactgctttcagctttaccattaacggttttggcgtttggagtagaagtgagaacattaccaagatcttctaaacatttagagattttctccagtcggactgaggttatatcagaactcctgccactctttttgtcctcgacaatttcataaaatggacctatgacacgcagcaattcttcaactttctcagtcattggcatagtttcaataatctttttcatttcttcaacatatgcaatcatggcttcctctttggtcatatcacccagtgaactccaagcatcccattcttcggcaaactctggatcaccttcacggccgcctcaaacctagtctcgtgcacggatctcgtgtccgccatctccagctgccagtgttggccccggtcccaaggtctgtcggcgggaatcaggcagcagcagcaccagctttcccaagagccgagaggaagagcatgtctagcagaagacagagggggtccgggcatcggtggccgcggagccgctctcccaccctggggaccctggcggagcagccacacc

SEQ ID NO: 13522 - RNA, 1912 nt, Homo sapiens
  source 1..1912: mol_type = other RNA
gctgggattacaggcatgagccaccacgcctggcccagtttgtttactcactgatttaaccaatcctatagagtgccttctaggagctaggtgatattgcttcaggccctgggaataccctagggatgatctagactcagatccctgtcctcgtggaacttacattctagtggaaagagagacagtgaacagttacagacacaacataatgtcatgtagtggtaaatactaggaagaaaaataaagcagggtgagaggatatgaagtgatggcacgagacttctttttagacagtgtggtcaggaggacctctgtgaagaggggcatttgagcagaaaccttctccttctttgatagtataaatacaccaaccactgtgcaataaaaggccatatgatggcaaacgttagcacaccaggagacatctcgaagggccaccaagatggtctctgtgaggtgggctgaggagcagtctgcaatgttgatgttgatgattttgcctgcaaagcagtcagcgtttccagtttctgcagtctctgaaggacattctgcatgtcctcctgcagtctcatcagcacgagggcgatctgctcattgaggctgcctcgggaccctctgtcggagccccagcgctccccatcacctccacttcccacctgccggcccttggttccttcgctcaagtgttgcatcctatgtcctcttcctcttctaacattagagaattcgtcagtttctccgcctcgcttctcccggtgtggtgctccgctgttattcctgccatcttctcctccatgcttgacttcaccttttccttcaactgcaaccacctgcatattcccaatgttgccatttccaggaggtacttgaatatcttcacgaaatccagaattttccatgggttgactggaatgaccacccaagtaatactgaaatggtccattgttggacgtaaagctgtctaaagactcttcttgtccaaattgttccatagaatcacagtaaacttcactgtctgaatcgcttgtcaaatgctgaattcctgtaacatcttcaacatgatcatcatttatatcttggtgaatgcaaacagcagattttccagtttgccccaagttttcatcaatgggctttacttcttcagtgcttctgccattcagggaagaactggcatgaatgtcattctgtatatcctgaacaaagccatctttatcatagccattagtgacaatgacttccaaattcttatggtctgctgacttcttcatcattttcttatcattatcactttgttctgctcctttcacttcttcttgggcctcttcttcctcagactcggctccactgtcactgctttcagctttaccattaacggttttggcgtttggagtagaagtgagaacattaccaagatcttctaaacatttagagattttctccagtcggactgaggttatatcagaactcctgccactctttttgtcctcgacaatttcataaaatggacctatgacacgcagcaattcttcaactttctcagtcattggcatagtttcaataatctttttcatttcttcaacatatgcaatcatggcttcctctttggtcatatcacccagtgaactccaagcatcccattcttcggcaaactctggatcaccttcacggccgcctcaaacctagtctcgtgcacggatctcgtgtccgccatctccagctgccagtgttggccccggtcccaaggtctgtcggcgggaatcaggcagcagcagcaccagctttcccaagagcctgcatgaaacgagaggaagagcatgtctagcagaagacagagggggtccgggcatcggtggccgcggagccgctctcccaccctggggaccctggcggagcagccacaccccccattccg

SEQ ID NO: 13523 - RNA, 2058 nt, Homo sapiens
  source 1..2058: mol_type = other RNA
gctgggattacaggcatgagccaccacgcctggcccagtttgtttactcactgatttaaccaatcctatagagtgccttctaggagctaggtgatattgcttcaggccctgggaataccctagggatgatctagactcagatccctgtcctcgtggaacttacattctagtggaaagagagacagtgaacagttacagacacaacataatgtcatgtagtggtaaatactaggaagaaaaataaagcagggtgagaggatatgaagtgatggcacgagacttctttttagacagtgtggtcaggaggacctctgtgaagaggggcatttgagcagaaaccttctccttctttgatagtataaatacaccaaccactgtgcaataaaaggccatatgatggcaaacgttagcacaccaggagacatctcgaagggccaccaagatggtctctgtgaggtgggctgaggagcagtctgcaatgttgatgttgatgattttgcctgcaaagcagtcagcgtttccagtttctgcagtctctgaaggacattctgcatgtcctcctgcagtctcatcagcacgagggcgatctgctcattgaggctgcctcgggaccctctgtcggagccccagcgctccccatcacctccacttcccacctgccggcccttggttccttcgctcaagtgttgcatcctatgtcctcttcctcttctaacattagagaattcgtcagtttctccgcctcgcttctcccggtgtggtgctccgctgttattcctgccatcttctcctccatgcttgacttcaccttttccttcaactgcaaccacctgcatattcccaatgttgccatttccaggaggtacttgaatatcttcacgaaatccagaattttccatgggttgactggaatgaccacccaagtaatactgaaatggtccattgttggacgtaaagctgtctaaagactcttcttgtccaaattgttccatagaatcacagtaaacttcactgtctgaatcgcttgtcaaatgctgaattcctgtaacatcttcaacatgatcatcatttatatcttggtgaatgcaaacagcagattttccagtttgccccaagttttcatcaatgggctttacttcttcagtgcttctgccattcagggaagaactggcatgaatgtcattctgtatatcctgaacaaagccatctttatcatagccattagtgacaatgacttccaaattcttatggtctgctgacttcttcatcattttcttatcattatcactttgttctgctcctttcacttcttcttgggcctcttcttcctcagactcggctccactgtcactgctttcagctttaccattaacggttttggcgtttggagtagaagtgagaacattaccaagatcttctaaacatttagagattttctccagtcggactgaggttatatcagaactcctgccactctttttgtcctcgacaatttcataaaatggacctatgacacgcagcaattcttcaactttctcagtcattggcatagtttcaataatctttttcatttcttcaacatatgcaatcatggcttcctctttggtcatatcacccagtgaactccaagcatcccatttatatcttccaataggatcccaaaatccaggccttgaaagtttacagggtccttcagttgcctgcttatagaagctataaaatttaagcatcatttcatttgttggctggaatgaaccattcttcggcaaactctggatcaccttcacggccgcctcaaacctagtctcgtgcacggatctcgtgtccgccatctccagctgccagtgttggccccggtcccaaggtctgtcggcgggaatcaggcagcagcagcaccagctttcccaagagccgagaggaagagcatgtctagcagaagacagagggggtccgggcatcggtggccgcggagccgctctcccaccctggggaccctggcggagcagccacaccccccattccgccggagtccgtctgtcagtccgtgccctccccaca

SEQ ID NO: 13524 - RNA, 2022 nt, Homo sapiens
  source 1..2022: mol_type = other RNA
gctgggattacaggcatgagccaccacgcctggcccagtttgtttactcactgatttaaccaatcctatagagtgccttctaggagctaggtgatattgcttcaggccctgggaataccctagggatgatctagactcagatccctgtcctcgtggaacttacattctagtggaaagagagacagtgaacagttacagacacaacataatgtcatgtagtggtaaatactaggaagaaaaataaagcagggtgagaggatatgaagtgatggcacgagacttctttttagacagtgtggtcaggaggacctctgtgaagaggggcatttgagcagaaaccttctccttctttgatagtataaatacaccaaccactgtgcaataaaaggccatatgatggcaaacgttagcacaccaggagacatctcgaagggccaccaagatggtctctgtgaggtgggctgaggagcagtctgcaatgttgatgttgatgattttgcctgcaaagcagtcagcgtttccagtttctgcagtctctgaaggacattctgcatgtcctcctgcagtctcatcagcacgagggcgatctgctcattgaggctgcctcgggaccctctgtcggagccccagcgctccccatcacctccacttcccacctgccggcccttggttccttcgctcaagtgttgcatcctatgtcctcttcctcttctaacattagagaattcgtcagtttctccgcctcgcttctcccggtgtggtgctccgctgttattcctgccatcttctcctccatgcttgacttcaccttttccttcaactgcaaccacctgcatattcccaatgttgccatttccaggaggtacttgaatatcttcacgaaatccagaattttccatgggttgactggaatgaccacccaagtaatactgaaatggtccattgttggacgtaaagctgtctaaagactcttcttgtccaaattgttccatagaatcacagtaaacttcactgtctgaatcgcttgtcaaatgctgaattcctgtaacatcttcaacatgatcatcatttatatcttggtgaatgcaaacagcagattttccagtttgccccaagttttcatcaatgggctttacttcttcagtgcttctgccattcagggaagaactggcatgaatgtcattctgtatatcctgaacaaagccatctttatcatagccattagtgacaatgacttccaaattcttatggtctgctgacttcttcatcattttcttatcattatcactttgttctgctcctttcacttcttcttgggcctcttcttcctcagactcggctccactgtcactgctttcagctttaccattaacggttttggcgtttggagtagaagtgagaacattaccaagatcttctaaacatttagagattttctccagtcggactgaggttatatcagaactcctgccactctttttgtcctcgacaatttcataaaatggacctatgacacgcagcaattcttcaactttctcagtcattggcatagtttcaataatctttttcatttcttcaacatatgcaatcatggcttcctctttggtcatatcacccagtgaactccaagcatcccatttatatcttccaataggatcccaaaatccaggccttgaaagtttacagggtccttcagttgcctgcttatagaagctataaaatttaagcatcatttcatttgttggctggaatgaaccattcttcggcaaactctggatcaccttcacggccgcctcaaacctagtctcgtgcacggatctcgtgtccgccatctccagctgccagtgttggccccggtcccaaggtctgtcggcgggaatcaggcagcagcagcaccagctttcccaagagcctgcatgaaacgagaggaagagcatgtctagcagaagacagagggggtccgggcatcggtggccgcggagccgctctcccaccctggggaccctggcggagcagccacac

SEQ ID NO: 13525 - RNA, 1995 nt, Homo sapiens
  source 1..1995: mol_type = other RNA
gctgggattacaggcatgagccaccacgcctggcccagtttgtttactcactgatttaaccaatcctatagagtgccttctaggagctaggtgatattgcttcaggccctgggaataccctagggatgatctagactcagatccctgtcctcgtggaacttacattctagtggaaagagagacagtgaacagttacagacacaacataatgtcatgtagtggtaaatactaggaagaaaaataaagcagggtgagaggatatgaagtgatggcacgagacttctttttagacagtgtggtcaggaggacctctgtgaagaggggcatttgagcagaaaccttctccttctttgatagtataaatacaccaaccactgtgcaataaaaggccatatgatggcaaacgttagcacaccaggagacatctcgaagggccaccaagatggtctctgtgaggtgggctgaggagcagtctgcaatgttgatgttgatgattttgcctgcaaagcagtcagcgtttccagtttctgcagtctctgaaggacattctgcatgtcctcctgcagtctcatcagcacgagggcgatctgctcattgaggctgcctcgggaccctctgtcggagccccagcgctccccatcacctccacttcccacctgccggcccttggttccttcgctcaagtgttgcatcctatgtcctcttcctcttctaacattagagaattcgtcagtttctccgcctcgcttctcccggtgtggtgctccgctgttattcctgccatcttctcctccatgcttgacttcaccttttccttcaactgcaaccacctgcatattcccaatgttgccatttccaggaggtacttgaatatcttcacgaaatccagaattttccatgggttgactggaatgaccacccaagtaatactgaaatggtccattgttggacgtaaagctgtctaaagactcttcttgtccaaattgttccatagaatcacagtaaacttcactgtctgaatcgcttgtcaaatgctgaattcctgtaacatcttcaacatgatcatcatttatatcttggtgaatgcaaacagcagattttccagtttgccccaagttttcatcaatgggctttacttcttcagtgcttctgccattcagggaagaactggcatgaatgtcattctgtatatcctgaacaaagccatctttatcatagccattagtgacaatgacttccaaattcttatggtctgctgacttcttcatcattttcttatcattatcactttgttctgctcctttcacttcttcttgggcctcttcttcctcagactcggctccactgtcactgctttcagctttaccattaacggttttggcgtttggagtagaagtgagaacattaccaagatcttctaaacatttagagattttctccagtcggactgaggttatatcagaactcctgccactctttttgtcctcgacaatttcataaaatggacctatgacacgcagcaattcttcaactttctcagtcattggcatagtttcaataatctttttcatttcttcaacatatgcaatcatggcttcctctttggtcatatcacccagtgaactccaagcatcccatttatatcttccaataggatcccaaaatccaggccttgaaagtttacagggtccttcagttgcctgcttatagaagctataaaatttaagcatcatttcatttgttggctggaatgaaccattcttcggcaaactctggatcaccttcacggccgcctcaaacctagtctcgtgcacggatctcgtgtccgccatctccagctgccagtgttggccccggtcccaaggtctgtcggcgggaatcaggcagcagcagcaccagctttcccaagagcctgcatgaaacttggtattgccggacaaggcctgtccggtaatgtccccgacgcccgcccctcgccctgccccgcgggcttat

SEQ ID NO: 13526 - RNA, 3396 nt, Homo sapiens
  source 1..3396: mol_type = other RNA
gctgggattacaggcatgagccaccacgcctggcccagtttgtttactcactgatttaaccaatcctatagagtgccttctaggagctaggtgatattgcttcaggccctgggaataccctagggatgatctagactcagatccctgtcctcgtggaacttacattctagtggaaagagagacagtgaacagttacagacacaacataatgtcatgtagtggtaaatactaggaagaaaaataaagcagggtgagaggatatgaagtgatggcacgagacttctttttagacagtgtggtcaggaggacctctgtgaagaggggcatttgagcagaaaccttctccttctttgatagtataaatacaccaaccactgtgcaataaaaggccatatgatggcaaacgttagcacaccaggagacatctcgaagggccaccaagatggtctctgtgaggtgggctgaggagcagtctgcaatgttgatgttgatgattttgcctgcaaagcagtcagcgtttccagtttctgcagtctctgaaggacattctgcatgtcctcctgcagtctcatcagcacgagggcgatctgctcattgaggctgcctcgggaccctctgtcggagccccagcgctccccatcacctccacttcccacctgccggcccttggttccttcgctcaagtgttgcatcctatgtcctcttcctcttctaacattagagaattcgtcagtttctccgcctcgcttctcccggtgtggtgctccgctgttattcctgccatcttctcctccatgcttgacttcaccttttccttcaactgcaaccacctgcatattcccaatgttgccatttccaggaggtacttgaatatcttcacgaaatccagaattttccatgggttgactggaatgaccacccaagtaatactgaaatggtccattgttggacgtaaagctgtctaaagactcttcttgtccaaattgttccatagaatcacagtaaacttcactgtctgaatcgcttgtcaaatgctgaattcctgtaacatcttcaacatgatcatcatttatatcttggtgaatgcaaacagcagattttccagtttgccccaagttttcatcaatgggctttacttcttcagtgcttctgccattcagggaagaactggcatgaatgtcattctgtatatcctgaacaaagccatctttatcatagccattagtgacaatgacttccaaattcttatggtctgctgacttcttcatcattttcttatcattatcactttgttctgctcctttcacttcttcttgggcctcttcttcctcagactcggctccactgtcactgctttcagctttaccattaacggttttggcgtttggagtagaagtgagaacattaccaagatcttctaaacatttagagattttctccagtcggactgaggttatatcagaactcctgccactctttttgtcctcgacaatttcataaaatggacctatgacacgcagcaattcttcaactttctcagtcattggcatagtttcaataatctttttcatttcttcaacatatgcaatcatggcttcctctttggtcatatcacccagtgaactccaagcatcccatttatatcttccaataggatcccaaaatccaggccttgaaagtttacagggtccttcagttgcctgcttatagaagctataaaatttaagcatcatttcatttgttggctggaatgaaccattcttcggcaaactctggatcaccttcacggccgcctcaaacctagtctcgtgcacggatctcgtgtccgccatctccagctgccagtgttggccccggtcccaaggtctgtcggcgggaatcaggcagcagcagcaccagctttcccaagagccttggtattgccggacaaggcctgtccggtaatgtccccgacgcccgcccctcgccctgccccgcgggcttatgggaaatgtagtccgccgttccgccgcgcttccggacacgtcccagcggcgtccggcgttcctgctagctcttccggttaggcgtctctgtcccgcggacgccgcagccgtgcggcggaatccctccttcctagccggttgcatttcgtgcctctttgaaatgccacattcgcttccagcttaagtgtcttgagattgtcgcggtgtctgcagctgcggcttctccagcgccctccggaggctttgcttcgggtttgtctaatacaacacagggggaaatcatttgatcgtggacgtttcacgtttctttgtcttcaaaaatgaagaggacattttgtaaaattatcacacaaagatgagaaatagattagagaaccaactttgggttgtaaatactaaagaattccaaatggtaatgtatgaatggctaaaaagcagtgacacttatctaacgcgttattactttattccataaaaggaacaaacctaaattgaaggaatattcatttcccccttattggatttaatagaacccttttcatttttaatgggaaataatcaatgtgacctatagatgtttcaattttttttttaaataaataaacctctttagggtgatttctggtgggattgaggaaaatgaacgggtttagggttatcttggcccaaagtctatcttggatttgccgctagttcactgtgtgactgcgtcaggaaacaagctctgaaaaatttcgttttctccaataaagtatgtgaaattacctagcatgtagtagccttcaagatttttgtatttcctcttttttgatacttagctgagcaataaatattggacagcagcaccagggaagaatctgaatcaggcagggaggatgagcactgcccaggaggaaaaagcgaaaaggaaagtgtgctgagcaggtgccttggcgggggagagaggaaaaggaaatgacttcacacacacacacacacacacgcgcacacacacacagagagaatgaagtttctttctgtctcttaagtgatgtgtgagtggatggacagattgccctcagctttaagggcagttcaggatgatctgtcttaagatcgatgctctgtggaatgagaaaaatgcgctctgcagggcatgcccactgcatgtgctgggaggctctcctacatccaatgggcagatgcgcagtctccacggaggcctcaggcctcggtgtgagccagggctgcttcaaacatgtcggctatctaaagtaagtcccagcaggggtcatttatttaaggaccgtggtgctttccatggctgatttgctggtaaatgacaggtgtgagtgtagtgaacatgtcttgcctccacctacttcacccaccatcctgtgcatcatggaaacctgtctcgatgatcagcagc

SEQ ID NO: 13527 - RNA, 2954 nt, Homo sapiens
  source 1..2954: mol_type = other RNA
gctgggattacaggcatgagccaccacgcctggccccaaactgactcttgaccaaagaatctgatttggcaaaccaaatcttagtgcagtgttcgctcctcgtccccttacccagaacatgattcagatcctaacataaacacaaaaacaggtcagggaaccaaaacactgtggtcttgtctattatacaaaatattgagataatgttcacgattcattctgttttcagcaattgtgacaattttgaagcttctctcgaagcttcgaaacacttcatttcctactaaataccaaaacgtgtcagacaggcatcaccagtgggaacttggttttgttttgtttttttttttgagatggagtctcgctctgttacccaggctggagtgcacaatctcggctcaccacaacttctgcctcccaggttcaagcaattcgcctgcctcagcagcctgaggagctgggactacaggcacgcgacaccatgcccggctaatttctgtatttttagtagagatggggtttcactatgttggccaggctggtctcgaactcctgacctcgtgatccgcccatcttggcctcccaaagtgctgggattacaggtgtgagccactgtgcctggccggggaactttgtttttaaacgtttacaaacaaaaagattttcgatgcataggccagtcctaatgcatcccataatggggaccaaggcaaaaacacacacacacaactacaaaatattccctagaaaaatgcaagatcctccgaaaatcaagatctctctaccaaacaacataccaagtcatcacagaagaggtgaagatgcctctcaaaagacatgtgccacagaaatagagcttgaaatactgaacacgatttctcgaagatccttctcaccaccccaagagaagcgccctgctctggtgagggaagaggaggcaaaggagaagagagaagtttcccttccatctggatctgggtggatgccaaccctgacgtgcagggcagagcaccaggctgcaggaactggatgctaattgcaatcgctttttgctttggaacatttgccaggaacttgtgaactgctaaggggatgaccaggaaactggatccatctctgtggctggggatgttttgaatgattctcgcgggctccctgtctgcttggtgaccctgttggtcctatgcgtatctgcgccagggaattaaactagccagtctgacgttctcaagcaccgccctggacacccccactgccagttcatggtctacagccacagtgaccccagcttttcacacaggtcctgaatgttatctggaatgcagacacaagtgctctgagctacactgcttggggaataattccacatggaaaggtacaacgtggccaagatctccgcagggacacggccctcagatgacagactccaggaagaaagagcatgagacactggtctctgtttaggtttgcccagagctcacggccgtctgcactgcaggcaacgcatcctcctgcggctcacggggggccaggaaccccagggcttctgatggagagttatgcaccgtcccctcggctgggttgtacattcactgattgtcagaagtttctgatactgctgtgggggccggggaaggagtcaccaacagtctggtcctgtcctttggactctacacatcatagcggttcaaactgtacgagtttgggtagctctgccggctgtattggaagtggtctgttaagatgttgttgcggccgtactgatagtccccgtgctgggggaagaggaggccgttgtggggcttctccagtgggctccggtgacgctccttgctgctcaggtctgctgtggtgacggggaggaggtgcttcctggcttgctggtttgcatcgtacttggtcttgttatagaggaagacccccaggatggcggtcatcatgcccaggacgttggtgctggtgactgggttgcgcagcatgatcagggacaccgtgatgaccatgattcttttggtggcattggcgaccgagtagctcagggggctaacgaggttgaggatgctgaaggcgataacattctgggcaaagttacagaagccgctgacagccaggagcaggagcgtccagggccactggtagacgtaggtcaagtcgctgctgaccaggaaagccgagaggtccaccagaacccaggtggggatcataaagaagacggcgtggcagcccaggatgttgagcagccggagatggtggatccgtgaatctcgcaagacctttttggagaaaatgttctgaagcgagaagcacagcgtggcggcgagggcgctgacgagtccccacatgtcaaaagacaactcggtgacggtggccagcaggacaccgctgatgatggggatgagtgacaagtataccttggtgctctgcttctccttcataatgatccgggacaggaggaccacccagatgggcatggtggccttgacggtgtgtgcataggacacgggcaccttccagatgctgacgtgcgctgacacggacgcgaagtacttgccgaaggcgagcggtagcacgtagcgcgggtagaagcgcggcggcagcagcgggccggacgacggatgcggactgggtccggggcccgagacgggcggcgcggggggcacgcgccaggcgcgcagcagcggcgggagcccagcgcacagagccaggatgtggcacagcgacacggtcaccgggaacgggaaggcgctcaggatcaccttgttgaccacgttgccgcccgcgctcagcgcgtaccacagcaggcacagcgccgccacccgcgcgccctcgcgcgccccaccactgctgctcgctgcgcccgggccccccgcgccgtggcccgcgcccaccgcggccgccgccatcctgcccgagcggccgccccttccagcccgtccgacggcccgacgccgggc

SEQ ID NO: 13528 - RNA, 2481 nt, Homo sapiens
  source 1..2481: mol_type = other RNA
gctgggattacaggcatgagccaccacgcctggcccctcctgtatgctttctaagcatcctatatttctttgcactcagctaggctgtgccctcaggacctagttccaccccagaaacaaagaggggcactgtgaattgagaagaaatgaatgatggggcttgtgaggttcagcatttattcctcaggaggtgaccaggctggtcagaggcacctggatctggggacagctgagccctccctgctgctcaagactggcctgggcactgcagtggggccagtcctggcccctgacaactcaagctcctaggtccagtctagactccagggacctccaggccagcccaaggctctttgaagcaagaatctgagtctactaacctgccttgtccaacccaacaccccaaactcctcagctagctgcatccctggtggctacagcttcagatggctcccccatacaactcatagataacgggttctggggcctcacccctaattcattgggcccaaggataccctagtattagcctttcctaagaggaggagtttccccaactctcccgaaacatccagaatgttcccacaccttctcctcagtctttctttcctgaatttcttgggagtggaccattcctgggcactgggaaccagaagtaccaaactaccatctatctctcagtgcctctgtttacccatttgtaaaacttgggctgcatttcctgcttcttacggagttttgggggccattaatattaaagccccggatgatctctggaagacagggactctgttttcatgattttgtcctctagctgccccacaacctccctggaaccttctggaatgtgctgcacaggtcaaactagagcggggaacccaagaactggtgggggccggcaagtggatggcctggggcctgggaacattgaaccatggcagtgattttgagtgtcttttcaaagggaagtggctcaacgccactcgtcgttgaggtgggtctttgggtctcagggagtgcccagccctgggcctgcggagggcagcaggggatgggaccttcagaagtgaggggaggcctgcaggaagggcctccaggttggagtcagcctcggcaccaggcccagctgctccagctgcagccgcgtgggcctgtaggcccccaggttgctgtagacagcggcgggcgggccgtcgtggggccgcggggagaggtgggcctggggactcggggctccccaagggccttggtggggctggaaccggggcggtggaggcgggtgtggggccgcggggctacagggccctgaagacgcggacacacttcgggtaccggggtggctgcctgccgagcggccgctgaaggggttggaggacgtgcggtcactggcggagccactgctgctgctaaggcggccattggccggggctgctccgggcgggacgggggcgaccagccgcggggacttcaggcccatcacaggcttggaggaggcgtagaggtggcggaactcctcgtcaaacagctccaccgcctggcctgtgaacttggagaggatgttccggtgcacgtgtccgcagagccaggtgaagctgtaagatccagacaggacaaatctccagtccgagatgatgaacttctcccggatttggccagcgaatttcctgcctgacttggcacagtatatctctccttccacactccggatggaaatgttctggctagtccgggtgatgcagcggcggacgaggtctctgatgttgttgtgcttgacggtctggaagtacacagtggcgctggatttttccttcaggtagggcttctcagctgaggcccagctgtgcagtagggccggctcgctgccctctgaggccacagggaagtaggtgccggactgtagggagctggagtccagtcccttagggcctgcttccgcccctcccagggtgtctgggggacacgggggctccctggcctgggcctggatgtactgggcctccaccgaggacaagaagtccacctcgccttcctggctgagcacccgccagtaggcttcagaacccccatccaagagggcgtccgtggccagccgggcactctcgttgtcactaaagtcagccctggctggccggacccactggctcttgacatcttccagacgcttccggattttgcccaggtgccttgaccggctcatgcctcccgtccctgggtggtgctgggggaggctggcacgtcagctcctccagatgtgggaagcaaatggaacacaccacggaggagtggggctcccgcacccccgggaggccgcctgctcccaggaccggcgtgcagggcacctccaagaagtgatttaccgctgtcctgagcaatgcttctcagaactcctcatctgcagctgcgggattggcttatctctcagggccacctgccctgccctcgggccgggagggctggctcagacacctccttggcacagtc

SEQ ID NO: 13529 - RNA, 3294 nt, Homo sapiens
  source 1..3294: mol_type = other RNA
gctgggattacaggcatgagccaccacgcctggcccctcctgtatgctttctaagcatcctatatttctttgcactcagctaggctgtgccctcaggacctagttccaccccagaaacaaagaggggcactgtgaattgagaagaaatgaatgatggggcttgtgaggttcagcatttattcctcaggaggtgaccaggctggtcagaggcacctggatctggggacagctgagccctccctgctgctcaagactggcctgggcactgcagtggggccagtcctggcccctgacaactcaagctcctaggtccagtctagactccagggacctccaggccagcccaaggctctttgaagcaagaatctgagtctactaacctgccttgtccaacccaacaccccaaactcctcagctagctgcatccctggtggctacagcttcagatggctcccccatacaactcatagataacgggttctggggcctcacccctaattcattgggcccaaggataccctagtattagcctttcctaagaggaggagtttccccaactctcccgaaacatccagaatgttcccacaccttctcctcagtctttctttcctgaatttcttgggagtggaccattcctgggcactgggaaccagaagtaccaaactaccatctatctctcagtgcctctgtttacccatttgtaaaacttgggctgcatttcctgcttcttacggagttttgggggccattaatattaaagccccggatgatctctggaagacagggactctgttttcatgattttgtcctctagctgccccacaacctccctggaaccttctggaatgtgctgcacaggtcaaactagagcggggaacccaagaactggtgggggccggcaagtggatggcctggggcctgggaacattgaaccatggcagtgattttgagtgtcttttcaaagggaagtggctcaacgccactcgtcgttgaggtgggtctttgggtctcagggagtgcccagccctgggcctgcggagggcagcaggggatgggaccttcagaagtgaggggaggcctgcaggaagggcctccaggttggagtcagcctcggcaccaggcccagctgctccagctgcagccgcgtgggcctgtaggcccccaggttgctgtagacagcggcgggcgggccgtcgtggggccgcggggagaggtgggcctggggactcggggctccccaagggccttggtggggctggaaccggggcggtggaggcgggtgtggggccgcggggctacagggccctgaagacgcggacacacttcgggtaccggggtggctgcctgccgagcggccgctgaaggggttggaggacgtgcggtcactggcggagccactgctgctgctaaggcggccattggccggggctgctccgggcgggacgggggcgaccagccgcggggacttcaggcccatcacaggcttggaggaggcgtagaggtggcggaactcctcgtcaaacagctccaccgcctggcctgtgaacttggagaggatgttccggtgcacgtgtccgcagagccaggtgaagctgtaagatccagacaggacaaatctccagtccgagatgatgaacttctcccggatttggccagcgaatttcctgcctgacttggcacagtatatctctccttccacactccggatggaaatgttcttgaggtgactgtcagagatctggactttgtcacacatctcctggaagagcttcacacctccctggtccaggagcacacaaacgaacaccccacgcttgttggctgcctctagaatgtcacagaagatctccacatccgtgaacacatccatcaggatgaccaggacctggctagtccgggtgatgcagcggcggacgaggtctctgatgttgttgtgcttgacggtctggaagtacacagtggcgctggatttttccttcaggtagggcttctcagctgaggcccagctgtgcagtagggccggctcgctgccctctgaggccacagggaagtaggtgccggactgtagggagctggagtccagtcccttagggcctgcttccgcccctcccagggtgtctgggggacacgggggctccctggcctgggcctggatgtactgggcctccaccgaggacaagaagtccacctcgccttcctggctgagcacccgccagtaggcttcagaacccccatccaagagggcgtccgtggccagccgggcactctcgttgtcactaaagtcagccctggctggccggacccactggctcttgacatcttccagacgcttccggattttgcccaggtgccttgaccggctcatgcctcccgtccctgggtggtgctgggggaggctggcacgtcagctcctccagatgtgggaagcaaatggaacacaccacggaggagtggggctcccgcacccccgggaggccgcctgctcccaggaccggcgtgcagggcacctccaagaagtgatttaccgctgtcctgagcaatgcttctcagaactcctcatctgcagctgcgggattggcttatctctcagggccacctgccctgccctcgggccgggagggctggctcagacacctccttggcacagtcagccatgggatatttcctctcctcccagccgcagggggaggcgaaggtgagccggctttcctgctgggtttcgcaactctccctcaggcctttgttaccaagcagggagcctccctggcaccaccagcccagctggaggatgggcctgaaggaggcctgcctgcctctgctcccctcctgggtgcctcgattcccatgctgtttcaaagataagaatttccctgtgggggggaaagatgccatccctgagatgcgcccccctctctgtgtgaggagggagctggacacgggccagggagagctgttgaccaggcgcgcctcctctccttggtcacacccaagtgcccacccctccctgccctatgaaggagctcctttctcccatgccctctcaagtgtttgtcattgtcgtgtttgcagagaccgcagaggttccagttctcaggccaacgcttcctcgctggaagtggcttcttggaacactgtctggagaacgagccgaggctgccggcggcccacgagcccaggggaccagtcagtgttggcgctgagaaactgcacaaaatggtcccacatgttcattccagcatggcttctcccatacttggccatcgctgagtgctcactgcatgctggctgtctgta

SEQ ID NO: 13530 - RNA, 3049 nt, Homo sapiens
  source 1..3049: mol_type = other RNA
gctgggattacaggcatgagccaccacgcctggccctgaccacttctttctactcctctgctatactcgtccaagtcaccatcatctcttaccttgtcaactgcaacagcttccacaaacccccaccagcaagtagtagtatattaataatatagtatttctcaaggtatctgtgactgagagtcagagttttaccatctcaatctgccataatcaatacttctagaaagctgatcccacatgcgactcaccatgcaagttcaacaccccacagcaccgtttcagatgcgtactctcctgactgcttgcctctgtggctcagtgcgaatactctgcattcatgctggagtacttgagaagggcacacactctagagctacactgtctgagtgcaaatgctggcactcattcttgttacacaaatgaccttgagcaaggtgtttaacttcccttacttttatcatctataaaataattctacctaacaggattctacctaataaaaaaagaattacctaattctttttaacctaattcttttttttttttgtatcaaagaaaatattttattcaagttcccaaaacaaacttcaggagttatgctgggtttgaattgaagaaaaaaggccaagttaaaataggaaaacaaatggttttcatttggtggcagctgaaatcaaagtatacatgtatatacattctaatccatcatctatcccatgtggcattttccaaggttttaagagtctaccacgccaaaccctttgccactttcactgcttttgctttgcttttcccctttcttttctctcgctttgccgtcagcctttttctttgcctttggttcatccatattgggtactgtccatgctggtctagaagagtctttttgtttctcttagtatcagtctcccttttcatgtcatctttttcatcttttacctcacattgcattttctcttggcaatgtttgggtaccaccacagttgctatctcttgaacatctttcattaaaacatcaccgtctagtttgagaatacttttaagcctgctggcctcctttggggcattcttttttctcttttcagcacgcatctttcttttccacttactccgtaagcttttagccatgtttcacctgagaaacgaacacccacacctcagctctttttaacctaattctaattacctaataattctacttaataggattattgaaaggattaaaccagttaataagaatgatgaggctgggcatggtggctcacacctgtaatcccagcccactgggaggctgaggcaggtagattgtttgaactcagagtttgagaccagcctgggcaacatggcaaaaccccatctctactaaaaatataaaaaattagccaggtgtggtggcgtacacctgtagttccagctacctgggacgctgaggtgggaggatcacctaagcccaggaggtcgtggctgcagtgagccatgatcaatgccaatgcactccagcctgggctgcagagtaagaccctatctcaaaaaaaagtaaaataaataataataataatacctgacacatggcaaatgcaaagcatgttcatttctattgatattactatagcttactcaccctacaaaagtcataggagtgactcttttataagtgttaagtaagatcatagcaatcttgctgttcaaaatccttctactcatttaccattgtactcactgctaacagtggcctacatggtctcatgtgatctcctagtacctctcatccccacacttagttccagccacacaccagcctccttagaatccctcaagcatgcctttacaccatgcccaaaaacgtttctttccaacaccctcatctattcagttctctgctcaaactcctcagacagaccttctctgaatactccatctaaaaagacccaccactgccattcctatcccccttctctactttattctgttttacagcattcttttttttttttttgagacggagtctcactctgtcgcccaggctagagtgcagtggtgagatctcggctcactgcaagctccgcctcccgggttcacaccattttcctgcctcagcctcctgagcagctgggactataggcgcccgccaccacgcccggctaattttttgtatttttggtagagatgaggtttcaccgtgttagccaggatggtctcgatctcctgacctcatgatctgcccacctcggcctcccaaagtgctgggattacaggtgtgagccaccgcgcccggcctcttacagcattctttaccaccaggcataaaacctatgtctttctccactggaatgtatactccaagaaggcagagacttcattttgttcaccagtgcatcatcagcatatatacatgcgcctggcacatagcaggcaatcaataaatatggcaagaaagaatacctgacactgaggcagaagtacggaaaattgttgcatctccctccctgaactcccagtaagcatattctgaattaagtcgctgagactgagcatctccattcaaggacctgtgtgcttatcaccgtgcaaagtatggcaagaggaaataaggttgctctgtgtccatgagtcctcatctacctgaagtgtaagaagtcacatccctgcccagccaagctgacctgagtgcatcaagtgagaagagagacctcccaggagagctggtgggtcaccctacaatgccccactggccactgctataccaggcactgcagttactgcagtgtgacgagcagggaggaaagagcactacgacgagacccacagagtctactttatcttccttcagcaacacaggtaaaagcgattgtaatagttctcctaaatctcaaacacagttgacaaaatctctgatgtttccattaaaaatcttcaacgacaaaagagctctaccacatcaaactacccagcatctattaaaatgagagtattctggctgggcatggtagctcacgcctgctgttatcctaacactttgggaggccaaggcaggcagattgcctga

SEQ ID NO: 13531 - RNA, 2301 nt, Homo sapiens
  source 1..2301: mol_type = other RNA
gctgggattacaggcatgagccaccacgcctggcctaatctcatcgatctaacctataaaaaagagaataataacttactcacctcattggatagttatgaagataagatagagtataaagggtttggcagagcgtctgtcctatggtaaatgctcgctaactggttagctactataattttctatttgtatctattcaaatctcactgcttctgcaagtctcctaacaaaaagttttgccaaaatttattttgccattgaaagtaatggcaaaagccacaattttgcacaaaccaagaagccttctctgcttatcttccagtccaagattatctcctcttcctagtattcttattttgtgacttttatagaatcacttggttggtctgggtttatgtttaaagttcctgactacaggtgaaatactcttggagaaagagacctaaacttctagcgtaacgctgagacacatcttcatagaatagaattgttattttatgtccccaattaaagggattttatttttgtggatgttttcttgggttgagtgttctactgatttattgaatggtctactgatttctcattatgtgaaaactccagagtcctaggtgtgtttcttccaagagcctaattaattcaggctgctaaggctgccacatggactctggtttaaagactaggctatttggtgagcaattctaagtcctattttggaacactaaggtcatatacctttggaatgccaaattacaagatgctttgaaggaacttttagggtaaatcacaatctcatccgtgtgcatctgcagttaaggtttataaagagaagtttggttcctgattttcagtagcagtatcattagttttttaaaaactacaggaaattttacatgtattttgcctcacaaataccaacaattaggtcagaattcagaaaagtggattctgtttgcatagaattacattaattctgcattctctcatagcaaagttgaaagagaggattaatcacttattcatgcaaaaccaattcacatgaatcatttatttatcttgttctggtaattttgcagagctcatttttacatgcctcaggttgcagataaagtgaaaactcagagggtgatttaccctccacaataaagacctgatggccgtgtaaacagcatgcttcctataggaaatcaataggtaaccatggaaatgactccacaatgggaaattctatttctttatgaacaaatcatcaaaaagatcaattgtaagatgaaaaggctttgcctgtgccctatctttcgcaaaggcttttggtctatgtaaagaagaaaatatgtgccttggtgacagtaaagaattatcttaaagctgtattgagaatgaacatcacttgttactttataaagtttgggctgaaatgtcttgtcctccattcctggaggcctagctaagaaacttatatctaatggcaagaagaatgttccagaatacaggatgcttgaattcttgatccagcttaatttctttcttttttttaggaaaaaaacaagacaaaacaaaaaaacaagggtaataatatccaacgccaaagagcctttgataattaaataagataatagttggtaaagaatatagtacagtgcccagcacagagcaagtggaaaatgctattaacagccacttgtacagtgatgataattgcccaaacaatattaatcccactagtaaagggttttcacattacaggtattttttttaaaactttcatcttaggttcggggtacatgtgaaggtttgttacataggtaaagtcatgttatgggggtttattatacagattatttcatcacccaggaattaaacccagtacccaataattatcttttctgctcctctccctcctcccacctttcccactcaactagaccccagtgtctgatgtttccttctttgtgttcataagttcttatcatttagctcccacttataagtgagaatatgcagtatttggttttttgttcctgcattcatttgctgaggataatagcctccagctccatccatgttcctgcaaaagacaagatttcattttttatggctgtatagtattccatggtgtatatgtaccacaatttctttatccaatctgtcactgatgggcatttagattgatttcatgtctttgctattgtgaacagtgccacagtgaacatttgtgtgcatgtgtctatatggtagagtgctttatatccctctgggtatatacccagtaataggattgacccaggctaatttccagca

SEQ ID NO: 13532 - RNA, 2607 nt, Homo sapiens
  source 1..2607: mol_type = other RNA
gctgggattacaggcatgagccaccacgcctggcctattatgccatatttttactaaaactctgtctttaacctatccattgcgttataattgcctacagctttcactacaggaacatgccgtgcaggtgtatagtctaggagcaatgggctataccgtatagcctcggcgtgtggtaggctgtaccatttatgactgtgtaagcacattcaaggatgctcacacgacagaatcacctaaccgtgcatttctcaggacatatccccacacatgtggagatgtgaggcatggaaagcaagttctgcatgaaagatgcagtaatgcgcctcagcagatgagacgtgcagagcccagagcagcgcggttaacgccgtggccggccgttcagggaactggctcatcttgcacgtggtgcgtgtggttcctccctaatgcacgttccatggatggaggaggaaggaagttggatgtgaccaccgcaaacaccatattaggatgtgggtggaacgcagactgcagctgcaaggaattttgtaagtaaatcctgcaaaaagaagacacagctggctgggcacggtggctcacacatgtaaccccaccactttgggaggccgaggctggcggatcacctgaagtcgggagttcaagaccagcctggccgacatggtgaaaccctgtctctaccaaaaatacaaaaatgagccaggcgtggtggcgggcgcctataatcccagctactcaggaggctgagacatgagaatcgcttgaacctgggagacagaggttgcagtgagccgagatcgcgccactgcactccagcctgggtgacaaagtgagactgtgtctcaaaaaaaaaaaaaaaaagtgaacctgaaggagggtccagacgtggtttggcaggagggaagggtgtttcaggagaagaaactacacgtgcaaagtgtcaagagccgcagagtccttggcccggagggtttggggagatgttgggtgacagggaaaggagggatcaggagagtccagcaggggacagaccatgcaaagcctgcagaggaaacacggccgctcagactgtggaggaactggatgaggaggcatctggaagcagtctggagtctggagattagtccgtgacagcgtctgcagcctccatgcccaatgctgcccttgctgccttcctcctgcaagacctcactctgaggaggatgaggcagaggcagagaagcaggatcttcatagccacctccccaacagccaccagaaccacccccgtcatgggccctgatttgcagtgcacggagaagctgagagagacgcgctgggagcccagcgggtgccgagcgtggcaggtgaactctccttcgtgctccatttgaacccgaggcagctccaggaccccagggtctgagggctgggaggggcccacggtctgtccccaccgggtccagctcagcctggctggggggctgctgtgtgtgacacagaccagacgcaggctttggccctccaggacccggagggatgtgccgttcctcaggttttccaggactgtcctgtttgcttgggaaaccatcactctcaggttctctggaggatactgcacagagaggtccagggctcgctgctgggagccaagcctgttctccgctcggcaggtgtagcgccctgaatccccggcccttaccccacgcagctccagccccagggttctggggccccaggggtgggacgaggagaggactctgtcctgcaggacccagctcagcgtggcagggggctggctgtcagcagcacagaggagccgcaggaactggcctttctgaacttccagatatatgacgtttccctggagttccagggaggccacacggagtcggacggtcctctgtgcgctcacaccctttctggagaagtccacatggcaggtgaggtcggtgtcgtggtcctgggggctgggcgtgaagctgagcactgagaagtgggaggtgcttggtctggttcttctaggggagagggcagcccccgtccaggagaaagaaggggctggacatttcttgaaagcccagttaaacacacagatgaccgtcaccggctgcccgggctccagggtctcggggatgtagacatcaggcttctgagtcagggctgttacttttagaaagaacaaattgttcacgaaactatgtctcacacggcttcctctctccacccgaaagaagtaccatgcctcatcctccctctgcgcgtctctgatcaccaaggagcagctccctttgccgggatccccagtgagctggaatcggtcccgggtgctcatttccacctctcgactctggttgttagtggccacaggagcacccgtctttgggctggtccatcctttgaaccagtagccataagcagcagtagactcgtcccagccatcccgggggtaggagaggttgcaagacacgatgacacacaggccctccggcaccggcacctgcctctgcacttgaagactgtaactgggatccttgttcagggaccccgcccccagcacgggcagcagcaggggcagcagcagcatctctgggctctggggctgggcctgtcccgggaccatct

SEQ ID NO: 13533 - RNA, 2603 nt, Homo sapiens
  source 1..2603: mol_type = other RNA
gctgggattacaggcatgagccaccacgcctggcctattatgccatatttttactaaaactctgtctttaacctatccattgcgttataattgcctacagctttcactacaggaacatgccgtgcaggtgtatagtctaggagcaatgggctataccgtatagcctcggcgtgtggtaggctgtaccatttatgactgtgtaagcacattcaaggatgctcacacgacagaatcacctaaccgtgcatttctcaggacatatccccacacatgtggagatgtgaggcatggaaagcaagttctgcatgaaagatgcagtaatgcgcctcagcagatgagacgtgcagagcccagagcagcgcggttaacgccgtggccggccgttcagggaactggctcatcttgcacgtggtgcgtgtggttcctccctaatgcacgttccatggatggaggaggaaggaagttggatgtgaccaccgcaaacaccatattaggatgtgggtggaacgcagactgcagctgcaaggaattttgtaagtaaatcctgcaaaaagaagacacagctggctgggcacggtggctcacacatgtaaccccaccactttgggaggccgaggctggcggatcacctgaagtcgggagttcaagaccagcctggccgacatggtgaaaccctgtctctaccaaaaatacaaaaatgagccaggcgtggtggcgggcgcctataatcccagctactcaggaggctgagacatgagaatcgcttgaacctgggagacagaggttgcagtgagccgagatcgcgccactgcactccagcctgggtgacaaagtgagactgtgtctcaaaaaaaaaaaaaaaaagtgaacctgaaggagggtccagacgtggtttggcaggagggaagggtgtttcaggagaagaaactacacgtgcaaagtgtcaagagccgcagagtccttggcccggagggtttggggagatgttgggtgacagggaaaggagggatcaggagagtccagcaggggacagaccatgcaaagcctgcagaggaaacacggccgctcagactgtggaggaactggatgaggaggcatctggaagcagtctggagtctggagattagtccgtgacagcgtctgcagcctccatgcccaatgctgcccttgctgccttcctcctgcaagacctcactctgaggaggatgaggcagaggcagagaagcaggatcttcatagccacctccccaacagccaccagaaccacccccgtcatgggccctgatttgcagtgcacggagaagctgagagagacgcgctgggagcccagcgggtgccgagcgtggcaggtgaactctccttcgtgctccatttgaacccgaggcagctccaggaccccagggtctgagggctgggaggggcccacggtctgtccccaccgggtccagctcagcctggctggggggctgctgtgtgtgacacagaccagacgcaggctttggccctccaggacccggagggatgtgccgttcctcaggttttccaggactgtcctgtttgcttgggaaaccatcactctcaggttctctggaggatactgcacagagaggtccagggctcgctgctgggagccaagcctgttctccgctcggcaggtgtagcgccctgaatccccggcccttaccccacgcagctccagccccagggttctggggccccaggggtgggacgaggagaggactctgtcctgcaggacccagctcagcgtggcagggggctggctgtcagcagcacagaggagccgcaggaactggcctttctgaacttccagatatatgacgtttccctggagttccagggaggccacacggagtcggacggtcctctgtgcgctcacaccctttctggagaagtccacatggcaggtgaggtcggtgtcgtggtcctgggggctgggcgtgaagctgagcactgagaagtgggaggtgcttggtctggttcttctaggggagagggcagcccccgtccaggagaaagaaggggctggacatttcttgaaagcccagttaaacacacagatgaccgtcaccggctgcccgggctccagggtctcggggatgtagacatcaggcttctgagtcagggctgttacttttagaacaaattgttcacgaaactatgtctcacacggcttcctctctccacccgaaagaagtaccatgcctcatcctccctctgcgcgtctctgatcaccaaggagcagctccctttgccgggatccccagtgagctggaatcggtcccgggtgctcatttccacctctcgactctggttgttagtggccacaggagcacccgtctttgggctggtccatcctttgaaccagtagccataagcagcagtagactcgtcccagccatcccgggggtaggagaggttgcaagacacgatgacacacaggccctccggcaccggcacctgcctctgcacttgaagactgtaactgggatccttgttcagggaccccgcccccagcacgggcagcagcaggggcagcagcagcatctctgggctctggggctgggcctgtcccgggaccatct

SEQ ID NO: 13534 - RNA, 1608 nt, Homo sapiens
  source 1..1608: mol_type = other RNA
gctgggattacaggcatgagccaccacgcctggcctcttcagttacttttataaagaggaactttctttcattatcacccatttggttgttcaaagtacaattttttatggaaagacagaaaaaatgtttgcttctttccctttaattactgattttcagaatagttagttaattctctagtattctccaaaggtgactgatatggttttgctgtgtccccacccaaatctcatcttgaattctcatatattatgtgagggactggtggaaggtaattgaatcatgggggaaggtctttcccgtgctgatagtagataagtgtcacgagatctgatggttttaaaaaaggagttccccagcacaagctcttttcccttgtctgctatcatgtgagatgtgcctttcgccttccaccatgattgtgaggcttccccagccacacgtggaactgtaagtccaattaaacatttcttttgtaaattgcccagtcatgggtatgtctttatcaacagcatgaaaacagacttaatacagtgaccaatgattttatttgtttgcttagtatcattattgactcagatttaaacttattttatgtaagcaatatgtgatgctcaaaatgatccaaagtagattgtcttttaaagttagtaataggactcaataagtaaaatcagtttaaatttatggagatgctacttcggaatttgctaaaaggtaaatgaaactcaatatttactcaaataaaatggatttacttataagtgctgtcatacgcctaaattttagttggggtatcatgctgagaagcctttcattgtacacaatttcaaagaaatgagagtcatggcaactttttcttaccttcgaattactgcattgtagttacatttaagtgtcatcaaacattgatcaacataacacgttactccatgtactaagaaaaatgtttagaaatttactaacataaggagactcagccatcagcagtcactggagacgtatatgttggcacttggtgaagcagtacactaaatagaacatgttggtcaataggcaatactaattaacttagcaaaatattaaaacttttatcatagaatatagatcaagaaattggcaatttttaaggaaaaaatatactcactgcggagcccaaagtgtcctttggcaggattacttcacagcatatacaatgaatgtctttttttccttttctcatttgcttcctgatattttgaaagcatgagttactgtgaaaccatcgccaaaatcaagatcatgaccgtatccacaaatttcatgattctgtaggtcaaggattagagcagccataagcagagagtttgtccctgatacacgatgtttttggccacagctgtagttgtttggatagctgggggctcctgggatggctagagtgggatcatatgcctggagtcttcattcttctccattggatgtttgctgggatgagaaggtccaagatagtcctttgataatgtgtcgtggtgcctgggctgggatggctgaaacacaggagacctagcagaaattctctatactcaccgccatctccggatagtcagacttctcactcggcagct

SEQ ID NO: 13535 - RNA, 2217 nt, Homo sapiens
  source 1..2217: mol_type = other RNA
gctgggattacaggcatgagccaccacgcctggcctgaacacctttagagttctaatgtacaacataaggactaaaattagtaaaattctattagagatttttattaagtaaactgtagctgctcttgtcacaacaaaagcaactatgtgagatgacagatccattaatctgcttcactaaacactttactatctatacatatcccataacatgttgtaagcctcaaaaatacacattaaatttatttttaaaaaataaaatcatgactttgggaggccgaggccggcggatcacgaggtcaggaaatcgaaatcattctggctaacatggtgaaacccagtctctactaaaaaatacaaaaaaattagccgggcgtggtggcgggcgcttgtagtcccagctacttgggaggctgaggcaggagaatggcgtgaactcaggaggtggagcttgcagtgagccgagatcatgccactacactccagcctgggcgatagagcgagactccatctcaaaataaaataaaataaaataaaataataaaataaaatcatgtttgtggactgatatcagtaactggtagtacctatgtgaaacacattttcaaagatgaaatatgtgaaagctcattacaattcaacattagcagatgatgatttgcaatagattttgatgacatagaatagtaacaaagaacctcaattaagcaaaatgttaaccaccccaaaagaattccacttttctcattagtagacctgtattgcaaaacactataacacaatcatgattatattttgaatttcatcaacaaaaactggcggtagcctgggcaatgtggcaaaaccccatcttcacagaaattttttaaattagcagctcatggcgggatgtggcagcgtggtggctgtgtggtcccagctactcaggaggctgacgtggaagaatcacttgagcctaggaggtctaggctgcagtgagccgtgatcacaccattgcacttcagcctggcaacagagtgaggccaaagacctcatatcaaaacaaacaaacaaaataaaacaaaacaaaacaaaaattgtgtaaatttcttctgtctcttgctcaataagtcctacatatatccttgattttatttcttggtccacaaagcataaaatattcgctatctggctctttacaaaagacgttagctaactcctggaaagaagaattgatcctacaaaataagacattaagagatattggtcccaaattcatggtgcaaaagaaagatggggaaattatctcccagagtttctttatgagcctccaggtaaatccaggtgccatttgcaaagactgggaagtgcaaagaaagaggctgggcaaaaggtaagggctagaggggtctcggacatgttgtgctcgaagtgtctgtggaacgggcaggcagggatcttcaggagggagctggatgagtggttctggagctcagaagggaagcccgtaatgaagctgaggactgcggagtcactggcatgttggtggctgctgaaaccagcagtgaatcagatggctcccaaggaaaggcaaaagtactggggccaggtctgagggaacccacacaggtacctgggatctgttcattttctactgatcttggaaaaatgtgaagagtaaaggtaatgctgggaaagaggaggtaagaataaagttaggagaaatctggcccgccttgctgctcctggatccaacttcctaaaatgctacacagaagagaccatttgaacaatgtggagacatctctatgaccagattgtgttgagcttagacatgcaatttttcactgggtgaaagtaaacacatgtatcccaatgattaacaatttatgtcgctaagacacaaaaaaatttaaaatacaaacaattcataaatgacaggatcctaatatagaaagtgtcttcattaaaattgatgtggtaggaaacactcatgttgtgctgtttatctgttttcctatgaatataatactgggaatattgttgaacaattcacagaaactctaaaaaatagaatgaatgcttcagtacaagatttttttaaatatttgttctaatttgattacagtttcacaatcttttgataagacttgtttcagctatgcaaaggaataaagaaatcacgaaactttttttttttgaaacagtcttgctccgtcgcccaggctggcatgcagt

SEQ ID NO: 13536 - RNA, 2306 nt, Homo sapiens
  source 1..2306: mol_type = other RNA
gctgggattacaggcatgagccaccacgcctggcctgacctagtttaagcacaccaaaagctactttacatttttaaaaagtgaatttgatgtcttttgaaatctcctctgtgcacttggggaagtccctgtcctctatcaacttgagaggctggctgctgtgctcacaagccttcatttacacagcaagccttcctttcaggacggctgcaaaacggaagcctaaaacagtagatggtgacagaatggtattgttaccagcagggaaatggcaagctcgccccctggtgacaagctggggagacaacagaaaaagcaaatttttttttttttttgagacggagtctcactctatcgcccaggctggagggcagtggcgcaatctcagctcactgcaagctccgcctcccgggttcaagcaattctcctgcctcagcctccccagtagctgggactacaggcgcctgccaccacgcccggctaattttttgtattttttagtagagatggggtttccccgtgttagccaggatggtcatgatctcctgatctcgtgatccacccgccttggccacccaaagtgctggggttacaggcgtgagccaccgtgcccggccacaaatgttcttaaaaggcacaaccaccacaaagaacatactctctacggtacctggaatctggaaagaacactaattaacacaaaccgtaggtcactcaaaattgttcattcacagggacagttaaaaaggctcagttccaggggacaaatgtgtcacaaagtccttgcttacaaactcctagctgaagctgccttgggaagaatctgctccctcagcatgatgggcagtgccaggcgactacactggaggtgctaatttttaactgccaatgtctcttctagacgatggcaggctgatgtttcatcttcttcagcaaccctgaagcataacagcctttaagctgtatgttgcacgtccctcttgatctctgtgaatttactgaaagatgtgactctaaaggcaaaacgaagcccacaccaatgattatgtaagtcagagggtggtagttgtgactatttaactgttcttagttctttaagacctcaattacgtaaaccaagatacgttctgattttcaagccatcctaaccaaaataataatgatgaaaatgatgacagctgattcctttaggccccggggctgctaatttttcaaacttcctgctatcctcccttccctactaccaatctccagggctctctagtttgctcctatttttcacagagttgccagagtttgaaaactaagacccccataaacatggctatcttcacagaacatccagatgaaggaatattgactgtaataaacattgtacagaacacccagataaaggaatattgactgaaataaacattgtaggctatactccagtagctggggcaatggatccatgtaaatggagctacaaattcaagtcccaagtttttttgctccagcaggttgaccttcaagggctgcatcagtcttcagaaacaggagctgccagcctcaagcagtttgttgcctgggagggagggtggaccacattacccaaatgttaagggttggacacctttctgctgttctttgtgtagctgctgggctcgattttttagcacctcggccttggcctcatccttatcaacaccatcccccagcttgtacatgcgactggcattggcacaggcccagatatgacccaggtcacaggctttcatggagtatttacatgccaggtccatgtccttgggaaagcctggggcaccctgcaggaacatggcactgaggttgaagcaactggaagtatagccaccatcacaggcccttgtgtagtagtccctggcctttcccaagtcaggctggccatcctcattaacctgtccatcatgtgccaggaggccaacgttgtgacatgctgctattgacttctttccaggcttctcacacgccatcaaaaagcacctggcggcagctttcaggtcctgggtcagaccaccttttccagtcacatagtaggcccccagtttgtagcagctatcactgtgctggttctcttcacagttaaacttcaacaccttggcagcctcatcaaaattcttccggatcccttccaaatagtccaccagccgatagcaaccgtccgggtccttctcgtggtagcagtggtagttgcactccacctccatgttctccaaaaaggacttgacctgctcctcatcctggaagtccaccatgccggccatggttcgcgccggcccaaagac

SEQ ID NO: 13537 - RNA, 8041 nt, Homo sapiens
  source 1..8041: mol_type = other RNA
gctgggattacaggcatgagccaccacgcctggcctgagaacttgctttattttagccaaaattattttatcacttctttcccttctcacaggttctagctcttatcttcttgtaccccttccctgccgcaatatattatcttacgcaaagcaagtaaactttcagtttcctattcccattactctatttagcaaacctaggaccttccttaggacccagcatcctcacaaggcagggtggggttgtaaatagcccccagtttttgctgtgtcataaattattttattccttgttacattagcaaaacagacatttcaatgtgaatcctccccgttgataagcttaaattaagaatataaagtacaacactgtaaaacctttgccctgatgttaaaagcctttcagaaggtttttgaaatccctatttcccacttgatctgggttcctcttcaccctgtgagacactccagctgcattgaactgccagtgttcccaatcagctgtgctctgttaaacatccacattttagaaaagcatgcttaatttttcactaaatgataattatttccccagcatttaatgtattactcattctctccacatcaaggaccttgtaaacaaattcagagcattatctgtaggttcttttaagatcatctttaaataattttcaaggtgggatgcggggagtgtcagcaaggcttctctcattaaaaaaccttaaaatctccatttgtccctgtcaaagcctgaattggaagcagggtcagcattagggtgagacaagagatgcagggttgtgcaagtgcagggttgttaaaaaggaaaaaaattgaaattgcttaagaaagtcattgcttttgaggggtaatagcaggtgtacttccctaagtacaatagcaaatctttcaaagaaaatttctatcctatttttccttgaaaataaccatattgaatacagttatagaactgtattttatttatttgtatgtgctacaatttggtgcatgcagcaaccacagttccttaaatttttggccattgttttcaggactcaaaatagctcagcattccattctataaggcccatgtttctttcccatggtacagtatgagtactttttaaagtaggtgaacataaaataaaagtttgctagttgtagtgcatatgaacaaaataaccacatgggttttatggcacatgttctaaaaagataaagatataatggagagatatctcattcaaacaggttaacattataaacagtgcaagtgagggccatagaagcaaagtaacatagtaaaattaacaaatataaaaacctaagctgaaagaggaggtatggagattttttaaatagtcctgaaagataatagagattgctcataatttgaagtagacataattcaggatttgaaataaatcatctaaaattttaaacatgtcatattgtttaaatcattctctgtcctataggaatgacggtaataacttgactatgtactttgtagtgtcctgaaaatagtatgctcagttaagtttataaattgcaaaataaccatctctttaaagtggaacagcattcatcagggaattgttcacttatgaagaggtcatccagacctggagacaagctacttttttggtgaatagaatatattgccattgctactatttatcctccttgttttcaggaatgcttcactacttattctcattatgataaactctatctcaggcttttaggtatcatttaaaacccacttgtgtggggaggttctatcactctccaaataactttgcagggcccaaggctataaatatgaatatatttatacaaacctattttgttataatagggccttgggcctactatacaaacctattttgtttaaggctataaatatgaatgtatttatataaacctgttttgttataatagagcccaaggccctattataacaaaataggtatgttataaaactattataacaaaataggtatgtcatagaactattataacaaaataggtttgtataaatatattacaggacaattatttaccattattacaggaaaattatttctcatctgtatatccaataattacacaaaatggttgtgttttgaagttggagaacaaccacattctaaaaaggcacagagcaaaaaagaaaataagctcatattttactatacgaaaaaggtaaacaaagaagtggttgaaaaatccatgttctatttaaagtcctctcattccagaattatagaatataattgattttatgtgattatcaagtataagctcttggaaattttatgatgtaaaaatagaggcaaagctgtactcattaataaaataaaacatttgattagcatatattgataaaataaaatattcatgattgtagtttattttttgttgaatttattaataatctttatatatatttatatatgtatggctttgagcaaagacaaaagaaatactctaactcatccctgatcatacagttgttgtaagaatcagctattctattatctttccagcagcagaaagaccaatgaataatacatttctttctgtacagattaaaactccatacatacgggcttcactatgtacagagaaaagaggtcacttttcaactagcaatggacctttatattacaggaatgtgagtcatttttttttcttaatctaagtatatatacattcatacatatatgtatataatttaccctgtacctttttattagtttaatatataaaccttagtttttttgtccattctattacaaagtgaataaaaattgtatggttgcactgaaagaccatgcatttcaattttgcttatgtttcccaatagtgctcaaaataaaaaaccaaaaatttatatatataaaaatatttcactaccaaatccattaatcctatcaaatgtaaacctttaataatttaaaggaccaatacgtaatcttaataaattgaagttaattctcatattttaataaaataaaggagttttgtactgatatgtaaatggtcttgcagctttcccataggttctaggtagactgaacaatccctttcttacaacagtattcctgacatgccatcatatgtcaccagcatattgatgattacattacatcgactagcagttaattacttccacaccagttgggatttgtttgaaattaaacataacaactcattttggtattataggtattatatccacaaaaggcataacaggcagcaaggatccactttagagtttctgcttttgtttttgttttctgtcctcaagtctatctgcaggccctgtcccacataatgtgtgatctctgtatgttcttaaatgtattgccagtgccagagatactgaagacctccactttaagtcatgctcttaacttgggttatttaccgcagccagttgttaggaatctttcaattgtgttccagtcatactccacatgtgtgggatgcattaggcacaaatgattactaagggagttctttgagaagaagcaggtgctcacagatcatgtaaagagttaagaaaacagacagacaatgctcatagacgttcaactttacccctgctttctgtcaccatgtctgtactattttcaacacattaaaaatgacaaacctcctatctaagggctacgttagtcaccacatgccttaaagtttactaaccatttagttacaatatacatagagcaaaatgtgtgttcccaaacagacgtgatgctgtattgaatttatttctttaaattaataccatagtaaattaccagctacagtgaagacacagacaacacttaactccaaatcaagctgtggtttacaaataattatttaaataataatagcaataatattaaataaaagtgaaaacctcacttctagacttaagtcagagatccaagtcagccttataggaattataagataggcaattaatgaattgttatgcttttctagaaacgagaaatactgtaagcctttctctacaatgactgatttgaacctatttttttttccccagaagcatgcagggactattttcagatgcttgattatggcaagaagaaagaaaagtaacgatttttggtgtaatacaagcaatttgtagattcgagcatacaattttgcataaaacattgcaggttaaaataatattgtaggtttcaagccattgcattacaattgaataattctcacaatcaggttttgtaaaatttaaaactctaagttttgaagtgaagcaataaaactaaattcttaaacaatgacttttaccttcatacaacacagaatagctatttttatttgggttgaaaaagttatttacaactaacattgatcgagtcttggtaaaagtccgataacacatgaagacaaatattaattttccctcagctttctgaaagatcaatgaacatgtttgaggttagtgatattcttaacaaacagtggcaatgctagtctcctacggtggccaagcaagtagtgcattctttaacctaatttgaaattgaaagcaccgaaatacaatttagatctataaaatgggatttgttatttaattctccaccattaatgattaacaatttagatgcagagacacagctaatgaaagaaagttttgattggtgctatttactagttcatttgagttgcctttttaaaatcagttttgtttccattgaatccaagaactcttcataaaatagagaaatatacatatcaaaggacttaagtaaaagtaggttagaaataaataatcttacaacgacattttaaatcctttaatgatttaaagaaaggaagacatataacactgaatgctaaacaggtcttttgaccctctcttgggaatttagatatatattttatagtatatgtatatatatttttacatttcacgtgtaggccacagctgtctaaaatatctcttcatagtaggctagagggatctatcaggagatagaataaaataagatctgagtatagtctcagtttatgagagtatttctttctgctttgacaatcagcagggatcataaatttgaagcaaatcgtggcttttctgcgtctgggtctgtgtttaagactgaggaagattctcttggaagagcagctgctggtggagggggtgctggagggactcctcggttcggggggatggctcccgacgacatctgtcggaagagggtgacgcgctgcgggacagtgctcctgccccctgcctgaaggcccgttccggggaccgccgtcacgggttgagggatggaggccagggactcgcccacagtgggatgaggtctggaaatcagagtggacacctcatggggcagcgagggctgcgaggcggagagtggcctgacttcccgggtcaggttggtgttgtgaagcgcctgcgtgctcttgtgcacttcatttttcggcgtggagctgccaggtgtctgtggctgcggggacggctgctgtggctgagtctgcggcggctgggactgctgtacctgctgctgcggctgctgttgcatgagtgacagctgggaggcggtgggggaggcatagtggaaagttcgagcggccagagggctctgtacaggagggctgcagaccgcggtggtgtaggagcagggtgacaggatggctgatggctggggggtctgtgtgctgggactgggggagtgcaggttgctgtgagacaggctggtcgctgtgtacaccggtggagattgtgtcctcatgcgggaggtcggggtcgtagtagacgatgtggaattcagggttgtcatttgaggataattgatgggagcgattgcctgcaccatctccctgtcatgtttcacaatctgcttgaggatttcgttctcctgattgttgaaaacaccagtgttcagatccttctggaacttttgcagaagaattgaatttttctttcctattcgatctagtcggtcaatggcaactgtctcaaaggctctcctcatcattggatattcctccaggacctcgttgaaattgtccacggaaagtgagtaaagacgacaatatgtatcagctcgaacactggcagtacgacgtcctttggtcagcaggcaaatctctccaaagtaagagccatctgtcagcttcatttctttactggattttgtaatgacaccagcaacaccgtgttgaatgaaatacatttttttacccacggctccttctcgtatgatataatctccaggttgaaacacctcaaatctcaacttgctcagcatggcagtcacaaaattaggatccgcattagcaaataaaggcattgtagccaccagtttccgacagttgaagttgactatctcctctctcagaggatcattgagttcattgagaatattttcctcatcaaagattttgccttggtatctgtgttcatagtaatcatgtatcttctgacgcatatcagctggtaacttatggaatgacatgtattgttccacttgcttatacttctcttgatactgccgcctcgaagaatccagagactggattaaagcggtggcatggccgacaaacatggcatagcaggtggccccgacgatcatgctcagcatggtaatccagaggtcagacatgctgactggggcttgggctccatacccaatgcacagcatgtgactcatagctttgaagagtgcgtatgaatactgctttccccaagaatcattaaccatttcatttaaagacacccagcaatctggtgggaagtcctgcagtagtggtactaagaactgaagacaaccatcccagtggcacaggagcagcatcatgccgatgagattaaaaattctcaccactgcactggcgagatcatatgtcatgtggaatatctcttcccattgatgtatgtatctaattaaccttgaaagtcgtaataaacgcaagagactgagaatttttgtaaacctcacaatgcgaagtgccctggctgtcttgtaaacttcagaatccattcctttttctacaataagaaagatataatccactgggatggatgagatgaagtcaaccacaaaccagctttttaaataattcatcttgatcactttggggtccaggatgatttcagaactgtcttcattgacagtcccagtcctaaaattcatgatcaggtccaataggaaaactgtatctgatgccacattgaaaataatccatggtgttgttgtttgctctgtaaagaatgtgattccaactggtatgatgactagatttccaaccatcattataagcattattaaatcccagtaaaacctgaaatcactgtaagggtggataatccagaagcctgcagttttaaccctttcctgctccttttccaccgccttctggctcccaaacatgcggagggagaatttgttgaccccgggctgcagcatggaggtgaactgcctctgcatgaagccgtactgccgccggggcccctcggcgtcttcgaagccccccgccggctcctcgccgccgccgccgccgccgccaccgccgccaccgccgtccaccttgaagcacacggagttgccgtgctccttcgcgccggccccgccgccccccggcggggtgcccaggcgcttctcggccgcggccggccccgcgcccgtcgcggacgccttggcggggaagacgctgttgccatcgtcccggctgttagacgaagagttgggcttgccgcctccttccatgcccggaggacgcggccggcgacggcgcgggctccagactcgccggccgcccggcgccggagacacgtagccgagagggtaggggcccgagccggctgccggcgagcccagctgcccgtcgcggcggcggcggcggcggcggcggctgctgcttcccgaccgcgccgctgctagctgcgcgcctggctcccgccgccgccgctgcccttagtggctgcggtccgggctccggtgcggctggtgctgaagctgaggctgccggagctaggcgaggctcagctcggctc

SEQ ID NO: 13538 - RNA, 11263 nt, Homo sapiens
  source 1..11263: mol_type = other RNA
gctgggattacaggcatgagccaccacgcctggcctgggaggggtttttgaaagcatactgccctccccatgccccctcccccggacaccctcaaatcccactttggcagcagataatggaaacaaccactgggctaggcaaagtttctgctgcgtgctccaggaaatctataatgagaagtcctggggtagccagcagagattctcttgaccctgaagtccaagagaggggtgttgccccctggggacattgggcaatgtctgatgacatacttgattgttaccgttggcaggacactgctacaggtatcttgtggatggaggccaggaatgctgctcagcttcctacagtacccaagacggcccccacaagaaagaattacccagccccaaatgccaatagtgctaaggttgacagaccctgcgctacagtctcctagaacttaggagtcaaatctgggcacttcgatgtcctggagttactttctaaaagactacaggaagcagtgcatggaggcagatttgttcccgcctgccagggccatctcgttaataacggactgtgttttgggccagacgggcatagccccgcttgaccagaactgtttgggtattttagaacaaaacaaactcatataaacatactaaggcatattgacagctgaccacctccctcgcacatggctttgataagtattaataggaaacagactctcgacagacactgctttccacgggtgaaagtgtacctgggtccttacatttggggaagggcagcttttcttttggggcccctttgccacaaggcagggactggcagtgggccaaggatagggagtgtgagataaagggcagaggccaggccaggttggcctccaaagtcaaatccctgttcatggggaacatctatgttgactccctgggaggcaggccccttccctcagaccctcagacctgtgtttccttaatcccagcacctggtctttcattttaattttttttagagacagggtcttgctctgtcactcaggctggagtgcagtggtgcgatcctagctcactgtcgcctcaaactcctgggaccaagtgatcctcctgcctcagcctcccaagtagctgggaccacaggagcatgccatcatgcccagctaatttttttttttttttttttttagtagagacgagattgcgctgtgttgcccaagctggtctcaaactcctggccccaagtgatcctcccacctcagtctcccaaagtgctattacaggcatgaaccaccatgcctggcctactttttgagccaaagaggacatttggatgcaggagactatgaaggttggggacagccagagagtatgaatgggttataaaggaagactagttagtgtttctctctccttgttgcttcctggcagtctcagactacattcctgatacagacagaaggctttgaggacatggtggccacagcggcatgctgggtatgtggggcagcgggtagggaaatatacaaggaaacatggctggtttaaaacacaggctagaagtccacagatttcctaatggcaagaatgaaaaggctgcattaggcgctggtgctgtcggagtgaaggggctcaggcatctggattgcccatcctattaggaccatttgccctatgagctaggtcaggacacctctcacttgttttgagcttagggcaagacctgacctctttcaaagtccagagcaggcagctgctgaaagcgtgtttggtcagaagattctgtgttcttagccaatgtctactggctgggggtcagttttccctccgggcatctgggcatggctggacttgggaaggattcaccctgttgactccagagaagctgactatcacatcagctctgaaaactcatcttttccctgagcctgctcttcagagacctctctctcagctaggggcaagatgttttattttattttattttattttattttttttgagataagagtcttgctctgtcacccaggctggagtgcagtggtacaatcttggctcactgcagcctccacctcctgggctcaagcgatcctccttcctcagcctcccaggtagctgagactacaggcgcatgccaccatgcccagctaatttttgtattttcttagtagagtcagggtttctactaactggctgactggtctccaactcctgacctcaactgatacacccacctcggcctcccaaagtgctgggattacagacatgagctaccgcgcccagcctgcaagatgctttaatttctcctttattctcaccctctacaatggatggggtgccaggtacgctgattcagttcctggagtctctttatcactacatccgcctcttccctcactcaagccttggttgcagcaataacccccccaacagctcaacgggccatgctctgtactgtggccagaactttcttttccaagtataactccaatcgccttaatgtccctttttgaaaaacattcttagggactccctgttgccttctgaataaagcctaaatttcttgtaatgccactcacctctccccacggtctggtcccagcccaccttttctcaccctcctcagccttccaaagccagcctcaatttatcttacatgctccctgtccgtgcctttcctctcactcttcccaattcctggacaactcttaccttccagaagctaccagtgaaatcccgcccatttctcaaaccccagaaatttatgtcagttccaagacgggtgtctctctccatcagattataacctttggctgggcgtggtggctcatgcctgtaatccagcactttgggaggctgaggtgcgtggatcatttgaggtcaggaattcaagaccagcctggccaacatggtgaaaccctgactctactaaaaatacaaaacttagctgggcgtggtggtaggcgcctgtagtcccagttactcaggaggccgaggcagaagaatcacttgaactgggggaggcagaggatgcagtgagctgagatcgtaccactgtacgccagcctgggtgacagagcaagactctgtcaaaaaaaaaaatagattctaaccttctgcacgagaggaactgtgttttgcttatctctgcaaactgcccggtgccttccacacactggagaagcaagacatgttataagttaagtgaaaaattaaaatgcagtaagttttgaaccaggtactgtaactgggcatttcgtgggcattgtctcattcaatccaccttgttatacaggtgggtatgcagactctaaaaggtcaagtgagccgcccacagccatctgcaccaacaggggcagaattaggatttgcactcaggtcggctcccaaaattccatattgatgggtctgaagtgtccccccgcaaaagaaagacacctggctgtctcactccagggaaaccaaaagaagccctctctcctcccaaggagtttaacatcatctctctgctctttcacgacacaagctgtgggaactggatgcatagtgatggcaggtgagcatgatgttccggtgttcctatttcaggagacgtctcattcctcctggccaaactcacttttgtgaaatggggctggagctgctactggtcaattcagggggaagagggaaataaatgggccataacccgaataacccccaaatatcttgtcaaccctattttgcttacccattgcttaattctattttgcacttaaacggttggctacgaggcctggatgaaaagccaccacgagagggcagtatttccccacccttgatctgagcctaacaatctggactccactctggtccttgagaggttactcaacagagagagaggcttttggtatcaggaattctggcaaatgaaagaaacacatcagatcgctctcctgccttctagcctggagttgtgaagcagcttgtgttggggattgaaaggtgtttacttaaaaaaaaatctttctggagaagaaggatgaatcctggttttataatcatttctttggactccttgacaaaatgagacaatgtttccatctgtctgctactagaaaggcaggcacatgcagaaaggaggtgcctggcaccttgtaagcgcttctaagtatttattccctgatggaaaagcattcctgcataaagcttgacttggagtgggaagcactgatcaatttgtctttaatggggattggacacaacagtttccttccctggggaattggggaggcgtctccaaagctataaaggattggaaagaaagcctttgggaggaaagctactaggagctggaaatgggtttgcaggaaaggagtttagaatgggcttcccttcaggattagaaggggtgagtgtgggatgctaagtgtttgttctttatatctgtggaagagtgagcaggggaaattgggattaaaggaaggcaggggagattatagctggcatgaagtcaagctccatgtggcaggaacaggacaccggtgggggctgccagggatggcagagcaaggtgagtcatagattgccttttcactttaacagtctcctggcctgggccctttggggtcttggtgcccccactgtaaagccctttcaaagagggccagtgcacttcctctttagcagacacccaaactgaacaacaagatatgcccacgtacagtatataaaagaaatgtggtttttctgtatagcaagacacaacaaacagggtagaaccagcagaacattccctttccatccttggggaccctgcagtctgggaggccactaggatttcttgtctctttctgggaactgcctgacactaatttgtagtatttaaaaaagtatacaaagggatcccttcccaccatttactctgagagagtaaattcaacaggttgcctcttagggaggaattacaccggctccaattcctaccgaagacttggctgcccatttttgatctgagttgagggtaacttatttgtcaaaattaatttaacaggtttaaaactttggagatcaactgcagagggcaacaagcctgagggacaagttcttcccaccccaagttgtggctcctatcgaagaagccacgtgggacctcattatggcaactctttccaacctcatccactttaaccagcttccattatttcatccccaagggtgaagcagcaagcccgctttgggggaataaaaaaataataatcatattgttacttgatattgtttccaggcaccaaagctttaacatttaatccattcatattctttaggttcgtatgacattatgactaggaaaaactgaggacaagtgacccatccaaagtcatccagtggcaaagtgggaagatccttattgccaccaggcttctttgaacaacataacttccaggccccttggatgctattgctggaggagggggtcagtcaatggatgtggcaaagtcaagtgattctagctggtatgggtgggtttggggaggggatttgcacaatccattggatgggttcatgtcacatgagggctctgctcactggtatcaaaatctaaatgcagcaaattctgggaatgcctctttcattgggagacagcccctttaatcaatttcccactcctctccccatgccctgaaccctttctaactagaacaattatggggcttccaaatgtttcaggtacatgggcgtggaccctaattatggacacacgagggattaatatgggccagggacacgtttcttggcattgagggtcttcaatgaaagcagtggcaatctaagatcgacacacttgtgcagggaagaggacggacagagacctggcccatcacacacacacacacacacacacacacacacacaggcacgcacaaccaaaatgtcatcataaaaaaggagaaagggggacttcagtggctgagggactggctcagagagcttgtgcctagttcctgcagcctttccaggggaaccccagagaaaaaaacccccacagcgacggccatgttccagtggtttcatgcacccgtgagttgcccttgtcggcaagagagggagtgggaacagagttttgtaagagccactgcagattagaaaagcattgcatcgcagcaggaaaactcaaggagtaaacccaggagggccgaggaaaccactgaggggcgagaagcccgaggagggaaaccagggcacagcgacaaggacaggaggcagagcgagggccacagggggtcccagaggaaaggttcagcagtgtctgtccgcgcttacaaaacttgcagccggctgggcaagagggtccagttaggagctgaaaacctcatcggtgtcttttttgctctcttcaatgaaggcaatggactcagatctaaggcggttggtcacttcgtacgttcgcagggtgactccaaaaatatcctcatggtatcggttgtcatccctcatccggctgatgaatacgccggcgtcctctgccgagagcttcccctgctgggtcatgatgcgctggatggctttgaggacatcagcagccatggtgacgtccccacagacgtatatgtggcccccttgctccttcagggctcggtacacagactccgccagctgctcctgcaggatgtcctgcacgtacttctttggtttgtctggctcccgggagtaagccgtgtacagctctctgaagacccccttgttcttggcctgcagggtctcttccctgtagatatgatctatcttggattgccggcacccgaagaccaggaccatggggcaggggttcattcctttgtgttggatatcaaattgccgctgttgccagaagcttcggaaaggggcaatgccggtgcctggtccaacgaggatgcaggggacttgggggttccggggcaggtggaagctgggtgctcctctcacgaaacaggggaccagttcgtcagcctgtatccggttgagccaggaggagcatacgccgtggtgaattggtccttctccatctcgagtgcggtaggaaacgatggccacagtgaggtgcacttcatcagggtacatgtctggggaggagctgatggaatagtagcggggctgcagcagggacagctgggtcaggagcagggtggccggcatctggatagatgggaactcctccagcacctccacgatggtggggttcttgccccatttccattcctcgtactcctgcaaacccttgctgaggaccagcagacgctgcttctccttctcgctggtagctagggaggcaaactgctgcagctgcagaggcgttggtggcgtggtgatgtccaggtagtacttgaaggcctggaagatggtgcagggcgggaggcggagctcgtctgtccagttactgatgacacctaaagccgtgttccgctcctccagcagttccactttcaccatctggttgacaggcggcgcgtcctccagccgctcgatcagggcattcacgaggtcctcgtggttgccagggaagacacccaggtggtccccaggctggtactgcagctcctggctcccgttggtgtggagacgcacgaagatagttgaccgactggatttagggctctggaggttttgacggctaaggagccgggcagctgagactcgctttttgtggacattggatagaccttgtgtgagttctggagcttcggccacaaaggtgaggcggaacttgtttctcttccagctgcgatcattgctgatgagggaattgttggccttttcaatgttgacatcatctcccacacagaagacatcacaggctgccttgaagaccttcttggcccaggtcctgaaagcctcttcctgcccacagagctcatccccttccctcatcttcaggatcctctcccctcccagttcttccaggagggtgtccacagcgtgtccgaaggcgcaaaagtgagggtatgctcgtgagccgaggccaaaaactgagaacctcacattggccaggggtccagcactctcaaagttgtctctgaggtcgggcccatcgcctgatgatttttgggagtcagagtaggaggagacgctgttgaatcggaccttgtagctcctgtgctggctgtcacgggctgcagccagaccgtggacttctgtgtcaccattggggaggggaggccctttacggggaaagaaacgcaagggttccgggtacttcctttcttcctgcacagagttggggtgcctcatttccatcaaagcacagccgaatttctccccattctcagggggatctccattgccaaaggtgctggtgaccacaaggaccagagtttcatgttccaggtgcacaatgtcatattcttccatggacatcaccttggcatcaaaggcgtgtttgaagatctcacacaaggtcttggcataagcttgcgatttgcctgtctctgtggcatagaggatggtcgctttcaccctcttggccatagcctgccccatcagcttggccgagaacttgacagcttctgctagcttcttgaagccaatggctcgccgctttgtgggggtcccgttggtgcctttccagacatgcgtgttccagggatcaggctggtattcgaaggagggggtgagccggtagttgagcatctcctggtggaacacaggggtgatgcttccggacatggggggcacgatccacacccagtcggcagggcagcccccccggcagcggtactcattctccatgtgcttaatgaaggactcggtggcggagtgatggtcaacaatggtcactttgtcactctggaagctatagagaaccgcgatattgatctccaccagcgcctggtccttccacagggaggacgtcttcctcatgtctaagttcatcttcttggccacttcctccaggatattgtagcgggagttgtcacagtagtcgcggacaccaatctctgtgcccatgtaccagccactgaagggacaggcgctgaactccaggccgccaatctctaggagcatgttggacacggcggggaggccgtaccacttcagccccaggtccttgaaccactcaaacttggggtgcctgatgggaacttccaacaccagctctggaggaatctggaagagctcagggtcattgccgttggcctgaagcaggagcggcaggacatcgaagcggcctctaggcggtttccagccctgctgtatgcatatctctgtgaactgcacattggctgggtcccccagggtggagccgtcaggctgcttgtagccagcgtagcggatgagctgggagttccagactcggaagtcgtgcttgccgtctgtcctctgggggaatatggtgatggcagacctgaggttccctttgttggtggcatacttgacatggttacagatgtagttgaacatcccgtgggccgtggtgcagtcacgggcatcgaatacctgcagcttggaccactggatcctgcccacacagcgcgaggcattccgccaggcgtgcttggccccatagatgagctctgtgtccttgagctggtaagtgctagtggtgtcgatctctttgttcacctcttccagcctttccatgtgggctttggagccaaatcttttaattgatgaatagtattgatcaataaactctttggcgagagggaagagctgtccttttgtgcggacgtcttcaggcctccttgcatgctgagaaggatgcatgatggagcccatgcagatgtactcagtgcatcccgtttccaatgtgctcttaaggtggagggtgtcagtgagaaccacctcagtctcccagttcttgaccttgaggaagcgtggacacttggaggggctgccattctttgtgggggactgttttcctgaggtggggggctgctccttctctgaatatgggttgttgaggacgacaggcacattgcccttcccccataggtcattgaagactcggtcgttctccacgccgaggggcagaggtttgtgtgacttgccgtccaaatctctgtccacctggattcccatatctttcatctctgccttggcaggtgcccctcccttgacccctctgctcccactggtgagaaggctcagcacaggctctatctccttgagcagttcattgttctcccctctgccttggaggctgactctggttgctttcttcgcggggtcctggcctgggggcctgggggccaggccgttggcatgggggagtgagccagcctcctgcccatcatcgtaggcatgctgaggcccattcccgggacccgaggccccatccactgccaggggctgttctttgccggccggtggctggtgggacagatccacggctttggtggggggacccaggggctgtgtcacccggatggtcttgggggtcccatcacctgtaaaggtggtctccaggtgcgtggtgaaaccttcagggcccctcagaatgaggaccacgtgggtctcagaggcaatgcctctgagtacctccagggcgctgtcatagctcaggtccaccaagggccggccgttgaccgcaagaatgatgtctccggcctggatgaggccactctgctctgcggcgcccccacgaatcaggtcagagatgatcacgggcggcttactgacccgctccttcaccagaaatcccaggcccccaactttgcgcttgaagagacgaacagaaatgacattgggctggatttgctgaacaccgaacatgtgatcctccatggtaactagcttccgaggggtcctgtctgaagacctcacaatgctatcaggccaagatgatttcaccaggaggatccaggcttcaggctacacggagagcaggagccggggtgacaggtgctgacaaggcttcagccctctctgtctttgacgtcagctcagcgtcacccactcatggctggtggcccgtcggtggcatgatttcctgcatccgcctctctccttattctctaaggaagtgatggttgaccaggcagacgtcaagagaggcggtgggacgtgtccctaaggtcaggcagaaaggggaggagatgcgtctgatggctgtgtctagaagtgacgcatgatagatgtgaactattctctgggtatcttcattgccagcctgttagatgcggatcagatctgaggcatcatgagcccgtccgctcggccgctgctcgctgcccggccgcccctcggaggagccgcggcgctaagtagctcctcacccagcggctggaaacgcggcataaatatgtagggactgagccgt

SEQ ID NO: 13539 - RNA, 11161 nt, Homo sapiens
  source 1..11161: mol_type = other RNA
gctgggattacaggcatgagccaccacgcctggcctgggaggggtttttgaaagcatactgccctccccatgccccctcccccggacaccctcaaatcccactttggcagcagataatggaaacaaccactgggctaggcaaagtttctgctgcgtgctccaggaaatctataatgagaagtcctggggtagccagcagagattctcttgaccctgaagtccaagagaggggtgttgccccctggggacattgggcaatgtctgatgacatacttgattgttaccgttggcaggacactgctacaggtatcttgtggatggaggccaggaatgctgctcagcttcctacagtacccaagacggcccccacaagaaagaattacccagccccaaatgccaatagtgctaaggttgacagaccctgcgctacagtctcctagaacttaggagtcaaatctgggcacttcgatgtcctggagttactttctaaaagactacaggaagcagtgcatggaggcagatttgttcccgcctgccagggccatctcgttaataacggactgtgttttgggccagacgggcatagccccgcttgaccagaactgtttgggtattttagaacaaaacaaactcatataaacatactaaggcatattgacagctgaccacctccctcgcacatggctttgataagtattaataggaaacagactctcgacagacactgctttccacgggtgaaagtgtacctgggtccttacatttggggaagggcagcttttcttttggggcccctttgccacaaggcagggactggcagtgggccaaggatagggagtgtgagataaagggcagaggccaggccaggttggcctccaaagtcaaatccctgttcatggggaacatctatgttgactccctgggaggcaggccccttccctcagaccctcagacctgtgtttccttaatcccagcacctggtctttcattttaattttttttagagacagggtcttgctctgtcactcaggctggagtgcagtggtgcgatcctagctcactgtcgcctcaaactcctgggaccaagtgatcctcctgcctcagcctcccaagtagctgggaccacaggagcatgccatcatgcccagctaatttttttttttttttttttttagtagagacgagattgcgctgtgttgcccaagctggtctcaaactcctggccccaagtgatcctcccacctcagtctcccaaagtgctattacaggcatgaaccaccatgcctggcctactttttgagccaaagaggacatttggatgcaggagactatgaaggttggggacagccagagagtatgaatgggttataaaggaagactagttagtgtttctctctccttgttgcttcctggcagtctcagactacattcctgatacagacagaaggctttgaggacatggtggccacagcggcatgctgggtatgtggggcagcgggtagggaaatatacaaggaaacatggctggtttaaaacacaggctagaagtccacagatttcctaatggcaagaatgaaaaggctgcattaggcgctggtgctgtcggagtgaaggggctcaggcatctggattgcccatcctattaggaccatttgccctatgagctaggtcaggacacctctcacttgttttgagcttagggcaagacctgacctctttcaaagtccagagcaggcagctgctgaaagcgtgtttggtcagaagattctgtgttcttagccaatgtctactggctgggggtcagttttccctccgggcatctgggcatggctggacttgggaaggattcaccctgttgactccagagaagctgactatcacatcagctctgaaaactcatcttttccctgagcctgctcttcagagacctctctctcagctaggggcaagatgttttattttattttattttattttattttttttgagataagagtcttgctctgtcacccaggctggagtgcagtggtacaatcttggctcactgcagcctccacctcctgggctcaagcgatcctccttcctcagcctcccaggtagctgagactacaggcgcatgccaccatgcccagctaatttttgtattttcttagtagagtcagggtttctactaactggctgactggtctccaactcctgacctcaactgatacacccacctcggcctcccaaagtgctgggattacagacatgagctaccgcgcccagcctgcaagatgctttaatttctcctttattctcaccctctacaatggatggggtgccaggtacgctgattcagttcctggagtctctttatcactacatccgcctcttccctcactcaagccttggttgcagcaataacccccccaacagctcaacgggccatgctctgtactgtggccagaactttcttttccaagtataactccaatcgccttaatgtccctttttgaaaaacattcttagggactccctgttgccttctgaataaagcctaaatttcttgtaatgccactcacctctccccacggtctggtcccagcccaccttttctcaccctcctcagccttccaaagccagcctcaatttatcttacatgctccctgtccgtgcctttcctctcactcttcccaattcctggacaactcttaccttccagaagctaccagtgaaatcccgcccatttctcaaaccccagaaatttatgtcagttccaagacgggtgtctctctccatcagattataacctttggctgggcgtggtggctcatgcctgtaatccagcactttgggaggctgaggtgcgtggatcatttgaggtcaggaattcaagaccagcctggccaacatggtgaaaccctgactctactaaaaatacaaaacttagctgggcgtggtggtaggcgcctgtagtcccagttactcaggaggccgaggcagaagaatcacttgaactgggggaggcagaggatgcagtgagctgagatcgtaccactgtacgccagcctgggtgacagagcaagactctgtcaaaaaaaaaaatagattctaaccttctgcacgagaggaactgtgttttgcttatctctgcaaactgcccggtgccttccacacactggagaagcaagacatgttataagttaagtgaaaaattaaaatgcagtaagttttgaaccaggtactgtaactgggcatttcgtgggcattgtctcattcaatccaccttgttatacaggtgggtatgcagactctaaaaggtcaagtgagccgcccacagccatctgcaccaacaggggcagaattaggatttgcactcaggtcggctcccaaaattccatattgatgggtctgaagtgtccccccgcaaaagaaagacacctggctgtctcactccagggaaaccaaaagaagccctctctcctcccaaggagtttaacatcatctctctgctctttcacgacacaagctgtgggaactggatgcatagtgatggcaggtgagcatgatgttccggtgttcctatttcaggagacgtctcattcctcctggccaaactcacttttgtgaaatggggctggagctgctactggtcaattcagggggaagagggaaataaatgggccataacccgaataacccccaaatatcttgtcaaccctattttgcttacccattgcttaattctattttgcacttaaacggttggctacgaggcctggatgaaaagccaccacgagagggcagtatttccccacccttgatctgagcctaacaatctggactccactctggtccttgagaggttactcaacagagagagaggcttttggtatcaggaattctggcaaatgaaagaaacacatcagatcgctctcctgccttctagcctggagttgtgaagcagcttgtgttggggattgaaaggtgtttacttaaaaaaaaatctttctggagaagaaggatgaatcctggttttataatcatttctttggactccttgacaaaatgagacaatgtttccatctgtctgctactagaaaggcaggcacatgcagaaaggaggtgcctggcaccttgtaagcgcttctaagtatttattccctgatggaaaagcattcctgcataaagcttgacttggagtgggaagcactgatcaatttgtctttaatggggattggacacaacagtttccttccctggggaattggggaggcgtctccaaagctataaaggattggaaagaaagcctttgggaggaaagctactaggagctggaaatgggtttgcaggaaaggagtttagaatgggcttcccttcaggattagaaggggtgagtgtgggatgctaagtgtttgttctttatatctgtggaagagtgagcaggggaaattgggattaaaggaaggcaggggagattatagctggcatgaagtcaagctccatgtggcaggaacaggacaccggtgggggctgccagggatggcagagcaaggtgagtcatagattgccttttcactttaacagtctcctggcctgggccctttggggtcttggtgcccccactgtaaagccctttcaaagagggccagtgcacttcctctttagcagacacccaaactgaacaacaagatatgcccacgtacagtatataaaagaaatgtggtttttctgtatagcaagacacaacaaacagggtagaaccagcagaacattccctttccatccttggggaccctgcagtctgggaggccactaggatttcttgtctctttctgggaactgcctgacactaatttgtagtatttaaaaaagtatacaaagggatcccttcccaccatttactctgagagagtaaattcaacaggttgcctcttagggaggaattacaccggctccaattcctaccgaagacttggctgcccatttttgatctgagttgagggtaacttatttgtcaaaattaatttaacaggtttaaaactttggagatcaactgcagagggcaacaagcctgagggacaagttcttcccaccccaagttgtggctcctatcgaagaagccacgtgggacctcattatggcaactctttccaacctcatccactttaaccagcttccattatttcatccccaagggtgaagcagcaagcccgctttgggggaataaaaaaataataatcatattgttacttgatattgtttccaggcaccaaagctttaacatttaatccattcatattctttaggttcgtatgacattatgactaggaaaaactgaggacaagtgacccatccaaagtcatccagtggcaaagtgggaagatccttattgccaccaggcttctttgaacaacataacttccaggccccttggatgctattgctggaggagggggtcagtcaatggatgtggcaaagtcaagtgattctagctggtatgggtgggtttggggaggggatttgcacaatccattggatgggttcatgtcacatgagggctctgctcactggtatcaaaatctaaatgcagcaaattctgggaatgcctctttcattgggagacagcccctttaatcaatttcccactcctctccccatgccctgaaccctttctaactagaacaattatggggcttccaaatgtttcaggtacatgggcgtggaccctaattatggacacacgagggattaatatgggccagggacacgtttcttggcattgagggtcttcaatgaaagcagtggcaatctaagatcgacacacttgtgcagggaagaggacggacagagacctggcccatcacacacacacacacacacacacacacacacacaggcacgcacaaccaaaatgtcatcataaaaaaggagaaagggggacttcagtggctgagggactggctcagagagcttgtgcctagttcctgcagcctttccaggggaaccccagagaaaaaaacccccacagcgacggccatgttccagtggtttcatgcacccgtgagttgcccttgtcggcaagagagggagtgggaacagagttttgtaagagccactgcagattagaaaagcattgcatcgcagcaggaaaactcaaggagtaaacccaggagggccgaggaaaccactgaggggcgagaagcccgaggagggaaaccagggcacagcgacaaggacaggaggcagagcgagggccacagggggtcccagaggaaaggttcagcagtgtctgtccgcgcttacaaaacttgcagccggctgggcaagagggtccagttaggagctgaaaacctcatcggtgtcttttttgctctcttcaatgaaggcaatggactcagatctaaggcggttggtcacttcgtacgttcgcagggtgactccaaaaatatcctcatggtatcggttgtcatccctcatccggctgatgaatacgccggcgtcctctgccgagagcttcccctgctgggtcatgatgcgctggatggctttgaggacatcagcagccatggtgacgtccccacagacgtatatgtggcccccttgctccttcagggctcggtacacagactccgccagctgctcctgcaggatgtcctgcacgtacttctttggtttgtctggctcccgggagtaagccgtgtacagctctctgaagacccccttgttcttggcctgcagggtctcttccctgtagatatgatctatcttggattgccggcacccgaagaccaggaccatggggcaggggttcattcctttgtgttggatatcaaattgccgctgttgccagaagcttcggaaaggggcaatgccggtgcctggtccaacgaggatgcaggggacttgggggttccggggcaggtggaagctgggtgctcctctcacgaaacaggggaccagttcgtcagcctgtatccggttgagccaggaggagcatacgccgtggtgaattggtccttctccatctcgagtgcggtaggaaacgatggccacagtgaggtgcacttcatcagggtacatgtctggggaggagctgatggaatagtagcggggctgcagcagggacagctgggtcaggagcagggtggccggcatctggatagatgggaactcctccagcacctccacgatggtggggttcttgccccatttccattcctcgtactcctgcaaacccttgctgaggaccagcagacgctgcttctccttctcgctggtagctagggaggcaaactgctgcagctgcagaggcgttggtggcgtggtgatgtccaggtagtacttgaaggcctggaagatggtgcagggcgggaggcggagctcgtctgtccagttactgatgacacctaaagccgtgttccgctcctccagcagttccactttcaccatctggttgacaggcggcgcgtcctccagccgctcgatcagggcattcacgaggtcctcgtggttgccagggaagacacccaggtggtccccaggctggtactgcagctcctggctcccgttggtgtggagacgcacgaagatagttgaccgactggatttagggctctggaggttttgacggctaaggagccgggcagctgagactcgctttttgtggacattggatagaccttgtgtgagttctggagcttcggccacaaaggtgaggcggaacttgtttctcttccagctgcgatcattgctgatgagggaattgttggccttttcaatgttgacatcatctcccacacagaagacatcacaggctgccttgaagaccttcttggcccaggtcctgaaagcctcttcctgcccacagagctcatccccttccctcatcttcaggatcctctcccctcccagttcttccaggagggtgtccacagcgtgtccgaaggcgcaaaagtgagggtatgctcgtgagccgaggccaaaaactgagaacctcacattggccaggggtccagcactctcaaagttgtctctgaggtcgggcccatcgcctgatgatttttgggagtcagagtaggaggagacgctgttgaatcggaccttgtagctcttcctttcttcctgcacagagttggggtgcctcatttccatcaaagcacagccgaatttctccccattctcagggggatctccattgccaaaggtgctggtgaccacaaggaccagagtttcatgttccaggtgcacaatgtcatattcttccatggacatcaccttggcatcaaaggcgtgtttgaagatctcacacaaggtcttggcataagcttgcgatttgcctgtctctgtggcatagaggatggtcgctttcaccctcttggccatagcctgccccatcagcttggccgagaacttgacagcttctgctagcttcttgaagccaatggctcgccgctttgtgggggtcccgttggtgcctttccagacatgcgtgttccagggatcaggctggtattcgaaggagggggtgagccggtagttgagcatctcctggtggaacacaggggtgatgcttccggacatggggggcacgatccacacccagtcggcagggcagcccccccggcagcggtactcattctccatgtgcttaatgaaggactcggtggcggagtgatggtcaacaatggtcactttgtcactctggaagctatagagaaccgcgatattgatctccaccagcgcctggtccttccacagggaggacgtcttcctcatgtctaagttcatcttcttggccacttcctccaggatattgtagcgggagttgtcacagtagtcgcggacaccaatctctgtgcccatgtaccagccactgaagggacaggcgctgaactccaggccgccaatctctaggagcatgttggacacggcggggaggccgtaccacttcagccccaggtccttgaaccactcaaacttggggtgcctgatgggaacttccaacaccagctctggaggaatctggaagagctcagggtcattgccgttggcctgaagcaggagcggcaggacatcgaagcggcctctaggcggtttccagccctgctgtatgcatatctctgtgaactgcacattggctgggtcccccagggtggagccgtcaggctgcttgtagccagcgtagcggatgagctgggagttccagactcggaagtcgtgcttgccgtctgtcctctgggggaatatggtgatggcagacctgaggttccctttgttggtggcatacttgacatggttacagatgtagttgaacatcccgtgggccgtggtgcagtcacgggcatcgaatacctgcagcttggaccactggatcctgcccacacagcgcgaggcattccgccaggcgtgcttggccccatagatgagctctgtgtccttgagctggtaagtgctagtggtgtcgatctctttgttcacctcttccagcctttccatgtgggctttggagccaaatcttttaattgatgaatagtattgatcaataaactctttggcgagagggaagagctgtccttttgtgcggacgtcttcaggcctccttgcatgctgagaaggatgcatgatggagcccatgcagatgtactcagtgcatcccgtttccaatgtgctcttaaggtggagggtgtcagtgagaaccacctcagtctcccagttcttgaccttgaggaagcgtggacacttggaggggctgccattctttgtgggggactgttttcctgaggtggggggctgctccttctctgaatatgggttgttgaggacgacaggcacattgcccttcccccataggtcattgaagactcggtcgttctccacgccgaggggcagaggtttgtgtgacttgccgtccaaatctctgtccacctggattcccatatctttcatctctgccttggcaggtgcccctcccttgacccctctgctcccactggtgagaaggctcagcacaggctctatctccttgagcagttcattgttctcccctctgccttggaggctgactctggttgctttcttcgcggggtcctggcctgggggcctgggggccaggccgttggcatgggggagtgagccagcctcctgcccatcatcgtaggcatgctgaggcccattcccgggacccgaggccccatccactgccaggggctgttctttgccggccggtggctggtgggacagatccacggctttggtggggggacccaggggctgtgtcacccggatggtcttgggggtcccatcacctgtaaaggtggtctccaggtgcgtggtgaaaccttcagggcccctcagaatgaggaccacgtgggtctcagaggcaatgcctctgagtacctccagggcgctgtcatagctcaggtccaccaagggccggccgttgaccgcaagaatgatgtctccggcctggatgaggccactctgctctgcggcgcccccacgaatcaggtcagagatgatcacgggcggcttactgacccgctccttcaccagaaatcccaggcccccaactttgcgcttgaagagacgaacagaaatgacattgggctggatttgctgaacaccgaacatgtgatcctccatggtaactagcttccgaggggtcctgtctgaagacctcacaatgctatcaggccaagatgatttcaccaggaggatccaggcttcaggctacacggagagcaggagccggggtgacaggtgctgacaaggcttcagccctctctgtctttgacgtcagctcagcgtcacccactcatggctggtggcccgtcggtggcatgatttcctgcatccgcctctctccttattctctaaggaagtgatggttgaccaggcagacgtcaagagaggcggtgggacgtgtccctaaggtcaggcagaaaggggaggagatgcgtctgatggctgtgtctagaagtgacgcatgatagatgtgaactattctctgggtatcttcattgccagcctgttagatgcggatcagatctgaggcatcatgagcccgtccgctcggccgctgctcgctgcccggccgcccctcggaggagccgcggcgctaagtagctcctcacccagcggctggaaacgcggcataaatatgtagggactgagccgt

SEQ ID NO: 13540 - RNA, 9924 nt, Homo sapiens
  source 1..9924: mol_type = other RNA
gctgggattacaggcatgagccaccacgcctggcctgggaggggtttttgaaagcatactgccctccccatgccccctcccccggacaccctcaaatcccactttggcagcagataatggaaacaaccactgggctaggcaaagtttctgctgcgtgctccaggaaatctataatgagaagtcctggggtagccagcagagattctcttgaccctgaagtccaagagaggggtgttgccccctggggacattgggcaatgtctgatgacatacttgattgttaccgttggcaggacactgctacaggtatcttgtggatggaggccaggaatgctgctcagcttcctacagtacccaagacggcccccacaagaaagaattacccagccccaaatgccaatagtgctaaggttgacagaccctgcgctacagtctcctagaacttaggagtcaaatctgggcacttcgatgtcctggagttactttctaaaagactacaggaagcagtgcatggaggcagatttgttcccgcctgccagggccatctcgttaataacggactgtgttttgggccagacgggcatagccccgcttgaccagaactgtttgggtattttagaacaaaacaaactcatataaacatactaaggcatattgacagctgaccacctccctcgcacatggctttgataagtattaataggaaacagactctcgacagacactgctttccacgggtgaaagtgtacctgggtccttacatttggggaagggcagcttttcttttggggcccctttgccacaaggcagggactggcagtgggccaaggatagggagtgtgagataaagggcagaggccaggccaggttggcctccaaagtcaaatccctgttcatggggaacatctatgttgactccctgggaggcaggccccttccctcagaccctcagacctgtgtttccttaatcccagcacctggtctttcattttaattttttttagagacagggtcttgctctgtcactcaggctggagtgcagtggtgcgatcctagctcactgtcgcctcaaactcctgggaccaagtgatcctcctgcctcagcctcccaagtagctgggaccacaggagcatgccatcatgcccagctaatttttttttttttttttttttagtagagacgagattgcgctgtgttgcccaagctggtctcaaactcctggccccaagtgatcctcccacctcagtctcccaaagtgctattacaggcatgaaccaccatgcctggcctactttttgagccaaagaggacatttggatgcaggagactatgaaggttggggacagccagagagtatgaatgggttataaaggaagactagttagtgtttctctctccttgttgcttcctggcagtctcagactacattcctgatacagacagaaggctttgaggacatggtggccacagcggcatgctgggtatgtggggcagcgggtagggaaatatacaaggaaacatggctggtttaaaacacaggctagaagtccacagatttcctaatggcaagaatgaaaaggctgcattaggcgctggtgctgtcggagtgaaggggctcaggcatctggattgcccatcctattaggaccatttgccctatgagctaggtcaggacacctctcacttgttttgagcttagggcaagacctgacctctttcaaagtccagagcaggcagctgctgaaagcgtgtttggtcagaagattctgtgttcttagccaatgtctactggctgggggtcagttttccctccgggcatctgggcatggctggacttgggaaggattcaccctgttgactccagagaagctgactatcacatcagctctgaaaactcatcttttccctgagcctgctcttcagagacctctctctcagctaggggcaagatgttttattttattttattttattttattttttttgagataagagtcttgctctgtcacccaggctggagtgcagtggtacaatcttggctcactgcagcctccacctcctgggctcaagcgatcctccttcctcagcctcccaggtagctgagactacaggcgcatgccaccatgcccagctaatttttgtattttcttagtagagtcagggtttctactaactggctgactggtctccaactcctgacctcaactgatacacccacctcggcctcccaaagtgctgggattacagacatgagctaccgcgcccagcctgcaagatgctttaatttctcctttattctcaccctctacaatggatggggtgccaggtacgctgattcagttcctggagtctctttatcactacatccgcctcttccctcactcaagccttggttgcagcaataacccccccaacagctcaacgggccatgctctgtactgtggccagaactttcttttccaagtataactccaatcgccttaatgtccctttttgaaaaacattcttagggactccctgttgccttctgaataaagcctaaatttcttgtaatgccactcacctctccccacggtctggtcccagcccaccttttctcaccctcctcagccttccaaagccagcctcaatttatcttacatgctccctgtccgtgcctttcctctcactcttcccaattcctggacaactcttaccttccagaagctaccagtgaaatcccgcccatttctcaaaccccagaaatttatgtcagttccaagacgggtgtctctctccatcagattataacctttggctgggcgtggtggctcatgcctgtaatccagcactttgggaggctgaggtgcgtggatcatttgaggtcaggaattcaagaccagcctggccaacatggtgaaaccctgactctactaaaaatacaaaacttagctgggcgtggtggtaggcgcctgtagtcccagttactcaggaggccgaggcagaagaatcacttgaactgggggaggcagaggatgcagtgagctgagatcgtaccactgtacgccagcctgggtgacagagcaagactctgtcaaaaaaaaaaatagattctaaccttctgcacgagaggaactgtgttttgcttatctctgcaaactgcccggtgccttccacacactggagaagcaagacatgttataagttaagtgaaaaattaaaatgcagtaagttttgaaccaggtactgtaactgggcatttcgtgggcattgtctcattcaatccaccttgttatacaggtgggtatgcagactctaaaaggtcaagtgagccgcccacagccatctgcaccaacaggggcagaattaggatttgcactcaggtcggctcccaaaattccatattgatgggtctgaagtgtccccccgcaaaagaaagacacctggctgtctcactccagggaaaccaaaagaagccctctctcctcccaaggagtttaacatcatctctctgctctttcacgacacaagctgtgggaactggatgcatagtgatggcaggtgagcatgatgttccggtgttcctatttcaggagacgtctcattcctcctggccaaactcacttttgtgaaatggggctggagctgctactggtcaattcagggggaagagggaaataaatgggccataacccgaataacccccaaatatcttgtcaaccctattttgcttacccattgcttaattctattttgcacttaaacggttggctacgaggcctggatgaaaagccaccacgagagggcagtatttccccacccttgatctgagcctaacaatctggactccactctggtccttgagaggttactcaacagagagagaggcttttggtatcaggaattctggcaaatgaaagaaacacatcagatcgctctcctgccttctagcctggagttgtgaagcagcttgtgttggggattgaaaggtgtttacttaaaaaaaaatctttctggagaagaaggatgaatcctggttttataatcatttctttggactccttgacaaaatgagacaatgtttccatctgtctgctactagaaaggcaggcacatgcagaaaggaggtgcctggcaccttgtaagcgcttctaagtatttattccctgatggaaaagcattcctgcataaagcttgacttggagtgggaagcactgatcaatttgtctttaatggggattggacacaacagtttccttccctggggaattggggaggcgtctccaaagctataaaggattggaaagaaagcctttgggaggaaagctactaggagctggaaatgggtttgcaggaaaggagtttagaatgggcttcccttcaggattagaaggggtgagtgtgggatgctaagtgtttgttctttatatctgtggaagagtgagcaggggaaattgggattaaaggaaggcaggggagattatagctggcatgaagtcaagctccatgtggcaggaacaggacaccggtgggggctgccagggatggcagagcaaggtgagtcatagattgccttttcactttaacagtctcctggcctgggccctttggggtcttggtgcccccactgtaaagccctttcaaagagggccagtgcacttcctctttagcagacacccaaactgaacaacaagatatgcccacgtacagtatataaaagaaatgtggtttttctgtatagcaagacacaacaaacagggtagaaccagcagaacattccctttccatccttggggaccctgcagtctgggaggccactaggatttcttgtctctttctgggaactgcctgacactaatttgtagtatttaaaaaagtatacaaagggatcccttcccaccatttactctgagagagtaaattcaacaggttgcctcttagggaggaattacaccggctccaattcctaccgaagacttggctgcccatttttgatctgagttgagggtaacttatttgtcaaaattaatttaacaggtttaaaactttggagatcaactgcagagggcaacaagcctgagggacaagttcttcccaccccaagttgtggctcctatcgaagaagccacgtgggacctcattatggcaactctttccaacctcatccactttaaccagcttccattatttcatccccaagggtgaagcagcaagcccgctttgggggaataaaaaaataataatcatattgttacttgatattgtttccaggcaccaaagctttaacatttaatccattcatattctttaggttcgtatgacattatgactaggaaaaactgaggacaagtgacccatccaaagtcatccagtggcaaagtgggaagatccttattgccaccaggcttctttgaacaacataacttccaggccccttggatgctattgctggaggagggggtcagtcaatggatgtggcaaagtcaagtgattctagctggtatgggtgggtttggggaggggatttgcacaatccattggatgggttcatgtcacatgagggctctgctcactggtatcaaaatctaaatgcagcaaattctgggaatgcctctttcattgggagacagcccctttaatcaatttcccactcctctccccatgccctgaaccctttctaactagaacaattatggggcttccaaatgtttcaggtacatgggcgtggaccctaattatggacacacgagggattaatatgggccagggacacgtttcttggcattgagggtcttcaatgaaagcagtggcaatctaagatcgacacacttgtgcagggaagaggacggacagagacctggcccatcacacacacacacacacacacacacacacacacaggcacgcacaaccaaaatgtcatcataaaaaaggagaaagggggacttcagtggctgagggactggctcagagagcttgtgcctagttcctgcagcctttccaggggaaccccagagaaaaaaacccccacagcgacggccatgttccagtggtttcatgcacccgtgagttgcccttgtcggcaagagagggagtgggaacagagttttgtaagagccactgcagattagaaaagcattgcatcgcagcaggaaaactcaaggagtaaacccaggagggccgaggaaaccactgaggggcgagaagcccgaggagggaaaccagggcacagcgacaaggacaggaggcagagcgagggccacagggggtcccagaggaaaggttcagcagtgtctgtccgcgcttacaaaacttgcagccggctgggcaagagggtccagttaggagctgaaaacctcatcggtgtcttttttgctctcttcaatgaaggcaatggactcagatctaaggcggttggtcacttcgtacgttcgcagggtgactccaaaaatatcctcatggtatcggttgtcatccctcatccggctgatgaatacgccggcgtcctctgccgagagcttcccctgctgggtcatgatgcgctggatggctttgaggacatcagcagccatggtgacgtccccacagacgtatatgtggcccccttgctccttcagggctcggtacacagactccgccagctgctcctgcaggatgtcctgcacgtacttctttggtttgtctggctcccgggagtaagccgtgtacagctctctgaagacccccttgttcttggcctgcagggtctcttccctgtagatatgatctatcttggattgccggcacccgaagaccaggaccatggggcaggggttcattcctttgtgttggatatcaaattgccgctgttgccagaagcttcggaaaggggcaatgccggtgcctggtccaacgaggatgcaggggacttgggggttccggggcaggtggaagctgggtgctcctctcacgaaacaggggaccagttcgtcagcctgtatccggttgagccaggaggagcatacgccgtggtgaattggtccttctccatctcgagtgcggtaggaaacgatggccacagtgaggtgcacttcatcagggtacatgtctggggaggagctgatggaatagtagcggggctgcagcagggacagctgggtcaggagcagggtggccggcatctggatagatgggaactcctccagcacctccacgatggtggggttcttgccccatttccattcctcgtactcctgcaaacccttgctgaggaccagcagacgctgcttctccttctcgctggtagctagggaggcaaactgctgcagctgcagaggcgttggtggcgtggtgatgtccaggtagtacttgaaggcctggaagatggtgcagggcgggaggcggagctcgtctgtccagttactgatgacacctaaagccgtgttccgctcctccagcagttccactttcaccatctggttgacaggcggcgcgtcctccagccgctcgatcagggcattcacgaggtcctcgtggttgccagggaagacacccaggtggtccccaggctggtactgcagctcctggctcccgttggtgtggagacgcacgaagatagttgaccgactggatttagggctctggaggttttgacggctaaggagccgggcagctgagactcgctttttgtggacattggatagaccttgtgtgagttctggagcttcggccacaaaggtgaggcggaacttgtttctcttccagctgcgatcattgctgatgagggaattgttggccttttcaatgttgacatcatctcccacacagaagacatcacaggctgccttgaagaccttcttggcccaggtcctgaaagcctcttcctgcccacagagctcatccccttccctcatcttcaggatcctctcccctcccagttcttccaggagggtgtccacagcgtgtccgaaggcgcaaaagtgagggtatgctcgtgagccgaggccaaaaactgagaacctcacattggccaggggtccagcactctcaaagttgtctctgaggtcgggcccatcgcctgatgatttttgggagtcagagtaggaggagacgctgttgaatcggaccttgtagctcttcctttcttcctgcacagagttggggtgcctcatttccatcaaagcacagccgaatttctccccattctcagggggatctccattgccaaaggtgctggtgaccacaaggaccagagtttcatgttccaggtgcacaatgtcatattcttccatggacatcaccttggcatcaaaggcgtgtttgaagatctcacacaaggtcttggcataagcttgcgatttgcctgtctctgtggcatagaggatggtcgctttcaccctcttggccatagcctgccccatcagcttggccgagaacttgacagcttctgctagcttcttgaagccaatggctcgccgctttgtgggggtcccgttggtgcctttccagacatgcgtgttccagggatcaggctggtattcgaaggagggggtgagccggtagttgagcatctcctggtggaacacaggggtgatgcttccggacatggggggcacgatccacacccagtcggcagggcagcccccccggcagcggtactcattctccatgtgcttaatgaaggactcggtggcggagtgatggtcaacaatggtcactttgtcactctggaagctatagagaaccgcgatattgatctccaccagcgcctggtccttccacagggaggacgtcttcctcatgtctaagttcatcttcttggccacttcctccaggatattgtagcgggagttgtcacagtagtcgcggacaccaatctctgtgcccatgtaccagccactgaagggacaggcgctgaactccaggccgccaatctctaggagcatgttggacacggcggggaggccgtaccacttcagccccaggtccttgaaccactcaaacttggggtgcctgatgggaacttccaacaccagctctggaggaatctggaagagctcagggtcattgccgttggcctgaagcaggagcggcaggacatcgaagcggcctctaggcggtttccagccctgctgtatgcatatctctgtgaactgcacattggctgggtcccccagggtggagccgtcaggctgcttgtagccagcgtagcggatgagctgggagttccagactcggaagtcgtgcttgccgtctgtcctctgggggaatatggtgatggcagacctgaggttccctttgttggtggcatacttgacatggttacagatgtagttgaacatcccgtgggccgtggtgcagtcacgggcatcgaatacctgcagcttggaccactggatcctgcccacacagcgcgaggcattccgccaggcgtgcttggccccatagatgagctctgtgtccttgagctggtaagtgctagtggtgtcgatctctttgttcacctcttccagcctttccatgtgggctttggagccaaatcttttaattgatgaatagtattgatcaataaactctttggcgagagggaagagctgtccttttgtgcggacgtcttcaggcctccttgcatgctgagaaggatgcatgatggagcccatgcagatgtactcagtgcatcccgtttccaatgtgctcttaaggtggagggtgtcagtgagaaccacctcagtctcccagttcttgaccttgaggaagcgtggacacttggaggggctgccattctttgtgggggactgttttcctgaggtggggggtggttatgtgaccctcgttgagcaccaaaaccctctgtgattctcagtttcctcatcacagaatccctgatgtccttatcttcctggccagccatcagcggctaaggaaagcagttaccaccaaggctctagaatgtctcatcctccccg

SEQ ID NO: 13541 - RNA, 9929 nt, Homo sapiens
  source 1..9929: mol_type = other RNA
gctgggattacaggcatgagccaccacgcctggcctgggaggggtttttgaaagcatactgccctccccatgccccctcccccggacaccctcaaatcccactttggcagcagataatggaaacaaccactgggctaggcaaagtttctgctgcgtgctccaggaaatctataatgagaagtcctggggtagccagcagagattctcttgaccctgaagtccaagagaggggtgttgccccctggggacattgggcaatgtctgatgacatacttgattgttaccgttggcaggacactgctacaggtatcttgtggatggaggccaggaatgctgctcagcttcctacagtacccaagacggcccccacaagaaagaattacccagccccaaatgccaatagtgctaaggttgacagaccctgcgctacagtctcctagaacttaggagtcaaatctgggcacttcgatgtcctggagttactttctaaaagactacaggaagcagtgcatggaggcagatttgttcccgcctgccagggccatctcgttaataacggactgtgttttgggccagacgggcatagccccgcttgaccagaactgtttgggtattttagaacaaaacaaactcatataaacatactaaggcatattgacagctgaccacctccctcgcacatggctttgataagtattaataggaaacagactctcgacagacactgctttccacgggtgaaagtgtacctgggtccttacatttggggaagggcagcttttcttttggggcccctttgccacaaggcagggactggcagtgggccaaggatagggagtgtgagataaagggcagaggccaggccaggttggcctccaaagtcaaatccctgttcatggggaacatctatgttgactccctgggaggcaggccccttccctcagaccctcagacctgtgtttccttaatcccagcacctggtctttcattttaattttttttagagacagggtcttgctctgtcactcaggctggagtgcagtggtgcgatcctagctcactgtcgcctcaaactcctgggaccaagtgatcctcctgcctcagcctcccaagtagctgggaccacaggagcatgccatcatgcccagctaatttttttttttttttttttttagtagagacgagattgcgctgtgttgcccaagctggtctcaaactcctggccccaagtgatcctcccacctcagtctcccaaagtgctattacaggcatgaaccaccatgcctggcctactttttgagccaaagaggacatttggatgcaggagactatgaaggttggggacagccagagagtatgaatgggttataaaggaagactagttagtgtttctctctccttgttgcttcctggcagtctcagactacattcctgatacagacagaaggctttgaggacatggtggccacagcggcatgctgggtatgtggggcagcgggtagggaaatatacaaggaaacatggctggtttaaaacacaggctagaagtccacagatttcctaatggcaagaatgaaaaggctgcattaggcgctggtgctgtcggagtgaaggggctcaggcatctggattgcccatcctattaggaccatttgccctatgagctaggtcaggacacctctcacttgttttgagcttagggcaagacctgacctctttcaaagtccagagcaggcagctgctgaaagcgtgtttggtcagaagattctgtgttcttagccaatgtctactggctgggggtcagttttccctccgggcatctgggcatggctggacttgggaaggattcaccctgttgactccagagaagctgactatcacatcagctctgaaaactcatcttttccctgagcctgctcttcagagacctctctctcagctaggggcaagatgttttattttattttattttattttattttttttgagataagagtcttgctctgtcacccaggctggagtgcagtggtacaatcttggctcactgcagcctccacctcctgggctcaagcgatcctccttcctcagcctcccaggtagctgagactacaggcgcatgccaccatgcccagctaatttttgtattttcttagtagagtcagggtttctactaactggctgactggtctccaactcctgacctcaactgatacacccacctcggcctcccaaagtgctgggattacagacatgagctaccgcgcccagcctgcaagatgctttaatttctcctttattctcaccctctacaatggatggggtgccaggtacgctgattcagttcctggagtctctttatcactacatccgcctcttccctcactcaagccttggttgcagcaataacccccccaacagctcaacgggccatgctctgtactgtggccagaactttcttttccaagtataactccaatcgccttaatgtccctttttgaaaaacattcttagggactccctgttgccttctgaataaagcctaaatttcttgtaatgccactcacctctccccacggtctggtcccagcccaccttttctcaccctcctcagccttccaaagccagcctcaatttatcttacatgctccctgtccgtgcctttcctctcactcttcccaattcctggacaactcttaccttccagaagctaccagtgaaatcccgcccatttctcaaaccccagaaatttatgtcagttccaagacgggtgtctctctccatcagattataacctttggctgggcgtggtggctcatgcctgtaatccagcactttgggaggctgaggtgcgtggatcatttgaggtcaggaattcaagaccagcctggccaacatggtgaaaccctgactctactaaaaatacaaaacttagctgggcgtggtggtaggcgcctgtagtcccagttactcaggaggccgaggcagaagaatcacttgaactgggggaggcagaggatgcagtgagctgagatcgtaccactgtacgccagcctgggtgacagagcaagactctgtcaaaaaaaaaaatagattctaaccttctgcacgagaggaactgtgttttgcttatctctgcaaactgcccggtgccttccacacactggagaagcaagacatgttataagttaagtgaaaaattaaaatgcagtaagttttgaaccaggtactgtaactgggcatttcgtgggcattgtctcattcaatccaccttgttatacaggtgggtatgcagactctaaaaggtcaagtgagccgcccacagccatctgcaccaacaggggcagaattaggatttgcactcaggtcggctcccaaaattccatattgatgggtctgaagtgtccccccgcaaaagaaagacacctggctgtctcactccagggaaaccaaaagaagccctctctcctcccaaggagtttaacatcatctctctgctctttcacgacacaagctgtgggaactggatgcatagtgatggcaggtgagcatgatgttccggtgttcctatttcaggagacgtctcattcctcctggccaaactcacttttgtgaaatggggctggagctgctactggtcaattcagggggaagagggaaataaatgggccataacccgaataacccccaaatatcttgtcaaccctattttgcttacccattgcttaattctattttgcacttaaacggttggctacgaggcctggatgaaaagccaccacgagagggcagtatttccccacccttgatctgagcctaacaatctggactccactctggtccttgagaggttactcaacagagagagaggcttttggtatcaggaattctggcaaatgaaagaaacacatcagatcgctctcctgccttctagcctggagttgtgaagcagcttgtgttggggattgaaaggtgtttacttaaaaaaaaatctttctggagaagaaggatgaatcctggttttataatcatttctttggactccttgacaaaatgagacaatgtttccatctgtctgctactagaaaggcaggcacatgcagaaaggaggtgcctggcaccttgtaagcgcttctaagtatttattccctgatggaaaagcattcctgcataaagcttgacttggagtgggaagcactgatcaatttgtctttaatggggattggacacaacagtttccttccctggggaattggggaggcgtctccaaagctataaaggattggaaagaaagcctttgggaggaaagctactaggagctggaaatgggtttgcaggaaaggagtttagaatgggcttcccttcaggattagaaggggtgagtgtgggatgctaagtgtttgttctttatatctgtggaagagtgagcaggggaaattgggattaaaggaaggcaggggagattatagctggcatgaagtcaagctccatgtggcaggaacaggacaccggtgggggctgccagggatggcagagcaaggtgagtcatagattgccttttcactttaacagtctcctggcctgggccctttggggtcttggtgcccccactgtaaagccctttcaaagagggccagtgcacttcctctttagcagacacccaaactgaacaacaagatatgcccacgtacagtatataaaagaaatgtggtttttctgtatagcaagacacaacaaacagggtagaaccagcagaacattccctttccatccttggggaccctgcagtctgggaggccactaggatttcttgtctctttctgggaactgcctgacactaatttgtagtatttaaaaaagtatacaaagggatcccttcccaccatttactctgagagagtaaattcaacaggttgcctcttagggaggaattacaccggctccaattcctaccgaagacttggctgcccatttttgatctgagttgagggtaacttatttgtcaaaattaatttaacaggtttaaaactttggagatcaactgcagagggcaacaagcctgagggacaagttcttcccaccccaagttgtggctcctatcgaagaagccacgtgggacctcattatggcaactctttccaacctcatccactttaaccagcttccattatttcatccccaagggtgaagcagcaagcccgctttgggggaataaaaaaataataatcatattgttacttgatattgtttccaggcaccaaagctttaacatttaatccattcatattctttaggttcgtatgacattatgactaggaaaaactgaggacaagtgacccatccaaagtcatccagtggcaaagtgggaagatccttattgccaccaggcttctttgaacaacataacttccaggccccttggatgctattgctggaggagggggtcagtcaatggatgtggcaaagtcaagtgattctagctggtatgggtgggtttggggaggggatttgcacaatccattggatgggttcatgtcacatgagggctctgctcactggtatcaaaatctaaatgcagcaaattctgggaatgcctctttcattgggagacagcccctttaatcaatttcccactcctctccccatgccctgaaccctttctaactagaacaattatggggcttccaaatgtttcaggtacatgggcgtggaccctaattatggacacacgagggattaatatgggccagggacacgtttcttggcattgagggtcttcaatgaaagcagtggcaatctaagatcgacacacttgtgcagggaagaggacggacagagacctggcccatcacacacacacacacacacacacacacacacacaggcacgcacaaccaaaatgtcatcataaaaaaggagaaagggggacttcagtggctgagggactggctcagagagcttgtgcctagttcctgcagcctttccaggggaaccccagagaaaaaaacccccacagcgacggccatgttccagtggtttcatgcacccgtgagttgcccttgtcggcaagagagggagtgggaacagagttttgtaagagccactgcagattagaaaagcattgcatcgcagcaggaaaactcaaggagtaaacccaggagggccgaggaaaccactgaggggcgagaagcccgaggagggaaaccagggcacagcgacaaggacaggaggcagagcgagggccacagggggtcccagaggaaaggttcagcagtgtctgtccgcgcttacaaaacttgcagccggctgggcaagagggtccagttaggagctgaaaacctcatcggtgtcttttttgctctcttcaatgaaggcaatggactcagatctaaggcggttggtcacttcgtacgttcgcagggtgactccaaaaatatcctcatggtatcggttgtcatccctcatccggctgatgaatacgccggcgtcctctgccgagagcttcccctgctgggtcatgatgcgctggatggctttgaggacatcagcagccatggtgacgtccccacagacgtatatgtggcccccttgctccttcagggctcggtacacagactccgccagctgctcctgcaggatgtcctgcacgtacttctttggtttgtctggctcccgggagtaagccgtgtacagctctctgaagacccccttgttcttggcctgcagggtctcttccctgtagatatgatctatcttggattgccggcacccgaagaccaggaccatggggcaggggttcattcctttgtgttggatatcaaattgccgctgttgccagaagcttcggaaaggggcaatgccggtgcctggtccaacgaggatgcaggggacttgggggttccggggcaggtggaagctgggtgctcctctcacgaaacaggggaccagttcgtcagcctgtatccggttgagccaggaggagcatacgccgtggtgaattggtccttctccatctcgagtgcggtaggaaacgatggccacagtgaggtgcacttcatcagggtacatgtctggggaggagctgatggaatagtagcggggctgcagcagggacagctgggtcaggagcagggtggccggcatctggatagatgggaactcctccagcacctccacgatggtggggttcttgccccatttccattcctcgtactcctgcaaacccttgctgaggaccagcagacgctgcttctccttctcgctggtagctagggaggcaaactgctgcagctgcagaggcgttggtggcgtggtgatgtccaggtagtacttgaaggcctggaagatggtgcagggcgggaggcggagctcgtctgtccagttactgatgacacctaaagccgtgttccgctcctccagcagttccactttcaccatctggttgacaggcggcgcgtcctccagccgctcgatcagggcattcacgaggtcctcgtggttgccagggaagacacccaggtggtccccaggctggtactgcagctcctggctcccgttggtgtggagacgcacgaagatagttgaccgactggatttagggctctggaggttttgacggctaaggagccgggcagctgagactcgctttttgtggacattggatagaccttgtgtgagttctggagcttcggccacaaaggtgaggcggaacttgtttctcttccagctgcgatcattgctgatgagggaattgttggccttttcaatgttgacatcatctcccacacagaagacatcacaggctgccttgaagaccttcttggcccaggtcctgaaagcctcttcctgcccacagagctcatccccttccctcatcttcaggatcctctcccctcccagttcttccaggagggtgtccacagcgtgtccgaaggcgcaaaagtgagggtatgctcgtgagccgaggccaaaaactgagaacctcacattggccaggggtccagcactctcaaagttgtctctgaggtcgggcccatcgcctgatgatttttgggagtcagagtaggaggagacgctgttgaatcggaccttgtagctcttcctttcttcctgcacagagttggggtgcctcatttccatcaaagcacagccgaatttctccccattctcagggggatctccattgccaaaggtgctggtgaccacaaggaccagagtttcatgttccaggtgcacaatgtcatattcttccatggacatcaccttggcatcaaaggcgtgtttgaagatctcacacaaggtcttggcataagcttgcgatttgcctgtctctgtggcatagaggatggtcgctttcaccctcttggccatagcctgccccatcagcttggccgagaacttgacagcttctgctagcttcttgaagccaatggctcgccgctttgtgggggtcccgttggtgcctttccagacatgcgtgttccagggatcaggctggtattcgaaggagggggtgagccggtagttgagcatctcctggtggaacacaggggtgatgcttccggacatggggggcacgatccacacccagtcggcagggcagcccccccggcagcggtactcattctccatgtgcttaatgaaggactcggtggcggagtgatggtcaacaatggtcactttgtcactctggaagctatagagaaccgcgatattgatctccaccagcgcctggtccttccacagggaggacgtcttcctcatgtctaagttcatcttcttggccacttcctccaggatattgtagcgggagttgtcacagtagtcgcggacaccaatctctgtgcccatgtaccagccactgaagggacaggcgctgaactccaggccgccaatctctaggagcatgttggacacggcggggaggccgtaccacttcagccccaggtccttgaaccactcaaacttggggtgcctgatgggaacttccaacaccagctctggaggaatctggaagagctcagggtcattgccgttggcctgaagcaggagcggcaggacatcgaagcggcctctaggcggtttccagccctgctgtatgcatatctctgtgaactgcacattggctgggtcccccagggtggagccgtcaggctgcttgtagccagcgtagcggatgagctgggagttccagactcggaagtcgtgcttgccgtctgtcctctgggggaatatggtgatggcagacctgaggttccctttgttggtggcatacttgacatggttacagatgtagttgaacatcccgtgggccgtggtgcagtcacgggcatcgaatacctgcagcttggaccactggatcctgcccacacagcgcgaggcattccgccaggcgtgcttggccccatagatgagctctgtgtccttgagctggtaagtgctagtggtgtcgatctctttgttcacctcttccagcctttccatgtgggctttggagccaaatcttttaattgatgaatagtattgatcaataaactctttggcgagagggaagagctgtccttttgtgcggacgtcttcaggcctccttgcatgctgagaaggatgcatgatggagcccatgcagatgtactcagtgcatcccgtttccaatgtgctcttaaggtggagggtgtcagtgagaaccacctcagtctcccagttcttgaccttgaggaagcgtggacacttggaggggctgccattctttgtgggggactgttttcctgaggtggggggtggttatgtgaccctcgttgagcaccaaaaccctctgtgattctcagtttcctcatctgcattcgtcctgcttcaattgcattctattgccttttgcccagtccttggcagttgctttgctgccctgcccagccatttctcaacccccacctatc

SEQ ID NO: 13542 - RNA, 88 nt, Homo sapiens
  source 1..88: mol_type = other RNA
gctgggattacaggcatgagccaccacgcctggcttcaaaaagacctgtttctaccacttcggttttgtggatgagtctgttgtaaat

SEQ ID NO: 13543 - RNA, 4310 nt, Homo sapiens
  source 1..4310: mol_type = other RNA
gctgggattacaggcatgagccaccacgcctggcttgtggttgaaatcttaacccacaatatgatggtgttgggatgtggagcctttgggaggtgattagataatgaaggtggagacctcaagaatgggattagtgacattctttaaaaggccctggagactgggtacagtggctcatgcctgtaatctcagcactttgggaggctgaggtgggcagatcacttgaggtcaggagtttgagaccaacctggccaatatggtgaaacccagtgtctacaaaaatacaaaaattagctgggcatggtggtgcatccctgtagtcccagctcctcaggaggctgaggcaggagaattgcttgaactcaggaggcagagagaggcagaggttgcagtgagccgagattgtgccactgcactccagcctgggcgacagagccagactccatctcaaaaaaaaaaaaaaaaaaaaaaaaatggccctggagagctgtctcccatcttctacgataagaggacacagctagaaggcactgtctttgaaaaagtgggccctcatcagacagcactggtggcttgatcttggacttcccagtctccagacttgtgagaagaacatttgtttataagttacccagtcttttttttttttttgagatggagtcttgctctgtcacccaggctggagtgcaatggcgtgatcttggctcactgcaacctccgcctcctgggttcaagcgattctcctgcctcagcttcccgaggagctgggattacaggtatgtgcgaccatgcctcgctaattttgtatttttagtagaggaggggcttcgccatgttggccaggctgttcttgaatgcctgacctcaggtgattcatccccctcggcctcccacagtgctgggattacaggcatgagccactgcatccagccaagttacccactcttaaggtattttgttataaccacctgaacaagaacaaagacattctctaagccatgtagtacacattcataaatctggggttttaaataccttcctcctataattgtcacgagggacagattcaagtttcatttggttgaagcttctaaacctggaaggaacctaaaatgagcttcagcttcaaggctaatgtgcctgttctccctccacgtaaagcagaaaatgccagatctcccttgccctgcttgctttgcagggaggatgtgactccacaatccaggttcccccaatctgtggccacacccaggatgaggatcagaagctagtgaccaccagcatcgctcctggtagctgatggcaacgtgagggaaactgcctcatttcacaggtaacagggtcagaagttctgttggcagccaacacagttcccagaccagctctgtgttccaatgtgacttgggttcatttatgtggctaactcaacttccctgtcctttccagaggttccatgagctcttcttttaaacatgtactgggcacttataggctctcatttcctgagctcgggactaaaccctctacacatccagcattcctttactaagcccctttgcccccagagctaggaggtgtggctcacaggcagggatcatcctctgctttcctccaaggcctggaccagaaggaccaagggaagacagttccagcccagagccatttcccttccaacctcttggcaagcctgatgagttccactccccgctgacgggcacacctgccttccaggcactgatcctgctttccccctcttgctctgccactcactgtgcctggcttgctgcccagccctccccagccttctctcctcctacctttcccacttattgcctccttccaggcttgtccagcatgataaactctggtctcagcattcacagcctcctctatctctcagctgtgtccctggtcatgactctgcttgctcttccctaaagcaattaaaataggaaaatctgacccttctcacccaggaggcaggtcctctcctatccactggagacccagagcaaaagctctctcctcccttcatcctccttctcaccatgtgatttcagacaagtcctttcacttccgagttttgccatgtgtgcctgtgtgcatatgtatgtgatgtacagacctctggagccatttcaccacagtgcctctccactcccagccagtgccagggcaccccctcagctgctgcaggatgtgtcaccagaaggagagagttaaaggggaagaaagcccttgagtaggagccaagtcatctgaacgcacaccctgtgcccagaggaggaggggcaagagttgctttccatgaagagtgcacctgatgagaaggcagctccagaggactcaaaggaaaaccaagaatcaagagagaaagaaacgtgcagtccttgcctacttggggagggggaggggtcgtaccacaaactccttggtcaatatagggacctgcttctccgtgcgccccagccccctctgcaccatgcactctcctcccgggcctagcgcctgctacaactgtggcctccactaatttcgggggtgcgaggcggtggatgatgcccaagtgaagccgttcaggcctcgtggcagcaccagatcaagggcgaggttgcgctgctcgtcctcagagtacacaggccggtagcccagcagctgcagcgcaccagcgcacagttcctgcacgcggcggatcttggcaaagggcagcgcatggcgccaggcctgggagacgttgagcgcattcctggacgaagtcttgaaggcttcgcggcgcgcaccaggtccagatccgtgggtgatgttatggatccaggcctcgagctgtggcgtgagactgagcccagtgaaggcgtagagcgcacggatttctgccagcggctcccgcgccaggtcctcgaagcgcaccaggcggtagcggccgcgcagaaagggtggcggcttgagtgtggcggcctcggcgatgcgtacgtggctacggcacacctcgcgcaccacgcgcaggccggggtcggcctccacccacgtgccgttggtgcccagcacgatgccgttgtcacgcgccagagccttggctgtctgctcccgggagcgcagcacggcccgcgggtcgcgcaccaggtgcacgatgcgtaggttgagcgcggggtcgctgagcagcgggtagagcacctgcaggttgaagaagcgcacctccttgagcaccacgtggctgtaggagcggcaggcctcccgggccagggtgaaggactgccgcgcgcacagtggcttgcacacggcctcgctgctgatggcgcctcggggaaaggcactgcaggcgggtggcgagcacagtgcacggctcacggcccactggaagaggtcggacaggttgcggcgccaaggcagataggcatcaaacacgtccatgtcgcacaggaagacggagcgcaccaggtcgcgcacagccatgtgcagcgttgcggcgctgccctgcgacagggtggtccacacgtgccacgcgggctccattaggtagaagacgtcggggtgctggttgaagagttggcccacgaaggacgagcccgagcgccacgaggacagcaccagcacatgcacgcgcgcctcgccgcctgctggggacgagggccctggccgggaaaccagaaagaggaggaggaaggtctgcgccaggaggagcgcggtcactgctgtgctggagacgcgcggcagccacatgctgactgctgggggccactgtccagggctgctgggagagctgcaacgctgatcacaaatccatgggagatgattagaggttcctcagcaccccaaagcttggcggctctgcccgagctgcagcggcacggtgggggacgcctctctccctggactcagcaaaggctcccaaacgtcgtctcttccaaattccaccgcacagccagctctttctcttcactgggagggtccgcaggggctgacttgctccttaaggtcccaagactattaagcgacacccggtgaggccgggaaaggggctctaagaggcatggacgagagttggcggtgaccaagccactggaagctcctggagactcgaggtagaacgaatgtgggaacagggcaggagtcccagaatgggatgttgaggctgggggtgtcctggggctaccacagggaaggacccggcgcagagctccctctggaacccggcactgcggcccgcgccctctactccccgcgcgccggccggcaaccctcggcgctgcccggtgcagcccgcccgagcgcacacaatgaggcgctttcagacgtggctgcggtcccgaggt

SEQ ID NO: 13544 - RNA, 383 nt, Homo sapiens
  source 1..383: mol_type = other RNA
gctgggattacaggcatgagccaccacgctcagctagtgaaataactttggtgataaagttttagtaacacccgccaattggaagtcaggtaaaaaagaagataaagattctgcagtggttatacagagttaaatggctttgactctttcagtgtgcaaggctgtgtacattattttacaaaagtgtttataaaaatttgtaaaataatatttccctctggaatattttatttttacctgtgctcagcgatttctacccttggaaggtatgagatctgcccctatgttctattgatacagtgctgctctagacatttagtctgcagggagattttggtattagaactgaggctgcaatgctagggaatattcctgcagttttt

SEQ ID NO: 13545 - RNA, 890 nt, Homo sapiens
  source 1..890: mol_type = other RNA
gctgggattacaggcatgagccaccacgctcggccaggagggacatttcttaaaacctaggatggtggcactgaaggggccctcagaaaccctgcaggccagctccatcctcccccaggagggaactgcggcgcagagaggctagtgtggaggtgggctgagggcctttcactacgcagctctgcttccttggcgttaatgacctccccgccctgtctctgatcccctgagctgcccacatcagcgctgggcacactcatagctccttggagactggccactgttttccctcggagacagatgaccttcatacacattgtgaaaggtataggcccagacccttctgtgcacatttcactgacactggaagacccggggcccaccgtgggtcacctttgccgtctcacttgtgaatacctgccagtgtcccagtagatgaagccgacagacagctcaggcccagtgaaggtgtgtcccatgggccacgggatctcgcctggcagagatctgctttaagatgccatctccaggagccaaggtcatctccagaatctctccccacatcttcccaacagagcagtgttgagtcagctcccctttttctgcctctccgaggtactctcagccatgccctccttctggctttcgtaggatctgactcaagatccactttaggcaggcagtatctgtggaaccttctcgtgtagggcccacctgattccccgagctggcgccagggctgcggtgcactgtgttagctctgagaggggtgtccctgcccacgccagctctgaatcttgcaagccactgcaccttttgagagttgctcccgaactgcctcctacacaggtggttcccaagcggttcatatcaaggtcccttttattatc

SEQ ID NO: 13546 - RNA, 4221 nt, Homo sapiens
  source 1..4221: mol_type = other RNA
gctgggattacaggcatgagccaccacgctcggcccattactcttaaaattataagatctcacccaaggtggaggaaatcacctaactcatccagggataagaagttctgtcaaagggttggtttattcctttacacacttcacacacacacaatccttcccccacccctgacacccttttcaactatttaaggtctgggggctacttccgggtatttttgggtatcagcagggagacagaaatgagcaggatttatgggagagtcaaatgcccctctcaaaacagttaaaggccttccttataaatggcctctctctgtaaatataaaaactaactataagaatctcaaacggtcagccctaaaagaccaggtcttgtgggattgtagagttggccgctatgaagggaagactggaaaaagtgcctccagagacacggggtggtccacagcctaacagttaaaatgctcatcacttttaagaactttcctaacccctttagttctttgatgctaagcagggaagagggaggcttggagaccagggatgtcctcccaggtggtgctggggcctgggtaaccctcagggttgccctcaggagccctctgcctctggaacaccgtgcttggtaggagttattgaagggctgtgtacagtgagtaagccctttcttgtcagcaaaccttcatcaagtcttcagagcgatactgagggtgctctcatttctctgtggaaaaggctctcctcacagagttcctcagacagtgtcccaggtgatggacatggagacttgggctgagtctgagtaagcatctttgtagtctaaaaatgcagctcatatgaaaatatcagctgtgtaacatcagaagcatgacgcctacaggaagatggcctcgagaaagtcttggaaagaagcactttctgctatcaaaacttgatcatttcccatgagaaaaaatgctcaagaaagttggatggcagcttggcacacttaagagaaagctcactcacaactaaagaacaactgcattctgctacagtaatctgggatgggtatgacagcaccagcataacactggctggagtgtggcaaggagagggagttggcaatctactgatgctggggacattggataccgatttttttctactgttttccagatctttgagttcattctcgatttttgtgattaattccctgagttcatcaagattagtgcaaataagctgaaactctggtacagtaggtgactttatgacagttttcctcttctttgtgattgcttttttagagacggatttttttccagatttgtgcttcttgtgttttgctttttttttgatgatcaataacttattctggatctcaggtttgtaagacttgaatgcaagagaatgaagaccttcacgctttctctgtaagttttcattcaaaacatctttcaatttcttttttttctttttcttcttttttgccctcattttagttagtttgagtttcttgtggctctgtagtgactgctctaatagaatatcccttacaactttgtggcagttaatttctggatgatcactgtgacttccatttacatgtatttggcaagattttagagtattttcttttaatggactgggttcaatctttattctggaagcttcaccgtatttttcctgattttctataaaccttatttcacctggactaagaggctctccaaagccagtaacttcccctggactccttggtttctctaaattttctttacaacaatcagtttttttaatttcacaaggcctgcgaattctaatttcatagttggattttactcccatttcaacagagatgtcatgattatccaagatcattttagcaggacagcaagctggatcaaaattattttcctgctctttcttgaaggaagagggcaggctatctctgctacatctatgttctccattacttgtactaacatagtcacacttcaatttctccaatttaatccgaggtactctttgtattttaatgggtggaattggaaattctggggcctgaaagggtctctgtttataaatccgtacatctgcaccacagaactgtggaaaatgtacataagcattctccaaataatcataaccaagaataacttccctgcattcatggataggctgtccaagtacagcatcttgaacttccttttgtgtttcatacacaaagtcacaaagacccttaagtagccacactttttggtaaaaaggtagttcgtgaaaaggtttttcttccaatggattaacttctccaagaactttaaaaaactgaggacacaaccccagtttttcagcacagttatcaggattttcagtttgccctacagcagtgtaccactgttgtactttctgcctcagcgctgcttcccaggtcctataaggcaaagtaggtcttcgatgtaaggtaggtctgcgatggggaggacttaatagagaagtcattattttcgatagaaaagcattacactgaggcatcagaagacaacgttccaattcgtaaaagactatttctggcaaatttagaatttgctgagctaaacaaaggaaatgcccaatagctggaatttcccacatggtctccatacaagttggagctgcttgagctagaagttttctttcccattcttctatttccttttgactagcttcttctgcttcttttctttcctgctcccgaagccttttttcttcttttgctctcagctgttcttcctgtctcaaaacttgaaccattatagattcaaaaactccacttgtcaagcctgccaaacttcgcggtgttgaccgacgccttgttgaggtacatgcagttcccttctcatcctccaatccataatagcctctagatgtaactgctatcgttgtcttttctctcaagtgccgagagagaagcgctaacttctgctccagcatcatctccagcttctggccctgtttggagatccagtggtccactccgtgcaggcggtagcacgtctccagcatcaacctgaagtccgccacgaactcggtgatgcccccgtactggccgctggcgaacttctcttccatctgcagcagacacatgccctgtccgggctgctgcgggaaggcgcgaccgccccggcccccgctgcgcggcccttccgccacctcctcctccgcggtggcaacgccccccaagggctgcagaaagggggcggtgaggccccggtgcttctcctgcaggaactcgcccaggatgcggtagccctgctgtagctcgtaggtcagctcctgctccttgcagcaaccgcctccgatcaccatcgcctccatctcttcctcctgatcgtccgcgtcctccagcgaggaggcactccttccgtgggccggccctgaggtctgggccgccgctgccacctcctcctcgtcgtcctctccttcggccgccggtggcggccgctcttcctccccagccggctccatcgctcccggcgtcccgggcacactcatgccccggcaggcctaggctgggcggtgtggaacagccgctcgaggtgctgggggacgcgtgagcgcgagccgcttcctcacggctcggccgcggcgcgtagcccccgccacatcgggcctggctctcctcagccgccggctcggctcggtgcgcgcgggggtcttgagctcaccgccggcggggcggggttacatggcgcgcgaggaggggggagagaagaggagagcctaggtgccctcctctcccctcccccccggcggcggcgcgcgcacggccctcgccggcctcacccctccgcaccccgcccgcctgctcttcaccggccaggccctgccgggtcgccgcggcctcggcgccccaccccctcccgggccagcggggggctgggagggggcgaggaggaagggggttctcctctcccctccccggagggggccgcagcggcggctccggctcctcctctccctcacaccccctcccgcccccctctacctgcgggggacacgggcagaaggaggcggtgcacggacggggcccggcgacaactgtcagttagaagccccgctgggcggtgaggggggagaaaggggaggggcagggagagaagggggagggcactcagccccccggctgggaagagctgtggagagaagcaaagaaagaggccctgtcgccatccccggtgcgcatgcgtagtagaa

SEQ ID NO: 13547 - RNA, 4393 nt, Homo sapiens
  source 1..4393: mol_type = other RNA
gctgggattacaggcatgagccaccacgctcggcccattactcttaaaattataagatctcacccaaggtggaggaaatcacctaactcatccagggataagaagttctgtcaaagggttggtttattcctttacacacttcacacacacacaatccttcccccacccctgacacccttttcaactatttaaggtctgggggctacttccgggtatttttgggtatcagcagggagacagaaatgagcaggatttatgggagagtcaaatgcccctctcaaaacagttaaaggccttccttataaatggcctctctctgtaaatataaaaactaactataagaatctcaaacggtcagccctaaaagaccaggtcttgtgggattgtagagttggccgctatgaagggaagactggaaaaagtgcctccagagacacggggtggtccacagcctaacagttaaaatgctcatcacttttaagaactttcctaacccctttagttctttgatgctaagcagggaagagggaggcttggagaccagggatgtcctcccaggtggtgctggggcctgggtaaccctcagggttgccctcaggagccctctgcctctggaacaccgtgcttggtaggagttattgaagggctgtgtacagtgagtaagccctttcttgtcagcaaaccttcatcaagtcttcagagcgatactgagggtgctctcatttctctgtggaaaaggctctcctcacagagttcctcagacagtgtcccaggtgatggacatggagacttgggctgagtctgagtaagcatctttgtagtctaaaaatgcagctcatatgaaaatatcagctgtgtaacatcagaagcatgacgcctacaggaagatggcctcgagaaagtcttggaaagaagcactttctgctatcaaaacttgatcatttcccatgagaaaaaatgctcaagaaagttggatggcagcttggcacacttaagagaaagctcactgaatcaaagtgatctttctccaggatatccagaggttctgttgagtctatagacttactgatttctcccttaggagagtcttttccaagatctccttcaccttcatcagtggtccatagttctctattaaatgtatcatgatcaggttgtcttctgaaatcatcatagtctttcttcaggcggctcctgtttctttggaaagccttcattaactttggttcccatggcagcaattcatttaaaagacgtatcaatgtactatgtaattcttttacagcttgcctccgatgataccattttcccgatttttttctactgttttccagatctttgagttcattctcgatttttgtgattaattccctgagttcatcaagattagtgcaaataagctgaaactctggtacagtaggtgactttatgacagttttcctcttctttgtgattgcttttttagagacggatttttttccagatttgtgcttcttgtgttttgctttttttttgatgatcaataacttattctggatctcaggtttgtaagacttgaatgcaagagaatgaagaccttcacgctttctctgtaagttttcattcaaaacatctttcaatttcttttttttctttttcttcttttttgccctcattttagttagtttgagtttcttgtggctctgtagtgactgctctaatagaatatcccttacaactttgtggcagttaatttctggatgatcactgtgacttccatttacatgtatttggcaagattttagagtattttcttttaatggactgggttcaatctttattctggaagcttcaccgtatttttcctgattttctataaaccttatttcacctggactaagaggctctccaaagccagtaacttcccctggactccttggtttctctaaattttctttacaacaatcagtttttttaatttcacaaggcctgcgaattctaatttcatagttggattttactcccatttcaacagagatgtcatgattatccaagatcattttagcaggacagcaagctggatcaaaattattttcctgctctttcttgaaggaagagggcaggctatctctgctacatctatgttctccattacttgtactaacatagtcacacttcaatttctccaatttaatccgaggtactctttgtattttaatgggtggaattggaaattctggggcctgaaagggtctctgtttataaatccgtacatctgcaccacagaactgtggaaaatgtacataagcattctccaaataatcataaccaagaataacttccctgcattcatggataggctgtccaagtacagcatcttgaacttccttttgtgtttcatacacaaagtcacaaagacccttaagtagccacactttttggtaaaaaggtagttcgtgaaaaggtttttcttccaatggattaacttctccaagaactttaaaaaactgaggacacaaccccagtttttcagcacagttatcaggattttcagtttgccctacagcagtgtaccactgttgtactttctgcctcagcgctgcttcccaggtcctataaggcaaagtaggtcttcgatgtaaggtaggtctgcgatggggaggacttaatagagaagtcattattttcgatagaaaagcattacactgaggcatcagaagacaacgttccaattcgtaaaagactatttctggcaaatttagaatttgctgagctaaacaaaggaaatgcccaatagctggaatttcccacatggtctccatacaagttggagctgcttgagctagaagttttctttcccattcttctatttccttttgactagcttcttctgcttcttttctttcctgctcccgaagccttttttcttcttttgctctcagctgttcttcctgtctcaaaacttgaaccattatagattcaaaaactccacttgtcaagcctgccaaacttcgcggtgttgaccgacgccttgttgaggtacatgcagttcccttctcatcctccaatccataatagcctctagatgtaactgctatcgttgtcttttctctcaagtgccgagagagaagcgctaacttctgctccagcatcatctccagcttctggccctgtttggagatccagtggtccactccgtgcaggcggtagcacgtctccagcatcaacctgaagtccgccacgaactcggtgatgcccccgtactggccgctggcgaacttctcttccatctgcagcagacacatgccctgtccgggctgctgcgggaaggcgcgaccgccccggcccccgctgcgcggcccttccgccacctcctcctccgcggtggcaacgccccccaagggctgcagaaagggggcggtgaggccccggtgcttctcctgcaggaactcgcccaggatgcggtagccctgctgtagctcgtaggtcagctcctgctccttgcagcaaccgcctccgatcaccatcgcctccatctcttcctcctgatcgtccgcgtcctccagcgaggaggcactccttccgtgggccggccctgaggtctgggccgccgctgccacctcctcctcgtcgtcctctccttcggccgccggtggcggccgctcttcctccccagccggctccatcgctcccggcgtcccgggcacactcatgccccggcaggcctaggctgggcggtgtggaacagccgctcgaggtgctgggggacgcgtgagcgcgagccgcttcctcacggctcggccgcggcgcgtagcccccgccacatcgggcctggctctcctcagccgccggctcggctcggtgcgcgcgggggtcttgagctcaccgccggcggggcggggttacatggcgcgcgaggaggggggagagaagaggagagcctaggtgccctcctctcccctcccccccggcggcggcgcgcgcacggccctcgccggcctcacccctccgcaccccgcccgcctgctcttcaccggccaggccctgccgggtcgccgcggcctcggcgccccaccccctcccgggccagcggggggctgggagggggcgaggaggaagggggttctcctctcccctccccggagggggccgcagcggcggctccggctcctcctctccctcacaccccctcccgcccccctctacctgcgggggacacgggcagaaggaggcggtgcacggacggggcccggcgacaactgtcagttagaagccccgctgggcggtgaggggggagaaaggggaggggcagggagagaagggggagggcactcagccccccggctgggaagagctgtggagagaagcaaagaaagaggccctgtcgccatccccggtgcgcatgcgtagtaga

SEQ ID NO: 13548 - RNA, 5098 nt, Homo sapiens
  source 1..5098: mol_type = other RNA
gctgggattacaggcatgagccaccacgctcggcccattactcttaaaattataagatctcacccaaggtggaggaaatcacctaactcatccagggataagaagttctgtcaaagggttggtttattcctttacacacttcacacacacacaatccttcccccacccctgacacccttttcaactatttaaggtctgggggctacttccgggtatttttgggtatcagcagggagacagaaatgagcaggatttatgggagagtcaaatgcccctctcaaaacagttaaaggccttccttataaatggcctctctctgtaaatataaaaactaactataagaatctcaaacggtcagccctaaaagaccaggtcttgtgggattgtagagttggccgctatgaagggaagactggaaaaagtgcctccagagacacggggtggtccacagcctaacagttaaaatgctcatcacttttaagaactttcctaacccctttagttctttgatgctaagcagggaagagggaggcttggagaccagggatgtcctcccaggtggtgctggggcctgggtaaccctcagggttgccctcaggagccctctgcctctggaacaccgtgcttggtaggagttattgaagggctgtgtacagtgagtaagccctttcttgtcagcaaaccttcatcaagtcttcagagcgatactgagggtgctctcatttctctgtggaaaaggctctcctcacagagttcctcagacagtgtcccaggtgatggacatggagacttgggctgagtctgagtaagcatctttgtagtctaaaaatgcagctcatatgaaaatatcagctgtgtaacatcagaagcatgacgcctacaggaagatggcctcgagaaagtcttggaaagaagcactttctgctatcaaaacttgatcatttcccatgagaaaaaatgctcaagaaagttggatggcagcttggcacacttaagagaaagctcactttctgttgaagtggtggcacttcttttgcaactgcttttccttctttatgctgaatcacaaaattcttaggcagaataagaacttgctgcatgattttttctcctgttttaggatccaccataggctgcacctgaatctttacagagctattttgaagatctattggcaaccactggccacagggcattttgtataccatttgtaaaggaccttttgtattggtgtggcaggtcaatgctggctttatcgggcttgcttccggaggagataaaactggtttttccacagcaagagcatttctacctgtggaaggaggcagttgatttgttaaggtcactttattcccaatattctttgcaagcaaagcctgaatgggtttggtccctttctggagagtagacactggtactgaatccaatgaggcaaatgactctggaaatgatggctctgtatgctttgattcactgaaacagtcaatctgcacatcactttctagattctcaactgttgtctcatttgtgcttaactttgccttcttccttggagaaagctcttttgtgctgtcatccacataatcagtttgtttggactgtcgtttaagtgttttaagcagtgtcttcggtaagtcttttgaaggcaattcctttttcaacagcttgcttctagccataggaaaatctatttctgacaacttcatatcatctgaatcaaagtgatctttctccaggatatccagaggttctgttgagtctatagacttactgatttctcccttaggagagtcttttccaagatctccttcaccttcatcagtggtccatagttctctattaaatgtatcatgatcaggttgtcttctgaaatcatcatagtctttcttcaggcggctcctgtttctttggaaagccttcattaactttggttcccatggcagcaattcatttaaaagacgtatcaatgtactatgtaattcttttacagcttgcctccgatgataccattttcccgatttttttctactgttttccagatctttgagttcattctcgatttttgtgattaattccctgagttcatcaagattagtgcaaataagctgaaactctggtacagtaggtgactttatgacagttttcctcttctttgtgattgcttttttagagacggatttttttccagatttgtgcttcttgtgttttgctttttttttgatgatcaataacttattctggatctcaggtttgtaagacttgaatgcaagagaatgaagaccttcacgctttctctgtaagttttcattcaaaacatctttcaatttcttttttttctttttcttcttttttgccctcattttagttagtttgagtttcttgtggctctgtagtgactgctctaatagaatatcccttacaactttgtggcagttaatttctggatgatcactgtgacttccatttacatgtatttggcaagattttagagtattttcttttaatggactgggttcaatctttattctggaagcttcaccgtatttttcctgattttctataaaccttatttcacctggactaagaggctctccaaagccagtaacttcccctggactccttggtttctctaaattttctttacaacaatcagtttttttaatttcacaaggcctgcgaattctaatttcatagttggattttactcccatttcaacagagatgtcatgattatccaagatcattttagcaggacagcaagctggatcaaaattattttcctgctctttcttgaaggaagagggcaggctatctctgctacatctatgttctccattacttgtactaacatagtcacacttcaatttctccaatttaatccgaggtactctttgtattttaatgggtggaattggaaattctggggcctgaaagggtctctgtttataaatccgtacatctgcaccacagaactgtggaaaatgtacataagcattctccaaataatcataaccaagaataacttccctgcattcatggataggctgtccaagtacagcatcttgaacttccttttgtgtttcatacacaaagtcacaaagacccttaagtagccacactttttggtaaaaaggtagttcgtgaaaaggtttttcttccaatggattaacttctccaagaactttaaaaaactgaggacacaaccccagtttttcagcacagttatcaggattttcagtttgccctacagcagtgtaccactgttgtactttctgcctcagcgctgcttcccaggtcctataaggcaaagtaggtcttcgatgtaaggtaggtctgcgatggggaggacttaatagagaagtcattattttcgatagaaaagcattacactgaggcatcagaagacaacgttccaattcgtaaaagactatttctggcaaatttagaatttgctgagctaaacaaaggaaatgcccaatagctggaatttcccacatggtctccatacaagttggagctgcttgagctagaagttttctttcccattcttctatttccttttgactagcttcttctgcttcttttctttcctgctcccgaagccttttttcttcttttgctctcagctgttcttcctgtctcaaaacttgaaccattatagattcaaaaactccacttgtcaagcctgccaaacttcgcggtgttgaccgacgccttgttgaggtacatgcagttcccttctcatcctccaatccataatagcctctagatgtaactgctatcgttgtcttttctctcaagtgccgagagagaagcgctaacttctgctccagcatcatctccagcttctggccctgtttggagatccagtggtccactccgtgcaggcggtagcacgtctccagcatcaacctgaagtccgccacgaactcggtgatgcccccgtactggccgctggcgaacttctcttccatctgcagcagacacatgccctgtccgggctgctgcgggaaggcgcgaccgccccggcccccgctgcgcggcccttccgccacctcctcctccgcggtggcaacgccccccaagggctgcagaaagggggcggtgaggccccggtgcttctcctgcaggaactcgcccaggatgcggtagccctgctgtagctcgtaggtcagctcctgctccttgcagcaaccgcctccgatcaccatcgcctccatctcttcctcctgatcgtccgcgtcctccagcgaggaggcactccttccgtgggccggccctgaggtctgggccgccgctgccacctcctcctcgtcgtcctctccttcggccgccggtggcggccgctcttcctccccagccggctccatcgctcccggcgtcccgggcacactcatgccccggcaggcctaggctgggcggtgtggaacagccgctcgaggtgctgggggacgcgtgagcgcgagccgcttcctcacggctcggccgcggcgcgtagcccccgccacatcgggcctggctctcctcagccgccggctcggctcggtgcgcgcgggggtcttgagctcaccgccggcggggcggggttacatggcgcgcgaggaggggggagagaagaggagagcctaggtgccctcctctcccctcccccccggcggcggcgcgcgcacggccctcgccggcctcacccctccgcaccccgcccgcctgctcttcaccggccaggccctgccgggtcgccgcggcctcggcgccccaccccctcccgggccagcggggggctgggagggggcgaggaggaagggggttctcctctcccctccccggagggggccgcagcggcggctccggctcctcctctccctcacaccccctcccgcccccctctacctgcgggggacacgggcagaaggaggcggtgcacggacggggcccggcgacaactgtcagttagaagccccgctgggcggtgaggggggagaaaggggaggggcagggagagaagggggagggcactcagccccccggctgggaagagctgtggagagaagcaaagaaagaggccctgtcgccatccccggtgcgcatgcgtagtaga

SEQ ID NO: 13549 - RNA, 1170 nt, Homo sapiens
  source 1..1170: mol_type = other RNA
gctgggattacaggcatgagccaccacggccagccactgttgtagttttaaatcatatattttataaggagcacataattttctgttcacttgagtggaccccttccaaggccctgaagttaattatttgtaattttaaattctttttcttgaagaagaatctctaaactgtaataatatcaggttccagaaaacctggatacaccctcagctcagatctttcctggttaaatccgtctcttctcttcccccacccttcactgctagtaacttcagaaattgtttttcgctctctttagcccaatttttttcttcactacatttagcggtatctgaatttattcatttaaaatgtattcattttctgtccctctttactagaatgtaagctcattgatggcaggtacttcatttgtttcatttgctcctgtgaccccagaacccagaataatgattcacaaagaataggtgccaatcaatacattttcaatgactgacctcggatccaccaaactgctacatttcagccatgtttgtggcacagctatgtttggctactgggagtcccaggcttatgttccagcctccatgaagcagccattcattttgagatcctgtcacattctggctacttccagagatctgtgagcaaatccctgctgttcaagagaccaacagacttctctctcattcttttgagccttggtgtcacttattattctcagtgaaatccttctttcccatggaagcacccaaagatggcttgggtgaacccctctgcttggttccacccattaaaaccctcggccacacagaccccacttttaaaaggttattaattctgacatgcccaagttcatctgagttccttagaaagatcaaccagcagcacctacttcacgacctatcctccattccattcaaataacgcggccaataggaaaatcctccgccctgagccaacgactcggcgtagctgagacagcacgggaggcagatctgccctgtagagccttgcggttccactgctggcctccggattcccgggagcccccagcccgacaggacaaccttccttccccgcttcctcctttccaggtctgtcccagcccccgctgcctgggccacacccgcttccctctggtggcccagccaccaccgccgcagttc

SEQ ID NO: 13550 - RNA, 1295 nt, Homo sapiens
  source 1..1295: mol_type = other RNA
gctgggattacaggcatgagccaccacggccagccactgttgtagttttaaatcatatattttataaggagcacataattttctgttcacttgagtggaccccttccaaggccctgaagttaattatttgtaattttaaattctttttcttgaagaagaatctctaaactgtaataatatcaggttccagaaaacctggatacaccctcagctcagatctttcctggttaaatccgtctcttctcttcccccacccttcactgctagtaacttcagaaattgtttttcgctctctttagcccaatttttttcttcactacatttagcggtatctgaatttattcatttaaaatgtattcattttctgtccctctttactagaatgtaagctcattgatggcaggtacttcatttgtttcatttgctcctgtgaccccagaacccagaataatgattcacaaagaataggtgccaatcaatacattttcaatgactgacctcggatccaccaaactgctacatttcagccatgtttgtggcacagctatgtttggctactgggagtcccaggcttatgttccagcctccatgaagcagccattcattttgagatcctgtcacattctggctacttccagagatctgtgagcaaatccctgctgttcaagagaccaacagacttctctctcattcttttgagccttggtgtcacttattattctcagtgaaatccttctttcccatggaagcacccaaagatggcttgggtgaacccctctgcttggttccacccttgtaatccagaggcaaggcaaagattagatgctatgatctagaaatcaggattgatctagcaatggagtctgaagcaagttagggtggttccatgttggttctggtcaactccctgggtaggacattaaaaccctcggccacacagaccccacttttaaaaggttattaattctgacatgcccaagttcatctgagttccttagaaagatcaaccagcagcacctacttcacgacctatcctccattccattcaaataacgcggccaataggaaaatcctccgccctgagccaacgactcggcgtagctgagacagcacgggaggcagatctgccctgtagagccttgcggttccactgctggcctccggattcccgggagcccccagcccgacaggacaaccttccttccccgcttcctcctttccaggtctgtcccagcccccgctgcctgggccacacccgcttccctctggtggcccagccaccaccgccgcagttc

SEQ ID NO: 13551 - RNA, 1066 nt, Homo sapiens
  source 1..1066: mol_type = other RNA
gctgggattacaggcatgagccaccacggccagccactgttgtagttttaaatcatatattttataaggagcacataattttctgttcacttgagtggaccccttccaaggccctgaagttaattatttgtaattttaaattctttttcttgaagaagaatctctaaactgtaataatatcaggttccagaaaacctggatacaccctcagctcagatctttcctggttaaatccgtctcttctcttcccccacccttcactgctagtaacttcagaaattgtttttcgctctctttagcccaatttttttcttcactacatttagcggtatctgaatttattcatttaaaatgtattcattttctgtccctctttactagaatgtaagctcattgatggcaggtacttcatttgtttcatttgctcctgtgaccccagaacccagaataatgattcacaaagaataggtgccaatcaatacattttcaatgactgacctcggatccaccaaactgctacatttcagccatgtttgtggcacagctatgtttggctactgggagtcccaggcttatgttccagcctccatgaagcagccattcattttgagatcctgtcacattctggctacttccagagatctgtgagcaaatccctgctgttcaagagaccaacagacttctctctcattcttttgagccttggtgtcacttattattctcagtgaaatccttctttcccatggaagcacccaaagatggcttgggtgaacccctctgcttggttccaccttcacgacctatcctccattccattcaaataacgcggccaataggaaaatcctccgccctgagccaacgactcggcgtagctgagacagcacgggaggcagatctgccctgtagagccttgcggttccactgctggcctccggattcccgggagcccccagcccgacaggacaaccttccttccccgcttcctcctttccaggtctgtcccagcccccgctgcctgggccacacccgcttccctctggtggcccagccaccaccgccgcagttc

SEQ ID NO: 13552 - RNA, 1364 nt, Homo sapiens
  source 1..1364: mol_type = other RNA
gctgggattacaggcatgagccaccacggctggcaagttgtcccctttttcttgtaatcacttttctgtattgtaatataaagatttcaaagtagtaaacaagggtgggcagcctttactgaagttaaccctcaggaacttatccattagttctctaaatctttcacctgggacaagagtcaaaggtaatcttctgggtgtaattgctttggggtgctgcttactaatttcttcataaatttgaagcctctcttctaaagtgctaatttgtagagctttttccaagccttcataataacaccaattttctgcatttcgatcaatcaagtttttgaacacttcactggcttcttttaatcttcccaatttcaacagtatttcccctttaatttcttccaccaaaagtttatcacatatttgtttctcatacatttctatatgttccaaagattcctgcaacagatctgcctctctcatcacttgattctggtataatatcaattcactatattcataatctattttgtttggaggaacttgctgagtttgtctaaattcttccaacagttttagggccatatcataatctttcagcaaatggtatgcaatagcatatccaatccaggaggcacgctgtgtggggcgcaactgaagaagctggtatcttgtctctcggtaaccttcaaggtctctcatttggatctgcaacagtgagagatccctcaaaatttgcaggttatctttatctaatttgagggcatttcggtaacattttatagcttcatcatattttttatcagaacgctgcaagagtccatatacatgccaacagacatgactcttgacatcattacgaagtcctttacgaacaaactcataagcttcttctttttttcctaaacagttcagtgttaatcctttcatagccaaagtctctccatgttcagcaaattttgggttcgacagaatcatcttgcaaaacttgaggccatttttgtactgcttctgttcataacatttcaagatgcgtttgaagaggttgctctccttgggcggcagcagcacgttcggcatcgtggccggcagggaggctaggtggccggcagggaggctaggtgcccgggcgctccgcttcgcgggggtgggcaccgggacgaaccgctgctgagagtcgggctgcgggcgatggattagttcattggtctacagttgcaattgggcagcctggctgttcggcacgggtggcaatggagaaggaaggcggtctgagcaggacacgcttcccctgggctccgctttttggccagcggcggcggcggcggttcccgcgcactgcaagatggcagccagggtccgcctcccga

SEQ ID NO: 13553 - RNA, 2544 nt, Homo sapiens
  source 1..2544: mol_type = other RNA
gctgggattacaggcatgagccaccacgtccggcctcaatgagggctttttaaggcaagtcaggagtttcctattagaaagatcactctaccataaatggagaaaattgggcaaaggggaggggatggctagtgggtgaaatcatggagactagaaggaaggaagctgttgaattaatctagacaagaaatgataaggtcctaatagtggcagtggagatggagtaaagtggacgatgggaaaatgggatgaggcctctggagagcagctcacaggcaatttttttttcattccctacaatgacatttgcctacggcaacacactctgccacatgcaatgaggtagtgactggctcaagctaaggaaataatcttgttactgacgtggtatcaccgggaatcatggctgtataactgtagtttcataatcaaattttggaactctacatttaattgcttaatggtgatgatgattatgacaggaataatactgataatagctgcaacccaattttattggacacttattctgtgctagttactgttccaagcattctgaatttactaacccacttaatcttcaagtgactctatcgggtaggttctattcttactcttaaagaatagatgaggacactgaggcagcacagacaggtttaataccttgtctaaggtcacacagctaggaagtgagaaaataaggatctgagccttggaaatctggttctaggacgcaaacttccaaaaattctcctatcaatttacaatgacaaacataaattatggtctttctccataaaactcaatttgagcactaaaactgactttttaccatttgttatgaacattctgaacaatcacaataaaaagtagtgcggagacactattcaagtctctaaaaacatcttaggagtggtacatgaagcaaaatgctgggtgtgagtgtttttgcagattcaggctccaaagaacaaaaaagcagaaaaaacaaacaatggtgtttttaaacaatgaatgttgttttcctttagccataagggaattttaaaacttgacaaactcattcagctttcaaagcattccacattccccacccacaagcaaatgccagaaggtgccagtttgagccaactcagctcaggaatgactttctaaatactggatcagatttcttgaatgtccgcgctccacagatggatacttactattgtcctaattggtctgatgaaaagtacttagcaatttatcaagcaattaatttaacaaaaacatttcagcaagagatgagatggtgtggcacaaatgcagaaacagaaatttgaaaagattcaaatgtattacttcaaaaagattgaaaaattgctgcctaaaatctttgaaactttagagctaggttgtgcataggcttaatttttaatgaagaatcttctgggaaaataagtttttgattatataaagaaagcaatttccttgatttgcaggaaataattctttttggggaaaaacaaataaattaatatttaatatactcattacatccatccagctaacatttactggaagcatgctgtgtgcctggcaccatgctaggcactgagacacaaaaatgaaaaagacaagaatcttgttctttagcctaggtggggagatagataagcaaaggaatagtgtaataaatgcaataaaagaaatacgtactagctagacctgtgggaagaaaggttagaaagatgaacagaaactgtgctagaattttggacctaattctgtaagtgttggagagccattaagcagaagtgatcgttagatttaattttagaaggatcatgctgttatcaatgtgaagaatgggctgtagtggggaaacgccaaaggcagattctgttccactcttcataaaaatcgtaccacagcactctgataccctttttgctctctaatccatttctcttttccccccaacacagataatttagaaattatttagtcttttaaaagcgctggtgtccaagtttttgaggttttcccagatatttgttattggttaataatttaattccattgtggtcagagaacatattttctatgacttgaatccttttaaatttatcaagatttgtttcatggctcaaaatacggtctatcttggtacatgtttcatgtactcttggaaagaatgtgtgatttattgttgttggggactgctgtgctctacaaatgtcatttaagtcaaattgtttgatagtcttgttctaatcttctatatccttactgattttgtgtattcttgttctactaaacattgaaaggatattaaaatctccaggctgcgtgcagtggctcatgcctgtaatcccagcactttgggaggccgaggcaggcagatcacgaggtcaggagatcgagaccatcctggctaacacggtgaaaccccgtctctactaaaaatacaaaaaaattagccaggcgtggtggtggccgcctgtagtcccagctactggggaggctgaagcaggagaatggcgtgaacctgggaggcggagc

SEQ ID NO: 13554 - RNA, 1810 nt, Homo sapiens
  source 1..1810: mol_type = other RNA
gctgggattacaggcatgagccaccacgtgatatggggcttttttgtgtgtgtgtgtgatggagtctcacttttgtcgcccaggctggagtgcaatggcgtgatctcggctcactgcaacctccacctcccaggttcaagcgattctcctgcctcggcctcccgagtagctgagattacaggtgcccaccaccatgcccagttaatttttttgtatttttagtagagacggggtttcaccatgttggccaggctagtcttgaactcctgacctcaggtgatccacccgcctcagcctcccaaagtgctgggattacaagcgtgagccaccgtacccagccgatatggggccttcttatgttgcccaggctggtctcaaactcctgggctcaggtgatccccctgcctcctgccaaagcactggctacgcccggccaaatgagttctttcatgaagtctaaggtaatttgaaaaagtaaagactttaccacactgtttacaatcaaagggtttttctccagtgtgagtcatttcatgtcttcggagggaactgcaccacccaaaggctttaccacaccttgtacattcatatggcttttctccactatgagtttttttatgtcttcgaaaacaactgggataattgaaggttttaccacatttattacattcataaggtctttctccagtgtgagctctttcatgtgcttgaagggacgtgggacatctaaagactttggcacatttttgacattcgtagagttttcctccactatgagttctttcatgtctgtgaagggaactggaacaactgagttttttcccacattcctgacattggtgggatttctccagcgcgtgagatctgatttcatgtgtccgaaggtaacctgcggaaatgaaggctttaccacattgtttacatttgtaaggtttttctccagtgtgagttctaacatgaatttgaaataaactgggataatcgataggttttccacagtatttacattcatagcgtttttctccagtatgcatttttccatgttttcgaaagaaactggaaactgtgaaggctctcactatttccctacatttataggacctctttccagtgtgagttctttgatggatttgaaataaattgggagaattaaaggctttcccgcacaccttgcattcataaggtctctttcgagttggtgttactgtgcgccgtgcaccactactgggggaaatggaggctttcccatgttgtttctgtttacggggcgtctctctccattccccaccacactcagatcgtttgtgtccagcatgagctctcatgtgcctgtccaggaatgaatgacggaggaagactttcccacacacgctgcatttgcatggtttcactccagtttgacttttcttgttcaggtgacaatcaggaatctggctgaaagtttctctgtgttcattcccttctttacgtccacagagtctctccaccagacttcttagcttaatccccaggttttggtacagattctcaatgtcctggtctttccattggattccgaccgaggccaggttcctgaaggtttccagcgtcacatctctgtagagattcttctgggaaggactcagcaaagcccactcctcctgggtgaagttcacagccacatcctcaaaggccactgagtccatttccggcttccgggtgtcctgggtccttcctggggctggagcagccagaacaggtcccacacgacaaaatcagccgtatccggggcaccaggggctccccgaggaactaaaacccggacccgaat

SEQ ID NO: 13555 - RNA, 1904 nt, Homo sapiens
  source 1..1904: mol_type = other RNA
gctgggattacaggcatgagccaccacgtgatatggggcttttttgtgtgtgtgtgtgatggagtctcacttttgtcgcccaggctggagtgcaatggcgtgatctcggctcactgcaacctccacctcccaggttcaagcgattctcctgcctcggcctcccgagtagctgagattacaggtgcccaccaccatgcccagttaatttttttgtatttttagtagagacggggtttcaccatgttggccaggctagtcttgaactcctgacctcaggtgatccacccgcctcagcctcccaaagtgctgggattacaagcgtgagccaccgtacccagccgatatggggccttcttatgttgcccaggctggtctcaaactcctgggctcaggtgatccccctgcctcctgccaaagcactggctacgcccggccaaatgagttctttcatgaagtctaaggtaatttgaaaaagtaaagactttaccacactgtttacaatcaaagggtttttctccagtgtgagtcatttcatgtcttcggagggaactgcaccacccaaaggctttaccacaccttgtacattcatatggcttttctccactatgagtttttttatgtcttcgaaaacaactgggataattgaaggttttaccacatttattacattcataaggtctttctccagtgtgagctctttcatgtgcttgaagggacgtgggacatctaaagactttggcacatttttgacattcgtagagttttcctccactatgagttctttcatgtctgtgaagggaactggaacaactgagttttttcccacattcctgacattggtgggatttctccagcgcgtgagatctgatttcatgtgtccgaaggtaacctgcggaaatgaaggctttaccacattgtttacatttgtaaggtttttctccagtgtgagttctaacatgaatttgaaataaactgggataatcgataggttttccacagtatttacattcatagcgtttttctccagtatgcatttttccatgttttcgaaagaaactggaaactgtgaaggctctcactatttccctacatttataggacctctttccagtgtgagttctttgatggatttgaaataaattgggagaattaaaggctttcccgcacaccttgcattcataaggtctctttcgagttggtgttactgtgcgccgtgcaccactactgggggaaatggaggctttcccatgttgtttctgtttacggggcgtctctctccattccccaccacactcagatcgtttgtgtccagcatgagctctcatgtgcctgtccaggaatgaatgacggaggaagactttcccacacacgctgcatttgcatggtttcactccagtttgacttttcttgttcaggtgacaatcaggaatctggctgaaagtttctctgtgttcattcccttctttacgtccacagagtctctccaccagacttcttagcttaatccccaggttttggtacagattctcaatgtcctggtctttccattggattccgaccgaggccaggttcctgaaggtttccagcgtcacatctctgtagagattcttctgggaaggactcagcaaagcccactcctcctgggtgaagttcacagccacatcctcaaaggccactgagtcctaacaccaaagatttccaaaccatcacattcaggacagcatactattagcagagagataaacaaatagatcaaggaaaaagaagagtcttcaatgggccagtattcatatgaaaacttggttaataacagagcaggcatgtagagtagtagggtggaccacttgaggtcaggagttaaagaccagcctggcctacatagtgaaaactggtctctattaaaa

SEQ ID NO: 13556 - RNA, 1805 nt, Homo sapiens
  source 1..1805: mol_type = other RNA
gctgggattacaggcatgagccaccacgtgatatggggcttttttgtgtgtgtgtgtgatggagtctcacttttgtcgcccaggctggagtgcaatggcgtgatctcggctcactgcaacctccacctcccaggttcaagcgattctcctgcctcggcctcccgagtagctgagattacaggtgcccaccaccatgcccagttaatttttttgtatttttagtagagacggggtttcaccatgttggccaggctagtcttgaactcctgacctcaggtgatccacccgcctcagcctcccaaagtgctgggattacaagcgtgagccaccgtacccagccgatatggggccttcttatgttgcccaggctggtctcaaactcctgggctcaggtgatccccctgcctcctgccaaagcactggctacgcccggccaaatgagttctttcatgaagtctaaggtaatttgaaaaagtaaagactttaccacactgtttacaatcaaagggtttttctccagtgtgagtcatttcatgtcttcggagggaactgcaccacccaaaggctttaccacaccttgtacattcatatggcttttctccactatgagtttttttatgtcttcgaaaacaactgggataattgaaggttttaccacatttattacattcataaggtctttctccagtgtgagctctttcatgtgcttgaagggacgtgggacatctaaagactttggcacatttttgacattcgtagagttttcctccactatgagttctttcatgtctgtgaagggaactggaacaactgagttttttcccacattcctgacattggtgggatttctccagcgcgtgagatctgatttcatgtgtccgaaggtaacctgcggaaatgaaggctttaccacattgtttacatttgtaaggtttttctccagtgtgagttctaacatgaatttgaaataaactgggataatcgataggttttccacagtatttacattcatagcgtttttctccagtatgcatttttccatgttttcgaaagaaactggaaactgtgaaggctctcactatttccctacatttataggacctctttccagtgtgagttctttgatggatttgaaataaattgggagaattaaaggctttcccgcacaccttgcattcataaggtctctttcgagttggtgttactgtgcgccgtgcaccactactgggggaaatggaggctttcccatgttgtttctgtttacggggcgtctctctccattccccaccacactcagatcgtttgtgtccagcatgagctctcatgtgcctgtccaggaatgaatgacggaggaagactttcccacacacgctgcatttgcatggtttcactccagtttgacttttcttgttcaggtgacaatcaggaatctggctgaaagtttctctgtgttcattcccttctttacgtccacagagtctctccaccagacttcttagcttaatccccaggttttggtacagattctcaatgtcctggtctttccattggattccgaggccaggttcctgaaggtttccagcgtcacatctctgtagagattcttctgggaaggactcagcaaagcccactcctcctgggtgaagttcacagccacatcctcaaaggccactgagtccatttccggcttccgggtgtcctgggtccttcctggggctggagcagccagaacaggtcccacacgacaaaatcagccgtatccggggcaccaggggctccccgaggaactaaaacccggacccgaa

SEQ ID NO: 13557 - RNA, 1934 nt, Homo sapiens
  source 1..1934: mol_type = other RNA
gctgggattacaggcatgagccaccacgtgatatggggcttttttgtgtgtgtgtgtgatggagtctcacttttgtcgcccaggctggagtgcaatggcgtgatctcggctcactgcaacctccacctcccaggttcaagcgattctcctgcctcggcctcccgagtagctgagattacaggtgcccaccaccatgcccagttaatttttttgtatttttagtagagacggggtttcaccatgttggccaggctagtcttgaactcctgacctcaggtgatccacccgcctcagcctcccaaagtgctgggattacaagcgtgagccaccgtacccagccgatatggggccttcttatgttgcccaggctggtctcaaactcctgggctcaggtgatccccctgcctcctgccaaagcactggctacgcccggccaaatgagttctttcatgaagtctaaggtaatttgaaaaagtaaagactttaccacactgtttacaatcaaagggtttttctccagtgtgagtcatttcatgtcttcggagggaactgcaccacccaaaggctttaccacaccttgtacattcatatggcttttctccactatgagtttttttatgtcttcgaaaacaactgggataattgaaggttttaccacatttattacattcataaggtctttctccagtgtgagctctttcatgtgcttgaagggacgtgggacatctaaagactttggcacatttttgacattcgtagagttttcctccactatgagttctttcatgtctgtgaagggaactggaacaactgagttttttcccacattcctgacattggtgggatttctccagcgcgtgagatctgatttcatgtgtccgaaggtaacctgcggaaatgaaggctttaccacattgtttacatttgtaaggtttttctccagtgtgagttctaacatgaatttgaaataaactgggataatcgataggttttccacagtatttacattcatagcgtttttctccagtatgcatttttccatgttttcgaaagaaactggaaactgtgaaggctctcactatttccctacatttataggacctctttccagtgtgagttctttgatggatttgaaataaattgggagaattaaaggctttcccgcacaccttgcattcataaggtctctttcgagttggtgttactgtgcgccgtgcaccactactgggggaaatggaggctttcccatgttgtttctgtttacggggcgtctctctccattccccaccacactcagatcgtttgtgtccagcatgagctctcatgtgcctgtccaggaatgaatgacggaggaagactttcccacacacgctgcatttgcatggtttcactccagtttgacttttcttgttcaggtgacaatcaggaatctggctgaaagtttctctgtgttcattcccttctttacgtccacagagtctctccaccagacttcttagcttaatccccaggttttggtacagattctcaatgtcctggtctttccattggattccgaggccaggttcctgaaggtttccagcgtcacatctctgtagagattcttctgggaaggactcagcaaagcccactcctcctgggtgaagttcacagccacatcctcaaaggccactgagtcctgggcatggtggtggacgccggtaatcccagctacttgggaggcagaggcaggagaatcccatgaacccgggaggcggaggttgcagtgagccgagatcatgccattacactccagcttgactgacttcaggtctcttcgtcctttcggctgaccttacagctcctggttttccggagcaggccctgtcggcttcctgtactcagtgggtccttcctgctgctttttttttttttttttgagacggagtttcgct

SEQ ID NO: 13558 - RNA, 1733 nt, Homo sapiens
  source 1..1733: mol_type = other RNA
gctgggattacaggcatgagccaccacgtgatatggggcttttttgtgtgtgtgtgtgatggagtctcacttttgtcgcccaggctggagtgcaatggcgtgatctcggctcactgcaacctccacctcccaggttcaagcgattctcctgcctcggcctcccgagtagctgagattacaggtgcccaccaccatgcccagttaatttttttgtatttttagtagagacggggtttcaccatgttggccaggctagtcttgaactcctgacctcaggtgatccacccgcctcagcctcccaaagtgctgggattacaagcgtgagccaccgtacccagccgatatggggccttcttatgttgcccaggctggtctcaaactcctgggctcaggtgatccccctgcctcctgccaaagcactggctacgcccggccaaatgagttctttcatgaagtctaaggtaatttgaaaaagtaaagactttaccacactgtttacaatcaaagggtttttctccagtgtgagtcatttcatgtcttcggagggaactgcaccacccaaaggctttaccacaccttgtacattcatatggcttttctccactatgagtttttttatgtcttcgaaaacaactgggataattgaaggttttaccacatttattacattcataaggtctttctccagtgtgagctctttcatgtgcttgaagggacgtgggacatctaaagactttggcacatttttgacattcgtagagttttcctccactatgagttctttcatgtctgtgaagggaactggaacaactgagttttttcccacattcctgacattggtgggatttctccagcgcgtgagatctgatttcatgtgtccgaaggtaacctgcggaaatgaaggctttaccacattgtttacatttgtaaggtttttctccagtgtgagttctaacatgaatttgaaataaactgggataatcgataggttttccacagtatttacattcatagcgtttttctccagtatgcatttttccatgttttcgaaagaaactggaaactgtgaaggctctcactatttccctacatttataggacctctttccagtgtgagttctttgatggatttgaaataaattgggagaattaaaggctttcccgcacaccttgcattcataaggtctctttcgagttggtgttactgtgcgccgtgcaccactactgggggaaatggaggctttcccatgttgtttctgtttacggggcgtctctctccattccccaccacactcagatcgtttgtgtccagcatgagctctcatgtgcctgtccaggaatgaatgacggaggaagactttcccacacacgctgcatttgcatggtttcactccagtttgacttttcttgttcaggtgacaatcaggaatctggctgaaagtttctctgtgttcattcccttctttacgtccacagagtctctccaccagacttcttagcttaatccccaggttttggtacagattctcaatgtcctggtctttccattggattccgaggccaggttcctgaaggtttccagcgtcacatctctgtagagattcttctgggaaggactcagcaaagcccactcctcctgggtgaagttcacagccacatcctcaaaggccactgagtcttgactgacttcaggtctcttcgtcctttcggctgaccttacagctcctggtttt

SEQ ID NO: 13559 - RNA, 1176 nt, Homo sapiens
  source 1..1176: mol_type = other RNA
gctgggattacaggcatgagccaccacgtgcggccaggtcatcttttcatccaagctgctcacaatgtttccgcacaccaaccaatctcttaatccttaccacaatgatcaggcagtaaaaactattactcttacttcccatttgggaaaactaaagctgagaaactcaaaaacttgtgtagcattaagtatgaattgcctacgtcaacgctgtgtccctaattttcagaccctatccttctttaattcccaactgattctagtaagcacccgaaagagaaccagaacatgttacaactcttttttctacctggagaaaggcataattctcaagaaataacatagttcatatcttatgttaaagttaattactctagtagagaagattctcttaattgacttggaagtagttcactgaagagtattaagtgctgctttaaggtaccaattagtctgtttagatgcttgagtctttaatgtgtattaacaatgtgttgaatcagaaactcaagagtctgagttctgagcagagggaaaattacagcaggaaatacacaggatcaaagtatgtccaagtatttaatattctctcagaaaccagatgcctaatctacgtaacatataaaatctgctgggaagaggggatgggatgcagtggatgtggatttattaacattagaacatctgatgggaaacaatatagtgatgttaaatacaaaacacttccattcacacacccaaggaaaaataaaatgctccagagaaacttgccagaagcttggaatcaaccccaagcagcttggaagagtcagtcagaaaggcctagggcagaatccagcacagagttgaatggatgctacctgcctttctcttgtcttagtcataaaggaaaactttatatatgtgtgtttaacacgttttcacttttatttgagatgcttgctttcctatgacctgatttatcttgggttcggagcaattctgcttgtagacctgggaattttcttccatgttataatactcagtctcccttgagacaacggccagtatcagctcagtagaaccaataggtcaggaaactttcagtatggcaaaaacaggatcctgctaatttacaaagataaatttccggcacagtcacaccccaatctgacaatacacagccccttgactggt

SEQ ID NO: 13560 - RNA, 3554 nt, Homo sapiens
  source 1..3554: mol_type = other RNA
gctgggattacaggcatgagccaccactcccagccaatagtgaattttctaagagcatgtatccctatcagtaacagggatacatgaagatacttataaaatacagaaaaactgcccagcaaatcagggccctaaacagttggtagattccataaattcaactggctaccatgtatagccctcactgtaaggtaggtggttaggtttctagagagcattagtcttagaattatgaagagccatattaacccaaatgatttctaaatttagatatatattttccctgctacataaaaactctgggtaataactagaaatagacccacaatttagagacaatgtatactagatttatctcctttgtttttagttgaaggcaaaaaaaaaaaaaaaaaaaaaaaactattccagttgtcatcacaaataaatgccaaatgcctcatattcagcggttcattacagtgtataaaaaaaaactgatcatttccctagtcagtgctgttatcaatataaaagattaatttacaaaaacgtaaatattcataacccaatccagctgtattttctgcttttgcaccacaggtcaaaagatattttaaaaactaaaacctgaaagcctcaaaataagctagattcaccttcaccttaccttttcaaaaggagaagggccaaaccacacaagaactgtttacctgcaggaagttcaaacacatgaccagcatctgctaagtcacttcccagtcttcacaaaatacaagctgtgattgatttgtaggtcaaatctataaaaatattttgcacacttaagtcagaagagctgagaactaaattagcactctgtttctttgctgtcaacacgattctgacgctgcagtttaaaggaggcagccttttcacttctggtgaccggatggtccgtgagatcctcaaatgacttggcagctgtgctgctatttgggaaggggtccttctcaaacccatcctcgtccatatgtgagtctgtgctggggtcttcctggatggtgtccattctctggtggtccagttttggagctgctggcgccgaagggatcacaggggcaggctgcaggcggcctggagtctggggcgcaggaaagggtttgataatgcgaaccgatgcagaatccatgctgctcagcatttcgacgttactggggtgaaacagagacagagattcatactgtttatccaatttcttatccacacaatggacaagaatgctgaaaggaatccaaaatatcaaggagaaaaccaggacagacccaacgatgttgtctgctaaaaactttccaaaagtattgatgctcagctggtcaatgaaatcccaaaatcgttcaattacatcctgtactcgtttctcacatttgccattcatgtcacaaaatcctactgtacagggctttcctttcctcaaaaataagttcttttgttcagcatcgacatagggcacacagcggccagaaaggtccctgcagcacaccttgcaggagttgtcagtttcattacatgcacaggactccagctgctgttccctctcgcagaaagggatgcatttcccatccttacacttgccaagatccaagcaaacagtgtcatcttcagcatttcctggaggcgggcactcactgctattacctgtgcagtaggacacgcctttgcaagtagcattaatcgcctcctggcacttcttctgggcagtctcaaactgacagtttttacagcaaggactgttcctgtcactgcactggacaccttccttcaacgtgcagtcgctgttgcagcaggtgtcgttgttcagatacatgatgccaggatcacactcttctccttcatccaccctcgagttcccacaaactttattgctgcgttcttgaaaacactcctgggccttactttcaatggtcttatagattgattgtttactgcagtttgaaaacatcttattgttctcgtgatcgccactcacagctatgggatacatgacatatttccctccctggtcctcattcggggcacattctgctagaccatccggatcatgttctgctccaaaattatgtcccaattcatgagttgtaaccaggtcagcttcctttgtaaggatggttttaccataattctttgtgctcgtcaaaccactattcaaatagatatttttcttcccaactgggctataataagcctttggacaaacacctccatggctgtttgctctgggagagccaacataagctaatccaagagttcccatatcaaaatcttggtatgtgaaaaggtgtgccaagcaaactttagatgcttcctcagctatatcaaagctaaattgctctagcaacatcttcacatcccaagcatccttttcttcatttgggtaactttttgccatgttgtagtgcttttcaccaggttttacctcttgtggagacttgagaatgcgaatctatactgctctatctgtattccatagcctttaaaacctgcattatcccatgaagtgttccgatagatgtcatcaactctgtcaattagctctattaagtaatttgtagttgtactctcttcccctctgcccatgtatctgtagaagcgatgatctgctaccaccaataatttacacgtgttcttcatgggatctgggtcagctcttcttttcactcgatgaacaagctctaatatgaatttgtatgcacttcaggtggttctctgtctactaacccttttgggagcaactcttcattatccacttttaaataaccacacacttttggagactgcaaacgtgaaacattcttgatatcttcagatttataaactaacattcttttgtctttggtatcattaacaaatctccaaagtggctctatgttatattcggccccatctgtgttgattctgattataacatcatcatctcttatgtgggctagaaccctagagtcaggctcaccaaccacgtgtccagtgaagaagtcctgccattttacagtgtactcgctttcgtttttaccatccaccaccacgaccttgaaattttgtgaaaaacgttcagtacttgatgtcaggtataatttaaaatgccttttcaaagctgaaaaagttagtagtgtttctacatgtgttgaagtctgtagatctctttttcttaccgaatgctgctggatattagataaagagagaatatcgtagtctgagagcaaagaatcaagcttctcgagtctctggtgggggccgaagcccgggtcatccggaggtcgcggcgccagcacgaaaggaaccacgctggtcaggaataggagagactgcctcatgttcccggccccgctaccgactccacctctctgggcagccttcgcctgacggggtttcggaaaactgctcacatcgggggaggacgggatccgcccggcctagcccctcaatcctcttttccctcccgcgccgcctactgggaagattctaccgccaggctcgacgcccccagaagtgcaggtggcgttaccaaaggccggctcagccagcttccggccgccgct

SEQ ID NO: 13561 - RNA, 3540 nt, Homo sapiens
  source 1..3540: mol_type = other RNA
gctgggattacaggcatgagccaccactcccagccaatagtgaattttctaagagcatgtatccctatcagtaacagggatacatgaagatacttataaaatacagaaaaactgcccagcaaatcagggccctaaacagttggtagattccataaattcaactggctaccatgtatagccctcactgtaaggtaggtggttaggtttctagagagcattagtcttagaattatgaagagccatattaacccaaatgatttctaaatttagatatatattttccctgctacataaaaactctgggtaataactagaaatagacccacaatttagagacaatgtatactagatttatctcctttgtttttagttgaaggcaaaaaaaaaaaaaaaaaaaaaaaactattccagttgtcatcacaaataaatgccaaatgcctcatattcagcggttcattacagtgtataaaaaaaaactgatcatttccctagtcagtgctgttatcaatataaaagattaatttacaaaaacgtaaatattcataacccaatccagctgtattttctgcttttgcaccacaggtcaaaagatattttaaaaactaaaacctgaaagcctcaaaataagctagattcaccttcaccttaccttttcaaaaggagaagggccaaaccacacaagaactgtttacctgcaggaagttcaaacacatgaccagcatctgctaagtcacttcccagtcttcacaaaatacaagctgtgattgatttgtaggtcaaatctataaaaatattttgcacacttaagtcagaagagctgagaactaaattagcactctgtttctttgctgtcaacacgattctgacgctgcagtttaaaggaggcagccttttcacttctggtgaccggatggtccgtgagatcctcaaatgacttggcagctgtgctgctatttgggaaggggtccttctcaaacccatcctcgtccatatgtgagtctgtgctggggtcttcctggatggtgtccattctctggtggtccagttttggagctgctggcgccgaagggatcacaggggcaggctgcaggcggcctggagtctggggcgcaggaaagggtttgataatgcgaaccgatgcagaatccatgctgctcagcatttcgacgttactggggtgaaacagagacagagattcatactgtttatccaatttcttatccacacaatggacaagaatgctgaaaggaatccaaaatatcaaggagaaaaccaggacagacccaacgatgttgtctgctaaaaactttccaaaagtattgatgctcagctggtcaatgaaatcccaaaatcgttcaattacatcctgtactcgtttctcacatttgccattcatgtcacaaaatcctactgtacagggctttcctttcctcaaaaataagttcttttgttcagcatcgacatagggcacacagcggccagaaaggtccctgcagcacaccttgcaggagttgtcagtttcattacatgcacaggactccagctgctgttccctctcgcagaaagggatgcatttcccatccttacacttgccaagatccaagcaaacagtgtcatcttcagcatttcctggaggcgggcactcactgctattacctgtgcagtaggacacgcctttgcaagtagcattaatcgcctcctggcacttcttctgggcagtctcaaactgacagtttttacagcaaggactgttcctgtcactgcactggacaccttccttcaacgtgcagtcgctgttgcagcaggtgtcgttgttcagatacatgatgccaggatcacactcttctccttcatccaccctcgagttcccacaaactttattgctgcgttcttgaaaacactcctgggccttactttcaatggtcttatagattgattgtttactgcagtttgaaaacatcttattgttctcgtgatcgccactcacagctatgggatacatgacatatttccctccctggtcctcattcggggcacattctgctagaccatccggatcatgttctgctccaaaattatgtcccaattcatgagttgtaaccaggtcagcttcctttgtaaggatggttttaccataattctttgtgctcgtcaaaccactattcaaatagatatttttcttcccaactgggctataataagcctttggacaaacacctccatggctgtttgctctgggagagccaacataagctaatccaagagttcccatatcaaaatcttggtatgtgaaaaggtgtgccaagcaaactttagatgcttcctcagctatatcaaagctaaattgctctagcaacatcttcacatcccaagcatccttttcttcatttgggtaactttttgccatgttgtagtgcttttcaccaggttttacctcttgtggagacttgagaatgcgaatctatactgctctatctgtattccatagcctttaaaacctgcattatcccatgaagtgttccgatagatgtcatcaactctgtcaattagctctattaagtaatttgtagttgtactctcttcccctctgcccatgtatctgtagaagcgatgatctgctaccaccaataatttacacgtgttcttcatgggatctgggtcagctcttcttttcactcgatgaacaagctcttcaggtggttctctgtctactaacccttttgggagcaactcttcattatccacttttaaataaccacacacttttggagactgcaaacgtgaaacattcttgatatcttcagatttataaactaacattcttttgtctttggtatcattaacaaatctccaaagtggctctatgttatattcggccccatctgtgttgattctgattataacatcatcatctcttatgtgggctagaaccctagagtcaggctcaccaaccacgtgtccagtgaagaagtcctgccattttacagtgtactcgctttcgtttttaccatccaccaccacgaccttgaaattttgtgaaaaacgttcagtacttgatgtcaggtataatttaaaatgccttttcaaagctgaaaaagttagtagtgtttctacatgtgttgaagtctgtagatctctttttcttaccgaatgctgctggatattagataaagagagaatatcgtagtctgagagcaaagaatcaagcttcttcatgtgtggaagctaaaaaagtggatctcgtggaggtagacagcagaatggtggttaccagaggctgagaagggaagtgggagtggtggagatgaacagaaagtggttagtgttacaaaaatacagtttgattagtaagttctaatatttgatagtacagtacagaaattatagttaacaatttattgtatacttcaaaacagctagaagacttgtaatattcctaacacagaaaagatgtttcaaatgatgggtatcccaatcaccctgatttgatcactacatattatacacaggtatcaaaatatcacatgtacccaaaaaaca

SEQ ID NO: 13562 - RNA, 5487 nt, Homo sapiens
  source 1..5487: mol_type = other RNA
gctgggattacaggcatgagccaccactcccagccaatagtgaattttctaagagcatgtatccctatcagtaacagggatacatgaagatacttataaaatacagaaaaactgcccagcaaatcagggccctaaacagttggtagattccataaattcaactggctaccatgtatagccctcactgtaaggtaggtggttaggtttctagagagcattagtcttagaattatgaagagccatattaacccaaatgatttctaaatttagatatatattttccctgctacataaaaactctgggtaataactagaaatagacccacaatttagagacaatgtatactagatttatctcctttgtttttagttgaaggcaaaaaaaaaaaaaaaaaaaaaaaactattccagttgtcatcacaaataaatgccaaatgcctcatattcagcggttcattacagtgtataaaaaaaaactgatcatttccctagtcagtgctgttatcaatataaaagattaatttacaaaaacgtaaatattcataacccaatccagctgtattttctgcttttgcaccacaggtcaaaagatattttaaaaactaaaacctgaaagcctcaaaataagctagattcaccttcaccttaccttttcaaaaggagaagggccaaaccacacaagaactgtttacctgcaggaagttcaaacacatgaccagcatctgctaagtcacttcccagtcttcacaaaatacaagctgtgattgatttgtaggtcaaatctataaaaatattttgcacacttaagtcagaagagctgagaactaaattagcactctgtttctttgctgtcaacacgattctgacgctgcagtttaaaggaggcagccttttcacttctggtgaccggatggtccgtgagatcctcaaatgacttggcagctgtgctgctatttgggaaggggtccttctcaaacccatcctcgtccatatgtgagtctgtgctggggtcttcctggatggtgtccattctctggtggtccagttttggagctgctggcgccgaagggatcacaggggcaggctgcaggcggcctggagtctggggcgcaggaaagggtttgataatgcgaaccgatgcagaatccatgctgctcagcatttcgacgttactggggtgaaacagagacagagattcatactgtttatccaatttcttatccacacaatggacaagaatgctgaaaggaatccaaaatatcaaggagaaaaccaggacagacccaacgatgttgtctgctaaaaactttccaaaagtattgatgctcagctggtcaatgaaatcccaaaatcgttcaattacatcctgtactcgtttctcacatttgccattcatgtcacaaaatcctactgtacagggctttcctttcctcaaaaataagttcttttgttcagcatcgacatagggcacacagcggccagaaaggtccctgcagcacaccttgcaggagttgtcagtttcattacatgcacaggactccagctgctgttccctctcgcagaaagggatgcatttcccatccttacacttgccaagatccaagcaaacagtgtcatcttcagcatttcctggaggcgggcactcactgctattacctgtgcagtaggacacgcctttgcaagtagcattaatcgcctcctggcacttcttctgggcagtctcaaactgacagtttttacagcaaggactgttcctgtcactgcactggacaccttccttcaacgtgcagtcgctgttgcagcaggtgtcgttgttcagatacatgatgccaggatcacactcttctccttcatccaccctcgagttcccacaaactttattgctgcgttcttgaaaacactcctgggccttactttcaatggtcttatagattgattgtttactgcagtttgaaaacatcttattgttctcgtgatcgccactcacagctatgggatacatgacatatttccctccctggtcctcattcggggcacattctgctagaccatccggatcatgttctgctccaaaattatgtcccaattcatgagttgtaaccaggtcagcttcctttgtaaggatggttttaccataattctttgtgctcgtcaaaccactattcaaatagatatttttcttcccaactgggctataataagcctttggacaaacacctccatggctgtttgctctgggagagccaacataagctaatccaagagttcccatatcaaaatcttggtatgtgaaaaggtgtgccaagcaaactttagatgcttcctcagctatatcaaagctaaattgctctagcaacatcttcacatcccaagcatccttttcttcatttgggtaactttttgccatgttgtagtgcttttcaccaggttttacctcttgtggagacttgagaatgcgaatctatacttaaagagatcatatacttagaacacttccaaaataagtcagaaggctctgaatactgcattattttatctgttcaaaaaaagaatcgttctagaaaaaaaacattttaaaaccaaaattcataaattcttcagtaccaatattcaatgtttgaaacaaacagagaagcatatggtatggaaaacatatgtcaatgaattatttataatattataaatgtactcttaaattttcatatcctccatgtttattttgaaaaaataagaacttgggttacaggagcctaaaatatttattacgactacagtcgacaactcaggaaagaataataaaatatacatctctttgtgcatcaaaggaataaaaggctaagaatagagtcttctccttatacaggcatttcagacaaattcatattaaacctgcaaagaagaaaaaaaaaagtaacaaaggctcccattagtaagtgtgagataaagaaggaaaccatgctcagctcagagtttctgtgagtctctctgcctgcctgcctgcctgcctgcctgcagagaaggcccattctggtctcctctgccactgtgtggtaagtttactggggtggactctgcagttttgatggtggctggtcaaggtcaaatctgggatagaactacttagaagcccaccatgatacacatctaaaccacaccctccaatccatccttcatcagatgtaaagaagttaatgttttaatctcctatattattcctgtttcttcgactggttccaaatgcctaaagcaaaaagaaaatttacaggttccctgaaactcaaacatgatgcagctatttataataaaacaagtgaagcagctttacatgcatgaacatgaagtactctccaacatactgtgaaatgaaaaagcaaggtgtaaaagtgtactgcatagcaccgttgtgtcaaatacagacatatacatacactatacctgcatacgacatctctagaaagatacatatgaaactagtgacatgaatgtctttggggaaaggaactggtttgacaataaacaggctgcagagacttacttttcactggcttttgtactgtgtacatgttacctattcaaataataacttaaaaagaaaatgcgtaacagtgaaagagaatgaaaagggaaaaataattctcttagttttatacaagtaatatcaaagtttaacatttataaacatggtgaatgatttttaaaaattttttcaacctctaaattctatactatataacttataaaaatatggtttactacaaaaagcttggaaaaaaatagagataacaatttatataatttacatatcaaaatgtctctctgcccaaagcaataccctttgtcagaagcctttttaattagtcctagcaatttgaaataacttttaatatgagctattattaagatgacattaatataacattactagacacactctgttaacagattacaagaaatcagaaggagatatctgagaggaaagaacctaaaggttctgtatatataaatacagccttgcaaaggtacacagtattttttagtaaattttctgactaaggattcaatggtgcatgccagagttttaactaaagacttaagcataatcggaggggggaagaaaactacagagaatataaaggccatgaattcaaagaaggaacaaagcacagcagcataaaaggctttctacctaaagcgagactaaggacagaaaacttcacaatctagaactaattaacatcaaaaatactgcacaattcatcataaaaaatcattggcatctgagaaaacttatttacaattattgttaaggacaagtttttaggttttgaatacaagtgacaaatatttacattacaaaacttaagtaatataagccatatctattgataaatacctgctctatctgtattccatagcctttaaaacctgcattatcccatgaagtgttccgatagatgtcatcaactctgtcaattagctctattaagtaatttgtagttgtactctcttcccctctgcccatgtatctgtagaagcgatgatctgctaccaccaataatttacacgtgttcttcatgggatctgggtcagctcttcttttcactcgatgaacaagctctaatatgaatttgtatgcacttcaggtggttctctgtctactaacccttttgggagcaactcttcattatccacttttaaataaccacacacttttggagactgcaaacgtgaaacattcttgatatcttcagatttataaactaacattcttttgtctttggtatcattaacaaatctccaaagtggctctatgttatattcggccccatctgtgttgattctgattataacatcatcatctcttatgtgggctagaaccctagagtcaggctcaccaaccacgtgtccagtgaagaagtcctgccattttacagtgtactcgctttcgtttttaccatccaccaccacgaccttgaaattttgtgaaaaacgttcagtacttgatgtcaggtataatttaaaatgccttttcaaagctgaaaaagttagtagtgtttctacatgtgttgaagtctgtagatctctttttcttaccgaatgctgctggatattagataaagagagaatatcgtagtctgagagcaaagaatcaagcttcttcatgtgtggaagctaaaaaagtggatctcgtggaggtagacagcagaatggtggttaccagaggctgagaagggaagtgggagtggtggagatgaacagaaagtggttagtgttacaaaaatacagtttgattagtaagttctaatatttgatagtacagtacagaaattatagttaacaatttattgtatacttcaaaacagctagaagacttgtaatattcctaacacagaaaagatgtttcaaatgatgggtatcccaatcaccctgatttgatcactacatattatacacaggtatcaaaatatcacatgtacccaaaaaaca

SEQ ID NO: 13563 - RNA, 3549 nt, Homo sapiens
  source 1..3549: mol_type = other RNA
gctgggattacaggcatgagccaccactcccagccaatagtgaattttctaagagcatgtatccctatcagtaacagggatacatgaagatacttataaaatacagaaaaactgcccagcaaatcagggccctaaacagttggtagattccataaattcaactggctaccatgtatagccctcactgtaaggtaggtggttaggtttctagagagcattagtcttagaattatgaagagccatattaacccaaatgatttctaaatttagatatatattttccctgctacataaaaactctgggtaataactagaaatagacccacaatttagagacaatgtatactagatttatctcctttgtttttagttgaaggcaaaaaaaaaaaaaaaaaaaaaaaactattccagttgtcatcacaaataaatgccaaatgcctcatattcagcggttcattacagtgtataaaaaaaaactgatcatttccctagtcagtgctgttatcaatataaaagattaatttacaaaaacgtaaatattcataacccaatccagctgtattttctgcttttgcaccacaggtcaaaagatattttaaaaactaaaacctgaaagcctcaaaataagctagattcaccttcaccttaccttttcaaaaggagaagggccaaaccacacaagaactgtttacctgcaggaagttcaaacacatgaccagcatctgctaagtcacttcccagtcttcacaaaatacaagctgtgattgatttgtaggtcaaatctataaaaatattttgcacacttaagtcagaagagctgagaactaaattagcactctgtttctttgctgtcaacacgattctgacgctgcagtttaaaggaggcagccttttcacttctggtgaccggatggtccgtgagatcctcaaatgacttggcagctgtgctgctatttgggaaggggtccttctcaaacccatcctcgtccatatgtgagtctgtgctggggtcttcctggatggtgtccattctctggtggtccagttttggagctgctggcgccgaagggatcacaggggcaggctgcaggcggcctggagtctggggcgcaggaaagggtttgataatgcgaaccgatgcagaatccatgctgctcagcatttcgacgttactggggtgaaacagagacagagattcatactgtttatccaatttcttatccacacaatggacaagaatgctgaaaggaatccaaaatatcaaggagaaaaccaggacagacccaacgatgttgtctgctaaaaactttccaaaagtattgatgctcagctggtcaatgaaatcccaaaatcgttcaattacatcctgtactcgtttctcacatttgccattcatgtcacaaaatcctactgtacagggctttcctttcctcaaaaataagttcttttgttcagcatcgacatagggcacacagcggccagaaaggtccctgcagcacaccttgcaggagttgtcagtttcattacatgcacaggactccagctgctgttccctctcgcagaaagggatgcatttcccatccttacacttgccaagatccaagcaaacagtgtcatcttcagcatttcctggaggcgggcactcactgctattacctgtgcagtaggacacgcctttgcaagtagcattaatcgcctcctggcacttcttctgggcagtctcaaactgacagtttttacagcaaggactgttcctgtcactgcactggacaccttccttcaacgtgcagtcgctgttgcagcaggtgtcgttgttcagatacatgatgccaggatcacactcttctccttcatccaccctcgagttcccacaaactttattgctgcgttcttgaaaacactcctgggccttactttcaatggtcttatagattgattgtttactgcagtttgaaaacatcttattgttctcgtgatcgccactcacagctatgggatacatgacatatttccctccctggtcctcattcggggcacattctgctagaccatccggatcatgttctgctccaaaattatgtcccaattcatgagttgtaaccaggtcagcttcctttgtaaggatggttttaccataattctttgtgctcgtcaaaccactattcaaatagatatttttcttcccaactgggctataataagcctttggacaaacacctccatggctgtttgctctgggagagccaacataagctaatccaagagttcccatatcaaaatcttggtatgtgaaaaggtgtgccaagcaaactttagatgcttcctcagctatatcaaagctaaattgctctagcaacatcttcacatcccaagcatccttttcttcatttgggtaactttttgccatgttgtagtgcttttcaccaggttttacctcttgtggagacttgagaatgcgaatctgctctatctgtattccatagcctttaaaacctgcattatcccatgaagtgttccgatagatgtcatcaactctgtcaattagctctattaagtaatttgtagttgtactctcttcccctctgcccatgtatctgtagaagcgatgatctgctaccaccaataatttacacgtgttcttcatgggatctgggtcagctcttcttttcactcgatgaacaagctctaatatgaatttgtatgcacttcaggtggttctctgtctactaacccttttgggagcaactcttcattatccacttttaaataaccacacacttttggagactgcaaacgtgaaacattcttgatatcttcagatttataaactaacattcttttgtctttggtatcattaacaaatctccaaagtggctctatgttatattcggccccatctgtgttgattctgattataacatcatcatctcttatgtgggctagaaccctagagtcaggctcaccaaccacgtgtccagtgaagaagtcctgccattttacagtgtactcgctttcgtttttaccatccaccaccacgaccttgaaattttgtgaaaaacgttcagtacttgatgtcaggtataatttaaaatgccttttcaaagctgaaaaagttagtagtgtttctacatgtgttgaagtctgtagatctctttttcttaccgaatgctgctggatattagataaagagagaatatcgtagtctgagagcaaagaatcaagcttctcgagtctctggtgggggccgaagcccgggtcatccggaggtcgcggcgccagcacgaaaggaaccacgctggtcaggaataggagagactgcctcatgttcccggccccgctaccgactccacctctctgggcagccttcgcctgacggggtttcggaaaactgctcacatcgggggaggacgggatccgcccggcctagcccctcaatcctcttttccctcccgcgccgcctactgggaagattctaccgccaggctcgacgcccccagaagtgcaggtggcgttaccaaaggccggctcagccagcttccggccgccgct

SEQ ID NO: 13564 - RNA, 3529 nt, Homo sapiens
  source 1..3529: mol_type = other RNA
gctgggattacaggcatgagccaccactcccagccaatagtgaattttctaagagcatgtatccctatcagtaacagggatacatgaagatacttataaaatacagaaaaactgcccagcaaatcagggccctaaacagttggtagattccataaattcaactggctaccatgtatagccctcactgtaaggtaggtggttaggtttctagagagcattagtcttagaattatgaagagccatattaacccaaatgatttctaaatttagatatatattttccctgctacataaaaactctgggtaataactagaaatagacccacaatttagagacaatgtatactagatttatctcctttgtttttagttgaaggcaaaaaaaaaaaaaaaaaaaaaaaactattccagttgtcatcacaaataaatgccaaatgcctcatattcagcggttcattacagtgtataaaaaaaaactgatcatttccctagtcagtgctgttatcaatataaaagattaatttacaaaaacgtaaatattcataacccaatccagctgtattttctgcttttgcaccacaggtcaaaagatattttaaaaactaaaacctgaaagcctcaaaataagctagattcaccttcaccttaccttttcaaaaggagaagggccaaaccacacaagaactgtttacctgcaggaagttcaaacacatgaccagcatctgctaagtcacttcccagtcttcacaaaatacaagctgtgattgatttgtaggtcaaatctataaaaatattttgcacacttaagtcagaagagctgagaactaaattagcactctgtttctttgctgtcaacacgattctgacgctgcagtttaaaggaggcagccttttcacttctggtgaccggatggtccgtgagatcctcaaatgacttggcagctgtgctgctatttgggaaggggtccttctcaaacccatcctcgtccatatgtgagtctgtgctggggtcttcctggatggtgtccattctctggtggtccagttttggagctgctggcgccgaagggatcacaggggcaggctgcaggcggcctggagtctggggcgcaggaaagggtttgataatgcgaaccgatgcagaatccatgctgctcagcatttcgacgttactggggtgaaacagagacagagattcatactgtttatccaatttcttatccacacaatggacaagaatgctgaaaggaatccaaaatatcaaggagaaaaccaggacagacccaacgatgttgtctgctaaaaactttccaaaagtattgatgctcagctggtcaatgaaatcccaaaatcgttcaattacatcctgtactcgtttctcacatttgccattcatgtcacaaaatcctactgtacagggctttcctttcctcaaaaataagttcttttgttcagcatcgacatagggcacacagcggccagaaaggtccctgcagcacaccttgcaggagttgtcagtttcattacatgcacaggactccagctgctgttccctctcgcagaaagggatgcatttcccatccttacacttgccaagatccaagcaaacagtgtcatcttcagcatttcctggaggcgggcactcactgctattacctgtgcagtaggacacgcctttgcaagtagcattaatcgcctcctggcacttcttctgggcagtctcaaactgacagtttttacagcaaggactgttcctgtcactgcactggacaccttccttcaacgtgcagtcgctgttgcagcaggtgtcgttgttcagatacatgatgccaggatcacactcttctccttcatccaccctcgagttcccacaaactttattgctgcgttcttgaaaacactcctgggccttactttcaatggtcttatagattgattgtttactgcagtttgaaaacatcttattgttctcgtgatcgccactcacagctatgggatacatgacatatttccctccctggtcctcattcggggcacattctgctagaccatccggatcatgttctgctccaaaattatgtcccaattcatgagttgtaaccaggtcagcttcctttgtaaggatggttttaccataattctttgtgctcgtcaaaccactattcaaatagatatttttcttcccaactgggctataataagcctttggacaaacacctccatggctgtttgctctgggagagccaacataagctaatccaagagttcccatatcaaaatcttggtatgtgaaaaggtgtgccaagcaaactttagatgcttcctcagctatatcaaagctaaattgctctagcaacatcttcacatcccaagcatccttttcttcatttgggtaactttttgccatgttgtagtgcttttcaccaggttttacctcttgtggagacttgagaatgcgaatctgctctatctgtattccatagcctttaaaacctgcattatcccatgaagtgttccgatagatgtcatcaactctgtcaattagctctattaagtaatttgtagttgtactctcttcccctctgcccatgtatctgtagaagcgatgatctgctaccaccaataatttacacgtgttcttcatgggatctgggtcagctcttcttttcactcgatgaacaagctcttcaggtggttctctgtctactaacccttttgggagcaactcttcattatccacttttaaataaccacacacttttggagactgcaaacgtgaaacattcttgatatcttcagatttataaactaacattcttttgtctttggtatcattaacaaatctccaaagtggctctatgttatattcggccccatctgtgttgattctgattataacatcatcatctcttatgtgggctagaaccctagagtcaggctcaccaaccacgtgtccagtgaagaagtcctgccattttacagtgtactcgctttcgtttttaccatccaccaccacgaccttgaaattttgtgaaaaacgttcagtacttgatgtcaggtataatttaaaatgccttttcaaagctgaaaaagttagtagtgtttctacatgtgttgaagtctgtagatctctttttcttaccgaatgctgctggatattagataaagagagaatatcgtagtctgagagcaaagaatcaagcttctcgagtctctggtgggggccgaagcccgggtcatccggaggtcgcggcgccagcacgaaaggaaccacgctggtcaggaataggagagactgcctcatgttcccggccccgctaccgactccacctctctgggcagccttcgcctgacggggtttcggaaaactgctcacatcgggggaggacgggatccgcccggcctagcccctcaatcctcttttccctcccgcgccgcctactgggaagattctaccgccaggctcgacgcccccagaagtgcaggtggcgttaccaaaggccggctcagccagcttccggccgccgct

SEQ ID NO: 13565 - RNA, 3538 nt, Homo sapiens
  source 1..3538: mol_type = other RNA
gctgggattacaggcatgagccaccactcccagccaatagtgaattttctaagagcatgtatccctatcagtaacagggatacatgaagatacttataaaatacagaaaaactgcccagcaaatcagggccctaaacagttggtagattccataaattcaactggctaccatgtatagccctcactgtaaggtaggtggttaggtttctagagagcattagtcttagaattatgaagagccatattaacccaaatgatttctaaatttagatatatattttccctgctacataaaaactctgggtaataactagaaatagacccacaatttagagacaatgtatactagatttatctcctttgtttttagttgaaggcaaaaaaaaaaaaaaaaaaaaaaaactattccagttgtcatcacaaataaatgccaaatgcctcatattcagcggttcattacagtgtataaaaaaaaactgatcatttccctagtcagtgctgttatcaatataaaagattaatttacaaaaacgtaaatattcataacccaatccagctgtattttctgcttttgcaccacaggtcaaaagatattttaaaaactaaaacctgaaagcctcaaaataagctagattcaccttcaccttaccttttcaaaaggagaagggccaaaccacacaagaactgtttacctgcaggaagttcaaacacatgaccagcatctgctaagtcacttcccagtcttcacaaaatacaagctgtgattgatttgtaggtcaaatctataaaaatattttgcacacttaagtcagaagagctgagaactaaattagcactctgtttctttgctgtcaacacgattctgacgctgcagtttaaaggaggcagccttttcacttctggtgaccggatggtccgtgagatcctcaaatgacttggcagctgtgctgctatttgggaaggggtccttctcaaacccatcctcgtccatatgtgagtctgtgctggggtcttcctggatggtgtccattctctggtggtccagttttggagctgctggcgccgaagggatcacaggggcaggctgcaggcggcctggagtctggggcgcaggaaagggtttgataatgcgaaccgatgcagaatccatgctgctcagcatttcgacgttactggggtgaaacagagacagagattcatactgtttatccaatttcttatccacacaatggacaagaatgctgaaaggaatccaaaatatcaaggagaaaaccaggacagacccaacgatgttgtctgctaaaaactttccaaaagtattgatgctcagctggtcaatgaaatcccaaaatcgttcaattacatcctgtactcgtttctcacatttgccattcatgtcacaaaatcctactgtacagggctttcctttcctcaaaaataagttcttttgttcagcatcgacatagggcacacagcggccagaaaggtccctgcagcacaccttgcaggagttgtcagtttcattacatgcacaggactccagctgctgttccctctcgcagaaagggatgcatttcccatccttacacttgccaagatccaagcaaacagtgtcatcttcagcatttcctggaggcgggcactcactgctattacctgtgcagtaggacacgcctttgcaagtagcattaatcgcctcctggcacttcttctgggcagtctcaaactgacagtttttacagcaaggactgttcctgtcactgcactggacaccttccttcaacgtgcagtcgctgttgcagcaggtgtcgttgttcagatacatgatgccaggatcacactcttctccttcatccaccctcgagttcccacaaactttattgctgcgttcttgaaaacactcctgggccttactttcaatggtcttatagattgattgtttactgcagtttgaaaacatcttattgttctcgtgatcgccactcacagctatgggatacatgacatatttccctccctggtcctcattcggggcacattctgctagaccatccggatcatgttctgctccaaaattatgtcccaattcatgagttgtaaccaggtcagcttcctttgtaaggatggttttaccataattctttgtgctcgtcaaaccactattcaaatagatatttttcttcccaactgggctataataagcctttggacaaacacctccatggctgtttgctctgggagagccaacataagctaatccaagagttcccatatcaaaatcttggtatgtgaaaaggtgtgccaagcaaactttagatgcttcctcagctatatcaaagctaaattgctctagcaacatcttcacatcccaagcatccttttcttcatttgggtaactttttgccatgttgtagtgcttttcaccaggttttacctcttgtggagacttgagaatgcgaatctgctctatctgtattccatagcctttaaaacctgcattatcccatgaagtgttccgatagatgtcatcaactctgtcaattagctctattaagtaatttgtagttgtactctcttcccctctgcccatgtatctgtagaagcgatgatctgctaccaccaataatttacacgtgttcttcatgggatctgggtcagctcttcttttcactcgatgaacaagctcttcaggtggttctctgtctactaacccttttgggagcaactcttcattatccacttttaaataaccacacacttttggagactgcaaacgtgaaacattcttgatatcttcagatttataaactaacattcttttgtctttggtatcattaacaaatctccaaagtggctctatgttatattcggccccatctgtgttgattctgattataacatcatcatctcttatgtgggctagaaccctagagtcaggctcaccaaccacgtgtccagtgaagaagtcctgccattttacagtgtactcgctttcgtttttaccatccaccaccacgaccttgaaattttgtgaaaaacgttcagtacttgatgtcaggtataatttaaaatgccttttcaaagctgaaaaagttagtagtgtttctacatgtgttgaagtctgtagatctctttttcttaccgaatgctgctggatattagataaagagagaatatcgtagtctgagagcaaagaatcaagcttcttcatgtgtggaagctaaaaaagtggatctcgtggaggtagacagcagaatggtggttaccagaggctgagaagggaagtgggagtggtggagatgaacagaaagtggttagtgttacaaaaatacagtttgattagtaagttctaatatttgatagtacagtacagaaattatagttaacaatttattgtatacttcaaaacagctagaagacttgtaatattcctaacacagaaaagatgtttcaaatgatgggtatcccaatcaccctgatttgatcactacatattatacacaggtatcaaaatatcacatgtacccaaaaaacacat

SEQ ID NO: 13566 - RNA, 1088 nt, Homo sapiens
  source 1..1088: mol_type = other RNA
gctgggattacaggcatgagccaccactcccagccactatgcattcagaaagatgagaaatcgtgaagtcatgaccactcacctctaataccaacctgacaacgtctctaagataatttataaagcggtgttgaagtaaagggaatgggctttgagtgtctgctggtaacattgacccacatgctcttgcagttgctgcttggcagagatctctctctttgcggatttaaagttaacagaagacctttggggactgtggagagggaactgggcctaaaataccccactaaactgcttgatgaaaactggagactaatcttacaaaaaggaatcttcctgcccagtccagtttccaacctctaagaaaagttgcagaaataaaaatattcgccattgtaccttgaaccagttgtcattttagcacccaacagttttcccctttctaccttccgcagattagttacatgaaaaagcttgttgaaatagttcaaaggatgagttcatgaatccaatcccagaaacatgaataaactgatgactagttggccttggagaacatcttgagtattatcctctgcaatctgtacaactgccccagacgcactttaggagttatgcatcggagatgacaggtaacatgccaccacatcacagaacacaaatgtcttgggtccactccttggattcactctggagactgatgtcggcttgtcaattcaagtttcagatgtccggactccaagtgccagttccttcccggtgttcagccactgtgttaatcctccacaggggcctgctacgtgctgttctggtgaggcgttccacccaggcaattttctacccaggagtgctctttggatcacgtcactcaggctggccagagtcccctgcagggatgctccacagggcaggcctaagctgcctaaggggctacctcggccatccctcagttacctcgattcccggtcaggggaccaagaaatgtagaaggacgagccgcagacaaaacctctcagacaccaagttgtagaaggaagggctttattcagctgggaggatcggcaagctgctgccttaaaatccgagca

SEQ ID NO: 13567 - RNA, 1153 nt, Homo sapiens
  source 1..1153: mol_type = other RNA
gctgggattacaggcatgagccaccactcccagccagtaatacttaaggctcatgctaggcttgaaaacaggtctactatactggcacagagaaataggtaagcatgagaccccggcactgggcacagctctctgctggggaaaccctgggagatggctcccctgcagggcggtttactcctggcctccagaagcttatctgttagtggaccgtgggcacacaagttttctttcccctttgtgtattcaccctcaaaagggcaaatttctacactataagttgttgctggactaacatcgaataataaagtacttctttagcaagattcaagttgaattcaatccttgtgaattctagaagcaattaacattatgagaatacagtagtccccctttatgtgaagtttcactttctgtggtttgttatccacagtcaacggcagctcaaaaatgggtgaacacacagcacaacaggatattttgagagagagagaaaacaaattcacataacttttaatagaacatatagttataactgttctattcttacttatttttgttaatttcttcctgtgcctaatttataaattaaactttatcacaggtatgtattacatacaggggaaaaacataatatatagagacttcagtactatcagtggtttcagacatccactggagatcttggaggtggataaggggggaccatggtgtttcaaaatcttgtttggagtttacaaagggaatgcttaatttctgatttatctaacaaaagatacctgtagacttacctgtcatacaaaataaccacactgaataatagcttgtcatagcaaatcttcccctccaactactcatacccctttctctctcttcaagtcctaaattcaagtaatacttcacttgacacttatttatctccaggattatcatataactaccattgacagttagatccacttttttgcaattgactgaacaacccaatcaatagcaacaaggacactctgctttcacaagatgacagctgctccagctgctggctccctggggctgatgttggggaatcaggccagcacaacatgacacattcacagggacacggacaccaggtacaacactacatctacatgggtcattagcttgactatag

SEQ ID NO: 13568 - RNA, 6885 nt, Homo sapiens
  source 1..6885: mol_type = other RNA
gctgggattacaggcatgagccaccactcccagcctgataactgttttatttatttatttttatttttttggagatatggggtctgtgttgcccagactgatcttgaactcctggcctcaaggaatccttctgactgagcttcccagtgtgctgggattaaaagtgtgagccactatgaccagccagaagagataattttaactttttaaaatattttgcagtattggccgggcacagtggcttgtgcctgtaatcccagtactttgggagtatgaggcatgcagatcacctgaggtcaggagtttgagaccagcctggccaacttgatgaaaccgtctctactaaaaatacaaaaatcagccaggcaaggtggaggctgtctgtaatctcagctactcgggaggctgaggcaggagaaccactggaacccaggaggtggaatttgcagtaagttgagatcacaccattgcactccagcctgggcaacgagtgaaacactaactcaaaaacaaagaaacaaacaccaactcaaaaacaaagaaacaaaccaaaaaaatgaaaatatcttgtagtatttttaaatagagatgtggtttcgctatgttgcccaggctggtttgaactccttggctcaagggatctttttgcctcagcctccaaaagtgctgggattacaggcctgagccactattcccaacctagatgactcttatagattaagaatttagaaatagtaggaacatgccccactacagtatatgacagtcattatatacaaatatcattaagggacaattttttaaaaatcacaatgttattcaaacatagctccataacatattagtaaaggtcatgaagtatttttaagtgatccattatgtcacagtcgagcttatccaggaatacaaggttgatgtaacattggaaaagcaataaatacaaataccacatttatttaatttaatttatttatttttgacagagtcgcaccctgtcacccagcatggagtgcagtggtgcaatcttggctcaatgcaacctccacctcccaggttcaagtgattctcctgcttcagcctcccaagtagctgggattacaggtgcacatcaccacacccagctaatttttgtattgttagtagagatggggtttcaccatgttggctgggctggtctcgaactcttgacctcaaatgatctgcccacccccacctcccaaattgctgggattacaggcataagcccccacacccagcctgaccacatttgttttagaaaagcgcctttccatgcattcacttcttcaagttttttttttgttttgtttttgtttttttttttgagatggggtcttgctatgttgcctaagctggtctagaacccctgggctcaggccaccctcccaagtagctaaaactataggcatgcatcaccacatcatttcattgaagtatttattaggtaccatcatgagctaggtgcagttctaggtattgagttttatcagtaaataaacatgatcatcacagaggatgtgaaggaagcatttaataaattcaagaggaattcagcctcataaactatgaaatattgggaaataattcatcatgtaaaaactggatataaagaaaaaacttttcctgcaggacattgttgcaggaagtcagggaccccaaacggggggactggctgaagccatggcagaaaaacatggattgtgaaggtttcatggacatttattagttccccaaattaatacttttataatttcttatgcctgtctttactgcaatctctaaacataaattgtaaagatttcatggacacttatcacttccccagtcaatacccttgtgatttcctatgcctgtctttactttaatctctcaatcctgtcagctgaggaggatgtatattacctcaggaccctgtaataattgcattaactgcacaaattatacagcatgtgtgtttgagcaatatgaaatctgggcaccttgaaaaaagaacaggataacagcaatgtttaggaaacaagagagataaccttaaattctgaccgccggtgagccaggtggaacaaagccacatttctcttctttcacaagcaaatgggagaaatatcactgaattctttttctcagcaaggaacatccttgagaaagagaatgcacacctgggagtgggtctctgaactggcccccctgggtgtagccatctcttatggtcgagactgcaggggtgaaatagaccccagtctcccatagcactcccaggcttattaggaagaggaaattcccacctaataaattttagtcagaccagttgatctcaaaaccgtctcctgataagatgttatcaatgacaatggtgcccaaaacttcattagcaattttaatttcaccttggtcctgtgatctcgccctgcctccacttgccttgtgatattctattaccttgtaaagtacttgatgtctgtgacccacacctatttgcacactccctccccttttgaaaatccctaataaaaacttgctggtttttgcggcttgtggggcatcacggaacctaccgacatgtgatgtctgccccggacacccagctttaaaatttctctcttttgtactctgtccctttatttctcaagttggctgacacttagggaaaatagaaaagaacctatgtgaatatcggggctggttccctgacaggacataacctcttcaaaaaataaaaaagaaataaaagcctacagccaaaccaacaaaatagagtgcatatctcaccagaactgcaaagacaagtatgctggtattactacttttagttggtgttgtgcagcgggttaaaatcagtccagtaaagcaagaaaatatttagagagagcttcatcatcatacgaattttgggggtcattgttcagtccaaagtacttaatatgattcttttctctttccacatagagaatcagataatctataaataatgactcttactgttccactttaggagttaggtatacatacatatgtgtatatatatgtatatatatatacacatacacacacacacacacacacacacagtgaccccccaaatttcatatgaagttccaaacctcaatgtgactgtatgtgaaaagagaagggggcggggaggggggagaccgaccgacctatttgttggtctccatcgtgtgaaaacatgaggaagtgggcacttacatgccaggaagagagctctcactagaggttgaccatgctggcactctgatctcagacttccagcctccagatatgtgagaatataaatttgtgttttgggccagatacggtggctcaggcctgtaatcccagcactttgggaggccaaggcaggtggatcaccaaaggtcagatctgaccaacatggagatcagcctaaccaacatggagaaaccctgtctctactaaaaatacaaacttagctaaggtttgtggtgcatgccaataatcccagctactgagggtgaggcaggagaatcactggaactcaggaggtggaggttgcggtgagccaagatcataccattgcactccagcctgggcaacaagagcaaaactccatctcaaaaaaaaaaaaaaaaaaaaaaaaaaaatcctgtgtttttaacctcattgatttaaaattaaattaatttctaagccatttggtctgcggtattctcttatggttgtctgagctgactaaggcagatattggtactgagaagtgaggtactgcaattaaaaacaaacaaaaaaactaaaaatgtgaagcagctttgaaactgacaaatgagtagaggctggaaaaattctgatgtgcaagctggaaataaggttggtaagggttattctggtgaggtgtcattggggaatgaggaacatgctattgggaaatgaagaaaagacaacccttgatataaagtggtgaagaacttggcagaactgtattctagcattttacggaaggtagagcttgagacagataaaatggtatgtatcactaagatctgtaattaaagtgttaaaggacacaggaagcttcattattcctgagtgcttacaggaaaatgtgctgggaacaggccccccaaatctggccataaacaggcaatgagaaactggccataaacaaaatctctgcagcactgtgacatgctcgtgatggctatgacgcccatgctggaggctgctggtttaccagaatgagggcaagcaacacctggcccacccagggcagaaaactggaaaactgctcaaggcattcctaaaccacaaacaatagcatgagtgatttgtgccttaaggacatattcctgttgcagataacaagccagagcctgtccctttctttctcataaggaatacttatagctgatctacaatctataggaataatgtttatcacaggcttactgtcaataaatatgtgggtcaaactctgttcaagctcagctctgaaggctgtgagccccgattcccactctgcactatatttctgtgtctttgtcttaattcctctagagccactgggttagggtctccacgacccagctggtctcggcaaaaatgcaaaaggagacctgaattgcagaagaaattgttaaggaaaaaggaaccagaacttggagatttggaaaattctcagcctatccatactgcaaaaattagaaaacttgtactgaagagaatcctcaaagtgtggctgaacaatcatttgataaagagatcatgagtgggattcatggactatatcagccatcttaacagaagtgagaagagagactggattatactataagagacactgccacttacattgtgccacctaaaatggacagagaagacagaacagaacagtcaaggttgtcacacttcttattttacaagaaggggacatagaaataatcagctgtgaaagggcactggcagttatggatggtttcactcctgacatgctctgcaggatccatgggaacagaagagaaccttggaggagcatctttttaacaatccacctctggggcctacatcatcttggcttctggtaaattttgacatgaatgtgccacactggcagccactaaccaacaggggctgggatcaatctgcatgatttatctcgtacagaacttgttaatgctatgatcttaggaatctaatcaccaaggtgaggcagcctgcagtactgacctcaccatccatgacccttcttcacagatgcccagactcaggtaaccatgatgttgtattcagaacctgtaggtttaatttcagaccctcgggatgcatctaaggccaatctgtgagccattacaacctccaaaaggcatttaggactaatctgatgatctttgcactgccaataattaaagatggcaaccaatgggctaaatggtaacaacactcatatccttacattcatagtatttctccccagtgtgaattctttcatgcatacttaggcatgaggaaagagcaaatgctttcccaaattctttacatacaaaaggtttctctctggtaggagttcacaggtggggtgaggaatacagaaattctttcccacatatcttgcatttacctttctccactgtgagttttcaaatgtttactacgatgggaagaagtaatgaaggtcttcccacattcaacacattcataaggcttctctcctgtgtgaattcttctatgttgagtaagcgttgaagatctattgaaggctttcccacattccttacactgatagggtttctctccagtgtgatttcgtatgtgtatagcaaggcccgtgtactgagtgaaggcttggccacattccttacattcatagggttttattccagtgtgagttcttacatgttgagtaaggtgagttgatctagtgaaggctttcccacattccgtacatttgtgtggttttattccagtgtgaatttgaatgtgaacattaaaggatgaggaatttctaaaggatcttccacattctttacattcaaaggacttctctcctttatgagtttttgcatgtgcagaaagttgagaaaaattagtgaaggatttcccacagttcttagtcttttcggatttctttccagtatgaactgctacacactgctttaagtgtgaggaagttgtgatggctctctcacattcctgaaattcacagagtttctctccaatgtggattcccatgtgattatcaaggcttgcaaaatacttaaagccttttccacattccttacatttgtagggttgtcttccattgagaatttcaagatgcacagcaaggcctggagttaaggtgaagacttttccacatggattaaatttggaaagttcttgtccaatagaggcttccttgtgcacactgatgctgtcttttccataacaattaccctcaaaagtgttccctccattctgagctctcatgtgtgtcttaaggcaaaactgttcactgaagacctctccacaattctcacagagtttccatccactgtagcttcttgtctgcatttgtatcccagtgaatatttgattcttcaaaaaaccctgctgaagtgatgaccgtttggttctaggttgtatttcccattctgaagttaagcagaaaaagaaatcatgggacatatcaaaggctgacatcctctgaagctgatggtgagatgtgcctcaatgctgtctttcttgatgccaagatcgcctcagggcagcttatgaatctaggtggatacaggcaatctccattcccctttgtacagggttatctgaggcccacagcggggtggactccaccacaataaaggttaaacggcactgaccatgctgagccacagccggtaaagatggcggtggcacact

SEQ ID NO: 13569 - RNA, 7048 nt, Homo sapiens
  source 1..7048: mol_type = other RNA
gctgggattacaggcatgagccaccactcccagcctgataactgttttatttatttatttttatttttttggagatatggggtctgtgttgcccagactgatcttgaactcctggcctcaaggaatccttctgactgagcttcccagtgtgctgggattaaaagtgtgagccactatgaccagccagaagagataattttaactttttaaaatattttgcagtattggccgggcacagtggcttgtgcctgtaatcccagtactttgggagtatgaggcatgcagatcacctgaggtcaggagtttgagaccagcctggccaacttgatgaaaccgtctctactaaaaatacaaaaatcagccaggcaaggtggaggctgtctgtaatctcagctactcgggaggctgaggcaggagaaccactggaacccaggaggtggaatttgcagtaagttgagatcacaccattgcactccagcctgggcaacgagtgaaacactaactcaaaaacaaagaaacaaacaccaactcaaaaacaaagaaacaaaccaaaaaaatgaaaatatcttgtagtatttttaaatagagatgtggtttcgctatgttgcccaggctggtttgaactccttggctcaagggatctttttgcctcagcctccaaaagtgctgggattacaggcctgagccactattcccaacctagatgactcttatagattaagaatttagaaatagtaggaacatgccccactacagtatatgacagtcattatatacaaatatcattaagggacaattttttaaaaatcacaatgttattcaaacatagctccataacatattagtaaaggtcatgaagtatttttaagtgatccattatgtcacagtcgagcttatccaggaatacaaggttgatgtaacattggaaaagcaataaatacaaataccacatttatttaatttaatttatttatttttgacagagtcgcaccctgtcacccagcatggagtgcagtggtgcaatcttggctcaatgcaacctccacctcccaggttcaagtgattctcctgcttcagcctcccaagtagctgggattacaggtgcacatcaccacacccagctaatttttgtattgttagtagagatggggtttcaccatgttggctgggctggtctcgaactcttgacctcaaatgatctgcccacccccacctcccaaattgctgggattacaggcataagcccccacacccagcctgaccacatttgttttagaaaagcgcctttccatgcattcacttcttcaagttttttttttgttttgtttttgtttttttttttgagatggggtcttgctatgttgcctaagctggtctagaacccctgggctcaggccaccctcccaagtagctaaaactataggcatgcatcaccacatcatttcattgaagtatttattaggtaccatcatgagctaggtgcagttctaggtattgagttttatcagtaaataaacatgatcatcacagaggatgtgaaggaagcatttaataaattcaagaggaattcagcctcataaactatgaaatattgggaaataattcatcatgtaaaaactggatataaagaaaaaacttttcctgcaggacattgttgcaggaagtcagggaccccaaacggggggactggctgaagccatggcagaaaaacatggattgtgaaggtttcatggacatttattagttccccaaattaatacttttataatttcttatgcctgtctttactgcaatctctaaacataaattgtaaagatttcatggacacttatcacttccccagtcaatacccttgtgatttcctatgcctgtctttactttaatctctcaatcctgtcagctgaggaggatgtatattacctcaggaccctgtaataattgcattaactgcacaaattatacagcatgtgtgtttgagcaatatgaaatctgggcaccttgaaaaaagaacaggataacagcaatgtttaggaaacaagagagataaccttaaattctgaccgccggtgagccaggtggaacaaagccacatttctcttctttcacaagcaaatgggagaaatatcactgaattctttttctcagcaaggaacatccttgagaaagagaatgcacacctgggagtgggtctctgaactggcccccctgggtgtagccatctcttatggtcgagactgcaggggtgaaatagaccccagtctcccatagcactcccaggcttattaggaagaggaaattcccacctaataaattttagtcagaccagttgatctcaaaaccgtctcctgataagatgttatcaatgacaatggtgcccaaaacttcattagcaattttaatttcaccttggtcctgtgatctcgccctgcctccacttgccttgtgatattctattaccttgtaaagtacttgatgtctgtgacccacacctatttgcacactccctccccttttgaaaatccctaataaaaacttgctggtttttgcggcttgtggggcatcacggaacctaccgacatgtgatgtctgccccggacacccagctttaaaatttctctcttttgtactctgtccctttatttctcaagttggctgacacttagggaaaatagaaaagaacctatgtgaatatcggggctggttccctgacaggacataacctcttcaaaaaataaaaaagaaataaaagcctacagccaaaccaacaaaatagagtgcatatctcaccagaactgcaaagacaagtatgctggtattactacttttagttggtgttgtgcagcgggttaaaatcagtccagtaaagcaagaaaatatttagagagagcttcatcatcatacgaattttgggggtcattgttcagtccaaagtacttaatatgattcttttctctttccacatagagaatcagataatctataaataatgactcttactgttccactttaggagttaggtatacatacatatgtgtatatatatgtatatatatatacacatacacacacacacacacacacacacagtgaccccccaaatttcatatgaagttccaaacctcaatgtgactgtatgtgaaaagagaagggggcggggaggggggagaccgaccgacctatttgttggtctccatcgtgtgaaaacatgaggaagtgggcacttacatgccaggaagagagctctcactagaggttgaccatgctggcactctgatctcagacttccagcctccagatatgtgagaatataaatttgtgttttgggccagatacggtggctcaggcctgtaatcccagcactttgggaggccaaggcaggtggatcaccaaaggtcagatctgaccaacatggagatcagcctaaccaacatggagaaaccctgtctctactaaaaatacaaacttagctaaggtttgtggtgcatgccaataatcccagctactgagggtgaggcaggagaatcactggaactcaggaggtggaggttgcggtgagccaagatcataccattgcactccagcctgggcaacaagagcaaaactccatctcaaaaaaaaaaaaaaaaaaaaaaaaaaaatcctgtgtttttaacctcattgatttaaaattaaattaatttctaagccatttggtctgcggtattctcttatggttgtctgagctgactaaggcagatattggtactgagaagtgaggtactgcaattaaaaacaaacaaaaaaactaaaaatgtgaagcagctttgaaactgacaaatgagtagaggctggaaaaattctgatgtgcaagctggaaataaggttggtaagggttattctggtgaggtgtcattggggaatgaggaacatgctattgggaaatgaagaaaagacaacccttgatataaagtggtgaagaacttggcagaactgtattctagcattttacggaaggtagagcttgagacagataaaatggtatgtatcactaagatctgtaattaaagtgttaaaggacacaggaagcttcattattcctgagtgcttacaggaaaatgtgctgggaacaggccccccaaatctggccataaacaggcaatgagaaactggccataaacaaaatctctgcagcactgtgacatgctcgtgatggctatgacgcccatgctggaggctgctggtttaccagaatgagggcaagcaacacctggcccacccagggcagaaaactggaaaactgctcaaggcattcctaaaccacaaacaatagcatgagtgatttgtgccttaaggacatattcctgttgcagataacaagccagagcctgtccctttctttctcataaggaatacttatagctgatctacaatctataggaataatgtttatcacaggcttactgtcaataaatatgtgggtcaaactctgttcaagctcagctctgaaggctgtgagccccgattcccactctgcactatatttctgtgtctttgtcttaattcctctagagccactgggttagggtctccacgacccagctggtctcggcaaaaatgcaaaaggagacctgaattgcagaagaaattgttaaggaaaaaggaaccagaacttggagatttggaaaattctcagcctatccatactgcaaaaattagaaaacttgtactgaagagaatcctcaaagtgtggctgaacaatcatttgataaagagatcatgagtgggattcatggactatatcagccatcttaacagaagtgagaagagagactggattatactataagagacactgccacttacattgtgccacctaaaatggacagagaagacagaacagaacagtcaaggttgtcacacttcttattttacaagaaggggacatagaaataatcagctgtgaaagggcactggcagttatggatggtttcactcctgacatgctctgcaggatccatgggaacagaagagaaccttggaggagcatctttttaacaatccacctctggggcctacatcatcttggcttctggtaaattttgacatgaatgtgccacactggcagccactaaccaacaggggctgggatcaatctgcatgatttatctcgtacagaacttgttaatgctatgatcttaggaatctaatcaccaaggtgaggcagcctgcagtactgacctcaccatccatgacccttcttcacagatgcccagactcaggtaaccatgatgttgtattcagaacctgtaggtttaatttcagaccctcgggatgcatctaaggccaatctgtgagccattacaacctccaaaaggcatttaggactaatctgatgatctttgcactgccaataattaaagatggcaaccaatgggctaaatggtaacaacactcatatccttacattcatagtatttctccccagtgtgaattctttcatgcatacttaggcatgaggaaagagcaaatgctttcccaaattctttacatacaaaaggtttctctctggtaggagttcacaggtggggtgaggaatacagaaattctttcccacatatcttgcatttacctttctccactgtgagttttcaaatgtttactacgatgggaagaagtaatgaaggtcttcccacattcaacacattcataaggcttctctcctgtgtgaattcttctatgttgagtaagcgttgaagatctattgaaggctttcccacattccttacactgatagggtttctctccagtgtgatttcgtatgtgtatagcaaggcccgtgtactgagtgaaggcttggccacattccttacattcatagggttttattccagtgtgagttcttacatgttgagtaaggtgagttgatctagtgaaggctttcccacattccgtacatttgtgtggttttattccagtgtgaatttgaatgtgaacattaaaggatgaggaatttctaaaggatcttccacattctttacattcaaaggacttctctcctttatgagtttttgcatgtgcagaaagttgagaaaaattagtgaaggatttcccacagttcttagtcttttcggatttctttccagtatgaactgctacacactgctttaagtgtgaggaagttgtgatggctctctcacattcctgaaattcacagagtttctctccaatgtggattcccatgtgattatcaaggcttgcaaaatacttaaagccttttccacattccttacatttgtagggttgtcttccattgagaatttcaagatgcacagcaaggcctggagttaaggtgaagacttttccacatggattaaatttggaaagttcttgtccaatagaggcttccttgtgcacactgatgctgtcttttccataacaattaccctcaaaagtgttccctccattctgagctctcatgtgtgtcttaaggcaaaactgttcactgaagacctctccacaattctcacagagtttccatccactgtagcttcttgtctgcatttgtatcccagtgaatatttgattcttcaaaaaaccctgctgaagtgatgaccgtttggttctaggttgtatttcccattctgaagttaagcagaaaaagaaatccacagaggccaggttcatgtagttctccagcatcacatctctgtagaggtatttctgagttgtgtccagtaaagcccactcctctggggtgaactccacagccacatcatcaaacgtcactgaatcctggtaagaatttgaccggtggtcctctaccatcgttcctatctttgtcttttcttcaaaaggacagattggttccctgggaaaaaacccatgggacatatcaaaggctgacatcctctgaagctgatggtgagatgtgcctcaatgctgtctttcttgatgccaagatcgcctcagggcagcttatgaatcacagcggggtggactccaccacaataaaggttaaacggcactgaccatgctgagccacagccggtaaagatggcggtggcacact

SEQ ID NO: 13570 - RNA, 7101 nt, Homo sapiens
  source 1..7101: mol_type = other RNA
gctgggattacaggcatgagccaccactcccagcctgataactgttttatttatttatttttatttttttggagatatggggtctgtgttgcccagactgatcttgaactcctggcctcaaggaatccttctgactgagcttcccagtgtgctgggattaaaagtgtgagccactatgaccagccagaagagataattttaactttttaaaatattttgcagtattggccgggcacagtggcttgtgcctgtaatcccagtactttgggagtatgaggcatgcagatcacctgaggtcaggagtttgagaccagcctggccaacttgatgaaaccgtctctactaaaaatacaaaaatcagccaggcaaggtggaggctgtctgtaatctcagctactcgggaggctgaggcaggagaaccactggaacccaggaggtggaatttgcagtaagttgagatcacaccattgcactccagcctgggcaacgagtgaaacactaactcaaaaacaaagaaacaaacaccaactcaaaaacaaagaaacaaaccaaaaaaatgaaaatatcttgtagtatttttaaatagagatgtggtttcgctatgttgcccaggctggtttgaactccttggctcaagggatctttttgcctcagcctccaaaagtgctgggattacaggcctgagccactattcccaacctagatgactcttatagattaagaatttagaaatagtaggaacatgccccactacagtatatgacagtcattatatacaaatatcattaagggacaattttttaaaaatcacaatgttattcaaacatagctccataacatattagtaaaggtcatgaagtatttttaagtgatccattatgtcacagtcgagcttatccaggaatacaaggttgatgtaacattggaaaagcaataaatacaaataccacatttatttaatttaatttatttatttttgacagagtcgcaccctgtcacccagcatggagtgcagtggtgcaatcttggctcaatgcaacctccacctcccaggttcaagtgattctcctgcttcagcctcccaagtagctgggattacaggtgcacatcaccacacccagctaatttttgtattgttagtagagatggggtttcaccatgttggctgggctggtctcgaactcttgacctcaaatgatctgcccacccccacctcccaaattgctgggattacaggcataagcccccacacccagcctgaccacatttgttttagaaaagcgcctttccatgcattcacttcttcaagttttttttttgttttgtttttgtttttttttttgagatggggtcttgctatgttgcctaagctggtctagaacccctgggctcaggccaccctcccaagtagctaaaactataggcatgcatcaccacatcatttcattgaagtatttattaggtaccatcatgagctaggtgcagttctaggtattgagttttatcagtaaataaacatgatcatcacagaggatgtgaaggaagcatttaataaattcaagaggaattcagcctcataaactatgaaatattgggaaataattcatcatgtaaaaactggatataaagaaaaaacttttcctgcaggacattgttgcaggaagtcagggaccccaaacggggggactggctgaagccatggcagaaaaacatggattgtgaaggtttcatggacatttattagttccccaaattaatacttttataatttcttatgcctgtctttactgcaatctctaaacataaattgtaaagatttcatggacacttatcacttccccagtcaatacccttgtgatttcctatgcctgtctttactttaatctctcaatcctgtcagctgaggaggatgtatattacctcaggaccctgtaataattgcattaactgcacaaattatacagcatgtgtgtttgagcaatatgaaatctgggcaccttgaaaaaagaacaggataacagcaatgtttaggaaacaagagagataaccttaaattctgaccgccggtgagccaggtggaacaaagccacatttctcttctttcacaagcaaatgggagaaatatcactgaattctttttctcagcaaggaacatccttgagaaagagaatgcacacctgggagtgggtctctgaactggcccccctgggtgtagccatctcttatggtcgagactgcaggggtgaaatagaccccagtctcccatagcactcccaggcttattaggaagaggaaattcccacctaataaattttagtcagaccagttgatctcaaaaccgtctcctgataagatgttatcaatgacaatggtgcccaaaacttcattagcaattttaatttcaccttggtcctgtgatctcgccctgcctccacttgccttgtgatattctattaccttgtaaagtacttgatgtctgtgacccacacctatttgcacactccctccccttttgaaaatccctaataaaaacttgctggtttttgcggcttgtggggcatcacggaacctaccgacatgtgatgtctgccccggacacccagctttaaaatttctctcttttgtactctgtccctttatttctcaagttggctgacacttagggaaaatagaaaagaacctatgtgaatatcggggctggttccctgacaggacataacctcttcaaaaaataaaaaagaaataaaagcctacagccaaaccaacaaaatagagtgcatatctcaccagaactgcaaagacaagtatgctggtattactacttttagttggtgttgtgcagcgggttaaaatcagtccagtaaagcaagaaaatatttagagagagcttcatcatcatacgaattttgggggtcattgttcagtccaaagtacttaatatgattcttttctctttccacatagagaatcagataatctataaataatgactcttactgttccactttaggagttaggtatacatacatatgtgtatatatatgtatatatatatacacatacacacacacacacacacacacacagtgaccccccaaatttcatatgaagttccaaacctcaatgtgactgtatgtgaaaagagaagggggcggggaggggggagaccgaccgacctatttgttggtctccatcgtgtgaaaacatgaggaagtgggcacttacatgccaggaagagagctctcactagaggttgaccatgctggcactctgatctcagacttccagcctccagatatgtgagaatataaatttgtgttttgggccagatacggtggctcaggcctgtaatcccagcactttgggaggccaaggcaggtggatcaccaaaggtcagatctgaccaacatggagatcagcctaaccaacatggagaaaccctgtctctactaaaaatacaaacttagctaaggtttgtggtgcatgccaataatcccagctactgagggtgaggcaggagaatcactggaactcaggaggtggaggttgcggtgagccaagatcataccattgcactccagcctgggcaacaagagcaaaactccatctcaaaaaaaaaaaaaaaaaaaaaaaaaaaatcctgtgtttttaacctcattgatttaaaattaaattaatttctaagccatttggtctgcggtattctcttatggttgtctgagctgactaaggcagatattggtactgagaagtgaggtactgcaattaaaaacaaacaaaaaaactaaaaatgtgaagcagctttgaaactgacaaatgagtagaggctggaaaaattctgatgtgcaagctggaaataaggttggtaagggttattctggtgaggtgtcattggggaatgaggaacatgctattgggaaatgaagaaaagacaacccttgatataaagtggtgaagaacttggcagaactgtattctagcattttacggaaggtagagcttgagacagataaaatggtatgtatcactaagatctgtaattaaagtgttaaaggacacaggaagcttcattattcctgagtgcttacaggaaaatgtgctgggaacaggccccccaaatctggccataaacaggcaatgagaaactggccataaacaaaatctctgcagcactgtgacatgctcgtgatggctatgacgcccatgctggaggctgctggtttaccagaatgagggcaagcaacacctggcccacccagggcagaaaactggaaaactgctcaaggcattcctaaaccacaaacaatagcatgagtgatttgtgccttaaggacatattcctgttgcagataacaagccagagcctgtccctttctttctcataaggaatacttatagctgatctacaatctataggaataatgtttatcacaggcttactgtcaataaatatgtgggtcaaactctgttcaagctcagctctgaaggctgtgagccccgattcccactctgcactatatttctgtgtctttgtcttaattcctctagagccactgggttagggtctccacgacccagctggtctcggcaaaaatgcaaaaggagacctgaattgcagaagaaattgttaaggaaaaaggaaccagaacttggagatttggaaaattctcagcctatccatactgcaaaaattagaaaacttgtactgaagagaatcctcaaagtgtggctgaacaatcatttgataaagagatcatgagtgggattcatggactatatcagccatcttaacagaagtgagaagagagactggattatactataagagacactgccacttacattgtgccacctaaaatggacagagaagacagaacagaacagtcaaggttgtcacacttcttattttacaagaaggggacatagaaataatcagctgtgaaagggcactggcagttatggatggtttcactcctgacatgctctgcaggatccatgggaacagaagagaaccttggaggagcatctttttaacaatccacctctggggcctacatcatcttggcttctggtaaattttgacatgaatgtgccacactggcagccactaaccaacaggggctgggatcaatctgcatgatttatctcgtacagaacttgttaatgctatgatcttaggaatctaatcaccaaggtgaggcagcctgcagtactgacctcaccatccatgacccttcttcacagatgcccagactcaggtaaccatgatgttgtattcagaacctgtaggtttaatttcagaccctcgggatgcatctaaggccaatctgtgagccattacaacctccaaaaggcatttaggactaatctgatgatctttgcactgccaataattaaagatggcaaccaatgggctaaatggtaacaacactcatatccttacattcatagtatttctccccagtgtgaattctttcatgcatacttaggcatgaggaaagagcaaatgctttcccaaattctttacatacaaaaggtttctctctggtaggagttcacaggtggggtgaggaatacagaaattctttcccacatatcttgcatttacctttctccactgtgagttttcaaatgtttactacgatgggaagaagtaatgaaggtcttcccacattcaacacattcataaggcttctctcctgtgtgaattcttctatgttgagtaagcgttgaagatctattgaaggctttcccacattccttacactgatagggtttctctccagtgtgatttcgtatgtgtatagcaaggcccgtgtactgagtgaaggcttggccacattccttacattcatagggttttattccagtgtgagttcttacatgttgagtaaggtgagttgatctagtgaaggctttcccacattccgtacatttgtgtggttttattccagtgtgaatttgaatgtgaacattaaaggatgaggaatttctaaaggatcttccacattctttacattcaaaggacttctctcctttatgagtttttgcatgtgcagaaagttgagaaaaattagtgaaggatttcccacagttcttagtcttttcggatttctttccagtatgaactgctacacactgctttaagtgtgaggaagttgtgatggctctctcacattcctgaaattcacagagtttctctccaatgtggattcccatgtgattatcaaggcttgcaaaatacttaaagccttttccacattccttacatttgtagggttgtcttccattgagaatttcaagatgcacagcaaggcctggagttaaggtgaagacttttccacatggattaaatttggaaagttcttgtccaatagaggcttccttgtgcacactgatgctgtcttttccataacaattaccctcaaaagtgttccctccattctgagctctcatgtgtgtcttaaggcaaaactgttcactgaagacctctccacaattctcacagagtttccatccactgtagcttcttgtctgcatttgtatcccagtgaatatttgattcttcaaaaaaccctgctgaagtgatgaccgtttggttctaggttgtatttcccattctgaagttaagcagaaaaagaaatccacagaggccaggttcatgtagttctccagcatcacatctctgtagaggtatttctgagttgtgtccagtaaagcccactcctctggggtgaactccacagccacatcatcaaacgtcactgaatcctggtaagaatttgaccggtggtcctctaccatcgttcctatctttgtcttttcttcaaaaggacagattggttccctgggaaaaaacccatgggacatatcaaaggctgacatcctctgaagctgatggtgagatgtgcctcaatgctgtctttcttgatgccaagatcgcctcagggcagcttatgaatctaggtggatacaggcaatctccattcccctttgtacagggttatctgaggcccacagcggggtggactccaccacaataaaggttaaacggcactgaccatgctgagccacagccggtaaagatggcggtggcacact

SEQ ID NO: 13571 - RNA, 1862 nt, Homo sapiens
  source 1..1862: mol_type = other RNA
gctgggattacaggcatgagccaccactcccggccaatgttttgtatttttagtagagatggggtttcatcatgttggccagactggtctcaaactctggacctcaggtgatccacctgcctcagcctcccaaagtgtagggattacaggtgtgagccaccgcgcccagcctatgtttctattttatacatattcaacaaacatgattccccaacttctgcaaaataatttctttttcaagaacattgattttagagctcacactaagaaaaagaatacaaaaataatggcatagaaagtgaaaaaacaaaaataaaaagtagaaagctaaagtttcccattaaaatgatcaatatactgtgcagtaagtcaaatgtgtacaatgaattaagaaaatatgatatataaaaatccaaatttacaaaattaagtacaaataggtgtttatattacaaagtgatactggtttataaaaggattcaacatagattttttttaaatggttgttttcctcaatcaatttaacaatgattttaaatgtataaaattttaatatctctttgagacagtgatccaagcttcttcccttgatgatgttaccagttcatactttgtttcaataacctgtccctccacagaaagtaggtgcagtctcttcaccaatacactaagaagtactgtggtcaccatatatgcaaacctcaactctggacactcctgtgtgcctgagaatccaagtgaggaaaaagttttcattactaattcatcatcaaaccgatctggatcaaacttgtgtggagatggccaagtattaggatcctgaagtaccacaccaagggcataaaggacgagggtctctctaggaataataaatcggtcaatttttccttcaatatcttgaagctgggcagaaactggagtcagtttggcagttcgaacagtttcacaaagcacatgctgacaatatattttgcagttattatgcaactggccagagaaaatatcatactgtcttctaggatctgttggtcattaaggttcccttgtactaaggagtcaatgaaaatatgttgactgaagttccttccttttcgttcttttatgatgttccttaaaacagactccagttgcatgagggcatcttcatattgttttttccgagtcatgtttttatcaagtgacccatctagaaagccttttccaatctcagaccaaactgtgccatgattcttctggaagcgaatgacttcctgatcatcttcaaatgtactacccattaccatctgtgtaacagacttcatagcaaaaccaagcatatgctggctgaggggcacgtgctgggtctctgggtaggagagccatttatctaataattcttctgaaagctttaggaggagggcaaagttactcttcagagaatcagtcacaccattttcatacaattttttcctcatgtggttttcactcacactgccaccaccagattgataccttaataatgacttcagcatggtttcaaaagggtccgatgtcttattgggattgatatgctgcttcagtacatcaacagtgcccaaactaaccacgaggcgcctgccaaaccagaaggagaccacaggcccatatctctcatgcaaattaaccaggaactcatgcaaacttccactattcacaatatctggaagattaccatctttttcttcagttggagtaatccctggaattcctgcagcttgtctggaagccggatagaggtagagcacggctcccaccaacgccagcaagaaggtaacggcgaagatcgcgaagtccaacatggttctgccgcccagggagccacgtctcggatcggccgctccagc

SEQ ID NO: 13572 - RNA, 1783 nt, Homo sapiens
  source 1..1783: mol_type = other RNA
gctgggattacaggcatgagccaccactcccggccaatgttttgtatttttagtagagatggggtttcatcatgttggccagactggtctcaaactctggacctcaggtgatccacctgcctcagcctcccaaagtgtagggattacaggtgtgagccaccgcgcccagcctatgtttctattttatacatattcaacaaacatgattccccaacttctgcaaaataatttctttttcaagaacattgattttagagctcacactaagaaaaagaatacaaaaataatggcatagaaagtgaaaaaacaaaaataaaaagtagaaagctaaagtttcccattaaaatgatcaatatactgtgcagtaagtcaaatgtgtacaatgaattaagaaaatatgatatataaaaatccaaatttacaaaattaagtacaaataggtgtttatattacaaagtgatactggtttataaaaggattcaacatagattttttttaaatggttgttttcctcaatcaatttaacaatgattttaaatgtataaaattttaatatctctttgagacagtgatccaagcttcttcccttgatgatgttaccagttcatactttgtttcaataacctgtccctccacagaaagtaggtgcagtctcttcaccaatacactaagaagtactgtggtcaccatatatgcaaacctcaactctggacactcctgtgtgcctgagaatccaagtgaggaaaaagttttcattactaattcatcatcaaaccgatctggatcaaacttgtgtggagatggccaagtattaggatcctgaagtaccacaccaagggcataaaggacgagggtctctctaggaataataaatcggtcaatttttccttcaatatcttgaagctgggcagaaactggagtcagtttggcagttcgaacagtttcacaaagcacatgctgacaatatattttgcagttattatgcaactggccagagaaaatatcatactgtcttctaggatctgttggtcattaaggttcccttgtactaaggagtcaatgaaaatatgttgactgaagttccttccttttcgttcttttatgatgttccttaaaacagactccagttgcatgagggtgtgccatgattcttctggaagcgaatgacttcctgatcatcttcaaatgtactacccattaccatctgtgtaacagacttcatagcaaaaccaagcatatgctggctgaggggcacgtgctgggtctctgggtaggagagccatttatctaataattcttctgaaagctttaggaggagggcaaagttactcttcagagaatcagtcacaccattttcatacaattttttcctcatgtggttttcactcacactgccaccaccagattgataccttaataatgacttcagcatggtttcaaaagggtccgatgtcttattgggattgatatgctgcttcagtacatcaacagtgcccaaactaaccacgaggcgcctgccaaaccagaaggagaccacaggcccatatctctcatgcaaattaaccaggaactcatgcaaacttccactattcacaatatctggaagattaccatctttttcttcagttggagtaatccctggaattcctgcagcttgtctggaagccggatagaggtagagcacggctcccaccaacgccagcaagaaggtaacggcgaagatcgcgaagtccaacatggttctgccgcccagggagccacgtctcggatcggccgctccagc

SEQ ID NO: 13573 - RNA, 1566 nt, Homo sapiens
  source 1..1566: mol_type = other RNA
gctgggattacaggcatgagccaccactcccggccaatgttttgtatttttagtagagatggggtttcatcatgttggccagactggtctcaaactctggacctcaggtgatccacctgcctcagcctcccaaagtgtagggattacaggtgtgagccaccgcgcccagcctatgtttctattttatacatattcaacaaacatgattccccaacttctgcaaaataatttctttttcaagaacattgattttagagctcacactaagaaaaagaatacaaaaataatggcatagaaagtgaaaaaacaaaaataaaaagtagaaagctaaagtttcccattaaaatgatcaatatactgtgcagtaagtcaaatgtgtacaatgaattaagaaaatatgatatataaaaatccaaatttacaaaattaagtacaaataggtgtttatattacaaagtgatactggtttataaaaggattcaacatagattttttttaaatggttgttttcctcaatcaatttaacaatgattttaaatgtataaaattttaatatctctttgagacagtgatccaagcttcttcccttgatgatgttaccagttcatactttgtttcaataacctgtccctccacagaaagtaggtgcagtctcttcaccaatacactaagaagtactgtggtcaccatatatgcaaacctcaactctggacactcctgtgtgcctgagaatccaagtgaggaaaaagttttcattactaattcatcatcaaaccgatctggatcaaacttgtgtggagatggccaagtattaggatcctgaagtaccacaccaagggcataaaggacgagggtctctctaggaataataaatcggtcaatttttccttcaatatcttgaagctgggcagaaactggagtcagtttggcagttcgaacagtttcacaaagcacatgctgacaatatattttgcagttattatgcaactggccagagaaaatatcatactgtcttctaggatctgttggtcattaaggttcccttgtactaaggagtcaatgaaaatatgttgactgaagttccttccttttcgttcttttatgatgttccttaaaacagactccagttgcatgagggtgtgccatgattcttctggaagcgaatgacttcctgatcatcttcaaatgtactacccattaccatctgtgtaacagacttcatagcaaaaccaagcatatgctggctgaggggcacgtgctgggtctctgggtaggagagccatttatctaataattcttctgaaagctttaggaggagggcaaagttactcttcagagaatcagtcacaccattttcatacaattttttcctcatgtggttttcactcacactgccaccaccagattgataccttaataatgacttcagcatggtttcaaaagggtccgcggatagaggtagagcacggctcccaccaacgccagcaagaaggtaacggcgaagatcgcgaagtccaacatggttctgccgcccagggagccacgtctcggatcggccgctccagc

SEQ ID NO: 13574 - RNA, 2007 nt, Homo sapiens
  source 1..2007: mol_type = other RNA
gctgggattacaggcatgagccaccactcccggccaatgttttgtatttttagtagagatggggtttcatcatgttggccagactggtctcaaactctggacctcaggtgatccacctgcctcagcctcccaaagtgtagggattacaggtgtgagccaccgcgcccagcctatgtttctattttatacatattcaacaaacatgattccccaacttctgcaaaataatttctttttcaagaacattgattttagagctcacactaagaaaaagaatacaaaaataatggcatagaaagtgaaaaaacaaaaataaaaagtagaaagctaaagtttcccattaaaatgatcaatatactgtgcagtaagtcaaatgtgtacaatgaattaagaaaatatgatatataaaaatccaaatttacaaaattaagtacaaataggtgtttatattacaaagtgatactggtttataaaaggattcaacatagattttttttaaatggttgttttcctcaatcaatttaacaatgattttaaatgtataaaattttaatatctctttgagacagtgatccaagcttcttcccttgatgatgttaccagttcatactttgtttcaataacctgtccctccacagaaagtaggtgcagtctcttcaccaatacactaagaagtactgtggtcaccatatatgcaaacctcaactctggacactcctgtgtgcctgagaatccaagtgaggaaaaagttttcattactaattcatcatcaaaccgatctggatcaaacttgtgtggagatggccaagtattaggatcctgaagtaccacaccaagggcataaaggacgagggtctctctaggaataataaatcggtcaatttttccttcaatatcttgaagctgggcagaaactggagtcagtttggcagttcgaacagtttcacaaagcacatgctgacaatatctgagctgctcaattttctctggagtaacaggaccatttccaaaaacttggtttatctcttcatataattttttttgaacttcttcagaggtggttaaaaaacagattgcccaggtacacaattttgcagttattatgcaactggccagagaaaatatcatactgtcttctaggatctgttggtcattaaggttcccttgtactaaggagtcaatgaaaatatgttgactgaagttccttccttttcgttcttttatgatgttccttaaaacagactccagttgcatgagggcatcttcatattgttttttccgagtcatgtttttatcaagtgacccatctagaaagccttttccaatctcagaccaaacctgaaaataggtaaatatacataatgtgccatgattcttctggaagcgaatgacttcctgatcatcttcaaatgtactacccattaccatctgtgtaacagacttcatagcaaaaccaagcatatgctggctgaggggcacgtgctgggtctctgggtaggagagccatttatctaataattcttctgaaagctttaggaggagggcaaagttactcttcagagaatcagtcacaccattttcatacaattttttcctcatgtggttttcactcacactgccaccaccagattgataccttaataatgacttcagcatggtttcaaaagggtccgatgtcttattgggattgatatgctgcttcagtacatcaacagtgcccaaactaaccacgaggcgcctgccaaaccagaaggagaccacaggcccatatctctcatgcaaattaaccaggaactcatgcaaacttccactattcacaatatctggaagattaccatctttttcttcagttggagtaatccctggaattcctgcagcttgtctggaagccggatagaggtagagcacggctcccaccaacgccagcaagaaggtaacggcgaagatcgcgaagtccaacatggttctgccgcccagggagccacgtctcggatcggccgctccagc

SEQ ID NO: 13575 - RNA, 1710 nt, Homo sapiens
  source 1..1710: mol_type = other RNA
gctgggattacaggcatgagccaccactcccggccaatgttttgtatttttagtagagatggggtttcatcatgttggccagactggtctcaaactctggacctcaggtgatccacctgcctcagcctcccaaagtgtagggattacaggtgtgagccaccgcgcccagcctatgtttctattttatacatattcaacaaacatgattccccaacttctgcaaaataatttctttttcaagaacattgattttagagctcacactaagaaaaagaatacaaaaataatggcatagaaagtgaaaaaacaaaaataaaaagtagaaagctaaagtttcccattaaaatgatcaatatactgtgcagtaagtcaaatgtgtacaatgaattaagaaaatatgatatataaaaatccaaatttacaaaattaagtacaaataggtgtttatattacaaagtgatactggtttataaaaggattcaacatagattttttttaaatggttgttttcctcaatcaatttaacaatgattttaaatgtataaaattttaatatctctttgagacagtgatccaagcttcttcccttgatgatgttaccagttcatactttgtttcaataacctgtccctccacagaaagtaggtgcagtctcttcaccaatacactaagaagtactgtggtcaccatatatgcaaacctcaactctggacactcctgtgtgcctgagaatccaagtgaggaaaaagttttcattactaattcatcatcaaaccgatctggatcaaacttgtgtggagatggccaagtattaggatcctgaagtaccacaccaagggcataaaggacgagggtctctctaggaataataaatcggtcaatttttccttcaatatcttgaagctgggcagaaactggagtcagtttggcagttcgaacagtttcacaaagcacatgctgacaatatctgagctgctcaattttctctggagtaacaggaccatttccaaaaacttggtttatctcttcatataattttttttgaacttcttcagaggtggttaaaaaacagattgcccaggtacacaattttgcagttattatgcaactggccagagaaaatatcatactgtcttctaggatctgttggtcattaaggttcccttgtactaaggagtcaatgaaaatatgttgactgaagttccttccttttcgttcttttatgatgttccttaaaacagactccagttgcatgagggcatcttcatattgttttttccgagtcatgtttttatcaagtgacccatctagaaagccttttccaatctcagaccaaactgtgccatgattcttctggaagcgaatgacttcctgatcatcttcaaatgtactacccattaccatctgtgtaacagacttcatagcaaaaccaagcatatgctggctgaggggcacgtgctgggtctctgggtaggagagccatttatctaataattcttctgaaagcttaataatgacttcagcatggtttcaaaagggtccgttttcttcagttggagtaatccctggaattcctgcagcttgtctggaagccggatagaggtagagcacggctcccaccaacgccagcaagaaggtaacggcgaagatcgcgaagtccaacatggttctgccgcccagggagccacgtctcggatcggccgctccagc

SEQ ID NO: 13576 - RNA, 1983 nt, Homo sapiens
  source 1..1983: mol_type = other RNA
gctgggattacaggcatgagccaccactcccggccaatgttttgtatttttagtagagatggggtttcatcatgttggccagactggtctcaaactctggacctcaggtgatccacctgcctcagcctcccaaagtgtagggattacaggtgtgagccaccgcgcccagcctatgtttctattttatacatattcaacaaacatgattccccaacttctgcaaaataatttctttttcaagaacattgattttagagctcacactaagaaaaagaatacaaaaataatggcatagaaagtgaaaaaacaaaaataaaaagtagaaagctaaagtttcccattaaaatgatcaatatactgtgcagtaagtcaaatgtgtacaatgaattaagaaaatatgatatataaaaatccaaatttacaaaattaagtacaaataggtgtttatattacaaagtgatactggtttataaaaggattcaacatagattttttttaaatggttgttttcctcaatcaatttaacaatgattttaaatgtataaaattttaatatctctttgagacagtgatccaagcttcttcccttgatgatgttaccagttcatactttgtttcaataacctgtccctccacagaaagtaggtgcagtctcttcaccaatacactaagaagtactgtggtcaccatatatgcaaacctcaactctggacactcctgtgtgcctgagaatccaagtgaggaaaaagttttcattactaattcatcatcaaaccgatctggatcaaacttgtgtggagatggccaagtattaggatcctgaagtaccacaccaagggcataaaggacgagggtctctctaggaataataaatcggtcaatttttccttcaatatcttgaagctgggcagaaactggagtcagtttggcagttcgaacagtttcacaaagcacatgctgacaatatctgagctgctcaattttctctggagtaacaggaccatttccaaaaacttggtttatctcttcatataattttttttgaacttcttcagaggtggttaaaaaacagattgcccaggtacacaattttgcagttattatgcaactggccagagaaaatatcatactgtcttctaggatctgttggtcattaaggttcccttgtactaaggagtcaatgaaaatatgttgactgaagttccttccttttcgttcttttatgatgttccttaaaacagactccagttgcatgagggcatcttcatattgttttttccgagtcatgtttttatcaagtgacccatctagaaagccttttccaatctcagaccaaactgtgccatgattcttctggaagcgaatgacttcctgatcatcttcaaatgtactacccattaccatctgtgtaacagacttcatagcaaaaccaagcatatgctggctgaggggcacgtgctgggtctctgggtaggagagccatttatctaataattcttctgaaagctttaggaggagggcaaagttactcttcagagaatcagtcacaccattttcatacaattttttcctcatgtggttttcactcacactgccaccaccagattgataccttaataatgacttcagcatggtttcaaaagggtccgatgtcttattgggattgatatgctgcttcagtacatcaacagtgcccaaactaaccacgaggcgcctgccaaaccagaaggagaccacaggcccatatctctcatgcaaattaaccaggaactcatgcaaacttccactattcacaatatctggaagattaccatctttttcttcagttggagtaatccctggaattcctgcagcttgtctggaagccggatagaggtagagcacggctcccaccaacgccagcaagaaggtaacggcgaagatcgcgaagtccaacatggttctgccgcccagggagccacgtctcggatcggccgctccagc

SEQ ID NO: 13577 - RNA, 1766 nt, Homo sapiens
  source 1..1766: mol_type = other RNA
gctgggattacaggcatgagccaccactcccggccaatgttttgtatttttagtagagatggggtttcatcatgttggccagactggtctcaaactctggacctcaggtgatccacctgcctcagcctcccaaagtgtagggattacaggtgtgagccaccgcgcccagcctatgtttctattttatacatattcaacaaacatgattccccaacttctgcaaaataatttctttttcaagaacattgattttagagctcacactaagaaaaagaatacaaaaataatggcatagaaagtgaaaaaacaaaaataaaaagtagaaagctaaagtttcccattaaaatgatcaatatactgtgcagtaagtcaaatgtgtacaatgaattaagaaaatatgatatataaaaatccaaatttacaaaattaagtacaaataggtgtttatattacaaagtgatactggtttataaaaggattcaacatagattttttttaaatggttgttttcctcaatcaatttaacaatgattttaaatgtataaaattttaatatctctttgagacagtgatccaagcttcttcccttgatgatgttaccagttcatactttgtttcaataacctgtccctccacagaaagtaggtgcagtctcttcaccaatacactaagaagtactgtggtcaccatatatgcaaacctcaactctggacactcctgtgtgcctgagaatccaagtgaggaaaaagttttcattactaattcatcatcaaaccgatctggatcaaacttgtgtggagatggccaagtattaggatcctgaagtaccacaccaagggcataaaggacgagggtctctctaggaataataaatcggtcaatttttccttcaatatcttgaagctgggcagaaactggagtcagtttggcagttcgaacagtttcacaaagcacatgctgacaatatctgagctgctcaattttctctggagtaacaggaccatttccaaaaacttggtttatctcttcatataattttttttgaacttcttcagaggtggttaaaaaacagattgcccaggtacacaattttgcagttattatgcaactggccagagaaaatatcatactgtcttctaggatctgttggtcattaaggttcccttgtactaaggagtcaatgaaaatatgttgactgaagttccttccttttcgttcttttatgatgttccttaaaacagactccagttgcatgagggcatcttcatattgttttttccgagtcatgtttttatcaagtgacccatctagaaagccttttccaatctcagaccaaactgtgccatgattcttctggaagcgaatgacttcctgatcatcttcaaatgtactacccattaccatctgtgtaacagacttcatagcaaaaccaagcatatgctggctgaggggcacgtgctgggtctctgggtaggagagccatttatctaataattcttctgaaagctttaggaggagggcaaagttactcttcagagaatcagtcacaccattttcatacaattttttcctcatgtggttttcactcacactgccaccaccagattgataccttaataatgacttcagcatggtttcaaaagggtccgcggatagaggtagagcacggctcccaccaacgccagcaagaaggtaacggcgaagatcgcgaagtccaacatggttctgccgcccagggagccacgtctcggatcggccgctccagc

SEQ ID NO: 13578 - RNA, 2535 nt, Homo sapiens
  source 1..2535: mol_type = other RNA
gctgggattacaggcatgagccaccactcccggccaatgttttgtatttttagtagagatggggtttcatcatgttggccagactggtctcaaactctggacctcaggtgatccacctgcctcagcctcccaaagtgtagggattacaggtgtgagccaccgcgcccagcctatgtttctattttatacatattcaacaaacatgattccccaacttctgcaaaataatttctttttcaagaacattgattttagagctcacactaagaaaaagaatacaaaaataatggcatagaaagtgaaaaaacaaaaataaaaagtagaaagctaaagtttcccattaaaatgatcaatatactgtgcagtaagtcaaatgtgtacaatgaattaagaaaatatgatatataaaaatccaaatttacaaaattaagtacaaataggtgtttatattacaaagtgatactggtttataaaaggattcaacatagattttttttaaatggttgttttcctcaatcaatttaacaatgattttaaatgtataaaattttaatatctctttgagacagtgatccaagcttcttcccttgatgatgttaccagttcatactttgtttcaataacctgtccctccacagaaagtaggtgcagtctcttcaccaatacactaagaagtactgtggtcaccatatatgcaaacctcaactctggacactcctgtgtgcctgagaatccaagtgaggaaaaagttttcattactaattcatcatcaaaccgatctggatcaaacttgtgtggagatggccaagtattaggatcctgaagtaccacaccaagggcataaaggacgagggtctctctaggaataataaatcggtcaatttttccttcaatatcttgaagctgggcagaaactggagtcagtttggcagttcgaacagtttcacaaagcacatgctgacaatatctgagctgctcaattttctctggagtaacaggaccatttccaaaaacttggtttatctcttcatataattttttttgaacttcttcagaggtggttaaaaaacagattgcccaggtacacaattttgcagttattatgcaactggccagagaaaatatcatactgtcttctaggatctgttggtcattaaggttcccttgtactaaggagtcaatgaaaatatgttgactgaagttccttccttttcgttcttttatgatgttccttaaaacagactccagttgcatgagggcatcttcatattgttttttccgagtcatgtttttatcaagtgacccatctagaaagccttttccaatctcagaccaaactgtgccatgattcttctggaagcgaatgacttcctgatcatcttcaaatgtactacccattaccatctgtgtaacagacttcatagcaaaaccaagcatatgctggctgaggggcacgtgctgggtctctgggtaggagagccatttatctaataattcttctgaaagctttaggaggagggcaaagttactcttcagagaatcagtcacaccattttcatacaattttttcctcatgtggttttcactcacactgccaccaccagattgataccttaataatgacttcagcatggtttcaaaagggtccgctgctcggaaaagaacatttaagaaggtgtatggtcaattccagcagttcagctacttttcaactttcactgtaaaaccaccaccttgctttgtagaacaggtgttttttgtttgtttgtttgtttgttttgagataagagtctggctctgtcgccaggctgcagtgcagtggtgcgatcttggctcactgcaagctccgcctcccaggttcaagcgattctcctgcctcagcctcctgagtagctgggattacaggcgcccgccaccacagccagctaatgtttgtatttttagtagagacggtgtgtcaccatgttggccaggatggtctcgatatcctgacctcgtgatccgcccgcctcagcctcccaaagtgtgtagaacaggttttaaagacggtcctcagtcatcaacacttttgttttcagaccctccctctctcgctgacggaggcaagtggagagaggaggaccggaggctcgcagaggcgtcagcggcagaggaaacctcgcacccgaacccgcagcgcggcgctctccccaaagaagcatttgcctggagcccctaagaggagcaagacctggacctcgagcactttggattccagtcaggatagatcgatggacagatggaaaagaggaatacacaagtgctgggagaatcctcaagaaaggagaaaggagtggcgcgcccaggagtctcgtcctgacacactgggaaatgaaatttgggtttggcgagttatggccaaaaagctgcccaaagtacttgagagccgccttggagagtggcgcggggtgcctggcaaggtgagaccggcctgcgggggcgcgggcttttcctcagcagctctacgcccgcctggcccggcgcctgaggggtagc

SEQ ID NO: 13579 - RNA, 1816 nt, Homo sapiens
  source 1..1816: mol_type = other RNA
gctgggattacaggcatgagccaccactcccggccaatgttttgtatttttagtagagatggggtttcatcatgttggccagactggtctcaaactctggacctcaggtgatccacctgcctcagcctcccaaagtgtagggattacaggtgtgagccaccgcgcccagcctatgtttctattttatacatattcaacaaacatgattccccaacttctgcaaaataatttctttttcaagaacattgattttagagctcacactaagaaaaagaatacaaaaataatggcatagaaagtgaaaaaacaaaaataaaaagtagaaagctaaagtttcccattaaaatgatcaatatactgtgcagtaagtcaaatgtgtacaatgaattaagaaaatatgatatataaaaatccaaatttacaaaattaagtacaaataggtgtttatattacaaagtgatactggtttataaaaggattcaacatagattttttttaaatggttgttttcctcaatcaatttaacaatgattttaaatgtataaaattttaatatctctttgagacagtgatccaagcttcttcccttgatgatgttaccagttcatactttgtttcaataacctgtccctccacagaaagtaggtgcagtctcttcaccaatacactaagaagtactgtggtcaccatatatgcaaacctcaactctggacactcctgtgtgcctgagaatccaagtgaggaaaaagttttcattactaattcatcatcaaaccgatctggatcaaacttgtgtggagatggccaagtattaggatcctgaagtaccacaccaagggcataaaggacgagggtctctctaggaataataaatcggtcaatttttccttcaatatcttgaagctgggcagaaactggagtcagtttggcagttcgaacagtttcacaaagcacatgctgacaatatctgagctgctcaattttctctggagtaacaggaccatttccaaaaacttggtttatctcttcatataattttttttgaacttcttcagaggtggttaaaaaacagattgcccaggtacacaattttgcagttattatgcaactggccagagaaaatatcatactgtcttctaggatctgttggtcattaaggttcccttgtactaaggagtcaatgaaaatatgttgactgaagttccttccttttcgttcttttatgatgttccttaaaacagactccagttgcatgagggcatcttcatattgttttttccgagtcatgtttttatcaagtgacccatctagaaagccttttccaatctcagaccaaactgtgccatgattcttctggaagcgaatgacttcctgatcatcttcaaatgtactacccattaccatctgtgtaacagacttcatagcaaaaccaagcatatgctggctgaggggcacgtgctgggtctctgggtaggagagccatttatctaataattcttctgaaagctttaggaggagggcaaagttactcttcagagaatcagtcacaccattttcatacaattttttcctcatgtggttttcactcacactgccaccaccagattgataccttaataatgacttcagcatggtttcaaaagggtccgttttcttcagttggagtaatccctggaattcctgcagcttgtctggaagccggatagaggtagagcacggctcccaccaacgccagcaagaaggtaacggcgaagatcgcgaagtccaacatggttctgccgcccagggagccacgtctcggatcggccgctccagc

SEQ ID NO: 13580 - RNA, 1631 nt, Homo sapiens
  source 1..1631: mol_type = other RNA
gctgggattacaggcatgagccaccactcccggccaatgttttgtatttttagtagagatggggtttcatcatgttggccagactggtctcaaactctggacctcaggtgatccacctgcctcagcctcccaaagtgtagggattacaggtgtgagccaccgcgcccagcctatgtttctattttatacatattcaacaaacatgattccccaacttctgcaaaataatttctttttcaagaacattgattttagagctcacactaagaaaaagaatacaaaaataatggcatagaaagtgaaaaaacaaaaataaaaagtagaaagctaaagtttcccattaaaatgatcaatatactgtgcagtaagtcaaatgtgtacaatgaattaagaaaatatgatatataaaaatccaaatttacaaaattaagtacaaataggtgtttatattacaaagtgatactggtttataaaaggattcaacatagattttttttaaatggttgttttcctcaatcaatttaacaatgattttaaatgtataaaattttaatatctctttgagacagtgatccaagcttcttcccttgatgatgttaccagttcatactttgtttcaataacctgtccctccacagaaagtaggtgcagtctcttcaccaatacactaagaagtactgtggtcaccatatatgcaaacctcaactctggacactcctgtgtgcctgagaatccaagtgaggaaaaagttttcattactaattcatcatcaaaccgatctggatcaaacttgtgtggagatggccaagtattaggatcctgaagtaccacaccaagggcataaaggacgagggtctctctaggaataataaatcggtcaatttttccttcaatatcttgaagctgggcagaaactggagtcagtttggcagttcgaacagtttcacaaagcacatgctgacaatatctgagctgctcaattttctctggagtaacaggaccatttccaaaaacttggtttatctcttcatataattttttttgaacttcttcagaggtggttaaaaaacagattgcccaggtacacaattttgcagttattatgcaactggccagagaaaatatcatactgtcttctaggatctgttggtcattaaggttcccttgtactaaggagtcaatgaaaatatgttgactgaagttccttccttttcgttcttttatgatgttccttaaaacagactccagttgcatgagggtgtgccatgattcttctggaagcgaatgacttcctgatcatcttcaaatgtactacccattaccatctgtgtaacagacttcatagcaaaaccaagcatatgctggctgaggggcacgtgctgggtctctgggtaggagagccatttatctaataattcttctgaaagcttaataatgacttcagcatggtttcaaaagggtccgttttcttcagttggagtaatccctggaattcctgcagcttgtctggaagccggatagaggtagagcacggctcccaccaacgccagcaagaaggtaacggcgaagatcgcgaagtccaacatggttctgccgcccagggagccacgtctcggatcggccgctccagc

SEQ ID NO: 13581 - RNA, 1904 nt, Homo sapiens
  source 1..1904: mol_type = other RNA
gctgggattacaggcatgagccaccactcccggccaatgttttgtatttttagtagagatggggtttcatcatgttggccagactggtctcaaactctggacctcaggtgatccacctgcctcagcctcccaaagtgtagggattacaggtgtgagccaccgcgcccagcctatgtttctattttatacatattcaacaaacatgattccccaacttctgcaaaataatttctttttcaagaacattgattttagagctcacactaagaaaaagaatacaaaaataatggcatagaaagtgaaaaaacaaaaataaaaagtagaaagctaaagtttcccattaaaatgatcaatatactgtgcagtaagtcaaatgtgtacaatgaattaagaaaatatgatatataaaaatccaaatttacaaaattaagtacaaataggtgtttatattacaaagtgatactggtttataaaaggattcaacatagattttttttaaatggttgttttcctcaatcaatttaacaatgattttaaatgtataaaattttaatatctctttgagacagtgatccaagcttcttcccttgatgatgttaccagttcatactttgtttcaataacctgtccctccacagaaagtaggtgcagtctcttcaccaatacactaagaagtactgtggtcaccatatatgcaaacctcaactctggacactcctgtgtgcctgagaatccaagtgaggaaaaagttttcattactaattcatcatcaaaccgatctggatcaaacttgtgtggagatggccaagtattaggatcctgaagtaccacaccaagggcataaaggacgagggtctctctaggaataataaatcggtcaatttttccttcaatatcttgaagctgggcagaaactggagtcagtttggcagttcgaacagtttcacaaagcacatgctgacaatatctgagctgctcaattttctctggagtaacaggaccatttccaaaaacttggtttatctcttcatataattttttttgaacttcttcagaggtggttaaaaaacagattgcccaggtacacaattttgcagttattatgcaactggccagagaaaatatcatactgtcttctaggatctgttggtcattaaggttcccttgtactaaggagtcaatgaaaatatgttgactgaagttccttccttttcgttcttttatgatgttccttaaaacagactccagttgcatgagggtgtgccatgattcttctggaagcgaatgacttcctgatcatcttcaaatgtactacccattaccatctgtgtaacagacttcatagcaaaaccaagcatatgctggctgaggggcacgtgctgggtctctgggtaggagagccatttatctaataattcttctgaaagctttaggaggagggcaaagttactcttcagagaatcagtcacaccattttcatacaattttttcctcatgtggttttcactcacactgccaccaccagattgataccttaataatgacttcagcatggtttcaaaagggtccgatgtcttattgggattgatatgctgcttcagtacatcaacagtgcccaaactaaccacgaggcgcctgccaaaccagaaggagaccacaggcccatatctctcatgcaaattaaccaggaactcatgcaaacttccactattcacaatatctggaagattaccatctttttcttcagttggagtaatccctggaattcctgcagcttgtctggaagccggatagaggtagagcacggctcccaccaacgccagcaagaaggtaacggcgaagatcgcgaagtccaacatggttctgccgcccagggagccacgtctcggatcggccgctccagc

SEQ ID NO: 13582 - RNA, 1687 nt, Homo sapiens
  source 1..1687: mol_type = other RNA
gctgggattacaggcatgagccaccactcccggccaatgttttgtatttttagtagagatggggtttcatcatgttggccagactggtctcaaactctggacctcaggtgatccacctgcctcagcctcccaaagtgtagggattacaggtgtgagccaccgcgcccagcctatgtttctattttatacatattcaacaaacatgattccccaacttctgcaaaataatttctttttcaagaacattgattttagagctcacactaagaaaaagaatacaaaaataatggcatagaaagtgaaaaaacaaaaataaaaagtagaaagctaaagtttcccattaaaatgatcaatatactgtgcagtaagtcaaatgtgtacaatgaattaagaaaatatgatatataaaaatccaaatttacaaaattaagtacaaataggtgtttatattacaaagtgatactggtttataaaaggattcaacatagattttttttaaatggttgttttcctcaatcaatttaacaatgattttaaatgtataaaattttaatatctctttgagacagtgatccaagcttcttcccttgatgatgttaccagttcatactttgtttcaataacctgtccctccacagaaagtaggtgcagtctcttcaccaatacactaagaagtactgtggtcaccatatatgcaaacctcaactctggacactcctgtgtgcctgagaatccaagtgaggaaaaagttttcattactaattcatcatcaaaccgatctggatcaaacttgtgtggagatggccaagtattaggatcctgaagtaccacaccaagggcataaaggacgagggtctctctaggaataataaatcggtcaatttttccttcaatatcttgaagctgggcagaaactggagtcagtttggcagttcgaacagtttcacaaagcacatgctgacaatatctgagctgctcaattttctctggagtaacaggaccatttccaaaaacttggtttatctcttcatataattttttttgaacttcttcagaggtggttaaaaaacagattgcccaggtacacaattttgcagttattatgcaactggccagagaaaatatcatactgtcttctaggatctgttggtcattaaggttcccttgtactaaggagtcaatgaaaatatgttgactgaagttccttccttttcgttcttttatgatgttccttaaaacagactccagttgcatgagggtgtgccatgattcttctggaagcgaatgacttcctgatcatcttcaaatgtactacccattaccatctgtgtaacagacttcatagcaaaaccaagcatatgctggctgaggggcacgtgctgggtctctgggtaggagagccatttatctaataattcttctgaaagctttaggaggagggcaaagttactcttcagagaatcagtcacaccattttcatacaattttttcctcatgtggttttcactcacactgccaccaccagattgataccttaataatgacttcagcatggtttcaaaagggtccgcggatagaggtagagcacggctcccaccaacgccagcaagaaggtaacggcgaagatcgcgaagtccaacatggttctgccgcccagggagccacgtctcggatcggccgctccagc

SEQ ID NO: 13583 - RNA, 2456 nt, Homo sapiens
  source 1..2456: mol_type = other RNA
gctgggattacaggcatgagccaccactcccggccaatgttttgtatttttagtagagatggggtttcatcatgttggccagactggtctcaaactctggacctcaggtgatccacctgcctcagcctcccaaagtgtagggattacaggtgtgagccaccgcgcccagcctatgtttctattttatacatattcaacaaacatgattccccaacttctgcaaaataatttctttttcaagaacattgattttagagctcacactaagaaaaagaatacaaaaataatggcatagaaagtgaaaaaacaaaaataaaaagtagaaagctaaagtttcccattaaaatgatcaatatactgtgcagtaagtcaaatgtgtacaatgaattaagaaaatatgatatataaaaatccaaatttacaaaattaagtacaaataggtgtttatattacaaagtgatactggtttataaaaggattcaacatagattttttttaaatggttgttttcctcaatcaatttaacaatgattttaaatgtataaaattttaatatctctttgagacagtgatccaagcttcttcccttgatgatgttaccagttcatactttgtttcaataacctgtccctccacagaaagtaggtgcagtctcttcaccaatacactaagaagtactgtggtcaccatatatgcaaacctcaactctggacactcctgtgtgcctgagaatccaagtgaggaaaaagttttcattactaattcatcatcaaaccgatctggatcaaacttgtgtggagatggccaagtattaggatcctgaagtaccacaccaagggcataaaggacgagggtctctctaggaataataaatcggtcaatttttccttcaatatcttgaagctgggcagaaactggagtcagtttggcagttcgaacagtttcacaaagcacatgctgacaatatctgagctgctcaattttctctggagtaacaggaccatttccaaaaacttggtttatctcttcatataattttttttgaacttcttcagaggtggttaaaaaacagattgcccaggtacacaattttgcagttattatgcaactggccagagaaaatatcatactgtcttctaggatctgttggtcattaaggttcccttgtactaaggagtcaatgaaaatatgttgactgaagttccttccttttcgttcttttatgatgttccttaaaacagactccagttgcatgagggtgtgccatgattcttctggaagcgaatgacttcctgatcatcttcaaatgtactacccattaccatctgtgtaacagacttcatagcaaaaccaagcatatgctggctgaggggcacgtgctgggtctctgggtaggagagccatttatctaataattcttctgaaagctttaggaggagggcaaagttactcttcagagaatcagtcacaccattttcatacaattttttcctcatgtggttttcactcacactgccaccaccagattgataccttaataatgacttcagcatggtttcaaaagggtccgctgctcggaaaagaacatttaagaaggtgtatggtcaattccagcagttcagctacttttcaactttcactgtaaaaccaccaccttgctttgtagaacaggtgttttttgtttgtttgtttgtttgttttgagataagagtctggctctgtcgccaggctgcagtgcagtggtgcgatcttggctcactgcaagctccgcctcccaggttcaagcgattctcctgcctcagcctcctgagtagctgggattacaggcgcccgccaccacagccagctaatgtttgtatttttagtagagacggtgtgtcaccatgttggccaggatggtctcgatatcctgacctcgtgatccgcccgcctcagcctcccaaagtgtgtagaacaggttttaaagacggtcctcagtcatcaacacttttgttttcagaccctccctctctcgctgacggaggcaagtggagagaggaggaccggaggctcgcagaggcgtcagcggcagaggaaacctcgcacccgaacccgcagcgcggcgctctccccaaagaagcatttgcctggagcccctaagaggagcaagacctggacctcgagcactttggattccagtcaggatagatcgatggacagatggaaaagaggaatacacaagtgctgggagaatcctcaagaaaggagaaaggagtggcgcgcccaggagtctcgtcctgacacactgggaaatgaaatttgggtttggcgagttatggccaaaaagctgcccaaagtacttgagagccgccttggagagtggcgcggggtgcctggcaaggtgagaccggcctgcgggggcgcgggcttttcctcagcagctctacgcccgcctggcccggcgcctgaggggtagc

SEQ ID NO: 13584 - RNA, 1737 nt, Homo sapiens
  source 1..1737: mol_type = other RNA
gctgggattacaggcatgagccaccactcccggccaatgttttgtatttttagtagagatggggtttcatcatgttggccagactggtctcaaactctggacctcaggtgatccacctgcctcagcctcccaaagtgtagggattacaggtgtgagccaccgcgcccagcctatgtttctattttatacatattcaacaaacatgattccccaacttctgcaaaataatttctttttcaagaacattgattttagagctcacactaagaaaaagaatacaaaaataatggcatagaaagtgaaaaaacaaaaataaaaagtagaaagctaaagtttcccattaaaatgatcaatatactgtgcagtaagtcaaatgtgtacaatgaattaagaaaatatgatatataaaaatccaaatttacaaaattaagtacaaataggtgtttatattacaaagtgatactggtttataaaaggattcaacatagattttttttaaatggttgttttcctcaatcaatttaacaatgattttaaatgtataaaattttaatatctctttgagacagtgatccaagcttcttcccttgatgatgttaccagttcatactttgtttcaataacctgtccctccacagaaagtaggtgcagtctcttcaccaatacactaagaagtactgtggtcaccatatatgcaaacctcaactctggacactcctgtgtgcctgagaatccaagtgaggaaaaagttttcattactaattcatcatcaaaccgatctggatcaaacttgtgtggagatggccaagtattaggatcctgaagtaccacaccaagggcataaaggacgagggtctctctaggaataataaatcggtcaatttttccttcaatatcttgaagctgggcagaaactggagtcagtttggcagttcgaacagtttcacaaagcacatgctgacaatatctgagctgctcaattttctctggagtaacaggaccatttccaaaaacttggtttatctcttcatataattttttttgaacttcttcagaggtggttaaaaaacagattgcccaggtacacaattttgcagttattatgcaactggccagagaaaatatcatactgtcttctaggatctgttggtcattaaggttcccttgtactaaggagtcaatgaaaatatgttgactgaagttccttccttttcgttcttttatgatgttccttaaaacagactccagttgcatgagggtgtgccatgattcttctggaagcgaatgacttcctgatcatcttcaaatgtactacccattaccatctgtgtaacagacttcatagcaaaaccaagcatatgctggctgaggggcacgtgctgggtctctgggtaggagagccatttatctaataattcttctgaaagctttaggaggagggcaaagttactcttcagagaatcagtcacaccattttcatacaattttttcctcatgtggttttcactcacactgccaccaccagattgataccttaataatgacttcagcatggtttcaaaagggtccgttttcttcagttggagtaatccctggaattcctgcagcttgtctggaagccggatagaggtagagcacggctcccaccaacgccagcaagaaggtaacggcgaagatcgcgaagtccaacatggttctgccgcccagggagccacgtctcggatcggccgctccagc

SEQ ID NO: 13585 - RNA, 1571 nt, Homo sapiens
  source 1..1571: mol_type = other RNA
gctgggattacaggcatgagccaccactcccggccaatgttttgtatttttagtagagatggggtttcatcatgttggccagactggtctcaaactctggacctcaggtgatccacctgcctcagcctcccaaagtgtagggattacaggtgtgagccaccgcgcccagcctatgtttctattttatacatattcaacaaacatgattccccaacttctgcaaaataatttctttttcaagaacattgattttagagctcacactaagaaaaagaatacaaaaataatggcatagaaagtgaaaaaacaaaaataaaaagtagaaagctaaagtttcccattaaaatgatcaatatactgtgcagtaagtcaaatgtgtacaatgaattaagaaaatatgatatataaaaatccaaatttacaaaattaagtacaaataggtgtttatattacaaagtgatactggtttataaaaggattcaacatagattttttttaaatggttgttttcctcaatcaatttaacaatgattttaaatgtataaaattttaatatctctttgagacagtgatccaagcttcttcccttgatgatgttaccagttcatactttgtttcaataacctgtccctccacagaaagtaggtgcagtctcttcaccaatacactaagaagtactgtggtcaccatatatgcaaacctcaactctggacactcctgtgtgcctgagaatccaagtgaggaaaaagttttcattactaattcatcatcaaaccgatctggatcaaacttgtgtggagatggccaagtattaggatcctgaagtaccacaccaagggcataaaggacgagggtctctctaggaataataaatcggtcaatttttccttcaatatcttgaagctgggcagaaactggagtcagtttggcagttcgaacagtttcacaaagcacatgctgacaatatctgagctgctcaattttctctggagtaacaggaccatttccaaaaacttggtttatctcttcatataattttttttgaacttcttcagaggtggttaaaaaacagattgcccaggtacacaattttgcagttattatgcaactggccagagaaaatatcatactgtcttctaggattgtgccatgattcttctggaagcgaatgacttcctgatcatcttcaaatgtactacccattaccatctgtgtaacagacttcatagcaaaaccaagcatatgctggctgaggggcacgtgctgggtctctgggtaggagagccatttatctaataattcttctgaaagctttaggaggagggcaaagttactcttcagagaatcagtcacaccattttcatacaattttttcctcatgtggttttcactcacactgccaccaccagattgataccttaataatgacttcagcatggtttcaaaagggtccgcggatagaggtagagcacggctcccaccaacgccagcaagaaggtaacggcgaagatcgcgaagtccaacatggttctgccgcccagggagccacgtctcggatcggccgctccagc

SEQ ID NO: 13586 - RNA, 1621 nt, Homo sapiens
  source 1..1621: mol_type = other RNA
gctgggattacaggcatgagccaccactcccggccaatgttttgtatttttagtagagatggggtttcatcatgttggccagactggtctcaaactctggacctcaggtgatccacctgcctcagcctcccaaagtgtagggattacaggtgtgagccaccgcgcccagcctatgtttctattttatacatattcaacaaacatgattccccaacttctgcaaaataatttctttttcaagaacattgattttagagctcacactaagaaaaagaatacaaaaataatggcatagaaagtgaaaaaacaaaaataaaaagtagaaagctaaagtttcccattaaaatgatcaatatactgtgcagtaagtcaaatgtgtacaatgaattaagaaaatatgatatataaaaatccaaatttacaaaattaagtacaaataggtgtttatattacaaagtgatactggtttataaaaggattcaacatagattttttttaaatggttgttttcctcaatcaatttaacaatgattttaaatgtataaaattttaatatctctttgagacagtgatccaagcttcttcccttgatgatgttaccagttcatactttgtttcaataacctgtccctccacagaaagtaggtgcagtctcttcaccaatacactaagaagtactgtggtcaccatatatgcaaacctcaactctggacactcctgtgtgcctgagaatccaagtgaggaaaaagttttcattactaattcatcatcaaaccgatctggatcaaacttgtgtggagatggccaagtattaggatcctgaagtaccacaccaagggcataaaggacgagggtctctctaggaataataaatcggtcaatttttccttcaatatcttgaagctgggcagaaactggagtcagtttggcagttcgaacagtttcacaaagcacatgctgacaatatctgagctgctcaattttctctggagtaacaggaccatttccaaaaacttggtttatctcttcatataattttttttgaacttcttcagaggtggttaaaaaacagattgcccaggtacacaattttgcagttattatgcaactggccagagaaaatatcatactgtcttctaggattgtgccatgattcttctggaagcgaatgacttcctgatcatcttcaaatgtactacccattaccatctgtgtaacagacttcatagcaaaaccaagcatatgctggctgaggggcacgtgctgggtctctgggtaggagagccatttatctaataattcttctgaaagctttaggaggagggcaaagttactcttcagagaatcagtcacaccattttcatacaattttttcctcatgtggttttcactcacactgccaccaccagattgataccttaataatgacttcagcatggtttcaaaagggtccgttttcttcagttggagtaatccctggaattcctgcagcttgtctggaagccggatagaggtagagcacggctcccaccaacgccagcaagaaggtaacggcgaagatcgcgaagtccaacatggttctgccgcccagggagccacgtctcggatcggccgctccagc

SEQ ID NO: 13587 - RNA, 1871 nt, Homo sapiens
  source 1..1871: mol_type = other RNA
gctgggattacaggcatgagccaccactcccggccaatgttttgtatttttagtagagatggggtttcatcatgttggccagactggtctcaaactctggacctcaggtgatccacctgcctcagcctcccaaagtgtagggattacaggtgtgagccaccgcgcccagcctatgtttctattttatacatattcaacaaacatgattccccaacttctgcaaaataatttctttttcaagaacattgattttagagctcacactaagaaaaagaatacaaaaataatggcatagaaagtgaaaaaacaaaaataaaaagtagaaagctaaagtttcccattaaaatgatcaatatactgtgcagtaagtcaaatgtgtacaatgaattaagaaaatatgatatataaaaatccaaatttacaaaattaagtacaaataggtgtttatattacaaagtgatactggtttataaaaggattcaacatagattttttttaaatggttgttttcctcaatcaatttaacaatgattttaaatgtataaaattttaatatctctttgagacagtgatccaagcttcttcccttgatgatgttaccagttcatactttgtttcaataacctgtccctccacagaaagtaggtgcagtctcttcaccaatacactaagaagtactgtggtcaccatatatgcaaacctcaactctggacactcctgtgtgcctgagaatccaagtgaggaaaaagttttcattactaattcatcatcaaaccgatctggatcaaacttgtgtggagatggccaagtattaggatcctgaagtaccacaccaagggcataaaggacgagggtctgagctgctcaattttctctggagtaacaggaccatttccaaaaacttggtttatctcttcatataattttttttgaacttcttcagaggtggttaaaaaacagattgcccaggtacacaattttgcagttattatgcaactggccagagaaaatatcatactgtcttctaggatctgttggtcattaaggttcccttgtactaaggagtcaatgaaaatatgttgactgaagttccttccttttcgttcttttatgatgttccttaaaacagactccagttgcatgagggcatcttcatattgttttttccgagtcatgtttttatcaagtgacccatctagaaagccttttccaatctcagaccaaactgtgccatgattcttctggaagcgaatgacttcctgatcatcttcaaatgtactacccattaccatctgtgtaacagacttcatagcaaaaccaagcatatgctggctgaggggcacgtgctgggtctctgggtaggagagccatttatctaataattcttctgaaagctttaggaggagggcaaagttactcttcagagaatcagtcacaccattttcatacaattttttcctcatgtggttttcactcacactgccaccaccagattgataccttaataatgacttcagcatggtttcaaaagggtccgatgtcttattgggattgatatgctgcttcagtacatcaacagtgcccaaactaaccacgaggcgcctgccaaaccagaaggagaccacaggcccatatctctcatgcaaattaaccaggaactcatgcaaacttccactattcacaatatctggaagattaccatctttttcttcagttggagtaatccctggaattcctgcagcttgtctggaagccggatagaggtagagcacggctcccaccaacgccagcaagaaggtaacggcgaagatcgcgaagtccaacatggttctgccgcccagggagccacgtctcggatcggccgctccagc

SEQ ID NO: 13588 - RNA, 1625 nt, Homo sapiens
  source 1..1625: mol_type = other RNA
gctgggattacaggcatgagccaccactcccggccaatgttttgtatttttagtagagatggggtttcatcatgttggccagactggtctcaaactctggacctcaggtgatccacctgcctcagcctcccaaagtgtagggattacaggtgtgagccaccgcgcccagcctatgtttctattttatacatattcaacaaacatgattccccaacttctgcaaaataatttctttttcaagaacattgattttagagctcacactaagaaaaagaatacaaaaataatggcatagaaagtgaaaaaacaaaaataaaaagtagaaagctaaagtttcccattaaaatgatcaatatactgtgcagtaagtcaaatgtgtacaatgaattaagaaaatatgatatataaaaatccaaatttacaaaattaagtacaaataggtgtttatattacaaagtgatactggtttataaaaggattcaacatagattttttttaaatggttgttttcctcaatcaatttaacaatgattttaaatgtataaaattttaatatctctttgagacagtgatccaagcttcttcccttgatgatgttaccagttcatactttgtttcaataacctgtccctccacagaaagtaggtgcagtctcttcaccaatacactaagaagtactgtggtcaccatatatgcaaacctcaactctggacactcctgtgtgcctgagaatccaagtgaggaaaaagttttcattactaattcatcatcaaaccgatctggatcaaacttgtgtggagatggccaagtattaggatcctgaagtaccacaccaagggcataaaggacgagggtctgagctgctcaattttctctggagtaacaggaccatttccaaaaacttggtttatctcttcatataattttttttgaacttcttcagaggtggttaaaaaacagattgcccaggtacacaattttgcagttattatgcaactggccagagaaaatatcatactgtcttctaggatctgttggtcattaaggttcccttgtactaaggagtcaatgaaaatatgttgactgaagttccttccttttcgttcttttatgatgttccttaaaacagactccagttgcatgagggtgtgccatgattcttctggaagcgaatgacttcctgatcatcttcaaatgtactacccattaccatctgtgtaacagacttcatagcaaaaccaagcatatgctggctgaggggcacgtgctgggtctctgggtaggagagccatttatctaataattcttctgaaagctttaggaggagggcaaagttactcttcagagaatcagtcacaccattttcatacaattttttcctcatgtggttttcactcacactgccaccaccagattgataccttaataatgacttcagcatggtttcaaaagggtccgttttcttcagttggagtaatccctggaattcctgcagcttgtctggaagccggatagaggtagagcacggctcccaccaacgccagcaagaaggtaacggcgaagatcgcgaagtccaacatggttctgccgcccagggagccacgtctcggatcggccgctccagc

SEQ ID NO: 13589 - RNA, 3314 nt, Homo sapiens
  source 1..3314: mol_type = other RNA
gctgggattacaggcatgagccaccactcccggcccaagttgcagaacaagtgacaaacatcccttctgcttgacagacgccgaggccagaagccttgtccaaggcagggcattgaggcagagggctctgagccgacagttgtccggcactgctccttgggtgggccagcagatttggcttgggctcctgttcagggttgccccccaagtcctgcccggggggcccagtctgacggcctgacgcctctgggctcttgaagtttgaatgtagcatccccaccgaaccgccttcgggctggggacagatagcggaggcggtgggcggggggcaggggcagggcaccgccccacggaggtcgggagtccacttccccccaggggcctcctccagtgccccgctgcctcatcagagccttggctggagtgtccttggagccccaggatttcttgagctcgttgtccccatcactggagccagacagctgggacaggcggcttaggtcccacatggagcggctgggccgggccggggggccgctgggggtccgggcgcgctgcacactccttagaatgtcactgagtgccggccccggggtagcaggggagacgcggcaggcggccaggcggtgggccagcgggccgtcaggcggcggaggcgacgcgggggccacggagcggcggcgggacacgcggtgcgggctgcggccccgctgcaggccacctatgaccgagggtttctgggggggcgcaggtgggagcgggcaggaggccgcgtacagcgtccggaactcaaggctgaaggcgtcaacaatttcaccagtcagcagggtcaccaggcctcggtgcaggcgtgcgtcactccacgtgaagctgtaggatcctgagatgaccctctcgccgtccagcagcacaaacttctcccgcacggtgccgctcacctgccgtcgccagcggctctggaagctgcagccccgcacgacacggacatccacgttctccgtgttccaggggttcacccccagctgctgggccagttccaggaaggcaggcagctgctggcggtccaggagcaggtagacaggtacccagcggcgcgtggcagcatccaccaagtccaaaagcaggtctgggtcagtgaagacgtccatgaccacggccaccagcttgtgggcagcctggatctccagccgcaccagctccttgaggggcggctgaccctctccaggaggctgggtgtacagctgcgcccgggtgatgcctttccacgcagagtccactggccagcccagccgcaggacgggcgccggctgctccgactgcccaggccagtagctcaggctgcccgcgtccacatcggtggtggtggctccctctgccatcccgctgggctcctgcttggccactgtccagtcttcagctgccgctgccaagccctgaacctcatccgcactgaggaagggccacagctcctcgcgctgcacgcaggtctggaacgcctccgcgcccttgctcaacagagcctccagtgccagccgctggccctcggaatatagaaagccggggctggccccgggcaccctgggaccggagtccactccttccagcgccgccagctgggaggccgccatcggggtcactcgggtgggaggactgactgtgagaggctgggtccccgggggtctggctgtctctggggactgtgatcatctgggggttctcctgataggcagaccctacgtggccatccgaggcctccggcggggccctgcagatgtccaaatggctccctgcagcagcccctgccacactgttctgacaatcacgctgcccaaataagcgaccatccaatgtgtcaggccactcagatccgccacctgcctgcacccagtggcaccatgcctggctggccttccgtgaccttcctgccagccgtctctgctggtcaggttgacctcctgacaccatccccaactgtgtgacccatcagctggccatctctgctcagccacacgacagcctccaacccaccagtcacacagtgcccagtcagacccttcagctgtcctgaatttggtcaggctgaccacttgatcatttccaggcggcaagctgcctgcctgtctctaatcacccaaaggtccttaaaggcacgacaggttgcctgcctgcccccggccaagagcacgacgaactgaccctctccttccactgtctggcaaacgccaatggcttccgactgacagtcacagtatctgcctgttggagcatctgtctctggccaaatctgacagcccccacgagtttctcctgctcatcagctctcacccgcagaccagccaggatgcctctccactgggcctgctcgctcagccttaaaggccgaaggcttggcaaacccttccctaccctgtcaatgggggaccctgctccctggaccctcctcacactccttccagctgctgcagtggagggtgaaatgcgctacaggggtctccattactatgggacaggtctatgatcttcacagcccatctaggtgtgagtgccacctaaccagccaccctcctcaggctggctgcccctgcctggggcctggccctgggacctgttccaggccgtcctctgatctgcggggagccctacccaagctgcccccagcctggtttctgcctaaatgctatctcctgccagctacccggacgcttcttcccggacaggggccagtctctatctcgccctgtctccctcccaagcctcagttatccccttgaggctcctgacccaacctcggggaccctggacccttgatccctgcaaaccagaagcccttcattccaatcccaccaacccaggccgctgcttcctccagaccacagcagggagaccggctagtgccgggctcaatggcctcccttccagtgcctgctttttccgagaacgtaggctgtggctccccggcttctacttctgcggtgcttcccggcttctggcctcactcatcaggcctcgacctgtgctctcccagggggtgaacgcccctctagactcaggcttcccggtccccggggggttgagattgcctcacctgttcccaggcagtctctccctccccacagccctgccagcctgcaccctgcacttcccggtccacgccccacccgccatcccagcaccagggaggggcacaggatcctttaagaggggcgggcgtggctgacccaaggaagccggtgtgggaacacctgccacctggctgttgggaaggaggcagggagcttccggggcagtgggggcaggaagagggctggtcttca

SEQ ID NO: 13590 - RNA, 3017 nt, Homo sapiens
  source 1..3017: mol_type = other RNA
gctgggattacaggcatgagccaccactcccggcccaagttgcagaacaagtgacaaacatcccttctgcttgacagacgccgaggccagaagccttgtccaaggcagggcattgaggcagagggctctgagccgacagttgtccggcactgctccttgggtgggccagcagatttggcttgggctcctgttcagggttgccccccaagtcctgcccggggggcccagtctgacggcctgacgcctctgggctcttgaagtttgaatgtagcatccccaccgaaccgccttcgggctggggacagatagcggaggcggtgggcggggggcaggggcagggcaccgccccacggaggtcgggagtccacttccccccaggggcctcctccagtgccccgctgcctcatcagagccttggctggagtgtccttggagccccaggatttcttgagctcgttgtccccatcactggagccagacagctgggacaggcggcttaggtcccacatggagcggctgggccgggccggggggccgctgggggtccgggcgcgctgcacactccttagaatgtcactgagtgccggccccggggtagcaggggagacgcggcaggcggccaggcggtgggccagcgggccgtcaggcggcggaggcgacgcgggggccacggagcggcggcgggacacgcggtgcgggctgcggccccgctgcaggccacctatgaccgagggtttctgggggggcgcaggtgggagcgggcaggaggccgcgtacagcgtccggaactcaaggctgaaggcgtcaacaatttcaccagtcagcagggtcaccaggcctcggtgcaggcgtgcgtcactccacgtgaagctgtaggatcctgagatgaccctctcgccgtccagcagcacaaacttctcccgcacggtgccgctcacctgccgtcgccagcggctctggaagctgcagccccgcacgacacggacatccacgttctccgtgttccaggggttcacccccagctgctgggccagttccaggaaggcaggcagctgctggcggtccaggagcaggtagacaggtacccagcggcgcgtggcagcatccaccaagtccaaaagcaggtctgggtcagtgaagacgtccatgaccacggccaccagcttgtgggcagcctggatctccagccgcaccagctccttgaggggcggctgaccctctccaggaggctgggtgtacagctgcgcccgggtgatgcctttccacgcagagtccactggccagcccagccgcaggacgggcgccggctgctccgactgcccaggccagtagctcaggctgcccgcgtccacatcggtggtggtggctccctctgccatcccgctgggctcctgcttggccactgtccagtcttcagctgccgctgccaagccctgaacctcatccgcactgaggaagggccacagctcctcgcgctgcacgcaggtctggaacgcctccgcgcccttgctcaacagagcctccagtgccagccgctggccctcggaatatagaaagccggggctggccccgggcaccctgggaccggagtccactccttccagcgccgccagctgggaggccgccatcggggtcactcgggtgggaggactgactgtgagaggctgggtccccgggggtctggctgtctctggggactgtgatcatctgggggttctcctgataggcagaccctacgtggccatccgaggcctccggcggggccctgcagatgtccaaatggctccctgcagcagcccctgccacactgttctgacaatcacgctgcccaaataagcgaccatccaatgtgtcaggccactcagatccgccacctgcctgcacccagtggcaccatgcctggctggccttccgtgaccttcctgccagccgtctctgctggtcaggttgacctcctgacaccatccccaactgtgtgacccatcagctggccatctctgctcagccacacgacagcctccaacccaccagtcacacagtgcccagtcagacccttcagctgtcctgaatttggtcaggctgaccacttgatcatttccaggcggcaagctgcctgcctgtctctaatcacccaaaggtccttaaaggcacgacaggttgcctgcctgcccccggccaagagcacgacgaactgaccctctccttccactgtctggcaaacgccaatggcttccgactgacagtcacagtatctgcctgttggagcatctgtctctggccaaatctgacagcccccacgagtttctcctgctcatcagctctcacccgcagaccagccaggatgcctctccactgggcctgctcgctcagccttaaaggccgaaggcttggcaaacccttccctaccctgtcaatgggggaccctgctccctggaccctcctcacactccttccagctgctgcagtggagggtgaaatgcgctacaggggtctccattactatgggacaggtctatgatcttcacagcccatctaggtgtgagtgccacctaaccagccaccctcctcaggctggctgcccctgcctggggcctggccctgggacctgttccaggccgtcctctgatctgcggggagccctacccaagctgcccccagcctggtttctgcctaaatgctatctcctgccagctacccggacgcttcttcccggacaggggccagtctctatctcgccctgtctccctcccaagcctcagttatccccttgaggctcctgacccaacctcggggaccctggacccttgatccctgcaaaccagaagcccttcattccaatcccaccaacccaggccgctgcttcctccagaccacagcagggagccacaccggctagtgccgggctcaatggcctcccttccagtgcctgctttttccgagaacgtaggctgtggctccccggcttctacttctgcggtgcttcccggcttctggcctcactcatcaggcctcgacct

SEQ ID NO: 13591 - RNA, 3155 nt, Homo sapiens
  source 1..3155: mol_type = other RNA
gctgggattacaggcatgagccaccactcccggcccaagttgcagaacaagtgacaaacatcccttctgcttgacagacgccgaggccagaagccttgtccaaggcagggcattgaggcagagggctctgagccgacagttgtccggcactgctccttgggtgggccagcagatttggcttgggctcctgttcagggttgccccccaagtcctgcccggggggcccagtctgacggcctgacgcctctgggctcttgaagtttgaatgtagcatccccaccgaaccgccttcgggctggggacagatagcggaggcggtgggcggggggcaggggcagggcaccgccccacggaggtcgggagtccacttccccccaggggcctcctccagtgccccgctgcctcatcagagccttggctggagtgtccttggagccccaggatttcttgagctcgttgtccccatcactggagccagacagctgggacaggcggcttaggtcccacatggagcggctgggccgggccggggggccgctgggggtccgggcgcgctgcacactccttagaatgtcactgagtgccggccccggggtagcaggggagacgcggcaggcggccaggcggtgggccagcgggccgtcaggcggcggaggcgacgcgggggccacggagcggcggcgggacacgcggtgcgggctgcggccccgctgcaggccacctatgaccgagggtttctgggggggcgcaggtgggagcgggcaggaggccgcgtacagcgtccggaactcaaggctgaaggcgtcaacaatttcaccagtcagcagggtcaccaggcctcggtgcaggcgtgcgtcactccacgtgaagctgtaggatcctgagatgaccctctcgccgtccagcagcacaaacttctcccgcacggtgccgctcacctgccgtcgccagcggctctggaagctgcagccccgcacgacacggacatccacgttctccgtgttccaggggttcacccccagctgctgggccagttccaggaaggcaggcagctgctggcggtccaggagcaggtagacaggtacccagcggcgcgtggcagcatccaccaagtccaaaagcaggtctgggtcagtgaagacgtccatgaccacggccaccagcttgtgggcagcctggatctccagccgcaccagctccttgaggggcggctgaccctctccaggaggctgggtgtacagctgcgcccgggtgatgcctttccacgcagagtccactggccagcccagccgcaggacgggcgccggctgctccgactgcccaggccagtagctcaggctgcccgcgtccacatcggtggtggtggctccctctgccatcccgctgggctcctgcttggccactgtccagtcttcagctgccgctgccaagccctgaacctcatccgcactgaggaagggccacagctcctcgcgctgcacgcaggtctggaacgcctccgcgcccttgctcaacagagcctccagtgccagccgctggccctcggaatatagaaagccggggctggccccgggcaccctgggaccggagtccactccttccagcgccgccagctgggaggccgccatcggggtcactcgggtgggaggactgactgtgagaggctgggtccccgggggtctggctgtctctggggactgtgatcatctgggggttctcctgataggcagaccctacgtggccatccgaggcctccggcggggccctgcagatgtccaaatggctccctgcagcagcccctgccacactgttctgacaatcacgctgcccaaataagcgaccatccaatgtgtcaggccactcagatccgccacctgcctgcacccagtggcaccatgcctggctggccttccgtgaccttcctgccagccgtctctgctggtcaggttgacctcctgacaccatccccaactgtgtgacccatcagctggccatctctgctcagccacacgacagcctccaacccaccagtcacacagtgcccagtcagacccttcagctgtcctgaatttggtcaggctgaccacttgatcatttccaggcggcaagctgcctgcctgtctctaatcacccaaaggtccttaaaggcacgacaggttgcctgcctgcccccggccaagagcacgacgaactgaccctctccttccactgtctggcaaacgccaatggcttccgactgacagtcacagtatctgcctgttggagcatctgtctctggccaaatctgacagcccccacgagtttctcctgctcatcagctctcacccgcagaccagccaggatgcctctccactgggcctgctcgctcagccttaaaggccgaaggcttggcaaacccttccctaccctgtcaatgggggaccctgctccctggaccctcctcacactccttccagctgctgcagtggagggtgaaatgcgctacaggggtctccattactatgggacaggtctatgatcttcacagcccatctaggtgtgagtgccacctaaccagccaccctcctcaggctggctgcccctgcctggggcctggccctgggacctgttccaggccgtcctctgatctgcggggagccctacccaagctgcccccagcctggtttctgcctaaatgctatctcctgccagctacccggacgcttcttcccggacaggggccagtctctatctcgccctgtctccctcccaagcctcagttatccccttgaggctcctgacccaacctcggggaccctggacccttgatccctgcaaaccagaagcccttcattccaatcccaccaacccaggccgctgcttcctccagaccacagcagggagccacaccggctagtgccgggctcaatggcctcccttccagtgcctgctttttccgagaacgtaggctgtggctccccggcttctacttctgcggtgcttcccggcttctggcctcactcatcaggcctcgacctgtgctctcccagggggtgaacgcccctctagactcaggcttcccggtccccggggggttgagattgcctcacctgttcccaggcagtctctccctccccacagccctgccagcctgcaccctgcacttcccggtccac

SEQ ID NO: 13592 - RNA, 1671 nt, Homo sapiens
  source 1..1671: mol_type = other RNA
gctgggattacaggcatgagccaccactcctgactctccttgtttacttttaagcaagaaaggaaaattaaatgtagaacaattatgatagacttgtaaaaggaataaacaccccagatttgcaggccaattctactctgaatcccaaaatacatagtttcttcaactctaatgggtcagagaactatgtggaaagttttttccagaaaagatctttgattaaaacacacacacacacacacacgcacacacacacacacacacacactcattttggggtaagagatttttcctaaataagtatagccatcttgtttctatcatttataattcaatcaggtgcaaagagaggactatataaccatttctccctttaaatgagaaactgggatacaagtggtttgaggtggggaagaaatgatacattttaaaaactcaaatgacaagttcttcctggctggagagtgagacaagagaaaccacaaaaccccagactgtgcaatctgtaaagacagtgataaagtgactacttcatagatgaagatggacaacttgaacttccccttgagtttcacaagggagtcctgtgtgtgagaaggaaggaacatatttgagtgtaatgtgcagttgcatttagatctaaggaaacttaaaatgaatttaagtttccttaattcaaaatgaatttttgagcagttctccacggtaactttaataagtctccatttcaactttctgttctcaatcccatctacagctcaaacatatgcagtatctgccagccctgtccatgaattcctgaagtcccagccaagtgcctctcagctcaaaaagccccttgcttgccaggggtcagccatgtctggaaggctctgaaagaggtctgctgggcagtaggactgcttctgtggatgagaggcctcttgttggactggagagaccaggagccgagataacagcagaagcaaaaatccaccggtgcgtcagcaagcagggcactcggccattcatctccatccttccttctgagctgttctccagcaggctccggccgcagctccaggccactagagcagatagataatgtaggacagaatgaccaggcctatgatggcaaagaacatcaggatgaaaatatccagcattgtggattcctaggccgaccaagcccctggattctggtgaaccgtgagctgtgagcacggaggttgcagtcggtggagagaaatggctccccttcactccacagctcagccctggttctttcccctccccctcccaggggcctgagactgaaggatgctgcagctccaccagcagcttcctgcccccccaccaaccacagccaaccaatcacaaagcctgggggtggatagccaaggagatgccagatttagacccacagaaccgcagaatcaaaggggctcaatttctccccaggaacccaatcccacccctttgtatctaaatggagcctgcatgctctggatgtaggaggagataggatcctacccagctcccccaagagtgaatcctcctgactgccttcttcgcgtttcctctcacacacctcgggcagattatctcagaaaaatcatggttgggtattgggtgggccattggcaacttctaaaggtcacattatggggagacacagacaaaagtttcgtg

SEQ ID NO: 13593 - RNA, 3650 nt, Homo sapiens
  source 1..3650: mol_type = other RNA
gctgggattacaggcatgagccaccactgtgcctggcctaaaaattttttgttaaaaatgctttccaccggccgggtgcagtggctcatgcctataatcccagcactttgggaggccaaggtaggtggatcacctgaggtcaggaatttgagaccagctggccaacatggtgaaaccgcctttctactaaaaatacaaaaactagccaggcatgggggctgacacctgtaatcctagctactcaggaggctgaggcaggagaatcgcttgaacccgggaggtagaggttgcagtgagccaagatcatgccactgcactccagctggagcgacagagtgaaactctgtctcacacacacacacacacacaaaaatactttccacctaattctgaggcagagccaagtttgtgaacactaatgtagaacccacaataaatattgcttccttcttgggaggacttttttcagagattattttttcttctaagttaccttcctgtcaaaaaaggaacggtcttggctacagatttttttttttttttttttttgagatggagtctcgttctgtcacccaggctggagtgcagtggcatgatcacagctcactgcaacctctgcctcccaggttcaagcagttctctgcctcagcctcccgagtagctgggattacaggcgtccgccaccacgcccggctaatttttgtatttttagtagaaacggggtttcaccatctcggccaggctggtcttgaactcctgacctcatgatccatccgccttggcctcccaaagtgctgggattacaggcatgagctaccgcgcccggccttggctgcagattaacgggaatacctcccttgggcttcctaggtgacactgtgatattcggtatgacctcccttgctctattccttggaagaagtacaggcactggtcaagagtgcccgggacccacattgcctggttttgaatcccagcacctccacatgttacgcgtcggacctccaggaagttacttaaactctctgtgcttcagtttcccgagtggcctaaccctaaggggggttacagaacctgcctcatagtgttgattggaagaaataaaggagctcagacctgccaagggctgaggatggtgcctatctagcacatggcaatgctccataagcataagcagctattattattgtggttcctattttttaaatcagatatatcctgcggagccactagcagaatgtgctaaatagctgtctggtgaatgaaagaatgaccaaatggtcctgtatttccttatctagatcatctctaaacaccttctaatggtatggtttcagacctaaatcttcccacaaatctttacggatgcagtaacttttgttaaatcccttcgccccaacttttcatctaccctctgacaacaaaagctgggaaatagagggaagcaaaggaatcatgtacggctgatgggatttagacagcacagagcaagtggttaggtttaaagaacgtcatccaaataccctggcaggaaaccttgtatactgacagttgcaatatgtgtaagaaaagaatgcatccaatggtatcctcaattaattaattaattaattaatttttgagacagtctctctctgtcgcccaggctggagtgcaatggtgcaatctcagctcactgcaacctccacctcctgggttcaagcaattctcctgcctcagcctcccaagtagctgggactacaggcacatgccaccacggctaattttctgtatttttagtagagacagggtttcaccatgttggccaggatggtcttgatctcctgacttcatgatccgcccgcctcagcctcccaaagtgctgggattataggcatgagccaccacgcccagcctctcaatttttttgttttttcagaagatgggaggcaacatggtaggttcacaattaaaattgtcttgaaagtatttattgtttaataattctttctcccctcagccccatccggccactctctctttctgcttttctgatcatcctaaaggctgaatacatcctcctcctgtgtggaggacacgaagcaatactaaaatcaatacactcgatcaggtcttcatcagataccacgtcactgtgggtagagtgctagttttcaacaaatgtggtgttcttagggctccacaaggtagtcctttctcaaggtcgctgggccactcatggagttgaaatgccgctgcccatctaagtacaacatggactctccatatgtttttgggaaaaccaatggcacttctttttccgacatgaacgtgaaatgaaagacattggtggttgtatgctgcttctcctgcagggaggccacttcactgtgtactctgacttgaatataattattctgagtaaagcatacctgtgaagaaagaaagagcaatgagccaacctcaacaggtttctgaaacatgatgtcatctactgctaccacaaacggtcgagaaccaccaaagctacaagcagtagcccacgcaagttcatatgccttcctcataaggaaaccaccaaagatccgattgaaaatgttccgctcctgagggtggcaaatttccaaactcttcagttttgaattctccatccacactgcattagagggtaaaactcgactccgaaaacttatagtctttggatccagtgtgctgagaaacatctcatgtatggtggtcctctcctcagcgctgggggccattttcagtaacgacgtggagctgaaggcaattcttctccccttgttcaattccccttgtctaaagagctcctcttcctctgggctttcagggatgagtggatttacaaatgccggccctttattttcagaatcacgagccaccattacaaatgttgcatccaaaacaggacaaaattcatcaccatgtaactggaacatttgcatcttcacttccatggatgtcttcccgacccagctaacatggccactgaacttaatgtcctgttctgggctcaagctcttcttacacatatcaatcttatccaccagggctgtaactatcgataaaggagacatcttggcggagtggattttgttgtgcatgtaacaaataagaactcccaagctgtcaagatcctcaagaatcctgccaaatcttacggtgttttgaacagtcaaatatttctctcgtaattcaggctcactgcccaaaggcaagagaacttcaatataactgtccttcattctcctaggaggcagtccatcctgtgatttagccaagaaactatgaagtaatttcctttcttccattgccttcacatggtctctccagtttgtggatgctcctactatctcccgcaacttatctcgaacatgattcacatgtatagatgaacatgcttcatgaatgtggaagattccctgtttcttggggttctggggtccttgagtcagtcctcttccaggagtaagctgccctttgcccaaggcacaaagccgcagtgctgcccgcctcattgcgctaggctgccgtgcgcgcgatggagaaccgggccccgcgcgctagtcggcggagggaaactgaggcgataaaagacgcacgagtaccagaccgcgcccttgctgaggacagcccgggagccggacagc

SEQ ID NO: 13594 - RNA, 3525 nt, Homo sapiens
  source 1..3525: mol_type = other RNA
gctgggattacaggcatgagccaccactgtgcctggcctaaaaattttttgttaaaaatgctttccaccggccgggtgcagtggctcatgcctataatcccagcactttgggaggccaaggtaggtggatcacctgaggtcaggaatttgagaccagctggccaacatggtgaaaccgcctttctactaaaaatacaaaaactagccaggcatgggggctgacacctgtaatcctagctactcaggaggctgaggcaggagaatcgcttgaacccgggaggtagaggttgcagtgagccaagatcatgccactgcactccagctggagcgacagagtgaaactctgtctcacacacacacacacacacaaaaatactttccacctaattctgaggcagagccaagtttgtgaacactaatgtagaacccacaataaatattgcttccttcttgggaggacttttttcagagattattttttcttctaagttaccttcctgtcaaaaaaggaacggtcttggctacagatttttttttttttttttttttgagatggagtctcgttctgtcacccaggctggagtgcagtggcatgatcacagctcactgcaacctctgcctcccaggttcaagcagttctctgcctcagcctcccgagtagctgggattacaggcgtccgccaccacgcccggctaatttttgtatttttagtagaaacggggtttcaccatctcggccaggctggtcttgaactcctgacctcatgatccatccgccttggcctcccaaagtgctgggattacaggcatgagctaccgcgcccggccttggctgcagattaacgggaatacctcccttgggcttcctaggtgacactgtgatattcggtatgacctcccttgctctattccttggaagaagtacaggcactggtcaagagtgcccgggacccacattgcctggttttgaatcccagcacctccacatgttacgcgtcggacctccaggaagttacttaaactctctgtgcttcagtttcccgagtggcctaaccctaaggggggttacagaacctgcctcatagtgttgattggaagaaataaaggagctcagacctgccaagggctgaggatggtgcctatctagcacatggcaatgctccataagcataagcagctattattattgtggttcctattttttaaatcagatatatcctgcggagccactagcagaatgtgctaaatagctgtctggtgaatgaaagaatgaccaaatggtcctgtatttccttatctagatcatctctaaacaccttctaatggtatggtttcagacctaaatcttcccacaaatctttacggatgcagtaacttttgttaaatcccttcgccccaacttttcatctaccctctgacaacaaaagctgggaaatagagggaagcaaaggaatcatgtacggctgatgggatttagacagcacagagcaagtggttaggtttaaagaacgtcatccaaataccctggcaggaaaccttgtatactgacagttgcaatatgtgtaagaaaagaatgcatccaatggtatcctcaattaattaattaattaattaatttttgagacagtctctctctgtcgcccaggctggagtgcaatggtgcaatctcagctcactgcaacctccacctcctgggttcaagcaattctcctgcctcagcctcccaagtagctgggactacaggcacatgccaccacggctaattttctgtatttttagtagagacagggtttcaccatgttggccaggatggtcttgatctcctgacttcatgatccgcccgcctcagcctcccaaagtgctgggattataggcatgagccaccacgcccagcctctcaatttttttgttttttcagaagatgggaggcaacatggtaggttcacaattaaaattgtcttgaaagtatttattgtttaataattctttctcccctcagccccatccggccactctctctttctgcttttctgatcatcctaaaggctgaatacatcctcctcctgtgtggaggacacgaagcaatactaaaatcaatacactcgatcaggtcttcatcagataccacgtcactgtgggtagagtgctagttttcaacaaatgtggtgttcttagggctccacaaggtagtcctttctcaaggtcgctgggccactcatggagttgaaatgccgctgcccatctaagtacaacatggactctccatatgtttttgggaaaaccaatggcacttctttttccgacatgaacgtgaaatgaaagacattggtggttgtatgctgcttctcctgcagggaggccacttcactgtgtactctgacttgaatataattattctgagtaaagcatacctgtgaagaaagaaagagcaatgagccaacctcaacaggtttctgaaacatgatgtcatctactgctaccacaaacggtcgagaaccaccaaagctacaagcagtagcccacgcaagttcatatgccttcctcataaggaaaccaccaaagatccgattgaaaatgttccgctcctgagggtggcaaatttccaaactcttcagttttgaattctccatccacactgcattagagggtaaaactcgactccgaaaacttatagtctttggatccagtgtgctgagaaacatctcatgtatggtggtcctctcctcagcgctgggggccattttcagtaacgacgtggagctgaaggcaattcttctccccttgttcaattccccttgtctaaagagctcctcttcctctgggctttcagggatgagtggatttacaaatgccggccctttattttcagaatcacgagccaccattacaaatgttgcatccaaaacaggacaaaattcatcaccatgtaactggaacatttgcatcttcacttccatggatgtcttcccgacccagctaacatggccactgaacttaatgtcctgttctgggctcaagctcttcttacacatatcaatcttatccaccagggctgtaactatcgataaaggagacatcttggcggagtggattttgttgtgcatgtaacaaataagaactcccaagctgtcaagatcctcaagaatcctgccaaatcttacggtgttttgaacagtcaaatatttctctcgtaattcaggctcactgcccaaaggcaagagaacttcaatataactgtccttcattctcctaggaggcagtccatcctgtgatttagccaagaaactatgaagtaatttcctttcttccattgccttcacatggtctctccagtttgtggatgctcctactatctcccgcaacttatctcgaacgcagtgctgcccgcctcattgcgctaggctgccgtgcgcgcgatggagaaccgggccccgcgcgctagtcggcggagggaaactgaggcgataaaagacgcacgagtaccagaccgcgcccttgctgaggacagcccgggagccggacagc

SEQ ID NO: 13595 - RNA, 3623 nt, Homo sapiens
  source 1..3623: mol_type = other RNA
gctgggattacaggcatgagccaccactgtgcctggcctaaaaattttttgttaaaaatgctttccaccggccgggtgcagtggctcatgcctataatcccagcactttgggaggccaaggtaggtggatcacctgaggtcaggaatttgagaccagctggccaacatggtgaaaccgcctttctactaaaaatacaaaaactagccaggcatgggggctgacacctgtaatcctagctactcaggaggctgaggcaggagaatcgcttgaacccgggaggtagaggttgcagtgagccaagatcatgccactgcactccagctggagcgacagagtgaaactctgtctcacacacacacacacacacaaaaatactttccacctaattctgaggcagagccaagtttgtgaacactaatgtagaacccacaataaatattgcttccttcttgggaggacttttttcagagattattttttcttctaagttaccttcctgtcaaaaaaggaacggtcttggctacagatttttttttttttttttttttgagatggagtctcgttctgtcacccaggctggagtgcagtggcatgatcacagctcactgcaacctctgcctcccaggttcaagcagttctctgcctcagcctcccgagtagctgggattacaggcgtccgccaccacgcccggctaatttttgtatttttagtagaaacggggtttcaccatctcggccaggctggtcttgaactcctgacctcatgatccatccgccttggcctcccaaagtgctgggattacaggcatgagctaccgcgcccggccttggctgcagattaacgggaatacctcccttgggcttcctaggtgacactgtgatattcggtatgacctcccttgctctattccttggaagaagtacaggcactggtcaagagtgcccgggacccacattgcctggttttgaatcccagcacctccacatgttacgcgtcggacctccaggaagttacttaaactctctgtgcttcagtttcccgagtggcctaaccctaaggggggttacagaacctgcctcatagtgttgattggaagaaataaaggagctcagacctgccaagggctgaggatggtgcctatctagcacatggcaatgctccataagcataagcagctattattattgtggttcctattttttaaatcagatatatcctgcggagccactagcagaatgtgctaaatagctgtctggtgaatgaaagaatgaccaaatggtcctgtatttccttatctagatcatctctaaacaccttctaatggtatggtttcagacctaaatcttcccacaaatctttacggatgcagtaacttttgttaaatcccttcgccccaacttttcatctaccctctgacaacaaaagctgggaaatagagggaagcaaaggaatcatgtacggctgatgggatttagacagcacagagcaagtggttaggtttaaagaacgtcatccaaataccctggcaggaaaccttgtatactgacagttgcaatatgtgtaagaaaagaatgcatccaatggtatcctcaattaattaattaattaattaatttttgagacagtctctctctgtcgcccaggctggagtgcaatggtgcaatctcagctcactgcaacctccacctcctgggttcaagcaattctcctgcctcagcctcccaagtagctgggactacaggcacatgccaccacggctaattttctgtatttttagtagagacagggtttcaccatgttggccaggatggtcttgatctcctgacttcatgatccgcccgcctcagcctcccaaagtgctgggattataggcatgagccaccacgcccagcctctcaatttttttgttttttcagaagatgggaggcaacatggtaggttcacaattaaaattgtcttgaaagtatttattgtttaataattctttctcccctcagccccatccggccactctctctttctgcttttctgatcatcctaaaggctgaatacatcctcctcctgtgtggaggacacgaagcaatactaaaatcaatacactcgatcaggtcttcatcagataccacgtcactgtgggtagagtgctagttttcaacaaatgtggtgttcttagggctccacaaggtagtcctttctcaaggtcgctgggccactcatggagttgaaatgccgctgcccatctaagtacaacatggactctccatatgtttttgggaaaaccaatggcacttctttttccgacatgaacgtgaaatgaaagacattggtggttgtatgctgcttctcctgcagggaggccacttcactgtgtactctgacttgaatataattattctgagtaaagcatacctgtgaagaaagaaagagcaatgagccaacctcaacaggtttctgaaacatgatgtcatctactgctaccacaaacggtcgagaaccaccaaagctacaagcagtagcccacgcaagttcatatgccttcctcataaggaaaccaccaaagatccgattgaaaatgttccgctcctgagggtggcaaatttccaaactcttcagttttgaattctccatccacactgcattagagggtaaaactcgactccgaaaacttatagtctttggatccagtgtgctgagaaacatctcatgtatggtggtcctctcctcagcgctgggggccattttcagtaacgacgtggagctgaaggcaattcttctccccttgttcaattccccttgtctaaagagctcctcttcctctgggctttcagggatgagtggatttacaaatgccggccctttattttcagaatcacgagccaccattacaaatgttgcatccaaaacaggacaaaattcatcaccatgtaactggaacatttgcatcttcacttccatggatgtcttcccgacccagctaacatggccactgaacttaatgtcctgttctgggctcaagctcttcttacacatatcaatcttatccaccagggctgtaactatcgataaaggagacatcttggcggagtggattttgttgtgcatgtaacaaataagaactcccaagctgtcaagatcctcaagaatcctgccaaatcttacggtgttttgaacagtcaaatatttctctcgtaattcaggctcactgcccaaaggcaagagaacttcaatataactgtccttcattctcctaggaggcagtccatcctgtgatttagccaagaaactatgaagtaatttcctttcttccattgccttcacatggtctctccagtttgtggatgctcctactatctcccgcaacttatctcgaacttcatgaatgtggaagattccctgtttcttggggttctggggtccttgagtcagtcctcttccaggagtaagctgccctttgcccaaggcacaaagccgcagtgctgcccgcctcattgcgctaggctgccgtgcgcgcgatggagaaccgggccccgcgcgctagtcggcggagggaaactgaggcgataaaagacgcacgagtaccagaccgcgcccttgctgaggacagcccgggagccggacagc

SEQ ID NO: 13596 - RNA, 4210 nt, Homo sapiens
  source 1..4210: mol_type = other RNA
gctgggattacaggcatgagccaccagacccggcctgtgttaggcatttataaggagatggcagtccagctcctggtgataagaaaatgtagactcccaagattcatgttttaactttcttcataagttaagcaggagtcatttgcctctgtcatgaattccaagactacaaagttttaagagatgctgggatagcaaatgaggcttgaattctgtgttgacaagcccacacacctcatttcatttagtatccaagagataaacaaacaccacctcttctactccaggactggcatctctggacttttctgccataatcccaaatcaggccaactctccttcctctaggattcgcgtggtgggatgccaggcagtgacacccttagagcaggaagtctgactgtagacccagctacaccccaaccagtgagggtctgcattgggcacttgggcctcctcgtgaggcgggggtccagggttctggtgcaatgcccaaggcagggccacttctcagccctagctctgggccagcacagtgccccggtttggctgcaccaactcacaggctcttagctggggttctggcaggtggggctcggctagaaacagattagacagtgttgctaattcttcagcaaagtcccctggccactgggcctggtggaggctgcccaggcaggcctctatctccatccgtcccatcagacccttctccaccagctcccgtagcaagaatagcagcaagtcccactcccttggccttgtgtctgccagaagccccacatttcttgggctcagcagcagctgcagcggaaccggcccctgaaagtcttccttccacaaggaaagcagcatgtgcagaagccttcgagcctgccctctctccagcctgtactgtgccgggggccctaggataggaatttgatctgcaacgaggagggaagctaactccacagagcactttgccagatgctgctcagcaggtgggcacaggaactggcggcaccgcagcgtctggcccagctggcctaggagctgttccagatgctctggggagactccctcgtcagggtcccgtggccccacggccaaggagagcacgtcaggcgcgggagcagcccctccgctccccccgggcagcaggttcaggaccctgggctcgaagtgtgcgactcactgctgctttcacctccctcctgatcagtgctgtgatgttggctgacagccaagcacaggctttctctgttgcaagccccacagcaatgttctctgcactgctcagaacggctgccggggtctcctctggaagcagcgcccgcacagccccagggctcttcctttgacagaactcccgccccagggccaatgcctgggccccgtgagggcacagctgggaacacaagatctccaacagctgggctgggtctcccccttcctctccctgtgtcaccagctgctcttggagaagtgactctgcctggcgcaccagatctgccaccagtgtagccttgatatgtttgacacagtttgatccaattctttctgccacgaactctacggtccggcgcaaggagggcggctggttgtggaaaaaggcctgggcgagctgtgcctgcagcccctggctggtctgggaaggctgggctcccaggctggtggtagtggtgggggtgattttcctcatgaagcccccactccgtccactactgcctgacacccacgaagcgagcagtttccggagctctccgatgtaggggcagcaggtgtagagcagctgctggtccaccacaggcgcattgtccaagccatgctctggggctactgtgtccacctcaaaggcatatgagggaccctcttccagaaagaacaagtcctcagggactgtgggaatctggaaaagccagcccaggacagcaagtagcagcagcttgttcaggaaacacatcttcccctcactctcctgcgacaacaccaagctccggtgcaggcgcagcaggagagtgaagatgtcccggtaatattccagcaagggaacaacatggtcagcaaaggagagaaactccaccagccagggcacggtgagcaccgcccggcgggcctgcagccctcgctgcagcagagtccgcacatccaggaccggagggacctggctcctgagggccagaatggagtcctgaagctcaccggtcgggggaggttcaggcccccggtatggcaggaaagccacaaagcccaggaatttagccaaaagtctcaggctaagaagcaccacagcaaattgcttccgctcaccctgccagtctacgtctgactccccgtcttcatcattgggctcatgctggggcagggcaagaccattgagctcctggatcttcaagctcagactgtccatgagatgctggttaaactggaagctgctggcactaaggatgaagtccctaaagaagccttgacagcctgggaaggtggggggtgggcagggccccccactgctctgaggagccataagccgttcctgtaggcgccacaaccgccccagcttgtcagctcccagcatactcaacacatctggggcctcgcccaagacggtgcccccagcaccaccagggctctgacacatctggagtagttgtttttggaaaagccgaacaaagtggctgtggctgcaggctgcggagagctgacccatcatggccctgattctgctgcccaagcccttctcaaaatcccagccaggctcctcatggtgatcttcccactctcgcagcacctcataaaacacatccctctgtttcttaaaagtatgaaaggctcggtcactggagaagttggcacgattgtcagtctctggctgaaaggagacagcttgagtagagggaggcatcaccagagagaccttggcaacactgccctcataggcagctcgaaggcggccttgcagagctggtgagaagcacagcagccgctcattctcagccagcagcttcaaggtccctttgtccaggttggaaagaacctgaaagtgacactccaaaacctgcactgcaaagaagacacaatcgtggatgctttggaacagtggactttccagggaatctaggacagctggacttagttcagggtcgctgtccttggcagtcaccatcctccgggcagtgaggagctgaaagacgaagaaaagctccaagaagaggtttggtaccaggttctcagcaatgcacgaggagtaaacaagggctacaagctccaggcgctggcgggaagacactctggcagggtctgcaggttcatctgtgaggcttcctgtccggctggggaggggcgaccccaattctggggtgggacaggtgggggtaggtgactgctgcagctgcttagagcgctccttcctgagcatctctcgctcctcttgcagacttctgcaccctgggggaaggccaaggccccaagggctagtgtccagggctgagggttgggaactggggacacagctgattgggggtgaggtgaagcaggtcttgggcttggagagtgaccgctcttcgctcaccggagttgggttgatcctgcgagaaggcttcgtcctgcctgtagggccggggggaaccgagcctacgggagggaactcctccaggttgctgaggtttggcggatcagacagcgtgaggctggggcggctggggctgccagagcccctaagcctccggcccccggctccgggcaggctctccccgctgaccccctcctccaggccgcggcctccacgctcgcgggccggccccgggccccgcctcctgcccccgcggcgggccagaggggcctcggcagcggtgctctgggcctcggtcggagggaaaagctggctgcgcgccccgcggctaccccgcggcgggcctcccggcctccctggcaaggctgccgaggcgcccggggtcttggcgggggtcgggggcccctgcgggaggacgcggctgctctgctccctcaggaagttcaacaggaacggtacgaattctttccgcagggcccggagtgagctcagcgcggccgcctccccagcgttatcctgggggcgtgtcaccgctgttacctccgaaccctgggtgctgcgcgcgatccaccgcacgacggctgcgaccgacacctcttctcgcagcagcgactccaaaacggccgccatcccggtcggggcgctctggggcgactgcgc

SEQ ID NO: 13597 - RNA, 3303 nt, Homo sapiens
  source 1..3303: mol_type = other RNA
gctgggattacaggcatgagccaccagacccggcctgtgttaggcatttataaggagatggcagtccagctcctggtgataagaaaatgtagactcccaagattcatgttttaactttcttcataagttaagcaggagtcatttgcctctgtcatgaattccaagactacaaagttttaagagatgctgggatagcaaatgaggcttgaattctgtgttgacaagcccacacacctcatttcatttagtatccaagagataaacaaacaccacctcttctactccaggactggcatctctggacttttctgccataatcccaaatcaggccaactctccttcctctaggattcgcgtggtgggatgccaggcagtgacacccttagagcaggaagtctgactgtagacccagctacaccccaaccagtgagggtctgcattgggcacttgggcctcctcgtgaggcgggggtccagggttctggtgcaatgcccaaggcagggccacttctcagccctagctctgggccagcacagtgccccggtttggctgcaccaactcacaggctcttagctggggttctggcaggtggggctcggctagaaacagattagacagtgttgctaattcttcagcaaagtcccctggccactgggcctggtggaggctgcccaggcaggcctctatctccatccgtcccatcagacccttctccaccagctcccgtagcaagaatagcagcaagtcccactcccttggccttgtgtctgccagaagccccacatttcttgggctcagcagcagctgcagcggaaccggcccctgaaagtcttccttccacaaggaaagcagcatgtgcagaagccttcgagcctgccctctctccagcctgtactgtgccgggggccctaggataggaatttgatctgcaacgaggagggaagctaactccacagagcactttgccagatgctgctcagcaggtgggcacaggaactggcggcaccgcagcgtctggcccagctggcctaggagctgttccagatgctctggggagactccctcgtcagggtcccgtggccccacggccaaggagagcacgtcttttatctcggagatgaggtgggaggggaggggagcatggtgctcacaggcgcgggagcagcccctccgctccccccgggcagcaggttcaggaccctgggctcgaagtgtgcgactcactgctgctttcacctccctcctgatcagtgctgtgatgttggctgacagccaagcacaggctttctctgttgcaagccccacagcaatgttctctgcactgctcagaacggctgccggggtctcctctggaagcagcgcccgcacagccccagggctcttcctttgacagaactcccgccccagggccaatgcctgggccccgtgagggcacagctgggaacacaagatctccaacagctgggctgggtctcccccttcctctccctgtgtcaccagctgctcttggagaagtgactctgcctggcgcaccagatctgccaccagtgtagccttgatatgtttgacacagtttgatccaattctttctgccacgaactctacggtccggcgcaaggagggcggctggttgtggaaaaaggcctgggcgagctgtgcctgcagcccctggctggtctgggaaggctgggctcccaggctggtggtagtggtgggggtgattttcctcatgaagcccccactccgtccactactgcctgacacccacgaagcgagcagtttccggagctctccgatgtaggggcagcaggtgtagagcagctgctggtccaccacaggcgcattgtccaagccatgctctggggctactgtgtccacctcaaaggcatatgagggaccctcttccagaaagaacaagtcctcagggactgtgggaatctggaaaagccagcccaggacagcaagtagcagcagcttgttcaggaaacacatcttcccctcactctcctgcgacaacaccaagctccggtgcaggcgcagcaggagagtgaagatgtcccggtaatattccagcaagggaacaacatggtcagcaaaggagagaaactccaccagccagggcacggtgagcaccgcccggcgggcctgcagccctcgctgcagcagagtccgcacatccaggaccggagggacctggctcctgagggccagaatggagtcctgaagctcaccggtcgggggaggttcaggcccccggtatggcaggaaagccacaaagcccaggaatttagccaaaagtctcaggctaagaagcaccacagcaaattgcttccgctcaccctgccagtctacgtctgactccccgtcttcatcattgggctcatgctggggcagggcaagaccattgagctcctggatcttcaagctcagactgtccatgagatgctggttaaactggaagctgctggcactaaggatgaagtccctaaagaagccttgacagcctgggaaggtggggggtgggcagggccccccactgctctgaggagccataagccgttcctgtaggcgccacaaccgccccagcttgtcagctcccagcatactcaacacatctggggcctcgcccaagacggtgcccccagcaccaccagggctctgacacatctggagtagttgtttttggaaaagccgaacaaagtggctgtggctgcaggctgcggagagctgacccatcatggccctgattctgctgcccaagcccttctcaaaatcccagccaggctcctcatggtgatcttcccactctcgcagcacctcataaaacacatccctctgtttcttaaaagtatgaaaggctcggtcactggagaagttggcacgattgtcagtctctggctgaaaggagacagcttgagtagagggaggcatcaccagagagaccttggcaacactgccctcataggcagctcgaaggcggccttgcagagctggtgagaagcacagcagccgctcattctcagccagcagcttcaaggtccctttgtccaggttggaaagaacctgaaagtgacactccaaaacctgcactgcaaagaagacacaatcgtggatgctttggaacagtggactttccagggaatctaggacagctggacttagttcagggtcgctgtccttggcagtcaccatcctccgggcagtgaggagcagcaatgcacgaggagtaaacaagggctacaagctccaggcgctggcgggaagacactctggcagggtctgcaggttcatctgtgaggcttc

SEQ ID NO: 13598 - RNA, 4226 nt, Homo sapiens
  source 1..4226: mol_type = other RNA
gctgggattacaggcatgagccaccagacccggcctgtgttaggcatttataaggagatggcagtccagctcctggtgataagaaaatgtagactcccaagattcatgttttaactttcttcataagttaagcaggagtcatttgcctctgtcatgaattccaagactacaaagttttaagagatgctgggatagcaaatgaggcttgaattctgtgttgacaagcccacacacctcatttcatttagtatccaagagataaacaaacaccacctcttctactccaggactggcatctctggacttttctgccataatcccaaatcaggccaactctccttcctctaggattcgcgtggtgggatgccaggcagtgacacccttagagcaggaagtctgactgtagacccagctacaccccaaccagtgagggtctgcattgggcacttgggcctcctcgtgaggcgggggtccagggttctggtgcaatgcccaaggcagggccacttctcagccctagctctgggccagcacagtgccccggtttggctgcaccaactcacaggctcttagctggggttctggcaggtggggctcggctagaaacagattagacagtgttgctaattcttcagcaaagtcccctggccactgggcctggtggaggctgcccaggcaggcctctatctccatccgtcccatcagacccttctccaccagctcccgtagcaagaatagcagcaagtcccactcccttggccttgtgtctgccagaagccccacatttcttgggctcagcagcagctgcagcggaaccggcccctgaaagtcttccttccacaaggaaagcagcatgtgcagaagccttcgagcctgccctctctccagcctgtactgtgccgggggccctaggataggaatttgatctgcaacgaggagggaagctaactccacagagcactttgccagatgctgctcagcaggtgggcacaggaactggcggcaccgcagcgtctggcccagctggcctaggagctgttccagatgctctggggagactccctcgtcagggtcccgtggccccacggccaaggagagcacgtcttttatctcggagatgaggtgggaggggaggggagcatggtgctcacaggcgcgggagcagcccctccgctccccccgggcagcaggttcaggaccctgggctcgaagtgtgcgactcactgctgctttcacctccctcctgatcagtgctgtgatgttggctgacagccaagcacaggctttctctgttgcaagccccacagcaatgttctctgcactgctcagaacggctgccggggtctcctctggaagcagcgcccgcacagccccagggctcttcctttgacagaactcccgccccagggccaatgcctgggccccgtgagggcacagctgggaacacaagatctccaacagctgggctgggtctcccccttcctctccctgtgtcaccagctgctcttggagaagtgactctgcctggcgcaccagatctgccaccagtgtagccttgatatgtttgacacagtttgatccaattctttctgccacgaactctacggtccggcgcaaggagggcggctggttgtggaaaaaggcctgggcgagctgtgcctgcagcccctggctggtctgggaaggctgggctcccaggctggtggtagtggtgggggtgattttcctcatgaagcccccactccgtccactactgcctgacacccacgaagcgagcagtttccggagctctccgatgtaggggcagcaggtgtagagcagctgctggtccaccacaggcgcattgtccaagccatgctctggggctactgtgtccacctcaaaggcatatgagggaccctcttccagaaagaacaagtcctcagggactgtgggaatctggaaaagccagcccaggacagcaagtagcagcagcttgttcaggaaacacatcttcccctcactctcctgcgacaacaccaagctccggtgcaggcgcagcaggagagtgaagatgtcccggtaatattccagcaagggaacaacatggtcagcaaaggagagaaactccaccagccagggcacggtgagcaccgcccggcgggcctgcagccctcgctgcagcagagtccgcacatccaggaccggagggacctggctcctgagggccagaatggagtcctgaagctcaccggtcgggggaggttcaggcccccggtatggcaggaaagccacaaagcccaggaatttagccaaaagtctcaggctaagaagcaccacagcaaattgcttccgctcaccctgccagtctacgtctgactccccgtcttcatcattgggctcatgctggggcagggcaagaccattgagctcctggatcttcaagctcagactgtccatgagatgctggttaaactggaagctgctggcactaaggatgaagtccctaaagaagccttgacagcctgggaaggtggggggtgggcagggccccccactgctctgaggagccataagccgttcctgtaggcgccacaaccgccccagcttgtcagctcccagcatactcaacacatctggggcctcgcccaagacggtgcccccagcaccaccagggctctgacacatctggagtagttgtttttggaaaagccgaacaaagtggctgtggctgcaggctgcggagagctgacccatcatggccctgattctgctgcccaagcccttctcaaaatcccagccaggctcctcatggtgatcttcccactctcgcagcacctcataaaacacatccctctgtttcttaaaagtatgaaaggctcggtcactggagaagttggcacgattgtcagtctctggctgaaaggagacagcttgagtagagggaggcatcaccagagagaccttggcaacactgccctcataggcagctcgaaggcggccttgcagagctggtgagaagcacagcagccgctcattctcagccagcagcttcaaggtccctttgtccaggttggaaagaacctgaaagtgacactccaaaacctgcactgcaaagaagacacaatcgtggatgctttggaacagtggactttccagggaatctaggacagctggacttagttcagggtcgctgtccttggcagtcaccatcctccgggcagtgaggagctgaaagacgaagaaaagctccaagaagaggtttggtaccaggttctcagcaatgcacgaggagtaaacaagggctacaagctccaggcgctggcgggaagacactctggcagggtctgcaggttcatctgtgaggcttcctgtccggctggggaggggcgaccccaattctggggtgggacaggtgggggtaggtgactgctgcagctgcttagagcgctccttcctgagcatctctcgctcctcttgcagacttctgcaccctgggggaaggccaaggccccaagggctagtgtccagggctgagggttgggaactggggacacagctgattgggggtgaggtgaagcaggtcttgggcttggagagtgaccgctcttcgctcaccggagttgggttgatcctgcgagaaggcttcgtccctgtagggccggggggaaccgagcctacgggagggaactcctccaggttgctgaggtttggcggatcagacagcgtgaggctggggcggctggggctgccagagcccctaagcctccggcccccggctccgggcaggctctccccgctgaccccctcctccaggccgcggcctccacgctcgcgggccggccccgggccccgcctcctgcccccgcggcgggccagaggggcctcggcagcggtgctctgggcctcggtcggagggaaaagctggctgcgcgccccgcggctaccccgcggcgggcctcccggcctccctggcaaggctgccgaggcgcccggggtcttggcgggggtcgggggcccctgcgggaggacgcggctgctctgctccctcaggaagttcaacaggaacggtacgaattctttccgcagggcccggagtgagctcagcgcggccgcctccccagcgttatcctccgaaccctgggtgctgcgcgcgatccaccgcacgacggctgcgaccgacacctcttctcgcagcagcgactccaaaacggccgccatcccggtcggggcgctctggggcgact

SEQ ID NO: 13599 - RNA, 4254 nt, Homo sapiens
  source 1..4254: mol_type = other RNA
gctgggattacaggcatgagccaccagacccggcctgtgttaggcatttataaggagatggcagtccagctcctggtgataagaaaatgtagactcccaagattcatgttttaactttcttcataagttaagcaggagtcatttgcctctgtcatgaattccaagactacaaagttttaagagatgctgggatagcaaatgaggcttgaattctgtgttgacaagcccacacacctcatttcatttagtatccaagagataaacaaacaccacctcttctactccaggactggcatctctggacttttctgccataatcccaaatcaggccaactctccttcctctaggattcgcgtggtgggatgccaggcagtgacacccttagagcaggaagtctgactgtagacccagctacaccccaaccagtgagggtctgcattgggcacttgggcctcctcgtgaggcgggggtccagggttctggtgcaatgcccaaggcagggccacttctcagccctagctctgggccagcacagtgccccggtttggctgcaccaactcacaggctcttagctggggttctggcaggtggggctcggctagaaacagattagacagtgttgctaattcttcagcaaagtcccctggccactgggcctggtggaggctgcccaggcaggcctctatctccatccgtcccatcagacccttctccaccagctcccgtagcaagaatagcagcaagtcccactcccttggccttgtgtctgccagaagccccacatttcttgggctcagcagcagctgcagcggaaccggcccctgaaagtcttccttccacaaggaaagcagcatgtgcagaagccttcgagcctgccctctctccagcctgtactgtgccgggggccctaggataggaatttgatctgcaacgaggagggaagctaactccacagagcactttgccagatgctgctcagcaggtgggcacaggaactggcggcaccgcagcgtctggcccagctggcctaggagctgttccagatgctctggggagactccctcgtcagggtcccgtggccccacggccaaggagagcacgtcttttatctcggagatgaggtgggaggggaggggagcatggtgctcacaggcgcgggagcagcccctccgctccccccgggcagcaggttcaggaccctgggctcgaagtgtgcgactcactgctgctttcacctccctcctgatcagtgctgtgatgttggctgacagccaagcacaggctttctctgttgcaagccccacagcaatgttctctgcactgctcagaacggctgccggggtctcctctggaagcagcgcccgcacagccccagggctcttcctttgacagaactcccgccccagggccaatgcctgggccccgtgagggcacagctgggaacacaagatctccaacagctgggctgggtctcccccttcctctccctgtgtcaccagctgctcttggagaagtgactctgcctggcgcaccagatctgccaccagtgtagccttgatatgtttgacacagtttgatccaattctttctgccacgaactctacggtccggcgcaaggagggcggctggttgtggaaaaaggcctgggcgagctgtgcctgcagcccctggctggtctgggaaggctgggctcccaggctggtggtagtggtgggggtgattttcctcatgaagcccccactccgtccactactgcctgacacccacgaagcgagcagtttccggagctctccgatgtaggggcagcaggtgtagagcagctgctggtccaccacaggcgcattgtccaagccatgctctggggctactgtgtccacctcaaaggcatatgagggaccctcttccagaaagaacaagtcctcagggactgtgggaatctggaaaagccagcccaggacagcaagtagcagcagcttgttcaggaaacacatcttcccctcactctcctgcgacaacaccaagctccggtgcaggcgcagcaggagagtgaagatgtcccggtaatattccagcaagggaacaacatggtcagcaaaggagagaaactccaccagccagggcacggtgagcaccgcccggcgggcctgcagccctcgctgcagcagagtccgcacatccaggaccggagggacctggctcctgagggccagaatggagtcctgaagctcaccggtcgggggaggttcaggcccccggtatggcaggaaagccacaaagcccaggaatttagccaaaagtctcaggctaagaagcaccacagcaaattgcttccgctcaccctgccagtctacgtctgactccccgtcttcatcattgggctcatgctggggcagggcaagaccattgagctcctggatcttcaagctcagactgtccatgagatgctggttaaactggaagctgctggcactaaggatgaagtccctaaagaagccttgacagcctgggaaggtggggggtgggcagggccccccactgctctgaggagccataagccgttcctgtaggcgccacaaccgccccagcttgtcagctcccagcatactcaacacatctggggcctcgcccaagacggtgcccccagcaccaccagggctctgacacatctggagtagttgtttttggaaaagccgaacaaagtggctgtggctgcaggctgcggagagctgacccatcatggccctgattctgctgcccaagcccttctcaaaatcccagccaggctcctcatggtgatcttcccactctcgcagcacctcataaaacacatccctctgtttcttaaaagtatgaaaggctcggtcactggagaagttggcacgattgtcagtctctggctgaaaggagacagcttgagtagagggaggcatcaccagagagaccttggcaacactgccctcataggcagctcgaaggcggccttgcagagctggtgagaagcacagcagccgctcattctcagccagcagcttcaaggtccctttgtccaggttggaaagaacctgaaagtgacactccaaaacctgcactgcaaagaagacacaatcgtggatgctttggaacagtggactttccagggaatctaggacagctggacttagttcagggtcgctgtccttggcagtcaccatcctccgggcagtgaggagctgaaagacgaagaaaagctccaagaagaggtttggtaccaggttctcagcaatgcacgaggagtaaacaagggctacaagctccaggcgctggcgggaagacactctggcagggtctgcaggttcatctgtgaggcttcctgtccggctggggaggggcgaccccaattctggggtgggacaggtgggggtaggtgactgctgcagctgcttagagcgctccttcctgagcatctctcgctcctcttgcagacttctgcaccctgggggaaggccaaggccccaagggctagtgtccagggctgagggttgggaactggggacacagctgattgggggtgaggtgaagcaggtcttgggcttggagagtgaccgctcttcgctcaccggagttgggttgatcctgcgagaaggcttcgtccctgtagggccggggggaaccgagcctacgggagggaactcctccaggttgctgaggtttggcggatcagacagcgtgaggctggggcggctggggctgccagagcccctaagcctccggcccccggctccgggcaggctctccccgctgaccccctcctccaggccgcggcctccacgctcgcgggccggccccgggccccgcctcctgcccccgcggcgggccagaggggcctcggcagcggtgctctgggcctcggtcggagggaaaagctggctgcgcgccccgcggctaccccgcggcgggcctcccggcctccctggcaaggctgccgaggcgcccggggtcttggcgggggtcgggggcccctgcgggaggacgcggctgctctgctccctcaggaagttcaacaggaacggtacgaattctttccgcagggcccggagtgagctcagcgcggccgcctccccagcgttatcctgggggcgtgtcaccgctgttacctccgaaccctgggtgctgcgcgcgatccaccgcacgacggctgcgaccgacacctcttctcgcagcagcgactccaaaacggccgccatcccggtcggggcgctctggggcgactgcgc

SEQ ID NO: 13600 - RNA, 4232 nt, Homo sapiens
  source 1..4232: mol_type = other RNA
gctgggattacaggcatgagccaccagacccggcctgtgttaggcatttataaggagatggcagtccagctcctggtgataagaaaatgtagactcccaagattcatgttttaactttcttcataagttaagcaggagtcatttgcctctgtcatgaattccaagactacaaagttttaagagatgctgggatagcaaatgaggcttgaattctgtgttgacaagcccacacacctcatttcatttagtatccaagagataaacaaacaccacctcttctactccaggactggcatctctggacttttctgccataatcccaaatcaggccaactctccttcctctaggattcgcgtggtgggatgccaggcagtgacacccttagagcaggaagtctgactgtagacccagctacaccccaaccagtgagggtctgcattgggcacttgggcctcctcgtgaggcgggggtccagggttctggtgcaatgcccaaggcagggccacttctcagccctagctctgggccagcacagtgccccggtttggctgcaccaactcacaggctcttagctggggttctggcaggtggggctcggctagaaacagattagacagtgttgctaattcttcagcaaagtcccctggccactgggcctggtggaggctgcccaggcaggcctctatctccatccgtcccatcagacccttctccaccagctcccgtagcaagaatagcagcaagtcccactcccttggccttgtgtctgccagaagccccacatttcttgggctcagcagcagctgcagcggaaccggcccctgaaagtcttccttccacaaggaaagcagcatgtgcagaagccttcgagcctgccctctctccagcctgtactgtgccgggggccctaggataggaatttgatctgcaacgaggagggaagctaactccacagagcactttgccagatgctgctcagcaggtgggcacaggaactggcggcaccgcagcgtctggcccagctggcctaggagctgttccagatgctctggggagactccctcgtcagggtcccgtggccccacggccaaggagagcacgtcttttatctcggagatgaggtgggaggggaggggagcatggtgctcacaggcgcgggagcagcccctccgctccccccgggcagcaggttcaggaccctgggctcgaagtgtgcgactcactgctgctttcacctccctcctgatcagtgctgtgatgttggctgacagccaagcacaggctttctctgttgcaagccccacagcaatgttctctgcactgctcagaacggctgccggggtctcctctggaagcagcgcccgcacagccccagggctcttcctttgacagaactcccgccccagggccaatgcctgggccccgtgagggcacagctgggaacacaagatctccaacagctgggctgggtctcccccttcctctccctgtgtcaccagctgctcttggagaagtgactctgcctggcgcaccagatctgccaccagtgtagccttgatatgtttgacacagtttgatccaattctttctgccacgaactctacggtccggcgcaaggagggcggctggttgtggaaaaaggcctgggcgagctgtgcctgcagcccctggctggtctgggaaggctgggctcccaggctggtggtagtggtgggggtgattttcctcatgaagcccccactccgtccactactgcctgacacccacgaagcgagcagtttccggagctctccgatgtaggggcagcaggtgtagagcagctgctggtccaccacaggcgcattgtccaagccatgctctggggctactgtgtccacctcaaaggcatatgagggaccctcttccagaaagaacaagtcctcagggactgtgggaatctggaaaagccagcccaggacagcaagtagcagcagcttgttcaggaaacacatcttcccctcactctcctgcgacaacaccaagctccggtgcaggcgcagcaggagagtgaagatgtcccggtaatattccagcaagggaacaacatggtcagcaaaggagagaaactccaccagccagggcacggtgagcaccgcccggcgggcctgcagccctcgctgcagcagagtccgcacatccaggaccggagggacctggctcctgagggccagaatggagtcctgaagctcaccggtcgggggaggttcaggcccccggtatggcaggaaagccacaaagcccaggaatttagccaaaagtctcaggctaagaagcaccacagcaaattgcttccgctcaccctgccagtctacgtctgactccccgtcttcatcattgggctcatgctggggcagggcaagaccattgagctcctggatcttcaagctcagactgtccatgagatgctggttaaactggaagctgctggcactaaggatgaagtccctaaagaagccttgacagcctgggaaggtggggggtgggcagggccccccactgctctgaggagccataagccgttcctgtaggcgccacaaccgccccagcttgtcagctcccagcatactcaacacatctggggcctcgcccaagacggtgcccccagcaccaccagggctctgacacatctggagtagttgtttttggaaaagccgaacaaagtggctgtggctgcaggctgcggagagctgacccatcatggccctgattctgctgcccaagcccttctcaaaatcccagccaggctcctcatggtgatcttcccactctcgcagcacctcataaaacacatccctctgtttcttaaaagtatgaaaggctcggtcactggagaagttggcacgattgtcagtctctggctgaaaggagacagcttgagtagagggaggcatcaccagagagaccttggcaacactgccctcataggcagctcgaaggcggccttgcagagctggtgagaagcacagcagccgctcattctcagccagcagcttcaaggtccctttgtccaggttggaaagaacctgaaagtgacactccaaaacctgcactgcaaagaagacacaatcgtggatgctttggaacagtggactttccagggaatctaggacagctggacttagttcagggtcgctgtccttggcagtcaccatcctccgggcagtgaggagctgaaagacgaagaaaagctccaagaagaggtttggtaccaggttctcagcaatgcacgaggagtaaacaagggctacaagctccaggcgctggcgggaagacactctggcagggtctgcaggttcatctgtgaggcttcctgtccggctggggaggggcgaccccaattctggggtgggacaggtgggggtaggtgactgctgcagctgcttagagcgctccttcctgagcatctctcgctcctcttgcagacttctgcaccctgggggaaggccaaggccccaagggctagtgtccagggctgagggttgggaactggggacacagctgattgggggtgaggtgaagcaggtcttgggcttggagagtgaccgctcttcgctcaccggagttgggttgatcctgcgagaaggcttcgtcctgcctgtagggccggggggaaccgagcctacgggagggaactcctccaggttgctgaggtttggcggatcagacagcgtgaggctggggcggctggggctgccagagcccctaagcctccggcccccggctccgggcaggctctccccgctgaccccctcctccaggccgcggcctccacgctcgcgggccggccccgggccccgcctcctgcccccgcggcgggccagaggggcctcggcagcggtgctctgggcctcggtcggagggaaaagctggctgcgcgccccgcggctaccccgcggcgggcctcccggcctccctggcaaggctgccgaggcgcccggggtcttggcgggggtcgggggcccctgcgggaggacgcggctgctctgctccctcaggaagttcaacaggaacggtacgaattctttccgcagggcccggagtgagctcagcgcggccgcctccccagcgttatcctccgaaccctgggtgctgcgcgcgatccaccgcacgacggctgcgaccgacacctcttctcgcagcagcgactccaaaacggccgccatcccggtcggggcgctctggggcgactgcg

SEQ ID NO: 13601 - RNA, 4257 nt, Homo sapiens
  source 1..4257: mol_type = other RNA
gctgggattacaggcatgagccaccagacccggcctgtgttaggcatttataaggagatggcagtccagctcctggtgataagaaaatgtagactcccaagattcatgttttaactttcttcataagttaagcaggagtcatttgcctctgtcatgaattccaagactacaaagttttaagagatgctgggatagcaaatgaggcttgaattctgtgttgacaagcccacacacctcatttcatttagtatccaagagataaacaaacaccacctcttctactccaggactggcatctctggacttttctgccataatcccaaatcaggccaactctccttcctctaggattcgcgtggtgggatgccaggcagtgacacccttagagcaggaagtctgactgtagacccagctacaccccaaccagtgagggtctgcattgggcacttgggcctcctcgtgaggcgggggtccagggttctggtgcaatgcccaaggcagggccacttctcagccctagctctgggccagcacagtgccccggtttggctgcaccaactcacaggctcttagctggggttctggcaggtggggctcggctagaaacagattagacagtgttgctaattcttcagcaaagtcccctggccactgggcctggtggaggctgcccaggcaggcctctatctccatccgtcccatcagacccttctccaccagctcccgtagcaagaatagcagcaagtcccactcccttggccttgtgtctgccagaagccccacatttcttgggctcagcagcagctgcagcggaaccggcccctgaaagtcttccttccacaaggaaagcagcatgtgcagaagccttcgagcctgccctctctccagcctgtactgtgccgggggccctaggataggaatttgatctgcaacgaggagggaagctaactccacagagcactttgccagatgctgctcagcaggtgggcacaggaactggcggcaccgcagcgtctggcccagctggcctaggagctgttccagatgctctggggagactccctcgtcagggtcccgtggccccacggccaaggagagcacgtcttttatctcggagatgaggtgggaggggaggggagcatggtgctcacaggcgcgggagcagcccctccgctccccccgggcagcaggttcaggaccctgggctcgaagtgtgcgactcactgctgctttcacctccctcctgatcagtgctgtgatgttggctgacagccaagcacaggctttctctgttgcaagccccacagcaatgttctctgcactgctcagaacggctgccggggtctcctctggaagcagcgcccgcacagccccagggctcttcctttgacagaactcccgccccagggccaatgcctgggccccgtgagggcacagctgggaacacaagatctccaacagctgggctgggtctcccccttcctctccctgtgtcaccagctgctcttggagaagtgactctgcctggcgcaccagatctgccaccagtgtagccttgatatgtttgacacagtttgatccaattctttctgccacgaactctacggtccggcgcaaggagggcggctggttgtggaaaaaggcctgggcgagctgtgcctgcagcccctggctggtctgggaaggctgggctcccaggctggtggtagtggtgggggtgattttcctcatgaagcccccactccgtccactactgcctgacacccacgaagcgagcagtttccggagctctccgatgtaggggcagcaggtgtagagcagctgctggtccaccacaggcgcattgtccaagccatgctctggggctactgtgtccacctcaaaggcatatgagggaccctcttccagaaagaacaagtcctcagggactgtgggaatctggaaaagccagcccaggacagcaagtagcagcagcttgttcaggaaacacatcttcccctcactctcctgcgacaacaccaagctccggtgcaggcgcagcaggagagtgaagatgtcccggtaatattccagcaagggaacaacatggtcagcaaaggagagaaactccaccagccagggcacggtgagcaccgcccggcgggcctgcagccctcgctgcagcagagtccgcacatccaggaccggagggacctggctcctgagggccagaatggagtcctgaagctcaccggtcgggggaggttcaggcccccggtatggcaggaaagccacaaagcccaggaatttagccaaaagtctcaggctaagaagcaccacagcaaattgcttccgctcaccctgccagtctacgtctgactccccgtcttcatcattgggctcatgctggggcagggcaagaccattgagctcctggatcttcaagctcagactgtccatgagatgctggttaaactggaagctgctggcactaaggatgaagtccctaaagaagccttgacagcctgggaaggtggggggtgggcagggccccccactgctctgaggagccataagccgttcctgtaggcgccacaaccgccccagcttgtcagctcccagcatactcaacacatctggggcctcgcccaagacggtgcccccagcaccaccagggctctgacacatctggagtagttgtttttggaaaagccgaacaaagtggctgtggctgcaggctgcggagagctgacccatcatggccctgattctgctgcccaagcccttctcaaaatcccagccaggctcctcatggtgatcttcccactctcgcagcacctcataaaacacatccctctgtttcttaaaagtatgaaaggctcggtcactggagaagttggcacgattgtcagtctctggctgaaaggagacagcttgagtagagggaggcatcaccagagagaccttggcaacactgccctcataggcagctcgaaggcggccttgcagagctggtgagaagcacagcagccgctcattctcagccagcagcttcaaggtccctttgtccaggttggaaagaacctgaaagtgacactccaaaacctgcactgcaaagaagacacaatcgtggatgctttggaacagtggactttccagggaatctaggacagctggacttagttcagggtcgctgtccttggcagtcaccatcctccgggcagtgaggagctgaaagacgaagaaaagctccaagaagaggtttggtaccaggttctcagcaatgcacgaggagtaaacaagggctacaagctccaggcgctggcgggaagacactctggcagggtctgcaggttcatctgtgaggcttcctgtccggctggggaggggcgaccccaattctggggtgggacaggtgggggtaggtgactgctgcagctgcttagagcgctccttcctgagcatctctcgctcctcttgcagacttctgcaccctgggggaaggccaaggccccaagggctagtgtccagggctgagggttgggaactggggacacagctgattgggggtgaggtgaagcaggtcttgggcttggagagtgaccgctcttcgctcaccggagttgggttgatcctgcgagaaggcttcgtcctgcctgtagggccggggggaaccgagcctacgggagggaactcctccaggttgctgaggtttggcggatcagacagcgtgaggctggggcggctggggctgccagagcccctaagcctccggcccccggctccgggcaggctctccccgctgaccccctcctccaggccgcggcctccacgctcgcgggccggccccgggccccgcctcctgcccccgcggcgggccagaggggcctcggcagcggtgctctgggcctcggtcggagggaaaagctggctgcgcgccccgcggctaccccgcggcgggcctcccggcctccctggcaaggctgccgaggcgcccggggtcttggcgggggtcgggggcccctgcgggaggacgcggctgctctgctccctcaggaagttcaacaggaacggtacgaattctttccgcagggcccggagtgagctcagcgcggccgcctccccagcgttatcctgggggcgtgtcaccgctgttacctccgaaccctgggtgctgcgcgcgatccaccgcacgacggctgcgaccgacacctcttctcgcagcagcgactccaaaacggccgccatcccggtcggggcgctctggggcgactgcgc

SEQ ID NO: 13602 - RNA, 4193 nt, Homo sapiens
  source 1..4193: mol_type = other RNA
gctgggattacaggcatgagccaccagacccggcctgtgttaggcatttataaggagatggcagtccagctcctggtgataagaaaatgtagactcccaagattcatgttttaactttcttcataagttaagcaggagtcatttgcctctgtcatgaattccaagactacaaagttttaagagatgctgggatagcaaatgaggcttgaattctgtgttgacaagcccacacacctcatttcatttagtatccaagagataaacaaacaccacctcttctactccaggactggcatctctggacttttctgccataatcccaaatcaggccaactctccttcctctaggattcgcgtggtgggatgccaggcagtgacacccttagagcaggaagtctgactgtagacccagctacaccccaaccagtgagggtctgcattgggcacttgggcctcctcgtgaggcgggggtccagggttctggtgcaatgcccaaggcagggccacttctcagccctagctctgggccagcacagtgccccggtttggctgcaccaactcacaggctcttagctggggttctggcaggtggggctcggctagaaacagattagacagtgttgctaattcttcagcaaagtcccctggccactgggcctggtggaggctgcccaggcaggcctctatctccatccgtcccatcagacccttctccaccagctcccgtagcaagaatagcagcaagtcccactcccttggccttgtgtctgccagaagccccacatttcttgggctcagcagcagctgcagcggaaccggcccctgaaagtcttccttccacaaggaaagcagcatgtgcagaagccttcgagcctgccctctctccagcctgtactgtgccgggggccctaggataggaatttgatctgcaactggcggcaccgcagcgtctggcccagctggcctaggagctgttccagatgctctggggagactccctcgtcagggtcccgtggccccacggccaaggagagcacgtcttttatctcggagatgaggtgggaggggaggggagcatggtgctcacaggcgcgggagcagcccctccgctccccccgggcagcaggttcaggaccctgggctcgaagtgtgcgactcactgctgctttcacctccctcctgatcagtgctgtgatgttggctgacagccaagcacaggctttctctgttgcaagccccacagcaatgttctctgcactgctcagaacggctgccggggtctcctctggaagcagcgcccgcacagccccagggctcttcctttgacagaactcccgccccagggccaatgcctgggccccgtgagggcacagctgggaacacaagatctccaacagctgggctgggtctcccccttcctctccctgtgtcaccagctgctcttggagaagtgactctgcctggcgcaccagatctgccaccagtgtagccttgatatgtttgacacagtttgatccaattctttctgccacgaactctacggtccggcgcaaggagggcggctggttgtggaaaaaggcctgggcgagctgtgcctgcagcccctggctggtctgggaaggctgggctcccaggctggtggtagtggtgggggtgattttcctcatgaagcccccactccgtccactactgcctgacacccacgaagcgagcagtttccggagctctccgatgtaggggcagcaggtgtagagcagctgctggtccaccacaggcgcattgtccaagccatgctctggggctactgtgtccacctcaaaggcatatgagggaccctcttccagaaagaacaagtcctcagggactgtgggaatctggaaaagccagcccaggacagcaagtagcagcagcttgttcaggaaacacatcttcccctcactctcctgcgacaacaccaagctccggtgcaggcgcagcaggagagtgaagatgtcccggtaatattccagcaagggaacaacatggtcagcaaaggagagaaactccaccagccagggcacggtgagcaccgcccggcgggcctgcagccctcgctgcagcagagtccgcacatccaggaccggagggacctggctcctgagggccagaatggagtcctgaagctcaccggtcgggggaggttcaggcccccggtatggcaggaaagccacaaagcccaggaatttagccaaaagtctcaggctaagaagcaccacagcaaattgcttccgctcaccctgccagtctacgtctgactccccgtcttcatcattgggctcatgctggggcagggcaagaccattgagctcctggatcttcaagctcagactgtccatgagatgctggttaaactggaagctgctggcactaaggatgaagtccctaaagaagccttgacagcctgggaaggtggggggtgggcagggccccccactgctctgaggagccataagccgttcctgtaggcgccacaaccgccccagcttgtcagctcccagcatactcaacacatctggggcctcgcccaagacggtgcccccagcaccaccagggctctgacacatctggagtagttgtttttggaaaagccgaacaaagtggctgtggctgcaggctgcggagagctgacccatcatggccctgattctgctgcccaagcccttctcaaaatcccagccaggctcctcatggtgatcttcccactctcgcagcacctcataaaacacatccctctgtttcttaaaagtatgaaaggctcggtcactggagaagttggcacgattgtcagtctctggctgaaaggagacagcttgagtagagggaggcatcaccagagagaccttggcaacactgccctcataggcagctcgaaggcggccttgcagagctggtgagaagcacagcagccgctcattctcagccagcagcttcaaggtccctttgtccaggttggaaagaacctgaaagtgacactccaaaacctgcactgcaaagaagacacaatcgtggatgctttggaacagtggactttccagggaatctaggacagctggacttagttcagggtcgctgtccttggcagtcaccatcctccgggcagtgaggagctgaaagacgaagaaaagctccaagaagaggtttggtaccaggttctcagcaatgcacgaggagtaaacaagggctacaagctccaggcgctggcgggaagacactctggcagggtctgcaggttcatctgtgaggcttcctgtccggctggggaggggcgaccccaattctggggtgggacaggtgggggtaggtgactgctgcagctgcttagagcgctccttcctgagcatctctcgctcctcttgcagacttctgcaccctgggggaaggccaaggccccaagggctagtgtccagggctgagggttgggaactggggacacagctgattgggggtgaggtgaagcaggtcttgggcttggagagtgaccgctcttcgctcaccggagttgggttgatcctgcgagaaggcttcgtcctgcctgtagggccggggggaaccgagcctacgggagggaactcctccaggttgctgaggtttggcggatcagacagcgtgaggctggggcggctggggctgccagagcccctaagcctccggcccccggctccgggcaggctctccccgctgaccccctcctccaggccgcggcctccacgctcgcgggccggccccgggccccgcctcctgcccccgcggcgggccagaggggcctcggcagcggtgctctgggcctcggtcggagggaaaagctggctgcgcgccccgcggctaccccgcggcgggcctcccggcctccctggcaaggctgccgaggcgcccggggtcttggcgggggtcgggggcccctgcgggaggacgcggctgctctgctccctcaggaagttcaacaggaacggtacgaattctttccgcagggcccggagtgagctcagcgcggccgcctccccagcgttatcctgggggcgtgtcaccgctgttacctccgaaccctgggtgctgcgcgcgatccaccgcacgacggctgcgaccgacacctcttctcgcagcagcgactccaaaacggccgccatcccggtcggggcgctctggggcgactgcgc

SEQ ID NO: 13603 - RNA, 1760 nt, Homo sapiens
  source 1..1760: mol_type = other RNA
gctgggattacaggcatgagccaccagagctattttatatactatttactcctacatactctgaggtctcagttagctacactttatcttgttctcaactatgattggataaccaagaatcagcagacacttgaggaaggctcataatatagaagaagcagacaacaaaacaaagatgtgaccactgagtggagggatatagttcaaggaacagaagagagtttgaaaacatcagtaatcaaagaaccaaaaaaacttttcgaaataaaaatacagtctctaaaatcaatatttgatccaaggattggaagggaaagtacaagcatgaaataaacaatataaaaagctccccaaatgtagaacaaagcccacagatatggaaaatataaaacaggagagaaaaaatgaatcgattcaggagggaaagggagagaaagagggaagggaccatctaaagaaagtggggagagaccgggaaagaagtcagttcgggcgtcagcagaacaagtagattacaacagcagccaggggaaagtgtgcagggatagggaggatgaaatcagggcaagaggaggctaacgagaaaaggcaatttctccattcctgaccttccccactgagcccagctttggcttcagagtgatttcagagtggcttcagagtgactcatgatcccagtggaagtgttcctgggggaaggggcagtgggtcagacagcccagggcaggaagaggcaatgagatgtcttacagtggggctgcctggaagaagcctggggcatgggctttctccagcaaggctgggtgtgagtcctgtgcactgtggtcttcccaaagtgctcctctccctgcactcctcatggctggccttgtccgtcctctcctccaggcagtagatcccgcagctcctcaatgcttgggttcctcctggctcctcctgctccttggctcctacgtgcactcccgtgcaaacctgaccagtcccggacacattttcttttccacatgcacaaaagtttgggcacaccttgcaacatacactgtaccttagtcttttcaaagaatgacacctcttttctcctaatatgtaaaaagagaagtagctacagatgtaacaggaagtgagcaagagacttgaaggagattcgagtaggtttgcggtgttgacttccgagcttggattcaagtccctgaagggcaccagacacctgtgatcaccaaggagaggagaggagacaggaccatgtggctgtccccatctctgctgcttctcatcctcccaggtgagtgtggctggagctttaaggcactggaatgacagcggctggcttggagacagagacgctctgttctcaggaaggagacatgtcagggaaaatgacagcgccaattcatccatccatgcccatattcattaaatagcaatcaagtttttgttatctgacaggttctgtgttagatgcttaattgttgtctttccattctgatgtagaacttttttcagagtgaacaaatgaagcccctatacccatctttccccaggaggtcgtgtgtagtttcttagttcccttcagatgccatagaaagcagatttgggcatggagtccaatttctgttccaggaattccttgggttgtggagctctgcctgtttatggtgaaattgtcttccgctcccaccatggtgaccctgatatcccagtacctctttagggcactgatcttgtatctgctgccgctcccagtacctctttagggcact

SEQ ID NO: 13604 - RNA, 1924 nt, Homo sapiens
  source 1..1924: mol_type = other RNA
gctgggattacaggcatgagccaccagagctattttatatactatttactcctacatactctgaggtctcagttagctacactttatcttgttctcaactatgattggataaccaagaatcagcagacacttgaggaaggctcataatatagaagaagcagacaacaaaacaaagatgtgaccactgagtggagggatatagttcaaggaacagaagagagtttgaaaacatcagtaatcaaagaaccaaaaaaacttttcgaaataaaaatacagtctctaaaatcaatatttgatccaaggattggaagggaaagtacaagcatgaaataaacaatataaaaagctccccaaatgtagaacaaagcccacagatatggaaaatataaaacaggagagaaaaaatgaatcgattcaggagggaaagggagagaaagagggaagggaccatctaaagaaagtggggagagaccgggaaagaagtcagttcgggcgtcagcagaacaagtagattacaacagcagccaggggaaagtgtgcagggatagggaggatgaaatcagggcaagaggaggctaacgagaaaaggcaatttctccattcctgaccttccccactgagcccagctttggcttcagagtgatttcagagtggcttcagagtgactcatgatcccagtggaagtgttcctgggggaaggggcagtgggtcagacagcccagggcaggaagaggcaatgagatgtcttacagtggggctgcctggaagaagcctggggcatgggctttctccagcaaggctgggtgtgagtcctgtgcactgtggtcttcccaaagtgctcctctccctgcactcctcatggctggccttgtccgtcctctcctccaggcagtagatcccgcagctcctcaatgcttgggttcctcctggctcctcctgctccttggctcctacgtgcactcccgtgcaaacctgaccagtcccggacacattttcttttccacatgcacaaaagtttgggcacaccttgcaacatacactgtaccttagtcttttcaaagaatgacacctcttttctcctaatatgtaaaaagagaagtagctacagatgtaacaggaagtgagcaagagacttgaaggagattcgagtaggtttgcggtgttgacttccgagcttggattcaagtccctgaagggcaccagacacctgtgatcaccaaggagaggagaggagacaggaccatgtggctgtccccatctctgctgcttctcatcctcccaggtgagtgtggctggagctttaaggcactggaatgacagcggctggcttggagacagagacgctctgttctcaggaaggagacatgtcagggaaaatgacagcgccaattcatccatccatgcccatattcattaaatagcaatcaagtttttgttatctgacaggttctgtgttagatgcttaattgttgtctttccattctgatgtagaacttttttcagagtgaacaaatgaagcccctatacccatctttccccaggaggtcgtgtgtagtttcttagttcccttcagatgccatagaaagcagatttgggcatggagtccaatttctgttccaggaattccttgggttgtggagctctgcctgtttatggtgaaattgtcttccgctcccaccatggtgacccttttattggctgccggcagacttgttccagggtttctcgttcgtcttgtcagtttctctttctctgctccagcagaccttctttgctcacgttcctgtcccggccaccacttgtcgctgttggttgctaggggattgaacaaaggggggacgaatgcagaaatgaagacaaagacaaagagatctgttttgaaagaaggggtcagggagctccttgcttctagtgaacaagggcc

SEQ ID NO: 13605 - RNA, 16916 nt, Homo sapiens
  source 1..16916: mol_type = other RNA
gctgggattacaggcatgagccaccataataaggattctgatgaacatttgattccttggactactgttatactcaaaagccttccttaatcttctaattgtcaccctaaatatcctaaaatttctgtcttcctagtagttcttcatagtcctaaaaatttgtcagagagaaaggtaaatcaagaaacatgattttcaaatgatttaaggtggtactagggtttaggatttcctttgctttttatcatttaacacactgcttatcatacagctggaagtgctctgggccagtgtctctacttcgagggaagaaggaggtagtgagacagaaggaaatagcacaattcctggccctgacagaagggtgttcaggagacctgctctcctctcactttattccatctcatctggacctgtggcttccaatccacatctctttcctttaatatcctgcattggctaggctgtataaatcctttggtgcatcgaaaaactaagtgcattttttgtttttgtgattatgcaatacttataggaaaagttataattttagaatatttaagtacacttacatttttgagaaaaagactattgaaatgtttgtgccatgtcaaatttcagttgaacattttgggtattcttaatataagaccaggccaggcaccgtggctcaggccgggcacagtggctcacacctataatcccagcacttagggaggccaaggcgggaagatcacctgaagtcaggagttcaagaccagcctggctaacaaggtgaaactctgtctctactaaaaatacaaaaattagccgggcgtggtggctggcgcttgtaatcccagctacttgggaggctgagacaggagaatcacttgaacctgggaagcagaggttgtggtgagctgagatcgcaccattgcactccagcctgggcaacaaagagcgaaactccgtctcaaaaaaataaaaaataaaccctagaattatagtatgttagaattggaagggaagaattgtctaaggttattctagctaataagcaacagacttggaaaggaaaaggtcctgacaaagctaagcctcccgttcaggtttcctgactcgtgaattcagtgctgctgccactacacgatgcatgctctttgtatcaagggtgagacagcattacacatacatagaaaattatctatttaaactctatttgaacttttgatgagtttgtctccccctcccccactccttttcagaataacttgacgtttacaggtaccatcagtggtgatgtctgtgtgtggaaagatcacatattgtgtagaatcgtggcgagagctcacaacgggcctgtgtttgccatgtacaccaccctgcgagatggacttatcgtgactgggggaaaggaaaggccgtgagtcctctttcttttcacagaatatttatgcatttgtgacctacctgaggtttgcagttaattattctagttgtttctaggctacacagagtgtcctctccgaccttcctcctcatatgcttctcctttattaccttttatgtgccttctatttgattctcatttctggtcttaattcacttccaatttttttcatgttggggtgatactttttctgaggtgtggataggtagttgtcctacaagttgagttacttttcttaatgtctgtatgcctgtgtatgatttgctgagtaggaggcccatgggggaatctggagccagggttgtattttgactgcctgctctctttttgttcagaatggattctaaggagtagaatgcacattgttgctttagaaaaggatgagggaactagagagaactgccttgtttccttttgcttgaggcaaatttaaactgttttatacaagacctcaaaatttgagaagaggtctcttctgagtgattttcaaatctcccaacagtaaccagatacttatgatttgatttgtcaccaacatagtcatatgcatgttgaaacatgacatgtaggccaggcacagtggctcacacctgtaatcttatcactttgggaggctgaggcaggtggatcgcttgagcccaggagttcaagaccagcctgggcaacatggtgaaaccccatcgctataaaaaacaacaattagccgggtgtggtggcacatgcctgtagtccctgctactcaggaggctgaggtgggaggatcacttgagcctggggaggtcaaggctttagtgagctgtgatggtgccactgcactccagcctgggtgacagagtgagaccccatttaaaaaacaaaaacaaaaacaaaaaaaaatgtgacatatagttgactaagaagtacatttcaatacaggattgaaagaacccacatatgttaattaaacacaagcgcagaatttgtgccttttacataaaggaagaatgcacataggcatgctttcagacaagcaattcatctagcagaaaaggaaggaatacatttttcagcccttccaggaataaaatccataaatgggctctatttcgtcctccaacacttgtatttcccacgtcatttactcctgcacacccccactcactagaagcctgctaaactgttccagtgagatattttaacacctgatagggaataaatatgcttctgttttggccttcaaaaataagctctgggccagttgcagtggctcacgcctgtaatcccaacactttgggaggccgaggtgggcggatcacgaggtcaggagtttgggatcagcctggccaatatggtgaaactccatctctactaaaaatacaaaaattagccaggcatggtgcctgtaatcccagctacttgggaggctgaaggagaagaatcgcttgaacctgggaggcacaggttgcagtgagccgagatcacaccactgcactccaggccaggtgacagagcgacactctgtctcaaaaaaataaataaatcaactctgtagcatagcatttgtaattctattattttgccttacatttccattatccttttaataaaattgtttttttacatcttcctaatcaagaagtattatgaggccaggcacagtggctcatacctggaatcccagcactttgggaggccgaggcaggcagatcacctgaggtcaaggtatttgagaccagcctggccaacatggtgaaaccccatctctactaaaaatacagaaattagctgggtgtggtggtgcacacctgtaatgctagctactcgggaggctgaggtaggagaatcgcttgaacctgggaggcagaggttgcaataagcctagatcatgccactgcactcaagcctgggagacagagcgagactacatcttaaaaaaaaaaaaaaaagtattatgagagaggataatgtattgtaatgtattgtagaggctaaataaaattatgctcatgtcagaaaaaaagagtatttctcaaaataaaattcactgaaactggatgtttattttgactgagatatagtatatcctcaaattgccatagaaagtttacaagaatattagaggtaaattataaatatcagggcctttttaaaaaaaaaagattctgcttataacttggtatttgtttataataaaaattatagtagccaataatgaacacttactctggcttggttatttacttaggtcaaaagaaggaggagcggttaaactgtgggatcaggaactgaggcggtgccgtgccttcaggcttgagacaggacaagccacagattgtgttcgttctgtgtgcagaggcaaagtaagatgttccatgagctgatacagtgcagcagaaaacagaaagtggttattactgtgattccctcaccctttgcagcctaatgaacaatacttaataatgcataacgatggatttgcttgccaacattactctgtctttgctgctttctttgccaaagttagcaccagtgtggtgcataagctaggaagctattctgtctaaatactgtatgtaaacctccaatattttctagaatctgccaatttaacaactctagtagacataattgaaagcccttggcagttgactcatattaggacagctgtctccattttttaaaaaaacacacattccctagataaaacgtgcagtaaacaaacaatgaaatactactcagccataaaaaataatgaaattctgtcattcttggtggcaacatggatgagactggaggacatgatgtgaagtgaaataagccaggcacagaaagataaatacatgttctcactcctgtgcagaaactaaaaaagttgatcccacagaggtggagagtagaatagtggttactggaggcggacaagggggagggggagggggatagggaaggactggttaaaggatacaagtttacacagccagataggaatagtatgttttagtattctgtagtactgtaggatgactatagttaagaatcacgtatttatgtattttcaggtatttacaagagaggattttgaaagtttccatcacaaagaaatgataaatgtctgaggtgatggttatgcgtattaccctatgccctatagatatgtataattatgtgtcaatttcaaaataaaaattcaaaactacaactcctatgaaaatttttgagcgtgtttgtacttattaagtgtatttataaatcatacggatattatcttcagcctgcatattaaattgtagttaagcttttactttttaactaaaaaataaattctattattttttcctatatcccactgcactgaccccagtttggaaatcctaagattatcaaataaaaactttgattattgaagaatccaggtgtactgccacagaaaagttctattctgtagcatggactctaatatgtaatctagcccattgtgcttacagatagatgtgtgcctgtagtcatagaaaaatttgcatgagctaatgactgccttgctactagattagctcaaagcaaaaagttctctgaaagcaggtcaatagggtcatttttatattatgaagaagaaaagcagctgttgtattacattcactgtattggtcctgcttgtgtttcagggcaagatccttgttgggacaaggaatgctgaaataatcgaagttggagagaaaaatgcagcttgtaatattttagttaacggtcatgtggatgggccaatctggggactagcaacacatccttccagggattttttcctttctgctgcagaagatgggacagtgagactttgggatattgctgataaagtaagtacagataatttttttaaaagaggttacaacttctaaaaagaaaagttggaagttctaaattgctagtacttaaagaactgccagaattctgttgagcattttgaggggaaactggtataatttagaagtacttcacttaatgtttcctatgactctttttttttttttttttaaatgcagaagatgttaaacaaagtgaatttgggacatgctgctcgtactgtgtgttacagccctgaaggggacatggtggctattggaatgaaaaatggagaatttatcattttactagtgagttctctaaaaatatggggaaagaagagagacaggagatgtgcaatccatgatatcaggttagtgaacaaatggaatagagtttctagtatatacttgatttaacttccatttgtaaaattttccatagccttgccttcaaaaagaggtccccagggcctgtagcatttcccgtattataaattgtatgctaaaatatggctgtttgtatactacttaattcttcttgctaaattataaacccactgggcaccaactataatagcaagtactagtaggtaatgtttgatgaattcatgttaacacttagccatgtccattaagttcatcccaccaagaggtatctcccactgtaatacaagagagctatctgcccttcaaaagttgtcaccctggaaaactaaagttgtgatttcaaacatatcttctcttagtaacctcagtttgggaatatgtagttcattaatttaatcaatacctattgattaaatgttccagaatccaaattaatttaaatgtttcttaaacctttgtttttcagtgcttaagcatttttcaacagtggctaccatttacggagtacttccgtgtgatcagtagataagattattgaatctaggtctgtcaaaagcttgtacacttttcatcagtaaaatccttttacaaatgaaaccttcctcagaacttcaatatataaaatagtaacagtggcttcccttagcttttacatgtctctatcgtacctcagtaagactcatgggccatttcaagagactgaattgtcccatatgactccaaagattgctaggcaaatagcatttcactttgtcttttaaataagttcttcaggccgggcgcggtggctcatgcctgtaatcccagcactttgggaggccgaggcaggcagatcacctgaagtcaggagtactcgaccagcctggccaacatagtgaaaccccatctcaactaaaaatacaaaaatcagccgggcgtggtggcaggcgcctgtaatcccagctactcagggggctgaaacaggagaatcgcttgaacccgggaggcggaggttgcgccatcgcactccagcctgggagacaagagcgagacttcgtctcaaaaaaaaaaaattcttcttccaagattcaagttgtgtcatttcaccttaataactggaggttagttaagctgggctgtgttctttgcttaatattaagacaacgttttttccagatggaagaaaactatcttaatgaattgttagcttattaattatgtaatgctaatggcttttaaaagctgagatgttctgactgggtgttgtggctcacacctgtaatcccagtaccttgggaggccaagggggaaggattgcttgaggccaggagtttgggaccatagtgagaccccgcctctatttaaaaaattaaattttgttttgttttgttttgagttggagttttgctcttgttgcccatgctgaagtgcaatggtgcaatctcagctcaccacaacctgtgcctcctgggttcaagcgattctcctgcttcagcctcccgagtagatgggattacaggcgtgcaccaccatgcctggctaattttgtatttttagtagagacagggtttctctatgttggtcaggctggtctcaaactctcgacctcaggtgatctgcccgcctccgcttcccaaagttctgggattataggtgtgagccactgggcctggcctaagaaagtttttttaagccattagacgtttttaaaggaattgggagatgacaattggggaaatatttaaaatttaagtaaaatataaagcttccttatttcatgtaacccagacaatctcagtatacatgatcagttgtgtctgacaggtaaatctatttgaggccttatcacacgttacttttaagaactagaaaggaaaagtcactgatcttaagtatttataatacttcatgtggtctaatactttttacgttttgttttgattcagatttagtccggattcccggtatctggcagtaggttctagtgagaactcagtggatttttatgacctaacgctgggccccactcttaacagaatcagctactgcaaagacattccaagctttgtcattcaaatggacttctctgcagatagcagttatctccaggtacagtaccaatactgtatacccaggtggcaagttcttctgcttttacatttcgtgttagtgaatgcatttaaagttcctgagctccagagctccagcttctcaactcctccctttgtaccttctgacctacagctcccctttcctcccccacttatcagagcttttctcctattaagtttttgtagtgatcttttgcatacttaataatgttagacatgtaaatcaagtagcaatatgctagtattctgtaaaccccctgtggattttgtctctcacctaatggaattcttgtcccattttaatctgatgaaaaaggtctctagtggctgctataaacggcatgtctatgaagtgccttcaggaaaacatcttatggatcatgccgctattgacagaattacttgggctacatggactaggtaaatacttatatattcacaaggcaagaactgactttgaaggccagttagaaaatcctatttctgaactgttagagccattccaataaggaatagtaattgagtttcaagtttttgttaccatattttgaaatggtatgttcatgttgggacccctttttattgaatatatttccatgttttatcagtttccatgatttatcaagttttttttttaaggaaatcaaagttttaactttaaagataccctgatatttttcttaatgctaaatttaatgactggcaaaaaggtattgggtgctgttaagcaactgttattaattctctatctaaaggaatgctatcttgaatctattagaagtcaaagcttccaaatttgttcaaatttcctggctgtatgacaggtaaccatgactatccatttttttggccaatgaaaaatgccatcaaattcctgtatcagccaggcatatagtggctcatgcctgtaatctctgatgtagcaggccgaggtgggaggatcacttgagcctagaagttttgataccagcctgggcaacatagcaagaccccatctctgaaatttttttaattcctatgtcataagtcatttttatttttgtagagatagggatctcacaatattgcccaggctggtctcaaactcttggcctcaagcagtcctcctgcctcagcctcccaaaatgttgggattactggtatgtgctgctggacccagccaagtagcacttttaatttgaaaaatagttctatcagttttcagtcaggcgcggtggctcagcctgtaatcccagcactttgggaggccgagcgggggtgatcacctgaggtcgggagttcgagactagcctgaccaacatggagaaaccctgtctctactaaaaatacaaaataagccgggcatgttagcgcatgcctgtgatcccagctactcgggaggctgaggcaggagaattgcttgaacccaggaggcagaggttgcggtgagccgagatcatgccattgcactccagcctgggtaacaagagcgaaaactccgtctcaaaaaaaaaaaaagaaaaaatagttctatcagttttcataaagtactactttaatcttaaaaagattaatctagaaacccttcaaattataaaatgtcatttttaaaaggcaggagttgatatcctgatgaaattcaggtctccaaacaacttaccataatttacttcctgtattttaagtaacatgatagggtacttagagattaattgccaagaaactttttgaatatagtcaacctgcccgcacttgccatgatgagttttcttttgttccttccctctagtattctaggagatgaggttttgggaatctggtccagacatgctgagaaagctgatgtcaactgtgcctgtgtatctcattcaggaatcagtcttgttacaggagatgactttggcatggttaagttatttgacttcccatgtccagaaaaatttgtaagtttgtgttttgtttactattatcagtttactcctaattttgatgtcttatcatcagcacttttccccatatatttaaaatgttttgtcctaatttctaaatttttccccaaactttctaaatctatttactttgaaataaaagctattagaaacaaatcctctccctcgagtaataccatctttggaaccatcctacaaaagctgtaattagcttttcaccaaacctataatcagttatcaaatttcaaatgcttttccttagagaaaaatggtcagagtacctggagacatctgactgcccacacagcctggttttgcagatccactactcatgctgaaaagcattctaatcactggctgcggtgctaactccctactctctccacagctcttgtcatagagattatagttcctaataagagcctttgacttctgtgtgcaccaaatgccctgagcttgtctgtcattgttttttaggcaaaacacaaaaggttcttgggtcattcgccccatgtgacaaatattcgatttaccagtggtgatcgacatgttgttagtgctggaggtgatgactgcaggttagtaactttctcagcccatgaagagcagactatgttactagttaagagacttaatacaacaactcctacagctttggtttatgaaatcagctagtcaacattagtagaaggtagtataaccagatggctcttcagaatctcatatttatgcaaatacagaataaaaggagttaaagaggaaaaatattacacatgtaacctgaaagcacaactgaaaaatattaaactgttatgaaaatctaaaaacataattaactccctgcaattttcttctctgattgcagcttatttgtctggaaatgtgtacatacacctcactgagagatgctgagatgactacagaaattaactttgagaccagaattacagagaagaaaaaccaaaacccaaccctgcatggtcaagtggtgctaacccaagactgtaacagggagaaatgcccagaatcatcaaaatagtgaaagactgatctgttcaaaatatttgctatatgcactgggtataatccgtaatccatacactgccagataatgccatttcaaggaaggatcgaatacttgatggtaaaggccaagtccccctgtattgggaagtgtgtgatttcggcagacctgctgggaaaatttagggtagagcactctttacagaagaactcaaaaacccaatttggataattttcattatctttttagcaaaatggtttcttaatgtttatattttattttcaaggttcattgtttaatgaaatattttattcttgcatttccataaggaaagggaaagtcatgatcatcctaaaggatcacagtttttaaaaggcaaacattttccctaaggaaacagacacaagctttcctagagaatatgatgttttttaggcattaataaggtccttttttataaaggacacttttctcctagtagttttgaattcaggaacagatccaaagttagcagtatatggctgctacatttccattttcattttcgagccatcagtttatgttcagatgccatctctgtaatcgcacatttaaaacataactgtagcctcactaatggaaaagtagtatgatgaacaatcattcccaatggtgtacaatgtaagggttttagggagcaacagtatttaactggaagaaagaattgcatatttaatgtagtctaatatatacacatttgtttaacatgtaaacaaaagtgttaaattcacatatacaacattatacaatttaatcactcttggaataaaatttttatagccttttttctattgggaaaatttgtttagatgtgtgccactccataggtttatttccaaaatgaatgagcccaactccatttgtaaaaacttgtcagttagaattcctttttttagtggattagggctgaattcttagatccttatttcttttcactttaaatgctgccaaagatcactactcatcattcaggaattcgctgtctagcctatctgtagtttcctgaagattgaaaattatgtagactgctatttaaaaatatatttttctaagtgtgaggtttaagatgctgtattgaccctatgagtttttaatgtgttaattatctttatagcataatagatcgctttaggttcctggaatcccatttggtctgacaggatatatgaagattcttaatacctattttctgtgtctaatacttggttaatactaaaaatagaaatgactaaattacatcacagaaagcataaccagtgattgaacctggtagttttaaagctctaaatagctgtggctgaaggactgattatggggctaagaagcttgaaacgtaagttggtacttgttcatcagtggattctcctaaattaagccaaattttgaaatacatgactattaagtttctactcatgtatttacagtcagtcaataaattaaaggaggaaaaaaatccctgaacaacctgcccataaaaagaaaaatactctacatttgagcctgctgcagttttaaattttccctctgggtcaagtttgccagcttttggctacagagaaattatatttccattacagtgcaggtagaaactctgtaaccttaagcatgtaaactacatagaataaaactgtttccactgcatttctgtccttcaaagtggccaacctgattaagtcagccttaatcactgctgctgtcagtttcacgactaaaggtcatattgactaagtagtcatcagctgaccacctcgctgtatcagccagcaacgaggggaaggtgaagaaacatgataggccatatagaatctgccctatgtttacttttttaacccagataattatttttgtgtgcagtatctaagctcctgattgtgtaacctgggacttctggcaccttttgttccattcattttatgtataaaatgcatgccaaagcacactgtgccctctggtacccttgcttccaatcgccaaccatgctcatttccttcctttttttgtggtccctttttgtggtgatcattttaaaccacgtcatccaacaaatgttttatggtcaaccttagcttgttcataagccatagcaactgaaagattaaactcttaaatatgtgtctgggcagtggctattaaatagcaaaaaacaatcagattttagtattttattatttccttgtaaaatggctgaactaaattaaacccttgtttcccatttgttctataatttatagtgaaactgagaacaaaactatctttataaatgatagctaaaagtatttccagatatttaaacaatttaaaataaatttcttctgcagagatgcaaagcatctcaacactggaatgaacaaatgccttaaattcaatggagtaaacctttagaatgaagaggaactgtcatttcacccaagccgaagacaacagccttatgcacttgtgtgctctgtctttgctgcttctcgtgtttcaagcctttcctgtgggatcagcacagcaaagtgcaacttaccaaatggtttaatgactggttaattctttcttctcccaatggaaaagcaatggcaacacaacagtagactgctggcttgacaatcttaaacgtgagcctttgcacatgtaggtttatcatcatttgagtatacgactaagcaagtcaatgaactttttttttttttttagcagtttaatttggtcctgagaatgttgcagtctttattaccccttttgcattaatccacttttctaaccaccttttaagctttaatttttaacactatacaccaagtctttgaaatcagtgatctgttatttaactctaaagcatttgacacttcttgccttaacagttttaaaaaccacacacaaaaaaactctgtaagtaatacagtaggccaaaagtttcatcctatctatcttgcagtttacctatctgatctgatctctgtaattatagttctgtcatttaaaatatactatttaaatctaatttttacatttcaaaaattatcttcagtagtaactaagtatattttctgtggattctgagaatgttatttttcagaatgtgagaatatatatgtacatttataatcttgtgactttaaagtctgttttcagatacagtatgtaaatacttgtaaaaaaatttgtataattttgtgataatgtagtttcccaaaaaaattatttagaaggcattatgttattagtaaatgagagcactgtatagaactgttcctattttctgcacttgccattccagctgcctccactgtccatacccacctcattcatcctgtcacagaaggcaggaaaactgggaactttaccaaagtagcactcagcctgagaggcctgtataatcatgcttttcaaactaaattcacttaaaaattaaaaagcagaattgaatattttaagcagcctcagtacctttggccaatgctgttttcatggtggattatgaacattatataatctttgggaaaagtgaaagtagtacaatttttagaataatgacaactgcctcactgcatctctccactcacacagcaaccgtgtagccccctaagctgcagtaccatgactaaccatgatgtcaatttcatatgctgatcctcacaacagcagtgcacaaacatgccccaaatattttaacagaatttagctcttccttaagctgtcttttcatagtaaaaacaaaacaaaaacacccaatgttaaaaccacataataaacttacaaacttgaaaaattagacacttcagatagataggcaataaaacttcatattatgaaagcaatatattccaagtttcaaagatttgacaagttctgtagagtatctttcatcagtacatgaaaacttccaaactgcatgatcttctgccaggcaggactgggtgctattcgctggtttgaggtcgaatccatttcaaggcatgtcgtggtgggacattaatggtgggatggtagaatgtgcagtccggtcttgtacattgagtgttaaacctacaatgttttggatgatagaagggacattccatcttcttacaagcagggaagtaacggcagagctgactactggaaggtggtgctggtggtgcaactgctggttttggagacagtactggaattcttctactcacatgagtgaagggacaatctggtttagtacactttgcatcatatttacaatttgggtgaacaaacaaacatttttcagcaaatttacaattggggaaggctttgcagggtgagatggggtgatggtaggcacactcatccccatttttacaagcaggccagtacttgcagcgctccaaaagtttttctggtttctgtgccacactcagttcactcatctcagcatttgggtcctcaagctgcctgctcagcaagtgcaactgctgtgggtggaggagacctctgagtcccttgtttgaggctgcagtttggtttacgggtttcattccttcaaagcacatgtcctcctcttgatctgacatgtatcctggggggctggggacaccatccagcgtcactataaacttgggacttgcaggtttatctggttgtacaagatctcgtgtctgcataaggtgtcctgaaagtacccgaagggaatctgcagtcttcatccccgactcttggtttggtgccactactacttcctcagacagctttggcttcttcagaataaatgatcttgtgtctgcatggaccatggattccatgtcatagtaatcttgactcatctgcagagtttctgccattactgggtcgatttgcagtcgggataataattgcctctgttgagttccttgatttttttctacagaatctccttttgtttcctcttctttaatggggggacttattctgggggtcctactttgtccctggaccacttctgctagcaattcttcttgagaagttcgagttctgggagcaactggaagtgtctgtttctgtggaactgtagagtagttagttgtttttgttacggattcttgagcttcagatatagccttcaaaatcagattcttgttagcttgtttagaaggtggaagagaaggtctcctttcaggctttgcaggcacagacacactgctggagatgcttcctgttcgagacccgtaatcatcatcttcttcctcctcttctccatcatgattgaatttttttactttaacaactgaacttaccacaggcaactttctcttccgaaagttttcatcctccatactcattttctccgagttgtttctaaagaacggactatacgtttcttctaagctgttaagcacctctggttcacacaaacgtcctgtttcatatacccaactactctgcatatcaagctgcttggcagcatgaatactattctgctgctgttgaaattgcaacctgtttaaatgaacaccactatctgcatttctacttgcaggtggtcgataaatttcaatagaagggcgagaagaaccatatgtaagtgtcactgtaggttttttctgagataagggattctcctgcacaaagttgaggtcttcgtcaatgagatcatctggttctggcttaatatcaatcacatcttcagagggtgctggctccctcaaaggtttcactgttgacattagtcgggttgcagctccatcatcgtaagtctgtctgacatttgtggtttttgactcctgcgaacttgtagaaactctggaatctcttttttcaggtctcgcgctaggaatggcaagtggtggcactgcagcttcatgcctcctctcatctccccgactgaaattgctcttgtttgaaggcacgttactatcaaagatgttggtatcagaagacttcagactagagggttcagttgtaacagagcgaagtttatctaatacaccatgaagccatacggtgaatcgaattgtgttgttccctagaaacagggacagatcctctgtcatttggtcctgacttttcttgttggccaccatcaccataatgtaatcaggaagttcttcatcaacataagctcctaattcttgtaatttccccttaatggcactccggatcttgcggctgatctcggtgccgatctccatggctctgcggcgtgcgggaactcagcactgcgcggcgcttggcttacccggaggctgccgcggactcctaccccgcagccgggacaccaccgcctcc

SEQ ID NO: 13606 - RNA, 16841 nt, Homo sapiens
  source 1..16841: mol_type = other RNA
gctgggattacaggcatgagccaccataataaggattctgatgaacatttgattccttggactactgttatactcaaaagccttccttaatcttctaattgtcaccctaaatatcctaaaatttctgtcttcctagtagttcttcatagtcctaaaaatttgtcagagagaaaggtaaatcaagaaacatgattttcaaatgatttaaggtggtactagggtttaggatttcctttgctttttatcatttaacacactgcttatcatacagctggaagtgctctgggccagtgtctctacttcgagggaagaaggaggtagtgagacagaaggaaatagcacaattcctggccctgacagaagggtgttcaggagacctgctctcctctcactttattccatctcatctggacctgtggcttccaatccacatctctttcctttaatatcctgcattggctaggctgtataaatcctttggtgcatcgaaaaactaagtgcattttttgtttttgtgattatgcaatacttataggaaaagttataattttagaatatttaagtacacttacatttttgagaaaaagactattgaaatgtttgtgccatgtcaaatttcagttgaacattttgggtattcttaatataagaccaggccaggcaccgtggctcaggccgggcacagtggctcacacctataatcccagcacttagggaggccaaggcgggaagatcacctgaagtcaggagttcaagaccagcctggctaacaaggtgaaactctgtctctactaaaaatacaaaaattagccgggcgtggtggctggcgcttgtaatcccagctacttgggaggctgagacaggagaatcacttgaacctgggaagcagaggttgtggtgagctgagatcgcaccattgcactccagcctgggcaacaaagagcgaaactccgtctcaaaaaaataaaaaataaaccctagaattatagtatgttagaattggaagggaagaattgtctaaggttattctagctaataagcaacagacttggaaaggaaaaggtcctgacaaagctaagcctcccgttcaggtttcctgactcgtgaattcagtgctgctgccactacacgatgcatgctctttgtatcaagggtgagacagcattacacatacatagaaaattatctatttaaactctatttgaacttttgatgagtttgtctccccctcccccactccttttcagaataacttgacgtttacaggtaccatcagtggtgatgtctgtgtgtggaaagatcacatattgtgtagaatcgtggcgagagctcacaacgggcctgtgtttgccatgtacaccaccctgcgagatggacttatcgtgactgggggaaaggaaaggccgtgagtcctctttcttttcacagaatatttatgcatttgtgacctacctgaggtttgcagttaattattctagttgtttctaggctacacagagtgtcctctccgaccttcctcctcatatgcttctcctttattaccttttatgtgccttctatttgattctcatttctggtcttaattcacttccaatttttttcatgttggggtgatactttttctgaggtgtggataggtagttgtcctacaagttgagttacttttcttaatgtctgtatgcctgtgtatgatttgctgagtaggaggcccatgggggaatctggagccagggttgtattttgactgcctgctctctttttgttcagaatggattctaaggagtagaatgcacattgttgctttagaaaaggatgagggaactagagagaactgccttgtttccttttgcttgaggcaaatttaaactgttttatacaagacctcaaaatttgagaagaggtctcttctgagtgattttcaaatctcccaacagtaaccagatacttatgatttgatttgtcaccaacatagtcatatgcatgttgaaacatgacatgtaggccaggcacagtggctcacacctgtaatcttatcactttgggaggctgaggcaggtggatcgcttgagcccaggagttcaagaccagcctgggcaacatggtgaaaccccatcgctataaaaaacaacaattagccgggtgtggtggcacatgcctgtagtccctgctactcaggaggctgaggtgggaggatcacttgagcctggggaggtcaaggctttagtgagctgtgatggtgccactgcactccagcctgggtgacagagtgagaccccatttaaaaaacaaaaacaaaaacaaaaaaaaatgtgacatatagttgactaagaagtacatttcaatacaggattgaaagaacccacatatgttaattaaacacaagcgcagaatttgtgccttttacataaaggaagaatgcacataggcatgctttcagacaagcaattcatctagcagaaaaggaaggaatacatttttcagcccttccaggaataaaatccataaatgggctctatttcgtcctccaacacttgtatttcccacgtcatttactcctgcacacccccactcactagaagcctgctaaactgttccagtgagatattttaacacctgatagggaataaatatgcttctgttttggccttcaaaaataagctctgggccagttgcagtggctcacgcctgtaatcccaacactttgggaggccgaggtgggcggatcacgaggtcaggagtttgggatcagcctggccaatatggtgaaactccatctctactaaaaatacaaaaattagccaggcatggtgcctgtaatcccagctacttgggaggctgaaggagaagaatcgcttgaacctgggaggcacaggttgcagtgagccgagatcacaccactgcactccaggccaggtgacagagcgacactctgtctcaaaaaaataaataaatcaactctgtagcatagcatttgtaattctattattttgccttacatttccattatccttttaataaaattgtttttttacatcttcctaatcaagaagtattatgaggccaggcacagtggctcatacctggaatcccagcactttgggaggccgaggcaggcagatcacctgaggtcaaggtatttgagaccagcctggccaacatggtgaaaccccatctctactaaaaatacagaaattagctgggtgtggtggtgcacacctgtaatgctagctactcgggaggctgaggtaggagaatcgcttgaacctgggaggcagaggttgcaataagcctagatcatgccactgcactcaagcctgggagacagagcgagactacatcttaaaaaaaaaaaaaaaagtattatgagagaggataatgtattgtaatgtattgtagaggctaaataaaattatgctcatgtcagaaaaaaagagtatttctcaaaataaaattcactgaaactggatgtttattttgactgagatatagtatatcctcaaattgccatagaaagtttacaagaatattagaggtaaattataaatatcagggcctttttaaaaaaaaaagattctgcttataacttggtatttgtttataataaaaattatagtagccaataatgaacacttactctggcttggttatttacttaggtcaaaagaaggaggagcggttaaactgtgggatcaggaactgaggcggtgccgtgccttcaggcttgagacaggacaagccacagattgtgttcgttctgtgtgcagaggcaaagtaagatgttccatgagctgatacagtgcagcagaaaacagaaagtggttattactgtgattccctcaccctttgcagcctaatgaacaatacttaataatgcataacgatggatttgcttgccaacattactctgtctttgctgctttctttgccaaagttagcaccagtgtggtgcataagctaggaagctattctgtctaaatactgtatgtaaacctccaatattttctagaatctgccaatttaacaactctagtagacataattgaaagcccttggcagttgactcatattaggacagctgtctccattttttaaaaaaacacacattccctagataaaacgtgcagtaaacaaacaatgaaatactactcagccataaaaaataatgaaattctgtcattcttggtggcaacatggatgagactggaggacatgatgtgaagtgaaataagccaggcacagaaagataaatacatgttctcactcctgtgcagaaactaaaaaagttgatcccacagaggtggagagtagaatagtggttactggaggcggacaagggggagggggagggggatagggaaggactggttaaaggatacaagtttacacagccagataggaatagtatgttttagtattctgtagtactgtaggatgactatagttaagaatcacgtatttatgtattttcaggtatttacaagagaggattttgaaagtttccatcacaaagaaatgataaatgtctgaggtgatggttatgcgtattaccctatgccctatagatatgtataattatgtgtcaatttcaaaataaaaattcaaaactacaactcctatgaaaatttttgagcgtgtttgtacttattaagtgtatttataaatcatacggatattatcttcagcctgcatattaaattgtagttaagcttttactttttaactaaaaaataaattctattattttttcctatatcccactgcactgaccccagtttggaaatcctaagattatcaaataaaaactttgattattgaagaatccaggtgtactgccacagaaaagttctattctgtagcatggactctaatatgtaatctagcccattgtgcttacagatagatgtgtgcctgtagtcatagaaaaatttgcatgagctaatgactgccttgctactagattagctcaaagcaaaaagttctctgaaagcaggtcaatagggtcatttttatattatgaagaagaaaagcagctgttgtattacattcactgtattggtcctgcttgtgtttcagggcaagatccttgttgggacaaggaatgctgaaataatcgaagttggagagaaaaatgcagcttgtaatattttagttaacggtcatgtggatgggccaatctggggactagcaacacatccttccagggattttttcctttctgctgcagaagatgggacagtgagactttgggatattgctgataaagtaagtacagataatttttttaaaagaggttacaacttctaaaaagaaaagttggaagttctaaattgctagtacttaaagaactgccagaattctgttgagcattttgaggggaaactggtataatttagaagtacttcacttaatgtttcctatgactctttttttttttttttttaaatgcagaagatgttaaacaaagtgaatttgggacatgctgctcgtactgtgtgttacagccctgaaggggacatggtggctattggaatgaaaaatggagaatttatcattttactagtgagttctctaaaaatatggggaaagaagagagacaggagatgtgcaatccatgatatcaggttagtgaacaaatggaatagagtttctagtatatacttgatttaacttccatttgtaaaattttccatagccttgccttcaaaaagaggtccccagggcctgtagcatttcccgtattataaattgtatgctaaaatatggctgtttgtatactacttaattcttcttgctaaattataaacccactgggcaccaactataatagcaagtactagtaggtaatgtttgatgaattcatgttaacacttagccatgtccattaagttcatcccaccaagaggtatctcccactgtaatacaagagagctatctgcccttcaaaagttgtcaccctggaaaactaaagttgtgatttcaaacatatcttctcttagtaacctcagtttgggaatatgtagttcattaatttaatcaatacctattgattaaatgttccagaatccaaattaatttaaatgtttcttaaacctttgtttttcagtgcttaagcatttttcaacagtggctaccatttacggagtacttccgtgtgatcagtagataagattattgaatctaggtctgtcaaaagcttgtacacttttcatcagtaaaatccttttacaaatgaaaccttcctcagaacttcaatatataaaatagtaacagtggcttcccttagcttttacatgtctctatcgtacctcagtaagactcatgggccatttcaagagactgaattgtcccatatgactccaaagattgctaggcaaatagcatttcactttgtcttttaaataagttcttcaggccgggcgcggtggctcatgcctgtaatcccagcactttgggaggccgaggcaggcagatcacctgaagtcaggagtactcgaccagcctggccaacatagtgaaaccccatctcaactaaaaatacaaaaatcagccgggcgtggtggcaggcgcctgtaatcccagctactcagggggctgaaacaggagaatcgcttgaacccgggaggcggaggttgcgccatcgcactccagcctgggagacaagagcgagacttcgtctcaaaaaaaaaaaattcttcttccaagattcaagttgtgtcatttcaccttaataactggaggttagttaagctgggctgtgttctttgcttaatattaagacaacgttttttccagatggaagaaaactatcttaatgaattgttagcttattaattatgtaatgctaatggcttttaaaagctgagatgttctgactgggtgttgtggctcacacctgtaatcccagtaccttgggaggccaagggggaaggattgcttgaggccaggagtttgggaccatagtgagaccccgcctctatttaaaaaattaaattttgttttgttttgttttgagttggagttttgctcttgttgcccatgctgaagtgcaatggtgcaatctcagctcaccacaacctgtgcctcctgggttcaagcgattctcctgcttcagcctcccgagtagatgggattacaggcgtgcaccaccatgcctggctaattttgtatttttagtagagacagggtttctctatgttggtcaggctggtctcaaactctcgacctcaggtgatctgcccgcctccgcttcccaaagttctgggattataggtgtgagccactgggcctggcctaagaaagtttttttaagccattagacgtttttaaaggaattgggagatgacaattggggaaatatttaaaatttaagtaaaatataaagcttccttatttcatgtaacccagacaatctcagtatacatgatcagttgtgtctgacaggtaaatctatttgaggccttatcacacgttacttttaagaactagaaaggaaaagtcactgatcttaagtatttataatacttcatgtggtctaatactttttacgttttgttttgattcagatttagtccggattcccggtatctggcagtaggttctagtgagaactcagtggatttttatgacctaacgctgggccccactcttaacagaatcagctactgcaaagacattccaagctttgtcattcaaatggacttctctgcagatagcagttatctccaggtacagtaccaatactgtatacccaggtggcaagttcttctgcttttacatttcgtgttagtgaatgcatttaaagttcctgagctccagagctccagcttctcaactcctccctttgtaccttctgacctacagctcccctttcctcccccacttatcagagcttttctcctattaagtttttgtagtgatcttttgcatacttaataatgttagacatgtaaatcaagtagcaatatgctagtattctgtaaaccccctgtggattttgtctctcacctaatggaattcttgtcccattttaatctgatgaaaaaggtctctagtggctgctataaacggcatgtctatgaagtgccttcaggaaaacatcttatggatcatgccgctattgacagaattacttgggctacatggactaggtaaatacttatatattcacaaggcaagaactgactttgaaggccagttagaaaatcctatttctgaactgttagagccattccaataaggaatagtaattgagtttcaagtttttgttaccatattttgaaatggtatgttcatgttgggacccctttttattgaatatatttccatgttttatcagtttccatgatttatcaagttttttttttaaggaaatcaaagttttaactttaaagataccctgatatttttcttaatgctaaatttaatgactggcaaaaaggtattgggtgctgttaagcaactgttattaattctctatctaaaggaatgctatcttgaatctattagaagtcaaagcttccaaatttgttcaaatttcctggctgtatgacaggtaaccatgactatccatttttttggccaatgaaaaatgccatcaaattcctgtatcagccaggcatatagtggctcatgcctgtaatctctgatgtagcaggccgaggtgggaggatcacttgagcctagaagttttgataccagcctgggcaacatagcaagaccccatctctgaaatttttttaattcctatgtcataagtcatttttatttttgtagagatagggatctcacaatattgcccaggctggtctcaaactcttggcctcaagcagtcctcctgcctcagcctcccaaaatgttgggattactggtatgtgctgctggacccagccaagtagcacttttaatttgaaaaatagttctatcagttttcagtcaggcgcggtggctcagcctgtaatcccagcactttgggaggccgagcgggggtgatcacctgaggtcgggagttcgagactagcctgaccaacatggagaaaccctgtctctactaaaaatacaaaataagccgggcatgttagcgcatgcctgtgatcccagctactcgggaggctgaggcaggagaattgcttgaacccaggaggcagaggttgcggtgagccgagatcatgccattgcactccagcctgggtaacaagagcgaaaactccgtctcaaaaaaaaaaaaagaaaaaatagttctatcagttttcataaagtactactttaatcttaaaaagattaatctagaaacccttcaaattataaaatgtcatttttaaaaggcaggagttgatatcctgatgaaattcaggtctccaaacaacttaccataatttacttcctgtattttaagtaacatgatagggtacttagagattaattgccaagaaactttttgaatatagtcaacctgcccgcacttgccatgatgagttttcttttgttccttccctctagtattctaggagatgaggttttgggaatctggtccagacatgctgagaaagctgatgtcaactgtgcctgtgtatctcattcaggaatcagtcttgttacaggagatgactttggcatggttaagttatttgacttcccatgtccagaaaaatttgtaagtttgtgttttgtttactattatcagtttactcctaattttgatgtcttatcatcagcacttttccccatatatttaaaatgttttgtcctaatttctaaatttttccccaaactttctaaatctatttactttgaaataaaagctattagaaacaaatcctctccctcgagtaataccatctttggaaccatcctacaaaagctgtaattagcttttcaccaaacctataatcagttatcaaatttcaaatgcttttccttagagaaaaatggtcagagtacctggagacatctgactgcccacacagcctggttttgcagatccactactcatgctgaaaagcattctaatcactggctgcggtgctaactccctactctctccacagctcttgtcatagagattatagttcctaataagagcctttgacttctgtgtgcaccaaatgccctgagcttgtctgtcattgttttttaggcaaaacacaaaaggttcttgggtcattcgccccatgtgacaaatattcgatttaccagtggtgatcgacatgttgttagtgctggaggtgatgactgcaggttagtaactttctcagcccatgaagagcagactatgttactagttaagagacttaatacaacaactcctacagctttggtttatgaaatcagctagtcaacattagtagaaggtagtataaccagatggctcttcagaatctcatatttatgcaaatacagaataaaaggagttaaagaggaaaaatattacacatgtaacctgaaagcacaactgaaaaatattaaactgttatgaaaatctaaaaacataattaactccctgcaattttcttctctgattgcagcttatttgtctggaaatgtgtacatacacctcactgagagatgctgagatgactacagaaattaactttgagaccagaattacagagaagaaaaaccaaaacccaaccctgcatggtcaagtggtgctaacccaagactgtaacagggagaaatgcccagaatcatcaaaatagtgaaagactgatctgttcaaaatatttgctatatgcactgggtataatccgtaatccatacactgccagataatgccatttcaaggaaggatcgaatacttgatggtaaaggccaagtccccctgtattgggaagtgtgtgatttcggcagacctgctgggaaaatttagggtagagcactctttacagaagaactcaaaaacccaatttggataattttcattatctttttagcaaaatggtttcttaatgtttatattttattttcaaggttcattgtttaatgaaatattttattcttgcatttccataaggaaagggaaagtcatgatcatcctaaaggatcacagtttttaaaaggcaaacattttccctaaggaaacagacacaagctttcctagagaatatgatgttttttaggcattaataaggtccttttttataaaggacacttttctcctagtagttttgaattcaggaacagatccaaagttagcagtatatggctgctacatttccattttcattttcgagccatcagtttatgttcagatgccatctctgtaatcgcacatttaaaacataactgtagcctcactaatggaaaagtagtatgatgaacaatcattcccaatggtgtacaatgtaagggttttagggagcaacagtatttaactggaagaaagaattgcatatttaatgtagtctaatatatacacatttgtttaacatgtaaacaaaagtgttaaattcacatatacaacattatacaatttaatcactcttggaataaaatttttatagccttttttctattgggaaaatttgtttagatgtgtgccactccataggtttatttccaaaatgaatgagcccaactccatttgtaaaaacttgtcagttagaattcctttttttagtggattagggctgaattcttagatccttatttcttttcactttaaatgctgccaaagatcactactcatcattcaggaattcgctgtctagcctatctgtagtttcctgaagattgaaaattatgtagactgctatttaaaaatatatttttctaagtgtgaggtttaagatgctgtattgaccctatgagtttttaatgtgttaattatctttatagcataatagatcgctttaggttcctggaatcccatttggtctgacaggatatatgaagattcttaatacctattttctgtgtctaatacttggttaatactaaaaatagaaatgactaaattacatcacagaaagcataaccagtgattgaacctggtagttttaaagctctaaatagctgtggctgaaggactgattatggggctaagaagcttgaaacgtaagttggtacttgttcatcagtggattctcctaaattaagccaaattttgaaatacatgactattaagtttctactcatgtatttacagtcagtcaataaattaaaggaggaaaaaaatccctgaacaacctgcccataaaaagaaaaatactctacatttgagcctgctgcagttttaaattttccctctgggtcaagtttgccagcttttggctacagagaaattatatttccattacagtgcaggtagaaactctgtaaccttaagcatgtaaactacatagaataaaactgtttccactgcatttctgtccttcaaagtggccaacctgattaagtcagccttaatcactgctgctgtcagtttcacgactaaaggtcatattgactaagtagtcatcagctgaccacctcgctgtatcagccagcaacgaggggaaggtgaagaaacatgataggccatatagaatctgccctatgtttacttttttaacccagataattatttttgtgtgcagtatctaagctcctgattgtgtaacctgggacttctggcaccttttgttccattcattttatgtataaaatgcatgccaaagcacactgtgccctctggtacccttgcttccaatcgccaaccatgctcatttccttcctttttttgtggtccctttttgtggtgatcattttaaaccacgtcatccaacaaatgttttatggtcaaccttagcttgttcataagccatagcaactgaaagattaaactcttaaatatgtgtctgggcagtggctattaaatagcaaaaaacaatcagattttagtattttattatttccttgtaaaatggctgaactaaattaaacccttgtttcccatttgttctataatttatagtgaaactgagaacaaaactatctttataaatgatagctaaaagtatttccagatatttaaacaatttaaaataaatttcttctgcagagatgcaaagcatctcaacactggaatgaacaaatgccttaaattcaatggagtaaacctttagaatgaagaggaactgtcatttcacccaagccgaagacaacagccttatgcacttgtgtgctctgtctttgctgcttctcgtgtttcaagcctttcctgtgggatcagcacagcaaagtgcaacttaccaaatggtttaatgactggttaattctttcttctcccaatggaaaagcaatggcaacacaacagtagactgctggcttgacaatcttaaacgtgagcctttgcacatgtaggtttatcatcatttgagtatacgactaagcaagtcaatgaactttttttttttttttagcagtttaatttggtcctgagaatgttgcagtctttattaccccttttgcattaatccacttttctaaccaccttttaagctttaatttttaacactatacaccaagtctttgaaatcagtgatctgttatttaactctaaagcatttgacacttcttgccttaacagttttaaaaaccacacacaaaaaaactctgtaagtaatacagtaggccaaaagtttcatcctatctatcttgcagtttacctatctgatctgatctctgtaattatagttctgtcatttaaaatatactatttaaatctaatttttacatttcaaaaattatcttcagtagtaactaagtatattttctgtggattctgagaatgttatttttcagaatgtgagaatatatatgtacatttataatcttgtgactttaaagtctgttttcagatacagtatgtaaatacttgtaaaaaaatttgtataattttgtgataatgtagtttcccaaaaaaattatttagaaggcattatgttattagtaaatgagagcactgtatagaactgttcctattttctgcacttgccattccagctgcctccactgtccatacccacctcattcatcctgtcacagaaggcaggaaaactgggaactttaccaaagtagcactcagcctgagaggcctgtataatcatgcttttcaaactaaattcacttaaaaattaaaaagcagaattgaatattttaagcagcctcagtacctttggccaatgctgttttcatggtggattatgaacattatataatctttgggaaaagtgaaagtagtacaatttttagaataatgacaactgcctcactgcatctctccactcacacagcaaccgtgtagccccctaagctgcagtaccatgactaaccatgatgtcaatttcatatgctgatcctcacaacagcagtgcacaaacatgccccaaatattttaacagaatttagctcttccttaagctgtcttttcatagtaaaaacaaaacaaaaacacccaatgttaaaaccacataataaacttacaaacttgaaaaattagacacttcagatagataggcaataaaacttcatattatgaaagcaatatattccaagtttcaaagatttgacaagttctgtagagtatctttcatcagtacatgaaaacttccaaactgcatgatcttctgccaggcaggactgggtgctattcgctggtttgaggtcgaatccatttcaaggcatgtcgtggtgggacattaatggtgggatggtagaatgtgcagtccggtcttgtacattgagtgttaaacctacaatgttttggatgatagaagggacattccatcttcttacaagcagggaagtaacggcagagctgactactggaaggtggtgctggtggtgcaactgctggttttggagacagtactggaattcttctactcacatgagtgaagggacaatctggtttagtacactttgcatcatatttacaatttgggtgaacaaacaaacatttttcagcaaatttacaattggggaaggctttgcagggtgagatggggtgatggtaggcacactcatccccatttttacaagcaggccagtacttgcagcgctccaaaagtttttctggtttctgtgccacactcagttcactcatctcagcatttgggtcctcaagctgcctgctcagcaagtgcaactgctgtgggtggaggagacctctgagtcccttgtttgaggctgcagtttggtttacgggtttcattccttcaaagcacatgtcctcctcttgatctgacatgtatcctggggggctggggacaccatccagcgtcactataaacttgggacttgcaggtttatctggttgtacaagatctcgtgtctgcataaggtgtcctgaaagtacccgaagggaatctgcagtcttcatccccgactcttggtttggtgccactactacttcctcagacagctttggcttcttcagaataaatgatcttgtgtctgcatggaccatggattccatgtcatagtaatcttgatttttttctacagaatctccttttgtttcctcttctttaatggggggacttattctgggggtcctactttgtccctggaccacttctgctagcaattcttcttgagaagttcgagttctgggagcaactggaagtgtctgtttctgtggaactgtagagtagttagttgtttttgttacggattcttgagcttcagatatagccttcaaaatcagattcttgttagcttgtttagaaggtggaagagaaggtctcctttcaggctttgcaggcacagacacactgctggagatgcttcctgttcgagacccgtaatcatcatcttcttcctcctcttctccatcatgattgaatttttttactttaacaactgaacttaccacaggcaactttctcttccgaaagttttcatcctccatactcattttctccgagttgtttctaaagaacggactatacgtttcttctaagctgttaagcacctctggttcacacaaacgtcctgtttcatatacccaactactctgcatatcaagctgcttggcagcatgaatactattctgctgctgttgaaattgcaacctgtttaaatgaacaccactatctgcatttctacttgcaggtggtcgataaatttcaatagaagggcgagaagaaccatatgtaagtgtcactgtaggttttttctgagataagggattctcctgcacaaagttgaggtcttcgtcaatgagatcatctggttctggcttaatatcaatcacatcttcagagggtgctggctccctcaaaggtttcactgttgacattagtcgggttgcagctccatcatcgtaagtctgtctgacatttgtggtttttgactcctgcgaacttgtagaaactctggaatctcttttttcaggtctcgcgctaggaatggcaagtggtggcactgcagcttcatgcctcctctcatctccccgactgaaattgctcttgtttgaaggcacgttactatcaaagatgttggtatcagaagacttcagactagagggttcagttgtaacagagcgaagtttatctaatacaccatgaagccatacggtgaatcgaattgtgttgttccctagaaacagggacagatcctctgtcatttggtcctgacttttcttgttggccaccatcaccataatgtaatcaggaagttcttcatcaacataagctcctaattcttgtaatttccccttaatggcactccggatcttgcggctgatctcggtgccgatctccatggctctgcggcgtgcgggaactcagcactgcgcggcgcttggcttacccggaggctgccgcggactcctaccccgcagccgggacaccaccgcctcc

SEQ ID NO: 13607 - RNA, 16816 nt, Homo sapiens
  source 1..16816: mol_type = other RNA
gctgggattacaggcatgagccaccataataaggattctgatgaacatttgattccttggactactgttatactcaaaagccttccttaatcttctaattgtcaccctaaatatcctaaaatttctgtcttcctagtagttcttcatagtcctaaaaatttgtcagagagaaaggtaaatcaagaaacatgattttcaaatgatttaaggtggtactagggtttaggatttcctttgctttttatcatttaacacactgcttatcatacagctggaagtgctctgggccagtgtctctacttcgagggaagaaggaggtagtgagacagaaggaaatagcacaattcctggccctgacagaagggtgttcaggagacctgctctcctctcactttattccatctcatctggacctgtggcttccaatccacatctctttcctttaatatcctgcattggctaggctgtataaatcctttggtgcatcgaaaaactaagtgcattttttgtttttgtgattatgcaatacttataggaaaagttataattttagaatatttaagtacacttacatttttgagaaaaagactattgaaatgtttgtgccatgtcaaatttcagttgaacattttgggtattcttaatataagaccaggccaggcaccgtggctcaggccgggcacagtggctcacacctataatcccagcacttagggaggccaaggcgggaagatcacctgaagtcaggagttcaagaccagcctggctaacaaggtgaaactctgtctctactaaaaatacaaaaattagccgggcgtggtggctggcgcttgtaatcccagctacttgggaggctgagacaggagaatcacttgaacctgggaagcagaggttgtggtgagctgagatcgcaccattgcactccagcctgggcaacaaagagcgaaactccgtctcaaaaaaataaaaaataaaccctagaattatagtatgttagaattggaagggaagaattgtctaaggttattctagctaataagcaacagacttggaaaggaaaaggtcctgacaaagctaagcctcccgttcaggtttcctgactcgtgaattcagtgctgctgccactacacgatgcatgctctttgtatcaagggtgagacagcattacacatacatagaaaattatctatttaaactctatttgaacttttgatgagtttgtctccccctcccccactccttttcagaataacttgacgtttacaggtaccatcagtggtgatgtctgtgtgtggaaagatcacatattgtgtagaatcgtggcgagagctcacaacgggcctgtgtttgccatgtacaccaccctgcgagatggacttatcgtgactgggggaaaggaaaggccgtgagtcctctttcttttcacagaatatttatgcatttgtgacctacctgaggtttgcagttaattattctagttgtttctaggctacacagagtgtcctctccgaccttcctcctcatatgcttctcctttattaccttttatgtgccttctatttgattctcatttctggtcttaattcacttccaatttttttcatgttggggtgatactttttctgaggtgtggataggtagttgtcctacaagttgagttacttttcttaatgtctgtatgcctgtgtatgatttgctgagtaggaggcccatgggggaatctggagccagggttgtattttgactgcctgctctctttttgttcagaatggattctaaggagtagaatgcacattgttgctttagaaaaggatgagggaactagagagaactgccttgtttccttttgcttgaggcaaatttaaactgttttatacaagacctcaaaatttgagaagaggtctcttctgagtgattttcaaatctcccaacagtaaccagatacttatgatttgatttgtcaccaacatagtcatatgcatgttgaaacatgacatgtaggccaggcacagtggctcacacctgtaatcttatcactttgggaggctgaggcaggtggatcgcttgagcccaggagttcaagaccagcctgggcaacatggtgaaaccccatcgctataaaaaacaacaattagccgggtgtggtggcacatgcctgtagtccctgctactcaggaggctgaggtgggaggatcacttgagcctggggaggtcaaggctttagtgagctgtgatggtgccactgcactccagcctgggtgacagagtgagaccccatttaaaaaacaaaaacaaaaacaaaaaaaaatgtgacatatagttgactaagaagtacatttcaatacaggattgaaagaacccacatatgttaattaaacacaagcgcagaatttgtgccttttacataaaggaagaatgcacataggcatgctttcagacaagcaattcatctagcagaaaaggaaggaatacatttttcagcccttccaggaataaaatccataaatgggctctatttcgtcctccaacacttgtatttcccacgtcatttactcctgcacacccccactcactagaagcctgctaaactgttccagtgagatattttaacacctgatagggaataaatatgcttctgttttggccttcaaaaataagctctgggccagttgcagtggctcacgcctgtaatcccaacactttgggaggccgaggtgggcggatcacgaggtcaggagtttgggatcagcctggccaatatggtgaaactccatctctactaaaaatacaaaaattagccaggcatggtgcctgtaatcccagctacttgggaggctgaaggagaagaatcgcttgaacctgggaggcacaggttgcagtgagccgagatcacaccactgcactccaggccaggtgacagagcgacactctgtctcaaaaaaataaataaatcaactctgtagcatagcatttgtaattctattattttgccttacatttccattatccttttaataaaattgtttttttacatcttcctaatcaagaagtattatgaggccaggcacagtggctcatacctggaatcccagcactttgggaggccgaggcaggcagatcacctgaggtcaaggtatttgagaccagcctggccaacatggtgaaaccccatctctactaaaaatacagaaattagctgggtgtggtggtgcacacctgtaatgctagctactcgggaggctgaggtaggagaatcgcttgaacctgggaggcagaggttgcaataagcctagatcatgccactgcactcaagcctgggagacagagcgagactacatcttaaaaaaaaaaaaaaaagtattatgagagaggataatgtattgtaatgtattgtagaggctaaataaaattatgctcatgtcagaaaaaaagagtatttctcaaaataaaattcactgaaactggatgtttattttgactgagatatagtatatcctcaaattgccatagaaagtttacaagaatattagaggtaaattataaatatcagggcctttttaaaaaaaaaagattctgcttataacttggtatttgtttataataaaaattatagtagccaataatgaacacttactctggcttggttatttacttaggtcaaaagaaggaggagcggttaaactgtgggatcaggaactgaggcggtgccgtgccttcaggcttgagacaggacaagccacagattgtgttcgttctgtgtgcagaggcaaagtaagatgttccatgagctgatacagtgcagcagaaaacagaaagtggttattactgtgattccctcaccctttgcagcctaatgaacaatacttaataatgcataacgatggatttgcttgccaacattactctgtctttgctgctttctttgccaaagttagcaccagtgtggtgcataagctaggaagctattctgtctaaatactgtatgtaaacctccaatattttctagaatctgccaatttaacaactctagtagacataattgaaagcccttggcagttgactcatattaggacagctgtctccattttttaaaaaaacacacattccctagataaaacgtgcagtaaacaaacaatgaaatactactcagccataaaaaataatgaaattctgtcattcttggtggcaacatggatgagactggaggacatgatgtgaagtgaaataagccaggcacagaaagataaatacatgttctcactcctgtgcagaaactaaaaaagttgatcccacagaggtggagagtagaatagtggttactggaggcggacaagggggagggggagggggatagggaaggactggttaaaggatacaagtttacacagccagataggaatagtatgttttagtattctgtagtactgtaggatgactatagttaagaatcacgtatttatgtattttcaggtatttacaagagaggattttgaaagtttccatcacaaagaaatgataaatgtctgaggtgatggttatgcgtattaccctatgccctatagatatgtataattatgtgtcaatttcaaaataaaaattcaaaactacaactcctatgaaaatttttgagcgtgtttgtacttattaagtgtatttataaatcatacggatattatcttcagcctgcatattaaattgtagttaagcttttactttttaactaaaaaataaattctattattttttcctatatcccactgcactgaccccagtttggaaatcctaagattatcaaataaaaactttgattattgaagaatccaggtgtactgccacagaaaagttctattctgtagcatggactctaatatgtaatctagcccattgtgcttacagatagatgtgtgcctgtagtcatagaaaaatttgcatgagctaatgactgccttgctactagattagctcaaagcaaaaagttctctgaaagcaggtcaatagggtcatttttatattatgaagaagaaaagcagctgttgtattacattcactgtattggtcctgcttgtgtttcagggcaagatccttgttgggacaaggaatgctgaaataatcgaagttggagagaaaaatgcagcttgtaatattttagttaacggtcatgtggatgggccaatctggggactagcaacacatccttccagggattttttcctttctgctgcagaagatgggacagtgagactttgggatattgctgataaagtaagtacagataatttttttaaaagaggttacaacttctaaaaagaaaagttggaagttctaaattgctagtacttaaagaactgccagaattctgttgagcattttgaggggaaactggtataatttagaagtacttcacttaatgtttcctatgactctttttttttttttttttaaatgcagaagatgttaaacaaagtgaatttgggacatgctgctcgtactgtgtgttacagccctgaaggggacatggtggctattggaatgaaaaatggagaatttatcattttactagtgagttctctaaaaatatggggaaagaagagagacaggagatgtgcaatccatgatatcaggttagtgaacaaatggaatagagtttctagtatatacttgatttaacttccatttgtaaaattttccatagccttgccttcaaaaagaggtccccagggcctgtagcatttcccgtattataaattgtatgctaaaatatggctgtttgtatactacttaattcttcttgctaaattataaacccactgggcaccaactataatagcaagtactagtaggtaatgtttgatgaattcatgttaacacttagccatgtccattaagttcatcccaccaagaggtatctcccactgtaatacaagagagctatctgcccttcaaaagttgtcaccctggaaaactaaagttgtgatttcaaacatatcttctcttagtaacctcagtttgggaatatgtagttcattaatttaatcaatacctattgattaaatgttccagaatccaaattaatttaaatgtttcttaaacctttgtttttcagtgcttaagcatttttcaacagtggctaccatttacggagtacttccgtgtgatcagtagataagattattgaatctaggtctgtcaaaagcttgtacacttttcatcagtaaaatccttttacaaatgaaaccttcctcagaacttcaatatataaaatagtaacagtggcttcccttagcttttacatgtctctatcgtacctcagtaagactcatgggccatttcaagagactgaattgtcccatatgactccaaagattgctaggcaaatagcatttcactttgtcttttaaataagttcttcaggccgggcgcggtggctcatgcctgtaatcccagcactttgggaggccgaggcaggcagatcacctgaagtcaggagtactcgaccagcctggccaacatagtgaaaccccatctcaactaaaaatacaaaaatcagccgggcgtggtggcaggcgcctgtaatcccagctactcagggggctgaaacaggagaatcgcttgaacccgggaggcggaggttgcgccatcgcactccagcctgggagacaagagcgagacttcgtctcaaaaaaaaaaaattcttcttccaagattcaagttgtgtcatttcaccttaataactggaggttagttaagctgggctgtgttctttgcttaatattaagacaacgttttttccagatggaagaaaactatcttaatgaattgttagcttattaattatgtaatgctaatggcttttaaaagctgagatgttctgactgggtgttgtggctcacacctgtaatcccagtaccttgggaggccaagggggaaggattgcttgaggccaggagtttgggaccatagtgagaccccgcctctatttaaaaaattaaattttgttttgttttgttttgagttggagttttgctcttgttgcccatgctgaagtgcaatggtgcaatctcagctcaccacaacctgtgcctcctgggttcaagcgattctcctgcttcagcctcccgagtagatgggattacaggcgtgcaccaccatgcctggctaattttgtatttttagtagagacagggtttctctatgttggtcaggctggtctcaaactctcgacctcaggtgatctgcccgcctccgcttcccaaagttctgggattataggtgtgagccactgggcctggcctaagaaagtttttttaagccattagacgtttttaaaggaattgggagatgacaattggggaaatatttaaaatttaagtaaaatataaagcttccttatttcatgtaacccagacaatctcagtatacatgatcagttgtgtctgacaggtaaatctatttgaggccttatcacacgttacttttaagaactagaaaggaaaagtcactgatcttaagtatttataatacttcatgtggtctaatactttttacgttttgttttgattcagatttagtccggattcccggtatctggcagtaggttctagtgagaactcagtggatttttatgacctaacgctgggccccactcttaacagaatcagctactgcaaagacattccaagctttgtcattcaaatggacttctctgcagatagcagttatctccaggtacagtaccaatactgtatacccaggtggcaagttcttctgcttttacatttcgtgttagtgaatgcatttaaagttcctgagctccagagctccagcttctcaactcctccctttgtaccttctgacctacagctcccctttcctcccccacttatcagagcttttctcctattaagtttttgtagtgatcttttgcatacttaataatgttagacatgtaaatcaagtagcaatatgctagtattctgtaaaccccctgtggattttgtctctcacctaatggaattcttgtcccattttaatctgatgaaaaaggtctctagtggctgctataaacggcatgtctatgaagtgccttcaggaaaacatcttatggatcatgccgctattgacagaattacttgggctacatggactaggtaaatacttatatattcacaaggcaagaactgactttgaaggccagttagaaaatcctatttctgaactgttagagccattccaataaggaatagtaattgagtttcaagtttttgttaccatattttgaaatggtatgttcatgttgggacccctttttattgaatatatttccatgttttatcagtttccatgatttatcaagttttttttttaaggaaatcaaagttttaactttaaagataccctgatatttttcttaatgctaaatttaatgactggcaaaaaggtattgggtgctgttaagcaactgttattaattctctatctaaaggaatgctatcttgaatctattagaagtcaaagcttccaaatttgttcaaatttcctggctgtatgacaggtaaccatgactatccatttttttggccaatgaaaaatgccatcaaattcctgtatcagccaggcatatagtggctcatgcctgtaatctctgatgtagcaggccgaggtgggaggatcacttgagcctagaagttttgataccagcctgggcaacatagcaagaccccatctctgaaatttttttaattcctatgtcataagtcatttttatttttgtagagatagggatctcacaatattgcccaggctggtctcaaactcttggcctcaagcagtcctcctgcctcagcctcccaaaatgttgggattactggtatgtgctgctggacccagccaagtagcacttttaatttgaaaaatagttctatcagttttcagtcaggcgcggtggctcagcctgtaatcccagcactttgggaggccgagcgggggtgatcacctgaggtcgggagttcgagactagcctgaccaacatggagaaaccctgtctctactaaaaatacaaaataagccgggcatgttagcgcatgcctgtgatcccagctactcgggaggctgaggcaggagaattgcttgaacccaggaggcagaggttgcggtgagccgagatcatgccattgcactccagcctgggtaacaagagcgaaaactccgtctcaaaaaaaaaaaaagaaaaaatagttctatcagttttcataaagtactactttaatcttaaaaagattaatctagaaacccttcaaattataaaatgtcatttttaaaaggcaggagttgatatcctgatgaaattcaggtctccaaacaacttaccataatttacttcctgtattttaagtaacatgatagggtacttagagattaattgccaagaaactttttgaatatagtcaacctgcccgcacttgccatgatgagttttcttttgttccttccctctagtattctaggagatgaggttttgggaatctggtccagacatgctgagaaagctgatgtcaactgtgcctgtgtatctcattcaggaatcagtcttgttacaggagatgactttggcatggttaagttatttgacttcccatgtccagaaaaatttgtaagtttgtgttttgtttactattatcagtttactcctaattttgatgtcttatcatcagcacttttccccatatatttaaaatgttttgtcctaatttctaaatttttccccaaactttctaaatctatttactttgaaataaaagctattagaaacaaatcctctccctcgagtaataccatctttggaaccatcctacaaaagctgtaattagcttttcaccaaacctataatcagttatcaaatttcaaatgcttttccttagagaaaaatggtcagagtacctggagacatctgactgcccacacagcctggttttgcagatccactactcatgctgaaaagcattctaatcactggctgcggtgctaactccctactctctccacagctcttgtcatagagattatagttcctaataagagcctttgacttctgtgtgcaccaaatgccctgagcttgtctgtcattgttttttaggcaaaacacaaaaggttcttgggtcattcgccccatgtgacaaatattcgatttaccagtggtgatcgacatgttgttagtgctggaggtgatgactgcaggttagtaactttctcagcccatgaagagcagactatgttactagttaagagacttaatacaacaactcctacagctttggtttatgaaatcagctagtcaacattagtagaaggtagtataaccagatggctcttcagaatctcatatttatgcaaatacagaataaaaggagttaaagaggaaaaatattacacatgtaacctgaaagcacaactgaaaaatattaaactgttatgaaaatctaaaaacataattaactccctgcaattttcttctctgattgcagcttatttgtctggaaatgtgtacatacacctcactgagagatgctgagatgactacagaaattaactttgagaccagaattacagagaagaaaaaccaaaacccaaccctgcatggtcaagtggtgctaacccaagactgtaacagggagaaatgcccagaatcatcaaaatagtgaaagactgatctgttcaaaatatttgctatatgcactgggtataatccgtaatccatacactgccagataatgccatttcaaggaaggatcgaatacttgatggtaaaggccaagtccccctgtattgggaagtgtgtgatttcggcagacctgctgggaaaatttagggtagagcactctttacagaagaactcaaaaacccaatttggataattttcattatctttttagcaaaatggtttcttaatgtttatattttattttcaaggttcattgtttaatgaaatattttattcttgcatttccataaggaaagggaaagtcatgatcatcctaaaggatcacagtttttaaaaggcaaacattttccctaaggaaacagacacaagctttcctagagaatatgatgttttttaggcattaataaggtccttttttataaaggacacttttctcctagtagttttgaattcaggaacagatccaaagttagcagtatatggctgctacatttccattttcattttcgagccatcagtttatgttcagatgccatctctgtaatcgcacatttaaaacataactgtagcctcactaatggaaaagtagtatgatgaacaatcattcccaatggtgtacaatgtaagggttttagggagcaacagtatttaactggaagaaagaattgcatatttaatgtagtctaatatatacacatttgtttaacatgtaaacaaaagtgttaaattcacatatacaacattatacaatttaatcactcttggaataaaatttttatagccttttttctattgggaaaatttgtttagatgtgtgccactccataggtttatttccaaaatgaatgagcccaactccatttgtaaaaacttgtcagttagaattcctttttttagtggattagggctgaattcttagatccttatttcttttcactttaaatgctgccaaagatcactactcatcattcaggaattcgctgtctagcctatctgtagtttcctgaagattgaaaattatgtagactgctatttaaaaatatatttttctaagtgtgaggtttaagatgctgtattgaccctatgagtttttaatgtgttaattatctttatagcataatagatcgctttaggttcctggaatcccatttggtctgacaggatatatgaagattcttaatacctattttctgtgtctaatacttggttaatactaaaaatagaaatgactaaattacatcacagaaagcataaccagtgattgaacctggtagttttaaagctctaaatagctgtggctgaaggactgattatggggctaagaagcttgaaacgtaagttggtacttgttcatcagtggattctcctaaattaagccaaattttgaaatacatgactattaagtttctactcatgtatttacagtcagtcaataaattaaaggaggaaaaaaatccctgaacaacctgcccataaaaagaaaaatactctacatttgagcctgctgcagttttaaattttccctctgggtcaagtttgccagcttttggctacagagaaattatatttccattacagtgcaggtagaaactctgtaaccttaagcatgtaaactacatagaataaaactgtttccactgcatttctgtccttcaaagtggccaacctgattaagtcagccttaatcactgctgctgtcagtttcacgactaaaggtcatattgactaagtagtcatcagctgaccacctcgctgtatcagccagcaacgaggggaaggtgaagaaacatgataggccatatagaatctgccctatgtttacttttttaacccagataattatttttgtgtgcagtatctaagctcctgattgtgtaacctgggacttctggcaccttttgttccattcattttatgtataaaatgcatgccaaagcacactgtgccctctggtacccttgcttccaatcgccaaccatgctcatttccttcctttttttgtggtccctttttgtggtgatcattttaaaccacgtcatccaacaaatgttttatggtcaaccttagcttgttcataagccatagcaactgaaagattaaactcttaaatatgtgtctgggcagtggctattaaatagcaaaaaacaatcagattttagtattttattatttccttgtaaaatggctgaactaaattaaacccttgtttcccatttgttctataatttatagtgaaactgagaacaaaactatctttataaatgatagctaaaagtatttccagatatttaaacaatttaaaataaatttcttctgcagagatgcaaagcatctcaacactggaatgaacaaatgccttaaattcaatggagtaaacctttagaatgaagaggaactgtcatttcacccaagccgaagacaacagccttatgcacttgtgtgctctgtctttgctgcttctcgtgtttcaagcctttcctgtgggatcagcacagcaaagtgcaacttaccaaatggtttaatgactggttaattctttcttctcccaatggaaaagcaatggcaacacaacagtagactgctggcttgacaatcttaaacgtgagcctttgcacatgtaggtttatcatcatttgagtatacgactaagcaagtcaatgaactttttttttttttttagcagtttaatttggtcctgagaatgttgcagtctttattaccccttttgcattaatccacttttctaaccaccttttaagctttaatttttaacactatacaccaagtctttgaaatcagtgatctgttatttaactctaaagcatttgacacttcttgccttaacagttttaaaaaccacacacaaaaaaactctgtaagtaatacagtaggccaaaagtttcatcctatctatcttgcagtttacctatctgatctgatctctgtaattatagttctgtcatttaaaatatactatttaaatctaatttttacatttcaaaaattatcttcagtagtaactaagtatattttctgtggattctgagaatgttatttttcagaatgtgagaatatatatgtacatttataatcttgtgactttaaagtctgttttcagatacagtatgtaaatacttgtaaaaaaatttgtataattttgtgataatgtagtttcccaaaaaaattatttagaaggcattatgttattagtaaatgagagcactgtatagaactgttcctattttctgcacttgccattccagctgcctccactgtccatacccacctcattcatcctgtcacagaaggcaggaaaactgggaactttaccaaagtagcactcagcctgagaggcctgtataatcatgcttttcaaactaaattcacttaaaaattaaaaagcagaattgaatattttaagcagcctcagtacctttggccaatgctgttttcatggtggattatgaacattatataatctttgggaaaagtgaaagtagtacaatttttagaataatgacaactgcctcactgcatctctccactcacacagcaaccgtgtagccccctaagctgcagtaccatgactaaccatgatgtcaatttcatatgctgatcctcacaacagcagtgcacaaacatgccccaaatattttaacagaatttagctcttccttaagctgtcttttcatagtaaaaacaaaacaaaaacacccaatgttaaaaccacataataaacttacaaacttgaaaaattagacacttcagatagataggcaataaaacttcatattatgaaagcaatatattccaagtttcaaagatttgacaagttctgtagagtatctttcatcagtacatgaaaacttccaaactgcatgatcttctgccaggcaggactgggtgctattcgctggtttgaggtcgaatccatttcaaggcatgtcgtggtgggacattaatggtgggatggtagaatgtgcagtccggtcttgtacattgagtgttaaacctacaatgttttggatgatagaagggacattccatcttcttacaagcagggaagtaacggcagagctgactactggaaggtggtgctggtggtgcaactgctggttttggagacagtactggaattcttctactcacatgagtgaagggacaatctggtttagtacactttgcatcatatttacaatttgggtgaacaaacaaacatttttcagcaaatttacaattggggaaggctttgcagggtgagatggggtgatggtaggcacactcatccccatttttacaagcaggccagtacttgcagcgctccaaaagtttttctggtttctgtgccacactcagttcactcatctcagcgttagaaaagctaccatttgggtcctcaagctgcctgctcagcaagtgcaactgctgtgggtggaggagacctctgagtcccttgtttgaggctgcagtttggtttacgggtttcattccttcaaagcacatgtcctcctcttgatctgacatgtatcctggggggctggggacaccatccagcgtcactataaacttgggacttgcaggtttatctggttgtacaagatctcgtgtctgcataaggtgtcctgaaagtacccgaagggaatctgcagtcttcatccccgactcttggtttggtgccactactacttcctcagacagctttggcttcttcagaataaatgatcttgtgtctgcatggaccatggattccatgtcatagtaatcttgactcatctgcagagtttctgccattactgggtcgatttgcagtcgggataataattgcctctgttgagttccttgatttttttctacagaatctccttttgtttcctcttctttaatggggggacttattctgggggtcctactttgtccctggaccacttctgctagcaattcttcttgagaagttcgagttctgggagcaactggaagtgtctgtttctgtggaactgtagagtagttagttgtttttgttacggattcttgagcttcagatatagccttcaaaatcagattcttgttagcttgtttagaaggtggaagagaaggtctcctttcaggctttgcaggcacagacacactgctggagatgcttcctgttcgagacccgtaatcatcatcttcttcctcctcttctccatcatgattgaatttttttactttaacaactgaacttaccacaggcaactttctcttccgaaagttttcatcctccatactcattttctccgagttgtttctaaagaacggactatacgtttcttctaagctgttaagcacctctggttcacacaaacgtcctgtttcatatacccaactactctgcatatcaagctgcttggcagcatgaatactattctgctgctgttgaaattgcaacctgtttaaatgaacaccactatctgcatttctacttgcaggtggtcgataaatttcaatagaagggcgagaagaaccatatgtaagtgtcactgtaggttttttctgagataagggattctcctgcacaaagttgaggtcttcgtcaatgagatcatctggttctggcttaatatcaatcacatcttcagagggtgctggctccctcaaaggtttcactgttgacattagtcgggttgcagctccatcatcgtaagtctgtctgacatttgtggtttttgactcctgcgaacttgtagaaactctggaatctcttttttcaggtctcgcgctaggaatggcaagtggtggcactgcagcttcatgcctcctctcatctccccgactgaaattgctcttgtttgaaggcacgttactatcaaagatgttggtatcagaagacttcagactagagggttcagttgtaacagagcgaagtttatctaatacaccatgaagccaacataagctcctaattcttgtaatttccccttaatggcactccggatcttgcggctgatctcggtgccgatctccatggctctgcggcgtgcgggaactcagcactgcgcggcgcttggcttacccggaggctgccgcggactcctaccccgcagccgggacaccaccgcctcc

SEQ ID NO: 13608 - RNA, 16931 nt, Homo sapiens
  source 1..16931: mol_type = other RNA
gctgggattacaggcatgagccaccataataaggattctgatgaacatttgattccttggactactgttatactcaaaagccttccttaatcttctaattgtcaccctaaatatcctaaaatttctgtcttcctagtagttcttcatagtcctaaaaatttgtcagagagaaaggtaaatcaagaaacatgattttcaaatgatttaaggtggtactagggtttaggatttcctttgctttttatcatttaacacactgcttatcatacagctggaagtgctctgggccagtgtctctacttcgagggaagaaggaggtagtgagacagaaggaaatagcacaattcctggccctgacagaagggtgttcaggagacctgctctcctctcactttattccatctcatctggacctgtggcttccaatccacatctctttcctttaatatcctgcattggctaggctgtataaatcctttggtgcatcgaaaaactaagtgcattttttgtttttgtgattatgcaatacttataggaaaagttataattttagaatatttaagtacacttacatttttgagaaaaagactattgaaatgtttgtgccatgtcaaatttcagttgaacattttgggtattcttaatataagaccaggccaggcaccgtggctcaggccgggcacagtggctcacacctataatcccagcacttagggaggccaaggcgggaagatcacctgaagtcaggagttcaagaccagcctggctaacaaggtgaaactctgtctctactaaaaatacaaaaattagccgggcgtggtggctggcgcttgtaatcccagctacttgggaggctgagacaggagaatcacttgaacctgggaagcagaggttgtggtgagctgagatcgcaccattgcactccagcctgggcaacaaagagcgaaactccgtctcaaaaaaataaaaaataaaccctagaattatagtatgttagaattggaagggaagaattgtctaaggttattctagctaataagcaacagacttggaaaggaaaaggtcctgacaaagctaagcctcccgttcaggtttcctgactcgtgaattcagtgctgctgccactacacgatgcatgctctttgtatcaagggtgagacagcattacacatacatagaaaattatctatttaaactctatttgaacttttgatgagtttgtctccccctcccccactccttttcagaataacttgacgtttacaggtaccatcagtggtgatgtctgtgtgtggaaagatcacatattgtgtagaatcgtggcgagagctcacaacgggcctgtgtttgccatgtacaccaccctgcgagatggacttatcgtgactgggggaaaggaaaggccgtgagtcctctttcttttcacagaatatttatgcatttgtgacctacctgaggtttgcagttaattattctagttgtttctaggctacacagagtgtcctctccgaccttcctcctcatatgcttctcctttattaccttttatgtgccttctatttgattctcatttctggtcttaattcacttccaatttttttcatgttggggtgatactttttctgaggtgtggataggtagttgtcctacaagttgagttacttttcttaatgtctgtatgcctgtgtatgatttgctgagtaggaggcccatgggggaatctggagccagggttgtattttgactgcctgctctctttttgttcagaatggattctaaggagtagaatgcacattgttgctttagaaaaggatgagggaactagagagaactgccttgtttccttttgcttgaggcaaatttaaactgttttatacaagacctcaaaatttgagaagaggtctcttctgagtgattttcaaatctcccaacagtaaccagatacttatgatttgatttgtcaccaacatagtcatatgcatgttgaaacatgacatgtaggccaggcacagtggctcacacctgtaatcttatcactttgggaggctgaggcaggtggatcgcttgagcccaggagttcaagaccagcctgggcaacatggtgaaaccccatcgctataaaaaacaacaattagccgggtgtggtggcacatgcctgtagtccctgctactcaggaggctgaggtgggaggatcacttgagcctggggaggtcaaggctttagtgagctgtgatggtgccactgcactccagcctgggtgacagagtgagaccccatttaaaaaacaaaaacaaaaacaaaaaaaaatgtgacatatagttgactaagaagtacatttcaatacaggattgaaagaacccacatatgttaattaaacacaagcgcagaatttgtgccttttacataaaggaagaatgcacataggcatgctttcagacaagcaattcatctagcagaaaaggaaggaatacatttttcagcccttccaggaataaaatccataaatgggctctatttcgtcctccaacacttgtatttcccacgtcatttactcctgcacacccccactcactagaagcctgctaaactgttccagtgagatattttaacacctgatagggaataaatatgcttctgttttggccttcaaaaataagctctgggccagttgcagtggctcacgcctgtaatcccaacactttgggaggccgaggtgggcggatcacgaggtcaggagtttgggatcagcctggccaatatggtgaaactccatctctactaaaaatacaaaaattagccaggcatggtgcctgtaatcccagctacttgggaggctgaaggagaagaatcgcttgaacctgggaggcacaggttgcagtgagccgagatcacaccactgcactccaggccaggtgacagagcgacactctgtctcaaaaaaataaataaatcaactctgtagcatagcatttgtaattctattattttgccttacatttccattatccttttaataaaattgtttttttacatcttcctaatcaagaagtattatgaggccaggcacagtggctcatacctggaatcccagcactttgggaggccgaggcaggcagatcacctgaggtcaaggtatttgagaccagcctggccaacatggtgaaaccccatctctactaaaaatacagaaattagctgggtgtggtggtgcacacctgtaatgctagctactcgggaggctgaggtaggagaatcgcttgaacctgggaggcagaggttgcaataagcctagatcatgccactgcactcaagcctgggagacagagcgagactacatcttaaaaaaaaaaaaaaaagtattatgagagaggataatgtattgtaatgtattgtagaggctaaataaaattatgctcatgtcagaaaaaaagagtatttctcaaaataaaattcactgaaactggatgtttattttgactgagatatagtatatcctcaaattgccatagaaagtttacaagaatattagaggtaaattataaatatcagggcctttttaaaaaaaaaagattctgcttataacttggtatttgtttataataaaaattatagtagccaataatgaacacttactctggcttggttatttacttaggtcaaaagaaggaggagcggttaaactgtgggatcaggaactgaggcggtgccgtgccttcaggcttgagacaggacaagccacagattgtgttcgttctgtgtgcagaggcaaagtaagatgttccatgagctgatacagtgcagcagaaaacagaaagtggttattactgtgattccctcaccctttgcagcctaatgaacaatacttaataatgcataacgatggatttgcttgccaacattactctgtctttgctgctttctttgccaaagttagcaccagtgtggtgcataagctaggaagctattctgtctaaatactgtatgtaaacctccaatattttctagaatctgccaatttaacaactctagtagacataattgaaagcccttggcagttgactcatattaggacagctgtctccattttttaaaaaaacacacattccctagataaaacgtgcagtaaacaaacaatgaaatactactcagccataaaaaataatgaaattctgtcattcttggtggcaacatggatgagactggaggacatgatgtgaagtgaaataagccaggcacagaaagataaatacatgttctcactcctgtgcagaaactaaaaaagttgatcccacagaggtggagagtagaatagtggttactggaggcggacaagggggagggggagggggatagggaaggactggttaaaggatacaagtttacacagccagataggaatagtatgttttagtattctgtagtactgtaggatgactatagttaagaatcacgtatttatgtattttcaggtatttacaagagaggattttgaaagtttccatcacaaagaaatgataaatgtctgaggtgatggttatgcgtattaccctatgccctatagatatgtataattatgtgtcaatttcaaaataaaaattcaaaactacaactcctatgaaaatttttgagcgtgtttgtacttattaagtgtatttataaatcatacggatattatcttcagcctgcatattaaattgtagttaagcttttactttttaactaaaaaataaattctattattttttcctatatcccactgcactgaccccagtttggaaatcctaagattatcaaataaaaactttgattattgaagaatccaggtgtactgccacagaaaagttctattctgtagcatggactctaatatgtaatctagcccattgtgcttacagatagatgtgtgcctgtagtcatagaaaaatttgcatgagctaatgactgccttgctactagattagctcaaagcaaaaagttctctgaaagcaggtcaatagggtcatttttatattatgaagaagaaaagcagctgttgtattacattcactgtattggtcctgcttgtgtttcagggcaagatccttgttgggacaaggaatgctgaaataatcgaagttggagagaaaaatgcagcttgtaatattttagttaacggtcatgtggatgggccaatctggggactagcaacacatccttccagggattttttcctttctgctgcagaagatgggacagtgagactttgggatattgctgataaagtaagtacagataatttttttaaaagaggttacaacttctaaaaagaaaagttggaagttctaaattgctagtacttaaagaactgccagaattctgttgagcattttgaggggaaactggtataatttagaagtacttcacttaatgtttcctatgactctttttttttttttttttaaatgcagaagatgttaaacaaagtgaatttgggacatgctgctcgtactgtgtgttacagccctgaaggggacatggtggctattggaatgaaaaatggagaatttatcattttactagtgagttctctaaaaatatggggaaagaagagagacaggagatgtgcaatccatgatatcaggttagtgaacaaatggaatagagtttctagtatatacttgatttaacttccatttgtaaaattttccatagccttgccttcaaaaagaggtccccagggcctgtagcatttcccgtattataaattgtatgctaaaatatggctgtttgtatactacttaattcttcttgctaaattataaacccactgggcaccaactataatagcaagtactagtaggtaatgtttgatgaattcatgttaacacttagccatgtccattaagttcatcccaccaagaggtatctcccactgtaatacaagagagctatctgcccttcaaaagttgtcaccctggaaaactaaagttgtgatttcaaacatatcttctcttagtaacctcagtttgggaatatgtagttcattaatttaatcaatacctattgattaaatgttccagaatccaaattaatttaaatgtttcttaaacctttgtttttcagtgcttaagcatttttcaacagtggctaccatttacggagtacttccgtgtgatcagtagataagattattgaatctaggtctgtcaaaagcttgtacacttttcatcagtaaaatccttttacaaatgaaaccttcctcagaacttcaatatataaaatagtaacagtggcttcccttagcttttacatgtctctatcgtacctcagtaagactcatgggccatttcaagagactgaattgtcccatatgactccaaagattgctaggcaaatagcatttcactttgtcttttaaataagttcttcaggccgggcgcggtggctcatgcctgtaatcccagcactttgggaggccgaggcaggcagatcacctgaagtcaggagtactcgaccagcctggccaacatagtgaaaccccatctcaactaaaaatacaaaaatcagccgggcgtggtggcaggcgcctgtaatcccagctactcagggggctgaaacaggagaatcgcttgaacccgggaggcggaggttgcgccatcgcactccagcctgggagacaagagcgagacttcgtctcaaaaaaaaaaaattcttcttccaagattcaagttgtgtcatttcaccttaataactggaggttagttaagctgggctgtgttctttgcttaatattaagacaacgttttttccagatggaagaaaactatcttaatgaattgttagcttattaattatgtaatgctaatggcttttaaaagctgagatgttctgactgggtgttgtggctcacacctgtaatcccagtaccttgggaggccaagggggaaggattgcttgaggccaggagtttgggaccatagtgagaccccgcctctatttaaaaaattaaattttgttttgttttgttttgagttggagttttgctcttgttgcccatgctgaagtgcaatggtgcaatctcagctcaccacaacctgtgcctcctgggttcaagcgattctcctgcttcagcctcccgagtagatgggattacaggcgtgcaccaccatgcctggctaattttgtatttttagtagagacagggtttctctatgttggtcaggctggtctcaaactctcgacctcaggtgatctgcccgcctccgcttcccaaagttctgggattataggtgtgagccactgggcctggcctaagaaagtttttttaagccattagacgtttttaaaggaattgggagatgacaattggggaaatatttaaaatttaagtaaaatataaagcttccttatttcatgtaacccagacaatctcagtatacatgatcagttgtgtctgacaggtaaatctatttgaggccttatcacacgttacttttaagaactagaaaggaaaagtcactgatcttaagtatttataatacttcatgtggtctaatactttttacgttttgttttgattcagatttagtccggattcccggtatctggcagtaggttctagtgagaactcagtggatttttatgacctaacgctgggccccactcttaacagaatcagctactgcaaagacattccaagctttgtcattcaaatggacttctctgcagatagcagttatctccaggtacagtaccaatactgtatacccaggtggcaagttcttctgcttttacatttcgtgttagtgaatgcatttaaagttcctgagctccagagctccagcttctcaactcctccctttgtaccttctgacctacagctcccctttcctcccccacttatcagagcttttctcctattaagtttttgtagtgatcttttgcatacttaataatgttagacatgtaaatcaagtagcaatatgctagtattctgtaaaccccctgtggattttgtctctcacctaatggaattcttgtcccattttaatctgatgaaaaaggtctctagtggctgctataaacggcatgtctatgaagtgccttcaggaaaacatcttatggatcatgccgctattgacagaattacttgggctacatggactaggtaaatacttatatattcacaaggcaagaactgactttgaaggccagttagaaaatcctatttctgaactgttagagccattccaataaggaatagtaattgagtttcaagtttttgttaccatattttgaaatggtatgttcatgttgggacccctttttattgaatatatttccatgttttatcagtttccatgatttatcaagttttttttttaaggaaatcaaagttttaactttaaagataccctgatatttttcttaatgctaaatttaatgactggcaaaaaggtattgggtgctgttaagcaactgttattaattctctatctaaaggaatgctatcttgaatctattagaagtcaaagcttccaaatttgttcaaatttcctggctgtatgacaggtaaccatgactatccatttttttggccaatgaaaaatgccatcaaattcctgtatcagccaggcatatagtggctcatgcctgtaatctctgatgtagcaggccgaggtgggaggatcacttgagcctagaagttttgataccagcctgggcaacatagcaagaccccatctctgaaatttttttaattcctatgtcataagtcatttttatttttgtagagatagggatctcacaatattgcccaggctggtctcaaactcttggcctcaagcagtcctcctgcctcagcctcccaaaatgttgggattactggtatgtgctgctggacccagccaagtagcacttttaatttgaaaaatagttctatcagttttcagtcaggcgcggtggctcagcctgtaatcccagcactttgggaggccgagcgggggtgatcacctgaggtcgggagttcgagactagcctgaccaacatggagaaaccctgtctctactaaaaatacaaaataagccgggcatgttagcgcatgcctgtgatcccagctactcgggaggctgaggcaggagaattgcttgaacccaggaggcagaggttgcggtgagccgagatcatgccattgcactccagcctgggtaacaagagcgaaaactccgtctcaaaaaaaaaaaaagaaaaaatagttctatcagttttcataaagtactactttaatcttaaaaagattaatctagaaacccttcaaattataaaatgtcatttttaaaaggcaggagttgatatcctgatgaaattcaggtctccaaacaacttaccataatttacttcctgtattttaagtaacatgatagggtacttagagattaattgccaagaaactttttgaatatagtcaacctgcccgcacttgccatgatgagttttcttttgttccttccctctagtattctaggagatgaggttttgggaatctggtccagacatgctgagaaagctgatgtcaactgtgcctgtgtatctcattcaggaatcagtcttgttacaggagatgactttggcatggttaagttatttgacttcccatgtccagaaaaatttgtaagtttgtgttttgtttactattatcagtttactcctaattttgatgtcttatcatcagcacttttccccatatatttaaaatgttttgtcctaatttctaaatttttccccaaactttctaaatctatttactttgaaataaaagctattagaaacaaatcctctccctcgagtaataccatctttggaaccatcctacaaaagctgtaattagcttttcaccaaacctataatcagttatcaaatttcaaatgcttttccttagagaaaaatggtcagagtacctggagacatctgactgcccacacagcctggttttgcagatccactactcatgctgaaaagcattctaatcactggctgcggtgctaactccctactctctccacagctcttgtcatagagattatagttcctaataagagcctttgacttctgtgtgcaccaaatgccctgagcttgtctgtcattgttttttaggcaaaacacaaaaggttcttgggtcattcgccccatgtgacaaatattcgatttaccagtggtgatcgacatgttgttagtgctggaggtgatgactgcaggttagtaactttctcagcccatgaagagcagactatgttactagttaagagacttaatacaacaactcctacagctttggtttatgaaatcagctagtcaacattagtagaaggtagtataaccagatggctcttcagaatctcatatttatgcaaatacagaataaaaggagttaaagaggaaaaatattacacatgtaacctgaaagcacaactgaaaaatattaaactgttatgaaaatctaaaaacataattaactccctgcaattttcttctctgattgcagcttatttgtctggaaatgtgtacatacacctcactgagagatgctgagatgactacagaaattaactttgagaccagaattacagagaagaaaaaccaaaacccaaccctgcatggtcaagtggtgctaacccaagactgtaacagggagaaatgcccagaatcatcaaaatagtgaaagactgatctgttcaaaatatttgctatatgcactgggtataatccgtaatccatacactgccagataatgccatttcaaggaaggatcgaatacttgatggtaaaggccaagtccccctgtattgggaagtgtgtgatttcggcagacctgctgggaaaatttagggtagagcactctttacagaagaactcaaaaacccaatttggataattttcattatctttttagcaaaatggtttcttaatgtttatattttattttcaaggttcattgtttaatgaaatattttattcttgcatttccataaggaaagggaaagtcatgatcatcctaaaggatcacagtttttaaaaggcaaacattttccctaaggaaacagacacaagctttcctagagaatatgatgttttttaggcattaataaggtccttttttataaaggacacttttctcctagtagttttgaattcaggaacagatccaaagttagcagtatatggctgctacatttccattttcattttcgagccatcagtttatgttcagatgccatctctgtaatcgcacatttaaaacataactgtagcctcactaatggaaaagtagtatgatgaacaatcattcccaatggtgtacaatgtaagggttttagggagcaacagtatttaactggaagaaagaattgcatatttaatgtagtctaatatatacacatttgtttaacatgtaaacaaaagtgttaaattcacatatacaacattatacaatttaatcactcttggaataaaatttttatagccttttttctattgggaaaatttgtttagatgtgtgccactccataggtttatttccaaaatgaatgagcccaactccatttgtaaaaacttgtcagttagaattcctttttttagtggattagggctgaattcttagatccttatttcttttcactttaaatgctgccaaagatcactactcatcattcaggaattcgctgtctagcctatctgtagtttcctgaagattgaaaattatgtagactgctatttaaaaatatatttttctaagtgtgaggtttaagatgctgtattgaccctatgagtttttaatgtgttaattatctttatagcataatagatcgctttaggttcctggaatcccatttggtctgacaggatatatgaagattcttaatacctattttctgtgtctaatacttggttaatactaaaaatagaaatgactaaattacatcacagaaagcataaccagtgattgaacctggtagttttaaagctctaaatagctgtggctgaaggactgattatggggctaagaagcttgaaacgtaagttggtacttgttcatcagtggattctcctaaattaagccaaattttgaaatacatgactattaagtttctactcatgtatttacagtcagtcaataaattaaaggaggaaaaaaatccctgaacaacctgcccataaaaagaaaaatactctacatttgagcctgctgcagttttaaattttccctctgggtcaagtttgccagcttttggctacagagaaattatatttccattacagtgcaggtagaaactctgtaaccttaagcatgtaaactacatagaataaaactgtttccactgcatttctgtccttcaaagtggccaacctgattaagtcagccttaatcactgctgctgtcagtttcacgactaaaggtcatattgactaagtagtcatcagctgaccacctcgctgtatcagccagcaacgaggggaaggtgaagaaacatgataggccatatagaatctgccctatgtttacttttttaacccagataattatttttgtgtgcagtatctaagctcctgattgtgtaacctgggacttctggcaccttttgttccattcattttatgtataaaatgcatgccaaagcacactgtgccctctggtacccttgcttccaatcgccaaccatgctcatttccttcctttttttgtggtccctttttgtggtgatcattttaaaccacgtcatccaacaaatgttttatggtcaaccttagcttgttcataagccatagcaactgaaagattaaactcttaaatatgtgtctgggcagtggctattaaatagcaaaaaacaatcagattttagtattttattatttccttgtaaaatggctgaactaaattaaacccttgtttcccatttgttctataatttatagtgaaactgagaacaaaactatctttataaatgatagctaaaagtatttccagatatttaaacaatttaaaataaatttcttctgcagagatgcaaagcatctcaacactggaatgaacaaatgccttaaattcaatggagtaaacctttagaatgaagaggaactgtcatttcacccaagccgaagacaacagccttatgcacttgtgtgctctgtctttgctgcttctcgtgtttcaagcctttcctgtgggatcagcacagcaaagtgcaacttaccaaatggtttaatgactggttaattctttcttctcccaatggaaaagcaatggcaacacaacagtagactgctggcttgacaatcttaaacgtgagcctttgcacatgtaggtttatcatcatttgagtatacgactaagcaagtcaatgaactttttttttttttttagcagtttaatttggtcctgagaatgttgcagtctttattaccccttttgcattaatccacttttctaaccaccttttaagctttaatttttaacactatacaccaagtctttgaaatcagtgatctgttatttaactctaaagcatttgacacttcttgccttaacagttttaaaaaccacacacaaaaaaactctgtaagtaatacagtaggccaaaagtttcatcctatctatcttgcagtttacctatctgatctgatctctgtaattatagttctgtcatttaaaatatactatttaaatctaatttttacatttcaaaaattatcttcagtagtaactaagtatattttctgtggattctgagaatgttatttttcagaatgtgagaatatatatgtacatttataatcttgtgactttaaagtctgttttcagatacagtatgtaaatacttgtaaaaaaatttgtataattttgtgataatgtagtttcccaaaaaaattatttagaaggcattatgttattagtaaatgagagcactgtatagaactgttcctattttctgcacttgccattccagctgcctccactgtccatacccacctcattcatcctgtcacagaaggcaggaaaactgggaactttaccaaagtagcactcagcctgagaggcctgtataatcatgcttttcaaactaaattcacttaaaaattaaaaagcagaattgaatattttaagcagcctcagtacctttggccaatgctgttttcatggtggattatgaacattatataatctttgggaaaagtgaaagtagtacaatttttagaataatgacaactgcctcactgcatctctccactcacacagcaaccgtgtagccccctaagctgcagtaccatgactaaccatgatgtcaatttcatatgctgatcctcacaacagcagtgcacaaacatgccccaaatattttaacagaatttagctcttccttaagctgtcttttcatagtaaaaacaaaacaaaaacacccaatgttaaaaccacataataaacttacaaacttgaaaaattagacacttcagatagataggcaataaaacttcatattatgaaagcaatatattccaagtttcaaagatttgacaagttctgtagagtatctttcatcagtacatgaaaacttccaaactgcatgatcttctgccaggcaggactgggtgctattcgctggtttgaggtcgaatccatttcaaggcatgtcgtggtgggacattaatggtgggatggtagaatgtgcagtccggtcttgtacattgagtgttaaacctacaatgttttggatgatagaagggacattccatcttcttacaagcagggaagtaacggcagagctgactactggaaggtggtgctggtggtgcaactgctggttttggagacagtactggaattcttctactcacatgagtgaagggacaatctggtttagtacactttgcatcatatttacaatttgggtgaacaaacaaacatttttcagcaaatttacaattggggaaggctttgcagggtgagatggggtgatggtaggcacactcatccccatttttacaagcaggccagtacttgcagcgctccaaaagtttttctggtttctgtgccacactcagttcactcatctcagcgttagaaaagctaccatttgggtcctcaagctgcctgctcagcaagtgcaactgctgtgggtggaggagacctctgagtcccttgtttgaggctgcagtttggtttacgggtttcattccttcaaagcacatgtcctcctcttgatctgacatgtatcctggggggctggggacaccatccagcgtcactataaacttgggacttgcaggtttatctggttgtacaagatctcgtgtctgcataaggtgtcctgaaagtacccgaagggaatctgcagtcttcatccccgactcttggtttggtgccactactacttcctcagacagctttggcttcttcagaataaatgatcttgtgtctgcatggaccatggattccatgtcatagtaatcttgactcatctgcagagtttctgccattactgggtcgatttgcagtcgggataataattgcctctgttgagttccttgatttttttctacagaatctccttttgtttcctcttctttaatggggggacttattctgggggtcctactttgtccctggaccacttctgctagcaattcttcttgagaagttcgagttctgggagcaactggaagtgtctgtttctgtggaactgtagagtagttagttgtttttgttacggattcttgagcttcagatatagccttcaaaatcagattcttgttagcttgtttagaaggtggaagagaaggtctcctttcaggctttgcaggcacagacacactgctggagatgcttcctgttcgagacccgtaatcatcatcttcttcctcctcttctccatcatgattgaatttttttactttaacaactgaacttaccacaggcaactttctcttccgaaagttttcatcctccatactcattttctccgagttgtttctaaagaacggactatacgtttcttctaagctgttaagcacctctggttcacacaaacgtcctgtttcatatacccaactactctgcatatcaagctgcttggcagcatgaatactattctgctgctgttgaaattgcaacctgtttaaatgaacaccactatctgcatttctacttgcaggtggtcgataaatttcaatagaagggcgagaagaaccatatgtaagtgtcactgtaggttttttctgagataagggattctcctgcacaaagttgaggtcttcgtcaatgagatcatctggttctggcttaatatcaatcacatcttcagagggtgctggctccctcaaaggtttcactgttgacattagtcgggttgcagctccatcatcgtaagtctgtctgacatttgtggtttttgactcctgcgaacttgtagaaactctggaatctcttttttcaggtctcgcgctaggaatggcaagtggtggcactgcagcttcatgcctcctctcatctccccgactgaaattgctcttgtttgaaggcacgttactatcaaagatgttggtatcagaagacttcagactagagggttcagttgtaacagagcgaagtttatctaatacaccatgaagccatacggtgaatcgaattgtgttgttccctagaaacagggacagatcctctgtcatttggtcctgacttttcttgttggccaccatcaccataatgtaatcaggaagttcttcatcaacataagctcctaattcttgtaatttccccttaatggcactccggatcttgcggctgatctcggtgccgatctccatggctctgcggcgtgcgggaactcagcactgcgcggcgcttggcttacccggaggctgccgcggactcctaccccgcagccgggacaccaccgcctcc

SEQ ID NO: 13609 - RNA, 17112 nt, Homo sapiens
  source 1..17112: mol_type = other RNA
gctgggattacaggcatgagccaccataataaggattctgatgaacatttgattccttggactactgttatactcaaaagccttccttaatcttctaattgtcaccctaaatatcctaaaatttctgtcttcctagtagttcttcatagtcctaaaaatttgtcagagagaaaggtaaatcaagaaacatgattttcaaatgatttaaggtggtactagggtttaggatttcctttgctttttatcatttaacacactgcttatcatacagctggaagtgctctgggccagtgtctctacttcgagggaagaaggaggtagtgagacagaaggaaatagcacaattcctggccctgacagaagggtgttcaggagacctgctctcctctcactttattccatctcatctggacctgtggcttccaatccacatctctttcctttaatatcctgcattggctaggctgtataaatcctttggtgcatcgaaaaactaagtgcattttttgtttttgtgattatgcaatacttataggaaaagttataattttagaatatttaagtacacttacatttttgagaaaaagactattgaaatgtttgtgccatgtcaaatttcagttgaacattttgggtattcttaatataagaccaggccaggcaccgtggctcaggccgggcacagtggctcacacctataatcccagcacttagggaggccaaggcgggaagatcacctgaagtcaggagttcaagaccagcctggctaacaaggtgaaactctgtctctactaaaaatacaaaaattagccgggcgtggtggctggcgcttgtaatcccagctacttgggaggctgagacaggagaatcacttgaacctgggaagcagaggttgtggtgagctgagatcgcaccattgcactccagcctgggcaacaaagagcgaaactccgtctcaaaaaaataaaaaataaaccctagaattatagtatgttagaattggaagggaagaattgtctaaggttattctagctaataagcaacagacttggaaaggaaaaggtcctgacaaagctaagcctcccgttcaggtttcctgactcgtgaattcagtgctgctgccactacacgatgcatgctctttgtatcaagggtgagacagcattacacatacatagaaaattatctatttaaactctatttgaacttttgatgagtttgtctccccctcccccactccttttcagaataacttgacgtttacaggtaccatcagtggtgatgtctgtgtgtggaaagatcacatattgtgtagaatcgtggcgagagctcacaacgggcctgtgtttgccatgtacaccaccctgcgagatggacttatcgtgactgggggaaaggaaaggccgtgagtcctctttcttttcacagaatatttatgcatttgtgacctacctgaggtttgcagttaattattctagttgtttctaggctacacagagtgtcctctccgaccttcctcctcatatgcttctcctttattaccttttatgtgccttctatttgattctcatttctggtcttaattcacttccaatttttttcatgttggggtgatactttttctgaggtgtggataggtagttgtcctacaagttgagttacttttcttaatgtctgtatgcctgtgtatgatttgctgagtaggaggcccatgggggaatctggagccagggttgtattttgactgcctgctctctttttgttcagaatggattctaaggagtagaatgcacattgttgctttagaaaaggatgagggaactagagagaactgccttgtttccttttgcttgaggcaaatttaaactgttttatacaagacctcaaaatttgagaagaggtctcttctgagtgattttcaaatctcccaacagtaaccagatacttatgatttgatttgtcaccaacatagtcatatgcatgttgaaacatgacatgtaggccaggcacagtggctcacacctgtaatcttatcactttgggaggctgaggcaggtggatcgcttgagcccaggagttcaagaccagcctgggcaacatggtgaaaccccatcgctataaaaaacaacaattagccgggtgtggtggcacatgcctgtagtccctgctactcaggaggctgaggtgggaggatcacttgagcctggggaggtcaaggctttagtgagctgtgatggtgccactgcactccagcctgggtgacagagtgagaccccatttaaaaaacaaaaacaaaaacaaaaaaaaatgtgacatatagttgactaagaagtacatttcaatacaggattgaaagaacccacatatgttaattaaacacaagcgcagaatttgtgccttttacataaaggaagaatgcacataggcatgctttcagacaagcaattcatctagcagaaaaggaaggaatacatttttcagcccttccaggaataaaatccataaatgggctctatttcgtcctccaacacttgtatttcccacgtcatttactcctgcacacccccactcactagaagcctgctaaactgttccagtgagatattttaacacctgatagggaataaatatgcttctgttttggccttcaaaaataagctctgggccagttgcagtggctcacgcctgtaatcccaacactttgggaggccgaggtgggcggatcacgaggtcaggagtttgggatcagcctggccaatatggtgaaactccatctctactaaaaatacaaaaattagccaggcatggtgcctgtaatcccagctacttgggaggctgaaggagaagaatcgcttgaacctgggaggcacaggttgcagtgagccgagatcacaccactgcactccaggccaggtgacagagcgacactctgtctcaaaaaaataaataaatcaactctgtagcatagcatttgtaattctattattttgccttacatttccattatccttttaataaaattgtttttttacatcttcctaatcaagaagtattatgaggccaggcacagtggctcatacctggaatcccagcactttgggaggccgaggcaggcagatcacctgaggtcaaggtatttgagaccagcctggccaacatggtgaaaccccatctctactaaaaatacagaaattagctgggtgtggtggtgcacacctgtaatgctagctactcgggaggctgaggtaggagaatcgcttgaacctgggaggcagaggttgcaataagcctagatcatgccactgcactcaagcctgggagacagagcgagactacatcttaaaaaaaaaaaaaaaagtattatgagagaggataatgtattgtaatgtattgtagaggctaaataaaattatgctcatgtcagaaaaaaagagtatttctcaaaataaaattcactgaaactggatgtttattttgactgagatatagtatatcctcaaattgccatagaaagtttacaagaatattagaggtaaattataaatatcagggcctttttaaaaaaaaaagattctgcttataacttggtatttgtttataataaaaattatagtagccaataatgaacacttactctggcttggttatttacttaggtcaaaagaaggaggagcggttaaactgtgggatcaggaactgaggcggtgccgtgccttcaggcttgagacaggacaagccacagattgtgttcgttctgtgtgcagaggcaaagtaagatgttccatgagctgatacagtgcagcagaaaacagaaagtggttattactgtgattccctcaccctttgcagcctaatgaacaatacttaataatgcataacgatggatttgcttgccaacattactctgtctttgctgctttctttgccaaagttagcaccagtgtggtgcataagctaggaagctattctgtctaaatactgtatgtaaacctccaatattttctagaatctgccaatttaacaactctagtagacataattgaaagcccttggcagttgactcatattaggacagctgtctccattttttaaaaaaacacacattccctagataaaacgtgcagtaaacaaacaatgaaatactactcagccataaaaaataatgaaattctgtcattcttggtggcaacatggatgagactggaggacatgatgtgaagtgaaataagccaggcacagaaagataaatacatgttctcactcctgtgcagaaactaaaaaagttgatcccacagaggtggagagtagaatagtggttactggaggcggacaagggggagggggagggggatagggaaggactggttaaaggatacaagtttacacagccagataggaatagtatgttttagtattctgtagtactgtaggatgactatagttaagaatcacgtatttatgtattttcaggtatttacaagagaggattttgaaagtttccatcacaaagaaatgataaatgtctgaggtgatggttatgcgtattaccctatgccctatagatatgtataattatgtgtcaatttcaaaataaaaattcaaaactacaactcctatgaaaatttttgagcgtgtttgtacttattaagtgtatttataaatcatacggatattatcttcagcctgcatattaaattgtagttaagcttttactttttaactaaaaaataaattctattattttttcctatatcccactgcactgaccccagtttggaaatcctaagattatcaaataaaaactttgattattgaagaatccaggtgtactgccacagaaaagttctattctgtagcatggactctaatatgtaatctagcccattgtgcttacagatagatgtgtgcctgtagtcatagaaaaatttgcatgagctaatgactgccttgctactagattagctcaaagcaaaaagttctctgaaagcaggtcaatagggtcatttttatattatgaagaagaaaagcagctgttgtattacattcactgtattggtcctgcttgtgtttcagggcaagatccttgttgggacaaggaatgctgaaataatcgaagttggagagaaaaatgcagcttgtaatattttagttaacggtcatgtggatgggccaatctggggactagcaacacatccttccagggattttttcctttctgctgcagaagatgggacagtgagactttgggatattgctgataaagtaagtacagataatttttttaaaagaggttacaacttctaaaaagaaaagttggaagttctaaattgctagtacttaaagaactgccagaattctgttgagcattttgaggggaaactggtataatttagaagtacttcacttaatgtttcctatgactctttttttttttttttttaaatgcagaagatgttaaacaaagtgaatttgggacatgctgctcgtactgtgtgttacagccctgaaggggacatggtggctattggaatgaaaaatggagaatttatcattttactagtgagttctctaaaaatatggggaaagaagagagacaggagatgtgcaatccatgatatcaggttagtgaacaaatggaatagagtttctagtatatacttgatttaacttccatttgtaaaattttccatagccttgccttcaaaaagaggtccccagggcctgtagcatttcccgtattataaattgtatgctaaaatatggctgtttgtatactacttaattcttcttgctaaattataaacccactgggcaccaactataatagcaagtactagtaggtaatgtttgatgaattcatgttaacacttagccatgtccattaagttcatcccaccaagaggtatctcccactgtaatacaagagagctatctgcccttcaaaagttgtcaccctggaaaactaaagttgtgatttcaaacatatcttctcttagtaacctcagtttgggaatatgtagttcattaatttaatcaatacctattgattaaatgttccagaatccaaattaatttaaatgtttcttaaacctttgtttttcagtgcttaagcatttttcaacagtggctaccatttacggagtacttccgtgtgatcagtagataagattattgaatctaggtctgtcaaaagcttgtacacttttcatcagtaaaatccttttacaaatgaaaccttcctcagaacttcaatatataaaatagtaacagtggcttcccttagcttttacatgtctctatcgtacctcagtaagactcatgggccatttcaagagactgaattgtcccatatgactccaaagattgctaggcaaatagcatttcactttgtcttttaaataagttcttcaggccgggcgcggtggctcatgcctgtaatcccagcactttgggaggccgaggcaggcagatcacctgaagtcaggagtactcgaccagcctggccaacatagtgaaaccccatctcaactaaaaatacaaaaatcagccgggcgtggtggcaggcgcctgtaatcccagctactcagggggctgaaacaggagaatcgcttgaacccgggaggcggaggttgcgccatcgcactccagcctgggagacaagagcgagacttcgtctcaaaaaaaaaaaattcttcttccaagattcaagttgtgtcatttcaccttaataactggaggttagttaagctgggctgtgttctttgcttaatattaagacaacgttttttccagatggaagaaaactatcttaatgaattgttagcttattaattatgtaatgctaatggcttttaaaagctgagatgttctgactgggtgttgtggctcacacctgtaatcccagtaccttgggaggccaagggggaaggattgcttgaggccaggagtttgggaccatagtgagaccccgcctctatttaaaaaattaaattttgttttgttttgttttgagttggagttttgctcttgttgcccatgctgaagtgcaatggtgcaatctcagctcaccacaacctgtgcctcctgggttcaagcgattctcctgcttcagcctcccgagtagatgggattacaggcgtgcaccaccatgcctggctaattttgtatttttagtagagacagggtttctctatgttggtcaggctggtctcaaactctcgacctcaggtgatctgcccgcctccgcttcccaaagttctgggattataggtgtgagccactgggcctggcctaagaaagtttttttaagccattagacgtttttaaaggaattgggagatgacaattggggaaatatttaaaatttaagtaaaatataaagcttccttatttcatgtaacccagacaatctcagtatacatgatcagttgtgtctgacaggtaaatctatttgaggccttatcacacgttacttttaagaactagaaaggaaaagtcactgatcttaagtatttataatacttcatgtggtctaatactttttacgttttgttttgattcagatttagtccggattcccggtatctggcagtaggttctagtgagaactcagtggatttttatgacctaacgctgggccccactcttaacagaatcagctactgcaaagacattccaagctttgtcattcaaatggacttctctgcagatagcagttatctccaggtacagtaccaatactgtatacccaggtggcaagttcttctgcttttacatttcgtgttagtgaatgcatttaaagttcctgagctccagagctccagcttctcaactcctccctttgtaccttctgacctacagctcccctttcctcccccacttatcagagcttttctcctattaagtttttgtagtgatcttttgcatacttaataatgttagacatgtaaatcaagtagcaatatgctagtattctgtaaaccccctgtggattttgtctctcacctaatggaattcttgtcccattttaatctgatgaaaaaggtctctagtggctgctataaacggcatgtctatgaagtgccttcaggaaaacatcttatggatcatgccgctattgacagaattacttgggctacatggactaggtaaatacttatatattcacaaggcaagaactgactttgaaggccagttagaaaatcctatttctgaactgttagagccattccaataaggaatagtaattgagtttcaagtttttgttaccatattttgaaatggtatgttcatgttgggacccctttttattgaatatatttccatgttttatcagtttccatgatttatcaagttttttttttaaggaaatcaaagttttaactttaaagataccctgatatttttcttaatgctaaatttaatgactggcaaaaaggtattgggtgctgttaagcaactgttattaattctctatctaaaggaatgctatcttgaatctattagaagtcaaagcttccaaatttgttcaaatttcctggctgtatgacaggtaaccatgactatccatttttttggccaatgaaaaatgccatcaaattcctgtatcagccaggcatatagtggctcatgcctgtaatctctgatgtagcaggccgaggtgggaggatcacttgagcctagaagttttgataccagcctgggcaacatagcaagaccccatctctgaaatttttttaattcctatgtcataagtcatttttatttttgtagagatagggatctcacaatattgcccaggctggtctcaaactcttggcctcaagcagtcctcctgcctcagcctcccaaaatgttgggattactggtatgtgctgctggacccagccaagtagcacttttaatttgaaaaatagttctatcagttttcagtcaggcgcggtggctcagcctgtaatcccagcactttgggaggccgagcgggggtgatcacctgaggtcgggagttcgagactagcctgaccaacatggagaaaccctgtctctactaaaaatacaaaataagccgggcatgttagcgcatgcctgtgatcccagctactcgggaggctgaggcaggagaattgcttgaacccaggaggcagaggttgcggtgagccgagatcatgccattgcactccagcctgggtaacaagagcgaaaactccgtctcaaaaaaaaaaaaagaaaaaatagttctatcagttttcataaagtactactttaatcttaaaaagattaatctagaaacccttcaaattataaaatgtcatttttaaaaggcaggagttgatatcctgatgaaattcaggtctccaaacaacttaccataatttacttcctgtattttaagtaacatgatagggtacttagagattaattgccaagaaactttttgaatatagtcaacctgcccgcacttgccatgatgagttttcttttgttccttccctctagtattctaggagatgaggttttgggaatctggtccagacatgctgagaaagctgatgtcaactgtgcctgtgtatctcattcaggaatcagtcttgttacaggagatgactttggcatggttaagttatttgacttcccatgtccagaaaaatttgtaagtttgtgttttgtttactattatcagtttactcctaattttgatgtcttatcatcagcacttttccccatatatttaaaatgttttgtcctaatttctaaatttttccccaaactttctaaatctatttactttgaaataaaagctattagaaacaaatcctctccctcgagtaataccatctttggaaccatcctacaaaagctgtaattagcttttcaccaaacctataatcagttatcaaatttcaaatgcttttccttagagaaaaatggtcagagtacctggagacatctgactgcccacacagcctggttttgcagatccactactcatgctgaaaagcattctaatcactggctgcggtgctaactccctactctctccacagctcttgtcatagagattatagttcctaataagagcctttgacttctgtgtgcaccaaatgccctgagcttgtctgtcattgttttttaggcaaaacacaaaaggttcttgggtcattcgccccatgtgacaaatattcgatttaccagtggtgatcgacatgttgttagtgctggaggtgatgactgcaggttagtaactttctcagcccatgaagagcagactatgttactagttaagagacttaatacaacaactcctacagctttggtttatgaaatcagctagtcaacattagtagaaggtagtataaccagatggctcttcagaatctcatatttatgcaaatacagaataaaaggagttaaagaggaaaaatattacacatgtaacctgaaagcacaactgaaaaatattaaactgttatgaaaatctaaaaacataattaactccctgcaattttcttctctgattgcagcttatttgtctggaaatgtgtacatacacctcactgagagatgctgagatgactacagaaattaactttgagaccagaattacagagaagaaaaaccaaaacccaaccctgcatggtcaagtggtgctaacccaagactgtaacagggagaaatgcccagaatcatcaaaatagtgaaagactgatctgttcaaaatatttgctatatgcactgggtataatccgtaatccatacactgccagataatgccatttcaaggaaggatcgaatacttgatggtaaaggccaagtccccctgtattgggaagtgtgtgatttcggcagacctgctgggaaaatttagggtagagcactctttacagaagaactcaaaaacccaatttggataattttcattatctttttagcaaaatggtttcttaatgtttatattttattttcaaggttcattgtttaatgaaatattttattcttgcatttccataaggaaagggaaagtcatgatcatcctaaaggatcacagtttttaaaaggcaaacattttccctaaggaaacagacacaagctttcctagagaatatgatgttttttaggcattaataaggtccttttttataaaggacacttttctcctagtagttttgaattcaggaacagatccaaagttagcagtatatggctgctacatttccattttcattttcgagccatcagtttatgttcagatgccatctctgtaatcgcacatttaaaacataactgtagcctcactaatggaaaagtagtatgatgaacaatcattcccaatggtgtacaatgtaagggttttagggagcaacagtatttaactggaagaaagaattgcatatttaatgtagtctaatatatacacatttgtttaacatgtaaacaaaagtgttaaattcacatatacaacattatacaatttaatcactcttggaataaaatttttatagccttttttctattgggaaaatttgtttagatgtgtgccactccataggtttatttccaaaatgaatgagcccaactccatttgtaaaaacttgtcagttagaattcctttttttagtggattagggctgaattcttagatccttatttcttttcactttaaatgctgccaaagatcactactcatcattcaggaattcgctgtctagcctatctgtagtttcctgaagattgaaaattatgtagactgctatttaaaaatatatttttctaagtgtgaggtttaagatgctgtattgaccctatgagtttttaatgtgttaattatctttatagcataatagatcgctttaggttcctggaatcccatttggtctgacaggatatatgaagattcttaatacctattttctgtgtctaatacttggttaatactaaaaatagaaatgactaaattacatcacagaaagcataaccagtgattgaacctggtagttttaaagctctaaatagctgtggctgaaggactgattatggggctaagaagcttgaaacgtaagttggtacttgttcatcagtggattctcctaaattaagccaaattttgaaatacatgactattaagtttctactcatgtatttacagtcagtcaataaattaaaggaggaaaaaaatccctgaacaacctgcccataaaaagaaaaatactctacatttgagcctgctgcagttttaaattttccctctgggtcaagtttgccagcttttggctacagagaaattatatttccattacagtgcaggtagaaactctgtaaccttaagcatgtaaactacatagaataaaactgtttccactgcatttctgtccttcaaagtggccaacctgattaagtcagccttaatcactgctgctgtcagtttcacgactaaaggtcatattgactaagtagtcatcagctgaccacctcgctgtatcagccagcaacgaggggaaggtgaagaaacatgataggccatatagaatctgccctatgtttacttttttaacccagataattatttttgtgtgcagtatctaagctcctgattgtgtaacctgggacttctggcaccttttgttccattcattttatgtataaaatgcatgccaaagcacactgtgccctctggtacccttgcttccaatcgccaaccatgctcatttccttcctttttttgtggtccctttttgtggtgatcattttaaaccacgtcatccaacaaatgttttatggtcaaccttagcttgttcataagccatagcaactgaaagattaaactcttaaatatgtgtctgggcagtggctattaaatagcaaaaaacaatcagattttagtattttattatttccttgtaaaatggctgaactaaattaaacccttgtttcccatttgttctataatttatagtgaaactgagaacaaaactatctttataaatgatagctaaaagtatttccagatatttaaacaatttaaaataaatttcttctgcagagatgcaaagcatctcaacactggaatgaacaaatgccttaaattcaatggagtaaacctttagaatgaagaggaactgtcatttcacccaagccgaagacaacagccttatgcacttgtgtgctctgtctttgctgcttctcgtgtttcaagcctttcctgtgggatcagcacagcaaagtgcaacttaccaaatggtttaatgactggttaattctttcttctcccaatggaaaagcaatggcaacacaacagtagactgctggcttgacaatcttaaacgtgagcctttgcacatgtaggtttatcatcatttgagtatacgactaagcaagtcaatgaactttttttttttttttagcagtttaatttggtcctgagaatgttgcagtctttattaccccttttgcattaatccacttttctaaccaccttttaagctttaatttttaacactatacaccaagtctttgaaatcagtgatctgttatttaactctaaagcatttgacacttcttgccttaacagttttaaaaaccacacacaaaaaaactctgtaagtaatacagtaggccaaaagtttcatcctatctatcttgcagtttacctatctgatctgatctctgtaattatagttctgtcatttaaaatatactatttaaatctaatttttacatttcaaaaattatcttcagtagtaactaagtatattttctgtggattctgagaatgttatttttcagaatgtgagaatatatatgtacatttataatcttgtgactttaaagtctgttttcagatacagtatgtaaatacttgtaaaaaaatttgtataattttgtgataatgtagtttcccaaaaaaattatttagaaggcattatgttattagtaaatgagagcactgtatagaactgttcctattttctgcacttgccattccagctgcctccactgtccatacccacctcattcatcctgtcacagaaggcaggaaaactgggaactttaccaaagtagcactcagcctgagaggcctgtataatcatgcttttcaaactaaattcacttaaaaattaaaaagcagaattgaatattttaagcagcctcagtacctttggccaatgctgttttcatggtggattatgaacattatataatctttgggaaaagtgaaagtagtacaatttttagaataatgacaactgcctcactgcatctctccactcacacagcaaccgtgtagccccctaagctgcagtaccatgactaaccatgatgtcaatttcatatgctgatcctcacaacagcagtgcacaaacatgccccaaatattttaacagaatttagctcttccttaagctgtcttttcatagtaaaaacaaaacaaaaacacccaatgttaaaaccacataataaacttacaaacttgaaaaattagacacttcagatagataggcaataaaacttcatattatgaaagcaatatattccaagtttcaaagatttgacaagttctgtagagtatctttcatcagtacatgaaaacttccaaactgcatgatcttctgccaggcaggactgggtgctattcgctggtttgaggtcgaatccatttcaaggcatgtcgtggtgggacattaatggtgggatggtagaatgtgcagtccggtcttgtacattgagtgttaaacctacaatgttttggatgatagaagggacattccatcttcttacaagcagggaagtaacggcagagctgactactggaaggtggtgctggtggtgcaactgctggttttggagacagtactggaattcttctactcacatgagtgaagggacaatctggtttagtacactttgcatcatatttacaatttgggtgaacaaacaaacatttttcagcaaatttacaattggggaaggctttgcagggtgagatggggtgatggtaggcacactcatccccatttttacaagcaggccagtacttgcagcgctccaaaagtttttctggtttctgtgccacactcagttcactcatctcagcgttagaaaagctaccatttgggtcctcaagctgcctgctcagcaagtgcaactgctgtgggtggaggagacctctgagtcccttgtttgaggctgcagtttggtttacgggtttcattccttcaaagcacatgtcctcctcttgatctgacatgtatcctggggggctggggacaccatccagcgtcactataaacttgggacttgcaggtttatctggttgtacaagatctcgtgtctgcataaggtgtcctgaaagtacccgaagggaatctgcagtcttcatccccgactcttggtttggtgccactactacttcctcagacagctttggcttcttcagaataaatgatcttgtgtctgcatggaccatggattccatgtcatagtaatcttgactcatctgcagagtttctgccattactgggtcgatttgcagtcgggataataattgcctctgttgagttccttgatttttttctacagaatctccttttgtttcctcttctttaatggggggacttattctgggggtcctactttgtccctggaccacttctgctagcaattcttcttgagaagttcgagttctgggagcaactggaagtgtctgtttctgtggaactgtagagtagttagttgtttttgttacggattcttgagcttcagatatagccttcaaaatcagattcttgttagcttgtttagaaggtggaagagaaggtctcctttcaggctttgcaggcacagacacactgctggagatgcttcctgttcgagacccgtaatcatcatcttcttcctcctcttctccatcatgattgaatttttttactttaacaactgaacttaccacaggcaactttctcttccgaaagttttcatcctccatactcattttctccgagttgtttctaaagaacggactatacgtttcttctaagctgttaagcacctctggttcacacaaacgtcctgtttcatatacccaactactctgcatatcaagctgcttggcagcatgaatactattctgctgctgttgaaattgcaacctgtttaaatgaacaccactatctgcatttctacttgcaggtggtcgataaatttcaatagaagggcgagaagaaccatatgtaagtgtcactgtaggttttttctgagataagggattctcctgcacaaagttgaggtcttcgtcaatgagatcatctggttctggcttaatatcaatcacatcttcagagggtgctggctccctcaaaggtttcactgttgacattagtcgggttgcagctccatcatcgtaagtctgtctgacatttgtggtttttgactcctgcgaacttgtagaaactctggaatctcttttttcaggtctcgcgctaggaatggcaagtggtggcactgcagcttcatgcctcctctcatctccccgactgaaattgctcttgtttgaaggcacgttactatcaaagatgttggtatcagaagacttcagactagagggttcagttgtaacagagcgaagtttatctaatacaccatgaagccatacggtgaatcgaattgtgttgttccctagaaacagggacagatcctctgtcatttggtcctgacttttcttgttggccaccatcaccataatgtaatcaggaagttcttcatctatttaaaaggaaaggtagatcaaaactttgtttcctcaaaactttcttcttaaagttgatgtgcttgaaaatatagatgtagctctaagctttagagtcgcagagctctactggaattacattggacaagatggcttagctttaatttttttctcttcattccacaggtatttcaaatacaacataagctcctaattcttgtaatttccccttaatggcactccggatcttgcggctgatctcggtgccgatctccatggctctgcggcgtgcgggaactcagcactgcgcggcgcttggcttacccggaggctgccgcggactcctaccccgcagccgggacaccaccgcctcc

SEQ ID NO: 13610 - RNA, 16741 nt, Homo sapiens
  source 1..16741: mol_type = other RNA
gctgggattacaggcatgagccaccataataaggattctgatgaacatttgattccttggactactgttatactcaaaagccttccttaatcttctaattgtcaccctaaatatcctaaaatttctgtcttcctagtagttcttcatagtcctaaaaatttgtcagagagaaaggtaaatcaagaaacatgattttcaaatgatttaaggtggtactagggtttaggatttcctttgctttttatcatttaacacactgcttatcatacagctggaagtgctctgggccagtgtctctacttcgagggaagaaggaggtagtgagacagaaggaaatagcacaattcctggccctgacagaagggtgttcaggagacctgctctcctctcactttattccatctcatctggacctgtggcttccaatccacatctctttcctttaatatcctgcattggctaggctgtataaatcctttggtgcatcgaaaaactaagtgcattttttgtttttgtgattatgcaatacttataggaaaagttataattttagaatatttaagtacacttacatttttgagaaaaagactattgaaatgtttgtgccatgtcaaatttcagttgaacattttgggtattcttaatataagaccaggccaggcaccgtggctcaggccgggcacagtggctcacacctataatcccagcacttagggaggccaaggcgggaagatcacctgaagtcaggagttcaagaccagcctggctaacaaggtgaaactctgtctctactaaaaatacaaaaattagccgggcgtggtggctggcgcttgtaatcccagctacttgggaggctgagacaggagaatcacttgaacctgggaagcagaggttgtggtgagctgagatcgcaccattgcactccagcctgggcaacaaagagcgaaactccgtctcaaaaaaataaaaaataaaccctagaattatagtatgttagaattggaagggaagaattgtctaaggttattctagctaataagcaacagacttggaaaggaaaaggtcctgacaaagctaagcctcccgttcaggtttcctgactcgtgaattcagtgctgctgccactacacgatgcatgctctttgtatcaagggtgagacagcattacacatacatagaaaattatctatttaaactctatttgaacttttgatgagtttgtctccccctcccccactccttttcagaataacttgacgtttacaggtaccatcagtggtgatgtctgtgtgtggaaagatcacatattgtgtagaatcgtggcgagagctcacaacgggcctgtgtttgccatgtacaccaccctgcgagatggacttatcgtgactgggggaaaggaaaggccgtgagtcctctttcttttcacagaatatttatgcatttgtgacctacctgaggtttgcagttaattattctagttgtttctaggctacacagagtgtcctctccgaccttcctcctcatatgcttctcctttattaccttttatgtgccttctatttgattctcatttctggtcttaattcacttccaatttttttcatgttggggtgatactttttctgaggtgtggataggtagttgtcctacaagttgagttacttttcttaatgtctgtatgcctgtgtatgatttgctgagtaggaggcccatgggggaatctggagccagggttgtattttgactgcctgctctctttttgttcagaatggattctaaggagtagaatgcacattgttgctttagaaaaggatgagggaactagagagaactgccttgtttccttttgcttgaggcaaatttaaactgttttatacaagacctcaaaatttgagaagaggtctcttctgagtgattttcaaatctcccaacagtaaccagatacttatgatttgatttgtcaccaacatagtcatatgcatgttgaaacatgacatgtaggccaggcacagtggctcacacctgtaatcttatcactttgggaggctgaggcaggtggatcgcttgagcccaggagttcaagaccagcctgggcaacatggtgaaaccccatcgctataaaaaacaacaattagccgggtgtggtggcacatgcctgtagtccctgctactcaggaggctgaggtgggaggatcacttgagcctggggaggtcaaggctttagtgagctgtgatggtgccactgcactccagcctgggtgacagagtgagaccccatttaaaaaacaaaaacaaaaacaaaaaaaaatgtgacatatagttgactaagaagtacatttcaatacaggattgaaagaacccacatatgttaattaaacacaagcgcagaatttgtgccttttacataaaggaagaatgcacataggcatgctttcagacaagcaattcatctagcagaaaaggaaggaatacatttttcagcccttccaggaataaaatccataaatgggctctatttcgtcctccaacacttgtatttcccacgtcatttactcctgcacacccccactcactagaagcctgctaaactgttccagtgagatattttaacacctgatagggaataaatatgcttctgttttggccttcaaaaataagctctgggccagttgcagtggctcacgcctgtaatcccaacactttgggaggccgaggtgggcggatcacgaggtcaggagtttgggatcagcctggccaatatggtgaaactccatctctactaaaaatacaaaaattagccaggcatggtgcctgtaatcccagctacttgggaggctgaaggagaagaatcgcttgaacctgggaggcacaggttgcagtgagccgagatcacaccactgcactccaggccaggtgacagagcgacactctgtctcaaaaaaataaataaatcaactctgtagcatagcatttgtaattctattattttgccttacatttccattatccttttaataaaattgtttttttacatcttcctaatcaagaagtattatgaggccaggcacagtggctcatacctggaatcccagcactttgggaggccgaggcaggcagatcacctgaggtcaaggtatttgagaccagcctggccaacatggtgaaaccccatctctactaaaaatacagaaattagctgggtgtggtggtgcacacctgtaatgctagctactcgggaggctgaggtaggagaatcgcttgaacctgggaggcagaggttgcaataagcctagatcatgccactgcactcaagcctgggagacagagcgagactacatcttaaaaaaaaaaaaaaaagtattatgagagaggataatgtattgtaatgtattgtagaggctaaataaaattatgctcatgtcagaaaaaaagagtatttctcaaaataaaattcactgaaactggatgtttattttgactgagatatagtatatcctcaaattgccatagaaagtttacaagaatattagaggtaaattataaatatcagggcctttttaaaaaaaaaagattctgcttataacttggtatttgtttataataaaaattatagtagccaataatgaacacttactctggcttggttatttacttaggtcaaaagaaggaggagcggttaaactgtgggatcaggaactgaggcggtgccgtgccttcaggcttgagacaggacaagccacagattgtgttcgttctgtgtgcagaggcaaagtaagatgttccatgagctgatacagtgcagcagaaaacagaaagtggttattactgtgattccctcaccctttgcagcctaatgaacaatacttaataatgcataacgatggatttgcttgccaacattactctgtctttgctgctttctttgccaaagttagcaccagtgtggtgcataagctaggaagctattctgtctaaatactgtatgtaaacctccaatattttctagaatctgccaatttaacaactctagtagacataattgaaagcccttggcagttgactcatattaggacagctgtctccattttttaaaaaaacacacattccctagataaaacgtgcagtaaacaaacaatgaaatactactcagccataaaaaataatgaaattctgtcattcttggtggcaacatggatgagactggaggacatgatgtgaagtgaaataagccaggcacagaaagataaatacatgttctcactcctgtgcagaaactaaaaaagttgatcccacagaggtggagagtagaatagtggttactggaggcggacaagggggagggggagggggatagggaaggactggttaaaggatacaagtttacacagccagataggaatagtatgttttagtattctgtagtactgtaggatgactatagttaagaatcacgtatttatgtattttcaggtatttacaagagaggattttgaaagtttccatcacaaagaaatgataaatgtctgaggtgatggttatgcgtattaccctatgccctatagatatgtataattatgtgtcaatttcaaaataaaaattcaaaactacaactcctatgaaaatttttgagcgtgtttgtacttattaagtgtatttataaatcatacggatattatcttcagcctgcatattaaattgtagttaagcttttactttttaactaaaaaataaattctattattttttcctatatcccactgcactgaccccagtttggaaatcctaagattatcaaataaaaactttgattattgaagaatccaggtgtactgccacagaaaagttctattctgtagcatggactctaatatgtaatctagcccattgtgcttacagatagatgtgtgcctgtagtcatagaaaaatttgcatgagctaatgactgccttgctactagattagctcaaagcaaaaagttctctgaaagcaggtcaatagggtcatttttatattatgaagaagaaaagcagctgttgtattacattcactgtattggtcctgcttgtgtttcagggcaagatccttgttgggacaaggaatgctgaaataatcgaagttggagagaaaaatgcagcttgtaatattttagttaacggtcatgtggatgggccaatctggggactagcaacacatccttccagggattttttcctttctgctgcagaagatgggacagtgagactttgggatattgctgataaagtaagtacagataatttttttaaaagaggttacaacttctaaaaagaaaagttggaagttctaaattgctagtacttaaagaactgccagaattctgttgagcattttgaggggaaactggtataatttagaagtacttcacttaatgtttcctatgactctttttttttttttttttaaatgcagaagatgttaaacaaagtgaatttgggacatgctgctcgtactgtgtgttacagccctgaaggggacatggtggctattggaatgaaaaatggagaatttatcattttactagtgagttctctaaaaatatggggaaagaagagagacaggagatgtgcaatccatgatatcaggttagtgaacaaatggaatagagtttctagtatatacttgatttaacttccatttgtaaaattttccatagccttgccttcaaaaagaggtccccagggcctgtagcatttcccgtattataaattgtatgctaaaatatggctgtttgtatactacttaattcttcttgctaaattataaacccactgggcaccaactataatagcaagtactagtaggtaatgtttgatgaattcatgttaacacttagccatgtccattaagttcatcccaccaagaggtatctcccactgtaatacaagagagctatctgcccttcaaaagttgtcaccctggaaaactaaagttgtgatttcaaacatatcttctcttagtaacctcagtttgggaatatgtagttcattaatttaatcaatacctattgattaaatgttccagaatccaaattaatttaaatgtttcttaaacctttgtttttcagtgcttaagcatttttcaacagtggctaccatttacggagtacttccgtgtgatcagtagataagattattgaatctaggtctgtcaaaagcttgtacacttttcatcagtaaaatccttttacaaatgaaaccttcctcagaacttcaatatataaaatagtaacagtggcttcccttagcttttacatgtctctatcgtacctcagtaagactcatgggccatttcaagagactgaattgtcccatatgactccaaagattgctaggcaaatagcatttcactttgtcttttaaataagttcttcaggccgggcgcggtggctcatgcctgtaatcccagcactttgggaggccgaggcaggcagatcacctgaagtcaggagtactcgaccagcctggccaacatagtgaaaccccatctcaactaaaaatacaaaaatcagccgggcgtggtggcaggcgcctgtaatcccagctactcagggggctgaaacaggagaatcgcttgaacccgggaggcggaggttgcgccatcgcactccagcctgggagacaagagcgagacttcgtctcaaaaaaaaaaaattcttcttccaagattcaagttgtgtcatttcaccttaataactggaggttagttaagctgggctgtgttctttgcttaatattaagacaacgttttttccagatggaagaaaactatcttaatgaattgttagcttattaattatgtaatgctaatggcttttaaaagctgagatgttctgactgggtgttgtggctcacacctgtaatcccagtaccttgggaggccaagggggaaggattgcttgaggccaggagtttgggaccatagtgagaccccgcctctatttaaaaaattaaattttgttttgttttgttttgagttggagttttgctcttgttgcccatgctgaagtgcaatggtgcaatctcagctcaccacaacctgtgcctcctgggttcaagcgattctcctgcttcagcctcccgagtagatgggattacaggcgtgcaccaccatgcctggctaattttgtatttttagtagagacagggtttctctatgttggtcaggctggtctcaaactctcgacctcaggtgatctgcccgcctccgcttcccaaagttctgggattataggtgtgagccactgggcctggcctaagaaagtttttttaagccattagacgtttttaaaggaattgggagatgacaattggggaaatatttaaaatttaagtaaaatataaagcttccttatttcatgtaacccagacaatctcagtatacatgatcagttgtgtctgacaggtaaatctatttgaggccttatcacacgttacttttaagaactagaaaggaaaagtcactgatcttaagtatttataatacttcatgtggtctaatactttttacgttttgttttgattcagatttagtccggattcccggtatctggcagtaggttctagtgagaactcagtggatttttatgacctaacgctgggccccactcttaacagaatcagctactgcaaagacattccaagctttgtcattcaaatggacttctctgcagatagcagttatctccaggtacagtaccaatactgtatacccaggtggcaagttcttctgcttttacatttcgtgttagtgaatgcatttaaagttcctgagctccagagctccagcttctcaactcctccctttgtaccttctgacctacagctcccctttcctcccccacttatcagagcttttctcctattaagtttttgtagtgatcttttgcatacttaataatgttagacatgtaaatcaagtagcaatatgctagtattctgtaaaccccctgtggattttgtctctcacctaatggaattcttgtcccattttaatctgatgaaaaaggtctctagtggctgctataaacggcatgtctatgaagtgccttcaggaaaacatcttatggatcatgccgctattgacagaattacttgggctacatggactaggtaaatacttatatattcacaaggcaagaactgactttgaaggccagttagaaaatcctatttctgaactgttagagccattccaataaggaatagtaattgagtttcaagtttttgttaccatattttgaaatggtatgttcatgttgggacccctttttattgaatatatttccatgttttatcagtttccatgatttatcaagttttttttttaaggaaatcaaagttttaactttaaagataccctgatatttttcttaatgctaaatttaatgactggcaaaaaggtattgggtgctgttaagcaactgttattaattctctatctaaaggaatgctatcttgaatctattagaagtcaaagcttccaaatttgttcaaatttcctggctgtatgacaggtaaccatgactatccatttttttggccaatgaaaaatgccatcaaattcctgtatcagccaggcatatagtggctcatgcctgtaatctctgatgtagcaggccgaggtgggaggatcacttgagcctagaagttttgataccagcctgggcaacatagcaagaccccatctctgaaatttttttaattcctatgtcataagtcatttttatttttgtagagatagggatctcacaatattgcccaggctggtctcaaactcttggcctcaagcagtcctcctgcctcagcctcccaaaatgttgggattactggtatgtgctgctggacccagccaagtagcacttttaatttgaaaaatagttctatcagttttcagtcaggcgcggtggctcagcctgtaatcccagcactttgggaggccgagcgggggtgatcacctgaggtcgggagttcgagactagcctgaccaacatggagaaaccctgtctctactaaaaatacaaaataagccgggcatgttagcgcatgcctgtgatcccagctactcgggaggctgaggcaggagaattgcttgaacccaggaggcagaggttgcggtgagccgagatcatgccattgcactccagcctgggtaacaagagcgaaaactccgtctcaaaaaaaaaaaaagaaaaaatagttctatcagttttcataaagtactactttaatcttaaaaagattaatctagaaacccttcaaattataaaatgtcatttttaaaaggcaggagttgatatcctgatgaaattcaggtctccaaacaacttaccataatttacttcctgtattttaagtaacatgatagggtacttagagattaattgccaagaaactttttgaatatagtcaacctgcccgcacttgccatgatgagttttcttttgttccttccctctagtattctaggagatgaggttttgggaatctggtccagacatgctgagaaagctgatgtcaactgtgcctgtgtatctcattcaggaatcagtcttgttacaggagatgactttggcatggttaagttatttgacttcccatgtccagaaaaatttgtaagtttgtgttttgtttactattatcagtttactcctaattttgatgtcttatcatcagcacttttccccatatatttaaaatgttttgtcctaatttctaaatttttccccaaactttctaaatctatttactttgaaataaaagctattagaaacaaatcctctccctcgagtaataccatctttggaaccatcctacaaaagctgtaattagcttttcaccaaacctataatcagttatcaaatttcaaatgcttttccttagagaaaaatggtcagagtacctggagacatctgactgcccacacagcctggttttgcagatccactactcatgctgaaaagcattctaatcactggctgcggtgctaactccctactctctccacagctcttgtcatagagattatagttcctaataagagcctttgacttctgtgtgcaccaaatgccctgagcttgtctgtcattgttttttaggcaaaacacaaaaggttcttgggtcattcgccccatgtgacaaatattcgatttaccagtggtgatcgacatgttgttagtgctggaggtgatgactgcaggttagtaactttctcagcccatgaagagcagactatgttactagttaagagacttaatacaacaactcctacagctttggtttatgaaatcagctagtcaacattagtagaaggtagtataaccagatggctcttcagaatctcatatttatgcaaatacagaataaaaggagttaaagaggaaaaatattacacatgtaacctgaaagcacaactgaaaaatattaaactgttatgaaaatctaaaaacataattaactccctgcaattttcttctctgattgcagcttatttgtctggaaatgtgtacatacacctcactgagagatgctgagatgactacagaaattaactttgagaccagaattacagagaagaaaaaccaaaacccaaccctgcatggtcaagtggtgctaacccaagactgtaacagggagaaatgcccagaatcatcaaaatagtgaaagactgatctgttcaaaatatttgctatatgcactgggtataatccgtaatccatacactgccagataatgccatttcaaggaaggatcgaatacttgatggtaaaggccaagtccccctgtattgggaagtgtgtgatttcggcagacctgctgggaaaatttagggtagagcactctttacagaagaactcaaaaacccaatttggataattttcattatctttttagcaaaatggtttcttaatgtttatattttattttcaaggttcattgtttaatgaaatattttattcttgcatttccataaggaaagggaaagtcatgatcatcctaaaggatcacagtttttaaaaggcaaacattttccctaaggaaacagacacaagctttcctagagaatatgatgttttttaggcattaataaggtccttttttataaaggacacttttctcctagtagttttgaattcaggaacagatccaaagttagcagtatatggctgctacatttccattttcattttcgagccatcagtttatgttcagatgccatctctgtaatcgcacatttaaaacataactgtagcctcactaatggaaaagtagtatgatgaacaatcattcccaatggtgtacaatgtaagggttttagggagcaacagtatttaactggaagaaagaattgcatatttaatgtagtctaatatatacacatttgtttaacatgtaaacaaaagtgttaaattcacatatacaacattatacaatttaatcactcttggaataaaatttttatagccttttttctattgggaaaatttgtttagatgtgtgccactccataggtttatttccaaaatgaatgagcccaactccatttgtaaaaacttgtcagttagaattcctttttttagtggattagggctgaattcttagatccttatttcttttcactttaaatgctgccaaagatcactactcatcattcaggaattcgctgtctagcctatctgtagtttcctgaagattgaaaattatgtagactgctatttaaaaatatatttttctaagtgtgaggtttaagatgctgtattgaccctatgagtttttaatgtgttaattatctttatagcataatagatcgctttaggttcctggaatcccatttggtctgacaggatatatgaagattcttaatacctattttctgtgtctaatacttggttaatactaaaaatagaaatgactaaattacatcacagaaagcataaccagtgattgaacctggtagttttaaagctctaaatagctgtggctgaaggactgattatggggctaagaagcttgaaacgtaagttggtacttgttcatcagtggattctcctaaattaagccaaattttgaaatacatgactattaagtttctactcatgtatttacagtcagtcaataaattaaaggaggaaaaaaatccctgaacaacctgcccataaaaagaaaaatactctacatttgagcctgctgcagttttaaattttccctctgggtcaagtttgccagcttttggctacagagaaattatatttccattacagtgcaggtagaaactctgtaaccttaagcatgtaaactacatagaataaaactgtttccactgcatttctgtccttcaaagtggccaacctgattaagtcagccttaatcactgctgctgtcagtttcacgactaaaggtcatattgactaagtagtcatcagctgaccacctcgctgtatcagccagcaacgaggggaaggtgaagaaacatgataggccatatagaatctgccctatgtttacttttttaacccagataattatttttgtgtgcagtatctaagctcctgattgtgtaacctgggacttctggcaccttttgttccattcattttatgtataaaatgcatgccaaagcacactgtgccctctggtacccttgcttccaatcgccaaccatgctcatttccttcctttttttgtggtccctttttgtggtgatcattttaaaccacgtcatccaacaaatgttttatggtcaaccttagcttgttcataagccatagcaactgaaagattaaactcttaaatatgtgtctgggcagtggctattaaatagcaaaaaacaatcagattttagtattttattatttccttgtaaaatggctgaactaaattaaacccttgtttcccatttgttctataatttatagtgaaactgagaacaaaactatctttataaatgatagctaaaagtatttccagatatttaaacaatttaaaataaatttcttctgcagagatgcaaagcatctcaacactggaatgaacaaatgccttaaattcaatggagtaaacctttagaatgaagaggaactgtcatttcacccaagccgaagacaacagccttatgcacttgtgtgctctgtctttgctgcttctcgtgtttcaagcctttcctgtgggatcagcacagcaaagtgcaacttaccaaatggtttaatgactggttaattctttcttctcccaatggaaaagcaatggcaacacaacagtagactgctggcttgacaatcttaaacgtgagcctttgcacatgtaggtttatcatcatttgagtatacgactaagcaagtcaatgaactttttttttttttttagcagtttaatttggtcctgagaatgttgcagtctttattaccccttttgcattaatccacttttctaaccaccttttaagctttaatttttaacactatacaccaagtctttgaaatcagtgatctgttatttaactctaaagcatttgacacttcttgccttaacagttttaaaaaccacacacaaaaaaactctgtaagtaatacagtaggccaaaagtttcatcctatctatcttgcagtttacctatctgatctgatctctgtaattatagttctgtcatttaaaatatactatttaaatctaatttttacatttcaaaaattatcttcagtagtaactaagtatattttctgtggattctgagaatgttatttttcagaatgtgagaatatatatgtacatttataatcttgtgactttaaagtctgttttcagatacagtatgtaaatacttgtaaaaaaatttgtataattttgtgataatgtagtttcccaaaaaaattatttagaaggcattatgttattagtaaatgagagcactgtatagaactgttcctattttctgcacttgccattccagctgcctccactgtccatacccacctcattcatcctgtcacagaaggcaggaaaactgggaactttaccaaagtagcactcagcctgagaggcctgtataatcatgcttttcaaactaaattcacttaaaaattaaaaagcagaattgaatattttaagcagcctcagtacctttggccaatgctgttttcatggtggattatgaacattatataatctttgggaaaagtgaaagtagtacaatttttagaataatgacaactgcctcactgcatctctccactcacacagcaaccgtgtagccccctaagctgcagtaccatgactaaccatgatgtcaatttcatatgctgatcctcacaacagcagtgcacaaacatgccccaaatattttaacagaatttagctcttccttaagctgtcttttcatagtaaaaacaaaacaaaaacacccaatgttaaaaccacataataaacttacaaacttgaaaaattagacacttcagatagataggcaataaaacttcatattatgaaagcaatatattccaagtttcaaagatttgacaagttctgtagagtatctttcatcagtacatgaaaacttccaaactgcatgatcttctgccaggcaggactgggtgctattcgctggtttgaggtcgaatccatttcaaggcatgtcgtggtgggacattaatggtgggatggtagaatgtgcagtccggtcttgtacattgagtgttaaacctacaatgttttggatgatagaagggacattccatcttcttacaagcagggaagtaacggcagagctgactactggaaggtggtgctggtggtgcaactgctggttttggagacagtactggaattcttctactcacatgagtgaagggacaatctggtttagtacactttgcatcatatttacaatttgggtgaacaaacaaacatttttcagcaaatttacaattggggaaggctttgcagggtgagatggggtgatggtaggcacactcatccccatttttacaagcaggccagtacttgcagcgctccaaaagtttttctggtttctgtgccacactcagttcactcatctcagcgttagaaaagctaccatttgggtcctcaagctgcctgctcagcaagtgcaactgctgtgggtggaggagacctctgagtcccttgtttgaggctgcagtttggtttacgggtttcattccttcaaagcacatgtcctcctcttgatctgacatgtatcctggggggctggggacaccatccagcgtcactataaacttgggacttgcaggtttatctggttgtacaagatctcgtgtctgcataaggtgtcctgaaagtacccgaagggaatctgcagtcttcatccccgactcttggtttggtgccactactacttcctcagacagctttggcttcttcagaataaatgatcttgtgtctgcatggaccatggattccatgtcatagtaatcttgatttttttctacagaatctccttttgtttcctcttctttaatggggggacttattctgggggtcctactttgtccctggaccacttctgctagcaattcttcttgagaagttcgagttctgggagcaactggaagtgtctgtttctgtggaactgtagagtagttagttgtttttgttacggattcttgagcttcagatatagccttcaaaatcagattcttgttagcttgtttagaaggtggaagagaaggtctcctttcaggctttgcaggcacagacacactgctggagatgcttcctgttcgagacccgtaatcatcatcttcttcctcctcttctccatcatgattgaatttttttactttaacaactgaacttaccacaggcaactttctcttccgaaagttttcatcctccatactcattttctccgagttgtttctaaagaacggactatacgtttcttctaagctgttaagcacctctggttcacacaaacgtcctgtttcatatacccaactactctgcatatcaagctgcttggcagcatgaatactattctgctgctgttgaaattgcaacctgtttaaatgaacaccactatctgcatttctacttgcaggtggtcgataaatttcaatagaagggcgagaagaaccatatgtaagtgtcactgtaggttttttctgagataagggattctcctgcacaaagttgaggtcttcgtcaatgagatcatctggttctggcttaatatcaatcacatcttcagagggtgctggctccctcaaaggtttcactgttgacattagtcgggttgcagctccatcatcgtaagtctgtctgacatttgtggtttttgactcctgcgaacttgtagaaactctggaatctcttttttcaggtctcgcgctaggaatggcaagtggtggcactgcagcttcatgcctcctctcatctccccgactgaaattgctcttgtttgaaggcacgttactatcaaagatgttggtatcagaagacttcagactagagggttcagttgtaacagagcgaagtttatctaatacaccatgaagccaacataagctcctaattcttgtaatttccccttaatggcactccggatcttgcggctgatctcggtgccgatctccatggctctgcggcgtgcgggaactcagcactgcgcggcgcttggcttacccggaggctgccgcggactcctaccccgcagccgggacaccaccgcctcc

SEQ ID NO: 13611 - RNA, 16856 nt, Homo sapiens
  source 1..16856: mol_type = other RNA
gctgggattacaggcatgagccaccataataaggattctgatgaacatttgattccttggactactgttatactcaaaagccttccttaatcttctaattgtcaccctaaatatcctaaaatttctgtcttcctagtagttcttcatagtcctaaaaatttgtcagagagaaaggtaaatcaagaaacatgattttcaaatgatttaaggtggtactagggtttaggatttcctttgctttttatcatttaacacactgcttatcatacagctggaagtgctctgggccagtgtctctacttcgagggaagaaggaggtagtgagacagaaggaaatagcacaattcctggccctgacagaagggtgttcaggagacctgctctcctctcactttattccatctcatctggacctgtggcttccaatccacatctctttcctttaatatcctgcattggctaggctgtataaatcctttggtgcatcgaaaaactaagtgcattttttgtttttgtgattatgcaatacttataggaaaagttataattttagaatatttaagtacacttacatttttgagaaaaagactattgaaatgtttgtgccatgtcaaatttcagttgaacattttgggtattcttaatataagaccaggccaggcaccgtggctcaggccgggcacagtggctcacacctataatcccagcacttagggaggccaaggcgggaagatcacctgaagtcaggagttcaagaccagcctggctaacaaggtgaaactctgtctctactaaaaatacaaaaattagccgggcgtggtggctggcgcttgtaatcccagctacttgggaggctgagacaggagaatcacttgaacctgggaagcagaggttgtggtgagctgagatcgcaccattgcactccagcctgggcaacaaagagcgaaactccgtctcaaaaaaataaaaaataaaccctagaattatagtatgttagaattggaagggaagaattgtctaaggttattctagctaataagcaacagacttggaaaggaaaaggtcctgacaaagctaagcctcccgttcaggtttcctgactcgtgaattcagtgctgctgccactacacgatgcatgctctttgtatcaagggtgagacagcattacacatacatagaaaattatctatttaaactctatttgaacttttgatgagtttgtctccccctcccccactccttttcagaataacttgacgtttacaggtaccatcagtggtgatgtctgtgtgtggaaagatcacatattgtgtagaatcgtggcgagagctcacaacgggcctgtgtttgccatgtacaccaccctgcgagatggacttatcgtgactgggggaaaggaaaggccgtgagtcctctttcttttcacagaatatttatgcatttgtgacctacctgaggtttgcagttaattattctagttgtttctaggctacacagagtgtcctctccgaccttcctcctcatatgcttctcctttattaccttttatgtgccttctatttgattctcatttctggtcttaattcacttccaatttttttcatgttggggtgatactttttctgaggtgtggataggtagttgtcctacaagttgagttacttttcttaatgtctgtatgcctgtgtatgatttgctgagtaggaggcccatgggggaatctggagccagggttgtattttgactgcctgctctctttttgttcagaatggattctaaggagtagaatgcacattgttgctttagaaaaggatgagggaactagagagaactgccttgtttccttttgcttgaggcaaatttaaactgttttatacaagacctcaaaatttgagaagaggtctcttctgagtgattttcaaatctcccaacagtaaccagatacttatgatttgatttgtcaccaacatagtcatatgcatgttgaaacatgacatgtaggccaggcacagtggctcacacctgtaatcttatcactttgggaggctgaggcaggtggatcgcttgagcccaggagttcaagaccagcctgggcaacatggtgaaaccccatcgctataaaaaacaacaattagccgggtgtggtggcacatgcctgtagtccctgctactcaggaggctgaggtgggaggatcacttgagcctggggaggtcaaggctttagtgagctgtgatggtgccactgcactccagcctgggtgacagagtgagaccccatttaaaaaacaaaaacaaaaacaaaaaaaaatgtgacatatagttgactaagaagtacatttcaatacaggattgaaagaacccacatatgttaattaaacacaagcgcagaatttgtgccttttacataaaggaagaatgcacataggcatgctttcagacaagcaattcatctagcagaaaaggaaggaatacatttttcagcccttccaggaataaaatccataaatgggctctatttcgtcctccaacacttgtatttcccacgtcatttactcctgcacacccccactcactagaagcctgctaaactgttccagtgagatattttaacacctgatagggaataaatatgcttctgttttggccttcaaaaataagctctgggccagttgcagtggctcacgcctgtaatcccaacactttgggaggccgaggtgggcggatcacgaggtcaggagtttgggatcagcctggccaatatggtgaaactccatctctactaaaaatacaaaaattagccaggcatggtgcctgtaatcccagctacttgggaggctgaaggagaagaatcgcttgaacctgggaggcacaggttgcagtgagccgagatcacaccactgcactccaggccaggtgacagagcgacactctgtctcaaaaaaataaataaatcaactctgtagcatagcatttgtaattctattattttgccttacatttccattatccttttaataaaattgtttttttacatcttcctaatcaagaagtattatgaggccaggcacagtggctcatacctggaatcccagcactttgggaggccgaggcaggcagatcacctgaggtcaaggtatttgagaccagcctggccaacatggtgaaaccccatctctactaaaaatacagaaattagctgggtgtggtggtgcacacctgtaatgctagctactcgggaggctgaggtaggagaatcgcttgaacctgggaggcagaggttgcaataagcctagatcatgccactgcactcaagcctgggagacagagcgagactacatcttaaaaaaaaaaaaaaaagtattatgagagaggataatgtattgtaatgtattgtagaggctaaataaaattatgctcatgtcagaaaaaaagagtatttctcaaaataaaattcactgaaactggatgtttattttgactgagatatagtatatcctcaaattgccatagaaagtttacaagaatattagaggtaaattataaatatcagggcctttttaaaaaaaaaagattctgcttataacttggtatttgtttataataaaaattatagtagccaataatgaacacttactctggcttggttatttacttaggtcaaaagaaggaggagcggttaaactgtgggatcaggaactgaggcggtgccgtgccttcaggcttgagacaggacaagccacagattgtgttcgttctgtgtgcagaggcaaagtaagatgttccatgagctgatacagtgcagcagaaaacagaaagtggttattactgtgattccctcaccctttgcagcctaatgaacaatacttaataatgcataacgatggatttgcttgccaacattactctgtctttgctgctttctttgccaaagttagcaccagtgtggtgcataagctaggaagctattctgtctaaatactgtatgtaaacctccaatattttctagaatctgccaatttaacaactctagtagacataattgaaagcccttggcagttgactcatattaggacagctgtctccattttttaaaaaaacacacattccctagataaaacgtgcagtaaacaaacaatgaaatactactcagccataaaaaataatgaaattctgtcattcttggtggcaacatggatgagactggaggacatgatgtgaagtgaaataagccaggcacagaaagataaatacatgttctcactcctgtgcagaaactaaaaaagttgatcccacagaggtggagagtagaatagtggttactggaggcggacaagggggagggggagggggatagggaaggactggttaaaggatacaagtttacacagccagataggaatagtatgttttagtattctgtagtactgtaggatgactatagttaagaatcacgtatttatgtattttcaggtatttacaagagaggattttgaaagtttccatcacaaagaaatgataaatgtctgaggtgatggttatgcgtattaccctatgccctatagatatgtataattatgtgtcaatttcaaaataaaaattcaaaactacaactcctatgaaaatttttgagcgtgtttgtacttattaagtgtatttataaatcatacggatattatcttcagcctgcatattaaattgtagttaagcttttactttttaactaaaaaataaattctattattttttcctatatcccactgcactgaccccagtttggaaatcctaagattatcaaataaaaactttgattattgaagaatccaggtgtactgccacagaaaagttctattctgtagcatggactctaatatgtaatctagcccattgtgcttacagatagatgtgtgcctgtagtcatagaaaaatttgcatgagctaatgactgccttgctactagattagctcaaagcaaaaagttctctgaaagcaggtcaatagggtcatttttatattatgaagaagaaaagcagctgttgtattacattcactgtattggtcctgcttgtgtttcagggcaagatccttgttgggacaaggaatgctgaaataatcgaagttggagagaaaaatgcagcttgtaatattttagttaacggtcatgtggatgggccaatctggggactagcaacacatccttccagggattttttcctttctgctgcagaagatgggacagtgagactttgggatattgctgataaagtaagtacagataatttttttaaaagaggttacaacttctaaaaagaaaagttggaagttctaaattgctagtacttaaagaactgccagaattctgttgagcattttgaggggaaactggtataatttagaagtacttcacttaatgtttcctatgactctttttttttttttttttaaatgcagaagatgttaaacaaagtgaatttgggacatgctgctcgtactgtgtgttacagccctgaaggggacatggtggctattggaatgaaaaatggagaatttatcattttactagtgagttctctaaaaatatggggaaagaagagagacaggagatgtgcaatccatgatatcaggttagtgaacaaatggaatagagtttctagtatatacttgatttaacttccatttgtaaaattttccatagccttgccttcaaaaagaggtccccagggcctgtagcatttcccgtattataaattgtatgctaaaatatggctgtttgtatactacttaattcttcttgctaaattataaacccactgggcaccaactataatagcaagtactagtaggtaatgtttgatgaattcatgttaacacttagccatgtccattaagttcatcccaccaagaggtatctcccactgtaatacaagagagctatctgcccttcaaaagttgtcaccctggaaaactaaagttgtgatttcaaacatatcttctcttagtaacctcagtttgggaatatgtagttcattaatttaatcaatacctattgattaaatgttccagaatccaaattaatttaaatgtttcttaaacctttgtttttcagtgcttaagcatttttcaacagtggctaccatttacggagtacttccgtgtgatcagtagataagattattgaatctaggtctgtcaaaagcttgtacacttttcatcagtaaaatccttttacaaatgaaaccttcctcagaacttcaatatataaaatagtaacagtggcttcccttagcttttacatgtctctatcgtacctcagtaagactcatgggccatttcaagagactgaattgtcccatatgactccaaagattgctaggcaaatagcatttcactttgtcttttaaataagttcttcaggccgggcgcggtggctcatgcctgtaatcccagcactttgggaggccgaggcaggcagatcacctgaagtcaggagtactcgaccagcctggccaacatagtgaaaccccatctcaactaaaaatacaaaaatcagccgggcgtggtggcaggcgcctgtaatcccagctactcagggggctgaaacaggagaatcgcttgaacccgggaggcggaggttgcgccatcgcactccagcctgggagacaagagcgagacttcgtctcaaaaaaaaaaaattcttcttccaagattcaagttgtgtcatttcaccttaataactggaggttagttaagctgggctgtgttctttgcttaatattaagacaacgttttttccagatggaagaaaactatcttaatgaattgttagcttattaattatgtaatgctaatggcttttaaaagctgagatgttctgactgggtgttgtggctcacacctgtaatcccagtaccttgggaggccaagggggaaggattgcttgaggccaggagtttgggaccatagtgagaccccgcctctatttaaaaaattaaattttgttttgttttgttttgagttggagttttgctcttgttgcccatgctgaagtgcaatggtgcaatctcagctcaccacaacctgtgcctcctgggttcaagcgattctcctgcttcagcctcccgagtagatgggattacaggcgtgcaccaccatgcctggctaattttgtatttttagtagagacagggtttctctatgttggtcaggctggtctcaaactctcgacctcaggtgatctgcccgcctccgcttcccaaagttctgggattataggtgtgagccactgggcctggcctaagaaagtttttttaagccattagacgtttttaaaggaattgggagatgacaattggggaaatatttaaaatttaagtaaaatataaagcttccttatttcatgtaacccagacaatctcagtatacatgatcagttgtgtctgacaggtaaatctatttgaggccttatcacacgttacttttaagaactagaaaggaaaagtcactgatcttaagtatttataatacttcatgtggtctaatactttttacgttttgttttgattcagatttagtccggattcccggtatctggcagtaggttctagtgagaactcagtggatttttatgacctaacgctgggccccactcttaacagaatcagctactgcaaagacattccaagctttgtcattcaaatggacttctctgcagatagcagttatctccaggtacagtaccaatactgtatacccaggtggcaagttcttctgcttttacatttcgtgttagtgaatgcatttaaagttcctgagctccagagctccagcttctcaactcctccctttgtaccttctgacctacagctcccctttcctcccccacttatcagagcttttctcctattaagtttttgtagtgatcttttgcatacttaataatgttagacatgtaaatcaagtagcaatatgctagtattctgtaaaccccctgtggattttgtctctcacctaatggaattcttgtcccattttaatctgatgaaaaaggtctctagtggctgctataaacggcatgtctatgaagtgccttcaggaaaacatcttatggatcatgccgctattgacagaattacttgggctacatggactaggtaaatacttatatattcacaaggcaagaactgactttgaaggccagttagaaaatcctatttctgaactgttagagccattccaataaggaatagtaattgagtttcaagtttttgttaccatattttgaaatggtatgttcatgttgggacccctttttattgaatatatttccatgttttatcagtttccatgatttatcaagttttttttttaaggaaatcaaagttttaactttaaagataccctgatatttttcttaatgctaaatttaatgactggcaaaaaggtattgggtgctgttaagcaactgttattaattctctatctaaaggaatgctatcttgaatctattagaagtcaaagcttccaaatttgttcaaatttcctggctgtatgacaggtaaccatgactatccatttttttggccaatgaaaaatgccatcaaattcctgtatcagccaggcatatagtggctcatgcctgtaatctctgatgtagcaggccgaggtgggaggatcacttgagcctagaagttttgataccagcctgggcaacatagcaagaccccatctctgaaatttttttaattcctatgtcataagtcatttttatttttgtagagatagggatctcacaatattgcccaggctggtctcaaactcttggcctcaagcagtcctcctgcctcagcctcccaaaatgttgggattactggtatgtgctgctggacccagccaagtagcacttttaatttgaaaaatagttctatcagttttcagtcaggcgcggtggctcagcctgtaatcccagcactttgggaggccgagcgggggtgatcacctgaggtcgggagttcgagactagcctgaccaacatggagaaaccctgtctctactaaaaatacaaaataagccgggcatgttagcgcatgcctgtgatcccagctactcgggaggctgaggcaggagaattgcttgaacccaggaggcagaggttgcggtgagccgagatcatgccattgcactccagcctgggtaacaagagcgaaaactccgtctcaaaaaaaaaaaaagaaaaaatagttctatcagttttcataaagtactactttaatcttaaaaagattaatctagaaacccttcaaattataaaatgtcatttttaaaaggcaggagttgatatcctgatgaaattcaggtctccaaacaacttaccataatttacttcctgtattttaagtaacatgatagggtacttagagattaattgccaagaaactttttgaatatagtcaacctgcccgcacttgccatgatgagttttcttttgttccttccctctagtattctaggagatgaggttttgggaatctggtccagacatgctgagaaagctgatgtcaactgtgcctgtgtatctcattcaggaatcagtcttgttacaggagatgactttggcatggttaagttatttgacttcccatgtccagaaaaatttgtaagtttgtgttttgtttactattatcagtttactcctaattttgatgtcttatcatcagcacttttccccatatatttaaaatgttttgtcctaatttctaaatttttccccaaactttctaaatctatttactttgaaataaaagctattagaaacaaatcctctccctcgagtaataccatctttggaaccatcctacaaaagctgtaattagcttttcaccaaacctataatcagttatcaaatttcaaatgcttttccttagagaaaaatggtcagagtacctggagacatctgactgcccacacagcctggttttgcagatccactactcatgctgaaaagcattctaatcactggctgcggtgctaactccctactctctccacagctcttgtcatagagattatagttcctaataagagcctttgacttctgtgtgcaccaaatgccctgagcttgtctgtcattgttttttaggcaaaacacaaaaggttcttgggtcattcgccccatgtgacaaatattcgatttaccagtggtgatcgacatgttgttagtgctggaggtgatgactgcaggttagtaactttctcagcccatgaagagcagactatgttactagttaagagacttaatacaacaactcctacagctttggtttatgaaatcagctagtcaacattagtagaaggtagtataaccagatggctcttcagaatctcatatttatgcaaatacagaataaaaggagttaaagaggaaaaatattacacatgtaacctgaaagcacaactgaaaaatattaaactgttatgaaaatctaaaaacataattaactccctgcaattttcttctctgattgcagcttatttgtctggaaatgtgtacatacacctcactgagagatgctgagatgactacagaaattaactttgagaccagaattacagagaagaaaaaccaaaacccaaccctgcatggtcaagtggtgctaacccaagactgtaacagggagaaatgcccagaatcatcaaaatagtgaaagactgatctgttcaaaatatttgctatatgcactgggtataatccgtaatccatacactgccagataatgccatttcaaggaaggatcgaatacttgatggtaaaggccaagtccccctgtattgggaagtgtgtgatttcggcagacctgctgggaaaatttagggtagagcactctttacagaagaactcaaaaacccaatttggataattttcattatctttttagcaaaatggtttcttaatgtttatattttattttcaaggttcattgtttaatgaaatattttattcttgcatttccataaggaaagggaaagtcatgatcatcctaaaggatcacagtttttaaaaggcaaacattttccctaaggaaacagacacaagctttcctagagaatatgatgttttttaggcattaataaggtccttttttataaaggacacttttctcctagtagttttgaattcaggaacagatccaaagttagcagtatatggctgctacatttccattttcattttcgagccatcagtttatgttcagatgccatctctgtaatcgcacatttaaaacataactgtagcctcactaatggaaaagtagtatgatgaacaatcattcccaatggtgtacaatgtaagggttttagggagcaacagtatttaactggaagaaagaattgcatatttaatgtagtctaatatatacacatttgtttaacatgtaaacaaaagtgttaaattcacatatacaacattatacaatttaatcactcttggaataaaatttttatagccttttttctattgggaaaatttgtttagatgtgtgccactccataggtttatttccaaaatgaatgagcccaactccatttgtaaaaacttgtcagttagaattcctttttttagtggattagggctgaattcttagatccttatttcttttcactttaaatgctgccaaagatcactactcatcattcaggaattcgctgtctagcctatctgtagtttcctgaagattgaaaattatgtagactgctatttaaaaatatatttttctaagtgtgaggtttaagatgctgtattgaccctatgagtttttaatgtgttaattatctttatagcataatagatcgctttaggttcctggaatcccatttggtctgacaggatatatgaagattcttaatacctattttctgtgtctaatacttggttaatactaaaaatagaaatgactaaattacatcacagaaagcataaccagtgattgaacctggtagttttaaagctctaaatagctgtggctgaaggactgattatggggctaagaagcttgaaacgtaagttggtacttgttcatcagtggattctcctaaattaagccaaattttgaaatacatgactattaagtttctactcatgtatttacagtcagtcaataaattaaaggaggaaaaaaatccctgaacaacctgcccataaaaagaaaaatactctacatttgagcctgctgcagttttaaattttccctctgggtcaagtttgccagcttttggctacagagaaattatatttccattacagtgcaggtagaaactctgtaaccttaagcatgtaaactacatagaataaaactgtttccactgcatttctgtccttcaaagtggccaacctgattaagtcagccttaatcactgctgctgtcagtttcacgactaaaggtcatattgactaagtagtcatcagctgaccacctcgctgtatcagccagcaacgaggggaaggtgaagaaacatgataggccatatagaatctgccctatgtttacttttttaacccagataattatttttgtgtgcagtatctaagctcctgattgtgtaacctgggacttctggcaccttttgttccattcattttatgtataaaatgcatgccaaagcacactgtgccctctggtacccttgcttccaatcgccaaccatgctcatttccttcctttttttgtggtccctttttgtggtgatcattttaaaccacgtcatccaacaaatgttttatggtcaaccttagcttgttcataagccatagcaactgaaagattaaactcttaaatatgtgtctgggcagtggctattaaatagcaaaaaacaatcagattttagtattttattatttccttgtaaaatggctgaactaaattaaacccttgtttcccatttgttctataatttatagtgaaactgagaacaaaactatctttataaatgatagctaaaagtatttccagatatttaaacaatttaaaataaatttcttctgcagagatgcaaagcatctcaacactggaatgaacaaatgccttaaattcaatggagtaaacctttagaatgaagaggaactgtcatttcacccaagccgaagacaacagccttatgcacttgtgtgctctgtctttgctgcttctcgtgtttcaagcctttcctgtgggatcagcacagcaaagtgcaacttaccaaatggtttaatgactggttaattctttcttctcccaatggaaaagcaatggcaacacaacagtagactgctggcttgacaatcttaaacgtgagcctttgcacatgtaggtttatcatcatttgagtatacgactaagcaagtcaatgaactttttttttttttttagcagtttaatttggtcctgagaatgttgcagtctttattaccccttttgcattaatccacttttctaaccaccttttaagctttaatttttaacactatacaccaagtctttgaaatcagtgatctgttatttaactctaaagcatttgacacttcttgccttaacagttttaaaaaccacacacaaaaaaactctgtaagtaatacagtaggccaaaagtttcatcctatctatcttgcagtttacctatctgatctgatctctgtaattatagttctgtcatttaaaatatactatttaaatctaatttttacatttcaaaaattatcttcagtagtaactaagtatattttctgtggattctgagaatgttatttttcagaatgtgagaatatatatgtacatttataatcttgtgactttaaagtctgttttcagatacagtatgtaaatacttgtaaaaaaatttgtataattttgtgataatgtagtttcccaaaaaaattatttagaaggcattatgttattagtaaatgagagcactgtatagaactgttcctattttctgcacttgccattccagctgcctccactgtccatacccacctcattcatcctgtcacagaaggcaggaaaactgggaactttaccaaagtagcactcagcctgagaggcctgtataatcatgcttttcaaactaaattcacttaaaaattaaaaagcagaattgaatattttaagcagcctcagtacctttggccaatgctgttttcatggtggattatgaacattatataatctttgggaaaagtgaaagtagtacaatttttagaataatgacaactgcctcactgcatctctccactcacacagcaaccgtgtagccccctaagctgcagtaccatgactaaccatgatgtcaatttcatatgctgatcctcacaacagcagtgcacaaacatgccccaaatattttaacagaatttagctcttccttaagctgtcttttcatagtaaaaacaaaacaaaaacacccaatgttaaaaccacataataaacttacaaacttgaaaaattagacacttcagatagataggcaataaaacttcatattatgaaagcaatatattccaagtttcaaagatttgacaagttctgtagagtatctttcatcagtacatgaaaacttccaaactgcatgatcttctgccaggcaggactgggtgctattcgctggtttgaggtcgaatccatttcaaggcatgtcgtggtgggacattaatggtgggatggtagaatgtgcagtccggtcttgtacattgagtgttaaacctacaatgttttggatgatagaagggacattccatcttcttacaagcagggaagtaacggcagagctgactactggaaggtggtgctggtggtgcaactgctggttttggagacagtactggaattcttctactcacatgagtgaagggacaatctggtttagtacactttgcatcatatttacaatttgggtgaacaaacaaacatttttcagcaaatttacaattggggaaggctttgcagggtgagatggggtgatggtaggcacactcatccccatttttacaagcaggccagtacttgcagcgctccaaaagtttttctggtttctgtgccacactcagttcactcatctcagcgttagaaaagctaccatttgggtcctcaagctgcctgctcagcaagtgcaactgctgtgggtggaggagacctctgagtcccttgtttgaggctgcagtttggtttacgggtttcattccttcaaagcacatgtcctcctcttgatctgacatgtatcctggggggctggggacaccatccagcgtcactataaacttgggacttgcaggtttatctggttgtacaagatctcgtgtctgcataaggtgtcctgaaagtacccgaagggaatctgcagtcttcatccccgactcttggtttggtgccactactacttcctcagacagctttggcttcttcagaataaatgatcttgtgtctgcatggaccatggattccatgtcatagtaatcttgatttttttctacagaatctccttttgtttcctcttctttaatggggggacttattctgggggtcctactttgtccctggaccacttctgctagcaattcttcttgagaagttcgagttctgggagcaactggaagtgtctgtttctgtggaactgtagagtagttagttgtttttgttacggattcttgagcttcagatatagccttcaaaatcagattcttgttagcttgtttagaaggtggaagagaaggtctcctttcaggctttgcaggcacagacacactgctggagatgcttcctgttcgagacccgtaatcatcatcttcttcctcctcttctccatcatgattgaatttttttactttaacaactgaacttaccacaggcaactttctcttccgaaagttttcatcctccatactcattttctccgagttgtttctaaagaacggactatacgtttcttctaagctgttaagcacctctggttcacacaaacgtcctgtttcatatacccaactactctgcatatcaagctgcttggcagcatgaatactattctgctgctgttgaaattgcaacctgtttaaatgaacaccactatctgcatttctacttgcaggtggtcgataaatttcaatagaagggcgagaagaaccatatgtaagtgtcactgtaggttttttctgagataagggattctcctgcacaaagttgaggtcttcgtcaatgagatcatctggttctggcttaatatcaatcacatcttcagagggtgctggctccctcaaaggtttcactgttgacattagtcgggttgcagctccatcatcgtaagtctgtctgacatttgtggtttttgactcctgcgaacttgtagaaactctggaatctcttttttcaggtctcgcgctaggaatggcaagtggtggcactgcagcttcatgcctcctctcatctccccgactgaaattgctcttgtttgaaggcacgttactatcaaagatgttggtatcagaagacttcagactagagggttcagttgtaacagagcgaagtttatctaatacaccatgaagccatacggtgaatcgaattgtgttgttccctagaaacagggacagatcctctgtcatttggtcctgacttttcttgttggccaccatcaccataatgtaatcaggaagttcttcatcaacataagctcctaattcttgtaatttccccttaatggcactccggatcttgcggctgatctcggtgccgatctccatggctctgcggcgtgcgggaactcagcactgcgcggcgcttggcttacccggaggctgccgcggactcctaccccgcagccgggacaccaccgcctcc

SEQ ID NO: 13612 - RNA, 17037 nt, Homo sapiens
  source 1..17037: mol_type = other RNA
gctgggattacaggcatgagccaccataataaggattctgatgaacatttgattccttggactactgttatactcaaaagccttccttaatcttctaattgtcaccctaaatatcctaaaatttctgtcttcctagtagttcttcatagtcctaaaaatttgtcagagagaaaggtaaatcaagaaacatgattttcaaatgatttaaggtggtactagggtttaggatttcctttgctttttatcatttaacacactgcttatcatacagctggaagtgctctgggccagtgtctctacttcgagggaagaaggaggtagtgagacagaaggaaatagcacaattcctggccctgacagaagggtgttcaggagacctgctctcctctcactttattccatctcatctggacctgtggcttccaatccacatctctttcctttaatatcctgcattggctaggctgtataaatcctttggtgcatcgaaaaactaagtgcattttttgtttttgtgattatgcaatacttataggaaaagttataattttagaatatttaagtacacttacatttttgagaaaaagactattgaaatgtttgtgccatgtcaaatttcagttgaacattttgggtattcttaatataagaccaggccaggcaccgtggctcaggccgggcacagtggctcacacctataatcccagcacttagggaggccaaggcgggaagatcacctgaagtcaggagttcaagaccagcctggctaacaaggtgaaactctgtctctactaaaaatacaaaaattagccgggcgtggtggctggcgcttgtaatcccagctacttgggaggctgagacaggagaatcacttgaacctgggaagcagaggttgtggtgagctgagatcgcaccattgcactccagcctgggcaacaaagagcgaaactccgtctcaaaaaaataaaaaataaaccctagaattatagtatgttagaattggaagggaagaattgtctaaggttattctagctaataagcaacagacttggaaaggaaaaggtcctgacaaagctaagcctcccgttcaggtttcctgactcgtgaattcagtgctgctgccactacacgatgcatgctctttgtatcaagggtgagacagcattacacatacatagaaaattatctatttaaactctatttgaacttttgatgagtttgtctccccctcccccactccttttcagaataacttgacgtttacaggtaccatcagtggtgatgtctgtgtgtggaaagatcacatattgtgtagaatcgtggcgagagctcacaacgggcctgtgtttgccatgtacaccaccctgcgagatggacttatcgtgactgggggaaaggaaaggccgtgagtcctctttcttttcacagaatatttatgcatttgtgacctacctgaggtttgcagttaattattctagttgtttctaggctacacagagtgtcctctccgaccttcctcctcatatgcttctcctttattaccttttatgtgccttctatttgattctcatttctggtcttaattcacttccaatttttttcatgttggggtgatactttttctgaggtgtggataggtagttgtcctacaagttgagttacttttcttaatgtctgtatgcctgtgtatgatttgctgagtaggaggcccatgggggaatctggagccagggttgtattttgactgcctgctctctttttgttcagaatggattctaaggagtagaatgcacattgttgctttagaaaaggatgagggaactagagagaactgccttgtttccttttgcttgaggcaaatttaaactgttttatacaagacctcaaaatttgagaagaggtctcttctgagtgattttcaaatctcccaacagtaaccagatacttatgatttgatttgtcaccaacatagtcatatgcatgttgaaacatgacatgtaggccaggcacagtggctcacacctgtaatcttatcactttgggaggctgaggcaggtggatcgcttgagcccaggagttcaagaccagcctgggcaacatggtgaaaccccatcgctataaaaaacaacaattagccgggtgtggtggcacatgcctgtagtccctgctactcaggaggctgaggtgggaggatcacttgagcctggggaggtcaaggctttagtgagctgtgatggtgccactgcactccagcctgggtgacagagtgagaccccatttaaaaaacaaaaacaaaaacaaaaaaaaatgtgacatatagttgactaagaagtacatttcaatacaggattgaaagaacccacatatgttaattaaacacaagcgcagaatttgtgccttttacataaaggaagaatgcacataggcatgctttcagacaagcaattcatctagcagaaaaggaaggaatacatttttcagcccttccaggaataaaatccataaatgggctctatttcgtcctccaacacttgtatttcccacgtcatttactcctgcacacccccactcactagaagcctgctaaactgttccagtgagatattttaacacctgatagggaataaatatgcttctgttttggccttcaaaaataagctctgggccagttgcagtggctcacgcctgtaatcccaacactttgggaggccgaggtgggcggatcacgaggtcaggagtttgggatcagcctggccaatatggtgaaactccatctctactaaaaatacaaaaattagccaggcatggtgcctgtaatcccagctacttgggaggctgaaggagaagaatcgcttgaacctgggaggcacaggttgcagtgagccgagatcacaccactgcactccaggccaggtgacagagcgacactctgtctcaaaaaaataaataaatcaactctgtagcatagcatttgtaattctattattttgccttacatttccattatccttttaataaaattgtttttttacatcttcctaatcaagaagtattatgaggccaggcacagtggctcatacctggaatcccagcactttgggaggccgaggcaggcagatcacctgaggtcaaggtatttgagaccagcctggccaacatggtgaaaccccatctctactaaaaatacagaaattagctgggtgtggtggtgcacacctgtaatgctagctactcgggaggctgaggtaggagaatcgcttgaacctgggaggcagaggttgcaataagcctagatcatgccactgcactcaagcctgggagacagagcgagactacatcttaaaaaaaaaaaaaaaagtattatgagagaggataatgtattgtaatgtattgtagaggctaaataaaattatgctcatgtcagaaaaaaagagtatttctcaaaataaaattcactgaaactggatgtttattttgactgagatatagtatatcctcaaattgccatagaaagtttacaagaatattagaggtaaattataaatatcagggcctttttaaaaaaaaaagattctgcttataacttggtatttgtttataataaaaattatagtagccaataatgaacacttactctggcttggttatttacttaggtcaaaagaaggaggagcggttaaactgtgggatcaggaactgaggcggtgccgtgccttcaggcttgagacaggacaagccacagattgtgttcgttctgtgtgcagaggcaaagtaagatgttccatgagctgatacagtgcagcagaaaacagaaagtggttattactgtgattccctcaccctttgcagcctaatgaacaatacttaataatgcataacgatggatttgcttgccaacattactctgtctttgctgctttctttgccaaagttagcaccagtgtggtgcataagctaggaagctattctgtctaaatactgtatgtaaacctccaatattttctagaatctgccaatttaacaactctagtagacataattgaaagcccttggcagttgactcatattaggacagctgtctccattttttaaaaaaacacacattccctagataaaacgtgcagtaaacaaacaatgaaatactactcagccataaaaaataatgaaattctgtcattcttggtggcaacatggatgagactggaggacatgatgtgaagtgaaataagccaggcacagaaagataaatacatgttctcactcctgtgcagaaactaaaaaagttgatcccacagaggtggagagtagaatagtggttactggaggcggacaagggggagggggagggggatagggaaggactggttaaaggatacaagtttacacagccagataggaatagtatgttttagtattctgtagtactgtaggatgactatagttaagaatcacgtatttatgtattttcaggtatttacaagagaggattttgaaagtttccatcacaaagaaatgataaatgtctgaggtgatggttatgcgtattaccctatgccctatagatatgtataattatgtgtcaatttcaaaataaaaattcaaaactacaactcctatgaaaatttttgagcgtgtttgtacttattaagtgtatttataaatcatacggatattatcttcagcctgcatattaaattgtagttaagcttttactttttaactaaaaaataaattctattattttttcctatatcccactgcactgaccccagtttggaaatcctaagattatcaaataaaaactttgattattgaagaatccaggtgtactgccacagaaaagttctattctgtagcatggactctaatatgtaatctagcccattgtgcttacagatagatgtgtgcctgtagtcatagaaaaatttgcatgagctaatgactgccttgctactagattagctcaaagcaaaaagttctctgaaagcaggtcaatagggtcatttttatattatgaagaagaaaagcagctgttgtattacattcactgtattggtcctgcttgtgtttcagggcaagatccttgttgggacaaggaatgctgaaataatcgaagttggagagaaaaatgcagcttgtaatattttagttaacggtcatgtggatgggccaatctggggactagcaacacatccttccagggattttttcctttctgctgcagaagatgggacagtgagactttgggatattgctgataaagtaagtacagataatttttttaaaagaggttacaacttctaaaaagaaaagttggaagttctaaattgctagtacttaaagaactgccagaattctgttgagcattttgaggggaaactggtataatttagaagtacttcacttaatgtttcctatgactctttttttttttttttttaaatgcagaagatgttaaacaaagtgaatttgggacatgctgctcgtactgtgtgttacagccctgaaggggacatggtggctattggaatgaaaaatggagaatttatcattttactagtgagttctctaaaaatatggggaaagaagagagacaggagatgtgcaatccatgatatcaggttagtgaacaaatggaatagagtttctagtatatacttgatttaacttccatttgtaaaattttccatagccttgccttcaaaaagaggtccccagggcctgtagcatttcccgtattataaattgtatgctaaaatatggctgtttgtatactacttaattcttcttgctaaattataaacccactgggcaccaactataatagcaagtactagtaggtaatgtttgatgaattcatgttaacacttagccatgtccattaagttcatcccaccaagaggtatctcccactgtaatacaagagagctatctgcccttcaaaagttgtcaccctggaaaactaaagttgtgatttcaaacatatcttctcttagtaacctcagtttgggaatatgtagttcattaatttaatcaatacctattgattaaatgttccagaatccaaattaatttaaatgtttcttaaacctttgtttttcagtgcttaagcatttttcaacagtggctaccatttacggagtacttccgtgtgatcagtagataagattattgaatctaggtctgtcaaaagcttgtacacttttcatcagtaaaatccttttacaaatgaaaccttcctcagaacttcaatatataaaatagtaacagtggcttcccttagcttttacatgtctctatcgtacctcagtaagactcatgggccatttcaagagactgaattgtcccatatgactccaaagattgctaggcaaatagcatttcactttgtcttttaaataagttcttcaggccgggcgcggtggctcatgcctgtaatcccagcactttgggaggccgaggcaggcagatcacctgaagtcaggagtactcgaccagcctggccaacatagtgaaaccccatctcaactaaaaatacaaaaatcagccgggcgtggtggcaggcgcctgtaatcccagctactcagggggctgaaacaggagaatcgcttgaacccgggaggcggaggttgcgccatcgcactccagcctgggagacaagagcgagacttcgtctcaaaaaaaaaaaattcttcttccaagattcaagttgtgtcatttcaccttaataactggaggttagttaagctgggctgtgttctttgcttaatattaagacaacgttttttccagatggaagaaaactatcttaatgaattgttagcttattaattatgtaatgctaatggcttttaaaagctgagatgttctgactgggtgttgtggctcacacctgtaatcccagtaccttgggaggccaagggggaaggattgcttgaggccaggagtttgggaccatagtgagaccccgcctctatttaaaaaattaaattttgttttgttttgttttgagttggagttttgctcttgttgcccatgctgaagtgcaatggtgcaatctcagctcaccacaacctgtgcctcctgggttcaagcgattctcctgcttcagcctcccgagtagatgggattacaggcgtgcaccaccatgcctggctaattttgtatttttagtagagacagggtttctctatgttggtcaggctggtctcaaactctcgacctcaggtgatctgcccgcctccgcttcccaaagttctgggattataggtgtgagccactgggcctggcctaagaaagtttttttaagccattagacgtttttaaaggaattgggagatgacaattggggaaatatttaaaatttaagtaaaatataaagcttccttatttcatgtaacccagacaatctcagtatacatgatcagttgtgtctgacaggtaaatctatttgaggccttatcacacgttacttttaagaactagaaaggaaaagtcactgatcttaagtatttataatacttcatgtggtctaatactttttacgttttgttttgattcagatttagtccggattcccggtatctggcagtaggttctagtgagaactcagtggatttttatgacctaacgctgggccccactcttaacagaatcagctactgcaaagacattccaagctttgtcattcaaatggacttctctgcagatagcagttatctccaggtacagtaccaatactgtatacccaggtggcaagttcttctgcttttacatttcgtgttagtgaatgcatttaaagttcctgagctccagagctccagcttctcaactcctccctttgtaccttctgacctacagctcccctttcctcccccacttatcagagcttttctcctattaagtttttgtagtgatcttttgcatacttaataatgttagacatgtaaatcaagtagcaatatgctagtattctgtaaaccccctgtggattttgtctctcacctaatggaattcttgtcccattttaatctgatgaaaaaggtctctagtggctgctataaacggcatgtctatgaagtgccttcaggaaaacatcttatggatcatgccgctattgacagaattacttgggctacatggactaggtaaatacttatatattcacaaggcaagaactgactttgaaggccagttagaaaatcctatttctgaactgttagagccattccaataaggaatagtaattgagtttcaagtttttgttaccatattttgaaatggtatgttcatgttgggacccctttttattgaatatatttccatgttttatcagtttccatgatttatcaagttttttttttaaggaaatcaaagttttaactttaaagataccctgatatttttcttaatgctaaatttaatgactggcaaaaaggtattgggtgctgttaagcaactgttattaattctctatctaaaggaatgctatcttgaatctattagaagtcaaagcttccaaatttgttcaaatttcctggctgtatgacaggtaaccatgactatccatttttttggccaatgaaaaatgccatcaaattcctgtatcagccaggcatatagtggctcatgcctgtaatctctgatgtagcaggccgaggtgggaggatcacttgagcctagaagttttgataccagcctgggcaacatagcaagaccccatctctgaaatttttttaattcctatgtcataagtcatttttatttttgtagagatagggatctcacaatattgcccaggctggtctcaaactcttggcctcaagcagtcctcctgcctcagcctcccaaaatgttgggattactggtatgtgctgctggacccagccaagtagcacttttaatttgaaaaatagttctatcagttttcagtcaggcgcggtggctcagcctgtaatcccagcactttgggaggccgagcgggggtgatcacctgaggtcgggagttcgagactagcctgaccaacatggagaaaccctgtctctactaaaaatacaaaataagccgggcatgttagcgcatgcctgtgatcccagctactcgggaggctgaggcaggagaattgcttgaacccaggaggcagaggttgcggtgagccgagatcatgccattgcactccagcctgggtaacaagagcgaaaactccgtctcaaaaaaaaaaaaagaaaaaatagttctatcagttttcataaagtactactttaatcttaaaaagattaatctagaaacccttcaaattataaaatgtcatttttaaaaggcaggagttgatatcctgatgaaattcaggtctccaaacaacttaccataatttacttcctgtattttaagtaacatgatagggtacttagagattaattgccaagaaactttttgaatatagtcaacctgcccgcacttgccatgatgagttttcttttgttccttccctctagtattctaggagatgaggttttgggaatctggtccagacatgctgagaaagctgatgtcaactgtgcctgtgtatctcattcaggaatcagtcttgttacaggagatgactttggcatggttaagttatttgacttcccatgtccagaaaaatttgtaagtttgtgttttgtttactattatcagtttactcctaattttgatgtcttatcatcagcacttttccccatatatttaaaatgttttgtcctaatttctaaatttttccccaaactttctaaatctatttactttgaaataaaagctattagaaacaaatcctctccctcgagtaataccatctttggaaccatcctacaaaagctgtaattagcttttcaccaaacctataatcagttatcaaatttcaaatgcttttccttagagaaaaatggtcagagtacctggagacatctgactgcccacacagcctggttttgcagatccactactcatgctgaaaagcattctaatcactggctgcggtgctaactccctactctctccacagctcttgtcatagagattatagttcctaataagagcctttgacttctgtgtgcaccaaatgccctgagcttgtctgtcattgttttttaggcaaaacacaaaaggttcttgggtcattcgccccatgtgacaaatattcgatttaccagtggtgatcgacatgttgttagtgctggaggtgatgactgcaggttagtaactttctcagcccatgaagagcagactatgttactagttaagagacttaatacaacaactcctacagctttggtttatgaaatcagctagtcaacattagtagaaggtagtataaccagatggctcttcagaatctcatatttatgcaaatacagaataaaaggagttaaagaggaaaaatattacacatgtaacctgaaagcacaactgaaaaatattaaactgttatgaaaatctaaaaacataattaactccctgcaattttcttctctgattgcagcttatttgtctggaaatgtgtacatacacctcactgagagatgctgagatgactacagaaattaactttgagaccagaattacagagaagaaaaaccaaaacccaaccctgcatggtcaagtggtgctaacccaagactgtaacagggagaaatgcccagaatcatcaaaatagtgaaagactgatctgttcaaaatatttgctatatgcactgggtataatccgtaatccatacactgccagataatgccatttcaaggaaggatcgaatacttgatggtaaaggccaagtccccctgtattgggaagtgtgtgatttcggcagacctgctgggaaaatttagggtagagcactctttacagaagaactcaaaaacccaatttggataattttcattatctttttagcaaaatggtttcttaatgtttatattttattttcaaggttcattgtttaatgaaatattttattcttgcatttccataaggaaagggaaagtcatgatcatcctaaaggatcacagtttttaaaaggcaaacattttccctaaggaaacagacacaagctttcctagagaatatgatgttttttaggcattaataaggtccttttttataaaggacacttttctcctagtagttttgaattcaggaacagatccaaagttagcagtatatggctgctacatttccattttcattttcgagccatcagtttatgttcagatgccatctctgtaatcgcacatttaaaacataactgtagcctcactaatggaaaagtagtatgatgaacaatcattcccaatggtgtacaatgtaagggttttagggagcaacagtatttaactggaagaaagaattgcatatttaatgtagtctaatatatacacatttgtttaacatgtaaacaaaagtgttaaattcacatatacaacattatacaatttaatcactcttggaataaaatttttatagccttttttctattgggaaaatttgtttagatgtgtgccactccataggtttatttccaaaatgaatgagcccaactccatttgtaaaaacttgtcagttagaattcctttttttagtggattagggctgaattcttagatccttatttcttttcactttaaatgctgccaaagatcactactcatcattcaggaattcgctgtctagcctatctgtagtttcctgaagattgaaaattatgtagactgctatttaaaaatatatttttctaagtgtgaggtttaagatgctgtattgaccctatgagtttttaatgtgttaattatctttatagcataatagatcgctttaggttcctggaatcccatttggtctgacaggatatatgaagattcttaatacctattttctgtgtctaatacttggttaatactaaaaatagaaatgactaaattacatcacagaaagcataaccagtgattgaacctggtagttttaaagctctaaatagctgtggctgaaggactgattatggggctaagaagcttgaaacgtaagttggtacttgttcatcagtggattctcctaaattaagccaaattttgaaatacatgactattaagtttctactcatgtatttacagtcagtcaataaattaaaggaggaaaaaaatccctgaacaacctgcccataaaaagaaaaatactctacatttgagcctgctgcagttttaaattttccctctgggtcaagtttgccagcttttggctacagagaaattatatttccattacagtgcaggtagaaactctgtaaccttaagcatgtaaactacatagaataaaactgtttccactgcatttctgtccttcaaagtggccaacctgattaagtcagccttaatcactgctgctgtcagtttcacgactaaaggtcatattgactaagtagtcatcagctgaccacctcgctgtatcagccagcaacgaggggaaggtgaagaaacatgataggccatatagaatctgccctatgtttacttttttaacccagataattatttttgtgtgcagtatctaagctcctgattgtgtaacctgggacttctggcaccttttgttccattcattttatgtataaaatgcatgccaaagcacactgtgccctctggtacccttgcttccaatcgccaaccatgctcatttccttcctttttttgtggtccctttttgtggtgatcattttaaaccacgtcatccaacaaatgttttatggtcaaccttagcttgttcataagccatagcaactgaaagattaaactcttaaatatgtgtctgggcagtggctattaaatagcaaaaaacaatcagattttagtattttattatttccttgtaaaatggctgaactaaattaaacccttgtttcccatttgttctataatttatagtgaaactgagaacaaaactatctttataaatgatagctaaaagtatttccagatatttaaacaatttaaaataaatttcttctgcagagatgcaaagcatctcaacactggaatgaacaaatgccttaaattcaatggagtaaacctttagaatgaagaggaactgtcatttcacccaagccgaagacaacagccttatgcacttgtgtgctctgtctttgctgcttctcgtgtttcaagcctttcctgtgggatcagcacagcaaagtgcaacttaccaaatggtttaatgactggttaattctttcttctcccaatggaaaagcaatggcaacacaacagtagactgctggcttgacaatcttaaacgtgagcctttgcacatgtaggtttatcatcatttgagtatacgactaagcaagtcaatgaactttttttttttttttagcagtttaatttggtcctgagaatgttgcagtctttattaccccttttgcattaatccacttttctaaccaccttttaagctttaatttttaacactatacaccaagtctttgaaatcagtgatctgttatttaactctaaagcatttgacacttcttgccttaacagttttaaaaaccacacacaaaaaaactctgtaagtaatacagtaggccaaaagtttcatcctatctatcttgcagtttacctatctgatctgatctctgtaattatagttctgtcatttaaaatatactatttaaatctaatttttacatttcaaaaattatcttcagtagtaactaagtatattttctgtggattctgagaatgttatttttcagaatgtgagaatatatatgtacatttataatcttgtgactttaaagtctgttttcagatacagtatgtaaatacttgtaaaaaaatttgtataattttgtgataatgtagtttcccaaaaaaattatttagaaggcattatgttattagtaaatgagagcactgtatagaactgttcctattttctgcacttgccattccagctgcctccactgtccatacccacctcattcatcctgtcacagaaggcaggaaaactgggaactttaccaaagtagcactcagcctgagaggcctgtataatcatgcttttcaaactaaattcacttaaaaattaaaaagcagaattgaatattttaagcagcctcagtacctttggccaatgctgttttcatggtggattatgaacattatataatctttgggaaaagtgaaagtagtacaatttttagaataatgacaactgcctcactgcatctctccactcacacagcaaccgtgtagccccctaagctgcagtaccatgactaaccatgatgtcaatttcatatgctgatcctcacaacagcagtgcacaaacatgccccaaatattttaacagaatttagctcttccttaagctgtcttttcatagtaaaaacaaaacaaaaacacccaatgttaaaaccacataataaacttacaaacttgaaaaattagacacttcagatagataggcaataaaacttcatattatgaaagcaatatattccaagtttcaaagatttgacaagttctgtagagtatctttcatcagtacatgaaaacttccaaactgcatgatcttctgccaggcaggactgggtgctattcgctggtttgaggtcgaatccatttcaaggcatgtcgtggtgggacattaatggtgggatggtagaatgtgcagtccggtcttgtacattgagtgttaaacctacaatgttttggatgatagaagggacattccatcttcttacaagcagggaagtaacggcagagctgactactggaaggtggtgctggtggtgcaactgctggttttggagacagtactggaattcttctactcacatgagtgaagggacaatctggtttagtacactttgcatcatatttacaatttgggtgaacaaacaaacatttttcagcaaatttacaattggggaaggctttgcagggtgagatggggtgatggtaggcacactcatccccatttttacaagcaggccagtacttgcagcgctccaaaagtttttctggtttctgtgccacactcagttcactcatctcagcgttagaaaagctaccatttgggtcctcaagctgcctgctcagcaagtgcaactgctgtgggtggaggagacctctgagtcccttgtttgaggctgcagtttggtttacgggtttcattccttcaaagcacatgtcctcctcttgatctgacatgtatcctggggggctggggacaccatccagcgtcactataaacttgggacttgcaggtttatctggttgtacaagatctcgtgtctgcataaggtgtcctgaaagtacccgaagggaatctgcagtcttcatccccgactcttggtttggtgccactactacttcctcagacagctttggcttcttcagaataaatgatcttgtgtctgcatggaccatggattccatgtcatagtaatcttgatttttttctacagaatctccttttgtttcctcttctttaatggggggacttattctgggggtcctactttgtccctggaccacttctgctagcaattcttcttgagaagttcgagttctgggagcaactggaagtgtctgtttctgtggaactgtagagtagttagttgtttttgttacggattcttgagcttcagatatagccttcaaaatcagattcttgttagcttgtttagaaggtggaagagaaggtctcctttcaggctttgcaggcacagacacactgctggagatgcttcctgttcgagacccgtaatcatcatcttcttcctcctcttctccatcatgattgaatttttttactttaacaactgaacttaccacaggcaactttctcttccgaaagttttcatcctccatactcattttctccgagttgtttctaaagaacggactatacgtttcttctaagctgttaagcacctctggttcacacaaacgtcctgtttcatatacccaactactctgcatatcaagctgcttggcagcatgaatactattctgctgctgttgaaattgcaacctgtttaaatgaacaccactatctgcatttctacttgcaggtggtcgataaatttcaatagaagggcgagaagaaccatatgtaagtgtcactgtaggttttttctgagataagggattctcctgcacaaagttgaggtcttcgtcaatgagatcatctggttctggcttaatatcaatcacatcttcagagggtgctggctccctcaaaggtttcactgttgacattagtcgggttgcagctccatcatcgtaagtctgtctgacatttgtggtttttgactcctgcgaacttgtagaaactctggaatctcttttttcaggtctcgcgctaggaatggcaagtggtggcactgcagcttcatgcctcctctcatctccccgactgaaattgctcttgtttgaaggcacgttactatcaaagatgttggtatcagaagacttcagactagagggttcagttgtaacagagcgaagtttatctaatacaccatgaagccatacggtgaatcgaattgtgttgttccctagaaacagggacagatcctctgtcatttggtcctgacttttcttgttggccaccatcaccataatgtaatcaggaagttcttcatctatttaaaaggaaaggtagatcaaaactttgtttcctcaaaactttcttcttaaagttgatgtgcttgaaaatatagatgtagctctaagctttagagtcgcagagctctactggaattacattggacaagatggcttagctttaatttttttctcttcattccacaggtatttcaaatacaacataagctcctaattcttgtaatttccccttaatggcactccggatcttgcggctgatctcggtgccgatctccatggctctgcggcgtgcgggaactcagcactgcgcggcgcttggcttacccggaggctgccgcggactcctaccccgcagccgggacaccaccgcctcc

SEQ ID NO: 13613 - RNA, 16771 nt, Homo sapiens
  source 1..16771: mol_type = other RNA
gctgggattacaggcatgagccaccataataaggattctgatgaacatttgattccttggactactgttatactcaaaagccttccttaatcttctaattgtcaccctaaatatcctaaaatttctgtcttcctagtagttcttcatagtcctaaaaatttgtcagagagaaaggtaaatcaagaaacatgattttcaaatgatttaaggtggtactagggtttaggatttcctttgctttttatcatttaacacactgcttatcatacagctggaagtgctctgggccagtgtctctacttcgagggaagaaggaggtagtgagacagaaggaaatagcacaattcctggccctgacagaagggtgttcaggagacctgctctcctctcactttattccatctcatctggacctgtggcttccaatccacatctctttcctttaatatcctgcattggctaggctgtataaatcctttggtgcatcgaaaaactaagtgcattttttgtttttgtgattatgcaatacttataggaaaagttataattttagaatatttaagtacacttacatttttgagaaaaagactattgaaatgtttgtgccatgtcaaatttcagttgaacattttgggtattcttaatataagaccaggccaggcaccgtggctcaggccgggcacagtggctcacacctataatcccagcacttagggaggccaaggcgggaagatcacctgaagtcaggagttcaagaccagcctggctaacaaggtgaaactctgtctctactaaaaatacaaaaattagccgggcgtggtggctggcgcttgtaatcccagctacttgggaggctgagacaggagaatcacttgaacctgggaagcagaggttgtggtgagctgagatcgcaccattgcactccagcctgggcaacaaagagcgaaactccgtctcaaaaaaataaaaaataaaccctagaattatagtatgttagaattggaagggaagaattgtctaaggttattctagctaataagcaacagacttggaaaggaaaaggtcctgacaaagctaagcctcccgttcaggtttcctgactcgtgaattcagtgctgctgccactacacgatgcatgctctttgtatcaagggtgagacagcattacacatacatagaaaattatctatttaaactctatttgaacttttgatgagtttgtctccccctcccccactccttttcagaataacttgacgtttacaggtaccatcagtggtgatgtctgtgtgtggaaagatcacatattgtgtagaatcgtggcgagagctcacaacgggcctgtgtttgccatgtacaccaccctgcgagatggacttatcgtgactgggggaaaggaaaggccgtgagtcctctttcttttcacagaatatttatgcatttgtgacctacctgaggtttgcagttaattattctagttgtttctaggctacacagagtgtcctctccgaccttcctcctcatatgcttctcctttattaccttttatgtgccttctatttgattctcatttctggtcttaattcacttccaatttttttcatgttggggtgatactttttctgaggtgtggataggtagttgtcctacaagttgagttacttttcttaatgtctgtatgcctgtgtatgatttgctgagtaggaggcccatgggggaatctggagccagggttgtattttgactgcctgctctctttttgttcagaatggattctaaggagtagaatgcacattgttgctttagaaaaggatgagggaactagagagaactgccttgtttccttttgcttgaggcaaatttaaactgttttatacaagacctcaaaatttgagaagaggtctcttctgagtgattttcaaatctcccaacagtaaccagatacttatgatttgatttgtcaccaacatagtcatatgcatgttgaaacatgacatgtaggccaggcacagtggctcacacctgtaatcttatcactttgggaggctgaggcaggtggatcgcttgagcccaggagttcaagaccagcctgggcaacatggtgaaaccccatcgctataaaaaacaacaattagccgggtgtggtggcacatgcctgtagtccctgctactcaggaggctgaggtgggaggatcacttgagcctggggaggtcaaggctttagtgagctgtgatggtgccactgcactccagcctgggtgacagagtgagaccccatttaaaaaacaaaaacaaaaacaaaaaaaaatgtgacatatagttgactaagaagtacatttcaatacaggattgaaagaacccacatatgttaattaaacacaagcgcagaatttgtgccttttacataaaggaagaatgcacataggcatgctttcagacaagcaattcatctagcagaaaaggaaggaatacatttttcagcccttccaggaataaaatccataaatgggctctatttcgtcctccaacacttgtatttcccacgtcatttactcctgcacacccccactcactagaagcctgctaaactgttccagtgagatattttaacacctgatagggaataaatatgcttctgttttggccttcaaaaataagctctgggccagttgcagtggctcacgcctgtaatcccaacactttgggaggccgaggtgggcggatcacgaggtcaggagtttgggatcagcctggccaatatggtgaaactccatctctactaaaaatacaaaaattagccaggcatggtgcctgtaatcccagctacttgggaggctgaaggagaagaatcgcttgaacctgggaggcacaggttgcagtgagccgagatcacaccactgcactccaggccaggtgacagagcgacactctgtctcaaaaaaataaataaatcaactctgtagcatagcatttgtaattctattattttgccttacatttccattatccttttaataaaattgtttttttacatcttcctaatcaagaagtattatgaggccaggcacagtggctcatacctggaatcccagcactttgggaggccgaggcaggcagatcacctgaggtcaaggtatttgagaccagcctggccaacatggtgaaaccccatctctactaaaaatacagaaattagctgggtgtggtggtgcacacctgtaatgctagctactcgggaggctgaggtaggagaatcgcttgaacctgggaggcagaggttgcaataagcctagatcatgccactgcactcaagcctgggagacagagcgagactacatcttaaaaaaaaaaaaaaaagtattatgagagaggataatgtattgtaatgtattgtagaggctaaataaaattatgctcatgtcagaaaaaaagagtatttctcaaaataaaattcactgaaactggatgtttattttgactgagatatagtatatcctcaaattgccatagaaagtttacaagaatattagaggtaaattataaatatcagggcctttttaaaaaaaaaagattctgcttataacttggtatttgtttataataaaaattatagtagccaataatgaacacttactctggcttggttatttacttaggtcaaaagaaggaggagcggttaaactgtgggatcaggaactgaggcggtgccgtgccttcaggcttgagacaggacaagccacagattgtgttcgttctgtgtgcagaggcaaagtaagatgttccatgagctgatacagtgcagcagaaaacagaaagtggttattactgtgattccctcaccctttgcagcctaatgaacaatacttaataatgcataacgatggatttgcttgccaacattactctgtctttgctgctttctttgccaaagttagcaccagtgtggtgcataagctaggaagctattctgtctaaatactgtatgtaaacctccaatattttctagaatctgccaatttaacaactctagtagacataattgaaagcccttggcagttgactcatattaggacagctgtctccattttttaaaaaaacacacattccctagataaaacgtgcagtaaacaaacaatgaaatactactcagccataaaaaataatgaaattctgtcattcttggtggcaacatggatgagactggaggacatgatgtgaagtgaaataagccaggcacagaaagataaatacatgttctcactcctgtgcagaaactaaaaaagttgatcccacagaggtggagagtagaatagtggttactggaggcggacaagggggagggggagggggatagggaaggactggttaaaggatacaagtttacacagccagataggaatagtatgttttagtattctgtagtactgtaggatgactatagttaagaatcacgtatttatgtattttcaggtatttacaagagaggattttgaaagtttccatcacaaagaaatgataaatgtctgaggtgatggttatgcgtattaccctatgccctatagatatgtataattatgtgtcaatttcaaaataaaaattcaaaactacaactcctatgaaaatttttgagcgtgtttgtacttattaagtgtatttataaatcatacggatattatcttcagcctgcatattaaattgtagttaagcttttactttttaactaaaaaataaattctattattttttcctatatcccactgcactgaccccagtttggaaatcctaagattatcaaataaaaactttgattattgaagaatccaggtgtactgccacagaaaagttctattctgtagcatggactctaatatgtaatctagcccattgtgcttacagatagatgtgtgcctgtagtcatagaaaaatttgcatgagctaatgactgccttgctactagattagctcaaagcaaaaagttctctgaaagcaggtcaatagggtcatttttatattatgaagaagaaaagcagctgttgtattacattcactgtattggtcctgcttgtgtttcagggcaagatccttgttgggacaaggaatgctgaaataatcgaagttggagagaaaaatgcagcttgtaatattttagttaacggtcatgtggatgggccaatctggggactagcaacacatccttccagggattttttcctttctgctgcagaagatgggacagtgagactttgggatattgctgataaagtaagtacagataatttttttaaaagaggttacaacttctaaaaagaaaagttggaagttctaaattgctagtacttaaagaactgccagaattctgttgagcattttgaggggaaactggtataatttagaagtacttcacttaatgtttcctatgactctttttttttttttttttaaatgcagaagatgttaaacaaagtgaatttgggacatgctgctcgtactgtgtgttacagccctgaaggggacatggtggctattggaatgaaaaatggagaatttatcattttactagtgagttctctaaaaatatggggaaagaagagagacaggagatgtgcaatccatgatatcaggttagtgaacaaatggaatagagtttctagtatatacttgatttaacttccatttgtaaaattttccatagccttgccttcaaaaagaggtccccagggcctgtagcatttcccgtattataaattgtatgctaaaatatggctgtttgtatactacttaattcttcttgctaaattataaacccactgggcaccaactataatagcaagtactagtaggtaatgtttgatgaattcatgttaacacttagccatgtccattaagttcatcccaccaagaggtatctcccactgtaatacaagagagctatctgcccttcaaaagttgtcaccctggaaaactaaagttgtgatttcaaacatatcttctcttagtaacctcagtttgggaatatgtagttcattaatttaatcaatacctattgattaaatgttccagaatccaaattaatttaaatgtttcttaaacctttgtttttcagtgcttaagcatttttcaacagtggctaccatttacggagtacttccgtgtgatcagtagataagattattgaatctaggtctgtcaaaagcttgtacacttttcatcagtaaaatccttttacaaatgaaaccttcctcagaacttcaatatataaaatagtaacagtggcttcccttagcttttacatgtctctatcgtacctcagtaagactcatgggccatttcaagagactgaattgtcccatatgactccaaagattgctaggcaaatagcatttcactttgtcttttaaataagttcttcaggccgggcgcggtggctcatgcctgtaatcccagcactttgggaggccgaggcaggcagatcacctgaagtcaggagtactcgaccagcctggccaacatagtgaaaccccatctcaactaaaaatacaaaaatcagccgggcgtggtggcaggcgcctgtaatcccagctactcagggggctgaaacaggagaatcgcttgaacccgggaggcggaggttgcgccatcgcactccagcctgggagacaagagcgagacttcgtctcaaaaaaaaaaaattcttcttccaagattcaagttgtgtcatttcaccttaataactggaggttagttaagctgggctgtgttctttgcttaatattaagacaacgttttttccagatggaagaaaactatcttaatgaattgttagcttattaattatgtaatgctaatggcttttaaaagctgagatgttctgactgggtgttgtggctcacacctgtaatcccagtaccttgggaggccaagggggaaggattgcttgaggccaggagtttgggaccatagtgagaccccgcctctatttaaaaaattaaattttgttttgttttgttttgagttggagttttgctcttgttgcccatgctgaagtgcaatggtgcaatctcagctcaccacaacctgtgcctcctgggttcaagcgattctcctgcttcagcctcccgagtagatgggattacaggcgtgcaccaccatgcctggctaattttgtatttttagtagagacagggtttctctatgttggtcaggctggtctcaaactctcgacctcaggtgatctgcccgcctccgcttcccaaagttctgggattataggtgtgagccactgggcctggcctaagaaagtttttttaagccattagacgtttttaaaggaattgggagatgacaattggggaaatatttaaaatttaagtaaaatataaagcttccttatttcatgtaacccagacaatctcagtatacatgatcagttgtgtctgacaggtaaatctatttgaggccttatcacacgttacttttaagaactagaaaggaaaagtcactgatcttaagtatttataatacttcatgtggtctaatactttttacgttttgttttgattcagatttagtccggattcccggtatctggcagtaggttctagtgagaactcagtggatttttatgacctaacgctgggccccactcttaacagaatcagctactgcaaagacattccaagctttgtcattcaaatggacttctctgcagatagcagttatctccaggtacagtaccaatactgtatacccaggtggcaagttcttctgcttttacatttcgtgttagtgaatgcatttaaagttcctgagctccagagctccagcttctcaactcctccctttgtaccttctgacctacagctcccctttcctcccccacttatcagagcttttctcctattaagtttttgtagtgatcttttgcatacttaataatgttagacatgtaaatcaagtagcaatatgctagtattctgtaaaccccctgtggattttgtctctcacctaatggaattcttgtcccattttaatctgatgaaaaaggtctctagtggctgctataaacggcatgtctatgaagtgccttcaggaaaacatcttatggatcatgccgctattgacagaattacttgggctacatggactaggtaaatacttatatattcacaaggcaagaactgactttgaaggccagttagaaaatcctatttctgaactgttagagccattccaataaggaatagtaattgagtttcaagtttttgttaccatattttgaaatggtatgttcatgttgggacccctttttattgaatatatttccatgttttatcagtttccatgatttatcaagttttttttttaaggaaatcaaagttttaactttaaagataccctgatatttttcttaatgctaaatttaatgactggcaaaaaggtattgggtgctgttaagcaactgttattaattctctatctaaaggaatgctatcttgaatctattagaagtcaaagcttccaaatttgttcaaatttcctggctgtatgacaggtaaccatgactatccatttttttggccaatgaaaaatgccatcaaattcctgtatcagccaggcatatagtggctcatgcctgtaatctctgatgtagcaggccgaggtgggaggatcacttgagcctagaagttttgataccagcctgggcaacatagcaagaccccatctctgaaatttttttaattcctatgtcataagtcatttttatttttgtagagatagggatctcacaatattgcccaggctggtctcaaactcttggcctcaagcagtcctcctgcctcagcctcccaaaatgttgggattactggtatgtgctgctggacccagccaagtagcacttttaatttgaaaaatagttctatcagttttcagtcaggcgcggtggctcagcctgtaatcccagcactttgggaggccgagcgggggtgatcacctgaggtcgggagttcgagactagcctgaccaacatggagaaaccctgtctctactaaaaatacaaaataagccgggcatgttagcgcatgcctgtgatcccagctactcgggaggctgaggcaggagaattgcttgaacccaggaggcagaggttgcggtgagccgagatcatgccattgcactccagcctgggtaacaagagcgaaaactccgtctcaaaaaaaaaaaaagaaaaaatagttctatcagttttcataaagtactactttaatcttaaaaagattaatctagaaacccttcaaattataaaatgtcatttttaaaaggcaggagttgatatcctgatgaaattcaggtctccaaacaacttaccataatttacttcctgtattttaagtaacatgatagggtacttagagattaattgccaagaaactttttgaatatagtcaacctgcccgcacttgccatgatgagttttcttttgttccttccctctagtattctaggagatgaggttttgggaatctggtccagacatgctgagaaagctgatgtcaactgtgcctgtgtatctcattcaggaatcagtcttgttacaggagatgactttggcatggttaagttatttgacttcccatgtccagaaaaatttgtaagtttgtgttttgtttactattatcagtttactcctaattttgatgtcttatcatcagcacttttccccatatatttaaaatgttttgtcctaatttctaaatttttccccaaactttctaaatctatttactttgaaataaaagctattagaaacaaatcctctccctcgagtaataccatctttggaaccatcctacaaaagctgtaattagcttttcaccaaacctataatcagttatcaaatttcaaatgcttttccttagagaaaaatggtcagagtacctggagacatctgactgcccacacagcctggttttgcagatccactactcatgctgaaaagcattctaatcactggctgcggtgctaactccctactctctccacagctcttgtcatagagattatagttcctaataagagcctttgacttctgtgtgcaccaaatgccctgagcttgtctgtcattgttttttaggcaaaacacaaaaggttcttgggtcattcgccccatgtgacaaatattcgatttaccagtggtgatcgacatgttgttagtgctggaggtgatgactgcaggttagtaactttctcagcccatgaagagcagactatgttactagttaagagacttaatacaacaactcctacagctttggtttatgaaatcagctagtcaacattagtagaaggtagtataaccagatggctcttcagaatctcatatttatgcaaatacagaataaaaggagttaaagaggaaaaatattacacatgtaacctgaaagcacaactgaaaaatattaaactgttatgaaaatctaaaaacataattaactccctgcaattttcttctctgattgcagcttatttgtctggaaatgtgtacatacacctcactgagagatgctgagatgactacagaaattaactttgagaccagaattacagagaagaaaaaccaaaacccaaccctgcatggtcaagtggtgctaacccaagactgtaacagggagaaatgcccagaatcatcaaaatagtgaaagactgatctgttcaaaatatttgctatatgcactgggtataatccgtaatccatacactgccagataatgccatttcaaggaaggatcgaatacttgatggtaaaggccaagtccccctgtattgggaagtgtgtgatttcggcagacctgctgggaaaatttagggtagagcactctttacagaagaactcaaaaacccaatttggataattttcattatctttttagcaaaatggtttcttaatgtttatattttattttcaaggttcattgtttaatgaaatattttattcttgcatttccataaggaaagggaaagtcatgatcatcctaaaggatcacagtttttaaaaggcaaacattttccctaaggaaacagacacaagctttcctagagaatatgatgttttttaggcattaataaggtccttttttataaaggacacttttctcctagtagttttgaattcaggaacagatccaaagttagcagtatatggctgctacatttccattttcattttcgagccatcagtttatgttcagatgccatctctgtaatcgcacatttaaaacataactgtagcctcactaatggaaaagtagtatgatgaacaatcattcccaatggtgtacaatgtaagggttttagggagcaacagtatttaactggaagaaagaattgcatatttaatgtagtctaatatatacacatttgtttaacatgtaaacaaaagtgttaaattcacatatacaacattatacaatttaatcactcttggaataaaatttttatagccttttttctattgggaaaatttgtttagatgtgtgccactccataggtttatttccaaaatgaatgagcccaactccatttgtaaaaacttgtcagttagaattcctttttttagtggattagggctgaattcttagatccttatttcttttcactttaaatgctgccaaagatcactactcatcattcaggaattcgctgtctagcctatctgtagtttcctgaagattgaaaattatgtagactgctatttaaaaatatatttttctaagtgtgaggtttaagatgctgtattgaccctatgagtttttaatgtgttaattatctttatagcataatagatcgctttaggttcctggaatcccatttggtctgacaggatatatgaagattcttaatacctattttctgtgtctaatacttggttaatactaaaaatagaaatgactaaattacatcacagaaagcataaccagtgattgaacctggtagttttaaagctctaaatagctgtggctgaaggactgattatggggctaagaagcttgaaacgtaagttggtacttgttcatcagtggattctcctaaattaagccaaattttgaaatacatgactattaagtttctactcatgtatttacagtcagtcaataaattaaaggaggaaaaaaatccctgaacaacctgcccataaaaagaaaaatactctacatttgagcctgctgcagttttaaattttccctctgggtcaagtttgccagcttttggctacagagaaattatatttccattacagtgcaggtagaaactctgtaaccttaagcatgtaaactacatagaataaaactgtttccactgcatttctgtccttcaaagtggccaacctgattaagtcagccttaatcactgctgctgtcagtttcacgactaaaggtcatattgactaagtagtcatcagctgaccacctcgctgtatcagccagcaacgaggggaaggtgaagaaacatgataggccatatagaatctgccctatgtttacttttttaacccagataattatttttgtgtgcagtatctaagctcctgattgtgtaacctgggacttctggcaccttttgttccattcattttatgtataaaatgcatgccaaagcacactgtgccctctggtacccttgcttccaatcgccaaccatgctcatttccttcctttttttgtggtccctttttgtggtgatcattttaaaccacgtcatccaacaaatgttttatggtcaaccttagcttgttcataagccatagcaactgaaagattaaactcttaaatatgtgtctgggcagtggctattaaatagcaaaaaacaatcagattttagtattttattatttccttgtaaaatggctgaactaaattaaacccttgtttcccatttgttctataatttatagtgaaactgagaacaaaactatctttataaatgatagctaaaagtatttccagatatttaaacaatttaaaataaatttcttctgcagagatgcaaagcatctcaacactggaatgaacaaatgccttaaattcaatggagtaaacctttagaatgaagaggaactgtcatttcacccaagccgaagacaacagccttatgcacttgtgtgctctgtctttgctgcttctcgtgtttcaagcctttcctgtgggatcagcacagcaaagtgcaacttaccaaatggtttaatgactggttaattctttcttctcccaatggaaaagcaatggcaacacaacagtagactgctggcttgacaatcttaaacgtgagcctttgcacatgtaggtttatcatcatttgagtatacgactaagcaagtcaatgaactttttttttttttttagcagtttaatttggtcctgagaatgttgcagtctttattaccccttttgcattaatccacttttctaaccaccttttaagctttaatttttaacactatacaccaagtctttgaaatcagtgatctgttatttaactctaaagcatttgacacttcttgccttaacagttttaaaaaccacacacaaaaaaactctgtaagtaatacagtaggccaaaagtttcatcctatctatcttgcagtttacctatctgatctgatctctgtaattatagttctgtcatttaaaatatactatttaaatctaatttttacatttcaaaaattatcttcagtagtaactaagtatattttctgtggattctgagaatgttatttttcagaatgtgagaatatatatgtacatttataatcttgtgactttaaagtctgttttcagatacagtatgtaaatacttgtaaaaaaatttgtataattttgtgataatgtagtttcccaaaaaaattatttagaaggcattatgttattagtaaatgagagcactgtatagaactgttcctattttctgcacttgccattccagctgcctccactgtccatacccacctcattcatcctgtcacagaaggcaggaaaactgggaactttaccaaagtagcactcagcctgagaggcctgtataatcatgcttttcaaactaaattcacttaaaaattaaaaagcagaattgaatattttaagcagcctcagtacctttggccaatgctgttttcatggtggattatgaacattatataatctttgggaaaagtgaaagtagtacaatttttagaataatgacaactgcctcactgcatctctccactcacacagcaaccgtgtagccccctaagctgcagtaccatgactaaccatgatgtcaatttcatatgctgatcctcacaacagcagtgcacaaacatgccccaaatattttaacagaatttagctcttccttaagctgtcttttcatagtaaaaacaaaacaaaaacacccaatgttaaaaccacataataaacttacaaacttgaaaaattagacacttcagatagataggcaataaaacttcatattatgaaagcaatatattccaagtttcaaagatttgacaagttctgtagagtatctttcatcagtacatgaaaacttccaaactgcatgatcttctgccaggcaggactgggtgctattcgctggtttgaggtcgaatccatttcaaggcatgtcgtggtgggacattaatggtgggatggtagaatgtgcagtccggtcttgtacattgagtgttaaacctacaatgttttggatgatagaagggacattccatcttcttacaagcagggaagtaacggcagagctgactactggaaggtggtgctggtggtgcaactgctggttttggagacagtactggaattcttctactcacatgagtgaagggacaatctggtttagtacactttgcatcatatttacaatttgggtgaacaaacaaacatttttcagcaaatttacaattggggaaggctttgcagggtgagatggggtgatggtaggcacactcatccccatttttacaagcaggccagtacttgcagcgctccaaaagtttttctggtttctgtgccacactcagttcactcatctcagcgttagaaaagctaccatttgggtcctcaagctgcctgctcagcaagtgcaactgctgtgggtggaggagacctctgagtcccttgtttgaggctgcagtttggtttacgggtttcattccttcaaagcacatgtcctcctcttgatctgacatgtatcctggggggctggggacaccatccagcgtcactataaacttgggacttgcaggtttatctggttgtacaagatctcttgactcatctgcagagtttctgccattactgggtcgatttgcagtcgggataataattgcctctgttgagttccttgatttttttctacagaatctccttttgtttcctcttctttaatggggggacttattctgggggtcctactttgtccctggaccacttctgctagcaattcttcttgagaagttcgagttctgggagcaactggaagtgtctgtttctgtggaactgtagagtagttagttgtttttgttacggattcttgagcttcagatatagccttcaaaatcagattcttgttagcttgtttagaaggtggaagagaaggtctcctttcaggctttgcaggcacagacacactgctggagatgcttcctgttcgagacccgtaatcatcatcttcttcctcctcttctccatcatgattgaatttttttactttaacaactgaacttaccacaggcaactttctcttccgaaagttttcatcctccatactcattttctccgagttgtttctaaagaacggactatacgtttcttctaagctgttaagcacctctggttcacacaaacgtcctgtttcatatacccaactactctgcatatcaagctgcttggcagcatgaatactattctgctgctgttgaaattgcaacctgtttaaatgaacaccactatctgcatttctacttgcaggtggtcgataaatttcaatagaagggcgagaagaaccatatgtaagtgtcactgtaggttttttctgagataagggattctcctgcacaaagttgaggtcttcgtcaatgagatcatctggttctggcttaatatcaatcacatcttcagagggtgctggctccctcaaaggtttcactgttgacattagtcgggttgcagctccatcatcgtaagtctgtctgacatttgtggtttttgactcctgcgaacttgtagaaactctggaatctcttttttcaggtctcgcgctaggaatggcaagtggtggcactgcagcttcatgcctcctctcatctccccgactgaaattgctcttgtttgaaggcacgttactatcaaagatgttggtatcagaagacttcagactagagggttcagttgtaacagagcgaagtttatctaatacaccatgaagccatacggtgaatcgaattgtgttgttccctagaaacagggacagatcctctgtcatttggtcctgacttttcttgttggccaccatcaccataatgtaatcaggaagttcttcatcaacataagctcctaattcttgtaatttccccttaatggcactccggatcttgcggctgatctcggtgccgatctccatggctctgcggcgtgcgggaactcagcactgcgcggcgcttggcttacccggaggctgccgcggactcctaccccgcagccgggacaccaccgcctcc

SEQ ID NO: 13614 - RNA, 16307 nt, Homo sapiens
  source 1..16307: mol_type = other RNA
gctgggattacaggcatgagccaccataataaggattctgatgaacatttgattccttggactactgttatactcaaaagccttccttaatcttctaattgtcaccctaaatatcctaaaatttctgtcttcctagtagttcttcatagtcctaaaaatttgtcagagagaaaggtaaatcaagaaacatgattttcaaatgatttaaggtggtactagggtttaggatttcctttgctttttatcatttaacacactgcttatcatacagctggaagtgctctgggccagtgtctctacttcgagggaagaaggaggtagtgagacagaaggaaatagcacaattcctggccctgacagaagggtgttcaggagacctgctctcctctcactttattccatctcatctggacctgtggcttccaatccacatctctttcctttaatatcctgcattggctaggctgtataaatcctttggtgcatcgaaaaactaagtgcattttttgtttttgtgattatgcaatacttataggaaaagttataattttagaatatttaagtacacttacatttttgagaaaaagactattgaaatgtttgtgccatgtcaaatttcagttgaacattttgggtattcttaatataagaccaggccaggcaccgtggctcaggccgggcacagtggctcacacctataatcccagcacttagggaggccaaggcgggaagatcacctgaagtcaggagttcaagaccagcctggctaacaaggtgaaactctgtctctactaaaaatacaaaaattagccgggcgtggtggctggcgcttgtaatcccagctacttgggaggctgagacaggagaatcacttgaacctgggaagcagaggttgtggtgagctgagatcgcaccattgcactccagcctgggcaacaaagagcgaaactccgtctcaaaaaaataaaaaataaaccctagaattatagtatgttagaattggaagggaagaattgtctaaggttattctagctaataagcaacagacttggaaaggaaaaggtcctgacaaagctaagcctcccgttcaggtttcctgactcgtgaattcagtgctgctgccactacacgatgcatgctctttgtatcaagggtgagacagcattacacatacatagaaaattatctatttaaactctatttgaacttttgatgagtttgtctccccctcccccactccttttcagaataacttgacgtttacaggtaccatcagtggtgatgtctgtgtgtggaaagatcacatattgtgtagaatcgtggcgagagctcacaacgggcctgtgtttgccatgtacaccaccctgcgagatggacttatcgtgactgggggaaaggaaaggccgtgagtcctctttcttttcacagaatatttatgcatttgtgacctacctgaggtttgcagttaattattctagttgtttctaggctacacagagtgtcctctccgaccttcctcctcatatgcttctcctttattaccttttatgtgccttctatttgattctcatttctggtcttaattcacttccaatttttttcatgttggggtgatactttttctgaggtgtggataggtagttgtcctacaagttgagttacttttcttaatgtctgtatgcctgtgtatgatttgctgagtaggaggcccatgggggaatctggagccagggttgtattttgactgcctgctctctttttgttcagaatggattctaaggagtagaatgcacattgttgctttagaaaaggatgagggaactagagagaactgccttgtttccttttgcttgaggcaaatttaaactgttttatacaagacctcaaaatttgagaagaggtctcttctgagtgattttcaaatctcccaacagtaaccagatacttatgatttgatttgtcaccaacatagtcatatgcatgttgaaacatgacatgtaggccaggcacagtggctcacacctgtaatcttatcactttgggaggctgaggcaggtggatcgcttgagcccaggagttcaagaccagcctgggcaacatggtgaaaccccatcgctataaaaaacaacaattagccgggtgtggtggcacatgcctgtagtccctgctactcaggaggctgaggtgggaggatcacttgagcctggggaggtcaaggctttagtgagctgtgatggtgccactgcactccagcctgggtgacagagtgagaccccatttaaaaaacaaaaacaaaaacaaaaaaaaatgtgacatatagttgactaagaagtacatttcaatacaggattgaaagaacccacatatgttaattaaacacaagcgcagaatttgtgccttttacataaaggaagaatgcacataggcatgctttcagacaagcaattcatctagcagaaaaggaaggaatacatttttcagcccttccaggaataaaatccataaatgggctctatttcgtcctccaacacttgtatttcccacgtcatttactcctgcacacccccactcactagaagcctgctaaactgttccagtgagatattttaacacctgatagggaataaatatgcttctgttttggccttcaaaaataagctctgggccagttgcagtggctcacgcctgtaatcccaacactttgggaggccgaggtgggcggatcacgaggtcaggagtttgggatcagcctggccaatatggtgaaactccatctctactaaaaatacaaaaattagccaggcatggtgcctgtaatcccagctacttgggaggctgaaggagaagaatcgcttgaacctgggaggcacaggttgcagtgagccgagatcacaccactgcactccaggccaggtgacagagcgacactctgtctcaaaaaaataaataaatcaactctgtagcatagcatttgtaattctattattttgccttacatttccattatccttttaataaaattgtttttttacatcttcctaatcaagaagtattatgaggccaggcacagtggctcatacctggaatcccagcactttgggaggccgaggcaggcagatcacctgaggtcaaggtatttgagaccagcctggccaacatggtgaaaccccatctctactaaaaatacagaaattagctgggtgtggtggtgcacacctgtaatgctagctactcgggaggctgaggtaggagaatcgcttgaacctgggaggcagaggttgcaataagcctagatcatgccactgcactcaagcctgggagacagagcgagactacatcttaaaaaaaaaaaaaaaagtattatgagagaggataatgtattgtaatgtattgtagaggctaaataaaattatgctcatgtcagaaaaaaagagtatttctcaaaataaaattcactgaaactggatgtttattttgactgagatatagtatatcctcaaattgccatagaaagtttacaagaatattagaggtaaattataaatatcagggcctttttaaaaaaaaaagattctgcttataacttggtatttgtttataataaaaattatagtagccaataatgaacacttactctggcttggttatttacttaggtcaaaagaaggaggagcggttaaactgtgggatcaggaactgaggcggtgccgtgccttcaggcttgagacaggacaagccacagattgtgttcgttctgtgtgcagaggcaaagtaagatgttccatgagctgatacagtgcagcagaaaacagaaagtggttattactgtgattccctcaccctttgcagcctaatgaacaatacttaataatgcataacgatggatttgcttgccaacattactctgtctttgctgctttctttgccaaagttagcaccagtgtggtgcataagctaggaagctattctgtctaaatactgtatgtaaacctccaatattttctagaatctgccaatttaacaactctagtagacataattgaaagcccttggcagttgactcatattaggacagctgtctccattttttaaaaaaacacacattccctagataaaacgtgcagtaaacaaacaatgaaatactactcagccataaaaaataatgaaattctgtcattcttggtggcaacatggatgagactggaggacatgatgtgaagtgaaataagccaggcacagaaagataaatacatgttctcactcctgtgcagaaactaaaaaagttgatcccacagaggtggagagtagaatagtggttactggaggcggacaagggggagggggagggggatagggaaggactggttaaaggatacaagtttacacagccagataggaatagtatgttttagtattctgtagtactgtaggatgactatagttaagaatcacgtatttatgtattttcaggtatttacaagagaggattttgaaagtttccatcacaaagaaatgataaatgtctgaggtgatggttatgcgtattaccctatgccctatagatatgtataattatgtgtcaatttcaaaataaaaattcaaaactacaactcctatgaaaatttttgagcgtgtttgtacttattaagtgtatttataaatcatacggatattatcttcagcctgcatattaaattgtagttaagcttttactttttaactaaaaaataaattctattattttttcctatatcccactgcactgaccccagtttggaaatcctaagattatcaaataaaaactttgattattgaagaatccaggtgtactgccacagaaaagttctattctgtagcatggactctaatatgtaatctagcccattgtgcttacagatagatgtgtgcctgtagtcatagaaaaatttgcatgagctaatgactgccttgctactagattagctcaaagcaaaaagttctctgaaagcaggtcaatagggtcatttttatattatgaagaagaaaagcagctgttgtattacattcactgtattggtcctgcttgtgtttcagggcaagatccttgttgggacaaggaatgctgaaataatcgaagttggagagaaaaatgcagcttgtaatattttagttaacggtcatgtggatgggccaatctggggactagcaacacatccttccagggattttttcctttctgctgcagaagatgggacagtgagactttgggatattgctgataaagtaagtacagataatttttttaaaagaggttacaacttctaaaaagaaaagttggaagttctaaattgctagtacttaaagaactgccagaattctgttgagcattttgaggggaaactggtataatttagaagtacttcacttaatgtttcctatgactctttttttttttttttttaaatgcagaagatgttaaacaaagtgaatttgggacatgctgctcgtactgtgtgttacagccctgaaggggacatggtggctattggaatgaaaaatggagaatttatcattttactagtgagttctctaaaaatatggggaaagaagagagacaggagatgtgcaatccatgatatcaggttagtgaacaaatggaatagagtttctagtatatacttgatttaacttccatttgtaaaattttccatagccttgccttcaaaaagaggtccccagggcctgtagcatttcccgtattataaattgtatgctaaaatatggctgtttgtatactacttaattcttcttgctaaattataaacccactgggcaccaactataatagcaagtactagtaggtaatgtttgatgaattcatgttaacacttagccatgtccattaagttcatcccaccaagaggtatctcccactgtaatacaagagagctatctgcccttcaaaagttgtcaccctggaaaactaaagttgtgatttcaaacatatcttctcttagtaacctcagtttgggaatatgtagttcattaatttaatcaatacctattgattaaatgttccagaatccaaattaatttaaatgtttcttaaacctttgtttttcagtgcttaagcatttttcaacagtggctaccatttacggagtacttccgtgtgatcagtagataagattattgaatctaggtctgtcaaaagcttgtacacttttcatcagtaaaatccttttacaaatgaaaccttcctcagaacttcaatatataaaatagtaacagtggcttcccttagcttttacatgtctctatcgtacctcagtaagactcatgggccatttcaagagactgaattgtcccatatgactccaaagattgctaggcaaatagcatttcactttgtcttttaaataagttcttcaggccgggcgcggtggctcatgcctgtaatcccagcactttgggaggccgaggcaggcagatcacctgaagtcaggagtactcgaccagcctggccaacatagtgaaaccccatctcaactaaaaatacaaaaatcagccgggcgtggtggcaggcgcctgtaatcccagctactcagggggctgaaacaggagaatcgcttgaacccgggaggcggaggttgcgccatcgcactccagcctgggagacaagagcgagacttcgtctcaaaaaaaaaaaattcttcttccaagattcaagttgtgtcatttcaccttaataactggaggttagttaagctgggctgtgttctttgcttaatattaagacaacgttttttccagatggaagaaaactatcttaatgaattgttagcttattaattatgtaatgctaatggcttttaaaagctgagatgttctgactgggtgttgtggctcacacctgtaatcccagtaccttgggaggccaagggggaaggattgcttgaggccaggagtttgggaccatagtgagaccccgcctctatttaaaaaattaaattttgttttgttttgttttgagttggagttttgctcttgttgcccatgctgaagtgcaatggtgcaatctcagctcaccacaacctgtgcctcctgggttcaagcgattctcctgcttcagcctcccgagtagatgggattacaggcgtgcaccaccatgcctggctaattttgtatttttagtagagacagggtttctctatgttggtcaggctggtctcaaactctcgacctcaggtgatctgcccgcctccgcttcccaaagttctgggattataggtgtgagccactgggcctggcctaagaaagtttttttaagccattagacgtttttaaaggaattgggagatgacaattggggaaatatttaaaatttaagtaaaatataaagcttccttatttcatgtaacccagacaatctcagtatacatgatcagttgtgtctgacaggtaaatctatttgaggccttatcacacgttacttttaagaactagaaaggaaaagtcactgatcttaagtatttataatacttcatgtggtctaatactttttacgttttgttttgattcagatttagtccggattcccggtatctggcagtaggttctagtgagaactcagtggatttttatgacctaacgctgggccccactcttaacagaatcagctactgcaaagacattccaagctttgtcattcaaatggacttctctgcagatagcagttatctccaggtacagtaccaatactgtatacccaggtggcaagttcttctgcttttacatttcgtgttagtgaatgcatttaaagttcctgagctccagagctccagcttctcaactcctccctttgtaccttctgacctacagctcccctttcctcccccacttatcagagcttttctcctattaagtttttgtagtgatcttttgcatacttaataatgttagacatgtaaatcaagtagcaatatgctagtattctgtaaaccccctgtggattttgtctctcacctaatggaattcttgtcccattttaatctgatgaaaaaggtctctagtggctgctataaacggcatgtctatgaagtgccttcaggaaaacatcttatggatcatgccgctattgacagaattacttgggctacatggactaggtaaatacttatatattcacaaggcaagaactgactttgaaggccagttagaaaatcctatttctgaactgttagagccattccaataaggaatagtaattgagtttcaagtttttgttaccatattttgaaatggtatgttcatgttgggacccctttttattgaatatatttccatgttttatcagtttccatgatttatcaagttttttttttaaggaaatcaaagttttaactttaaagataccctgatatttttcttaatgctaaatttaatgactggcaaaaaggtattgggtgctgttaagcaactgttattaattctctatctaaaggaatgctatcttgaatctattagaagtcaaagcttccaaatttgttcaaatttcctggctgtatgacaggtaaccatgactatccatttttttggccaatgaaaaatgccatcaaattcctgtatcagccaggcatatagtggctcatgcctgtaatctctgatgtagcaggccgaggtgggaggatcacttgagcctagaagttttgataccagcctgggcaacatagcaagaccccatctctgaaatttttttaattcctatgtcataagtcatttttatttttgtagagatagggatctcacaatattgcccaggctggtctcaaactcttggcctcaagcagtcctcctgcctcagcctcccaaaatgttgggattactggtatgtgctgctggacccagccaagtagcacttttaatttgaaaaatagttctatcagttttcagtcaggcgcggtggctcagcctgtaatcccagcactttgggaggccgagcgggggtgatcacctgaggtcgggagttcgagactagcctgaccaacatggagaaaccctgtctctactaaaaatacaaaataagccgggcatgttagcgcatgcctgtgatcccagctactcgggaggctgaggcaggagaattgcttgaacccaggaggcagaggttgcggtgagccgagatcatgccattgcactccagcctgggtaacaagagcgaaaactccgtctcaaaaaaaaaaaaagaaaaaatagttctatcagttttcataaagtactactttaatcttaaaaagattaatctagaaacccttcaaattataaaatgtcatttttaaaaggcaggagttgatatcctgatgaaattcaggtctccaaacaacttaccataatttacttcctgtattttaagtaacatgatagggtacttagagattaattgccaagaaactttttgaatatagtcaacctgcccgcacttgccatgatgagttttcttttgttccttccctctagtattctaggagatgaggttttgggaatctggtccagacatgctgagaaagctgatgtcaactgtgcctgtgtatctcattcaggaatcagtcttgttacaggagatgactttggcatggttaagttatttgacttcccatgtccagaaaaatttgtaagtttgtgttttgtttactattatcagtttactcctaattttgatgtcttatcatcagcacttttccccatatatttaaaatgttttgtcctaatttctaaatttttccccaaactttctaaatctatttactttgaaataaaagctattagaaacaaatcctctccctcgagtaataccatctttggaaccatcctacaaaagctgtaattagcttttcaccaaacctataatcagttatcaaatttcaaatgcttttccttagagaaaaatggtcagagtacctggagacatctgactgcccacacagcctggttttgcagatccactactcatgctgaaaagcattctaatcactggctgcggtgctaactccctactctctccacagctcttgtcatagagattatagttcctaataagagcctttgacttctgtgtgcaccaaatgccctgagcttgtctgtcattgttttttaggcaaaacacaaaaggttcttgggtcattcgccccatgtgacaaatattcgatttaccagtggtgatcgacatgttgttagtgctggaggtgatgactgcaggttagtaactttctcagcccatgaagagcagactatgttactagttaagagacttaatacaacaactcctacagctttggtttatgaaatcagctagtcaacattagtagaaggtagtataaccagatggctcttcagaatctcatatttatgcaaatacagaataaaaggagttaaagaggaaaaatattacacatgtaacctgaaagcacaactgaaaaatattaaactgttatgaaaatctaaaaacataattaactccctgcaattttcttctctgattgcagcttatttgtctggaaatgtgtacatacacctcactgagagatgctgagatgactacagaaattaactttgagaccagaattacagagaagaaaaaccaaaacccaaccctgcatggtcaagtggtgctaacccaagactgtaacagggagaaatgcccagaatcatcaaaatagtgaaagactgatctgttcaaaatatttgctatatgcactgggtataatccgtaatccatacactgccagataatgccatttcaaggaaggatcgaatacttgatggtaaaggccaagtccccctgtattgggaagtgtgtgatttcggcagacctgctgggaaaatttagggtagagcactctttacagaagaactcaaaaacccaatttggataattttcattatctttttagcaaaatggtttcttaatgtttatattttattttcaaggttcattgtttaatgaaatattttattcttgcatttccataaggaaagggaaagtcatgatcatcctaaaggatcacagtttttaaaaggcaaacattttccctaaggaaacagacacaagctttcctagagaatatgatgttttttaggcattaataaggtccttttttataaaggacacttttctcctagtagttttgaattcaggaacagatccaaagttagcagtatatggctgctacatttccattttcattttcgagccatcagtttatgttcagatgccatctctgtaatcgcacatttaaaacataactgtagcctcactaatggaaaagtagtatgatgaacaatcattcccaatggtgtacaatgtaagggttttagggagcaacagtatttaactggaagaaagaattgcatatttaatgtagtctaatatatacacatttgtttaacatgtaaacaaaagtgttaaattcacatatacaacattatacaatttaatcactcttggaataaaatttttatagccttttttctattgggaaaatttgtttagatgtgtgccactccataggtttatttccaaaatgaatgagcccaactccatttgtaaaaacttgtcagttagaattcctttttttagtggattagggctgaattcttagatccttatttcttttcactttaaatgctgccaaagatcactactcatcattcaggaattcgctgtctagcctatctgtagtttcctgaagattgaaaattatgtagactgctatttaaaaatatatttttctaagtgtgaggtttaagatgctgtattgaccctatgagtttttaatgtgttaattatctttatagcataatagatcgctttaggttcctggaatcccatttggtctgacaggatatatgaagattcttaatacctattttctgtgtctaatacttggttaatactaaaaatagaaatgactaaattacatcacagaaagcataaccagtgattgaacctggtagttttaaagctctaaatagctgtggctgaaggactgattatggggctaagaagcttgaaacgtaagttggtacttgttcatcagtggattctcctaaattaagccaaattttgaaatacatgactattaagtttctactcatgtatttacagtcagtcaataaattaaaggaggaaaaaaatccctgaacaacctgcccataaaaagaaaaatactctacatttgagcctgctgcagttttaaattttccctctgggtcaagtttgccagcttttggctacagagaaattatatttccattacagtgcaggtagaaactctgtaaccttaagcatgtaaactacatagaataaaactgtttccactgcatttctgtccttcaaagtggccaacctgattaagtcagccttaatcactgctgctgtcagtttcacgactaaaggtcatattgactaagtagtcatcagctgaccacctcgctgtatcagccagcaacgaggggaaggtgaagaaacatgataggccatatagaatctgccctatgtttacttttttaacccagataattatttttgtgtgcagtatctaagctcctgattgtgtaacctgggacttctggcaccttttgttccattcattttatgtataaaatgcatgccaaagcacactgtgccctctggtacccttgcttccaatcgccaaccatgctcatttccttcctttttttgtggtccctttttgtggtgatcattttaaaccacgtcatccaacaaatgttttatggtcaaccttagcttgttcataagccatagcaactgaaagattaaactcttaaatatgtgtctgggcagtggctattaaatagcaaaaaacaatcagattttagtattttattatttccttgtaaaatggctgaactaaattaaacccttgtttcccatttgttctataatttatagtgaaactgagaacaaaactatctttataaatgatagctaaaagtatttccagatatttaaacaatttaaaataaatttcttctgcagagatgcaaagcatctcaacactggaatgaacaaatgccttaaattcaatggagtaaacctttagaatgaagaggaactgtcatttcacccaagccgaagacaacagccttatgcacttgtgtgctctgtctttgctgcttctcgtgtttcaagcctttcctgtgggatcagcacagcaaagtgcaacttaccaaatggtttaatgactggttaattctttcttctcccaatggaaaagcaatggcaacacaacagtagactgctggcttgacaatcttaaacgtgagcctttgcacatgtaggtttatcatcatttgagtatacgactaagcaagtcaatgaactttttttttttttttagcagtttaatttggtcctgagaatgttgcagtctttattaccccttttgcattaatccacttttctaaccaccttttaagctttaatttttaacactatacaccaagtctttgaaatcagtgatctgttatttaactctaaagcatttgacacttcttgccttaacagttttaaaaaccacacacaaaaaaactctgtaagtaatacagtaggccaaaagtttcatcctatctatcttgcagtttacctatctgatctgatctctgtaattatagttctgtcatttaaaatatactatttaaatctaatttttacatttcaaaaattatcttcagtagtaactaagtatattttctgtggattctgagaatgttatttttcagaatgtgagaatatatatgtacatttataatcttgtgactttaaagtctgttttcagatacagtatgtaaatacttgtaaaaaaatttgtataattttgtgataatgtagtttcccaaaaaaattatttagaaggcattatgttattagtaaatgagagcactgtatagaactgttcctattttctgcacttgccattccagctgcctccactgtccatacccacctcattcatcctgtcacagaaggcaggaaaactgggaactttaccaaagtagcactcagcctgagaggcctgtataatcatgcttttcaaactaaattcacttaaaaattaaaaagcagaattgaatattttaagcagcctcagtacctttggccaatgctgttttcatggtggattatgaacattatataatctttgggaaaagtgaaagtagtacaatttttagaataatgacaactgcctcactgcatctctccactcacacagcaaccgtgtagccccctaagctgcagtaccatgactaaccatgatgtcaatttcatatgctgatcctcacaacagcagtgcacaaacatgccccaaatattttaacagaatttagctcttccttaagctgtcttttcatagtaaaaacaaaacaaaaacacccaatgttaaaaccacataataaacttacaaacttgaaaaattagacacttcagatagataggcaataaaacttcatattatgaaagcaatatattccaagtttcaaagatttgacaagttctgtagagtatctttcatcagtacatgaaaacttccaaactgcatgatcttctgccaggcaggactgggtgctattcgctggtttgaggtcgaatccatttcaaggcatgtcgtggtgggacattaatggtgggatggtagaatgtgcagtccggtcttgtacattgagtgttaaacctacaatgttttggatgatagaagggacattccatcttcttacaagcagggaagtaacggcagagctgactactggaaggtggtgctggtggtgcaactgctggttttggagacagtactggaattcttctactcacatgagtgaagggacaatctggtttagtacactttgcatcatatttacaatttgggtgaacaaacaaacatttttcagcaaatttacaattggggaaggctttgcagggtgagatggggtgatggtaggcacactcatccccatttttacaagcaggccagtacttgcagcgctccaaaagtttttctggtttctgtgccacactcagttcactcatctcagctgtagagtagttagttgtttttgttacggattcttgagcttcagatatagccttcaaaatcagattcttgttagcttgtttagaaggtggaagagaaggtctcctttcaggctttgcaggcacagacacactgctggagatgcttcctgttcgagacccgtaatcatcatcttcttcctcctcttctccatcatgattgaatttttttactttaacaactgaacttaccacaggcaactttctcttccgaaagttttcatcctccatactcattttctccgagttgtttctaaagaacggactatacgtttcttctaagctgttaagcacctctggttcacacaaacgtcctgtttcatatacccaactactctgcatatcaagctgcttggcagcatgaatactattctgctgctgttgaaattgcaacctgtttaaatgaacaccactatctgcatttctacttgcaggtggtcgataaatttcaatagaagggcgagaagaaccatatgtaagtgtcactgtaggttttttctgagataagggattctcctgcacaaagttgaggtcttcgtcaatgagatcatctggttctggcttaatatcaatcacatcttcagagggtgctggctccctcaaaggtttcactgttgacattagtcgggttgcagctccatcatcgtaagtctgtctgacatttgtggtttttgactcctgcgaacttgtagaaactctggaatctcttttttcaggtctcgcgctaggaatggcaagtggtggcactgcagcttcatgcctcctctcatctccccgactgaaattgctcttgtttgaaggcacgttactatcaaagatgttggtatcagaagacttcagactagagggttcagttgtaacagagcgaagtttatctaatacaccatgaagccatacggtgaatcgaattgtgttgttccctagaaacagggacagatcctctgtcatttggtcctgacttttcttgttggccaccatcaccataatgtaatcaggaagttcttcatcaacataagctcctaattcttgtaatttccccttaatggcactccggatcttgcggctgatctcggtgccgatctccatggctctgcggcgtgcgggaactcagcactgcgcggcgcttggcttacccggaggctgccgcggactcctaccccgcagccgggacaccaccgcctcc

SEQ ID NO: 13615 - RNA, 16423 nt, Homo sapiens
  source 1..16423: mol_type = other RNA
gctgggattacaggcatgagccaccataataaggattctgatgaacatttgattccttggactactgttatactcaaaagccttccttaatcttctaattgtcaccctaaatatcctaaaatttctgtcttcctagtagttcttcatagtcctaaaaatttgtcagagagaaaggtaaatcaagaaacatgattttcaaatgatttaaggtggtactagggtttaggatttcctttgctttttatcatttaacacactgcttatcatacagctggaagtgctctgggccagtgtctctacttcgagggaagaaggaggtagtgagacagaaggaaatagcacaattcctggccctgacagaagggtgttcaggagacctgctctcctctcactttattccatctcatctggacctgtggcttccaatccacatctctttcctttaatatcctgcattggctaggctgtataaatcctttggtgcatcgaaaaactaagtgcattttttgtttttgtgattatgcaatacttataggaaaagttataattttagaatatttaagtacacttacatttttgagaaaaagactattgaaatgtttgtgccatgtcaaatttcagttgaacattttgggtattcttaatataagaccaggccaggcaccgtggctcaggccgggcacagtggctcacacctataatcccagcacttagggaggccaaggcgggaagatcacctgaagtcaggagttcaagaccagcctggctaacaaggtgaaactctgtctctactaaaaatacaaaaattagccgggcgtggtggctggcgcttgtaatcccagctacttgggaggctgagacaggagaatcacttgaacctgggaagcagaggttgtggtgagctgagatcgcaccattgcactccagcctgggcaacaaagagcgaaactccgtctcaaaaaaataaaaaataaaccctagaattatagtatgttagaattggaagggaagaattgtctaaggttattctagctaataagcaacagacttggaaaggaaaaggtcctgacaaagctaagcctcccgttcaggtttcctgactcgtgaattcagtgctgctgccactacacgatgcatgctctttgtatcaagggtgagacagcattacacatacatagaaaattatctatttaaactctatttgaacttttgatgagtttgtctccccctcccccactccttttcagaataacttgacgtttacaggtaccatcagtggtgatgtctgtgtgtggaaagatcacatattgtgtagaatcgtggcgagagctcacaacgggcctgtgtttgccatgtacaccaccctgcgagatggacttatcgtgactgggggaaaggaaaggccgtgagtcctctttcttttcacagaatatttatgcatttgtgacctacctgaggtttgcagttaattattctagttgtttctaggctacacagagtgtcctctccgaccttcctcctcatatgcttctcctttattaccttttatgtgccttctatttgattctcatttctggtcttaattcacttccaatttttttcatgttggggtgatactttttctgaggtgtggataggtagttgtcctacaagttgagttacttttcttaatgtctgtatgcctgtgtatgatttgctgagtaggaggcccatgggggaatctggagccagggttgtattttgactgcctgctctctttttgttcagaatggattctaaggagtagaatgcacattgttgctttagaaaaggatgagggaactagagagaactgccttgtttccttttgcttgaggcaaatttaaactgttttatacaagacctcaaaatttgagaagaggtctcttctgagtgattttcaaatctcccaacagtaaccagatacttatgatttgatttgtcaccaacatagtcatatgcatgttgaaacatgacatgtaggccaggcacagtggctcacacctgtaatcttatcactttgggaggctgaggcaggtggatcgcttgagcccaggagttcaagaccagcctgggcaacatggtgaaaccccatcgctataaaaaacaacaattagccgggtgtggtggcacatgcctgtagtccctgctactcaggaggctgaggtgggaggatcacttgagcctggggaggtcaaggctttagtgagctgtgatggtgccactgcactccagcctgggtgacagagtgagaccccatttaaaaaacaaaaacaaaaacaaaaaaaaatgtgacatatagttgactaagaagtacatttcaatacaggattgaaagaacccacatatgttaattaaacacaagcgcagaatttgtgccttttacataaaggaagaatgcacataggcatgctttcagacaagcaattcatctagcagaaaaggaaggaatacatttttcagcccttccaggaataaaatccataaatgggctctatttcgtcctccaacacttgtatttcccacgtcatttactcctgcacacccccactcactagaagcctgctaaactgttccagtgagatattttaacacctgatagggaataaatatgcttctgttttggccttcaaaaataagctctgggccagttgcagtggctcacgcctgtaatcccaacactttgggaggccgaggtgggcggatcacgaggtcaggagtttgggatcagcctggccaatatggtgaaactccatctctactaaaaatacaaaaattagccaggcatggtgcctgtaatcccagctacttgggaggctgaaggagaagaatcgcttgaacctgggaggcacaggttgcagtgagccgagatcacaccactgcactccaggccaggtgacagagcgacactctgtctcaaaaaaataaataaatcaactctgtagcatagcatttgtaattctattattttgccttacatttccattatccttttaataaaattgtttttttacatcttcctaatcaagaagtattatgaggccaggcacagtggctcatacctggaatcccagcactttgggaggccgaggcaggcagatcacctgaggtcaaggtatttgagaccagcctggccaacatggtgaaaccccatctctactaaaaatacagaaattagctgggtgtggtggtgcacacctgtaatgctagctactcgggaggctgaggtaggagaatcgcttgaacctgggaggcagaggttgcaataagcctagatcatgccactgcactcaagcctgggagacagagcgagactacatcttaaaaaaaaaaaaaaaagtattatgagagaggataatgtattgtaatgtattgtagaggctaaataaaattatgctcatgtcagaaaaaaagagtatttctcaaaataaaattcactgaaactggatgtttattttgactgagatatagtatatcctcaaattgccatagaaagtttacaagaatattagaggtaaattataaatatcagggcctttttaaaaaaaaaagattctgcttataacttggtatttgtttataataaaaattatagtagccaataatgaacacttactctggcttggttatttacttaggtcaaaagaaggaggagcggttaaactgtgggatcaggaactgaggcggtgccgtgccttcaggcttgagacaggacaagccacagattgtgttcgttctgtgtgcagaggcaaagtaagatgttccatgagctgatacagtgcagcagaaaacagaaagtggttattactgtgattccctcaccctttgcagcctaatgaacaatacttaataatgcataacgatggatttgcttgccaacattactctgtctttgctgctttctttgccaaagttagcaccagtgtggtgcataagctaggaagctattctgtctaaatactgtatgtaaacctccaatattttctagaatctgccaatttaacaactctagtagacataattgaaagcccttggcagttgactcatattaggacagctgtctccattttttaaaaaaacacacattccctagataaaacgtgcagtaaacaaacaatgaaatactactcagccataaaaaataatgaaattctgtcattcttggtggcaacatggatgagactggaggacatgatgtgaagtgaaataagccaggcacagaaagataaatacatgttctcactcctgtgcagaaactaaaaaagttgatcccacagaggtggagagtagaatagtggttactggaggcggacaagggggagggggagggggatagggaaggactggttaaaggatacaagtttacacagccagataggaatagtatgttttagtattctgtagtactgtaggatgactatagttaagaatcacgtatttatgtattttcaggtatttacaagagaggattttgaaagtttccatcacaaagaaatgataaatgtctgaggtgatggttatgcgtattaccctatgccctatagatatgtataattatgtgtcaatttcaaaataaaaattcaaaactacaactcctatgaaaatttttgagcgtgtttgtacttattaagtgtatttataaatcatacggatattatcttcagcctgcatattaaattgtagttaagcttttactttttaactaaaaaataaattctattattttttcctatatcccactgcactgaccccagtttggaaatcctaagattatcaaataaaaactttgattattgaagaatccaggtgtactgccacagaaaagttctattctgtagcatggactctaatatgtaatctagcccattgtgcttacagatagatgtgtgcctgtagtcatagaaaaatttgcatgagctaatgactgccttgctactagattagctcaaagcaaaaagttctctgaaagcaggtcaatagggtcatttttatattatgaagaagaaaagcagctgttgtattacattcactgtattggtcctgcttgtgtttcagggcaagatccttgttgggacaaggaatgctgaaataatcgaagttggagagaaaaatgcagcttgtaatattttagttaacggtcatgtggatgggccaatctggggactagcaacacatccttccagggattttttcctttctgctgcagaagatgggacagtgagactttgggatattgctgataaagtaagtacagataatttttttaaaagaggttacaacttctaaaaagaaaagttggaagttctaaattgctagtacttaaagaactgccagaattctgttgagcattttgaggggaaactggtataatttagaagtacttcacttaatgtttcctatgactctttttttttttttttttaaatgcagaagatgttaaacaaagtgaatttgggacatgctgctcgtactgtgtgttacagccctgaaggggacatggtggctattggaatgaaaaatggagaatttatcattttactagtgagttctctaaaaatatggggaaagaagagagacaggagatgtgcaatccatgatatcaggttagtgaacaaatggaatagagtttctagtatatacttgatttaacttccatttgtaaaattttccatagccttgccttcaaaaagaggtccccagggcctgtagcatttcccgtattataaattgtatgctaaaatatggctgtttgtatactacttaattcttcttgctaaattataaacccactgggcaccaactataatagcaagtactagtaggtaatgtttgatgaattcatgttaacacttagccatgtccattaagttcatcccaccaagaggtatctcccactgtaatacaagagagctatctgcccttcaaaagttgtcaccctggaaaactaaagttgtgatttcaaacatatcttctcttagtaacctcagtttgggaatatgtagttcattaatttaatcaatacctattgattaaatgttccagaatccaaattaatttaaatgtttcttaaacctttgtttttcagtgcttaagcatttttcaacagtggctaccatttacggagtacttccgtgtgatcagtagataagattattgaatctaggtctgtcaaaagcttgtacacttttcatcagtaaaatccttttacaaatgaaaccttcctcagaacttcaatatataaaatagtaacagtggcttcccttagcttttacatgtctctatcgtacctcagtaagactcatgggccatttcaagagactgaattgtcccatatgactccaaagattgctaggcaaatagcatttcactttgtcttttaaataagttcttcaggccgggcgcggtggctcatgcctgtaatcccagcactttgggaggccgaggcaggcagatcacctgaagtcaggagtactcgaccagcctggccaacatagtgaaaccccatctcaactaaaaatacaaaaatcagccgggcgtggtggcaggcgcctgtaatcccagctactcagggggctgaaacaggagaatcgcttgaacccgggaggcggaggttgcgccatcgcactccagcctgggagacaagagcgagacttcgtctcaaaaaaaaaaaattcttcttccaagattcaagttgtgtcatttcaccttaataactggaggttagttaagctgggctgtgttctttgcttaatattaagacaacgttttttccagatggaagaaaactatcttaatgaattgttagcttattaattatgtaatgctaatggcttttaaaagctgagatgttctgactgggtgttgtggctcacacctgtaatcccagtaccttgggaggccaagggggaaggattgcttgaggccaggagtttgggaccatagtgagaccccgcctctatttaaaaaattaaattttgttttgttttgttttgagttggagttttgctcttgttgcccatgctgaagtgcaatggtgcaatctcagctcaccacaacctgtgcctcctgggttcaagcgattctcctgcttcagcctcccgagtagatgggattacaggcgtgcaccaccatgcctggctaattttgtatttttagtagagacagggtttctctatgttggtcaggctggtctcaaactctcgacctcaggtgatctgcccgcctccgcttcccaaagttctgggattataggtgtgagccactgggcctggcctaagaaagtttttttaagccattagacgtttttaaaggaattgggagatgacaattggggaaatatttaaaatttaagtaaaatataaagcttccttatttcatgtaacccagacaatctcagtatacatgatcagttgtgtctgacaggtaaatctatttgaggccttatcacacgttacttttaagaactagaaaggaaaagtcactgatcttaagtatttataatacttcatgtggtctaatactttttacgttttgttttgattcagatttagtccggattcccggtatctggcagtaggttctagtgagaactcagtggatttttatgacctaacgctgggccccactcttaacagaatcagctactgcaaagacattccaagctttgtcattcaaatggacttctctgcagatagcagttatctccaggtacagtaccaatactgtatacccaggtggcaagttcttctgcttttacatttcgtgttagtgaatgcatttaaagttcctgagctccagagctccagcttctcaactcctccctttgtaccttctgacctacagctcccctttcctcccccacttatcagagcttttctcctattaagtttttgtagtgatcttttgcatacttaataatgttagacatgtaaatcaagtagcaatatgctagtattctgtaaaccccctgtggattttgtctctcacctaatggaattcttgtcccattttaatctgatgaaaaaggtctctagtggctgctataaacggcatgtctatgaagtgccttcaggaaaacatcttatggatcatgccgctattgacagaattacttgggctacatggactaggtaaatacttatatattcacaaggcaagaactgactttgaaggccagttagaaaatcctatttctgaactgttagagccattccaataaggaatagtaattgagtttcaagtttttgttaccatattttgaaatggtatgttcatgttgggacccctttttattgaatatatttccatgttttatcagtttccatgatttatcaagttttttttttaaggaaatcaaagttttaactttaaagataccctgatatttttcttaatgctaaatttaatgactggcaaaaaggtattgggtgctgttaagcaactgttattaattctctatctaaaggaatgctatcttgaatctattagaagtcaaagcttccaaatttgttcaaatttcctggctgtatgacaggtaaccatgactatccatttttttggccaatgaaaaatgccatcaaattcctgtatcagccaggcatatagtggctcatgcctgtaatctctgatgtagcaggccgaggtgggaggatcacttgagcctagaagttttgataccagcctgggcaacatagcaagaccccatctctgaaatttttttaattcctatgtcataagtcatttttatttttgtagagatagggatctcacaatattgcccaggctggtctcaaactcttggcctcaagcagtcctcctgcctcagcctcccaaaatgttgggattactggtatgtgctgctggacccagccaagtagcacttttaatttgaaaaatagttctatcagttttcagtcaggcgcggtggctcagcctgtaatcccagcactttgggaggccgagcgggggtgatcacctgaggtcgggagttcgagactagcctgaccaacatggagaaaccctgtctctactaaaaatacaaaataagccgggcatgttagcgcatgcctgtgatcccagctactcgggaggctgaggcaggagaattgcttgaacccaggaggcagaggttgcggtgagccgagatcatgccattgcactccagcctgggtaacaagagcgaaaactccgtctcaaaaaaaaaaaaagaaaaaatagttctatcagttttcataaagtactactttaatcttaaaaagattaatctagaaacccttcaaattataaaatgtcatttttaaaaggcaggagttgatatcctgatgaaattcaggtctccaaacaacttaccataatttacttcctgtattttaagtaacatgatagggtacttagagattaattgccaagaaactttttgaatatagtcaacctgcccgcacttgccatgatgagttttcttttgttccttccctctagtattctaggagatgaggttttgggaatctggtccagacatgctgagaaagctgatgtcaactgtgcctgtgtatctcattcaggaatcagtcttgttacaggagatgactttggcatggttaagttatttgacttcccatgtccagaaaaatttgtaagtttgtgttttgtttactattatcagtttactcctaattttgatgtcttatcatcagcacttttccccatatatttaaaatgttttgtcctaatttctaaatttttccccaaactttctaaatctatttactttgaaataaaagctattagaaacaaatcctctccctcgagtaataccatctttggaaccatcctacaaaagctgtaattagcttttcaccaaacctataatcagttatcaaatttcaaatgcttttccttagagaaaaatggtcagagtacctggagacatctgactgcccacacagcctggttttgcagatccactactcatgctgaaaagcattctaatcactggctgcggtgctaactccctactctctccacagctcttgtcatagagattatagttcctaataagagcctttgacttctgtgtgcaccaaatgccctgagcttgtctgtcattgttttttaggcaaaacacaaaaggttcttgggtcattcgccccatgtgacaaatattcgatttaccagtggtgatcgacatgttgttagtgctggaggtgatgactgcaggttagtaactttctcagcccatgaagagcagactatgttactagttaagagacttaatacaacaactcctacagctttggtttatgaaatcagctagtcaacattagtagaaggtagtataaccagatggctcttcagaatctcatatttatgcaaatacagaataaaaggagttaaagaggaaaaatattacacatgtaacctgaaagcacaactgaaaaatattaaactgttatgaaaatctaaaaacataattaactccctgcaattttcttctctgattgcagcttatttgtctggaaatgtgtacatacacctcactgagagatgctgagatgactacagaaattaactttgagaccagaattacagagaagaaaaaccaaaacccaaccctgcatggtcaagtggtgctaacccaagactgtaacagggagaaatgcccagaatcatcaaaatagtgaaagactgatctgttcaaaatatttgctatatgcactgggtataatccgtaatccatacactgccagataatgccatttcaaggaaggatcgaatacttgatggtaaaggccaagtccccctgtattgggaagtgtgtgatttcggcagacctgctgggaaaatttagggtagagcactctttacagaagaactcaaaaacccaatttggataattttcattatctttttagcaaaatggtttcttaatgtttatattttattttcaaggttcattgtttaatgaaatattttattcttgcatttccataaggaaagggaaagtcatgatcatcctaaaggatcacagtttttaaaaggcaaacattttccctaaggaaacagacacaagctttcctagagaatatgatgttttttaggcattaataaggtccttttttataaaggacacttttctcctagtagttttgaattcaggaacagatccaaagttagcagtatatggctgctacatttccattttcattttcgagccatcagtttatgttcagatgccatctctgtaatcgcacatttaaaacataactgtagcctcactaatggaaaagtagtatgatgaacaatcattcccaatggtgtacaatgtaagggttttagggagcaacagtatttaactggaagaaagaattgcatatttaatgtagtctaatatatacacatttgtttaacatgtaaacaaaagtgttaaattcacatatacaacattatacaatttaatcactcttggaataaaatttttatagccttttttctattgggaaaatttgtttagatgtgtgccactccataggtttatttccaaaatgaatgagcccaactccatttgtaaaaacttgtcagttagaattcctttttttagtggattagggctgaattcttagatccttatttcttttcactttaaatgctgccaaagatcactactcatcattcaggaattcgctgtctagcctatctgtagtttcctgaagattgaaaattatgtagactgctatttaaaaatatatttttctaagtgtgaggtttaagatgctgtattgaccctatgagtttttaatgtgttaattatctttatagcataatagatcgctttaggttcctggaatcccatttggtctgacaggatatatgaagattcttaatacctattttctgtgtctaatacttggttaatactaaaaatagaaatgactaaattacatcacagaaagcataaccagtgattgaacctggtagttttaaagctctaaatagctgtggctgaaggactgattatggggctaagaagcttgaaacgtaagttggtacttgttcatcagtggattctcctaaattaagccaaattttgaaatacatgactattaagtttctactcatgtatttacagtcagtcaataaattaaaggaggaaaaaaatccctgaacaacctgcccataaaaagaaaaatactctacatttgagcctgctgcagttttaaattttccctctgggtcaagtttgccagcttttggctacagagaaattatatttccattacagtgcaggtagaaactctgtaaccttaagcatgtaaactacatagaataaaactgtttccactgcatttctgtccttcaaagtggccaacctgattaagtcagccttaatcactgctgctgtcagtttcacgactaaaggtcatattgactaagtagtcatcagctgaccacctcgctgtatcagccagcaacgaggggaaggtgaagaaacatgataggccatatagaatctgccctatgtttacttttttaacccagataattatttttgtgtgcagtatctaagctcctgattgtgtaacctgggacttctggcaccttttgttccattcattttatgtataaaatgcatgccaaagcacactgtgccctctggtacccttgcttccaatcgccaaccatgctcatttccttcctttttttgtggtccctttttgtggtgatcattttaaaccacgtcatccaacaaatgttttatggtcaaccttagcttgttcataagccatagcaactgaaagattaaactcttaaatatgtgtctgggcagtggctattaaatagcaaaaaacaatcagattttagtattttattatttccttgtaaaatggctgaactaaattaaacccttgtttcccatttgttctataatttatagtgaaactgagaacaaaactatctttataaatgatagctaaaagtatttccagatatttaaacaatttaaaataaatttcttctgcagagatgcaaagcatctcaacactggaatgaacaaatgccttaaattcaatggagtaaacctttagaatgaagaggaactgtcatttcacccaagccgaagacaacagccttatgcacttgtgtgctctgtctttgctgcttctcgtgtttcaagcctttcctgtgggatcagcacagcaaagtgcaacttaccaaatggtttaatgactggttaattctttcttctcccaatggaaaagcaatggcaacacaacagtagactgctggcttgacaatcttaaacgtgagcctttgcacatgtaggtttatcatcatttgagtatacgactaagcaagtcaatgaactttttttttttttttagcagtttaatttggtcctgagaatgttgcagtctttattaccccttttgcattaatccacttttctaaccaccttttaagctttaatttttaacactatacaccaagtctttgaaatcagtgatctgttatttaactctaaagcatttgacacttcttgccttaacagttttaaaaaccacacacaaaaaaactctgtaagtaatacagtaggccaaaagtttcatcctatctatcttgcagtttacctatctgatctgatctctgtaattatagttctgtcatttaaaatatactatttaaatctaatttttacatttcaaaaattatcttcagtagtaactaagtatattttctgtggattctgagaatgttatttttcagaatgtgagaatatatatgtacatttataatcttgtgactttaaagtctgttttcagatacagtatgtaaatacttgtaaaaaaatttgtataattttgtgataatgtagtttcccaaaaaaattatttagaaggcattatgttattagtaaatgagagcactgtatagaactgttcctattttctgcacttgccattccagctgcctccactgtccatacccacctcattcatcctgtcacagaaggcaggaaaactgggaactttaccaaagtagcactcagcctgagaggcctgtataatcatgcttttcaaactaaattcacttaaaaattaaaaagcagaattgaatattttaagcagcctcagtacctttggccaatgctgttttcatggtggattatgaacattatataatctttgggaaaagtgaaagtagtacaatttttagaataatgacaactgcctcactgcatctctccactcacacagcaaccgtgtagccccctaagctgcagtaccatgactaaccatgatgtcaatttcatatgctgatcctcacaacagcagtgcacaaacatgccccaaatattttaacagaatttagctcttccttaagctgtcttttcatagtaaaaacaaaacaaaaacacccaatgttaaaaccacataataaacttacaaacttgaaaaattagacacttcagatagataggcaataaaacttcatattatgaaagcaatatattccaagtttcaaagatttgacaagttctgtagagtatctttcatcagtacatgaaaacttccaaactgcatgatcttctgccaggcaggactgggtgctattcgctggtttgaggtcgaatccatttcaaggcatgtcgtggtgggacattaatggtgggatggtagaatgtgcagtccggtcttgtacattgagtgttaaacctacaatgttttggatgatagaagggacattccatcttcttacaagcagggaagtaacggcagagctgactactggaaggtggtgctggtggtgcaactgctggttttggagacagtactggaattcttctactcacatgagtgaagggacaatctggtttagtacactttgcatcatatttacaatttgggtgaacaaacaaacatttttcagcaaatttacaattggggaaggctttgcagggtgagatggggtgatggtaggcacactcatccccatttttacaagcaggccagtacttgcagcgctccaaaagtttttctggtttctgtgccacactcagttcactcatctcagcttgactcatctgcagagtttctgccattactgggtcgatttgcagtcgggataataattgcctctgttgagttccttgatttttttctacagaatctccttttgtttcctcttctttaatggggggacttattctgggggtcctactttgtccctggaccacttctgctagcaattcttcttgagaagttcgagttctgggagcaactggaagtgtctgtttctgtggaactgtagagtagttagttgtttttgttacggattcttgagcttcagatatagccttcaaaatcagattcttgttagcttgtttagaaggtggaagagaaggtctcctttcaggctttgcaggcacagacacactgctggagatgcttcctgttcgagacccgtaatcatcatcttcttcctcctcttctccatcatgattgaatttttttactttaacaactgaacttaccacaggcaactttctcttccgaaagttttcatcctccatactcattttctccgagttgtttctaaagaacggactatacgtttcttctaagctgttaagcacctctggttcacacaaacgtcctgtttcatatacccaactactctgcatatcaagctgcttggcagcatgaatactattctgctgctgttgaaattgcaacctgtttaaatgaacaccactatctgcatttctacttgcaggtggtcgataaatttcaatagaagggcgagaagaaccatatgtaagtgtcactgtaggttttttctgagataagggattctcctgcacaaagttgaggtcttcgtcaatgagatcatctggttctggcttaatatcaatcacatcttcagagggtgctggctccctcaaaggtttcactgttgacattagtcgggttgcagctccatcatcgtaagtctgtctgacatttgtggtttttgactcctgcgaacttgtagaaactctggaatctcttttttcaggtctcgcgctaggaatggcaagtggtggcactgcagcttcatgcctcctctcatctccccgactgaaattgctcttgtttgaaggcacgttactatcaaagatgttggtatcagaagacttcagactagagggttcagttgtaacagagcgaagtttatctaatacaccatgaagccaacataagctcctaattcttgtaatttccccttaatggcactccggatcttgcggctgatctcggtgccgatctccatggctctgcggcgtgcgggaactcagcactgcgcggcgcttggcttacccggaggctgccgcggactcctaccccgcagccgggacaccaccgcctcc

SEQ ID NO: 13616 - RNA, 16538 nt, Homo sapiens
  source 1..16538: mol_type = other RNA
gctgggattacaggcatgagccaccataataaggattctgatgaacatttgattccttggactactgttatactcaaaagccttccttaatcttctaattgtcaccctaaatatcctaaaatttctgtcttcctagtagttcttcatagtcctaaaaatttgtcagagagaaaggtaaatcaagaaacatgattttcaaatgatttaaggtggtactagggtttaggatttcctttgctttttatcatttaacacactgcttatcatacagctggaagtgctctgggccagtgtctctacttcgagggaagaaggaggtagtgagacagaaggaaatagcacaattcctggccctgacagaagggtgttcaggagacctgctctcctctcactttattccatctcatctggacctgtggcttccaatccacatctctttcctttaatatcctgcattggctaggctgtataaatcctttggtgcatcgaaaaactaagtgcattttttgtttttgtgattatgcaatacttataggaaaagttataattttagaatatttaagtacacttacatttttgagaaaaagactattgaaatgtttgtgccatgtcaaatttcagttgaacattttgggtattcttaatataagaccaggccaggcaccgtggctcaggccgggcacagtggctcacacctataatcccagcacttagggaggccaaggcgggaagatcacctgaagtcaggagttcaagaccagcctggctaacaaggtgaaactctgtctctactaaaaatacaaaaattagccgggcgtggtggctggcgcttgtaatcccagctacttgggaggctgagacaggagaatcacttgaacctgggaagcagaggttgtggtgagctgagatcgcaccattgcactccagcctgggcaacaaagagcgaaactccgtctcaaaaaaataaaaaataaaccctagaattatagtatgttagaattggaagggaagaattgtctaaggttattctagctaataagcaacagacttggaaaggaaaaggtcctgacaaagctaagcctcccgttcaggtttcctgactcgtgaattcagtgctgctgccactacacgatgcatgctctttgtatcaagggtgagacagcattacacatacatagaaaattatctatttaaactctatttgaacttttgatgagtttgtctccccctcccccactccttttcagaataacttgacgtttacaggtaccatcagtggtgatgtctgtgtgtggaaagatcacatattgtgtagaatcgtggcgagagctcacaacgggcctgtgtttgccatgtacaccaccctgcgagatggacttatcgtgactgggggaaaggaaaggccgtgagtcctctttcttttcacagaatatttatgcatttgtgacctacctgaggtttgcagttaattattctagttgtttctaggctacacagagtgtcctctccgaccttcctcctcatatgcttctcctttattaccttttatgtgccttctatttgattctcatttctggtcttaattcacttccaatttttttcatgttggggtgatactttttctgaggtgtggataggtagttgtcctacaagttgagttacttttcttaatgtctgtatgcctgtgtatgatttgctgagtaggaggcccatgggggaatctggagccagggttgtattttgactgcctgctctctttttgttcagaatggattctaaggagtagaatgcacattgttgctttagaaaaggatgagggaactagagagaactgccttgtttccttttgcttgaggcaaatttaaactgttttatacaagacctcaaaatttgagaagaggtctcttctgagtgattttcaaatctcccaacagtaaccagatacttatgatttgatttgtcaccaacatagtcatatgcatgttgaaacatgacatgtaggccaggcacagtggctcacacctgtaatcttatcactttgggaggctgaggcaggtggatcgcttgagcccaggagttcaagaccagcctgggcaacatggtgaaaccccatcgctataaaaaacaacaattagccgggtgtggtggcacatgcctgtagtccctgctactcaggaggctgaggtgggaggatcacttgagcctggggaggtcaaggctttagtgagctgtgatggtgccactgcactccagcctgggtgacagagtgagaccccatttaaaaaacaaaaacaaaaacaaaaaaaaatgtgacatatagttgactaagaagtacatttcaatacaggattgaaagaacccacatatgttaattaaacacaagcgcagaatttgtgccttttacataaaggaagaatgcacataggcatgctttcagacaagcaattcatctagcagaaaaggaaggaatacatttttcagcccttccaggaataaaatccataaatgggctctatttcgtcctccaacacttgtatttcccacgtcatttactcctgcacacccccactcactagaagcctgctaaactgttccagtgagatattttaacacctgatagggaataaatatgcttctgttttggccttcaaaaataagctctgggccagttgcagtggctcacgcctgtaatcccaacactttgggaggccgaggtgggcggatcacgaggtcaggagtttgggatcagcctggccaatatggtgaaactccatctctactaaaaatacaaaaattagccaggcatggtgcctgtaatcccagctacttgggaggctgaaggagaagaatcgcttgaacctgggaggcacaggttgcagtgagccgagatcacaccactgcactccaggccaggtgacagagcgacactctgtctcaaaaaaataaataaatcaactctgtagcatagcatttgtaattctattattttgccttacatttccattatccttttaataaaattgtttttttacatcttcctaatcaagaagtattatgaggccaggcacagtggctcatacctggaatcccagcactttgggaggccgaggcaggcagatcacctgaggtcaaggtatttgagaccagcctggccaacatggtgaaaccccatctctactaaaaatacagaaattagctgggtgtggtggtgcacacctgtaatgctagctactcgggaggctgaggtaggagaatcgcttgaacctgggaggcagaggttgcaataagcctagatcatgccactgcactcaagcctgggagacagagcgagactacatcttaaaaaaaaaaaaaaaagtattatgagagaggataatgtattgtaatgtattgtagaggctaaataaaattatgctcatgtcagaaaaaaagagtatttctcaaaataaaattcactgaaactggatgtttattttgactgagatatagtatatcctcaaattgccatagaaagtttacaagaatattagaggtaaattataaatatcagggcctttttaaaaaaaaaagattctgcttataacttggtatttgtttataataaaaattatagtagccaataatgaacacttactctggcttggttatttacttaggtcaaaagaaggaggagcggttaaactgtgggatcaggaactgaggcggtgccgtgccttcaggcttgagacaggacaagccacagattgtgttcgttctgtgtgcagaggcaaagtaagatgttccatgagctgatacagtgcagcagaaaacagaaagtggttattactgtgattccctcaccctttgcagcctaatgaacaatacttaataatgcataacgatggatttgcttgccaacattactctgtctttgctgctttctttgccaaagttagcaccagtgtggtgcataagctaggaagctattctgtctaaatactgtatgtaaacctccaatattttctagaatctgccaatttaacaactctagtagacataattgaaagcccttggcagttgactcatattaggacagctgtctccattttttaaaaaaacacacattccctagataaaacgtgcagtaaacaaacaatgaaatactactcagccataaaaaataatgaaattctgtcattcttggtggcaacatggatgagactggaggacatgatgtgaagtgaaataagccaggcacagaaagataaatacatgttctcactcctgtgcagaaactaaaaaagttgatcccacagaggtggagagtagaatagtggttactggaggcggacaagggggagggggagggggatagggaaggactggttaaaggatacaagtttacacagccagataggaatagtatgttttagtattctgtagtactgtaggatgactatagttaagaatcacgtatttatgtattttcaggtatttacaagagaggattttgaaagtttccatcacaaagaaatgataaatgtctgaggtgatggttatgcgtattaccctatgccctatagatatgtataattatgtgtcaatttcaaaataaaaattcaaaactacaactcctatgaaaatttttgagcgtgtttgtacttattaagtgtatttataaatcatacggatattatcttcagcctgcatattaaattgtagttaagcttttactttttaactaaaaaataaattctattattttttcctatatcccactgcactgaccccagtttggaaatcctaagattatcaaataaaaactttgattattgaagaatccaggtgtactgccacagaaaagttctattctgtagcatggactctaatatgtaatctagcccattgtgcttacagatagatgtgtgcctgtagtcatagaaaaatttgcatgagctaatgactgccttgctactagattagctcaaagcaaaaagttctctgaaagcaggtcaatagggtcatttttatattatgaagaagaaaagcagctgttgtattacattcactgtattggtcctgcttgtgtttcagggcaagatccttgttgggacaaggaatgctgaaataatcgaagttggagagaaaaatgcagcttgtaatattttagttaacggtcatgtggatgggccaatctggggactagcaacacatccttccagggattttttcctttctgctgcagaagatgggacagtgagactttgggatattgctgataaagtaagtacagataatttttttaaaagaggttacaacttctaaaaagaaaagttggaagttctaaattgctagtacttaaagaactgccagaattctgttgagcattttgaggggaaactggtataatttagaagtacttcacttaatgtttcctatgactctttttttttttttttttaaatgcagaagatgttaaacaaagtgaatttgggacatgctgctcgtactgtgtgttacagccctgaaggggacatggtggctattggaatgaaaaatggagaatttatcattttactagtgagttctctaaaaatatggggaaagaagagagacaggagatgtgcaatccatgatatcaggttagtgaacaaatggaatagagtttctagtatatacttgatttaacttccatttgtaaaattttccatagccttgccttcaaaaagaggtccccagggcctgtagcatttcccgtattataaattgtatgctaaaatatggctgtttgtatactacttaattcttcttgctaaattataaacccactgggcaccaactataatagcaagtactagtaggtaatgtttgatgaattcatgttaacacttagccatgtccattaagttcatcccaccaagaggtatctcccactgtaatacaagagagctatctgcccttcaaaagttgtcaccctggaaaactaaagttgtgatttcaaacatatcttctcttagtaacctcagtttgggaatatgtagttcattaatttaatcaatacctattgattaaatgttccagaatccaaattaatttaaatgtttcttaaacctttgtttttcagtgcttaagcatttttcaacagtggctaccatttacggagtacttccgtgtgatcagtagataagattattgaatctaggtctgtcaaaagcttgtacacttttcatcagtaaaatccttttacaaatgaaaccttcctcagaacttcaatatataaaatagtaacagtggcttcccttagcttttacatgtctctatcgtacctcagtaagactcatgggccatttcaagagactgaattgtcccatatgactccaaagattgctaggcaaatagcatttcactttgtcttttaaataagttcttcaggccgggcgcggtggctcatgcctgtaatcccagcactttgggaggccgaggcaggcagatcacctgaagtcaggagtactcgaccagcctggccaacatagtgaaaccccatctcaactaaaaatacaaaaatcagccgggcgtggtggcaggcgcctgtaatcccagctactcagggggctgaaacaggagaatcgcttgaacccgggaggcggaggttgcgccatcgcactccagcctgggagacaagagcgagacttcgtctcaaaaaaaaaaaattcttcttccaagattcaagttgtgtcatttcaccttaataactggaggttagttaagctgggctgtgttctttgcttaatattaagacaacgttttttccagatggaagaaaactatcttaatgaattgttagcttattaattatgtaatgctaatggcttttaaaagctgagatgttctgactgggtgttgtggctcacacctgtaatcccagtaccttgggaggccaagggggaaggattgcttgaggccaggagtttgggaccatagtgagaccccgcctctatttaaaaaattaaattttgttttgttttgttttgagttggagttttgctcttgttgcccatgctgaagtgcaatggtgcaatctcagctcaccacaacctgtgcctcctgggttcaagcgattctcctgcttcagcctcccgagtagatgggattacaggcgtgcaccaccatgcctggctaattttgtatttttagtagagacagggtttctctatgttggtcaggctggtctcaaactctcgacctcaggtgatctgcccgcctccgcttcccaaagttctgggattataggtgtgagccactgggcctggcctaagaaagtttttttaagccattagacgtttttaaaggaattgggagatgacaattggggaaatatttaaaatttaagtaaaatataaagcttccttatttcatgtaacccagacaatctcagtatacatgatcagttgtgtctgacaggtaaatctatttgaggccttatcacacgttacttttaagaactagaaaggaaaagtcactgatcttaagtatttataatacttcatgtggtctaatactttttacgttttgttttgattcagatttagtccggattcccggtatctggcagtaggttctagtgagaactcagtggatttttatgacctaacgctgggccccactcttaacagaatcagctactgcaaagacattccaagctttgtcattcaaatggacttctctgcagatagcagttatctccaggtacagtaccaatactgtatacccaggtggcaagttcttctgcttttacatttcgtgttagtgaatgcatttaaagttcctgagctccagagctccagcttctcaactcctccctttgtaccttctgacctacagctcccctttcctcccccacttatcagagcttttctcctattaagtttttgtagtgatcttttgcatacttaataatgttagacatgtaaatcaagtagcaatatgctagtattctgtaaaccccctgtggattttgtctctcacctaatggaattcttgtcccattttaatctgatgaaaaaggtctctagtggctgctataaacggcatgtctatgaagtgccttcaggaaaacatcttatggatcatgccgctattgacagaattacttgggctacatggactaggtaaatacttatatattcacaaggcaagaactgactttgaaggccagttagaaaatcctatttctgaactgttagagccattccaataaggaatagtaattgagtttcaagtttttgttaccatattttgaaatggtatgttcatgttgggacccctttttattgaatatatttccatgttttatcagtttccatgatttatcaagttttttttttaaggaaatcaaagttttaactttaaagataccctgatatttttcttaatgctaaatttaatgactggcaaaaaggtattgggtgctgttaagcaactgttattaattctctatctaaaggaatgctatcttgaatctattagaagtcaaagcttccaaatttgttcaaatttcctggctgtatgacaggtaaccatgactatccatttttttggccaatgaaaaatgccatcaaattcctgtatcagccaggcatatagtggctcatgcctgtaatctctgatgtagcaggccgaggtgggaggatcacttgagcctagaagttttgataccagcctgggcaacatagcaagaccccatctctgaaatttttttaattcctatgtcataagtcatttttatttttgtagagatagggatctcacaatattgcccaggctggtctcaaactcttggcctcaagcagtcctcctgcctcagcctcccaaaatgttgggattactggtatgtgctgctggacccagccaagtagcacttttaatttgaaaaatagttctatcagttttcagtcaggcgcggtggctcagcctgtaatcccagcactttgggaggccgagcgggggtgatcacctgaggtcgggagttcgagactagcctgaccaacatggagaaaccctgtctctactaaaaatacaaaataagccgggcatgttagcgcatgcctgtgatcccagctactcgggaggctgaggcaggagaattgcttgaacccaggaggcagaggttgcggtgagccgagatcatgccattgcactccagcctgggtaacaagagcgaaaactccgtctcaaaaaaaaaaaaagaaaaaatagttctatcagttttcataaagtactactttaatcttaaaaagattaatctagaaacccttcaaattataaaatgtcatttttaaaaggcaggagttgatatcctgatgaaattcaggtctccaaacaacttaccataatttacttcctgtattttaagtaacatgatagggtacttagagattaattgccaagaaactttttgaatatagtcaacctgcccgcacttgccatgatgagttttcttttgttccttccctctagtattctaggagatgaggttttgggaatctggtccagacatgctgagaaagctgatgtcaactgtgcctgtgtatctcattcaggaatcagtcttgttacaggagatgactttggcatggttaagttatttgacttcccatgtccagaaaaatttgtaagtttgtgttttgtttactattatcagtttactcctaattttgatgtcttatcatcagcacttttccccatatatttaaaatgttttgtcctaatttctaaatttttccccaaactttctaaatctatttactttgaaataaaagctattagaaacaaatcctctccctcgagtaataccatctttggaaccatcctacaaaagctgtaattagcttttcaccaaacctataatcagttatcaaatttcaaatgcttttccttagagaaaaatggtcagagtacctggagacatctgactgcccacacagcctggttttgcagatccactactcatgctgaaaagcattctaatcactggctgcggtgctaactccctactctctccacagctcttgtcatagagattatagttcctaataagagcctttgacttctgtgtgcaccaaatgccctgagcttgtctgtcattgttttttaggcaaaacacaaaaggttcttgggtcattcgccccatgtgacaaatattcgatttaccagtggtgatcgacatgttgttagtgctggaggtgatgactgcaggttagtaactttctcagcccatgaagagcagactatgttactagttaagagacttaatacaacaactcctacagctttggtttatgaaatcagctagtcaacattagtagaaggtagtataaccagatggctcttcagaatctcatatttatgcaaatacagaataaaaggagttaaagaggaaaaatattacacatgtaacctgaaagcacaactgaaaaatattaaactgttatgaaaatctaaaaacataattaactccctgcaattttcttctctgattgcagcttatttgtctggaaatgtgtacatacacctcactgagagatgctgagatgactacagaaattaactttgagaccagaattacagagaagaaaaaccaaaacccaaccctgcatggtcaagtggtgctaacccaagactgtaacagggagaaatgcccagaatcatcaaaatagtgaaagactgatctgttcaaaatatttgctatatgcactgggtataatccgtaatccatacactgccagataatgccatttcaaggaaggatcgaatacttgatggtaaaggccaagtccccctgtattgggaagtgtgtgatttcggcagacctgctgggaaaatttagggtagagcactctttacagaagaactcaaaaacccaatttggataattttcattatctttttagcaaaatggtttcttaatgtttatattttattttcaaggttcattgtttaatgaaatattttattcttgcatttccataaggaaagggaaagtcatgatcatcctaaaggatcacagtttttaaaaggcaaacattttccctaaggaaacagacacaagctttcctagagaatatgatgttttttaggcattaataaggtccttttttataaaggacacttttctcctagtagttttgaattcaggaacagatccaaagttagcagtatatggctgctacatttccattttcattttcgagccatcagtttatgttcagatgccatctctgtaatcgcacatttaaaacataactgtagcctcactaatggaaaagtagtatgatgaacaatcattcccaatggtgtacaatgtaagggttttagggagcaacagtatttaactggaagaaagaattgcatatttaatgtagtctaatatatacacatttgtttaacatgtaaacaaaagtgttaaattcacatatacaacattatacaatttaatcactcttggaataaaatttttatagccttttttctattgggaaaatttgtttagatgtgtgccactccataggtttatttccaaaatgaatgagcccaactccatttgtaaaaacttgtcagttagaattcctttttttagtggattagggctgaattcttagatccttatttcttttcactttaaatgctgccaaagatcactactcatcattcaggaattcgctgtctagcctatctgtagtttcctgaagattgaaaattatgtagactgctatttaaaaatatatttttctaagtgtgaggtttaagatgctgtattgaccctatgagtttttaatgtgttaattatctttatagcataatagatcgctttaggttcctggaatcccatttggtctgacaggatatatgaagattcttaatacctattttctgtgtctaatacttggttaatactaaaaatagaaatgactaaattacatcacagaaagcataaccagtgattgaacctggtagttttaaagctctaaatagctgtggctgaaggactgattatggggctaagaagcttgaaacgtaagttggtacttgttcatcagtggattctcctaaattaagccaaattttgaaatacatgactattaagtttctactcatgtatttacagtcagtcaataaattaaaggaggaaaaaaatccctgaacaacctgcccataaaaagaaaaatactctacatttgagcctgctgcagttttaaattttccctctgggtcaagtttgccagcttttggctacagagaaattatatttccattacagtgcaggtagaaactctgtaaccttaagcatgtaaactacatagaataaaactgtttccactgcatttctgtccttcaaagtggccaacctgattaagtcagccttaatcactgctgctgtcagtttcacgactaaaggtcatattgactaagtagtcatcagctgaccacctcgctgtatcagccagcaacgaggggaaggtgaagaaacatgataggccatatagaatctgccctatgtttacttttttaacccagataattatttttgtgtgcagtatctaagctcctgattgtgtaacctgggacttctggcaccttttgttccattcattttatgtataaaatgcatgccaaagcacactgtgccctctggtacccttgcttccaatcgccaaccatgctcatttccttcctttttttgtggtccctttttgtggtgatcattttaaaccacgtcatccaacaaatgttttatggtcaaccttagcttgttcataagccatagcaactgaaagattaaactcttaaatatgtgtctgggcagtggctattaaatagcaaaaaacaatcagattttagtattttattatttccttgtaaaatggctgaactaaattaaacccttgtttcccatttgttctataatttatagtgaaactgagaacaaaactatctttataaatgatagctaaaagtatttccagatatttaaacaatttaaaataaatttcttctgcagagatgcaaagcatctcaacactggaatgaacaaatgccttaaattcaatggagtaaacctttagaatgaagaggaactgtcatttcacccaagccgaagacaacagccttatgcacttgtgtgctctgtctttgctgcttctcgtgtttcaagcctttcctgtgggatcagcacagcaaagtgcaacttaccaaatggtttaatgactggttaattctttcttctcccaatggaaaagcaatggcaacacaacagtagactgctggcttgacaatcttaaacgtgagcctttgcacatgtaggtttatcatcatttgagtatacgactaagcaagtcaatgaactttttttttttttttagcagtttaatttggtcctgagaatgttgcagtctttattaccccttttgcattaatccacttttctaaccaccttttaagctttaatttttaacactatacaccaagtctttgaaatcagtgatctgttatttaactctaaagcatttgacacttcttgccttaacagttttaaaaaccacacacaaaaaaactctgtaagtaatacagtaggccaaaagtttcatcctatctatcttgcagtttacctatctgatctgatctctgtaattatagttctgtcatttaaaatatactatttaaatctaatttttacatttcaaaaattatcttcagtagtaactaagtatattttctgtggattctgagaatgttatttttcagaatgtgagaatatatatgtacatttataatcttgtgactttaaagtctgttttcagatacagtatgtaaatacttgtaaaaaaatttgtataattttgtgataatgtagtttcccaaaaaaattatttagaaggcattatgttattagtaaatgagagcactgtatagaactgttcctattttctgcacttgccattccagctgcctccactgtccatacccacctcattcatcctgtcacagaaggcaggaaaactgggaactttaccaaagtagcactcagcctgagaggcctgtataatcatgcttttcaaactaaattcacttaaaaattaaaaagcagaattgaatattttaagcagcctcagtacctttggccaatgctgttttcatggtggattatgaacattatataatctttgggaaaagtgaaagtagtacaatttttagaataatgacaactgcctcactgcatctctccactcacacagcaaccgtgtagccccctaagctgcagtaccatgactaaccatgatgtcaatttcatatgctgatcctcacaacagcagtgcacaaacatgccccaaatattttaacagaatttagctcttccttaagctgtcttttcatagtaaaaacaaaacaaaaacacccaatgttaaaaccacataataaacttacaaacttgaaaaattagacacttcagatagataggcaataaaacttcatattatgaaagcaatatattccaagtttcaaagatttgacaagttctgtagagtatctttcatcagtacatgaaaacttccaaactgcatgatcttctgccaggcaggactgggtgctattcgctggtttgaggtcgaatccatttcaaggcatgtcgtggtgggacattaatggtgggatggtagaatgtgcagtccggtcttgtacattgagtgttaaacctacaatgttttggatgatagaagggacattccatcttcttacaagcagggaagtaacggcagagctgactactggaaggtggtgctggtggtgcaactgctggttttggagacagtactggaattcttctactcacatgagtgaagggacaatctggtttagtacactttgcatcatatttacaatttgggtgaacaaacaaacatttttcagcaaatttacaattggggaaggctttgcagggtgagatggggtgatggtaggcacactcatccccatttttacaagcaggccagtacttgcagcgctccaaaagtttttctggtttctgtgccacactcagttcactcatctcagcttgactcatctgcagagtttctgccattactgggtcgatttgcagtcgggataataattgcctctgttgagttccttgatttttttctacagaatctccttttgtttcctcttctttaatggggggacttattctgggggtcctactttgtccctggaccacttctgctagcaattcttcttgagaagttcgagttctgggagcaactggaagtgtctgtttctgtggaactgtagagtagttagttgtttttgttacggattcttgagcttcagatatagccttcaaaatcagattcttgttagcttgtttagaaggtggaagagaaggtctcctttcaggctttgcaggcacagacacactgctggagatgcttcctgttcgagacccgtaatcatcatcttcttcctcctcttctccatcatgattgaatttttttactttaacaactgaacttaccacaggcaactttctcttccgaaagttttcatcctccatactcattttctccgagttgtttctaaagaacggactatacgtttcttctaagctgttaagcacctctggttcacacaaacgtcctgtttcatatacccaactactctgcatatcaagctgcttggcagcatgaatactattctgctgctgttgaaattgcaacctgtttaaatgaacaccactatctgcatttctacttgcaggtggtcgataaatttcaatagaagggcgagaagaaccatatgtaagtgtcactgtaggttttttctgagataagggattctcctgcacaaagttgaggtcttcgtcaatgagatcatctggttctggcttaatatcaatcacatcttcagagggtgctggctccctcaaaggtttcactgttgacattagtcgggttgcagctccatcatcgtaagtctgtctgacatttgtggtttttgactcctgcgaacttgtagaaactctggaatctcttttttcaggtctcgcgctaggaatggcaagtggtggcactgcagcttcatgcctcctctcatctccccgactgaaattgctcttgtttgaaggcacgttactatcaaagatgttggtatcagaagacttcagactagagggttcagttgtaacagagcgaagtttatctaatacaccatgaagccatacggtgaatcgaattgtgttgttccctagaaacagggacagatcctctgtcatttggtcctgacttttcttgttggccaccatcaccataatgtaatcaggaagttcttcatcaacataagctcctaattcttgtaatttccccttaatggcactccggatcttgcggctgatctcggtgccgatctccatggctctgcggcgtgcgggaactcagcactgcgcggcgcttggcttacccggaggctgccgcggactcctaccccgcagccgggacaccaccgcctcc

SEQ ID NO: 13617 - RNA, 16514 nt, Homo sapiens
  source 1..16514: mol_type = other RNA
gctgggattacaggcatgagccaccataataaggattctgatgaacatttgattccttggactactgttatactcaaaagccttccttaatcttctaattgtcaccctaaatatcctaaaatttctgtcttcctagtagttcttcatagtcctaaaaatttgtcagagagaaaggtaaatcaagaaacatgattttcaaatgatttaaggtggtactagggtttaggatttcctttgctttttatcatttaacacactgcttatcatacagctggaagtgctctgggccagtgtctctacttcgagggaagaaggaggtagtgagacagaaggaaatagcacaattcctggccctgacagaagggtgttcaggagacctgctctcctctcactttattccatctcatctggacctgtggcttccaatccacatctctttcctttaatatcctgcattggctaggctgtataaatcctttggtgcatcgaaaaactaagtgcattttttgtttttgtgattatgcaatacttataggaaaagttataattttagaatatttaagtacacttacatttttgagaaaaagactattgaaatgtttgtgccatgtcaaatttcagttgaacattttgggtattcttaatataagaccaggccaggcaccgtggctcaggccgggcacagtggctcacacctataatcccagcacttagggaggccaaggcgggaagatcacctgaagtcaggagttcaagaccagcctggctaacaaggtgaaactctgtctctactaaaaatacaaaaattagccgggcgtggtggctggcgcttgtaatcccagctacttgggaggctgagacaggagaatcacttgaacctgggaagcagaggttgtggtgagctgagatcgcaccattgcactccagcctgggcaacaaagagcgaaactccgtctcaaaaaaataaaaaataaaccctagaattatagtatgttagaattggaagggaagaattgtctaaggttattctagctaataagcaacagacttggaaaggaaaaggtcctgacaaagctaagcctcccgttcaggtttcctgactcgtgaattcagtgctgctgccactacacgatgcatgctctttgtatcaagggtgagacagcattacacatacatagaaaattatctatttaaactctatttgaacttttgatgagtttgtctccccctcccccactccttttcagaataacttgacgtttacaggtaccatcagtggtgatgtctgtgtgtggaaagatcacatattgtgtagaatcgtggcgagagctcacaacgggcctgtgtttgccatgtacaccaccctgcgagatggacttatcgtgactgggggaaaggaaaggccgtgagtcctctttcttttcacagaatatttatgcatttgtgacctacctgaggtttgcagttaattattctagttgtttctaggctacacagagtgtcctctccgaccttcctcctcatatgcttctcctttattaccttttatgtgccttctatttgattctcatttctggtcttaattcacttccaatttttttcatgttggggtgatactttttctgaggtgtggataggtagttgtcctacaagttgagttacttttcttaatgtctgtatgcctgtgtatgatttgctgagtaggaggcccatgggggaatctggagccagggttgtattttgactgcctgctctctttttgttcagaatggattctaaggagtagaatgcacattgttgctttagaaaaggatgagggaactagagagaactgccttgtttccttttgcttgaggcaaatttaaactgttttatacaagacctcaaaatttgagaagaggtctcttctgagtgattttcaaatctcccaacagtaaccagatacttatgatttgatttgtcaccaacatagtcatatgcatgttgaaacatgacatgtaggccaggcacagtggctcacacctgtaatcttatcactttgggaggctgaggcaggtggatcgcttgagcccaggagttcaagaccagcctgggcaacatggtgaaaccccatcgctataaaaaacaacaattagccgggtgtggtggcacatgcctgtagtccctgctactcaggaggctgaggtgggaggatcacttgagcctggggaggtcaaggctttagtgagctgtgatggtgccactgcactccagcctgggtgacagagtgagaccccatttaaaaaacaaaaacaaaaacaaaaaaaaatgtgacatatagttgactaagaagtacatttcaatacaggattgaaagaacccacatatgttaattaaacacaagcgcagaatttgtgccttttacataaaggaagaatgcacataggcatgctttcagacaagcaattcatctagcagaaaaggaaggaatacatttttcagcccttccaggaataaaatccataaatgggctctatttcgtcctccaacacttgtatttcccacgtcatttactcctgcacacccccactcactagaagcctgctaaactgttccagtgagatattttaacacctgatagggaataaatatgcttctgttttggccttcaaaaataagctctgggccagttgcagtggctcacgcctgtaatcccaacactttgggaggccgaggtgggcggatcacgaggtcaggagtttgggatcagcctggccaatatggtgaaactccatctctactaaaaatacaaaaattagccaggcatggtgcctgtaatcccagctacttgggaggctgaaggagaagaatcgcttgaacctgggaggcacaggttgcagtgagccgagatcacaccactgcactccaggccaggtgacagagcgacactctgtctcaaaaaaataaataaatcaactctgtagcatagcatttgtaattctattattttgccttacatttccattatccttttaataaaattgtttttttacatcttcctaatcaagaagtattatgaggccaggcacagtggctcatacctggaatcccagcactttgggaggccgaggcaggcagatcacctgaggtcaaggtatttgagaccagcctggccaacatggtgaaaccccatctctactaaaaatacagaaattagctgggtgtggtggtgcacacctgtaatgctagctactcgggaggctgaggtaggagaatcgcttgaacctgggaggcagaggttgcaataagcctagatcatgccactgcactcaagcctgggagacagagcgagactacatcttaaaaaaaaaaaaaaaagtattatgagagaggataatgtattgtaatgtattgtagaggctaaataaaattatgctcatgtcagaaaaaaagagtatttctcaaaataaaattcactgaaactggatgtttattttgactgagatatagtatatcctcaaattgccatagaaagtttacaagaatattagaggtaaattataaatatcagggcctttttaaaaaaaaaagattctgcttataacttggtatttgtttataataaaaattatagtagccaataatgaacacttactctggcttggttatttacttaggtcaaaagaaggaggagcggttaaactgtgggatcaggaactgaggcggtgccgtgccttcaggcttgagacaggacaagccacagattgtgttcgttctgtgtgcagaggcaaagtaagatgttccatgagctgatacagtgcagcagaaaacagaaagtggttattactgtgattccctcaccctttgcagcctaatgaacaatacttaataatgcataacgatggatttgcttgccaacattactctgtctttgctgctttctttgccaaagttagcaccagtgtggtgcataagctaggaagctattctgtctaaatactgtatgtaaacctccaatattttctagaatctgccaatttaacaactctagtagacataattgaaagcccttggcagttgactcatattaggacagctgtctccattttttaaaaaaacacacattccctagataaaacgtgcagtaaacaaacaatgaaatactactcagccataaaaaataatgaaattctgtcattcttggtggcaacatggatgagactggaggacatgatgtgaagtgaaataagccaggcacagaaagataaatacatgttctcactcctgtgcagaaactaaaaaagttgatcccacagaggtggagagtagaatagtggttactggaggcggacaagggggagggggagggggatagggaaggactggttaaaggatacaagtttacacagccagataggaatagtatgttttagtattctgtagtactgtaggatgactatagttaagaatcacgtatttatgtattttcaggtatttacaagagaggattttgaaagtttccatcacaaagaaatgataaatgtctgaggtgatggttatgcgtattaccctatgccctatagatatgtataattatgtgtcaatttcaaaataaaaattcaaaactacaactcctatgaaaatttttgagcgtgtttgtacttattaagtgtatttataaatcatacggatattatcttcagcctgcatattaaattgtagttaagcttttactttttaactaaaaaataaattctattattttttcctatatcccactgcactgaccccagtttggaaatcctaagattatcaaataaaaactttgattattgaagaatccaggtgtactgccacagaaaagttctattctgtagcatggactctaatatgtaatctagcccattgtgcttacagatagatgtgtgcctgtagtcatagaaaaatttgcatgagctaatgactgccttgctactagattagctcaaagcaaaaagttctctgaaagcaggtcaatagggtcatttttatattatgaagaagaaaagcagctgttgtattacattcactgtattggtcctgcttgtgtttcagggcaagatccttgttgggacaaggaatgctgaaataatcgaagttggagagaaaaatgcagcttgtaatattttagttaacggtcatgtggatgggccaatctggggactagcaacacatccttccagggattttttcctttctgctgcagaagatgggacagtgagactttgggatattgctgataaagtaagtacagataatttttttaaaagaggttacaacttctaaaaagaaaagttggaagttctaaattgctagtacttaaagaactgccagaattctgttgagcattttgaggggaaactggtataatttagaagtacttcacttaatgtttcctatgactctttttttttttttttttaaatgcagaagatgttaaacaaagtgaatttgggacatgctgctcgtactgtgtgttacagccctgaaggggacatggtggctattggaatgaaaaatggagaatttatcattttactagtgagttctctaaaaatatggggaaagaagagagacaggagatgtgcaatccatgatatcaggttagtgaacaaatggaatagagtttctagtatatacttgatttaacttccatttgtaaaattttccatagccttgccttcaaaaagaggtccccagggcctgtagcatttcccgtattataaattgtatgctaaaatatggctgtttgtatactacttaattcttcttgctaaattataaacccactgggcaccaactataatagcaagtactagtaggtaatgtttgatgaattcatgttaacacttagccatgtccattaagttcatcccaccaagaggtatctcccactgtaatacaagagagctatctgcccttcaaaagttgtcaccctggaaaactaaagttgtgatttcaaacatatcttctcttagtaacctcagtttgggaatatgtagttcattaatttaatcaatacctattgattaaatgttccagaatccaaattaatttaaatgtttcttaaacctttgtttttcagtgcttaagcatttttcaacagtggctaccatttacggagtacttccgtgtgatcagtagataagattattgaatctaggtctgtcaaaagcttgtacacttttcatcagtaaaatccttttacaaatgaaaccttcctcagaacttcaatatataaaatagtaacagtggcttcccttagcttttacatgtctctatcgtacctcagtaagactcatgggccatttcaagagactgaattgtcccatatgactccaaagattgctaggcaaatagcatttcactttgtcttttaaataagttcttcaggccgggcgcggtggctcatgcctgtaatcccagcactttgggaggccgaggcaggcagatcacctgaagtcaggagtactcgaccagcctggccaacatagtgaaaccccatctcaactaaaaatacaaaaatcagccgggcgtggtggcaggcgcctgtaatcccagctactcagggggctgaaacaggagaatcgcttgaacccgggaggcggaggttgcgccatcgcactccagcctgggagacaagagcgagacttcgtctcaaaaaaaaaaaattcttcttccaagattcaagttgtgtcatttcaccttaataactggaggttagttaagctgggctgtgttctttgcttaatattaagacaacgttttttccagatggaagaaaactatcttaatgaattgttagcttattaattatgtaatgctaatggcttttaaaagctgagatgttctgactgggtgttgtggctcacacctgtaatcccagtaccttgggaggccaagggggaaggattgcttgaggccaggagtttgggaccatagtgagaccccgcctctatttaaaaaattaaattttgttttgttttgttttgagttggagttttgctcttgttgcccatgctgaagtgcaatggtgcaatctcagctcaccacaacctgtgcctcctgggttcaagcgattctcctgcttcagcctcccgagtagatgggattacaggcgtgcaccaccatgcctggctaattttgtatttttagtagagacagggtttctctatgttggtcaggctggtctcaaactctcgacctcaggtgatctgcccgcctccgcttcccaaagttctgggattataggtgtgagccactgggcctggcctaagaaagtttttttaagccattagacgtttttaaaggaattgggagatgacaattggggaaatatttaaaatttaagtaaaatataaagcttccttatttcatgtaacccagacaatctcagtatacatgatcagttgtgtctgacaggtaaatctatttgaggccttatcacacgttacttttaagaactagaaaggaaaagtcactgatcttaagtatttataatacttcatgtggtctaatactttttacgttttgttttgattcagatttagtccggattcccggtatctggcagtaggttctagtgagaactcagtggatttttatgacctaacgctgggccccactcttaacagaatcagctactgcaaagacattccaagctttgtcattcaaatggacttctctgcagatagcagttatctccaggtacagtaccaatactgtatacccaggtggcaagttcttctgcttttacatttcgtgttagtgaatgcatttaaagttcctgagctccagagctccagcttctcaactcctccctttgtaccttctgacctacagctcccctttcctcccccacttatcagagcttttctcctattaagtttttgtagtgatcttttgcatacttaataatgttagacatgtaaatcaagtagcaatatgctagtattctgtaaaccccctgtggattttgtctctcacctaatggaattcttgtcccattttaatctgatgaaaaaggtctctagtggctgctataaacggcatgtctatgaagtgccttcaggaaaacatcttatggatcatgccgctattgacagaattacttgggctacatggactaggtaaatacttatatattcacaaggcaagaactgactttgaaggccagttagaaaatcctatttctgaactgttagagccattccaataaggaatagtaattgagtttcaagtttttgttaccatattttgaaatggtatgttcatgttgggacccctttttattgaatatatttccatgttttatcagtttccatgatttatcaagttttttttttaaggaaatcaaagttttaactttaaagataccctgatatttttcttaatgctaaatttaatgactggcaaaaaggtattgggtgctgttaagcaactgttattaattctctatctaaaggaatgctatcttgaatctattagaagtcaaagcttccaaatttgttcaaatttcctggctgtatgacaggtaaccatgactatccatttttttggccaatgaaaaatgccatcaaattcctgtatcagccaggcatatagtggctcatgcctgtaatctctgatgtagcaggccgaggtgggaggatcacttgagcctagaagttttgataccagcctgggcaacatagcaagaccccatctctgaaatttttttaattcctatgtcataagtcatttttatttttgtagagatagggatctcacaatattgcccaggctggtctcaaactcttggcctcaagcagtcctcctgcctcagcctcccaaaatgttgggattactggtatgtgctgctggacccagccaagtagcacttttaatttgaaaaatagttctatcagttttcagtcaggcgcggtggctcagcctgtaatcccagcactttgggaggccgagcgggggtgatcacctgaggtcgggagttcgagactagcctgaccaacatggagaaaccctgtctctactaaaaatacaaaataagccgggcatgttagcgcatgcctgtgatcccagctactcgggaggctgaggcaggagaattgcttgaacccaggaggcagaggttgcggtgagccgagatcatgccattgcactccagcctgggtaacaagagcgaaaactccgtctcaaaaaaaaaaaaagaaaaaatagttctatcagttttcataaagtactactttaatcttaaaaagattaatctagaaacccttcaaattataaaatgtcatttttaaaaggcaggagttgatatcctgatgaaattcaggtctccaaacaacttaccataatttacttcctgtattttaagtaacatgatagggtacttagagattaattgccaagaaactttttgaatatagtcaacctgcccgcacttgccatgatgagttttcttttgttccttccctctagtattctaggagatgaggttttgggaatctggtccagacatgctgagaaagctgatgtcaactgtgcctgtgtatctcattcaggaatcagtcttgttacaggagatgactttggcatggttaagttatttgacttcccatgtccagaaaaatttgtaagtttgtgttttgtttactattatcagtttactcctaattttgatgtcttatcatcagcacttttccccatatatttaaaatgttttgtcctaatttctaaatttttccccaaactttctaaatctatttactttgaaataaaagctattagaaacaaatcctctccctcgagtaataccatctttggaaccatcctacaaaagctgtaattagcttttcaccaaacctataatcagttatcaaatttcaaatgcttttccttagagaaaaatggtcagagtacctggagacatctgactgcccacacagcctggttttgcagatccactactcatgctgaaaagcattctaatcactggctgcggtgctaactccctactctctccacagctcttgtcatagagattatagttcctaataagagcctttgacttctgtgtgcaccaaatgccctgagcttgtctgtcattgttttttaggcaaaacacaaaaggttcttgggtcattcgccccatgtgacaaatattcgatttaccagtggtgatcgacatgttgttagtgctggaggtgatgactgcaggttagtaactttctcagcccatgaagagcagactatgttactagttaagagacttaatacaacaactcctacagctttggtttatgaaatcagctagtcaacattagtagaaggtagtataaccagatggctcttcagaatctcatatttatgcaaatacagaataaaaggagttaaagaggaaaaatattacacatgtaacctgaaagcacaactgaaaaatattaaactgttatgaaaatctaaaaacataattaactccctgcaattttcttctctgattgcagcttatttgtctggaaatgtgtacatacacctcactgagagatgctgagatgactacagaaattaactttgagaccagaattacagagaagaaaaaccaaaacccaaccctgcatggtcaagtggtgctaacccaagactgtaacagggagaaatgcccagaatcatcaaaatagtgaaagactgatctgttcaaaatatttgctatatgcactgggtataatccgtaatccatacactgccagataatgccatttcaaggaaggatcgaatacttgatggtaaaggccaagtccccctgtattgggaagtgtgtgatttcggcagacctgctgggaaaatttagggtagagcactctttacagaagaactcaaaaacccaatttggataattttcattatctttttagcaaaatggtttcttaatgtttatattttattttcaaggttcattgtttaatgaaatattttattcttgcatttccataaggaaagggaaagtcatgatcatcctaaaggatcacagtttttaaaaggcaaacattttccctaaggaaacagacacaagctttcctagagaatatgatgttttttaggcattaataaggtccttttttataaaggacacttttctcctagtagttttgaattcaggaacagatccaaagttagcagtatatggctgctacatttccattttcattttcgagccatcagtttatgttcagatgccatctctgtaatcgcacatttaaaacataactgtagcctcactaatggaaaagtagtatgatgaacaatcattcccaatggtgtacaatgtaagggttttagggagcaacagtatttaactggaagaaagaattgcatatttaatgtagtctaatatatacacatttgtttaacatgtaaacaaaagtgttaaattcacatatacaacattatacaatttaatcactcttggaataaaatttttatagccttttttctattgggaaaatttgtttagatgtgtgccactccataggtttatttccaaaatgaatgagcccaactccatttgtaaaaacttgtcagttagaattcctttttttagtggattagggctgaattcttagatccttatttcttttcactttaaatgctgccaaagatcactactcatcattcaggaattcgctgtctagcctatctgtagtttcctgaagattgaaaattatgtagactgctatttaaaaatatatttttctaagtgtgaggtttaagatgctgtattgaccctatgagtttttaatgtgttaattatctttatagcataatagatcgctttaggttcctggaatcccatttggtctgacaggatatatgaagattcttaatacctattttctgtgtctaatacttggttaatactaaaaatagaaatgactaaattacatcacagaaagcataaccagtgattgaacctggtagttttaaagctctaaatagctgtggctgaaggactgattatggggctaagaagcttgaaacgtaagttggtacttgttcatcagtggattctcctaaattaagccaaattttgaaatacatgactattaagtttctactcatgtatttacagtcagtcaataaattaaaggaggaaaaaaatccctgaacaacctgcccataaaaagaaaaatactctacatttgagcctgctgcagttttaaattttccctctgggtcaagtttgccagcttttggctacagagaaattatatttccattacagtgcaggtagaaactctgtaaccttaagcatgtaaactacatagaataaaactgtttccactgcatttctgtccttcaaagtggccaacctgattaagtcagccttaatcactgctgctgtcagtttcacgactaaaggtcatattgactaagtagtcatcagctgaccacctcgctgtatcagccagcaacgaggggaaggtgaagaaacatgataggccatatagaatctgccctatgtttacttttttaacccagataattatttttgtgtgcagtatctaagctcctgattgtgtaacctgggacttctggcaccttttgttccattcattttatgtataaaatgcatgccaaagcacactgtgccctctggtacccttgcttccaatcgccaaccatgctcatttccttcctttttttgtggtccctttttgtggtgatcattttaaaccacgtcatccaacaaatgttttatggtcaaccttagcttgttcataagccatagcaactgaaagattaaactcttaaatatgtgtctgggcagtggctattaaatagcaaaaaacaatcagattttagtattttattatttccttgtaaaatggctgaactaaattaaacccttgtttcccatttgttctataatttatagtgaaactgagaacaaaactatctttataaatgatagctaaaagtatttccagatatttaaacaatttaaaataaatttcttctgcagagatgcaaagcatctcaacactggaatgaacaaatgccttaaattcaatggagtaaacctttagaatgaagaggaactgtcatttcacccaagccgaagacaacagccttatgcacttgtgtgctctgtctttgctgcttctcgtgtttcaagcctttcctgtgggatcagcacagcaaagtgcaacttaccaaatggtttaatgactggttaattctttcttctcccaatggaaaagcaatggcaacacaacagtagactgctggcttgacaatcttaaacgtgagcctttgcacatgtaggtttatcatcatttgagtatacgactaagcaagtcaatgaactttttttttttttttagcagtttaatttggtcctgagaatgttgcagtctttattaccccttttgcattaatccacttttctaaccaccttttaagctttaatttttaacactatacaccaagtctttgaaatcagtgatctgttatttaactctaaagcatttgacacttcttgccttaacagttttaaaaaccacacacaaaaaaactctgtaagtaatacagtaggccaaaagtttcatcctatctatcttgcagtttacctatctgatctgatctctgtaattatagttctgtcatttaaaatatactatttaaatctaatttttacatttcaaaaattatcttcagtagtaactaagtatattttctgtggattctgagaatgttatttttcagaatgtgagaatatatatgtacatttataatcttgtgactttaaagtctgttttcagatacagtatgtaaatacttgtaaaaaaatttgtataattttgtgataatgtagtttcccaaaaaaattatttagaaggcattatgttattagtaaatgagagcactgtatagaactgttcctattttctgcacttgccattccagctgcctccactgtccatacccacctcattcatcctgtcacagaaggcaggaaaactgggaactttaccaaagtagcactcagcctgagaggcctgtataatcatgcttttcaaactaaattcacttaaaaattaaaaagcagaattgaatattttaagcagcctcagtacctttggccaatgctgttttcatggtggattatgaacattatataatctttgggaaaagtgaaagtagtacaatttttagaataatgacaactgcctcactgcatctctccactcacacagcaaccgtgtagccccctaagctgcagtaccatgactaaccatgatgtcaatttcatatgctgatcctcacaacagcagtgcacaaacatgccccaaatattttaacagaatttagctcttccttaagctgtcttttcatagtaaaaacaaaacaaaaacacccaatgttaaaaccacataataaacttacaaacttgaaaaattagacacttcagatagataggcaataaaacttcatattatgaaagcaatatattccaagtttcaaagatttgacaagttctgtagagtatctttcatcagtacatgaaaacttccaaactgcatgatcttctgccaggcaggactgggtgctattcgctggtttgaggtcgaatccatttcaaggcatgtcgtggtgggacattaatggtgggatggtagaatgtgcagtccggtcttgtacattgagtgttaaacctacaatgttttggatgatagaagggacattccatcttcttacaagcagggaagtaacggcagagctgactactggaaggtggtgctggtggtgcaactgctggttttggagacagtactggaattcttctactcacatgagtgaagggacaatctggtttagtacactttgcatcatatttacaatttgggtgaacaaacaaacatttttcagcaaatttacaattggggaaggctttgcagggtgagatggggtgatggtaggcacactcatccccatttttacaagcaggccagtacttgcagcgctccaaaagtttttctggtttctgtgccacactcagttcactcatctcagcttgactcatctgcagagtttctgccattactgggtcgatttgcagtcgggataataattgcctctgttgagttccttgatttttttctacagaatctccttttgtttcctcttctttaatggggggacttattctgggggtcctactttgtccctggaccacttctgctagcaattcttcttgagaagttcgagttctgggagcaactggaagtgtctgtttctgtggaactgtagagtagttagttgtttttgttacggattcttgagcttcagatatagccttcaaaatcagattcttgttagcttgtttagaaggtggaagagaaggtctcctttcaggctttgcaggcacagacacactgctggagatgcttcctgttcgagacccgtaatcatcatcttcttcctcctcttctccatcatgattgaatttttttactttaacaactgaacttaccacaggcaactttctcttccgaaagttttcatcctccatactcattttctccgagttgtttctaaagaacggactatacgtttcttctaagctgttaagcacctctggttcacacaaacgtcctgtttcatatacccaactactctgcatatcaagctgcttggcagcatgaatactattctgctgctgttgaaattgcaacctgtttaaatgaacaccactatctgcatttctacttgcaggtggtcgataaatttcaatagaagggcgagaagaaccatatgtaagtgtcactgtaggttttttctgagataagggattctcctgcacaaagttgaggtcttcgtcaatgagatcatctggttctggcttaatatcaatcacatcttcagagggtgctggctccctcaaaggtttcactgttgacattagtcgggttgcagctccatcatcgtaagtctgtctgacatttgtggtttttgactcctgcgaacttgtagaaactctggaatctcttttttcaggtctcgcgctaggaatggcaagtggtggcactgcagcttcatgcctcctctcatctccccgactgaaattgctcttgtttgaaggcacgttactatcaaagatgttggtatcagaagacttcagactagagggttcagttgtaacagagcgaagtttatctaatacaccatgaagccatacggtgaatcgaattgtgttgttccctagaaacagggacagatcctctgtcatttggtcctgacttttcttgttggccaccatcaccataatgtaatcaggaagttcttcatcaacataagctcctaattcttgtaatttccccttaatggcactctcccgcagcggatccaaagcggcgccgtgcgccgcggtggtggctccagccgggcctgcgcctgtccttccatttcccggcggctacttcagccgcagccacgctccg

SEQ ID NO: 13618 - RNA, 16348 nt, Homo sapiens
  source 1..16348: mol_type = other RNA
gctgggattacaggcatgagccaccataataaggattctgatgaacatttgattccttggactactgttatactcaaaagccttccttaatcttctaattgtcaccctaaatatcctaaaatttctgtcttcctagtagttcttcatagtcctaaaaatttgtcagagagaaaggtaaatcaagaaacatgattttcaaatgatttaaggtggtactagggtttaggatttcctttgctttttatcatttaacacactgcttatcatacagctggaagtgctctgggccagtgtctctacttcgagggaagaaggaggtagtgagacagaaggaaatagcacaattcctggccctgacagaagggtgttcaggagacctgctctcctctcactttattccatctcatctggacctgtggcttccaatccacatctctttcctttaatatcctgcattggctaggctgtataaatcctttggtgcatcgaaaaactaagtgcattttttgtttttgtgattatgcaatacttataggaaaagttataattttagaatatttaagtacacttacatttttgagaaaaagactattgaaatgtttgtgccatgtcaaatttcagttgaacattttgggtattcttaatataagaccaggccaggcaccgtggctcaggccgggcacagtggctcacacctataatcccagcacttagggaggccaaggcgggaagatcacctgaagtcaggagttcaagaccagcctggctaacaaggtgaaactctgtctctactaaaaatacaaaaattagccgggcgtggtggctggcgcttgtaatcccagctacttgggaggctgagacaggagaatcacttgaacctgggaagcagaggttgtggtgagctgagatcgcaccattgcactccagcctgggcaacaaagagcgaaactccgtctcaaaaaaataaaaaataaaccctagaattatagtatgttagaattggaagggaagaattgtctaaggttattctagctaataagcaacagacttggaaaggaaaaggtcctgacaaagctaagcctcccgttcaggtttcctgactcgtgaattcagtgctgctgccactacacgatgcatgctctttgtatcaagggtgagacagcattacacatacatagaaaattatctatttaaactctatttgaacttttgatgagtttgtctccccctcccccactccttttcagaataacttgacgtttacaggtaccatcagtggtgatgtctgtgtgtggaaagatcacatattgtgtagaatcgtggcgagagctcacaacgggcctgtgtttgccatgtacaccaccctgcgagatggacttatcgtgactgggggaaaggaaaggccgtgagtcctctttcttttcacagaatatttatgcatttgtgacctacctgaggtttgcagttaattattctagttgtttctaggctacacagagtgtcctctccgaccttcctcctcatatgcttctcctttattaccttttatgtgccttctatttgattctcatttctggtcttaattcacttccaatttttttcatgttggggtgatactttttctgaggtgtggataggtagttgtcctacaagttgagttacttttcttaatgtctgtatgcctgtgtatgatttgctgagtaggaggcccatgggggaatctggagccagggttgtattttgactgcctgctctctttttgttcagaatggattctaaggagtagaatgcacattgttgctttagaaaaggatgagggaactagagagaactgccttgtttccttttgcttgaggcaaatttaaactgttttatacaagacctcaaaatttgagaagaggtctcttctgagtgattttcaaatctcccaacagtaaccagatacttatgatttgatttgtcaccaacatagtcatatgcatgttgaaacatgacatgtaggccaggcacagtggctcacacctgtaatcttatcactttgggaggctgaggcaggtggatcgcttgagcccaggagttcaagaccagcctgggcaacatggtgaaaccccatcgctataaaaaacaacaattagccgggtgtggtggcacatgcctgtagtccctgctactcaggaggctgaggtgggaggatcacttgagcctggggaggtcaaggctttagtgagctgtgatggtgccactgcactccagcctgggtgacagagtgagaccccatttaaaaaacaaaaacaaaaacaaaaaaaaatgtgacatatagttgactaagaagtacatttcaatacaggattgaaagaacccacatatgttaattaaacacaagcgcagaatttgtgccttttacataaaggaagaatgcacataggcatgctttcagacaagcaattcatctagcagaaaaggaaggaatacatttttcagcccttccaggaataaaatccataaatgggctctatttcgtcctccaacacttgtatttcccacgtcatttactcctgcacacccccactcactagaagcctgctaaactgttccagtgagatattttaacacctgatagggaataaatatgcttctgttttggccttcaaaaataagctctgggccagttgcagtggctcacgcctgtaatcccaacactttgggaggccgaggtgggcggatcacgaggtcaggagtttgggatcagcctggccaatatggtgaaactccatctctactaaaaatacaaaaattagccaggcatggtgcctgtaatcccagctacttgggaggctgaaggagaagaatcgcttgaacctgggaggcacaggttgcagtgagccgagatcacaccactgcactccaggccaggtgacagagcgacactctgtctcaaaaaaataaataaatcaactctgtagcatagcatttgtaattctattattttgccttacatttccattatccttttaataaaattgtttttttacatcttcctaatcaagaagtattatgaggccaggcacagtggctcatacctggaatcccagcactttgggaggccgaggcaggcagatcacctgaggtcaaggtatttgagaccagcctggccaacatggtgaaaccccatctctactaaaaatacagaaattagctgggtgtggtggtgcacacctgtaatgctagctactcgggaggctgaggtaggagaatcgcttgaacctgggaggcagaggttgcaataagcctagatcatgccactgcactcaagcctgggagacagagcgagactacatcttaaaaaaaaaaaaaaaagtattatgagagaggataatgtattgtaatgtattgtagaggctaaataaaattatgctcatgtcagaaaaaaagagtatttctcaaaataaaattcactgaaactggatgtttattttgactgagatatagtatatcctcaaattgccatagaaagtttacaagaatattagaggtaaattataaatatcagggcctttttaaaaaaaaaagattctgcttataacttggtatttgtttataataaaaattatagtagccaataatgaacacttactctggcttggttatttacttaggtcaaaagaaggaggagcggttaaactgtgggatcaggaactgaggcggtgccgtgccttcaggcttgagacaggacaagccacagattgtgttcgttctgtgtgcagaggcaaagtaagatgttccatgagctgatacagtgcagcagaaaacagaaagtggttattactgtgattccctcaccctttgcagcctaatgaacaatacttaataatgcataacgatggatttgcttgccaacattactctgtctttgctgctttctttgccaaagttagcaccagtgtggtgcataagctaggaagctattctgtctaaatactgtatgtaaacctccaatattttctagaatctgccaatttaacaactctagtagacataattgaaagcccttggcagttgactcatattaggacagctgtctccattttttaaaaaaacacacattccctagataaaacgtgcagtaaacaaacaatgaaatactactcagccataaaaaataatgaaattctgtcattcttggtggcaacatggatgagactggaggacatgatgtgaagtgaaataagccaggcacagaaagataaatacatgttctcactcctgtgcagaaactaaaaaagttgatcccacagaggtggagagtagaatagtggttactggaggcggacaagggggagggggagggggatagggaaggactggttaaaggatacaagtttacacagccagataggaatagtatgttttagtattctgtagtactgtaggatgactatagttaagaatcacgtatttatgtattttcaggtatttacaagagaggattttgaaagtttccatcacaaagaaatgataaatgtctgaggtgatggttatgcgtattaccctatgccctatagatatgtataattatgtgtcaatttcaaaataaaaattcaaaactacaactcctatgaaaatttttgagcgtgtttgtacttattaagtgtatttataaatcatacggatattatcttcagcctgcatattaaattgtagttaagcttttactttttaactaaaaaataaattctattattttttcctatatcccactgcactgaccccagtttggaaatcctaagattatcaaataaaaactttgattattgaagaatccaggtgtactgccacagaaaagttctattctgtagcatggactctaatatgtaatctagcccattgtgcttacagatagatgtgtgcctgtagtcatagaaaaatttgcatgagctaatgactgccttgctactagattagctcaaagcaaaaagttctctgaaagcaggtcaatagggtcatttttatattatgaagaagaaaagcagctgttgtattacattcactgtattggtcctgcttgtgtttcagggcaagatccttgttgggacaaggaatgctgaaataatcgaagttggagagaaaaatgcagcttgtaatattttagttaacggtcatgtggatgggccaatctggggactagcaacacatccttccagggattttttcctttctgctgcagaagatgggacagtgagactttgggatattgctgataaagtaagtacagataatttttttaaaagaggttacaacttctaaaaagaaaagttggaagttctaaattgctagtacttaaagaactgccagaattctgttgagcattttgaggggaaactggtataatttagaagtacttcacttaatgtttcctatgactctttttttttttttttttaaatgcagaagatgttaaacaaagtgaatttgggacatgctgctcgtactgtgtgttacagccctgaaggggacatggtggctattggaatgaaaaatggagaatttatcattttactagtgagttctctaaaaatatggggaaagaagagagacaggagatgtgcaatccatgatatcaggttagtgaacaaatggaatagagtttctagtatatacttgatttaacttccatttgtaaaattttccatagccttgccttcaaaaagaggtccccagggcctgtagcatttcccgtattataaattgtatgctaaaatatggctgtttgtatactacttaattcttcttgctaaattataaacccactgggcaccaactataatagcaagtactagtaggtaatgtttgatgaattcatgttaacacttagccatgtccattaagttcatcccaccaagaggtatctcccactgtaatacaagagagctatctgcccttcaaaagttgtcaccctggaaaactaaagttgtgatttcaaacatatcttctcttagtaacctcagtttgggaatatgtagttcattaatttaatcaatacctattgattaaatgttccagaatccaaattaatttaaatgtttcttaaacctttgtttttcagtgcttaagcatttttcaacagtggctaccatttacggagtacttccgtgtgatcagtagataagattattgaatctaggtctgtcaaaagcttgtacacttttcatcagtaaaatccttttacaaatgaaaccttcctcagaacttcaatatataaaatagtaacagtggcttcccttagcttttacatgtctctatcgtacctcagtaagactcatgggccatttcaagagactgaattgtcccatatgactccaaagattgctaggcaaatagcatttcactttgtcttttaaataagttcttcaggccgggcgcggtggctcatgcctgtaatcccagcactttgggaggccgaggcaggcagatcacctgaagtcaggagtactcgaccagcctggccaacatagtgaaaccccatctcaactaaaaatacaaaaatcagccgggcgtggtggcaggcgcctgtaatcccagctactcagggggctgaaacaggagaatcgcttgaacccgggaggcggaggttgcgccatcgcactccagcctgggagacaagagcgagacttcgtctcaaaaaaaaaaaattcttcttccaagattcaagttgtgtcatttcaccttaataactggaggttagttaagctgggctgtgttctttgcttaatattaagacaacgttttttccagatggaagaaaactatcttaatgaattgttagcttattaattatgtaatgctaatggcttttaaaagctgagatgttctgactgggtgttgtggctcacacctgtaatcccagtaccttgggaggccaagggggaaggattgcttgaggccaggagtttgggaccatagtgagaccccgcctctatttaaaaaattaaattttgttttgttttgttttgagttggagttttgctcttgttgcccatgctgaagtgcaatggtgcaatctcagctcaccacaacctgtgcctcctgggttcaagcgattctcctgcttcagcctcccgagtagatgggattacaggcgtgcaccaccatgcctggctaattttgtatttttagtagagacagggtttctctatgttggtcaggctggtctcaaactctcgacctcaggtgatctgcccgcctccgcttcccaaagttctgggattataggtgtgagccactgggcctggcctaagaaagtttttttaagccattagacgtttttaaaggaattgggagatgacaattggggaaatatttaaaatttaagtaaaatataaagcttccttatttcatgtaacccagacaatctcagtatacatgatcagttgtgtctgacaggtaaatctatttgaggccttatcacacgttacttttaagaactagaaaggaaaagtcactgatcttaagtatttataatacttcatgtggtctaatactttttacgttttgttttgattcagatttagtccggattcccggtatctggcagtaggttctagtgagaactcagtggatttttatgacctaacgctgggccccactcttaacagaatcagctactgcaaagacattccaagctttgtcattcaaatggacttctctgcagatagcagttatctccaggtacagtaccaatactgtatacccaggtggcaagttcttctgcttttacatttcgtgttagtgaatgcatttaaagttcctgagctccagagctccagcttctcaactcctccctttgtaccttctgacctacagctcccctttcctcccccacttatcagagcttttctcctattaagtttttgtagtgatcttttgcatacttaataatgttagacatgtaaatcaagtagcaatatgctagtattctgtaaaccccctgtggattttgtctctcacctaatggaattcttgtcccattttaatctgatgaaaaaggtctctagtggctgctataaacggcatgtctatgaagtgccttcaggaaaacatcttatggatcatgccgctattgacagaattacttgggctacatggactaggtaaatacttatatattcacaaggcaagaactgactttgaaggccagttagaaaatcctatttctgaactgttagagccattccaataaggaatagtaattgagtttcaagtttttgttaccatattttgaaatggtatgttcatgttgggacccctttttattgaatatatttccatgttttatcagtttccatgatttatcaagttttttttttaaggaaatcaaagttttaactttaaagataccctgatatttttcttaatgctaaatttaatgactggcaaaaaggtattgggtgctgttaagcaactgttattaattctctatctaaaggaatgctatcttgaatctattagaagtcaaagcttccaaatttgttcaaatttcctggctgtatgacaggtaaccatgactatccatttttttggccaatgaaaaatgccatcaaattcctgtatcagccaggcatatagtggctcatgcctgtaatctctgatgtagcaggccgaggtgggaggatcacttgagcctagaagttttgataccagcctgggcaacatagcaagaccccatctctgaaatttttttaattcctatgtcataagtcatttttatttttgtagagatagggatctcacaatattgcccaggctggtctcaaactcttggcctcaagcagtcctcctgcctcagcctcccaaaatgttgggattactggtatgtgctgctggacccagccaagtagcacttttaatttgaaaaatagttctatcagttttcagtcaggcgcggtggctcagcctgtaatcccagcactttgggaggccgagcgggggtgatcacctgaggtcgggagttcgagactagcctgaccaacatggagaaaccctgtctctactaaaaatacaaaataagccgggcatgttagcgcatgcctgtgatcccagctactcgggaggctgaggcaggagaattgcttgaacccaggaggcagaggttgcggtgagccgagatcatgccattgcactccagcctgggtaacaagagcgaaaactccgtctcaaaaaaaaaaaaagaaaaaatagttctatcagttttcataaagtactactttaatcttaaaaagattaatctagaaacccttcaaattataaaatgtcatttttaaaaggcaggagttgatatcctgatgaaattcaggtctccaaacaacttaccataatttacttcctgtattttaagtaacatgatagggtacttagagattaattgccaagaaactttttgaatatagtcaacctgcccgcacttgccatgatgagttttcttttgttccttccctctagtattctaggagatgaggttttgggaatctggtccagacatgctgagaaagctgatgtcaactgtgcctgtgtatctcattcaggaatcagtcttgttacaggagatgactttggcatggttaagttatttgacttcccatgtccagaaaaatttgtaagtttgtgttttgtttactattatcagtttactcctaattttgatgtcttatcatcagcacttttccccatatatttaaaatgttttgtcctaatttctaaatttttccccaaactttctaaatctatttactttgaaataaaagctattagaaacaaatcctctccctcgagtaataccatctttggaaccatcctacaaaagctgtaattagcttttcaccaaacctataatcagttatcaaatttcaaatgcttttccttagagaaaaatggtcagagtacctggagacatctgactgcccacacagcctggttttgcagatccactactcatgctgaaaagcattctaatcactggctgcggtgctaactccctactctctccacagctcttgtcatagagattatagttcctaataagagcctttgacttctgtgtgcaccaaatgccctgagcttgtctgtcattgttttttaggcaaaacacaaaaggttcttgggtcattcgccccatgtgacaaatattcgatttaccagtggtgatcgacatgttgttagtgctggaggtgatgactgcaggttagtaactttctcagcccatgaagagcagactatgttactagttaagagacttaatacaacaactcctacagctttggtttatgaaatcagctagtcaacattagtagaaggtagtataaccagatggctcttcagaatctcatatttatgcaaatacagaataaaaggagttaaagaggaaaaatattacacatgtaacctgaaagcacaactgaaaaatattaaactgttatgaaaatctaaaaacataattaactccctgcaattttcttctctgattgcagcttatttgtctggaaatgtgtacatacacctcactgagagatgctgagatgactacagaaattaactttgagaccagaattacagagaagaaaaaccaaaacccaaccctgcatggtcaagtggtgctaacccaagactgtaacagggagaaatgcccagaatcatcaaaatagtgaaagactgatctgttcaaaatatttgctatatgcactgggtataatccgtaatccatacactgccagataatgccatttcaaggaaggatcgaatacttgatggtaaaggccaagtccccctgtattgggaagtgtgtgatttcggcagacctgctgggaaaatttagggtagagcactctttacagaagaactcaaaaacccaatttggataattttcattatctttttagcaaaatggtttcttaatgtttatattttattttcaaggttcattgtttaatgaaatattttattcttgcatttccataaggaaagggaaagtcatgatcatcctaaaggatcacagtttttaaaaggcaaacattttccctaaggaaacagacacaagctttcctagagaatatgatgttttttaggcattaataaggtccttttttataaaggacacttttctcctagtagttttgaattcaggaacagatccaaagttagcagtatatggctgctacatttccattttcattttcgagccatcagtttatgttcagatgccatctctgtaatcgcacatttaaaacataactgtagcctcactaatggaaaagtagtatgatgaacaatcattcccaatggtgtacaatgtaagggttttagggagcaacagtatttaactggaagaaagaattgcatatttaatgtagtctaatatatacacatttgtttaacatgtaaacaaaagtgttaaattcacatatacaacattatacaatttaatcactcttggaataaaatttttatagccttttttctattgggaaaatttgtttagatgtgtgccactccataggtttatttccaaaatgaatgagcccaactccatttgtaaaaacttgtcagttagaattcctttttttagtggattagggctgaattcttagatccttatttcttttcactttaaatgctgccaaagatcactactcatcattcaggaattcgctgtctagcctatctgtagtttcctgaagattgaaaattatgtagactgctatttaaaaatatatttttctaagtgtgaggtttaagatgctgtattgaccctatgagtttttaatgtgttaattatctttatagcataatagatcgctttaggttcctggaatcccatttggtctgacaggatatatgaagattcttaatacctattttctgtgtctaatacttggttaatactaaaaatagaaatgactaaattacatcacagaaagcataaccagtgattgaacctggtagttttaaagctctaaatagctgtggctgaaggactgattatggggctaagaagcttgaaacgtaagttggtacttgttcatcagtggattctcctaaattaagccaaattttgaaatacatgactattaagtttctactcatgtatttacagtcagtcaataaattaaaggaggaaaaaaatccctgaacaacctgcccataaaaagaaaaatactctacatttgagcctgctgcagttttaaattttccctctgggtcaagtttgccagcttttggctacagagaaattatatttccattacagtgcaggtagaaactctgtaaccttaagcatgtaaactacatagaataaaactgtttccactgcatttctgtccttcaaagtggccaacctgattaagtcagccttaatcactgctgctgtcagtttcacgactaaaggtcatattgactaagtagtcatcagctgaccacctcgctgtatcagccagcaacgaggggaaggtgaagaaacatgataggccatatagaatctgccctatgtttacttttttaacccagataattatttttgtgtgcagtatctaagctcctgattgtgtaacctgggacttctggcaccttttgttccattcattttatgtataaaatgcatgccaaagcacactgtgccctctggtacccttgcttccaatcgccaaccatgctcatttccttcctttttttgtggtccctttttgtggtgatcattttaaaccacgtcatccaacaaatgttttatggtcaaccttagcttgttcataagccatagcaactgaaagattaaactcttaaatatgtgtctgggcagtggctattaaatagcaaaaaacaatcagattttagtattttattatttccttgtaaaatggctgaactaaattaaacccttgtttcccatttgttctataatttatagtgaaactgagaacaaaactatctttataaatgatagctaaaagtatttccagatatttaaacaatttaaaataaatttcttctgcagagatgcaaagcatctcaacactggaatgaacaaatgccttaaattcaatggagtaaacctttagaatgaagaggaactgtcatttcacccaagccgaagacaacagccttatgcacttgtgtgctctgtctttgctgcttctcgtgtttcaagcctttcctgtgggatcagcacagcaaagtgcaacttaccaaatggtttaatgactggttaattctttcttctcccaatggaaaagcaatggcaacacaacagtagactgctggcttgacaatcttaaacgtgagcctttgcacatgtaggtttatcatcatttgagtatacgactaagcaagtcaatgaactttttttttttttttagcagtttaatttggtcctgagaatgttgcagtctttattaccccttttgcattaatccacttttctaaccaccttttaagctttaatttttaacactatacaccaagtctttgaaatcagtgatctgttatttaactctaaagcatttgacacttcttgccttaacagttttaaaaaccacacacaaaaaaactctgtaagtaatacagtaggccaaaagtttcatcctatctatcttgcagtttacctatctgatctgatctctgtaattatagttctgtcatttaaaatatactatttaaatctaatttttacatttcaaaaattatcttcagtagtaactaagtatattttctgtggattctgagaatgttatttttcagaatgtgagaatatatatgtacatttataatcttgtgactttaaagtctgttttcagatacagtatgtaaatacttgtaaaaaaatttgtataattttgtgataatgtagtttcccaaaaaaattatttagaaggcattatgttattagtaaatgagagcactgtatagaactgttcctattttctgcacttgccattccagctgcctccactgtccatacccacctcattcatcctgtcacagaaggcaggaaaactgggaactttaccaaagtagcactcagcctgagaggcctgtataatcatgcttttcaaactaaattcacttaaaaattaaaaagcagaattgaatattttaagcagcctcagtacctttggccaatgctgttttcatggtggattatgaacattatataatctttgggaaaagtgaaagtagtacaatttttagaataatgacaactgcctcactgcatctctccactcacacagcaaccgtgtagccccctaagctgcagtaccatgactaaccatgatgtcaatttcatatgctgatcctcacaacagcagtgcacaaacatgccccaaatattttaacagaatttagctcttccttaagctgtcttttcatagtaaaaacaaaacaaaaacacccaatgttaaaaccacataataaacttacaaacttgaaaaattagacacttcagatagataggcaataaaacttcatattatgaaagcaatatattccaagtttcaaagatttgacaagttctgtagagtatctttcatcagtacatgaaaacttccaaactgcatgatcttctgccaggcaggactgggtgctattcgctggtttgaggtcgaatccatttcaaggcatgtcgtggtgggacattaatggtgggatggtagaatgtgcagtccggtcttgtacattgagtgttaaacctacaatgttttggatgatagaagggacattccatcttcttacaagcagggaagtaacggcagagctgactactggaaggtggtgctggtggtgcaactgctggttttggagacagtactggaattcttctactcacatgagtgaagggacaatctggtttagtacactttgcatcatatttacaatttgggtgaacaaacaaacatttttcagcaaatttacaattggggaaggctttgcagggtgagatggggtgatggtaggcacactcatccccatttttacaagcaggccagtacttgcagcgctccaaaagtttttctggtttctgtgccacactcagttcactcatctcagcttgatttttttctacagaatctccttttgtttcctcttctttaatggggggacttattctgggggtcctactttgtccctggaccacttctgctagcaattcttcttgagaagttcgagttctgggagcaactggaagtgtctgtttctgtggaactgtagagtagttagttgtttttgttacggattcttgagcttcagatatagccttcaaaatcagattcttgttagcttgtttagaaggtggaagagaaggtctcctttcaggctttgcaggcacagacacactgctggagatgcttcctgttcgagacccgtaatcatcatcttcttcctcctcttctccatcatgattgaatttttttactttaacaactgaacttaccacaggcaactttctcttccgaaagttttcatcctccatactcattttctccgagttgtttctaaagaacggactatacgtttcttctaagctgttaagcacctctggttcacacaaacgtcctgtttcatatacccaactactctgcatatcaagctgcttggcagcatgaatactattctgctgctgttgaaattgcaacctgtttaaatgaacaccactatctgcatttctacttgcaggtggtcgataaatttcaatagaagggcgagaagaaccatatgtaagtgtcactgtaggttttttctgagataagggattctcctgcacaaagttgaggtcttcgtcaatgagatcatctggttctggcttaatatcaatcacatcttcagagggtgctggctccctcaaaggtttcactgttgacattagtcgggttgcagctccatcatcgtaagtctgtctgacatttgtggtttttgactcctgcgaacttgtagaaactctggaatctcttttttcaggtctcgcgctaggaatggcaagtggtggcactgcagcttcatgcctcctctcatctccccgactgaaattgctcttgtttgaaggcacgttactatcaaagatgttggtatcagaagacttcagactagagggttcagttgtaacagagcgaagtttatctaatacaccatgaagccaacataagctcctaattcttgtaatttccccttaatggcactccggatcttgcggctgatctcggtgccgatctccatggctctgcggcgtgcgggaactcagcactgcgcggcgcttggcttacccggaggctgccgcggactcctaccccgcagccgggacaccaccgcctcc

SEQ ID NO: 13619 - RNA, 16463 nt, Homo sapiens
  source 1..16463: mol_type = other RNA
gctgggattacaggcatgagccaccataataaggattctgatgaacatttgattccttggactactgttatactcaaaagccttccttaatcttctaattgtcaccctaaatatcctaaaatttctgtcttcctagtagttcttcatagtcctaaaaatttgtcagagagaaaggtaaatcaagaaacatgattttcaaatgatttaaggtggtactagggtttaggatttcctttgctttttatcatttaacacactgcttatcatacagctggaagtgctctgggccagtgtctctacttcgagggaagaaggaggtagtgagacagaaggaaatagcacaattcctggccctgacagaagggtgttcaggagacctgctctcctctcactttattccatctcatctggacctgtggcttccaatccacatctctttcctttaatatcctgcattggctaggctgtataaatcctttggtgcatcgaaaaactaagtgcattttttgtttttgtgattatgcaatacttataggaaaagttataattttagaatatttaagtacacttacatttttgagaaaaagactattgaaatgtttgtgccatgtcaaatttcagttgaacattttgggtattcttaatataagaccaggccaggcaccgtggctcaggccgggcacagtggctcacacctataatcccagcacttagggaggccaaggcgggaagatcacctgaagtcaggagttcaagaccagcctggctaacaaggtgaaactctgtctctactaaaaatacaaaaattagccgggcgtggtggctggcgcttgtaatcccagctacttgggaggctgagacaggagaatcacttgaacctgggaagcagaggttgtggtgagctgagatcgcaccattgcactccagcctgggcaacaaagagcgaaactccgtctcaaaaaaataaaaaataaaccctagaattatagtatgttagaattggaagggaagaattgtctaaggttattctagctaataagcaacagacttggaaaggaaaaggtcctgacaaagctaagcctcccgttcaggtttcctgactcgtgaattcagtgctgctgccactacacgatgcatgctctttgtatcaagggtgagacagcattacacatacatagaaaattatctatttaaactctatttgaacttttgatgagtttgtctccccctcccccactccttttcagaataacttgacgtttacaggtaccatcagtggtgatgtctgtgtgtggaaagatcacatattgtgtagaatcgtggcgagagctcacaacgggcctgtgtttgccatgtacaccaccctgcgagatggacttatcgtgactgggggaaaggaaaggccgtgagtcctctttcttttcacagaatatttatgcatttgtgacctacctgaggtttgcagttaattattctagttgtttctaggctacacagagtgtcctctccgaccttcctcctcatatgcttctcctttattaccttttatgtgccttctatttgattctcatttctggtcttaattcacttccaatttttttcatgttggggtgatactttttctgaggtgtggataggtagttgtcctacaagttgagttacttttcttaatgtctgtatgcctgtgtatgatttgctgagtaggaggcccatgggggaatctggagccagggttgtattttgactgcctgctctctttttgttcagaatggattctaaggagtagaatgcacattgttgctttagaaaaggatgagggaactagagagaactgccttgtttccttttgcttgaggcaaatttaaactgttttatacaagacctcaaaatttgagaagaggtctcttctgagtgattttcaaatctcccaacagtaaccagatacttatgatttgatttgtcaccaacatagtcatatgcatgttgaaacatgacatgtaggccaggcacagtggctcacacctgtaatcttatcactttgggaggctgaggcaggtggatcgcttgagcccaggagttcaagaccagcctgggcaacatggtgaaaccccatcgctataaaaaacaacaattagccgggtgtggtggcacatgcctgtagtccctgctactcaggaggctgaggtgggaggatcacttgagcctggggaggtcaaggctttagtgagctgtgatggtgccactgcactccagcctgggtgacagagtgagaccccatttaaaaaacaaaaacaaaaacaaaaaaaaatgtgacatatagttgactaagaagtacatttcaatacaggattgaaagaacccacatatgttaattaaacacaagcgcagaatttgtgccttttacataaaggaagaatgcacataggcatgctttcagacaagcaattcatctagcagaaaaggaaggaatacatttttcagcccttccaggaataaaatccataaatgggctctatttcgtcctccaacacttgtatttcccacgtcatttactcctgcacacccccactcactagaagcctgctaaactgttccagtgagatattttaacacctgatagggaataaatatgcttctgttttggccttcaaaaataagctctgggccagttgcagtggctcacgcctgtaatcccaacactttgggaggccgaggtgggcggatcacgaggtcaggagtttgggatcagcctggccaatatggtgaaactccatctctactaaaaatacaaaaattagccaggcatggtgcctgtaatcccagctacttgggaggctgaaggagaagaatcgcttgaacctgggaggcacaggttgcagtgagccgagatcacaccactgcactccaggccaggtgacagagcgacactctgtctcaaaaaaataaataaatcaactctgtagcatagcatttgtaattctattattttgccttacatttccattatccttttaataaaattgtttttttacatcttcctaatcaagaagtattatgaggccaggcacagtggctcatacctggaatcccagcactttgggaggccgaggcaggcagatcacctgaggtcaaggtatttgagaccagcctggccaacatggtgaaaccccatctctactaaaaatacagaaattagctgggtgtggtggtgcacacctgtaatgctagctactcgggaggctgaggtaggagaatcgcttgaacctgggaggcagaggttgcaataagcctagatcatgccactgcactcaagcctgggagacagagcgagactacatcttaaaaaaaaaaaaaaaagtattatgagagaggataatgtattgtaatgtattgtagaggctaaataaaattatgctcatgtcagaaaaaaagagtatttctcaaaataaaattcactgaaactggatgtttattttgactgagatatagtatatcctcaaattgccatagaaagtttacaagaatattagaggtaaattataaatatcagggcctttttaaaaaaaaaagattctgcttataacttggtatttgtttataataaaaattatagtagccaataatgaacacttactctggcttggttatttacttaggtcaaaagaaggaggagcggttaaactgtgggatcaggaactgaggcggtgccgtgccttcaggcttgagacaggacaagccacagattgtgttcgttctgtgtgcagaggcaaagtaagatgttccatgagctgatacagtgcagcagaaaacagaaagtggttattactgtgattccctcaccctttgcagcctaatgaacaatacttaataatgcataacgatggatttgcttgccaacattactctgtctttgctgctttctttgccaaagttagcaccagtgtggtgcataagctaggaagctattctgtctaaatactgtatgtaaacctccaatattttctagaatctgccaatttaacaactctagtagacataattgaaagcccttggcagttgactcatattaggacagctgtctccattttttaaaaaaacacacattccctagataaaacgtgcagtaaacaaacaatgaaatactactcagccataaaaaataatgaaattctgtcattcttggtggcaacatggatgagactggaggacatgatgtgaagtgaaataagccaggcacagaaagataaatacatgttctcactcctgtgcagaaactaaaaaagttgatcccacagaggtggagagtagaatagtggttactggaggcggacaagggggagggggagggggatagggaaggactggttaaaggatacaagtttacacagccagataggaatagtatgttttagtattctgtagtactgtaggatgactatagttaagaatcacgtatttatgtattttcaggtatttacaagagaggattttgaaagtttccatcacaaagaaatgataaatgtctgaggtgatggttatgcgtattaccctatgccctatagatatgtataattatgtgtcaatttcaaaataaaaattcaaaactacaactcctatgaaaatttttgagcgtgtttgtacttattaagtgtatttataaatcatacggatattatcttcagcctgcatattaaattgtagttaagcttttactttttaactaaaaaataaattctattattttttcctatatcccactgcactgaccccagtttggaaatcctaagattatcaaataaaaactttgattattgaagaatccaggtgtactgccacagaaaagttctattctgtagcatggactctaatatgtaatctagcccattgtgcttacagatagatgtgtgcctgtagtcatagaaaaatttgcatgagctaatgactgccttgctactagattagctcaaagcaaaaagttctctgaaagcaggtcaatagggtcatttttatattatgaagaagaaaagcagctgttgtattacattcactgtattggtcctgcttgtgtttcagggcaagatccttgttgggacaaggaatgctgaaataatcgaagttggagagaaaaatgcagcttgtaatattttagttaacggtcatgtggatgggccaatctggggactagcaacacatccttccagggattttttcctttctgctgcagaagatgggacagtgagactttgggatattgctgataaagtaagtacagataatttttttaaaagaggttacaacttctaaaaagaaaagttggaagttctaaattgctagtacttaaagaactgccagaattctgttgagcattttgaggggaaactggtataatttagaagtacttcacttaatgtttcctatgactctttttttttttttttttaaatgcagaagatgttaaacaaagtgaatttgggacatgctgctcgtactgtgtgttacagccctgaaggggacatggtggctattggaatgaaaaatggagaatttatcattttactagtgagttctctaaaaatatggggaaagaagagagacaggagatgtgcaatccatgatatcaggttagtgaacaaatggaatagagtttctagtatatacttgatttaacttccatttgtaaaattttccatagccttgccttcaaaaagaggtccccagggcctgtagcatttcccgtattataaattgtatgctaaaatatggctgtttgtatactacttaattcttcttgctaaattataaacccactgggcaccaactataatagcaagtactagtaggtaatgtttgatgaattcatgttaacacttagccatgtccattaagttcatcccaccaagaggtatctcccactgtaatacaagagagctatctgcccttcaaaagttgtcaccctggaaaactaaagttgtgatttcaaacatatcttctcttagtaacctcagtttgggaatatgtagttcattaatttaatcaatacctattgattaaatgttccagaatccaaattaatttaaatgtttcttaaacctttgtttttcagtgcttaagcatttttcaacagtggctaccatttacggagtacttccgtgtgatcagtagataagattattgaatctaggtctgtcaaaagcttgtacacttttcatcagtaaaatccttttacaaatgaaaccttcctcagaacttcaatatataaaatagtaacagtggcttcccttagcttttacatgtctctatcgtacctcagtaagactcatgggccatttcaagagactgaattgtcccatatgactccaaagattgctaggcaaatagcatttcactttgtcttttaaataagttcttcaggccgggcgcggtggctcatgcctgtaatcccagcactttgggaggccgaggcaggcagatcacctgaagtcaggagtactcgaccagcctggccaacatagtgaaaccccatctcaactaaaaatacaaaaatcagccgggcgtggtggcaggcgcctgtaatcccagctactcagggggctgaaacaggagaatcgcttgaacccgggaggcggaggttgcgccatcgcactccagcctgggagacaagagcgagacttcgtctcaaaaaaaaaaaattcttcttccaagattcaagttgtgtcatttcaccttaataactggaggttagttaagctgggctgtgttctttgcttaatattaagacaacgttttttccagatggaagaaaactatcttaatgaattgttagcttattaattatgtaatgctaatggcttttaaaagctgagatgttctgactgggtgttgtggctcacacctgtaatcccagtaccttgggaggccaagggggaaggattgcttgaggccaggagtttgggaccatagtgagaccccgcctctatttaaaaaattaaattttgttttgttttgttttgagttggagttttgctcttgttgcccatgctgaagtgcaatggtgcaatctcagctcaccacaacctgtgcctcctgggttcaagcgattctcctgcttcagcctcccgagtagatgggattacaggcgtgcaccaccatgcctggctaattttgtatttttagtagagacagggtttctctatgttggtcaggctggtctcaaactctcgacctcaggtgatctgcccgcctccgcttcccaaagttctgggattataggtgtgagccactgggcctggcctaagaaagtttttttaagccattagacgtttttaaaggaattgggagatgacaattggggaaatatttaaaatttaagtaaaatataaagcttccttatttcatgtaacccagacaatctcagtatacatgatcagttgtgtctgacaggtaaatctatttgaggccttatcacacgttacttttaagaactagaaaggaaaagtcactgatcttaagtatttataatacttcatgtggtctaatactttttacgttttgttttgattcagatttagtccggattcccggtatctggcagtaggttctagtgagaactcagtggatttttatgacctaacgctgggccccactcttaacagaatcagctactgcaaagacattccaagctttgtcattcaaatggacttctctgcagatagcagttatctccaggtacagtaccaatactgtatacccaggtggcaagttcttctgcttttacatttcgtgttagtgaatgcatttaaagttcctgagctccagagctccagcttctcaactcctccctttgtaccttctgacctacagctcccctttcctcccccacttatcagagcttttctcctattaagtttttgtagtgatcttttgcatacttaataatgttagacatgtaaatcaagtagcaatatgctagtattctgtaaaccccctgtggattttgtctctcacctaatggaattcttgtcccattttaatctgatgaaaaaggtctctagtggctgctataaacggcatgtctatgaagtgccttcaggaaaacatcttatggatcatgccgctattgacagaattacttgggctacatggactaggtaaatacttatatattcacaaggcaagaactgactttgaaggccagttagaaaatcctatttctgaactgttagagccattccaataaggaatagtaattgagtttcaagtttttgttaccatattttgaaatggtatgttcatgttgggacccctttttattgaatatatttccatgttttatcagtttccatgatttatcaagttttttttttaaggaaatcaaagttttaactttaaagataccctgatatttttcttaatgctaaatttaatgactggcaaaaaggtattgggtgctgttaagcaactgttattaattctctatctaaaggaatgctatcttgaatctattagaagtcaaagcttccaaatttgttcaaatttcctggctgtatgacaggtaaccatgactatccatttttttggccaatgaaaaatgccatcaaattcctgtatcagccaggcatatagtggctcatgcctgtaatctctgatgtagcaggccgaggtgggaggatcacttgagcctagaagttttgataccagcctgggcaacatagcaagaccccatctctgaaatttttttaattcctatgtcataagtcatttttatttttgtagagatagggatctcacaatattgcccaggctggtctcaaactcttggcctcaagcagtcctcctgcctcagcctcccaaaatgttgggattactggtatgtgctgctggacccagccaagtagcacttttaatttgaaaaatagttctatcagttttcagtcaggcgcggtggctcagcctgtaatcccagcactttgggaggccgagcgggggtgatcacctgaggtcgggagttcgagactagcctgaccaacatggagaaaccctgtctctactaaaaatacaaaataagccgggcatgttagcgcatgcctgtgatcccagctactcgggaggctgaggcaggagaattgcttgaacccaggaggcagaggttgcggtgagccgagatcatgccattgcactccagcctgggtaacaagagcgaaaactccgtctcaaaaaaaaaaaaagaaaaaatagttctatcagttttcataaagtactactttaatcttaaaaagattaatctagaaacccttcaaattataaaatgtcatttttaaaaggcaggagttgatatcctgatgaaattcaggtctccaaacaacttaccataatttacttcctgtattttaagtaacatgatagggtacttagagattaattgccaagaaactttttgaatatagtcaacctgcccgcacttgccatgatgagttttcttttgttccttccctctagtattctaggagatgaggttttgggaatctggtccagacatgctgagaaagctgatgtcaactgtgcctgtgtatctcattcaggaatcagtcttgttacaggagatgactttggcatggttaagttatttgacttcccatgtccagaaaaatttgtaagtttgtgttttgtttactattatcagtttactcctaattttgatgtcttatcatcagcacttttccccatatatttaaaatgttttgtcctaatttctaaatttttccccaaactttctaaatctatttactttgaaataaaagctattagaaacaaatcctctccctcgagtaataccatctttggaaccatcctacaaaagctgtaattagcttttcaccaaacctataatcagttatcaaatttcaaatgcttttccttagagaaaaatggtcagagtacctggagacatctgactgcccacacagcctggttttgcagatccactactcatgctgaaaagcattctaatcactggctgcggtgctaactccctactctctccacagctcttgtcatagagattatagttcctaataagagcctttgacttctgtgtgcaccaaatgccctgagcttgtctgtcattgttttttaggcaaaacacaaaaggttcttgggtcattcgccccatgtgacaaatattcgatttaccagtggtgatcgacatgttgttagtgctggaggtgatgactgcaggttagtaactttctcagcccatgaagagcagactatgttactagttaagagacttaatacaacaactcctacagctttggtttatgaaatcagctagtcaacattagtagaaggtagtataaccagatggctcttcagaatctcatatttatgcaaatacagaataaaaggagttaaagaggaaaaatattacacatgtaacctgaaagcacaactgaaaaatattaaactgttatgaaaatctaaaaacataattaactccctgcaattttcttctctgattgcagcttatttgtctggaaatgtgtacatacacctcactgagagatgctgagatgactacagaaattaactttgagaccagaattacagagaagaaaaaccaaaacccaaccctgcatggtcaagtggtgctaacccaagactgtaacagggagaaatgcccagaatcatcaaaatagtgaaagactgatctgttcaaaatatttgctatatgcactgggtataatccgtaatccatacactgccagataatgccatttcaaggaaggatcgaatacttgatggtaaaggccaagtccccctgtattgggaagtgtgtgatttcggcagacctgctgggaaaatttagggtagagcactctttacagaagaactcaaaaacccaatttggataattttcattatctttttagcaaaatggtttcttaatgtttatattttattttcaaggttcattgtttaatgaaatattttattcttgcatttccataaggaaagggaaagtcatgatcatcctaaaggatcacagtttttaaaaggcaaacattttccctaaggaaacagacacaagctttcctagagaatatgatgttttttaggcattaataaggtccttttttataaaggacacttttctcctagtagttttgaattcaggaacagatccaaagttagcagtatatggctgctacatttccattttcattttcgagccatcagtttatgttcagatgccatctctgtaatcgcacatttaaaacataactgtagcctcactaatggaaaagtagtatgatgaacaatcattcccaatggtgtacaatgtaagggttttagggagcaacagtatttaactggaagaaagaattgcatatttaatgtagtctaatatatacacatttgtttaacatgtaaacaaaagtgttaaattcacatatacaacattatacaatttaatcactcttggaataaaatttttatagccttttttctattgggaaaatttgtttagatgtgtgccactccataggtttatttccaaaatgaatgagcccaactccatttgtaaaaacttgtcagttagaattcctttttttagtggattagggctgaattcttagatccttatttcttttcactttaaatgctgccaaagatcactactcatcattcaggaattcgctgtctagcctatctgtagtttcctgaagattgaaaattatgtagactgctatttaaaaatatatttttctaagtgtgaggtttaagatgctgtattgaccctatgagtttttaatgtgttaattatctttatagcataatagatcgctttaggttcctggaatcccatttggtctgacaggatatatgaagattcttaatacctattttctgtgtctaatacttggttaatactaaaaatagaaatgactaaattacatcacagaaagcataaccagtgattgaacctggtagttttaaagctctaaatagctgtggctgaaggactgattatggggctaagaagcttgaaacgtaagttggtacttgttcatcagtggattctcctaaattaagccaaattttgaaatacatgactattaagtttctactcatgtatttacagtcagtcaataaattaaaggaggaaaaaaatccctgaacaacctgcccataaaaagaaaaatactctacatttgagcctgctgcagttttaaattttccctctgggtcaagtttgccagcttttggctacagagaaattatatttccattacagtgcaggtagaaactctgtaaccttaagcatgtaaactacatagaataaaactgtttccactgcatttctgtccttcaaagtggccaacctgattaagtcagccttaatcactgctgctgtcagtttcacgactaaaggtcatattgactaagtagtcatcagctgaccacctcgctgtatcagccagcaacgaggggaaggtgaagaaacatgataggccatatagaatctgccctatgtttacttttttaacccagataattatttttgtgtgcagtatctaagctcctgattgtgtaacctgggacttctggcaccttttgttccattcattttatgtataaaatgcatgccaaagcacactgtgccctctggtacccttgcttccaatcgccaaccatgctcatttccttcctttttttgtggtccctttttgtggtgatcattttaaaccacgtcatccaacaaatgttttatggtcaaccttagcttgttcataagccatagcaactgaaagattaaactcttaaatatgtgtctgggcagtggctattaaatagcaaaaaacaatcagattttagtattttattatttccttgtaaaatggctgaactaaattaaacccttgtttcccatttgttctataatttatagtgaaactgagaacaaaactatctttataaatgatagctaaaagtatttccagatatttaaacaatttaaaataaatttcttctgcagagatgcaaagcatctcaacactggaatgaacaaatgccttaaattcaatggagtaaacctttagaatgaagaggaactgtcatttcacccaagccgaagacaacagccttatgcacttgtgtgctctgtctttgctgcttctcgtgtttcaagcctttcctgtgggatcagcacagcaaagtgcaacttaccaaatggtttaatgactggttaattctttcttctcccaatggaaaagcaatggcaacacaacagtagactgctggcttgacaatcttaaacgtgagcctttgcacatgtaggtttatcatcatttgagtatacgactaagcaagtcaatgaactttttttttttttttagcagtttaatttggtcctgagaatgttgcagtctttattaccccttttgcattaatccacttttctaaccaccttttaagctttaatttttaacactatacaccaagtctttgaaatcagtgatctgttatttaactctaaagcatttgacacttcttgccttaacagttttaaaaaccacacacaaaaaaactctgtaagtaatacagtaggccaaaagtttcatcctatctatcttgcagtttacctatctgatctgatctctgtaattatagttctgtcatttaaaatatactatttaaatctaatttttacatttcaaaaattatcttcagtagtaactaagtatattttctgtggattctgagaatgttatttttcagaatgtgagaatatatatgtacatttataatcttgtgactttaaagtctgttttcagatacagtatgtaaatacttgtaaaaaaatttgtataattttgtgataatgtagtttcccaaaaaaattatttagaaggcattatgttattagtaaatgagagcactgtatagaactgttcctattttctgcacttgccattccagctgcctccactgtccatacccacctcattcatcctgtcacagaaggcaggaaaactgggaactttaccaaagtagcactcagcctgagaggcctgtataatcatgcttttcaaactaaattcacttaaaaattaaaaagcagaattgaatattttaagcagcctcagtacctttggccaatgctgttttcatggtggattatgaacattatataatctttgggaaaagtgaaagtagtacaatttttagaataatgacaactgcctcactgcatctctccactcacacagcaaccgtgtagccccctaagctgcagtaccatgactaaccatgatgtcaatttcatatgctgatcctcacaacagcagtgcacaaacatgccccaaatattttaacagaatttagctcttccttaagctgtcttttcatagtaaaaacaaaacaaaaacacccaatgttaaaaccacataataaacttacaaacttgaaaaattagacacttcagatagataggcaataaaacttcatattatgaaagcaatatattccaagtttcaaagatttgacaagttctgtagagtatctttcatcagtacatgaaaacttccaaactgcatgatcttctgccaggcaggactgggtgctattcgctggtttgaggtcgaatccatttcaaggcatgtcgtggtgggacattaatggtgggatggtagaatgtgcagtccggtcttgtacattgagtgttaaacctacaatgttttggatgatagaagggacattccatcttcttacaagcagggaagtaacggcagagctgactactggaaggtggtgctggtggtgcaactgctggttttggagacagtactggaattcttctactcacatgagtgaagggacaatctggtttagtacactttgcatcatatttacaatttgggtgaacaaacaaacatttttcagcaaatttacaattggggaaggctttgcagggtgagatggggtgatggtaggcacactcatccccatttttacaagcaggccagtacttgcagcgctccaaaagtttttctggtttctgtgccacactcagttcactcatctcagcttgatttttttctacagaatctccttttgtttcctcttctttaatggggggacttattctgggggtcctactttgtccctggaccacttctgctagcaattcttcttgagaagttcgagttctgggagcaactggaagtgtctgtttctgtggaactgtagagtagttagttgtttttgttacggattcttgagcttcagatatagccttcaaaatcagattcttgttagcttgtttagaaggtggaagagaaggtctcctttcaggctttgcaggcacagacacactgctggagatgcttcctgttcgagacccgtaatcatcatcttcttcctcctcttctccatcatgattgaatttttttactttaacaactgaacttaccacaggcaactttctcttccgaaagttttcatcctccatactcattttctccgagttgtttctaaagaacggactatacgtttcttctaagctgttaagcacctctggttcacacaaacgtcctgtttcatatacccaactactctgcatatcaagctgcttggcagcatgaatactattctgctgctgttgaaattgcaacctgtttaaatgaacaccactatctgcatttctacttgcaggtggtcgataaatttcaatagaagggcgagaagaaccatatgtaagtgtcactgtaggttttttctgagataagggattctcctgcacaaagttgaggtcttcgtcaatgagatcatctggttctggcttaatatcaatcacatcttcagagggtgctggctccctcaaaggtttcactgttgacattagtcgggttgcagctccatcatcgtaagtctgtctgacatttgtggtttttgactcctgcgaacttgtagaaactctggaatctcttttttcaggtctcgcgctaggaatggcaagtggtggcactgcagcttcatgcctcctctcatctccccgactgaaattgctcttgtttgaaggcacgttactatcaaagatgttggtatcagaagacttcagactagagggttcagttgtaacagagcgaagtttatctaatacaccatgaagccatacggtgaatcgaattgtgttgttccctagaaacagggacagatcctctgtcatttggtcctgacttttcttgttggccaccatcaccataatgtaatcaggaagttcttcatcaacataagctcctaattcttgtaatttccccttaatggcactccggatcttgcggctgatctcggtgccgatctccatggctctgcggcgtgcgggaactcagcactgcgcggcgcttggcttacccggaggctgccgcggactcctaccccgcagccgggacaccaccgcctcc

SEQ ID NO: 13620 - RNA, 16913 nt, Homo sapiens
  source 1..16913: mol_type = other RNA
gctgggattacaggcatgagccaccataataaggattctgatgaacatttgattccttggactactgttatactcaaaagccttccttaatcttctaattgtcaccctaaatatcctaaaatttctgtcttcctagtagttcttcatagtcctaaaaatttgtcagagagaaaggtaaatcaagaaacatgattttcaaatgatttaaggtggtactagggtttaggatttcctttgctttttatcatttaacacactgcttatcatacagctggaagtgctctgggccagtgtctctacttcgagggaagaaggaggtagtgagacagaaggaaatagcacaattcctggccctgacagaagggtgttcaggagacctgctctcctctcactttattccatctcatctggacctgtggcttccaatccacatctctttcctttaatatcctgcattggctaggctgtataaatcctttggtgcatcgaaaaactaagtgcattttttgtttttgtgattatgcaatacttataggaaaagttataattttagaatatttaagtacacttacatttttgagaaaaagactattgaaatgtttgtgccatgtcaaatttcagttgaacattttgggtattcttaatataagaccaggccaggcaccgtggctcaggccgggcacagtggctcacacctataatcccagcacttagggaggccaaggcgggaagatcacctgaagtcaggagttcaagaccagcctggctaacaaggtgaaactctgtctctactaaaaatacaaaaattagccgggcgtggtggctggcgcttgtaatcccagctacttgggaggctgagacaggagaatcacttgaacctgggaagcagaggttgtggtgagctgagatcgcaccattgcactccagcctgggcaacaaagagcgaaactccgtctcaaaaaaataaaaaataaaccctagaattatagtatgttagaattggaagggaagaattgtctaaggttattctagctaataagcaacagacttggaaaggaaaaggtcctgacaaagctaagcctcccgttcaggtttcctgactcgtgaattcagtgctgctgccactacacgatgcatgctctttgtatcaagggtgagacagcattacacatacatagaaaattatctatttaaactctatttgaacttttgatgagtttgtctccccctcccccactccttttcagaataacttgacgtttacaggtaccatcagtggtgatgtctgtgtgtggaaagatcacatattgtgtagaatcgtggcgagagctcacaacgggcctgtgtttgccatgtacaccaccctgcgagatggacttatcgtgactgggggaaaggaaaggccgtgagtcctctttcttttcacagaatatttatgcatttgtgacctacctgaggtttgcagttaattattctagttgtttctaggctacacagagtgtcctctccgaccttcctcctcatatgcttctcctttattaccttttatgtgccttctatttgattctcatttctggtcttaattcacttccaatttttttcatgttggggtgatactttttctgaggtgtggataggtagttgtcctacaagttgagttacttttcttaatgtctgtatgcctgtgtatgatttgctgagtaggaggcccatgggggaatctggagccagggttgtattttgactgcctgctctctttttgttcagaatggattctaaggagtagaatgcacattgttgctttagaaaaggatgagggaactagagagaactgccttgtttccttttgcttgaggcaaatttaaactgttttatacaagacctcaaaatttgagaagaggtctcttctgagtgattttcaaatctcccaacagtaaccagatacttatgatttgatttgtcaccaacatagtcatatgcatgttgaaacatgacatgtaggccaggcacagtggctcacacctgtaatcttatcactttgggaggctgaggcaggtggatcgcttgagcccaggagttcaagaccagcctgggcaacatggtgaaaccccatcgctataaaaaacaacaattagccgggtgtggtggcacatgcctgtagtccctgctactcaggaggctgaggtgggaggatcacttgagcctggggaggtcaaggctttagtgagctgtgatggtgccactgcactccagcctgggtgacagagtgagaccccatttaaaaaacaaaaacaaaaacaaaaaaaaatgtgacatatagttgactaagaagtacatttcaatacaggattgaaagaacccacatatgttaattaaacacaagcgcagaatttgtgccttttacataaaggaagaatgcacataggcatgctttcagacaagcaattcatctagcagaaaaggaaggaatacatttttcagcccttccaggaataaaatccataaatgggctctatttcgtcctccaacacttgtatttcccacgtcatttactcctgcacacccccactcactagaagcctgctaaactgttccagtgagatattttaacacctgatagggaataaatatgcttctgttttggccttcaaaaataagctctgggccagttgcagtggctcacgcctgtaatcccaacactttgggaggccgaggtgggcggatcacgaggtcaggagtttgggatcagcctggccaatatggtgaaactccatctctactaaaaatacaaaaattagccaggcatggtgcctgtaatcccagctacttgggaggctgaaggagaagaatcgcttgaacctgggaggcacaggttgcagtgagccgagatcacaccactgcactccaggccaggtgacagagcgacactctgtctcaaaaaaataaataaatcaactctgtagcatagcatttgtaattctattattttgccttacatttccattatccttttaataaaattgtttttttacatcttcctaatcaagaagtattatgaggccaggcacagtggctcatacctggaatcccagcactttgggaggccgaggcaggcagatcacctgaggtcaaggtatttgagaccagcctggccaacatggtgaaaccccatctctactaaaaatacagaaattagctgggtgtggtggtgcacacctgtaatgctagctactcgggaggctgaggtaggagaatcgcttgaacctgggaggcagaggttgcaataagcctagatcatgccactgcactcaagcctgggagacagagcgagactacatcttaaaaaaaaaaaaaaaagtattatgagagaggataatgtattgtaatgtattgtagaggctaaataaaattatgctcatgtcagaaaaaaagagtatttctcaaaataaaattcactgaaactggatgtttattttgactgagatatagtatatcctcaaattgccatagaaagtttacaagaatattagaggtaaattataaatatcagggcctttttaaaaaaaaaagattctgcttataacttggtatttgtttataataaaaattatagtagccaataatgaacacttactctggcttggttatttacttaggtcaaaagaaggaggagcggttaaactgtgggatcaggaactgaggcggtgccgtgccttcaggcttgagacaggacaagccacagattgtgttcgttctgtgtgcagaggcaaagtaagatgttccatgagctgatacagtgcagcagaaaacagaaagtggttattactgtgattccctcaccctttgcagcctaatgaacaatacttaataatgcataacgatggatttgcttgccaacattactctgtctttgctgctttctttgccaaagttagcaccagtgtggtgcataagctaggaagctattctgtctaaatactgtatgtaaacctccaatattttctagaatctgccaatttaacaactctagtagacataattgaaagcccttggcagttgactcatattaggacagctgtctccattttttaaaaaaacacacattccctagataaaacgtgcagtaaacaaacaatgaaatactactcagccataaaaaataatgaaattctgtcattcttggtggcaacatggatgagactggaggacatgatgtgaagtgaaataagccaggcacagaaagataaatacatgttctcactcctgtgcagaaactaaaaaagttgatcccacagaggtggagagtagaatagtggttactggaggcggacaagggggagggggagggggatagggaaggactggttaaaggatacaagtttacacagccagataggaatagtatgttttagtattctgtagtactgtaggatgactatagttaagaatcacgtatttatgtattttcaggtatttacaagagaggattttgaaagtttccatcacaaagaaatgataaatgtctgaggtgatggttatgcgtattaccctatgccctatagatatgtataattatgtgtcaatttcaaaataaaaattcaaaactacaactcctatgaaaatttttgagcgtgtttgtacttattaagtgtatttataaatcatacggatattatcttcagcctgcatattaaattgtagttaagcttttactttttaactaaaaaataaattctattattttttcctatatcccactgcactgaccccagtttggaaatcctaagattatcaaataaaaactttgattattgaagaatccaggtgtactgccacagaaaagttctattctgtagcatggactctaatatgtaatctagcccattgtgcttacagatagatgtgtgcctgtagtcatagaaaaatttgcatgagctaatgactgccttgctactagattagctcaaagcaaaaagttctctgaaagcaggtcaatagggtcatttttatattatgaagaagaaaagcagctgttgtattacattcactgtattggtcctgcttgtgtttcagggcaagatccttgttgggacaaggaatgctgaaataatcgaagttggagagaaaaatgcagcttgtaatattttagttaacggtcatgtggatgggccaatctggggactagcaacacatccttccagggattttttcctttctgctgcagaagatgggacagtgagactttgggatattgctgataaagtaagtacagataatttttttaaaagaggttacaacttctaaaaagaaaagttggaagttctaaattgctagtacttaaagaactgccagaattctgttgagcattttgaggggaaactggtataatttagaagtacttcacttaatgtttcctatgactctttttttttttttttttaaatgcagaagatgttaaacaaagtgaatttgggacatgctgctcgtactgtgtgttacagccctgaaggggacatggtggctattggaatgaaaaatggagaatttatcattttactagtgagttctctaaaaatatggggaaagaagagagacaggagatgtgcaatccatgatatcaggttagtgaacaaatggaatagagtttctagtatatacttgatttaacttccatttgtaaaattttccatagccttgccttcaaaaagaggtccccagggcctgtagcatttcccgtattataaattgtatgctaaaatatggctgtttgtatactacttaattcttcttgctaaattataaacccactgggcaccaactataatagcaagtactagtaggtaatgtttgatgaattcatgttaacacttagccatgtccattaagttcatcccaccaagaggtatctcccactgtaatacaagagagctatctgcccttcaaaagttgtcaccctggaaaactaaagttgtgatttcaaacatatcttctcttagtaacctcagtttgggaatatgtagttcattaatttaatcaatacctattgattaaatgttccagaatccaaattaatttaaatgtttcttaaacctttgtttttcagtgcttaagcatttttcaacagtggctaccatttacggagtacttccgtgtgatcagtagataagattattgaatctaggtctgtcaaaagcttgtacacttttcatcagtaaaatccttttacaaatgaaaccttcctcagaacttcaatatataaaatagtaacagtggcttcccttagcttttacatgtctctatcgtacctcagtaagactcatgggccatttcaagagactgaattgtcccatatgactccaaagattgctaggcaaatagcatttcactttgtcttttaaataagttcttcaggccgggcgcggtggctcatgcctgtaatcccagcactttgggaggccgaggcaggcagatcacctgaagtcaggagtactcgaccagcctggccaacatagtgaaaccccatctcaactaaaaatacaaaaatcagccgggcgtggtggcaggcgcctgtaatcccagctactcagggggctgaaacaggagaatcgcttgaacccgggaggcggaggttgcgccatcgcactccagcctgggagacaagagcgagacttcgtctcaaaaaaaaaaaattcttcttccaagattcaagttgtgtcatttcaccttaataactggaggttagttaagctgggctgtgttctttgcttaatattaagacaacgttttttccagatggaagaaaactatcttaatgaattgttagcttattaattatgtaatgctaatggcttttaaaagctgagatgttctgactgggtgttgtggctcacacctgtaatcccagtaccttgggaggccaagggggaaggattgcttgaggccaggagtttgggaccatagtgagaccccgcctctatttaaaaaattaaattttgttttgttttgttttgagttggagttttgctcttgttgcccatgctgaagtgcaatggtgcaatctcagctcaccacaacctgtgcctcctgggttcaagcgattctcctgcttcagcctcccgagtagatgggattacaggcgtgcaccaccatgcctggctaattttgtatttttagtagagacagggtttctctatgttggtcaggctggtctcaaactctcgacctcaggtgatctgcccgcctccgcttcccaaagttctgggattataggtgtgagccactgggcctggcctaagaaagtttttttaagccattagacgtttttaaaggaattgggagatgacaattggggaaatatttaaaatttaagtaaaatataaagcttccttatttcatgtaacccagacaatctcagtatacatgatcagttgtgtctgacaggtaaatctatttgaggccttatcacacgttacttttaagaactagaaaggaaaagtcactgatcttaagtatttataatacttcatgtggtctaatactttttacgttttgttttgattcagatttagtccggattcccggtatctggcagtaggttctagtgagaactcagtggatttttatgacctaacgctgggccccactcttaacagaatcagctactgcaaagacattccaagctttgtcattcaaatggacttctctgcagatagcagttatctccaggtacagtaccaatactgtatacccaggtggcaagttcttctgcttttacatttcgtgttagtgaatgcatttaaagttcctgagctccagagctccagcttctcaactcctccctttgtaccttctgacctacagctcccctttcctcccccacttatcagagcttttctcctattaagtttttgtagtgatcttttgcatacttaataatgttagacatgtaaatcaagtagcaatatgctagtattctgtaaaccccctgtggattttgtctctcacctaatggaattcttgtcccattttaatctgatgaaaaaggtctctagtggctgctataaacggcatgtctatgaagtgccttcaggaaaacatcttatggatcatgccgctattgacagaattacttgggctacatggactaggtaaatacttatatattcacaaggcaagaactgactttgaaggccagttagaaaatcctatttctgaactgttagagccattccaataaggaatagtaattgagtttcaagtttttgttaccatattttgaaatggtatgttcatgttgggacccctttttattgaatatatttccatgttttatcagtttccatgatttatcaagttttttttttaaggaaatcaaagttttaactttaaagataccctgatatttttcttaatgctaaatttaatgactggcaaaaaggtattgggtgctgttaagcaactgttattaattctctatctaaaggaatgctatcttgaatctattagaagtcaaagcttccaaatttgttcaaatttcctggctgtatgacaggtaaccatgactatccatttttttggccaatgaaaaatgccatcaaattcctgtatcagccaggcatatagtggctcatgcctgtaatctctgatgtagcaggccgaggtgggaggatcacttgagcctagaagttttgataccagcctgggcaacatagcaagaccccatctctgaaatttttttaattcctatgtcataagtcatttttatttttgtagagatagggatctcacaatattgcccaggctggtctcaaactcttggcctcaagcagtcctcctgcctcagcctcccaaaatgttgggattactggtatgtgctgctggacccagccaagtagcacttttaatttgaaaaatagttctatcagttttcagtcaggcgcggtggctcagcctgtaatcccagcactttgggaggccgagcgggggtgatcacctgaggtcgggagttcgagactagcctgaccaacatggagaaaccctgtctctactaaaaatacaaaataagccgggcatgttagcgcatgcctgtgatcccagctactcgggaggctgaggcaggagaattgcttgaacccaggaggcagaggttgcggtgagccgagatcatgccattgcactccagcctgggtaacaagagcgaaaactccgtctcaaaaaaaaaaaaagaaaaaatagttctatcagttttcataaagtactactttaatcttaaaaagattaatctagaaacccttcaaattataaaatgtcatttttaaaaggcaggagttgatatcctgatgaaattcaggtctccaaacaacttaccataatttacttcctgtattttaagtaacatgatagggtacttagagattaattgccaagaaactttttgaatatagtcaacctgcccgcacttgccatgatgagttttcttttgttccttccctctagtattctaggagatgaggttttgggaatctggtccagacatgctgagaaagctgatgtcaactgtgcctgtgtatctcattcaggaatcagtcttgttacaggagatgactttggcatggttaagttatttgacttcccatgtccagaaaaatttgtaagtttgtgttttgtttactattatcagtttactcctaattttgatgtcttatcatcagcacttttccccatatatttaaaatgttttgtcctaatttctaaatttttccccaaactttctaaatctatttactttgaaataaaagctattagaaacaaatcctctccctcgagtaataccatctttggaaccatcctacaaaagctgtaattagcttttcaccaaacctataatcagttatcaaatttcaaatgcttttccttagagaaaaatggtcagagtacctggagacatctgactgcccacacagcctggttttgcagatccactactcatgctgaaaagcattctaatcactggctgcggtgctaactccctactctctccacagctcttgtcatagagattatagttcctaataagagcctttgacttctgtgtgcaccaaatgccctgagcttgtctgtcattgttttttaggcaaaacacaaaaggttcttgggtcattcgccccatgtgacaaatattcgatttaccagtggtgatcgacatgttgttagtgctggaggtgatgactgcaggttagtaactttctcagcccatgaagagcagactatgttactagttaagagacttaatacaacaactcctacagctttggtttatgaaatcagctagtcaacattagtagaaggtagtataaccagatggctcttcagaatctcatatttatgcaaatacagaataaaaggagttaaagaggaaaaatattacacatgtaacctgaaagcacaactgaaaaatattaaactgttatgaaaatctaaaaacataattaactccctgcaattttcttctctgattgcagcttatttgtctggaaatgtgtacatacacctcactgagagatgctgagatgactacagaaattaactttgagaccagaattacagagaagaaaaaccaaaacccaaccctgcatggtcaagtggtgctaacccaagactgtaacagggagaaatgcccagaatcatcaaaatagtgaaagactgatctgttcaaaatatttgctatatgcactgggtataatccgtaatccatacactgccagataatgccatttcaaggaaggatcgaatacttgatggtaaaggccaagtccccctgtattgggaagtgtgtgatttcggcagacctgctgggaaaatttagggtagagcactctttacagaagaactcaaaaacccaatttggataattttcattatctttttagcaaaatggtttcttaatgtttatattttattttcaaggttcattgtttaatgaaatattttattcttgcatttccataaggaaagggaaagtcatgatcatcctaaaggatcacagtttttaaaaggcaaacattttccctaaggaaacagacacaagctttcctagagaatatgatgttttttaggcattaataaggtccttttttataaaggacacttttctcctagtagttttgaattcaggaacagatccaaagttagcagtatatggctgctacatttccattttcattttcgagccatcagtttatgttcagatgccatctctgtaatcgcacatttaaaacataactgtagcctcactaatggaaaagtagtatgatgaacaatcattcccaatggtgtacaatgtaagggttttagggagcaacagtatttaactggaagaaagaattgcatatttaatgtagtctaatatatacacatttgtttaacatgtaaacaaaagtgttaaattcacatatacaacattatacaatttaatcactcttggaataaaatttttatagccttttttctattgggaaaatttgtttagatgtgtgccactccataggtttatttccaaaatgaatgagcccaactccatttgtaaaaacttgtcagttagaattcctttttttagtggattagggctgaattcttagatccttatttcttttcactttaaatgctgccaaagatcactactcatcattcaggaattcgctgtctagcctatctgtagtttcctgaagattgaaaattatgtagactgctatttaaaaatatatttttctaagtgtgaggtttaagatgctgtattgaccctatgagtttttaatgtgttaattatctttatagcataatagatcgctttaggttcctggaatcccatttggtctgacaggatatatgaagattcttaatacctattttctgtgtctaatacttggttaatactaaaaatagaaatgactaaattacatcacagaaagcataaccagtgattgaacctggtagttttaaagctctaaatagctgtggctgaaggactgattatggggctaagaagcttgaaacgtaagttggtacttgttcatcagtggattctcctaaattaagccaaattttgaaatacatgactattaagtttctactcatgtatttacagtcagtcaataaattaaaggaggaaaaaaatccctgaacaacctgcccataaaaagaaaaatactctacatttgagcctgctgcagttttaaattttccctctgggtcaagtttgccagcttttggctacagagaaattatatttccattacagtgcaggtagaaactctgtaaccttaagcatgtaaactacatagaataaaactgtttccactgcatttctgtccttcaaagtggccaacctgattaagtcagccttaatcactgctgctgtcagtttcacgactaaaggtcatattgactaagtagtcatcagctgaccacctcgctgtatcagccagcaacgaggggaaggtgaagaaacatgataggccatatagaatctgccctatgtttacttttttaacccagataattatttttgtgtgcagtatctaagctcctgattgtgtaacctgggacttctggcaccttttgttccattcattttatgtataaaatgcatgccaaagcacactgtgccctctggtacccttgcttccaatcgccaaccatgctcatttccttcctttttttgtggtccctttttgtggtgatcattttaaaccacgtcatccaacaaatgttttatggtcaaccttagcttgttcataagccatagcaactgaaagattaaactcttaaatatgtgtctgggcagtggctattaaatagcaaaaaacaatcagattttagtattttattatttccttgtaaaatggctgaactaaattaaacccttgtttcccatttgttctataatttatagtgaaactgagaacaaaactatctttataaatgatagctaaaagtatttccagatatttaaacaatttaaaataaatttcttctgcagagatgcaaagcatctcaacactggaatgaacaaatgccttaaattcaatggagtaaacctttagaatgaagaggaactgtcatttcacccaagccgaagacaacagccttatgcacttgtgtgctctgtctttgctgcttctcgtgtttcaagcctttcctgtgggatcagcacagcaaagtgcaacttaccaaatggtttaatgactggttaattctttcttctcccaatggaaaagcaatggcaacacaacagtagactgctggcttgacaatcttaaacgtgagcctttgcacatgtaggtttatcatcatttgagtatacgactaagcaagtcaatgaactttttttttttttttagcagtttaatttggtcctgagaatgttgcagtctttattaccccttttgcattaatccacttttctaaccaccttttaagctttaatttttaacactatacaccaagtctttgaaatcagtgatctgttatttaactctaaagcatttgacacttcttgccttaacagttttaaaaaccacacacaaaaaaactctgtaagtaatacagtaggccaaaagtttcatcctatctatcttgcagtttacctatctgatctgatctctgtaattatagttctgtcatttaaaatatactatttaaatctaatttttacatttcaaaaattatcttcagtagtaactaagtatattttctgtggattctgagaatgttatttttcagaatgtgagaatatatatgtacatttataatcttgtgactttaaagtctgttttcagatacagtatgtaaatacttgtaaaaaaatttgtataattttgtgataatgtagtttcccaaaaaaattatttagaaggcattatgttattagtaaatgagagcactgtatagaactgttcctattttctgcacttgccattccagctgcctccactgtccatacccacctcattcatcctgtcacagaaggcaggaaaactgggaactttaccaaagtagcactcagcctgagaggcctgtataatcatgcttttcaaactaaattcacttaaaaattaaaaagcagaattgaatattttaagcagcctcagtacctttggccaatgctgttttcatggtggattatgaacattatataatctttgggaaaagtgaaagtagtacaatttttagaataatgacaactgcctcactgcatctctccactcacacagcaaccgtgtagccccctaagctgcagtaccatgactaaccatgatgtcaatttcatatgctgatcctcacaacagcagtgcacaaacatgccccaaatattttaacagaatttagctcttccttaagctgtcttttcatagtaaaaacaaaacaaaaacacccaatgttaaaaccacataataaacttacaaacttgaaaaattagacacttcagatagataggcaataaaacttcatattatgaaagcaatatattccaagtttcaaagatttgacaagttctgtagagtatctttcatcagtacatgaaaacttccaaactgcatgatcttctgccaggcaggactgggtgctattcgctggtttgaggtcgaatccatttcaaggcatgtcgtggtgggacattaatggtgggatggtagaatgtgcagtccggtcttgtacattgagtgttaaacctacaatgttttggatgatagaagggacattccatcttcttacaagcagggaagtaacggcagagctgactactggaaggtggtgctggtggtgcaactggttttggagacagtactggaattcttctactcacatgagtgaagggacaatctggtttagtacactttgcatcatatttacaatttgggtgaacaaacaaacatttttcagcaaatttacaattggggaaggctttgcagggtgagatggggtgatggtaggcacactcatccccatttttacaagcaggccagtacttgcagcgctccaaaagtttttctggtttctgtgccacactcagttcactcatctcagcatttgggtcctcaagctgcctgctcagcaagtgcaactgctgtgggtggaggagacctctgagtcccttgtttgaggctgcagtttggtttacgggtttcattccttcaaagcacatgtcctcctcttgatctgacatgtatcctggggggctggggacaccatccagcgtcactataaacttgggacttgcaggtttatctggttgtacaagatctcgtgtctgcataaggtgtcctgaaagtacccgaagggaatctgcagtcttcatccccgactcttggtttggtgccactactacttcctcagacagctttggcttcttcagaataaatgatcttgtgtctgcatggaccatggattccatgtcatagtaatcttgactcatctgcagagtttctgccattactgggtcgatttgcagtcgggataataattgcctctgttgagttccttgatttttttctacagaatctccttttgtttcctcttctttaatggggggacttattctgggggtcctactttgtccctggaccacttctgctagcaattcttcttgagaagttcgagttctgggagcaactggaagtgtctgtttctgtggaactgtagagtagttagttgtttttgttacggattcttgagcttcagatatagccttcaaaatcagattcttgttagcttgtttagaaggtggaagagaaggtctcctttcaggctttgcaggcacagacacactgctggagatgcttcctgttcgagacccgtaatcatcatcttcttcctcctcttctccatcatgattgaatttttttactttaacaactgaacttaccacaggcaactttctcttccgaaagttttcatcctccatactcattttctccgagttgtttctaaagaacggactatacgtttcttctaagctgttaagcacctctggttcacacaaacgtcctgtttcatatacccaactactctgcatatcaagctgcttggcagcatgaatactattctgctgctgttgaaattgcaacctgtttaaatgaacaccactatctgcatttctacttgcaggtggtcgataaatttcaatagaagggcgagaagaaccatatgtaagtgtcactgtaggttttttctgagataagggattctcctgcacaaagttgaggtcttcgtcaatgagatcatctggttctggcttaatatcaatcacatcttcagagggtgctggctccctcaaaggtttcactgttgacattagtcgggttgcagctccatcatcgtaagtctgtctgacatttgtggtttttgactcctgcgaacttgtagaaactctggaatctcttttttcaggtctcgcgctaggaatggcaagtggtggcactgcagcttcatgcctcctctcatctccccgactgaaattgctcttgtttgaaggcacgttactatcaaagatgttggtatcagaagacttcagactagagggttcagttgtaacagagcgaagtttatctaatacaccatgaagccatacggtgaatcgaattgtgttgttccctagaaacagggacagatcctctgtcatttggtcctgacttttcttgttggccaccatcaccataatgtaatcaggaagttcttcatcaacataagctcctaattcttgtaatttccccttaatggcactccggatcttgcggctgatctcggtgccgatctccatggctctgcggcgtgcgggaactcagcactgcgcggcgcttggcttacccggaggctgccgcggactcctaccccgcagccgggacaccaccgcctcc

SEQ ID NO: 13621 - RNA, 16838 nt, Homo sapiens
  source 1..16838: mol_type = other RNA
gctgggattacaggcatgagccaccataataaggattctgatgaacatttgattccttggactactgttatactcaaaagccttccttaatcttctaattgtcaccctaaatatcctaaaatttctgtcttcctagtagttcttcatagtcctaaaaatttgtcagagagaaaggtaaatcaagaaacatgattttcaaatgatttaaggtggtactagggtttaggatttcctttgctttttatcatttaacacactgcttatcatacagctggaagtgctctgggccagtgtctctacttcgagggaagaaggaggtagtgagacagaaggaaatagcacaattcctggccctgacagaagggtgttcaggagacctgctctcctctcactttattccatctcatctggacctgtggcttccaatccacatctctttcctttaatatcctgcattggctaggctgtataaatcctttggtgcatcgaaaaactaagtgcattttttgtttttgtgattatgcaatacttataggaaaagttataattttagaatatttaagtacacttacatttttgagaaaaagactattgaaatgtttgtgccatgtcaaatttcagttgaacattttgggtattcttaatataagaccaggccaggcaccgtggctcaggccgggcacagtggctcacacctataatcccagcacttagggaggccaaggcgggaagatcacctgaagtcaggagttcaagaccagcctggctaacaaggtgaaactctgtctctactaaaaatacaaaaattagccgggcgtggtggctggcgcttgtaatcccagctacttgggaggctgagacaggagaatcacttgaacctgggaagcagaggttgtggtgagctgagatcgcaccattgcactccagcctgggcaacaaagagcgaaactccgtctcaaaaaaataaaaaataaaccctagaattatagtatgttagaattggaagggaagaattgtctaaggttattctagctaataagcaacagacttggaaaggaaaaggtcctgacaaagctaagcctcccgttcaggtttcctgactcgtgaattcagtgctgctgccactacacgatgcatgctctttgtatcaagggtgagacagcattacacatacatagaaaattatctatttaaactctatttgaacttttgatgagtttgtctccccctcccccactccttttcagaataacttgacgtttacaggtaccatcagtggtgatgtctgtgtgtggaaagatcacatattgtgtagaatcgtggcgagagctcacaacgggcctgtgtttgccatgtacaccaccctgcgagatggacttatcgtgactgggggaaaggaaaggccgtgagtcctctttcttttcacagaatatttatgcatttgtgacctacctgaggtttgcagttaattattctagttgtttctaggctacacagagtgtcctctccgaccttcctcctcatatgcttctcctttattaccttttatgtgccttctatttgattctcatttctggtcttaattcacttccaatttttttcatgttggggtgatactttttctgaggtgtggataggtagttgtcctacaagttgagttacttttcttaatgtctgtatgcctgtgtatgatttgctgagtaggaggcccatgggggaatctggagccagggttgtattttgactgcctgctctctttttgttcagaatggattctaaggagtagaatgcacattgttgctttagaaaaggatgagggaactagagagaactgccttgtttccttttgcttgaggcaaatttaaactgttttatacaagacctcaaaatttgagaagaggtctcttctgagtgattttcaaatctcccaacagtaaccagatacttatgatttgatttgtcaccaacatagtcatatgcatgttgaaacatgacatgtaggccaggcacagtggctcacacctgtaatcttatcactttgggaggctgaggcaggtggatcgcttgagcccaggagttcaagaccagcctgggcaacatggtgaaaccccatcgctataaaaaacaacaattagccgggtgtggtggcacatgcctgtagtccctgctactcaggaggctgaggtgggaggatcacttgagcctggggaggtcaaggctttagtgagctgtgatggtgccactgcactccagcctgggtgacagagtgagaccccatttaaaaaacaaaaacaaaaacaaaaaaaaatgtgacatatagttgactaagaagtacatttcaatacaggattgaaagaacccacatatgttaattaaacacaagcgcagaatttgtgccttttacataaaggaagaatgcacataggcatgctttcagacaagcaattcatctagcagaaaaggaaggaatacatttttcagcccttccaggaataaaatccataaatgggctctatttcgtcctccaacacttgtatttcccacgtcatttactcctgcacacccccactcactagaagcctgctaaactgttccagtgagatattttaacacctgatagggaataaatatgcttctgttttggccttcaaaaataagctctgggccagttgcagtggctcacgcctgtaatcccaacactttgggaggccgaggtgggcggatcacgaggtcaggagtttgggatcagcctggccaatatggtgaaactccatctctactaaaaatacaaaaattagccaggcatggtgcctgtaatcccagctacttgggaggctgaaggagaagaatcgcttgaacctgggaggcacaggttgcagtgagccgagatcacaccactgcactccaggccaggtgacagagcgacactctgtctcaaaaaaataaataaatcaactctgtagcatagcatttgtaattctattattttgccttacatttccattatccttttaataaaattgtttttttacatcttcctaatcaagaagtattatgaggccaggcacagtggctcatacctggaatcccagcactttgggaggccgaggcaggcagatcacctgaggtcaaggtatttgagaccagcctggccaacatggtgaaaccccatctctactaaaaatacagaaattagctgggtgtggtggtgcacacctgtaatgctagctactcgggaggctgaggtaggagaatcgcttgaacctgggaggcagaggttgcaataagcctagatcatgccactgcactcaagcctgggagacagagcgagactacatcttaaaaaaaaaaaaaaaagtattatgagagaggataatgtattgtaatgtattgtagaggctaaataaaattatgctcatgtcagaaaaaaagagtatttctcaaaataaaattcactgaaactggatgtttattttgactgagatatagtatatcctcaaattgccatagaaagtttacaagaatattagaggtaaattataaatatcagggcctttttaaaaaaaaaagattctgcttataacttggtatttgtttataataaaaattatagtagccaataatgaacacttactctggcttggttatttacttaggtcaaaagaaggaggagcggttaaactgtgggatcaggaactgaggcggtgccgtgccttcaggcttgagacaggacaagccacagattgtgttcgttctgtgtgcagaggcaaagtaagatgttccatgagctgatacagtgcagcagaaaacagaaagtggttattactgtgattccctcaccctttgcagcctaatgaacaatacttaataatgcataacgatggatttgcttgccaacattactctgtctttgctgctttctttgccaaagttagcaccagtgtggtgcataagctaggaagctattctgtctaaatactgtatgtaaacctccaatattttctagaatctgccaatttaacaactctagtagacataattgaaagcccttggcagttgactcatattaggacagctgtctccattttttaaaaaaacacacattccctagataaaacgtgcagtaaacaaacaatgaaatactactcagccataaaaaataatgaaattctgtcattcttggtggcaacatggatgagactggaggacatgatgtgaagtgaaataagccaggcacagaaagataaatacatgttctcactcctgtgcagaaactaaaaaagttgatcccacagaggtggagagtagaatagtggttactggaggcggacaagggggagggggagggggatagggaaggactggttaaaggatacaagtttacacagccagataggaatagtatgttttagtattctgtagtactgtaggatgactatagttaagaatcacgtatttatgtattttcaggtatttacaagagaggattttgaaagtttccatcacaaagaaatgataaatgtctgaggtgatggttatgcgtattaccctatgccctatagatatgtataattatgtgtcaatttcaaaataaaaattcaaaactacaactcctatgaaaatttttgagcgtgtttgtacttattaagtgtatttataaatcatacggatattatcttcagcctgcatattaaattgtagttaagcttttactttttaactaaaaaataaattctattattttttcctatatcccactgcactgaccccagtttggaaatcctaagattatcaaataaaaactttgattattgaagaatccaggtgtactgccacagaaaagttctattctgtagcatggactctaatatgtaatctagcccattgtgcttacagatagatgtgtgcctgtagtcatagaaaaatttgcatgagctaatgactgccttgctactagattagctcaaagcaaaaagttctctgaaagcaggtcaatagggtcatttttatattatgaagaagaaaagcagctgttgtattacattcactgtattggtcctgcttgtgtttcagggcaagatccttgttgggacaaggaatgctgaaataatcgaagttggagagaaaaatgcagcttgtaatattttagttaacggtcatgtggatgggccaatctggggactagcaacacatccttccagggattttttcctttctgctgcagaagatgggacagtgagactttgggatattgctgataaagtaagtacagataatttttttaaaagaggttacaacttctaaaaagaaaagttggaagttctaaattgctagtacttaaagaactgccagaattctgttgagcattttgaggggaaactggtataatttagaagtacttcacttaatgtttcctatgactctttttttttttttttttaaatgcagaagatgttaaacaaagtgaatttgggacatgctgctcgtactgtgtgttacagccctgaaggggacatggtggctattggaatgaaaaatggagaatttatcattttactagtgagttctctaaaaatatggggaaagaagagagacaggagatgtgcaatccatgatatcaggttagtgaacaaatggaatagagtttctagtatatacttgatttaacttccatttgtaaaattttccatagccttgccttcaaaaagaggtccccagggcctgtagcatttcccgtattataaattgtatgctaaaatatggctgtttgtatactacttaattcttcttgctaaattataaacccactgggcaccaactataatagcaagtactagtaggtaatgtttgatgaattcatgttaacacttagccatgtccattaagttcatcccaccaagaggtatctcccactgtaatacaagagagctatctgcccttcaaaagttgtcaccctggaaaactaaagttgtgatttcaaacatatcttctcttagtaacctcagtttgggaatatgtagttcattaatttaatcaatacctattgattaaatgttccagaatccaaattaatttaaatgtttcttaaacctttgtttttcagtgcttaagcatttttcaacagtggctaccatttacggagtacttccgtgtgatcagtagataagattattgaatctaggtctgtcaaaagcttgtacacttttcatcagtaaaatccttttacaaatgaaaccttcctcagaacttcaatatataaaatagtaacagtggcttcccttagcttttacatgtctctatcgtacctcagtaagactcatgggccatttcaagagactgaattgtcccatatgactccaaagattgctaggcaaatagcatttcactttgtcttttaaataagttcttcaggccgggcgcggtggctcatgcctgtaatcccagcactttgggaggccgaggcaggcagatcacctgaagtcaggagtactcgaccagcctggccaacatagtgaaaccccatctcaactaaaaatacaaaaatcagccgggcgtggtggcaggcgcctgtaatcccagctactcagggggctgaaacaggagaatcgcttgaacccgggaggcggaggttgcgccatcgcactccagcctgggagacaagagcgagacttcgtctcaaaaaaaaaaaattcttcttccaagattcaagttgtgtcatttcaccttaataactggaggttagttaagctgggctgtgttctttgcttaatattaagacaacgttttttccagatggaagaaaactatcttaatgaattgttagcttattaattatgtaatgctaatggcttttaaaagctgagatgttctgactgggtgttgtggctcacacctgtaatcccagtaccttgggaggccaagggggaaggattgcttgaggccaggagtttgggaccatagtgagaccccgcctctatttaaaaaattaaattttgttttgttttgttttgagttggagttttgctcttgttgcccatgctgaagtgcaatggtgcaatctcagctcaccacaacctgtgcctcctgggttcaagcgattctcctgcttcagcctcccgagtagatgggattacaggcgtgcaccaccatgcctggctaattttgtatttttagtagagacagggtttctctatgttggtcaggctggtctcaaactctcgacctcaggtgatctgcccgcctccgcttcccaaagttctgggattataggtgtgagccactgggcctggcctaagaaagtttttttaagccattagacgtttttaaaggaattgggagatgacaattggggaaatatttaaaatttaagtaaaatataaagcttccttatttcatgtaacccagacaatctcagtatacatgatcagttgtgtctgacaggtaaatctatttgaggccttatcacacgttacttttaagaactagaaaggaaaagtcactgatcttaagtatttataatacttcatgtggtctaatactttttacgttttgttttgattcagatttagtccggattcccggtatctggcagtaggttctagtgagaactcagtggatttttatgacctaacgctgggccccactcttaacagaatcagctactgcaaagacattccaagctttgtcattcaaatggacttctctgcagatagcagttatctccaggtacagtaccaatactgtatacccaggtggcaagttcttctgcttttacatttcgtgttagtgaatgcatttaaagttcctgagctccagagctccagcttctcaactcctccctttgtaccttctgacctacagctcccctttcctcccccacttatcagagcttttctcctattaagtttttgtagtgatcttttgcatacttaataatgttagacatgtaaatcaagtagcaatatgctagtattctgtaaaccccctgtggattttgtctctcacctaatggaattcttgtcccattttaatctgatgaaaaaggtctctagtggctgctataaacggcatgtctatgaagtgccttcaggaaaacatcttatggatcatgccgctattgacagaattacttgggctacatggactaggtaaatacttatatattcacaaggcaagaactgactttgaaggccagttagaaaatcctatttctgaactgttagagccattccaataaggaatagtaattgagtttcaagtttttgttaccatattttgaaatggtatgttcatgttgggacccctttttattgaatatatttccatgttttatcagtttccatgatttatcaagttttttttttaaggaaatcaaagttttaactttaaagataccctgatatttttcttaatgctaaatttaatgactggcaaaaaggtattgggtgctgttaagcaactgttattaattctctatctaaaggaatgctatcttgaatctattagaagtcaaagcttccaaatttgttcaaatttcctggctgtatgacaggtaaccatgactatccatttttttggccaatgaaaaatgccatcaaattcctgtatcagccaggcatatagtggctcatgcctgtaatctctgatgtagcaggccgaggtgggaggatcacttgagcctagaagttttgataccagcctgggcaacatagcaagaccccatctctgaaatttttttaattcctatgtcataagtcatttttatttttgtagagatagggatctcacaatattgcccaggctggtctcaaactcttggcctcaagcagtcctcctgcctcagcctcccaaaatgttgggattactggtatgtgctgctggacccagccaagtagcacttttaatttgaaaaatagttctatcagttttcagtcaggcgcggtggctcagcctgtaatcccagcactttgggaggccgagcgggggtgatcacctgaggtcgggagttcgagactagcctgaccaacatggagaaaccctgtctctactaaaaatacaaaataagccgggcatgttagcgcatgcctgtgatcccagctactcgggaggctgaggcaggagaattgcttgaacccaggaggcagaggttgcggtgagccgagatcatgccattgcactccagcctgggtaacaagagcgaaaactccgtctcaaaaaaaaaaaaagaaaaaatagttctatcagttttcataaagtactactttaatcttaaaaagattaatctagaaacccttcaaattataaaatgtcatttttaaaaggcaggagttgatatcctgatgaaattcaggtctccaaacaacttaccataatttacttcctgtattttaagtaacatgatagggtacttagagattaattgccaagaaactttttgaatatagtcaacctgcccgcacttgccatgatgagttttcttttgttccttccctctagtattctaggagatgaggttttgggaatctggtccagacatgctgagaaagctgatgtcaactgtgcctgtgtatctcattcaggaatcagtcttgttacaggagatgactttggcatggttaagttatttgacttcccatgtccagaaaaatttgtaagtttgtgttttgtttactattatcagtttactcctaattttgatgtcttatcatcagcacttttccccatatatttaaaatgttttgtcctaatttctaaatttttccccaaactttctaaatctatttactttgaaataaaagctattagaaacaaatcctctccctcgagtaataccatctttggaaccatcctacaaaagctgtaattagcttttcaccaaacctataatcagttatcaaatttcaaatgcttttccttagagaaaaatggtcagagtacctggagacatctgactgcccacacagcctggttttgcagatccactactcatgctgaaaagcattctaatcactggctgcggtgctaactccctactctctccacagctcttgtcatagagattatagttcctaataagagcctttgacttctgtgtgcaccaaatgccctgagcttgtctgtcattgttttttaggcaaaacacaaaaggttcttgggtcattcgccccatgtgacaaatattcgatttaccagtggtgatcgacatgttgttagtgctggaggtgatgactgcaggttagtaactttctcagcccatgaagagcagactatgttactagttaagagacttaatacaacaactcctacagctttggtttatgaaatcagctagtcaacattagtagaaggtagtataaccagatggctcttcagaatctcatatttatgcaaatacagaataaaaggagttaaagaggaaaaatattacacatgtaacctgaaagcacaactgaaaaatattaaactgttatgaaaatctaaaaacataattaactccctgcaattttcttctctgattgcagcttatttgtctggaaatgtgtacatacacctcactgagagatgctgagatgactacagaaattaactttgagaccagaattacagagaagaaaaaccaaaacccaaccctgcatggtcaagtggtgctaacccaagactgtaacagggagaaatgcccagaatcatcaaaatagtgaaagactgatctgttcaaaatatttgctatatgcactgggtataatccgtaatccatacactgccagataatgccatttcaaggaaggatcgaatacttgatggtaaaggccaagtccccctgtattgggaagtgtgtgatttcggcagacctgctgggaaaatttagggtagagcactctttacagaagaactcaaaaacccaatttggataattttcattatctttttagcaaaatggtttcttaatgtttatattttattttcaaggttcattgtttaatgaaatattttattcttgcatttccataaggaaagggaaagtcatgatcatcctaaaggatcacagtttttaaaaggcaaacattttccctaaggaaacagacacaagctttcctagagaatatgatgttttttaggcattaataaggtccttttttataaaggacacttttctcctagtagttttgaattcaggaacagatccaaagttagcagtatatggctgctacatttccattttcattttcgagccatcagtttatgttcagatgccatctctgtaatcgcacatttaaaacataactgtagcctcactaatggaaaagtagtatgatgaacaatcattcccaatggtgtacaatgtaagggttttagggagcaacagtatttaactggaagaaagaattgcatatttaatgtagtctaatatatacacatttgtttaacatgtaaacaaaagtgttaaattcacatatacaacattatacaatttaatcactcttggaataaaatttttatagccttttttctattgggaaaatttgtttagatgtgtgccactccataggtttatttccaaaatgaatgagcccaactccatttgtaaaaacttgtcagttagaattcctttttttagtggattagggctgaattcttagatccttatttcttttcactttaaatgctgccaaagatcactactcatcattcaggaattcgctgtctagcctatctgtagtttcctgaagattgaaaattatgtagactgctatttaaaaatatatttttctaagtgtgaggtttaagatgctgtattgaccctatgagtttttaatgtgttaattatctttatagcataatagatcgctttaggttcctggaatcccatttggtctgacaggatatatgaagattcttaatacctattttctgtgtctaatacttggttaatactaaaaatagaaatgactaaattacatcacagaaagcataaccagtgattgaacctggtagttttaaagctctaaatagctgtggctgaaggactgattatggggctaagaagcttgaaacgtaagttggtacttgttcatcagtggattctcctaaattaagccaaattttgaaatacatgactattaagtttctactcatgtatttacagtcagtcaataaattaaaggaggaaaaaaatccctgaacaacctgcccataaaaagaaaaatactctacatttgagcctgctgcagttttaaattttccctctgggtcaagtttgccagcttttggctacagagaaattatatttccattacagtgcaggtagaaactctgtaaccttaagcatgtaaactacatagaataaaactgtttccactgcatttctgtccttcaaagtggccaacctgattaagtcagccttaatcactgctgctgtcagtttcacgactaaaggtcatattgactaagtagtcatcagctgaccacctcgctgtatcagccagcaacgaggggaaggtgaagaaacatgataggccatatagaatctgccctatgtttacttttttaacccagataattatttttgtgtgcagtatctaagctcctgattgtgtaacctgggacttctggcaccttttgttccattcattttatgtataaaatgcatgccaaagcacactgtgccctctggtacccttgcttccaatcgccaaccatgctcatttccttcctttttttgtggtccctttttgtggtgatcattttaaaccacgtcatccaacaaatgttttatggtcaaccttagcttgttcataagccatagcaactgaaagattaaactcttaaatatgtgtctgggcagtggctattaaatagcaaaaaacaatcagattttagtattttattatttccttgtaaaatggctgaactaaattaaacccttgtttcccatttgttctataatttatagtgaaactgagaacaaaactatctttataaatgatagctaaaagtatttccagatatttaaacaatttaaaataaatttcttctgcagagatgcaaagcatctcaacactggaatgaacaaatgccttaaattcaatggagtaaacctttagaatgaagaggaactgtcatttcacccaagccgaagacaacagccttatgcacttgtgtgctctgtctttgctgcttctcgtgtttcaagcctttcctgtgggatcagcacagcaaagtgcaacttaccaaatggtttaatgactggttaattctttcttctcccaatggaaaagcaatggcaacacaacagtagactgctggcttgacaatcttaaacgtgagcctttgcacatgtaggtttatcatcatttgagtatacgactaagcaagtcaatgaactttttttttttttttagcagtttaatttggtcctgagaatgttgcagtctttattaccccttttgcattaatccacttttctaaccaccttttaagctttaatttttaacactatacaccaagtctttgaaatcagtgatctgttatttaactctaaagcatttgacacttcttgccttaacagttttaaaaaccacacacaaaaaaactctgtaagtaatacagtaggccaaaagtttcatcctatctatcttgcagtttacctatctgatctgatctctgtaattatagttctgtcatttaaaatatactatttaaatctaatttttacatttcaaaaattatcttcagtagtaactaagtatattttctgtggattctgagaatgttatttttcagaatgtgagaatatatatgtacatttataatcttgtgactttaaagtctgttttcagatacagtatgtaaatacttgtaaaaaaatttgtataattttgtgataatgtagtttcccaaaaaaattatttagaaggcattatgttattagtaaatgagagcactgtatagaactgttcctattttctgcacttgccattccagctgcctccactgtccatacccacctcattcatcctgtcacagaaggcaggaaaactgggaactttaccaaagtagcactcagcctgagaggcctgtataatcatgcttttcaaactaaattcacttaaaaattaaaaagcagaattgaatattttaagcagcctcagtacctttggccaatgctgttttcatggtggattatgaacattatataatctttgggaaaagtgaaagtagtacaatttttagaataatgacaactgcctcactgcatctctccactcacacagcaaccgtgtagccccctaagctgcagtaccatgactaaccatgatgtcaatttcatatgctgatcctcacaacagcagtgcacaaacatgccccaaatattttaacagaatttagctcttccttaagctgtcttttcatagtaaaaacaaaacaaaaacacccaatgttaaaaccacataataaacttacaaacttgaaaaattagacacttcagatagataggcaataaaacttcatattatgaaagcaatatattccaagtttcaaagatttgacaagttctgtagagtatctttcatcagtacatgaaaacttccaaactgcatgatcttctgccaggcaggactgggtgctattcgctggtttgaggtcgaatccatttcaaggcatgtcgtggtgggacattaatggtgggatggtagaatgtgcagtccggtcttgtacattgagtgttaaacctacaatgttttggatgatagaagggacattccatcttcttacaagcagggaagtaacggcagagctgactactggaaggtggtgctggtggtgcaactggttttggagacagtactggaattcttctactcacatgagtgaagggacaatctggtttagtacactttgcatcatatttacaatttgggtgaacaaacaaacatttttcagcaaatttacaattggggaaggctttgcagggtgagatggggtgatggtaggcacactcatccccatttttacaagcaggccagtacttgcagcgctccaaaagtttttctggtttctgtgccacactcagttcactcatctcagcatttgggtcctcaagctgcctgctcagcaagtgcaactgctgtgggtggaggagacctctgagtcccttgtttgaggctgcagtttggtttacgggtttcattccttcaaagcacatgtcctcctcttgatctgacatgtatcctggggggctggggacaccatccagcgtcactataaacttgggacttgcaggtttatctggttgtacaagatctcgtgtctgcataaggtgtcctgaaagtacccgaagggaatctgcagtcttcatccccgactcttggtttggtgccactactacttcctcagacagctttggcttcttcagaataaatgatcttgtgtctgcatggaccatggattccatgtcatagtaatcttgatttttttctacagaatctccttttgtttcctcttctttaatggggggacttattctgggggtcctactttgtccctggaccacttctgctagcaattcttcttgagaagttcgagttctgggagcaactggaagtgtctgtttctgtggaactgtagagtagttagttgtttttgttacggattcttgagcttcagatatagccttcaaaatcagattcttgttagcttgtttagaaggtggaagagaaggtctcctttcaggctttgcaggcacagacacactgctggagatgcttcctgttcgagacccgtaatcatcatcttcttcctcctcttctccatcatgattgaatttttttactttaacaactgaacttaccacaggcaactttctcttccgaaagttttcatcctccatactcattttctccgagttgtttctaaagaacggactatacgtttcttctaagctgttaagcacctctggttcacacaaacgtcctgtttcatatacccaactactctgcatatcaagctgcttggcagcatgaatactattctgctgctgttgaaattgcaacctgtttaaatgaacaccactatctgcatttctacttgcaggtggtcgataaatttcaatagaagggcgagaagaaccatatgtaagtgtcactgtaggttttttctgagataagggattctcctgcacaaagttgaggtcttcgtcaatgagatcatctggttctggcttaatatcaatcacatcttcagagggtgctggctccctcaaaggtttcactgttgacattagtcgggttgcagctccatcatcgtaagtctgtctgacatttgtggtttttgactcctgcgaacttgtagaaactctggaatctcttttttcaggtctcgcgctaggaatggcaagtggtggcactgcagcttcatgcctcctctcatctccccgactgaaattgctcttgtttgaaggcacgttactatcaaagatgttggtatcagaagacttcagactagagggttcagttgtaacagagcgaagtttatctaatacaccatgaagccatacggtgaatcgaattgtgttgttccctagaaacagggacagatcctctgtcatttggtcctgacttttcttgttggccaccatcaccataatgtaatcaggaagttcttcatcaacataagctcctaattcttgtaatttccccttaatggcactccggatcttgcggctgatctcggtgccgatctccatggctctgcggcgtgcgggaactcagcactgcgcggcgcttggcttacccggaggctgccgcggactcctaccccgcagccgggacaccaccgcctcc

SEQ ID NO: 13622 - RNA, 16813 nt, Homo sapiens
  source 1..16813: mol_type = other RNA
gctgggattacaggcatgagccaccataataaggattctgatgaacatttgattccttggactactgttatactcaaaagccttccttaatcttctaattgtcaccctaaatatcctaaaatttctgtcttcctagtagttcttcatagtcctaaaaatttgtcagagagaaaggtaaatcaagaaacatgattttcaaatgatttaaggtggtactagggtttaggatttcctttgctttttatcatttaacacactgcttatcatacagctggaagtgctctgggccagtgtctctacttcgagggaagaaggaggtagtgagacagaaggaaatagcacaattcctggccctgacagaagggtgttcaggagacctgctctcctctcactttattccatctcatctggacctgtggcttccaatccacatctctttcctttaatatcctgcattggctaggctgtataaatcctttggtgcatcgaaaaactaagtgcattttttgtttttgtgattatgcaatacttataggaaaagttataattttagaatatttaagtacacttacatttttgagaaaaagactattgaaatgtttgtgccatgtcaaatttcagttgaacattttgggtattcttaatataagaccaggccaggcaccgtggctcaggccgggcacagtggctcacacctataatcccagcacttagggaggccaaggcgggaagatcacctgaagtcaggagttcaagaccagcctggctaacaaggtgaaactctgtctctactaaaaatacaaaaattagccgggcgtggtggctggcgcttgtaatcccagctacttgggaggctgagacaggagaatcacttgaacctgggaagcagaggttgtggtgagctgagatcgcaccattgcactccagcctgggcaacaaagagcgaaactccgtctcaaaaaaataaaaaataaaccctagaattatagtatgttagaattggaagggaagaattgtctaaggttattctagctaataagcaacagacttggaaaggaaaaggtcctgacaaagctaagcctcccgttcaggtttcctgactcgtgaattcagtgctgctgccactacacgatgcatgctctttgtatcaagggtgagacagcattacacatacatagaaaattatctatttaaactctatttgaacttttgatgagtttgtctccccctcccccactccttttcagaataacttgacgtttacaggtaccatcagtggtgatgtctgtgtgtggaaagatcacatattgtgtagaatcgtggcgagagctcacaacgggcctgtgtttgccatgtacaccaccctgcgagatggacttatcgtgactgggggaaaggaaaggccgtgagtcctctttcttttcacagaatatttatgcatttgtgacctacctgaggtttgcagttaattattctagttgtttctaggctacacagagtgtcctctccgaccttcctcctcatatgcttctcctttattaccttttatgtgccttctatttgattctcatttctggtcttaattcacttccaatttttttcatgttggggtgatactttttctgaggtgtggataggtagttgtcctacaagttgagttacttttcttaatgtctgtatgcctgtgtatgatttgctgagtaggaggcccatgggggaatctggagccagggttgtattttgactgcctgctctctttttgttcagaatggattctaaggagtagaatgcacattgttgctttagaaaaggatgagggaactagagagaactgccttgtttccttttgcttgaggcaaatttaaactgttttatacaagacctcaaaatttgagaagaggtctcttctgagtgattttcaaatctcccaacagtaaccagatacttatgatttgatttgtcaccaacatagtcatatgcatgttgaaacatgacatgtaggccaggcacagtggctcacacctgtaatcttatcactttgggaggctgaggcaggtggatcgcttgagcccaggagttcaagaccagcctgggcaacatggtgaaaccccatcgctataaaaaacaacaattagccgggtgtggtggcacatgcctgtagtccctgctactcaggaggctgaggtgggaggatcacttgagcctggggaggtcaaggctttagtgagctgtgatggtgccactgcactccagcctgggtgacagagtgagaccccatttaaaaaacaaaaacaaaaacaaaaaaaaatgtgacatatagttgactaagaagtacatttcaatacaggattgaaagaacccacatatgttaattaaacacaagcgcagaatttgtgccttttacataaaggaagaatgcacataggcatgctttcagacaagcaattcatctagcagaaaaggaaggaatacatttttcagcccttccaggaataaaatccataaatgggctctatttcgtcctccaacacttgtatttcccacgtcatttactcctgcacacccccactcactagaagcctgctaaactgttccagtgagatattttaacacctgatagggaataaatatgcttctgttttggccttcaaaaataagctctgggccagttgcagtggctcacgcctgtaatcccaacactttgggaggccgaggtgggcggatcacgaggtcaggagtttgggatcagcctggccaatatggtgaaactccatctctactaaaaatacaaaaattagccaggcatggtgcctgtaatcccagctacttgggaggctgaaggagaagaatcgcttgaacctgggaggcacaggttgcagtgagccgagatcacaccactgcactccaggccaggtgacagagcgacactctgtctcaaaaaaataaataaatcaactctgtagcatagcatttgtaattctattattttgccttacatttccattatccttttaataaaattgtttttttacatcttcctaatcaagaagtattatgaggccaggcacagtggctcatacctggaatcccagcactttgggaggccgaggcaggcagatcacctgaggtcaaggtatttgagaccagcctggccaacatggtgaaaccccatctctactaaaaatacagaaattagctgggtgtggtggtgcacacctgtaatgctagctactcgggaggctgaggtaggagaatcgcttgaacctgggaggcagaggttgcaataagcctagatcatgccactgcactcaagcctgggagacagagcgagactacatcttaaaaaaaaaaaaaaaagtattatgagagaggataatgtattgtaatgtattgtagaggctaaataaaattatgctcatgtcagaaaaaaagagtatttctcaaaataaaattcactgaaactggatgtttattttgactgagatatagtatatcctcaaattgccatagaaagtttacaagaatattagaggtaaattataaatatcagggcctttttaaaaaaaaaagattctgcttataacttggtatttgtttataataaaaattatagtagccaataatgaacacttactctggcttggttatttacttaggtcaaaagaaggaggagcggttaaactgtgggatcaggaactgaggcggtgccgtgccttcaggcttgagacaggacaagccacagattgtgttcgttctgtgtgcagaggcaaagtaagatgttccatgagctgatacagtgcagcagaaaacagaaagtggttattactgtgattccctcaccctttgcagcctaatgaacaatacttaataatgcataacgatggatttgcttgccaacattactctgtctttgctgctttctttgccaaagttagcaccagtgtggtgcataagctaggaagctattctgtctaaatactgtatgtaaacctccaatattttctagaatctgccaatttaacaactctagtagacataattgaaagcccttggcagttgactcatattaggacagctgtctccattttttaaaaaaacacacattccctagataaaacgtgcagtaaacaaacaatgaaatactactcagccataaaaaataatgaaattctgtcattcttggtggcaacatggatgagactggaggacatgatgtgaagtgaaataagccaggcacagaaagataaatacatgttctcactcctgtgcagaaactaaaaaagttgatcccacagaggtggagagtagaatagtggttactggaggcggacaagggggagggggagggggatagggaaggactggttaaaggatacaagtttacacagccagataggaatagtatgttttagtattctgtagtactgtaggatgactatagttaagaatcacgtatttatgtattttcaggtatttacaagagaggattttgaaagtttccatcacaaagaaatgataaatgtctgaggtgatggttatgcgtattaccctatgccctatagatatgtataattatgtgtcaatttcaaaataaaaattcaaaactacaactcctatgaaaatttttgagcgtgtttgtacttattaagtgtatttataaatcatacggatattatcttcagcctgcatattaaattgtagttaagcttttactttttaactaaaaaataaattctattattttttcctatatcccactgcactgaccccagtttggaaatcctaagattatcaaataaaaactttgattattgaagaatccaggtgtactgccacagaaaagttctattctgtagcatggactctaatatgtaatctagcccattgtgcttacagatagatgtgtgcctgtagtcatagaaaaatttgcatgagctaatgactgccttgctactagattagctcaaagcaaaaagttctctgaaagcaggtcaatagggtcatttttatattatgaagaagaaaagcagctgttgtattacattcactgtattggtcctgcttgtgtttcagggcaagatccttgttgggacaaggaatgctgaaataatcgaagttggagagaaaaatgcagcttgtaatattttagttaacggtcatgtggatgggccaatctggggactagcaacacatccttccagggattttttcctttctgctgcagaagatgggacagtgagactttgggatattgctgataaagtaagtacagataatttttttaaaagaggttacaacttctaaaaagaaaagttggaagttctaaattgctagtacttaaagaactgccagaattctgttgagcattttgaggggaaactggtataatttagaagtacttcacttaatgtttcctatgactctttttttttttttttttaaatgcagaagatgttaaacaaagtgaatttgggacatgctgctcgtactgtgtgttacagccctgaaggggacatggtggctattggaatgaaaaatggagaatttatcattttactagtgagttctctaaaaatatggggaaagaagagagacaggagatgtgcaatccatgatatcaggttagtgaacaaatggaatagagtttctagtatatacttgatttaacttccatttgtaaaattttccatagccttgccttcaaaaagaggtccccagggcctgtagcatttcccgtattataaattgtatgctaaaatatggctgtttgtatactacttaattcttcttgctaaattataaacccactgggcaccaactataatagcaagtactagtaggtaatgtttgatgaattcatgttaacacttagccatgtccattaagttcatcccaccaagaggtatctcccactgtaatacaagagagctatctgcccttcaaaagttgtcaccctggaaaactaaagttgtgatttcaaacatatcttctcttagtaacctcagtttgggaatatgtagttcattaatttaatcaatacctattgattaaatgttccagaatccaaattaatttaaatgtttcttaaacctttgtttttcagtgcttaagcatttttcaacagtggctaccatttacggagtacttccgtgtgatcagtagataagattattgaatctaggtctgtcaaaagcttgtacacttttcatcagtaaaatccttttacaaatgaaaccttcctcagaacttcaatatataaaatagtaacagtggcttcccttagcttttacatgtctctatcgtacctcagtaagactcatgggccatttcaagagactgaattgtcccatatgactccaaagattgctaggcaaatagcatttcactttgtcttttaaataagttcttcaggccgggcgcggtggctcatgcctgtaatcccagcactttgggaggccgaggcaggcagatcacctgaagtcaggagtactcgaccagcctggccaacatagtgaaaccccatctcaactaaaaatacaaaaatcagccgggcgtggtggcaggcgcctgtaatcccagctactcagggggctgaaacaggagaatcgcttgaacccgggaggcggaggttgcgccatcgcactccagcctgggagacaagagcgagacttcgtctcaaaaaaaaaaaattcttcttccaagattcaagttgtgtcatttcaccttaataactggaggttagttaagctgggctgtgttctttgcttaatattaagacaacgttttttccagatggaagaaaactatcttaatgaattgttagcttattaattatgtaatgctaatggcttttaaaagctgagatgttctgactgggtgttgtggctcacacctgtaatcccagtaccttgggaggccaagggggaaggattgcttgaggccaggagtttgggaccatagtgagaccccgcctctatttaaaaaattaaattttgttttgttttgttttgagttggagttttgctcttgttgcccatgctgaagtgcaatggtgcaatctcagctcaccacaacctgtgcctcctgggttcaagcgattctcctgcttcagcctcccgagtagatgggattacaggcgtgcaccaccatgcctggctaattttgtatttttagtagagacagggtttctctatgttggtcaggctggtctcaaactctcgacctcaggtgatctgcccgcctccgcttcccaaagttctgggattataggtgtgagccactgggcctggcctaagaaagtttttttaagccattagacgtttttaaaggaattgggagatgacaattggggaaatatttaaaatttaagtaaaatataaagcttccttatttcatgtaacccagacaatctcagtatacatgatcagttgtgtctgacaggtaaatctatttgaggccttatcacacgttacttttaagaactagaaaggaaaagtcactgatcttaagtatttataatacttcatgtggtctaatactttttacgttttgttttgattcagatttagtccggattcccggtatctggcagtaggttctagtgagaactcagtggatttttatgacctaacgctgggccccactcttaacagaatcagctactgcaaagacattccaagctttgtcattcaaatggacttctctgcagatagcagttatctccaggtacagtaccaatactgtatacccaggtggcaagttcttctgcttttacatttcgtgttagtgaatgcatttaaagttcctgagctccagagctccagcttctcaactcctccctttgtaccttctgacctacagctcccctttcctcccccacttatcagagcttttctcctattaagtttttgtagtgatcttttgcatacttaataatgttagacatgtaaatcaagtagcaatatgctagtattctgtaaaccccctgtggattttgtctctcacctaatggaattcttgtcccattttaatctgatgaaaaaggtctctagtggctgctataaacggcatgtctatgaagtgccttcaggaaaacatcttatggatcatgccgctattgacagaattacttgggctacatggactaggtaaatacttatatattcacaaggcaagaactgactttgaaggccagttagaaaatcctatttctgaactgttagagccattccaataaggaatagtaattgagtttcaagtttttgttaccatattttgaaatggtatgttcatgttgggacccctttttattgaatatatttccatgttttatcagtttccatgatttatcaagttttttttttaaggaaatcaaagttttaactttaaagataccctgatatttttcttaatgctaaatttaatgactggcaaaaaggtattgggtgctgttaagcaactgttattaattctctatctaaaggaatgctatcttgaatctattagaagtcaaagcttccaaatttgttcaaatttcctggctgtatgacaggtaaccatgactatccatttttttggccaatgaaaaatgccatcaaattcctgtatcagccaggcatatagtggctcatgcctgtaatctctgatgtagcaggccgaggtgggaggatcacttgagcctagaagttttgataccagcctgggcaacatagcaagaccccatctctgaaatttttttaattcctatgtcataagtcatttttatttttgtagagatagggatctcacaatattgcccaggctggtctcaaactcttggcctcaagcagtcctcctgcctcagcctcccaaaatgttgggattactggtatgtgctgctggacccagccaagtagcacttttaatttgaaaaatagttctatcagttttcagtcaggcgcggtggctcagcctgtaatcccagcactttgggaggccgagcgggggtgatcacctgaggtcgggagttcgagactagcctgaccaacatggagaaaccctgtctctactaaaaatacaaaataagccgggcatgttagcgcatgcctgtgatcccagctactcgggaggctgaggcaggagaattgcttgaacccaggaggcagaggttgcggtgagccgagatcatgccattgcactccagcctgggtaacaagagcgaaaactccgtctcaaaaaaaaaaaaagaaaaaatagttctatcagttttcataaagtactactttaatcttaaaaagattaatctagaaacccttcaaattataaaatgtcatttttaaaaggcaggagttgatatcctgatgaaattcaggtctccaaacaacttaccataatttacttcctgtattttaagtaacatgatagggtacttagagattaattgccaagaaactttttgaatatagtcaacctgcccgcacttgccatgatgagttttcttttgttccttccctctagtattctaggagatgaggttttgggaatctggtccagacatgctgagaaagctgatgtcaactgtgcctgtgtatctcattcaggaatcagtcttgttacaggagatgactttggcatggttaagttatttgacttcccatgtccagaaaaatttgtaagtttgtgttttgtttactattatcagtttactcctaattttgatgtcttatcatcagcacttttccccatatatttaaaatgttttgtcctaatttctaaatttttccccaaactttctaaatctatttactttgaaataaaagctattagaaacaaatcctctccctcgagtaataccatctttggaaccatcctacaaaagctgtaattagcttttcaccaaacctataatcagttatcaaatttcaaatgcttttccttagagaaaaatggtcagagtacctggagacatctgactgcccacacagcctggttttgcagatccactactcatgctgaaaagcattctaatcactggctgcggtgctaactccctactctctccacagctcttgtcatagagattatagttcctaataagagcctttgacttctgtgtgcaccaaatgccctgagcttgtctgtcattgttttttaggcaaaacacaaaaggttcttgggtcattcgccccatgtgacaaatattcgatttaccagtggtgatcgacatgttgttagtgctggaggtgatgactgcaggttagtaactttctcagcccatgaagagcagactatgttactagttaagagacttaatacaacaactcctacagctttggtttatgaaatcagctagtcaacattagtagaaggtagtataaccagatggctcttcagaatctcatatttatgcaaatacagaataaaaggagttaaagaggaaaaatattacacatgtaacctgaaagcacaactgaaaaatattaaactgttatgaaaatctaaaaacataattaactccctgcaattttcttctctgattgcagcttatttgtctggaaatgtgtacatacacctcactgagagatgctgagatgactacagaaattaactttgagaccagaattacagagaagaaaaaccaaaacccaaccctgcatggtcaagtggtgctaacccaagactgtaacagggagaaatgcccagaatcatcaaaatagtgaaagactgatctgttcaaaatatttgctatatgcactgggtataatccgtaatccatacactgccagataatgccatttcaaggaaggatcgaatacttgatggtaaaggccaagtccccctgtattgggaagtgtgtgatttcggcagacctgctgggaaaatttagggtagagcactctttacagaagaactcaaaaacccaatttggataattttcattatctttttagcaaaatggtttcttaatgtttatattttattttcaaggttcattgtttaatgaaatattttattcttgcatttccataaggaaagggaaagtcatgatcatcctaaaggatcacagtttttaaaaggcaaacattttccctaaggaaacagacacaagctttcctagagaatatgatgttttttaggcattaataaggtccttttttataaaggacacttttctcctagtagttttgaattcaggaacagatccaaagttagcagtatatggctgctacatttccattttcattttcgagccatcagtttatgttcagatgccatctctgtaatcgcacatttaaaacataactgtagcctcactaatggaaaagtagtatgatgaacaatcattcccaatggtgtacaatgtaagggttttagggagcaacagtatttaactggaagaaagaattgcatatttaatgtagtctaatatatacacatttgtttaacatgtaaacaaaagtgttaaattcacatatacaacattatacaatttaatcactcttggaataaaatttttatagccttttttctattgggaaaatttgtttagatgtgtgccactccataggtttatttccaaaatgaatgagcccaactccatttgtaaaaacttgtcagttagaattcctttttttagtggattagggctgaattcttagatccttatttcttttcactttaaatgctgccaaagatcactactcatcattcaggaattcgctgtctagcctatctgtagtttcctgaagattgaaaattatgtagactgctatttaaaaatatatttttctaagtgtgaggtttaagatgctgtattgaccctatgagtttttaatgtgttaattatctttatagcataatagatcgctttaggttcctggaatcccatttggtctgacaggatatatgaagattcttaatacctattttctgtgtctaatacttggttaatactaaaaatagaaatgactaaattacatcacagaaagcataaccagtgattgaacctggtagttttaaagctctaaatagctgtggctgaaggactgattatggggctaagaagcttgaaacgtaagttggtacttgttcatcagtggattctcctaaattaagccaaattttgaaatacatgactattaagtttctactcatgtatttacagtcagtcaataaattaaaggaggaaaaaaatccctgaacaacctgcccataaaaagaaaaatactctacatttgagcctgctgcagttttaaattttccctctgggtcaagtttgccagcttttggctacagagaaattatatttccattacagtgcaggtagaaactctgtaaccttaagcatgtaaactacatagaataaaactgtttccactgcatttctgtccttcaaagtggccaacctgattaagtcagccttaatcactgctgctgtcagtttcacgactaaaggtcatattgactaagtagtcatcagctgaccacctcgctgtatcagccagcaacgaggggaaggtgaagaaacatgataggccatatagaatctgccctatgtttacttttttaacccagataattatttttgtgtgcagtatctaagctcctgattgtgtaacctgggacttctggcaccttttgttccattcattttatgtataaaatgcatgccaaagcacactgtgccctctggtacccttgcttccaatcgccaaccatgctcatttccttcctttttttgtggtccctttttgtggtgatcattttaaaccacgtcatccaacaaatgttttatggtcaaccttagcttgttcataagccatagcaactgaaagattaaactcttaaatatgtgtctgggcagtggctattaaatagcaaaaaacaatcagattttagtattttattatttccttgtaaaatggctgaactaaattaaacccttgtttcccatttgttctataatttatagtgaaactgagaacaaaactatctttataaatgatagctaaaagtatttccagatatttaaacaatttaaaataaatttcttctgcagagatgcaaagcatctcaacactggaatgaacaaatgccttaaattcaatggagtaaacctttagaatgaagaggaactgtcatttcacccaagccgaagacaacagccttatgcacttgtgtgctctgtctttgctgcttctcgtgtttcaagcctttcctgtgggatcagcacagcaaagtgcaacttaccaaatggtttaatgactggttaattctttcttctcccaatggaaaagcaatggcaacacaacagtagactgctggcttgacaatcttaaacgtgagcctttgcacatgtaggtttatcatcatttgagtatacgactaagcaagtcaatgaactttttttttttttttagcagtttaatttggtcctgagaatgttgcagtctttattaccccttttgcattaatccacttttctaaccaccttttaagctttaatttttaacactatacaccaagtctttgaaatcagtgatctgttatttaactctaaagcatttgacacttcttgccttaacagttttaaaaaccacacacaaaaaaactctgtaagtaatacagtaggccaaaagtttcatcctatctatcttgcagtttacctatctgatctgatctctgtaattatagttctgtcatttaaaatatactatttaaatctaatttttacatttcaaaaattatcttcagtagtaactaagtatattttctgtggattctgagaatgttatttttcagaatgtgagaatatatatgtacatttataatcttgtgactttaaagtctgttttcagatacagtatgtaaatacttgtaaaaaaatttgtataattttgtgataatgtagtttcccaaaaaaattatttagaaggcattatgttattagtaaatgagagcactgtatagaactgttcctattttctgcacttgccattccagctgcctccactgtccatacccacctcattcatcctgtcacagaaggcaggaaaactgggaactttaccaaagtagcactcagcctgagaggcctgtataatcatgcttttcaaactaaattcacttaaaaattaaaaagcagaattgaatattttaagcagcctcagtacctttggccaatgctgttttcatggtggattatgaacattatataatctttgggaaaagtgaaagtagtacaatttttagaataatgacaactgcctcactgcatctctccactcacacagcaaccgtgtagccccctaagctgcagtaccatgactaaccatgatgtcaatttcatatgctgatcctcacaacagcagtgcacaaacatgccccaaatattttaacagaatttagctcttccttaagctgtcttttcatagtaaaaacaaaacaaaaacacccaatgttaaaaccacataataaacttacaaacttgaaaaattagacacttcagatagataggcaataaaacttcatattatgaaagcaatatattccaagtttcaaagatttgacaagttctgtagagtatctttcatcagtacatgaaaacttccaaactgcatgatcttctgccaggcaggactgggtgctattcgctggtttgaggtcgaatccatttcaaggcatgtcgtggtgggacattaatggtgggatggtagaatgtgcagtccggtcttgtacattgagtgttaaacctacaatgttttggatgatagaagggacattccatcttcttacaagcagggaagtaacggcagagctgactactggaaggtggtgctggtggtgcaactggttttggagacagtactggaattcttctactcacatgagtgaagggacaatctggtttagtacactttgcatcatatttacaatttgggtgaacaaacaaacatttttcagcaaatttacaattggggaaggctttgcagggtgagatggggtgatggtaggcacactcatccccatttttacaagcaggccagtacttgcagcgctccaaaagtttttctggtttctgtgccacactcagttcactcatctcagcgttagaaaagctaccatttgggtcctcaagctgcctgctcagcaagtgcaactgctgtgggtggaggagacctctgagtcccttgtttgaggctgcagtttggtttacgggtttcattccttcaaagcacatgtcctcctcttgatctgacatgtatcctggggggctggggacaccatccagcgtcactataaacttgggacttgcaggtttatctggttgtacaagatctcgtgtctgcataaggtgtcctgaaagtacccgaagggaatctgcagtcttcatccccgactcttggtttggtgccactactacttcctcagacagctttggcttcttcagaataaatgatcttgtgtctgcatggaccatggattccatgtcatagtaatcttgactcatctgcagagtttctgccattactgggtcgatttgcagtcgggataataattgcctctgttgagttccttgatttttttctacagaatctccttttgtttcctcttctttaatggggggacttattctgggggtcctactttgtccctggaccacttctgctagcaattcttcttgagaagttcgagttctgggagcaactggaagtgtctgtttctgtggaactgtagagtagttagttgtttttgttacggattcttgagcttcagatatagccttcaaaatcagattcttgttagcttgtttagaaggtggaagagaaggtctcctttcaggctttgcaggcacagacacactgctggagatgcttcctgttcgagacccgtaatcatcatcttcttcctcctcttctccatcatgattgaatttttttactttaacaactgaacttaccacaggcaactttctcttccgaaagttttcatcctccatactcattttctccgagttgtttctaaagaacggactatacgtttcttctaagctgttaagcacctctggttcacacaaacgtcctgtttcatatacccaactactctgcatatcaagctgcttggcagcatgaatactattctgctgctgttgaaattgcaacctgtttaaatgaacaccactatctgcatttctacttgcaggtggtcgataaatttcaatagaagggcgagaagaaccatatgtaagtgtcactgtaggttttttctgagataagggattctcctgcacaaagttgaggtcttcgtcaatgagatcatctggttctggcttaatatcaatcacatcttcagagggtgctggctccctcaaaggtttcactgttgacattagtcgggttgcagctccatcatcgtaagtctgtctgacatttgtggtttttgactcctgcgaacttgtagaaactctggaatctcttttttcaggtctcgcgctaggaatggcaagtggtggcactgcagcttcatgcctcctctcatctccccgactgaaattgctcttgtttgaaggcacgttactatcaaagatgttggtatcagaagacttcagactagagggttcagttgtaacagagcgaagtttatctaatacaccatgaagccaacataagctcctaattcttgtaatttccccttaatggcactccggatcttgcggctgatctcggtgccgatctccatggctctgcggcgtgcgggaactcagcactgcgcggcgcttggcttacccggaggctgccgcggactcctaccccgcagccgggacaccaccgcctcc

SEQ ID NO: 13623 - RNA, 16928 nt, Homo sapiens
  source 1..16928: mol_type = other RNA
gctgggattacaggcatgagccaccataataaggattctgatgaacatttgattccttggactactgttatactcaaaagccttccttaatcttctaattgtcaccctaaatatcctaaaatttctgtcttcctagtagttcttcatagtcctaaaaatttgtcagagagaaaggtaaatcaagaaacatgattttcaaatgatttaaggtggtactagggtttaggatttcctttgctttttatcatttaacacactgcttatcatacagctggaagtgctctgggccagtgtctctacttcgagggaagaaggaggtagtgagacagaaggaaatagcacaattcctggccctgacagaagggtgttcaggagacctgctctcctctcactttattccatctcatctggacctgtggcttccaatccacatctctttcctttaatatcctgcattggctaggctgtataaatcctttggtgcatcgaaaaactaagtgcattttttgtttttgtgattatgcaatacttataggaaaagttataattttagaatatttaagtacacttacatttttgagaaaaagactattgaaatgtttgtgccatgtcaaatttcagttgaacattttgggtattcttaatataagaccaggccaggcaccgtggctcaggccgggcacagtggctcacacctataatcccagcacttagggaggccaaggcgggaagatcacctgaagtcaggagttcaagaccagcctggctaacaaggtgaaactctgtctctactaaaaatacaaaaattagccgggcgtggtggctggcgcttgtaatcccagctacttgggaggctgagacaggagaatcacttgaacctgggaagcagaggttgtggtgagctgagatcgcaccattgcactccagcctgggcaacaaagagcgaaactccgtctcaaaaaaataaaaaataaaccctagaattatagtatgttagaattggaagggaagaattgtctaaggttattctagctaataagcaacagacttggaaaggaaaaggtcctgacaaagctaagcctcccgttcaggtttcctgactcgtgaattcagtgctgctgccactacacgatgcatgctctttgtatcaagggtgagacagcattacacatacatagaaaattatctatttaaactctatttgaacttttgatgagtttgtctccccctcccccactccttttcagaataacttgacgtttacaggtaccatcagtggtgatgtctgtgtgtggaaagatcacatattgtgtagaatcgtggcgagagctcacaacgggcctgtgtttgccatgtacaccaccctgcgagatggacttatcgtgactgggggaaaggaaaggccgtgagtcctctttcttttcacagaatatttatgcatttgtgacctacctgaggtttgcagttaattattctagttgtttctaggctacacagagtgtcctctccgaccttcctcctcatatgcttctcctttattaccttttatgtgccttctatttgattctcatttctggtcttaattcacttccaatttttttcatgttggggtgatactttttctgaggtgtggataggtagttgtcctacaagttgagttacttttcttaatgtctgtatgcctgtgtatgatttgctgagtaggaggcccatgggggaatctggagccagggttgtattttgactgcctgctctctttttgttcagaatggattctaaggagtagaatgcacattgttgctttagaaaaggatgagggaactagagagaactgccttgtttccttttgcttgaggcaaatttaaactgttttatacaagacctcaaaatttgagaagaggtctcttctgagtgattttcaaatctcccaacagtaaccagatacttatgatttgatttgtcaccaacatagtcatatgcatgttgaaacatgacatgtaggccaggcacagtggctcacacctgtaatcttatcactttgggaggctgaggcaggtggatcgcttgagcccaggagttcaagaccagcctgggcaacatggtgaaaccccatcgctataaaaaacaacaattagccgggtgtggtggcacatgcctgtagtccctgctactcaggaggctgaggtgggaggatcacttgagcctggggaggtcaaggctttagtgagctgtgatggtgccactgcactccagcctgggtgacagagtgagaccccatttaaaaaacaaaaacaaaaacaaaaaaaaatgtgacatatagttgactaagaagtacatttcaatacaggattgaaagaacccacatatgttaattaaacacaagcgcagaatttgtgccttttacataaaggaagaatgcacataggcatgctttcagacaagcaattcatctagcagaaaaggaaggaatacatttttcagcccttccaggaataaaatccataaatgggctctatttcgtcctccaacacttgtatttcccacgtcatttactcctgcacacccccactcactagaagcctgctaaactgttccagtgagatattttaacacctgatagggaataaatatgcttctgttttggccttcaaaaataagctctgggccagttgcagtggctcacgcctgtaatcccaacactttgggaggccgaggtgggcggatcacgaggtcaggagtttgggatcagcctggccaatatggtgaaactccatctctactaaaaatacaaaaattagccaggcatggtgcctgtaatcccagctacttgggaggctgaaggagaagaatcgcttgaacctgggaggcacaggttgcagtgagccgagatcacaccactgcactccaggccaggtgacagagcgacactctgtctcaaaaaaataaataaatcaactctgtagcatagcatttgtaattctattattttgccttacatttccattatccttttaataaaattgtttttttacatcttcctaatcaagaagtattatgaggccaggcacagtggctcatacctggaatcccagcactttgggaggccgaggcaggcagatcacctgaggtcaaggtatttgagaccagcctggccaacatggtgaaaccccatctctactaaaaatacagaaattagctgggtgtggtggtgcacacctgtaatgctagctactcgggaggctgaggtaggagaatcgcttgaacctgggaggcagaggttgcaataagcctagatcatgccactgcactcaagcctgggagacagagcgagactacatcttaaaaaaaaaaaaaaaagtattatgagagaggataatgtattgtaatgtattgtagaggctaaataaaattatgctcatgtcagaaaaaaagagtatttctcaaaataaaattcactgaaactggatgtttattttgactgagatatagtatatcctcaaattgccatagaaagtttacaagaatattagaggtaaattataaatatcagggcctttttaaaaaaaaaagattctgcttataacttggtatttgtttataataaaaattatagtagccaataatgaacacttactctggcttggttatttacttaggtcaaaagaaggaggagcggttaaactgtgggatcaggaactgaggcggtgccgtgccttcaggcttgagacaggacaagccacagattgtgttcgttctgtgtgcagaggcaaagtaagatgttccatgagctgatacagtgcagcagaaaacagaaagtggttattactgtgattccctcaccctttgcagcctaatgaacaatacttaataatgcataacgatggatttgcttgccaacattactctgtctttgctgctttctttgccaaagttagcaccagtgtggtgcataagctaggaagctattctgtctaaatactgtatgtaaacctccaatattttctagaatctgccaatttaacaactctagtagacataattgaaagcccttggcagttgactcatattaggacagctgtctccattttttaaaaaaacacacattccctagataaaacgtgcagtaaacaaacaatgaaatactactcagccataaaaaataatgaaattctgtcattcttggtggcaacatggatgagactggaggacatgatgtgaagtgaaataagccaggcacagaaagataaatacatgttctcactcctgtgcagaaactaaaaaagttgatcccacagaggtggagagtagaatagtggttactggaggcggacaagggggagggggagggggatagggaaggactggttaaaggatacaagtttacacagccagataggaatagtatgttttagtattctgtagtactgtaggatgactatagttaagaatcacgtatttatgtattttcaggtatttacaagagaggattttgaaagtttccatcacaaagaaatgataaatgtctgaggtgatggttatgcgtattaccctatgccctatagatatgtataattatgtgtcaatttcaaaataaaaattcaaaactacaactcctatgaaaatttttgagcgtgtttgtacttattaagtgtatttataaatcatacggatattatcttcagcctgcatattaaattgtagttaagcttttactttttaactaaaaaataaattctattattttttcctatatcccactgcactgaccccagtttggaaatcctaagattatcaaataaaaactttgattattgaagaatccaggtgtactgccacagaaaagttctattctgtagcatggactctaatatgtaatctagcccattgtgcttacagatagatgtgtgcctgtagtcatagaaaaatttgcatgagctaatgactgccttgctactagattagctcaaagcaaaaagttctctgaaagcaggtcaatagggtcatttttatattatgaagaagaaaagcagctgttgtattacattcactgtattggtcctgcttgtgtttcagggcaagatccttgttgggacaaggaatgctgaaataatcgaagttggagagaaaaatgcagcttgtaatattttagttaacggtcatgtggatgggccaatctggggactagcaacacatccttccagggattttttcctttctgctgcagaagatgggacagtgagactttgggatattgctgataaagtaagtacagataatttttttaaaagaggttacaacttctaaaaagaaaagttggaagttctaaattgctagtacttaaagaactgccagaattctgttgagcattttgaggggaaactggtataatttagaagtacttcacttaatgtttcctatgactctttttttttttttttttaaatgcagaagatgttaaacaaagtgaatttgggacatgctgctcgtactgtgtgttacagccctgaaggggacatggtggctattggaatgaaaaatggagaatttatcattttactagtgagttctctaaaaatatggggaaagaagagagacaggagatgtgcaatccatgatatcaggttagtgaacaaatggaatagagtttctagtatatacttgatttaacttccatttgtaaaattttccatagccttgccttcaaaaagaggtccccagggcctgtagcatttcccgtattataaattgtatgctaaaatatggctgtttgtatactacttaattcttcttgctaaattataaacccactgggcaccaactataatagcaagtactagtaggtaatgtttgatgaattcatgttaacacttagccatgtccattaagttcatcccaccaagaggtatctcccactgtaatacaagagagctatctgcccttcaaaagttgtcaccctggaaaactaaagttgtgatttcaaacatatcttctcttagtaacctcagtttgggaatatgtagttcattaatttaatcaatacctattgattaaatgttccagaatccaaattaatttaaatgtttcttaaacctttgtttttcagtgcttaagcatttttcaacagtggctaccatttacggagtacttccgtgtgatcagtagataagattattgaatctaggtctgtcaaaagcttgtacacttttcatcagtaaaatccttttacaaatgaaaccttcctcagaacttcaatatataaaatagtaacagtggcttcccttagcttttacatgtctctatcgtacctcagtaagactcatgggccatttcaagagactgaattgtcccatatgactccaaagattgctaggcaaatagcatttcactttgtcttttaaataagttcttcaggccgggcgcggtggctcatgcctgtaatcccagcactttgggaggccgaggcaggcagatcacctgaagtcaggagtactcgaccagcctggccaacatagtgaaaccccatctcaactaaaaatacaaaaatcagccgggcgtggtggcaggcgcctgtaatcccagctactcagggggctgaaacaggagaatcgcttgaacccgggaggcggaggttgcgccatcgcactccagcctgggagacaagagcgagacttcgtctcaaaaaaaaaaaattcttcttccaagattcaagttgtgtcatttcaccttaataactggaggttagttaagctgggctgtgttctttgcttaatattaagacaacgttttttccagatggaagaaaactatcttaatgaattgttagcttattaattatgtaatgctaatggcttttaaaagctgagatgttctgactgggtgttgtggctcacacctgtaatcccagtaccttgggaggccaagggggaaggattgcttgaggccaggagtttgggaccatagtgagaccccgcctctatttaaaaaattaaattttgttttgttttgttttgagttggagttttgctcttgttgcccatgctgaagtgcaatggtgcaatctcagctcaccacaacctgtgcctcctgggttcaagcgattctcctgcttcagcctcccgagtagatgggattacaggcgtgcaccaccatgcctggctaattttgtatttttagtagagacagggtttctctatgttggtcaggctggtctcaaactctcgacctcaggtgatctgcccgcctccgcttcccaaagttctgggattataggtgtgagccactgggcctggcctaagaaagtttttttaagccattagacgtttttaaaggaattgggagatgacaattggggaaatatttaaaatttaagtaaaatataaagcttccttatttcatgtaacccagacaatctcagtatacatgatcagttgtgtctgacaggtaaatctatttgaggccttatcacacgttacttttaagaactagaaaggaaaagtcactgatcttaagtatttataatacttcatgtggtctaatactttttacgttttgttttgattcagatttagtccggattcccggtatctggcagtaggttctagtgagaactcagtggatttttatgacctaacgctgggccccactcttaacagaatcagctactgcaaagacattccaagctttgtcattcaaatggacttctctgcagatagcagttatctccaggtacagtaccaatactgtatacccaggtggcaagttcttctgcttttacatttcgtgttagtgaatgcatttaaagttcctgagctccagagctccagcttctcaactcctccctttgtaccttctgacctacagctcccctttcctcccccacttatcagagcttttctcctattaagtttttgtagtgatcttttgcatacttaataatgttagacatgtaaatcaagtagcaatatgctagtattctgtaaaccccctgtggattttgtctctcacctaatggaattcttgtcccattttaatctgatgaaaaaggtctctagtggctgctataaacggcatgtctatgaagtgccttcaggaaaacatcttatggatcatgccgctattgacagaattacttgggctacatggactaggtaaatacttatatattcacaaggcaagaactgactttgaaggccagttagaaaatcctatttctgaactgttagagccattccaataaggaatagtaattgagtttcaagtttttgttaccatattttgaaatggtatgttcatgttgggacccctttttattgaatatatttccatgttttatcagtttccatgatttatcaagttttttttttaaggaaatcaaagttttaactttaaagataccctgatatttttcttaatgctaaatttaatgactggcaaaaaggtattgggtgctgttaagcaactgttattaattctctatctaaaggaatgctatcttgaatctattagaagtcaaagcttccaaatttgttcaaatttcctggctgtatgacaggtaaccatgactatccatttttttggccaatgaaaaatgccatcaaattcctgtatcagccaggcatatagtggctcatgcctgtaatctctgatgtagcaggccgaggtgggaggatcacttgagcctagaagttttgataccagcctgggcaacatagcaagaccccatctctgaaatttttttaattcctatgtcataagtcatttttatttttgtagagatagggatctcacaatattgcccaggctggtctcaaactcttggcctcaagcagtcctcctgcctcagcctcccaaaatgttgggattactggtatgtgctgctggacccagccaagtagcacttttaatttgaaaaatagttctatcagttttcagtcaggcgcggtggctcagcctgtaatcccagcactttgggaggccgagcgggggtgatcacctgaggtcgggagttcgagactagcctgaccaacatggagaaaccctgtctctactaaaaatacaaaataagccgggcatgttagcgcatgcctgtgatcccagctactcgggaggctgaggcaggagaattgcttgaacccaggaggcagaggttgcggtgagccgagatcatgccattgcactccagcctgggtaacaagagcgaaaactccgtctcaaaaaaaaaaaaagaaaaaatagttctatcagttttcataaagtactactttaatcttaaaaagattaatctagaaacccttcaaattataaaatgtcatttttaaaaggcaggagttgatatcctgatgaaattcaggtctccaaacaacttaccataatttacttcctgtattttaagtaacatgatagggtacttagagattaattgccaagaaactttttgaatatagtcaacctgcccgcacttgccatgatgagttttcttttgttccttccctctagtattctaggagatgaggttttgggaatctggtccagacatgctgagaaagctgatgtcaactgtgcctgtgtatctcattcaggaatcagtcttgttacaggagatgactttggcatggttaagttatttgacttcccatgtccagaaaaatttgtaagtttgtgttttgtttactattatcagtttactcctaattttgatgtcttatcatcagcacttttccccatatatttaaaatgttttgtcctaatttctaaatttttccccaaactttctaaatctatttactttgaaataaaagctattagaaacaaatcctctccctcgagtaataccatctttggaaccatcctacaaaagctgtaattagcttttcaccaaacctataatcagttatcaaatttcaaatgcttttccttagagaaaaatggtcagagtacctggagacatctgactgcccacacagcctggttttgcagatccactactcatgctgaaaagcattctaatcactggctgcggtgctaactccctactctctccacagctcttgtcatagagattatagttcctaataagagcctttgacttctgtgtgcaccaaatgccctgagcttgtctgtcattgttttttaggcaaaacacaaaaggttcttgggtcattcgccccatgtgacaaatattcgatttaccagtggtgatcgacatgttgttagtgctggaggtgatgactgcaggttagtaactttctcagcccatgaagagcagactatgttactagttaagagacttaatacaacaactcctacagctttggtttatgaaatcagctagtcaacattagtagaaggtagtataaccagatggctcttcagaatctcatatttatgcaaatacagaataaaaggagttaaagaggaaaaatattacacatgtaacctgaaagcacaactgaaaaatattaaactgttatgaaaatctaaaaacataattaactccctgcaattttcttctctgattgcagcttatttgtctggaaatgtgtacatacacctcactgagagatgctgagatgactacagaaattaactttgagaccagaattacagagaagaaaaaccaaaacccaaccctgcatggtcaagtggtgctaacccaagactgtaacagggagaaatgcccagaatcatcaaaatagtgaaagactgatctgttcaaaatatttgctatatgcactgggtataatccgtaatccatacactgccagataatgccatttcaaggaaggatcgaatacttgatggtaaaggccaagtccccctgtattgggaagtgtgtgatttcggcagacctgctgggaaaatttagggtagagcactctttacagaagaactcaaaaacccaatttggataattttcattatctttttagcaaaatggtttcttaatgtttatattttattttcaaggttcattgtttaatgaaatattttattcttgcatttccataaggaaagggaaagtcatgatcatcctaaaggatcacagtttttaaaaggcaaacattttccctaaggaaacagacacaagctttcctagagaatatgatgttttttaggcattaataaggtccttttttataaaggacacttttctcctagtagttttgaattcaggaacagatccaaagttagcagtatatggctgctacatttccattttcattttcgagccatcagtttatgttcagatgccatctctgtaatcgcacatttaaaacataactgtagcctcactaatggaaaagtagtatgatgaacaatcattcccaatggtgtacaatgtaagggttttagggagcaacagtatttaactggaagaaagaattgcatatttaatgtagtctaatatatacacatttgtttaacatgtaaacaaaagtgttaaattcacatatacaacattatacaatttaatcactcttggaataaaatttttatagccttttttctattgggaaaatttgtttagatgtgtgccactccataggtttatttccaaaatgaatgagcccaactccatttgtaaaaacttgtcagttagaattcctttttttagtggattagggctgaattcttagatccttatttcttttcactttaaatgctgccaaagatcactactcatcattcaggaattcgctgtctagcctatctgtagtttcctgaagattgaaaattatgtagactgctatttaaaaatatatttttctaagtgtgaggtttaagatgctgtattgaccctatgagtttttaatgtgttaattatctttatagcataatagatcgctttaggttcctggaatcccatttggtctgacaggatatatgaagattcttaatacctattttctgtgtctaatacttggttaatactaaaaatagaaatgactaaattacatcacagaaagcataaccagtgattgaacctggtagttttaaagctctaaatagctgtggctgaaggactgattatggggctaagaagcttgaaacgtaagttggtacttgttcatcagtggattctcctaaattaagccaaattttgaaatacatgactattaagtttctactcatgtatttacagtcagtcaataaattaaaggaggaaaaaaatccctgaacaacctgcccataaaaagaaaaatactctacatttgagcctgctgcagttttaaattttccctctgggtcaagtttgccagcttttggctacagagaaattatatttccattacagtgcaggtagaaactctgtaaccttaagcatgtaaactacatagaataaaactgtttccactgcatttctgtccttcaaagtggccaacctgattaagtcagccttaatcactgctgctgtcagtttcacgactaaaggtcatattgactaagtagtcatcagctgaccacctcgctgtatcagccagcaacgaggggaaggtgaagaaacatgataggccatatagaatctgccctatgtttacttttttaacccagataattatttttgtgtgcagtatctaagctcctgattgtgtaacctgggacttctggcaccttttgttccattcattttatgtataaaatgcatgccaaagcacactgtgccctctggtacccttgcttccaatcgccaaccatgctcatttccttcctttttttgtggtccctttttgtggtgatcattttaaaccacgtcatccaacaaatgttttatggtcaaccttagcttgttcataagccatagcaactgaaagattaaactcttaaatatgtgtctgggcagtggctattaaatagcaaaaaacaatcagattttagtattttattatttccttgtaaaatggctgaactaaattaaacccttgtttcccatttgttctataatttatagtgaaactgagaacaaaactatctttataaatgatagctaaaagtatttccagatatttaaacaatttaaaataaatttcttctgcagagatgcaaagcatctcaacactggaatgaacaaatgccttaaattcaatggagtaaacctttagaatgaagaggaactgtcatttcacccaagccgaagacaacagccttatgcacttgtgtgctctgtctttgctgcttctcgtgtttcaagcctttcctgtgggatcagcacagcaaagtgcaacttaccaaatggtttaatgactggttaattctttcttctcccaatggaaaagcaatggcaacacaacagtagactgctggcttgacaatcttaaacgtgagcctttgcacatgtaggtttatcatcatttgagtatacgactaagcaagtcaatgaactttttttttttttttagcagtttaatttggtcctgagaatgttgcagtctttattaccccttttgcattaatccacttttctaaccaccttttaagctttaatttttaacactatacaccaagtctttgaaatcagtgatctgttatttaactctaaagcatttgacacttcttgccttaacagttttaaaaaccacacacaaaaaaactctgtaagtaatacagtaggccaaaagtttcatcctatctatcttgcagtttacctatctgatctgatctctgtaattatagttctgtcatttaaaatatactatttaaatctaatttttacatttcaaaaattatcttcagtagtaactaagtatattttctgtggattctgagaatgttatttttcagaatgtgagaatatatatgtacatttataatcttgtgactttaaagtctgttttcagatacagtatgtaaatacttgtaaaaaaatttgtataattttgtgataatgtagtttcccaaaaaaattatttagaaggcattatgttattagtaaatgagagcactgtatagaactgttcctattttctgcacttgccattccagctgcctccactgtccatacccacctcattcatcctgtcacagaaggcaggaaaactgggaactttaccaaagtagcactcagcctgagaggcctgtataatcatgcttttcaaactaaattcacttaaaaattaaaaagcagaattgaatattttaagcagcctcagtacctttggccaatgctgttttcatggtggattatgaacattatataatctttgggaaaagtgaaagtagtacaatttttagaataatgacaactgcctcactgcatctctccactcacacagcaaccgtgtagccccctaagctgcagtaccatgactaaccatgatgtcaatttcatatgctgatcctcacaacagcagtgcacaaacatgccccaaatattttaacagaatttagctcttccttaagctgtcttttcatagtaaaaacaaaacaaaaacacccaatgttaaaaccacataataaacttacaaacttgaaaaattagacacttcagatagataggcaataaaacttcatattatgaaagcaatatattccaagtttcaaagatttgacaagttctgtagagtatctttcatcagtacatgaaaacttccaaactgcatgatcttctgccaggcaggactgggtgctattcgctggtttgaggtcgaatccatttcaaggcatgtcgtggtgggacattaatggtgggatggtagaatgtgcagtccggtcttgtacattgagtgttaaacctacaatgttttggatgatagaagggacattccatcttcttacaagcagggaagtaacggcagagctgactactggaaggtggtgctggtggtgcaactggttttggagacagtactggaattcttctactcacatgagtgaagggacaatctggtttagtacactttgcatcatatttacaatttgggtgaacaaacaaacatttttcagcaaatttacaattggggaaggctttgcagggtgagatggggtgatggtaggcacactcatccccatttttacaagcaggccagtacttgcagcgctccaaaagtttttctggtttctgtgccacactcagttcactcatctcagcgttagaaaagctaccatttgggtcctcaagctgcctgctcagcaagtgcaactgctgtgggtggaggagacctctgagtcccttgtttgaggctgcagtttggtttacgggtttcattccttcaaagcacatgtcctcctcttgatctgacatgtatcctggggggctggggacaccatccagcgtcactataaacttgggacttgcaggtttatctggttgtacaagatctcgtgtctgcataaggtgtcctgaaagtacccgaagggaatctgcagtcttcatccccgactcttggtttggtgccactactacttcctcagacagctttggcttcttcagaataaatgatcttgtgtctgcatggaccatggattccatgtcatagtaatcttgactcatctgcagagtttctgccattactgggtcgatttgcagtcgggataataattgcctctgttgagttccttgatttttttctacagaatctccttttgtttcctcttctttaatggggggacttattctgggggtcctactttgtccctggaccacttctgctagcaattcttcttgagaagttcgagttctgggagcaactggaagtgtctgtttctgtggaactgtagagtagttagttgtttttgttacggattcttgagcttcagatatagccttcaaaatcagattcttgttagcttgtttagaaggtggaagagaaggtctcctttcaggctttgcaggcacagacacactgctggagatgcttcctgttcgagacccgtaatcatcatcttcttcctcctcttctccatcatgattgaatttttttactttaacaactgaacttaccacaggcaactttctcttccgaaagttttcatcctccatactcattttctccgagttgtttctaaagaacggactatacgtttcttctaagctgttaagcacctctggttcacacaaacgtcctgtttcatatacccaactactctgcatatcaagctgcttggcagcatgaatactattctgctgctgttgaaattgcaacctgtttaaatgaacaccactatctgcatttctacttgcaggtggtcgataaatttcaatagaagggcgagaagaaccatatgtaagtgtcactgtaggttttttctgagataagggattctcctgcacaaagttgaggtcttcgtcaatgagatcatctggttctggcttaatatcaatcacatcttcagagggtgctggctccctcaaaggtttcactgttgacattagtcgggttgcagctccatcatcgtaagtctgtctgacatttgtggtttttgactcctgcgaacttgtagaaactctggaatctcttttttcaggtctcgcgctaggaatggcaagtggtggcactgcagcttcatgcctcctctcatctccccgactgaaattgctcttgtttgaaggcacgttactatcaaagatgttggtatcagaagacttcagactagagggttcagttgtaacagagcgaagtttatctaatacaccatgaagccatacggtgaatcgaattgtgttgttccctagaaacagggacagatcctctgtcatttggtcctgacttttcttgttggccaccatcaccataatgtaatcaggaagttcttcatcaacataagctcctaattcttgtaatttccccttaatggcactccggatcttgcggctgatctcggtgccgatctccatggctctgcggcgtgcgggaactcagcactgcgcggcgcttggcttacccggaggctgccgcggactcctaccccgcagccgggacaccaccgcctcc

SEQ ID NO: 13624 - RNA, 16904 nt, Homo sapiens
  source 1..16904: mol_type = other RNA
gctgggattacaggcatgagccaccataataaggattctgatgaacatttgattccttggactactgttatactcaaaagccttccttaatcttctaattgtcaccctaaatatcctaaaatttctgtcttcctagtagttcttcatagtcctaaaaatttgtcagagagaaaggtaaatcaagaaacatgattttcaaatgatttaaggtggtactagggtttaggatttcctttgctttttatcatttaacacactgcttatcatacagctggaagtgctctgggccagtgtctctacttcgagggaagaaggaggtagtgagacagaaggaaatagcacaattcctggccctgacagaagggtgttcaggagacctgctctcctctcactttattccatctcatctggacctgtggcttccaatccacatctctttcctttaatatcctgcattggctaggctgtataaatcctttggtgcatcgaaaaactaagtgcattttttgtttttgtgattatgcaatacttataggaaaagttataattttagaatatttaagtacacttacatttttgagaaaaagactattgaaatgtttgtgccatgtcaaatttcagttgaacattttgggtattcttaatataagaccaggccaggcaccgtggctcaggccgggcacagtggctcacacctataatcccagcacttagggaggccaaggcgggaagatcacctgaagtcaggagttcaagaccagcctggctaacaaggtgaaactctgtctctactaaaaatacaaaaattagccgggcgtggtggctggcgcttgtaatcccagctacttgggaggctgagacaggagaatcacttgaacctgggaagcagaggttgtggtgagctgagatcgcaccattgcactccagcctgggcaacaaagagcgaaactccgtctcaaaaaaataaaaaataaaccctagaattatagtatgttagaattggaagggaagaattgtctaaggttattctagctaataagcaacagacttggaaaggaaaaggtcctgacaaagctaagcctcccgttcaggtttcctgactcgtgaattcagtgctgctgccactacacgatgcatgctctttgtatcaagggtgagacagcattacacatacatagaaaattatctatttaaactctatttgaacttttgatgagtttgtctccccctcccccactccttttcagaataacttgacgtttacaggtaccatcagtggtgatgtctgtgtgtggaaagatcacatattgtgtagaatcgtggcgagagctcacaacgggcctgtgtttgccatgtacaccaccctgcgagatggacttatcgtgactgggggaaaggaaaggccgtgagtcctctttcttttcacagaatatttatgcatttgtgacctacctgaggtttgcagttaattattctagttgtttctaggctacacagagtgtcctctccgaccttcctcctcatatgcttctcctttattaccttttatgtgccttctatttgattctcatttctggtcttaattcacttccaatttttttcatgttggggtgatactttttctgaggtgtggataggtagttgtcctacaagttgagttacttttcttaatgtctgtatgcctgtgtatgatttgctgagtaggaggcccatgggggaatctggagccagggttgtattttgactgcctgctctctttttgttcagaatggattctaaggagtagaatgcacattgttgctttagaaaaggatgagggaactagagagaactgccttgtttccttttgcttgaggcaaatttaaactgttttatacaagacctcaaaatttgagaagaggtctcttctgagtgattttcaaatctcccaacagtaaccagatacttatgatttgatttgtcaccaacatagtcatatgcatgttgaaacatgacatgtaggccaggcacagtggctcacacctgtaatcttatcactttgggaggctgaggcaggtggatcgcttgagcccaggagttcaagaccagcctgggcaacatggtgaaaccccatcgctataaaaaacaacaattagccgggtgtggtggcacatgcctgtagtccctgctactcaggaggctgaggtgggaggatcacttgagcctggggaggtcaaggctttagtgagctgtgatggtgccactgcactccagcctgggtgacagagtgagaccccatttaaaaaacaaaaacaaaaacaaaaaaaaatgtgacatatagttgactaagaagtacatttcaatacaggattgaaagaacccacatatgttaattaaacacaagcgcagaatttgtgccttttacataaaggaagaatgcacataggcatgctttcagacaagcaattcatctagcagaaaaggaaggaatacatttttcagcccttccaggaataaaatccataaatgggctctatttcgtcctccaacacttgtatttcccacgtcatttactcctgcacacccccactcactagaagcctgctaaactgttccagtgagatattttaacacctgatagggaataaatatgcttctgttttggccttcaaaaataagctctgggccagttgcagtggctcacgcctgtaatcccaacactttgggaggccgaggtgggcggatcacgaggtcaggagtttgggatcagcctggccaatatggtgaaactccatctctactaaaaatacaaaaattagccaggcatggtgcctgtaatcccagctacttgggaggctgaaggagaagaatcgcttgaacctgggaggcacaggttgcagtgagccgagatcacaccactgcactccaggccaggtgacagagcgacactctgtctcaaaaaaataaataaatcaactctgtagcatagcatttgtaattctattattttgccttacatttccattatccttttaataaaattgtttttttacatcttcctaatcaagaagtattatgaggccaggcacagtggctcatacctggaatcccagcactttgggaggccgaggcaggcagatcacctgaggtcaaggtatttgagaccagcctggccaacatggtgaaaccccatctctactaaaaatacagaaattagctgggtgtggtggtgcacacctgtaatgctagctactcgggaggctgaggtaggagaatcgcttgaacctgggaggcagaggttgcaataagcctagatcatgccactgcactcaagcctgggagacagagcgagactacatcttaaaaaaaaaaaaaaaagtattatgagagaggataatgtattgtaatgtattgtagaggctaaataaaattatgctcatgtcagaaaaaaagagtatttctcaaaataaaattcactgaaactggatgtttattttgactgagatatagtatatcctcaaattgccatagaaagtttacaagaatattagaggtaaattataaatatcagggcctttttaaaaaaaaaagattctgcttataacttggtatttgtttataataaaaattatagtagccaataatgaacacttactctggcttggttatttacttaggtcaaaagaaggaggagcggttaaactgtgggatcaggaactgaggcggtgccgtgccttcaggcttgagacaggacaagccacagattgtgttcgttctgtgtgcagaggcaaagtaagatgttccatgagctgatacagtgcagcagaaaacagaaagtggttattactgtgattccctcaccctttgcagcctaatgaacaatacttaataatgcataacgatggatttgcttgccaacattactctgtctttgctgctttctttgccaaagttagcaccagtgtggtgcataagctaggaagctattctgtctaaatactgtatgtaaacctccaatattttctagaatctgccaatttaacaactctagtagacataattgaaagcccttggcagttgactcatattaggacagctgtctccattttttaaaaaaacacacattccctagataaaacgtgcagtaaacaaacaatgaaatactactcagccataaaaaataatgaaattctgtcattcttggtggcaacatggatgagactggaggacatgatgtgaagtgaaataagccaggcacagaaagataaatacatgttctcactcctgtgcagaaactaaaaaagttgatcccacagaggtggagagtagaatagtggttactggaggcggacaagggggagggggagggggatagggaaggactggttaaaggatacaagtttacacagccagataggaatagtatgttttagtattctgtagtactgtaggatgactatagttaagaatcacgtatttatgtattttcaggtatttacaagagaggattttgaaagtttccatcacaaagaaatgataaatgtctgaggtgatggttatgcgtattaccctatgccctatagatatgtataattatgtgtcaatttcaaaataaaaattcaaaactacaactcctatgaaaatttttgagcgtgtttgtacttattaagtgtatttataaatcatacggatattatcttcagcctgcatattaaattgtagttaagcttttactttttaactaaaaaataaattctattattttttcctatatcccactgcactgaccccagtttggaaatcctaagattatcaaataaaaactttgattattgaagaatccaggtgtactgccacagaaaagttctattctgtagcatggactctaatatgtaatctagcccattgtgcttacagatagatgtgtgcctgtagtcatagaaaaatttgcatgagctaatgactgccttgctactagattagctcaaagcaaaaagttctctgaaagcaggtcaatagggtcatttttatattatgaagaagaaaagcagctgttgtattacattcactgtattggtcctgcttgtgtttcagggcaagatccttgttgggacaaggaatgctgaaataatcgaagttggagagaaaaatgcagcttgtaatattttagttaacggtcatgtggatgggccaatctggggactagcaacacatccttccagggattttttcctttctgctgcagaagatgggacagtgagactttgggatattgctgataaagtaagtacagataatttttttaaaagaggttacaacttctaaaaagaaaagttggaagttctaaattgctagtacttaaagaactgccagaattctgttgagcattttgaggggaaactggtataatttagaagtacttcacttaatgtttcctatgactctttttttttttttttttaaatgcagaagatgttaaacaaagtgaatttgggacatgctgctcgtactgtgtgttacagccctgaaggggacatggtggctattggaatgaaaaatggagaatttatcattttactagtgagttctctaaaaatatggggaaagaagagagacaggagatgtgcaatccatgatatcaggttagtgaacaaatggaatagagtttctagtatatacttgatttaacttccatttgtaaaattttccatagccttgccttcaaaaagaggtccccagggcctgtagcatttcccgtattataaattgtatgctaaaatatggctgtttgtatactacttaattcttcttgctaaattataaacccactgggcaccaactataatagcaagtactagtaggtaatgtttgatgaattcatgttaacacttagccatgtccattaagttcatcccaccaagaggtatctcccactgtaatacaagagagctatctgcccttcaaaagttgtcaccctggaaaactaaagttgtgatttcaaacatatcttctcttagtaacctcagtttgggaatatgtagttcattaatttaatcaatacctattgattaaatgttccagaatccaaattaatttaaatgtttcttaaacctttgtttttcagtgcttaagcatttttcaacagtggctaccatttacggagtacttccgtgtgatcagtagataagattattgaatctaggtctgtcaaaagcttgtacacttttcatcagtaaaatccttttacaaatgaaaccttcctcagaacttcaatatataaaatagtaacagtggcttcccttagcttttacatgtctctatcgtacctcagtaagactcatgggccatttcaagagactgaattgtcccatatgactccaaagattgctaggcaaatagcatttcactttgtcttttaaataagttcttcaggccgggcgcggtggctcatgcctgtaatcccagcactttgggaggccgaggcaggcagatcacctgaagtcaggagtactcgaccagcctggccaacatagtgaaaccccatctcaactaaaaatacaaaaatcagccgggcgtggtggcaggcgcctgtaatcccagctactcagggggctgaaacaggagaatcgcttgaacccgggaggcggaggttgcgccatcgcactccagcctgggagacaagagcgagacttcgtctcaaaaaaaaaaaattcttcttccaagattcaagttgtgtcatttcaccttaataactggaggttagttaagctgggctgtgttctttgcttaatattaagacaacgttttttccagatggaagaaaactatcttaatgaattgttagcttattaattatgtaatgctaatggcttttaaaagctgagatgttctgactgggtgttgtggctcacacctgtaatcccagtaccttgggaggccaagggggaaggattgcttgaggccaggagtttgggaccatagtgagaccccgcctctatttaaaaaattaaattttgttttgttttgttttgagttggagttttgctcttgttgcccatgctgaagtgcaatggtgcaatctcagctcaccacaacctgtgcctcctgggttcaagcgattctcctgcttcagcctcccgagtagatgggattacaggcgtgcaccaccatgcctggctaattttgtatttttagtagagacagggtttctctatgttggtcaggctggtctcaaactctcgacctcaggtgatctgcccgcctccgcttcccaaagttctgggattataggtgtgagccactgggcctggcctaagaaagtttttttaagccattagacgtttttaaaggaattgggagatgacaattggggaaatatttaaaatttaagtaaaatataaagcttccttatttcatgtaacccagacaatctcagtatacatgatcagttgtgtctgacaggtaaatctatttgaggccttatcacacgttacttttaagaactagaaaggaaaagtcactgatcttaagtatttataatacttcatgtggtctaatactttttacgttttgttttgattcagatttagtccggattcccggtatctggcagtaggttctagtgagaactcagtggatttttatgacctaacgctgggccccactcttaacagaatcagctactgcaaagacattccaagctttgtcattcaaatggacttctctgcagatagcagttatctccaggtacagtaccaatactgtatacccaggtggcaagttcttctgcttttacatttcgtgttagtgaatgcatttaaagttcctgagctccagagctccagcttctcaactcctccctttgtaccttctgacctacagctcccctttcctcccccacttatcagagcttttctcctattaagtttttgtagtgatcttttgcatacttaataatgttagacatgtaaatcaagtagcaatatgctagtattctgtaaaccccctgtggattttgtctctcacctaatggaattcttgtcccattttaatctgatgaaaaaggtctctagtggctgctataaacggcatgtctatgaagtgccttcaggaaaacatcttatggatcatgccgctattgacagaattacttgggctacatggactaggtaaatacttatatattcacaaggcaagaactgactttgaaggccagttagaaaatcctatttctgaactgttagagccattccaataaggaatagtaattgagtttcaagtttttgttaccatattttgaaatggtatgttcatgttgggacccctttttattgaatatatttccatgttttatcagtttccatgatttatcaagttttttttttaaggaaatcaaagttttaactttaaagataccctgatatttttcttaatgctaaatttaatgactggcaaaaaggtattgggtgctgttaagcaactgttattaattctctatctaaaggaatgctatcttgaatctattagaagtcaaagcttccaaatttgttcaaatttcctggctgtatgacaggtaaccatgactatccatttttttggccaatgaaaaatgccatcaaattcctgtatcagccaggcatatagtggctcatgcctgtaatctctgatgtagcaggccgaggtgggaggatcacttgagcctagaagttttgataccagcctgggcaacatagcaagaccccatctctgaaatttttttaattcctatgtcataagtcatttttatttttgtagagatagggatctcacaatattgcccaggctggtctcaaactcttggcctcaagcagtcctcctgcctcagcctcccaaaatgttgggattactggtatgtgctgctggacccagccaagtagcacttttaatttgaaaaatagttctatcagttttcagtcaggcgcggtggctcagcctgtaatcccagcactttgggaggccgagcgggggtgatcacctgaggtcgggagttcgagactagcctgaccaacatggagaaaccctgtctctactaaaaatacaaaataagccgggcatgttagcgcatgcctgtgatcccagctactcgggaggctgaggcaggagaattgcttgaacccaggaggcagaggttgcggtgagccgagatcatgccattgcactccagcctgggtaacaagagcgaaaactccgtctcaaaaaaaaaaaaagaaaaaatagttctatcagttttcataaagtactactttaatcttaaaaagattaatctagaaacccttcaaattataaaatgtcatttttaaaaggcaggagttgatatcctgatgaaattcaggtctccaaacaacttaccataatttacttcctgtattttaagtaacatgatagggtacttagagattaattgccaagaaactttttgaatatagtcaacctgcccgcacttgccatgatgagttttcttttgttccttccctctagtattctaggagatgaggttttgggaatctggtccagacatgctgagaaagctgatgtcaactgtgcctgtgtatctcattcaggaatcagtcttgttacaggagatgactttggcatggttaagttatttgacttcccatgtccagaaaaatttgtaagtttgtgttttgtttactattatcagtttactcctaattttgatgtcttatcatcagcacttttccccatatatttaaaatgttttgtcctaatttctaaatttttccccaaactttctaaatctatttactttgaaataaaagctattagaaacaaatcctctccctcgagtaataccatctttggaaccatcctacaaaagctgtaattagcttttcaccaaacctataatcagttatcaaatttcaaatgcttttccttagagaaaaatggtcagagtacctggagacatctgactgcccacacagcctggttttgcagatccactactcatgctgaaaagcattctaatcactggctgcggtgctaactccctactctctccacagctcttgtcatagagattatagttcctaataagagcctttgacttctgtgtgcaccaaatgccctgagcttgtctgtcattgttttttaggcaaaacacaaaaggttcttgggtcattcgccccatgtgacaaatattcgatttaccagtggtgatcgacatgttgttagtgctggaggtgatgactgcaggttagtaactttctcagcccatgaagagcagactatgttactagttaagagacttaatacaacaactcctacagctttggtttatgaaatcagctagtcaacattagtagaaggtagtataaccagatggctcttcagaatctcatatttatgcaaatacagaataaaaggagttaaagaggaaaaatattacacatgtaacctgaaagcacaactgaaaaatattaaactgttatgaaaatctaaaaacataattaactccctgcaattttcttctctgattgcagcttatttgtctggaaatgtgtacatacacctcactgagagatgctgagatgactacagaaattaactttgagaccagaattacagagaagaaaaaccaaaacccaaccctgcatggtcaagtggtgctaacccaagactgtaacagggagaaatgcccagaatcatcaaaatagtgaaagactgatctgttcaaaatatttgctatatgcactgggtataatccgtaatccatacactgccagataatgccatttcaaggaaggatcgaatacttgatggtaaaggccaagtccccctgtattgggaagtgtgtgatttcggcagacctgctgggaaaatttagggtagagcactctttacagaagaactcaaaaacccaatttggataattttcattatctttttagcaaaatggtttcttaatgtttatattttattttcaaggttcattgtttaatgaaatattttattcttgcatttccataaggaaagggaaagtcatgatcatcctaaaggatcacagtttttaaaaggcaaacattttccctaaggaaacagacacaagctttcctagagaatatgatgttttttaggcattaataaggtccttttttataaaggacacttttctcctagtagttttgaattcaggaacagatccaaagttagcagtatatggctgctacatttccattttcattttcgagccatcagtttatgttcagatgccatctctgtaatcgcacatttaaaacataactgtagcctcactaatggaaaagtagtatgatgaacaatcattcccaatggtgtacaatgtaagggttttagggagcaacagtatttaactggaagaaagaattgcatatttaatgtagtctaatatatacacatttgtttaacatgtaaacaaaagtgttaaattcacatatacaacattatacaatttaatcactcttggaataaaatttttatagccttttttctattgggaaaatttgtttagatgtgtgccactccataggtttatttccaaaatgaatgagcccaactccatttgtaaaaacttgtcagttagaattcctttttttagtggattagggctgaattcttagatccttatttcttttcactttaaatgctgccaaagatcactactcatcattcaggaattcgctgtctagcctatctgtagtttcctgaagattgaaaattatgtagactgctatttaaaaatatatttttctaagtgtgaggtttaagatgctgtattgaccctatgagtttttaatgtgttaattatctttatagcataatagatcgctttaggttcctggaatcccatttggtctgacaggatatatgaagattcttaatacctattttctgtgtctaatacttggttaatactaaaaatagaaatgactaaattacatcacagaaagcataaccagtgattgaacctggtagttttaaagctctaaatagctgtggctgaaggactgattatggggctaagaagcttgaaacgtaagttggtacttgttcatcagtggattctcctaaattaagccaaattttgaaatacatgactattaagtttctactcatgtatttacagtcagtcaataaattaaaggaggaaaaaaatccctgaacaacctgcccataaaaagaaaaatactctacatttgagcctgctgcagttttaaattttccctctgggtcaagtttgccagcttttggctacagagaaattatatttccattacagtgcaggtagaaactctgtaaccttaagcatgtaaactacatagaataaaactgtttccactgcatttctgtccttcaaagtggccaacctgattaagtcagccttaatcactgctgctgtcagtttcacgactaaaggtcatattgactaagtagtcatcagctgaccacctcgctgtatcagccagcaacgaggggaaggtgaagaaacatgataggccatatagaatctgccctatgtttacttttttaacccagataattatttttgtgtgcagtatctaagctcctgattgtgtaacctgggacttctggcaccttttgttccattcattttatgtataaaatgcatgccaaagcacactgtgccctctggtacccttgcttccaatcgccaaccatgctcatttccttcctttttttgtggtccctttttgtggtgatcattttaaaccacgtcatccaacaaatgttttatggtcaaccttagcttgttcataagccatagcaactgaaagattaaactcttaaatatgtgtctgggcagtggctattaaatagcaaaaaacaatcagattttagtattttattatttccttgtaaaatggctgaactaaattaaacccttgtttcccatttgttctataatttatagtgaaactgagaacaaaactatctttataaatgatagctaaaagtatttccagatatttaaacaatttaaaataaatttcttctgcagagatgcaaagcatctcaacactggaatgaacaaatgccttaaattcaatggagtaaacctttagaatgaagaggaactgtcatttcacccaagccgaagacaacagccttatgcacttgtgtgctctgtctttgctgcttctcgtgtttcaagcctttcctgtgggatcagcacagcaaagtgcaacttaccaaatggtttaatgactggttaattctttcttctcccaatggaaaagcaatggcaacacaacagtagactgctggcttgacaatcttaaacgtgagcctttgcacatgtaggtttatcatcatttgagtatacgactaagcaagtcaatgaactttttttttttttttagcagtttaatttggtcctgagaatgttgcagtctttattaccccttttgcattaatccacttttctaaccaccttttaagctttaatttttaacactatacaccaagtctttgaaatcagtgatctgttatttaactctaaagcatttgacacttcttgccttaacagttttaaaaaccacacacaaaaaaactctgtaagtaatacagtaggccaaaagtttcatcctatctatcttgcagtttacctatctgatctgatctctgtaattatagttctgtcatttaaaatatactatttaaatctaatttttacatttcaaaaattatcttcagtagtaactaagtatattttctgtggattctgagaatgttatttttcagaatgtgagaatatatatgtacatttataatcttgtgactttaaagtctgttttcagatacagtatgtaaatacttgtaaaaaaatttgtataattttgtgataatgtagtttcccaaaaaaattatttagaaggcattatgttattagtaaatgagagcactgtatagaactgttcctattttctgcacttgccattccagctgcctccactgtccatacccacctcattcatcctgtcacagaaggcaggaaaactgggaactttaccaaagtagcactcagcctgagaggcctgtataatcatgcttttcaaactaaattcacttaaaaattaaaaagcagaattgaatattttaagcagcctcagtacctttggccaatgctgttttcatggtggattatgaacattatataatctttgggaaaagtgaaagtagtacaatttttagaataatgacaactgcctcactgcatctctccactcacacagcaaccgtgtagccccctaagctgcagtaccatgactaaccatgatgtcaatttcatatgctgatcctcacaacagcagtgcacaaacatgccccaaatattttaacagaatttagctcttccttaagctgtcttttcatagtaaaaacaaaacaaaaacacccaatgttaaaaccacataataaacttacaaacttgaaaaattagacacttcagatagataggcaataaaacttcatattatgaaagcaatatattccaagtttcaaagatttgacaagttctgtagagtatctttcatcagtacatgaaaacttccaaactgcatgatcttctgccaggcaggactgggtgctattcgctggtttgaggtcgaatccatttcaaggcatgtcgtggtgggacattaatggtgggatggtagaatgtgcagtccggtcttgtacattgagtgttaaacctacaatgttttggatgatagaagggacattccatcttcttacaagcagggaagtaacggcagagctgactactggaaggtggtgctggtggtgcaactggttttggagacagtactggaattcttctactcacatgagtgaagggacaatctggtttagtacactttgcatcatatttacaatttgggtgaacaaacaaacatttttcagcaaatttacaattggggaaggctttgcagggtgagatggggtgatggtaggcacactcatccccatttttacaagcaggccagtacttgcagcgctccaaaagtttttctggtttctgtgccacactcagttcactcatctcagcgttagaaaagctaccatttgggtcctcaagctgcctgctcagcaagtgcaactgctgtgggtggaggagacctctgagtcccttgtttgaggctgcagtttggtttacgggtttcattccttcaaagcacatgtcctcctcttgatctgacatgtatcctggggggctggggacaccatccagcgtcactataaacttgggacttgcaggtttatctggttgtacaagatctcgtgtctgcataaggtgtcctgaaagtacccgaagggaatctgcagtcttcatccccgactcttggtttggtgccactactacttcctcagacagctttggcttcttcagaataaatgatcttgtgtctgcatggaccatggattccatgtcatagtaatcttgactcatctgcagagtttctgccattactgggtcgatttgcagtcgggataataattgcctctgttgagttccttgatttttttctacagaatctccttttgtttcctcttctttaatggggggacttattctgggggtcctactttgtccctggaccacttctgctagcaattcttcttgagaagttcgagttctgggagcaactggaagtgtctgtttctgtggaactgtagagtagttagttgtttttgttacggattcttgagcttcagatatagccttcaaaatcagattcttgttagcttgtttagaaggtggaagagaaggtctcctttcaggctttgcaggcacagacacactgctggagatgcttcctgttcgagacccgtaatcatcatcttcttcctcctcttctccatcatgattgaatttttttactttaacaactgaacttaccacaggcaactttctcttccgaaagttttcatcctccatactcattttctccgagttgtttctaaagaacggactatacgtttcttctaagctgttaagcacctctggttcacacaaacgtcctgtttcatatacccaactactctgcatatcaagctgcttggcagcatgaatactattctgctgctgttgaaattgcaacctgtttaaatgaacaccactatctgcatttctacttgcaggtggtcgataaatttcaatagaagggcgagaagaaccatatgtaagtgtcactgtaggttttttctgagataagggattctcctgcacaaagttgaggtcttcgtcaatgagatcatctggttctggcttaatatcaatcacatcttcagagggtgctggctccctcaaaggtttcactgttgacattagtcgggttgcagctccatcatcgtaagtctgtctgacatttgtggtttttgactcctgcgaacttgtagaaactctggaatctcttttttcaggtctcgcgctaggaatggcaagtggtggcactgcagcttcatgcctcctctcatctccccgactgaaattgctcttgtttgaaggcacgttactatcaaagatgttggtatcagaagacttcagactagagggttcagttgtaacagagcgaagtttatctaatacaccatgaagccatacggtgaatcgaattgtgttgttccctagaaacagggacagatcctctgtcatttggtcctgacttttcttgttggccaccatcaccataatgtaatcaggaagttcttcatcaacataagctcctaattcttgtaatttccccttaatggcactctcccgcagcggatccaaagcggcgccgtgcgccgcggtggtggctccagccgggcctgcgcctgtccttccatttcccggcggctacttcagccgcagccacgctccg

SEQ ID NO: 13625 - RNA, 17109 nt, Homo sapiens
  source 1..17109: mol_type = other RNA
gctgggattacaggcatgagccaccataataaggattctgatgaacatttgattccttggactactgttatactcaaaagccttccttaatcttctaattgtcaccctaaatatcctaaaatttctgtcttcctagtagttcttcatagtcctaaaaatttgtcagagagaaaggtaaatcaagaaacatgattttcaaatgatttaaggtggtactagggtttaggatttcctttgctttttatcatttaacacactgcttatcatacagctggaagtgctctgggccagtgtctctacttcgagggaagaaggaggtagtgagacagaaggaaatagcacaattcctggccctgacagaagggtgttcaggagacctgctctcctctcactttattccatctcatctggacctgtggcttccaatccacatctctttcctttaatatcctgcattggctaggctgtataaatcctttggtgcatcgaaaaactaagtgcattttttgtttttgtgattatgcaatacttataggaaaagttataattttagaatatttaagtacacttacatttttgagaaaaagactattgaaatgtttgtgccatgtcaaatttcagttgaacattttgggtattcttaatataagaccaggccaggcaccgtggctcaggccgggcacagtggctcacacctataatcccagcacttagggaggccaaggcgggaagatcacctgaagtcaggagttcaagaccagcctggctaacaaggtgaaactctgtctctactaaaaatacaaaaattagccgggcgtggtggctggcgcttgtaatcccagctacttgggaggctgagacaggagaatcacttgaacctgggaagcagaggttgtggtgagctgagatcgcaccattgcactccagcctgggcaacaaagagcgaaactccgtctcaaaaaaataaaaaataaaccctagaattatagtatgttagaattggaagggaagaattgtctaaggttattctagctaataagcaacagacttggaaaggaaaaggtcctgacaaagctaagcctcccgttcaggtttcctgactcgtgaattcagtgctgctgccactacacgatgcatgctctttgtatcaagggtgagacagcattacacatacatagaaaattatctatttaaactctatttgaacttttgatgagtttgtctccccctcccccactccttttcagaataacttgacgtttacaggtaccatcagtggtgatgtctgtgtgtggaaagatcacatattgtgtagaatcgtggcgagagctcacaacgggcctgtgtttgccatgtacaccaccctgcgagatggacttatcgtgactgggggaaaggaaaggccgtgagtcctctttcttttcacagaatatttatgcatttgtgacctacctgaggtttgcagttaattattctagttgtttctaggctacacagagtgtcctctccgaccttcctcctcatatgcttctcctttattaccttttatgtgccttctatttgattctcatttctggtcttaattcacttccaatttttttcatgttggggtgatactttttctgaggtgtggataggtagttgtcctacaagttgagttacttttcttaatgtctgtatgcctgtgtatgatttgctgagtaggaggcccatgggggaatctggagccagggttgtattttgactgcctgctctctttttgttcagaatggattctaaggagtagaatgcacattgttgctttagaaaaggatgagggaactagagagaactgccttgtttccttttgcttgaggcaaatttaaactgttttatacaagacctcaaaatttgagaagaggtctcttctgagtgattttcaaatctcccaacagtaaccagatacttatgatttgatttgtcaccaacatagtcatatgcatgttgaaacatgacatgtaggccaggcacagtggctcacacctgtaatcttatcactttgggaggctgaggcaggtggatcgcttgagcccaggagttcaagaccagcctgggcaacatggtgaaaccccatcgctataaaaaacaacaattagccgggtgtggtggcacatgcctgtagtccctgctactcaggaggctgaggtgggaggatcacttgagcctggggaggtcaaggctttagtgagctgtgatggtgccactgcactccagcctgggtgacagagtgagaccccatttaaaaaacaaaaacaaaaacaaaaaaaaatgtgacatatagttgactaagaagtacatttcaatacaggattgaaagaacccacatatgttaattaaacacaagcgcagaatttgtgccttttacataaaggaagaatgcacataggcatgctttcagacaagcaattcatctagcagaaaaggaaggaatacatttttcagcccttccaggaataaaatccataaatgggctctatttcgtcctccaacacttgtatttcccacgtcatttactcctgcacacccccactcactagaagcctgctaaactgttccagtgagatattttaacacctgatagggaataaatatgcttctgttttggccttcaaaaataagctctgggccagttgcagtggctcacgcctgtaatcccaacactttgggaggccgaggtgggcggatcacgaggtcaggagtttgggatcagcctggccaatatggtgaaactccatctctactaaaaatacaaaaattagccaggcatggtgcctgtaatcccagctacttgggaggctgaaggagaagaatcgcttgaacctgggaggcacaggttgcagtgagccgagatcacaccactgcactccaggccaggtgacagagcgacactctgtctcaaaaaaataaataaatcaactctgtagcatagcatttgtaattctattattttgccttacatttccattatccttttaataaaattgtttttttacatcttcctaatcaagaagtattatgaggccaggcacagtggctcatacctggaatcccagcactttgggaggccgaggcaggcagatcacctgaggtcaaggtatttgagaccagcctggccaacatggtgaaaccccatctctactaaaaatacagaaattagctgggtgtggtggtgcacacctgtaatgctagctactcgggaggctgaggtaggagaatcgcttgaacctgggaggcagaggttgcaataagcctagatcatgccactgcactcaagcctgggagacagagcgagactacatcttaaaaaaaaaaaaaaaagtattatgagagaggataatgtattgtaatgtattgtagaggctaaataaaattatgctcatgtcagaaaaaaagagtatttctcaaaataaaattcactgaaactggatgtttattttgactgagatatagtatatcctcaaattgccatagaaagtttacaagaatattagaggtaaattataaatatcagggcctttttaaaaaaaaaagattctgcttataacttggtatttgtttataataaaaattatagtagccaataatgaacacttactctggcttggttatttacttaggtcaaaagaaggaggagcggttaaactgtgggatcaggaactgaggcggtgccgtgccttcaggcttgagacaggacaagccacagattgtgttcgttctgtgtgcagaggcaaagtaagatgttccatgagctgatacagtgcagcagaaaacagaaagtggttattactgtgattccctcaccctttgcagcctaatgaacaatacttaataatgcataacgatggatttgcttgccaacattactctgtctttgctgctttctttgccaaagttagcaccagtgtggtgcataagctaggaagctattctgtctaaatactgtatgtaaacctccaatattttctagaatctgccaatttaacaactctagtagacataattgaaagcccttggcagttgactcatattaggacagctgtctccattttttaaaaaaacacacattccctagataaaacgtgcagtaaacaaacaatgaaatactactcagccataaaaaataatgaaattctgtcattcttggtggcaacatggatgagactggaggacatgatgtgaagtgaaataagccaggcacagaaagataaatacatgttctcactcctgtgcagaaactaaaaaagttgatcccacagaggtggagagtagaatagtggttactggaggcggacaagggggagggggagggggatagggaaggactggttaaaggatacaagtttacacagccagataggaatagtatgttttagtattctgtagtactgtaggatgactatagttaagaatcacgtatttatgtattttcaggtatttacaagagaggattttgaaagtttccatcacaaagaaatgataaatgtctgaggtgatggttatgcgtattaccctatgccctatagatatgtataattatgtgtcaatttcaaaataaaaattcaaaactacaactcctatgaaaatttttgagcgtgtttgtacttattaagtgtatttataaatcatacggatattatcttcagcctgcatattaaattgtagttaagcttttactttttaactaaaaaataaattctattattttttcctatatcccactgcactgaccccagtttggaaatcctaagattatcaaataaaaactttgattattgaagaatccaggtgtactgccacagaaaagttctattctgtagcatggactctaatatgtaatctagcccattgtgcttacagatagatgtgtgcctgtagtcatagaaaaatttgcatgagctaatgactgccttgctactagattagctcaaagcaaaaagttctctgaaagcaggtcaatagggtcatttttatattatgaagaagaaaagcagctgttgtattacattcactgtattggtcctgcttgtgtttcagggcaagatccttgttgggacaaggaatgctgaaataatcgaagttggagagaaaaatgcagcttgtaatattttagttaacggtcatgtggatgggccaatctggggactagcaacacatccttccagggattttttcctttctgctgcagaagatgggacagtgagactttgggatattgctgataaagtaagtacagataatttttttaaaagaggttacaacttctaaaaagaaaagttggaagttctaaattgctagtacttaaagaactgccagaattctgttgagcattttgaggggaaactggtataatttagaagtacttcacttaatgtttcctatgactctttttttttttttttttaaatgcagaagatgttaaacaaagtgaatttgggacatgctgctcgtactgtgtgttacagccctgaaggggacatggtggctattggaatgaaaaatggagaatttatcattttactagtgagttctctaaaaatatggggaaagaagagagacaggagatgtgcaatccatgatatcaggttagtgaacaaatggaatagagtttctagtatatacttgatttaacttccatttgtaaaattttccatagccttgccttcaaaaagaggtccccagggcctgtagcatttcccgtattataaattgtatgctaaaatatggctgtttgtatactacttaattcttcttgctaaattataaacccactgggcaccaactataatagcaagtactagtaggtaatgtttgatgaattcatgttaacacttagccatgtccattaagttcatcccaccaagaggtatctcccactgtaatacaagagagctatctgcccttcaaaagttgtcaccctggaaaactaaagttgtgatttcaaacatatcttctcttagtaacctcagtttgggaatatgtagttcattaatttaatcaatacctattgattaaatgttccagaatccaaattaatttaaatgtttcttaaacctttgtttttcagtgcttaagcatttttcaacagtggctaccatttacggagtacttccgtgtgatcagtagataagattattgaatctaggtctgtcaaaagcttgtacacttttcatcagtaaaatccttttacaaatgaaaccttcctcagaacttcaatatataaaatagtaacagtggcttcccttagcttttacatgtctctatcgtacctcagtaagactcatgggccatttcaagagactgaattgtcccatatgactccaaagattgctaggcaaatagcatttcactttgtcttttaaataagttcttcaggccgggcgcggtggctcatgcctgtaatcccagcactttgggaggccgaggcaggcagatcacctgaagtcaggagtactcgaccagcctggccaacatagtgaaaccccatctcaactaaaaatacaaaaatcagccgggcgtggtggcaggcgcctgtaatcccagctactcagggggctgaaacaggagaatcgcttgaacccgggaggcggaggttgcgccatcgcactccagcctgggagacaagagcgagacttcgtctcaaaaaaaaaaaattcttcttccaagattcaagttgtgtcatttcaccttaataactggaggttagttaagctgggctgtgttctttgcttaatattaagacaacgttttttccagatggaagaaaactatcttaatgaattgttagcttattaattatgtaatgctaatggcttttaaaagctgagatgttctgactgggtgttgtggctcacacctgtaatcccagtaccttgggaggccaagggggaaggattgcttgaggccaggagtttgggaccatagtgagaccccgcctctatttaaaaaattaaattttgttttgttttgttttgagttggagttttgctcttgttgcccatgctgaagtgcaatggtgcaatctcagctcaccacaacctgtgcctcctgggttcaagcgattctcctgcttcagcctcccgagtagatgggattacaggcgtgcaccaccatgcctggctaattttgtatttttagtagagacagggtttctctatgttggtcaggctggtctcaaactctcgacctcaggtgatctgcccgcctccgcttcccaaagttctgggattataggtgtgagccactgggcctggcctaagaaagtttttttaagccattagacgtttttaaaggaattgggagatgacaattggggaaatatttaaaatttaagtaaaatataaagcttccttatttcatgtaacccagacaatctcagtatacatgatcagttgtgtctgacaggtaaatctatttgaggccttatcacacgttacttttaagaactagaaaggaaaagtcactgatcttaagtatttataatacttcatgtggtctaatactttttacgttttgttttgattcagatttagtccggattcccggtatctggcagtaggttctagtgagaactcagtggatttttatgacctaacgctgggccccactcttaacagaatcagctactgcaaagacattccaagctttgtcattcaaatggacttctctgcagatagcagttatctccaggtacagtaccaatactgtatacccaggtggcaagttcttctgcttttacatttcgtgttagtgaatgcatttaaagttcctgagctccagagctccagcttctcaactcctccctttgtaccttctgacctacagctcccctttcctcccccacttatcagagcttttctcctattaagtttttgtagtgatcttttgcatacttaataatgttagacatgtaaatcaagtagcaatatgctagtattctgtaaaccccctgtggattttgtctctcacctaatggaattcttgtcccattttaatctgatgaaaaaggtctctagtggctgctataaacggcatgtctatgaagtgccttcaggaaaacatcttatggatcatgccgctattgacagaattacttgggctacatggactaggtaaatacttatatattcacaaggcaagaactgactttgaaggccagttagaaaatcctatttctgaactgttagagccattccaataaggaatagtaattgagtttcaagtttttgttaccatattttgaaatggtatgttcatgttgggacccctttttattgaatatatttccatgttttatcagtttccatgatttatcaagttttttttttaaggaaatcaaagttttaactttaaagataccctgatatttttcttaatgctaaatttaatgactggcaaaaaggtattgggtgctgttaagcaactgttattaattctctatctaaaggaatgctatcttgaatctattagaagtcaaagcttccaaatttgttcaaatttcctggctgtatgacaggtaaccatgactatccatttttttggccaatgaaaaatgccatcaaattcctgtatcagccaggcatatagtggctcatgcctgtaatctctgatgtagcaggccgaggtgggaggatcacttgagcctagaagttttgataccagcctgggcaacatagcaagaccccatctctgaaatttttttaattcctatgtcataagtcatttttatttttgtagagatagggatctcacaatattgcccaggctggtctcaaactcttggcctcaagcagtcctcctgcctcagcctcccaaaatgttgggattactggtatgtgctgctggacccagccaagtagcacttttaatttgaaaaatagttctatcagttttcagtcaggcgcggtggctcagcctgtaatcccagcactttgggaggccgagcgggggtgatcacctgaggtcgggagttcgagactagcctgaccaacatggagaaaccctgtctctactaaaaatacaaaataagccgggcatgttagcgcatgcctgtgatcccagctactcgggaggctgaggcaggagaattgcttgaacccaggaggcagaggttgcggtgagccgagatcatgccattgcactccagcctgggtaacaagagcgaaaactccgtctcaaaaaaaaaaaaagaaaaaatagttctatcagttttcataaagtactactttaatcttaaaaagattaatctagaaacccttcaaattataaaatgtcatttttaaaaggcaggagttgatatcctgatgaaattcaggtctccaaacaacttaccataatttacttcctgtattttaagtaacatgatagggtacttagagattaattgccaagaaactttttgaatatagtcaacctgcccgcacttgccatgatgagttttcttttgttccttccctctagtattctaggagatgaggttttgggaatctggtccagacatgctgagaaagctgatgtcaactgtgcctgtgtatctcattcaggaatcagtcttgttacaggagatgactttggcatggttaagttatttgacttcccatgtccagaaaaatttgtaagtttgtgttttgtttactattatcagtttactcctaattttgatgtcttatcatcagcacttttccccatatatttaaaatgttttgtcctaatttctaaatttttccccaaactttctaaatctatttactttgaaataaaagctattagaaacaaatcctctccctcgagtaataccatctttggaaccatcctacaaaagctgtaattagcttttcaccaaacctataatcagttatcaaatttcaaatgcttttccttagagaaaaatggtcagagtacctggagacatctgactgcccacacagcctggttttgcagatccactactcatgctgaaaagcattctaatcactggctgcggtgctaactccctactctctccacagctcttgtcatagagattatagttcctaataagagcctttgacttctgtgtgcaccaaatgccctgagcttgtctgtcattgttttttaggcaaaacacaaaaggttcttgggtcattcgccccatgtgacaaatattcgatttaccagtggtgatcgacatgttgttagtgctggaggtgatgactgcaggttagtaactttctcagcccatgaagagcagactatgttactagttaagagacttaatacaacaactcctacagctttggtttatgaaatcagctagtcaacattagtagaaggtagtataaccagatggctcttcagaatctcatatttatgcaaatacagaataaaaggagttaaagaggaaaaatattacacatgtaacctgaaagcacaactgaaaaatattaaactgttatgaaaatctaaaaacataattaactccctgcaattttcttctctgattgcagcttatttgtctggaaatgtgtacatacacctcactgagagatgctgagatgactacagaaattaactttgagaccagaattacagagaagaaaaaccaaaacccaaccctgcatggtcaagtggtgctaacccaagactgtaacagggagaaatgcccagaatcatcaaaatagtgaaagactgatctgttcaaaatatttgctatatgcactgggtataatccgtaatccatacactgccagataatgccatttcaaggaaggatcgaatacttgatggtaaaggccaagtccccctgtattgggaagtgtgtgatttcggcagacctgctgggaaaatttagggtagagcactctttacagaagaactcaaaaacccaatttggataattttcattatctttttagcaaaatggtttcttaatgtttatattttattttcaaggttcattgtttaatgaaatattttattcttgcatttccataaggaaagggaaagtcatgatcatcctaaaggatcacagtttttaaaaggcaaacattttccctaaggaaacagacacaagctttcctagagaatatgatgttttttaggcattaataaggtccttttttataaaggacacttttctcctagtagttttgaattcaggaacagatccaaagttagcagtatatggctgctacatttccattttcattttcgagccatcagtttatgttcagatgccatctctgtaatcgcacatttaaaacataactgtagcctcactaatggaaaagtagtatgatgaacaatcattcccaatggtgtacaatgtaagggttttagggagcaacagtatttaactggaagaaagaattgcatatttaatgtagtctaatatatacacatttgtttaacatgtaaacaaaagtgttaaattcacatatacaacattatacaatttaatcactcttggaataaaatttttatagccttttttctattgggaaaatttgtttagatgtgtgccactccataggtttatttccaaaatgaatgagcccaactccatttgtaaaaacttgtcagttagaattcctttttttagtggattagggctgaattcttagatccttatttcttttcactttaaatgctgccaaagatcactactcatcattcaggaattcgctgtctagcctatctgtagtttcctgaagattgaaaattatgtagactgctatttaaaaatatatttttctaagtgtgaggtttaagatgctgtattgaccctatgagtttttaatgtgttaattatctttatagcataatagatcgctttaggttcctggaatcccatttggtctgacaggatatatgaagattcttaatacctattttctgtgtctaatacttggttaatactaaaaatagaaatgactaaattacatcacagaaagcataaccagtgattgaacctggtagttttaaagctctaaatagctgtggctgaaggactgattatggggctaagaagcttgaaacgtaagttggtacttgttcatcagtggattctcctaaattaagccaaattttgaaatacatgactattaagtttctactcatgtatttacagtcagtcaataaattaaaggaggaaaaaaatccctgaacaacctgcccataaaaagaaaaatactctacatttgagcctgctgcagttttaaattttccctctgggtcaagtttgccagcttttggctacagagaaattatatttccattacagtgcaggtagaaactctgtaaccttaagcatgtaaactacatagaataaaactgtttccactgcatttctgtccttcaaagtggccaacctgattaagtcagccttaatcactgctgctgtcagtttcacgactaaaggtcatattgactaagtagtcatcagctgaccacctcgctgtatcagccagcaacgaggggaaggtgaagaaacatgataggccatatagaatctgccctatgtttacttttttaacccagataattatttttgtgtgcagtatctaagctcctgattgtgtaacctgggacttctggcaccttttgttccattcattttatgtataaaatgcatgccaaagcacactgtgccctctggtacccttgcttccaatcgccaaccatgctcatttccttcctttttttgtggtccctttttgtggtgatcattttaaaccacgtcatccaacaaatgttttatggtcaaccttagcttgttcataagccatagcaactgaaagattaaactcttaaatatgtgtctgggcagtggctattaaatagcaaaaaacaatcagattttagtattttattatttccttgtaaaatggctgaactaaattaaacccttgtttcccatttgttctataatttatagtgaaactgagaacaaaactatctttataaatgatagctaaaagtatttccagatatttaaacaatttaaaataaatttcttctgcagagatgcaaagcatctcaacactggaatgaacaaatgccttaaattcaatggagtaaacctttagaatgaagaggaactgtcatttcacccaagccgaagacaacagccttatgcacttgtgtgctctgtctttgctgcttctcgtgtttcaagcctttcctgtgggatcagcacagcaaagtgcaacttaccaaatggtttaatgactggttaattctttcttctcccaatggaaaagcaatggcaacacaacagtagactgctggcttgacaatcttaaacgtgagcctttgcacatgtaggtttatcatcatttgagtatacgactaagcaagtcaatgaactttttttttttttttagcagtttaatttggtcctgagaatgttgcagtctttattaccccttttgcattaatccacttttctaaccaccttttaagctttaatttttaacactatacaccaagtctttgaaatcagtgatctgttatttaactctaaagcatttgacacttcttgccttaacagttttaaaaaccacacacaaaaaaactctgtaagtaatacagtaggccaaaagtttcatcctatctatcttgcagtttacctatctgatctgatctctgtaattatagttctgtcatttaaaatatactatttaaatctaatttttacatttcaaaaattatcttcagtagtaactaagtatattttctgtggattctgagaatgttatttttcagaatgtgagaatatatatgtacatttataatcttgtgactttaaagtctgttttcagatacagtatgtaaatacttgtaaaaaaatttgtataattttgtgataatgtagtttcccaaaaaaattatttagaaggcattatgttattagtaaatgagagcactgtatagaactgttcctattttctgcacttgccattccagctgcctccactgtccatacccacctcattcatcctgtcacagaaggcaggaaaactgggaactttaccaaagtagcactcagcctgagaggcctgtataatcatgcttttcaaactaaattcacttaaaaattaaaaagcagaattgaatattttaagcagcctcagtacctttggccaatgctgttttcatggtggattatgaacattatataatctttgggaaaagtgaaagtagtacaatttttagaataatgacaactgcctcactgcatctctccactcacacagcaaccgtgtagccccctaagctgcagtaccatgactaaccatgatgtcaatttcatatgctgatcctcacaacagcagtgcacaaacatgccccaaatattttaacagaatttagctcttccttaagctgtcttttcatagtaaaaacaaaacaaaaacacccaatgttaaaaccacataataaacttacaaacttgaaaaattagacacttcagatagataggcaataaaacttcatattatgaaagcaatatattccaagtttcaaagatttgacaagttctgtagagtatctttcatcagtacatgaaaacttccaaactgcatgatcttctgccaggcaggactgggtgctattcgctggtttgaggtcgaatccatttcaaggcatgtcgtggtgggacattaatggtgggatggtagaatgtgcagtccggtcttgtacattgagtgttaaacctacaatgttttggatgatagaagggacattccatcttcttacaagcagggaagtaacggcagagctgactactggaaggtggtgctggtggtgcaactggttttggagacagtactggaattcttctactcacatgagtgaagggacaatctggtttagtacactttgcatcatatttacaatttgggtgaacaaacaaacatttttcagcaaatttacaattggggaaggctttgcagggtgagatggggtgatggtaggcacactcatccccatttttacaagcaggccagtacttgcagcgctccaaaagtttttctggtttctgtgccacactcagttcactcatctcagcgttagaaaagctaccatttgggtcctcaagctgcctgctcagcaagtgcaactgctgtgggtggaggagacctctgagtcccttgtttgaggctgcagtttggtttacgggtttcattccttcaaagcacatgtcctcctcttgatctgacatgtatcctggggggctggggacaccatccagcgtcactataaacttgggacttgcaggtttatctggttgtacaagatctcgtgtctgcataaggtgtcctgaaagtacccgaagggaatctgcagtcttcatccccgactcttggtttggtgccactactacttcctcagacagctttggcttcttcagaataaatgatcttgtgtctgcatggaccatggattccatgtcatagtaatcttgactcatctgcagagtttctgccattactgggtcgatttgcagtcgggataataattgcctctgttgagttccttgatttttttctacagaatctccttttgtttcctcttctttaatggggggacttattctgggggtcctactttgtccctggaccacttctgctagcaattcttcttgagaagttcgagttctgggagcaactggaagtgtctgtttctgtggaactgtagagtagttagttgtttttgttacggattcttgagcttcagatatagccttcaaaatcagattcttgttagcttgtttagaaggtggaagagaaggtctcctttcaggctttgcaggcacagacacactgctggagatgcttcctgttcgagacccgtaatcatcatcttcttcctcctcttctccatcatgattgaatttttttactttaacaactgaacttaccacaggcaactttctcttccgaaagttttcatcctccatactcattttctccgagttgtttctaaagaacggactatacgtttcttctaagctgttaagcacctctggttcacacaaacgtcctgtttcatatacccaactactctgcatatcaagctgcttggcagcatgaatactattctgctgctgttgaaattgcaacctgtttaaatgaacaccactatctgcatttctacttgcaggtggtcgataaatttcaatagaagggcgagaagaaccatatgtaagtgtcactgtaggttttttctgagataagggattctcctgcacaaagttgaggtcttcgtcaatgagatcatctggttctggcttaatatcaatcacatcttcagagggtgctggctccctcaaaggtttcactgttgacattagtcgggttgcagctccatcatcgtaagtctgtctgacatttgtggtttttgactcctgcgaacttgtagaaactctggaatctcttttttcaggtctcgcgctaggaatggcaagtggtggcactgcagcttcatgcctcctctcatctccccgactgaaattgctcttgtttgaaggcacgttactatcaaagatgttggtatcagaagacttcagactagagggttcagttgtaacagagcgaagtttatctaatacaccatgaagccatacggtgaatcgaattgtgttgttccctagaaacagggacagatcctctgtcatttggtcctgacttttcttgttggccaccatcaccataatgtaatcaggaagttcttcatctatttaaaaggaaaggtagatcaaaactttgtttcctcaaaactttcttcttaaagttgatgtgcttgaaaatatagatgtagctctaagctttagagtcgcagagctctactggaattacattggacaagatggcttagctttaatttttttctcttcattccacaggtatttcaaatacaacataagctcctaattcttgtaatttccccttaatggcactccggatcttgcggctgatctcggtgccgatctccatggctctgcggcgtgcgggaactcagcactgcgcggcgcttggcttacccggaggctgccgcggactcctaccccgcagccgggacaccaccgcctcc

SEQ ID NO: 13626 - RNA, 16738 nt, Homo sapiens
  source 1..16738: mol_type = other RNA
gctgggattacaggcatgagccaccataataaggattctgatgaacatttgattccttggactactgttatactcaaaagccttccttaatcttctaattgtcaccctaaatatcctaaaatttctgtcttcctagtagttcttcatagtcctaaaaatttgtcagagagaaaggtaaatcaagaaacatgattttcaaatgatttaaggtggtactagggtttaggatttcctttgctttttatcatttaacacactgcttatcatacagctggaagtgctctgggccagtgtctctacttcgagggaagaaggaggtagtgagacagaaggaaatagcacaattcctggccctgacagaagggtgttcaggagacctgctctcctctcactttattccatctcatctggacctgtggcttccaatccacatctctttcctttaatatcctgcattggctaggctgtataaatcctttggtgcatcgaaaaactaagtgcattttttgtttttgtgattatgcaatacttataggaaaagttataattttagaatatttaagtacacttacatttttgagaaaaagactattgaaatgtttgtgccatgtcaaatttcagttgaacattttgggtattcttaatataagaccaggccaggcaccgtggctcaggccgggcacagtggctcacacctataatcccagcacttagggaggccaaggcgggaagatcacctgaagtcaggagttcaagaccagcctggctaacaaggtgaaactctgtctctactaaaaatacaaaaattagccgggcgtggtggctggcgcttgtaatcccagctacttgggaggctgagacaggagaatcacttgaacctgggaagcagaggttgtggtgagctgagatcgcaccattgcactccagcctgggcaacaaagagcgaaactccgtctcaaaaaaataaaaaataaaccctagaattatagtatgttagaattggaagggaagaattgtctaaggttattctagctaataagcaacagacttggaaaggaaaaggtcctgacaaagctaagcctcccgttcaggtttcctgactcgtgaattcagtgctgctgccactacacgatgcatgctctttgtatcaagggtgagacagcattacacatacatagaaaattatctatttaaactctatttgaacttttgatgagtttgtctccccctcccccactccttttcagaataacttgacgtttacaggtaccatcagtggtgatgtctgtgtgtggaaagatcacatattgtgtagaatcgtggcgagagctcacaacgggcctgtgtttgccatgtacaccaccctgcgagatggacttatcgtgactgggggaaaggaaaggccgtgagtcctctttcttttcacagaatatttatgcatttgtgacctacctgaggtttgcagttaattattctagttgtttctaggctacacagagtgtcctctccgaccttcctcctcatatgcttctcctttattaccttttatgtgccttctatttgattctcatttctggtcttaattcacttccaatttttttcatgttggggtgatactttttctgaggtgtggataggtagttgtcctacaagttgagttacttttcttaatgtctgtatgcctgtgtatgatttgctgagtaggaggcccatgggggaatctggagccagggttgtattttgactgcctgctctctttttgttcagaatggattctaaggagtagaatgcacattgttgctttagaaaaggatgagggaactagagagaactgccttgtttccttttgcttgaggcaaatttaaactgttttatacaagacctcaaaatttgagaagaggtctcttctgagtgattttcaaatctcccaacagtaaccagatacttatgatttgatttgtcaccaacatagtcatatgcatgttgaaacatgacatgtaggccaggcacagtggctcacacctgtaatcttatcactttgggaggctgaggcaggtggatcgcttgagcccaggagttcaagaccagcctgggcaacatggtgaaaccccatcgctataaaaaacaacaattagccgggtgtggtggcacatgcctgtagtccctgctactcaggaggctgaggtgggaggatcacttgagcctggggaggtcaaggctttagtgagctgtgatggtgccactgcactccagcctgggtgacagagtgagaccccatttaaaaaacaaaaacaaaaacaaaaaaaaatgtgacatatagttgactaagaagtacatttcaatacaggattgaaagaacccacatatgttaattaaacacaagcgcagaatttgtgccttttacataaaggaagaatgcacataggcatgctttcagacaagcaattcatctagcagaaaaggaaggaatacatttttcagcccttccaggaataaaatccataaatgggctctatttcgtcctccaacacttgtatttcccacgtcatttactcctgcacacccccactcactagaagcctgctaaactgttccagtgagatattttaacacctgatagggaataaatatgcttctgttttggccttcaaaaataagctctgggccagttgcagtggctcacgcctgtaatcccaacactttgggaggccgaggtgggcggatcacgaggtcaggagtttgggatcagcctggccaatatggtgaaactccatctctactaaaaatacaaaaattagccaggcatggtgcctgtaatcccagctacttgggaggctgaaggagaagaatcgcttgaacctgggaggcacaggttgcagtgagccgagatcacaccactgcactccaggccaggtgacagagcgacactctgtctcaaaaaaataaataaatcaactctgtagcatagcatttgtaattctattattttgccttacatttccattatccttttaataaaattgtttttttacatcttcctaatcaagaagtattatgaggccaggcacagtggctcatacctggaatcccagcactttgggaggccgaggcaggcagatcacctgaggtcaaggtatttgagaccagcctggccaacatggtgaaaccccatctctactaaaaatacagaaattagctgggtgtggtggtgcacacctgtaatgctagctactcgggaggctgaggtaggagaatcgcttgaacctgggaggcagaggttgcaataagcctagatcatgccactgcactcaagcctgggagacagagcgagactacatcttaaaaaaaaaaaaaaaagtattatgagagaggataatgtattgtaatgtattgtagaggctaaataaaattatgctcatgtcagaaaaaaagagtatttctcaaaataaaattcactgaaactggatgtttattttgactgagatatagtatatcctcaaattgccatagaaagtttacaagaatattagaggtaaattataaatatcagggcctttttaaaaaaaaaagattctgcttataacttggtatttgtttataataaaaattatagtagccaataatgaacacttactctggcttggttatttacttaggtcaaaagaaggaggagcggttaaactgtgggatcaggaactgaggcggtgccgtgccttcaggcttgagacaggacaagccacagattgtgttcgttctgtgtgcagaggcaaagtaagatgttccatgagctgatacagtgcagcagaaaacagaaagtggttattactgtgattccctcaccctttgcagcctaatgaacaatacttaataatgcataacgatggatttgcttgccaacattactctgtctttgctgctttctttgccaaagttagcaccagtgtggtgcataagctaggaagctattctgtctaaatactgtatgtaaacctccaatattttctagaatctgccaatttaacaactctagtagacataattgaaagcccttggcagttgactcatattaggacagctgtctccattttttaaaaaaacacacattccctagataaaacgtgcagtaaacaaacaatgaaatactactcagccataaaaaataatgaaattctgtcattcttggtggcaacatggatgagactggaggacatgatgtgaagtgaaataagccaggcacagaaagataaatacatgttctcactcctgtgcagaaactaaaaaagttgatcccacagaggtggagagtagaatagtggttactggaggcggacaagggggagggggagggggatagggaaggactggttaaaggatacaagtttacacagccagataggaatagtatgttttagtattctgtagtactgtaggatgactatagttaagaatcacgtatttatgtattttcaggtatttacaagagaggattttgaaagtttccatcacaaagaaatgataaatgtctgaggtgatggttatgcgtattaccctatgccctatagatatgtataattatgtgtcaatttcaaaataaaaattcaaaactacaactcctatgaaaatttttgagcgtgtttgtacttattaagtgtatttataaatcatacggatattatcttcagcctgcatattaaattgtagttaagcttttactttttaactaaaaaataaattctattattttttcctatatcccactgcactgaccccagtttggaaatcctaagattatcaaataaaaactttgattattgaagaatccaggtgtactgccacagaaaagttctattctgtagcatggactctaatatgtaatctagcccattgtgcttacagatagatgtgtgcctgtagtcatagaaaaatttgcatgagctaatgactgccttgctactagattagctcaaagcaaaaagttctctgaaagcaggtcaatagggtcatttttatattatgaagaagaaaagcagctgttgtattacattcactgtattggtcctgcttgtgtttcagggcaagatccttgttgggacaaggaatgctgaaataatcgaagttggagagaaaaatgcagcttgtaatattttagttaacggtcatgtggatgggccaatctggggactagcaacacatccttccagggattttttcctttctgctgcagaagatgggacagtgagactttgggatattgctgataaagtaagtacagataatttttttaaaagaggttacaacttctaaaaagaaaagttggaagttctaaattgctagtacttaaagaactgccagaattctgttgagcattttgaggggaaactggtataatttagaagtacttcacttaatgtttcctatgactctttttttttttttttttaaatgcagaagatgttaaacaaagtgaatttgggacatgctgctcgtactgtgtgttacagccctgaaggggacatggtggctattggaatgaaaaatggagaatttatcattttactagtgagttctctaaaaatatggggaaagaagagagacaggagatgtgcaatccatgatatcaggttagtgaacaaatggaatagagtttctagtatatacttgatttaacttccatttgtaaaattttccatagccttgccttcaaaaagaggtccccagggcctgtagcatttcccgtattataaattgtatgctaaaatatggctgtttgtatactacttaattcttcttgctaaattataaacccactgggcaccaactataatagcaagtactagtaggtaatgtttgatgaattcatgttaacacttagccatgtccattaagttcatcccaccaagaggtatctcccactgtaatacaagagagctatctgcccttcaaaagttgtcaccctggaaaactaaagttgtgatttcaaacatatcttctcttagtaacctcagtttgggaatatgtagttcattaatttaatcaatacctattgattaaatgttccagaatccaaattaatttaaatgtttcttaaacctttgtttttcagtgcttaagcatttttcaacagtggctaccatttacggagtacttccgtgtgatcagtagataagattattgaatctaggtctgtcaaaagcttgtacacttttcatcagtaaaatccttttacaaatgaaaccttcctcagaacttcaatatataaaatagtaacagtggcttcccttagcttttacatgtctctatcgtacctcagtaagactcatgggccatttcaagagactgaattgtcccatatgactccaaagattgctaggcaaatagcatttcactttgtcttttaaataagttcttcaggccgggcgcggtggctcatgcctgtaatcccagcactttgggaggccgaggcaggcagatcacctgaagtcaggagtactcgaccagcctggccaacatagtgaaaccccatctcaactaaaaatacaaaaatcagccgggcgtggtggcaggcgcctgtaatcccagctactcagggggctgaaacaggagaatcgcttgaacccgggaggcggaggttgcgccatcgcactccagcctgggagacaagagcgagacttcgtctcaaaaaaaaaaaattcttcttccaagattcaagttgtgtcatttcaccttaataactggaggttagttaagctgggctgtgttctttgcttaatattaagacaacgttttttccagatggaagaaaactatcttaatgaattgttagcttattaattatgtaatgctaatggcttttaaaagctgagatgttctgactgggtgttgtggctcacacctgtaatcccagtaccttgggaggccaagggggaaggattgcttgaggccaggagtttgggaccatagtgagaccccgcctctatttaaaaaattaaattttgttttgttttgttttgagttggagttttgctcttgttgcccatgctgaagtgcaatggtgcaatctcagctcaccacaacctgtgcctcctgggttcaagcgattctcctgcttcagcctcccgagtagatgggattacaggcgtgcaccaccatgcctggctaattttgtatttttagtagagacagggtttctctatgttggtcaggctggtctcaaactctcgacctcaggtgatctgcccgcctccgcttcccaaagttctgggattataggtgtgagccactgggcctggcctaagaaagtttttttaagccattagacgtttttaaaggaattgggagatgacaattggggaaatatttaaaatttaagtaaaatataaagcttccttatttcatgtaacccagacaatctcagtatacatgatcagttgtgtctgacaggtaaatctatttgaggccttatcacacgttacttttaagaactagaaaggaaaagtcactgatcttaagtatttataatacttcatgtggtctaatactttttacgttttgttttgattcagatttagtccggattcccggtatctggcagtaggttctagtgagaactcagtggatttttatgacctaacgctgggccccactcttaacagaatcagctactgcaaagacattccaagctttgtcattcaaatggacttctctgcagatagcagttatctccaggtacagtaccaatactgtatacccaggtggcaagttcttctgcttttacatttcgtgttagtgaatgcatttaaagttcctgagctccagagctccagcttctcaactcctccctttgtaccttctgacctacagctcccctttcctcccccacttatcagagcttttctcctattaagtttttgtagtgatcttttgcatacttaataatgttagacatgtaaatcaagtagcaatatgctagtattctgtaaaccccctgtggattttgtctctcacctaatggaattcttgtcccattttaatctgatgaaaaaggtctctagtggctgctataaacggcatgtctatgaagtgccttcaggaaaacatcttatggatcatgccgctattgacagaattacttgggctacatggactaggtaaatacttatatattcacaaggcaagaactgactttgaaggccagttagaaaatcctatttctgaactgttagagccattccaataaggaatagtaattgagtttcaagtttttgttaccatattttgaaatggtatgttcatgttgggacccctttttattgaatatatttccatgttttatcagtttccatgatttatcaagttttttttttaaggaaatcaaagttttaactttaaagataccctgatatttttcttaatgctaaatttaatgactggcaaaaaggtattgggtgctgttaagcaactgttattaattctctatctaaaggaatgctatcttgaatctattagaagtcaaagcttccaaatttgttcaaatttcctggctgtatgacaggtaaccatgactatccatttttttggccaatgaaaaatgccatcaaattcctgtatcagccaggcatatagtggctcatgcctgtaatctctgatgtagcaggccgaggtgggaggatcacttgagcctagaagttttgataccagcctgggcaacatagcaagaccccatctctgaaatttttttaattcctatgtcataagtcatttttatttttgtagagatagggatctcacaatattgcccaggctggtctcaaactcttggcctcaagcagtcctcctgcctcagcctcccaaaatgttgggattactggtatgtgctgctggacccagccaagtagcacttttaatttgaaaaatagttctatcagttttcagtcaggcgcggtggctcagcctgtaatcccagcactttgggaggccgagcgggggtgatcacctgaggtcgggagttcgagactagcctgaccaacatggagaaaccctgtctctactaaaaatacaaaataagccgggcatgttagcgcatgcctgtgatcccagctactcgggaggctgaggcaggagaattgcttgaacccaggaggcagaggttgcggtgagccgagatcatgccattgcactccagcctgggtaacaagagcgaaaactccgtctcaaaaaaaaaaaaagaaaaaatagttctatcagttttcataaagtactactttaatcttaaaaagattaatctagaaacccttcaaattataaaatgtcatttttaaaaggcaggagttgatatcctgatgaaattcaggtctccaaacaacttaccataatttacttcctgtattttaagtaacatgatagggtacttagagattaattgccaagaaactttttgaatatagtcaacctgcccgcacttgccatgatgagttttcttttgttccttccctctagtattctaggagatgaggttttgggaatctggtccagacatgctgagaaagctgatgtcaactgtgcctgtgtatctcattcaggaatcagtcttgttacaggagatgactttggcatggttaagttatttgacttcccatgtccagaaaaatttgtaagtttgtgttttgtttactattatcagtttactcctaattttgatgtcttatcatcagcacttttccccatatatttaaaatgttttgtcctaatttctaaatttttccccaaactttctaaatctatttactttgaaataaaagctattagaaacaaatcctctccctcgagtaataccatctttggaaccatcctacaaaagctgtaattagcttttcaccaaacctataatcagttatcaaatttcaaatgcttttccttagagaaaaatggtcagagtacctggagacatctgactgcccacacagcctggttttgcagatccactactcatgctgaaaagcattctaatcactggctgcggtgctaactccctactctctccacagctcttgtcatagagattatagttcctaataagagcctttgacttctgtgtgcaccaaatgccctgagcttgtctgtcattgttttttaggcaaaacacaaaaggttcttgggtcattcgccccatgtgacaaatattcgatttaccagtggtgatcgacatgttgttagtgctggaggtgatgactgcaggttagtaactttctcagcccatgaagagcagactatgttactagttaagagacttaatacaacaactcctacagctttggtttatgaaatcagctagtcaacattagtagaaggtagtataaccagatggctcttcagaatctcatatttatgcaaatacagaataaaaggagttaaagaggaaaaatattacacatgtaacctgaaagcacaactgaaaaatattaaactgttatgaaaatctaaaaacataattaactccctgcaattttcttctctgattgcagcttatttgtctggaaatgtgtacatacacctcactgagagatgctgagatgactacagaaattaactttgagaccagaattacagagaagaaaaaccaaaacccaaccctgcatggtcaagtggtgctaacccaagactgtaacagggagaaatgcccagaatcatcaaaatagtgaaagactgatctgttcaaaatatttgctatatgcactgggtataatccgtaatccatacactgccagataatgccatttcaaggaaggatcgaatacttgatggtaaaggccaagtccccctgtattgggaagtgtgtgatttcggcagacctgctgggaaaatttagggtagagcactctttacagaagaactcaaaaacccaatttggataattttcattatctttttagcaaaatggtttcttaatgtttatattttattttcaaggttcattgtttaatgaaatattttattcttgcatttccataaggaaagggaaagtcatgatcatcctaaaggatcacagtttttaaaaggcaaacattttccctaaggaaacagacacaagctttcctagagaatatgatgttttttaggcattaataaggtccttttttataaaggacacttttctcctagtagttttgaattcaggaacagatccaaagttagcagtatatggctgctacatttccattttcattttcgagccatcagtttatgttcagatgccatctctgtaatcgcacatttaaaacataactgtagcctcactaatggaaaagtagtatgatgaacaatcattcccaatggtgtacaatgtaagggttttagggagcaacagtatttaactggaagaaagaattgcatatttaatgtagtctaatatatacacatttgtttaacatgtaaacaaaagtgttaaattcacatatacaacattatacaatttaatcactcttggaataaaatttttatagccttttttctattgggaaaatttgtttagatgtgtgccactccataggtttatttccaaaatgaatgagcccaactccatttgtaaaaacttgtcagttagaattcctttttttagtggattagggctgaattcttagatccttatttcttttcactttaaatgctgccaaagatcactactcatcattcaggaattcgctgtctagcctatctgtagtttcctgaagattgaaaattatgtagactgctatttaaaaatatatttttctaagtgtgaggtttaagatgctgtattgaccctatgagtttttaatgtgttaattatctttatagcataatagatcgctttaggttcctggaatcccatttggtctgacaggatatatgaagattcttaatacctattttctgtgtctaatacttggttaatactaaaaatagaaatgactaaattacatcacagaaagcataaccagtgattgaacctggtagttttaaagctctaaatagctgtggctgaaggactgattatggggctaagaagcttgaaacgtaagttggtacttgttcatcagtggattctcctaaattaagccaaattttgaaatacatgactattaagtttctactcatgtatttacagtcagtcaataaattaaaggaggaaaaaaatccctgaacaacctgcccataaaaagaaaaatactctacatttgagcctgctgcagttttaaattttccctctgggtcaagtttgccagcttttggctacagagaaattatatttccattacagtgcaggtagaaactctgtaaccttaagcatgtaaactacatagaataaaactgtttccactgcatttctgtccttcaaagtggccaacctgattaagtcagccttaatcactgctgctgtcagtttcacgactaaaggtcatattgactaagtagtcatcagctgaccacctcgctgtatcagccagcaacgaggggaaggtgaagaaacatgataggccatatagaatctgccctatgtttacttttttaacccagataattatttttgtgtgcagtatctaagctcctgattgtgtaacctgggacttctggcaccttttgttccattcattttatgtataaaatgcatgccaaagcacactgtgccctctggtacccttgcttccaatcgccaaccatgctcatttccttcctttttttgtggtccctttttgtggtgatcattttaaaccacgtcatccaacaaatgttttatggtcaaccttagcttgttcataagccatagcaactgaaagattaaactcttaaatatgtgtctgggcagtggctattaaatagcaaaaaacaatcagattttagtattttattatttccttgtaaaatggctgaactaaattaaacccttgtttcccatttgttctataatttatagtgaaactgagaacaaaactatctttataaatgatagctaaaagtatttccagatatttaaacaatttaaaataaatttcttctgcagagatgcaaagcatctcaacactggaatgaacaaatgccttaaattcaatggagtaaacctttagaatgaagaggaactgtcatttcacccaagccgaagacaacagccttatgcacttgtgtgctctgtctttgctgcttctcgtgtttcaagcctttcctgtgggatcagcacagcaaagtgcaacttaccaaatggtttaatgactggttaattctttcttctcccaatggaaaagcaatggcaacacaacagtagactgctggcttgacaatcttaaacgtgagcctttgcacatgtaggtttatcatcatttgagtatacgactaagcaagtcaatgaactttttttttttttttagcagtttaatttggtcctgagaatgttgcagtctttattaccccttttgcattaatccacttttctaaccaccttttaagctttaatttttaacactatacaccaagtctttgaaatcagtgatctgttatttaactctaaagcatttgacacttcttgccttaacagttttaaaaaccacacacaaaaaaactctgtaagtaatacagtaggccaaaagtttcatcctatctatcttgcagtttacctatctgatctgatctctgtaattatagttctgtcatttaaaatatactatttaaatctaatttttacatttcaaaaattatcttcagtagtaactaagtatattttctgtggattctgagaatgttatttttcagaatgtgagaatatatatgtacatttataatcttgtgactttaaagtctgttttcagatacagtatgtaaatacttgtaaaaaaatttgtataattttgtgataatgtagtttcccaaaaaaattatttagaaggcattatgttattagtaaatgagagcactgtatagaactgttcctattttctgcacttgccattccagctgcctccactgtccatacccacctcattcatcctgtcacagaaggcaggaaaactgggaactttaccaaagtagcactcagcctgagaggcctgtataatcatgcttttcaaactaaattcacttaaaaattaaaaagcagaattgaatattttaagcagcctcagtacctttggccaatgctgttttcatggtggattatgaacattatataatctttgggaaaagtgaaagtagtacaatttttagaataatgacaactgcctcactgcatctctccactcacacagcaaccgtgtagccccctaagctgcagtaccatgactaaccatgatgtcaatttcatatgctgatcctcacaacagcagtgcacaaacatgccccaaatattttaacagaatttagctcttccttaagctgtcttttcatagtaaaaacaaaacaaaaacacccaatgttaaaaccacataataaacttacaaacttgaaaaattagacacttcagatagataggcaataaaacttcatattatgaaagcaatatattccaagtttcaaagatttgacaagttctgtagagtatctttcatcagtacatgaaaacttccaaactgcatgatcttctgccaggcaggactgggtgctattcgctggtttgaggtcgaatccatttcaaggcatgtcgtggtgggacattaatggtgggatggtagaatgtgcagtccggtcttgtacattgagtgttaaacctacaatgttttggatgatagaagggacattccatcttcttacaagcagggaagtaacggcagagctgactactggaaggtggtgctggtggtgcaactggttttggagacagtactggaattcttctactcacatgagtgaagggacaatctggtttagtacactttgcatcatatttacaatttgggtgaacaaacaaacatttttcagcaaatttacaattggggaaggctttgcagggtgagatggggtgatggtaggcacactcatccccatttttacaagcaggccagtacttgcagcgctccaaaagtttttctggtttctgtgccacactcagttcactcatctcagcgttagaaaagctaccatttgggtcctcaagctgcctgctcagcaagtgcaactgctgtgggtggaggagacctctgagtcccttgtttgaggctgcagtttggtttacgggtttcattccttcaaagcacatgtcctcctcttgatctgacatgtatcctggggggctggggacaccatccagcgtcactataaacttgggacttgcaggtttatctggttgtacaagatctcgtgtctgcataaggtgtcctgaaagtacccgaagggaatctgcagtcttcatccccgactcttggtttggtgccactactacttcctcagacagctttggcttcttcagaataaatgatcttgtgtctgcatggaccatggattccatgtcatagtaatcttgatttttttctacagaatctccttttgtttcctcttctttaatggggggacttattctgggggtcctactttgtccctggaccacttctgctagcaattcttcttgagaagttcgagttctgggagcaactggaagtgtctgtttctgtggaactgtagagtagttagttgtttttgttacggattcttgagcttcagatatagccttcaaaatcagattcttgttagcttgtttagaaggtggaagagaaggtctcctttcaggctttgcaggcacagacacactgctggagatgcttcctgttcgagacccgtaatcatcatcttcttcctcctcttctccatcatgattgaatttttttactttaacaactgaacttaccacaggcaactttctcttccgaaagttttcatcctccatactcattttctccgagttgtttctaaagaacggactatacgtttcttctaagctgttaagcacctctggttcacacaaacgtcctgtttcatatacccaactactctgcatatcaagctgcttggcagcatgaatactattctgctgctgttgaaattgcaacctgtttaaatgaacaccactatctgcatttctacttgcaggtggtcgataaatttcaatagaagggcgagaagaaccatatgtaagtgtcactgtaggttttttctgagataagggattctcctgcacaaagttgaggtcttcgtcaatgagatcatctggttctggcttaatatcaatcacatcttcagagggtgctggctccctcaaaggtttcactgttgacattagtcgggttgcagctccatcatcgtaagtctgtctgacatttgtggtttttgactcctgcgaacttgtagaaactctggaatctcttttttcaggtctcgcgctaggaatggcaagtggtggcactgcagcttcatgcctcctctcatctccccgactgaaattgctcttgtttgaaggcacgttactatcaaagatgttggtatcagaagacttcagactagagggttcagttgtaacagagcgaagtttatctaatacaccatgaagccaacataagctcctaattcttgtaatttccccttaatggcactccggatcttgcggctgatctcggtgccgatctccatggctctgcggcgtgcgggaactcagcactgcgcggcgcttggcttacccggaggctgccgcggactcctaccccgcagccgggacaccaccgcctcc

SEQ ID NO: 13627 - RNA, 16853 nt, Homo sapiens
  source 1..16853: mol_type = other RNA
gctgggattacaggcatgagccaccataataaggattctgatgaacatttgattccttggactactgttatactcaaaagccttccttaatcttctaattgtcaccctaaatatcctaaaatttctgtcttcctagtagttcttcatagtcctaaaaatttgtcagagagaaaggtaaatcaagaaacatgattttcaaatgatttaaggtggtactagggtttaggatttcctttgctttttatcatttaacacactgcttatcatacagctggaagtgctctgggccagtgtctctacttcgagggaagaaggaggtagtgagacagaaggaaatagcacaattcctggccctgacagaagggtgttcaggagacctgctctcctctcactttattccatctcatctggacctgtggcttccaatccacatctctttcctttaatatcctgcattggctaggctgtataaatcctttggtgcatcgaaaaactaagtgcattttttgtttttgtgattatgcaatacttataggaaaagttataattttagaatatttaagtacacttacatttttgagaaaaagactattgaaatgtttgtgccatgtcaaatttcagttgaacattttgggtattcttaatataagaccaggccaggcaccgtggctcaggccgggcacagtggctcacacctataatcccagcacttagggaggccaaggcgggaagatcacctgaagtcaggagttcaagaccagcctggctaacaaggtgaaactctgtctctactaaaaatacaaaaattagccgggcgtggtggctggcgcttgtaatcccagctacttgggaggctgagacaggagaatcacttgaacctgggaagcagaggttgtggtgagctgagatcgcaccattgcactccagcctgggcaacaaagagcgaaactccgtctcaaaaaaataaaaaataaaccctagaattatagtatgttagaattggaagggaagaattgtctaaggttattctagctaataagcaacagacttggaaaggaaaaggtcctgacaaagctaagcctcccgttcaggtttcctgactcgtgaattcagtgctgctgccactacacgatgcatgctctttgtatcaagggtgagacagcattacacatacatagaaaattatctatttaaactctatttgaacttttgatgagtttgtctccccctcccccactccttttcagaataacttgacgtttacaggtaccatcagtggtgatgtctgtgtgtggaaagatcacatattgtgtagaatcgtggcgagagctcacaacgggcctgtgtttgccatgtacaccaccctgcgagatggacttatcgtgactgggggaaaggaaaggccgtgagtcctctttcttttcacagaatatttatgcatttgtgacctacctgaggtttgcagttaattattctagttgtttctaggctacacagagtgtcctctccgaccttcctcctcatatgcttctcctttattaccttttatgtgccttctatttgattctcatttctggtcttaattcacttccaatttttttcatgttggggtgatactttttctgaggtgtggataggtagttgtcctacaagttgagttacttttcttaatgtctgtatgcctgtgtatgatttgctgagtaggaggcccatgggggaatctggagccagggttgtattttgactgcctgctctctttttgttcagaatggattctaaggagtagaatgcacattgttgctttagaaaaggatgagggaactagagagaactgccttgtttccttttgcttgaggcaaatttaaactgttttatacaagacctcaaaatttgagaagaggtctcttctgagtgattttcaaatctcccaacagtaaccagatacttatgatttgatttgtcaccaacatagtcatatgcatgttgaaacatgacatgtaggccaggcacagtggctcacacctgtaatcttatcactttgggaggctgaggcaggtggatcgcttgagcccaggagttcaagaccagcctgggcaacatggtgaaaccccatcgctataaaaaacaacaattagccgggtgtggtggcacatgcctgtagtccctgctactcaggaggctgaggtgggaggatcacttgagcctggggaggtcaaggctttagtgagctgtgatggtgccactgcactccagcctgggtgacagagtgagaccccatttaaaaaacaaaaacaaaaacaaaaaaaaatgtgacatatagttgactaagaagtacatttcaatacaggattgaaagaacccacatatgttaattaaacacaagcgcagaatttgtgccttttacataaaggaagaatgcacataggcatgctttcagacaagcaattcatctagcagaaaaggaaggaatacatttttcagcccttccaggaataaaatccataaatgggctctatttcgtcctccaacacttgtatttcccacgtcatttactcctgcacacccccactcactagaagcctgctaaactgttccagtgagatattttaacacctgatagggaataaatatgcttctgttttggccttcaaaaataagctctgggccagttgcagtggctcacgcctgtaatcccaacactttgggaggccgaggtgggcggatcacgaggtcaggagtttgggatcagcctggccaatatggtgaaactccatctctactaaaaatacaaaaattagccaggcatggtgcctgtaatcccagctacttgggaggctgaaggagaagaatcgcttgaacctgggaggcacaggttgcagtgagccgagatcacaccactgcactccaggccaggtgacagagcgacactctgtctcaaaaaaataaataaatcaactctgtagcatagcatttgtaattctattattttgccttacatttccattatccttttaataaaattgtttttttacatcttcctaatcaagaagtattatgaggccaggcacagtggctcatacctggaatcccagcactttgggaggccgaggcaggcagatcacctgaggtcaaggtatttgagaccagcctggccaacatggtgaaaccccatctctactaaaaatacagaaattagctgggtgtggtggtgcacacctgtaatgctagctactcgggaggctgaggtaggagaatcgcttgaacctgggaggcagaggttgcaataagcctagatcatgccactgcactcaagcctgggagacagagcgagactacatcttaaaaaaaaaaaaaaaagtattatgagagaggataatgtattgtaatgtattgtagaggctaaataaaattatgctcatgtcagaaaaaaagagtatttctcaaaataaaattcactgaaactggatgtttattttgactgagatatagtatatcctcaaattgccatagaaagtttacaagaatattagaggtaaattataaatatcagggcctttttaaaaaaaaaagattctgcttataacttggtatttgtttataataaaaattatagtagccaataatgaacacttactctggcttggttatttacttaggtcaaaagaaggaggagcggttaaactgtgggatcaggaactgaggcggtgccgtgccttcaggcttgagacaggacaagccacagattgtgttcgttctgtgtgcagaggcaaagtaagatgttccatgagctgatacagtgcagcagaaaacagaaagtggttattactgtgattccctcaccctttgcagcctaatgaacaatacttaataatgcataacgatggatttgcttgccaacattactctgtctttgctgctttctttgccaaagttagcaccagtgtggtgcataagctaggaagctattctgtctaaatactgtatgtaaacctccaatattttctagaatctgccaatttaacaactctagtagacataattgaaagcccttggcagttgactcatattaggacagctgtctccattttttaaaaaaacacacattccctagataaaacgtgcagtaaacaaacaatgaaatactactcagccataaaaaataatgaaattctgtcattcttggtggcaacatggatgagactggaggacatgatgtgaagtgaaataagccaggcacagaaagataaatacatgttctcactcctgtgcagaaactaaaaaagttgatcccacagaggtggagagtagaatagtggttactggaggcggacaagggggagggggagggggatagggaaggactggttaaaggatacaagtttacacagccagataggaatagtatgttttagtattctgtagtactgtaggatgactatagttaagaatcacgtatttatgtattttcaggtatttacaagagaggattttgaaagtttccatcacaaagaaatgataaatgtctgaggtgatggttatgcgtattaccctatgccctatagatatgtataattatgtgtcaatttcaaaataaaaattcaaaactacaactcctatgaaaatttttgagcgtgtttgtacttattaagtgtatttataaatcatacggatattatcttcagcctgcatattaaattgtagttaagcttttactttttaactaaaaaataaattctattattttttcctatatcccactgcactgaccccagtttggaaatcctaagattatcaaataaaaactttgattattgaagaatccaggtgtactgccacagaaaagttctattctgtagcatggactctaatatgtaatctagcccattgtgcttacagatagatgtgtgcctgtagtcatagaaaaatttgcatgagctaatgactgccttgctactagattagctcaaagcaaaaagttctctgaaagcaggtcaatagggtcatttttatattatgaagaagaaaagcagctgttgtattacattcactgtattggtcctgcttgtgtttcagggcaagatccttgttgggacaaggaatgctgaaataatcgaagttggagagaaaaatgcagcttgtaatattttagttaacggtcatgtggatgggccaatctggggactagcaacacatccttccagggattttttcctttctgctgcagaagatgggacagtgagactttgggatattgctgataaagtaagtacagataatttttttaaaagaggttacaacttctaaaaagaaaagttggaagttctaaattgctagtacttaaagaactgccagaattctgttgagcattttgaggggaaactggtataatttagaagtacttcacttaatgtttcctatgactctttttttttttttttttaaatgcagaagatgttaaacaaagtgaatttgggacatgctgctcgtactgtgtgttacagccctgaaggggacatggtggctattggaatgaaaaatggagaatttatcattttactagtgagttctctaaaaatatggggaaagaagagagacaggagatgtgcaatccatgatatcaggttagtgaacaaatggaatagagtttctagtatatacttgatttaacttccatttgtaaaattttccatagccttgccttcaaaaagaggtccccagggcctgtagcatttcccgtattataaattgtatgctaaaatatggctgtttgtatactacttaattcttcttgctaaattataaacccactgggcaccaactataatagcaagtactagtaggtaatgtttgatgaattcatgttaacacttagccatgtccattaagttcatcccaccaagaggtatctcccactgtaatacaagagagctatctgcccttcaaaagttgtcaccctggaaaactaaagttgtgatttcaaacatatcttctcttagtaacctcagtttgggaatatgtagttcattaatttaatcaatacctattgattaaatgttccagaatccaaattaatttaaatgtttcttaaacctttgtttttcagtgcttaagcatttttcaacagtggctaccatttacggagtacttccgtgtgatcagtagataagattattgaatctaggtctgtcaaaagcttgtacacttttcatcagtaaaatccttttacaaatgaaaccttcctcagaacttcaatatataaaatagtaacagtggcttcccttagcttttacatgtctctatcgtacctcagtaagactcatgggccatttcaagagactgaattgtcccatatgactccaaagattgctaggcaaatagcatttcactttgtcttttaaataagttcttcaggccgggcgcggtggctcatgcctgtaatcccagcactttgggaggccgaggcaggcagatcacctgaagtcaggagtactcgaccagcctggccaacatagtgaaaccccatctcaactaaaaatacaaaaatcagccgggcgtggtggcaggcgcctgtaatcccagctactcagggggctgaaacaggagaatcgcttgaacccgggaggcggaggttgcgccatcgcactccagcctgggagacaagagcgagacttcgtctcaaaaaaaaaaaattcttcttccaagattcaagttgtgtcatttcaccttaataactggaggttagttaagctgggctgtgttctttgcttaatattaagacaacgttttttccagatggaagaaaactatcttaatgaattgttagcttattaattatgtaatgctaatggcttttaaaagctgagatgttctgactgggtgttgtggctcacacctgtaatcccagtaccttgggaggccaagggggaaggattgcttgaggccaggagtttgggaccatagtgagaccccgcctctatttaaaaaattaaattttgttttgttttgttttgagttggagttttgctcttgttgcccatgctgaagtgcaatggtgcaatctcagctcaccacaacctgtgcctcctgggttcaagcgattctcctgcttcagcctcccgagtagatgggattacaggcgtgcaccaccatgcctggctaattttgtatttttagtagagacagggtttctctatgttggtcaggctggtctcaaactctcgacctcaggtgatctgcccgcctccgcttcccaaagttctgggattataggtgtgagccactgggcctggcctaagaaagtttttttaagccattagacgtttttaaaggaattgggagatgacaattggggaaatatttaaaatttaagtaaaatataaagcttccttatttcatgtaacccagacaatctcagtatacatgatcagttgtgtctgacaggtaaatctatttgaggccttatcacacgttacttttaagaactagaaaggaaaagtcactgatcttaagtatttataatacttcatgtggtctaatactttttacgttttgttttgattcagatttagtccggattcccggtatctggcagtaggttctagtgagaactcagtggatttttatgacctaacgctgggccccactcttaacagaatcagctactgcaaagacattccaagctttgtcattcaaatggacttctctgcagatagcagttatctccaggtacagtaccaatactgtatacccaggtggcaagttcttctgcttttacatttcgtgttagtgaatgcatttaaagttcctgagctccagagctccagcttctcaactcctccctttgtaccttctgacctacagctcccctttcctcccccacttatcagagcttttctcctattaagtttttgtagtgatcttttgcatacttaataatgttagacatgtaaatcaagtagcaatatgctagtattctgtaaaccccctgtggattttgtctctcacctaatggaattcttgtcccattttaatctgatgaaaaaggtctctagtggctgctataaacggcatgtctatgaagtgccttcaggaaaacatcttatggatcatgccgctattgacagaattacttgggctacatggactaggtaaatacttatatattcacaaggcaagaactgactttgaaggccagttagaaaatcctatttctgaactgttagagccattccaataaggaatagtaattgagtttcaagtttttgttaccatattttgaaatggtatgttcatgttgggacccctttttattgaatatatttccatgttttatcagtttccatgatttatcaagttttttttttaaggaaatcaaagttttaactttaaagataccctgatatttttcttaatgctaaatttaatgactggcaaaaaggtattgggtgctgttaagcaactgttattaattctctatctaaaggaatgctatcttgaatctattagaagtcaaagcttccaaatttgttcaaatttcctggctgtatgacaggtaaccatgactatccatttttttggccaatgaaaaatgccatcaaattcctgtatcagccaggcatatagtggctcatgcctgtaatctctgatgtagcaggccgaggtgggaggatcacttgagcctagaagttttgataccagcctgggcaacatagcaagaccccatctctgaaatttttttaattcctatgtcataagtcatttttatttttgtagagatagggatctcacaatattgcccaggctggtctcaaactcttggcctcaagcagtcctcctgcctcagcctcccaaaatgttgggattactggtatgtgctgctggacccagccaagtagcacttttaatttgaaaaatagttctatcagttttcagtcaggcgcggtggctcagcctgtaatcccagcactttgggaggccgagcgggggtgatcacctgaggtcgggagttcgagactagcctgaccaacatggagaaaccctgtctctactaaaaatacaaaataagccgggcatgttagcgcatgcctgtgatcccagctactcgggaggctgaggcaggagaattgcttgaacccaggaggcagaggttgcggtgagccgagatcatgccattgcactccagcctgggtaacaagagcgaaaactccgtctcaaaaaaaaaaaaagaaaaaatagttctatcagttttcataaagtactactttaatcttaaaaagattaatctagaaacccttcaaattataaaatgtcatttttaaaaggcaggagttgatatcctgatgaaattcaggtctccaaacaacttaccataatttacttcctgtattttaagtaacatgatagggtacttagagattaattgccaagaaactttttgaatatagtcaacctgcccgcacttgccatgatgagttttcttttgttccttccctctagtattctaggagatgaggttttgggaatctggtccagacatgctgagaaagctgatgtcaactgtgcctgtgtatctcattcaggaatcagtcttgttacaggagatgactttggcatggttaagttatttgacttcccatgtccagaaaaatttgtaagtttgtgttttgtttactattatcagtttactcctaattttgatgtcttatcatcagcacttttccccatatatttaaaatgttttgtcctaatttctaaatttttccccaaactttctaaatctatttactttgaaataaaagctattagaaacaaatcctctccctcgagtaataccatctttggaaccatcctacaaaagctgtaattagcttttcaccaaacctataatcagttatcaaatttcaaatgcttttccttagagaaaaatggtcagagtacctggagacatctgactgcccacacagcctggttttgcagatccactactcatgctgaaaagcattctaatcactggctgcggtgctaactccctactctctccacagctcttgtcatagagattatagttcctaataagagcctttgacttctgtgtgcaccaaatgccctgagcttgtctgtcattgttttttaggcaaaacacaaaaggttcttgggtcattcgccccatgtgacaaatattcgatttaccagtggtgatcgacatgttgttagtgctggaggtgatgactgcaggttagtaactttctcagcccatgaagagcagactatgttactagttaagagacttaatacaacaactcctacagctttggtttatgaaatcagctagtcaacattagtagaaggtagtataaccagatggctcttcagaatctcatatttatgcaaatacagaataaaaggagttaaagaggaaaaatattacacatgtaacctgaaagcacaactgaaaaatattaaactgttatgaaaatctaaaaacataattaactccctgcaattttcttctctgattgcagcttatttgtctggaaatgtgtacatacacctcactgagagatgctgagatgactacagaaattaactttgagaccagaattacagagaagaaaaaccaaaacccaaccctgcatggtcaagtggtgctaacccaagactgtaacagggagaaatgcccagaatcatcaaaatagtgaaagactgatctgttcaaaatatttgctatatgcactgggtataatccgtaatccatacactgccagataatgccatttcaaggaaggatcgaatacttgatggtaaaggccaagtccccctgtattgggaagtgtgtgatttcggcagacctgctgggaaaatttagggtagagcactctttacagaagaactcaaaaacccaatttggataattttcattatctttttagcaaaatggtttcttaatgtttatattttattttcaaggttcattgtttaatgaaatattttattcttgcatttccataaggaaagggaaagtcatgatcatcctaaaggatcacagtttttaaaaggcaaacattttccctaaggaaacagacacaagctttcctagagaatatgatgttttttaggcattaataaggtccttttttataaaggacacttttctcctagtagttttgaattcaggaacagatccaaagttagcagtatatggctgctacatttccattttcattttcgagccatcagtttatgttcagatgccatctctgtaatcgcacatttaaaacataactgtagcctcactaatggaaaagtagtatgatgaacaatcattcccaatggtgtacaatgtaagggttttagggagcaacagtatttaactggaagaaagaattgcatatttaatgtagtctaatatatacacatttgtttaacatgtaaacaaaagtgttaaattcacatatacaacattatacaatttaatcactcttggaataaaatttttatagccttttttctattgggaaaatttgtttagatgtgtgccactccataggtttatttccaaaatgaatgagcccaactccatttgtaaaaacttgtcagttagaattcctttttttagtggattagggctgaattcttagatccttatttcttttcactttaaatgctgccaaagatcactactcatcattcaggaattcgctgtctagcctatctgtagtttcctgaagattgaaaattatgtagactgctatttaaaaatatatttttctaagtgtgaggtttaagatgctgtattgaccctatgagtttttaatgtgttaattatctttatagcataatagatcgctttaggttcctggaatcccatttggtctgacaggatatatgaagattcttaatacctattttctgtgtctaatacttggttaatactaaaaatagaaatgactaaattacatcacagaaagcataaccagtgattgaacctggtagttttaaagctctaaatagctgtggctgaaggactgattatggggctaagaagcttgaaacgtaagttggtacttgttcatcagtggattctcctaaattaagccaaattttgaaatacatgactattaagtttctactcatgtatttacagtcagtcaataaattaaaggaggaaaaaaatccctgaacaacctgcccataaaaagaaaaatactctacatttgagcctgctgcagttttaaattttccctctgggtcaagtttgccagcttttggctacagagaaattatatttccattacagtgcaggtagaaactctgtaaccttaagcatgtaaactacatagaataaaactgtttccactgcatttctgtccttcaaagtggccaacctgattaagtcagccttaatcactgctgctgtcagtttcacgactaaaggtcatattgactaagtagtcatcagctgaccacctcgctgtatcagccagcaacgaggggaaggtgaagaaacatgataggccatatagaatctgccctatgtttacttttttaacccagataattatttttgtgtgcagtatctaagctcctgattgtgtaacctgggacttctggcaccttttgttccattcattttatgtataaaatgcatgccaaagcacactgtgccctctggtacccttgcttccaatcgccaaccatgctcatttccttcctttttttgtggtccctttttgtggtgatcattttaaaccacgtcatccaacaaatgttttatggtcaaccttagcttgttcataagccatagcaactgaaagattaaactcttaaatatgtgtctgggcagtggctattaaatagcaaaaaacaatcagattttagtattttattatttccttgtaaaatggctgaactaaattaaacccttgtttcccatttgttctataatttatagtgaaactgagaacaaaactatctttataaatgatagctaaaagtatttccagatatttaaacaatttaaaataaatttcttctgcagagatgcaaagcatctcaacactggaatgaacaaatgccttaaattcaatggagtaaacctttagaatgaagaggaactgtcatttcacccaagccgaagacaacagccttatgcacttgtgtgctctgtctttgctgcttctcgtgtttcaagcctttcctgtgggatcagcacagcaaagtgcaacttaccaaatggtttaatgactggttaattctttcttctcccaatggaaaagcaatggcaacacaacagtagactgctggcttgacaatcttaaacgtgagcctttgcacatgtaggtttatcatcatttgagtatacgactaagcaagtcaatgaactttttttttttttttagcagtttaatttggtcctgagaatgttgcagtctttattaccccttttgcattaatccacttttctaaccaccttttaagctttaatttttaacactatacaccaagtctttgaaatcagtgatctgttatttaactctaaagcatttgacacttcttgccttaacagttttaaaaaccacacacaaaaaaactctgtaagtaatacagtaggccaaaagtttcatcctatctatcttgcagtttacctatctgatctgatctctgtaattatagttctgtcatttaaaatatactatttaaatctaatttttacatttcaaaaattatcttcagtagtaactaagtatattttctgtggattctgagaatgttatttttcagaatgtgagaatatatatgtacatttataatcttgtgactttaaagtctgttttcagatacagtatgtaaatacttgtaaaaaaatttgtataattttgtgataatgtagtttcccaaaaaaattatttagaaggcattatgttattagtaaatgagagcactgtatagaactgttcctattttctgcacttgccattccagctgcctccactgtccatacccacctcattcatcctgtcacagaaggcaggaaaactgggaactttaccaaagtagcactcagcctgagaggcctgtataatcatgcttttcaaactaaattcacttaaaaattaaaaagcagaattgaatattttaagcagcctcagtacctttggccaatgctgttttcatggtggattatgaacattatataatctttgggaaaagtgaaagtagtacaatttttagaataatgacaactgcctcactgcatctctccactcacacagcaaccgtgtagccccctaagctgcagtaccatgactaaccatgatgtcaatttcatatgctgatcctcacaacagcagtgcacaaacatgccccaaatattttaacagaatttagctcttccttaagctgtcttttcatagtaaaaacaaaacaaaaacacccaatgttaaaaccacataataaacttacaaacttgaaaaattagacacttcagatagataggcaataaaacttcatattatgaaagcaatatattccaagtttcaaagatttgacaagttctgtagagtatctttcatcagtacatgaaaacttccaaactgcatgatcttctgccaggcaggactgggtgctattcgctggtttgaggtcgaatccatttcaaggcatgtcgtggtgggacattaatggtgggatggtagaatgtgcagtccggtcttgtacattgagtgttaaacctacaatgttttggatgatagaagggacattccatcttcttacaagcagggaagtaacggcagagctgactactggaaggtggtgctggtggtgcaactggttttggagacagtactggaattcttctactcacatgagtgaagggacaatctggtttagtacactttgcatcatatttacaatttgggtgaacaaacaaacatttttcagcaaatttacaattggggaaggctttgcagggtgagatggggtgatggtaggcacactcatccccatttttacaagcaggccagtacttgcagcgctccaaaagtttttctggtttctgtgccacactcagttcactcatctcagcgttagaaaagctaccatttgggtcctcaagctgcctgctcagcaagtgcaactgctgtgggtggaggagacctctgagtcccttgtttgaggctgcagtttggtttacgggtttcattccttcaaagcacatgtcctcctcttgatctgacatgtatcctggggggctggggacaccatccagcgtcactataaacttgggacttgcaggtttatctggttgtacaagatctcgtgtctgcataaggtgtcctgaaagtacccgaagggaatctgcagtcttcatccccgactcttggtttggtgccactactacttcctcagacagctttggcttcttcagaataaatgatcttgtgtctgcatggaccatggattccatgtcatagtaatcttgatttttttctacagaatctccttttgtttcctcttctttaatggggggacttattctgggggtcctactttgtccctggaccacttctgctagcaattcttcttgagaagttcgagttctgggagcaactggaagtgtctgtttctgtggaactgtagagtagttagttgtttttgttacggattcttgagcttcagatatagccttcaaaatcagattcttgttagcttgtttagaaggtggaagagaaggtctcctttcaggctttgcaggcacagacacactgctggagatgcttcctgttcgagacccgtaatcatcatcttcttcctcctcttctccatcatgattgaatttttttactttaacaactgaacttaccacaggcaactttctcttccgaaagttttcatcctccatactcattttctccgagttgtttctaaagaacggactatacgtttcttctaagctgttaagcacctctggttcacacaaacgtcctgtttcatatacccaactactctgcatatcaagctgcttggcagcatgaatactattctgctgctgttgaaattgcaacctgtttaaatgaacaccactatctgcatttctacttgcaggtggtcgataaatttcaatagaagggcgagaagaaccatatgtaagtgtcactgtaggttttttctgagataagggattctcctgcacaaagttgaggtcttcgtcaatgagatcatctggttctggcttaatatcaatcacatcttcagagggtgctggctccctcaaaggtttcactgttgacattagtcgggttgcagctccatcatcgtaagtctgtctgacatttgtggtttttgactcctgcgaacttgtagaaactctggaatctcttttttcaggtctcgcgctaggaatggcaagtggtggcactgcagcttcatgcctcctctcatctccccgactgaaattgctcttgtttgaaggcacgttactatcaaagatgttggtatcagaagacttcagactagagggttcagttgtaacagagcgaagtttatctaatacaccatgaagccatacggtgaatcgaattgtgttgttccctagaaacagggacagatcctctgtcatttggtcctgacttttcttgttggccaccatcaccataatgtaatcaggaagttcttcatcaacataagctcctaattcttgtaatttccccttaatggcactccggatcttgcggctgatctcggtgccgatctccatggctctgcggcgtgcgggaactcagcactgcgcggcgcttggcttacccggaggctgccgcggactcctaccccgcagccgggacaccaccgcctcc

SEQ ID NO: 13628 - RNA, 16304 nt, Homo sapiens
  source 1..16304: mol_type = other RNA
gctgggattacaggcatgagccaccataataaggattctgatgaacatttgattccttggactactgttatactcaaaagccttccttaatcttctaattgtcaccctaaatatcctaaaatttctgtcttcctagtagttcttcatagtcctaaaaatttgtcagagagaaaggtaaatcaagaaacatgattttcaaatgatttaaggtggtactagggtttaggatttcctttgctttttatcatttaacacactgcttatcatacagctggaagtgctctgggccagtgtctctacttcgagggaagaaggaggtagtgagacagaaggaaatagcacaattcctggccctgacagaagggtgttcaggagacctgctctcctctcactttattccatctcatctggacctgtggcttccaatccacatctctttcctttaatatcctgcattggctaggctgtataaatcctttggtgcatcgaaaaactaagtgcattttttgtttttgtgattatgcaatacttataggaaaagttataattttagaatatttaagtacacttacatttttgagaaaaagactattgaaatgtttgtgccatgtcaaatttcagttgaacattttgggtattcttaatataagaccaggccaggcaccgtggctcaggccgggcacagtggctcacacctataatcccagcacttagggaggccaaggcgggaagatcacctgaagtcaggagttcaagaccagcctggctaacaaggtgaaactctgtctctactaaaaatacaaaaattagccgggcgtggtggctggcgcttgtaatcccagctacttgggaggctgagacaggagaatcacttgaacctgggaagcagaggttgtggtgagctgagatcgcaccattgcactccagcctgggcaacaaagagcgaaactccgtctcaaaaaaataaaaaataaaccctagaattatagtatgttagaattggaagggaagaattgtctaaggttattctagctaataagcaacagacttggaaaggaaaaggtcctgacaaagctaagcctcccgttcaggtttcctgactcgtgaattcagtgctgctgccactacacgatgcatgctctttgtatcaagggtgagacagcattacacatacatagaaaattatctatttaaactctatttgaacttttgatgagtttgtctccccctcccccactccttttcagaataacttgacgtttacaggtaccatcagtggtgatgtctgtgtgtggaaagatcacatattgtgtagaatcgtggcgagagctcacaacgggcctgtgtttgccatgtacaccaccctgcgagatggacttatcgtgactgggggaaaggaaaggccgtgagtcctctttcttttcacagaatatttatgcatttgtgacctacctgaggtttgcagttaattattctagttgtttctaggctacacagagtgtcctctccgaccttcctcctcatatgcttctcctttattaccttttatgtgccttctatttgattctcatttctggtcttaattcacttccaatttttttcatgttggggtgatactttttctgaggtgtggataggtagttgtcctacaagttgagttacttttcttaatgtctgtatgcctgtgtatgatttgctgagtaggaggcccatgggggaatctggagccagggttgtattttgactgcctgctctctttttgttcagaatggattctaaggagtagaatgcacattgttgctttagaaaaggatgagggaactagagagaactgccttgtttccttttgcttgaggcaaatttaaactgttttatacaagacctcaaaatttgagaagaggtctcttctgagtgattttcaaatctcccaacagtaaccagatacttatgatttgatttgtcaccaacatagtcatatgcatgttgaaacatgacatgtaggccaggcacagtggctcacacctgtaatcttatcactttgggaggctgaggcaggtggatcgcttgagcccaggagttcaagaccagcctgggcaacatggtgaaaccccatcgctataaaaaacaacaattagccgggtgtggtggcacatgcctgtagtccctgctactcaggaggctgaggtgggaggatcacttgagcctggggaggtcaaggctttagtgagctgtgatggtgccactgcactccagcctgggtgacagagtgagaccccatttaaaaaacaaaaacaaaaacaaaaaaaaatgtgacatatagttgactaagaagtacatttcaatacaggattgaaagaacccacatatgttaattaaacacaagcgcagaatttgtgccttttacataaaggaagaatgcacataggcatgctttcagacaagcaattcatctagcagaaaaggaaggaatacatttttcagcccttccaggaataaaatccataaatgggctctatttcgtcctccaacacttgtatttcccacgtcatttactcctgcacacccccactcactagaagcctgctaaactgttccagtgagatattttaacacctgatagggaataaatatgcttctgttttggccttcaaaaataagctctgggccagttgcagtggctcacgcctgtaatcccaacactttgggaggccgaggtgggcggatcacgaggtcaggagtttgggatcagcctggccaatatggtgaaactccatctctactaaaaatacaaaaattagccaggcatggtgcctgtaatcccagctacttgggaggctgaaggagaagaatcgcttgaacctgggaggcacaggttgcagtgagccgagatcacaccactgcactccaggccaggtgacagagcgacactctgtctcaaaaaaataaataaatcaactctgtagcatagcatttgtaattctattattttgccttacatttccattatccttttaataaaattgtttttttacatcttcctaatcaagaagtattatgaggccaggcacagtggctcatacctggaatcccagcactttgggaggccgaggcaggcagatcacctgaggtcaaggtatttgagaccagcctggccaacatggtgaaaccccatctctactaaaaatacagaaattagctgggtgtggtggtgcacacctgtaatgctagctactcgggaggctgaggtaggagaatcgcttgaacctgggaggcagaggttgcaataagcctagatcatgccactgcactcaagcctgggagacagagcgagactacatcttaaaaaaaaaaaaaaaagtattatgagagaggataatgtattgtaatgtattgtagaggctaaataaaattatgctcatgtcagaaaaaaagagtatttctcaaaataaaattcactgaaactggatgtttattttgactgagatatagtatatcctcaaattgccatagaaagtttacaagaatattagaggtaaattataaatatcagggcctttttaaaaaaaaaagattctgcttataacttggtatttgtttataataaaaattatagtagccaataatgaacacttactctggcttggttatttacttaggtcaaaagaaggaggagcggttaaactgtgggatcaggaactgaggcggtgccgtgccttcaggcttgagacaggacaagccacagattgtgttcgttctgtgtgcagaggcaaagtaagatgttccatgagctgatacagtgcagcagaaaacagaaagtggttattactgtgattccctcaccctttgcagcctaatgaacaatacttaataatgcataacgatggatttgcttgccaacattactctgtctttgctgctttctttgccaaagttagcaccagtgtggtgcataagctaggaagctattctgtctaaatactgtatgtaaacctccaatattttctagaatctgccaatttaacaactctagtagacataattgaaagcccttggcagttgactcatattaggacagctgtctccattttttaaaaaaacacacattccctagataaaacgtgcagtaaacaaacaatgaaatactactcagccataaaaaataatgaaattctgtcattcttggtggcaacatggatgagactggaggacatgatgtgaagtgaaataagccaggcacagaaagataaatacatgttctcactcctgtgcagaaactaaaaaagttgatcccacagaggtggagagtagaatagtggttactggaggcggacaagggggagggggagggggatagggaaggactggttaaaggatacaagtttacacagccagataggaatagtatgttttagtattctgtagtactgtaggatgactatagttaagaatcacgtatttatgtattttcaggtatttacaagagaggattttgaaagtttccatcacaaagaaatgataaatgtctgaggtgatggttatgcgtattaccctatgccctatagatatgtataattatgtgtcaatttcaaaataaaaattcaaaactacaactcctatgaaaatttttgagcgtgtttgtacttattaagtgtatttataaatcatacggatattatcttcagcctgcatattaaattgtagttaagcttttactttttaactaaaaaataaattctattattttttcctatatcccactgcactgaccccagtttggaaatcctaagattatcaaataaaaactttgattattgaagaatccaggtgtactgccacagaaaagttctattctgtagcatggactctaatatgtaatctagcccattgtgcttacagatagatgtgtgcctgtagtcatagaaaaatttgcatgagctaatgactgccttgctactagattagctcaaagcaaaaagttctctgaaagcaggtcaatagggtcatttttatattatgaagaagaaaagcagctgttgtattacattcactgtattggtcctgcttgtgtttcagggcaagatccttgttgggacaaggaatgctgaaataatcgaagttggagagaaaaatgcagcttgtaatattttagttaacggtcatgtggatgggccaatctggggactagcaacacatccttccagggattttttcctttctgctgcagaagatgggacagtgagactttgggatattgctgataaagtaagtacagataatttttttaaaagaggttacaacttctaaaaagaaaagttggaagttctaaattgctagtacttaaagaactgccagaattctgttgagcattttgaggggaaactggtataatttagaagtacttcacttaatgtttcctatgactctttttttttttttttttaaatgcagaagatgttaaacaaagtgaatttgggacatgctgctcgtactgtgtgttacagccctgaaggggacatggtggctattggaatgaaaaatggagaatttatcattttactagtgagttctctaaaaatatggggaaagaagagagacaggagatgtgcaatccatgatatcaggttagtgaacaaatggaatagagtttctagtatatacttgatttaacttccatttgtaaaattttccatagccttgccttcaaaaagaggtccccagggcctgtagcatttcccgtattataaattgtatgctaaaatatggctgtttgtatactacttaattcttcttgctaaattataaacccactgggcaccaactataatagcaagtactagtaggtaatgtttgatgaattcatgttaacacttagccatgtccattaagttcatcccaccaagaggtatctcccactgtaatacaagagagctatctgcccttcaaaagttgtcaccctggaaaactaaagttgtgatttcaaacatatcttctcttagtaacctcagtttgggaatatgtagttcattaatttaatcaatacctattgattaaatgttccagaatccaaattaatttaaatgtttcttaaacctttgtttttcagtgcttaagcatttttcaacagtggctaccatttacggagtacttccgtgtgatcagtagataagattattgaatctaggtctgtcaaaagcttgtacacttttcatcagtaaaatccttttacaaatgaaaccttcctcagaacttcaatatataaaatagtaacagtggcttcccttagcttttacatgtctctatcgtacctcagtaagactcatgggccatttcaagagactgaattgtcccatatgactccaaagattgctaggcaaatagcatttcactttgtcttttaaataagttcttcaggccgggcgcggtggctcatgcctgtaatcccagcactttgggaggccgaggcaggcagatcacctgaagtcaggagtactcgaccagcctggccaacatagtgaaaccccatctcaactaaaaatacaaaaatcagccgggcgtggtggcaggcgcctgtaatcccagctactcagggggctgaaacaggagaatcgcttgaacccgggaggcggaggttgcgccatcgcactccagcctgggagacaagagcgagacttcgtctcaaaaaaaaaaaattcttcttccaagattcaagttgtgtcatttcaccttaataactggaggttagttaagctgggctgtgttctttgcttaatattaagacaacgttttttccagatggaagaaaactatcttaatgaattgttagcttattaattatgtaatgctaatggcttttaaaagctgagatgttctgactgggtgttgtggctcacacctgtaatcccagtaccttgggaggccaagggggaaggattgcttgaggccaggagtttgggaccatagtgagaccccgcctctatttaaaaaattaaattttgttttgttttgttttgagttggagttttgctcttgttgcccatgctgaagtgcaatggtgcaatctcagctcaccacaacctgtgcctcctgggttcaagcgattctcctgcttcagcctcccgagtagatgggattacaggcgtgcaccaccatgcctggctaattttgtatttttagtagagacagggtttctctatgttggtcaggctggtctcaaactctcgacctcaggtgatctgcccgcctccgcttcccaaagttctgggattataggtgtgagccactgggcctggcctaagaaagtttttttaagccattagacgtttttaaaggaattgggagatgacaattggggaaatatttaaaatttaagtaaaatataaagcttccttatttcatgtaacccagacaatctcagtatacatgatcagttgtgtctgacaggtaaatctatttgaggccttatcacacgttacttttaagaactagaaaggaaaagtcactgatcttaagtatttataatacttcatgtggtctaatactttttacgttttgttttgattcagatttagtccggattcccggtatctggcagtaggttctagtgagaactcagtggatttttatgacctaacgctgggccccactcttaacagaatcagctactgcaaagacattccaagctttgtcattcaaatggacttctctgcagatagcagttatctccaggtacagtaccaatactgtatacccaggtggcaagttcttctgcttttacatttcgtgttagtgaatgcatttaaagttcctgagctccagagctccagcttctcaactcctccctttgtaccttctgacctacagctcccctttcctcccccacttatcagagcttttctcctattaagtttttgtagtgatcttttgcatacttaataatgttagacatgtaaatcaagtagcaatatgctagtattctgtaaaccccctgtggattttgtctctcacctaatggaattcttgtcccattttaatctgatgaaaaaggtctctagtggctgctataaacggcatgtctatgaagtgccttcaggaaaacatcttatggatcatgccgctattgacagaattacttgggctacatggactaggtaaatacttatatattcacaaggcaagaactgactttgaaggccagttagaaaatcctatttctgaactgttagagccattccaataaggaatagtaattgagtttcaagtttttgttaccatattttgaaatggtatgttcatgttgggacccctttttattgaatatatttccatgttttatcagtttccatgatttatcaagttttttttttaaggaaatcaaagttttaactttaaagataccctgatatttttcttaatgctaaatttaatgactggcaaaaaggtattgggtgctgttaagcaactgttattaattctctatctaaaggaatgctatcttgaatctattagaagtcaaagcttccaaatttgttcaaatttcctggctgtatgacaggtaaccatgactatccatttttttggccaatgaaaaatgccatcaaattcctgtatcagccaggcatatagtggctcatgcctgtaatctctgatgtagcaggccgaggtgggaggatcacttgagcctagaagttttgataccagcctgggcaacatagcaagaccccatctctgaaatttttttaattcctatgtcataagtcatttttatttttgtagagatagggatctcacaatattgcccaggctggtctcaaactcttggcctcaagcagtcctcctgcctcagcctcccaaaatgttgggattactggtatgtgctgctggacccagccaagtagcacttttaatttgaaaaatagttctatcagttttcagtcaggcgcggtggctcagcctgtaatcccagcactttgggaggccgagcgggggtgatcacctgaggtcgggagttcgagactagcctgaccaacatggagaaaccctgtctctactaaaaatacaaaataagccgggcatgttagcgcatgcctgtgatcccagctactcgggaggctgaggcaggagaattgcttgaacccaggaggcagaggttgcggtgagccgagatcatgccattgcactccagcctgggtaacaagagcgaaaactccgtctcaaaaaaaaaaaaagaaaaaatagttctatcagttttcataaagtactactttaatcttaaaaagattaatctagaaacccttcaaattataaaatgtcatttttaaaaggcaggagttgatatcctgatgaaattcaggtctccaaacaacttaccataatttacttcctgtattttaagtaacatgatagggtacttagagattaattgccaagaaactttttgaatatagtcaacctgcccgcacttgccatgatgagttttcttttgttccttccctctagtattctaggagatgaggttttgggaatctggtccagacatgctgagaaagctgatgtcaactgtgcctgtgtatctcattcaggaatcagtcttgttacaggagatgactttggcatggttaagttatttgacttcccatgtccagaaaaatttgtaagtttgtgttttgtttactattatcagtttactcctaattttgatgtcttatcatcagcacttttccccatatatttaaaatgttttgtcctaatttctaaatttttccccaaactttctaaatctatttactttgaaataaaagctattagaaacaaatcctctccctcgagtaataccatctttggaaccatcctacaaaagctgtaattagcttttcaccaaacctataatcagttatcaaatttcaaatgcttttccttagagaaaaatggtcagagtacctggagacatctgactgcccacacagcctggttttgcagatccactactcatgctgaaaagcattctaatcactggctgcggtgctaactccctactctctccacagctcttgtcatagagattatagttcctaataagagcctttgacttctgtgtgcaccaaatgccctgagcttgtctgtcattgttttttaggcaaaacacaaaaggttcttgggtcattcgccccatgtgacaaatattcgatttaccagtggtgatcgacatgttgttagtgctggaggtgatgactgcaggttagtaactttctcagcccatgaagagcagactatgttactagttaagagacttaatacaacaactcctacagctttggtttatgaaatcagctagtcaacattagtagaaggtagtataaccagatggctcttcagaatctcatatttatgcaaatacagaataaaaggagttaaagaggaaaaatattacacatgtaacctgaaagcacaactgaaaaatattaaactgttatgaaaatctaaaaacataattaactccctgcaattttcttctctgattgcagcttatttgtctggaaatgtgtacatacacctcactgagagatgctgagatgactacagaaattaactttgagaccagaattacagagaagaaaaaccaaaacccaaccctgcatggtcaagtggtgctaacccaagactgtaacagggagaaatgcccagaatcatcaaaatagtgaaagactgatctgttcaaaatatttgctatatgcactgggtataatccgtaatccatacactgccagataatgccatttcaaggaaggatcgaatacttgatggtaaaggccaagtccccctgtattgggaagtgtgtgatttcggcagacctgctgggaaaatttagggtagagcactctttacagaagaactcaaaaacccaatttggataattttcattatctttttagcaaaatggtttcttaatgtttatattttattttcaaggttcattgtttaatgaaatattttattcttgcatttccataaggaaagggaaagtcatgatcatcctaaaggatcacagtttttaaaaggcaaacattttccctaaggaaacagacacaagctttcctagagaatatgatgttttttaggcattaataaggtccttttttataaaggacacttttctcctagtagttttgaattcaggaacagatccaaagttagcagtatatggctgctacatttccattttcattttcgagccatcagtttatgttcagatgccatctctgtaatcgcacatttaaaacataactgtagcctcactaatggaaaagtagtatgatgaacaatcattcccaatggtgtacaatgtaagggttttagggagcaacagtatttaactggaagaaagaattgcatatttaatgtagtctaatatatacacatttgtttaacatgtaaacaaaagtgttaaattcacatatacaacattatacaatttaatcactcttggaataaaatttttatagccttttttctattgggaaaatttgtttagatgtgtgccactccataggtttatttccaaaatgaatgagcccaactccatttgtaaaaacttgtcagttagaattcctttttttagtggattagggctgaattcttagatccttatttcttttcactttaaatgctgccaaagatcactactcatcattcaggaattcgctgtctagcctatctgtagtttcctgaagattgaaaattatgtagactgctatttaaaaatatatttttctaagtgtgaggtttaagatgctgtattgaccctatgagtttttaatgtgttaattatctttatagcataatagatcgctttaggttcctggaatcccatttggtctgacaggatatatgaagattcttaatacctattttctgtgtctaatacttggttaatactaaaaatagaaatgactaaattacatcacagaaagcataaccagtgattgaacctggtagttttaaagctctaaatagctgtggctgaaggactgattatggggctaagaagcttgaaacgtaagttggtacttgttcatcagtggattctcctaaattaagccaaattttgaaatacatgactattaagtttctactcatgtatttacagtcagtcaataaattaaaggaggaaaaaaatccctgaacaacctgcccataaaaagaaaaatactctacatttgagcctgctgcagttttaaattttccctctgggtcaagtttgccagcttttggctacagagaaattatatttccattacagtgcaggtagaaactctgtaaccttaagcatgtaaactacatagaataaaactgtttccactgcatttctgtccttcaaagtggccaacctgattaagtcagccttaatcactgctgctgtcagtttcacgactaaaggtcatattgactaagtagtcatcagctgaccacctcgctgtatcagccagcaacgaggggaaggtgaagaaacatgataggccatatagaatctgccctatgtttacttttttaacccagataattatttttgtgtgcagtatctaagctcctgattgtgtaacctgggacttctggcaccttttgttccattcattttatgtataaaatgcatgccaaagcacactgtgccctctggtacccttgcttccaatcgccaaccatgctcatttccttcctttttttgtggtccctttttgtggtgatcattttaaaccacgtcatccaacaaatgttttatggtcaaccttagcttgttcataagccatagcaactgaaagattaaactcttaaatatgtgtctgggcagtggctattaaatagcaaaaaacaatcagattttagtattttattatttccttgtaaaatggctgaactaaattaaacccttgtttcccatttgttctataatttatagtgaaactgagaacaaaactatctttataaatgatagctaaaagtatttccagatatttaaacaatttaaaataaatttcttctgcagagatgcaaagcatctcaacactggaatgaacaaatgccttaaattcaatggagtaaacctttagaatgaagaggaactgtcatttcacccaagccgaagacaacagccttatgcacttgtgtgctctgtctttgctgcttctcgtgtttcaagcctttcctgtgggatcagcacagcaaagtgcaacttaccaaatggtttaatgactggttaattctttcttctcccaatggaaaagcaatggcaacacaacagtagactgctggcttgacaatcttaaacgtgagcctttgcacatgtaggtttatcatcatttgagtatacgactaagcaagtcaatgaactttttttttttttttagcagtttaatttggtcctgagaatgttgcagtctttattaccccttttgcattaatccacttttctaaccaccttttaagctttaatttttaacactatacaccaagtctttgaaatcagtgatctgttatttaactctaaagcatttgacacttcttgccttaacagttttaaaaaccacacacaaaaaaactctgtaagtaatacagtaggccaaaagtttcatcctatctatcttgcagtttacctatctgatctgatctctgtaattatagttctgtcatttaaaatatactatttaaatctaatttttacatttcaaaaattatcttcagtagtaactaagtatattttctgtggattctgagaatgttatttttcagaatgtgagaatatatatgtacatttataatcttgtgactttaaagtctgttttcagatacagtatgtaaatacttgtaaaaaaatttgtataattttgtgataatgtagtttcccaaaaaaattatttagaaggcattatgttattagtaaatgagagcactgtatagaactgttcctattttctgcacttgccattccagctgcctccactgtccatacccacctcattcatcctgtcacagaaggcaggaaaactgggaactttaccaaagtagcactcagcctgagaggcctgtataatcatgcttttcaaactaaattcacttaaaaattaaaaagcagaattgaatattttaagcagcctcagtacctttggccaatgctgttttcatggtggattatgaacattatataatctttgggaaaagtgaaagtagtacaatttttagaataatgacaactgcctcactgcatctctccactcacacagcaaccgtgtagccccctaagctgcagtaccatgactaaccatgatgtcaatttcatatgctgatcctcacaacagcagtgcacaaacatgccccaaatattttaacagaatttagctcttccttaagctgtcttttcatagtaaaaacaaaacaaaaacacccaatgttaaaaccacataataaacttacaaacttgaaaaattagacacttcagatagataggcaataaaacttcatattatgaaagcaatatattccaagtttcaaagatttgacaagttctgtagagtatctttcatcagtacatgaaaacttccaaactgcatgatcttctgccaggcaggactgggtgctattcgctggtttgaggtcgaatccatttcaaggcatgtcgtggtgggacattaatggtgggatggtagaatgtgcagtccggtcttgtacattgagtgttaaacctacaatgttttggatgatagaagggacattccatcttcttacaagcagggaagtaacggcagagctgactactggaaggtggtgctggtggtgcaactggttttggagacagtactggaattcttctactcacatgagtgaagggacaatctggtttagtacactttgcatcatatttacaatttgggtgaacaaacaaacatttttcagcaaatttacaattggggaaggctttgcagggtgagatggggtgatggtaggcacactcatccccatttttacaagcaggccagtacttgcagcgctccaaaagtttttctggtttctgtgccacactcagttcactcatctcagctgtagagtagttagttgtttttgttacggattcttgagcttcagatatagccttcaaaatcagattcttgttagcttgtttagaaggtggaagagaaggtctcctttcaggctttgcaggcacagacacactgctggagatgcttcctgttcgagacccgtaatcatcatcttcttcctcctcttctccatcatgattgaatttttttactttaacaactgaacttaccacaggcaactttctcttccgaaagttttcatcctccatactcattttctccgagttgtttctaaagaacggactatacgtttcttctaagctgttaagcacctctggttcacacaaacgtcctgtttcatatacccaactactctgcatatcaagctgcttggcagcatgaatactattctgctgctgttgaaattgcaacctgtttaaatgaacaccactatctgcatttctacttgcaggtggtcgataaatttcaatagaagggcgagaagaaccatatgtaagtgtcactgtaggttttttctgagataagggattctcctgcacaaagttgaggtcttcgtcaatgagatcatctggttctggcttaatatcaatcacatcttcagagggtgctggctccctcaaaggtttcactgttgacattagtcgggttgcagctccatcatcgtaagtctgtctgacatttgtggtttttgactcctgcgaacttgtagaaactctggaatctcttttttcaggtctcgcgctaggaatggcaagtggtggcactgcagcttcatgcctcctctcatctccccgactgaaattgctcttgtttgaaggcacgttactatcaaagatgttggtatcagaagacttcagactagagggttcagttgtaacagagcgaagtttatctaatacaccatgaagccatacggtgaatcgaattgtgttgttccctagaaacagggacagatcctctgtcatttggtcctgacttttcttgttggccaccatcaccataatgtaatcaggaagttcttcatcaacataagctcctaattcttgtaatttccccttaatggcactccggatcttgcggctgatctcggtgccgatctccatggctctgcggcgtgcgggaactcagcactgcgcggcgcttggcttacccggaggctgccgcggactcctaccccgcagccgggacaccaccgcctcc

SEQ ID NO: 13629 - RNA, 16420 nt, Homo sapiens
  source 1..16420: mol_type = other RNA
gctgggattacaggcatgagccaccataataaggattctgatgaacatttgattccttggactactgttatactcaaaagccttccttaatcttctaattgtcaccctaaatatcctaaaatttctgtcttcctagtagttcttcatagtcctaaaaatttgtcagagagaaaggtaaatcaagaaacatgattttcaaatgatttaaggtggtactagggtttaggatttcctttgctttttatcatttaacacactgcttatcatacagctggaagtgctctgggccagtgtctctacttcgagggaagaaggaggtagtgagacagaaggaaatagcacaattcctggccctgacagaagggtgttcaggagacctgctctcctctcactttattccatctcatctggacctgtggcttccaatccacatctctttcctttaatatcctgcattggctaggctgtataaatcctttggtgcatcgaaaaactaagtgcattttttgtttttgtgattatgcaatacttataggaaaagttataattttagaatatttaagtacacttacatttttgagaaaaagactattgaaatgtttgtgccatgtcaaatttcagttgaacattttgggtattcttaatataagaccaggccaggcaccgtggctcaggccgggcacagtggctcacacctataatcccagcacttagggaggccaaggcgggaagatcacctgaagtcaggagttcaagaccagcctggctaacaaggtgaaactctgtctctactaaaaatacaaaaattagccgggcgtggtggctggcgcttgtaatcccagctacttgggaggctgagacaggagaatcacttgaacctgggaagcagaggttgtggtgagctgagatcgcaccattgcactccagcctgggcaacaaagagcgaaactccgtctcaaaaaaataaaaaataaaccctagaattatagtatgttagaattggaagggaagaattgtctaaggttattctagctaataagcaacagacttggaaaggaaaaggtcctgacaaagctaagcctcccgttcaggtttcctgactcgtgaattcagtgctgctgccactacacgatgcatgctctttgtatcaagggtgagacagcattacacatacatagaaaattatctatttaaactctatttgaacttttgatgagtttgtctccccctcccccactccttttcagaataacttgacgtttacaggtaccatcagtggtgatgtctgtgtgtggaaagatcacatattgtgtagaatcgtggcgagagctcacaacgggcctgtgtttgccatgtacaccaccctgcgagatggacttatcgtgactgggggaaaggaaaggccgtgagtcctctttcttttcacagaatatttatgcatttgtgacctacctgaggtttgcagttaattattctagttgtttctaggctacacagagtgtcctctccgaccttcctcctcatatgcttctcctttattaccttttatgtgccttctatttgattctcatttctggtcttaattcacttccaatttttttcatgttggggtgatactttttctgaggtgtggataggtagttgtcctacaagttgagttacttttcttaatgtctgtatgcctgtgtatgatttgctgagtaggaggcccatgggggaatctggagccagggttgtattttgactgcctgctctctttttgttcagaatggattctaaggagtagaatgcacattgttgctttagaaaaggatgagggaactagagagaactgccttgtttccttttgcttgaggcaaatttaaactgttttatacaagacctcaaaatttgagaagaggtctcttctgagtgattttcaaatctcccaacagtaaccagatacttatgatttgatttgtcaccaacatagtcatatgcatgttgaaacatgacatgtaggccaggcacagtggctcacacctgtaatcttatcactttgggaggctgaggcaggtggatcgcttgagcccaggagttcaagaccagcctgggcaacatggtgaaaccccatcgctataaaaaacaacaattagccgggtgtggtggcacatgcctgtagtccctgctactcaggaggctgaggtgggaggatcacttgagcctggggaggtcaaggctttagtgagctgtgatggtgccactgcactccagcctgggtgacagagtgagaccccatttaaaaaacaaaaacaaaaacaaaaaaaaatgtgacatatagttgactaagaagtacatttcaatacaggattgaaagaacccacatatgttaattaaacacaagcgcagaatttgtgccttttacataaaggaagaatgcacataggcatgctttcagacaagcaattcatctagcagaaaaggaaggaatacatttttcagcccttccaggaataaaatccataaatgggctctatttcgtcctccaacacttgtatttcccacgtcatttactcctgcacacccccactcactagaagcctgctaaactgttccagtgagatattttaacacctgatagggaataaatatgcttctgttttggccttcaaaaataagctctgggccagttgcagtggctcacgcctgtaatcccaacactttgggaggccgaggtgggcggatcacgaggtcaggagtttgggatcagcctggccaatatggtgaaactccatctctactaaaaatacaaaaattagccaggcatggtgcctgtaatcccagctacttgggaggctgaaggagaagaatcgcttgaacctgggaggcacaggttgcagtgagccgagatcacaccactgcactccaggccaggtgacagagcgacactctgtctcaaaaaaataaataaatcaactctgtagcatagcatttgtaattctattattttgccttacatttccattatccttttaataaaattgtttttttacatcttcctaatcaagaagtattatgaggccaggcacagtggctcatacctggaatcccagcactttgggaggccgaggcaggcagatcacctgaggtcaaggtatttgagaccagcctggccaacatggtgaaaccccatctctactaaaaatacagaaattagctgggtgtggtggtgcacacctgtaatgctagctactcgggaggctgaggtaggagaatcgcttgaacctgggaggcagaggttgcaataagcctagatcatgccactgcactcaagcctgggagacagagcgagactacatcttaaaaaaaaaaaaaaaagtattatgagagaggataatgtattgtaatgtattgtagaggctaaataaaattatgctcatgtcagaaaaaaagagtatttctcaaaataaaattcactgaaactggatgtttattttgactgagatatagtatatcctcaaattgccatagaaagtttacaagaatattagaggtaaattataaatatcagggcctttttaaaaaaaaaagattctgcttataacttggtatttgtttataataaaaattatagtagccaataatgaacacttactctggcttggttatttacttaggtcaaaagaaggaggagcggttaaactgtgggatcaggaactgaggcggtgccgtgccttcaggcttgagacaggacaagccacagattgtgttcgttctgtgtgcagaggcaaagtaagatgttccatgagctgatacagtgcagcagaaaacagaaagtggttattactgtgattccctcaccctttgcagcctaatgaacaatacttaataatgcataacgatggatttgcttgccaacattactctgtctttgctgctttctttgccaaagttagcaccagtgtggtgcataagctaggaagctattctgtctaaatactgtatgtaaacctccaatattttctagaatctgccaatttaacaactctagtagacataattgaaagcccttggcagttgactcatattaggacagctgtctccattttttaaaaaaacacacattccctagataaaacgtgcagtaaacaaacaatgaaatactactcagccataaaaaataatgaaattctgtcattcttggtggcaacatggatgagactggaggacatgatgtgaagtgaaataagccaggcacagaaagataaatacatgttctcactcctgtgcagaaactaaaaaagttgatcccacagaggtggagagtagaatagtggttactggaggcggacaagggggagggggagggggatagggaaggactggttaaaggatacaagtttacacagccagataggaatagtatgttttagtattctgtagtactgtaggatgactatagttaagaatcacgtatttatgtattttcaggtatttacaagagaggattttgaaagtttccatcacaaagaaatgataaatgtctgaggtgatggttatgcgtattaccctatgccctatagatatgtataattatgtgtcaatttcaaaataaaaattcaaaactacaactcctatgaaaatttttgagcgtgtttgtacttattaagtgtatttataaatcatacggatattatcttcagcctgcatattaaattgtagttaagcttttactttttaactaaaaaataaattctattattttttcctatatcccactgcactgaccccagtttggaaatcctaagattatcaaataaaaactttgattattgaagaatccaggtgtactgccacagaaaagttctattctgtagcatggactctaatatgtaatctagcccattgtgcttacagatagatgtgtgcctgtagtcatagaaaaatttgcatgagctaatgactgccttgctactagattagctcaaagcaaaaagttctctgaaagcaggtcaatagggtcatttttatattatgaagaagaaaagcagctgttgtattacattcactgtattggtcctgcttgtgtttcagggcaagatccttgttgggacaaggaatgctgaaataatcgaagttggagagaaaaatgcagcttgtaatattttagttaacggtcatgtggatgggccaatctggggactagcaacacatccttccagggattttttcctttctgctgcagaagatgggacagtgagactttgggatattgctgataaagtaagtacagataatttttttaaaagaggttacaacttctaaaaagaaaagttggaagttctaaattgctagtacttaaagaactgccagaattctgttgagcattttgaggggaaactggtataatttagaagtacttcacttaatgtttcctatgactctttttttttttttttttaaatgcagaagatgttaaacaaagtgaatttgggacatgctgctcgtactgtgtgttacagccctgaaggggacatggtggctattggaatgaaaaatggagaatttatcattttactagtgagttctctaaaaatatggggaaagaagagagacaggagatgtgcaatccatgatatcaggttagtgaacaaatggaatagagtttctagtatatacttgatttaacttccatttgtaaaattttccatagccttgccttcaaaaagaggtccccagggcctgtagcatttcccgtattataaattgtatgctaaaatatggctgtttgtatactacttaattcttcttgctaaattataaacccactgggcaccaactataatagcaagtactagtaggtaatgtttgatgaattcatgttaacacttagccatgtccattaagttcatcccaccaagaggtatctcccactgtaatacaagagagctatctgcccttcaaaagttgtcaccctggaaaactaaagttgtgatttcaaacatatcttctcttagtaacctcagtttgggaatatgtagttcattaatttaatcaatacctattgattaaatgttccagaatccaaattaatttaaatgtttcttaaacctttgtttttcagtgcttaagcatttttcaacagtggctaccatttacggagtacttccgtgtgatcagtagataagattattgaatctaggtctgtcaaaagcttgtacacttttcatcagtaaaatccttttacaaatgaaaccttcctcagaacttcaatatataaaatagtaacagtggcttcccttagcttttacatgtctctatcgtacctcagtaagactcatgggccatttcaagagactgaattgtcccatatgactccaaagattgctaggcaaatagcatttcactttgtcttttaaataagttcttcaggccgggcgcggtggctcatgcctgtaatcccagcactttgggaggccgaggcaggcagatcacctgaagtcaggagtactcgaccagcctggccaacatagtgaaaccccatctcaactaaaaatacaaaaatcagccgggcgtggtggcaggcgcctgtaatcccagctactcagggggctgaaacaggagaatcgcttgaacccgggaggcggaggttgcgccatcgcactccagcctgggagacaagagcgagacttcgtctcaaaaaaaaaaaattcttcttccaagattcaagttgtgtcatttcaccttaataactggaggttagttaagctgggctgtgttctttgcttaatattaagacaacgttttttccagatggaagaaaactatcttaatgaattgttagcttattaattatgtaatgctaatggcttttaaaagctgagatgttctgactgggtgttgtggctcacacctgtaatcccagtaccttgggaggccaagggggaaggattgcttgaggccaggagtttgggaccatagtgagaccccgcctctatttaaaaaattaaattttgttttgttttgttttgagttggagttttgctcttgttgcccatgctgaagtgcaatggtgcaatctcagctcaccacaacctgtgcctcctgggttcaagcgattctcctgcttcagcctcccgagtagatgggattacaggcgtgcaccaccatgcctggctaattttgtatttttagtagagacagggtttctctatgttggtcaggctggtctcaaactctcgacctcaggtgatctgcccgcctccgcttcccaaagttctgggattataggtgtgagccactgggcctggcctaagaaagtttttttaagccattagacgtttttaaaggaattgggagatgacaattggggaaatatttaaaatttaagtaaaatataaagcttccttatttcatgtaacccagacaatctcagtatacatgatcagttgtgtctgacaggtaaatctatttgaggccttatcacacgttacttttaagaactagaaaggaaaagtcactgatcttaagtatttataatacttcatgtggtctaatactttttacgttttgttttgattcagatttagtccggattcccggtatctggcagtaggttctagtgagaactcagtggatttttatgacctaacgctgggccccactcttaacagaatcagctactgcaaagacattccaagctttgtcattcaaatggacttctctgcagatagcagttatctccaggtacagtaccaatactgtatacccaggtggcaagttcttctgcttttacatttcgtgttagtgaatgcatttaaagttcctgagctccagagctccagcttctcaactcctccctttgtaccttctgacctacagctcccctttcctcccccacttatcagagcttttctcctattaagtttttgtagtgatcttttgcatacttaataatgttagacatgtaaatcaagtagcaatatgctagtattctgtaaaccccctgtggattttgtctctcacctaatggaattcttgtcccattttaatctgatgaaaaaggtctctagtggctgctataaacggcatgtctatgaagtgccttcaggaaaacatcttatggatcatgccgctattgacagaattacttgggctacatggactaggtaaatacttatatattcacaaggcaagaactgactttgaaggccagttagaaaatcctatttctgaactgttagagccattccaataaggaatagtaattgagtttcaagtttttgttaccatattttgaaatggtatgttcatgttgggacccctttttattgaatatatttccatgttttatcagtttccatgatttatcaagttttttttttaaggaaatcaaagttttaactttaaagataccctgatatttttcttaatgctaaatttaatgactggcaaaaaggtattgggtgctgttaagcaactgttattaattctctatctaaaggaatgctatcttgaatctattagaagtcaaagcttccaaatttgttcaaatttcctggctgtatgacaggtaaccatgactatccatttttttggccaatgaaaaatgccatcaaattcctgtatcagccaggcatatagtggctcatgcctgtaatctctgatgtagcaggccgaggtgggaggatcacttgagcctagaagttttgataccagcctgggcaacatagcaagaccccatctctgaaatttttttaattcctatgtcataagtcatttttatttttgtagagatagggatctcacaatattgcccaggctggtctcaaactcttggcctcaagcagtcctcctgcctcagcctcccaaaatgttgggattactggtatgtgctgctggacccagccaagtagcacttttaatttgaaaaatagttctatcagttttcagtcaggcgcggtggctcagcctgtaatcccagcactttgggaggccgagcgggggtgatcacctgaggtcgggagttcgagactagcctgaccaacatggagaaaccctgtctctactaaaaatacaaaataagccgggcatgttagcgcatgcctgtgatcccagctactcgggaggctgaggcaggagaattgcttgaacccaggaggcagaggttgcggtgagccgagatcatgccattgcactccagcctgggtaacaagagcgaaaactccgtctcaaaaaaaaaaaaagaaaaaatagttctatcagttttcataaagtactactttaatcttaaaaagattaatctagaaacccttcaaattataaaatgtcatttttaaaaggcaggagttgatatcctgatgaaattcaggtctccaaacaacttaccataatttacttcctgtattttaagtaacatgatagggtacttagagattaattgccaagaaactttttgaatatagtcaacctgcccgcacttgccatgatgagttttcttttgttccttccctctagtattctaggagatgaggttttgggaatctggtccagacatgctgagaaagctgatgtcaactgtgcctgtgtatctcattcaggaatcagtcttgttacaggagatgactttggcatggttaagttatttgacttcccatgtccagaaaaatttgtaagtttgtgttttgtttactattatcagtttactcctaattttgatgtcttatcatcagcacttttccccatatatttaaaatgttttgtcctaatttctaaatttttccccaaactttctaaatctatttactttgaaataaaagctattagaaacaaatcctctccctcgagtaataccatctttggaaccatcctacaaaagctgtaattagcttttcaccaaacctataatcagttatcaaatttcaaatgcttttccttagagaaaaatggtcagagtacctggagacatctgactgcccacacagcctggttttgcagatccactactcatgctgaaaagcattctaatcactggctgcggtgctaactccctactctctccacagctcttgtcatagagattatagttcctaataagagcctttgacttctgtgtgcaccaaatgccctgagcttgtctgtcattgttttttaggcaaaacacaaaaggttcttgggtcattcgccccatgtgacaaatattcgatttaccagtggtgatcgacatgttgttagtgctggaggtgatgactgcaggttagtaactttctcagcccatgaagagcagactatgttactagttaagagacttaatacaacaactcctacagctttggtttatgaaatcagctagtcaacattagtagaaggtagtataaccagatggctcttcagaatctcatatttatgcaaatacagaataaaaggagttaaagaggaaaaatattacacatgtaacctgaaagcacaactgaaaaatattaaactgttatgaaaatctaaaaacataattaactccctgcaattttcttctctgattgcagcttatttgtctggaaatgtgtacatacacctcactgagagatgctgagatgactacagaaattaactttgagaccagaattacagagaagaaaaaccaaaacccaaccctgcatggtcaagtggtgctaacccaagactgtaacagggagaaatgcccagaatcatcaaaatagtgaaagactgatctgttcaaaatatttgctatatgcactgggtataatccgtaatccatacactgccagataatgccatttcaaggaaggatcgaatacttgatggtaaaggccaagtccccctgtattgggaagtgtgtgatttcggcagacctgctgggaaaatttagggtagagcactctttacagaagaactcaaaaacccaatttggataattttcattatctttttagcaaaatggtttcttaatgtttatattttattttcaaggttcattgtttaatgaaatattttattcttgcatttccataaggaaagggaaagtcatgatcatcctaaaggatcacagtttttaaaaggcaaacattttccctaaggaaacagacacaagctttcctagagaatatgatgttttttaggcattaataaggtccttttttataaaggacacttttctcctagtagttttgaattcaggaacagatccaaagttagcagtatatggctgctacatttccattttcattttcgagccatcagtttatgttcagatgccatctctgtaatcgcacatttaaaacataactgtagcctcactaatggaaaagtagtatgatgaacaatcattcccaatggtgtacaatgtaagggttttagggagcaacagtatttaactggaagaaagaattgcatatttaatgtagtctaatatatacacatttgtttaacatgtaaacaaaagtgttaaattcacatatacaacattatacaatttaatcactcttggaataaaatttttatagccttttttctattgggaaaatttgtttagatgtgtgccactccataggtttatttccaaaatgaatgagcccaactccatttgtaaaaacttgtcagttagaattcctttttttagtggattagggctgaattcttagatccttatttcttttcactttaaatgctgccaaagatcactactcatcattcaggaattcgctgtctagcctatctgtagtttcctgaagattgaaaattatgtagactgctatttaaaaatatatttttctaagtgtgaggtttaagatgctgtattgaccctatgagtttttaatgtgttaattatctttatagcataatagatcgctttaggttcctggaatcccatttggtctgacaggatatatgaagattcttaatacctattttctgtgtctaatacttggttaatactaaaaatagaaatgactaaattacatcacagaaagcataaccagtgattgaacctggtagttttaaagctctaaatagctgtggctgaaggactgattatggggctaagaagcttgaaacgtaagttggtacttgttcatcagtggattctcctaaattaagccaaattttgaaatacatgactattaagtttctactcatgtatttacagtcagtcaataaattaaaggaggaaaaaaatccctgaacaacctgcccataaaaagaaaaatactctacatttgagcctgctgcagttttaaattttccctctgggtcaagtttgccagcttttggctacagagaaattatatttccattacagtgcaggtagaaactctgtaaccttaagcatgtaaactacatagaataaaactgtttccactgcatttctgtccttcaaagtggccaacctgattaagtcagccttaatcactgctgctgtcagtttcacgactaaaggtcatattgactaagtagtcatcagctgaccacctcgctgtatcagccagcaacgaggggaaggtgaagaaacatgataggccatatagaatctgccctatgtttacttttttaacccagataattatttttgtgtgcagtatctaagctcctgattgtgtaacctgggacttctggcaccttttgttccattcattttatgtataaaatgcatgccaaagcacactgtgccctctggtacccttgcttccaatcgccaaccatgctcatttccttcctttttttgtggtccctttttgtggtgatcattttaaaccacgtcatccaacaaatgttttatggtcaaccttagcttgttcataagccatagcaactgaaagattaaactcttaaatatgtgtctgggcagtggctattaaatagcaaaaaacaatcagattttagtattttattatttccttgtaaaatggctgaactaaattaaacccttgtttcccatttgttctataatttatagtgaaactgagaacaaaactatctttataaatgatagctaaaagtatttccagatatttaaacaatttaaaataaatttcttctgcagagatgcaaagcatctcaacactggaatgaacaaatgccttaaattcaatggagtaaacctttagaatgaagaggaactgtcatttcacccaagccgaagacaacagccttatgcacttgtgtgctctgtctttgctgcttctcgtgtttcaagcctttcctgtgggatcagcacagcaaagtgcaacttaccaaatggtttaatgactggttaattctttcttctcccaatggaaaagcaatggcaacacaacagtagactgctggcttgacaatcttaaacgtgagcctttgcacatgtaggtttatcatcatttgagtatacgactaagcaagtcaatgaactttttttttttttttagcagtttaatttggtcctgagaatgttgcagtctttattaccccttttgcattaatccacttttctaaccaccttttaagctttaatttttaacactatacaccaagtctttgaaatcagtgatctgttatttaactctaaagcatttgacacttcttgccttaacagttttaaaaaccacacacaaaaaaactctgtaagtaatacagtaggccaaaagtttcatcctatctatcttgcagtttacctatctgatctgatctctgtaattatagttctgtcatttaaaatatactatttaaatctaatttttacatttcaaaaattatcttcagtagtaactaagtatattttctgtggattctgagaatgttatttttcagaatgtgagaatatatatgtacatttataatcttgtgactttaaagtctgttttcagatacagtatgtaaatacttgtaaaaaaatttgtataattttgtgataatgtagtttcccaaaaaaattatttagaaggcattatgttattagtaaatgagagcactgtatagaactgttcctattttctgcacttgccattccagctgcctccactgtccatacccacctcattcatcctgtcacagaaggcaggaaaactgggaactttaccaaagtagcactcagcctgagaggcctgtataatcatgcttttcaaactaaattcacttaaaaattaaaaagcagaattgaatattttaagcagcctcagtacctttggccaatgctgttttcatggtggattatgaacattatataatctttgggaaaagtgaaagtagtacaatttttagaataatgacaactgcctcactgcatctctccactcacacagcaaccgtgtagccccctaagctgcagtaccatgactaaccatgatgtcaatttcatatgctgatcctcacaacagcagtgcacaaacatgccccaaatattttaacagaatttagctcttccttaagctgtcttttcatagtaaaaacaaaacaaaaacacccaatgttaaaaccacataataaacttacaaacttgaaaaattagacacttcagatagataggcaataaaacttcatattatgaaagcaatatattccaagtttcaaagatttgacaagttctgtagagtatctttcatcagtacatgaaaacttccaaactgcatgatcttctgccaggcaggactgggtgctattcgctggtttgaggtcgaatccatttcaaggcatgtcgtggtgggacattaatggtgggatggtagaatgtgcagtccggtcttgtacattgagtgttaaacctacaatgttttggatgatagaagggacattccatcttcttacaagcagggaagtaacggcagagctgactactggaaggtggtgctggtggtgcaactggttttggagacagtactggaattcttctactcacatgagtgaagggacaatctggtttagtacactttgcatcatatttacaatttgggtgaacaaacaaacatttttcagcaaatttacaattggggaaggctttgcagggtgagatggggtgatggtaggcacactcatccccatttttacaagcaggccagtacttgcagcgctccaaaagtttttctggtttctgtgccacactcagttcactcatctcagcttgactcatctgcagagtttctgccattactgggtcgatttgcagtcgggataataattgcctctgttgagttccttgatttttttctacagaatctccttttgtttcctcttctttaatggggggacttattctgggggtcctactttgtccctggaccacttctgctagcaattcttcttgagaagttcgagttctgggagcaactggaagtgtctgtttctgtggaactgtagagtagttagttgtttttgttacggattcttgagcttcagatatagccttcaaaatcagattcttgttagcttgtttagaaggtggaagagaaggtctcctttcaggctttgcaggcacagacacactgctggagatgcttcctgttcgagacccgtaatcatcatcttcttcctcctcttctccatcatgattgaatttttttactttaacaactgaacttaccacaggcaactttctcttccgaaagttttcatcctccatactcattttctccgagttgtttctaaagaacggactatacgtttcttctaagctgttaagcacctctggttcacacaaacgtcctgtttcatatacccaactactctgcatatcaagctgcttggcagcatgaatactattctgctgctgttgaaattgcaacctgtttaaatgaacaccactatctgcatttctacttgcaggtggtcgataaatttcaatagaagggcgagaagaaccatatgtaagtgtcactgtaggttttttctgagataagggattctcctgcacaaagttgaggtcttcgtcaatgagatcatctggttctggcttaatatcaatcacatcttcagagggtgctggctccctcaaaggtttcactgttgacattagtcgggttgcagctccatcatcgtaagtctgtctgacatttgtggtttttgactcctgcgaacttgtagaaactctggaatctcttttttcaggtctcgcgctaggaatggcaagtggtggcactgcagcttcatgcctcctctcatctccccgactgaaattgctcttgtttgaaggcacgttactatcaaagatgttggtatcagaagacttcagactagagggttcagttgtaacagagcgaagtttatctaatacaccatgaagccaacataagctcctaattcttgtaatttccccttaatggcactccggatcttgcggctgatctcggtgccgatctccatggctctgcggcgtgcgggaactcagcactgcgcggcgcttggcttacccggaggctgccgcggactcctaccccgcagccgggacaccaccgcctcc

SEQ ID NO: 13630 - RNA, 15851 nt, Homo sapiens
  source 1..15851: mol_type = other RNA
gctgggattacaggcatgagccaccataataaggattctgatgaacatttgattccttggactactgttatactcaaaagccttccttaatcttctaattgtcaccctaaatatcctaaaatttctgtcttcctagtagttcttcatagtcctaaaaatttgtcagagagaaaggtaaatcaagaaacatgattttcaaatgatttaaggtggtactagggtttaggatttcctttgctttttatcatttaacacactgcttatcatacagctggaagtgctctgggccagtgtctctacttcgagggaagaaggaggtagtgagacagaaggaaatagcacaattcctggccctgacagaagggtgttcaggagacctgctctcctctcactttattccatctcatctggacctgtggcttccaatccacatctctttcctttaatatcctgcattggctaggctgtataaatcctttggtgcatcgaaaaactaagtgcattttttgtttttgtgattatgcaatacttataggaaaagttataattttagaatatttaagtacacttacatttttgagaaaaagactattgaaatgtttgtgccatgtcaaatttcagttgaacattttgggtattcttaatataagaccaggccaggcaccgtggctcaggccgggcacagtggctcacacctataatcccagcacttagggaggccaaggcgggaagatcacctgaagtcaggagttcaagaccagcctggctaacaaggtgaaactctgtctctactaaaaatacaaaaattagccgggcgtggtggctggcgcttgtaatcccagctacttgggaggctgagacaggagaatcacttgaacctgggaagcagaggttgtggtgagctgagatcgcaccattgcactccagcctgggcaacaaagagcgaaactccgtctcaaaaaaataaaaaataaaccctagaattatagtatgttagaattggaagggaagaattgtctaaggttattctagctaataagcaacagacttggaaaggaaaaggtcctgacaaagctaagcctcccgttcaggtttcctgactcgtgaattcagtgctgctgccactacacgatgcatgctctttgtatcaagggtgagacagcattacacatacatagaaaattatctatttaaactctatttgaacttttgatgagtttgtctccccctcccccactccttttcagaataacttgacgtttacaggtaccatcagtggtgatgtctgtgtgtggaaagatcacatattgtgtagaatcgtggcgagagctcacaacgggcctgtgtttgccatgtacaccaccctgcgagatggacttatcgtgactgggggaaaggaaaggccgtgagtcctctttcttttcacagaatatttatgcatttgtgacctacctgaggtttgcagttaattattctagttgtttctaggctacacagagtgtcctctccgaccttcctcctcatatgcttctcctttattaccttttatgtgccttctatttgattctcatttctggtcttaattcacttccaatttttttcatgttggggtgatactttttctgaggtgtggataggtagttgtcctacaagttgagttacttttcttaatgtctgtatgcctgtgtatgatttgctgagtaggaggcccatgggggaatctggagccagggttgtattttgactgcctgctctctttttgttcagaatggattctaaggagtagaatgcacattgttgctttagaaaaggatgagggaactagagagaactgccttgtttccttttgcttgaggcaaatttaaactgttttatacaagacctcaaaatttgagaagaggtctcttctgagtgattttcaaatctcccaacagtaaccagatacttatgatttgatttgtcaccaacatagtcatatgcatgttgaaacatgacatgtaggccaggcacagtggctcacacctgtaatcttatcactttgggaggctgaggcaggtggatcgcttgagcccaggagttcaagaccagcctgggcaacatggtgaaaccccatcgctataaaaaacaacaattagccgggtgtggtggcacatgcctgtagtccctgctactcaggaggctgaggtgggaggatcacttgagcctggggaggtcaaggctttagtgagctgtgatggtgccactgcactccagcctgggtgacagagtgagaccccatttaaaaaacaaaaacaaaaacaaaaaaaaatgtgacatatagttgactaagaagtacatttcaatacaggattgaaagaacccacatatgttaattaaacacaagcgcagaatttgtgccttttacataaaggaagaatgcacataggcatgctttcagacaagcaattcatctagcagaaaaggaaggaatacatttttcagcccttccaggaataaaatccataaatgggctctatttcgtcctccaacacttgtatttcccacgtcatttactcctgcacacccccactcactagaagcctgctaaactgttccagtgagatattttaacacctgatagggaataaatatgcttctgttttggccttcaaaaataagctctgggccagttgcagtggctcacgcctgtaatcccaacactttgggaggccgaggtgggcggatcacgaggtcaggagtttgggatcagcctggccaatatggtgaaactccatctctactaaaaatacaaaaattagccaggcatggtgcctgtaatcccagctacttgggaggctgaaggagaagaatcgcttgaacctgggaggcacaggttgcagtgagccgagatcacaccactgcactccaggccaggtgacagagcgacactctgtctcaaaaaaataaataaatcaactctgtagcatagcatttgtaattctattattttgccttacatttccattatccttttaataaaattgtttttttacatcttcctaatcaagaagtattatgaggccaggcacagtggctcatacctggaatcccagcactttgggaggccgaggcaggcagatcacctgaggtcaaggtatttgagaccagcctggccaacatggtgaaaccccatctctactaaaaatacagaaattagctgggtgtggtggtgcacacctgtaatgctagctactcgggaggctgaggtaggagaatcgcttgaacctgggaggcagaggttgcaataagcctagatcatgccactgcactcaagcctgggagacagagcgagactacatcttaaaaaaaaaaaaaaaagtattatgagagaggataatgtattgtaatgtattgtagaggctaaataaaattatgctcatgtcagaaaaaaagagtatttctcaaaataaaattcactgaaactggatgtttattttgactgagatatagtatatcctcaaattgccatagaaagtttacaagaatattagaggtaaattataaatatcagggcctttttaaaaaaaaaagattctgcttataacttggtatttgtttataataaaaattatagtagccaataatgaacacttactctggcttggttatttacttaggtcaaaagaaggaggagcggttaaactgtgggatcaggaactgaggcggtgccgtgccttcaggcttgagacaggacaagccacagattgtgttcgttctgtgtgcagaggcaaagtaagatgttccatgagctgatacagtgcagcagaaaacagaaagtggttattactgtgattccctcaccctttgcagcctaatgaacaatacttaataatgcataacgatggatttgcttgccaacattactctgtctttgctgctttctttgccaaagttagcaccagtgtggtgcataagctaggaagctattctgtctaaatactgtatgtaaacctccaatattttctagaatctgccaatttaacaactctagtagacataattgaaagcccttggcagttgactcatattaggacagctgtctccattttttaaaaaaacacacattccctagataaaacgtgcagtaaacaaacaatgaaatactactcagccataaaaaataatgaaattctgtcattcttggtggcaacatggatgagactggaggacatgatgtgaagtgaaataagccaggcacagaaagataaatacatgttctcactcctgtgcagaaactaaaaaagttgatcccacagaggtggagagtagaatagtggttactggaggcggacaagggggagggggagggggatagggaaggactggttaaaggatacaagtttacacagccagataggaatagtatgttttagtattctgtagtactgtaggatgactatagttaagaatcacgtatttatgtattttcaggtatttacaagagaggattttgaaagtttccatcacaaagaaatgataaatgtctgaggtgatggttatgcgtattaccctatgccctatagatatgtataattatgtgtcaatttcaaaataaaaattcaaaactacaactcctatgaaaatttttgagcgtgtttgtacttattaagtgtatttataaatcatacggatattatcttcagcctgcatattaaattgtagttaagcttttactttttaactaaaaaataaattctattattttttcctatatcccactgcactgaccccagtttggaaatcctaagattatcaaataaaaactttgattattgaagaatccaggtgtactgccacagaaaagttctattctgtagcatggactctaatatgtaatctagcccattgtgcttacagatagatgtgtgcctgtagtcatagaaaaatttgcatgagctaatgactgccttgctactagattagctcaaagcaaaaagttctctgaaagcaggtcaatagggtcatttttatattatgaagaagaaaagcagctgttgtattacattcactgtattggtcctgcttgtgtttcagggcaagatccttgttgggacaaggaatgctgaaataatcgaagttggagagaaaaatgcagcttgtaatattttagttaacggtcatgtggatgggccaatctggggactagcaacacatccttccagggattttttcctttctgctgcagaagatgggacagtgagactttgggatattgctgataaagtaagtacagataatttttttaaaagaggttacaacttctaaaaagaaaagttggaagttctaaattgctagtacttaaagaactgccagaattctgttgagcattttgaggggaaactggtataatttagaagtacttcacttaatgtttcctatgactctttttttttttttttttaaatgcagaagatgttaaacaaagtgaatttgggacatgctgctcgtactgtgtgttacagccctgaaggggacatggtggctattggaatgaaaaatggagaatttatcattttactagtgagttctctaaaaatatggggaaagaagagagacaggagatgtgcaatccatgatatcaggttagtgaacaaatggaatagagtttctagtatatacttgatttaacttccatttgtaaaattttccatagccttgccttcaaaaagaggtccccagggcctgtagcatttcccgtattataaattgtatgctaaaatatggctgtttgtatactacttaattcttcttgctaaattataaacccactgggcaccaactataatagcaagtactagtaggtaatgtttgatgaattcatgttaacacttagccatgtccattaagttcatcccaccaagaggtatctcccactgtaatacaagagagctatctgcccttcaaaagttgtcaccctggaaaactaaagttgtgatttcaaacatatcttctcttagtaacctcagtttgggaatatgtagttcattaatttaatcaatacctattgattaaatgttccagaatccaaattaatttaaatgtttcttaaacctttgtttttcagtgcttaagcatttttcaacagtggctaccatttacggagtacttccgtgtgatcagtagataagattattgaatctaggtctgtcaaaagcttgtacacttttcatcagtaaaatccttttacaaatgaaaccttcctcagaacttcaatatataaaatagtaacagtggcttcccttagcttttacatgtctctatcgtacctcagtaagactcatgggccatttcaagagactgaattgtcccatatgactccaaagattgctaggcaaatagcatttcactttgtcttttaaataagttcttcaggccgggcgcggtggctcatgcctgtaatcccagcactttgggaggccgaggcaggcagatcacctgaagtcaggagtactcgaccagcctggccaacatagtgaaaccccatctcaactaaaaatacaaaaatcagccgggcgtggtggcaggcgcctgtaatcccagctactcagggggctgaaacaggagaatcgcttgaacccgggaggcggaggttgcgccatcgcactccagcctgggagacaagagcgagacttcgtctcaaaaaaaaaaaattcttcttccaagattcaagttgtgtcatttcaccttaataactggaggttagttaagctgggctgtgttctttgcttaatattaagacaacgttttttccagatggaagaaaactatcttaatgaattgttagcttattaattatgtaatgctaatggcttttaaaagctgagatgttctgactgggtgttgtggctcacacctgtaatcccagtaccttgggaggccaagggggaaggattgcttgaggccaggagtttgggaccatagtgagaccccgcctctatttaaaaaattaaattttgttttgttttgttttgagttggagttttgctcttgttgcccatgctgaagtgcaatggtgcaatctcagctcaccacaacctgtgcctcctgggttcaagcgattctcctgcttcagcctcccgagtagatgggattacaggcgtgcaccaccatgcctggctaattttgtatttttagtagagacagggtttctctatgttggtcaggctggtctcaaactctcgacctcaggtgatctgcccgcctccgcttcccaaagttctgggattataggtgtgagccactgggcctggcctaagaaagtttttttaagccattagacgtttttaaaggaattgggagatgacaattggggaaatatttaaaatttaagtaaaatataaagcttccttatttcatgtaacccagacaatctcagtatacatgatcagttgtgtctgacaggtaaatctatttgaggccttatcacacgttacttttaagaactagaaaggaaaagtcactgatcttaagtatttataatacttcatgtggtctaatactttttacgttttgttttgattcagatttagtccggattcccggtatctggcagtaggttctagtgagaactcagtggatttttatgacctaacgctgggccccactcttaacagaatcagctactgcaaagacattccaagctttgtcattcaaatggacttctctgcagatagcagttatctccaggtacagtaccaatactgtatacccaggtggcaagttcttctgcttttacatttcgtgttagtgaatgcatttaaagttcctgagctccagagctccagcttctcaactcctccctttgtaccttctgacctacagctcccctttcctcccccacttatcagagcttttctcctattaagtttttgtagtgatcttttgcatacttaataatgttagacatgtaaatcaagtagcaatatgctagtattctgtaaaccccctgtggattttgtctctcacctaatggaattcttgtcccattttaatctgatgaaaaaggtctctagtggctgctataaacggcatgtctatgaagtgccttcaggaaaacatcttatggatcatgccgctattgacagaattacttgggctacatggactaggtaaatacttatatattcacaaggcaagaactgactttgaaggccagttagaaaatcctatttctgaactgttagagccattccaataaggaatagtaattgagtttcaagtttttgttaccatattttgaaatggtatgttcatgttgggacccctttttattgaatatatttccatgttttatcagtttccatgatttatcaagttttttttttaaggaaatcaaagttttaactttaaagataccctgatatttttcttaatgctaaatttaatgactggcaaaaaggtattgggtgctgttaagcaactgttattaattctctatctaaaggaatgctatcttgaatctattagaagtcaaagcttccaaatttgttcaaatttcctggctgtatgacaggtaaccatgactatccatttttttggccaatgaaaaatgccatcaaattcctgtatcagccaggcatatagtggctcatgcctgtaatctctgatgtagcaggccgaggtgggaggatcacttgagcctagaagttttgataccagcctgggcaacatagcaagaccccatctctgaaatttttttaattcctatgtcataagtcatttttatttttgtagagatagggatctcacaatattgcccaggctggtctcaaactcttggcctcaagcagtcctcctgcctcagcctcccaaaatgttgggattactggtatgtgctgctggacccagccaagtagcacttttaatttgaaaaatagttctatcagttttcagtcaggcgcggtggctcagcctgtaatcccagcactttgggaggccgagcgggggtgatcacctgaggtcgggagttcgagactagcctgaccaacatggagaaaccctgtctctactaaaaatacaaaataagccgggcatgttagcgcatgcctgtgatcccagctactcgggaggctgaggcaggagaattgcttgaacccaggaggcagaggttgcggtgagccgagatcatgccattgcactccagcctgggtaacaagagcgaaaactccgtctcaaaaaaaaaaaaagaaaaaatagttctatcagttttcataaagtactactttaatcttaaaaagattaatctagaaacccttcaaattataaaatgtcatttttaaaaggcaggagttgatatcctgatgaaattcaggtctccaaacaacttaccataatttacttcctgtattttaagtaacatgatagggtacttagagattaattgccaagaaactttttgaatatagtcaacctgcccgcacttgccatgatgagttttcttttgttccttccctctagtattctaggagatgaggttttgggaatctggtccagacatgctgagaaagctgatgtcaactgtgcctgtgtatctcattcaggaatcagtcttgttacaggagatgactttggcatggttaagttatttgacttcccatgtccagaaaaatttgtaagtttgtgttttgtttactattatcagtttactcctaattttgatgtcttatcatcagcacttttccccatatatttaaaatgttttgtcctaatttctaaatttttccccaaactttctaaatctatttactttgaaataaaagctattagaaacaaatcctctccctcgagtaataccatctttggaaccatcctacaaaagctgtaattagcttttcaccaaacctataatcagttatcaaatttcaaatgcttttccttagagaaaaatggtcagagtacctggagacatctgactgcccacacagcctggttttgcagatccactactcatgctgaaaagcattctaatcactggctgcggtgctaactccctactctctccacagctcttgtcatagagattatagttcctaataagagcctttgacttctgtgtgcaccaaatgccctgagcttgtctgtcattgttttttaggcaaaacacaaaaggttcttgggtcattcgccccatgtgacaaatattcgatttaccagtggtgatcgacatgttgttagtgctggaggtgatgactgcaggttagtaactttctcagcccatgaagagcagactatgttactagttaagagacttaatacaacaactcctacagctttggtttatgaaatcagctagtcaacattagtagaaggtagtataaccagatggctcttcagaatctcatatttatgcaaatacagaataaaaggagttaaagaggaaaaatattacacatgtaacctgaaagcacaactgaaaaatattaaactgttatgaaaatctaaaaacataattaactccctgcaattttcttctctgattgcagcttatttgtctggaaatgtgtacatacacctcactgagagatgctgagatgactacagaaattaactttgagaccagaattacagagaagaaaaaccaaaacccaaccctgcatggtcaagtggtgctaacccaagactgtaacagggagaaatgcccagaatcatcaaaatagtgaaagactgatctgttcaaaatatttgctatatgcactgggtataatccgtaatccatacactgccagataatgccatttcaaggaaggatcgaatacttgatggtaaaggccaagtccccctgtattgggaagtgtgtgatttcggcagacctgctgggaaaatttagggtagagcactctttacagaagaactcaaaaacccaatttggataattttcattatctttttagcaaaatggtttcttaatgtttatattttattttcaaggttcattgtttaatgaaatattttattcttgcatttccataaggaaagggaaagtcatgatcatcctaaaggatcacagtttttaaaaggcaaacattttccctaaggaaacagacacaagctttcctagagaatatgatgttttttaggcattaataaggtccttttttataaaggacacttttctcctagtagttttgaattcaggaacagatccaaagttagcagtatatggctgctacatttccattttcattttcgagccatcagtttatgttcagatgccatctctgtaatcgcacatttaaaacataactgtagcctcactaatggaaaagtagtatgatgaacaatcattcccaatggtgtacaatgtaagggttttagggagcaacagtatttaactggaagaaagaattgcatatttaatgtagtctaatatatacacatttgtttaacatgtaaacaaaagtgttaaattcacatatacaacattatacaatttaatcactcttggaataaaatttttatagccttttttctattgggaaaatttgtttagatgtgtgccactccataggtttatttccaaaatgaatgagcccaactccatttgtaaaaacttgtcagttagaattcctttttttagtggattagggctgaattcttagatccttatttcttttcactttaaatgctgccaaagatcactactcatcattcaggaattcgctgtctagcctatctgtagtttcctgaagattgaaaattatgtagactgctatttaaaaatatatttttctaagtgtgaggtttaagatgctgtattgaccctatgagtttttaatgtgttaattatctttatagcataatagatcgctttaggttcctggaatcccatttggtctgacaggatatatgaagattcttaatacctattttctgtgtctaatacttggttaatactaaaaatagaaatgactaaattacatcacagaaagcataaccagtgattgaacctggtagttttaaagctctaaatagctgtggctgaaggactgattatggggctaagaagcttgaaacgtaagttggtacttgttcatcagtggattctcctaaattaagccaaattttgaaatacatgactattaagtttctactcatgtatttacagtcagtcaataaattaaaggaggaaaaaaatccctgaacaacctgcccataaaaagaaaaatactctacatttgagcctgctgcagttttaaattttccctctgggtcaagtttgccagcttttggctacagagaaattatatttccattacagtgcaggtagaaactctgtaaccttaagcatgtaaactacatagaataaaactgtttccactgcatttctgtccttcaaagtggccaacctgattaagtcagccttaatcactgctgctgtcagtttcacgactaaaggtcatattgactaagtagtcatcagctgaccacctcgctgtatcagccagcaacgaggggaaggtgaagaaacatgataggccatatagaatctgccctatgtttacttttttaacccagataattatttttgtgtgcagtatctaagctcctgattgtgtaacctgggacttctggcaccttttgttccattcattttatgtataaaatgcatgccaaagcacactgtgccctctggtacccttgcttccaatcgccaaccatgctcatttccttcctttttttgtggtccctttttgtggtgatcattttaaaccacgtcatccaacaaatgttttatggtcaaccttagcttgttcataagccatagcaactgaaagattaaactcttaaatatgtgtctgggcagtggctattaaatagcaaaaaacaatcagattttagtattttattatttccttgtaaaatggctgaactaaattaaacccttgtttcccatttgttctataatttatagtgaaactgagaacaaaactatctttataaatgatagctaaaagtatttccagatatttaaacaatttaaaataaatttcttctgcagagatgcaaagcatctcaacactggaatgaacaaatgccttaaattcaatggagtaaacctttagaatgaagaggaactgtcatttcacccaagccgaagacaacagccttatgcacttgtgtgctctgtctttgctgcttctcgtgtttcaagcctttcctgtgggatcagcacagcaaagtgcaacttaccaaatggtttaatgactggttaattctttcttctcccaatggaaaagcaatggcaacacaacagtagactgctggcttgacaatcttaaacgtgagcctttgcacatgtaggtttatcatcatttgagtatacgactaagcaagtcaatgaactttttttttttttttagcagtttaatttggtcctgagaatgttgcagtctttattaccccttttgcattaatccacttttctaaccaccttttaagctttaatttttaacactatacaccaagtctttgaaatcagtgatctgttatttaactctaaagcatttgacacttcttgccttaacagttttaaaaaccacacacaaaaaaactctgtaagtaatacagtaggccaaaagtttcatcctatctatcttgcagtttacctatctgatctgatctctgtaattatagttctgtcatttaaaatatactatttaaatctaatttttacatttcaaaaattatcttcagtagtaactaagtatattttctgtggattctgagaatgttatttttcagaatgtgagaatatatatgtacatttataatcttgtgactttaaagtctgttttcagatacagtatgtaaatacttgtaaaaaaatttgtataattttgtgataatgtagtttcccaaaaaaattatttagaaggcattatgttattagtaaatgagagcactgtatagaactgttcctattttctgcacttgccattccagctgcctccactgtccatacccacctcattcatcctgtcacagaaggcaggaaaactgggaactttaccaaagtagcactcagcctgagaggcctgtataatcatgcttttcaaactaaattcacttaaaaattaaaaagcagaattgaatattttaagcagcctcagtacctttggccaatgctgttttcatggtggattatgaacattatataatctttgggaaaagtgaaagtagtacaatttttagaataatgacaactgcctcactgcatctctccactcacacagcaaccgtgtagccccctaagctgcagtaccatgactaaccatgatgtcaatttcatatgctgatcctcacaacagcagtgcacaaacatgccccaaatattttaacagaatttagctcttccttaagctgtcttttcatagtaaaaacaaaacaaaaacacccaatgttaaaaccacataataaacttacaaacttgaaaaattagacacttcagatagataggcaataaaacttcatattatgaaagcaatatattccaagtttcaaagatttgacaagttctgtagagtatctttcatcagtacatgaaaacttccaaactgcatgatcttctgccaggcaggactgggtgctattcgctggtttgaggtcgaatccatttcaaggcatgtcgtggtgggacattaatggtgggatggtagaatgtgcagtccggtcttgtacattgagtgttaaacctacaatgttttggatgatagaagggacattccatcttcttacaagcagggaagtaacggcagagctgactactggaaggtggtgctggtggtgcaactggttttggagacagtactggaattcttctactcacatgagtgaagggacaatctggtttagtacactttgcatcatatttacaatttgggtgaacaaacaaacatttttcagcaaatttacaattggggaaggctttgcagggtgagatggggtgatggtaggcacactcatccccatttttacaagcaggccagtacttgcagcgctccaaaagtttttctggtttctgtgccacactcagttcactcatctcagcttgactcatctgcagagtttctgccattactgggtcgatttgcagtcgggataataattgcctctgttgagttcctttctcaacgtttctaaggaagccgattatttttacatcagtagttcttgactgtgattcagtatcttcttcttgatcttcaaactgtctgttgcattcatatgttgttgaatattcattcattttaacctccaaagatgaaatttttgcttcattcttggacactctaacatttagatcaaaaagatttgcttccactgtcaaaatagctgctttcattcctttaatttcattgatatcagctgatattttccttaaaaggtgggaaatattgtctagctcattcagtgaacaagaggagcttgttatggaacctaagtccactggctccggtggaagaaaaattggtagaggtggtgatggaaactttgaagacattctcataaaggtgacaggaacctcaaagacattttcataaaattctctcccttaaaatctgataattttttcttcacagctcattaagttatttcatcgaaagtaaaagcagtgatcaaggctgttaccttaagacgtattaagagcaaataacatcttaaaacctgtaattcaaaagatggggttgtacatttctagagtcagaattcaaaactaaatgtgaaaaagctaaacgtaccagaccaattgctcttcgctacaactaagaagccctaatacgtagggccctacatcctctaagtaccatctgtat

SEQ ID NO: 13631 - RNA, 16345 nt, Homo sapiens
  source 1..16345: mol_type = other RNA
gctgggattacaggcatgagccaccataataaggattctgatgaacatttgattccttggactactgttatactcaaaagccttccttaatcttctaattgtcaccctaaatatcctaaaatttctgtcttcctagtagttcttcatagtcctaaaaatttgtcagagagaaaggtaaatcaagaaacatgattttcaaatgatttaaggtggtactagggtttaggatttcctttgctttttatcatttaacacactgcttatcatacagctggaagtgctctgggccagtgtctctacttcgagggaagaaggaggtagtgagacagaaggaaatagcacaattcctggccctgacagaagggtgttcaggagacctgctctcctctcactttattccatctcatctggacctgtggcttccaatccacatctctttcctttaatatcctgcattggctaggctgtataaatcctttggtgcatcgaaaaactaagtgcattttttgtttttgtgattatgcaatacttataggaaaagttataattttagaatatttaagtacacttacatttttgagaaaaagactattgaaatgtttgtgccatgtcaaatttcagttgaacattttgggtattcttaatataagaccaggccaggcaccgtggctcaggccgggcacagtggctcacacctataatcccagcacttagggaggccaaggcgggaagatcacctgaagtcaggagttcaagaccagcctggctaacaaggtgaaactctgtctctactaaaaatacaaaaattagccgggcgtggtggctggcgcttgtaatcccagctacttgggaggctgagacaggagaatcacttgaacctgggaagcagaggttgtggtgagctgagatcgcaccattgcactccagcctgggcaacaaagagcgaaactccgtctcaaaaaaataaaaaataaaccctagaattatagtatgttagaattggaagggaagaattgtctaaggttattctagctaataagcaacagacttggaaaggaaaaggtcctgacaaagctaagcctcccgttcaggtttcctgactcgtgaattcagtgctgctgccactacacgatgcatgctctttgtatcaagggtgagacagcattacacatacatagaaaattatctatttaaactctatttgaacttttgatgagtttgtctccccctcccccactccttttcagaataacttgacgtttacaggtaccatcagtggtgatgtctgtgtgtggaaagatcacatattgtgtagaatcgtggcgagagctcacaacgggcctgtgtttgccatgtacaccaccctgcgagatggacttatcgtgactgggggaaaggaaaggccgtgagtcctctttcttttcacagaatatttatgcatttgtgacctacctgaggtttgcagttaattattctagttgtttctaggctacacagagtgtcctctccgaccttcctcctcatatgcttctcctttattaccttttatgtgccttctatttgattctcatttctggtcttaattcacttccaatttttttcatgttggggtgatactttttctgaggtgtggataggtagttgtcctacaagttgagttacttttcttaatgtctgtatgcctgtgtatgatttgctgagtaggaggcccatgggggaatctggagccagggttgtattttgactgcctgctctctttttgttcagaatggattctaaggagtagaatgcacattgttgctttagaaaaggatgagggaactagagagaactgccttgtttccttttgcttgaggcaaatttaaactgttttatacaagacctcaaaatttgagaagaggtctcttctgagtgattttcaaatctcccaacagtaaccagatacttatgatttgatttgtcaccaacatagtcatatgcatgttgaaacatgacatgtaggccaggcacagtggctcacacctgtaatcttatcactttgggaggctgaggcaggtggatcgcttgagcccaggagttcaagaccagcctgggcaacatggtgaaaccccatcgctataaaaaacaacaattagccgggtgtggtggcacatgcctgtagtccctgctactcaggaggctgaggtgggaggatcacttgagcctggggaggtcaaggctttagtgagctgtgatggtgccactgcactccagcctgggtgacagagtgagaccccatttaaaaaacaaaaacaaaaacaaaaaaaaatgtgacatatagttgactaagaagtacatttcaatacaggattgaaagaacccacatatgttaattaaacacaagcgcagaatttgtgccttttacataaaggaagaatgcacataggcatgctttcagacaagcaattcatctagcagaaaaggaaggaatacatttttcagcccttccaggaataaaatccataaatgggctctatttcgtcctccaacacttgtatttcccacgtcatttactcctgcacacccccactcactagaagcctgctaaactgttccagtgagatattttaacacctgatagggaataaatatgcttctgttttggccttcaaaaataagctctgggccagttgcagtggctcacgcctgtaatcccaacactttgggaggccgaggtgggcggatcacgaggtcaggagtttgggatcagcctggccaatatggtgaaactccatctctactaaaaatacaaaaattagccaggcatggtgcctgtaatcccagctacttgggaggctgaaggagaagaatcgcttgaacctgggaggcacaggttgcagtgagccgagatcacaccactgcactccaggccaggtgacagagcgacactctgtctcaaaaaaataaataaatcaactctgtagcatagcatttgtaattctattattttgccttacatttccattatccttttaataaaattgtttttttacatcttcctaatcaagaagtattatgaggccaggcacagtggctcatacctggaatcccagcactttgggaggccgaggcaggcagatcacctgaggtcaaggtatttgagaccagcctggccaacatggtgaaaccccatctctactaaaaatacagaaattagctgggtgtggtggtgcacacctgtaatgctagctactcgggaggctgaggtaggagaatcgcttgaacctgggaggcagaggttgcaataagcctagatcatgccactgcactcaagcctgggagacagagcgagactacatcttaaaaaaaaaaaaaaaagtattatgagagaggataatgtattgtaatgtattgtagaggctaaataaaattatgctcatgtcagaaaaaaagagtatttctcaaaataaaattcactgaaactggatgtttattttgactgagatatagtatatcctcaaattgccatagaaagtttacaagaatattagaggtaaattataaatatcagggcctttttaaaaaaaaaagattctgcttataacttggtatttgtttataataaaaattatagtagccaataatgaacacttactctggcttggttatttacttaggtcaaaagaaggaggagcggttaaactgtgggatcaggaactgaggcggtgccgtgccttcaggcttgagacaggacaagccacagattgtgttcgttctgtgtgcagaggcaaagtaagatgttccatgagctgatacagtgcagcagaaaacagaaagtggttattactgtgattccctcaccctttgcagcctaatgaacaatacttaataatgcataacgatggatttgcttgccaacattactctgtctttgctgctttctttgccaaagttagcaccagtgtggtgcataagctaggaagctattctgtctaaatactgtatgtaaacctccaatattttctagaatctgccaatttaacaactctagtagacataattgaaagcccttggcagttgactcatattaggacagctgtctccattttttaaaaaaacacacattccctagataaaacgtgcagtaaacaaacaatgaaatactactcagccataaaaaataatgaaattctgtcattcttggtggcaacatggatgagactggaggacatgatgtgaagtgaaataagccaggcacagaaagataaatacatgttctcactcctgtgcagaaactaaaaaagttgatcccacagaggtggagagtagaatagtggttactggaggcggacaagggggagggggagggggatagggaaggactggttaaaggatacaagtttacacagccagataggaatagtatgttttagtattctgtagtactgtaggatgactatagttaagaatcacgtatttatgtattttcaggtatttacaagagaggattttgaaagtttccatcacaaagaaatgataaatgtctgaggtgatggttatgcgtattaccctatgccctatagatatgtataattatgtgtcaatttcaaaataaaaattcaaaactacaactcctatgaaaatttttgagcgtgtttgtacttattaagtgtatttataaatcatacggatattatcttcagcctgcatattaaattgtagttaagcttttactttttaactaaaaaataaattctattattttttcctatatcccactgcactgaccccagtttggaaatcctaagattatcaaataaaaactttgattattgaagaatccaggtgtactgccacagaaaagttctattctgtagcatggactctaatatgtaatctagcccattgtgcttacagatagatgtgtgcctgtagtcatagaaaaatttgcatgagctaatgactgccttgctactagattagctcaaagcaaaaagttctctgaaagcaggtcaatagggtcatttttatattatgaagaagaaaagcagctgttgtattacattcactgtattggtcctgcttgtgtttcagggcaagatccttgttgggacaaggaatgctgaaataatcgaagttggagagaaaaatgcagcttgtaatattttagttaacggtcatgtggatgggccaatctggggactagcaacacatccttccagggattttttcctttctgctgcagaagatgggacagtgagactttgggatattgctgataaagtaagtacagataatttttttaaaagaggttacaacttctaaaaagaaaagttggaagttctaaattgctagtacttaaagaactgccagaattctgttgagcattttgaggggaaactggtataatttagaagtacttcacttaatgtttcctatgactctttttttttttttttttaaatgcagaagatgttaaacaaagtgaatttgggacatgctgctcgtactgtgtgttacagccctgaaggggacatggtggctattggaatgaaaaatggagaatttatcattttactagtgagttctctaaaaatatggggaaagaagagagacaggagatgtgcaatccatgatatcaggttagtgaacaaatggaatagagtttctagtatatacttgatttaacttccatttgtaaaattttccatagccttgccttcaaaaagaggtccccagggcctgtagcatttcccgtattataaattgtatgctaaaatatggctgtttgtatactacttaattcttcttgctaaattataaacccactgggcaccaactataatagcaagtactagtaggtaatgtttgatgaattcatgttaacacttagccatgtccattaagttcatcccaccaagaggtatctcccactgtaatacaagagagctatctgcccttcaaaagttgtcaccctggaaaactaaagttgtgatttcaaacatatcttctcttagtaacctcagtttgggaatatgtagttcattaatttaatcaatacctattgattaaatgttccagaatccaaattaatttaaatgtttcttaaacctttgtttttcagtgcttaagcatttttcaacagtggctaccatttacggagtacttccgtgtgatcagtagataagattattgaatctaggtctgtcaaaagcttgtacacttttcatcagtaaaatccttttacaaatgaaaccttcctcagaacttcaatatataaaatagtaacagtggcttcccttagcttttacatgtctctatcgtacctcagtaagactcatgggccatttcaagagactgaattgtcccatatgactccaaagattgctaggcaaatagcatttcactttgtcttttaaataagttcttcaggccgggcgcggtggctcatgcctgtaatcccagcactttgggaggccgaggcaggcagatcacctgaagtcaggagtactcgaccagcctggccaacatagtgaaaccccatctcaactaaaaatacaaaaatcagccgggcgtggtggcaggcgcctgtaatcccagctactcagggggctgaaacaggagaatcgcttgaacccgggaggcggaggttgcgccatcgcactccagcctgggagacaagagcgagacttcgtctcaaaaaaaaaaaattcttcttccaagattcaagttgtgtcatttcaccttaataactggaggttagttaagctgggctgtgttctttgcttaatattaagacaacgttttttccagatggaagaaaactatcttaatgaattgttagcttattaattatgtaatgctaatggcttttaaaagctgagatgttctgactgggtgttgtggctcacacctgtaatcccagtaccttgggaggccaagggggaaggattgcttgaggccaggagtttgggaccatagtgagaccccgcctctatttaaaaaattaaattttgttttgttttgttttgagttggagttttgctcttgttgcccatgctgaagtgcaatggtgcaatctcagctcaccacaacctgtgcctcctgggttcaagcgattctcctgcttcagcctcccgagtagatgggattacaggcgtgcaccaccatgcctggctaattttgtatttttagtagagacagggtttctctatgttggtcaggctggtctcaaactctcgacctcaggtgatctgcccgcctccgcttcccaaagttctgggattataggtgtgagccactgggcctggcctaagaaagtttttttaagccattagacgtttttaaaggaattgggagatgacaattggggaaatatttaaaatttaagtaaaatataaagcttccttatttcatgtaacccagacaatctcagtatacatgatcagttgtgtctgacaggtaaatctatttgaggccttatcacacgttacttttaagaactagaaaggaaaagtcactgatcttaagtatttataatacttcatgtggtctaatactttttacgttttgttttgattcagatttagtccggattcccggtatctggcagtaggttctagtgagaactcagtggatttttatgacctaacgctgggccccactcttaacagaatcagctactgcaaagacattccaagctttgtcattcaaatggacttctctgcagatagcagttatctccaggtacagtaccaatactgtatacccaggtggcaagttcttctgcttttacatttcgtgttagtgaatgcatttaaagttcctgagctccagagctccagcttctcaactcctccctttgtaccttctgacctacagctcccctttcctcccccacttatcagagcttttctcctattaagtttttgtagtgatcttttgcatacttaataatgttagacatgtaaatcaagtagcaatatgctagtattctgtaaaccccctgtggattttgtctctcacctaatggaattcttgtcccattttaatctgatgaaaaaggtctctagtggctgctataaacggcatgtctatgaagtgccttcaggaaaacatcttatggatcatgccgctattgacagaattacttgggctacatggactaggtaaatacttatatattcacaaggcaagaactgactttgaaggccagttagaaaatcctatttctgaactgttagagccattccaataaggaatagtaattgagtttcaagtttttgttaccatattttgaaatggtatgttcatgttgggacccctttttattgaatatatttccatgttttatcagtttccatgatttatcaagttttttttttaaggaaatcaaagttttaactttaaagataccctgatatttttcttaatgctaaatttaatgactggcaaaaaggtattgggtgctgttaagcaactgttattaattctctatctaaaggaatgctatcttgaatctattagaagtcaaagcttccaaatttgttcaaatttcctggctgtatgacaggtaaccatgactatccatttttttggccaatgaaaaatgccatcaaattcctgtatcagccaggcatatagtggctcatgcctgtaatctctgatgtagcaggccgaggtgggaggatcacttgagcctagaagttttgataccagcctgggcaacatagcaagaccccatctctgaaatttttttaattcctatgtcataagtcatttttatttttgtagagatagggatctcacaatattgcccaggctggtctcaaactcttggcctcaagcagtcctcctgcctcagcctcccaaaatgttgggattactggtatgtgctgctggacccagccaagtagcacttttaatttgaaaaatagttctatcagttttcagtcaggcgcggtggctcagcctgtaatcccagcactttgggaggccgagcgggggtgatcacctgaggtcgggagttcgagactagcctgaccaacatggagaaaccctgtctctactaaaaatacaaaataagccgggcatgttagcgcatgcctgtgatcccagctactcgggaggctgaggcaggagaattgcttgaacccaggaggcagaggttgcggtgagccgagatcatgccattgcactccagcctgggtaacaagagcgaaaactccgtctcaaaaaaaaaaaaagaaaaaatagttctatcagttttcataaagtactactttaatcttaaaaagattaatctagaaacccttcaaattataaaatgtcatttttaaaaggcaggagttgatatcctgatgaaattcaggtctccaaacaacttaccataatttacttcctgtattttaagtaacatgatagggtacttagagattaattgccaagaaactttttgaatatagtcaacctgcccgcacttgccatgatgagttttcttttgttccttccctctagtattctaggagatgaggttttgggaatctggtccagacatgctgagaaagctgatgtcaactgtgcctgtgtatctcattcaggaatcagtcttgttacaggagatgactttggcatggttaagttatttgacttcccatgtccagaaaaatttgtaagtttgtgttttgtttactattatcagtttactcctaattttgatgtcttatcatcagcacttttccccatatatttaaaatgttttgtcctaatttctaaatttttccccaaactttctaaatctatttactttgaaataaaagctattagaaacaaatcctctccctcgagtaataccatctttggaaccatcctacaaaagctgtaattagcttttcaccaaacctataatcagttatcaaatttcaaatgcttttccttagagaaaaatggtcagagtacctggagacatctgactgcccacacagcctggttttgcagatccactactcatgctgaaaagcattctaatcactggctgcggtgctaactccctactctctccacagctcttgtcatagagattatagttcctaataagagcctttgacttctgtgtgcaccaaatgccctgagcttgtctgtcattgttttttaggcaaaacacaaaaggttcttgggtcattcgccccatgtgacaaatattcgatttaccagtggtgatcgacatgttgttagtgctggaggtgatgactgcaggttagtaactttctcagcccatgaagagcagactatgttactagttaagagacttaatacaacaactcctacagctttggtttatgaaatcagctagtcaacattagtagaaggtagtataaccagatggctcttcagaatctcatatttatgcaaatacagaataaaaggagttaaagaggaaaaatattacacatgtaacctgaaagcacaactgaaaaatattaaactgttatgaaaatctaaaaacataattaactccctgcaattttcttctctgattgcagcttatttgtctggaaatgtgtacatacacctcactgagagatgctgagatgactacagaaattaactttgagaccagaattacagagaagaaaaaccaaaacccaaccctgcatggtcaagtggtgctaacccaagactgtaacagggagaaatgcccagaatcatcaaaatagtgaaagactgatctgttcaaaatatttgctatatgcactgggtataatccgtaatccatacactgccagataatgccatttcaaggaaggatcgaatacttgatggtaaaggccaagtccccctgtattgggaagtgtgtgatttcggcagacctgctgggaaaatttagggtagagcactctttacagaagaactcaaaaacccaatttggataattttcattatctttttagcaaaatggtttcttaatgtttatattttattttcaaggttcattgtttaatgaaatattttattcttgcatttccataaggaaagggaaagtcatgatcatcctaaaggatcacagtttttaaaaggcaaacattttccctaaggaaacagacacaagctttcctagagaatatgatgttttttaggcattaataaggtccttttttataaaggacacttttctcctagtagttttgaattcaggaacagatccaaagttagcagtatatggctgctacatttccattttcattttcgagccatcagtttatgttcagatgccatctctgtaatcgcacatttaaaacataactgtagcctcactaatggaaaagtagtatgatgaacaatcattcccaatggtgtacaatgtaagggttttagggagcaacagtatttaactggaagaaagaattgcatatttaatgtagtctaatatatacacatttgtttaacatgtaaacaaaagtgttaaattcacatatacaacattatacaatttaatcactcttggaataaaatttttatagccttttttctattgggaaaatttgtttagatgtgtgccactccataggtttatttccaaaatgaatgagcccaactccatttgtaaaaacttgtcagttagaattcctttttttagtggattagggctgaattcttagatccttatttcttttcactttaaatgctgccaaagatcactactcatcattcaggaattcgctgtctagcctatctgtagtttcctgaagattgaaaattatgtagactgctatttaaaaatatatttttctaagtgtgaggtttaagatgctgtattgaccctatgagtttttaatgtgttaattatctttatagcataatagatcgctttaggttcctggaatcccatttggtctgacaggatatatgaagattcttaatacctattttctgtgtctaatacttggttaatactaaaaatagaaatgactaaattacatcacagaaagcataaccagtgattgaacctggtagttttaaagctctaaatagctgtggctgaaggactgattatggggctaagaagcttgaaacgtaagttggtacttgttcatcagtggattctcctaaattaagccaaattttgaaatacatgactattaagtttctactcatgtatttacagtcagtcaataaattaaaggaggaaaaaaatccctgaacaacctgcccataaaaagaaaaatactctacatttgagcctgctgcagttttaaattttccctctgggtcaagtttgccagcttttggctacagagaaattatatttccattacagtgcaggtagaaactctgtaaccttaagcatgtaaactacatagaataaaactgtttccactgcatttctgtccttcaaagtggccaacctgattaagtcagccttaatcactgctgctgtcagtttcacgactaaaggtcatattgactaagtagtcatcagctgaccacctcgctgtatcagccagcaacgaggggaaggtgaagaaacatgataggccatatagaatctgccctatgtttacttttttaacccagataattatttttgtgtgcagtatctaagctcctgattgtgtaacctgggacttctggcaccttttgttccattcattttatgtataaaatgcatgccaaagcacactgtgccctctggtacccttgcttccaatcgccaaccatgctcatttccttcctttttttgtggtccctttttgtggtgatcattttaaaccacgtcatccaacaaatgttttatggtcaaccttagcttgttcataagccatagcaactgaaagattaaactcttaaatatgtgtctgggcagtggctattaaatagcaaaaaacaatcagattttagtattttattatttccttgtaaaatggctgaactaaattaaacccttgtttcccatttgttctataatttatagtgaaactgagaacaaaactatctttataaatgatagctaaaagtatttccagatatttaaacaatttaaaataaatttcttctgcagagatgcaaagcatctcaacactggaatgaacaaatgccttaaattcaatggagtaaacctttagaatgaagaggaactgtcatttcacccaagccgaagacaacagccttatgcacttgtgtgctctgtctttgctgcttctcgtgtttcaagcctttcctgtgggatcagcacagcaaagtgcaacttaccaaatggtttaatgactggttaattctttcttctcccaatggaaaagcaatggcaacacaacagtagactgctggcttgacaatcttaaacgtgagcctttgcacatgtaggtttatcatcatttgagtatacgactaagcaagtcaatgaactttttttttttttttagcagtttaatttggtcctgagaatgttgcagtctttattaccccttttgcattaatccacttttctaaccaccttttaagctttaatttttaacactatacaccaagtctttgaaatcagtgatctgttatttaactctaaagcatttgacacttcttgccttaacagttttaaaaaccacacacaaaaaaactctgtaagtaatacagtaggccaaaagtttcatcctatctatcttgcagtttacctatctgatctgatctctgtaattatagttctgtcatttaaaatatactatttaaatctaatttttacatttcaaaaattatcttcagtagtaactaagtatattttctgtggattctgagaatgttatttttcagaatgtgagaatatatatgtacatttataatcttgtgactttaaagtctgttttcagatacagtatgtaaatacttgtaaaaaaatttgtataattttgtgataatgtagtttcccaaaaaaattatttagaaggcattatgttattagtaaatgagagcactgtatagaactgttcctattttctgcacttgccattccagctgcctccactgtccatacccacctcattcatcctgtcacagaaggcaggaaaactgggaactttaccaaagtagcactcagcctgagaggcctgtataatcatgcttttcaaactaaattcacttaaaaattaaaaagcagaattgaatattttaagcagcctcagtacctttggccaatgctgttttcatggtggattatgaacattatataatctttgggaaaagtgaaagtagtacaatttttagaataatgacaactgcctcactgcatctctccactcacacagcaaccgtgtagccccctaagctgcagtaccatgactaaccatgatgtcaatttcatatgctgatcctcacaacagcagtgcacaaacatgccccaaatattttaacagaatttagctcttccttaagctgtcttttcatagtaaaaacaaaacaaaaacacccaatgttaaaaccacataataaacttacaaacttgaaaaattagacacttcagatagataggcaataaaacttcatattatgaaagcaatatattccaagtttcaaagatttgacaagttctgtagagtatctttcatcagtacatgaaaacttccaaactgcatgatcttctgccaggcaggactgggtgctattcgctggtttgaggtcgaatccatttcaaggcatgtcgtggtgggacattaatggtgggatggtagaatgtgcagtccggtcttgtacattgagtgttaaacctacaatgttttggatgatagaagggacattccatcttcttacaagcagggaagtaacggcagagctgactactggaaggtggtgctggtggtgcaactggttttggagacagtactggaattcttctactcacatgagtgaagggacaatctggtttagtacactttgcatcatatttacaatttgggtgaacaaacaaacatttttcagcaaatttacaattggggaaggctttgcagggtgagatggggtgatggtaggcacactcatccccatttttacaagcaggccagtacttgcagcgctccaaaagtttttctggtttctgtgccacactcagttcactcatctcagcttgatttttttctacagaatctccttttgtttcctcttctttaatggggggacttattctgggggtcctactttgtccctggaccacttctgctagcaattcttcttgagaagttcgagttctgggagcaactggaagtgtctgtttctgtggaactgtagagtagttagttgtttttgttacggattcttgagcttcagatatagccttcaaaatcagattcttgttagcttgtttagaaggtggaagagaaggtctcctttcaggctttgcaggcacagacacactgctggagatgcttcctgttcgagacccgtaatcatcatcttcttcctcctcttctccatcatgattgaatttttttactttaacaactgaacttaccacaggcaactttctcttccgaaagttttcatcctccatactcattttctccgagttgtttctaaagaacggactatacgtttcttctaagctgttaagcacctctggttcacacaaacgtcctgtttcatatacccaactactctgcatatcaagctgcttggcagcatgaatactattctgctgctgttgaaattgcaacctgtttaaatgaacaccactatctgcatttctacttgcaggtggtcgataaatttcaatagaagggcgagaagaaccatatgtaagtgtcactgtaggttttttctgagataagggattctcctgcacaaagttgaggtcttcgtcaatgagatcatctggttctggcttaatatcaatcacatcttcagagggtgctggctccctcaaaggtttcactgttgacattagtcgggttgcagctccatcatcgtaagtctgtctgacatttgtggtttttgactcctgcgaacttgtagaaactctggaatctcttttttcaggtctcgcgctaggaatggcaagtggtggcactgcagcttcatgcctcctctcatctccccgactgaaattgctcttgtttgaaggcacgttactatcaaagatgttggtatcagaagacttcagactagagggttcagttgtaacagagcgaagtttatctaatacaccatgaagccaacataagctcctaattcttgtaatttccccttaatggcactccggatcttgcggctgatctcggtgccgatctccatggctctgcggcgtgcgggaactcagcactgcgcggcgcttggcttacccggaggctgccgcggactcctaccccgcagccgggacaccaccgcctcc

SEQ ID NO: 13632 - RNA, 16460 nt, Homo sapiens
  source 1..16460: mol_type = other RNA
gctgggattacaggcatgagccaccataataaggattctgatgaacatttgattccttggactactgttatactcaaaagccttccttaatcttctaattgtcaccctaaatatcctaaaatttctgtcttcctagtagttcttcatagtcctaaaaatttgtcagagagaaaggtaaatcaagaaacatgattttcaaatgatttaaggtggtactagggtttaggatttcctttgctttttatcatttaacacactgcttatcatacagctggaagtgctctgggccagtgtctctacttcgagggaagaaggaggtagtgagacagaaggaaatagcacaattcctggccctgacagaagggtgttcaggagacctgctctcctctcactttattccatctcatctggacctgtggcttccaatccacatctctttcctttaatatcctgcattggctaggctgtataaatcctttggtgcatcgaaaaactaagtgcattttttgtttttgtgattatgcaatacttataggaaaagttataattttagaatatttaagtacacttacatttttgagaaaaagactattgaaatgtttgtgccatgtcaaatttcagttgaacattttgggtattcttaatataagaccaggccaggcaccgtggctcaggccgggcacagtggctcacacctataatcccagcacttagggaggccaaggcgggaagatcacctgaagtcaggagttcaagaccagcctggctaacaaggtgaaactctgtctctactaaaaatacaaaaattagccgggcgtggtggctggcgcttgtaatcccagctacttgggaggctgagacaggagaatcacttgaacctgggaagcagaggttgtggtgagctgagatcgcaccattgcactccagcctgggcaacaaagagcgaaactccgtctcaaaaaaataaaaaataaaccctagaattatagtatgttagaattggaagggaagaattgtctaaggttattctagctaataagcaacagacttggaaaggaaaaggtcctgacaaagctaagcctcccgttcaggtttcctgactcgtgaattcagtgctgctgccactacacgatgcatgctctttgtatcaagggtgagacagcattacacatacatagaaaattatctatttaaactctatttgaacttttgatgagtttgtctccccctcccccactccttttcagaataacttgacgtttacaggtaccatcagtggtgatgtctgtgtgtggaaagatcacatattgtgtagaatcgtggcgagagctcacaacgggcctgtgtttgccatgtacaccaccctgcgagatggacttatcgtgactgggggaaaggaaaggccgtgagtcctctttcttttcacagaatatttatgcatttgtgacctacctgaggtttgcagttaattattctagttgtttctaggctacacagagtgtcctctccgaccttcctcctcatatgcttctcctttattaccttttatgtgccttctatttgattctcatttctggtcttaattcacttccaatttttttcatgttggggtgatactttttctgaggtgtggataggtagttgtcctacaagttgagttacttttcttaatgtctgtatgcctgtgtatgatttgctgagtaggaggcccatgggggaatctggagccagggttgtattttgactgcctgctctctttttgttcagaatggattctaaggagtagaatgcacattgttgctttagaaaaggatgagggaactagagagaactgccttgtttccttttgcttgaggcaaatttaaactgttttatacaagacctcaaaatttgagaagaggtctcttctgagtgattttcaaatctcccaacagtaaccagatacttatgatttgatttgtcaccaacatagtcatatgcatgttgaaacatgacatgtaggccaggcacagtggctcacacctgtaatcttatcactttgggaggctgaggcaggtggatcgcttgagcccaggagttcaagaccagcctgggcaacatggtgaaaccccatcgctataaaaaacaacaattagccgggtgtggtggcacatgcctgtagtccctgctactcaggaggctgaggtgggaggatcacttgagcctggggaggtcaaggctttagtgagctgtgatggtgccactgcactccagcctgggtgacagagtgagaccccatttaaaaaacaaaaacaaaaacaaaaaaaaatgtgacatatagttgactaagaagtacatttcaatacaggattgaaagaacccacatatgttaattaaacacaagcgcagaatttgtgccttttacataaaggaagaatgcacataggcatgctttcagacaagcaattcatctagcagaaaaggaaggaatacatttttcagcccttccaggaataaaatccataaatgggctctatttcgtcctccaacacttgtatttcccacgtcatttactcctgcacacccccactcactagaagcctgctaaactgttccagtgagatattttaacacctgatagggaataaatatgcttctgttttggccttcaaaaataagctctgggccagttgcagtggctcacgcctgtaatcccaacactttgggaggccgaggtgggcggatcacgaggtcaggagtttgggatcagcctggccaatatggtgaaactccatctctactaaaaatacaaaaattagccaggcatggtgcctgtaatcccagctacttgggaggctgaaggagaagaatcgcttgaacctgggaggcacaggttgcagtgagccgagatcacaccactgcactccaggccaggtgacagagcgacactctgtctcaaaaaaataaataaatcaactctgtagcatagcatttgtaattctattattttgccttacatttccattatccttttaataaaattgtttttttacatcttcctaatcaagaagtattatgaggccaggcacagtggctcatacctggaatcccagcactttgggaggccgaggcaggcagatcacctgaggtcaaggtatttgagaccagcctggccaacatggtgaaaccccatctctactaaaaatacagaaattagctgggtgtggtggtgcacacctgtaatgctagctactcgggaggctgaggtaggagaatcgcttgaacctgggaggcagaggttgcaataagcctagatcatgccactgcactcaagcctgggagacagagcgagactacatcttaaaaaaaaaaaaaaaagtattatgagagaggataatgtattgtaatgtattgtagaggctaaataaaattatgctcatgtcagaaaaaaagagtatttctcaaaataaaattcactgaaactggatgtttattttgactgagatatagtatatcctcaaattgccatagaaagtttacaagaatattagaggtaaattataaatatcagggcctttttaaaaaaaaaagattctgcttataacttggtatttgtttataataaaaattatagtagccaataatgaacacttactctggcttggttatttacttaggtcaaaagaaggaggagcggttaaactgtgggatcaggaactgaggcggtgccgtgccttcaggcttgagacaggacaagccacagattgtgttcgttctgtgtgcagaggcaaagtaagatgttccatgagctgatacagtgcagcagaaaacagaaagtggttattactgtgattccctcaccctttgcagcctaatgaacaatacttaataatgcataacgatggatttgcttgccaacattactctgtctttgctgctttctttgccaaagttagcaccagtgtggtgcataagctaggaagctattctgtctaaatactgtatgtaaacctccaatattttctagaatctgccaatttaacaactctagtagacataattgaaagcccttggcagttgactcatattaggacagctgtctccattttttaaaaaaacacacattccctagataaaacgtgcagtaaacaaacaatgaaatactactcagccataaaaaataatgaaattctgtcattcttggtggcaacatggatgagactggaggacatgatgtgaagtgaaataagccaggcacagaaagataaatacatgttctcactcctgtgcagaaactaaaaaagttgatcccacagaggtggagagtagaatagtggttactggaggcggacaagggggagggggagggggatagggaaggactggttaaaggatacaagtttacacagccagataggaatagtatgttttagtattctgtagtactgtaggatgactatagttaagaatcacgtatttatgtattttcaggtatttacaagagaggattttgaaagtttccatcacaaagaaatgataaatgtctgaggtgatggttatgcgtattaccctatgccctatagatatgtataattatgtgtcaatttcaaaataaaaattcaaaactacaactcctatgaaaatttttgagcgtgtttgtacttattaagtgtatttataaatcatacggatattatcttcagcctgcatattaaattgtagttaagcttttactttttaactaaaaaataaattctattattttttcctatatcccactgcactgaccccagtttggaaatcctaagattatcaaataaaaactttgattattgaagaatccaggtgtactgccacagaaaagttctattctgtagcatggactctaatatgtaatctagcccattgtgcttacagatagatgtgtgcctgtagtcatagaaaaatttgcatgagctaatgactgccttgctactagattagctcaaagcaaaaagttctctgaaagcaggtcaatagggtcatttttatattatgaagaagaaaagcagctgttgtattacattcactgtattggtcctgcttgtgtttcagggcaagatccttgttgggacaaggaatgctgaaataatcgaagttggagagaaaaatgcagcttgtaatattttagttaacggtcatgtggatgggccaatctggggactagcaacacatccttccagggattttttcctttctgctgcagaagatgggacagtgagactttgggatattgctgataaagtaagtacagataatttttttaaaagaggttacaacttctaaaaagaaaagttggaagttctaaattgctagtacttaaagaactgccagaattctgttgagcattttgaggggaaactggtataatttagaagtacttcacttaatgtttcctatgactctttttttttttttttttaaatgcagaagatgttaaacaaagtgaatttgggacatgctgctcgtactgtgtgttacagccctgaaggggacatggtggctattggaatgaaaaatggagaatttatcattttactagtgagttctctaaaaatatggggaaagaagagagacaggagatgtgcaatccatgatatcaggttagtgaacaaatggaatagagtttctagtatatacttgatttaacttccatttgtaaaattttccatagccttgccttcaaaaagaggtccccagggcctgtagcatttcccgtattataaattgtatgctaaaatatggctgtttgtatactacttaattcttcttgctaaattataaacccactgggcaccaactataatagcaagtactagtaggtaatgtttgatgaattcatgttaacacttagccatgtccattaagttcatcccaccaagaggtatctcccactgtaatacaagagagctatctgcccttcaaaagttgtcaccctggaaaactaaagttgtgatttcaaacatatcttctcttagtaacctcagtttgggaatatgtagttcattaatttaatcaatacctattgattaaatgttccagaatccaaattaatttaaatgtttcttaaacctttgtttttcagtgcttaagcatttttcaacagtggctaccatttacggagtacttccgtgtgatcagtagataagattattgaatctaggtctgtcaaaagcttgtacacttttcatcagtaaaatccttttacaaatgaaaccttcctcagaacttcaatatataaaatagtaacagtggcttcccttagcttttacatgtctctatcgtacctcagtaagactcatgggccatttcaagagactgaattgtcccatatgactccaaagattgctaggcaaatagcatttcactttgtcttttaaataagttcttcaggccgggcgcggtggctcatgcctgtaatcccagcactttgggaggccgaggcaggcagatcacctgaagtcaggagtactcgaccagcctggccaacatagtgaaaccccatctcaactaaaaatacaaaaatcagccgggcgtggtggcaggcgcctgtaatcccagctactcagggggctgaaacaggagaatcgcttgaacccgggaggcggaggttgcgccatcgcactccagcctgggagacaagagcgagacttcgtctcaaaaaaaaaaaattcttcttccaagattcaagttgtgtcatttcaccttaataactggaggttagttaagctgggctgtgttctttgcttaatattaagacaacgttttttccagatggaagaaaactatcttaatgaattgttagcttattaattatgtaatgctaatggcttttaaaagctgagatgttctgactgggtgttgtggctcacacctgtaatcccagtaccttgggaggccaagggggaaggattgcttgaggccaggagtttgggaccatagtgagaccccgcctctatttaaaaaattaaattttgttttgttttgttttgagttggagttttgctcttgttgcccatgctgaagtgcaatggtgcaatctcagctcaccacaacctgtgcctcctgggttcaagcgattctcctgcttcagcctcccgagtagatgggattacaggcgtgcaccaccatgcctggctaattttgtatttttagtagagacagggtttctctatgttggtcaggctggtctcaaactctcgacctcaggtgatctgcccgcctccgcttcccaaagttctgggattataggtgtgagccactgggcctggcctaagaaagtttttttaagccattagacgtttttaaaggaattgggagatgacaattggggaaatatttaaaatttaagtaaaatataaagcttccttatttcatgtaacccagacaatctcagtatacatgatcagttgtgtctgacaggtaaatctatttgaggccttatcacacgttacttttaagaactagaaaggaaaagtcactgatcttaagtatttataatacttcatgtggtctaatactttttacgttttgttttgattcagatttagtccggattcccggtatctggcagtaggttctagtgagaactcagtggatttttatgacctaacgctgggccccactcttaacagaatcagctactgcaaagacattccaagctttgtcattcaaatggacttctctgcagatagcagttatctccaggtacagtaccaatactgtatacccaggtggcaagttcttctgcttttacatttcgtgttagtgaatgcatttaaagttcctgagctccagagctccagcttctcaactcctccctttgtaccttctgacctacagctcccctttcctcccccacttatcagagcttttctcctattaagtttttgtagtgatcttttgcatacttaataatgttagacatgtaaatcaagtagcaatatgctagtattctgtaaaccccctgtggattttgtctctcacctaatggaattcttgtcccattttaatctgatgaaaaaggtctctagtggctgctataaacggcatgtctatgaagtgccttcaggaaaacatcttatggatcatgccgctattgacagaattacttgggctacatggactaggtaaatacttatatattcacaaggcaagaactgactttgaaggccagttagaaaatcctatttctgaactgttagagccattccaataaggaatagtaattgagtttcaagtttttgttaccatattttgaaatggtatgttcatgttgggacccctttttattgaatatatttccatgttttatcagtttccatgatttatcaagttttttttttaaggaaatcaaagttttaactttaaagataccctgatatttttcttaatgctaaatttaatgactggcaaaaaggtattgggtgctgttaagcaactgttattaattctctatctaaaggaatgctatcttgaatctattagaagtcaaagcttccaaatttgttcaaatttcctggctgtatgacaggtaaccatgactatccatttttttggccaatgaaaaatgccatcaaattcctgtatcagccaggcatatagtggctcatgcctgtaatctctgatgtagcaggccgaggtgggaggatcacttgagcctagaagttttgataccagcctgggcaacatagcaagaccccatctctgaaatttttttaattcctatgtcataagtcatttttatttttgtagagatagggatctcacaatattgcccaggctggtctcaaactcttggcctcaagcagtcctcctgcctcagcctcccaaaatgttgggattactggtatgtgctgctggacccagccaagtagcacttttaatttgaaaaatagttctatcagttttcagtcaggcgcggtggctcagcctgtaatcccagcactttgggaggccgagcgggggtgatcacctgaggtcgggagttcgagactagcctgaccaacatggagaaaccctgtctctactaaaaatacaaaataagccgggcatgttagcgcatgcctgtgatcccagctactcgggaggctgaggcaggagaattgcttgaacccaggaggcagaggttgcggtgagccgagatcatgccattgcactccagcctgggtaacaagagcgaaaactccgtctcaaaaaaaaaaaaagaaaaaatagttctatcagttttcataaagtactactttaatcttaaaaagattaatctagaaacccttcaaattataaaatgtcatttttaaaaggcaggagttgatatcctgatgaaattcaggtctccaaacaacttaccataatttacttcctgtattttaagtaacatgatagggtacttagagattaattgccaagaaactttttgaatatagtcaacctgcccgcacttgccatgatgagttttcttttgttccttccctctagtattctaggagatgaggttttgggaatctggtccagacatgctgagaaagctgatgtcaactgtgcctgtgtatctcattcaggaatcagtcttgttacaggagatgactttggcatggttaagttatttgacttcccatgtccagaaaaatttgtaagtttgtgttttgtttactattatcagtttactcctaattttgatgtcttatcatcagcacttttccccatatatttaaaatgttttgtcctaatttctaaatttttccccaaactttctaaatctatttactttgaaataaaagctattagaaacaaatcctctccctcgagtaataccatctttggaaccatcctacaaaagctgtaattagcttttcaccaaacctataatcagttatcaaatttcaaatgcttttccttagagaaaaatggtcagagtacctggagacatctgactgcccacacagcctggttttgcagatccactactcatgctgaaaagcattctaatcactggctgcggtgctaactccctactctctccacagctcttgtcatagagattatagttcctaataagagcctttgacttctgtgtgcaccaaatgccctgagcttgtctgtcattgttttttaggcaaaacacaaaaggttcttgggtcattcgccccatgtgacaaatattcgatttaccagtggtgatcgacatgttgttagtgctggaggtgatgactgcaggttagtaactttctcagcccatgaagagcagactatgttactagttaagagacttaatacaacaactcctacagctttggtttatgaaatcagctagtcaacattagtagaaggtagtataaccagatggctcttcagaatctcatatttatgcaaatacagaataaaaggagttaaagaggaaaaatattacacatgtaacctgaaagcacaactgaaaaatattaaactgttatgaaaatctaaaaacataattaactccctgcaattttcttctctgattgcagcttatttgtctggaaatgtgtacatacacctcactgagagatgctgagatgactacagaaattaactttgagaccagaattacagagaagaaaaaccaaaacccaaccctgcatggtcaagtggtgctaacccaagactgtaacagggagaaatgcccagaatcatcaaaatagtgaaagactgatctgttcaaaatatttgctatatgcactgggtataatccgtaatccatacactgccagataatgccatttcaaggaaggatcgaatacttgatggtaaaggccaagtccccctgtattgggaagtgtgtgatttcggcagacctgctgggaaaatttagggtagagcactctttacagaagaactcaaaaacccaatttggataattttcattatctttttagcaaaatggtttcttaatgtttatattttattttcaaggttcattgtttaatgaaatattttattcttgcatttccataaggaaagggaaagtcatgatcatcctaaaggatcacagtttttaaaaggcaaacattttccctaaggaaacagacacaagctttcctagagaatatgatgttttttaggcattaataaggtccttttttataaaggacacttttctcctagtagttttgaattcaggaacagatccaaagttagcagtatatggctgctacatttccattttcattttcgagccatcagtttatgttcagatgccatctctgtaatcgcacatttaaaacataactgtagcctcactaatggaaaagtagtatgatgaacaatcattcccaatggtgtacaatgtaagggttttagggagcaacagtatttaactggaagaaagaattgcatatttaatgtagtctaatatatacacatttgtttaacatgtaaacaaaagtgttaaattcacatatacaacattatacaatttaatcactcttggaataaaatttttatagccttttttctattgggaaaatttgtttagatgtgtgccactccataggtttatttccaaaatgaatgagcccaactccatttgtaaaaacttgtcagttagaattcctttttttagtggattagggctgaattcttagatccttatttcttttcactttaaatgctgccaaagatcactactcatcattcaggaattcgctgtctagcctatctgtagtttcctgaagattgaaaattatgtagactgctatttaaaaatatatttttctaagtgtgaggtttaagatgctgtattgaccctatgagtttttaatgtgttaattatctttatagcataatagatcgctttaggttcctggaatcccatttggtctgacaggatatatgaagattcttaatacctattttctgtgtctaatacttggttaatactaaaaatagaaatgactaaattacatcacagaaagcataaccagtgattgaacctggtagttttaaagctctaaatagctgtggctgaaggactgattatggggctaagaagcttgaaacgtaagttggtacttgttcatcagtggattctcctaaattaagccaaattttgaaatacatgactattaagtttctactcatgtatttacagtcagtcaataaattaaaggaggaaaaaaatccctgaacaacctgcccataaaaagaaaaatactctacatttgagcctgctgcagttttaaattttccctctgggtcaagtttgccagcttttggctacagagaaattatatttccattacagtgcaggtagaaactctgtaaccttaagcatgtaaactacatagaataaaactgtttccactgcatttctgtccttcaaagtggccaacctgattaagtcagccttaatcactgctgctgtcagtttcacgactaaaggtcatattgactaagtagtcatcagctgaccacctcgctgtatcagccagcaacgaggggaaggtgaagaaacatgataggccatatagaatctgccctatgtttacttttttaacccagataattatttttgtgtgcagtatctaagctcctgattgtgtaacctgggacttctggcaccttttgttccattcattttatgtataaaatgcatgccaaagcacactgtgccctctggtacccttgcttccaatcgccaaccatgctcatttccttcctttttttgtggtccctttttgtggtgatcattttaaaccacgtcatccaacaaatgttttatggtcaaccttagcttgttcataagccatagcaactgaaagattaaactcttaaatatgtgtctgggcagtggctattaaatagcaaaaaacaatcagattttagtattttattatttccttgtaaaatggctgaactaaattaaacccttgtttcccatttgttctataatttatagtgaaactgagaacaaaactatctttataaatgatagctaaaagtatttccagatatttaaacaatttaaaataaatttcttctgcagagatgcaaagcatctcaacactggaatgaacaaatgccttaaattcaatggagtaaacctttagaatgaagaggaactgtcatttcacccaagccgaagacaacagccttatgcacttgtgtgctctgtctttgctgcttctcgtgtttcaagcctttcctgtgggatcagcacagcaaagtgcaacttaccaaatggtttaatgactggttaattctttcttctcccaatggaaaagcaatggcaacacaacagtagactgctggcttgacaatcttaaacgtgagcctttgcacatgtaggtttatcatcatttgagtatacgactaagcaagtcaatgaactttttttttttttttagcagtttaatttggtcctgagaatgttgcagtctttattaccccttttgcattaatccacttttctaaccaccttttaagctttaatttttaacactatacaccaagtctttgaaatcagtgatctgttatttaactctaaagcatttgacacttcttgccttaacagttttaaaaaccacacacaaaaaaactctgtaagtaatacagtaggccaaaagtttcatcctatctatcttgcagtttacctatctgatctgatctctgtaattatagttctgtcatttaaaatatactatttaaatctaatttttacatttcaaaaattatcttcagtagtaactaagtatattttctgtggattctgagaatgttatttttcagaatgtgagaatatatatgtacatttataatcttgtgactttaaagtctgttttcagatacagtatgtaaatacttgtaaaaaaatttgtataattttgtgataatgtagtttcccaaaaaaattatttagaaggcattatgttattagtaaatgagagcactgtatagaactgttcctattttctgcacttgccattccagctgcctccactgtccatacccacctcattcatcctgtcacagaaggcaggaaaactgggaactttaccaaagtagcactcagcctgagaggcctgtataatcatgcttttcaaactaaattcacttaaaaattaaaaagcagaattgaatattttaagcagcctcagtacctttggccaatgctgttttcatggtggattatgaacattatataatctttgggaaaagtgaaagtagtacaatttttagaataatgacaactgcctcactgcatctctccactcacacagcaaccgtgtagccccctaagctgcagtaccatgactaaccatgatgtcaatttcatatgctgatcctcacaacagcagtgcacaaacatgccccaaatattttaacagaatttagctcttccttaagctgtcttttcatagtaaaaacaaaacaaaaacacccaatgttaaaaccacataataaacttacaaacttgaaaaattagacacttcagatagataggcaataaaacttcatattatgaaagcaatatattccaagtttcaaagatttgacaagttctgtagagtatctttcatcagtacatgaaaacttccaaactgcatgatcttctgccaggcaggactgggtgctattcgctggtttgaggtcgaatccatttcaaggcatgtcgtggtgggacattaatggtgggatggtagaatgtgcagtccggtcttgtacattgagtgttaaacctacaatgttttggatgatagaagggacattccatcttcttacaagcagggaagtaacggcagagctgactactggaaggtggtgctggtggtgcaactggttttggagacagtactggaattcttctactcacatgagtgaagggacaatctggtttagtacactttgcatcatatttacaatttgggtgaacaaacaaacatttttcagcaaatttacaattggggaaggctttgcagggtgagatggggtgatggtaggcacactcatccccatttttacaagcaggccagtacttgcagcgctccaaaagtttttctggtttctgtgccacactcagttcactcatctcagcttgatttttttctacagaatctccttttgtttcctcttctttaatggggggacttattctgggggtcctactttgtccctggaccacttctgctagcaattcttcttgagaagttcgagttctgggagcaactggaagtgtctgtttctgtggaactgtagagtagttagttgtttttgttacggattcttgagcttcagatatagccttcaaaatcagattcttgttagcttgtttagaaggtggaagagaaggtctcctttcaggctttgcaggcacagacacactgctggagatgcttcctgttcgagacccgtaatcatcatcttcttcctcctcttctccatcatgattgaatttttttactttaacaactgaacttaccacaggcaactttctcttccgaaagttttcatcctccatactcattttctccgagttgtttctaaagaacggactatacgtttcttctaagctgttaagcacctctggttcacacaaacgtcctgtttcatatacccaactactctgcatatcaagctgcttggcagcatgaatactattctgctgctgttgaaattgcaacctgtttaaatgaacaccactatctgcatttctacttgcaggtggtcgataaatttcaatagaagggcgagaagaaccatatgtaagtgtcactgtaggttttttctgagataagggattctcctgcacaaagttgaggtcttcgtcaatgagatcatctggttctggcttaatatcaatcacatcttcagagggtgctggctccctcaaaggtttcactgttgacattagtcgggttgcagctccatcatcgtaagtctgtctgacatttgtggtttttgactcctgcgaacttgtagaaactctggaatctcttttttcaggtctcgcgctaggaatggcaagtggtggcactgcagcttcatgcctcctctcatctccccgactgaaattgctcttgtttgaaggcacgttactatcaaagatgttggtatcagaagacttcagactagagggttcagttgtaacagagcgaagtttatctaatacaccatgaagccatacggtgaatcgaattgtgttgttccctagaaacagggacagatcctctgtcatttggtcctgacttttcttgttggccaccatcaccataatgtaatcaggaagttcttcatcaacataagctcctaattcttgtaatttccccttaatggcactccggatcttgcggctgatctcggtgccgatctccatggctctgcggcgtgcgggaactcagcactgcgcggcgcttggcttacccggaggctgccgcggactcctaccccgcagccgggacaccaccgcctcc

SEQ ID NO: 13633 - RNA, 16641 nt, Homo sapiens
  source 1..16641: mol_type = other RNA
gctgggattacaggcatgagccaccataataaggattctgatgaacatttgattccttggactactgttatactcaaaagccttccttaatcttctaattgtcaccctaaatatcctaaaatttctgtcttcctagtagttcttcatagtcctaaaaatttgtcagagagaaaggtaaatcaagaaacatgattttcaaatgatttaaggtggtactagggtttaggatttcctttgctttttatcatttaacacactgcttatcatacagctggaagtgctctgggccagtgtctctacttcgagggaagaaggaggtagtgagacagaaggaaatagcacaattcctggccctgacagaagggtgttcaggagacctgctctcctctcactttattccatctcatctggacctgtggcttccaatccacatctctttcctttaatatcctgcattggctaggctgtataaatcctttggtgcatcgaaaaactaagtgcattttttgtttttgtgattatgcaatacttataggaaaagttataattttagaatatttaagtacacttacatttttgagaaaaagactattgaaatgtttgtgccatgtcaaatttcagttgaacattttgggtattcttaatataagaccaggccaggcaccgtggctcaggccgggcacagtggctcacacctataatcccagcacttagggaggccaaggcgggaagatcacctgaagtcaggagttcaagaccagcctggctaacaaggtgaaactctgtctctactaaaaatacaaaaattagccgggcgtggtggctggcgcttgtaatcccagctacttgggaggctgagacaggagaatcacttgaacctgggaagcagaggttgtggtgagctgagatcgcaccattgcactccagcctgggcaacaaagagcgaaactccgtctcaaaaaaataaaaaataaaccctagaattatagtatgttagaattggaagggaagaattgtctaaggttattctagctaataagcaacagacttggaaaggaaaaggtcctgacaaagctaagcctcccgttcaggtttcctgactcgtgaattcagtgctgctgccactacacgatgcatgctctttgtatcaagggtgagacagcattacacatacatagaaaattatctatttaaactctatttgaacttttgatgagtttgtctccccctcccccactccttttcagaataacttgacgtttacaggtaccatcagtggtgatgtctgtgtgtggaaagatcacatattgtgtagaatcgtggcgagagctcacaacgggcctgtgtttgccatgtacaccaccctgcgagatggacttatcgtgactgggggaaaggaaaggccgtgagtcctctttcttttcacagaatatttatgcatttgtgacctacctgaggtttgcagttaattattctagttgtttctaggctacacagagtgtcctctccgaccttcctcctcatatgcttctcctttattaccttttatgtgccttctatttgattctcatttctggtcttaattcacttccaatttttttcatgttggggtgatactttttctgaggtgtggataggtagttgtcctacaagttgagttacttttcttaatgtctgtatgcctgtgtatgatttgctgagtaggaggcccatgggggaatctggagccagggttgtattttgactgcctgctctctttttgttcagaatggattctaaggagtagaatgcacattgttgctttagaaaaggatgagggaactagagagaactgccttgtttccttttgcttgaggcaaatttaaactgttttatacaagacctcaaaatttgagaagaggtctcttctgagtgattttcaaatctcccaacagtaaccagatacttatgatttgatttgtcaccaacatagtcatatgcatgttgaaacatgacatgtaggccaggcacagtggctcacacctgtaatcttatcactttgggaggctgaggcaggtggatcgcttgagcccaggagttcaagaccagcctgggcaacatggtgaaaccccatcgctataaaaaacaacaattagccgggtgtggtggcacatgcctgtagtccctgctactcaggaggctgaggtgggaggatcacttgagcctggggaggtcaaggctttagtgagctgtgatggtgccactgcactccagcctgggtgacagagtgagaccccatttaaaaaacaaaaacaaaaacaaaaaaaaatgtgacatatagttgactaagaagtacatttcaatacaggattgaaagaacccacatatgttaattaaacacaagcgcagaatttgtgccttttacataaaggaagaatgcacataggcatgctttcagacaagcaattcatctagcagaaaaggaaggaatacatttttcagcccttccaggaataaaatccataaatgggctctatttcgtcctccaacacttgtatttcccacgtcatttactcctgcacacccccactcactagaagcctgctaaactgttccagtgagatattttaacacctgatagggaataaatatgcttctgttttggccttcaaaaataagctctgggccagttgcagtggctcacgcctgtaatcccaacactttgggaggccgaggtgggcggatcacgaggtcaggagtttgggatcagcctggccaatatggtgaaactccatctctactaaaaatacaaaaattagccaggcatggtgcctgtaatcccagctacttgggaggctgaaggagaagaatcgcttgaacctgggaggcacaggttgcagtgagccgagatcacaccactgcactccaggccaggtgacagagcgacactctgtctcaaaaaaataaataaatcaactctgtagcatagcatttgtaattctattattttgccttacatttccattatccttttaataaaattgtttttttacatcttcctaatcaagaagtattatgaggccaggcacagtggctcatacctggaatcccagcactttgggaggccgaggcaggcagatcacctgaggtcaaggtatttgagaccagcctggccaacatggtgaaaccccatctctactaaaaatacagaaattagctgggtgtggtggtgcacacctgtaatgctagctactcgggaggctgaggtaggagaatcgcttgaacctgggaggcagaggttgcaataagcctagatcatgccactgcactcaagcctgggagacagagcgagactacatcttaaaaaaaaaaaaaaaagtattatgagagaggataatgtattgtaatgtattgtagaggctaaataaaattatgctcatgtcagaaaaaaagagtatttctcaaaataaaattcactgaaactggatgtttattttgactgagatatagtatatcctcaaattgccatagaaagtttacaagaatattagaggtaaattataaatatcagggcctttttaaaaaaaaaagattctgcttataacttggtatttgtttataataaaaattatagtagccaataatgaacacttactctggcttggttatttacttaggtcaaaagaaggaggagcggttaaactgtgggatcaggaactgaggcggtgccgtgccttcaggcttgagacaggacaagccacagattgtgttcgttctgtgtgcagaggcaaagtaagatgttccatgagctgatacagtgcagcagaaaacagaaagtggttattactgtgattccctcaccctttgcagcctaatgaacaatacttaataatgcataacgatggatttgcttgccaacattactctgtctttgctgctttctttgccaaagttagcaccagtgtggtgcataagctaggaagctattctgtctaaatactgtatgtaaacctccaatattttctagaatctgccaatttaacaactctagtagacataattgaaagcccttggcagttgactcatattaggacagctgtctccattttttaaaaaaacacacattccctagataaaacgtgcagtaaacaaacaatgaaatactactcagccataaaaaataatgaaattctgtcattcttggtggcaacatggatgagactggaggacatgatgtgaagtgaaataagccaggcacagaaagataaatacatgttctcactcctgtgcagaaactaaaaaagttgatcccacagaggtggagagtagaatagtggttactggaggcggacaagggggagggggagggggatagggaaggactggttaaaggatacaagtttacacagccagataggaatagtatgttttagtattctgtagtactgtaggatgactatagttaagaatcacgtatttatgtattttcaggtatttacaagagaggattttgaaagtttccatcacaaagaaatgataaatgtctgaggtgatggttatgcgtattaccctatgccctatagatatgtataattatgtgtcaatttcaaaataaaaattcaaaactacaactcctatgaaaatttttgagcgtgtttgtacttattaagtgtatttataaatcatacggatattatcttcagcctgcatattaaattgtagttaagcttttactttttaactaaaaaataaattctattattttttcctatatcccactgcactgaccccagtttggaaatcctaagattatcaaataaaaactttgattattgaagaatccaggtgtactgccacagaaaagttctattctgtagcatggactctaatatgtaatctagcccattgtgcttacagatagatgtgtgcctgtagtcatagaaaaatttgcatgagctaatgactgccttgctactagattagctcaaagcaaaaagttctctgaaagcaggtcaatagggtcatttttatattatgaagaagaaaagcagctgttgtattacattcactgtattggtcctgcttgtgtttcagggcaagatccttgttgggacaaggaatgctgaaataatcgaagttggagagaaaaatgcagcttgtaatattttagttaacggtcatgtggatgggccaatctggggactagcaacacatccttccagggattttttcctttctgctgcagaagatgggacagtgagactttgggatattgctgataaagtaagtacagataatttttttaaaagaggttacaacttctaaaaagaaaagttggaagttctaaattgctagtacttaaagaactgccagaattctgttgagcattttgaggggaaactggtataatttagaagtacttcacttaatgtttcctatgactctttttttttttttttttaaatgcagaagatgttaaacaaagtgaatttgggacatgctgctcgtactgtgtgttacagccctgaaggggacatggtggctattggaatgaaaaatggagaatttatcattttactagtgagttctctaaaaatatggggaaagaagagagacaggagatgtgcaatccatgatatcaggttagtgaacaaatggaatagagtttctagtatatacttgatttaacttccatttgtaaaattttccatagccttgccttcaaaaagaggtccccagggcctgtagcatttcccgtattataaattgtatgctaaaatatggctgtttgtatactacttaattcttcttgctaaattataaacccactgggcaccaactataatagcaagtactagtaggtaatgtttgatgaattcatgttaacacttagccatgtccattaagttcatcccaccaagaggtatctcccactgtaatacaagagagctatctgcccttcaaaagttgtcaccctggaaaactaaagttgtgatttcaaacatatcttctcttagtaacctcagtttgggaatatgtagttcattaatttaatcaatacctattgattaaatgttccagaatccaaattaatttaaatgtttcttaaacctttgtttttcagtgcttaagcatttttcaacagtggctaccatttacggagtacttccgtgtgatcagtagataagattattgaatctaggtctgtcaaaagcttgtacacttttcatcagtaaaatccttttacaaatgaaaccttcctcagaacttcaatatataaaatagtaacagtggcttcccttagcttttacatgtctctatcgtacctcagtaagactcatgggccatttcaagagactgaattgtcccatatgactccaaagattgctaggcaaatagcatttcactttgtcttttaaataagttcttcaggccgggcgcggtggctcatgcctgtaatcccagcactttgggaggccgaggcaggcagatcacctgaagtcaggagtactcgaccagcctggccaacatagtgaaaccccatctcaactaaaaatacaaaaatcagccgggcgtggtggcaggcgcctgtaatcccagctactcagggggctgaaacaggagaatcgcttgaacccgggaggcggaggttgcgccatcgcactccagcctgggagacaagagcgagacttcgtctcaaaaaaaaaaaattcttcttccaagattcaagttgtgtcatttcaccttaataactggaggttagttaagctgggctgtgttctttgcttaatattaagacaacgttttttccagatggaagaaaactatcttaatgaattgttagcttattaattatgtaatgctaatggcttttaaaagctgagatgttctgactgggtgttgtggctcacacctgtaatcccagtaccttgggaggccaagggggaaggattgcttgaggccaggagtttgggaccatagtgagaccccgcctctatttaaaaaattaaattttgttttgttttgttttgagttggagttttgctcttgttgcccatgctgaagtgcaatggtgcaatctcagctcaccacaacctgtgcctcctgggttcaagcgattctcctgcttcagcctcccgagtagatgggattacaggcgtgcaccaccatgcctggctaattttgtatttttagtagagacagggtttctctatgttggtcaggctggtctcaaactctcgacctcaggtgatctgcccgcctccgcttcccaaagttctgggattataggtgtgagccactgggcctggcctaagaaagtttttttaagccattagacgtttttaaaggaattgggagatgacaattggggaaatatttaaaatttaagtaaaatataaagcttccttatttcatgtaacccagacaatctcagtatacatgatcagttgtgtctgacaggtaaatctatttgaggccttatcacacgttacttttaagaactagaaaggaaaagtcactgatcttaagtatttataatacttcatgtggtctaatactttttacgttttgttttgattcagatttagtccggattcccggtatctggcagtaggttctagtgagaactcagtggatttttatgacctaacgctgggccccactcttaacagaatcagctactgcaaagacattccaagctttgtcattcaaatggacttctctgcagatagcagttatctccaggtacagtaccaatactgtatacccaggtggcaagttcttctgcttttacatttcgtgttagtgaatgcatttaaagttcctgagctccagagctccagcttctcaactcctccctttgtaccttctgacctacagctcccctttcctcccccacttatcagagcttttctcctattaagtttttgtagtgatcttttgcatacttaataatgttagacatgtaaatcaagtagcaatatgctagtattctgtaaaccccctgtggattttgtctctcacctaatggaattcttgtcccattttaatctgatgaaaaaggtctctagtggctgctataaacggcatgtctatgaagtgccttcaggaaaacatcttatggatcatgccgctattgacagaattacttgggctacatggactaggtaaatacttatatattcacaaggcaagaactgactttgaaggccagttagaaaatcctatttctgaactgttagagccattccaataaggaatagtaattgagtttcaagtttttgttaccatattttgaaatggtatgttcatgttgggacccctttttattgaatatatttccatgttttatcagtttccatgatttatcaagttttttttttaaggaaatcaaagttttaactttaaagataccctgatatttttcttaatgctaaatttaatgactggcaaaaaggtattgggtgctgttaagcaactgttattaattctctatctaaaggaatgctatcttgaatctattagaagtcaaagcttccaaatttgttcaaatttcctggctgtatgacaggtaaccatgactatccatttttttggccaatgaaaaatgccatcaaattcctgtatcagccaggcatatagtggctcatgcctgtaatctctgatgtagcaggccgaggtgggaggatcacttgagcctagaagttttgataccagcctgggcaacatagcaagaccccatctctgaaatttttttaattcctatgtcataagtcatttttatttttgtagagatagggatctcacaatattgcccaggctggtctcaaactcttggcctcaagcagtcctcctgcctcagcctcccaaaatgttgggattactggtatgtgctgctggacccagccaagtagcacttttaatttgaaaaatagttctatcagttttcagtcaggcgcggtggctcagcctgtaatcccagcactttgggaggccgagcgggggtgatcacctgaggtcgggagttcgagactagcctgaccaacatggagaaaccctgtctctactaaaaatacaaaataagccgggcatgttagcgcatgcctgtgatcccagctactcgggaggctgaggcaggagaattgcttgaacccaggaggcagaggttgcggtgagccgagatcatgccattgcactccagcctgggtaacaagagcgaaaactccgtctcaaaaaaaaaaaaagaaaaaatagttctatcagttttcataaagtactactttaatcttaaaaagattaatctagaaacccttcaaattataaaatgtcatttttaaaaggcaggagttgatatcctgatgaaattcaggtctccaaacaacttaccataatttacttcctgtattttaagtaacatgatagggtacttagagattaattgccaagaaactttttgaatatagtcaacctgcccgcacttgccatgatgagttttcttttgttccttccctctagtattctaggagatgaggttttgggaatctggtccagacatgctgagaaagctgatgtcaactgtgcctgtgtatctcattcaggaatcagtcttgttacaggagatgactttggcatggttaagttatttgacttcccatgtccagaaaaatttgtaagtttgtgttttgtttactattatcagtttactcctaattttgatgtcttatcatcagcacttttccccatatatttaaaatgttttgtcctaatttctaaatttttccccaaactttctaaatctatttactttgaaataaaagctattagaaacaaatcctctccctcgagtaataccatctttggaaccatcctacaaaagctgtaattagcttttcaccaaacctataatcagttatcaaatttcaaatgcttttccttagagaaaaatggtcagagtacctggagacatctgactgcccacacagcctggttttgcagatccactactcatgctgaaaagcattctaatcactggctgcggtgctaactccctactctctccacagctcttgtcatagagattatagttcctaataagagcctttgacttctgtgtgcaccaaatgccctgagcttgtctgtcattgttttttaggcaaaacacaaaaggttcttgggtcattcgccccatgtgacaaatattcgatttaccagtggtgatcgacatgttgttagtgctggaggtgatgactgcaggttagtaactttctcagcccatgaagagcagactatgttactagttaagagacttaatacaacaactcctacagctttggtttatgaaatcagctagtcaacattagtagaaggtagtataaccagatggctcttcagaatctcatatttatgcaaatacagaataaaaggagttaaagaggaaaaatattacacatgtaacctgaaagcacaactgaaaaatattaaactgttatgaaaatctaaaaacataattaactccctgcaattttcttctctgattgcagcttatttgtctggaaatgtgtacatacacctcactgagagatgctgagatgactacagaaattaactttgagaccagaattacagagaagaaaaaccaaaacccaaccctgcatggtcaagtggtgctaacccaagactgtaacagggagaaatgcccagaatcatcaaaatagtgaaagactgatctgttcaaaatatttgctatatgcactgggtataatccgtaatccatacactgccagataatgccatttcaaggaaggatcgaatacttgatggtaaaggccaagtccccctgtattgggaagtgtgtgatttcggcagacctgctgggaaaatttagggtagagcactctttacagaagaactcaaaaacccaatttggataattttcattatctttttagcaaaatggtttcttaatgtttatattttattttcaaggttcattgtttaatgaaatattttattcttgcatttccataaggaaagggaaagtcatgatcatcctaaaggatcacagtttttaaaaggcaaacattttccctaaggaaacagacacaagctttcctagagaatatgatgttttttaggcattaataaggtccttttttataaaggacacttttctcctagtagttttgaattcaggaacagatccaaagttagcagtatatggctgctacatttccattttcattttcgagccatcagtttatgttcagatgccatctctgtaatcgcacatttaaaacataactgtagcctcactaatggaaaagtagtatgatgaacaatcattcccaatggtgtacaatgtaagggttttagggagcaacagtatttaactggaagaaagaattgcatatttaatgtagtctaatatatacacatttgtttaacatgtaaacaaaagtgttaaattcacatatacaacattatacaatttaatcactcttggaataaaatttttatagccttttttctattgggaaaatttgtttagatgtgtgccactccataggtttatttccaaaatgaatgagcccaactccatttgtaaaaacttgtcagttagaattcctttttttagtggattagggctgaattcttagatccttatttcttttcactttaaatgctgccaaagatcactactcatcattcaggaattcgctgtctagcctatctgtagtttcctgaagattgaaaattatgtagactgctatttaaaaatatatttttctaagtgtgaggtttaagatgctgtattgaccctatgagtttttaatgtgttaattatctttatagcataatagatcgctttaggttcctggaatcccatttggtctgacaggatatatgaagattcttaatacctattttctgtgtctaatacttggttaatactaaaaatagaaatgactaaattacatcacagaaagcataaccagtgattgaacctggtagttttaaagctctaaatagctgtggctgaaggactgattatggggctaagaagcttgaaacgtaagttggtacttgttcatcagtggattctcctaaattaagccaaattttgaaatacatgactattaagtttctactcatgtatttacagtcagtcaataaattaaaggaggaaaaaaatccctgaacaacctgcccataaaaagaaaaatactctacatttgagcctgctgcagttttaaattttccctctgggtcaagtttgccagcttttggctacagagaaattatatttccattacagtgcaggtagaaactctgtaaccttaagcatgtaaactacatagaataaaactgtttccactgcatttctgtccttcaaagtggccaacctgattaagtcagccttaatcactgctgctgtcagtttcacgactaaaggtcatattgactaagtagtcatcagctgaccacctcgctgtatcagccagcaacgaggggaaggtgaagaaacatgataggccatatagaatctgccctatgtttacttttttaacccagataattatttttgtgtgcagtatctaagctcctgattgtgtaacctgggacttctggcaccttttgttccattcattttatgtataaaatgcatgccaaagcacactgtgccctctggtacccttgcttccaatcgccaaccatgctcatttccttcctttttttgtggtccctttttgtggtgatcattttaaaccacgtcatccaacaaatgttttatggtcaaccttagcttgttcataagccatagcaactgaaagattaaactcttaaatatgtgtctgggcagtggctattaaatagcaaaaaacaatcagattttagtattttattatttccttgtaaaatggctgaactaaattaaacccttgtttcccatttgttctataatttatagtgaaactgagaacaaaactatctttataaatgatagctaaaagtatttccagatatttaaacaatttaaaataaatttcttctgcagagatgcaaagcatctcaacactggaatgaacaaatgccttaaattcaatggagtaaacctttagaatgaagaggaactgtcatttcacccaagccgaagacaacagccttatgcacttgtgtgctctgtctttgctgcttctcgtgtttcaagcctttcctgtgggatcagcacagcaaagtgcaacttaccaaatggtttaatgactggttaattctttcttctcccaatggaaaagcaatggcaacacaacagtagactgctggcttgacaatcttaaacgtgagcctttgcacatgtaggtttatcatcatttgagtatacgactaagcaagtcaatgaactttttttttttttttagcagtttaatttggtcctgagaatgttgcagtctttattaccccttttgcattaatccacttttctaaccaccttttaagctttaatttttaacactatacaccaagtctttgaaatcagtgatctgttatttaactctaaagcatttgacacttcttgccttaacagttttaaaaaccacacacaaaaaaactctgtaagtaatacagtaggccaaaagtttcatcctatctatcttgcagtttacctatctgatctgatctctgtaattatagttctgtcatttaaaatatactatttaaatctaatttttacatttcaaaaattatcttcagtagtaactaagtatattttctgtggattctgagaatgttatttttcagaatgtgagaatatatatgtacatttataatcttgtgactttaaagtctgttttcagatacagtatgtaaatacttgtaaaaaaatttgtataattttgtgataatgtagtttcccaaaaaaattatttagaaggcattatgttattagtaaatgagagcactgtatagaactgttcctattttctgcacttgccattccagctgcctccactgtccatacccacctcattcatcctgtcacagaaggcaggaaaactgggaactttaccaaagtagcactcagcctgagaggcctgtataatcatgcttttcaaactaaattcacttaaaaattaaaaagcagaattgaatattttaagcagcctcagtacctttggccaatgctgttttcatggtggattatgaacattatataatctttgggaaaagtgaaagtagtacaatttttagaataatgacaactgcctcactgcatctctccactcacacagcaaccgtgtagccccctaagctgcagtaccatgactaaccatgatgtcaatttcatatgctgatcctcacaacagcagtgcacaaacatgccccaaatattttaacagaatttagctcttccttaagctgtcttttcatagtaaaaacaaaacaaaaacacccaatgttaaaaccacataataaacttacaaacttgaaaaattagacacttcagatagataggcaataaaacttcatattatgaaagcaatatattccaagtttcaaagatttgacaagttctgtagagtatctttcatcagtacatgaaaacttccaaactgcatgatcttctgccaggcaggactgggtgctattcgctggtttgaggtcgaatccatttcaaggcatgtcgtggtgggacattaatggtgggatggtagaatgtgcagtccggtcttgtacattgagtgttaaacctacaatgttttggatgatagaagggacattccatcttcttacaagcagggaagtaacggcagagctgactactggaaggtggtgctggtggtgcaactggttttggagacagtactggaattcttctactcacatgagtgaagggacaatctggtttagtacactttgcatcatatttacaatttgggtgaacaaacaaacatttttcagcaaatttacaattggggaaggctttgcagggtgagatggggtgatggtaggcacactcatccccatttttacaagcaggccagtacttgcagcgctccaaaagtttttctggtttctgtgccacactcagttcactcatctcagcttgatttttttctacagaatctccttttgtttcctcttctttaatggggggacttattctgggggtcctactttgtccctggaccacttctgctagcaattcttcttgagaagttcgagttctgggagcaactggaagtgtctgtttctgtggaactgtagagtagttagttgtttttgttacggattcttgagcttcagatatagccttcaaaatcagattcttgttagcttgtttagaaggtggaagagaaggtctcctttcaggctttgcaggcacagacacactgctggagatgcttcctgttcgagacccgtaatcatcatcttcttcctcctcttctccatcatgattgaatttttttactttaacaactgaacttaccacaggcaactttctcttccgaaagttttcatcctccatactcattttctccgagttgtttctaaagaacggactatacgtttcttctaagctgttaagcacctctggttcacacaaacgtcctgtttcatatacccaactactctgcatatcaagctgcttggcagcatgaatactattctgctgctgttgaaattgcaacctgtttaaatgaacaccactatctgcatttctacttgcaggtggtcgataaatttcaatagaagggcgagaagaaccatatgtaagtgtcactgtaggttttttctgagataagggattctcctgcacaaagttgaggtcttcgtcaatgagatcatctggttctggcttaatatcaatcacatcttcagagggtgctggctccctcaaaggtttcactgttgacattagtcgggttgcagctccatcatcgtaagtctgtctgacatttgtggtttttgactcctgcgaacttgtagaaactctggaatctcttttttcaggtctcgcgctaggaatggcaagtggtggcactgcagcttcatgcctcctctcatctccccgactgaaattgctcttgtttgaaggcacgttactatcaaagatgttggtatcagaagacttcagactagagggttcagttgtaacagagcgaagtttatctaatacaccatgaagccatacggtgaatcgaattgtgttgttccctagaaacagggacagatcctctgtcatttggtcctgacttttcttgttggccaccatcaccataatgtaatcaggaagttcttcatctatttaaaaggaaaggtagatcaaaactttgtttcctcaaaactttcttcttaaagttgatgtgcttgaaaatatagatgtagctctaagctttagagtcgcagagctctactggaattacattggacaagatggcttagctttaatttttttctcttcattccacaggtatttcaaatacaacataagctcctaattcttgtaatttccccttaatggcactccggatcttgcggctgatctcggtgccgatctccatggctctgcggcgtgcgggaactcagcactgcgcggcgcttggcttacccggaggctgccgcggactcctaccccgcagccgggacaccaccgcctcc

SEQ ID NO: 13634 - RNA, 1550 nt, Homo sapiens
  source 1..1550: mol_type = other RNA
gctgggattacaggcatgagccaccatacccagcctgcatcctaatttatgattcctattttgtgcctggtgaacagtccccatatttaacaataatacctacacataaaacaatccactgttacaatttatatagtcacaaagcattaagtatcttctgtagaccatagtttttaaccataattttctgcatcaaatccacagccagaatccccaagatcaaaaaaatttgcacaatacaaaccataatctaaagtacatgtacagacacatacacactctcacacacacttcttacagaactgtgcttggggaaactccatttgttgagtgccactgaaggcatattttgctacactgctgctccaggtatttttgtttggaaaaatctgtcacagtagggtatgactatttactggatgaacagaaaagaaagatatacctgtggcaaccagaaagttttaaggtctttcaagtcgtataaaatggacctgcagaaacgttggaatgttctcaggatgcaaagttggagctgaaatgtgatatcaaacagttgcaaaaaatgtatagcaaccatgccttgaggtcaaacctggtaccgagatctgcaacaaaaagcttcaagacacatagtttgttgggcttgtcccacatggtcgcataatctgctcatgtgtgaatttcacaaacgactcgtattgctctgctagtttggtattgaggattttctcatactcctcccaaatcttctcttcatagtttgagagacgtgtacatattgttctagcttgccggagggccaaggtgggctggtccatcttcacccaggagaaacctgcagcactgggtgctgggtgctgaggactgaggctggctttcctaagcacaagctgccctctgattaagaacaacttctaaatgtgtccacctctgataatgattctattatatgttgaaaaatgtgtttcggagttggaaggtgcctctggcggccaggcggggcaggctgctgcagggtcgcggtggggtttgcgtctgaaacgccggcggtggctcggcgtcccagggcctggggcccggagccgggcggggaagcggggagtggcgcggccgctttggggaaccaggctcagcagcgtcgcctcgagctccgtgggctgcttcggtgtcgccccgctcgccatgtggccggggaccgggaggggacgcggcagtagttgcgtcccaacctccggactcctcagcggggctctcaagcccagtaggctccaatccgttgagttcctcaatgttcctcggagtcgtccatagtttaaaatgacttctgcacctttcttataaccttgattgaagccctgttgaagagtaactgctttgccagcatctattccatctctataaccttctttgactcgtctttgcatgttactctgccattcccgctgcgccaggagcgactcgtctgcttcttcgtcaaacacgtcccctttgtctccagggccctggatcaaggaggctgcttgaacccacgacatcaccgaggcaattac

SEQ ID NO: 13635 - RNA, 635 nt, Homo sapiens
  source 1..635: mol_type = other RNA
gctgggattacaggcatgagccaccatacccagccttgttttcttcttgaaaccagttttcctgtcccttttaccttcattccagcccagcctggcttcatctcagtccttagattaacctccctcctctgctgccactgggtggggtctgcagttttccaccctgtggtcagccaacatactggatagcagaatcacagtcctaggttcatctccacaggctggagtgcaggtccaacttgcttcctcaaacagcacaacttgtttttctttctccggtgtctgctccctcctgatgcaggatccacttaagtctttctgaaactgacaccaggatcaagggaggaaaaaccaggcagcacaaagcctttggcaggctcctgcagcaagttctgtgctgcctgctcctcctgaaaatcctctctcagctctttccagatgtgccccagactctcacgagcacatttctctcaaacagcccatcaatcactccatgagtgtttacttagtgcccgcttcatgcgagacattgtcctctacgcccgggagcatgcctccatgtgggagaattgattcctgccttccagacctcatggcctctgcaaggaaacacgacatcagccaaagaaaataca

SEQ ID NO: 13636 - RNA, 622 nt, Homo sapiens
  source 1..622: mol_type = other RNA
gctgggattacaggcatgagccaccatacccagccttgttttcttcttgaaaccagttttccttcattccagcccagcctggcttcatctcagtccttagattaacctccctcctctgctgccactgggtggggtctgcagttttccaccctgtggtcagccaacatactggatagcagaatcacagtcctaggttcatctccacaggctggagtgcaggtccaacttgcttcctcaaacagcacaacttgtttttctttctccggtgtctgctccctcctgatgcaggatccacttaagtctttctgaaactgacaccaggatcaagggaggaaaaaccaggcagcacaaagcctttggcaggctcctgcagcaagttctgtgctgcctgctcctcctgaaaatcctctctcagctctttccagatgtgccccagactctcacgagcacatttctctcaaacagcccatcaatcactccatgagtgtttacttagtgcccgcttcatgcgagacattgtcctctacgcccgggagcatgcctccatgtgggagaattgattcctgccttccagacctcatggcctctgcaaggaaacacgacatcagccaaagaaaataca

SEQ ID NO: 13637 - RNA, 53 nt, Homo sapiens
  source 1..53: mol_type = other RNA
gctgggattacaggcatgagccaccatacccggccccaacatattattattaa

SEQ ID NO: 13638 - RNA, 2723 nt, Homo sapiens
  source 1..2723: mol_type = other RNA
gctgggattacaggcatgagccaccatacccggcgttttttctatacttttaaaaatggctcagagcagcaaaacaagttagaggatttattctgtgaaatgcactgcagagaaaaagaatgggcaaatagtataattaaaaatagttattgattcacactttccaaaatttttaaaaagtaaaccaccaaagaccaatacttctctctcctttcaatactaagccattttttccagtaaaattaatgaaataatgtatatttttataactaatcagtttgtgacagctgtggttctcactttttaaaaatacaaaatcatagttgcaaacagataatacacaatgatttttaaaactgaataggcaaagccttactctaactgatcaaatgaccaatcagctggattcaggcttttcaggctacagatgactttgatcaacagccctgcacatatcagaagcgtccccacagatgttctaaacacaaatgcggctgctgacaccctgacgctgcaaacaacagcaagggcatagagaggagaccttgatgattcagtgtgattcttcaacagatttctcttcttcactttcctcattggcttcatctttttccttgtaagaatcctggctgttggtatcaataaaataattttcttccccattctctctttcttctattttttcttcttcattaaagctttctttgtcttcagtgacacttttcgtctcttgattgttgaagtactcaagtacttttccactttggcctttctttgaaacaaactcatcagatattcctagtgcttttagggtattagaataatgcttttctgctgccattcttgcatttttctgagcaactctttcaaatagcagtggcctcttttttaatttttcttctctttcttctagttctcgttggtattctctcatcctttccttttcgctctttctgagacattttactctggatttagatatttgagctaaactttgatgtgagtcataagccttagcccgggttgtcaggagtttctgcaattctttcattctttgcttctgtttagttaggatccgatttctctcttcttccaacattttcttttcctcaagtgatctccttacggcttgttctcgtcctctggaagataccgtgggcacgggagggttgcagttacaaggcacagggtttacacctgcacatcttactggtgacttacgccttggagacaaataaggccaacgtgtttcttttaaattttcttcatctgcttcgatgtctgccaaaattttttctcttttaatagatgcatgtggagatgcatgaagatcaaatggtttacacactgttaagagttttggagacttgtgttctgagaggtgtttctggtatctctcaggaaggtcctcaaaatcaggagttgggcacctaaccttgtgtttacacttcaactttacagcctgttcaggacacctggggttcctgcatccacaagctgacctacaaggcagaggagatgagttctgtaaatgctcctgggctctcagctgtgtcctaaggtttcgatagagctcttcttcttttaacttgtcattggtagttgaaccataagtagatcgaggaatgggtctggctttaaatcgatttgttttctttttatacttaagaaagtctctcagctgcttttcccgggctgctcgcttctgttcctcccttgctataaatttaaatggcttttgtgaggccaaaagagcttctttgcttttctccttcagagaccttctccgttcttctttttgcttgactaaatcatggtaaagggggagaaagacagatgcaggaactggattggctcggaatttcttcttatactctggatcctcttcttgttttttgagcgctttatgtaccatttcgatatctgatttagatttcatggactcttcttttttcttctgttctcttatcatcatttgaaaaggctccggtactgtaattgtgggcacccattcttttcgtttcttccttcttttttcagctgcatggaagccagtatctttacagcgaatataatcctcaacacaaaagtctgtccacatattgttgatgagctccttagcataggtcatcattctgtttttcctaggatactctttttctaggttgggtaactcctcttcagaggaggacacatacaaggaggaagactggcctaaatcaggctctgaaaatgatgtcattaatgagacagggtgataggagttcttttctgatacagatctggaagagtcactaagagagtcttctctgatgaccactggctgaacttcctttaaatgtaatttatcctggtacattttctctaattttgccatagtttctatgtgggcagccttcaactcttctactttcttgaaatactcctcattagagtggtgaatatcaggaaagttcacaaagtcctcatagcttatcggtgcatgttcatccaccccagaaaagctggtgttcaaatcagccgatgccccagcgggctgagccactttctcctcctcttcgtcctccaagatcgcctccgctgccgccagggcctttaaggggtcttcgcgttcgtactgggcgacccgcgctccagtgatgggatttaccggggtctggagactggaggccaccagcttcgccactcggtgggaggtggccatcgccccgcctccgaggcct

SEQ ID NO: 13639 - RNA, 2733 nt, Homo sapiens
  source 1..2733: mol_type = other RNA
gctgggattacaggcatgagccaccatacccggcgttttttctatacttttaaaaatggctcagagcagcaaaacaagttagaggatttattctgtgaaatgcactgcagagaaaaagaatgggcaaatagtataattaaaaatagttattgattcacactttccaaaatttttaaaaagtaaaccaccaaagaccaatacttctctctcctttcaatactaagccattttttccagtaaaattaatgaaataatgtatatttttataactaatcagtttgtgacagctgtggttctcactttttaaaaatacaaaatcatagttgcaaacagataatacacaatgatttttaaaactgaataggcaaagccttactctaactgatcaaatgaccaatcagctggattcaggcttttcaggctacagatgactttgatcaacagccctgcacatatcagaagcgtccccacagatgttctaaacacaaatgcggctgctgacaccctgacgctgcaaacaacagcaagggcatagagaggagaccttgatgattcagtgtgattcttcaacagatttctcttcttcactttcctcattggcttcatctttttccttgtaagaatcctggctgttggtatcaataaaataattttcttccccattctctctttcttctattttttcttcttcattaaagctttctttgtcttcagtgacacttttcgtctcttgattgttgaagtactcaagtacttttccactttggcctttctttgaaacaaactcatcagatattcctagtgcttttagggtattagaataatgcttttctgctgccattcttgcatttttctgagcaactctttcaaatagcagtggcctcttttttaatttttcttctctttcttctagttctcgttggtattctctcatcctttccttttcgctctttctgagacattttactctggatttagatatttgagctaaactttgatgtgagtcataagccttagcccgggttgtcaggagtttctgcaattctttcattctttgcttctgtttagttaggatccgatttctctcttcttccaacattttcttttcctcaagtgatctccttacggcttgttctcgtcctctggaagataccgtgggcacgggagggttgcagttacaaggcacagggtttacacctgcacatcttactggtgacttacgccttggagacaaataaggccaacgtgtttcttttaaattttcttcatctgcttcgatgtctgccaaaattttttctcttttaatagatgcatgtggagatgcatgaagatcaaatggtttacacactgttaagagttttggagacttgtgttctgagaggtgtttctggtatctctcaggaaggtcctcaaaatcaggagttgggcacctaaccttgtgtttacacttcaactttacagcctgttcaggacacctggggttcctgcatccacaagctgacctacaaggcagaggagatgagttctgtaaatgctcctgggctctcagctgtgtcctaaggtttcgatagagctcttcttcttttaacttgtcattggtagttgaaccataagtagatcgaggaatgggtctggctttaaatcgatttgttttctttttatacttaagaaagtctctcagctgcttttcccgggctgctcgcttctgttcctcccttgctataaatttaaatggcttttgtgaggccaaaagagcttctttgcttttctccttcagagaccttctccgttcttctttttgcttgactaaatcatggtaaagggggagaaagacagatgcaggaactggattggctcggaatttcttcttatactctggatcctcttcttgttttttgagcgctttatgtaccatttcgatatctgatttagatttcatggactcttcttttttcttctgttctcttatcatcatttgaaaaggctccggtactgtaattgtgggcacccattcttttcgtttcttccttcttttttcagctgcatggaagccagtatctttacagcgaatataatcctcaacacaaaagtctgtccacatattgttgatgagctccttagcataggtcatcattctgtttttcctaggatactctttttctaggttgggtaactcctcttcagaggaggacacatacaaggaggaagactggcctaaatcaggctctggaagagtcactaagagagtcttctctgatgaccactggctgaacttcctttaaatgtaatttatcctggtacattttctctaattttgccatagtttctatgtgggcagccttcaactcttctactttcttgaaatactcctcattagagtggtgaatatcaggaaagttcacaaagtcctcatagcttatcggtgcatgttcatccaccccagaaaagctggtgttcaaatcagccgatgccccagcgggctgagccactttctcctcctcttcgtcctccaagatcgcctccgctgccgccagggcctttaaggggtcttcgcgttcgtactgggcgacccgcgctccagtgatgggatttaccggggtctggagactggaggccaccagcttcgccactcggtgggaggtggccatcgccccgcctccgaggcctgagcgcctgcgctggcccgggacgggaaagctggtgcggcccctggcaacccgggggcgcctagct

SEQ ID NO: 13640 - RNA, 2555 nt, Homo sapiens
  source 1..2555: mol_type = other RNA
gctgggattacaggcatgagccaccatacccggcgttttttctatacttttaaaaatggctcagagcagcaaaacaagttagaggatttattctgtgaaatgcactgcagagaaaaagaatgggcaaatagtataattaaaaatagttattgattcacactttccaaaatttttaaaaagtaaaccaccaaagaccaatacttctctctcctttcaatactaagccattttttccagtaaaattaatgaaataatgtatatttttataactaatcagtttgtgacagctgtggttctcactttttaaaaatacaaaatcatagttgcaaacagataatacacaatgatttttaaaactgaataggcaaagccttactctaactgatcaaatgaccaatcagctggattcaggcttttcaggctacagatgactttgatcaacagccctgcacatatcagaagcgtccccacagatgttctaaacacaaatgcggctgctgacaccctgacgctgcaaacaacagcaagggcatagagaggagaccttgatgattcagtgtgattcttcaacagatttctcttcttcactttcctcattggcttcatctttttccttgtaagaatcctggctgttggtatcaataaaataattttcttccccattctctctttcttctattttttcttcttcattaaagctttctttgtcttcagtgacacttttcgtctcttgattgttgaagtactcaagtacttttccactttggcctttctttgaaacaaactcatcagatattcctagtgcttttagggtattagaataatgcttttctgctgccattcttgcatttttctgagcaactctttcaaatagcagtggcctcttttttaatttttcttctctttcttctagttctcgttggtattctctcatcctttccttttcgctctttcttacggcttgttctcgtcctctggaagataccgtgggcacgggagggttgcagttacaaggcacagggtttacacctgcacatcttactggtgacttacgccttggagacaaataaggccaacgtgtttcttttaaattttcttcatctgcttcgatgtctgccaaaattttttctcttttaatagatgcatgtggagatgcatgaagatcaaatggtttacacactgttaagagttttggagacttgtgttctgagaggtgtttctggtatctctcaggaaggtcctcaaaatcaggagttgggcacctaaccttgtgtttacacttcaactttacagcctgttcaggacacctggggttcctgcatccacaagctgacctacaaggcagaggagatgagttctgtaaatgctcctgggctctcagctgtgtcctaaggtttcgatagagctcttcttcttttaacttgtcattggtagttgaaccataagtagatcgaggaatgggtctggctttaaatcgatttgttttctttttatacttaagaaagtctctcagctgcttttcccgggctgctcgcttctgttcctcccttgctataaatttaaatggcttttgtgaggccaaaagagcttctttgcttttctccttcagagaccttctccgttcttctttttgcttgactaaatcatggtaaagggggagaaagacagatgcaggaactggattggctcggaatttcttcttatactctggatcctcttcttgttttttgagcgctttatgtaccatttcgatatctgatttagatttcatggactcttcttttttcttctgttctcttatcatcatttgaaaaggctccggtactgtaattgtgggcacccattcttttcgtttcttccttcttttttcagctgcatggaagccagtatctttacagcgaatataatcctcaacacaaaagtctgtccacatattgttgatgagctccttagcataggtcatcattctgtttttcctaggatactctttttctaggttgggtaactcctcttcagaggaggacacatacaaggaggaagactggcctaaatcaggctctgaaaatgatgtcattaatgagacagggtgataggagttcttttctgatacagatctggaagagtcactaagagagtcttctctgatgaccactggctgaacttcctttaaatgtaatttatcctggtacattttctctaattttgccatagtttctatgtgggcagccttcaactcttctactttcttgaaatactcctcattagagtggtgaatatcaggaaagttcacaaagtcctcatagcttatcggtgcatgttcatccaccccagaaaagctggtgttcaaatcagccgatgccccagcgggctgagccactttctcctcctcttcgtcctccaagatcgcctccgctgccgccagggcctttaaggggtcttcgcgttcgtactgggcgacccgcgctccagtgatgggatttaccggggtctggagactggaggccaccagcttcgccactcggtgggaggtggccatcgccccgcctccgaggcct

SEQ ID NO: 13641 - RNA, 2591 nt, Homo sapiens
  source 1..2591: mol_type = other RNA
gctgggattacaggcatgagccaccatacccggcgttttttctatacttttaaaaatggctcagagcagcaaaacaagttagaggatttattctgtgaaatgcactgcagagaaaaagaatgggcaaatagtataattaaaaatagttattgattcacactttccaaaatttttaaaaagtaaaccaccaaagaccaatacttctctctcctttcaatactaagccattttttccagtaaaattaatgaaataatgtatatttttataactaatcagtttgtgacagctgtggttctcactttttaaaaatacaaaatcatagttgcaaacagataatacacaatgatttttaaaactgaataggcaaagccttactctaactgatcaaatgaccaatcagctggattcaggcttttcaggctacagatgactttgatcaacagccctgcacatatcagaagcgtccccacagatgttctaaacacaaatgcggctgctgacaccctgacgctgcaaacaacagcaagggcatagagaggagaccttgatgattcagtgtgattcttcaacagatttctcttcttcactttcctcattggcttcatctttttccttgtaagaatcctggctgttggtatcaataaaataattttcttccccattctctctttcttctattttttcttcttcattaaagctttctttgtcttcagtgacacttttcgtctcttgattgttgaagtactcaagtacttttccactttggcctttctttgaaacaaactcatcagatattcctagtgcttttagggtattagaataatgcttttctgctgccattcttgcatttttctgagcaactctttcaaatagcagtggcctcttttttaatttttcttctctttcttctagttctcgttggtattctctcatcctttccttttcgctctttcttacggcttgttctcgtcctctggaagataccgtgggcacgggagggttgcagttacaaggcacagggtttacacctgcacatcttactggtgacttacgccttggagacaaataaggccaacgtgtttcttttaaattttcttcatctgcttcgatgtctgccaaaattttttctcttttaatagatgcatgtggagatgcatgaagatcaaatggtttacacactgttaagagttttggagacttgtgttctgagaggtgtttctggtatctctcaggaaggtcctcaaaatcaggagttgggcacctaaccttgtgtttacacttcaactttacagcctgttcaggacacctggggttcctgcatccacaagctgacctacaaggcagaggagatgagttctgtaaatgctcctgggctctcagctgtgtcctaaggtttcgatagagctcttcttcttttaacttgtcattggtagttgaaccataagtagatcgaggaatgggtctggctttaaatcgatttgttttctttttatacttaagaaagtctctcagctgcttttcccgggctgctcgcttctgttcctcccttgctataaatttaaatggcttttgtgaggccaaaagagcttctttgcttttctccttcagagaccttctccgttcttctttttgcttgactaaatcatggtaaagggggagaaagacagatgcaggaactggattggctcggaatttcttcttatactctggatcctcttcttgttttttgagcgctttatgtaccatttcgatatctgatttagatttcatggactcttcttttttcttctgttctcttatcatcatttgaaaaggctccggtactgtaattgtgggcacccattcttttcgtttcttccttcttttttcagctgcatggaagccagtatctttacagcgaatataatcctcaacacaaaagtctgtccacatattgttgatgagctccttagcataggtcatcattctgtttttcctaggatactctttttctaggttgggtaactcctcttcagaggaggacacatacaaggaggaagactggcctaaatcaggctctgaaaatgatgtcattaatgagacagggtgataggagttcttttctgatacagatctggaagagtcactaagagagtcttctctgatgaccactggctgaacttcctttaaatgtaatttatcctggtacattttctctaattttgccatagtttctatgtgggcagccttcaactcttctactttcttgaaatactcctcattagagtggtgaatatcaggaaagttcacaaagtcctcatagcttatcggtgcatgttcatccaccccagaaaagctggtgttcaaatcagctcctttctgttagccctctgactgcttcctgtcggcttgtgtcagtctagcaacggttattcatctgggcagcagcagttcgttttagtagcagtgtctgaatccagtatgcagttttcactcgaaaaatcaacagaattggccaggcacagtggttcatgcctgtaatcccagcactttgggtcacttgaggtcaggaatccgagaccaatctggccaacatggtgaaaccccatct

SEQ ID NO: 13642 - RNA, 2499 nt, Homo sapiens
  source 1..2499: mol_type = other RNA
gctgggattacaggcatgagccaccatacccggcgttttttctatacttttaaaaatggctcagagcagcaaaacaagttagaggatttattctgtgaaatgcactgcagagaaaaagaatgggcaaatagtataattaaaaatagttattgattcacactttccaaaatttttaaaaagtaaaccaccaaagaccaatacttctctctcctttcaatactaagccattttttccagtaaaattaatgaaataatgtatatttttataactaatcagtttgtgacagctgtggttctcactttttaaaaatacaaaatcatagttgcaaacagataatacacaatgatttttaaaactgaataggcaaagccttactctaactgatcaaatgaccaatcagctggattcaggcttttcaggctacagatgactttgatcaacagccctgcacatatcagaagcgtccccacagatgttctaaacacaaatgcggctgctgacaccctgacgctgcaaacaacagcaagggcatagagaggagaccttgatgattcagtgtgattcttcaacagatttctcttcttcactttcctcattggcttcatctttttccttgtaagaatcctggctgttggtatcaataaaataattttcttccccattctctctttcttctattttttcttcttcattaaagctttctttgtcttcagtgacacttttcgtctcttgattgttgaagtactcaagtacttttccactttggcctttctttgaaacaaactcatcagatattcctagtgcttttagggtattagaataatgcttttctgctgccattcttgcatttttctgagcaactctttcaaatagcagtggcctcttttttaatttttcttctctttcttctagttctcgttggtattctctcatcctttccttttcgctctttcttacggcttgttctcgtcctctggaagataccgtgggcacgggagggttgcagttacaaggcacagggtttacacctgcacatcttactggtgacttacgccttggagacaaataaggccaacgtgtttcttttaaattttcttcatctgcttcgatgtctgccaaaattttttctcttttaatagatgcatgtggagatgcatgaagatcaaatggtttacacactgttaagagttttggagacttgtgttctgagaggtgtttctggtatctctcaggaaggtcctcaaaatcaggagttgggcacctaaccttgtgtttacacttcaactttacagcctgttcaggacacctggggttcctgcatccacaagctgacctacaaggcagaggagatgagttctgtaaatgctcctgggctctcagctgtgtcctaaggtttcgatagagctcttcttcttttaacttgtcattggtagttgaaccataagtagatcgaggaatgggtctggctttaaatcgatttgttttctttttatacttaagaaagtctctcagctgcttttcccgggctgctcgcttctgttcctcccttgctataaatttaaatggcttttgtgaggccaaaagagcttctttgcttttctccttcagagaccttctccgttcttctttttgcttgactaaatcatggtaaagggggagaaagacagatgcaggaactggattggctcggaatttcttcttatactctggatcctcttcttgttttttgagcgctttatgtaccatttcgatatctgatttagatttcatggactcttcttttttcttctgttctcttatcatcatttgaaaaggctccggtactgtaattgtgggcacccattcttttcgtttcttccttcttttttcagctgcatggaagccagtatctttacagcgaatataatcctcaacacaaaagtctgtccacatattgttgatgagctccttagcataggtcatcattctgtttttcctaggatactctttttctaggttgggtaactcctcttcagaggaggacacatacaaggaggaagactggcctaaatcaggctctggaagagtcactaagagagtcttctctgatgaccactggctgaacttcctttaaatgtaatttatcctggtacattttctctaattttgccatagtttctatgtgggcagccttcaactcttctactttcttgaaatactcctcattagagtggtgaatatcaggaaagttcacaaagtcctcatagcttatcggtgcatgttcatccaccccagaaaagctggtgttcaaatcagccgatgccccagcgggctgagccactttctcctcctcttcgtcctccaagatcgcctccgctgccgccagggcctttaaggggtcttcgcgttcgtactgggcgacccgcgctccagtgatgggatttaccggggtctggagactggaggccaccagcttcgccactcggtgggaggtggccatcgccccgcctccgaggcct

SEQ ID NO: 13643 - RNA, 2538 nt, Homo sapiens
  source 1..2538: mol_type = other RNA
gctgggattacaggcatgagccaccatacccggcgttttttctatacttttaaaaatggctcagagcagcaaaacaagttagaggatttattctgtgaaatgcactgcagagaaaaagaatgggcaaatagtataattaaaaatagttattgattcacactttccaaaatttttaaaaagtaaaccaccaaagaccaatacttctctctcctttcaatactaagccattttttccagtaaaattaatgaaataatgtatatttttataactaatcagtttgtgacagctgtggttctcactttttaaaaatacaaaatcatagttgcaaacagataatacacaatgatttttaaaactgaataggcaaagccttactctaactgatcaaatgaccaatcagctggattcaggcttttcaggctacagatgactttgatcaacagccctgcacatatcagaagcgtccccacagatgttctaaacacaaatgcggctgctgacaccctgacgctgcaaacaacagcaagggcatagagaggagaccttgatgattcagtgtgattcttcaacagatttctcttcttcactttcctcattggcttcatctttttccttgtaagaatcctggctgttggtatcaataaaataattttcttccccattctctctttcttctattttttcttcttcattaaagctttctttgtcttcagtgacacttttcgtctcttgattgttgaagtactcaagtacttttccactttggcctttctttgaaacaaactcatcagatattcctagtgcttttagggtattagaataatgcttttctgctgccattcttgcatttttctgagcaactctttcaaatagcagtggcctcttttttaatttttcttctctttcttctagttctcgttggtattctctcatcctttccttttcgctctttcttacggcttgttctcgtcctctggaagataccgtgggcacgggagggttgcagttacaaggcacagggtttacacctgcacatcttactggtgacttacgccttggagacaaataaggccaacgtgtttcttttaaattttcttcatctgcttcgatgtctgccaaaattttttctcttttaatagatgcatgtggagatgcatgaagatcaaatggtttacacactgttaagagttttggagacttgtgttctgagaggtgtttctggtatctctcaggaaggtcctcaaaatcaggagttgggcacctaaccttgtgtttacacttcaactttacagcctgttcaggacacctggggttcctgcatccacaagctgacctacaaggcagaggagatgagttctgtaaatgctcctgggctctcagctgtgtcctaaggtttcgatagagctcttcttcttttaacttgtcattggtagttgaaccataagtagatcgaggaatgggtctggctttaaatcgatttgttttctttttatacttaagaaagtctctcagctgcttttcccgggctgctcgcttctgttcctcccttgctataaatttaaatggcttttgtgaggccaaaagagcttctttgcttttctccttcagagaccttctccgttcttctttttgcttgactaaatcatggtaaagggggagaaagacagatgcaggaactggattggctcggaatttcttcttatactctggatcctcttcttgttttttgagcgctttatgtaccatttcgatatctgatttagatttcatggactcttcttttttcttctgttctcttatcatcatttgaaaaggctccggtactgtaattgtgggcacccattcttttcgtttcttccttcttttttcagctgcatggaagccagtatctttacagcgaatataatcctcaacacaaaagtctgtccacatattgttgatgagctccttagcataggtcatcattctgtttttcctaggatactctttttctaggttgggtaactcctcttcagaggaggacacatacaaggaggaagactggcctaaatcaggctctggaagagtcactaagagagtcttctctgatgaccactggctgaacttcctttaaatgtaatttatcctggtacattttctctaattttgccatagtttctatgtgggcagccttcaactcttctactttcttgaaatactcctcattagagtggtgaatatcaggaaagttcacaaagtcctcatagcttatcggtgcatgttcatccaccccagaaaagctggtgttcaaatcagctcctttctgttagccctctgactgcttcctgtcggcttgtgtcagtctagcaacggttattcatctgggcagcagcagttcgttttagtagcagtgtctgaatccagtatgcagttttcactcgaaaaatcaacagaattggccaggcacagtggttcatgcctgtaatcccagcactttgggtcacttgaggtcaggaatccgagaccaatctggccaacatggtgaaaccccatctcta

SEQ ID NO: 13644 - RNA, 1400 nt, Homo sapiens
  source 1..1400: mol_type = other RNA
gctgggattacaggcatgagccaccatacctgactgattctcagattctgaaatgacagttaagcccaggactcaagccagggacagaagcagataacctggttttggtgagaaggttatgcacttgcttctgaaaatgttgatgatgagactaagtcttatagtttcttgtgcacctcccttggtgcctagaagaaaggttaaaacaggatacattacagagggactatcttgagagaggagttacctgggcacagcccaggggcccttgggagtgacatgcaagggcagcactggcttgccttatttggttctcccgctctttcttctttcccttgtaaaagtaactgaagcttaaaggtgaaaatgacttaaataatagaaaccatgttagccttactccccttccccattagccacaaattggtggcgatcaccattttgtgcaccgagcctgggtctcacgcttgcaagtccttgggctcatctggagtcagcttcatcagtttgtccacacagagcaggatgagggtgaggaaccagaggctccagccaacagctgccgcgatccagccgtactcgtccactcctgtgcggcagcaccgggctgcttgtgggcagaagtccacgttgaggcactgctccagggtcccagggtctgggtggtgagcggtcaagcttgagctgttgctgctgcttgctgccgagcaagccgagtggagggaggcaaaggccaggctgaggatcagggtggcccgggtggcagcggggaggcgctgcatgctggaggctgtgctgagtgcccggtgcaggtgagccggtcctgcggagttgtgccgagtgcctgctgcaggtgagtcgactcccacctgcaggagctggaaagcaactctgccagaggtgaacttatgctgggtgtttgggggaaacaccatggggtggagcaaaggaaacttggcctgtcacaccttctctcacctctctagaagggaagccaaaccgttggctgaggaaggaagggaggggcaagctgtgcccttctcccctgagcgcaaatattgtccttattgagaaacaaggggaggacaagagagatctgtgtcatgctggttcctgggacatgagtttgctgcctctcccatctgcaggtgtagcatggatgctcaattccatttgggccaatattcactgagcacccactatgctgaagttgggagatacctgctgtcgaagtgcgttaattacaaacacgcatcattcaaccccagaaccgtgtttgaggaatggcttgggaggataaagcactgtgggtttcaacagtggaggccacatctgctgatgggatgcttcaagaagaaaatggcatttgaggttgggcatgggggctcaccctgtagtcc

SEQ ID NO: 13645 - RNA, 896 nt, Homo sapiens
  source 1..896: mol_type = other RNA
gctgggattacaggcatgagccaccatacctgactgattctcagattctgaaatgacagttaagcccaggactcaagccagggacagaagcagataacctggttttggtgagaaggttatgcacttgcttctgaaaatgttgatgatgagactaagtcttatagtttcttgtgcacctcccttggtgcctagaagaaaggttaaaacaggatacattacagagggactatcttgagagaggagttacctgggcacagcccaggggcccttgggagtgacatgcaagggcagcactggcttgccttatttggttctcccgctctttcttctttcccttgtaaaagtaactgaagcttaaaggtgaaaatgacttaaataatagaaaccatgttagccttactccccttccccattagccacaaattggtggcgatcaccattttgtgcaccgagcctgggtctcacgcttgcaagtccttgggctcatctggagtcagcttcatcagtttgtccacacagagcaggatgagggtgaggaaccagaggctccagccaacagctgccgcgatccagccgtactcgtccactcctgtgcggcagcaccgggctgcttgtgggcagaagtccacgttgaggcactgctccagggtcccagggtctgggtggtgagcggtcaagcttgagctgttgctgctgcttgcttctgccgagcaagccgagtggagggaggcaaaggccaggctgaggatcagggtggcccgggtggcagcggggaggcgctgcatgctggaggctgtgctgagtgcccggtgcaggtgagccggtcctgcggagttgtgccgagtgcctgctgcaggtgagtcgactcccacctgcaggagctggaaagcaactct

SEQ ID NO: 13646 - RNA, 1584 nt, Homo sapiens
  source 1..1584: mol_type = other RNA
gctgggattacaggcatgagccaccatacctggccaacatatcatacttttaaagtacttttaaatatagtacatttcccttgtaattcctttatataataagtccacctatgtgcattagtaagcttctttacaactcacctccaaatttaaagaattaattcatgcattggcttacagcaaaagaacttttgttttgattcatgtgtttaaaagaagaaatcaattaaagttcaattttaatatccaaagatgtaaggtggcaaatgttaccttctcaaggaagttttttctaccttcaagttcacagaaaatcataaaatgaaaacaatcactaggcataaatcagttataaagctacctttctaacacaatgcagctcactacatactccacaaaggtgaagtaaataacatcaaactcaaattttatcttgataactacacagtaatttttgctaattatatagcttaatttccaaatcttttcacatcattttaaaatatattctacatttctgagttttgatttgacaaaatggtaatcatttaaaatgaccctacttaaaaaaaaaattacaatttacaatttacaatcacttaaacaccaggatctaagttaaaacattagcaggcttcttgctctactttttacatttttatactaaacatatcccttaagtaaggatctacatttccatgttgtaataaaacattcagttacttaaattaagcagtgggggcatttatctgcaataagaagttacacaattacagtgctcatgtgcataaagtgatgatgctttcccaagcagctcatagacagaaacacagaaacactttttaaacatatttgttgatgaccctaaagacacacacttctaagtgtttgctttggaataaatgaacagccagcattttacttatcaagaaaccccaaggctttattagtattagaaatcagtaaagaaatccaaaactaaagaaaaacaaaaacgcctttttaaaaatacaacttcccttgttaagtgtattaatgcagtttttgtgtacctttgaaaattcttcaggttcctttatatctaatgaccttgttgcaaattctaatagttcttcagagttctccagggcattattacattgactaatctgactctgtaactcttgggatttacgagcttgttcctgcttgatacagttaatcatactttcttttacttcatccagtatagagtataaactatcaaattcttcatctaactctgagagtatgttggacgaattttcctgaactccttttagtgtatgatgtagtgtatcaataaagttctgaatttcatcatttttatttgccagagttgaaatgatcctctgtagagcttctttctgggagtccatggcgagtggctaagcccactgggctcgaacccgagacgacgaaccgtgtgaggaggctcagcgagatcgcacaccccaagaccgctactcactgcactgccccagcccgcaccggcaccgcccggccccacccgtccgcgcccagaccgcgcgcgccgtagtcacgccgcggttgccagggtgaaag

SEQ ID NO: 13647 - RNA, 4549 nt, Homo sapiens
  source 1..4549: mol_type = other RNA
gctgggattacaggcatgagccaccatacctggccgaaggcttgctgcattctaatagggctatttattaagaaatatgtaagtagggaaaaaatgtgtgcacaagtagagaaaaattgctagccaaaaaaaaaaaaaaaaagaataaaacagtatcatcaaaaccaaatcacagtgagactgttaatcacctctataaaagggagctaaactcattcagccaacctaaaattatgtttctttgtctttctctgtgatgagtgcctcaagtattgagttttaaaacttaatcttaaaaaaaaaattctgctgtgctgaagggtttaactaccatgttggatagtggtatatctaaaaataactttatagcatcttaattatggaaataatttataggtcccagtaagaagagaagcatacattttctattttcctcaaaacattttctagggcttcggcaaatatagctaaagatattgggaactaaactgtggaatccaatttttatgaacaggcagcaggagctgtatttttgattcttatttacaaattttataaaaatataaataaaatatatttctactcataaaaatgataaagggggtcataaggaacattaacaggtgtcaatattttctaagtacataaaaaagggttacatgatggaattacaggacagagaacaataattcaaggcctatggattatataccatgcaggagaaaaaaaccaattactaaatgaatcacgaatttcaattatgtgaatgttgacaaccttctttcaggaggttttaattaattggctattggtaggtaaggtgtaaggacatatgaccttttaggtttctatcactatgctgattttctgaatcactgtgtaaggtcaggagaaacttccctgaactccaaatccatgttagtttccaacactcttctttcctttatgtagatccaaggttccatctggtatcattttccttttgcctgagaacttcctttaacctgtagtatggttctgctgtttttgtctgaaaagtattcatattgcctctgaccaccactaagttcagttaggttttctttccaggtatttcccaaggcaaccttgaactccagaccatccaaaacagtttgaccctctggtggtgcaagcatagcattagcaccaggcaaaagagtagaaaaaatagacccaaagtccttgttcaccttttgccatgcaatatttagggcttggtttttcttctggtcaaggtcttctatagttgtaagaattttggatttgtcattttctacaattctcttcttcttcatcaagtcattgtatcgctcttcagcttctgtcaatacattcatagctctcatattgacatttcttcctagtttctccttcatttcttgcaacttctgaagtctctgaccagcttctttagggttgttagttttgaaatcataggcactattgggttggccaaagaggtgtctctctgcattaatccagtcataatctttcaacattttggatacctttgcagcaccatcttcagcctcccgtttatgtttgctgatgttgtggtctaattccttaattttaagctgagaatcattgttttgctccttgtgttttgccacttctgcatatttagctttaattacagtgtcttgggctgttatcacctctttttgcttggtcacctcttcttgagctttatttactgactccttatttttagccacctcagctgccattacttcaatctgactttcataggatttgatagcttcatttacagcttcaagctgttgtttgtaagatgtatgctctctcttgagctcttccagttccagagtgatagcttcaacttcctgttgtttttctttcatcttcttgctagatgcatctgcctttgttttggcacaatccagttttttctgagcatctttcagttctcgctctctttcagcttctgcatttttcattttattttccaatacttcatatttttcttctgcttttctttggatttctttagtgtttttcaaagtctcctcactttcctcaatggtttttttaagggcatctaattcttcttgttgcttgtgatatgagctttgctggagcttggtttgtaataaatctgcctcttcagttttcatctcccactgctgttttagttggcgatacttttcagcagtgtttttaagacctgctaattcctcttctagagcccgcagctcattctctttgattctcagttcatcctgaacatctttgagttcttgaaacttggttaaaatggaagctgcctgggatcgagcacctccactcaatgtcccatgaggatcaaacacatcacctccgagagttacagttctagtcattatcctcttatcaaaggccacttttttggcattatccatattgtcacaaacaaatgttgttccaaagacaaactccattgctttctgaagttctggtttatattcaaccaaggaaagagccacatgaacgttgtcagggccaacaagattctgagcaactctcagagtttctggtgcaatacatctggctgaaattttattgagtggaattatagtgtatcgacgtttcagttcccccctttctagtagctttttaccagtaacttctgtgtctactacaacattgtagagtcgttctccagccactaattctaaagctgtggttgcagaagtgtctttcacactaatcagagaagccacaagtcctttcacacaatttctattccagttcttctctggatccttgtatgcaaatcgaagattgggaaatctggctaatagagcttcatatgtttctttcaatctaccaatatcacgagacagctgcctgcgcttttccaaaaggctttcctctttattttcttcataatttagctttttcatttcagcttcaagtttttctttaagtctttttacagcttctagagcttcttgatccttcctgtagccactatccatcttcttaacttcagcttgtttattctttaattcctgttgagcatgcttcaacttcatctgagcctgtttggcttctgtctgagctttacttatatcatttttacaggccatcatttgaccagcaagagttgcttctgctccatcttcattactggacaggccagcggaaacagcattgaagtgctgctgtgcagctgccagagcttcagcatctttattacttgcttcttgaagggcatgcagtccatctgttatctttttaacctctttttcctttgctgctaaagtttttgagtcctcaaccatatttttttccagctctttgcgtttgctttcctcacatgccagatttttcttcttgagatcaaatgcgctttgagatttagtattaactcgctgagcctctgcaagagcatcttctaaagatcgaagtatacctccagtttccttatcttttcttttttccaattcttctatttcatgattaagtgcttttatttttttatcattctcagacaattcttcctgaagctttataactttatcttgcatttcttttaattcctcagctgagcgtactttggtatcttcagccagcaaaaactgataagcaatatataaacgactcaaatgttctatttctctcattactttttggtactccaagtaggacgatctttcctcttttaatttttgaatggttggagtaatctcttcttcaagtatcgtcttaatttctttcagcttagcctcctttttttctatagttttctgtgcagctatttttttgtattcatacatcctggttccagctgcttcttctatcatggataaaatctctggaggtttcatattcaatacttttgtaattcggccctgcatgatgagaaagtgagggttgttaacattaaggccaacagaacagaagagatcctgtactctggtgttgttggcattgactccattgattaaatatttatttctaccaccaataaccacctgccttgttactgtgatttcatcatgaacctcaaatcctaaaggactttgctttttgtcagaattatcaaaagtgattgacacagaggctttggtaataccagcctgcccatttttgtaaactaaatcttgtaaattagaagcccgaacctgagacaggttggagatgcccagcaaaaagcagatggagtccaatatgttggatttcccactaccatttaagccagtgatagcattgaagagggggtcaaaaccattgacttcggtcctctgagcataggacttgaatccctctagaataattgacttaatatgcattttcgatactgtcttgggtcagcaaacctctgacaggaatcaaacaggccacaaaccagttcgctgcctcaggccaggggcttgacgcaccccaaaagctcctccgggtcacaaaggcagggaacagaacaactctctagccggggccgctacaaagcgaacttcaccatagcggctacaacacctgccacaccgctctcaacacccgcgccggaactatttattccttt

SEQ ID NO: 13648 - RNA, 4922 nt, Homo sapiens
  source 1..4922: mol_type = other RNA
gctgggattacaggcatgagccaccatacctggcctaaacaaggcattttaacaaccaagaacaagtggcatctgtgccttagccattttgcttacatttctcctagctgcctaacgttcaccaggttgctgcttgcatccatgcattcattcgtctatttattaagtgctagtgtgcttctgaatgttgcagtacaaggggagggagatatatggatgacatagagctttaaaattaagaataaggctctagggtcagacttcttatattcacatgctggctccaccagcatgtaaatataagaactatgggagcttggacaagttacctgacctctgtgagcttccatttcctgaactgtgaaaactagggcaatataacttatctcagggtttcagtgaaaactaaagggataatacctagaaaagtggttagttagcaccaggactggctatctaatttaaagggcaaaaggaaaagcagaactccttgttcaaatatgattaagaaggcaatagtagagcattaaaccaagaacagggcccttctaagcatggggccctgtgtgactgcacaggttgcatgcctgtgaagctggccatggctgacacagtgcctgacatatggtgagtgcttgataaatgttaattattaattacccccagccactcctctgagagttcatctgttggtgagaaaagacacttaaccccaaaataactgcataagaaagagtatgacagacactgaagacatagttggagagttaggtgacatttcaggatccacgttttaaaaaagaacactgaaaagtaatttcctcttcagtggaaagaacacaggcttgtgagtcagacatttctgatatagctaataatagccactttttttttttaatagatggggtcttgctatttgcttaggctggagtgcagtggcaattcacaggcgtgatcatagtgcactacagtctcaaactcctgggctcaagcggtcctcctgcctcagcctcctgagtagctgggactacaggcgagtaccaccatgcctggctaatgagagccactattgactgagcatttcttatttctcagacactatgcaagatgcctactatatattatcttattaaatcttcccaacaatcttgggagaaaagtaacaattgttagtcccatttcacagataaggaaaacaagaatcagagcaatcaagtgactttcccaaggtcacccagctggtcattagaggcatggctcaaacctagccctatctggatctgggcttataacccctaagtcctacgctctgccactaatcagtgggtgattactggtcaggttatttttcctgctgtggtctccagctacctcagagggtgataaagtttgagtgaggctaaagtctgtaaaaccttaggtgggttaaaatatgtaacccctatagcaaagtggccacggttattctgggattttccttctttcctcttgagctaagcactggcacttaagagttaagtggttttatctttattggaaggaaatgtgttaaagacagactcactacagtgttgagacagtagtgagtagcacagtaaggagactgcccaggacttgaggtccttggtccctctatagaagtatcaagtgtttgtaaaaggtttagcacccatgtgacagaaagaagccatcatcctcttaatttctcttggttttacttaatatatagaagggcaaactagtgggcctctgagtgcaagatgaggacttcattagaataaagacatattgcctcctggatttctaacccatagctccaagagcctcagtgtcagaacataggtaagggacttgatttactgagagaccctaccctacaacatcctgtggacattagagctctgtgctcctgtcactgagtatcactgtgagcttaaaatatgtcagctgctccatttctctttccttttgtgtattcagagctctgattttaaaacactgaaatctggaagattccagtagctgcactctgtctaaagcatatgaggaatgactgtagaatttgcatgtcctctatagcttttgttcacatgtatgcaggcagggataatgttattgattgttcaacctatttaccttgaccaggggttgttagtaatgcccaatatgaatcaagttggcacaagtgtgatcagatgatcaggtcttgtctctttacactgcaccaccaatgcttcagcactgcctccctttgccttaaggactgggagtgcgatgctgtgaatgggatggaaggggttattcacatgtgctttcattacttcttcccttcctcagaagggaaggcaaagacatctataaaacctttacagctgtgcagacttctgtatccctccatcctcatttccaccctttgtaaagtcataaggatgctctccatttccctcttcccttctacttgttccctccccatatcccctaaaatcatgcagacaataaaggctggtattttgggtgccctggagaacgagggctacttcctagtcttctcttggtgtctccttgtgaaaaaagcatttcttcctcaggtggacaagctggtatttcctttggaatgaaatcctcatcctcttcctaggtcttcttcatttcccattccccactcttgggcttgctgctcacggagagccccagggctggccctcctgccagggactgctgcaagcgctccttcacagccaccagcttcagctccaggtcaatccggcgctcctcctttgcccgacactgagcttccagggtggccacggcttcttccagagcctttaattttgctcctgggctgctccgaatggcttccttcagttccctcttctcctgtctcagtgctatcagctctgtccgaatcgtctctttctctttctccagcttctctttttctaccaagtacctccgggcatcctcctcggctcggttcttgccatacttgtattgattggcactggaggcgtggcgtttgactttgacctgcgggtccacacgatgggacttctcactgcaggaggaggcgtgacgcttcacctgggcccctgtggggcgctcgggctcctcgtcctgcatcttttcataaggaacatcatcatagactcggggctcaggccactgattctggcaggatcttgcatataggaaggagttgcgcccagcactgacgatgctggttaaggtctccacatccacgtagtcatagtgcagcgcctccggagtgactctggagcccatctccaccagcagcagcccgagccagcgacccatgtcctctgaacagcttgcctccaagatggccacctcctgccggttgcgcaggatcctgaaggcaaatgggtgtcggggcccaaagcccggggccacctcacagccttgcagggcgatggcgttcacatgggttcgcaggtccatgtgatccttgtggaaatacagagtgttgcacttcaggcggcaccagcgttccttccagccctggttcaccagcacgttcaggtagccacagcagggaacctcctcctcggtggaggacgtctgcaggtcatcggccagtgtcttcttcttggagaagccaatgatacgggtgatcttgcggcccgcagccctgctcattgagcccttcagttctgccaggctgctcttcttccctttgccgtgatcacaggtctcccggcggccaagggtagaacagttgtcacccacacccacgctgtcagaatctgaggtctgcttctcttgggacagcctcttgtccaggtccaacttgcacaggaggactggggatctggggacctccactccctcagctcccccaactggcttgctcacttctcggatgaccttcagccactcctcggcctgctctcggctctgcagtgccagcaccaagacctcggtagccccctgggtgaaacgcagctcgtgcctcttgtgccggctgtccttgggcacgtagatgatgctgcaggtatccagtgccaacctcagatgtggctgccgatccttggagcttttgtaacacaggagctggtcctccctgatgaccgtcagctgcttggcccactgcccgaaacgctttttccgcagcaggaaggcacatatcctgcattccctcaccaggtgcatggaggcctcctctgagggccactggtgtcggggctgcgggctcttcccttcctcctcctcttcatcgtaggactcataggagctgctcattgcgtcagagtcattataggagctcttaagctcgccgttcaccctggttgcagggtagctgctgtctgcgtcctcatagtagccatccacaatcgagtgtgaggggctgcagccattgtgggagctgatgtactcaggcgacttgccgggtcccagaggaagggcctcttcatagtagtcctcagggggaggcttgttggggagcggtggaggcaggtcggccgcgtttctcaggcgtgggctcttggctagctcagggctggctcctttgctgggctccccatcatcctctggcatgtcccgaaggtcactcaggtcacagtcaaattcttcaaagagggattccacgaagctgggccccgagtggaggtctgctgtgttcacatacaggtaggagacctcctttgctggaaggggctgcaggctctgcaggatggaggccacggccatcttcttttccagggtggtatcgctgaggtactcgtggtccaggaggctgagcagcccggtgagctctgggagcagctgctccagcacctggcctcggtccatggcgccggcccggtccccggggagcgggccgcagggcgcaggggctccggcgcggctggtagcggccggcgcgctgcgctctcaggccagcccagcggccggcgctctct

SEQ ID NO: 13649 - RNA, 4631 nt, Homo sapiens
  source 1..4631: mol_type = other RNA
gctgggattacaggcatgagccaccatacctggcctaaacaaggcattttaacaaccaagaacaagtggcatctgtgccttagccattttgcttacatttctcctagctgcctaacgttcaccaggttgctgcttgcatccatgcattcattcgtctatttattaagtgctagtgtgcttctgaatgttgcagtacaaggggagggagatatatggatgacatagagctttaaaattaagaataaggctctagggtcagacttcttatattcacatgctggctccaccagcatgtaaatataagaactatgggagcttggacaagttacctgacctctgtgagcttccatttcctgaactgtgaaaactagggcaatataacttatctcagggtttcagtgaaaactaaagggataatacctagaaaagtggttagttagcaccaggactggctatctaatttaaagggcaaaaggaaaagcagaactccttgttcaaatatgattaagaaggcaatagtagagcattaaaccaagaacagggcccttctaagcatggggccctgtgtgactgcacaggttgcatgcctgtgaagctggccatggctgacacagtgcctgacatatggtgagtgcttgataaatgttaattattaattacccccagccactcctctgagagttcatctgttggtgagaaaagacacttaaccccaaaataactgcataagaaagagtatgacagacactgaagacatagttggagagttaggtgacatttcaggatccacgttttaaaaaagaacactgaaaagtaatttcctcttcagtggaaagaacacaggcttgtgagtcagacatttctgatatagctaataatagccactttttttttttaatagatggggtcttgctatttgcttaggctggagtgcagtggcaattcacaggcgtgatcatagtgcactacagtctcaaactcctgggctcaagcggtcctcctgcctcagcctcctgagtagctgggactacaggcgagtaccaccatgcctggctaatgagagccactattgactgagcatttcttatttctcagacactatgcaagatgcctactatatattatcttattaaatcttcccaacaatcttgggagaaaagtaacaattgttagtcccatttcacagataaggaaaacaagaatcagagcaatcaagtgactttcccaaggtcacccagctggtcattagaggcatggctcaaacctagccctatctggatctgggcttataacccctaagtcctacgctctgccactaatcagtgggtgattactggtcaggttatttttcctgctgtggtctccagctacctcagagggtgataaagtttgagtgaggctaaagtctgtaaaaccttaggtgggttaaaatatgtaacccctatagcaaagtggccacggttattctgggattttccttctttcctcttgagctaagcactggcacttaagagttaagtggttttatctttattggaaggaaatgtgttaaagacagactcactacagtgttgagacagtagtgagtagcacagtaaggagactgcccaggacttgaggtccttggtccctctatagaagtatcaagtgtttgtaaaaggtttagcacccatgtgacagaaagaagccatcatcctcttaatttctcttggttttacttaatatatagaagggcaaactagtgggcctctgagtgcaagatgaggacttcattagaataaagacatattgcctcctggatttctaacccatagctccaagagcctcagtgtcagaacataggtaagggacttgatttactgagagaccctaccctacaacatcctgtggacattagagctctgtgctcctgtcactgagtatcactgtgagcttaaaatatgtcagctgctccatttctctttccttttgtgtattcagagctctgattttaaaacactgaaatctggaagattccagtagctgcactctgtctaaagcatatgaggaatgactgtagaatttgcatgtcctctatagcttttgttcacatgtatgcaggcagggataatgttattgattgttcaacctatttaccttgaccaggggttgttagtaatgcccaatatgaatcaagttggcacaagtgtgatcagatgatcaggtcttgtctctttacactgcaccaccaatgcttcagcactgcctccctttgccttaaggactgggagtgcgatgctgtgaatgggatggaaggggttattcacatgtgctttcattacttcttcccttcctcagaagggaaggcaaagacatctataaaacctttacagctgtgcagacttctgtatccctccatcctcatttccaccctttgtaaagtcataaggatgctctccatttccctcttcccttctacttgttccctccccatatcccctaaaatcatgcagacaataaaggctggtattttgggtgccctggagaacgagggctacttcctagtcttctcttggtgtctccttgtgaaaaaagcatttcttcctcaggtggacaagctggtatttcctttggaatgaaatcctcatcctcttcctaggtcttcttcatttcccattccttggctttctgtagcacccttccttggttggaggctacgatggatgggctcctcttcctcagctcagaaacacagttgacagggagaggttgctctggaacgctgttctggggtttatttgcagtttccccactcttgggcttgctgctcacggagagccccagggctggccctcctgccagggactgctgcaagcgctccttcacagccaccagcttcagctccaggtcaatccggcgctcctcctttgcccgacactgagcttccagggtggccacggcttcttccagagcctttaattttgctcctgggctgctccgaatggcttccttcagttccctcttctcctgtctcagtgctatcagctctgtccgaatcgtctctttctctttctccagcttctctttttctaccaagtacctccgggcatcctcctcggctcggttcttgccatacttgtattgattggcactggaggcgtggcgtttgactttgacctgcgggtccacacgatgggacttctcactgcaggaggaggcgtgacgcttcacctgggcccctgtggggcgctcgggctcctcgtcctgcatcttttcataaggaacatcatcatagactcggggctcaggccactgattctggcaggatcttgcatataggaaggagttgcgcccagcactgacgatgctggttaaggtctccacatccacgtagtcatagtgcagcgcctccggagtgactctggagcccatctccaccagcagcagcccgagccagcgacccatgtcctctgaacagcttgcctccaagatggccacctcctgccggttgcgcaggatcctgaaggcaaatgggtgtcggggcccaaagcccggggccacctcacagccttgcagggcgatggcgttcacatgggttcgcaggtccatgtgatccttgtggaaatacagagtgttgcacttcaggcggcaccagcgttccttccagccctggttcaccagcacgttcaggtagccacagcagggaacctcctcctcggtggaggacgtctgcaggtcatcggccagtgtcttcttcttggagaagccaatgatacgggtgatcttgcggcccgcagccctgctcattgagcccttcagttctgccaggctgctcttcttccctttgccgtgatcacaggtctcccggcggccaagggtagaacagttgtcacccacacccacgctgtcagaatctgaggtctgcttctcttgggacagcctcttgtccaggtccaacttgcacaggaggactggggatctggggacctccactccctcagctcccccaactggcttgctcacttctcggatgaccttcagccactcctcggcctgctctcggctctgcagtgccagcaccaagacctcggtagccccctgggtgaaacgcagctcgtgcctcttgtgccggctgtccttgggcacgtagatgatgctgcaggtatccagtgccaacctcagatgtggctgccgatccttggagcttttgtaacacaggagctggtcctccctgatgaccgtcagctgcttggcccactgcccgaaacgctttttccgcagcaggaaggcacatatcctgcattccctcaccaggtgcatggaggcctcctctgagggccactggtgtcggggctgcgggctcttcccttcctcctcctcttcatcgtaggactcataggagctgctcattgcgtcagagtcattataggagctcttaagctcgccgttcaccctggttgcagggtagctgctgtctgcgtcctcatagtagccatccacaatcgagtgtgaggggctgcagccatctgatccaagcaccatagccaaaaggtgcaatcagcccaaggtccatcagctgaggaatggataagcacaatgtggtctatccgtatggtgggatagtgttcagccatagaaaggaaagaagttct

SEQ ID NO: 13650 - RNA, 5051 nt, Homo sapiens
  source 1..5051: mol_type = other RNA
gctgggattacaggcatgagccaccatacctggcctaaacaaggcattttaacaaccaagaacaagtggcatctgtgccttagccattttgcttacatttctcctagctgcctaacgttcaccaggttgctgcttgcatccatgcattcattcgtctatttattaagtgctagtgtgcttctgaatgttgcagtacaaggggagggagatatatggatgacatagagctttaaaattaagaataaggctctagggtcagacttcttatattcacatgctggctccaccagcatgtaaatataagaactatgggagcttggacaagttacctgacctctgtgagcttccatttcctgaactgtgaaaactagggcaatataacttatctcagggtttcagtgaaaactaaagggataatacctagaaaagtggttagttagcaccaggactggctatctaatttaaagggcaaaaggaaaagcagaactccttgttcaaatatgattaagaaggcaatagtagagcattaaaccaagaacagggcccttctaagcatggggccctgtgtgactgcacaggttgcatgcctgtgaagctggccatggctgacacagtgcctgacatatggtgagtgcttgataaatgttaattattaattacccccagccactcctctgagagttcatctgttggtgagaaaagacacttaaccccaaaataactgcataagaaagagtatgacagacactgaagacatagttggagagttaggtgacatttcaggatccacgttttaaaaaagaacactgaaaagtaatttcctcttcagtggaaagaacacaggcttgtgagtcagacatttctgatatagctaataatagccactttttttttttaatagatggggtcttgctatttgcttaggctggagtgcagtggcaattcacaggcgtgatcatagtgcactacagtctcaaactcctgggctcaagcggtcctcctgcctcagcctcctgagtagctgggactacaggcgagtaccaccatgcctggctaatgagagccactattgactgagcatttcttatttctcagacactatgcaagatgcctactatatattatcttattaaatcttcccaacaatcttgggagaaaagtaacaattgttagtcccatttcacagataaggaaaacaagaatcagagcaatcaagtgactttcccaaggtcacccagctggtcattagaggcatggctcaaacctagccctatctggatctgggcttataacccctaagtcctacgctctgccactaatcagtgggtgattactggtcaggttatttttcctgctgtggtctccagctacctcagagggtgataaagtttgagtgaggctaaagtctgtaaaaccttaggtgggttaaaatatgtaacccctatagcaaagtggccacggttattctgggattttccttctttcctcttgagctaagcactggcacttaagagttaagtggttttatctttattggaaggaaatgtgttaaagacagactcactacagtgttgagacagtagtgagtagcacagtaaggagactgcccaggacttgaggtccttggtccctctatagaagtatcaagtgtttgtaaaaggtttagcacccatgtgacagaaagaagccatcatcctcttaatttctcttggttttacttaatatatagaagggcaaactagtgggcctctgagtgcaagatgaggacttcattagaataaagacatattgcctcctggatttctaacccatagctccaagagcctcagtgtcagaacataggtaagggacttgatttactgagagaccctaccctacaacatcctgtggacattagagctctgtgctcctgtcactgagtatcactgtgagcttaaaatatgtcagctgctccatttctctttccttttgtgtattcagagctctgattttaaaacactgaaatctggaagattccagtagctgcactctgtctaaagcatatgaggaatgactgtagaatttgcatgtcctctatagcttttgttcacatgtatgcaggcagggataatgttattgattgttcaacctatttaccttgaccaggggttgttagtaatgcccaatatgaatcaagttggcacaagtgtgatcagatgatcaggtcttgtctctttacactgcaccaccaatgcttcagcactgcctccctttgccttaaggactgggagtgcgatgctgtgaatgggatggaaggggttattcacatgtgctttcattacttcttcccttcctcagaagggaaggcaaagacatctataaaacctttacagctgtgcagacttctgtatccctccatcctcatttccaccctttgtaaagtcataaggatgctctccatttccctcttcccttctacttgttccctccccatatcccctaaaatcatgcagacaataaaggctggtattttgggtgccctggagaacgagggctacttcctagtcttctcttggtgtctccttgtgaaaaaagcatttcttcctcaggtggacaagctggtatttcctttggaatgaaatcctcatcctcttcctaggtcttcttcatttcccattccttggctttctgtagcacccttccttggttggaggctacgatggatgggctcctcttcctcagctcagaaacacagttgacagggagaggttgctctggaacgctgttctggggtttatttgcagtttccccactcttgggcttgctgctcacggagagccccagggctggccctcctgccagggactgctgcaagcgctccttcacagccaccagcttcagctccaggtcaatccggcgctcctcctttgcccgacactgagcttccagggtggccacggcttcttccagagcctttaattttgctcctgggctgctccgaatggcttccttcagttccctcttctcctgtctcagtgctatcagctctgtccgaatcgtctctttctctttctccagcttctctttttctaccaagtacctccgggcatcctcctcggctcggttcttgccatacttgtattgattggcactggaggcgtggcgtttgactttgacctgcgggtccacacgatgggacttctcactgcaggaggaggcgtgacgcttcacctgggcccctgtggggcgctcgggctcctcgtcctgcatcttttcataaggaacatcatcatagactcggggctcaggccactgattctggcaggatcttgcatataggaaggagttgcgcccagcactgacgatgctggttaaggtctccacatccacgtagtcatagtgcagcgcctccggagtgactctggagcccatctccaccagcagcagcccgagccagcgacccatgtcctctgaacagcttgcctccaagatggccacctcctgccggttgcgcaggatcctgaaggcaaatgggtgtcggggcccaaagcccggggccacctcacagccttgcagggcgatggcgttcacatgggttcgcaggtccatgtgatccttgtggaaatacagagtgttgcacttcaggcggcaccagcgttccttccagccctggttcaccagcacgttcaggtagccacagcagggaacctcctcctcggtggaggacgtctgcaggtcatcggccagtgtcttcttcttggagaagccaatgatacgggtgatcttgcggcccgcagccctgctcattgagcccttcagttctgccaggctgctcttcttccctttgccgtgatcacaggtctcccggcggccaagggtagaacagttgtcacccacacccacgctgtcagaatctgaggtctgcttctcttgggacagcctcttgtccaggtccaacttgcacaggaggactggggatctggggacctccactccctcagctcccccaactggcttgctcacttctcggatgaccttcagccactcctcggcctgctctcggctctgcagtgccagcaccaagacctcggtagccccctgggtgaaacgcagctcgtgcctcttgtgccggctgtccttgggcacgtagatgatgctgcaggtatccagtgccaacctcagatgtggctgccgatccttggagcttttgtaacacaggagctggtcctccctgatgaccgtcagctgcttggcccactgcccgaaacgctttttccgcagcaggaaggcacatatcctgcattccctcaccaggtgcatggaggcctcctctgagggccactggtgtcggggctgcgggctcttcccttcctcctcctcttcatcgtaggactcataggagctgctcattgcgtcagagtcattataggagctcttaagctcgccgttcaccctggttgcagggtagctgctgtctgcgtcctcatagtagccatccacaatcgagtgtgaggggctgcagccattgtgggagctgatgtactcaggcgacttgccgggtcccagaggaagggcctcttcatagtagtcctcagggggaggcttgttggggagcggtggaggcaggtcggccgcgtttctcaggcgtgggctcttggctagctcagggctggctcctttgctgggctccccatcatcctctggcatgtcccgaaggtcactcaggtcacagtcaaattcttcaaagagggattccacgaagctgggccccgagtggaggtctgctgtgttcacatacaggtaggagacctcctttgctggaaggggctgcaggctctgcaggatggaggccacggccatcttcttttccagggtggtatcgctgaggtactcgtggtccaggaggctgagcagcccggtgagctctgggagcagctgctccagcacctggcctcggtccatggcgccggcccggtccccggggagcgggccgcagggcgcaggggctccggcgcggctggtagcggccggcgcgctgcgctctcaggccagcccagcggccggcgctctct

SEQ ID NO: 13651 - RNA, 5049 nt, Homo sapiens
  source 1..5049: mol_type = other RNA
gctgggattacaggcatgagccaccatacctggcctaaacaaggcattttaacaaccaagaacaagtggcatctgtgccttagccattttgcttacatttctcctagctgcctaacgttcaccaggttgctgcttgcatccatgcattcattcgtctatttattaagtgctagtgtgcttctgaatgttgcagtacaaggggagggagatatatggatgacatagagctttaaaattaagaataaggctctagggtcagacttcttatattcacatgctggctccaccagcatgtaaatataagaactatgggagcttggacaagttacctgacctctgtgagcttccatttcctgaactgtgaaaactagggcaatataacttatctcagggtttcagtgaaaactaaagggataatacctagaaaagtggttagttagcaccaggactggctatctaatttaaagggcaaaaggaaaagcagaactccttgttcaaatatgattaagaaggcaatagtagagcattaaaccaagaacagggcccttctaagcatggggccctgtgtgactgcacaggttgcatgcctgtgaagctggccatggctgacacagtgcctgacatatggtgagtgcttgataaatgttaattattaattacccccagccactcctctgagagttcatctgttggtgagaaaagacacttaaccccaaaataactgcataagaaagagtatgacagacactgaagacatagttggagagttaggtgacatttcaggatccacgttttaaaaaagaacactgaaaagtaatttcctcttcagtggaaagaacacaggcttgtgagtcagacatttctgatatagctaataatagccactttttttttttaatagatggggtcttgctatttgcttaggctggagtgcagtggcaattcacaggcgtgatcatagtgcactacagtctcaaactcctgggctcaagcggtcctcctgcctcagcctcctgagtagctgggactacaggcgagtaccaccatgcctggctaatgagagccactattgactgagcatttcttatttctcagacactatgcaagatgcctactatatattatcttattaaatcttcccaacaatcttgggagaaaagtaacaattgttagtcccatttcacagataaggaaaacaagaatcagagcaatcaagtgactttcccaaggtcacccagctggtcattagaggcatggctcaaacctagccctatctggatctgggcttataacccctaagtcctacgctctgccactaatcagtgggtgattactggtcaggttatttttcctgctgtggtctccagctacctcagagggtgataaagtttgagtgaggctaaagtctgtaaaaccttaggtgggttaaaatatgtaacccctatagcaaagtggccacggttattctgggattttccttctttcctcttgagctaagcactggcacttaagagttaagtggttttatctttattggaaggaaatgtgttaaagacagactcactacagtgttgagacagtagtgagtagcacagtaaggagactgcccaggacttgaggtccttggtccctctatagaagtatcaagtgtttgtaaaaggtttagcacccatgtgacagaaagaagccatcatcctcttaatttctcttggttttacttaatatatagaagggcaaactagtgggcctctgagtgcaagatgaggacttcattagaataaagacatattgcctcctggatttctaacccatagctccaagagcctcagtgtcagaacataggtaagggacttgatttactgagagaccctaccctacaacatcctgtggacattagagctctgtgctcctgtcactgagtatcactgtgagcttaaaatatgtcagctgctccatttctctttccttttgtgtattcagagctctgattttaaaacactgaaatctggaagattccagtagctgcactctgtctaaagcatatgaggaatgactgtagaatttgcatgtcctctatagcttttgttcacatgtatgcaggcagggataatgttattgattgttcaacctatttaccttgaccaggggttgttagtaatgcccaatatgaatcaagttggcacaagtgtgatcagatgatcaggtcttgtctctttacactgcaccaccaatgcttcagcactgcctccctttgccttaaggactgggagtgcgatgctgtgaatgggatggaaggggttattcacatgtgctttcattacttcttcccttcctcagaagggaaggcaaagacatctataaaacctttacagctgtgcagacttctgtatccctccatcctcatttccaccctttgtaaagtcataaggatgctctccatttccctcttcccttctacttgttccctccccatatcccctaaaatcatgcagacaataaaggctggtattttgggtgccctggagaacgagggctacttcctagtcttctcttggtgtctccttgtgaaaaaagcatttcttcctcaggtggacaagctggtatttcctttggaatgaaatcctcatcctcttcctaggtcttcttcatttcccattccttggctttctgtagcacccttccttggttggaggctacgatggatgggctcctcttcctcagctcagaaacacagttgacagggagaggttgctctggaacgctgttctggggtttatttgcagtttccccactcttgggcttgctgctcacggagagccccagggctggccctcctgccagggactgctgcaagcgctccttcacagccaccagcttcagctccaggtcaatccggcgctcctcctttgcccgacactgagcttccagggtggccacggcttcttccagagcctttaattttgctcctgggctgctccgaatggcttccttcagttccctcttctcctgtctcagtgctatcagctctgtccgaatcgtctctttctctttctccagcttctctttttctaccaagtacctccgggcatcctcctcggctcggttcttgccatacttgtattgattggcactggaggcgtggcgtttgactttgacctgcgggtccacacgatgggacttctcactgcaggaggaggcgtgacgcttcacctgggcccctgtggggcgctcgggctcctcgtcctgcatcttttcataaggaacatcatcatagactcggggctcaggccactgattctggcaggatcttgcatataggaaggagttgcgcccagcactgacgatgctggttaaggtctccacatccacgtagtcatagtgcagcgcctccggagtgactctggagcccatctccaccagcagcagcccgagccagcgacccatgtcctctgaacagcttgcctccaagatggccacctcctgccggttgcgcaggatcctgaaggcaaatgggtgtcggggcccaaagcccggggccacctcacagccttgcagggcgatggcgttcacatgggttcgcaggtccatgtgatccttgtggaaatacagagtgttgcacttcaggcggcaccagcgttccttccagccctggttcaccagcacgttcaggtagccacagcagggaacctcctcctcggtggaggacgtctgcaggtcatcggccagtgtcttcttcttggagaagccaatgatacgggtgatcttgcggcccgcagccctgctcattgagcccttcagttctgccaggctgctcttcttccctttgccgtgatcacaggtctcccggcggccaagggtagaacagttgtcacccacacccacgctgtcagaatctgaggtctgcttctcttgggacagcctcttgtccaggtccaacttgcacaggaggactggggatctggggacctccactccctcagctcccccaactggcttgctcacttctcggatgaccttcagccactcctcggcctgctctcggctctgcagtgccagcaccaagacctcggtagccccctgggtgaaacgcagctcgtgcctcttgtgccggctgtccttgggcacgtagatgatgctgcaggtatccagtgccaacctcagatgtggctgccgatccttggagcttttgtaacacaggagctggtcctccctgatgaccgtcagctgcttggcccactgcccgaaacgctttttccgcagcaggaaggcacatatcctgcattccctcaccaggtgcatggaggcctcctctgagggccactggtgtcggggctgcgggctcttcccttcctcctcctcttcatcgtaggactcataggagctgctcattgcgtcagagtcattataggagctcttaagctcgccgttcaccctggttgcagggtagctgctgtctgcgtcctcatagtagccatccacaatcgagtgtgaggggctgcagccattgtgggagctgatgtactcaggcgacttgccgggtcccagaggaagggcctcttcatagtagtcctcagggggaggcttgttggggagcggtggaggcaggtcggccgcgtttctcaggcgtgggctcttggctagctcagggctggctcctttgctgggctccccatcatcctctggcatgtcccgaaggtcactcaggtcacagtcaaattcttcaaagagggattccacgaagctgggccccgagtggaggtctgctgtgttcacatacaggtaggagacctcctttgctggaaggggctgcaggctctgcaggatggaggccacggccatcttcttttccagggtggtatcgctgaggtactcgtggtccaggaggctgagcagcccggtgagctctgggagcagctgctccagcactggggatcttgtcaaaatgcaaattctgattcaggaggtgtgcggtgggatccgagattctgcatttctgatccgcaccaagctgcagctgatgctggtggtcctggaccatctgagttgcaa

SEQ ID NO: 13652 - RNA, 4952 nt, Homo sapiens
  source 1..4952: mol_type = other RNA
gctgggattacaggcatgagccaccatacctggcctaaacaaggcattttaacaaccaagaacaagtggcatctgtgccttagccattttgcttacatttctcctagctgcctaacgttcaccaggttgctgcttgcatccatgcattcattcgtctatttattaagtgctagtgtgcttctgaatgttgcagtacaaggggagggagatatatggatgacatagagctttaaaattaagaataaggctctagggtcagacttcttatattcacatgctggctccaccagcatgtaaatataagaactatgggagcttggacaagttacctgacctctgtgagcttccatttcctgaactgtgaaaactagggcaatataacttatctcagggtttcagtgaaaactaaagggataatacctagaaaagtggttagttagcaccaggactggctatctaatttaaagggcaaaaggaaaagcagaactccttgttcaaatatgattaagaaggcaatagtagagcattaaaccaagaacagggcccttctaagcatggggccctgtgtgactgcacaggttgcatgcctgtgaagctggccatggctgacacagtgcctgacatatggtgagtgcttgataaatgttaattattaattacccccagccactcctctgagagttcatctgttggtgagaaaagacacttaaccccaaaataactgcataagaaagagtatgacagacactgaagacatagttggagagttaggtgacatttcaggatccacgttttaaaaaagaacactgaaaagtaatttcctcttcagtggaaagaacacaggcttgtgagtcagacatttctgatatagctaataatagccactttttttttttaatagatggggtcttgctatttgcttaggctggagtgcagtggcaattcacaggcgtgatcatagtgcactacagtctcaaactcctgggctcaagcggtcctcctgcctcagcctcctgagtagctgggactacaggcgagtaccaccatgcctggctaatgagagccactattgactgagcatttcttatttctcagacactatgcaagatgcctactatatattatcttattaaatcttcccaacaatcttgggagaaaagtaacaattgttagtcccatttcacagataaggaaaacaagaatcagagcaatcaagtgactttcccaaggtcacccagctggtcattagaggcatggctcaaacctagccctatctggatctgggcttataacccctaagtcctacgctctgccactaatcagtgggtgattactggtcaggttatttttcctgctgtggtctccagctacctcagagggtgataaagtttgagtgaggctaaagtctgtaaaaccttaggtgggttaaaatatgtaacccctatagcaaagtggccacggttattctgggattttccttctttcctcttgagctaagcactggcacttaagagttaagtggttttatctttattggaaggaaatgtgttaaagacagactcactacagtgttgagacagtagtgagtagcacagtaaggagactgcccaggacttgaggtccttggtccctctatagaagtatcaagtgtttgtaaaaggtttagcacccatgtgacagaaagaagccatcatcctcttaatttctcttggttttacttaatatatagaagggcaaactagtgggcctctgagtgcaagatgaggacttcattagaataaagacatattgcctcctggatttctaacccatagctccaagagcctcagtgtcagaacataggtaagggacttgatttactgagagaccctaccctacaacatcctgtggacattagagctctgtgctcctgtcactgagtatcactgtgagcttaaaatatgtcagctgctccatttctctttccttttgtgtattcagagctctgattttaaaacactgaaatctggaagattccagtagctgcactctgtctaaagcatatgaggaatgactgtagaatttgcatgtcctctatagcttttgttcacatgtatgcaggcagggataatgttattgattgttcaacctatttaccttgaccaggggttgttagtaatgcccaatatgaatcaagttggcacaagtgtgatcagatgatcaggtcttgtctctttacactgcaccaccaatgcttcagcactgcctccctttgccttaaggactgggagtgcgatgctgtgaatgggatggaaggggttattcacatgtgctttcattacttcttcccttcctcagaagggaaggcaaagacatctataaaacctttacagctgtgcagacttctgtatccctccatcctcatttccaccctttgtaaagtcataaggatgctctccatttccctcttcccttctacttgttccctccccatatcccctaaaatcatgcagacaataaaggctggtattttgggtgccctggagaacgagggctacttcctagtcttctcttggtgtctccttgtgaaaaaagcatttcttcctcaggtggacaagctggtatttcctttggaatgaaatcctcatcctcttcctaggtcttcttcatttcccattccttggctttctgtagcacccttccttggttggaggctacgatggatgggctcctcttcctcagctcagaaacacagttgacagggagaggttgctctggaacgctgttctggggtttatttgcagtttccccactcttgggcttgctgctcacggagagccccagggctggccctcctgccagggactgctgcaagcgctccttcacagccaccagcttcagctccaggtcaatccggcgctcctcctttgcccgacactgagcttccagggtggccacggcttcttccagagcctttaattttgctcctgggctgctccgaatggcttccttcagttccctcttctcctgtctcagtgctatcagctctgtccgaatcgtctctttctctttctccagcttctctttttctaccaagtacctccgggcatcctcctcggctcggttcttgccatacttgtattgattggcactggaggcgtggcgtttgactttgacctgcgggtccacacgatgggacttctcactgcaggaggaggcgtgacgcttcacctgggcccctgtggggcgctcgggctcctcgtcctgcatcttttcataaggaacatcatcatagactcggggctcaggccactgattctggcaggatcttgcatataggaaggagttgcgcccagcactgacgatgctggttaaggtctccacatccacgtagtcatagtgcagcgcctccggagtgactctggagcccatctccaccagcagcagcccgagccagcgacccatgtcctctgaacagcttgcctccaagatggccacctcctgccggttgcgcaggatcctgaaggcaaatgggtgtcggggcccaaagcccggggccacctcacagccttgcagggcgatggcgttcacatgggttcgcaggtccatgtgatccttgtggaaatacagagtgttgcacttcaggcggcaccagcgttccttccagccctggttcaccagcacgttcaggtagccacagcagggaacctcctcctcggtggaggacgtctgcaggtcatcggccagtgtcttcttcttggagaagccaatgatacgggtgatcttgcggcccgcagccctgctcattgagcccttcagttctgccaggctgctcttcttccctttgccgtgatcacaggtctcccggcggccaagggtagaacagttgtcacccacacccacgctgtcagaatctgaggtctgcttctcttgggacagcctcttgtccaggtccaacttgcacaggaggactggggatctggggacctccactccctcagctcccccaactggcttgctcacttctcggatgaccttcagccactcctcggcctgctctcggctctgcagtgccagcaccaagacctcggtagccccctgggtgaaacgcagctcgtgcctcttgtgccggctgtccttgggcacgtagatgatgctgcaggtatccagtgccaacctcagatgtggctgccgatccttggagcttttgtaacacaggagctggtcctccctgatgaccgtcagctgcttggcccactgcccgaaacgctttttccgcagcaggaaggcacatatcctgcattccctcaccaggtgcatggaggcctcctctgagggccactggtgtcggggctgcgggctcttcccttcctcctcctcttcatcgtaggactcataggagctgctcattgcgtcagagtcattattgtgggagctgatgtactcaggcgacttgccgggtcccagaggaagggcctcttcatagtagtcctcagggggaggcttgttggggagcggtggaggcaggtcggccgcgtttctcaggcgtgggctcttggctagctcagggctggctcctttgctgggctccccatcatcctctggcatgtcccgaaggtcactcaggtcacagtcaaattcttcaaagagggattccacgaagctgggccccgagtggaggtctgctgtgttcacatacaggtaggagacctcctttgctggaaggggctgcaggctctgcaggatggaggccacggccatcttcttttccagggtggtatcgctgaggtactcgtggtccaggaggctgagcagcccggtgagctctgggagcagctgctccagcacctggcctcggtccatggcgccggcccggtccccggggagcgggccgcagggcgcaggggctccggcgcggctggtagcggccggcgcgctgcgctctcaggccagcccagcggccggcgctctct

SEQ ID NO: 13653 - RNA, 684 nt, Homo sapiens
  source 1..684: mol_type = other RNA
gctgggattacaggcatgagccaccatatccggctaattttgtagtttttttcttttttttagtagagacgggatttcttcatgttggtcaggctggtctccgacctcgggtgatccgcccacctctgccttccaaagtgctgggattgcaggcctgagccactgcgcccgacggaaacccagaacggaaaacaaaagaaaaaccacaaagattagccggctgtggtgggccgcgcaggtagtcccagctactctgaaggctgatggaggaggattgcttcaccccggcttctaggtggcagtgagctatgatggcgctgctgcactccagactgggcgacagagcgggactagtttgaatgtcttctttcttcactagccgatgcatctgtgccagtaacacacggtgattctgtcctttcaccttcagttatgcctgggactgtcccctgacaggcagtgcgacgaggtcaggcccgcgcccgccgagtcctagggccgctgccgccgacggccatggaggacgagcagctcgacagcctggagggctgggcgccggtccggcaaggcctcttcgccgatgccgagaggcaccggctgcgcttcctggtggcgtggaatggcgcggagggcaagttagctgtgacttgtcacgacctcaccgcgcagcagccgcagcggcgc

SEQ ID NO: 13654 - RNA, 2487 nt, Homo sapiens
  source 1..2487: mol_type = other RNA
gctgggattacaggcatgagccaccatgaccagcctgaaaaagattttttgattggccaagaacttttaaatttaaaaactaaattcctgaaagtctgaattatattagctatggagtaaaatgagaaaatagaggactttcatttttactttatttctatactttaaaaagtgcttaaaagcgtgtattatttttataataaatacatttgatacaaggtttcaaatgttacttttctaacaaaattgcaatttaaggctttggggtttttttgtttgttttgttttttgtttttgagacagcgtctcactctgtcacccaggctagagtgcagtggtgcaatctcagctcactgcaacctccacctcctgggttcaagcgattctcccacctcagcctccggaatagttgggattacaggtgtgtgccaccacgcccggctatttaggctttgtattttaaatgagactatgaaaagcagtaaatattcatattacagagcacaggttttcaaaatgttctacttcatgctttaaaaataaaatgggccaggcacggtggctcacgcctgtaatcccaacactttgggaggccgaggcaggcggatcacgaggtcaagagatcgacaccatccttgccaacatggtgaaaccccttctctactaaaaatacaaaaattagctgggtgtggtgatgtgcgcctgtaagtctcagctactcgggaagctgaggcaggagaatcacttgaacccaggaggccgaggttgcagtgagccaagatcgcgccactgcaccccagcctggcgacagcgagactctgtctcataaaataaaaatacaataaaaaaaatcaataagtggtaagacaactccaggaccaaggaggaagagatgtccctttattgtattttgtgttatatgattttaggattcaaaaacctactttaagttacctaatgttccacaatatagcaggtatatttcttttaacctatttaagccatcagacagaataaacttatttggccagtacttaatgaaagacttctctaatactgagggaagtaggtttatgactaaatgaataaagccccatttgggagatgaaaacaaagcagcacctcagttttccctagagtctgtgtatagtaagaatgggtgaaagcggcataaagaaagtgtcattaagtcacatatagttatcatttaaatgtcatttggctgggcgtggtggctcacgcctgtaatcccaacactttgggaggccaagatgggcggatcacgaggtcaggggattgagaccatcctggctgacacagtgaaacaccgtctctactaaaaatacaaaaaattgcctggcgcggtggcgggcgcctgttgtcccagctactcgggaggctgaggcaggagaatggcgtgaacccgggaggcggagcttgcagtgagcagagatcgtgccacttcactccagcctgggcgacagagcgagactccgtctcaaaaaaaaaaaatgtcatttaaaacatctttaacacccaaaacatttatcttcaaagtatctttaaacgtccaatactacatgagctgctgtgagacagattttaaaaagtgatgaatcagctacaaagaatagcatgtcatcaatagcaaaataaattggaaatgctatttaagaaacgaaatcattatcaattatggataatataatatgagccaggcatggtggctcacattggtaaccttagcactttgggaggttgaggggggcggatcatttgaggtcaggagttcaaaaccatcctggccaacatggtgaaacccaatctctactaaaaatacaaaaaaattagccgggtctggtggcaagtgcctgtaatctcagctacttggaaggctgaggcgggagaatcgcttgaacctgggaggcagagattgtagtgagccaagatcacaccactgcactccagcctgggcaatagagtgagacttcatctcacacacacacacaaaaaaatcataatatagaatagaaataggtactatgttaaatataatggtggctgctgaactaaaatgatatataaataagagtacaggttttttatagaaaaaaaattgtgccatccattttttaatagaaaaaaagaaaaatacacacaaaaaaagaaaattaagaaacatggatgacattctcttcttcctaccaccccttcctcaccaaaaaataactaaatggatcattcagcttactgtctcttttaaaggctttacataaaacggtagattgattgtgaccttttaaaaatgctttgagacctataaataaataagtaagaataatcctgtctgggtgcagtggctcacgcctgtaatcccagcacgttgggaggccgaggtgggtggatcacctgaggttgggaatttgagaccagcctgaccaacatggtgaaaccctgtctctacttaaaatacaaaaattagtcagg

SEQ ID NO: 13655 - RNA, 6681 nt, Homo sapiens
  source 1..6681: mol_type = other RNA
gctgggattacaggcatgagccaccatgaccagcctgtaaaaagaaaattttttgataaattgagtgtagcctaaatgtatagtgctttaaagtctacattagtgcacagtaatgtcctgggccttcacattcactcaccattcactcattgactcatgcagataaatttccagccccgcagtctccattcatagggtaagtaccctattcaggtgtaccattttaaaaatctgtacaatgtttttactgtaccttttagatgtttagatatatttaggtatacaaatacttaccattgtgttacaattccctatagtattcagtacagttaacatatgtacaggtttgtagcctagaagcaatagatcatgtaacctaggtctgtagtaggctatactatctaggtttgtgtaaatatgtaagtacactctcatgtttgcacagtgatgaaatctcagaatgatacaattctcagaatgtatctccaatgactgtagtaggagattttggtatcctactttcaataaggaatagaacattcagacagaaaatcagcaaggaagcagaggacttgaacaacactatagctgaaatggaactaacagacatatacagaaaattccacccaacagcagcaaatatacagtcttctcaagcacactcagagcattttccaggataaatcacacgtcaggtcacaaaacaagtcttaacaaattcaagaaggttgaaatcctactaaatatcttttctgaccacagtggaataaaactagaaatcaatactggaattaaaactggaaaatctgcaaatatgtagaaattaaacaacagaattttgaacgaaattctgttcaaaatttcatttgaatgaaaggggaaatcaaaagatgaattagaaaatatgttaagataaacaaaaatgaaaacacaacacaataaaaacttacaggatacaacaaaagcagtactaagaaggaatattaagctgggcaagctcagtggctcacgcctgtaatcccagtgctttgggaatccaaggcacaaggatcacttgcagggagctatgatcgtgcctctgtacatcatagtgagatcttgtctcttaaacatgaaaacaaaaacaaagaagggagttgtaaatgcctacactaaaaatgaagaaagaagaaagatctcaaataaaaaacttaacaactcaaggaactagaaaaaaaggacaaatgaggaagcccaaagcaaagggaggaaatactataataaagattagagcaaaaataaatgaaaaaaagtttaaattaagtttttaaacttagttgattttttgaaaaaacaacaaaactgacaagccccttagctagactaagaaaaaaacaaaaagactggaagtcagaaacaaaagaggtggcattacacctgatgccacaattataagaggcttttaaaatcatataccaaaaaattcaataacctagaagaaattgattaattcctagaaacatacaaactaccaagacataatcataaaaaatctaaacaaagctgtaactagtaaggagattgaatcagtaatccaaacctcctaacaacaacaacaacaaaagcccaaaaccagatatctttcctggagaattctaccaaacttttaaagaagaatcaatgataattgttttcaaactcttccaaaaaaaaaaaattgaaggagagggaacacttccaaactcattttaaaagtccaacaaaaaaatggtagtaaaaaataaatcttcaaaagaaactacaatcagagtgaacaggcaacctacagaatgggagaaaatttttgcaatctacccatctgacaaagggctaatatccagaatctacaaagaacctaaacacatttacaagaaaaaaacaaaaaaccctatcaaaaagtgggcaaaggatatgaacagacacttctcaaaagaagacatttatgcagccaacagacacatgaaaaaatgcccatcatcactggtcatcagagaaatgcaaatcaaaaccacaatgagataccatctcacaccagttagaatggcaatcattaaaaagtcaggaaacaacacatgctggagaggatgtggagaaatagtaacgcttttacaccgttggtgggagtgtaaactagttcaaccattgtggaagacagtgtggcgattcctcaaggatctggaactagaaataccatttgacccattactgggtatatatctaaaggattataaatcatgctactataaagacacatgcacatgtatgtttattgcgacactattcacaatagcaaagacttggaaccaacccaaatgtccatcaatgatagaccggattaagaaaatgtgacacatatacaccatggaagactatgcagccgtaaaaaagggtgagttcatgtcctttgtagagacatggatgaagctggaaaccgtcattctgagcaaactatcacaagcacagaaaaccaaacactgcatgttctcactcataggtgggaattgaacaacgagagcacttggacacagggtggggaacatcacacactggggcctgttgaggtgtgggggactgggggagggatagcattaggagaaatacctaatgtaaatgatgagttgatgggtgcagcaaacgaacatggcacacatgtatacctatgtaacaaacctgcacgttgtgcacatgtatcctagaacttaaagtataataaaaataataagaagaaataaaaataaatcttgacccctacctcacaacaatgataaaaatatgtatattccaaatggattgtagatgtaatgtaaacaatgaaataaaagataccacagaaaattatctttgtgaaataggatcagaagcaaaaattgataaattgagtttaatcaaaattatgactttctattcaccaaaagacaaaaaagaattaaaaactagccatgaggttgaaaactactaaaaaaaggagttatgttcagaatacaagatttgtttaagtaataagaaaaacaagataaggaaataaataaagttctatggaagcaaaaagaagagaaaaaagaaaagaaaaacaacagactagagaaataggagatttgagcagctattgcacaaaataaggtataaaaattgccaaaataaaatagaaaggtactcaacttcatttaaatataaaataatttcaaaatgagattacaaaagtcacccagtaaaatggctaacatgaaaataacctgacaaatgtagagatgatgtggcccagcagaaagccttatgcactactaggaatgtaaacaggtaaaaacatcttggaaaattggttggtgttagctacaaaagacaaagatacacacatattctgtgacccacaaacacaactcttaggcaaaaacctgagagaaatctgtgtacatgggcatcaaagaaatgtacaatatatttatgatggcattatttgaaatagacattgaggcacaatgcaaattcctgaacagtagaataaataaggtatagtatatttatgaaatagtactagaaacagaaataaataaactacaactacatataacaacatggataatttcataaacaatgagtgataaatacaaataacacacaaatgcacagacaatacatgttgtgcaagtccaattagataacgttcccaaaacaggccccgaacaaacagttataaaaggcaaatgtgcggttacactggaggaaaaataagggaagtgatttggcaggtgcatgcgaggggcttcagcgatggaggcaacggagcttttcactttcatacaatttatggagctttattatttcagcctgtgcacatttgtttatatgtaataggttaaataatagtaaaatgttttctaaaatgttgattattaccaaaaacaaagagggtgaatatagtgaaaatttactagaaattacagttctgttaatatgcattgaataatgcagcataaaatgaaggaaggcaatatatattgctctgatgtcctataattccaaaagactttagttaaaatggatatgtaaaaagaggtaaaattttaacccagggaaatttgactcttagaaataaatttacgaagaagttgatagagaaaaacaatacgaaaattaaacaaaaggatgttatacactaacctttgcaaaggattcctcagttgtctgcagctgatcttctctgtccctagagtcaggtaaactggggctgaaggccatgaggtcggtcttgggtgggccctcaccagagcacaccctcggcctcctctgctgcgagtatgaccagctccccaccgcactggagcacaccagcgtgggcttgcccggagcgcacgcgccctcggtgggcagcgcagagcaccgcagcgcggtgtacagcagcagcgtgagcaccaaaaggctggacaccgcgcagatggcaatgatcaggtatacgttgacatccaccagcgcagcatcgggacccacagcgcccaccaacgcccgtgaggaggcctttggcgcctgtccactctccacaagtgacaccagcacagtggccgtggccgtcagcgcgggctcgccgtggtccttcaccagtaccagtaggcggtggcgcggagcgtccgtttcgtccagggcacgcgttgtgctgatctcgccagtgtacagccccacgcggaacgggatgcgcgcgccaccagtccccggctgcagctcgtacgaaagccacgcgttgtagcccgagtcagcatccaccgcgcgcacctttgccaccacgtggcccacacccaccgaccatggcaccagctcgctcactgcgccaccagtgccacccgcccgaggcgctagcagtgctggcgcgttgtcgttttcgtccagcacgaacacctgcagcgtcacgttgctgcccagaggtggcacgccggcatcgcgagcggtcacctgaaactgcagcagctctagctcctcgtggtccagcggctgcagcgcgtacaccttgccgctctccgcatgcaccgaaacgtagctcgacagcgcgcgctcccctacccgccgctctaccagcgagtaggacaccagcgcgttctcctgcgcgtccgcgtcccacgcagacacagtgaagatgtggcagcccggcgggttgttctccttcacgaacactgtgtactcgggctgcgcgaacgccggagcgttgtcgttcacatcagccacctccacagaaacactggccgtggcccacagcgaaggcgagcccccgtctcgcgcggtcaccaccagctcataggctgacacgctctcgcggtccagggcactgtccagcaccaacgagtagtaattcttgaaggtggacaccagcttgaaggggacgtgggacgtcaaggagcaggtgaccagcccattgacacccatgtctttgtcggacacgctgatcagggcgatgactgtacccagtggagcgtcctctctaattggaagtgataaagacttgaattccaaatctgggacattatcgttgttgtcttctacttccacaataactctacaatggccagaaagtgggagctgtcccttatcaatgccctctacaataatttcataggatttgctttcttcaaagtcaatatatccctttacaataatttgtccagtaattggatctatgtgaaacttggatttcacatttggcgaaatatcatttgagaatgaataaacaatgtccccattcaatccttcgtctaaatctgaggcgttaagtttaattaccaatgttccattaggaacattttctagtaatctcaccttataaatggttctgtcaaaagctggggcattgtcattggcatccagtactgtgatgagtaactgaacggtgccagtcaactcgggtttgcctccatcagtggctgtgagcactaaaaaaatctccggagcttcttctctgtctaaagatttccgtaatataagcccaagaccttttaccagctcgtcatcaggtggtttttccagagaaaagtattcatttgggctcagtctgtaagtgagcagggcgttctccccgatatctgcatccgaggcgccctctagtggaaaccgagagtcaagcggcctggattccgcgatggacaggttcttttgtgttgctgggaacaccggcgggttatcgttaatgtccctcacctccacgtccacatggaaaacctgcagcggcctgtctacgatcacctccaggtggatgctgcactccgcgctccgccggcacagctcctcccggtcgatccgagaattcacaaacaaaatgccattctgcagatttacctccagaaggcctccgcggcccttggacgccacccggaacaggcgcggcaccagctccgccagctccagtcccaggtcctgcgcgatgcggcccacgaaggtgccgtgtttggcctcctcggagaccgagtagtggagctgaccgttccctgcctcccaggctgcgaggagaagaagtaagagcagcagacgccgggattcctggccgcttccccaggaaaactccatctttagtgcacagtattttgttctgattaaatatcgtttctcaaagtcaagggaaatcttttaatcggtcagtcaagtgcagctgcatcctccatatttcagactccaaagagtgtatat

SEQ ID NO: 13656 - RNA, 2047 nt, Homo sapiens
  source 1..2047: mol_type = other RNA
gctgggattacaggcatgagccaccatgaccggccagctactgtcttttctttgacccttcctttccagtttttgaagataaagcaggaaataatcttctctgaagatacttgataaaaattcccaaaacaacaaaacacatgcttccacttcactgataaaaaatttaccgcagtttggcacctaagagtatgacaacagcaacaaaaagtaatttcaaagagttaagatttcttcagcaaaatagatgattcacatcttcaagtcctttttgaaatcagttaatattattctttccccatttccatctgaatgactgcagcaatagttttttttttttttttttttttttttcgagatggaatctcgctctgtcgcccagctggagtgcactggcgcaatcccggctcaccgcaatctctgcctcctgggttcaagcgattttcctgccttagcctctcgagtagctgggaccacaggcacgtgccaccacacccagctcacttttgcattccggtgtgggtctttttgagtttaccctatttagggttctttgagcctcttgaatatctagattcatgtatttcatcaaagctgggacattttctaccattatttcttcaaatattatgtccctttctctctttcttctccttctgggactcccctcatgcatatactggtatgcttgatagagtcccagaggtcttttatgctctgttcatttttcttcattctttttcctttctgctcctcagactgtataatcttaattgacctatcttgaagcctgttgattctttcttctgacttctccagtctgctgctgaatacctctagtgaattttcagttttagttataatacttttcaactccagaatttctatttggttcttttctacaatttcaatctctttattgatattctgtattggatgagacattgctttcctaatttttttgttctctgtccatggtttcctttagctcttctagcatatctaaaagagttgatgaaaagtctttgttttgtacatccgaagtctgtgcttcttcaggggtagtttctattaatttctttttttacctgtgtatgggccatacttttctggtttttccttgtcatgtaatctttgctaaaaatgtgacattttgaatagtattataatgtggtaactctggaaatcagattctcctccctccccatagttcattgttggtacttgttatggttaccactgtttggtaacttttctgaactttataaagtctgtattcgttgctgtgtgtgaccagctgagctcctgttctgttagcttaatttgcagctagtgatccaaaagagaaacagatttccttaaatgcctccaaaggactgattcttgaagaacttcaacatttggtagtggagtagacaaggacgactctgagaactttcacatgaattttctttcaccaatggacttcagcgaggaagaaacagaggagggaaaagtgagagataaagagagggtgggcagggcaccgctgggtatggaaaacgttagaaagggatggaaaacgttagaaaggggtgaaaagccgagcgcagtggctcacgcctgtaatcccagcactttgggaggccgaggcgggaggatcgcttcaggccaggggttcgagaccagcctgggtaacacagcgagaccctatctccggaaaaactttttttaaaaaattagccgggtgtggtggtgcatgcccgtggtgccagctacttagagggctgaggtgggatgacccgtaagccccggaggtcgaggctgcagtgagccgtgatcgcgtcactgcactcagactggacgacagcgcgagacctgtctcaaaaaaaaataacaaggggtagggtggggcagtgagatggttcagcgttgttcccaaggaactcatctccctaaatttccagtctcaagcgccgctttcattccctgccccgagcggcgctccccgctccgtgcacgcatctccgctgagggccgccctgacgcacggccttctgccttgaac

SEQ ID NO: 13657 - RNA, 4142 nt, Homo sapiens
  source 1..4142: mol_type = other RNA
gctgggattacaggcatgagccaccatgactggcctaaaacaaaataaattcttaatggcatttgtggaatgtgtttaagagccaaaactgtgaaaatgtaagctttatctttcttttttcctagattatttaaagaggattgtagccacacttcagatgaatgtttacaagccaaataatgatttaagagtgtgctcaataaaaaggccataggtttaagaattaaatggaataatataaattactaggtcaacaagaatatttcatgtatagtacactgtctaaggaatgcagagaaattttacaagaaacccaagactaaatacttcattaagaacactggttactaagtaaatagatggctcatgtaggaaaaagctaatatatgtagatgtaatgtcaactaagtgcatgtgacagaaatgaagaactaggaataagaatccagattttctggccaggcacggtggctcacatctgtaatcctagcactttgggaggccatagtgggtggatcacctgaggtcaggagtttgagaccagcctggcctacatggcgaaaccccatctctactaaagatacaaaaattagctgggcgtggtggtgggcacttataatcccagctactcaggaggctgaggaaggagaatcgctcgaacctgggggtggatgttgcagtgagccaaggtcgcgccacttcactccagcttgggcgaaagagcaaaactccatctcaaaacaacaaccaaaaagaatccagatttttaggtgtctaatactagacattctgtatccaagtttcagccatttcatccaataaagccttctaaagccttttttttttgagacagggtctcactctgtcactcaagctggagtgcagtggcgtgatcttggcttactgcaacctgtctcccaggctcaagcgattctcctgcctcagcctcccgagtagctaagactacaggccgtgtcaccaaacccggctaattttttgtaggcacggggtttcaccgtcttggccaggctggtctcaacctcctgacctcaagtgatccacctgccccagcctcccaaagtgctgggattacaggcatgagtcactgcgcccagctcccaaagccaattttcaattatttgtgagccatagattcagtgactacatcaatatctcttgccagggattggcctaacagctcagagaacagattgttaggatatatgggcaagccttctaagttcaagaggcaagagcagaaaatggaatgctatagggatttagctccatcttaagccattctggccctttctgctctactttaccagctatagagttaggaaggcttccagtaggccacagcaagaggaaaaacctttattctgtggggctcatttatccaggatttaacttacctgtgtcatgttaccgatctattaacacaagtaatttagagttggttatattatttcaagaaattgagcacaaagccaggatgtacaaggaggaattcaaacaatcaatattggattatataatgaaaagatgcccttacaatgtttatgatctagaatgtaatcataataaaggggggaaaataccttatgagtatcacaattgtatcagagactattaaacagtacaatgatacagagaatttattcaattcatacaagtaatttaccagatctaaacagtgaatagactgacctaaggggaaaaaaatccttacattgatagcaaaatatcttctagcccccataaataatctgcaatcatttgctaggaaaaaaacttcataaccatatgggtcatgcagacatttttatttatttatttattttgagacagagtctcgctctgtcgccctgattggagtgcagtggcacgatctcagcttactgcaacctccgtctcccaggttcaagcaatttcctgcctcagcttccccagtagctgggattataggcacacaccaccatgcctggctaatttttgcatttttagtagagataaggtttcaccatgttggtcaggctggtctcgaactcctgacctcaggtgattcgcctgcctcggcctcccaaagtgctgggattacaggcgtgagccaccgtgcccagcccatgcagacatttttaagtgctattggtattcactttatttcaaactgagcaaaacaatacaaccttttacttttttatacattttaaaatttctctcatattaacattccttcctaccccaatccatcccatcaccaaacaggaatgagataaggagtgaaaaaaagatgtatgtttctcattttccttcttttcccttgaagtaaaccagtaatttattaaaatattttataggtcagaggataacaaaagactcaatgtagtaaataagtaaataggcattcaaatatcagtaacctaacaggccctaatacagctttaagattttcttctttttttttttttgagagggagtctcgctctattgcttaggctggaatgcagtggtgcgatcttggttcactgcaacctccacctcccgggttcaagcaattctcctgctttggcctcctgagtagctgggattacaggcacatgcaccaaccctggctaatttttctgtatttttagtagagacagggtttcaccatgttggccaggctggtctcgaactcctgacctcaagtgatccacccacctcagcctcccaaagtgctgggattacaggtgtgagccactgcactggcctaagattttcattttaacagggaactgttagaacagaaaagaagcttcccaagaggcactcattttaaaaataaattatagcttaaattattactatgtggattatatcagcaaaggcagaaagaattaatgttttcctcctttcatgaaccttgtaaggctagtgttgagtggcttacaaatgtcatataatggactgtaaatcatctgccatattgatcaatcatgtttatttaaggttttcttaacattagagatttttaatgggagtataaaattagtaaacaaccatttcattttttctctcttcctattctagccacataagccagtttaatccatgacacagatttcagctgtaatttgcaaaacaatccaagagctaccacagtccccaaaactacagaaaactgccatccacaaataaactaccaaggtaaatgtaaatacagcgtggttctaattttctttcacacaatcccagacaaccccaaataactttataaataccttatgaaaaaaagcaatttaaaaacctatcaaatctatttaaaatatataaatgcagacctctcaaatttccttcaatcaggccagaaattatcacaaaaattataatcacagttacaaacagaatgagtggaatgtttgtaagtttaggacaaccaaaaaagccccatgtaactttttaaaaatataatcattcactcaaatatactgtaaataggaatggcagtaacacaggaagcaaaaataaacttgcaagtgaaatttctagaagctcatgaaaacaataccatcccatattgcagatacaaaaggaaaaacagttctaatggggttaagagtactctggtcatcttcgttcgtttggtcgtgcaaggtgttaactattttcacttcccatatcacaaagttagtccacaggaggagctggtggatcttgtccattatgaggactggttggctttccaggtaggctggatcctcttagattaggaggtctcagtaagaacaagatcaatgcaataaccatccaggctaccaagatcattgtaacactgatgccattatcaccagagggtcccggtaattcctgaagacactctgtgtctgtgcagtaggactgggactgccgtaacagattgatcagtcttctcattgcatgttcatgagagcaaacacattcacagggatcaaatccaccttctgccatgattacccagcttgattttacttgactgtttaaataaacagaaatttacttctcacggttctggaggctaggaagtccaagatcaaggcactggtagattcagtgtctgctgaggacccactctctggttggtagatggtgccttctcactgtgtcctactatggtggaagag

SEQ ID NO: 13658 - RNA, 4131 nt, Homo sapiens
  source 1..4131: mol_type = other RNA
gctgggattacaggcatgagccaccatgactggcctaaaacaaaataaattcttaatggcatttgtggaatgtgtttaagagccaaaactgtgaaaatgtaagctttatctttcttttttcctagattatttaaagaggattgtagccacacttcagatgaatgtttacaagccaaataatgatttaagagtgtgctcaataaaaaggccataggtttaagaattaaatggaataatataaattactaggtcaacaagaatatttcatgtatagtacactgtctaaggaatgcagagaaattttacaagaaacccaagactaaatacttcattaagaacactggttactaagtaaatagatggctcatgtaggaaaaagctaatatatgtagatgtaatgtcaactaagtgcatgtgacagaaatgaagaactaggaataagaatccagattttctggccaggcacggtggctcacatctgtaatcctagcactttgggaggccatagtgggtggatcacctgaggtcaggagtttgagaccagcctggcctacatggcgaaaccccatctctactaaagatacaaaaattagctgggcgtggtggtgggcacttataatcccagctactcaggaggctgaggaaggagaatcgctcgaacctgggggtggatgttgcagtgagccaaggtcgcgccacttcactccagcttgggcgaaagagcaaaactccatctcaaaacaacaaccaaaaagaatccagatttttaggtgtctaatactagacattctgtatccaagtttcagccatttcatccaataaagccttctaaagccttttttttttgagacagggtctcactctgtcactcaagctggagtgcagtggcgtgatcttggcttactgcaacctgtctcccaggctcaagcgattctcctgcctcagcctcccgagtagctaagactacaggccgtgtcaccaaacccggctaattttttgtaggcacggggtttcaccgtcttggccaggctggtctcaacctcctgacctcaagtgatccacctgccccagcctcccaaagtgctgggattacaggcatgagtcactgcgcccagctcccaaagccaattttcaattatttgtgagccatagattcagtgactacatcaatatctcttgccagggattggcctaacagctcagagaacagattgttaggatatatgggcaagccttctaagttcaagaggcaagagcagaaaatggaatgctatagggatttagctccatcttaagccattctggccctttctgctctactttaccagctatagagttaggaaggcttccagtaggccacagcaagaggaaaaacctttattctgtggggctcatttatccaggatttaacttacctgtgtcatgttaccgatctattaacacaagtaatttagagttggttatattatttcaagaaattgagcacaaagccaggatgtacaaggaggaattcaaacaatcaatattggattatataatgaaaagatgcccttacaatgtttatgatctagaatgtaatcataataaaggggggaaaataccttatgagtatcacaattgtatcagagactattaaacagtacaatgatacagagaatttattcaattcatacaagtaatttaccagatctaaacagtgaatagactgacctaaggggaaaaaaatccttacattgatagcaaaatatcttctagcccccataaataatctgcaatcatttgctaggaaaaaaacttcataaccatatgggtcatgcagacatttttatttatttatttattttgagacagagtctcgctctgtcgccctgattggagtgcagtggcacgatctcagcttactgcaacctccgtctcccaggttcaagcaatttcctgcctcagcttccccagtagctgggattataggcacacaccaccatgcctggctaatttttgcatttttagtagagataaggtttcaccatgttggtcaggctggtctcgaactcctgacctcaggtgattcgcctgcctcggcctcccaaagtgctgggattacaggcgtgagccaccgtgcccagcccatgcagacatttttaagtgctattggtattcactttatttcaaactgagcaaaacaatacaaccttttacttttttatacattttaaaatttctctcatattaacattccttcctaccccaatccatcccatcaccaaacaggaatgagataaggagtgaaaaaaagatgtatgtttctcattttccttcttttcccttgaagtaaaccagtaatttattaaaatattttataggtcagaggataacaaaagactcaatgtagtaaataagtaaataggcattcaaatatcagtaacctaacaggccctaatacagctttaagattttcttctttttttttttttgagagggagtctcgctctattgcttaggctggaatgcagtggtgcgatcttggttcactgcaacctccacctcccgggttcaagcaattctcctgctttggcctcctgagtagctgggattacaggcacatgcaccaaccctggctaatttttctgtatttttagtagagacagggtttcaccatgttggccaggctggtctcgaactcctgacctcaagtgatccacccacctcagcctcccaaagtgctgggattacaggtgtgagccactgcactggcctaagattttcattttaacagggaactgttagaacagaaaagaagcttcccaagaggcactcattttaaaaataaattatagcttaaattattactatgtggattatatcagcaaaggcagaaagaattaatgttttcctcctttcatgaaccttgtaaggctagtgttgagtggcttacaaatgtcatataatggactgtaaatcatctgccatattgatcaatcatgtttatttaaggttttcttaacattagagatttttaatgggagtataaaattagtaaacaaccatttcattttttctctcttcctattctagccacataagccagtttaatccatgacacagatttcagctgtaatttgcaaaacaatccaagagctaccacagtccccaaaactacagaaaactgccatccacaaataaactaccaaggtaaatgtaaatacagcgtggttctaattttctttcacacaatcccagacaaccccaaataactttataaataccttatgaaaaaaagcaatttaaaaacctatcaaatctatttaaaatatataaatgcagacctctcaaatttccttcaatcaggccagaaattatcacaaaaattataatcacagttacaaacagaatgagtggaatgtttgtaagtttaggacaaccaaaaaagccccatgtaactttttaaaaatataatcattcactcaaatatactgtaaataggaatggcagtaacacaggaagcaaaaataaacttgcaagtgaaatttctagaagctcatgaaaacaataccatcccatattgcagatacaaaaggaaaaacagttctaatggggttaagagtactctggtcatcttcgttcgtttggtcgtgcaaggtgttaactattttcacttcccatatcacaaagttagtccacaggaggagctggtggatcttgtccattatgaggactggttggctttccaggtaggctggatcctcttagattaggaggtctcagtaagaacaagatcaatgcaataaccatccaggctaccaagatcattgtaacactgatgccattatcaccagagggtcccggtaattcctgaagacactctgtgtctgtgcagtaggactgggactgccgtaacagattgatcagtcttctcattgcatgttcatgagagcaaacacattcacagggatcaaatccaccttctgccatgattacccagcttgattttacttgactgtttaaatccgcccagacaacaaccgatggggcggggaggatgggggccgggaccgaggctcggcagaaagaccgcctggagcttccagaaggctgcggctgctccggacgctgctgccactgccgtttctggcc

SEQ ID NO: 13659 - RNA, 4276 nt, Homo sapiens
  source 1..4276: mol_type = other RNA
gctgggattacaggcatgagccaccatgactggcctaaaacaaaataaattcttaatggcatttgtggaatgtgtttaagagccaaaactgtgaaaatgtaagctttatctttcttttttcctagattatttaaagaggattgtagccacacttcagatgaatgtttacaagccaaataatgatttaagagtgtgctcaataaaaaggccataggtttaagaattaaatggaataatataaattactaggtcaacaagaatatttcatgtatagtacactgtctaaggaatgcagagaaattttacaagaaacccaagactaaatacttcattaagaacactggttactaagtaaatagatggctcatgtaggaaaaagctaatatatgtagatgtaatgtcaactaagtgcatgtgacagaaatgaagaactaggaataagaatccagattttctggccaggcacggtggctcacatctgtaatcctagcactttgggaggccatagtgggtggatcacctgaggtcaggagtttgagaccagcctggcctacatggcgaaaccccatctctactaaagatacaaaaattagctgggcgtggtggtgggcacttataatcccagctactcaggaggctgaggaaggagaatcgctcgaacctgggggtggatgttgcagtgagccaaggtcgcgccacttcactccagcttgggcgaaagagcaaaactccatctcaaaacaacaaccaaaaagaatccagatttttaggtgtctaatactagacattctgtatccaagtttcagccatttcatccaataaagccttctaaagccttttttttttgagacagggtctcactctgtcactcaagctggagtgcagtggcgtgatcttggcttactgcaacctgtctcccaggctcaagcgattctcctgcctcagcctcccgagtagctaagactacaggccgtgtcaccaaacccggctaattttttgtaggcacggggtttcaccgtcttggccaggctggtctcaacctcctgacctcaagtgatccacctgccccagcctcccaaagtgctgggattacaggcatgagtcactgcgcccagctcccaaagccaattttcaattatttgtgagccatagattcagtgactacatcaatatctcttgccagggattggcctaacagctcagagaacagattgttaggatatatgggcaagccttctaagttcaagaggcaagagcagaaaatggaatgctatagggatttagctccatcttaagccattctggccctttctgctctactttaccagctatagagttaggaaggcttccagtaggccacagcaagaggaaaaacctttattctgtggggctcatttatccaggatttaacttacctgtgtcatgttaccgatctattaacacaagtaatttagagttggttatattatttcaagaaattgagcacaaagccaggatgtacaaggaggaattcaaacaatcaatattggattatataatgaaaagatgcccttacaatgtttatgatctagaatgtaatcataataaaggggggaaaataccttatgagtatcacaattgtatcagagactattaaacagtacaatgatacagagaatttattcaattcatacaagtaatttaccagatctaaacagtgaatagactgacctaaggggaaaaaaatccttacattgatagcaaaatatcttctagcccccataaataatctgcaatcatttgctaggaaaaaaacttcataaccatatgggtcatgcagacatttttatttatttatttattttgagacagagtctcgctctgtcgccctgattggagtgcagtggcacgatctcagcttactgcaacctccgtctcccaggttcaagcaatttcctgcctcagcttccccagtagctgggattataggcacacaccaccatgcctggctaatttttgcatttttagtagagataaggtttcaccatgttggtcaggctggtctcgaactcctgacctcaggtgattcgcctgcctcggcctcccaaagtgctgggattacaggcgtgagccaccgtgcccagcccatgcagacatttttaagtgctattggtattcactttatttcaaactgagcaaaacaatacaaccttttacttttttatacattttaaaatttctctcatattaacattccttcctaccccaatccatcccatcaccaaacaggaatgagataaggagtgaaaaaaagatgtatgtttctcattttccttcttttcccttgaagtaaaccagtaatttattaaaatattttataggtcagaggataacaaaagactcaatgtagtaaataagtaaataggcattcaaatatcagtaacctaacaggccctaatacagctttaagattttcttctttttttttttttgagagggagtctcgctctattgcttaggctggaatgcagtggtgcgatcttggttcactgcaacctccacctcccgggttcaagcaattctcctgctttggcctcctgagtagctgggattacaggcacatgcaccaaccctggctaatttttctgtatttttagtagagacagggtttcaccatgttggccaggctggtctcgaactcctgacctcaagtgatccacccacctcagcctcccaaagtgctgggattacaggtgtgagccactgcactggcctaagattttcattttaacagggaactgttagaacagaaaagaagcttcccaagaggcactcattttaaaaataaattatagcttaaattattactatgtggattatatcagcaaaggcagaaagaattaatgttttcctcctttcatgaaccttgtaaggctagtgttgagtggcttacaaatgtcatataatggactgtaaatcatctgccatattgatcaatcatgtttatttaaggttttcttaacattagagatttttaatgggagtataaaattagtaaacaaccatttcattttttctctcttcctattctagccacataagccagtttaatccatgacacagatttcagctgtaatttgcaaaacaatccaagagctaccacagtccccaaaactacagaaaactgccatccacaaataaactaccaaggtaaatgtaaatacagcgtggttctaattttctttcacacaatcccagacaaccccaaataactttataaataccttatgaaaaaaagcaatttaaaaacctatcaaatctatttaaaatatataaatgcagacctctcaaatttccttcaatcaggccagaaattatcacaaaaattataatcacagttacaaacagaatgagtggaatgtttgtaagtttaggacaaccaaaaaagccccatgtaactttttaaaaatataatcattcactcaaatatactgtaaataggaatggcagtaacacaggaagcaaaaataaacttgcaagtgaaatttctagaagctcatgaaaacaataccatcccatattgcagatacaaaaggaaaaacagttctaatggggttaagagtactctggtcatcttcgttcgtttggtcgtgcaaggtgttaactattttcacttcccatatcacaaagttagtccacaggaggagctggtggatcttgtccattatgaggactggttggctttccaggtaggctggatcctcttagattaggaggtctcagtaagaacaagatcaatgcaataaccatccaggctaccaagatcattgtaacactgatgccattatcaccagagggtcccggtaattcctgaagacactctgtgtctgtgcagtaggactgggactgccgtaacagattgatcagtcttctcattgcatgttcatgagagcaaacacattcacagggatcaaatccaccttctgccatgattacccagcttgattttacttgactgtttaaatctgagctaaggggagaaggggaggtgagaattggaaagggagatggagatgcggcctgagctggagaggctcactttccagaaggtaagcaacaccatatgcaaactctacttcacagttttgtctgaggccactctgtcaacacccgcccagacaacaaccgatggggcggggaggatgggggccgggaccgaggctcggcagaaagaccgcctggagcttccagaaggctgcggctgctccggacgctgctgccactgccgtttctggcc

SEQ ID NO: 13660 - RNA, 2636 nt, Homo sapiens
  source 1..2636: mol_type = other RNA
gctgggattacaggcatgagccaccatgccaagctggtagattccctcttctaaaagaagtacatgttgctttgcaatcaaacagaaaggcttttcatgtggatttgctgctaagttctacctcagtacagaagatgaaactgggtctacagtgcagaaggtgagaaattagtttttgatgaatggacacaacctgcgaaccaaaggtatcgagatggaactcaacacagcctcaacagtaatcagttgttttgtgtttccctgagatgaaaacatgaaacaggatctgcatttgatagcactatgaaattaataaggtaagtttcatgcatggtccatgcaaaaaaaaaaaaaaaagaaattaataagggaaggataagcaagttgtcaaggaaatactggattttctactgccttatgctgatagagtcagagaaaatcttatagagttttttgttaaaactcaatctgctaatttagtcagactgacatgttcctcaatgccaagtaggagtcctttttccctttcttccccttagtttacgttagtaacagttagcaagtaacagcttctaggttagcattgtcaggatcagaaagaaaaaaaaaaaggagaaaagcttgatttactgaaatgagaattctctcaaataaggacctaaatggtttttccagaaaaccttcctagacacatattctctaacaggtccatgggcttagggggcctataaactccccaagagaacaaataaaatttggcaattatgtgcaatgttttgaagagtctaaactttcattaaactctctaagtgagctattactcccaagctcccccagaaatactaaaactgactgtactggagataaaaaattcttttgtttagcatcaaagatatgcagtgcagtagttcagagttctaaaaggaaactttctttctgaagatatctcagacctcactcacagacctgtgagtgaaatatcagttctaagtcaataaccaactttatttataagtcagagttctttaaattactgtattgatctctgctaccttaaatcctttatgaaaaaaggggagacattttaaaaagtggttgacctctgtggttccctccctcttgacaatgactttacttcccccactaactttactatgccaaattgagttttatattcgatatgaggggaaaaaaggatataaaactgtacctattacacacactttcataaaacaccaagattggaaaggaacagaccaaaatattaatggggtttattgttgggctgggggactatgattaatttttataattatttatattaaattatgttttttggggttttatgcatgagtacacatttcttttataatcagaaaataaaatactttagcaatggcagagtcactggagaaaataagcttacagatttccaaataggatagaaggctaacaaaaaactcaaattctaaaataaagaacaatccaattaaaaaaaactatggcacatttttaaagcattttgaaatttctgtctttgtgtaaacaaacttacagtttcaatgacgatagtagctgaaaaagtcttctcattgatggattctagggtaccttcatttcctctgtagcctccatttaaaactagaattctttttcctggtgctggaattactgtctctaaatgagtctggtcaagtttcagcttgtctccagaatcaatcatcttcacaacagctgtatatttgtcaattacttccttaacaatagcctttttcttatgatatttctctcccagtttcttggttataattttcacaataatttcaggctgtagccagtagtctgttcgggcagttcttttcttttcctcttcaatctccatgatttcatccagtgcagatttctttttcttcttttctttagactgagttgagctctgggaagattcttttcgtttcactgatgctgaacttcctatcgtcttcagtgcactcggtcccagagtacttgacttggaagatgttgctccggatgagctacatgctcctttactcaaattaaacgtgactttctcttcatcattttctctgcttaattccgtaaaagtagggacctcctgttccttcccttccaggcctcttctcacttgctcttcaataaatttggcagttttttcttcatcatcaaggtcctgctttttctttttctccagttccagttgccggcggatagtttctgggtccctgtctatgtactgaatataccagccttttggtgtctcgtccactttgcacaagccttctctgcccagccacttagtaaaatcagtcagagtttcccactgagtggcattcatgtggatgtgctctcggtggctgatgtattcgttgtagacaatgttgttgtggacccttttagtgccaaagcgtctcctgagaagttctagaaagtcatttcggaattccctcgtcccggcactgcttctggcacatctggcaataccagcgtagcttctgcagccccttggacttgatcctgttggcgatagccttgggagtaagaaaatccgacttccccatggcgaccacggcagcgatcactttctggaccccagtactcagccagccggaaacgga

SEQ ID NO: 13661 - RNA, 2704 nt, Homo sapiens
  source 1..2704: mol_type = other RNA
gctgggattacaggcatgagccaccatgccaagctggtagattccctcttctaaaagaagtacatgttgctttgcaatcaaacagaaaggcttttcatgtggatttgctgctaagttctacctcagtacagaagatgaaactgggtctacagtgcagaaggtgagaaattagtttttgatgaatggacacaacctgcgaaccaaaggtatcgagatggaactcaacacagcctcaacagtaatcagttgttttgtgtttccctgagatgaaaacatgaaacaggatctgcatttgatagcactatgaaattaataaggtaagtttcatgcatggtccatgcaaaaaaaaaaaaaaaagaaattaataagggaaggataagcaagttgtcaaggaaatactggattttctactgccttatgctgatagagtcagagaaaatcttatagagttttttgttaaaactcaatctgctaatttagtcagactgacatgttcctcaatgccaagtaggagtcctttttccctttcttccccttagtttacgttagtaacagttagcaagtaacagcttctaggttagcattgtcaggatcagaaagaaaaaaaaaaaggagaaaagcttgatttactgaaatgagaattctctcaaataaggacctaaatggtttttccagaaaaccttcctagacacatattctctaacaggtccatgggcttagggggcctataaactccccaagagaacaaataaaatttggcaattatgtgcaatgttttgaagagtctaaactttcattaaactctctaagtgagctattactcccaagctcccccagaaatactaaaactgactgtactggagataaaaaattcttttgtttagcatcaaagatatgcagtgcagtagttcagagttctaaaaggaaactttctttctgaagatatctcagacctcactcacagacctgtgagtgaaatatcagttctaagtcaataaccaactttatttataagtcagagttctttaaattactgtattgatctctgctaccttaaatcctttatgaaaaaaggggagacattttaaaaagtggttgacctctgtggttccctccctcttgacaatgactttacttcccccactaactttactatgccaaattgagttttatattcgatatgaggggaaaaaaggatataaaactgtacctattacacacactttcataaaacaccaagattggaaaggaacagaccaaaatattaatggggtttattgttgggctgggggactatgattaatttttataattatttatattaaattatgttttttggggttttatgcatgagtacacatttcttttataatcagaaaataaaatactttagcaatggcagagtcactggagaaaataagcttacagatttccaaataggatagaaggctaacaaaaaactcaaattctaaaataaagaacaatccaattaaaaaaaactatggcacatttttaaagcattttgaaatttctgtctttgtgtaaacaaacttacagtttcaatgacgatagtagctgaaaaagtcttctcattgatggattctagggtaccttcatttcctctgtagcctccatttaaaactagaattctttttcctggtgctggaattactgtctctaaatgagtctggtcaagtttcagcttgtctccagaatcaatcatcttcacaacagctgtatatttgtcaattacttccttaacaatagcctttttcttatgatatttctctcccagtttcttggttataattttcacaataatttcaggctgtagccagtagtctgttcgggcagttcttttcttttcctcttcaatctccatgatttcatccagtgcagatttctttttcttcttttctttagactgagttgagctctgggaagattcttttcgtttcactgatgctgaacttcctatcgtcttcagtgcactcggtcccagagtacttgacttggaagatgttgctccggatgagctacatgctcctttactcaaattaaacgtgactttctcttcatcattttctctgcttaattccgtaaaagtagggacctcctgttccttcccttccaggcctcttctcacttgctcttcaataaatttggcagttttttcttcatcatcaaggtcctgctttttctttttctccagttccagttgccggcggatagtttctgggtccctgtctatgtactgaatataccagccttttggtgtctcgtccactttgcacaagccttctctgcccagccacttagtaaaatcagtcagagtttcccactgagtggcattcatgtggatgtgctctcggtggctgatgtattcgttgtagacaatgttgttgtggacccttttagtgccaaagcgtctcctgagaagttctagaaagtcatttcggaattcctctgaaaaataatccataaactgctgaggattttctgaagccagcaatagttgtctctgatgagattcggacatacaatgacacttaaagccattctcgtcccggcactgcttctggcacatctggcaataccagcgtagcttctgcagccccttggacttgatcctgttggcgatagccttgggagtaagaaaatccgacttccccatggcgaccacggcagcgatcactttctggac

SEQ ID NO: 13662 - RNA, 1299 nt, Homo sapiens
  source 1..1299: mol_type = other RNA
gctgggattacaggcatgagccaccatgccaggccgttttccagtttttatggtaaagttgtaatttgtagcagattcttaaaatggtcttttagaaaaacacaaattcttttgtaatacatcccagaagacttctttcacctgctggtttctgagagtataaatgaagggatttagtaaaggggcaattgaggtatagagcaaagctacacctttggatacagtcactctttcttttgcagatggtttaatatacataaagatacagctaccgtatgtcatggagacaacaatcatgtgggaagtacaggtggaaaatgctttgttcctttgctgtgcagaagagaatttcagaatggtcttaataatgcaagtgtaagagagaatcactaataccagtgtgaccacaagtgtcaccacagctaaggtaaaagacatcaattctaggacatgggtatctgtgcaggagatctgcagaataggagaagtttcacacataaagtggtcaatagttttggaagcacaaaaatccagcttgagtcccatgaccaatgggggaaatatgattaagaatccagttacccaagagctaagtacaagttggtagcagactttgctgctcataatgattggataatgcagtggtttgcagatggcaacgtagcggtcataggacatggcagccaggaggtaaaactcagtaactcccggtaaaaggataaaaaataattgagttgcacaattattataagaaatggttttgtctctagtcacaatggttatcaagaatctaggaatacacactgttgtgaatattacttccaaaaaggagaaattacggagaaagaaatacattggcgtcttgagccggggatccagcagggtgaggatgatgatgattaagttccccatcaggctcaaggtgtagttgagaaatagaaacaggaaaatcacaatttgcaactgtgggtcatctgtcaatcctaggagaatgaactctatttccattgatttgttcttcatttctcttttgtgatccttatcaaatcttttttggatctattattcatttctttctgtgtgcacggaagagatgcatgctaacataattagtgacaattctactcattttatgaccacattttattatccaataggcacatttattaccaatgatttttgtggggagaggcaatgtgtacgtattgtgtttctgtagagaatttccacatttcctcaacttcatcctcactataaagattgatactcagatattaataattttaatggacatctatc

SEQ ID NO: 13663 - RNA, 1715 nt, Homo sapiens
  source 1..1715: mol_type = other RNA
gctgggattacaggcatgagccaccatgcccacctgatcctcacattcttttttttttttttttttctgatacagagtcttgctctgccgcccaggctggagtgcagtggcatgatcttggctcactgcaacctccgcctccgaggttcaagagattctcctgcctcggcctcccaagtagctgggattacaggtgtgcaccaccacacctggctaatttttgtatttttagtagagacagggtttcaccatgttggccaggctgatctggaactcctgaccttgagtgatctgcccacctctgcctcccaaagtgctgggattacaggcatgagccaccatacctgactgattctcagattctgaaatgacagttaagcccaggactcaagccagggacagaagcagataacctggttttggtgagaaggttatgcacttgcttctgaaaatgttgatgatgagactaagtcttatagtttcttgtgcacctcccttggtgcctagaagaaaggttaaaacaggatacattacagagggactatcttgagagaggagttacctgggcacagcccaggggcccttgggagtgacatgcaagggcagcactggcttgccttatttggttctcccgctctttcttctttcccttgtaaaagtaactgaagcttaaaggtgaaaatgacttaaataatagaaaccatgttagccttactccccttccccattagccacaaattggtggcgatcaccattttgtgcaccgagcctgggtctcacgcttgcaagtccttgggctcatctggagtcagcttcatcagtttgtccacacagagcaggatgagggtgaggaaccagaggctccagccaacagctgccgcgatccagccgtactcgtccactcctgtgcggcagcaccgggctgcttgtgggcagaagtccacgttgaggcactgctccagggtcccagggtctgggtggtgagcggtcaagcttgagctgttgctgctgcttgctgccgagcaagccgagtggagggaggcaaaggccaggctgaggatcagggtggcccgggtggcagcggggaggcgctgcatgctggaggctgtgctgagtgcccggtgcaggtgagccggtcctgcggagttgtgccgagtgcctgctgcaggtgagtcgactcccacctgcaggagctggaaagcaactctgccagaggtgaacttatgctgggtgtttgggggaaacaccatggggtggagcaaaggaaacttggcctgtcacaccttctctcacctctctagaagggaagccaaaccgttggctgaggaaggaagggaggggcaagctgtgcccttctcccctgagcgcaaatattgtccttattgagaaacaaggggaggacaagagagatctgtgtcatgctggttcctgggacatgagtttgctgcctctcccatctgcaggtgtagcatggatgctcaattccatttgggccaatattcactgagcacccactatgctgaagttgggagatacctgctgtcgaagtgcgttaattacaaacacgcatcattcaaccccagaaccgtgtttgaggaatggcttgggaggataaagcactgtgggtttcaacagtggaggccacatctgctgatgggatgcttcaagaagaaaatggcatttgaggttgggcatgggggctcaccctgtagtcc

SEQ ID NO: 13664 - RNA, 1211 nt, Homo sapiens
  source 1..1211: mol_type = other RNA
gctgggattacaggcatgagccaccatgcccacctgatcctcacattcttttttttttttttttttctgatacagagtcttgctctgccgcccaggctggagtgcagtggcatgatcttggctcactgcaacctccgcctccgaggttcaagagattctcctgcctcggcctcccaagtagctgggattacaggtgtgcaccaccacacctggctaatttttgtatttttagtagagacagggtttcaccatgttggccaggctgatctggaactcctgaccttgagtgatctgcccacctctgcctcccaaagtgctgggattacaggcatgagccaccatacctgactgattctcagattctgaaatgacagttaagcccaggactcaagccagggacagaagcagataacctggttttggtgagaaggttatgcacttgcttctgaaaatgttgatgatgagactaagtcttatagtttcttgtgcacctcccttggtgcctagaagaaaggttaaaacaggatacattacagagggactatcttgagagaggagttacctgggcacagcccaggggcccttgggagtgacatgcaagggcagcactggcttgccttatttggttctcccgctctttcttctttcccttgtaaaagtaactgaagcttaaaggtgaaaatgacttaaataatagaaaccatgttagccttactccccttccccattagccacaaattggtggcgatcaccattttgtgcaccgagcctgggtctcacgcttgcaagtccttgggctcatctggagtcagcttcatcagtttgtccacacagagcaggatgagggtgaggaaccagaggctccagccaacagctgccgcgatccagccgtactcgtccactcctgtgcggcagcaccgggctgcttgtgggcagaagtccacgttgaggcactgctccagggtcccagggtctgggtggtgagcggtcaagcttgagctgttgctgctgcttgcttctgccgagcaagccgagtggagggaggcaaaggccaggctgaggatcagggtggcccgggtggcagcggggaggcgctgcatgctggaggctgtgctgagtgcccggtgcaggtgagccggtcctgcggagttgtgccgagtgcctgctgcaggtgagtcgactcccacctgcaggagctggaaagcaactct

SEQ ID NO: 13665 - RNA, 1772 nt, Homo sapiens
  source 1..1772: mol_type = other RNA
gctgggattacaggcatgagccaccatgcccagcatgttttctagcaagataacaaagaagggtgcatttggattcttgaatcttattccaagatcaactgagaatttagccataagtattttggaaagttattccacctccttcaaattgggttctctaccttatatattacataacaaatgaacacactttgatacttttcccaacaaagcctttggatagaaaccaagaagcttggtttgctattttcatgcttatggcatttgctcacctaacttttagttatgacctcaaaagaaaaggccctcctctcttcctcacactactttgctcattatatgtgaaattcaactgtccctttgaggccaactactaatttttcctttctgcttcccaagaaaattagagaaatttcagaattcaaatatgacaacttttacaagtcataggccaaccatcaagttgtcatctgtgatatggaaaggggaaggggatggatctaggttcatcaagccatggatttggcactgcttgacacaataagccttccagatgtctttagtgaattcataattaaaatagtcaaaaggatcaatacctttgaagaaacaatccaagctccaaggggcagaagtaggctgagtagtcactttaaattcaatcaatacatttaacaaatattcattgaatacatattaaatggtagtgttaggcactggctaataaaccaacagacattgtaccttatcaaatggaacttatgatctattgagggagacaggcaataaccaaaaaaaaaaaaaaacatataattatacattgtgataagaaaattaaagggaaagaaataggatgcaatgactaataatgaaaaacagcatatttactttagaaagagtgattagagaagaaatctgtgaaaaggtagtatttaaagccagatgtgaagggtaaaaagaagccagccagccgggcacggtggctcacacctgtaatcccagcactttgggaggccgagatgggcggatcatgaggtcaggagatcgagaccatcctggctaactaacacagtgaaaccccgtctctactaaaaatataaaaaattagccaagcgtggtggcgtgcacctgtagttccagctattcgggaggctgaggcaggagaatggtgtgaacccaggaggtggagcttgcagtgagcagagatcgtgccactgcactccagcccgggccacagcgagaccccgtctcaaaaaataaataaataaataaataaataaataaataaataaataaaagaagccagacattgaagccatccaagtttgcactttccatgtaatgtaagtaaagaaccaattgaggtagatagaggtcaggaaactgcagctaatgggccaaatctgacatgctgcatccttttttatagcctccaagctaagaatgatcttttacatttttattgatttttttttcgagttggagtcttgttctgttgcccaggatggagtgcactggcgcgatctcggctcactgcaacctctacctcctgggttcaagtgattctcctgccacagcctgctgagtagctgggattacagtgtgcaccatcatgctcagctaatttttgtatttttagtagagacagggtttcaccatgttggccacgctggtcttgaattcctgatctcgtgatccacccacctcagcctcccaaagtgctgggattacaggtgtgagccaccacacccagctgatcttttacattttta

SEQ ID NO: 13666 - RNA, 3581 nt, Homo sapiens
  source 1..3581: mol_type = other RNA
gctgggattacaggcatgagccaccatgcccagcatttctaaataattttgtggaatgtaagacatgtaaatataaagaagaccaaaaattagaagaggtcagagtaatgaaatttcattggaaacctttcctcaatgaatacacagtcattgcaaaaacaacacctcaacctttactgaaagtgaaagttagcaaaaactagtgaatcaattccatcctgctattaaaaaggccagattcattgtcaaagggataaattctgggtcttacattctttttccaccatctgctcttttttaaataactttttcctaaatatggtagatcatggctccccttaactttcaaccgacaaagcagccatacctacctctttctaagatgaaattgtgacactgatctcacaggtgcctatgccatgtaaacagcaggaatgtcaccttgggtaggcccagggtatggaacgtaatagagagccctgtgtataggacagggtcactccttagctgatacttctaaggacccatcacaggcaagtggaatttctctatcctgacttcattcccaggtcaatgctgacatatagagttctaaatctagataatttgtaattagtgaagttgaaaatataccataatttcagcaaaaaaaaaggggtcttgtactagatagtactaatgggttaagcgagttaaattaattaggcttttaaggatctcagccttatttcttctatcactcattccttatcttcaaactgagtctttggtggatgtaatataatctcatcttaggtatatatgagcacagaacggccattaaaatccatcacagaccaaaagaagagactgattttaggtcagtcctttttcattttgtaacaacagtaattctacttatagaaaacagactctcaaatctcaaaagtttaaagtttcattagaaaaatcataaaaataagaaaagtattcatcaagaatgataatagtataatttcattatcaaattcatttaaaacatgaattacagtacagcaagagaagtgacagcataaagtcttatataattttaaaaacaaacatcacaccatatggttttaataaaaggcaattgcagttccaatttccaagctgtatccttaagttgagggttttccgtagttggttttacattaaactatctccataacaagtttaaaggtgtatgtcatttcatcaccaagtattttagtcccaaaatgtataaaccaagcatctgataatgaggtatcttgtcgctgcctctcttttatttgaggaatataaaatttaaggtcaatccaagttcaagtccacaccacagtgctatctagcacatgaatatttgtcctcctttgcttcttaggaagcgtgattaggagtcatagccacaaaattgagattatgatgataaactttttttttttttttaagtctgcctgctaagttctatctcttctttcacccacccctggaatctccacctcccctatcaaatttagatttgggaagagtttttgttcaaagtctcttaatttcttcagtattcaaattatatctgagtttatttaaaacttaaaaaaaaagaagaaaaaagcttacctctttttattgtttcatcaagaaaatgttaaaaccctgacaaaagcttaccatcttttccaactctattctatcaaggccctgtcagcactagcatgataccacagactggatctttttccattatttattcccaaaaattagcaaaatcctttgtaattagctgaagtctatcagaataaattcagtctctgaagatgaagctacttgagttgttccattctgttcacgcacataacaaaaggcagaatcattcatttatcctgaaaaaaaccagacagtgtgtgtgacaactgcaagcaaggctcgctaagacattcttgcagctcagagaaattaaagcaaagtgcaagctggaagtgagttctaaagttaagtctcccacttgaaatttaattacaataaagaaggttagaggaggatgaataggttcaatgtcttcaacaattatcgaggtggaaagccacctctgtgtgctcctccacggccccctctaaagccacctctttctcctcggaagttagatctatttctttctcgtccacggccagcagaagttccacctcttcctccacctctgggagctccacctcctcggtcagatttagatttgggaggaggcgattttggtcgaagtctctcaatttcttctgtacaaccagtcaagtaggaattaggagcactgaaataggatgcatatgtttctgcattgtagttgctatttgtaagcgttggtccaactgtgagccagcctggtcgaattgtactatctcttccaaatagatgaaggcgtcttctaccaagacaaaaatgctcaattatatgaaaaatttctacaggtttttctatattgccaatttcaggttcttctgtgataattaagtcaatgtcaacattagcatgaatgaagtccccgtctgtgctacgcttcacagttcctttgatccccatgaggcagtgttcctttgttctctgaaagacagcctttggatctaaagtcttagtcttcccaggattgtttttattggttttaatccaacaaatatcttcacatcttctgtaaccccattttcgtaaacacactcttccaaggtccaacccctccccagaaccacaccagagaaaaataaatgatcgaggtgctgcaatctcatcaatttctaacttcataatatcatcccaagtccagcatttttcattagcagtgatgccagtttctctgtaatattcttctaaagggggttccagaagaatcacatcaaatttgggtgttagttctctgatgtcaaaggcttctatatcggcttgtaagtacatgggaggagtgttagatttagctattaactcatcctttagcctgatgagctccctcagtttaggatattcttcaaatctgtcagctaaacctacatccctgatgaaattctgaggtctatgtccagtgtctacaaaatgttggcagtaatcattatggggatttaagctctgtgttcccttaagaaaagtactagaatctttgtaaatctcttcttcatatggcaaattttcttcatcctgttgcatttctagttcatccttatattcttccattttgtcttcatctgtctctccttcatccagatacttacgttttgcatttggagcagaggtatcataggaagccctgcaagtttctcttgtttcagcaatttctctctgctcatctttgctatttaacacggcaccaatgctgtcggcactttcagctcccaactgctgcgcgaggagctgtcgccgtaacttctgccgctcccggatctcctgcaagcggctatccatgttccaactccggcttttcactatcccgagtacttgtcaatctccagtgaactcttatccaacctttcttccgagtctgtggaacaaaattcaccgggagcttacgaacagagtatcctcatagctttcctcagtagagactt

SEQ ID NO: 13667 - RNA, 7898 nt, Homo sapiens
  source 1..7898: mol_type = other RNA
gctgggattacaggcatgagccaccatgcccagccaaagactacattttcatgagaaaatgaatagttagcataacagaatgactgaataaatgttctcttccctcatctggatcagtaactagttggttggtcttcagctgtgctcaccagaaaaccaaatgttccttgagttgatgcttgggtatagtagccaatgatatatttgcagctataagtaaaattccaaataaatatattctaaagggaaggttctatatggtggcaaggcctgactggtggctttggtctaagacatatggatccctcctctgtcagccactcccacaccacctgcaattcctgagaggttgtccacaagatggggctttgctgaggaagcctctagcagacacagctgcctggtacttcttgagaactaccttgtcttctgtctgatagttctgtgcctttcagggagagtgggaagagatgcaaccagtggtccaaccaactgagagcagaagaaaggaaaaagtgctatcctgggccaggcatggtggttcacacctgtaatcccaacactttgggacgctgaggcaggaggatcacttgatcccaggagttagagaccagcctaggcaacatagtgaggccctgtctctccaaaaaaattaaaagatcagccaggtgtggtggtgcacgcttttagtctcagctacttggaaggctgagatgggaagactgcttgagtccaggagtttgaggctgcagcgagccatgatcacagcactacactccagcctatgggacagagtgagactctgtttccaaagaaaaaacaaaaaaaacaaaaacaaacaaacaaacaaacaaaaaaactctaccctgaaatggttgcaaatgtgaagaaacaaaatgccagatacagatgctggtgactcaactatttcttgaaaaggaaagaggcctggaagcttgggagagggggccaaactttctctggtcatcttcccactgttgccagcaatggtgagccggaaattgaaagaatgacacaaggttgcctgtacagacccacacaccctcccaggaaattggggaagctgggcatccctaacagtccatttaatggaggtggaaaagaggctgtggcttgagcttacaatgccctcacccagtcttcagatgaactcacagctcccaccctaaaatgagggggaaacattaaaatttagagtgggtcttgcctgcctgactttcctctgccaagataagctcaataaggcctgttcacagatgatgcatggctggtataatgggaccaaatgctgcccttgattctactcagaagtagaaagtgggtgagtaccaaacacaggccgaggacaggaggtccagggcttggacagagctcaggggtgaggtgagtaggggcaggccccacaggtttcatatgcctccaggccctgcagtggaaagctcaagttgctttcaaagtctctctggatggaagctgctgccaatatggttaacactcctgccagaactgctcctcaggaagtggctggaggagacatggggccagtttagcattctctactctgcctctctgtgccagggctgcttggggaacagcccactgtggcttctcttgctgcaatggaagagtacccgagccaagagaaatggaaaaagcagcatacccccaaaggagctacaaagcaaaggaaacacaccaggctcatgatgggtggctgatgggaagtctccaacacccaaagcctttactctatcagctgggtcctcacaggatctaactgcagagctaggaagagccttcccagaacccaaccacttcccaaacccagtctctgcttcatctactttctgattactatcttggctgaaaactatcaaaggttcttggattttaacctcaaatcaacttcagaacctgtggctagaaacgtgctatctttcagtgataaagacgctctagtttcctcctggcatggtgcctgtcagaggctatcatcctagaaggaagctaggatcacagggttattagcaacatctttggccaatgagagcaaagagggagcttgtctcttccagctcccagtctgcgtcagcacagaccagcatgatggtcactattttccaaaggcagcagagaaaccagcacttaaaaaccacaagttcaaagcccagctggaagtagatgaggctttggcagagaaaccagggtggtcagagctttgaacttgatgacactgagtaaaggatacagtggctgagcgtggggactcacgcccgtaatcccagcactttgggaggtcaaggcgtgcagatcacctgaggtcaggagttcgagaccagcctggctaacgtggtgaaaccctgcctctactaaaattacaaacaaattagccaggcgtggtggcaagcgcctgtaatcccagctactcaggaggctgaggcaggagaatcacttgaacctgggaggcggaggatgtagtgagccgagaccatgctattgttgcactccagcctgggtgacaagagcaagactctgtctcaaaaaaaaaaaaaaaaaaaaggatacagcagagcatcactggcaggaaagaacacaagattctgacaactaaagttgctgtttttctctttaattctcccagaaaaggaggtttatacctaaatgtgtgagggttggtaaaatacatgagataaacattttaacaactatgtaatgttaatcagcaaaataaaaaagtatttccagccctggcattccaagcaggcccatcccagttaggcccctgggggcaaagccagtggctcagtgtgcacttgggccagggccagttcaagttcgtcttctctataggccagtaagatgtgtttctttaaaaagatttcttaatctaaaaccagctgttgtctgctgtaggccagaacacgacattttaattagcatgattgttctgcttctgaaaccaggctctatggcatcccgaggacagatgatcctgacctaagcttatgggtgaggtttgctggttagcagctcagaaatacacgaacaataaagtggagtccctagcccactctgaatccatgaatcgccatcacctgctatatccctgtcttgaatttctacggtgactgtaccacctatctgttcatagggtaacatcacctttgaggttgtttcaagtgcctaggatataatgctccttctttaacataaattgttttatgctgtgttgcaagatctaacacccaatattcctgggagtaatgaggtactttaaatggagttgtaatgcctttaaagtccaatgactcctatgacgatgataaagtcacacagctctctagggctcacaatgaactcagatgaaagagttcctcttcccaaatcaaaggactctcaagattttaaaaaataaaaatttaaaaatgtaccctttgggagagaagctgcattagaaaccagccactaaggtagtgcattcgatgatgagcaaaagggcagaaatttgaagaaaccagggcaatatgacacatacacaatgccagcacagtccatagctttcagcagagatttcaatgtaagaccctcccctatacctgccccacatcttggaaaacaaactagaaaacccctagaaagattagaggtcctcactgtgcttgtcagcctctggtacctgggtgacaacagaaatatttttcctggctttctaccatatcgtccccaatattatgaatacatgagaccaaaatgctttcccatgtctcctactgaccagtacacattacccaaatcaaaagtatttggtaagcacctgtgtttgctgctgtcagaaactgaaaaaaatcacttcagtttctgcatttgcaaaatgaacatctgcagcttcagtttctgcatttgcaaaatgaacaaactggatgagatgatcgcttgccccctttggcaataatagtccatgattcgatcacttattcaaatgaaagaagacaaaactcttatgatttccacttccaactttgctacttctgaaactttctttgacctctcaaagtctggggaacacatctgaagtgactcttgatgaaactacagcataataactgcccaccttcatgtcactcaacagaacaatggatggtgtatgactgacgctgactggcaaaacaactaggtttctgtaattatatccatattctaagcaaattgttatgtattttgtgttttggggacatatgttgtggctaaagcccaaactgtggctaatcttaatatcagagccagataaatctgtttcgaatccataacatttaacattcgccagggtagatttgttcatcaactgggcttaaagaggtataattcacacatgtgcagtattagtaaatgctgaaatttaatgatttaaatataccagcaactgttgcaaagcagttgtatagcagcatttaacgttagccagaacctccctggctaatgttaagtttataccaaaagaatgagagaaattttggcatccccttgggatgggggtcacaattcccacaacttttacgggtaccagctagagcgactccttgcatggctagtacagaccctctgtttttctctgacaatacctttaaaacattgactggatctaatcaggaagcaaacagattcctctggaggtttctgagtcatctgttcttaaaatggttatgatttgggaccttcttacgcttgatgcagagggtatcagacattcctcctggcgtgtgttcccagacatgggcagaagactgttgtcaggccaaagacggagttaaatatatcaagggagaaaggtggttccttggactatcaggaattggtgtttaagacacagtagaaaaaggaataaaaaataattttaatcatatcaaaaagccaaaccaaagaggaatagctcatggaactgacaggatcctgactcagcggctggtgctcttcctgtgcacaagcccagcactccaggtcccaaggcatttatcaaatcccaccaagatgtttggcttttgcaccgaattctgggtttggttccctgaaagaactcattgatgtaaataactaaaagtgaggtctgggtaccctttacatgattccccagacctcaaatgggctaacacgcttctcttctccagcagtcttcctgtccgtgaagtttccttccagattgttacatggaactgaaaacaaagggagcctcagctggatttaaatctggagcatgccacaaagtcttccacttggcattttcgagaagaacccatcagagatcataagaaatacaagaacagaggttgcatagctcgaggtgcttggatattcattctaggttcttgttcttgagaaagtgggttaggtgggtgcatgccaagatccaagtaggtcaaccttccacccttaacctactactctgacatcagagtgctgggaggccttgttctctccctctgtcccagcctcacattcagacctccaccaatgacacgtttcataagctgccaatgttggggaagctcttcagcttctcaggaaagtcatctttgtacaggacagggtcagctcggtgttccaccaccttgagaggcatggtcccgaagactgaagcaaacttgttgatgcactctgacctctccaccatgtgtgtttggtctagtgaaagcccatctatggctgtgcactcaggacacttgaatttctttcgtggggttaccttgataactgcttttcccgtgacgttggccaccaggaagttcatggcaatatcttcacagttcatatgagcatctacccagttcttgatatccccaggcattttgtaggtatacaggtaattaaaatacttgtgataaaaagctgccccagtgagcaccatggacacttcattcgtccactcagactcatacttccacttattcatctcatggtcccagagatgcagacgacccgggtaacccaccaaccggtcaggaaattcccgccagacctcataaccaaattgcagctcgtcagaggtcagcataatgatatcatcatcaatggccagaacagcttctgtctcgatttcatcataagggaagaaacggttacttaacttgttttcagcagtcctcacaacttttaatggaacccggattttgggccagagagaatcttctggagggtttttattctgattattccagacgacaagtagtttggatagactgggcaccttggacacttcagtgatgacccggaagaggctctctactcggtcgtaggtgaggactatggcggtgaacccttgagactgtggtgggatcagcgggaggaagagtggattgctcacgctgccccacttcacagcaggagggtcattccattcttcataggagatggcagcatatggatagatccggtcattgataatctgcagggtggccagggcaatggctttaattgactggaagtacgcttcccagaaccaccgggcctgtctctgcatttcttcaatctgtctttgggggatgctctgcaaaatactgtacacatctgacatcttttcttctggtacaaccacagatgctctcttccagtcaagaacttcagagaaaggcaaaatataggagtctgcaatgacaaccgggacacagccagcttgtaacacatcgctcaatactgcctggcccagccgagctccacgaagaaccacacagaaagtagcctcctgtagcacctgtgggtaatcgaagacctggtgcttgtggcagcgcttacggacagaaaggacaccctctgagaggttggtgcatttatcgagtactaacactgactctccatgtttgacctggagggcttctaggtcctctctgtactcaggatggagacccacctgagatgacaggaggaagtattgccgtggacctggtcctttctctggaagatccacctcagctgacagtggactatagacaggaatgctgacatcgtagccttgccggtaagtccacgtagaaaagccgccaccagccaacagggccctgtctctggggacatccagggctgtgttataatctgggggacctccaggcaacatgttgaacaacaggtgattcgtacctcgatcccacctagagagctgggccatcgcttgtgctgtctccttgatgcgcagtgtgttctggttaagcacatcgatggagggaacaaacagacaggcccggttgatgtcatcagtgtagtagtcactgtctgagatggccatgagcagttcattatactcccgggagatggtgttgctgacagagacgccaaagtcatccacgtactttttcagagcatagatatacaccttgattttgttctttgggttgaagccacagcgatagacatcaaaacacgtgtgcattctgcaactgagatccccccgctctgggatgggactgtcggctggcagcctaacaaccggcacatcacggatgctgcgcttctctacattccagtcatttgaggactcgatagaatggggccaaaactgaaacatgccagtggcaatgaggcccaggaggacaatggagaagagggtgatatagtagattcggtgcttggtcttcattcttgggatgagggcaggaccccggatattatacttgaccgacgcacacataatgacacagacagcctcttcctcacactcctcggccacggctgcctcccgctcggccccgagcttggtcaccggctcatgccgcggggcgcgggccacctccgcccaggtcggatcggtccgaatcgccagccgccactgccagggccgagtctgggctggcgagcagcgagcgaggggccggtaaccgggatccgggccgtct

SEQ ID NO: 13668 - RNA, 7928 nt, Homo sapiens
  source 1..7928: mol_type = other RNA
gctgggattacaggcatgagccaccatgcccagccaaagactacattttcatgagaaaatgaatagttagcataacagaatgactgaataaatgttctcttccctcatctggatcagtaactagttggttggtcttcagctgtgctcaccagaaaaccaaatgttccttgagttgatgcttgggtatagtagccaatgatatatttgcagctataagtaaaattccaaataaatatattctaaagggaaggttctatatggtggcaaggcctgactggtggctttggtctaagacatatggatccctcctctgtcagccactcccacaccacctgcaattcctgagaggttgtccacaagatggggctttgctgaggaagcctctagcagacacagctgcctggtacttcttgagaactaccttgtcttctgtctgatagttctgtgcctttcagggagagtgggaagagatgcaaccagtggtccaaccaactgagagcagaagaaaggaaaaagtgctatcctgggccaggcatggtggttcacacctgtaatcccaacactttgggacgctgaggcaggaggatcacttgatcccaggagttagagaccagcctaggcaacatagtgaggccctgtctctccaaaaaaattaaaagatcagccaggtgtggtggtgcacgcttttagtctcagctacttggaaggctgagatgggaagactgcttgagtccaggagtttgaggctgcagcgagccatgatcacagcactacactccagcctatgggacagagtgagactctgtttccaaagaaaaaacaaaaaaaacaaaaacaaacaaacaaacaaacaaaaaaactctaccctgaaatggttgcaaatgtgaagaaacaaaatgccagatacagatgctggtgactcaactatttcttgaaaaggaaagaggcctggaagcttgggagagggggccaaactttctctggtcatcttcccactgttgccagcaatggtgagccggaaattgaaagaatgacacaaggttgcctgtacagacccacacaccctcccaggaaattggggaagctgggcatccctaacagtccatttaatggaggtggaaaagaggctgtggcttgagcttacaatgccctcacccagtcttcagatgaactcacagctcccaccctaaaatgagggggaaacattaaaatttagagtgggtcttgcctgcctgactttcctctgccaagataagctcaataaggcctgttcacagatgatgcatggctggtataatgggaccaaatgctgcccttgattctactcagaagtagaaagtgggtgagtaccaaacacaggccgaggacaggaggtccagggcttggacagagctcaggggtgaggtgagtaggggcaggccccacaggtttcatatgcctccaggccctgcagtggaaagctcaagttgctttcaaagtctctctggatggaagctgctgccaatatggttaacactcctgccagaactgctcctcaggaagtggctggaggagacatggggccagtttagcattctctactctgcctctctgtgccagggctgcttggggaacagcccactgtggcttctcttgctgcaatggaagagtacccgagccaagagaaatggaaaaagcagcatacccccaaaggagctacaaagcaaaggaaacacaccaggctcatgatgggtggctgatgggaagtctccaacacccaaagcctttactctatcagctgggtcctcacaggatctaactgcagagctaggaagagccttcccagaacccaaccacttcccaaacccagtctctgcttcatctactttctgattactatcttggctgaaaactatcaaaggttcttggattttaacctcaaatcaacttcagaacctgtggctagaaacgtgctatctttcagtgataaagacgctctagtttcctcctggcatggtgcctgtcagaggctatcatcctagaaggaagctaggatcacagggttattagcaacatctttggccaatgagagcaaagagggagcttgtctcttccagctcccagtctgcgtcagcacagaccagcatgatggtcactattttccaaaggcagcagagaaaccagcacttaaaaaccacaagttcaaagcccagctggaagtagatgaggctttggcagagaaaccagggtggtcagagctttgaacttgatgacactgagtaaaggatacagtggctgagcgtggggactcacgcccgtaatcccagcactttgggaggtcaaggcgtgcagatcacctgaggtcaggagttcgagaccagcctggctaacgtggtgaaaccctgcctctactaaaattacaaacaaattagccaggcgtggtggcaagcgcctgtaatcccagctactcaggaggctgaggcaggagaatcacttgaacctgggaggcggaggatgtagtgagccgagaccatgctattgttgcactccagcctgggtgacaagagcaagactctgtctcaaaaaaaaaaaaaaaaaaaaggatacagcagagcatcactggcaggaaagaacacaagattctgacaactaaagttgctgtttttctctttaattctcccagaaaaggaggtttatacctaaatgtgtgagggttggtaaaatacatgagataaacattttaacaactatgtaatgttaatcagcaaaataaaaaagtatttccagccctggcattccaagcaggcccatcccagttaggcccctgggggcaaagccagtggctcagtgtgcacttgggccagggccagttcaagttcgtcttctctataggccagtaagatgtgtttctttaaaaagatttcttaatctaaaaccagctgttgtctgctgtaggccagaacacgacattttaattagcatgattgttctgcttctgaaaccaggctctatggcatcccgaggacagatgatcctgacctaagcttatgggtgaggtttgctggttagcagctcagaaatacacgaacaataaagtggagtccctagcccactctgaatccatgaatcgccatcacctgctatatccctgtcttgaatttctacggtgactgtaccacctatctgttcatagggtaacatcacctttgaggttgtttcaagtgcctaggatataatgctccttctttaacataaattgttttatgctgtgttgcaagatctaacacccaatattcctgggagtaatgaggtactttaaatggagttgtaatgcctttaaagtccaatgactcctatgacgatgataaagtcacacagctctctagggctcacaatgaactcagatgaaagagttcctcttcccaaatcaaaggactctcaagattttaaaaaataaaaatttaaaaatgtaccctttgggagagaagctgcattagaaaccagccactaaggtagtgcattcgatgatgagcaaaagggcagaaatttgaagaaaccagggcaatatgacacatacacaatgccagcacagtccatagctttcagcagagatttcaatgtaagaccctcccctatacctgccccacatcttggaaaacaaactagaaaacccctagaaagattagaggtcctcactgtgcttgtcagcctctggtacctgggtgacaacagaaatatttttcctggctttctaccatatcgtccccaatattatgaatacatgagaccaaaatgctttcccatgtctcctactgaccagtacacattacccaaatcaaaagtatttggtaagcacctgtgtttgctgctgtcagaaactgaaaaaaatcacttcagtttctgcatttgcaaaatgaacatctgcagcttcagtttctgcatttgcaaaatgaacaaactggatgagatgatcgcttgccccctttggcaataatagtccatgattcgatcacttattcaaatgaaagaagacaaaactcttatgatttccacttccaactttgctacttctgaaactttctttgacctctcaaagtctggggaacacatctgaagtgactcttgatgaaactacagcataataactgcccaccttcatgtcactcaacagaacaatggatggtgtatgactgacgctgactggcaaaacaactaggtttctgtaattatatccatattctaagcaaattgttatgtattttgtgttttggggacatatgttgtggctaaagcccaaactgtggctaatcttaatatcagagccagataaatctgtttcgaatccataacatttaacattcgccagggtagatttgttcatcaactgggcttaaagaggtataattcacacatgtgcagtattagtaaatgctgaaatttaatgatttaaatataccagcaactgttgcaaagcagttgtatagcagcatttaacgttagccagaacctccctggctaatgttaagtttataccaaaagaatgagagaaattttggcatccccttgggatgggggtcacaattcccacaacttttacgggtaccagctagagcgactccttgcatggctagtacagaccctctgtttttctctgacaatacctttaaaacattgactggatctaatcaggaagcaaacagattcctctggaggtttctgagtcatctgttcttaaaatggttatgatttgggaccttcttacgcttgatgcagagggtatcagacattcctcctggcgtgtgttcccagacatgggcagaagactgttgtcaggccaaagacggagttaaatatatcaagggagaaaggtggttccttggactatcaggaattggtgtttaagacacagtagaaaaaggaataaaaaataattttaatcatatcaaaaagccaaaccaaagaggaatagctcatggaactgacaggatcctgactcagcggctggtgctcttcctgtgcacaagcccagcactccaggtcccaaggcatttatcaaatcccaccaagatgtttggcttttgcaccgaattctgggtttggttccctgaaagaactcattgatgtaaataactaaaagtgaggtctgggtaccctttacatgattccccagacctcaaatgggctaacacgcttctcttctccagcagtcttcctgtccgtgaagtttccttccagattgttacatggaactgaaaacaaagggagcctcagctggatttaaatctggagcatgccacaaagtcttccacttggcattttcgagaagaacccatcagagatcataagaaatacaagaacagaggttgcatagctcgaggtgcttggatattcattctaggttcttgttcttgagaaagtgggttaggtgggtgcatgccaagatccaagtaggtcaaccttccacccttaacctactactctgacatcagagtgctgggaggccttgttctctccctctgtcccagcctcacattcagacctccaccaatgacacgtttcataagctgccaatgttggggaagctcttcagcttctcaggaaagtcatctttgtacaggacagggtcagctcggtgttccaccaccttgagaggcatggtcccgaagactgaagcaaacttgttgatgcactctgacctctccaccatgtgtgtttggtctagtgaaagcccatctatggctgtgcactcaggacacttgaatttctttcgtggggttaccttgataactgcttttcccgtgacgttggccaccaggaagttcatggcaatatcttcacagttcatatgagcatctacccagttcttgatatccccaggcattttgtaggtatacaggtaattaaaatacttgtgataaaaagctgccccagtgagcaccatggacacttcattcgtccactcagactcatacttccacttattcatctcatggtcccagagatgcagacgacccgggtaacccaccaaccggtcaggaaattcccgccagacctcataaccaaattgcagctcgtcagaggtcagcataatgatatcatcatcaatggccagaacagcttctgtctcgatttcatcataagggaagaaacggttacttaacttgttttcagcagtcctcacaacttttaatggaacccggattttgggccagagagaatcttctggagggtttttattctgattattccagacgacaagtagtttggatagactgggcaccttggacacttcagtgatgacccggaagaggctctctactcggtcgtaggtgaggactatggcggtgaacccttgagactgtggtgggatcagcgggaggaagagtggattgctcacgctgccccacttcacagcaggagggtcattccattcttcataggagatggcagcatatggatagatccggtcattgataatctgtgaatcccactgttccctaggccagatcagggagttcatttggtgattagcagctgaccagttctctctcctggctggttccatgaagagctgtctctgcatttcttcaatctgtctttgggggatgctctgcaaaatactgtacacatctgacatcttttcttctggtacaaccacagatgctctcttccagtcaagaacttcagagaaaggcaaaatataggagtctgcaatgacaaccgggacacagccagcttgtaacacatcgctcaatactgcctggcccagccgagctccacgaagaaccacacagaaagtagcctcctgtagcacctgtgggtaatcgaagacctggtgcttgtggcagcgcttacggacagaaaggacaccctctgagaggttggtgcatttatcgagtactaacactgactctccatgtttgacctggagggcttctaggtcctctctgtactcaggatggagacccacctgagatgacaggaggaagtattgccgtggacctggtcctttctctggaagatccacctcagctgacagtggactatagacaggaatgctgacatcgtagccttgccggtaagtccacgtagaaaagccgccaccagccaacagggccctgtctctggggacatccagggctgtgttataatctgggggacctccaggcaacatgttgaacaacaggtgattcgtacctcgatcccacctagagagctgggccatcgcttgtgctgtctccttgatgcgcagtgtgttctggttaagcacatcgatggagggaacaaacagacaggcccggttgatgtcatcagtgtagtagtcactgtctgagatggccatgagcagttcattatactcccgggagatggtgttgctgacagagacgccaaagtcatccacgtactttttcagagcatagatatacaccttgattttgttctttgggttgaagccacagcgatagacatcaaaacacgtgtgcattctgcaactgagatccccccgctctgggatgggactgtcggctggcagcctaacaaccggcacatcacggatgctgcgcttctctacattccagtcatttgaggactcgatagaatggggccaaaactgaaacatgccagtggcaatgaggcccaggaggacaatggagaagagggtgatatagtagattcggtgcttggtcttcattcttgggatgagggcaggaccccggatattatacttgaccgacgcacacataatgacacagacagcctcttcctcacactcctcggccacggctgcctcccgctcggccccgagcttggtcaccggctcatgccgcggggcgcgggccacctccgcccaggtcggatcggtccgaatcgccagccgccactgccagggccgagtctgggctggcgagcagcgagcgaggggccggtaaccgggatccgggccgtct

SEQ ID NO: 13669 - RNA, 1999 nt, Homo sapiens
  source 1..1999: mol_type = other RNA
gctgggattacaggcatgagccaccatgcccagccaaatttttttttttttttaagggaagggatcttgctatgttgcccaggctggtctcaaactcctcagctcaagcaatctgcccacctcagcctctgaaagtgctgggattacaggcatgagccaccatgtccagcacactttaatattcactatgggccctcaaaaggaaatgtttgtggggccaccaaaagcaaatgtctcttgaacctagtcacctggggggacaagtgtgggaaagtgcacctgtgttcccatgagacccactcaagaggagcagaaatcctgttttgctatttccttaattgctactagggctgggattttttcatgtttattggcccctctacatttttttctttaaaaaaattcacaaagcatgtttatatttgttagctcttttgattctccctatgatagtgtgaagacagggacaaaacgctaccatttcacactcccagatctaacaatagctaccaagtaattatgccatgcgtttcttctaaccttcgcaatatcactacgaggtagttcttactatcctcattttacagataaggaaactgaggctaagtgacgctggcagacttgcccaaggccacacagctggtaacagggactggtagtcacttgagtcctacatgagcacccttgctactacagcagctcctcccctttctagaggcctagatggaaagatgctggtgtcagcggggggcacaaaggtccacccagtcccacacatgcagagaggcatcatttgttgctgataacaaagtccttggtctgcagggatgccaggtgtgggtggtgaccaaaggagcagggtccatcccatttccatctaggaagatgtgacctctgtgagtgaagagaggttctacttggctccgtgttccatcttggctccgtgttccatcccaagatgtggcatcatagacctggactgtaccatcaaaacctgagatggccaagcaattcttcaggcctggggcccaagtcactcgcagcagctctgggtcagggctaggtacggatactgggcactggactgagctcacaggatggcagagatcccgggggtcaagaagacaaagacgcccatctgagccaaggctggcaatgctgggcccagggccctggccccagctcccaacttcagcacaccatctctctccaccagacccagggccagggctgcgattctccaacggtgcccacttctgccgggtgtcaacaagccccagccggcctgaagcacagcagaaggcaaaggtgtctgcatctaggacctgcaggctactcagctcctcactgtcactgacatcattgtctgctcagctggttgggtgctggtccctgggactgcctaatcctgccccagcataggagcccttagaggccagggcttacctcttattcactgtgtatccccaacacctgaggtgtacgtggtcttccgggactccagatcaacgacctgcagacttcggagcctcgccccatggaggactccgggtgccaatgtggagaagacggccaccctaggccagagactctcctctttctcatgcacagcaatggtgctgacagctttaatgacatcactgtcctctgcaacctgccacacctgcagataacaacctggaaggccactggtaaccagcaatctggtatgtggcacatgctttagatcaaagatagacctgtctgaaaatcctccatggcgcactttgaaatctctttctgggaataagcccttgttttcctttacagaaagtctgagaggtaatttcagatgaagaatttcattctttttcaggctttcatagccagcaacaaagactcctttgtcatcaatccattcaaggactcgagtggctcctgacaggtcgaatgcatagaaatcctggtacaagcgcaaggattccaccagccagtcgtccccaggatccatggcaacgac

SEQ ID NO: 13670 - RNA, 1886 nt, Homo sapiens
  source 1..1886: mol_type = other RNA
gctgggattacaggcatgagccaccatgcccagccaaatttttttttttttttaagggaagggatcttgctatgttgcccaggctggtctcaaactcctcagctcaagcaatctgcccacctcagcctctgaaagtgctgggattacaggcatgagccaccatgtccagcacactttaatattcactatgggccctcaaaaggaaatgtttgtggggccaccaaaagcaaatgtctcttgaacctagtcacctggggggacaagtgtgggaaagtgcacctgtgttcccatgagacccactcaagaggagcagaaatcctgttttgctatttccttaattgctactagggctgggattttttcatgtttattggcccctctacatttttttctttaaaaaaattcacaaagcatgtttatatttgttagctcttttgattctccctatgatagtgtgaagacagggacaaaacgctaccatttcacactcccagatctaacaatagctaccaagtaattatgccatgcgtttcttctaaccttcgcaatatcactacgaggtagttcttactatcctcattttacagataaggaaactgaggctaagtgacgctggcagacttgcccaaggccacacagctggtaacagggactggtagtcacttgagtcctacatgagcacccttgctactacagcagctcctcccctttctagaggcctagatggaaagatgctggtgtcagcggggggcacaaaggtccacccagtcccacacatgcagagaggcatcatttgttgctgataacaaagtccttggtctgcagggatgccaggtgtgggtggtgaccaaaggagcagggtccatcccatttccatctaggaagatgtgacctctgtgagtgaagagaggttctacttggctccgtgttccatcttggctccgtgttccatcccaagatgtggcatcatagacctggactgtaccatcaaaacctgagatggccaagcaattcttcaggcctggggcccaagtcactcgcagcagctctgggtcagggctaggtacggatactgggcactggactgagctcacaggatggcagagatcccgggggtcaagaagacaaagacgcccatctgagccaaggctggcaatgctgggcccagggccctggccccagctcccaacttcagcacaccatctctctccaccagacccagggccagggctgcgattctccaacggtgcccacttctgccgggtgtcaacaagccccagccggcctgaagcacagcagaaggcaaaggtgtctgcatctaggacctgcaggctactcagctcctcactgtcactgacatctgaggtgtacgtggtcttccgggactccagatcaacgacctgcagacttcggagcctcgccccatggaggactccgggtgccaatgtggagaagacggccaccctaggccagagactctcctctttctcatgcacagcaatggtgctgacagctttaatgacatcactgtcctctgcaacctgccacacctgcagataacaacctggaaggccactggtaaccagcaatctggtatgtggcacatgctttagatcaaagatagacctgtctgaaaatcctccatggcgcactttgaaatctctttctgggaataagcccttgttttcctttacagaaagtctgagaggtaatttcagatgaagaatttcattctttttcaggctttcatagccagcaacaaagactcctttgtcatcaatccattcaaggactcgagtggctcctgacaggtcgaatgcatagaaatcctggtacaagcgcaaggattccaccagccagtcgtccccaggatccatggcaacgac

SEQ ID NO: 13671 - RNA, 2420 nt, Homo sapiens
  source 1..2420: mol_type = other RNA
gctgggattacaggcatgagccaccatgcccagccaaatttttttttttttttaagggaagggatcttgctatgttgcccaggctggtctcaaactcctcagctcaagcaatctgcccacctcagcctctgaaagtgctgggattacaggcatgagccaccatgtccagcacactttaatattcactatgggccctcaaaaggaaatgtttgtggggccaccaaaagcaaatgtctcttgaacctagtcacctggggggacaagtgtgggaaagtgcacctgtgttcccatgagacccactcaagaggagcagaaatcctgttttgctatttccttaattgctactagggctgggattttttcatgtttattggcccctctacatttttttctttaaaaaaattcacaaagcatgtttatatttgttagctcttttgattctccctatgatagtgtgaagacagggacaaaacgctaccatttcacactcccagatctaacaatagctaccaagtaattatgccatgcgtttcttctaaccttcgcaatatcactacgaggtagttcttactatcctcattttacagataaggaaactgaggctaagtgacgctggcagacttgcccaaggccacacagctggtaacagggactggtagtcacttgagtcctacatgagcacccttgctactacagcagctcctcccctttctagaggcctagatggaaagatgctggtgtcagcggggggcacaaaggtccacccagtcccacacatgcagagaggcatcatttgttgctgataacaaagtccttggtctgcagggatgccaggtgtgggtggtgaccaaaggagcagggtccatcccatttccatctaggaagatgtgacctctgtgagtgaagagaggttctacttggctccgtgttccatcttggctccgtgttccatcccaagatgtggcatcatagacctggactgtaccatcaaaacctgagatggccaagcaattcttcaggcctggggcccaagtcactcgcagcagctctgggtcagggctaggtacggatactgggcactggactgagctcacaggatggcagagatcccgggggtcaagaagacaaagacgcccatctgagccaaggctggcaatgctgggcccagggccctggccccagctcccaacttcagcacaccatctctctccaccagacccagggccagggctgcgattctccaacggtgcccacttctgccgggtgtcaacaagccccagccggcctgaagcacagcagaaggcaaaggtgtctgcatctaggacctgcaggctactcagctcctcactgtcactgacatctgaggtgtacgtggtcttccgggactccagatcaacgacctgcagacttcggagcctcgccccatggaggactccgggtgccaatgtggagaagacggccaccctaggccagagactctcctctttctcatgcacagcaatggtgctgacagctttaatgacatcactgtcctctgcaacctgccacacctgcagataacaacctggaaggccactggtaaccagcaatctggtatgtggcacatgctttagatcaaagatagacctgtctgaaaatcctccatggcgcactttgaaatctctttctgggaataagcccttgttttcctttacagaaagtctgagaggtaatttcagatgaagaatttcattctttttcaggctttcatagccagcaacaaagactcctttgtcatcaatccattcaaggactcgagtggctcctgacaggtcgaatgcatagaaatcctggtacctgcacaaaagggacacagaatcacacgatgcacagcacttcacagctcaaagaactccaagatggcagccgcatggttcagtggcccaaactctggagtcaggcagacgtgggactgagtttacttcccattttactccctgtttctgggaccaggccagtcccttgatgtccctgagcctcggtcctcatgtgtggacgtcccagggtacccagatttcccaaggttgacgtgaggaatcaatgagatcatctgtgttctgagctgaactcagaggctggcgcaaactaactgggcactgcgtcttcacaagcgcggctcttactagtaatctcacaacgcgcgcacgcaggaaggagccatttcctagagatgggggcctaggcccaggcggagtcctccacggtggcgagccccgaggccacagctggcccactctgcaccaggatccccaacgtgcctccacccacacccatccgcccgccaggcaagctccaggcccagctcccatgtcccagccccgtacgatttacaagcgcaaggattccaccagccagtcgtccccaggatccatggcaacgac

SEQ ID NO: 13672 - RNA, 1893 nt, Homo sapiens
  source 1..1893: mol_type = other RNA
gctgggattacaggcatgagccaccatgcccagccaaatttttttttttttttaagggaagggatcttgctatgttgcccaggctggtctcaaactcctcagctcaagcaatctgcccacctcagcctctgaaagtgctgggattacaggcatgagccaccatgtccagcacactttaatattcactatgggccctcaaaaggaaatgtttgtggggccaccaaaagcaaatgtctcttgaacctagtcacctggggggacaagtgtgggaaagtgcacctgtgttcccatgagacccactcaagaggagcagaaatcctgttttgctatttccttaattgctactagggctgggattttttcatgtttattggcccctctacatttttttctttaaaaaaattcacaaagcatgtttatatttgttagctcttttgattctccctatgatagtgtgaagacagggacaaaacgctaccatttcacactcccagatctaacaatagctaccaagtaattatgccatgcgtttcttctaaccttcgcaatatcactacgaggtagttcttactatcctcattttacagataaggaaactgaggctaagtgacgctggcagacttgcccaaggccacacagctggtaacagggactggtagtcacttgagtcctacatgagcacccttgctactacagcagctcctcccctttctagaggcctagatggaaagatgctggtgtcagcggggggcacaaaggtccacccagtcccacacatgcagagaggcatcatttgttgctgataacaaagtccttggtctgcagggatgccaggtgtgggtggtgaccaaaggagcagggtccatcccatttccatctaggaagatgtgacctctgtgagtgaagagaggttctacttggctccgtgttccatcttggctccgtgttccatcccaagatgtggcatcatagacctggactgtaccatcaaaacctgagatggccaagcaattcttcaggcctggggcccaagtcactcgcagcagctctgggtcagggctaggtacggatactgggcactggactgagctcacaggatggcagagatcccgggggtcaagaagacaaagacgcccatctgagccaaggctggcaatgctgggcccagggccctggccccagctcccaacttcagcacaccatctctctccaccagacccagggccagggctgcgattctccaacggtgcccacttctgccgggtgtcaacaagccccagccggcctgaagcacagcagaaggcaaaggtgtctgcatctaggacctgcaggctactcagctcctcactgtcactgacatctgaggtgtacgtggtcttccgggactccagatcaacgacctgcagacttcggagcctcgccccatggaggactccgggtgccaatgtggagaagacggccaccctaggccagagactctcctctttctcatgcacagcaatggtgctgacagctttaatgacatcactgtcctctgcaacctgccacacctgcagataacaacctggaaggccactggtaaccagcaatctggtatgtggcacatgctttagatcaaagatagacctgtctgaaaatcctccatggcgcactttgaaatctctttctgggaataagcccttgttttcctttacagaaagtctgagaggtaatttcagatgaagaatttcattctttttcaggctttcatagccagcaacaaagactcctttgtcatcaatccattcaaggactcgagtggctcctgacaggtcgaatgcatagaaatcctggtacgatttacaagcgcaaggattccaccagccagtcgtccccaggatccatggcaacgac

SEQ ID NO: 13673 - RNA, 1797 nt, Homo sapiens
  source 1..1797: mol_type = other RNA
gctgggattacaggcatgagccaccatgcccagccaaatttttttttttttttaagggaagggatcttgctatgttgcccaggctggtctcaaactcctcagctcaagcaatctgcccacctcagcctctgaaagtgctgggattacaggcatgagccaccatgtccagcacactttaatattcactatgggccctcaaaaggaaatgtttgtggggccaccaaaagcaaatgtctcttgaacctagtcacctggggggacaagtgtgggaaagtgcacctgtgttcccatgagacccactcaagaggagcagaaatcctgttttgctatttccttaattgctactagggctgggattttttcatgtttattggcccctctacatttttttctttaaaaaaattcacaaagcatgtttatatttgttagctcttttgattctccctatgatagtgtgaagacagggacaaaacgctaccatttcacactcccagatctaacaatagctaccaagtaattatgccatgcgtttcttctaaccttcgcaatatcactacgaggtagttcttactatcctcattttacagataaggaaactgaggctaagtgacgctggcagacttgcccaaggccacacagctggtaacagggactggtagtcacttgagtcctacatgagcacccttgctactacagcagctcctcccctttctagaggcctagatggaaagatgctggtgtcagcggggggcacaaaggtccacccagtcccacacatgcagagaggcatcatttgttgctgataacaaagtccttggtctgcagggatgccaggtgtgggtggtgaccaaaggagcagggtccatcccatttccatctaggaagatgtgacctctgtgagtgaagagaggttctacttggctccgtgttccatcttggctccgtgttccatcccaagatgtggcatcatagacctggactgtaccatcaaaacctgagatggccaagcaattcttcaggcctggggcccaagtcactcgcagcagctctgggtcagggctaggtacggatactgggcactggactgagctcacaggatggcagagatcccgggggtcaagaagacaaagacgcccatctgagccaaggctggcaatgctgggcccagggccctggccccagctcccaacttcagcacaccatctctctccaccagacccagggccagggctgcgattctccaacggtgcccacttctgccgggtgtcaacaagccccagccggcctgaagcacagcagaaggcaaaggtgtctgcatctaggacctgcaggctactcagctcctcactgtcactgacatctgaggtgtacgtggtcttccgggactccagatcaacgacctgcagacttcggagcctcgccccatggaggactccgggtgccaatgtggagaagacggccaccctaggccagagactctcctctttctcatgcacagcaatggtgctgacagctttaatgacatcactgtcctctgcaacctgccacacctgcagataacaacctggaaggccactggtaaccagcaatcttgttttcctttacagaaagtctgagaggtaatttcagatgaagaatttcattctttttcaggctttcatagccagcaacaaagactcctttgtcatcaatccattcaaggactcgagtggctcctgacaggtcgaatgcatagaaatcctggtacaagcgcaaggattccaccagccagtcgtccccaggatccatggcaacgac

SEQ ID NO: 13674 - RNA, 1492 nt, Homo sapiens
  source 1..1492: mol_type = other RNA
gctgggattacaggcatgagccaccatgcccagccagacatcttaatatgcactatctactatattataggctcttgagaaacatttcattccacagaatggttctgatttatccccagtgttgatgctaccaagaggaaaagattcactacaaaggtagttcaccttttaccaagtgtcaaatattctatattacctttgaaaaccagagattataggtattaatcccactgattcaactgtgtatatatatacacatatatacgtatatatgtgtatatatatacacacatatatatgtatacacatatatgtatacatacatacgtatatatacacatacatgtatacatacatactatatatacacatatgtatacatacatacgtatatatacacatatatgtatacatacgtatatatacacatatatatgtatacatatatatgaacacatatatgtgtgtgtgtatatatatatatatataagatttttcttgaccatgaatcaccatgtttgggagtacagtagggttaggaattacaatttactgatcccctatcatgtgccagacacaattatcaggtaaggaacttcaaaccctgcattctttttttataaaactatactccaaaaaagtgattgcttggtcatttctgcagattcaattagacattatacacacaaacacacccatgagaccgcatggcactgggaagattacccactatttcccacttattaagatctggatcatatttctcaatgctctgaagatacgttccctttgagtaggagtatcctccagtgacataaatacatccattcatgatgacggcaccgcactccatcctcctttccatcatgggagctatctctctccattcattttgttcagggtcatagcattctgtgattgtagtttgtccgccgactagatagagcttattttcaaacggaactgagcacaatccatattctggatgtggactggaggtgatgaggctccattcgttgatatcggaattgtagctctgaactttgtcataggtgcagcttcctctgtagccacagtggccaccaatgacgtagataacatcatgtaagacacaggcagtagcatttcccacacccaacttagtatttccaagacaatcttacttcagcattgggattaggataaacaatcatgacaatcttcagttttaaacatcagccagttgttttcaaatattactcctattctatatacagggaacagagtcttctggtttggagcaaaataatggaaacttcttaactccagcattattacgtggaacatctgatagaaaacccagtcccgccgtcggcagccgccccggcgcccgtgacgctcctgcgggttcagtcctttggcctcgccccacgcctgccctctcggcagccccactcacaagcccagctcgcaagcgcaggcgcctctcttctctagcccgaccgccaactgc

SEQ ID NO: 13675 - RNA, 2707 nt, Homo sapiens
  source 1..2707: mol_type = other RNA
gctgggattacaggcatgagccaccatgcccagccagacatcttaatatgcactatctactatattataggctcttgagaaacatttcattccacagaatggttctgatttatccccagtgttgatgctaccaagaggaaaagattcactacaaaggtagttcaccttttaccaagtgtcaaatattctatattacctttgaaaaccagagattataggtattaatcccactgattcaactgtgtatatatatacacatatatacgtatatatgtgtatatatatacacacatatatatgtatacacatatatgtatacatacatacgtatatatacacatacatgtatacatacatactatatatacacatatgtatacatacatacgtatatatacacatatatgtatacatacgtatatatacacatatatatgtatacatatatatgaacacatatatgtgtgtgtgtatatatatatatatataagatttttcttgaccatgaatcaccatgtttgggagtacagtagggttaggaattacaatttactgatcccctatcatgtgccagacacaattatcaggtaaggaacttcaaaccctgcattctttttttataaaactatactccaaaaaagtgattgcttggtcatttctgcagattcaattagacattatacacacaaacacacccatgagaccgcatggcactgggaagattacccactatttcccacttattaagatctggatcatatttctcaatgctctgaagatacgttccctttgagtaggagtatcctccagtgacataaatacatccattcatgatgacggcaccgcactccatcctcctttccatcatgggagctatctctctccattcattttgttcagggtcatagcattctgtgattgtagtttgtccgccgactagatagagcttattttcaaacggaactgagcacaatccatattctggatgtggactggaggtgatgaggctccattcgttgatatcggaattgtagctctgaactttgtcataggtgcagcttcctctgtagccacagtggccaccaatgacgtagataacatcatgtaagacacaggcagtagcatttcccacacctttaatcatgtttgcaataggaatccatttctcttttaaaggatcatagaactcagcctcttctgctggagccccttttctgtaaccacctaaagcatagacacagccacccaaggtgactgcacagtggtaatacctggcattgagcattggcaaaccttctgtccattcatcactttcactgttatagatccacactgtgtcaagagcttctatgttatccgtcctgtagcccccagttacataaatgttgggtcctaaacatgtaacaccatagctctccctggtataatctggtatttctgctccctgaatccaaacatttgtcaaaggatcccatatgtgaacctctgataaaggatgccagtaatagcctccaattatatacattgtggctgtggacctctgggaaatctctttatgcatgggattcaaggcattgtatattagggagcggatcttattttcggtgagcaggcagcttctttgaaggcctaaggctgtttttaagtacactggatctatatcaatgttgatatagctcagtagattatagaggcattcaattcgattttctacatcatgagcagtccacttaataactggctctatgatagcttcttctttccaaacactgagattctttctggacaagataaagagaaacttttcaaggctgatttccagaaattcttcttgttgccacacttccttaaactttgaacatagaattcttcgagattccttctctagttctggacacacatgaaattctgcaaaggagtgcattccaatacaattatcaatatccaagtgccttaccaaaaaccgctcacaagccttctttactgaaaggaactgtagcagatccgctgcctcaagcaggctttgaacatttcttttagttatttcaatttgggaagtgtatgcataatttacaaggccttccagaatatcatggtggatgccagagagttttattttatttttaaatttttctttcatgtcagctgtgaacattgccttaaaataattgctgcaagcagctaaaacggctcggtgacaatggaaaattatgcctgaaggacactgaagagtaatatcagtaaataatccatccaagtaaaatgttctgaatgcatccagaaaatccactggatgtgttgaatccttgaaaagataaatataatcttcttgtccttttagagccatggccaacttagtatttccaagacaatcttacttcagcattgggattaggataaacaatcatgacaatcttcagttttaaacatcagccagttgttttcaaatattactcctattctatatacagggaacagagtcttctggtttggagcaaaataatggaaacttcttaactccagcattattacgtggaacatctgatagaaaacccagtcccgccgtcggcagccgccccggcgcccgtgacgctcctgcgggttcagtcctttggcctcgccccacgcctgccctctcggcagccccactcacaagcccagctcgcaagcgcaggcgcctctcttctctagcccgaccgccaactgc

SEQ ID NO: 13676 - RNA, 2605 nt, Homo sapiens
  source 1..2605: mol_type = other RNA
gctgggattacaggcatgagccaccatgcccagccagacatcttaatatgcactatctactatattataggctcttgagaaacatttcattccacagaatggttctgatttatccccagtgttgatgctaccaagaggaaaagattcactacaaaggtagttcaccttttaccaagtgtcaaatattctatattacctttgaaaaccagagattataggtattaatcccactgattcaactgtgtatatatatacacatatatacgtatatatgtgtatatatatacacacatatatatgtatacacatatatgtatacatacatacgtatatatacacatacatgtatacatacatactatatatacacatatgtatacatacatacgtatatatacacatatatgtatacatacgtatatatacacatatatatgtatacatatatatgaacacatatatgtgtgtgtgtatatatatatatatataagatttttcttgaccatgaatcaccatgtttgggagtacagtagggttaggaattacaatttactgatcccctatcatgtgccagacacaattatcaggtaaggaacttcaaaccctgcattctttttttataaaactatactccaaaaaagtgattgcttggtcatttctgcagattcaattagacattatacacacaaacacacccatgagaccgcatggcactgggaagattacccactatttcccacttattaagatctggatcatatttctcaatgctctgaagatacgttccctttgagtaggagtatcctccagtgacataaatacatccattcatgatgacggcaccgcactccatcctcctttccatcatgggagctatctctctccattcattttgttcagggtcatagcattctgtgattgtagtttgtccgccgactagatagagcttattttcaaacggaactgagcacaatccatattctggatgtggactggaggtgatgaggctccattcgttgatatcggaattgtagctctgaactttgtcataggtgcagcttcctctgtagccacagtggccaccaatgacgtagataacatcatgtaagacacaggcagtagcatttcccacacctttaatcatgtttgcaataggaatccatttctcttttaaaggatcatagaactcagcctcttctgctggagccccttttctgtaaccacctaaagcatagacacagccacccaaggtgactgcacagtggtaatacctggcattgagcattggcaaaccttctgtccattcatcactttcactgttatagatccacactgtgtcaagagcttctatgttatccgtcctgtagcccccagttacataaatgttgggtcctaaacatgtaacaccatagctctccctggtataatctggtatttctgctccctgaatccaaacatttgtcaaaggatcccatatgtgaacctctgataaaggatgccagtaatagcctccaattatatacattgtggctgtggacctctgggaaatctctttatgcatgggattcaaggcattgtatattagggagcggatcttattttcggtgagcaggcagcttctttgaaggcctaaggctgtttttaagtacactggatctatatcaatgttgatatagctcagtagattatagaggcattcaattcgattttctacatcatgagcagtccacttaataactggctctatgatagcttcttctttccaaacactgagattctttctggacaagataaagagaaacttttcaaggctgatttccagaaattcttcttgttgccacacttccttaaactttgaacatagaattcttcgagattccttctctagttctggacacacatgaaattctgcaaaggagtgcattccaatacaattatcaatatccaagtgccttaccaaaaaccgctcacaagccttctttactgaaaggaactgtagcagatccgctgcctcaagcaggctttgaacatttcttttagttatttcaatttgggaagtgtatgcataatttacaaggccttccagaatatcatggtggatgccagagagttttattttatttttaaatttttctttcatgtcagctgtgaacattgccttaaaataattgctgcaagcagctaaaacggctcggtgacaatggaaaattatgcctgaaggacactgaagagtaatatcagtaaataatccatccaagtaaaatgttctgaatgcatccagaaaatccactggatgtgttgaatccttgaaaagataaatataatcttcttgtccttttagagccatggctcccgccggggctcgggacgcggcgctggcccgcgggctagtagcgagcgggagcggggacgcctccggcccctctgaccatctttggaagaggcgctcggaagccgccagctagtgccgctccaccccacaagcagctcctattttggtgtcccggcggctcccccgcctccacccgaacagccccccgcacggtctgggcgcgaggccactcgcgggaactcccccgtcgccgggccgtgcggcgagcggggc

SEQ ID NO: 13677 - RNA, 3921 nt, Homo sapiens
  source 1..3921: mol_type = other RNA
gctgggattacaggcatgagccaccatgcccagcccacgttaacattttttatgaagaataacttccaaaacaatccaaggagaagggtggcattttacagtctctttagtatcttgttataataaacagttgaattcttacagctgcttctacatccaaacttttttgttgaagtaagttgacttcacacagatacgcagttggaaaagtttttaaaatagccttttcagctaattgtggctattctttgataccacaccaagactacaagtgattttttttttttttttttttttttgaaatggagtctcgctctgtcacccaggctggagtccagtggcacgatctcgactcactgcaacctccacctcccgggttcaagctattctcctgcctcagcctcccgagtagctgggactacaagggatctgccaccacgcccggctaatttttgtaattttagtagagacggactttcaccatattggccaggctggtcttgaactcctgaccttgtgatccacccaccttggcctcccaaagtgttgggattacaggcgtgagccaccgcgcccggcttactacaagtcatagtttcttaaaggcaatgtagactccgaaaacttaatgcactcttatattgttaatacattaaaatccactggcctgtcttacacttttgaatcaatctttgagccatgcatgattttgtaacatcacgtactggtcacttggaaaaatggttcattgaattcttccaaatgaaatgcatttcattatacaaatcacatttgttaatatccccaacaataaagctcatggtggagtacagattttcggaaattccaatttttgcttgaaagctttatcactggcaacactatcagttgtttcccttgaggtgagaggctcattccattaatttccagaaaatatcagccaaatattcaagtctaaataccgtaatctgctagttctttcaattctaaagggcatgccttgaacacagccaattcagcttgcaactcaactgtgtaactgcttttcctcaaggcacccatacttcagtgcacagcagaggggctttatgcatgcttccagttttctcagaatattataaattctcaaggtcaactttttttttctttttgagacagggtttcactcttgttgcctgggctggagtgcaatggtatgatctcggctcactgcaacctccacctaccggattcaagcgattctcttgcctcagcctcccgagtagctggaattacaggcatgcaccaccatgcccagctaattttgtatttttagaagagacggggtttctccatgttggtcaggctggcctcgaactcccgacctcaggtgatccgcccgcctcagcctcccaaagtgctgggattacaggcatgagccactgcgctggctaggtcaacatttaatagttaaccattgctatttgttctatcaaggacatatcaaaactactagaagtttgctgccaccaccttgattcatgccacagtgccaacagttgacctcacagatcctccctgaaagggtcttgggactcccaggatctgcaggccgcattcttcgagaaccactattctaggtacagccccactgtccttctaaaatctaaggtcacagcttaaacttcagggaaggctgtagttttggaggccattgtcacattagaacccatttagaagtgactgtcaagagacaacttgagtgagtctgaaactgcctgctgatggcagtgtttctcaactggtttaaatcgccagtcccctaggaagccttcttcctgatcactccctgccatgaaaatggaatatcacagacacactatatgtgctgtgggccttaggagggccacaaacaactgcttgtgatttttttttatccttactgaagaaccaatttgcatccctgttgagaatacagggcttgtggccagtaataactctcccttttaggattcctgtctttccccattttttttctatccccagttgccatcacagcgtaacggtgcagggaggtatatgagggttgctaagggaaagcagaggtgcccctcactcaaacctacattcagaaaaaaatttccttcattattgattggatgtcttaaatgcaaagacttacacagaaactgggaagggaggacctatttcagacaaggattcaccatggaatttttatgaatatccttataaaataggacttgggatgcagatggattatttctttaagtcttgcaacttcagaaaagcctgagacacataccccctcctactatatatagtgattataaatagtatatttacctccaaaaaatttaacactgtgccctaatgcaagaaaaatctgtggtataacaatgtactcatgttctgtagctctttactgaaggcctcatgtcaaaggcggggaaggaaagcaattctgtggctctgcacttctacccaagtctgaagagaagtgagccaagttaaatgaaggtcaaggatgctcctcctggtcctctcaggggctggtaaagtcttatatgacgttttctggggagtcattactctgtccaaagtcgaggtagctcagaggccttcaggccgctgatacttccagaaggccacctccccatcatcactgcaggaggccagtagccctggctccttggggttccaggccacacagttgacatcctgggaatgggcctgatgcaagtgggctgtcagggagaaggtgggctgctgtggatccgagttgggatcctcctgaaacacgcggatcgcgtcatccccacaagctgtggccagagcccctgtcagctgacaccaagcaatgtcataaatggtccttgagtggaagccggacaaagtacagatacatttccaactggggtcagagccgctgcatgccaccccttgttcattgcctggtagatactgacgccagatacgcacagtacggtcatcactacaagacgccaggcgctggccactcgggtcaaaggccaagctccacacagtggattcatggccctcaagggtggcacagcatacccagtcatcctcttcctcccggtacagcttcactgtgtcatcatagctggcagaagctaagagctcctgacttgggtgccaaaccacatgcttgacatcctgtgtgtgggagttgagaacactgacacattcatactcatcctcttcatcaactgtgggagagaaaaaggggacccaagagccgaccctgtcagggacacagagggggctgtcaggtggttcccaatccacctggagggacctggcctcaccttcccagacccaaacgctcttatctcggctgcaagtggccaggaggttgccagatggggcccaagccactgacttgacctcattttcatggccctcgagagtggttacacactcaaagtcatcctggttcttcttccaaatgcaagtggtagcatcaaagctggcagaggccaggtaattaccgcagggggaccaggctaccttccgcacggtgcgctggtggccttcagaaaggacagacttgcagatccagctgtcaccctccgtgccccagatgcggattctccggtcgccgccgcacgaggccagcagggtccccgcggggttccaggccaggaaccagcagcgggagtccgggtgcgccgggacacggcccagcagcaccagcgagtccttcatgtcggcccgacgcagggggaggtgggggcgggcagagtccgctgagcagacagcgggtctcaccgcgcgcgtctgcgtaccgcccactccaggcttccgcggccgacagaggctcccgcttccgccggaggacctgggtcgccccggaaactcaactgcccactgctgcggccgccataccctctgggagtt

SEQ ID NO: 13678 - RNA, 3756 nt, Homo sapiens
  source 1..3756: mol_type = other RNA
gctgggattacaggcatgagccaccatgcccagcccacgttaacattttttatgaagaataacttccaaaacaatccaaggagaagggtggcattttacagtctctttagtatcttgttataataaacagttgaattcttacagctgcttctacatccaaacttttttgttgaagtaagttgacttcacacagatacgcagttggaaaagtttttaaaatagccttttcagctaattgtggctattctttgataccacaccaagactacaagtgattttttttttttttttttttttttgaaatggagtctcgctctgtcacccaggctggagtccagtggcacgatctcgactcactgcaacctccacctcccgggttcaagctattctcctgcctcagcctcccgagtagctgggactacaagggatctgccaccacgcccggctaatttttgtaattttagtagagacggactttcaccatattggccaggctggtcttgaactcctgaccttgtgatccacccaccttggcctcccaaagtgttgggattacaggcgtgagccaccgcgcccggcttactacaagtcatagtttcttaaaggcaatgtagactccgaaaacttaatgcactcttatattgttaatacattaaaatccactggcctgtcttacacttttgaatcaatctttgagccatgcatgattttgtaacatcacgtactggtcacttggaaaaatggttcattgaattcttccaaatgaaatgcatttcattatacaaatcacatttgttaatatccccaacaataaagctcatggtggagtacagattttcggaaattccaatttttgcttgaaagctttatcactggcaacactatcagttgtttcccttgaggtgagaggctcattccattaatttccagaaaatatcagccaaatattcaagtctaaataccgtaatctgctagttctttcaattctaaagggcatgccttgaacacagccaattcagcttgcaactcaactgtgtaactgcttttcctcaaggcacccatacttcagtgcacagcagaggggctttatgcatgcttccagttttctcagaatattataaattctcaaggtcaactttttttttctttttgagacagggtttcactcttgttgcctgggctggagtgcaatggtatgatctcggctcactgcaacctccacctaccggattcaagcgattctcttgcctcagcctcccgagtagctggaattacaggcatgcaccaccatgcccagctaattttgtatttttagaagagacggggtttctccatgttggtcaggctggcctcgaactcccgacctcaggtgatccgcccgcctcagcctcccaaagtgctgggattacaggcatgagccactgcgctggctaggtcaacatttaatagttaaccattgctatttgttctatcaaggacatatcaaaactactagaagtttgctgccaccaccttgattcatgccacagtgccaacagttgacctcacagatcctccctgaaagggtcttgggactcccaggatctgcaggccgcattcttcgagaaccactattctaggtacagccccactgtccttctaaaatctaaggtcacagcttaaacttcagggaaggctgtagttttggaggccattgtcacattagaacccatttagaagtgactgtcaagagacaacttgagtgagtctgaaactgcctgctgatggcagtgtttctcaactggtttaaatcgccagtcccctaggaagccttcttcctgatcactccctgccatgaaaatggaatatcacagacacactatatgtgctgtgggccttaggagggccacaaacaactgcttgtgatttttttttatccttactgaagaaccaatttgcatccctgttgagaatacagggcttgtggccagtaataactctcccttttaggattcctgtctttccccattttttttctatccccagttgccatcacagcgtaacggtgcagggaggtatatgagggttgctaagggaaagcagaggtgcccctcactcaaacctacattcagaaaaaaatttccttcattattgattggatgtcttaaatgcaaagacttacacagaaactgggaagggaggacctatttcagacaaggattcaccatggaatttttatgaatatccttataaaataggacttgggatgcagatggattatttctttaagtcttgcaacttcagaaaagcctgagacacataccccctcctactatatatagtgattataaatagtatatttacctccaaaaaatttaacactgtgccctaatgcaagaaaaatctgtggtataacaatgtactcatgttctgtagctctttactgaaggcctcatgtcaaaggcggggaaggaaagcaattctgtggctctgcacttctacccaagtctgaagagaagtgagccaagttaaatgaaggtcaaggatgctcctcctggtcctctcaggggctggtaaagtcttatatgacgttttctggggagtcattactctgtccaaagtcgaggtagctcagaggccttcaggccgctgatacttccagaaggccacctccccatcatcactgcaggaggccagtagccctggctccttggggttccaggccacacagttgacatcctgggaatgggcctgatgcaagtgggctgtcagggagaaggtgggctgctgtggatccgagttgggatcctcctgaaacacgcggatcgcgtcatccccacaagctgtggccagagcccctgtcagctgacaccaagcaatgtcataaatggtccttgagtggaagccggacaaagtacagatacatttccaactggggtcagagccgctgcatgccaccccttgttcattgcctggtagatactgacgccagatacgcacagtacggtcatcactacaagacgccaggcgctggccactcgggtcaaaggccaagctccacacagtggattcatggccctcaagggtggcacagcatacccagtcatcctcttcctcccggtacagcttcactgtgtcatcatagctggcagaagctaagagctcctgacttgggtgccaaaccacatgcttgacatcctgtgtgtgggagttgagaacactgacacattcatactcatcctcttcatcaacttcccagacccaaacgctcttatctcggctgcaagtggccaggaggttgccagatggggcccaagccactgacttgacctcattttcatggccctcgagagtggttacacactcaaagtcatcctggttcttcttccaaatgcaagtggtagcatcaaagctggcagaggccaggtaattaccgcagggggaccaggctaccttccgcacggtgcgctggtggccttcagaaaggacagacttgcagatccagctgtcaccctccgtgccccagatgcggattctccggtcgccgccgcacgaggccagcagggtccccgcggggttccaggccaggaaccagcagcgggagtccgggtgcgccgggacacggcccagcagcaccagcgagtccttcatgtcggcccgacgcagggggaggtgggggcgggcagagtccgctgagcagacagcgggtctcaccgcgcgcgtctgcgtaccgcccactccaggcttccgcggccgacagaggctcccgcttccgcc

SEQ ID NO: 13679 - RNA, 1563 nt, Homo sapiens
  source 1..1563: mol_type = other RNA
gctgggattacaggcatgagccaccatgcccagcccatgctgtacattttacttaactagaatctagtctatatttaagaagaatgtgagaaaatttttgttaaattccttgtgagtattatggttatagtaataactatctaattcttctgatatactaacttaacactcttaccccaaatcaaatgagttagacaaaatttatctgtaataaatccatgtttgtgtctagttatcaccatgttcattttttcctttgattgttcataatccataggtttaaattctatttgagaatttggggggactaaaatctgtaaaacaaaaataaaatcctaagccccctaaccaattatgaatccccctatgggccaaggggatcccagagaagtctgaaaaccaaattcctggccatgatggaaaaggaggttggacacacctcatcgtactccctccctttaggagttcaggcagcactgaccagcattaacattaaaacagacatcataagactgacacaacagactcttcgtggcaataaaattccaaattccagcctgactctggtgtagcatcacatggcagactgaaggaaataaaaatattttactaccaaatatatttctttgacatattttgaaatggcactgtgaagccatcttttggggggaactgcagagaactgcagagaatctcgcttaatacggttcagcctttcccaggtctagaggagattaagactctgacccctttaagggtccaaaaggagacatttaccacctattctctctgaaagcagttacccggaggcttcacctacgtaacaagaaccttggtctccacagctacccttagaactcaagcattcttttttactgacttcaaggctttacaaagcttaactcttaaccaagtgacaatcagaaaatctttgaatccacttacaacctgtcagcctcacttcaccttcaaaacatccaggctctttaggctgaaccaatgtacatttttaatgcacttatttatgattttacttacagttcctgtatccctaaaacataaaaaccaaactgtaacctgaccacttcaggcatactttctcagaacctgttgatactgttctccatgccatggtcactcatattcactcagaataaacctctaagtagtttacagagttgttgtttttgttgttttctcactgacccatcaaaataagtagttttctgaatccacttcctcttttggaaagtagtacacacgctcatctcttctgtgctgagctgatttcacaattggaagacatctcatctttgatgagctctgacagggctgatgagttggttcctggactctccacggttgctgttgggctttaggctagaactcttctgtactttcatctctttgaatacgtttcaggcagcagttaagcgggttctgctgttcatggccattggggtcctgtttagtttgtgatgatctccttctagacctgttctgtcagtgattctgttgctgaatttcctggtctctcactacgtgcatcgtactgcactaagt

SEQ ID NO: 13680 - RNA, 2238 nt, Homo sapiens
  source 1..2238: mol_type = other RNA
gctgggattacaggcatgagccaccatgcccagccctcaataggttttttaaaaacaaactcataagttatttactaaatacatagacataagtccagaagaaggcactgggaaaaggtattgtctgtgtaatacaaatttgcagtccagggcagtcctcctcaggaagccatatttgcagcacttcaaagcaaagactttgagccatgcaggcttcagttcccatcctgatccctccatgcgtgagctgcacaactcaggaaagacaccgtatctctgaacttcacctccagccacactgcactccagcctgggtgatagagtcagactacaacactgaagatgcatcatggttattttccacacagaggataccccaggaccttttgctgatttctgtagaaataacacaatatgcgttaatgtttgctaataataattaagctcagtgaacgagtccatgtaggatatcatgtaaaattgactggacttggaaactaactggaaatggagatgagagaggttttacaaaaggttgagtagagtgaggaggcgggtggtgaagcctttacatgaaaatggaatttcaggagtgggagcagggtgggagagggattgaaaggtggaggagcaggggaatagcagggaataaaattgattttagatatgttgtgtttgagatacctacaaaatgagaattgagaactgaaatgtaaaagaaaggtagaggctggagaaactgatttgagaatgatcatcataagagattattcctgaagccagggaagtagttgagaattgcagaaaaaagaagacagaggaagaaaagagaaagctaatctgtaagacatgttgccatgcttcttttgtctgtccccttttgggcacaagtctatttatggaagaatgagtaagtgttgtgactagagagagcttaggatggatggagagacagagcacagtacaagaacaagactgaggaggacacatttcagttaagaaagtccttattttctcagctttatcattagaagttaagccattctcttaacaccaaccaggaattcagtagtaaattaattcccagaatatgaatcagtcagcacagcaattgtggagagaaattgcaagcactttatgctaagtctactctcatacccagtaaaatacacaagtcctgctaaaactgtctgcatcacccatgcccccacaaacttatttattcacactggacaaggaagcttagtaatctactagacagatccagaaaacaaaactctactctatctgtggttagacaataaaaacccaatttattttttttctacaagatctcagaaaagtccacctaaaattttgcatgcgagcattgatttgttcaatcacaatcattattttccccatgataacaaaatctagattggaaatgttaactttcactttaaagttattcaactgtactcgatactagcgccaaggaacgtggtttctacctgctattatatcaatcatactgtaaatttatagaattataacagtcttgtgtctaggttaagtctgtactagtattgcccaataaaaaacacagattactggttcagtaatctgtgtttcatctcactggacactcaaggttctcccacatgggactttttaccaagccctacaacaattcggtagagtctcactgaaagttgctattctgtgcatctccttttgttaacatgactataaaagaaaagaagagaatgacacacaggcatcaggccaggcgcggtggctcacgccttttatcccagctctttgggaggctgaggcaggtggatcacctaaggtcaggagttgaaaaccagcctggccaacatagtgaaaccccatctctactaaaaatacaaaaattagccagacgtggtggtaggctcctgtaatttcagctacttgggagactgaggtgggaggatcacttgagcctgggaggttgaggttgaagtgaaccgacattgtgccactgcattccagcctgggtgacaaagtgagaccctcttctgccccagctcactgggtggggaaactcctgcatggtgctataatcaatttccacgtttcaggaccaggaagggactctgcccctattcagtcattcagcacatgtactgggtgccatcctttgatcagacctttggttgtaatttagatggttctgtgggaagagaagggtgttcacaatgcacaatacac

SEQ ID NO: 13681 - RNA, 3360 nt, Homo sapiens
  source 1..3360: mol_type = other RNA
gctgggattacaggcatgagccaccatgcccagccgaaacagctctcttactgctgttgtctgagtgtttatgtcctccccgaaatgtatatgttgaaatcgtaaatcccaaagtgatggaattaggaggcagggccttcaggaggcgatgggtcatgagagcggaatcctcatgaatgggactggtgcctttatattagagcccaaggagagacccccccgccccatcccttccaccatgtgaggacacaggagacggtgtcacctatgaaccaggaagcaaccctcattagacaccaaatctgccagtgccttgatcttagatgtcccagactctaggactgtgagagagcaatttctgttgttgacaacccaccagtttatggtattttcttatagcagcttaaacagactaagatacccacgagtctattaacaagataataaacaaagtataatttcaggaattaacaagaaacaggaataaaaagagctgtgaagaaacaaagtggggcaaatgaatagtccgtgagaaggaatgctatttgagtcgaggtcagggtgcctctttcaggaagcaacattcggacaaagacccgaacggaatgaggggacaaacaatgggcaacgttttgggggttggtgaggacagcagcaatgggcagagcctgaggcaggaaccagccaggcctttggaggaagagcaggaagccagtgtggggggaacagggagccaggcgaggcctggaggatacactagagatggcaggcagctcagtcaggtgaagccactgagagatgaaagccgacaacactgtgggaaactgacagcaggagagcctagggaaaagcggggtggttattcaaagagcaggttgcttagcacctttaaggaattttgggggtgggggcagcaggaacccaccatcacaaaaatcactgacatgccatatcatggatgaatctcaaaaacattataagtgaaagaagccagacacaaatgactgggtatagtctgattaagtgaaatatcctgaaaaggcagttctataaagatagaatgtagattagtgggtacctggagttggtggtgaagatggtaattaactacttgggcataaaggatctaaccgggatgacaaaaatgttctaaaactggatttcagtaacggttgcacaacctggtaaatgtattaaaaagtcattgaattgtacacttgaaatgtatgaattttatggtttgtaaatcataatgttatcgaaataatctctggtagtgaaataaagagaaaaaagagcaatgaccctttctggatgagtgccatccaggaatagccacctggagaactgcagagtcaagtaagaaaggcaggtgaccaggggcaactgagataaaagcttgcatatcaggcttaggcaaagaggatgagggctattttgagcagccgtctttaggtcagggttcacatttgcaggcaaaactgtccctctctctctctgagtttgctcctgtagatcaaatatcaggccggctgatagggtgtcctgagaatatgccctgcatccaccttacaggctttgctctgctcaggagctcagggcctcctgcagccacgtgaccgcagcactgagaagcaggcagggggaggcacgggcaaggagggttcgttcaatgccaagtaagtgactaaggaagctcttgtttactgtgcaagagaaaatgacttggtggccatttgtggaggttattaatgccaaataatctagaaattataaacaaaatatcataatggtaatatatgatttagaaactgatttacatctaattgacacaatattatagtgtcttccagttccaaagtatgaaaggctttgagaaacatcagaggaaagagcttccagtcacctctatggagagtcaaactgaggttaacctgaaaaccaaatcagcatcaaaacataaccaccctaaaactccagagaaaatgatggaagttaatacaggtagcactgagttatttccccaggacattcaggtgttggcgctgtgattggcatttttccagaggaccaggttgcctgcaacctcaggccccagaagatgcaggaacctgaacaccagggccaccccctgctctgtcactactctggtcttgccttggagtgtgaaatgctgcaattcatccaagatacagtcatgcagcatataacatttctgcatatgactgcatgtataatgatagtcccataagattataacaagctgaaaaattcctatcacctaatgacatcatagccaccatcatgtcgcagtgcaacacacatgtgtttgtggtgatactgttgtaaacagacctactgcagtgccggtcatataaaagtctagcacatacaagtatgtacagtacctaatacttgatcataacagctgttcctagtttacgtgttcactatattatagttttttatcattttgaagtatactcctaaaaacaaaaaaaggctaccctgtaagacagtctcaggcaagtccttcaggaggttttccagaagtagtcactgttataggagatcacagctccatgagcgttactggccctgaagaccttggaaggatgtgaagtggaagacaatgagcaatattgatgatcctaaccctgtgtaggcctaggctaaagtgtgtgtttgtgtcttagttaacaaaaaaagtttaaaaaaatatatatacatgaaaaaagaatagttttgtatagctgtacaatatatgtgttttaaactaagtgttattatttatttatttatttatttatttatttagacagagtttccctcttgtcacccaggctggagtgcagtggtgtgatctcagctcactgcaacctccacctcctgggttccagcgattctcctgcctcagcctcccgagtagctgggattacaggcgcccaccaccacacccaggtaatttttatatttttagtagagacagggttacaccatattgaccaggttggtctcgaactcctgacctcaggtgatccacgcccctcggcctccgaaagtgctaggattgcaggcacgagccaccgcgcaccagccaaggttatgcagttttagcaagaataccccagatgtgacattgtgctcttctcagtgcatcctattgggggcacatggtgttcatatgtcttattcctggtgacatcaatttggatcacttggttaaggtggtgtctgcctagtctctctactgtaaagtgactatttttccctcttaaagattaccttaaaatttaaggtaagttgtattttttgtcttaattcagatgcatatttaaataccacttttggaaaaatatt

SEQ ID NO: 13682 - RNA, 4196 nt, Homo sapiens
  source 1..4196: mol_type = other RNA
gctgggattacaggcatgagccaccatgcccagcctatgaacttgcttttctaacaagttccccagtaacgctgatgcttttgtcaggaccttgctttgagaaccacttccagtgagagaatatcattgatgctggcatctgaagtcctgagtttaaatcctgattctattattaccacctacataatcctagtcaagtaattttttctctcatttttagtctctttgtgacaatacttagatcccagagttatgagacatgaaataatgtaccaatcagagtttggtacagtccctggcatagaacacaataacaaatattaacttcctttttccattatacatggctagatggaacaattaagttaaatcgataacacataagttgaaacttcacaggaaaacaaagtacagctagttgaagcaaacaatatcttataattatacatgtaatacagaatgatagagaaatgttttaagtacttaaaaataccttcgttcaattttcaaaactttgaacgtaataatttaggtagtaggaacattagatgcaatctatagaagaaatattagactcaatctatgaagaacatgaatttttttacaacctataatggatcctgatacctcatctataattttagttttctatagaatcaataatataattagtgtacctgcttaaaactgtattacattgatcttcaatgctacttaatttctgagaaaacctaagttataagagtacatcagaatctctattatcaaccaaagcaaaacttctaccaacgacagaatggatactttttaaacaaatttacatataccaacaagcaaaaaactagagctttcattcctgcttgacatttttttcactttgtgtgtctcaaggctctctcaggaatcagtgtccaaaccatgaggtgaatcctgggaggtaagcaagcttgctgtagaagccgctgtacatgccttcaggaacagaaagggtaccagaggctgtgccctcctagtgtggctggttggagtgacaactagaatgttgtccgtgtttttctgtggaacctacaatgagtccagttgtctaagtgagtctcaaaggtattgaatagttgatgtcaaaaggcactttatgtcaggactgtttaaagcaagtttctccctataccagtagtgacccagaggcaaggtcttaccggacctcttattttcaaaagccttccctttccaattgagcctgatgccattatgtgacatctttttttccctgaatttctaaaagaaaatgtgatgattacctgcatatcttctttgttgctgcatcgtgttttgcatggtacccctttaatattgttttcaatacttagcctgctgatatacttttaacttctcacctgtttatgaattctcttaactaggctgtgaggcccttaagggtcttcaacttgtccctttcctccacgtaactttctcaaacgccccagttctcagtaacttttctcttttgctgtctgtaatataaacatgacccctacttacactgtcctacctatgtggccaataagagtgttgtcttcgcagttggaacccaaaagccctatgggatggaggatatgcactgtacttctttgtaaaagtgtcttgacaaagctgatgtccaatcaacatttaattaccagactgtccaagctagaaatgaaatacagttgattgcctgagtcctgataatcttgctaacaaaattataaaaggcctatagtatggccaatatatttggctaatggaaatgattttcttaaagccagaaaattcagctacccatagtgcttaaaaccagccttaaaagaacatgaacaggatggttcccaccttatcgagatcactggcattccatagtatccattcattcatatcctcctcctaggccgcatgaaacacctaccacatttccctacctcctaaagcaaacaaaactcttttcctccctcttgctgcaaaaaggtttattaaaagccgtatgtagtgtataaagcctttcaaaaatactagcaatccatgcctttctttttttgagatggagtcttgctctgtagcccaggctggagtgcagtggcgtgatcttggctcactgcaacctccgtctcccaggtcctggttcaaacagttctcctgcctcagcctcctgagtagctggaattacaggaacgcgccaccatgtccaggtaatttttgtattttcagtagacatggggtttcaccatgttggccaggctggtcttgaactcctgaccttgtgatctgcctgcctcggcctcccaaagtgctgagatgacaggtgtgagccgctgcacccggcctcattttaactaaatctgaagccagagttgatttgatgcccatcctgccagggaggcagttccttccctcaggtttgttagtagaaaccaaaaagtagcctgagagggttcaggtgccaccttggaggcactaccttatcttttgtccttttagagttttcttgctggggtgtttggctccagcactatagcccttaccacaatcattccacctggttcttcaataggactctgaggtatcaaaaaagtcactagggcagcccagagattggtacgatttacctttacacctcaaagttttttagatgtgagcagcgctggattatggcaatttaccttataataactcaccatagttggctgttataagaataaatattgttcttctaagatttttaattagttgcttcagttattacatttttttctattttttttttaaatagagatgaggttttgctatgttgcccaggctggtctcctggactcaagcaatctcccacttcaggctaccaaagtgctgggatttacaggcatgagccacctctcccagtctcagttattattttaataaatgagactgaacgtcctcttataaggctcactcccttgttcctactacatttgctctgtttaagtatctctttaaattcttcagttaagatcatcccttttatcagaaacctagacaccacaaagtagctttctcacctttaattctccatagggatcactattatactataatatttgcatacgtatgtgtatatatgtatttgcttttttaaaaaagtaaaaatgctcttctcactctttgtcgatataggcacccaggtacgtagttagaaattaaataaaggccacaataatttcccaaggaagatcattaaaaagaaaaatcctttcttcctctaatatcacatagctggcctttatggcatgccagctaagaaaaaaggtattgcctatggtgacaggaagactcaatctttctctctttgggttgtagctgaatttctatcaaaagtcctagtaaaatatataactcctcatttgttctaagccaagtcttttcttcagttttccttcaaacaatacctttactttcccattagaatatgaagaattggagactgtgaacagcaaggtttggggtgggtatcagtcacttcaaatctggctatgcagagagagggaaagacatggcagaatagcaggggtggagggtgagtgaaatgtatcttcattgggagtattgaaagagagcaagtttttcaaagttgttgccggtatctcatgaaagcccaggctgctaccatggtgagggcaaacactggcaccagcaccataaatatgggaataccacttgggtccccttcacctcgatgtcctataggtccattctgcacctgtaacctgtgctgcactctcagagacacagcatagcctgcattacgaaagaggtctacagcatcctggtgcagcaggttctttaggtcttggccatttaccgaaaggatcttatcaccctcctggagccgcccatccagggccgcagccccattttctttgatgcggctgacgtagatgccactgtcgttggagacatactgctgatctgtcccaccgacgatgttgaagcccagccctgagggccctctggtaagattgatctcttcctcagtgaccaaataatccactcttccgttcatgttttacagctcgtctggcttcctacttgggtcagctggagtgcagcacaggtgaaggtgaatcaatctcggcgctgcgcccacagcacagcggtttcggtttcagcagcctcgagacccggaaaag

SEQ ID NO: 13683 - RNA, 3493 nt, Homo sapiens
  source 1..3493: mol_type = other RNA
gctgggattacaggcatgagccaccatgcccagcctatgtcttaaatgcactgtatttccttgtactccagatccctattagtgaaatgcctattaaaacatttcgtaaggccagcatggcagtgtgcatcagtagtcccatctatttgggaggatggcttgaggccaggagttagagagagtagtgtgttataatcatgcctgtgaataaccactgcattccagcctaggcaatataacaagaccccatctttaaaaacaaacaaacaaacaaacgaacgaacaaacagaagtcttgtagtgcttccagcaaatcagcagaaaggaaaaaagagctctagagtaagaacagttgattctttttttaacaattagtgatgggggagtattcagatggccagctaaagagagaagttctagaactcagctagaccagtatattgctttatttaaattggctcaatatcctatctaaagctagaccagtggttttcaaagcatggagcctggactgcatcagctgagaatgtgttagaaatgcaaatttttgggtcccacctgaggtctactgtatcaaactctgggggtgggcctagcagccttgggttttaacaagccttccaagtgattctgatgtaagctaaatttggaagcccctgagatacacttactggaaagaagctggacccaggcccacagtgtacttgatgttcctgtggttggttcagttttcaaatttgtctgcacattggaatcacctggagagcttcaaaactaccaatgcctgtgacccgtcaccaaagattgtgatttaataggcctgggatatggcctgagctttggaatttttaaaggattctcaagtgatcctaatttgcagacaagtttggaaacccttggatgaatcaaaatacatcttgaatcaaggaccagagacagccaaaaacaaaagaaaagaaaacacacatattagtcaaattccattcaaagaagtttcctggctatttcagagtactggaatgttgtcacaataacattgctttacttaaattggctcaacaacctatctaaagaaatctttattcttgtaaactacattttctgaaataaattcctgcattattttgtttggaggaaatctgtaattttggaatcaataagggtttgtgtcactcttttcattaaatattcatctatgccatttaattgtccaaaaatggcatcaggaatgtctacacaagtggaaaggaactgtctaagtttctgtacacttgatatggcttctgtgatggtgacttttggttgctctggtaaagatacctccccttcatcttcacttcctgcttcactggtattttcgccagccaccatgtcctggatgatgtctgtgtcctgagagataatgagatcatcatctgcagtaacaaagtcctggaaatttacttcatttgggacacaggtggcaatagccactgtgtgccacaacttttcaatggcaatgtctggttcactggctgctgattctgtgtcacattctgcaaattccatagggacgatgcctgccttctgccaacatttcaccactgtggatggcttgactgaccaccacgctgcagcaatcatgtcgatggcctgcttgatgtccacctcttcttgatcctcactgctgttgagcttgaggaggatctgttttagaaggtggctctggtacagtactttcatggtgtgaattatgccaagattcagtggctgcaggacagcagtacagttggagggcagatacccaacctgaatcctttccaagtgtggaagcatgttatgagcagagcagttgtctatgagcaagaggatccggcgttccgccctcttcatcctggcatccacttgcatcagccactcattaaacagatcccttgtcatccaagcccactggttggctcggtaatcacaagggagggaatgaatgttcttgaggcagtgtgggctggctgacctaccaacaatcaatggtctcattttttcagtccccgaggcattgcaacaaaagagtgctgtcaaccgctgctttgctttcttgccccctctacagtggtctcctttagcagcaagtgtgtgctggggaagcaactggaaaaacactcctgtctcatcagcattaaagatatcatctgggctgtagtcagcaatcagttttataatttcccctgcatgccactcattaatcttatctattcctagaccattcattaacctgtcactatcttctctacagactgctttcaaagcaattccgtggcgatctctaaatctgttcagccagcccacacttgcttgaaaattgtcatagccaagcatgttggccaagtttagtgcttttttccgaatgacagaaccagtcacaagaatgtttttggcatggatttcttgaaaccaagcaaaaacagccttatcaatgtcatcataaagagcgctcctcatccttttccgctggggtcccacggatgcctcccgcaccttttcttcaaatttggtgcgatcctttaagaatgtagataaagtagagggagtgataccaaattcttttgccacatcacctttcctcttgcctgagtctacagctcccacaactttcattttctcctccagagagaactgccgacgcttcttgttccccttgtttgccatttccagggaatgagggctggccacaactaacaggactgtctggttcctcctcgcggcttgctttgccccaagtgtggaaagagtgcaaaatgatcaatctgactgcttcgtggagaatggattgtagaggggatgtggggagaactacatcagtccaggcaggagatgatggtggctagaaggttggtgatggcggtagatgcagagaagtaggcagactggaatacagtgagggttgtgcgggaacttgtacaaatgtggacaacttgtgacactggagagaaaggacaatccaatccaatccctatttgatttacggaagctctccatacggtcattcagctcagcttgagtcactccaggaactcactaccatcactattcgtgggccagtgggagagacggattgagggcagatcactggagtgatgaaggcgctacttgatgcggcactacgtatgaacccgatcctgaatgagagggaaagactgagacaggctgaggtcaggccttgaacgtcgtgctgaggagagggtggtattgtaggcttcccagcgcccgacgtggctctgaaaggtgaggcggggcctagatccctcacgctcagcacagccccgcccctgttacctgaacgccccacagcagtgcccgggggctgagcggccggggcgtcccaccgccggcagccacagcttcctcctccgcccgggacctctggccggaagcagtccgttcgccttactagacccgctccaagcctttgagcagttcgtgtgggtccgctcccaagctagggctgggctgttgc

SEQ ID NO: 13684 - RNA, 2947 nt, Homo sapiens
  source 1..2947: mol_type = other RNA
gctgggattacaggcatgagccaccatgcccagcctatgtcttaaatgcactgtatttccttgtactccagatccctattagtgaaatgcctattaaaacatttcgtaaggccagcatggcagtgtgcatcagtagtcccatctatttgggaggatggcttgaggccaggagttagagagagtagtgtgttataatcatgcctgtgaataaccactgcattccagcctaggcaatataacaagaccccatctttaaaaacaaacaaacaaacaaacgaacgaacaaacagaagtcttgtagtgcttccagcaaatcagcagaaaggaaaaaagagctctagagtaagaacagttgattctttttttaacaattagtgatgggggagtattcagatggccagctaaagagagaagttctagaactcagctagaccagtatattgctttatttaaattggctcaatatcctatctaaagctagaccagtggttttcaaagcatggagcctggactgcatcagctgagaatgtgttagaaatgcaaatttttgggtcccacctgaggtctactgtatcaaactctgggggtgggcctagcagccttgggttttaacaagccttccaagtgattctgatgtaagctaaatttggaagcccctgagatacacttactggaaagaagctggacccaggcccacagtgtacttgatgttcctgtggttggttcagttttcaaatttgtctgcacattggaatcacctggagagcttcaaaactaccaatgcctgtgacccgtcaccaaagattgtgatttaataggcctgggatatggcctgagctttggaatttttaaaggattctcaagtgatcctaatttgcagacaagtttggaaacccttggatgaatcaaaatacatcttgaatcaaggaccagagacagccaaaaacaaaagaaaagaaaacacacatattagtcaaattccattcaaagaagtttcctggctatttcagagtactggaatgttgtcacaataacattgctttacttaaattggctcaacaacctatctaaagaaatctttattcttgtaaactacattttctgaaataaattcctgcattattttgtttggaggaaatctgtaattttggaatcaataagggtttgtgtcactcttttcattaaatattcatctatgccatttaattgtccaaaaatggcatcaggaatgtctacacaagtggaaaggaactgtctaagtttctgtacacttgatatggcttctgtgatggtgacttttggttgctctggtaaagatacctccccttcatcttcacttcctgcttcactggtattttcgccagccaccatgtcctggatgatgtctgtgtcctgagagataatgagatcatcatctgcagtaacaaagtcctggaaatttacttcatttgggacacaggtggcaatagccactgtgtgccacaacttttcaatggcaatgtctggttcactggctgctgattctgtgtcacattctgcaaattccatagggacgatgcctgccttctgccaacatttcaccactgtggatggcttgactgaccaccacgctgcagcaatcatgtcgatggcctgcttgatgtccacctcttcttgatcctcactgctgttgagcttgaggaggatctgttttagaaggtggctctggtacagtactttcatggtgtgaattatgccaagattcagtggctgcaggacagcagtacagttggagggcagatacccaacctgaatcctttccaagtgtggaagcatgttatgagcagagcagttgtctatgagcaagaggatccggcgttccgccctcttcatcctggcatccacttgcatcagccactcattaaacagatcccttgtcatccaagcccactggttggctcggtaatcacaagggagggaatgaatgttcttgaggcagtgtgggctggctgacctaccaacaatcaatggtctcattttttcagtccccgaggcattgcaacaaaagagtgctgtcaaccgctgctttgctttcttgccccctctacagtggtctcctttagcagcaagtgtgtgctggggaagcaactggaaaaacactcctgtctcatcagcattaaagatatcatctgggctgtagtcagcaatcagttttataatttcccctgcatgccactcattaatcttatctattcctagaccattcattaacctgtcactatcttctctacagactgctttcaaagcaattccgtggcgatctctaaatctgttcagccagcccacacttgcttgaaaattgtcatagccaagcatgttggccaagtttagtgcttttttccgaatgacagaaccagtcacaagaatgtttttggcatggatttcttgaaaccaagcaaaaacagccttatcaatgtcatcataaagagcgctcctcatccttttccgctggggtcccacggatgcctcccgcaccttttcttcaaatttggtgcgatcctttaagaatgtagataaagtagagggagtgataccaaattcttttgccacatcacctttcctcttgcctgagtctacagctcccacaactttcattttctcctccagagagaactgccgacgcttcttgttccccttgtttgccatttccagggaatgagggctggccacaactaacaggactgtctggttcctcctcgcggcttgctttgccccaagtgtggaaagctgaacgccccacagcagtgcccgggggctgagcggccggggcgtcccaccgccggcagccacagcttcctcctccgcccgggacctctggccggaagcagtccgttcgccttactagacccgctccaagcctttgagcagttcgtgtgggtccgctcccaagctagggctgggctgttgc

SEQ ID NO: 13685 - RNA, 7721 nt, Homo sapiens
  source 1..7721: mol_type = other RNA
gctgggattacaggcatgagccaccatgcccagcctttttattaatgttttaatggcctgtgtttctaacaagtagttgaaacaatgttgaaaattaaagagtagacatgttaaaacttgcaacttcatttaaatttaaatatatcatttataccaaaatcagaatttatttaagatttatggctgggtgcttggctcacacctgtaatcctagcactttgggaggccaaggcaggtggactgcttgagcccaggagtttgaaaccagactggaaaacatggtaaaaccccatctctacaagaaataaataactctacctggccctttagcaaagaattaagaaaaatcaatacagaccagtggctcacacctgtaatcccagcactttgggaggctgagggtggatcacgaggtcaggagttcaagaccagcctggccaacatggtgaaaccccatctctactaaaaacacaaaaattagctgggcgtggtggcgtgtgcctgtaattccagctactagggaggctgaggcaggagaattgcttgaacccaggaggcagaggttgcagtgagccaagaacacaccactgcactccagcctggcaatacagcgagactccatctcaaaaaaaaaaaaaaaaatgcaaatactatgccatataaggagcttgagcatccacagggagtatctgtggttgcgggggggtcctccatgaatactgacaactgcatacttgctactctactggcagttccaaacatttgtttgtggtttattttgggtttcctaattacacgatcacatctccaattcatggcagttgtttctgcacccatccctaattcctcacattccttgttttcacaccttggctagatgttactcatttcataaaagtgatgcgcattcttgtaattttgctttgttttttacagacagggtctcactttgttgcccaggatggagtgcaggggcatgatcatagctcactgtagccttgaactactggactcaagctaacctcctgcctcagcctcctcagtaggtgggactaccggcacttgccactacacctggctgatcttttttttgagatggaggcttgttctgtcgcccagcctggagtgcagtggtgcaatcttggctcactgcaactgccacctcctaggttcaagcaattcttctgcctcagcctcccgagtagatgggattacaggcacgtgccaccacacctggctgacttttgtatttttagtagagacggggtttcaccatgttagccacactggtcttgaaatcctgacctcaagtgatctgcccacctcggcctcccaaagtgctgggattacaggcatgagccacggcgcctgaccacacctggctaatctttttaaaaagtttttgtacagacagggtctccctatattggtcaggcttgtctcgaactcctgggttccagcaatcctccagcctcagccttcccaagtgctggtattacatggatgagccactgcacctggctaattttactttaaaggaatctttctactattttatcattaagtatgacatttgtgttttcagaacatatattccctaccaagttacaggagttaattttaattcccaacttaatagtattttagtgtcatctatgggtgttaaattccatcaagtgatttatcagcatatactgagataatccttatgagttttatctggtagttaattaaaatattttctaatattaaatcttccaaacatactcttctgttttttgagacagggtctagttctgtcacccagggtggagtacagtggtacgatctcagctcactgcaacttccgcctcctagattcaagtgattctcccgtcccagcctcccaagtagctgggattataggtgtcagttaccatgccctgctatttttttgtatttttagtagagaggggtttcaccatgttggccaggctggtctcaaactcctgacctcaggtgatccaccatctcagcctcctgaagtgctgggattataggtgtgagccaccgtgcctggccccatatatctctttttaagtgggcatactgccattataaataatagtgattctgctggtaatgaacaaaggatgctggatccactaatagtctgttaaacctaatatcatgactttcttgttagctatacattggtttgctataattccatttagaatttttaaacctatgttcacaaatatggatttttaaacctatgttcacaaatatggatttttaaacctatgttcacaaatatggtttgcaagtcattttttctcctaaatttctatttgatggggaagttgtaaaatattggggttatttttccttggattttccttataataactattcctgaaaagtctctggaatgtctttcttttctggggctggggtagaaggactagatagatttacaaaccagtaactcaatttctgttttgtaaaattttcatttcattaaataataagtcctaatcaagtattattctttcccacagtatgtgagtgctgtcctcaatactgtcaacacttctggcttctaccaggcaaggctgcatgtagatttgcatctgaaaaaacaacaaactaaaatctaaccctaggtagtagtaaactgaatataaactttctcttatgaatttattctgtcttctttggtacatcaataataatatacacctttacagtatttcccagattgggggatacactttagcaagtatctgcgattatttgtttatgtaagatgtcccttcccttctgtgaatcatcattcttcaccccaagtatcttgagattggattctgtataagcagaatacaacagttaggcattcaggtatcattaaattcctccgcttcaaggatgaaaatttctttgggtatctaatagagtacaaagcagaaggtgtttcagaaatatttgcagtattgaatccgcatattcctccaagatagccctaatctaactggcagggtcccactcttcccagattaatgcccactcacataacaaacctgatgaggtagtgaagaaaactaactttgtgagtaagcaactggcagagtttttcaccactgtgactctatagctacatgtaactaagtagtatcactgacacataatcttaaattgaagttttaagatcattattctccatgttatacatgggtatcaaaagcattcccctcttgaccactccagaattctgtttaaaatttttcaatgacaacttatccatttccccaaagcctcagtgagcacatgatgccaacaattcatttcatgacttcatagcatgggccaagtttcttgcttaaaagacttccatcctgtcttgggaaacaaccatttccaaatatccacatatccttgcaagtttctgcctactcctctaccacccatttctgaagccatctgatttagtaagctgtatgcaaaagatacacaatggctaatgcaatcaaacaaggaatgtattaaaagcacacccaatagctcaaaataaaagacaagtgaacaaagttaagaaaatgacagtaacaaaagctgttctgggaacctctattgaaatagctacttattacatcaacatgctaccacagaacaaaagctcatgttgcttttctgaacttgaaaaacccattaacaatgtacagttctgagcctcagctgaccatagtgctcatgccaagtcctgagcagggcatcttgaatggtggttccctcatgactacatacaccgttagggaatgtttcgttaagaggaaatcaagatgttctaacctgtgaaggtagaatagattccaggctacacaaacacatgaagtgtgccttatattgattactaaagaggttgctgccaagactgcttccaaagggcagaagatagccctaaaaaatgtttgcagtgtggaaatgcatttttagtaagtcatattctagtaacaagttgcatttggtaagacacaaagaaacaatgttggtatgcagagtagaaatctctggaagatgatattgtcatatcagagatattgtcagtatcagagatactgaaatctctggaagatgatttttgtctcacatatggcattcgcaagtaaaatgccaaactgcaaaattcatattatgtagtacacataggaagatatctaaatatccctgtaggctctgggatgttatttcttattcttaacctccttactagattcacttgtacaatgaaataatctgtatcttattatttataattgagaattttctcaaaccttttcctgaaattttggaacacctggaataaaatttcttaaaatgattcctaaaagaaataattcttcaaaattaatattaagatataataacaggttggtttttttttttttttttttttttttttttagaatgaagcttctaaggtgaggttaacagtccagctgtggtttatttggtacattcataagatgttcactcctatatatattttttccctaggggtttctcatttctagatttacactttcccttatagcatggtccctccaaggtatatgcttccgatacataaaatgtttgtaattttgttaattctgccattcattagctcaataatttctctcattaaaattctgtaaactatgaatttcaaagaagtctattctatattcatctggttcatgaagtttcctctttgtgaatcttattttagtaaaatgactttacaacgtttaacatggttcctcacctgtatgaactttttaaaaaaaggtatgacttgctgctaaaaattttcagagtggttactaaattcagttttcctgtgtattgtctactatctttttgcatgtaaagaacagctttctgtggatgcctttccatatgctgtgcattcataaagtttctattcagtatgagttttctggaagatgacaagatgattccacttacagagtttctctttatatatgattgtttctatctcttgtgaatccacttttcagagtttcgtaaaattatcaatgtttgtcatctacatgagttctctgatgcataatgagctgtgacttccaacaaaaggctttcccacattcagtgcacttacaaggcttctctcctgtatgtgttctctgatgtgcactgagaattgatttttgagagaaggttttcccacattcattgcacccatagggtttctctcctgaatgagttctttgatgtacaatgagttgagaattcctaatgaaggcttttccacactcactgcattcatatggtttctctcttgtgtgcattctctggtgtacaagaaggcgtaatttcccactgaaggatttctcacattgactgcatttataagggttgacccctgcatgagttcgctcatgtacaatgagtagtgatttccaaatgaaggctttcccacattcattacattcatatggtttttcacctgaatgagttctcatgtgtataattaggtatgacttgctgctaaaagctttcccacattcactgcacccataaggcttttcccctgcatgagttcgctgatgtgaaatgagctggtctttcctattaaaggctttcccacattcactgcattcatagggattttctcctgtgtgaattctctgatgcacaatgagttgtgaattgaaactaaaggatttcccgcattccctgcactcatgtggtttctctcctgtatgagttctcatatgtataataaggtatgacttgctcctgaaggctttcccacactcactgcatccatatggttttactcctgtgtgacttctctgatgtacaatgagctgggacttcaaactaaaggtttttgcacattgactgcatccatagggttttactccagtgtgcactcctttatgtacaatgagctgtgatttgaacgtaaaggcttttccacattcattacaactatagggtttctctcctgtatgagttctctgatgtacaatcaggtttgactttgtattaaaggctttctgacactcactacattcaaatggtttctcccctgtatgagttctctggtgtataataagctgtgactttaaaccaaaagcctttccacagtcggtgcattcataaggcttctctcctgcatgagttctctggtgtgaaataagctggtatttccgactgaaggctttcccacattcatggcattcataggggttctctcctgtatgaatcctctgatgtataatgagctgtgatttaaaactgaaggctttcccacaattgttgcattcatggagtttttctcctgtatgagtccttgtatgtataataaggtatgacttgctcctgaaggctttgccacattcattgcatacataaggtttcattcctgtgtgacttctctgatgtacaatgagctgtgatttcaaactgaatcctttaccacactgaatacacccatagggctttactcctgtgtgaatcccctgatgtacaatgagctgtgacttgaatgtaaaggcttttccacaatcactacaaacataaggtttctcccctgtatgggttctctgatgtaccataaggtttgactttgtattaaaggctttctgacattcattgcattcatatggtttctctcctgtatgaattctttcatgtataatgagctgtgattttaaaccaaaagctttcccacattcattacacacatatggtttctgtcctgaatgagttttctggtgtgaaacaagctggtctttcctactgaagactttcccacattcacagcactcatagggattctcacctgtgtgaattctctgatgtataacaagctgtgaatggaaactgaatgttttcctgcattcactgcattcatgtagtttctctcctgtatgaattctctgatgtacaatgaggtatgatttactactgaagtctttcccacattcattacaaccatagggtttctcttcggcatgagtttgctgatgcactagaaggtatgacttgctgctgaaggctttctcacaacagctgcatccaaagggtttttcgcccatatacatttgttggcacataagttgcgatttcttattgacggtttttccagattcaatactttcacagtattttattccaataacagtttgctcatgtttagaatggaagaatgattttccatgtacctgaaacccattaggattatttctagcataatcactagtgaaatctatatatttcaaactctttccatgcgtgccacatttatgaggtttttgtcttgaaagatactttgtactaagaagacatagttttccaaatgtagtgcattcaaagctttttgccgtacttcccagcttgtctttattttcctgatgccaatccataagatcatcaattttccagactgtgtccaaatagaagctgtccggaccctggtggccatccctacggtcagttttgtgtgcctcgctggaagtgacaggacgcgagggatgctccggctcctccaaaccctgaaggggcagcagaatagagtccagggtactgcctccacctccagatctgcagccagaagggttcgcaaccactccagactcggctggcccgttgaccacgacgggcgatgaacgctatctgaggaacaaggatctcgccatcggcgcggaacaatggcggccgctacgtat

SEQ ID NO: 13686 - RNA, 7922 nt, Homo sapiens
  source 1..7922: mol_type = other RNA
gctgggattacaggcatgagccaccatgcccagcctttttattaatgttttaatggcctgtgtttctaacaagtagttgaaacaatgttgaaaattaaagagtagacatgttaaaacttgcaacttcatttaaatttaaatatatcatttataccaaaatcagaatttatttaagatttatggctgggtgcttggctcacacctgtaatcctagcactttgggaggccaaggcaggtggactgcttgagcccaggagtttgaaaccagactggaaaacatggtaaaaccccatctctacaagaaataaataactctacctggccctttagcaaagaattaagaaaaatcaatacagaccagtggctcacacctgtaatcccagcactttgggaggctgagggtggatcacgaggtcaggagttcaagaccagcctggccaacatggtgaaaccccatctctactaaaaacacaaaaattagctgggcgtggtggcgtgtgcctgtaattccagctactagggaggctgaggcaggagaattgcttgaacccaggaggcagaggttgcagtgagccaagaacacaccactgcactccagcctggcaatacagcgagactccatctcaaaaaaaaaaaaaaaaatgcaaatactatgccatataaggagcttgagcatccacagggagtatctgtggttgcgggggggtcctccatgaatactgacaactgcatacttgctactctactggcagttccaaacatttgtttgtggtttattttgggtttcctaattacacgatcacatctccaattcatggcagttgtttctgcacccatccctaattcctcacattccttgttttcacaccttggctagatgttactcatttcataaaagtgatgcgcattcttgtaattttgctttgttttttacagacagggtctcactttgttgcccaggatggagtgcaggggcatgatcatagctcactgtagccttgaactactggactcaagctaacctcctgcctcagcctcctcagtaggtgggactaccggcacttgccactacacctggctgatcttttttttgagatggaggcttgttctgtcgcccagcctggagtgcagtggtgcaatcttggctcactgcaactgccacctcctaggttcaagcaattcttctgcctcagcctcccgagtagatgggattacaggcacgtgccaccacacctggctgacttttgtatttttagtagagacggggtttcaccatgttagccacactggtcttgaaatcctgacctcaagtgatctgcccacctcggcctcccaaagtgctgggattacaggcatgagccacggcgcctgaccacacctggctaatctttttaaaaagtttttgtacagacagggtctccctatattggtcaggcttgtctcgaactcctgggttccagcaatcctccagcctcagccttcccaagtgctggtattacatggatgagccactgcacctggctaattttactttaaaggaatctttctactattttatcattaagtatgacatttgtgttttcagaacatatattccctaccaagttacaggagttaattttaattcccaacttaatagtattttagtgtcatctatgggtgttaaattccatcaagtgatttatcagcatatactgagataatccttatgagttttatctggtagttaattaaaatattttctaatattaaatcttccaaacatactcttctgttttttgagacagggtctagttctgtcacccagggtggagtacagtggtacgatctcagctcactgcaacttccgcctcctagattcaagtgattctcccgtcccagcctcccaagtagctgggattataggtgtcagttaccatgccctgctatttttttgtatttttagtagagaggggtttcaccatgttggccaggctggtctcaaactcctgacctcaggtgatccaccatctcagcctcctgaagtgctgggattataggtgtgagccaccgtgcctggccccatatatctctttttaagtgggcatactgccattataaataatagtgattctgctggtaatgaacaaaggatgctggatccactaatagtctgttaaacctaatatcatgactttcttgttagctatacattggtttgctataattccatttagaatttttaaacctatgttcacaaatatggatttttaaacctatgttcacaaatatggatttttaaacctatgttcacaaatatggtttgcaagtcattttttctcctaaatttctatttgatggggaagttgtaaaatattggggttatttttccttggattttccttataataactattcctgaaaagtctctggaatgtctttcttttctggggctggggtagaaggactagatagatttacaaaccagtaactcaatttctgttttgtaaaattttcatttcattaaataataagtcctaatcaagtattattctttcccacagtatgtgagtgctgtcctcaatactgtcaacacttctggcttctaccaggcaaggctgcatgtagatttgcatctgaaaaaacaacaaactaaaatctaaccctaggtagtagtaaactgaatataaactttctcttatgaatttattctgtcttctttggtacatcaataataatatacacctttacagtatttcccagattgggggatacactttagcaagtatctgcgattatttgtttatgtaagatgtcccttcccttctgtgaatcatcattcttcaccccaagtatcttgagattggattctgtataagcagaatacaacagttaggcattcaggtatcattaaattcctccgcttcaaggatgaaaatttctttgggtatctaatagagtacaaagcagaaggtgtttcagaaatatttgcagtattgaatccgcatattcctccaagatagccctaatctaactggcagggtcccactcttcccagattaatgcccactcacataacaaacctgatgaggtagtgaagaaaactaactttgtgagtaagcaactggcagagtttttcaccactgtgactctatagctacatgtaactaagtagtatcactgacacataatcttaaattgaagttttaagatcattattctccatgttatacatgggtatcaaaagcattcccctcttgaccactccagaattctgtttaaaatttttcaatgacaacttatccatttccccaaagcctcagtgagcacatgatgccaacaattcatttcatgacttcatagcatgggccaagtttcttgcttaaaagacttccatcctgtcttgggaaacaaccatttccaaatatccacatatccttgcaagtttctgcctactcctctaccacccatttctgaagccatctgatttagtaagctgtatgcaaaagatacacaatggctaatgcaatcaaacaaggaatgtattaaaagcacacccaatagctcaaaataaaagacaagtgaacaaagttaagaaaatgacagtaacaaaagctgttctgggaacctctattgaaatagctacttattacatcaacatgctaccacagaacaaaagctcatgttgcttttctgaacttgaaaaacccattaacaatgtacagttctgagcctcagctgaccatagtgctcatgccaagtcctgagcagggcatcttgaatggtggttccctcatgactacatacaccgttagggaatgtttcgttaagaggaaatcaagatgttctaacctgtgaaggtagaatagattccaggctacacaaacacatgaagtgtgccttatattgattactaaagaggttgctgccaagactgcttccaaagggcagaagatagccctaaaaaatgtttgcagtgtggaaatgcatttttagtaagtcatattctagtaacaagttgcatttggtaagacacaaagaaacaatgttggtatgcagagtagaaatctctggaagatgatattgtcatatcagagatattgtcagtatcagagatactgaaatctctggaagatgatttttgtctcacatatggcattcgcaagtaaaatgccaaactgcaaaattcatattatgtagtacacataggaagatatctaaatatccctgtaggctctgggatgttatttcttattcttaacctccttactagattcacttgtacaatgaaataatctgtatcttattatttataattgagaattttctcaaaccttttcctgaaattttggaacacctggaataaaatttcttaaaatgattcctaaaagaaataattcttcaaaattaatattaagatataataacaggttggtttttttttttttttttttttttttttttagaatgaagcttctaaggtgaggttaacagtccagctgtggtttatttggtacattcataagatgttcactcctatatatattttttccctaggggtttctcatttctagatttacactttcccttatagcatggtccctccaaggtatatgcttccgatacataaaatgtttgtaattttgttaattctgccattcattagctcaataatttctctcattaaaattctgtaaactatgaatttcaaagaagtctattctatattcatctggttcatgaagtttcctctttgtgaatcttattttagtaaaatgactttacaacgtttaacatggttcctcacctgtatgaactttttaaaaaaaggtatgacttgctgctaaaaattttcagagtggttactaaattcagttttcctgtgtattgtctactatctttttgcatgtaaagaacagctttctgtggatgcctttccatatgctgtgcattcataaagtttctattcagtatgagttttctggaagatgacaagatgattccacttacagagtttctctttatatatgattgtttctatctcttgtgaatccacttttcagagtttcgtaaaattatcaatgtttgtcatctacatgagttctctgatgcataatgagctgtgacttccaacaaaaggctttcccacattcagtgcacttacaaggcttctctcctgtatgtgttctctgatgtgcactgagaattgatttttgagagaaggttttcccacattcattgcacccatagggtttctctcctgaatgagttctttgatgtacaatgagttgagaattcctaatgaaggcttttccacactcactgcattcatatggtttctctcttgtgtgcattctctggtgtacaagaaggcgtaatttcccactgaaggatttctcacattgactgcatttataagggttgacccctgcatgagttcgctcatgtacaatgagtagtgatttccaaatgaaggctttcccacattcattacattcatatggtttttcacctgaatgagttctcatgtgtataattaggtatgacttgctgctaaaagctttcccacattcactgcacccataaggcttttcccctgcatgagttcgctgatgtgaaatgagctggtctttcctattaaaggctttcccacattcactgcattcatagggattttctcctgtgtgaattctctgatgcacaatgagttgtgaattgaaactaaaggatttcccgcattccctgcactcatgtggtttctctcctgtatgagttctcatatgtataataaggtatgacttgctcctgaaggctttcccacactcactgcatccatatggttttactcctgtgtgacttctctgatgtacaatgagctgggacttcaaactaaaggtttttgcacattgactgcatccatagggttttactccagtgtgcactcctttatgtacaatgagctgtgatttgaacgtaaaggcttttccacattcattacaactatagggtttctctcctgtatgagttctctgatgtacaatcaggtttgactttgtattaaaggctttctgacactcactacattcaaatggtttctcccctgtatgagttctctggtgtataataagctgtgactttaaaccaaaagcctttccacagtcggtgcattcataaggcttctctcctgcatgagttctctggtgtgaaataagctggtatttccgactgaaggctttcccacattcatggcattcataggggttctctcctgtatgaatcctctgatgtataatgagctgtgatttaaaactgaaggctttcccacaattgttgcattcatggagtttttctcctgtatgagtccttgtatgtataataaggtatgacttgctcctgaaggctttgccacattcattgcatacataaggtttcattcctgtgtgacttctctgatgtacaatgagctgtgatttcaaactgaatcctttaccacactgaatacacccatagggctttactcctgtgtgaatcccctgatgtacaatgagctgtgacttgaatgtaaaggcttttccacaatcactacaaacataaggtttctcccctgtatgggttctctgatgtaccataaggtttgactttgtattaaaggctttctgacattcattgcattcatatggtttctctcctgtatgaattctttcatgtataatgagctgtgattttaaaccaaaagctttcccacattcattacacacatatggtttctgtcctgaatgagttttctggtgtgaaacaagctggtctttcctactgaagactttcccacattcacagcactcatagggattctcacctgtgtgaattctctgatgtataacaagctgtgaatggaaactgaatgttttcctgcattcactgcattcatgtagtttctctcctgtatgaattctctgatgtacaatgaggtatgatttactactgaagtctttcccacattcattacaaccatagggtttctcttcggcatgagtttgctgatgcactagaaggtatgacttgctgctgaaggctttctcacaacagctgcatccaaagggtttttcgcccatatacatttgttggcacataagttgcgatttcttattgacggtttttccagattcaatactttcacagtattttattccaataacagtttgctcatgtttagaatggaagaatgattttccatgtacctgaaacccattaggattatttctagcataatcactagtgaaatctatatatttcaaactctttccatgcgtgccacatttatgaggtttttgtcttgaaagatactttgtactaagaagacatagttttccaaatgtagtgcattcaaagctttttgccgtacttcccagcttgtctttattttcctgatgccaatccataagatcatcaattttccagactgtgtccaggacttggtgatttttggctgctcttgggaaataaacagccactctaggactttctctattctgcgactcttctgcttctgcctgggtgttccagggagaggttgcagaccaggagtcccttggcccaagatggattcctgaccttggagctttctgatcctatcccatgaactgtttcgttcttggagaggtgggacccaaatagaagctgtccggaccctggtggccatccctacggtcagttttgtgtgcctcgctggaagtgacaggacgcgagggatgctccggctcctccaaaccctgaaggggcagcagaatagagtccagggtactgcctccacctccagatctgcagccagaagggttcgcaaccactccagactcggctggcccgttgaccacgacgggcgatgaacgctatctgaggaacaaggatctcgccatcggcgcggaacaatggcggccgctacgtat

SEQ ID NO: 13687 - RNA, 8050 nt, Homo sapiens
  source 1..8050: mol_type = other RNA
gctgggattacaggcatgagccaccatgcccagcctttttattaatgttttaatggcctgtgtttctaacaagtagttgaaacaatgttgaaaattaaagagtagacatgttaaaacttgcaacttcatttaaatttaaatatatcatttataccaaaatcagaatttatttaagatttatggctgggtgcttggctcacacctgtaatcctagcactttgggaggccaaggcaggtggactgcttgagcccaggagtttgaaaccagactggaaaacatggtaaaaccccatctctacaagaaataaataactctacctggccctttagcaaagaattaagaaaaatcaatacagaccagtggctcacacctgtaatcccagcactttgggaggctgagggtggatcacgaggtcaggagttcaagaccagcctggccaacatggtgaaaccccatctctactaaaaacacaaaaattagctgggcgtggtggcgtgtgcctgtaattccagctactagggaggctgaggcaggagaattgcttgaacccaggaggcagaggttgcagtgagccaagaacacaccactgcactccagcctggcaatacagcgagactccatctcaaaaaaaaaaaaaaaaatgcaaatactatgccatataaggagcttgagcatccacagggagtatctgtggttgcgggggggtcctccatgaatactgacaactgcatacttgctactctactggcagttccaaacatttgtttgtggtttattttgggtttcctaattacacgatcacatctccaattcatggcagttgtttctgcacccatccctaattcctcacattccttgttttcacaccttggctagatgttactcatttcataaaagtgatgcgcattcttgtaattttgctttgttttttacagacagggtctcactttgttgcccaggatggagtgcaggggcatgatcatagctcactgtagccttgaactactggactcaagctaacctcctgcctcagcctcctcagtaggtgggactaccggcacttgccactacacctggctgatcttttttttgagatggaggcttgttctgtcgcccagcctggagtgcagtggtgcaatcttggctcactgcaactgccacctcctaggttcaagcaattcttctgcctcagcctcccgagtagatgggattacaggcacgtgccaccacacctggctgacttttgtatttttagtagagacggggtttcaccatgttagccacactggtcttgaaatcctgacctcaagtgatctgcccacctcggcctcccaaagtgctgggattacaggcatgagccacggcgcctgaccacacctggctaatctttttaaaaagtttttgtacagacagggtctccctatattggtcaggcttgtctcgaactcctgggttccagcaatcctccagcctcagccttcccaagtgctggtattacatggatgagccactgcacctggctaattttactttaaaggaatctttctactattttatcattaagtatgacatttgtgttttcagaacatatattccctaccaagttacaggagttaattttaattcccaacttaatagtattttagtgtcatctatgggtgttaaattccatcaagtgatttatcagcatatactgagataatccttatgagttttatctggtagttaattaaaatattttctaatattaaatcttccaaacatactcttctgttttttgagacagggtctagttctgtcacccagggtggagtacagtggtacgatctcagctcactgcaacttccgcctcctagattcaagtgattctcccgtcccagcctcccaagtagctgggattataggtgtcagttaccatgccctgctatttttttgtatttttagtagagaggggtttcaccatgttggccaggctggtctcaaactcctgacctcaggtgatccaccatctcagcctcctgaagtgctgggattataggtgtgagccaccgtgcctggccccatatatctctttttaagtgggcatactgccattataaataatagtgattctgctggtaatgaacaaaggatgctggatccactaatagtctgttaaacctaatatcatgactttcttgttagctatacattggtttgctataattccatttagaatttttaaacctatgttcacaaatatggatttttaaacctatgttcacaaatatggatttttaaacctatgttcacaaatatggtttgcaagtcattttttctcctaaatttctatttgatggggaagttgtaaaatattggggttatttttccttggattttccttataataactattcctgaaaagtctctggaatgtctttcttttctggggctggggtagaaggactagatagatttacaaaccagtaactcaatttctgttttgtaaaattttcatttcattaaataataagtcctaatcaagtattattctttcccacagtatgtgagtgctgtcctcaatactgtcaacacttctggcttctaccaggcaaggctgcatgtagatttgcatctgaaaaaacaacaaactaaaatctaaccctaggtagtagtaaactgaatataaactttctcttatgaatttattctgtcttctttggtacatcaataataatatacacctttacagtatttcccagattgggggatacactttagcaagtatctgcgattatttgtttatgtaagatgtcccttcccttctgtgaatcatcattcttcaccccaagtatcttgagattggattctgtataagcagaatacaacagttaggcattcaggtatcattaaattcctccgcttcaaggatgaaaatttctttgggtatctaatagagtacaaagcagaaggtgtttcagaaatatttgcagtattgaatccgcatattcctccaagatagccctaatctaactggcagggtcccactcttcccagattaatgcccactcacataacaaacctgatgaggtagtgaagaaaactaactttgtgagtaagcaactggcagagtttttcaccactgtgactctatagctacatgtaactaagtagtatcactgacacataatcttaaattgaagttttaagatcattattctccatgttatacatgggtatcaaaagcattcccctcttgaccactccagaattctgtttaaaatttttcaatgacaacttatccatttccccaaagcctcagtgagcacatgatgccaacaattcatttcatgacttcatagcatgggccaagtttcttgcttaaaagacttccatcctgtcttgggaaacaaccatttccaaatatccacatatccttgcaagtttctgcctactcctctaccacccatttctgaagccatctgatttagtaagctgtatgcaaaagatacacaatggctaatgcaatcaaacaaggaatgtattaaaagcacacccaatagctcaaaataaaagacaagtgaacaaagttaagaaaatgacagtaacaaaagctgttctgggaacctctattgaaatagctacttattacatcaacatgctaccacagaacaaaagctcatgttgcttttctgaacttgaaaaacccattaacaatgtacagttctgagcctcagctgaccatagtgctcatgccaagtcctgagcagggcatcttgaatggtggttccctcatgactacatacaccgttagggaatgtttcgttaagaggaaatcaagatgttctaacctgtgaaggtagaatagattccaggctacacaaacacatgaagtgtgccttatattgattactaaagaggttgctgccaagactgcttccaaagggcagaagatagccctaaaaaatgtttgcagtgtggaaatgcatttttagtaagtcatattctagtaacaagttgcatttggtaagacacaaagaaacaatgttggtatgcagagtagaaatctctggaagatgatattgtcatatcagagatattgtcagtatcagagatactgaaatctctggaagatgatttttgtctcacatatggcattcgcaagtaaaatgccaaactgcaaaattcatattatgtagtacacataggaagatatctaaatatccctgtaggctctgggatgttatttcttattcttaacctccttactagattcacttgtacaatgaaataatctgtatcttattatttataattgagaattttctcaaaccttttcctgaaattttggaacacctggaataaaatttcttaaaatgattcctaaaagaaataattcttcaaaattaatattaagatataataacaggttggtttttttttttttttttttttttttttttagaatgaagcttctaaggtgaggttaacagtccagctgtggtttatttggtacattcataagatgttcactcctatatatattttttccctaggggtttctcatttctagatttacactttcccttatagcatggtccctccaaggtatatgcttccgatacataaaatgtttgtaattttgttaattctgccattcattagctcaataatttctctcattaaaattctgtaaactatgaatttcaaagaagtctattctatattcatctggttcatgaagtttcctctttgtgaatcttattttagtaaaatgactttacaacgtttaacatggttcctcacctgtatgaactttttaaaaaaaggtatgacttgctgctaaaaattttcagagtggttactaaattcagttttcctgtgtattgtctactatctttttgcatgtaaagaacagctttctgtggatgcctttccatatgctgtgcattcataaagtttctattcagtatgagttttctggaagatgacaagatgattccacttacagagtttctctttatatatgattgtttctatctcttgtgaatccacttttcagagtttcgtaaaattatcaatgtttgtcatctacatgagttctctgatgcataatgagctgtgacttccaacaaaaggctttcccacattcagtgcacttacaaggcttctctcctgtatgtgttctctgatgtgcactgagaattgatttttgagagaaggttttcccacattcattgcacccatagggtttctctcctgaatgagttctttgatgtacaatgagttgagaattcctaatgaaggcttttccacactcactgcattcatatggtttctctcttgtgtgcattctctggtgtacaagaaggcgtaatttcccactgaaggatttctcacattgactgcatttataagggttgacccctgcatgagttcgctcatgtacaatgagtagtgatttccaaatgaaggctttcccacattcattacattcatatggtttttcacctgaatgagttctcatgtgtataattaggtatgacttgctgctaaaagctttcccacattcactgcacccataaggcttttcccctgcatgagttcgctgatgtgaaatgagctggtctttcctattaaaggctttcccacattcactgcattcatagggattttctcctgtgtgaattctctgatgcacaatgagttgtgaattgaaactaaaggatttcccgcattccctgcactcatgtggtttctctcctgtatgagttctcatatgtataataaggtatgacttgctcctgaaggctttcccacactcactgcatccatatggttttactcctgtgtgacttctctgatgtacaatgagctgggacttcaaactaaaggtttttgcacattgactgcatccatagggttttactccagtgtgcactcctttatgtacaatgagctgtgatttgaacgtaaaggcttttccacattcattacaactatagggtttctctcctgtatgagttctctgatgtacaatcaggtttgactttgtattaaaggctttctgacactcactacattcaaatggtttctcccctgtatgagttctctggtgtataataagctgtgactttaaaccaaaagcctttccacagtcggtgcattcataaggcttctctcctgcatgagttctctggtgtgaaataagctggtatttccgactgaaggctttcccacattcatggcattcataggggttctctcctgtatgaatcctctgatgtataatgagctgtgatttaaaactgaaggctttcccacaattgttgcattcatggagtttttctcctgtatgagtccttgtatgtataataaggtatgacttgctcctgaaggctttgccacattcattgcatacataaggtttcattcctgtgtgacttctctgatgtacaatgagctgtgatttcaaactgaatcctttaccacactgaatacacccatagggctttactcctgtgtgaatcccctgatgtacaatgagctgtgacttgaatgtaaaggcttttccacaatcactacaaacataaggtttctcccctgtatgggttctctgatgtaccataaggtttgactttgtattaaaggctttctgacattcattgcattcatatggtttctctcctgtatgaattctttcatgtataatgagctgtgattttaaaccaaaagctttcccacattcattacacacatatggtttctgtcctgaatgagttttctggtgtgaaacaagctggtctttcctactgaagactttcccacattcacagcactcatagggattctcacctgtgtgaattctctgatgtataacaagctgtgaatggaaactgaatgttttcctgcattcactgcattcatgtagtttctctcctgtatgaattctctgatgtacaatgaggtatgatttactactgaagtctttcccacattcattacaaccatagggtttctcttcggcatgagtttgctgatgcactagaaggtatgacttgctgctgaaggctttctcacaacagctgcatccaaagggtttttcgcccatatacatttgttggcacataagttgcgatttcttattgacggtttttccagattcaatactttcacagtattttattccaataacagtttgctcatgtttagaatggaagaatgattttccatgtacctgaaacccattaggattatttctagcataatcactagtgaaatctatatatttcaaactctttccatgcgtgccacatttatgaggtttttgtcttgaaagatactttgtactaagaagacatagttttccaaatgtagtgcattcaaagctttttgccgtacttcccagcttgtctttattttcctgatgccaatccataagatcatcaattttccagactgtgtctccagaggatgcagcaacaaggcgtcatcttggaagcacagagcaggccctcaccagacaccaaacctgccagcaccttggctttggactttccagccttcaaaattggacaggtctgatttggaacttgggcctgcaccatacacagctcttctccttgttccaacttgaagatgatatcaggtttggtgtgttggtaccctagggacaccaggttgctatagttctccaacatcacactcctgtacaggcacttctgtgctgggtctagcagctgccactcctcccaggtaaaatccacaaacacatccatgaatgacaaaggtccccaaatagaagctgtccggaccctggtggccatccctacggtcagttttgtgtgcctcgctggaagtgacaggacgcgagggatgctccggctcctccaaaccctgaaggggcagcagaatagagtccagggtactgcctccacctccagatctgcagccagaagggttcgcaaccactccagactcggctggcccgttgaccacgacgggcgatgaacgctatctgaggaacaaggatctcgccatcggcgcggaacaatggcggccgctacgtat

SEQ ID NO: 13688 - RNA, 8251 nt, Homo sapiens
  source 1..8251: mol_type = other RNA
gctgggattacaggcatgagccaccatgcccagcctttttattaatgttttaatggcctgtgtttctaacaagtagttgaaacaatgttgaaaattaaagagtagacatgttaaaacttgcaacttcatttaaatttaaatatatcatttataccaaaatcagaatttatttaagatttatggctgggtgcttggctcacacctgtaatcctagcactttgggaggccaaggcaggtggactgcttgagcccaggagtttgaaaccagactggaaaacatggtaaaaccccatctctacaagaaataaataactctacctggccctttagcaaagaattaagaaaaatcaatacagaccagtggctcacacctgtaatcccagcactttgggaggctgagggtggatcacgaggtcaggagttcaagaccagcctggccaacatggtgaaaccccatctctactaaaaacacaaaaattagctgggcgtggtggcgtgtgcctgtaattccagctactagggaggctgaggcaggagaattgcttgaacccaggaggcagaggttgcagtgagccaagaacacaccactgcactccagcctggcaatacagcgagactccatctcaaaaaaaaaaaaaaaaatgcaaatactatgccatataaggagcttgagcatccacagggagtatctgtggttgcgggggggtcctccatgaatactgacaactgcatacttgctactctactggcagttccaaacatttgtttgtggtttattttgggtttcctaattacacgatcacatctccaattcatggcagttgtttctgcacccatccctaattcctcacattccttgttttcacaccttggctagatgttactcatttcataaaagtgatgcgcattcttgtaattttgctttgttttttacagacagggtctcactttgttgcccaggatggagtgcaggggcatgatcatagctcactgtagccttgaactactggactcaagctaacctcctgcctcagcctcctcagtaggtgggactaccggcacttgccactacacctggctgatcttttttttgagatggaggcttgttctgtcgcccagcctggagtgcagtggtgcaatcttggctcactgcaactgccacctcctaggttcaagcaattcttctgcctcagcctcccgagtagatgggattacaggcacgtgccaccacacctggctgacttttgtatttttagtagagacggggtttcaccatgttagccacactggtcttgaaatcctgacctcaagtgatctgcccacctcggcctcccaaagtgctgggattacaggcatgagccacggcgcctgaccacacctggctaatctttttaaaaagtttttgtacagacagggtctccctatattggtcaggcttgtctcgaactcctgggttccagcaatcctccagcctcagccttcccaagtgctggtattacatggatgagccactgcacctggctaattttactttaaaggaatctttctactattttatcattaagtatgacatttgtgttttcagaacatatattccctaccaagttacaggagttaattttaattcccaacttaatagtattttagtgtcatctatgggtgttaaattccatcaagtgatttatcagcatatactgagataatccttatgagttttatctggtagttaattaaaatattttctaatattaaatcttccaaacatactcttctgttttttgagacagggtctagttctgtcacccagggtggagtacagtggtacgatctcagctcactgcaacttccgcctcctagattcaagtgattctcccgtcccagcctcccaagtagctgggattataggtgtcagttaccatgccctgctatttttttgtatttttagtagagaggggtttcaccatgttggccaggctggtctcaaactcctgacctcaggtgatccaccatctcagcctcctgaagtgctgggattataggtgtgagccaccgtgcctggccccatatatctctttttaagtgggcatactgccattataaataatagtgattctgctggtaatgaacaaaggatgctggatccactaatagtctgttaaacctaatatcatgactttcttgttagctatacattggtttgctataattccatttagaatttttaaacctatgttcacaaatatggatttttaaacctatgttcacaaatatggatttttaaacctatgttcacaaatatggtttgcaagtcattttttctcctaaatttctatttgatggggaagttgtaaaatattggggttatttttccttggattttccttataataactattcctgaaaagtctctggaatgtctttcttttctggggctggggtagaaggactagatagatttacaaaccagtaactcaatttctgttttgtaaaattttcatttcattaaataataagtcctaatcaagtattattctttcccacagtatgtgagtgctgtcctcaatactgtcaacacttctggcttctaccaggcaaggctgcatgtagatttgcatctgaaaaaacaacaaactaaaatctaaccctaggtagtagtaaactgaatataaactttctcttatgaatttattctgtcttctttggtacatcaataataatatacacctttacagtatttcccagattgggggatacactttagcaagtatctgcgattatttgtttatgtaagatgtcccttcccttctgtgaatcatcattcttcaccccaagtatcttgagattggattctgtataagcagaatacaacagttaggcattcaggtatcattaaattcctccgcttcaaggatgaaaatttctttgggtatctaatagagtacaaagcagaaggtgtttcagaaatatttgcagtattgaatccgcatattcctccaagatagccctaatctaactggcagggtcccactcttcccagattaatgcccactcacataacaaacctgatgaggtagtgaagaaaactaactttgtgagtaagcaactggcagagtttttcaccactgtgactctatagctacatgtaactaagtagtatcactgacacataatcttaaattgaagttttaagatcattattctccatgttatacatgggtatcaaaagcattcccctcttgaccactccagaattctgtttaaaatttttcaatgacaacttatccatttccccaaagcctcagtgagcacatgatgccaacaattcatttcatgacttcatagcatgggccaagtttcttgcttaaaagacttccatcctgtcttgggaaacaaccatttccaaatatccacatatccttgcaagtttctgcctactcctctaccacccatttctgaagccatctgatttagtaagctgtatgcaaaagatacacaatggctaatgcaatcaaacaaggaatgtattaaaagcacacccaatagctcaaaataaaagacaagtgaacaaagttaagaaaatgacagtaacaaaagctgttctgggaacctctattgaaatagctacttattacatcaacatgctaccacagaacaaaagctcatgttgcttttctgaacttgaaaaacccattaacaatgtacagttctgagcctcagctgaccatagtgctcatgccaagtcctgagcagggcatcttgaatggtggttccctcatgactacatacaccgttagggaatgtttcgttaagaggaaatcaagatgttctaacctgtgaaggtagaatagattccaggctacacaaacacatgaagtgtgccttatattgattactaaagaggttgctgccaagactgcttccaaagggcagaagatagccctaaaaaatgtttgcagtgtggaaatgcatttttagtaagtcatattctagtaacaagttgcatttggtaagacacaaagaaacaatgttggtatgcagagtagaaatctctggaagatgatattgtcatatcagagatattgtcagtatcagagatactgaaatctctggaagatgatttttgtctcacatatggcattcgcaagtaaaatgccaaactgcaaaattcatattatgtagtacacataggaagatatctaaatatccctgtaggctctgggatgttatttcttattcttaacctccttactagattcacttgtacaatgaaataatctgtatcttattatttataattgagaattttctcaaaccttttcctgaaattttggaacacctggaataaaatttcttaaaatgattcctaaaagaaataattcttcaaaattaatattaagatataataacaggttggtttttttttttttttttttttttttttttagaatgaagcttctaaggtgaggttaacagtccagctgtggtttatttggtacattcataagatgttcactcctatatatattttttccctaggggtttctcatttctagatttacactttcccttatagcatggtccctccaaggtatatgcttccgatacataaaatgtttgtaattttgttaattctgccattcattagctcaataatttctctcattaaaattctgtaaactatgaatttcaaagaagtctattctatattcatctggttcatgaagtttcctctttgtgaatcttattttagtaaaatgactttacaacgtttaacatggttcctcacctgtatgaactttttaaaaaaaggtatgacttgctgctaaaaattttcagagtggttactaaattcagttttcctgtgtattgtctactatctttttgcatgtaaagaacagctttctgtggatgcctttccatatgctgtgcattcataaagtttctattcagtatgagttttctggaagatgacaagatgattccacttacagagtttctctttatatatgattgtttctatctcttgtgaatccacttttcagagtttcgtaaaattatcaatgtttgtcatctacatgagttctctgatgcataatgagctgtgacttccaacaaaaggctttcccacattcagtgcacttacaaggcttctctcctgtatgtgttctctgatgtgcactgagaattgatttttgagagaaggttttcccacattcattgcacccatagggtttctctcctgaatgagttctttgatgtacaatgagttgagaattcctaatgaaggcttttccacactcactgcattcatatggtttctctcttgtgtgcattctctggtgtacaagaaggcgtaatttcccactgaaggatttctcacattgactgcatttataagggttgacccctgcatgagttcgctcatgtacaatgagtagtgatttccaaatgaaggctttcccacattcattacattcatatggtttttcacctgaatgagttctcatgtgtataattaggtatgacttgctgctaaaagctttcccacattcactgcacccataaggcttttcccctgcatgagttcgctgatgtgaaatgagctggtctttcctattaaaggctttcccacattcactgcattcatagggattttctcctgtgtgaattctctgatgcacaatgagttgtgaattgaaactaaaggatttcccgcattccctgcactcatgtggtttctctcctgtatgagttctcatatgtataataaggtatgacttgctcctgaaggctttcccacactcactgcatccatatggttttactcctgtgtgacttctctgatgtacaatgagctgggacttcaaactaaaggtttttgcacattgactgcatccatagggttttactccagtgtgcactcctttatgtacaatgagctgtgatttgaacgtaaaggcttttccacattcattacaactatagggtttctctcctgtatgagttctctgatgtacaatcaggtttgactttgtattaaaggctttctgacactcactacattcaaatggtttctcccctgtatgagttctctggtgtataataagctgtgactttaaaccaaaagcctttccacagtcggtgcattcataaggcttctctcctgcatgagttctctggtgtgaaataagctggtatttccgactgaaggctttcccacattcatggcattcataggggttctctcctgtatgaatcctctgatgtataatgagctgtgatttaaaactgaaggctttcccacaattgttgcattcatggagtttttctcctgtatgagtccttgtatgtataataaggtatgacttgctcctgaaggctttgccacattcattgcatacataaggtttcattcctgtgtgacttctctgatgtacaatgagctgtgatttcaaactgaatcctttaccacactgaatacacccatagggctttactcctgtgtgaatcccctgatgtacaatgagctgtgacttgaatgtaaaggcttttccacaatcactacaaacataaggtttctcccctgtatgggttctctgatgtaccataaggtttgactttgtattaaaggctttctgacattcattgcattcatatggtttctctcctgtatgaattctttcatgtataatgagctgtgattttaaaccaaaagctttcccacattcattacacacatatggtttctgtcctgaatgagttttctggtgtgaaacaagctggtctttcctactgaagactttcccacattcacagcactcatagggattctcacctgtgtgaattctctgatgtataacaagctgtgaatggaaactgaatgttttcctgcattcactgcattcatgtagtttctctcctgtatgaattctctgatgtacaatgaggtatgatttactactgaagtctttcccacattcattacaaccatagggtttctcttcggcatgagtttgctgatgcactagaaggtatgacttgctgctgaaggctttctcacaacagctgcatccaaagggtttttcgcccatatacatttgttggcacataagttgcgatttcttattgacggtttttccagattcaatactttcacagtattttattccaataacagtttgctcatgtttagaatggaagaatgattttccatgtacctgaaacccattaggattatttctagcataatcactagtgaaatctatatatttcaaactctttccatgcgtgccacatttatgaggtttttgtcttgaaagatactttgtactaagaagacatagttttccaaatgtagtgcattcaaagctttttgccgtacttcccagcttgtctttattttcctgatgccaatccataagatcatcaattttccagactgtgtctccagaggatgcagcaacaaggcgtcatcttggaagcacagagcaggccctcaccagacaccaaacctgccagcaccttggctttggactttccagccttcaaaattggacaggtctgatttggaacttgggcctgcaccatacacagctcttctccttgttccaacttgaagatgatatcaggtttggtgtgttggtaccctagggacaccaggttgctatagttctccaacatcacactcctgtacaggcacttctgtgctgggtctagcagctgccactcctcccaggtaaaatccacaaacacatccatgaatgacaaaggtccccaggacttggtgatttttggctgctcttgggaaataaacagccactctaggactttctctattctgcgactcttctgcttctgcctgggtgttccagggagaggttgcagaccaggagtcccttggcccaagatggattcctgaccttggagctttctgatcctatcccatgaactgtttcgttcttggagaggtgggacccaaatagaagctgtccggaccctggtggccatccctacggtcagttttgtgtgcctcgctggaagtgacaggacgcgagggatgctccggctcctccaaaccctgaaggggcagcagaatagagtccagggtactgcctccacctccagatctgcagccagaagggttcgcaaccactccagactcggctggcccgttgaccacgacgggcgatgaacgctatctgaggaacaaggatctcgccatcggcgcggaacaatggcggccgctacgtat

SEQ ID NO: 13689 - RNA, 7817 nt, Homo sapiens
  source 1..7817: mol_type = other RNA
gctgggattacaggcatgagccaccatgcccagcctttttattaatgttttaatggcctgtgtttctaacaagtagttgaaacaatgttgaaaattaaagagtagacatgttaaaacttgcaacttcatttaaatttaaatatatcatttataccaaaatcagaatttatttaagatttatggctgggtgcttggctcacacctgtaatcctagcactttgggaggccaaggcaggtggactgcttgagcccaggagtttgaaaccagactggaaaacatggtaaaaccccatctctacaagaaataaataactctacctggccctttagcaaagaattaagaaaaatcaatacagaccagtggctcacacctgtaatcccagcactttgggaggctgagggtggatcacgaggtcaggagttcaagaccagcctggccaacatggtgaaaccccatctctactaaaaacacaaaaattagctgggcgtggtggcgtgtgcctgtaattccagctactagggaggctgaggcaggagaattgcttgaacccaggaggcagaggttgcagtgagccaagaacacaccactgcactccagcctggcaatacagcgagactccatctcaaaaaaaaaaaaaaaaatgcaaatactatgccatataaggagcttgagcatccacagggagtatctgtggttgcgggggggtcctccatgaatactgacaactgcatacttgctactctactggcagttccaaacatttgtttgtggtttattttgggtttcctaattacacgatcacatctccaattcatggcagttgtttctgcacccatccctaattcctcacattccttgttttcacaccttggctagatgttactcatttcataaaagtgatgcgcattcttgtaattttgctttgttttttacagacagggtctcactttgttgcccaggatggagtgcaggggcatgatcatagctcactgtagccttgaactactggactcaagctaacctcctgcctcagcctcctcagtaggtgggactaccggcacttgccactacacctggctgatcttttttttgagatggaggcttgttctgtcgcccagcctggagtgcagtggtgcaatcttggctcactgcaactgccacctcctaggttcaagcaattcttctgcctcagcctcccgagtagatgggattacaggcacgtgccaccacacctggctgacttttgtatttttagtagagacggggtttcaccatgttagccacactggtcttgaaatcctgacctcaagtgatctgcccacctcggcctcccaaagtgctgggattacaggcatgagccacggcgcctgaccacacctggctaatctttttaaaaagtttttgtacagacagggtctccctatattggtcaggcttgtctcgaactcctgggttccagcaatcctccagcctcagccttcccaagtgctggtattacatggatgagccactgcacctggctaattttactttaaaggaatctttctactattttatcattaagtatgacatttgtgttttcagaacatatattccctaccaagttacaggagttaattttaattcccaacttaatagtattttagtgtcatctatgggtgttaaattccatcaagtgatttatcagcatatactgagataatccttatgagttttatctggtagttaattaaaatattttctaatattaaatcttccaaacatactcttctgttttttgagacagggtctagttctgtcacccagggtggagtacagtggtacgatctcagctcactgcaacttccgcctcctagattcaagtgattctcccgtcccagcctcccaagtagctgggattataggtgtcagttaccatgccctgctatttttttgtatttttagtagagaggggtttcaccatgttggccaggctggtctcaaactcctgacctcaggtgatccaccatctcagcctcctgaagtgctgggattataggtgtgagccaccgtgcctggccccatatatctctttttaagtgggcatactgccattataaataatagtgattctgctggtaatgaacaaaggatgctggatccactaatagtctgttaaacctaatatcatgactttcttgttagctatacattggtttgctataattccatttagaatttttaaacctatgttcacaaatatggatttttaaacctatgttcacaaatatggatttttaaacctatgttcacaaatatggtttgcaagtcattttttctcctaaatttctatttgatggggaagttgtaaaatattggggttatttttccttggattttccttataataactattcctgaaaagtctctggaatgtctttcttttctggggctggggtagaaggactagatagatttacaaaccagtaactcaatttctgttttgtaaaattttcatttcattaaataataagtcctaatcaagtattattctttcccacagtatgtgagtgctgtcctcaatactgtcaacacttctggcttctaccaggcaaggctgcatgtagatttgcatctgaaaaaacaacaaactaaaatctaaccctaggtagtagtaaactgaatataaactttctcttatgaatttattctgtcttctttggtacatcaataataatatacacctttacagtatttcccagattgggggatacactttagcaagtatctgcgattatttgtttatgtaagatgtcccttcccttctgtgaatcatcattcttcaccccaagtatcttgagattggattctgtataagcagaatacaacagttaggcattcaggtatcattaaattcctccgcttcaaggatgaaaatttctttgggtatctaatagagtacaaagcagaaggtgtttcagaaatatttgcagtattgaatccgcatattcctccaagatagccctaatctaactggcagggtcccactcttcccagattaatgcccactcacataacaaacctgatgaggtagtgaagaaaactaactttgtgagtaagcaactggcagagtttttcaccactgtgactctatagctacatgtaactaagtagtatcactgacacataatcttaaattgaagttttaagatcattattctccatgttatacatgggtatcaaaagcattcccctcttgaccactccagaattctgtttaaaatttttcaatgacaacttatccatttccccaaagcctcagtgagcacatgatgccaacaattcatttcatgacttcatagcatgggccaagtttcttgcttaaaagacttccatcctgtcttgggaaacaaccatttccaaatatccacatatccttgcaagtttctgcctactcctctaccacccatttctgaagccatctgatttagtaagctgtatgcaaaagatacacaatggctaatgcaatcaaacaaggaatgtattaaaagcacacccaatagctcaaaataaaagacaagtgaacaaagttaagaaaatgacagtaacaaaagctgttctgggaacctctattgaaatagctacttattacatcaacatgctaccacagaacaaaagctcatgttgcttttctgaacttgaaaaacccattaacaatgtacagttctgagcctcagctgaccatagtgctcatgccaagtcctgagcagggcatcttgaatggtggttccctcatgactacatacaccgttagggaatgtttcgttaagaggaaatcaagatgttctaacctgtgaaggtagaatagattccaggctacacaaacacatgaagtgtgccttatattgattactaaagaggttgctgccaagactgcttccaaagggcagaagatagccctaaaaaatgtttgcagtgtggaaatgcatttttagtaagtcatattctagtaacaagttgcatttggtaagacacaaagaaacaatgttggtatgcagagtagaaatctctggaagatgatattgtcatatcagagatattgtcagtatcagagatactgaaatctctggaagatgatttttgtctcacatatggcattcgcaagtaaaatgccaaactgcaaaattcatattatgtagtacacataggaagatatctaaatatccctgtaggctctgggatgttatttcttattcttaacctccttactagattcacttgtacaatgaaataatctgtatcttattatttataattgagaattttctcaaaccttttcctgaaattttggaacacctggaataaaatttcttaaaatgattcctaaaagaaataattcttcaaaattaatattaagatataataacaggttggtttttttttttttttttttttttttttttagaatgaagcttctaaggtgaggttaacagtccagctgtggtttatttggtacattcataagatgttcactcctatatatattttttccctaggggtttctcatttctagatttacactttcccttatagcatggtccctccaaggtatatgcttccgatacataaaatgtttgtaattttgttaattctgccattcattagctcaataatttctctcattaaaattctgtaaactatgaatttcaaagaagtctattctatattcatctggttcatgaagtttcctctttgtgaatcttattttagtaaaatgactttacaacgtttaacatggttcctcacctgtatgaactttttaaaaaaaggtatgacttgctgctaaaaattttcagagtggttactaaattcagttttcctgtgtattgtctactatctttttgcatgtaaagaacagctttctgtggatgcctttccatatgctgtgcattcataaagtttctattcagtatgagttttctggaagatgacaagatgattccacttacagagtttctctttatatatgattgtttctatctcttgtgaatccacttttcagagtttcgtaaaattatcaatgtttgtcatctacatgagttctctgatgcataatgagctgtgacttccaacaaaaggctttcccacattcagtgcacttacaaggcttctctcctgtatgtgttctctgatgtgcactgagaattgatttttgagagaaggttttcccacattcattgcacccatagggtttctctcctgaatgagttctttgatgtacaatgagttgagaattcctaatgaaggcttttccacactcactgcattcatatggtttctctcttgtgtgcattctctggtgtacaagaaggcgtaatttcccactgaaggatttctcacattgactgcatttataagggttgacccctgcatgagttcgctcatgtacaatgagtagtgatttccaaatgaaggctttcccacattcattacattcatatggtttttcacctgaatgagttctcatgtgtataattaggtatgacttgctgctaaaagctttcccacattcactgcacccataaggcttttcccctgcatgagttcgctgatgtgaaatgagctggtctttcctattaaaggctttcccacattcactgcattcatagggattttctcctgtgtgaattctctgatgcacaatgagttgtgaattgaaactaaaggatttcccgcattccctgcactcatgtggtttctctcctgtatgagttctcatatgtataataaggtatgacttgctcctgaaggctttcccacactcactgcatccatatggttttactcctgtgtgacttctctgatgtacaatgagctgggacttcaaactaaaggtttttgcacattgactgcatccatagggttttactccagtgtgcactcctttatgtacaatgagctgtgatttgaacgtaaaggcttttccacattcattacaactatagggtttctctcctgtatgagttctctgatgtacaatcaggtttgactttgtattaaaggctttctgacactcactacattcaaatggtttctcccctgtatgagttctctggtgtataataagctgtgactttaaaccaaaagcctttccacagtcggtgcattcataaggcttctctcctgcatgagttctctggtgtgaaataagctggtatttccgactgaaggctttcccacattcatggcattcataggggttctctcctgtatgaatcctctgatgtataatgagctgtgatttaaaactgaaggctttcccacaattgttgcattcatggagtttttctcctgtatgagtccttgtatgtataataaggtatgacttgctcctgaaggctttgccacattcattgcatacataaggtttcattcctgtgtgacttctctgatgtacaatgagctgtgatttcaaactgaatcctttaccacactgaatacacccatagggctttactcctgtgtgaatcccctgatgtacaatgagctgtgacttgaatgtaaaggcttttccacaatcactacaaacataaggtttctcccctgtatgggttctctgatgtaccataaggtttgactttgtattaaaggctttctgacattcattgcattcatatggtttctctcctgtatgaattctttcatgtataatgagctgtgattttaaaccaaaagctttcccacattcattacacacatatggtttctgtcctgaatgagttttctggtgtgaaacaagctggtctttcctactgaagactttcccacattcacagcactcatagggattctcacctgtgtgaattctctgatgtataacaagctgtgaatggaaactgaatgttttcctgcattcactgcattcatgtagtttctctcctgtatgaattctctgatgtacaatgaggtatgatttactactgaagtctttcccacattcattacaaccatagggtttctcttcggcatgagtttgctgatgcactagaaggtatgacttgctgctgaaggctttctcacaacagctgcatccaaagggtttttcgcccatatacatttgttggcacataagttgcgatttcttattgacggtttttccagattcaatactttcacagtattttattccaataacagtttgctcatgtttagaatggaagaatgattttccatgtacctgaaacccattaggattatttctagcataatcactagtgaaatctatatatttcaaactctttccatgcgtgccacatttatgaggtttttgtcttgaaagatactttgtactaagaagacatagttttccaaatgtagtgcattcaaagctttttgccgtacttcccagcttgtctttattttcctgatgccaatccataagatcatcaattttccagactgtgtttggacaggtctgatttggaacttgggcctgcaccatacacagctcttctccttgttccaacttgaagatgatatcaggtttggtgtgttggtaccccaaatagaagctgtccggaccctggtggccatccctacggtcagttttgtgtgcctcgctggaagtgacaggacgcgagggatgctccggctcctccaaaccctgaaggggcagcagaatagagtccagggtactgcctccacctccagatctgcagccagaagggttcgcaaccactccagactcggctggcccgttgaccacgacgggcgatgaacgctatctgaggaacaaggatctcgccatcggcgcggaacaatggcggccgctacgtat

SEQ ID NO: 13690 - RNA, 8018 nt, Homo sapiens
  source 1..8018: mol_type = other RNA
gctgggattacaggcatgagccaccatgcccagcctttttattaatgttttaatggcctgtgtttctaacaagtagttgaaacaatgttgaaaattaaagagtagacatgttaaaacttgcaacttcatttaaatttaaatatatcatttataccaaaatcagaatttatttaagatttatggctgggtgcttggctcacacctgtaatcctagcactttgggaggccaaggcaggtggactgcttgagcccaggagtttgaaaccagactggaaaacatggtaaaaccccatctctacaagaaataaataactctacctggccctttagcaaagaattaagaaaaatcaatacagaccagtggctcacacctgtaatcccagcactttgggaggctgagggtggatcacgaggtcaggagttcaagaccagcctggccaacatggtgaaaccccatctctactaaaaacacaaaaattagctgggcgtggtggcgtgtgcctgtaattccagctactagggaggctgaggcaggagaattgcttgaacccaggaggcagaggttgcagtgagccaagaacacaccactgcactccagcctggcaatacagcgagactccatctcaaaaaaaaaaaaaaaaatgcaaatactatgccatataaggagcttgagcatccacagggagtatctgtggttgcgggggggtcctccatgaatactgacaactgcatacttgctactctactggcagttccaaacatttgtttgtggtttattttgggtttcctaattacacgatcacatctccaattcatggcagttgtttctgcacccatccctaattcctcacattccttgttttcacaccttggctagatgttactcatttcataaaagtgatgcgcattcttgtaattttgctttgttttttacagacagggtctcactttgttgcccaggatggagtgcaggggcatgatcatagctcactgtagccttgaactactggactcaagctaacctcctgcctcagcctcctcagtaggtgggactaccggcacttgccactacacctggctgatcttttttttgagatggaggcttgttctgtcgcccagcctggagtgcagtggtgcaatcttggctcactgcaactgccacctcctaggttcaagcaattcttctgcctcagcctcccgagtagatgggattacaggcacgtgccaccacacctggctgacttttgtatttttagtagagacggggtttcaccatgttagccacactggtcttgaaatcctgacctcaagtgatctgcccacctcggcctcccaaagtgctgggattacaggcatgagccacggcgcctgaccacacctggctaatctttttaaaaagtttttgtacagacagggtctccctatattggtcaggcttgtctcgaactcctgggttccagcaatcctccagcctcagccttcccaagtgctggtattacatggatgagccactgcacctggctaattttactttaaaggaatctttctactattttatcattaagtatgacatttgtgttttcagaacatatattccctaccaagttacaggagttaattttaattcccaacttaatagtattttagtgtcatctatgggtgttaaattccatcaagtgatttatcagcatatactgagataatccttatgagttttatctggtagttaattaaaatattttctaatattaaatcttccaaacatactcttctgttttttgagacagggtctagttctgtcacccagggtggagtacagtggtacgatctcagctcactgcaacttccgcctcctagattcaagtgattctcccgtcccagcctcccaagtagctgggattataggtgtcagttaccatgccctgctatttttttgtatttttagtagagaggggtttcaccatgttggccaggctggtctcaaactcctgacctcaggtgatccaccatctcagcctcctgaagtgctgggattataggtgtgagccaccgtgcctggccccatatatctctttttaagtgggcatactgccattataaataatagtgattctgctggtaatgaacaaaggatgctggatccactaatagtctgttaaacctaatatcatgactttcttgttagctatacattggtttgctataattccatttagaatttttaaacctatgttcacaaatatggatttttaaacctatgttcacaaatatggatttttaaacctatgttcacaaatatggtttgcaagtcattttttctcctaaatttctatttgatggggaagttgtaaaatattggggttatttttccttggattttccttataataactattcctgaaaagtctctggaatgtctttcttttctggggctggggtagaaggactagatagatttacaaaccagtaactcaatttctgttttgtaaaattttcatttcattaaataataagtcctaatcaagtattattctttcccacagtatgtgagtgctgtcctcaatactgtcaacacttctggcttctaccaggcaaggctgcatgtagatttgcatctgaaaaaacaacaaactaaaatctaaccctaggtagtagtaaactgaatataaactttctcttatgaatttattctgtcttctttggtacatcaataataatatacacctttacagtatttcccagattgggggatacactttagcaagtatctgcgattatttgtttatgtaagatgtcccttcccttctgtgaatcatcattcttcaccccaagtatcttgagattggattctgtataagcagaatacaacagttaggcattcaggtatcattaaattcctccgcttcaaggatgaaaatttctttgggtatctaatagagtacaaagcagaaggtgtttcagaaatatttgcagtattgaatccgcatattcctccaagatagccctaatctaactggcagggtcccactcttcccagattaatgcccactcacataacaaacctgatgaggtagtgaagaaaactaactttgtgagtaagcaactggcagagtttttcaccactgtgactctatagctacatgtaactaagtagtatcactgacacataatcttaaattgaagttttaagatcattattctccatgttatacatgggtatcaaaagcattcccctcttgaccactccagaattctgtttaaaatttttcaatgacaacttatccatttccccaaagcctcagtgagcacatgatgccaacaattcatttcatgacttcatagcatgggccaagtttcttgcttaaaagacttccatcctgtcttgggaaacaaccatttccaaatatccacatatccttgcaagtttctgcctactcctctaccacccatttctgaagccatctgatttagtaagctgtatgcaaaagatacacaatggctaatgcaatcaaacaaggaatgtattaaaagcacacccaatagctcaaaataaaagacaagtgaacaaagttaagaaaatgacagtaacaaaagctgttctgggaacctctattgaaatagctacttattacatcaacatgctaccacagaacaaaagctcatgttgcttttctgaacttgaaaaacccattaacaatgtacagttctgagcctcagctgaccatagtgctcatgccaagtcctgagcagggcatcttgaatggtggttccctcatgactacatacaccgttagggaatgtttcgttaagaggaaatcaagatgttctaacctgtgaaggtagaatagattccaggctacacaaacacatgaagtgtgccttatattgattactaaagaggttgctgccaagactgcttccaaagggcagaagatagccctaaaaaatgtttgcagtgtggaaatgcatttttagtaagtcatattctagtaacaagttgcatttggtaagacacaaagaaacaatgttggtatgcagagtagaaatctctggaagatgatattgtcatatcagagatattgtcagtatcagagatactgaaatctctggaagatgatttttgtctcacatatggcattcgcaagtaaaatgccaaactgcaaaattcatattatgtagtacacataggaagatatctaaatatccctgtaggctctgggatgttatttcttattcttaacctccttactagattcacttgtacaatgaaataatctgtatcttattatttataattgagaattttctcaaaccttttcctgaaattttggaacacctggaataaaatttcttaaaatgattcctaaaagaaataattcttcaaaattaatattaagatataataacaggttggtttttttttttttttttttttttttttttagaatgaagcttctaaggtgaggttaacagtccagctgtggtttatttggtacattcataagatgttcactcctatatatattttttccctaggggtttctcatttctagatttacactttcccttatagcatggtccctccaaggtatatgcttccgatacataaaatgtttgtaattttgttaattctgccattcattagctcaataatttctctcattaaaattctgtaaactatgaatttcaaagaagtctattctatattcatctggttcatgaagtttcctctttgtgaatcttattttagtaaaatgactttacaacgtttaacatggttcctcacctgtatgaactttttaaaaaaaggtatgacttgctgctaaaaattttcagagtggttactaaattcagttttcctgtgtattgtctactatctttttgcatgtaaagaacagctttctgtggatgcctttccatatgctgtgcattcataaagtttctattcagtatgagttttctggaagatgacaagatgattccacttacagagtttctctttatatatgattgtttctatctcttgtgaatccacttttcagagtttcgtaaaattatcaatgtttgtcatctacatgagttctctgatgcataatgagctgtgacttccaacaaaaggctttcccacattcagtgcacttacaaggcttctctcctgtatgtgttctctgatgtgcactgagaattgatttttgagagaaggttttcccacattcattgcacccatagggtttctctcctgaatgagttctttgatgtacaatgagttgagaattcctaatgaaggcttttccacactcactgcattcatatggtttctctcttgtgtgcattctctggtgtacaagaaggcgtaatttcccactgaaggatttctcacattgactgcatttataagggttgacccctgcatgagttcgctcatgtacaatgagtagtgatttccaaatgaaggctttcccacattcattacattcatatggtttttcacctgaatgagttctcatgtgtataattaggtatgacttgctgctaaaagctttcccacattcactgcacccataaggcttttcccctgcatgagttcgctgatgtgaaatgagctggtctttcctattaaaggctttcccacattcactgcattcatagggattttctcctgtgtgaattctctgatgcacaatgagttgtgaattgaaactaaaggatttcccgcattccctgcactcatgtggtttctctcctgtatgagttctcatatgtataataaggtatgacttgctcctgaaggctttcccacactcactgcatccatatggttttactcctgtgtgacttctctgatgtacaatgagctgggacttcaaactaaaggtttttgcacattgactgcatccatagggttttactccagtgtgcactcctttatgtacaatgagctgtgatttgaacgtaaaggcttttccacattcattacaactatagggtttctctcctgtatgagttctctgatgtacaatcaggtttgactttgtattaaaggctttctgacactcactacattcaaatggtttctcccctgtatgagttctctggtgtataataagctgtgactttaaaccaaaagcctttccacagtcggtgcattcataaggcttctctcctgcatgagttctctggtgtgaaataagctggtatttccgactgaaggctttcccacattcatggcattcataggggttctctcctgtatgaatcctctgatgtataatgagctgtgatttaaaactgaaggctttcccacaattgttgcattcatggagtttttctcctgtatgagtccttgtatgtataataaggtatgacttgctcctgaaggctttgccacattcattgcatacataaggtttcattcctgtgtgacttctctgatgtacaatgagctgtgatttcaaactgaatcctttaccacactgaatacacccatagggctttactcctgtgtgaatcccctgatgtacaatgagctgtgacttgaatgtaaaggcttttccacaatcactacaaacataaggtttctcccctgtatgggttctctgatgtaccataaggtttgactttgtattaaaggctttctgacattcattgcattcatatggtttctctcctgtatgaattctttcatgtataatgagctgtgattttaaaccaaaagctttcccacattcattacacacatatggtttctgtcctgaatgagttttctggtgtgaaacaagctggtctttcctactgaagactttcccacattcacagcactcatagggattctcacctgtgtgaattctctgatgtataacaagctgtgaatggaaactgaatgttttcctgcattcactgcattcatgtagtttctctcctgtatgaattctctgatgtacaatgaggtatgatttactactgaagtctttcccacattcattacaaccatagggtttctcttcggcatgagtttgctgatgcactagaaggtatgacttgctgctgaaggctttctcacaacagctgcatccaaagggtttttcgcccatatacatttgttggcacataagttgcgatttcttattgacggtttttccagattcaatactttcacagtattttattccaataacagtttgctcatgtttagaatggaagaatgattttccatgtacctgaaacccattaggattatttctagcataatcactagtgaaatctatatatttcaaactctttccatgcgtgccacatttatgaggtttttgtcttgaaagatactttgtactaagaagacatagttttccaaatgtagtgcattcaaagctttttgccgtacttcccagcttgtctttattttcctgatgccaatccataagatcatcaattttccagactgtgtttggacaggtctgatttggaacttgggcctgcaccatacacagctcttctccttgttccaacttgaagatgatatcaggtttggtgtgttggtaccccaggacttggtgatttttggctgctcttgggaaataaacagccactctaggactttctctattctgcgactcttctgcttctgcctgggtgttccagggagaggttgcagaccaggagtcccttggcccaagatggattcctgaccttggagctttctgatcctatcccatgaactgtttcgttcttggagaggtgggacccaaatagaagctgtccggaccctggtggccatccctacggtcagttttgtgtgcctcgctggaagtgacaggacgcgagggatgctccggctcctccaaaccctgaaggggcagcagaatagagtccagggtactgcctccacctccagatctgcagccagaagggttcgcaaccactccagactcggctggcccgttgaccacgacgggcgatgaacgctatctgaggaacaaggatctcgccatcggcgcggaacaatggcggccgctacgtat

SEQ ID NO: 13691 - RNA, 8086 nt, Homo sapiens
  source 1..8086: mol_type = other RNA
gctgggattacaggcatgagccaccatgcccagcctttttattaatgttttaatggcctgtgtttctaacaagtagttgaaacaatgttgaaaattaaagagtagacatgttaaaacttgcaacttcatttaaatttaaatatatcatttataccaaaatcagaatttatttaagatttatggctgggtgcttggctcacacctgtaatcctagcactttgggaggccaaggcaggtggactgcttgagcccaggagtttgaaaccagactggaaaacatggtaaaaccccatctctacaagaaataaataactctacctggccctttagcaaagaattaagaaaaatcaatacagaccagtggctcacacctgtaatcccagcactttgggaggctgagggtggatcacgaggtcaggagttcaagaccagcctggccaacatggtgaaaccccatctctactaaaaacacaaaaattagctgggcgtggtggcgtgtgcctgtaattccagctactagggaggctgaggcaggagaattgcttgaacccaggaggcagaggttgcagtgagccaagaacacaccactgcactccagcctggcaatacagcgagactccatctcaaaaaaaaaaaaaaaaatgcaaatactatgccatataaggagcttgagcatccacagggagtatctgtggttgcgggggggtcctccatgaatactgacaactgcatacttgctactctactggcagttccaaacatttgtttgtggtttattttgggtttcctaattacacgatcacatctccaattcatggcagttgtttctgcacccatccctaattcctcacattccttgttttcacaccttggctagatgttactcatttcataaaagtgatgcgcattcttgtaattttgctttgttttttacagacagggtctcactttgttgcccaggatggagtgcaggggcatgatcatagctcactgtagccttgaactactggactcaagctaacctcctgcctcagcctcctcagtaggtgggactaccggcacttgccactacacctggctgatcttttttttgagatggaggcttgttctgtcgcccagcctggagtgcagtggtgcaatcttggctcactgcaactgccacctcctaggttcaagcaattcttctgcctcagcctcccgagtagatgggattacaggcacgtgccaccacacctggctgacttttgtatttttagtagagacggggtttcaccatgttagccacactggtcttgaaatcctgacctcaagtgatctgcccacctcggcctcccaaagtgctgggattacaggcatgagccacggcgcctgaccacacctggctaatctttttaaaaagtttttgtacagacagggtctccctatattggtcaggcttgtctcgaactcctgggttccagcaatcctccagcctcagccttcccaagtgctggtattacatggatgagccactgcacctggctaattttactttaaaggaatctttctactattttatcattaagtatgacatttgtgttttcagaacatatattccctaccaagttacaggagttaattttaattcccaacttaatagtattttagtgtcatctatgggtgttaaattccatcaagtgatttatcagcatatactgagataatccttatgagttttatctggtagttaattaaaatattttctaatattaaatcttccaaacatactcttctgttttttgagacagggtctagttctgtcacccagggtggagtacagtggtacgatctcagctcactgcaacttccgcctcctagattcaagtgattctcccgtcccagcctcccaagtagctgggattataggtgtcagttaccatgccctgctatttttttgtatttttagtagagaggggtttcaccatgttggccaggctggtctcaaactcctgacctcaggtgatccaccatctcagcctcctgaagtgctgggattataggtgtgagccaccgtgcctggccccatatatctctttttaagtgggcatactgccattataaataatagtgattctgctggtaatgaacaaaggatgctggatccactaatagtctgttaaacctaatatcatgactttcttgttagctatacattggtttgctataattccatttagaatttttaaacctatgttcacaaatatggatttttaaacctatgttcacaaatatggatttttaaacctatgttcacaaatatggtttgcaagtcattttttctcctaaatttctatttgatggggaagttgtaaaatattggggttatttttccttggattttccttataataactattcctgaaaagtctctggaatgtctttcttttctggggctggggtagaaggactagatagatttacaaaccagtaactcaatttctgttttgtaaaattttcatttcattaaataataagtcctaatcaagtattattctttcccacagtatgtgagtgctgtcctcaatactgtcaacacttctggcttctaccaggcaaggctgcatgtagatttgcatctgaaaaaacaacaaactaaaatctaaccctaggtagtagtaaactgaatataaactttctcttatgaatttattctgtcttctttggtacatcaataataatatacacctttacagtatttcccagattgggggatacactttagcaagtatctgcgattatttgtttatgtaagatgtcccttcccttctgtgaatcatcattcttcaccccaagtatcttgagattggattctgtataagcagaatacaacagttaggcattcaggtatcattaaattcctccgcttcaaggatgaaaatttctttgggtatctaatagagtacaaagcagaaggtgtttcagaaatatttgcagtattgaatccgcatattcctccaagatagccctaatctaactggcagggtcccactcttcccagattaatgcccactcacataacaaacctgatgaggtagtgaagaaaactaactttgtgagtaagcaactggcagagtttttcaccactgtgactctatagctacatgtaactaagtagtatcactgacacataatcttaaattgaagttttaagatcattattctccatgttatacatgggtatcaaaagcattcccctcttgaccactccagaattctgtttaaaatttttcaatgacaacttatccatttccccaaagcctcagtgagcacatgatgccaacaattcatttcatgacttcatagcatgggccaagtttcttgcttaaaagacttccatcctgtcttgggaaacaaccatttccaaatatccacatatccttgcaagtttctgcctactcctctaccacccatttctgaagccatctgatttagtaagctgtatgcaaaagatacacaatggctaatgcaatcaaacaaggaatgtattaaaagcacacccaatagctcaaaataaaagacaagtgaacaaagttaagaaaatgacagtaacaaaagctgttctgggaacctctattgaaatagctacttattacatcaacatgctaccacagaacaaaagctcatgttgcttttctgaacttgaaaaacccattaacaatgtacagttctgagcctcagctgaccatagtgctcatgccaagtcctgagcagggcatcttgaatggtggttccctcatgactacatacaccgttagggaatgtttcgttaagaggaaatcaagatgttctaacctgtgaaggtagaatagattccaggctacacaaacacatgaagtgtgccttatattgattactaaagaggttgctgccaagactgcttccaaagggcagaagatagccctaaaaaatgtttgcagtgtggaaatgcatttttagtaagtcatattctagtaacaagttgcatttggtaagacacaaagaaacaatgttggtatgcagagtagaaatctctggaagatgatattgtcatatcagagatattgtcagtatcagagatactgaaatctctggaagatgatttttgtctcacatatggcattcgcaagtaaaatgccaaactgcaaaattcatattatgtagtacacataggaagatatctaaatatccctgtaggctctgggatgttatttcttattcttaacctccttactagattcacttgtacaatgaaataatctgtatcttattatttataattgagaattttctcaaaccttttcctgaaattttggaacacctggaataaaatttcttaaaatgattcctaaaagaaataattcttcaaaattaatattaagatataataacaggttggtttttttttttttttttttttttttttttagaatgaagcttctaaggtgaggttaacagtccagctgtggtttatttggtacattcataagatgttcactcctatatatattttttccctaggggtttctcatttctagatttacactttcccttatagcatggtccctccaaggtatatgcttccgatacataaaatgtttgtaattttgttaattctgccattcattagctcaataatttctctcattaaaattctgtaaactatgaatttcaaagaagtctattctatattcatctggttcatgaagtttcctctttgtgaatcttattttagtaaaatgactttacaacgtttaacatggttcctcacctgtatgaactttttaaaaaaaggtatgacttgctgctaaaaattttcagagtggttactaaattcagttttcctgtgtattgtctactatctttttgcatgtaaagaacagctttctgtggatgcctttccatatgctgtgcattcataaagtttctattcagtatgagttttctggaagatgacaagatgattccacttacagagtttctctttatatatgattgtttctatctcttgtgaatccacttttcagagtttcgtaaaattatcaatgtttgtcatctacatgagttctctgatgcataatgagctgtgacttccaacaaaaggctttcccacattcagtgcacttacaaggcttctctcctgtatgtgttctctgatgtgcactgagaattgatttttgagagaaggttttcccacattcattgcacccatagggtttctctcctgaatgagttctttgatgtacaatgagttgagaattcctaatgaaggcttttccacactcactgcattcatatggtttctctcttgtgtgcattctctggtgtacaagaaggcgtaatttcccactgaaggatttctcacattgactgcatttataagggttgacccctgcatgagttcgctcatgtacaatgagtagtgatttccaaatgaaggctttcccacattcattacattcatatggtttttcacctgaatgagttctcatgtgtataattaggtatgacttgctgctaaaagctttcccacattcactgcacccataaggcttttcccctgcatgagttcgctgatgtgaaatgagctggtctttcctattaaaggctttcccacattcactgcattcatagggattttctcctgtgtgaattctctgatgcacaatgagttgtgaattgaaactaaaggatttcccgcattccctgcactcatgtggtttctctcctgtatgagttctcatatgtataataaggtatgacttgctcctgaaggctttcccacactcactgcatccatatggttttactcctgtgtgacttctctgatgtacaatgagctgggacttcaaactaaaggtttttgcacattgactgcatccatagggttttactccagtgtgcactcctttatgtacaatgagctgtgatttgaacgtaaaggcttttccacattcattacaactatagggtttctctcctgtatgagttctctgatgtacaatcaggtttgactttgtattaaaggctttctgacactcactacattcaaatggtttctcccctgtatgagttctctggtgtataataagctgtgactttaaaccaaaagcctttccacagtcggtgcattcataaggcttctctcctgcatgagttctctggtgtgaaataagctggtatttccgactgaaggctttcccacattcatggcattcataggggttctctcctgtatgaatcctctgatgtataatgagctgtgatttaaaactgaaggctttcccacaattgttgcattcatggagtttttctcctgtatgagtccttgtatgtataataaggtatgacttgctcctgaaggctttgccacattcattgcatacataaggtttcattcctgtgtgacttctctgatgtacaatgagctgtgatttcaaactgaatcctttaccacactgaatacacccatagggctttactcctgtgtgaatcccctgatgtacaatgagctgtgacttgaatgtaaaggcttttccacaatcactacaaacataaggtttctcccctgtatgggttctctgatgtaccataaggtttgactttgtattaaaggctttctgacattcattgcattcatatggtttctctcctgtatgaattctttcatgtataatgagctgtgattttaaaccaaaagctttcccacattcattacacacatatggtttctgtcctgaatgagttttctggtgtgaaacaagctggtctttcctactgaagactttcccacattcacagcactcatagggattctcacctgtgtgaattctctgatgtataacaagctgtgaatggaaactgaatgttttcctgcattcactgcattcatgtagtttctctcctgtatgaattctctgatgtacaatgaggtatgatttactactgaagtctttcccacattcattacaaccatagggtttctcttcggcatgagtttgctgatgcactagaaggtatgacttgctgctgaaggctttctcacaacagctgcatccaaagggtttttcgcccatatacatttgttggcacataagttgcgatttcttattgacggtttttccagattcaatactttcacagtattttattccaataacagtttgctcatgtttagaatggaagaatgattttccatgtacctgaaacccattaggattatttctagcataatcactagtgaaatctatatatttcaaactctttccatgcgtgccacatttatgaggtttttgtcttgaaagatactttgtactaagaagacatagttttccaaatgtagtgcattcaaagctttttgccgtacttcccagcttgtctttattttcctgatgccaatccataagatcatcaattttccagactgtgtttggacaggtctgatttggaacttgggcctgcaccatacacagctcttctccttgttccaacttgaagatgatatcaggtttggtgtgttggtaccctagggacaccaggttgctatagttctccaacatcacactcctgtacaggcacttctgtgctgggtctagcagctgccactcctcccaggtaaaatccacaaacacatccatgaatgacaaaggtccccaggacttggtgatttttggctgctcttgggaaataaacagccactctaggactttctctattctgcgactcttctgcttctgcctgggtgttccagggagaggttgcagaccaggagtcccttggcccaagatggattcctgaccttggagctttctgatcctatcccatgaactgtttcgttcttggagaggtgggacccaaatagaagctgtccggaccctggtggccatccctacggtcagttttgtgtgcctcgctggaagtgacaggacgcgagggatgctccagatctgcagccagaagggttcgcaaccactccagactcggctggcccgttgaccacgacgggcgatgaacgctatctgaggaacaaggatctcgccatcggcgcggaacaatggcggccgctacgtat

SEQ ID NO: 13692 - RNA, 8145 nt, Homo sapiens
  source 1..8145: mol_type = other RNA
gctgggattacaggcatgagccaccatgcccagcctttttattaatgttttaatggcctgtgtttctaacaagtagttgaaacaatgttgaaaattaaagagtagacatgttaaaacttgcaacttcatttaaatttaaatatatcatttataccaaaatcagaatttatttaagatttatggctgggtgcttggctcacacctgtaatcctagcactttgggaggccaaggcaggtggactgcttgagcccaggagtttgaaaccagactggaaaacatggtaaaaccccatctctacaagaaataaataactctacctggccctttagcaaagaattaagaaaaatcaatacagaccagtggctcacacctgtaatcccagcactttgggaggctgagggtggatcacgaggtcaggagttcaagaccagcctggccaacatggtgaaaccccatctctactaaaaacacaaaaattagctgggcgtggtggcgtgtgcctgtaattccagctactagggaggctgaggcaggagaattgcttgaacccaggaggcagaggttgcagtgagccaagaacacaccactgcactccagcctggcaatacagcgagactccatctcaaaaaaaaaaaaaaaaatgcaaatactatgccatataaggagcttgagcatccacagggagtatctgtggttgcgggggggtcctccatgaatactgacaactgcatacttgctactctactggcagttccaaacatttgtttgtggtttattttgggtttcctaattacacgatcacatctccaattcatggcagttgtttctgcacccatccctaattcctcacattccttgttttcacaccttggctagatgttactcatttcataaaagtgatgcgcattcttgtaattttgctttgttttttacagacagggtctcactttgttgcccaggatggagtgcaggggcatgatcatagctcactgtagccttgaactactggactcaagctaacctcctgcctcagcctcctcagtaggtgggactaccggcacttgccactacacctggctgatcttttttttgagatggaggcttgttctgtcgcccagcctggagtgcagtggtgcaatcttggctcactgcaactgccacctcctaggttcaagcaattcttctgcctcagcctcccgagtagatgggattacaggcacgtgccaccacacctggctgacttttgtatttttagtagagacggggtttcaccatgttagccacactggtcttgaaatcctgacctcaagtgatctgcccacctcggcctcccaaagtgctgggattacaggcatgagccacggcgcctgaccacacctggctaatctttttaaaaagtttttgtacagacagggtctccctatattggtcaggcttgtctcgaactcctgggttccagcaatcctccagcctcagccttcccaagtgctggtattacatggatgagccactgcacctggctaattttactttaaaggaatctttctactattttatcattaagtatgacatttgtgttttcagaacatatattccctaccaagttacaggagttaattttaattcccaacttaatagtattttagtgtcatctatgggtgttaaattccatcaagtgatttatcagcatatactgagataatccttatgagttttatctggtagttaattaaaatattttctaatattaaatcttccaaacatactcttctgttttttgagacagggtctagttctgtcacccagggtggagtacagtggtacgatctcagctcactgcaacttccgcctcctagattcaagtgattctcccgtcccagcctcccaagtagctgggattataggtgtcagttaccatgccctgctatttttttgtatttttagtagagaggggtttcaccatgttggccaggctggtctcaaactcctgacctcaggtgatccaccatctcagcctcctgaagtgctgggattataggtgtgagccaccgtgcctggccccatatatctctttttaagtgggcatactgccattataaataatagtgattctgctggtaatgaacaaaggatgctggatccactaatagtctgttaaacctaatatcatgactttcttgttagctatacattggtttgctataattccatttagaatttttaaacctatgttcacaaatatggatttttaaacctatgttcacaaatatggatttttaaacctatgttcacaaatatggtttgcaagtcattttttctcctaaatttctatttgatggggaagttgtaaaatattggggttatttttccttggattttccttataataactattcctgaaaagtctctggaatgtctttcttttctggggctggggtagaaggactagatagatttacaaaccagtaactcaatttctgttttgtaaaattttcatttcattaaataataagtcctaatcaagtattattctttcccacagtatgtgagtgctgtcctcaatactgtcaacacttctggcttctaccaggcaaggctgcatgtagatttgcatctgaaaaaacaacaaactaaaatctaaccctaggtagtagtaaactgaatataaactttctcttatgaatttattctgtcttctttggtacatcaataataatatacacctttacagtatttcccagattgggggatacactttagcaagtatctgcgattatttgtttatgtaagatgtcccttcccttctgtgaatcatcattcttcaccccaagtatcttgagattggattctgtataagcagaatacaacagttaggcattcaggtatcattaaattcctccgcttcaaggatgaaaatttctttgggtatctaatagagtacaaagcagaaggtgtttcagaaatatttgcagtattgaatccgcatattcctccaagatagccctaatctaactggcagggtcccactcttcccagattaatgcccactcacataacaaacctgatgaggtagtgaagaaaactaactttgtgagtaagcaactggcagagtttttcaccactgtgactctatagctacatgtaactaagtagtatcactgacacataatcttaaattgaagttttaagatcattattctccatgttatacatgggtatcaaaagcattcccctcttgaccactccagaattctgtttaaaatttttcaatgacaacttatccatttccccaaagcctcagtgagcacatgatgccaacaattcatttcatgacttcatagcatgggccaagtttcttgcttaaaagacttccatcctgtcttgggaaacaaccatttccaaatatccacatatccttgcaagtttctgcctactcctctaccacccatttctgaagccatctgatttagtaagctgtatgcaaaagatacacaatggctaatgcaatcaaacaaggaatgtattaaaagcacacccaatagctcaaaataaaagacaagtgaacaaagttaagaaaatgacagtaacaaaagctgttctgggaacctctattgaaatagctacttattacatcaacatgctaccacagaacaaaagctcatgttgcttttctgaacttgaaaaacccattaacaatgtacagttctgagcctcagctgaccatagtgctcatgccaagtcctgagcagggcatcttgaatggtggttccctcatgactacatacaccgttagggaatgtttcgttaagaggaaatcaagatgttctaacctgtgaaggtagaatagattccaggctacacaaacacatgaagtgtgccttatattgattactaaagaggttgctgccaagactgcttccaaagggcagaagatagccctaaaaaatgtttgcagtgtggaaatgcatttttagtaagtcatattctagtaacaagttgcatttggtaagacacaaagaaacaatgttggtatgcagagtagaaatctctggaagatgatattgtcatatcagagatattgtcagtatcagagatactgaaatctctggaagatgatttttgtctcacatatggcattcgcaagtaaaatgccaaactgcaaaattcatattatgtagtacacataggaagatatctaaatatccctgtaggctctgggatgttatttcttattcttaacctccttactagattcacttgtacaatgaaataatctgtatcttattatttataattgagaattttctcaaaccttttcctgaaattttggaacacctggaataaaatttcttaaaatgattcctaaaagaaataattcttcaaaattaatattaagatataataacaggttggtttttttttttttttttttttttttttttagaatgaagcttctaaggtgaggttaacagtccagctgtggtttatttggtacattcataagatgttcactcctatatatattttttccctaggggtttctcatttctagatttacactttcccttatagcatggtccctccaaggtatatgcttccgatacataaaatgtttgtaattttgttaattctgccattcattagctcaataatttctctcattaaaattctgtaaactatgaatttcaaagaagtctattctatattcatctggttcatgaagtttcctctttgtgaatcttattttagtaaaatgactttacaacgtttaacatggttcctcacctgtatgaactttttaaaaaaaggtatgacttgctgctaaaaattttcagagtggttactaaattcagttttcctgtgtattgtctactatctttttgcatgtaaagaacagctttctgtggatgcctttccatatgctgtgcattcataaagtttctattcagtatgagttttctggaagatgacaagatgattccacttacagagtttctctttatatatgattgtttctatctcttgtgaatccacttttcagagtttcgtaaaattatcaatgtttgtcatctacatgagttctctgatgcataatgagctgtgacttccaacaaaaggctttcccacattcagtgcacttacaaggcttctctcctgtatgtgttctctgatgtgcactgagaattgatttttgagagaaggttttcccacattcattgcacccatagggtttctctcctgaatgagttctttgatgtacaatgagttgagaattcctaatgaaggcttttccacactcactgcattcatatggtttctctcttgtgtgcattctctggtgtacaagaaggcgtaatttcccactgaaggatttctcacattgactgcatttataagggttgacccctgcatgagttcgctcatgtacaatgagtagtgatttccaaatgaaggctttcccacattcattacattcatatggtttttcacctgaatgagttctcatgtgtataattaggtatgacttgctgctaaaagctttcccacattcactgcacccataaggcttttcccctgcatgagttcgctgatgtgaaatgagctggtctttcctattaaaggctttcccacattcactgcattcatagggattttctcctgtgtgaattctctgatgcacaatgagttgtgaattgaaactaaaggatttcccgcattccctgcactcatgtggtttctctcctgtatgagttctcatatgtataataaggtatgacttgctcctgaaggctttcccacactcactgcatccatatggttttactcctgtgtgacttctctgatgtacaatgagctgggacttcaaactaaaggtttttgcacattgactgcatccatagggttttactccagtgtgcactcctttatgtacaatgagctgtgatttgaacgtaaaggcttttccacattcattacaactatagggtttctctcctgtatgagttctctgatgtacaatcaggtttgactttgtattaaaggctttctgacactcactacattcaaatggtttctcccctgtatgagttctctggtgtataataagctgtgactttaaaccaaaagcctttccacagtcggtgcattcataaggcttctctcctgcatgagttctctggtgtgaaataagctggtatttccgactgaaggctttcccacattcatggcattcataggggttctctcctgtatgaatcctctgatgtataatgagctgtgatttaaaactgaaggctttcccacaattgttgcattcatggagtttttctcctgtatgagtccttgtatgtataataaggtatgacttgctcctgaaggctttgccacattcattgcatacataaggtttcattcctgtgtgacttctctgatgtacaatgagctgtgatttcaaactgaatcctttaccacactgaatacacccatagggctttactcctgtgtgaatcccctgatgtacaatgagctgtgacttgaatgtaaaggcttttccacaatcactacaaacataaggtttctcccctgtatgggttctctgatgtaccataaggtttgactttgtattaaaggctttctgacattcattgcattcatatggtttctctcctgtatgaattctttcatgtataatgagctgtgattttaaaccaaaagctttcccacattcattacacacatatggtttctgtcctgaatgagttttctggtgtgaaacaagctggtctttcctactgaagactttcccacattcacagcactcatagggattctcacctgtgtgaattctctgatgtataacaagctgtgaatggaaactgaatgttttcctgcattcactgcattcatgtagtttctctcctgtatgaattctctgatgtacaatgaggtatgatttactactgaagtctttcccacattcattacaaccatagggtttctcttcggcatgagtttgctgatgcactagaaggtatgacttgctgctgaaggctttctcacaacagctgcatccaaagggtttttcgcccatatacatttgttggcacataagttgcgatttcttattgacggtttttccagattcaatactttcacagtattttattccaataacagtttgctcatgtttagaatggaagaatgattttccatgtacctgaaacccattaggattatttctagcataatcactagtgaaatctatatatttcaaactctttccatgcgtgccacatttatgaggtttttgtcttgaaagatactttgtactaagaagacatagttttccaaatgtagtgcattcaaagctttttgccgtacttcccagcttgtctttattttcctgatgccaatccataagatcatcaattttccagactgtgtttggacaggtctgatttggaacttgggcctgcaccatacacagctcttctccttgttccaacttgaagatgatatcaggtttggtgtgttggtaccctagggacaccaggttgctatagttctccaacatcacactcctgtacaggcacttctgtgctgggtctagcagctgccactcctcccaggtaaaatccacaaacacatccatgaatgacaaaggtccccaggacttggtgatttttggctgctcttgggaaataaacagccactctaggactttctctattctgcgactcttctgcttctgcctgggtgttccagggagaggttgcagaccaggagtcccttggcccaagatggattcctgaccttggagctttctgatcctatcccatgaactgtttcgttcttggagaggtgggacccaaatagaagctgtccggaccctggtggccatccctacggtcagttttgtgtgcctcgctggaagtgacaggacgcgagggatgctccggctcctccaaaccctgaaggggcagcagaatagagtccagggtactgcctccacctccagatctgcagccagaagggttcgcaaccactccagactcggctggcccgttgaccacgacgggcgatgaacgctatctgaggaacaaggatctcgccatcggcgcggaacaatggcggccgctacgtat

SEQ ID NO: 13693 - RNA, 8093 nt, Homo sapiens
  source 1..8093: mol_type = other RNA
gctgggattacaggcatgagccaccatgcccagcctttttattaatgttttaatggcctgtgtttctaacaagtagttgaaacaatgttgaaaattaaagagtagacatgttaaaacttgcaacttcatttaaatttaaatatatcatttataccaaaatcagaatttatttaagatttatggctgggtgcttggctcacacctgtaatcctagcactttgggaggccaaggcaggtggactgcttgagcccaggagtttgaaaccagactggaaaacatggtaaaaccccatctctacaagaaataaataactctacctggccctttagcaaagaattaagaaaaatcaatacagaccagtggctcacacctgtaatcccagcactttgggaggctgagggtggatcacgaggtcaggagttcaagaccagcctggccaacatggtgaaaccccatctctactaaaaacacaaaaattagctgggcgtggtggcgtgtgcctgtaattccagctactagggaggctgaggcaggagaattgcttgaacccaggaggcagaggttgcagtgagccaagaacacaccactgcactccagcctggcaatacagcgagactccatctcaaaaaaaaaaaaaaaaatgcaaatactatgccatataaggagcttgagcatccacagggagtatctgtggttgcgggggggtcctccatgaatactgacaactgcatacttgctactctactggcagttccaaacatttgtttgtggtttattttgggtttcctaattacacgatcacatctccaattcatggcagttgtttctgcacccatccctaattcctcacattccttgttttcacaccttggctagatgttactcatttcataaaagtgatgcgcattcttgtaattttgctttgttttttacagacagggtctcactttgttgcccaggatggagtgcaggggcatgatcatagctcactgtagccttgaactactggactcaagctaacctcctgcctcagcctcctcagtaggtgggactaccggcacttgccactacacctggctgatcttttttttgagatggaggcttgttctgtcgcccagcctggagtgcagtggtgcaatcttggctcactgcaactgccacctcctaggttcaagcaattcttctgcctcagcctcccgagtagatgggattacaggcacgtgccaccacacctggctgacttttgtatttttagtagagacggggtttcaccatgttagccacactggtcttgaaatcctgacctcaagtgatctgcccacctcggcctcccaaagtgctgggattacaggcatgagccacggcgcctgaccacacctggctaatctttttaaaaagtttttgtacagacagggtctccctatattggtcaggcttgtctcgaactcctgggttccagcaatcctccagcctcagccttcccaagtgctggtattacatggatgagccactgcacctggctaattttactttaaaggaatctttctactattttatcattaagtatgacatttgtgttttcagaacatatattccctaccaagttacaggagttaattttaattcccaacttaatagtattttagtgtcatctatgggtgttaaattccatcaagtgatttatcagcatatactgagataatccttatgagttttatctggtagttaattaaaatattttctaatattaaatcttccaaacatactcttctgttttttgagacagggtctagttctgtcacccagggtggagtacagtggtacgatctcagctcactgcaacttccgcctcctagattcaagtgattctcccgtcccagcctcccaagtagctgggattataggtgtcagttaccatgccctgctatttttttgtatttttagtagagaggggtttcaccatgttggccaggctggtctcaaactcctgacctcaggtgatccaccatctcagcctcctgaagtgctgggattataggtgtgagccaccgtgcctggccccatatatctctttttaagtgggcatactgccattataaataatagtgattctgctggtaatgaacaaaggatgctggatccactaatagtctgttaaacctaatatcatgactttcttgttagctatacattggtttgctataattccatttagaatttttaaacctatgttcacaaatatggatttttaaacctatgttcacaaatatggatttttaaacctatgttcacaaatatggtttgcaagtcattttttctcctaaatttctatttgatggggaagttgtaaaatattggggttatttttccttggattttccttataataactattcctgaaaagtctctggaatgtctttcttttctggggctggggtagaaggactagatagatttacaaaccagtaactcaatttctgttttgtaaaattttcatttcattaaataataagtcctaatcaagtattattctttcccacagtatgtgagtgctgtcctcaatactgtcaacacttctggcttctaccaggcaaggctgcatgtagatttgcatctgaaaaaacaacaaactaaaatctaaccctaggtagtagtaaactgaatataaactttctcttatgaatttattctgtcttctttggtacatcaataataatatacacctttacagtatttcccagattgggggatacactttagcaagtatctgcgattatttgtttatgtaagatgtcccttcccttctgtgaatcatcattcttcaccccaagtatcttgagattggattctgtataagcagaatacaacagttaggcattcaggtatcattaaattcctccgcttcaaggatgaaaatttctttgggtatctaatagagtacaaagcagaaggtgtttcagaaatatttgcagtattgaatccgcatattcctccaagatagccctaatctaactggcagggtcccactcttcccagattaatgcccactcacataacaaacctgatgaggtagtgaagaaaactaactttgtgagtaagcaactggcagagtttttcaccactgtgactctatagctacatgtaactaagtagtatcactgacacataatcttaaattgaagttttaagatcattattctccatgttatacatgggtatcaaaagcattcccctcttgaccactccagaattctgtttaaaatttttcaatgacaacttatccatttccccaaagcctcagtgagcacatgatgccaacaattcatttcatgacttcatagcatgggccaagtttcttgcttaaaagacttccatcctgtcttgggaaacaaccatttccaaatatccacatatccttgcaagtttctgcctactcctctaccacccatttctgaagccatctgatttagtaagctgtatgcaaaagatacacaatggctaatgcaatcaaacaaggaatgtattaaaagcacacccaatagctcaaaataaaagacaagtgaacaaagttaagaaaatgacagtaacaaaagctgttctgggaacctctattgaaatagctacttattacatcaacatgctaccacagaacaaaagctcatgttgcttttctgaacttgaaaaacccattaacaatgtacagttctgagcctcagctgaccatagtgctcatgccaagtcctgagcagggcatcttgaatggtggttccctcatgactacatacaccgttagggaatgtttcgttaagaggaaatcaagatgttctaacctgtgaaggtagaatagattccaggctacacaaacacatgaagtgtgccttatattgattactaaagaggttgctgccaagactgcttccaaagggcagaagatagccctaaaaaatgtttgcagtgtggaaatgcatttttagtaagtcatattctagtaacaagttgcatttggtaagacacaaagaaacaatgttggtatgcagagtagaaatctctggaagatgatattgtcatatcagagatattgtcagtatcagagatactgaaatctctggaagatgatttttgtctcacatatggcattcgcaagtaaaatgccaaactgcaaaattcatattatgtagtacacataggaagatatctaaatatccctgtaggctctgggatgttatttcttattcttaacctccttactagattcacttgtacaatgaaataatctgtatcttattatttataattgagaattttctcaaaccttttcctgaaattttggaacacctggaataaaatttcttaaaatgattcctaaaagaaataattcttcaaaattaatattaagatataataacaggttggtttttttttttttttttttttttttttttagaatgaagcttctaaggtgaggttaacagtccagctgtggtttatttggtacattcataagatgttcactcctatatatattttttccctaggggtttctcatttctagatttacactttcccttatagcatggtccctccaaggtatatgcttccgatacataaaatgtttgtaattttgttaattctgccattcattagctcaataatttctctcattaaaattctgtaaactatgaatttcaaagaagtctattctatattcatctggttcatgaagtttcctctttgtgaatcttattttagtaaaatgactttacaacgtttaacatggttcctcacctgtatgaactttttaaaaaaaggtatgacttgctgctaaaaattttcagagtggttactaaattcagttttcctgtgtattgtctactatctttttgcatgtaaagaacagctttctgtggatgcctttccatatgctgtgcattcataaagtttctattcagtatgagttttctggaagatgacaagatgattccacttacagagtttctctttatatatgattgtttctatctcttgtgaatccacttttcagagtttcgtaaaattatcaatgtttgtcatctacatgagttctctgatgcataatgagctgtgacttccaacaaaaggctttcccacattcagtgcacttacaaggcttctctcctgtatgtgttctctgatgtgcactgagaattgatttttgagagaaggttttcccacattcattgcacccatagggtttctctcctgaatgagttctttgatgtacaatgagttgagaattcctaatgaaggcttttccacactcactgcattcatatggtttctctcttgtgtgcattctctggtgtacaagaaggcgtaatttcccactgaaggatttctcacattgactgcatttataagggttgacccctgcatgagttcgctcatgtacaatgagtagtgatttccaaatgaaggctttcccacattcattacattcatatggtttttcacctgaatgagttctcatgtgtataattaggtatgacttgctgctaaaagctttcccacattcactgcacccataaggcttttcccctgcatgagttcgctgatgtgaaatgagctggtctttcctattaaaggctttcccacattcactgcattcatagggattttctcctgtgtgaattctctgatgcacaatgagttgtgaattgaaactaaaggatttcccgcattccctgcactcatgtggtttctctcctgtatgagttctcatatgtataataaggtatgacttgctcctgaaggctttcccacactcactgcatccatatggttttactcctgtgtgacttctctgatgtacaatgagctgggacttcaaactaaaggtttttgcacattgactgcatccatagggttttactccagtgtgcactcctttatgtacaatgagctgtgatttgaacgtaaaggcttttccacattcattacaactatagggtttctctcctgtatgagttctctgatgtacaatcaggtttgactttgtattaaaggctttctgacactcactacattcaaatggtttctcccctgtatgagttctctggtgtataataagctgtgactttaaaccaaaagcctttccacagtcggtgcattcataaggcttctctcctgcatgagttctctggtgtgaaataagctggtatttccgactgaaggctttcccacattcatggcattcataggggttctctcctgtatgaatcctctgatgtataatgagctgtgatttaaaactgaaggctttcccacaattgttgcattcatggagtttttctcctgtatgagtccttgtatgtataataaggtatgacttgctcctgaaggctttgccacattcattgcatacataaggtttcattcctgtgtgacttctctgatgtacaatgagctgtgatttcaaactgaatcctttaccacactgaatacacccatagggctttactcctgtgtgaatcccctgatgtacaatgagctgtgacttgaatgtaaaggcttttccacaatcactacaaacataaggtttctcccctgtatgggttctctgatgtaccataaggtttgactttgtattaaaggctttctgacattcattgcattcatatggtttctctcctgtatgaattctttcatgtataatgagctgtgattttaaaccaaaagctttcccacattcattacacacatatggtttctgtcctgaatgagttttctggtgtgaaacaagctggtctttcctactgaagactttcccacattcacagcactcatagggattctcacctgtgtgaattctctgatgtataacaagctgtgaatggaaactgaatgttttcctgcattcactgcattcatgtagtttctctcctgtatgaattctctgatgtacaatgaggtatgatttactactgaagtctttcccacattcattacaaccatagggtttctcttcggcatgagtttgctgatgcactagaaggtatgacttgctgctgaaggctttctcacaacagctgcatccaaagggtttttcgcccatatacatttgttggcacataagttgcgatttcttattgacggtttttccagattcaatactttcacagtattttattccaataacagtttgctcatgtttagaatggaagaatgattttccatgtacctgaaacccattaggattatttctagcataatcactagtgaaatctatatatttcaaactctttccatgcgtgccacatttatgaggtttttgtcttgaaagatactttgtactaagaagacatagttttccaaatgtagtgcattcaaagctttttgccgtacttcccagcttgtctttattttcctgatgccaatccataagatcatcaattttccagactgtgtttggacaggtctgatttggaacttgggcctgcaccatacacagctcttctccttgttccaacttgaagatgatatcaggtttggtgtgttggtaccctagggacaccaggttgctatagttctccaacatcacactcctgtacaggcacttctgtgctgggtctagcagctgccactcctcccaggtaaaatccacaaacacatccatgaatgacaaaggtccccaggacttggtgatttttggctgctcttgggaaataaacagccactctaggactttctctattctgcgactcttctgcttctgcctgggtgttccagggagaggttgcagaccaggagtcccttggcccaagatggattcctgaccttggagctttctgatcctatcccatgaactgtttcgttcttggagaggtgggacctgtggaccaaatagaagctgtccggaccctggtggccatccctacggtcagttttgtgtgcctcgctggaagtgacaggacgcgagggatgctccagatctgcagccagaagggttcgcaaccactccagactcggctggcccgttgaccacgacgggcgatgaacgctatctgaggaacaaggatctcgccatcggcgcggaacaatggcggccgctacgtat

SEQ ID NO: 13694 - RNA, 11267 nt, Homo sapiens
  source 1..11267: mol_type = other RNA
gctgggattacaggcatgagccaccatgcccagctaatttttgtatttttagtagagacagggtttcaccatgttggccaggctggtcttgaactcctgagctcgggtgatctgcctgcttcagcctcccaaagtgctgggattacaagtgtgagccaccctgcacggcccctttctttctggcttcctcctcccttcttccttttctttcatttttaaaacatttttttaaaattattatttttaaatttttttttttgagatggagtctagctctgtcgcccaggctggagtgcagtggcatgatcttggctcactgcaatctctgcctcccgggttcaagcaattctcctgcttcagcctcccgagtagctgggattacaggtgtccaccaccacacccagctaatttttgtatttttagtagacggggtttcactgtgttggccaggctggtcttgaactcctaaccttgtgatccttggcctcccaaagtgctgggattacaaacgtgagctactgcgcctggcctattattattatttttgagacagagttttgctcttgttgcctgggtgggagtacaatggcgtgatcttggctcactgcaacatctgcctctcggtttcaagcgattctcctgcctcagcctctcaagtagctgggattacaggcgtgagccaccacacccggctaatttttgtatttttagtacagacggattttcaccatgttggccaagctggcctcgaactcctgacctcaggtgatctgcctgcctcagcctcccagagtgctgggattacaggcgtgagccaccgcgcccggcctaaaattatttttttagagacagggtctgactctgatgtccaggctggagtgcagtggcgctattatagctcactgctgtcttaaactcttgtgctcaagtaatcctcctgcctcagcctcccgagtaggtgggaccacaggcatgtgccaccatgcccagctcatatttttaattattgaaaaaaaaaaaacccaattttaaaaaccacacacagactcaaatgggcacagcaccaaattatgacacattagaatccttcctatgtgctcagagaacagggtttgtgctgagcttgagataaggcttctcttgctgtccctgtcaatcaaagagactgcaaggtgggcttcagacacagtgctagcatttgtaaacaattatctgtgagaatcagcggtcactttgtcctgtgctaccaaaatcaaacactgaaagaaaatggacattgagaccaacataagactacaactaccatcccagcccccagttcaaacatttgtgttcattgctcttcgccctgatggactgtatgctaagaaagaatttgcacttgcaaaatacatttttgctaactagatgctcattttatctttttaaaaatatgtatttcagttgcacatgaaatgtactttgaaagaatgagctccaaagttctggggggctgagacaggcgggctgagtgaaatgatgaagaaacagtggctttcagtgcgggccaagagagtagtgagcaatggtcagttattgagctgtggagtgccttcaacaagggtttttagacacatccatctggtgcctcatcccagaacctcacaggcctagggacctgaaatgctccccatgacaaggcaaacttcatatcctcacatgctgagacagactcaactttcagtctggaactgggctgggtgtctgtcagtccacgccacccatatccggagtacatcagagtctgggttcagtggcagccactttcgctgccctctcctgccccacacctagcgctctgcctggcccctttgctgtgggcgtgaaaatctggcacccgggccgacagggagagagctcagtctgcgtctgctgctttctgtttgattcatcactttccccttcaccctggagcccacgttggctgtggggcacctaactggctcctgaggcccctctggggggttgaggccctgggctgcatttggcctcggcagcctgctcacgcctctcctgactgggatgtcagaggactaggttcaaactccagcatggccagctgctggctgtgtgaccttgggcatgttaagcctcagtcccttcatccatacagtgggccaaggaagggatccctgatgtgccaacagatggatttatgaccacgtgtgtgcagcacctggcactagtttacacactgcagatgcccggtactgttgtcgccagcactcaggtctaggagagtggtcttcacaactctacctcaagggttgcctttggactgtgtccccacatggtcacatttgcatctccagacgccccaatgctgcttctcggatattctgaaggcatcctacactgtcaagctccccgactgttccccccagcaccccagtctccaactcagggtggccccatttcccccaggtcccaatcagatccctgggcccactgtggtcctggccatctcacatccaaaccctcagcaatggttgtgagtcagttctgttccagaatatctgatgccactgctacagaccccagccacctccagaccctggacaagttgcagcctcctgccccagcccctttttcctggcagccagaaagagcagcctcaatgcttctctaaccctgtaactcagctcaaaaagctctttaggcccctggtccccagaaatgcattcagagctcagccaaggggacctctcggcaccacctcacccctacatatccctacccgcatgtctgcagaactccaggcttttgtccagactgtccctactgcctggtatattcctgtcctatccgcccctcctcaagcctggtgtgatgactaaggcctccagctccaggtcactcagcctatgccagaatcacagctcagccagcctatgagcaagtttcttagccccagtttgtttcttcgtcagtataacgagagggttcacagcctccatctctgaggatgtcatgaaggttgagtaagataatcctggaagtacttggcgcaggatgcaccatattctataggaccctccacttggtatcatctccctggtgcctgacacaaagtaggtcttgagagactgaggccctggccctatacctcaggagatgcacccaggagcagctgcaggtcttctagaaagccctctagggacagccctggaaacccttgctcctgctccaagggtccacaagcccaggtaacttctgcgctaagctctgcaggggacagcccaggacctagttatgctggcctcagcgtctctgatagtcaaatggacaccaatggcagcctcatcctcccttcctgtccagctatgcaacctgacctgcaactgcaccctgctgagccttggtgtcctcaactttgtaatgtggggacaactaaaaaccccatgtgccagccctggcaacatagcaagaccccgtttctaaaaaaaaaaaaaaattaaaaattagccaggcagggttgttcacacctgtagtcctagtttgctttgcttggtcacgtagctcagcctcacactgacttccaggaacagcagagggacttggacgcctctccaggcaggcaggcctgttcctggaaagccaggtggggtggggggtcttcaggtggcaaaggaaggactggcagctgtgagccagagaagagacctggctcgtgccccagccctgctcctgtcctgctaagcctcagtttcctcatctgtaccacagggatctctgtgagcgcttcaggcaccaacaatctgctccctgggctcagtaggggatatctgatcccaccatttccccagccacatgccccagaagagggccgcagacctagtacaagagggagcaataaggtgacatcctctgctctgagaggtagagtgtttggggaagaccccagcccctgggaagggggccacttagccaggcctgcctgccacggggcatggctactctaagctgtctcaccctccccctttaggcatagctggggcaggtggaggtcagcccagttcagggctttccatgaagctgaggtaggcttccctgcctttcccactttgtgagctgtaaaattagcctttcctgaccattttcctgcaggactgctgtatgtgtgagaggtagtctttggaagaaaaggggcctctagaatttgaagcttctgatttctggttatgaggccaaagatcccaaaggtccttccagacacctcaggagggccctggggggcagaggctgggggctgtacagccaattacctcagaggggaaggcacccactcattccgcaagcgggggaaatcctgctctcctcccacagctaccagagcttcagatgggactcagatctgtctgcacacccagggctacagttggcctaatgtgactcttacctgcccataaacctggcccagagggctttatgggccagaatccctgggtttagtagctacatggacagccatatgagcaccacctaattgacttaattaactaaccccaggcctttggaagcaataggagatgagagcatcatactgggagtcaggagtcaagtgctgtgttacttcaagtaagccccatccctctctgggaaaaaagatcagggattgaatataagtcttgccatgatccaccccttccagtataaacaggccctcctggcttcatccaaagcgtatccaggtgatttggggccaagctgacccttgaacccaggtgtccatgctctctgtcccccagcttctcagctctgaaacccagcatgaggcccatgtctggcctcccagtagctctccatgtggctcctgggttaggactggcttcaggagccccaagccttggctgggtgggatggtgtctccagagtcctttagtacccctggaaagggaggtcctagtcccagcttggacagggacagggctgagggcaccagttggccaattcagttttaggaaccaggaggttgagaaccccagggatagccccactccaccataggaacagaatggtgacacagctctgctcaggcctatggcttacatggaggggccaggcccattagctcaaagtcaggggctgctgtgctcatttcacagatgcagtacctgcaacccagagagtacagggcccctgctcatcctcacacacccaaggggtcctgggccagtcacataactccacaggagagcaggaacaggcttggtcccagtctctgaggtcctctctggacccagtctctggagatgggccatggaggccagccttgcactttctccccacatcccagtcccattcctcacccactcccttctgggacccatgctggtcagtctttcagtcttctcactctgggaaagggccacctctctccaaatatgagtaaaaaaagggggggcctgggcagtttaggtctgaaggttgaggaagagttcccctggccacatcacctatcagaagagaggtggttaaggcaatttatcatgactctcaaaattcttccagcctctgcccatttccacgttgcaattccaaagccacttcaatcagtaggcgtgtgttacagcagcactctaatttgggcaccacaatctatattcgtttcccgtggctgctgtaacaaattatcacacatgtgttttcacacatgtgaaaacaacacaaatttatgatcttactgttctggaggtcagcaatctgaaatcagtttcacagggcttaaaatcaaggtattggcaggactgcattcttcttgaggccccagaggagaagaggctgtctgcattcctcggctcatggctcttcctccagcaattgcatcactctgacctctgcttccattgttacatacattttcttccgtcactctgacactcctgcctcctttacagaggcccttgtgattatactcagtttacctgaaaaatccaggatactccttccatctcaagatccttaatcacatctgcaaagtccattttgctatgtgaaggtaatatagtcacatgttaaggtttaggtgattaagacactgccattttggggggtcactgttcagcctaccagagcaggggtagagttgctttgacagtcccaaatccagttcagggggcttgtccagggcagaaggtcatgaggaggagatcaggtcactgtcctagccaggactctggctgggggctggctgaagccaagagctccaggaaacctggcgcctgctcctactgccgccaaggacagcctgttctcctggtgtggctgttgcgcagggatcaggtgcacttgagtcttcgaagtggccattgctcaacttgaatggctgcctgggtcgggcagaaggccaggtcctcatggcttcccatccctaatgaccggaatacatgggctgccaggtcagatgtgggccacatgggaagtcccagctctattctagaaaatgcatgtaccatcagcttactgatagacatttactgaacttgggtatgccagatccacagggggccccagagatgagggggataagaaggtttctgaaggcatggtacagaaggtgccagcagaggtatgggctaggggaggcagggagagcacagagcaggcatcctaaaggaggcagcatttgtgttggagcttgaagaagtggattgtttgcaccgcctgggcaaagggaaggtgtgtgttcagggcatcgagagtactgcacaaaggctgaagcccagggcagtagagaagagaatccactaagaaggagccaatgaagaaaaaaaagagaaaagaatcgaaggtggatagggaaagacatgctgtcccgcagaggttaaaggggttctcacctcaagccagcagttctcaaaccttgtcagcagtggagccctttgttctgatgacagcctactcagagcactgatggggccttgggaggggcccccagggcttttcccacagttgtcctcccccacctcttcagaactggattccataggacacaagagaacacacttaagtcatggggagccagctaagtgtttggggcaaggattgggagcagccaatagcccagggtccaggtgggggtaaaggagcaaaaaagagtattttttgcatttagggggttcggggcctatttcaataaggcagctgtatgagacccatggagaaacccactgacaactgggaaaagcatccaactgtgagacaaggcctcagtttccccaactatcagaagaggagatagaattactctcccagagtacatcaaacagggactcctacactcctgtctatgctctgggctctggctgaaggaggctgcacgggcagtgggcacatctctcaagacctcaggggcttgcacagcctggactccatcagctccatgtcctcctcccattctgcctgcaagtgctccttgacatatgctggtggtggtggggaggctgttcgagtctctggctttggcctcaggagcaagggaggggatagggcaggtgggcctggctttccctgagctagagccactggctgccctggcctgggcctcaaggcactggggccatagtgaggagaggctgaggggagatgtaggctgccaggctaccagcctgctggctccatctctagacaacagtgaggagtcaagagcccaagactgaaactcctgccttcccttctttccagactgccttgtatccctgcctgccttatgttggtcccatgcatcagatggacgcctgagggcactgggtccttcctccctgtgtctgccctccgaggaaggcaaggaaaaatgccacaatgtgccaagccaggcacatcccatgggctcctcacatgcatcctataaaataaagcattaagtcccatttctcagccttagaagccaaggctgagtgaggtgaagtcatctgcccaaggtcacatcctcgtgaggggcagattctgggattgaaatccaggctggtgtggctccaacatctgggctcaacgtccagggcccaatcaagccagtggctgcaggcttgaggccccgcctgccagtcctcttggcttggaccttttcctcagcagagtcaagctgcacatttttctgggcagaaagttgtgcccgaggccggctcctgcttgtggccccagctgccccgacagtgtcactctccaacactgcactctcttctggtgcaacatccacaagctcgccaaggcccttcctcaggaatgggcctgaggccaggagggagagaccatcagggaagccaggactggctgaggtgtaggggggcgacagactgctccgaggtcagggcagctaccctgagatgctgctgaagacagcaagagccaaagggcacaaggagaaagacagaaagggcaatactggtgaggaccttagcaggcaaaggtctgtgagcatgggggactaaggaagtggggagccttgccctggttgtgcacccccttcgccctccccacccaggttccttctggagcagcctccttaaaggaagccaggggcagctcagagtccatgcagctggggctgggcacagggcaggacactggggcactgggagctgcagtgtgacctctaccaaatgtgtcctccagccatagtgcagggcaacacttaggctgggtatgactccagcaatataggctccccaaagggagggatctaacttactgtctccacttggtcactgtcatgtgacctcaggcagtacataccttctcttgctctccatgcctggcgaatggacattcagatgccagcatgcacattccacttgactaagagtaaagaggttgccagttggcgttggccctggactcagaagagccagcttctcatagggaaaggagttgcccaaggtcccactgcaggacacagccctggaactcagctctcccagctgcagcagaggatgctgcctattggaccatactgcccatcagaccatactgccaggccctgggaagtgccagggtggcagggggcagtctagtggaatgagacagcctggtttgccatgtttcttaggacccaccctgatgtaggctcacatcaccagcactcaccaacctagagatttcctgtcgctgttgacaggaaggctggatctgcaggcctcctggtggccatgagtctgcacagaccagagctggggtggaggccacaaccctgtgcccagtatctcagcttctcactctccccagccccaaccagggacacatgggttatttgaaaccccagggggtcaactcgggagggatgttttagctaaaagctatggggataaaaaggaaacacccctcactggctcaagccttcagttaaatgaacgtggatgtgcgacccaggaactgtgcagcaaagacctccagaccctcccctccagaaagcaggcagtcatccttgagccaaaacgcagatgagcttcctgtgctcgagccaggcttggccagggaattgtgtacgcatgcacccagggcagtggaggactaatcaatccctgggagtgagctgctctatgccaggacccatggtatccaaggccaggagtgaggactcacgtgccttcctccacactgcacccccacaccactaccaagcaggggactgacggccagccctgctggggcagaaggaaacccttgccccagtgctacctgggagtaagggggtcaggggacctgcaagtcatggacaaaacattaggtcaccatttgttagtctctcaatactttactggccatatcccccgatacccccacagcaatttcaccaacacagagcaactgccctcagccactctgatgtgatggagccaatccaggtgtcctagaaatatcctagaaatgcagagcatggggaaatcacagaaccctgggaaatgccataagaacctgggctctggaaagtgccatccacctcccctctggtcaggctggcggcactgacaaggcatccacagggcagccatgctatggcccagacctccggatatgcaggaaccggggcctcccacagaagtccctgcgcacagccacaagattaaggtacaggtcaggccggctctgaagccagctgctgacaagctccgggtgccttgggtccacttctaagaagataccagagtctttcaggagccggggtgccaaggccagaatgtgggtaatgatgtccatgccctcctccccaccatccagggccgcggggtcttcatagctgcggatctcaggggccagctgctccatgtcctggtggaagacgtagggagggttgctgacaatcaggtccatggggccccagggcaggtgtgtccagctcctttctgaggtcatgtcgaggtggatgatccaaatcctgtcctgcaaccgaagcctctgagcattctcatgggtcagagagatagcagcttcccgcttatccacagcaatgactcggctctgggggagctggctcagcaggctgagggagatggctcctgatccgcagcccacctccagaatgagggggctgcctggggatcccacagcatgggacctctgggccacctcttccagcacccactcaaccagttcctctgtttctggccgaggaataaacactgggggcaccatccttaggctgagcccctggaagtcccactctccaaggatgtactgcaccggcatcctctgcaatcgacggctactcagctcccggatacactgtagttgctgagaggtcaagggctgggtccaaagtgccggcctcaggctctgaaatgttttggctccaaggacatgagccacgatgtactcactggattcccgggcctcagggatacccctcttctcaaagaccccagtccagtggctgaccagttctatggcactggataacccagccagaggtggttggggttgccatgagctgaaggcccagccccgggtacttcccctcctccctgggccagacaggagggcccacagcattcggccccaaagctccatgtctcagggaaaggttctccagagtgcttccaggttcccaagtctgctttatgatgtcagctgctgaggtgagtgctgagagtggcccctggacccagctgggtggagatggagaggtcacaagctctggtgccccaaaatggctctggtcctcagatatagttggttgccaccctgcctgaaaggctgccccacccacccaccagccggagaagctgccccgaact

SEQ ID NO: 13695 - RNA, 11203 nt, Homo sapiens
  source 1..11203: mol_type = other RNA
gctgggattacaggcatgagccaccatgcccagctaatttttgtatttttagtagagacagggtttcaccatgttggccaggctggtcttgaactcctgagctcgggtgatctgcctgcttcagcctcccaaagtgctgggattacaagtgtgagccaccctgcacggcccctttctttctggcttcctcctcccttcttccttttctttcatttttaaaacatttttttaaaattattatttttaaatttttttttttgagatggagtctagctctgtcgcccaggctggagtgcagtggcatgatcttggctcactgcaatctctgcctcccgggttcaagcaattctcctgcttcagcctcccgagtagctgggattacaggtgtccaccaccacacccagctaatttttgtatttttagtagacggggtttcactgtgttggccaggctggtcttgaactcctaaccttgtgatccttggcctcccaaagtgctgggattacaaacgtgagctactgcgcctggcctattattattatttttgagacagagttttgctcttgttgcctgggtgggagtacaatggcgtgatcttggctcactgcaacatctgcctctcggtttcaagcgattctcctgcctcagcctctcaagtagctgggattacaggcgtgagccaccacacccggctaatttttgtatttttagtacagacggattttcaccatgttggccaagctggcctcgaactcctgacctcaggtgatctgcctgcctcagcctcccagagtgctgggattacaggcgtgagccaccgcgcccggcctaaaattatttttttagagacagggtctgactctgatgtccaggctggagtgcagtggcgctattatagctcactgctgtcttaaactcttgtgctcaagtaatcctcctgcctcagcctcccgagtaggtgggaccacaggcatgtgccaccatgcccagctcatatttttaattattgaaaaaaaaaaaacccaattttaaaaaccacacacagactcaaatgggcacagcaccaaattatgacacattagaatccttcctatgtgctcagagaacagggtttgtgctgagcttgagataaggcttctcttgctgtccctgtcaatcaaagagactgcaaggtgggcttcagacacagtgctagcatttgtaaacaattatctgtgagaatcagcggtcactttgtcctgtgctaccaaaatcaaacactgaaagaaaatggacattgagaccaacataagactacaactaccatcccagcccccagttcaaacatttgtgttcattgctcttcgccctgatggactgtatgctaagaaagaatttgcacttgcaaaatacatttttgctaactagatgctcattttatctttttaaaaatatgtatttcagttgcacatgaaatgtactttgaaagaatgagctccaaagttctggggggctgagacaggcgggctgagtgaaatgatgaagaaacagtggctttcagtgcgggccaagagagtagtgagcaatggtcagttattgagctgtggagtgccttcaacaagggtttttagacacatccatctggtgcctcatcccagaacctcacaggcctagggacctgaaatgctccccatgacaaggcaaacttcatatcctcacatgctgagacagactcaactttcagtctggaactgggctgggtgtctgtcagtccacgccacccatatccggagtacatcagagtctgggttcagtggcagccactttcgctgccctctcctgccccacacctagcgctctgcctggcccctttgctgtgggcgtgaaaatctggcacccgggccgacagggagagagctcagtctgcgtctgctgctttctgtttgattcatcactttccccttcaccctggagcccacgttggctgtggggcacctaactggctcctgaggcccctctggggggttgaggccctgggctgcatttggcctcggcagcctgctcacgcctctcctgactgggatgtcagaggactaggttcaaactccagcatggccagctgctggctgtgtgaccttgggcatgttaagcctcagtcccttcatccatacagtgggccaaggaagggatccctgatgtgccaacagatggatttatgaccacgtgtgtgcagcacctggcactagtttacacactgcagatgcccggtactgttgtcgccagcactcaggtctaggagagtggtcttcacaactctacctcaagggttgcctttggactgtgtccccacatggtcacatttgcatctccagacgccccaatgctgcttctcggatattctgaaggcatcctacactgtcaagctccccgactgttccccccagcaccccagtctccaactcagggtggccccatttcccccaggtcccaatcagatccctgggcccactgtggtcctggccatctcacatccaaaccctcagcaatggttgtgagtcagttctgttccagaatatctgatgccactgctacagaccccagccacctccagaccctggacaagttgcagcctcctgccccagcccctttttcctggcagccagaaagagcagcctcaatgcttctctaaccctgtaactcagctcaaaaagctctttaggcccctggtccccagaaatgcattcagagctcagccaaggggacctctcggcaccacctcacccctacatatccctacccgcatgtctgcagaactccaggcttttgtccagactgtccctactgcctggtatattcctgtcctatccgcccctcctcaagcctggtgtgatgactaaggcctccagctccaggtcactcagcctatgccagaatcacagctcagccagcctatgagcaagtttcttagccccagtttgtttcttcgtcagtataacgagagggttcacagcctccatctctgaggatgtcatgaaggttgagtaagataatcctggaagtacttggcgcaggatgcaccatattctataggaccctccacttggtatcatctccctggtgcctgacacaaagtaggtcttgagagactgaggccctggccctatacctcaggagatgcacccaggagcagctgcaggtcttctagaaagccctctagggacagccctggaaacccttgctcctgctccaagggtccacaagcccaggtaacttctgcgctaagctctgcaggggacagcccaggacctagttatgctggcctcagcgtctctgatagtcaaatggacaccaatggcagcctcatcctcccttcctgtccagctatgcaacctgacctgcaactgcaccctgctgagccttggtgtcctcaactttgtaatgtggggacaactaaaaaccccatgtgccagccctggcaacatagcaagaccccgtttctaaaaaaaaaaaaaaattaaaaattagccaggcagggttgttcacacctgtagtcctagtttgctttgcttggtcacgtagctcagcctcacactgacttccaggaacagcagagggacttggacgcctctccaggcaggcaggcctgttcctggaaagccaggtggggtggggggtcttcaggtggcaaaggaaggactggcagctgtgagccagagaagagacctggctcgtgccccagccctgctcctgtcctgctaagcctcagtttcctcatctgtaccacagggatctctgtgagcgcttcaggcaccaacaatctgctccctgggctcagtaggggatatctgatcccaccatttccccagccacatgccccagaagagggccgcagacctagtacaagagggagcaataaggtgacatcctctgctctgagaggtagagtgtttggggaagaccccagcccctgggaagggggccacttagccaggcctgcctgccacggggcatggctactctaagctgtctcaccctccccctttaggcatagctggggcaggtggaggtcagcccagttcagggctttccatgaagctgaggtaggcttccctgcctttcccactttgtgagctgtaaaattagcctttcctgaccattttcctgcaggactgctgtatgtgtgagaggtagtctttggaagaaaaggggcctctagaatttgaagcttctgatttctggttatgaggccaaagatcccaaaggtccttccagacacctcaggagggccctggggggcagaggctgggggctgtacagccaattacctcagaggggaaggcacccactcattccgcaagcgggggaaatcctgctctcctcccacagctaccagagcttcagatgggactcagatctgtctgcacacccagggctacagttggcctaatgtgactcttacctgcccataaacctggcccagagggctttatgggccagaatccctgggtttagtagctacatggacagccatatgagcaccacctaattgacttaattaactaaccccaggcctttggaagcaataggagatgagagcatcatactgggagtcaggagtcaagtgctgtgttacttcaagtaagccccatccctctctgggaaaaaagatcagggattgaatataagtcttgccatgatccaccccttccagtataaacaggccctcctggcttcatccaaagcgtatccaggtgatttggggccaagctgacccttgaacccaggtgtccatgctctctgtcccccagcttctcagctctgaaacccagcatgaggcccatgtctggcctcccagtagctctccatgtggctcctgggttaggactggcttcaggagccccaagccttggctgggtgggatggtgtctccagagtcctttagtacccctggaaagggaggtcctagtcccagcttggacagggacagggctgagggcaccagttggccaattcagttttaggaaccaggaggttgagaaccccagggatagccccactccaccataggaacagaatggtgacacagctctgctcaggcctatggcttacatggaggggccaggcccattagctcaaagtcaggggctgctgtgctcatttcacagatgcagtacctgcaacccagagagtacagggcccctgctcatcctcacacacccaaggggtcctgggccagtcacataactccacaggagagcaggaacaggcttggtcccagtctctgaggtcctctctggacccagtctctggagatgggccatggaggccagccttgcactttctccccacatcccagtcccattcctcacccactcccttctgggacccatgctggtcagtctttcagtcttctcactctgggaaagggccacctctctccaaatatgagtaaaaaaagggggggcctgggcagtttaggtctgaaggttgaggaagagttcccctggccacatcacctatcagaagagaggtggttaaggcaatttatcatgactctcaaaattcttccagcctctgcccatttccacgttgcaattccaaagccacttcaatcagtaggcgtgtgttacagcagcactctaatttgggcaccacaatctatattcgtttcccgtggctgctgtaacaaattatcacacatgtgttttcacacatgtgaaaacaacacaaatttatgatcttactgttctggaggtcagcaatctgaaatcagtttcacagggcttaaaatcaaggtattggcaggactgcattcttcttgaggccccagaggagaagaggctgtctgcattcctcggctcatggctcttcctccagcaattgcatcactctgacctctgcttccattgttacatacattttcttccgtcactctgacactcctgcctcctttacagaggcccttgtgattatactcagtttacctgaaaaatccaggatactccttccatctcaagatccttaatcacatctgcaaagtccattttgctatgtgaaggtaatatagtcacatgttaaggtttaggtgattaagacactgccattttggggggtcactgttcagcctaccagagcaggggtagagttgctttgacagtcccaaatccagttcagggggcttgtccagggcagaaggtcatgaggaggagatcaggtcactgtcctagccaggactctggctgggggctggctgaagccaagagctccaggaaacctggcgcctgctcctactgccgccaaggacagcctgttctcctggtgtggctgttgcgcagggatcaggtgcacttgagtcttcgaagtggccattgctcaacttgaatggctgcctgggtcgggcagaaggccaggtcctcatggcttcccatccctaatgaccggaatacatgggctgccaggtcagatgtgggccacatgggaagtcccagctctattctagaaaatgcatgtaccatcagcttactgatagacatttactgaacttgggtatgccagatccacagggggccccagagatgagggggataagaaggtttctgaaggcatggtacagaaggtgccagcagaggtatgggctaggggaggcagggagagcacagagcaggcatcctaaaggaggcagcatttgtgttggagcttgaagaagtggattgtttgcaccgcctgggcaaagggaaggtgtgtgttcagggcatcgagagtactgcacaaaggctgaagcccagggcagtagagaagagaatccactaagaaggagccaatgaagaaaaaaaagagaaaagaatcgaaggtggatagggaaagacatgctgtcccgcagaggttaaaggggttctcacctcaagccagcagttctcaaaccttgtcagcagtggagccctttgttctgatgacagcctactcagagcactgatggggccttgggaggggcccccagggcttttcccacagttgtcctcccccacctcttcagaactggattccataggacacaagagaacacacttaagtcatggggagccagctaagtgtttggggcaaggattgggagcagccaatagcccagggtccaggtgggggtaaaggagcaaaaaagagtattttttgcatttagggggttcggggcctatttcaataaggcagctgtatgagacccatggagaaacccactgacaactgggaaaagcatccaactgtgagacaaggcctcagtttccccaactatcagaagaggagatagaattactctcccagagtacatcaaacagggactcctacactcctgtctatgctctgggctctggctgaaggaggctgcacgggcagtgggcacatctctcaagacctcaggggcttgcacagcctggactccatcagctccatgtcctcctcccattctgcctgcaagtgctccttgacatatgctggtggtggtggggaggctgttcgagtctctggctttggcctcaggagcaagggaggggatagggcaggtgggcctggctttccctgagctagagccactggctgccctggcctgggcctcaaggcactggggccatagtgaggagaggctgaggggagatgtaggctgccaggctaccagcctgctggctccatctctagacaacagtgaggagtcaagagcccaagactgaaactcctgccttcccttctttccagactgccttgtatccctgcctgccttatgttggtcccatgcatcagatggacgcctgagggcactgggtccttcctccctgtgtctgccctccgaggaaggcaaggaaaaatgccacaatgtgccaagccaggcacatcccatgggctcctcacatgcatcctataaaataaagcattaagtcccatttctcagccttagaagccaaggctgagtgaggtgaagtcatctgcccaaggtcacatcctcgtgaggggcagattctgggattgaaatccaggctggtgtggctccaacatctgggctcaacgtccagggcccaatcaagccagtggctgcaggcttgaggccccgcctgccagtcctcttggcttggaccttttcctcagcagagtcaagctgcacatttttctgggcagaaagttgtgcccgaggccggctcctgcttgtggccccagctgccccgacagtgtcactctccaacactgcactctcttctggtgcaacatccacaagctcgccaaggcccttcctcaggaatgggcctgaggccaggagggagagaccatcagggaagccaggactggctgaggtgtaggggggcgacagactgctccgaggtcagggcagctaccctgagatgctgctgaagacagcaagagccaaagggcacaaggagaaagacagaaagggcaatactggtgaggaccttagcaggcaaaggtctgtgagcatgggggactaaggaagtggggagccttgccctggttgtgcacccccttcgccctccccacccaggttccttctggagcagcctccttaaaggaagccaggggcagctcagagtccatgcagctggggctgggcacagggcaggacactggggcactgggagctgcagtgtgacctctaccaaatgtgtcctccagccatagtgcagggcaacacttaggctgggtatgactccagcaatataggctccccaaagggagggatctaacttactgtctccacttggtcactgtcatgtgacctcaggcagtacataccttctcttgctctccatgcctggcgaatggacattcagatgccagcatgcacattccacttgactaagagtaaagaggttgccagttggcgttggccctggactcagaagagccagcttctcatagggaaaggagttgcccaaggtcccactgcaggacacagccctggaactcagctctcccagctgcagcagaggatgctgcctattggaccatactgcccatcagaccatactgccaggccctgggaagtgccagggtggcagggggcagtctagtggaatgagacagcctggtttgccatgtttcttaggacccaccctgatgtaggctcacatcaccagcactcaccaacctagagatttcctgtcgctgttgacaggaaggctggatctgcaggcctcctggtggccatgagtctgcacagaccagagctggggtggaggccacaaccctgtgcccagtatctcagcttctcactctccccagccccaaccagggacacatgggttatttgaaaccccagggggtcaactcgggagggatgttttagctaaaagctatggggataaaaaggaaacacccctcactggctcaagccttcagttaaatgaacgtggatgtgcgacccaggaactgtgcagcaaagacctccagaccctcccctccagaaagcaggcagtcatccttgagccaaaacgcagatgagcttcctgtgctcgagccaggcttggccagggaattgtgtacgcatgcacccagggcagtggaggactaatcaatccctgggagtgagctgctctatgccaggacccatggtatccaaggccaggagtgaggactcacgtgccttcctccacactgcacccccacaccactaccaagcaggggactgacggccagccctgctggggcagaaggaaacccttgccccagtgctacctgggagtaagggggtcaggggacctgcaagtcatggacaaaacattaggtcaccatttgttagtctctcaatactttactggccatatcccccgatacccccacagcaatttcaccaacacagagcaactgccctcagccactctgatgtgatggagccaatccaggtgtcctagaaatatcctagaaatgcagagcatggggaaatcacagaaccctgggaaatgccataagaacctgggctctggaaagtgccatccacctcccctctggtcaggctggcggcactgacaaggcatccacagggcagccatgctatggcccagacctccggatatgcaggaaccggggcctcccacagaagtccctgcgcacagccacaagattaaggtacaggtcaggccggctctgaagccagctgctgacaagctccgggtgccttgggtccacttctaagaagatactaccagagtctttcaggagccggggtgccaaggccagaatgtgggtaatgatgtccatgccctcctccccaccatccagggccgcggggtcttcatagctgcggatctcaggggccagctgctccatgtcctggtggaagacgtagggagggttgctgacaatcaggtccatggggccccagggcaggtgtgtccagctcctttctgaggtcatgtcgaggtggatgatccaaatcctgtcctgcaaccgaagcctctgagcattctcatgggtcagagagatagcagcttcccgcttatccacagcaatgactcggctctgggggagctggctcagcaggctgagggagatggctcctgatccgcagcccacctccagaatgagggggctgcctggggatcccacagcatgggacctctgggccacctcttccagcacccactcaaccagttcctctgtttctggccgaggaataaacactgggggcaccatccttaggctgagcccctggaagtcccactctccaaggatgtactgcaccggcatcctctgcaatcgacggctactcagctcccggatacactgtagttgctgagaggtcaagggctgggtccaaagtgccggcctcaggctctgaaatggattcccgggcctcagggatacccctcttctcaaagaccccagtccagtggctgaccagttctatggcactggataacccagccagaggtggttggggttgccatgagctgaaggcccagccccgggtacttcccctcctccctgggccagacaggagggcccacagcattcggccccaaagctccatgtctcagggaaaggttctccagagtgcttccaggttcccaagtctgctttatgatgtcagctgctgaggtgagtgctgagagtggcccctggacccagctgggtggagatggagaggtcacaagctctggtgccccaaaatggctctggtcctcagatatagttggttgccacccagccggagaagctgccccgaact

SEQ ID NO: 13696 - RNA, 11232 nt, Homo sapiens
  source 1..11232: mol_type = other RNA
gctgggattacaggcatgagccaccatgcccagctaatttttgtatttttagtagagacagggtttcaccatgttggccaggctggtcttgaactcctgagctcgggtgatctgcctgcttcagcctcccaaagtgctgggattacaagtgtgagccaccctgcacggcccctttctttctggcttcctcctcccttcttccttttctttcatttttaaaacatttttttaaaattattatttttaaatttttttttttgagatggagtctagctctgtcgcccaggctggagtgcagtggcatgatcttggctcactgcaatctctgcctcccgggttcaagcaattctcctgcttcagcctcccgagtagctgggattacaggtgtccaccaccacacccagctaatttttgtatttttagtagacggggtttcactgtgttggccaggctggtcttgaactcctaaccttgtgatccttggcctcccaaagtgctgggattacaaacgtgagctactgcgcctggcctattattattatttttgagacagagttttgctcttgttgcctgggtgggagtacaatggcgtgatcttggctcactgcaacatctgcctctcggtttcaagcgattctcctgcctcagcctctcaagtagctgggattacaggcgtgagccaccacacccggctaatttttgtatttttagtacagacggattttcaccatgttggccaagctggcctcgaactcctgacctcaggtgatctgcctgcctcagcctcccagagtgctgggattacaggcgtgagccaccgcgcccggcctaaaattatttttttagagacagggtctgactctgatgtccaggctggagtgcagtggcgctattatagctcactgctgtcttaaactcttgtgctcaagtaatcctcctgcctcagcctcccgagtaggtgggaccacaggcatgtgccaccatgcccagctcatatttttaattattgaaaaaaaaaaaacccaattttaaaaaccacacacagactcaaatgggcacagcaccaaattatgacacattagaatccttcctatgtgctcagagaacagggtttgtgctgagcttgagataaggcttctcttgctgtccctgtcaatcaaagagactgcaaggtgggcttcagacacagtgctagcatttgtaaacaattatctgtgagaatcagcggtcactttgtcctgtgctaccaaaatcaaacactgaaagaaaatggacattgagaccaacataagactacaactaccatcccagcccccagttcaaacatttgtgttcattgctcttcgccctgatggactgtatgctaagaaagaatttgcacttgcaaaatacatttttgctaactagatgctcattttatctttttaaaaatatgtatttcagttgcacatgaaatgtactttgaaagaatgagctccaaagttctggggggctgagacaggcgggctgagtgaaatgatgaagaaacagtggctttcagtgcgggccaagagagtagtgagcaatggtcagttattgagctgtggagtgccttcaacaagggtttttagacacatccatctggtgcctcatcccagaacctcacaggcctagggacctgaaatgctccccatgacaaggcaaacttcatatcctcacatgctgagacagactcaactttcagtctggaactgggctgggtgtctgtcagtccacgccacccatatccggagtacatcagagtctgggttcagtggcagccactttcgctgccctctcctgccccacacctagcgctctgcctggcccctttgctgtgggcgtgaaaatctggcacccgggccgacagggagagagctcagtctgcgtctgctgctttctgtttgattcatcactttccccttcaccctggagcccacgttggctgtggggcacctaactggctcctgaggcccctctggggggttgaggccctgggctgcatttggcctcggcagcctgctcacgcctctcctgactgggatgtcagaggactaggttcaaactccagcatggccagctgctggctgtgtgaccttgggcatgttaagcctcagtcccttcatccatacagtgggccaaggaagggatccctgatgtgccaacagatggatttatgaccacgtgtgtgcagcacctggcactagtttacacactgcagatgcccggtactgttgtcgccagcactcaggtctaggagagtggtcttcacaactctacctcaagggttgcctttggactgtgtccccacatggtcacatttgcatctccagacgccccaatgctgcttctcggatattctgaaggcatcctacactgtcaagctccccgactgttccccccagcaccccagtctccaactcagggtggccccatttcccccaggtcccaatcagatccctgggcccactgtggtcctggccatctcacatccaaaccctcagcaatggttgtgagtcagttctgttccagaatatctgatgccactgctacagaccccagccacctccagaccctggacaagttgcagcctcctgccccagcccctttttcctggcagccagaaagagcagcctcaatgcttctctaaccctgtaactcagctcaaaaagctctttaggcccctggtccccagaaatgcattcagagctcagccaaggggacctctcggcaccacctcacccctacatatccctacccgcatgtctgcagaactccaggcttttgtccagactgtccctactgcctggtatattcctgtcctatccgcccctcctcaagcctggtgtgatgactaaggcctccagctccaggtcactcagcctatgccagaatcacagctcagccagcctatgagcaagtttcttagccccagtttgtttcttcgtcagtataacgagagggttcacagcctccatctctgaggatgtcatgaaggttgagtaagataatcctggaagtacttggcgcaggatgcaccatattctataggaccctccacttggtatcatctccctggtgcctgacacaaagtaggtcttgagagactgaggccctggccctatacctcaggagatgcacccaggagcagctgcaggtcttctagaaagccctctagggacagccctggaaacccttgctcctgctccaagggtccacaagcccaggtaacttctgcgctaagctctgcaggggacagcccaggacctagttatgctggcctcagcgtctctgatagtcaaatggacaccaatggcagcctcatcctcccttcctgtccagctatgcaacctgacctgcaactgcaccctgctgagccttggtgtcctcaactttgtaatgtggggacaactaaaaaccccatgtgccagccctggcaacatagcaagaccccgtttctaaaaaaaaaaaaaaattaaaaattagccaggcagggttgttcacacctgtagtcctagtttgctttgcttggtcacgtagctcagcctcacactgacttccaggaacagcagagggacttggacgcctctccaggcaggcaggcctgttcctggaaagccaggtggggtggggggtcttcaggtggcaaaggaaggactggcagctgtgagccagagaagagacctggctcgtgccccagccctgctcctgtcctgctaagcctcagtttcctcatctgtaccacagggatctctgtgagcgcttcaggcaccaacaatctgctccctgggctcagtaggggatatctgatcccaccatttccccagccacatgccccagaagagggccgcagacctagtacaagagggagcaataaggtgacatcctctgctctgagaggtagagtgtttggggaagaccccagcccctgggaagggggccacttagccaggcctgcctgccacggggcatggctactctaagctgtctcaccctccccctttaggcatagctggggcaggtggaggtcagcccagttcagggctttccatgaagctgaggtaggcttccctgcctttcccactttgtgagctgtaaaattagcctttcctgaccattttcctgcaggactgctgtatgtgtgagaggtagtctttggaagaaaaggggcctctagaatttgaagcttctgatttctggttatgaggccaaagatcccaaaggtccttccagacacctcaggagggccctggggggcagaggctgggggctgtacagccaattacctcagaggggaaggcacccactcattccgcaagcgggggaaatcctgctctcctcccacagctaccagagcttcagatgggactcagatctgtctgcacacccagggctacagttggcctaatgtgactcttacctgcccataaacctggcccagagggctttatgggccagaatccctgggtttagtagctacatggacagccatatgagcaccacctaattgacttaattaactaaccccaggcctttggaagcaataggagatgagagcatcatactgggagtcaggagtcaagtgctgtgttacttcaagtaagccccatccctctctgggaaaaaagatcagggattgaatataagtcttgccatgatccaccccttccagtataaacaggccctcctggcttcatccaaagcgtatccaggtgatttggggccaagctgacccttgaacccaggtgtccatgctctctgtcccccagcttctcagctctgaaacccagcatgaggcccatgtctggcctcccagtagctctccatgtggctcctgggttaggactggcttcaggagccccaagccttggctgggtgggatggtgtctccagagtcctttagtacccctggaaagggaggtcctagtcccagcttggacagggacagggctgagggcaccagttggccaattcagttttaggaaccaggaggttgagaaccccagggatagccccactccaccataggaacagaatggtgacacagctctgctcaggcctatggcttacatggaggggccaggcccattagctcaaagtcaggggctgctgtgctcatttcacagatgcagtacctgcaacccagagagtacagggcccctgctcatcctcacacacccaaggggtcctgggccagtcacataactccacaggagagcaggaacaggcttggtcccagtctctgaggtcctctctggacccagtctctggagatgggccatggaggccagccttgcactttctccccacatcccagtcccattcctcacccactcccttctgggacccatgctggtcagtctttcagtcttctcactctgggaaagggccacctctctccaaatatgagtaaaaaaagggggggcctgggcagtttaggtctgaaggttgaggaagagttcccctggccacatcacctatcagaagagaggtggttaaggcaatttatcatgactctcaaaattcttccagcctctgcccatttccacgttgcaattccaaagccacttcaatcagtaggcgtgtgttacagcagcactctaatttgggcaccacaatctatattcgtttcccgtggctgctgtaacaaattatcacacatgtgttttcacacatgtgaaaacaacacaaatttatgatcttactgttctggaggtcagcaatctgaaatcagtttcacagggcttaaaatcaaggtattggcaggactgcattcttcttgaggccccagaggagaagaggctgtctgcattcctcggctcatggctcttcctccagcaattgcatcactctgacctctgcttccattgttacatacattttcttccgtcactctgacactcctgcctcctttacagaggcccttgtgattatactcagtttacctgaaaaatccaggatactccttccatctcaagatccttaatcacatctgcaaagtccattttgctatgtgaaggtaatatagtcacatgttaaggtttaggtgattaagacactgccattttggggggtcactgttcagcctaccagagcaggggtagagttgctttgacagtcccaaatccagttcagggggcttgtccagggcagaaggtcatgaggaggagatcaggtcactgtcctagccaggactctggctgggggctggctgaagccaagagctccaggaaacctggcgcctgctcctactgccgccaaggacagcctgttctcctggtgtggctgttgcgcagggatcaggtgcacttgagtcttcgaagtggccattgctcaacttgaatggctgcctgggtcgggcagaaggccaggtcctcatggcttcccatccctaatgaccggaatacatgggctgccaggtcagatgtgggccacatgggaagtcccagctctattctagaaaatgcatgtaccatcagcttactgatagacatttactgaacttgggtatgccagatccacagggggccccagagatgagggggataagaaggtttctgaaggcatggtacagaaggtgccagcagaggtatgggctaggggaggcagggagagcacagagcaggcatcctaaaggaggcagcatttgtgttggagcttgaagaagtggattgtttgcaccgcctgggcaaagggaaggtgtgtgttcagggcatcgagagtactgcacaaaggctgaagcccagggcagtagagaagagaatccactaagaaggagccaatgaagaaaaaaaagagaaaagaatcgaaggtggatagggaaagacatgctgtcccgcagaggttaaaggggttctcacctcaagccagcagttctcaaaccttgtcagcagtggagccctttgttctgatgacagcctactcagagcactgatggggccttgggaggggcccccagggcttttcccacagttgtcctcccccacctcttcagaactggattccataggacacaagagaacacacttaagtcatggggagccagctaagtgtttggggcaaggattgggagcagccaatagcccagggtccaggtgggggtaaaggagcaaaaaagagtattttttgcatttagggggttcggggcctatttcaataaggcagctgtatgagacccatggagaaacccactgacaactgggaaaagcatccaactgtgagacaaggcctcagtttccccaactatcagaagaggagatagaattactctcccagagtacatcaaacagggactcctacactcctgtctatgctctgggctctggctgaaggaggctgcacgggcagtgggcacatctctcaagacctcaggggcttgcacagcctggactccatcagctccatgtcctcctcccattctgcctgcaagtgctccttgacatatgctggtggtggtggggaggctgttcgagtctctggctttggcctcaggagcaagggaggggatagggcaggtgggcctggctttccctgagctagagccactggctgccctggcctgggcctcaaggcactggggccatagtgaggagaggctgaggggagatgtaggctgccaggctaccagcctgctggctccatctctagacaacagtgaggagtcaagagcccaagactgaaactcctgccttcccttctttccagactgccttgtatccctgcctgccttatgttggtcccatgcatcagatggacgcctgagggcactgggtccttcctccctgtgtctgccctccgaggaaggcaaggaaaaatgccacaatgtgccaagccaggcacatcccatgggctcctcacatgcatcctataaaataaagcattaagtcccatttctcagccttagaagccaaggctgagtgaggtgaagtcatctgcccaaggtcacatcctcgtgaggggcagattctgggattgaaatccaggctggtgtggctccaacatctgggctcaacgtccagggcccaatcaagccagtggctgcaggcttgaggccccgcctgccagtcctcttggcttggaccttttcctcagcagagtcaagctgcacatttttctgggcagaaagttgtgcccgaggccggctcctgcttgtggccccagctgccccgacagtgtcactctccaacactgcactctcttctggtgcaacatccacaagctcgccaaggcccttcctcaggaatgggcctgaggccaggagggagagaccatcagggaagccaggactggctgaggtgtaggggggcgacagactgctccgaggtcagggcagctaccctgagatgctgctgaagacagcaagagccaaagggcacaaggagaaagacagaaagggcaatactggtgaggaccttagcaggcaaaggtctgtgagcatgggggactaaggaagtggggagccttgccctggttgtgcacccccttcgccctccccacccaggttccttctggagcagcctccttaaaggaagccaggggcagctcagagtccatgcagctggggctgggcacagggcaggacactggggcactgggagctgcagtgtgacctctaccaaatgtgtcctccagccatagtgcagggcaacacttaggctgggtatgactccagcaatataggctccccaaagggagggatctaacttactgtctccacttggtcactgtcatgtgacctcaggcagtacataccttctcttgctctccatgcctggcgaatggacattcagatgccagcatgcacattccacttgactaagagtaaagaggttgccagttggcgttggccctggactcagaagagccagcttctcatagggaaaggagttgcccaaggtcccactgcaggacacagccctggaactcagctctcccagctgcagcagaggatgctgcctattggaccatactgcccatcagaccatactgccaggccctgggaagtgccagggtggcagggggcagtctagtggaatgagacagcctggtttgccatgtttcttaggacccaccctgatgtaggctcacatcaccagcactcaccaacctagagatttcctgtcgctgttgacaggaaggctggatctgcaggcctcctggtggccatgagtctgcacagaccagagctggggtggaggccacaaccctgtgcccagtatctcagcttctcactctccccagccccaaccagggacacatgggttatttgaaaccccagggggtcaactcgggagggatgttttagctaaaagctatggggataaaaaggaaacacccctcactggctcaagccttcagttaaatgaacgtggatgtgcgacccaggaactgtgcagcaaagacctccagaccctcccctccagaaagcaggcagtcatccttgagccaaaacgcagatgagcttcctgtgctcgagccaggcttggccagggaattgtgtacgcatgcacccagggcagtggaggactaatcaatccctgggagtgagctgctctatgccaggacccatggtatccaaggccaggagtgaggactcacgtgccttcctccacactgcacccccacaccactaccaagcaggggactgacggccagccctgctggggcagaaggaaacccttgccccagtgctacctgggagtaagggggtcaggggacctgcaagtcatggacaaaacattaggtcaccatttgttagtctctcaatactttactggccatatcccccgatacccccacagcaatttcaccaacacagagcaactgccctcagccactctgatgtgatggagccaatccaggtgtcctagaaatatcctagaaatgcagagcatggggaaatcacagaaccctgggaaatgccataagaacctgggctctggaaagtgccatccacctcccctctggtcaggctggcggcactgacaaggcatccacagggcagccatgctatggcccagacctccggatatgcaggaaccggggcctcccacagaagtccctgcgcacagccacaagattaaggtacaggtcaggccggctctgaagccagctgctgacaagctccgggtgccttgggtccacttctaagaagatactaccagagtctttcaggagccggggtgccaaggccagaatgtgggtaatgatgtccatgccctcctccccaccatccagggccgcggggtcttcatagctgcggatctcaggggccagctgctccatgtcctggtggaagacgtagggagggttgctgacaatcaggtccatggggccccagggcaggtgtgtccagctcctttctgaggtcatgtcgaggtggatgatccaaatcctgtcctgcaaccgaagcctctgagcattctcatgggtcagagagatagcagcttcccgcttatccacagcaatgactcggctctgggggagctggctcagcaggctgagggagatggctcctgatccgcagcccacctccagaatgagggggctgcctggggatcccacagcatgggacctctgggccacctcttccagcacccactcaaccagttcctctgtttctggccgaggaataaacactgggggcaccatccttaggctgagcccctggaagtcccactctccaaggatgtactgcaccggcatcctctgcaatcgacggctactcagctcccggatacactgtagttgctgagaggtcaagggctgggtccaaagtgccggcctcaggctctgaaatggattcccgggcctcagggatacccctcttctcaaagaccccagtccagtggctgaccagttctatggcactggataacccagccagaggtggttggggttgccatgagctgaaggcccagccccgggtacttcccctcctccctgggccagacaggagggcccacagcattcggccccaaagctccatgtctcagggaaaggttctccagagtgcttccaggttcccaagtctgctttatgatgtcagctgctgaggtgagtgctgagagtggcccctggacccagctgggtggagatggagaggtcacaagctctggtgccccaaaatggctctggtcctcagatatagttggttgccaccctgcctgaaaggctgccccacccacccaccagccggagaagctgccccgaact

SEQ ID NO: 13697 - RNA, 11241 nt, Homo sapiens
  source 1..11241: mol_type = other RNA
gctgggattacaggcatgagccaccatgcccagctaatttttgtatttttagtagagacagggtttcaccatgttggccaggctggtcttgaactcctgagctcgggtgatctgcctgcttcagcctcccaaagtgctgggattacaagtgtgagccaccctgcacggcccctttctttctggcttcctcctcccttcttccttttctttcatttttaaaacatttttttaaaattattatttttaaatttttttttttgagatggagtctagctctgtcgcccaggctggagtgcagtggcatgatcttggctcactgcaatctctgcctcccgggttcaagcaattctcctgcttcagcctcccgagtagctgggattacaggtgtccaccaccacacccagctaatttttgtatttttagtagacggggtttcactgtgttggccaggctggtcttgaactcctaaccttgtgatccttggcctcccaaagtgctgggattacaaacgtgagctactgcgcctggcctattattattatttttgagacagagttttgctcttgttgcctgggtgggagtacaatggcgtgatcttggctcactgcaacatctgcctctcggtttcaagcgattctcctgcctcagcctctcaagtagctgggattacaggcgtgagccaccacacccggctaatttttgtatttttagtacagacggattttcaccatgttggccaagctggcctcgaactcctgacctcaggtgatctgcctgcctcagcctcccagagtgctgggattacaggcgtgagccaccgcgcccggcctaaaattatttttttagagacagggtctgactctgatgtccaggctggagtgcagtggcgctattatagctcactgctgtcttaaactcttgtgctcaagtaatcctcctgcctcagcctcccgagtaggtgggaccacaggcatgtgccaccatgcccagctcatatttttaattattgaaaaaaaaaaaacccaattttaaaaaccacacacagactcaaatgggcacagcaccaaattatgacacattagaatccttcctatgtgctcagagaacagggtttgtgctgagcttgagataaggcttctcttgctgtccctgtcaatcaaagagactgcaaggtgggcttcagacacagtgctagcatttgtaaacaattatctgtgagaatcagcggtcactttgtcctgtgctaccaaaatcaaacactgaaagaaaatggacattgagaccaacataagactacaactaccatcccagcccccagttcaaacatttgtgttcattgctcttcgccctgatggactgtatgctaagaaagaatttgcacttgcaaaatacatttttgctaactagatgctcattttatctttttaaaaatatgtatttcagttgcacatgaaatgtactttgaaagaatgagctccaaagttctggggggctgagacaggcgggctgagtgaaatgatgaagaaacagtggctttcagtgcgggccaagagagtagtgagcaatggtcagttattgagctgtggagtgccttcaacaagggtttttagacacatccatctggtgcctcatcccagaacctcacaggcctagggacctgaaatgctccccatgacaaggcaaacttcatatcctcacatgctgagacagactcaactttcagtctggaactgggctgggtgtctgtcagtccacgccacccatatccggagtacatcagagtctgggttcagtggcagccactttcgctgccctctcctgccccacacctagcgctctgcctggcccctttgctgtgggcgtgaaaatctggcacccgggccgacagggagagagctcagtctgcgtctgctgctttctgtttgattcatcactttccccttcaccctggagcccacgttggctgtggggcacctaactggctcctgaggcccctctggggggttgaggccctgggctgcatttggcctcggcagcctgctcacgcctctcctgactgggatgtcagaggactaggttcaaactccagcatggccagctgctggctgtgtgaccttgggcatgttaagcctcagtcccttcatccatacagtgggccaaggaagggatccctgatgtgccaacagatggatttatgaccacgtgtgtgcagcacctggcactagtttacacactgcagatgcccggtactgttgtcgccagcactcaggtctaggagagtggtcttcacaactctacctcaagggttgcctttggactgtgtccccacatggtcacatttgcatctccagacgccccaatgctgcttctcggatattctgaaggcatcctacactgtcaagctccccgactgttccccccagcaccccagtctccaactcagggtggccccatttcccccaggtcccaatcagatccctgggcccactgtggtcctggccatctcacatccaaaccctcagcaatggttgtgagtcagttctgttccagaatatctgatgccactgctacagaccccagccacctccagaccctggacaagttgcagcctcctgccccagcccctttttcctggcagccagaaagagcagcctcaatgcttctctaaccctgtaactcagctcaaaaagctctttaggcccctggtccccagaaatgcattcagagctcagccaaggggacctctcggcaccacctcacccctacatatccctacccgcatgtctgcagaactccaggcttttgtccagactgtccctactgcctggtatattcctgtcctatccgcccctcctcaagcctggtgtgatgactaaggcctccagctccaggtcactcagcctatgccagaatcacagctcagccagcctatgagcaagtttcttagccccagtttgtttcttcgtcagtataacgagagggttcacagcctccatctctgaggatgtcatgaaggttgagtaagataatcctggaagtacttggcgcaggatgcaccatattctataggaccctccacttggtatcatctccctggtgcctgacacaaagtaggtcttgagagactgaggccctggccctatacctcaggagatgcacccaggagcagctgcaggtcttctagaaagccctctagggacagccctggaaacccttgctcctgctccaagggtccacaagcccaggtaacttctgcgctaagctctgcaggggacagcccaggacctagttatgctggcctcagcgtctctgatagtcaaatggacaccaatggcagcctcatcctcccttcctgtccagctatgcaacctgacctgcaactgcaccctgctgagccttggtgtcctcaactttgtaatgtggggacaactaaaaaccccatgtgccagccctggcaacatagcaagaccccgtttctaaaaaaaaaaaaaaattaaaaattagccaggcagggttgttcacacctgtagtcctagtttgctttgcttggtcacgtagctcagcctcacactgacttccaggaacagcagagggacttggacgcctctccaggcaggcaggcctgttcctggaaagccaggtggggtggggggtcttcaggtggcaaaggaaggactggcagctgtgagccagagaagagacctggctcgtgccccagccctgctcctgtcctgctaagcctcagtttcctcatctgtaccacagggatctctgtgagcgcttcaggcaccaacaatctgctccctgggctcagtaggggatatctgatcccaccatttccccagccacatgccccagaagagggccgcagacctagtacaagagggagcaataaggtgacatcctctgctctgagaggtagagtgtttggggaagaccccagcccctgggaagggggccacttagccaggcctgcctgccacggggcatggctactctaagctgtctcaccctccccctttaggcatagctggggcaggtggaggtcagcccagttcagggctttccatgaagctgaggtaggcttccctgcctttcccactttgtgagctgtaaaattagcctttcctgaccattttcctgcaggactgctgtatgtgtgagaggtagtctttggaagaaaaggggcctctagaatttgaagcttctgatttctggttatgaggccaaagatcccaaaggtccttccagacacctcaggagggccctggggggcagaggctgggggctgtacagccaattacctcagaggggaaggcacccactcattccgcaagcgggggaaatcctgctctcctcccacagctaccagagcttcagatgggactcagatctgtctgcacacccagggctacagttggcctaatgtgactcttacctgcccataaacctggcccagagggctttatgggccagaatccctgggtttagtagctacatggacagccatatgagcaccacctaattgacttaattaactaaccccaggcctttggaagcaataggagatgagagcatcatactgggagtcaggagtcaagtgctgtgttacttcaagtaagccccatccctctctgggaaaaaagatcagggattgaatataagtcttgccatgatccaccccttccagtataaacaggccctcctggcttcatccaaagcgtatccaggtgatttggggccaagctgacccttgaacccaggtgtccatgctctctgtcccccagcttctcagctctgaaacccagcatgaggcccatgtctggcctcccagtagctctccatgtggctcctgggttaggactggcttcaggagccccaagccttggctgggtgggatggtgtctccagagtcctttagtacccctggaaagggaggtcctagtcccagcttggacagggacagggctgagggcaccagttggccaattcagttttaggaaccaggaggttgagaaccccagggatagccccactccaccataggaacagaatggtgacacagctctgctcaggcctatggcttacatggaggggccaggcccattagctcaaagtcaggggctgctgtgctcatttcacagatgcagtacctgcaacccagagagtacagggcccctgctcatcctcacacacccaaggggtcctgggccagtcacataactccacaggagagcaggaacaggcttggtcccagtctctgaggtcctctctggacccagtctctggagatgggccatggaggccagccttgcactttctccccacatcccagtcccattcctcacccactcccttctgggacccatgctggtcagtctttcagtcttctcactctgggaaagggccacctctctccaaatatgagtaaaaaaagggggggcctgggcagtttaggtctgaaggttgaggaagagttcccctggccacatcacctatcagaagagaggtggttaaggcaatttatcatgactctcaaaattcttccagcctctgcccatttccacgttgcaattccaaagccacttcaatcagtaggcgtgtgttacagcagcactctaatttgggcaccacaatctatattcgtttcccgtggctgctgtaacaaattatcacacatgtgttttcacacatgtgaaaacaacacaaatttatgatcttactgttctggaggtcagcaatctgaaatcagtttcacagggcttaaaatcaaggtattggcaggactgcattcttcttgaggccccagaggagaagaggctgtctgcattcctcggctcatggctcttcctccagcaattgcatcactctgacctctgcttccattgttacatacattttcttccgtcactctgacactcctgcctcctttacagaggcccttgtgattatactcagtttacctgaaaaatccaggatactccttccatctcaagatccttaatcacatctgcaaagtccattttgctatgtgaaggtaatatagtcacatgttaaggtttaggtgattaagacactgccattttggggggtcactgttcagcctaccagagcaggggtagagttgctttgacagtcccaaatccagttcagggggcttgtccagggcagaaggtcatgaggaggagatcaggtcactgtcctagccaggactctggctgggggctggctgaagccaagagctccaggaaacctggcgcctgctcctactgccgccaaggacagcctgttctcctggtgtggctgttgcgcagggatcaggtgcacttgagtcttcgaagtggccattgctcaacttgaatggctgcctgggtcgggcagaaggccaggtcctcatggcttcccatccctaatgaccggaatacatgggctgccaggtcagatgtgggccacatgggaagtcccagctctattctagaaaatgcatgtaccatcagcttactgatagacatttactgaacttgggtatgccagatccacagggggccccagagatgagggggataagaaggtttctgaaggcatggtacagaaggtgccagcagaggtatgggctaggggaggcagggagagcacagagcaggcatcctaaaggaggcagcatttgtgttggagcttgaagaagtggattgtttgcaccgcctgggcaaagggaaggtgtgtgttcagggcatcgagagtactgcacaaaggctgaagcccagggcagtagagaagagaatccactaagaaggagccaatgaagaaaaaaaagagaaaagaatcgaaggtggatagggaaagacatgctgtcccgcagaggttaaaggggttctcacctcaagccagcagttctcaaaccttgtcagcagtggagccctttgttctgatgacagcctactcagagcactgatggggccttgggaggggcccccagggcttttcccacagttgtcctcccccacctcttcagaactggattccataggacacaagagaacacacttaagtcatggggagccagctaagtgtttggggcaaggattgggagcagccaatagcccagggtccaggtgggggtaaaggagcaaaaaagagtattttttgcatttagggggttcggggcctatttcaataaggcagctgtatgagacccatggagaaacccactgacaactgggaaaagcatccaactgtgagacaaggcctcagtttccccaactatcagaagaggagatagaattactctcccagagtacatcaaacagggactcctacactcctgtctatgctctgggctctggctgaaggaggctgcacgggcagtgggcacatctctcaagacctcaggggcttgcacagcctggactccatcagctccatgtcctcctcccattctgcctgcaagtgctccttgacatatgctggtggtggtggggaggctgttcgagtctctggctttggcctcaggagcaagggaggggatagggcaggtgggcctggctttccctgagctagagccactggctgccctggcctgggcctcaaggcactggggccatagtgaggagaggctgaggggagatgtaggctgccaggctaccagcctgctggctccatctctagacaacagtgaggagtcaagagcccaagactgaaactcctgccttcccttctttccagactgccttgtatccctgcctgccttatgttggtcccatgcatcagatggacgcctgagggcactgggtccttcctccctgtgtctgccctccgaggaaggcaaggaaaaatgccacaatgtgccaagccaggcacatcccatgggctcctcacatgcatcctataaaataaagcattaagtcccatttctcagccttagaagccaaggctgagtgaggtgaagtcatctgcccaaggtcacatcctcgtgaggggcagattctgggattgaaatccaggctggtgtggctccaacatctgggctcaacgtccagggcccaatcaagccagtggctgcaggcttgaggccccgcctgccagtcctcttggcttggaccttttcctcagcagagtcaagctgcacatttttctgggcagaaagttgtgcccgaggccggctcctgcttgtggccccagctgccccgacagtgtcactctccaacactgcactctcttctggtgcaacatccacaagctcgccaaggcccttcctcaggaatgggcctgaggccaggagggagagaccatcagggaagccaggactggctgaggtgtaggggggcgacagactgctccgaggtcagggcagctaccctgagatgctgctgaagacagcaagagccaaagggcacaaggagaaagacagaaagggcaatactggtgaggaccttagcaggcaaaggtctgtgagcatgggggactaaggaagtggggagccttgccctggttgtgcacccccttcgccctccccacccaggttccttctggagcagcctccttaaaggaagccaggggcagctcagagtccatgcagctggggctgggcacagggcaggacactggggcactgggagctgcagtgtgacctctaccaaatgtgtcctccagccatagtgcagggcaacacttaggctgggtatgactccagcaatataggctccccaaagggagggatctaacttactgtctccacttggtcactgtcatgtgacctcaggcagtacataccttctcttgctctccatgcctggcgaatggacattcagatgccagcatgcacattccacttgactaagagtaaagaggttgccagttggcgttggccctggactcagaagagccagcttctcatagggaaaggagttgcccaaggtcccactgcaggacacagccctggaactcagctctcccagctgcagcagaggatgctgcctattggaccatactgcccatcagaccatactgccaggccctgggaagtgccagggtggcagggggcagtctagtggaatgagacagcctggtttgccatgtttcttaggacccaccctgatgtaggctcacatcaccagcactcaccaacctagagatttcctgtcgctgttgacaggaaggctggatctgcaggcctcctggtggccatgagtctgcacagaccagagctggggtggaggccacaaccctgtgcccagtatctcagcttctcactctccccagccccaaccagggacacatgggttatttgaaaccccagggggtcaactcgggagggatgttttagctaaaagctatggggataaaaaggaaacacccctcactggctcaagccttcagttaaatgaacgtggatgtgcgacccaggaactgtgcagcaaagacctccagaccctcccctccagaaagcaggcagtcatccttgagccaaaacgcagatgagcttcctgtgctcgagccaggcttggccagggaattgtgtacgcatgcacccagggcagtggaggactaatcaatccctgggagtgagctgctctatgccaggacccatggtatccaaggccaggagtgaggactcacgtgccttcctccacactgcacccccacaccactaccaagcaggggactgacggccagccctgctggggcagaaggaaacccttgccccagtgctacctgggagtaagggggtcaggggacctgcaagtcatggacaaaacattaggtcaccatttgttagtctctcaatactttactggccatatcccccgatacccccacagcaatttcaccaacacagagcaactgccctcagccactctgatgtgatggagccaatccaggtgtcctagaaatatcctagaaatgcagagcatggggaaatcacagaaccctgggaaatgccataagaacctgggctctggaaagtgccatccacctcccctctggtcaggctggcggcactgacaaggcatccacagggcagccatgctatggcccagacctccggatatgcaggaaccggggcctcccacagaagtccctgcgcacagccacaagattaaggtacaggtcaggccggctctgaagccagctgctgacaagctccgggtgccttgggtccacttctaagaagatactaccagagtctttcaggagccggggtgccaaggccagaatgtgggtaatgatgtccatgccctcctccccaccatccagggccgcggggtcttcatagctgcggatctcaggggccagctgctccatgtcctggtggaagacgtagggagggttgctgacaatcaggtccatggggccccagggcaggtgtgtccagctcctttctgaggtcatgtcgaggtggatgatccaaatcctgtcctgcaaccgaagcctctgagcattctcatgggtcagagagatagcagcttcccgcttatccacagcaatgactcggctctgggggagctggctcagcaggctgagggagatggctcctgatccgcagcccacctccagaatgagggggctgcctggggatcccacagcatgggacctctgggccacctcttccagcacccactcaaccagttcctctgtttctggccgaggaataaacactgggggcaccatccttaggctgagcccctggaagtcccactctccaaggatgtactgcaccggcatcctctgcaatcgacggctactcagctcccggatacactgtagttgctgagaggtcaagggctgggtccaaagtgccggcctcaggctctgaaatgttttggctccaaggacatgagccacgatgtactcactggattcccgggcctcagggatacccctcttctcaaagaccccagtccagtggctgaccagttctatggcactggataacccagccagaggtggttggggttgccatgagctgaaggcccagccccgggtacttcccctcctccctgggccagacaggagggcccacagcattcggccccaaagctccatgtctcagggaaaggttctccagagtgcttccaggttcccaagtctgctttatgatgtcagctgctgaggtgagtgctgagagtggcccctggacccagctgggtggagatggagaggtcacaagctctggtgccccaaaatggctctggtcctcagatatagttggttgccacccagccggagaagctgccccgaact

SEQ ID NO: 13698 - RNA, 11507 nt, Homo sapiens
  source 1..11507: mol_type = other RNA
gctgggattacaggcatgagccaccatgcccagctaatttttgtatttttagtagagacagggtttcaccatgttggccaggctggtcttgaactcctgagctcgggtgatctgcctgcttcagcctcccaaagtgctgggattacaagtgtgagccaccctgcacggcccctttctttctggcttcctcctcccttcttccttttctttcatttttaaaacatttttttaaaattattatttttaaatttttttttttgagatggagtctagctctgtcgcccaggctggagtgcagtggcatgatcttggctcactgcaatctctgcctcccgggttcaagcaattctcctgcttcagcctcccgagtagctgggattacaggtgtccaccaccacacccagctaatttttgtatttttagtagacggggtttcactgtgttggccaggctggtcttgaactcctaaccttgtgatccttggcctcccaaagtgctgggattacaaacgtgagctactgcgcctggcctattattattatttttgagacagagttttgctcttgttgcctgggtgggagtacaatggcgtgatcttggctcactgcaacatctgcctctcggtttcaagcgattctcctgcctcagcctctcaagtagctgggattacaggcgtgagccaccacacccggctaatttttgtatttttagtacagacggattttcaccatgttggccaagctggcctcgaactcctgacctcaggtgatctgcctgcctcagcctcccagagtgctgggattacaggcgtgagccaccgcgcccggcctaaaattatttttttagagacagggtctgactctgatgtccaggctggagtgcagtggcgctattatagctcactgctgtcttaaactcttgtgctcaagtaatcctcctgcctcagcctcccgagtaggtgggaccacaggcatgtgccaccatgcccagctcatatttttaattattgaaaaaaaaaaaacccaattttaaaaaccacacacagactcaaatgggcacagcaccaaattatgacacattagaatccttcctatgtgctcagagaacagggtttgtgctgagcttgagataaggcttctcttgctgtccctgtcaatcaaagagactgcaaggtgggcttcagacacagtgctagcatttgtaaacaattatctgtgagaatcagcggtcactttgtcctgtgctaccaaaatcaaacactgaaagaaaatggacattgagaccaacataagactacaactaccatcccagcccccagttcaaacatttgtgttcattgctcttcgccctgatggactgtatgctaagaaagaatttgcacttgcaaaatacatttttgctaactagatgctcattttatctttttaaaaatatgtatttcagttgcacatgaaatgtactttgaaagaatgagctccaaagttctggggggctgagacaggcgggctgagtgaaatgatgaagaaacagtggctttcagtgcgggccaagagagtagtgagcaatggtcagttattgagctgtggagtgccttcaacaagggtttttagacacatccatctggtgcctcatcccagaacctcacaggcctagggacctgaaatgctccccatgacaaggcaaacttcatatcctcacatgctgagacagactcaactttcagtctggaactgggctgggtgtctgtcagtccacgccacccatatccggagtacatcagagtctgggttcagtggcagccactttcgctgccctctcctgccccacacctagcgctctgcctggcccctttgctgtgggcgtgaaaatctggcacccgggccgacagggagagagctcagtctgcgtctgctgctttctgtttgattcatcactttccccttcaccctggagcccacgttggctgtggggcacctaactggctcctgaggcccctctggggggttgaggccctgggctgcatttggcctcggcagcctgctcacgcctctcctgactgggatgtcagaggactaggttcaaactccagcatggccagctgctggctgtgtgaccttgggcatgttaagcctcagtcccttcatccatacagtgggccaaggaagggatccctgatgtgccaacagatggatttatgaccacgtgtgtgcagcacctggcactagtttacacactgcagatgcccggtactgttgtcgccagcactcaggtctaggagagtggtcttcacaactctacctcaagggttgcctttggactgtgtccccacatggtcacatttgcatctccagacgccccaatgctgcttctcggatattctgaaggcatcctacactgtcaagctccccgactgttccccccagcaccccagtctccaactcagggtggccccatttcccccaggtcccaatcagatccctgggcccactgtggtcctggccatctcacatccaaaccctcagcaatggttgtgagtcagttctgttccagaatatctgatgccactgctacagaccccagccacctccagaccctggacaagttgcagcctcctgccccagcccctttttcctggcagccagaaagagcagcctcaatgcttctctaaccctgtaactcagctcaaaaagctctttaggcccctggtccccagaaatgcattcagagctcagccaaggggacctctcggcaccacctcacccctacatatccctacccgcatgtctgcagaactccaggcttttgtccagactgtccctactgcctggtatattcctgtcctatccgcccctcctcaagcctggtgtgatgactaaggcctccagctccaggtcactcagcctatgccagaatcacagctcagccagcctatgagcaagtttcttagccccagtttgtttcttcgtcagtataacgagagggttcacagcctccatctctgaggatgtcatgaaggttgagtaagataatcctggaagtacttggcgcaggatgcaccatattctataggaccctccacttggtatcatctccctggtgcctgacacaaagtaggtcttgagagactgaggccctggccctatacctcaggagatgcacccaggagcagctgcaggtcttctagaaagccctctagggacagccctggaaacccttgctcctgctccaagggtccacaagcccaggtaacttctgcgctaagctctgcaggggacagcccaggacctagttatgctggcctcagcgtctctgatagtcaaatggacaccaatggcagcctcatcctcccttcctgtccagctatgcaacctgacctgcaactgcaccctgctgagccttggtgtcctcaactttgtaatgtggggacaactaaaaaccccatgtgccagccctggcaacatagcaagaccccgtttctaaaaaaaaaaaaaaattaaaaattagccaggcagggttgttcacacctgtagtcctagtttgctttgcttggtcacgtagctcagcctcacactgacttccaggaacagcagagggacttggacgcctctccaggcaggcaggcctgttcctggaaagccaggtggggtggggggtcttcaggtggcaaaggaaggactggcagctgtgagccagagaagagacctggctcgtgccccagccctgctcctgtcctgctaagcctcagtttcctcatctgtaccacagggatctctgtgagcgcttcaggcaccaacaatctgctccctgggctcagtaggggatatctgatcccaccatttccccagccacatgccccagaagagggccgcagacctagtacaagagggagcaataaggtgacatcctctgctctgagaggtagagtgtttggggaagaccccagcccctgggaagggggccacttagccaggcctgcctgccacggggcatggctactctaagctgtctcaccctccccctttaggcatagctggggcaggtggaggtcagcccagttcagggctttccatgaagctgaggtaggcttccctgcctttcccactttgtgagctgtaaaattagcctttcctgaccattttcctgcaggactgctgtatgtgtgagaggtagtctttggaagaaaaggggcctctagaatttgaagcttctgatttctggttatgaggccaaagatcccaaaggtccttccagacacctcaggagggccctggggggcagaggctgggggctgtacagccaattacctcagaggggaaggcacccactcattccgcaagcgggggaaatcctgctctcctcccacagctaccagagcttcagatgggactcagatctgtctgcacacccagggctacagttggcctaatgtgactcttacctgcccataaacctggcccagagggctttatgggccagaatccctgggtttagtagctacatggacagccatatgagcaccacctaattgacttaattaactaaccccaggcctttggaagcaataggagatgagagcatcatactgggagtcaggagtcaagtgctgtgttacttcaagtaagccccatccctctctgggaaaaaagatcagggattgaatataagtcttgccatgatccaccccttccagtataaacaggccctcctggcttcatccaaagcgtatccaggtgatttggggccaagctgacccttgaacccaggtgtccatgctctctgtcccccagcttctcagctctgaaacccagcatgaggcccatgtctggcctcccagtagctctccatgtggctcctgggttaggactggcttcaggagccccaagccttggctgggtgggatggtgtctccagagtcctttagtacccctggaaagggaggtcctagtcccagcttggacagggacagggctgagggcaccagttggccaattcagttttaggaaccaggaggttgagaaccccagggatagccccactccaccataggaacagaatggtgacacagctctgctcaggcctatggcttacatggaggggccaggcccattagctcaaagtcaggggctgctgtgctcatttcacagatgcagtacctgcaacccagagagtacagggcccctgctcatcctcacacacccaaggggtcctgggccagtcacataactccacaggagagcaggaacaggcttggtcccagtctctgaggtcctctctggacccagtctctggagatgggccatggaggccagccttgcactttctccccacatcccagtcccattcctcacccactcccttctgggacccatgctggtcagtctttcagtcttctcactctgggaaagggccacctctctccaaatatgagtaaaaaaagggggggcctgggcagtttaggtctgaaggttgaggaagagttcccctggccacatcacctatcagaagagaggtggttaaggcaatttatcatgactctcaaaattcttccagcctctgcccatttccacgttgcaattccaaagccacttcaatcagtaggcgtgtgttacagcagcactctaatttgggcaccacaatctatattcgtttcccgtggctgctgtaacaaattatcacacatgtgttttcacacatgtgaaaacaacacaaatttatgatcttactgttctggaggtcagcaatctgaaatcagtttcacagggcttaaaatcaaggtattggcaggactgcattcttcttgaggccccagaggagaagaggctgtctgcattcctcggctcatggctcttcctccagcaattgcatcactctgacctctgcttccattgttacatacattttcttccgtcactctgacactcctgcctcctttacagaggcccttgtgattatactcagtttacctgaaaaatccaggatactccttccatctcaagatccttaatcacatctgcaaagtccattttgctatgtgaaggtaatatagtcacatgttaaggtttaggtgattaagacactgccattttggggggtcactgttcagcctaccagagcaggggtagagttgctttgacagtcccaaatccagttcagggggcttgtccagggcagaaggtcatgaggaggagatcaggtcactgtcctagccaggactctggctgggggctggctgaagccaagagctccaggaaacctggcgcctgctcctactgccgccaaggacagcctgttctcctggtgtggctgttgcgcagggatcaggtgcacttgagtcttcgaagtggccattgctcaacttgaatggctgcctgggtcgggcagaaggccaggtcctcatggcttcccatccctaatgaccggaatacatgggctgccaggtcagatgtgggccacatgggaagtcccagctctattctagaaaatgcatgtaccatcagcttactgatagacatttactgaacttgggtatgccagatccacagggggccccagagatgagggggataagaaggtttctgaaggcatggtacagaaggtgccagcagaggtatgggctaggggaggcagggagagcacagagcaggcatcctaaaggaggcagcatttgtgttggagcttgaagaagtggattgtttgcaccgcctgggcaaagggaaggtgtgtgttcagggcatcgagagtactgcacaaaggctgaagcccagggcagtagagaagagaatccactaagaaggagccaatgaagaaaaaaaagagaaaagaatcgaaggtggatagggaaagacatgctgtcccgcagaggttaaaggggttctcacctcaagccagcagttctcaaaccttgtcagcagtggagccctttgttctgatgacagcctactcagagcactgatggggccttgggaggggcccccagggcttttcccacagttgtcctcccccacctcttcagaactggattccataggacacaagagaacacacttaagtcatggggagccagctaagtgtttggggcaaggattgggagcagccaatagcccagggtccaggtgggggtaaaggagcaaaaaagagtattttttgcatttagggggttcggggcctatttcaataaggcagctgtatgagacccatggagaaacccactgacaactgggaaaagcatccaactgtgagacaaggcctcagtttccccaactatcagaagaggagatagaattactctcccagagtacatcaaacagggactcctacactcctgtctatgctctgggctctggctgaaggaggctgcacgggcagtgggcacatctctcaagacctcaggggcttgcacagcctggactccatcagctccatgtcctcctcccattctgcctgcaagtgctccttgacatatgctggtggtggtggggaggctgttcgagtctctggctttggcctcaggagcaagggaggggatagggcaggtgggcctggctttccctgagctagagccactggctgccctggcctgggcctcaaggcactggggccatagtgaggagaggctgaggggagatgtaggctgccaggctaccagcctgctggctccatctctagacaacagtgaggagtcaagagcccaagactgaaactcctgccttcccttctttccagactgccttgtatccctgcctgccttatgttggtcccatgcatcagatggacgcctgagggcactgggtccttcctccctgtgtctgccctccgaggaaggcaaggaaaaatgccacaatgtgccaagccaggcacatcccatgggctcctcacatgcatcctataaaataaagcattaagtcccatttctcagccttagaagccaaggctgagtgaggtgaagtcatctgcccaaggtcacatcctcgtgaggggcagattctgggattgaaatccaggctggtgtggctccaacatctgggctcaacgtccagggcccaatcaagccagtggctgcaggcttgaggccccgcctgccagtcctcttggcttggaccttttcctcagcagagtcaagctgcacatttttctgggcagaaagttgtgcccgaggccggctcctgcttgtggccccagctgccccgacagtgtcactctccaacactgcactctcttctggtgcaacatccacaagctcgccaaggcccttcctcaggaatgggcctgaggccaggagggagagaccatcagggaagccaggactggctgaggtgtaggggggcgacagactgctccgaggtcagggcagctaccctgagatgctgctgaagacagcaagagccaaagggcacaaggagaaagacagaaagggcaatactggtgaggaccttagcaggcaaaggtctgtgagcatgggggactaaggaagtggggagccttgccctggttgtgcacccccttcgccctccccacccaggttccttctggagcagcctccttaaaggaagccaggggcagctcagagtccatgcagctggggctgggcacagggcaggacactggggcactgggagctgcagtgtgacctctaccaaatgtgtcctccagccatagtgcagggcaacacttaggctgggtatgactccagcaatataggctccccaaagggagggatctaacttactgtctccacttggtcactgtcatgtgacctcaggcagtacataccttctcttgctctccatgcctggcgaatggacattcagatgccagcatgcacattccacttgactaagagtaaagaggttgccagttggcgttggccctggactcagaagagccagcttctcatagggaaaggagttgcccaaggtcccactgcaggacacagccctggaactcagctctcccagctgcagcagaggatgctgcctattggaccatactgcccatcagaccatactgccaggccctgggaagtgccagggtggcagggggcagtctagtggaatgagacagcctggtttgccatgtttcttaggacccaccctgatgtaggctcacatcaccagcactcaccaacctagagatttcctgtcgctgttgacaggaaggctggatctgcaggcctcctggtggccatgagtctgcacagaccagagctggggtggaggccacaaccctgtgcccagtatctcagcttctcactctccccagccccaaccagggacacatgggttatttgaaaccccagggggtcaactcgggagggatgttttagctaaaagctatggggataaaaaggaaacacccctcactggctcaagccttcagttaaatgaacgtggatgtgcgacccaggaactgtgcagcaaagacctccagaccctcccctccagaaagcaggcagtcatccttgagccaaaacgcagatgagcttcctgtgctcgagccaggcttggccagggaattgtgtacgcatgcacccagggcagtggaggactaatcaatccctgggagtgagctgctctatgccaggacccatggtatccaaggccaggagtgaggactcacgtgccttcctccacactgcacccccacaccactaccaagcaggggactgacggccagccctgctggggcagaaggaaacccttgccccagtgctacctgggagtaagggggtcaggggacctgcaagtcatggacaaaacattaggtcaccatttgttagtctctcaatactttactggccatatcccccgatacccccacagcaatttcaccaacacagagcaactgccctcagccactctgatgtgatggagccaatccaggtgtcctagaaatatcctagaaatgcagagcatggggaaatcacagaaccctgggaaatgccataagaacctgggctctggaaagtgccatccacctcccctctggtcaggctggcggcactgacaaggcatccacagggcagccatgctatggcccagacctccggatatgcaggaaccggggcctcccacagaagtccctgcgcacagccacaagattaaggtacaggtcaggccggctctgaagccagctgctgacaagctccgggtgccttgggtccacttctaagaagatactaccagagtctttcaggagccggggtgccaaggccagaatgtgggtaatgatgtccatgccctcctccccaccatccagggccgcggggtcttcatagctgcggatctcaggggccagctgctccatgtcctggtggaagacgtagggagggttgctgacaatcaggtccatggggccccagggcaggtgtgtccagctcctttctgaggtcatgtcgaggtggatgatccaaatcctgtcctgcaaccgaagcctctgagcattctcatgggtcagagagatagcagcttcccgcttatccacagcaatgactcggctctgggggagctggctcagcaggctgagggagatggctcctgatccgcagcccacctccagaatgagggggctgcctggggatcccacagcatgggacctctgggccacctcttccagcacccactcaaccagttcctctgtttctggccgaggaataaacactgggggcaccatccttaggctgagcccctggaagtcccactctccaaggatgtactgcaccggcatcctctgcaatcgacggctactcagctcccggatacactgtagttgctgagaggtcaagggctgggtccaaagtgccggcctcaggctctgaaatgttttggctccaaggacatgagccacgatgtactcactggattcccgggcctcagggatacccctcttctcaaagaccccagtccagtggctgaccagttctatggcactggataacccagccagaggtggttggggttgccatgagctgaaggcccagccccgggtacttcccctcctccctgggccagacaggagggcccacagcattcggccccaaagctccatgtctcagggaaaggttctccagagtgcttccaggttcccaagtctgctttatgatgtcagctgctgaggtgagtgctgagagtggcccctggacccagctgggtggagatggagaggtcacaagctctggtgccccaaaatggctctggtcctcagatatagttggttgccaccccgagtccaccagactccagaagcggctcttgcaccagtgcgccgtcccaggagccaaggcccgaagtcagaagtgtaaactccctcacagctacgcaccgcattgttaacgacccagatgaggccccctctctccaaccctgtttccccatctgcactatggagaatggtaccggccaggtctccaggcggttgcagtcgaaacaccccgttccgatccccacctcccatgcatacctgcctgaaaggctgccccacccacccaccagccggagaagctgccccgaact

SEQ ID NO: 13699 - RNA, 11408 nt, Homo sapiens
  source 1..11408: mol_type = other RNA
gctgggattacaggcatgagccaccatgcccagctaatttttgtatttttagtagagacagggtttcaccatgttggccaggctggtcttgaactcctgagctcgggtgatctgcctgcttcagcctcccaaagtgctgggattacaagtgtgagccaccctgcacggcccctttctttctggcttcctcctcccttcttccttttctttcatttttaaaacatttttttaaaattattatttttaaatttttttttttgagatggagtctagctctgtcgcccaggctggagtgcagtggcatgatcttggctcactgcaatctctgcctcccgggttcaagcaattctcctgcttcagcctcccgagtagctgggattacaggtgtccaccaccacacccagctaatttttgtatttttagtagacggggtttcactgtgttggccaggctggtcttgaactcctaaccttgtgatccttggcctcccaaagtgctgggattacaaacgtgagctactgcgcctggcctattattattatttttgagacagagttttgctcttgttgcctgggtgggagtacaatggcgtgatcttggctcactgcaacatctgcctctcggtttcaagcgattctcctgcctcagcctctcaagtagctgggattacaggcgtgagccaccacacccggctaatttttgtatttttagtacagacggattttcaccatgttggccaagctggcctcgaactcctgacctcaggtgatctgcctgcctcagcctcccagagtgctgggattacaggcgtgagccaccgcgcccggcctaaaattatttttttagagacagggtctgactctgatgtccaggctggagtgcagtggcgctattatagctcactgctgtcttaaactcttgtgctcaagtaatcctcctgcctcagcctcccgagtaggtgggaccacaggcatgtgccaccatgcccagctcatatttttaattattgaaaaaaaaaaaacccaattttaaaaaccacacacagactcaaatgggcacagcaccaaattatgacacattagaatccttcctatgtgctcagagaacagggtttgtgctgagcttgagataaggcttctcttgctgtccctgtcaatcaaagagactgcaaggtgggcttcagacacagtgctagcatttgtaaacaattatctgtgagaatcagcggtcactttgtcctgtgctaccaaaatcaaacactgaaagaaaatggacattgagaccaacataagactacaactaccatcccagcccccagttcaaacatttgtgttcattgctcttcgccctgatggactgtatgctaagaaagaatttgcacttgcaaaatacatttttgctaactagatgctcattttatctttttaaaaatatgtatttcagttgcacatgaaatgtactttgaaagaatgagctccaaagttctggggggctgagacaggcgggctgagtgaaatgatgaagaaacagtggctttcagtgcgggccaagagagtagtgagcaatggtcagttattgagctgtggagtgccttcaacaagggtttttagacacatccatctggtgcctcatcccagaacctcacaggcctagggacctgaaatgctccccatgacaaggcaaacttcatatcctcacatgctgagacagactcaactttcagtctggaactgggctgggtgtctgtcagtccacgccacccatatccggagtacatcagagtctgggttcagtggcagccactttcgctgccctctcctgccccacacctagcgctctgcctggcccctttgctgtgggcgtgaaaatctggcacccgggccgacagggagagagctcagtctgcgtctgctgctttctgtttgattcatcactttccccttcaccctggagcccacgttggctgtggggcacctaactggctcctgaggcccctctggggggttgaggccctgggctgcatttggcctcggcagcctgctcacgcctctcctgactgggatgtcagaggactaggttcaaactccagcatggccagctgctggctgtgtgaccttgggcatgttaagcctcagtcccttcatccatacagtgggccaaggaagggatccctgatgtgccaacagatggatttatgaccacgtgtgtgcagcacctggcactagtttacacactgcagatgcccggtactgttgtcgccagcactcaggtctaggagagtggtcttcacaactctacctcaagggttgcctttggactgtgtccccacatggtcacatttgcatctccagacgccccaatgctgcttctcggatattctgaaggcatcctacactgtcaagctccccgactgttccccccagcaccccagtctccaactcagggtggccccatttcccccaggtcccaatcagatccctgggcccactgtggtcctggccatctcacatccaaaccctcagcaatggttgtgagtcagttctgttccagaatatctgatgccactgctacagaccccagccacctccagaccctggacaagttgcagcctcctgccccagcccctttttcctggcagccagaaagagcagcctcaatgcttctctaaccctgtaactcagctcaaaaagctctttaggcccctggtccccagaaatgcattcagagctcagccaaggggacctctcggcaccacctcacccctacatatccctacccgcatgtctgcagaactccaggcttttgtccagactgtccctactgcctggtatattcctgtcctatccgcccctcctcaagcctggtgtgatgactaaggcctccagctccaggtcactcagcctatgccagaatcacagctcagccagcctatgagcaagtttcttagccccagtttgtttcttcgtcagtataacgagagggttcacagcctccatctctgaggatgtcatgaaggttgagtaagataatcctggaagtacttggcgcaggatgcaccatattctataggaccctccacttggtatcatctccctggtgcctgacacaaagtaggtcttgagagactgaggccctggccctatacctcaggagatgcacccaggagcagctgcaggtcttctagaaagccctctagggacagccctggaaacccttgctcctgctccaagggtccacaagcccaggtaacttctgcgctaagctctgcaggggacagcccaggacctagttatgctggcctcagcgtctctgatagtcaaatggacaccaatggcagcctcatcctcccttcctgtccagctatgcaacctgacctgcaactgcaccctgctgagccttggtgtcctcaactttgtaatgtggggacaactaaaaaccccatgtgccagccctggcaacatagcaagaccccgtttctaaaaaaaaaaaaaaattaaaaattagccaggcagggttgttcacacctgtagtcctagtttgctttgcttggtcacgtagctcagcctcacactgacttccaggaacagcagagggacttggacgcctctccaggcaggcaggcctgttcctggaaagccaggtggggtggggggtcttcaggtggcaaaggaaggactggcagctgtgagccagagaagagacctggctcgtgccccagccctgctcctgtcctgctaagcctcagtttcctcatctgtaccacagggatctctgtgagcgcttcaggcaccaacaatctgctccctgggctcagtaggggatatctgatcccaccatttccccagccacatgccccagaagagggccgcagacctagtacaagagggagcaataaggtgacatcctctgctctgagaggtagagtgtttggggaagaccccagcccctgggaagggggccacttagccaggcctgcctgccacggggcatggctactctaagctgtctcaccctccccctttaggcatagctggggcaggtggaggtcagcccagttcagggctttccatgaagctgaggtaggcttccctgcctttcccactttgtgagctgtaaaattagcctttcctgaccattttcctgcaggactgctgtatgtgtgagaggtagtctttggaagaaaaggggcctctagaatttgaagcttctgatttctggttatgaggccaaagatcccaaaggtccttccagacacctcaggagggccctggggggcagaggctgggggctgtacagccaattacctcagaggggaaggcacccactcattccgcaagcgggggaaatcctgctctcctcccacagctaccagagcttcagatgggactcagatctgtctgcacacccagggctacagttggcctaatgtgactcttacctgcccataaacctggcccagagggctttatgggccagaatccctgggtttagtagctacatggacagccatatgagcaccacctaattgacttaattaactaaccccaggcctttggaagcaataggagatgagagcatcatactgggagtcaggagtcaagtgctgtgttacttcaagtaagccccatccctctctgggaaaaaagatcagggattgaatataagtcttgccatgatccaccccttccagtataaacaggccctcctggcttcatccaaagcgtatccaggtgatttggggccaagctgacccttgaacccaggtgtccatgctctctgtcccccagcttctcagctctgaaacccagcatgaggcccatgtctggcctcccagtagctctccatgtggctcctgggttaggactggcttcaggagccccaagccttggctgggtgggatggtgtctccagagtcctttagtacccctggaaagggaggtcctagtcccagcttggacagggacagggctgagggcaccagttggccaattcagttttaggaaccaggaggttgagaaccccagggatagccccactccaccataggaacagaatggtgacacagctctgctcaggcctatggcttacatggaggggccaggcccattagctcaaagtcaggggctgctgtgctcatttcacagatgcagtacctgcaacccagagagtacagggcccctgctcatcctcacacacccaaggggtcctgggccagtcacataactccacaggagagcaggaacaggcttggtcccagtctctgaggtcctctctggacccagtctctggagatgggccatggaggccagccttgcactttctccccacatcccagtcccattcctcacccactcccttctgggacccatgctggtcagtctttcagtcttctcactctgggaaagggccacctctctccaaatatgagtaaaaaaagggggggcctgggcagtttaggtctgaaggttgaggaagagttcccctggccacatcacctatcagaagagaggtggttaaggcaatttatcatgactctcaaaattcttccagcctctgcccatttccacgttgcaattccaaagccacttcaatcagtaggcgtgtgttacagcagcactctaatttgggcaccacaatctatattcgtttcccgtggctgctgtaacaaattatcacacatgtgttttcacacatgtgaaaacaacacaaatttatgatcttactgttctggaggtcagcaatctgaaatcagtttcacagggcttaaaatcaaggtattggcaggactgcattcttcttgaggccccagaggagaagaggctgtctgcattcctcggctcatggctcttcctccagcaattgcatcactctgacctctgcttccattgttacatacattttcttccgtcactctgacactcctgcctcctttacagaggcccttgtgattatactcagtttacctgaaaaatccaggatactccttccatctcaagatccttaatcacatctgcaaagtccattttgctatgtgaaggtaatatagtcacatgttaaggtttaggtgattaagacactgccattttggggggtcactgttcagcctaccagagcaggggtagagttgctttgacagtcccaaatccagttcagggggcttgtccagggcagaaggtcatgaggaggagatcaggtcactgtcctagccaggactctggctgggggctggctgaagccaagagctccaggaaacctggcgcctgctcctactgccgccaaggacagcctgttctcctggtgtggctgttgcgcagggatcaggtgcacttgagtcttcgaagtggccattgctcaacttgaatggctgcctgggtcgggcagaaggccaggtcctcatggcttcccatccctaatgaccggaatacatgggctgccaggtcagatgtgggccacatgggaagtcccagctctattctagaaaatgcatgtaccatcagcttactgatagacatttactgaacttgggtatgccagatccacagggggccccagagatgagggggataagaaggtttctgaaggcatggtacagaaggtgccagcagaggtatgggctaggggaggcagggagagcacagagcaggcatcctaaaggaggcagcatttgtgttggagcttgaagaagtggattgtttgcaccgcctgggcaaagggaaggtgtgtgttcagggcatcgagagtactgcacaaaggctgaagcccagggcagtagagaagagaatccactaagaaggagccaatgaagaaaaaaaagagaaaagaatcgaaggtggatagggaaagacatgctgtcccgcagaggttaaaggggttctcacctcaagccagcagttctcaaaccttgtcagcagtggagccctttgttctgatgacagcctactcagagcactgatggggccttgggaggggcccccagggcttttcccacagttgtcctcccccacctcttcagaactggattccataggacacaagagaacacacttaagtcatggggagccagctaagtgtttggggcaaggattgggagcagccaatagcccagggtccaggtgggggtaaaggagcaaaaaagagtattttttgcatttagggggttcggggcctatttcaataaggcagctgtatgagacccatggagaaacccactgacaactgggaaaagcatccaactgtgagacaaggcctcagtttccccaactatcagaagaggagatagaattactctcccagagtacatcaaacagggactcctacactcctgtctatgctctgggctctggctgaaggaggctgcacgggcagtgggcacatctctcaagacctcaggggcttgcacagcctggactccatcagctccatgtcctcctcccattctgcctgcaagtgctccttgacatatgctggtggtggtggggaggctgttcgagtctctggctttggcctcaggagcaagggaggggatagggcaggtgggcctggctttccctgagctagagccactggctgccctggcctgggcctcaaggcactggggccatagtgaggagaggctgaggggagatgtaggctgccaggctaccagcctgctggctccatctctagacaacagtgaggagtcaagagcccaagactgaaactcctgccttcccttctttccagactgccttgtatccctgcctgccttatgttggtcccatgcatcagatggacgcctgagggcactgggtccttcctccctgtgtctgccctccgaggaaggcaaggaaaaatgccacaatgtgccaagccaggcacatcccatgggctcctcacatgcatcctataaaataaagcattaagtcccatttctcagccttagaagccaaggctgagtgaggtgaagtcatctgcccaaggtcacatcctcgtgaggggcagattctgggattgaaatccaggctggtgtggctccaacatctgggctcaacgtccagggcccaatcaagccagtggctgcaggcttgaggccccgcctgccagtcctcttggcttggaccttttcctcagcagagtcaagctgcacatttttctgggcagaaagttgtgcccgaggccggctcctgcttgtggccccagctgccccgacagtgtcactctccaacactgcactctcttctggtgcaacatccacaagctcgccaaggcccttcctcaggaatgggcctgaggccaggagggagagaccatcagggaagccaggactggctgaggtgtaggggggcgacagactgctccgaggtcagggcagctaccctgagatgctgctgaagacagcaagagccaaagggcacaaggagaaagacagaaagggcaatactggtgaggaccttagcaggcaaaggtctgtgagcatgggggactaaggaagtggggagccttgccctggttgtgcacccccttcgccctccccacccaggttccttctggagcagcctccttaaaggaagccaggggcagctcagagtccatgcagctggggctgggcacagggcaggacactggggcactgggagctgcagtgtgacctctaccaaatgtgtcctccagccatagtgcagggcaacacttaggctgggtatgactccagcaatataggctccccaaagggagggatctaacttactgtctccacttggtcactgtcatgtgacctcaggcagtacataccttctcttgctctccatgcctggcgaatggacattcagatgccagcatgcacattccacttgactaagagtaaagaggttgccagttggcgttggccctggactcagaagagccagcttctcatagggaaaggagttgcccaaggtcccactgcaggacacagccctggaactcagctctcccagctgcagcagaggatgctgcctattggaccatactgcccatcagaccatactgccaggccctgggaagtgccagggtggcagggggcagtctagtggaatgagacagcctggtttgccatgtttcttaggacccaccctgatgtaggctcacatcaccagcactcaccaacctagagatttcctgtcgctgttgacaggaaggctggatctgcaggcctcctggtggccatgagtctgcacagaccagagctggggtggaggccacaaccctgtgcccagtatctcagcttctcactctccccagccccaaccagggacacatgggttatttgaaaccccagggggtcaactcgggagggatgttttagctaaaagctatggggataaaaaggaaacacccctcactggctcaagccttcagttaaatgaacgtggatgtgcgacccaggaactgtgcagcaaagacctccagaccctcccctccagaaagcaggcagtcatccttgagccaaaacgcagatgagcttcctgtgctcgagccaggcttggccagggaattgtgtacgcatgcacccagggcagtggaggactaatcaatccctgggagtgagctgctctatgccaggacccatggtatccaaggccaggagtgaggactcacgtgccttcctccacactgcacccccacaccactaccaagcaggggactgacggccagccctgctggggcagaaggaaacccttgccccagtgctacctgggagtaagggggtcaggggacctgcaagtcatggacaaaacattaggtcaccatttgttagtctctcaatactttactggccatatcccccgatacccccacagcaatttcaccaacacagagcaactgccctcagccactctgatgtgatggagccaatccaggtgtcctagaaatatcctagaaatgcagagcatggggaaatcacagaaccctgggaaatgccataagaacctgggctctggaaagtgccatccacctcccctctggtcaggctggcggcactgacaaggcatccacagggcagccatgctatggcccagacctccggatatgcaggaaccggggcctcccacagaagtccctgcgcacagccacaagattaaggtacaggtcaggccggctctgaagccagctgctgacaagctccgggtgccttgggtccacttctaagaagatactaccagagtctttcaggagccggggtgccaaggccagaatgtgggtaatgatgtccatgccctcctccccaccatccagggccgcggggtcttcatagctgcggatctcaggggccagctgctccatgtcctggtggaagacgtagggagggttgctgacaatcaggtccatggggccccagggcaggtgtgtccagctcctttctgaggtcatgtcgaggtggatgatccaaatcctgtcctgcaaccgaagcctctgagcattctcatgggtcagagagatagcagcttcccgcttatccacagcaatgactcggctctgggggagctggctcagcaggctgagggagatggctcctgatccgcagcccacctccagaatgagggggctgcctggggatcccacagcatgggacctctgggccacctcttccagcacccactcaaccagttcctctgtttctggccgaggaataaacactgggggcaccatccttaggctgagcccctggaagtcccactctccaaggatgtactgcaccggcatcctctgcaatcgacggctactcagctcccggatacactgtagttgctgagaggtcaagggctgggtccaaagtgccggcctcaggctctgaaatgttttggctccaaggacatgagccacgatgtactcactggattcccgggcctcagggatacccctcttctcaaagaccccagtccagtggctgaccagttctatggcactggataacccagccagaggtggttggggttgccatgagctgaaggcccagccccgggtacttcccctcctccctgggccagacaggagggcccacagcattcggccccaaagctccatgtctcagggaaaggttctccagagtgcttccaggttcccaagtctgctttatgatgtcagctgctgaggtgagtgctgagagtggcccctggacccagctgggtggagatggagaggtcacaagctctggtgccccaaaatggctctggtcctcagatatagttggttgccacccgcattgttaacgacccagatgaggccccctctctccaaccctgtttccccatctgcactatggagaatggtaccggccaggtctccaggcggttgcagtcgaaacaccccgttccgatccccacctcccatgcatacctgcctgaaaggctgccccacccacccaccagccggagaagctgccccgaact

SEQ ID NO: 13700 - RNA, 11311 nt, Homo sapiens
  source 1..11311: mol_type = other RNA
gctgggattacaggcatgagccaccatgcccagctaatttttgtatttttagtagagacagggtttcaccatgttggccaggctggtcttgaactcctgagctcgggtgatctgcctgcttcagcctcccaaagtgctgggattacaagtgtgagccaccctgcacggcccctttctttctggcttcctcctcccttcttccttttctttcatttttaaaacatttttttaaaattattatttttaaatttttttttttgagatggagtctagctctgtcgcccaggctggagtgcagtggcatgatcttggctcactgcaatctctgcctcccgggttcaagcaattctcctgcttcagcctcccgagtagctgggattacaggtgtccaccaccacacccagctaatttttgtatttttagtagacggggtttcactgtgttggccaggctggtcttgaactcctaaccttgtgatccttggcctcccaaagtgctgggattacaaacgtgagctactgcgcctggcctattattattatttttgagacagagttttgctcttgttgcctgggtgggagtacaatggcgtgatcttggctcactgcaacatctgcctctcggtttcaagcgattctcctgcctcagcctctcaagtagctgggattacaggcgtgagccaccacacccggctaatttttgtatttttagtacagacggattttcaccatgttggccaagctggcctcgaactcctgacctcaggtgatctgcctgcctcagcctcccagagtgctgggattacaggcgtgagccaccgcgcccggcctaaaattatttttttagagacagggtctgactctgatgtccaggctggagtgcagtggcgctattatagctcactgctgtcttaaactcttgtgctcaagtaatcctcctgcctcagcctcccgagtaggtgggaccacaggcatgtgccaccatgcccagctcatatttttaattattgaaaaaaaaaaaacccaattttaaaaaccacacacagactcaaatgggcacagcaccaaattatgacacattagaatccttcctatgtgctcagagaacagggtttgtgctgagcttgagataaggcttctcttgctgtccctgtcaatcaaagagactgcaaggtgggcttcagacacagtgctagcatttgtaaacaattatctgtgagaatcagcggtcactttgtcctgtgctaccaaaatcaaacactgaaagaaaatggacattgagaccaacataagactacaactaccatcccagcccccagttcaaacatttgtgttcattgctcttcgccctgatggactgtatgctaagaaagaatttgcacttgcaaaatacatttttgctaactagatgctcattttatctttttaaaaatatgtatttcagttgcacatgaaatgtactttgaaagaatgagctccaaagttctggggggctgagacaggcgggctgagtgaaatgatgaagaaacagtggctttcagtgcgggccaagagagtagtgagcaatggtcagttattgagctgtggagtgccttcaacaagggtttttagacacatccatctggtgcctcatcccagaacctcacaggcctagggacctgaaatgctccccatgacaaggcaaacttcatatcctcacatgctgagacagactcaactttcagtctggaactgggctgggtgtctgtcagtccacgccacccatatccggagtacatcagagtctgggttcagtggcagccactttcgctgccctctcctgccccacacctagcgctctgcctggcccctttgctgtgggcgtgaaaatctggcacccgggccgacagggagagagctcagtctgcgtctgctgctttctgtttgattcatcactttccccttcaccctggagcccacgttggctgtggggcacctaactggctcctgaggcccctctggggggttgaggccctgggctgcatttggcctcggcagcctgctcacgcctctcctgactgggatgtcagaggactaggttcaaactccagcatggccagctgctggctgtgtgaccttgggcatgttaagcctcagtcccttcatccatacagtgggccaaggaagggatccctgatgtgccaacagatggatttatgaccacgtgtgtgcagcacctggcactagtttacacactgcagatgcccggtactgttgtcgccagcactcaggtctaggagagtggtcttcacaactctacctcaagggttgcctttggactgtgtccccacatggtcacatttgcatctccagacgccccaatgctgcttctcggatattctgaaggcatcctacactgtcaagctccccgactgttccccccagcaccccagtctccaactcagggtggccccatttcccccaggtcccaatcagatccctgggcccactgtggtcctggccatctcacatccaaaccctcagcaatggttgtgagtcagttctgttccagaatatctgatgccactgctacagaccccagccacctccagaccctggacaagttgcagcctcctgccccagcccctttttcctggcagccagaaagagcagcctcaatgcttctctaaccctgtaactcagctcaaaaagctctttaggcccctggtccccagaaatgcattcagagctcagccaaggggacctctcggcaccacctcacccctacatatccctacccgcatgtctgcagaactccaggcttttgtccagactgtccctactgcctggtatattcctgtcctatccgcccctcctcaagcctggtgtgatgactaaggcctccagctccaggtcactcagcctatgccagaatcacagctcagccagcctatgagcaagtttcttagccccagtttgtttcttcgtcagtataacgagagggttcacagcctccatctctgaggatgtcatgaaggttgagtaagataatcctggaagtacttggcgcaggatgcaccatattctataggaccctccacttggtatcatctccctggtgcctgacacaaagtaggtcttgagagactgaggccctggccctatacctcaggagatgcacccaggagcagctgcaggtcttctagaaagccctctagggacagccctggaaacccttgctcctgctccaagggtccacaagcccaggtaacttctgcgctaagctctgcaggggacagcccaggacctagttatgctggcctcagcgtctctgatagtcaaatggacaccaatggcagcctcatcctcccttcctgtccagctatgcaacctgacctgcaactgcaccctgctgagccttggtgtcctcaactttgtaatgtggggacaactaaaaaccccatgtgccagccctggcaacatagcaagaccccgtttctaaaaaaaaaaaaaaattaaaaattagccaggcagggttgttcacacctgtagtcctagtttgctttgcttggtcacgtagctcagcctcacactgacttccaggaacagcagagggacttggacgcctctccaggcaggcaggcctgttcctggaaagccaggtggggtggggggtcttcaggtggcaaaggaaggactggcagctgtgagccagagaagagacctggctcgtgccccagccctgctcctgtcctgctaagcctcagtttcctcatctgtaccacagggatctctgtgagcgcttcaggcaccaacaatctgctccctgggctcagtaggggatatctgatcccaccatttccccagccacatgccccagaagagggccgcagacctagtacaagagggagcaataaggtgacatcctctgctctgagaggtagagtgtttggggaagaccccagcccctgggaagggggccacttagccaggcctgcctgccacggggcatggctactctaagctgtctcaccctccccctttaggcatagctggggcaggtggaggtcagcccagttcagggctttccatgaagctgaggtaggcttccctgcctttcccactttgtgagctgtaaaattagcctttcctgaccattttcctgcaggactgctgtatgtgtgagaggtagtctttggaagaaaaggggcctctagaatttgaagcttctgatttctggttatgaggccaaagatcccaaaggtccttccagacacctcaggagggccctggggggcagaggctgggggctgtacagccaattacctcagaggggaaggcacccactcattccgcaagcgggggaaatcctgctctcctcccacagctaccagagcttcagatgggactcagatctgtctgcacacccagggctacagttggcctaatgtgactcttacctgcccataaacctggcccagagggctttatgggccagaatccctgggtttagtagctacatggacagccatatgagcaccacctaattgacttaattaactaaccccaggcctttggaagcaataggagatgagagcatcatactgggagtcaggagtcaagtgctgtgttacttcaagtaagccccatccctctctgggaaaaaagatcagggattgaatataagtcttgccatgatccaccccttccagtataaacaggccctcctggcttcatccaaagcgtatccaggtgatttggggccaagctgacccttgaacccaggtgtccatgctctctgtcccccagcttctcagctctgaaacccagcatgaggcccatgtctggcctcccagtagctctccatgtggctcctgggttaggactggcttcaggagccccaagccttggctgggtgggatggtgtctccagagtcctttagtacccctggaaagggaggtcctagtcccagcttggacagggacagggctgagggcaccagttggccaattcagttttaggaaccaggaggttgagaaccccagggatagccccactccaccataggaacagaatggtgacacagctctgctcaggcctatggcttacatggaggggccaggcccattagctcaaagtcaggggctgctgtgctcatttcacagatgcagtacctgcaacccagagagtacagggcccctgctcatcctcacacacccaaggggtcctgggccagtcacataactccacaggagagcaggaacaggcttggtcccagtctctgaggtcctctctggacccagtctctggagatgggccatggaggccagccttgcactttctccccacatcccagtcccattcctcacccactcccttctgggacccatgctggtcagtctttcagtcttctcactctgggaaagggccacctctctccaaatatgagtaaaaaaagggggggcctgggcagtttaggtctgaaggttgaggaagagttcccctggccacatcacctatcagaagagaggtggttaaggcaatttatcatgactctcaaaattcttccagcctctgcccatttccacgttgcaattccaaagccacttcaatcagtaggcgtgtgttacagcagcactctaatttgggcaccacaatctatattcgtttcccgtggctgctgtaacaaattatcacacatgtgttttcacacatgtgaaaacaacacaaatttatgatcttactgttctggaggtcagcaatctgaaatcagtttcacagggcttaaaatcaaggtattggcaggactgcattcttcttgaggccccagaggagaagaggctgtctgcattcctcggctcatggctcttcctccagcaattgcatcactctgacctctgcttccattgttacatacattttcttccgtcactctgacactcctgcctcctttacagaggcccttgtgattatactcagtttacctgaaaaatccaggatactccttccatctcaagatccttaatcacatctgcaaagtccattttgctatgtgaaggtaatatagtcacatgttaaggtttaggtgattaagacactgccattttggggggtcactgttcagcctaccagagcaggggtagagttgctttgacagtcccaaatccagttcagggggcttgtccagggcagaaggtcatgaggaggagatcaggtcactgtcctagccaggactctggctgggggctggctgaagccaagagctccaggaaacctggcgcctgctcctactgccgccaaggacagcctgttctcctggtgtggctgttgcgcagggatcaggtgcacttgagtcttcgaagtggccattgctcaacttgaatggctgcctgggtcgggcagaaggccaggtcctcatggcttcccatccctaatgaccggaatacatgggctgccaggtcagatgtgggccacatgggaagtcccagctctattctagaaaatgcatgtaccatcagcttactgatagacatttactgaacttgggtatgccagatccacagggggccccagagatgagggggataagaaggtttctgaaggcatggtacagaaggtgccagcagaggtatgggctaggggaggcagggagagcacagagcaggcatcctaaaggaggcagcatttgtgttggagcttgaagaagtggattgtttgcaccgcctgggcaaagggaaggtgtgtgttcagggcatcgagagtactgcacaaaggctgaagcccagggcagtagagaagagaatccactaagaaggagccaatgaagaaaaaaaagagaaaagaatcgaaggtggatagggaaagacatgctgtcccgcagaggttaaaggggttctcacctcaagccagcagttctcaaaccttgtcagcagtggagccctttgttctgatgacagcctactcagagcactgatggggccttgggaggggcccccagggcttttcccacagttgtcctcccccacctcttcagaactggattccataggacacaagagaacacacttaagtcatggggagccagctaagtgtttggggcaaggattgggagcagccaatagcccagggtccaggtgggggtaaaggagcaaaaaagagtattttttgcatttagggggttcggggcctatttcaataaggcagctgtatgagacccatggagaaacccactgacaactgggaaaagcatccaactgtgagacaaggcctcagtttccccaactatcagaagaggagatagaattactctcccagagtacatcaaacagggactcctacactcctgtctatgctctgggctctggctgaaggaggctgcacgggcagtgggcacatctctcaagacctcaggggcttgcacagcctggactccatcagctccatgtcctcctcccattctgcctgcaagtgctccttgacatatgctggtggtggtggggaggctgttcgagtctctggctttggcctcaggagcaagggaggggatagggcaggtgggcctggctttccctgagctagagccactggctgccctggcctgggcctcaaggcactggggccatagtgaggagaggctgaggggagatgtaggctgccaggctaccagcctgctggctccatctctagacaacagtgaggagtcaagagcccaagactgaaactcctgccttcccttctttccagactgccttgtatccctgcctgccttatgttggtcccatgcatcagatggacgcctgagggcactgggtccttcctccctgtgtctgccctccgaggaaggcaaggaaaaatgccacaatgtgccaagccaggcacatcccatgggctcctcacatgcatcctataaaataaagcattaagtcccatttctcagccttagaagccaaggctgagtgaggtgaagtcatctgcccaaggtcacatcctcgtgaggggcagattctgggattgaaatccaggctggtgtggctccaacatctgggctcaacgtccagggcccaatcaagccagtggctgcaggcttgaggccccgcctgccagtcctcttggcttggaccttttcctcagcagagtcaagctgcacatttttctgggcagaaagttgtgcccgaggccggctcctgcttgtggccccagctgccccgacagtgtcactctccaacactgcactctcttctggtgcaacatccacaagctcgccaaggcccttcctcaggaatgggcctgaggccaggagggagagaccatcagggaagccaggactggctgaggtgtaggggggcgacagactgctccgaggtcagggcagctaccctgagatgctgctgaagacagcaagagccaaagggcacaaggagaaagacagaaagggcaatactggtgaggaccttagcaggcaaaggtctgtgagcatgggggactaaggaagtggggagccttgccctggttgtgcacccccttcgccctccccacccaggttccttctggagcagcctccttaaaggaagccaggggcagctcagagtccatgcagctggggctgggcacagggcaggacactggggcactgggagctgcagtgtgacctctaccaaatgtgtcctccagccatagtgcagggcaacacttaggctgggtatgactccagcaatataggctccccaaagggagggatctaacttactgtctccacttggtcactgtcatgtgacctcaggcagtacataccttctcttgctctccatgcctggcgaatggacattcagatgccagcatgcacattccacttgactaagagtaaagaggttgccagttggcgttggccctggactcagaagagccagcttctcatagggaaaggagttgcccaaggtcccactgcaggacacagccctggaactcagctctcccagctgcagcagaggatgctgcctattggaccatactgcccatcagaccatactgccaggccctgggaagtgccagggtggcagggggcagtctagtggaatgagacagcctggtttgccatgtttcttaggacccaccctgatgtaggctcacatcaccagcactcaccaacctagagatttcctgtcgctgttgacaggaaggctggatctgcaggcctcctggtggccatgagtctgcacagaccagagctggggtggaggccacaaccctgtgcccagtatctcagcttctcactctccccagccccaaccagggacacatgggttatttgaaaccccagggggtcaactcgggagggatgttttagctaaaagctatggggataaaaaggaaacacccctcactggctcaagccttcagttaaatgaacgtggatgtgcgacccaggaactgtgcagcaaagacctccagaccctcccctccagaaagcaggcagtcatccttgagccaaaacgcagatgagcttcctgtgctcgagccaggcttggccagggaattgtgtacgcatgcacccagggcagtggaggactaatcaatccctgggagtgagctgctctatgccaggacccatggtatccaaggccaggagtgaggactcacgtgccttcctccacactgcacccccacaccactaccaagcaggggactgacggccagccctgctggggcagaaggaaacccttgccccagtgctacctgggagtaagggggtcaggggacctgcaagtcatggacaaaacattaggtcaccatttgttagtctctcaatactttactggccatatcccccgatacccccacagcaatttcaccaacacagagcaactgccctcagccactctgatgtgatggagccaatccaggtgtcctagaaatatcctagaaatgcagagcatggggaaatcacagaaccctgggaaatgccataagaacctgggctctggaaagtgccatccacctcccctctggtcaggctggcggcactgacaaggcatccacagggcagccatgctatggcccagacctccggatatgcaggaaccggggcctcccacagaagtccctgcgcacagccacaagattaaggtacaggtcaggccggctctgaagccagctgctgacaagctccgggtgccttgggtccacttctaagaagatactaccagagtctttcaggagccggggtgccaaggccagaatgtgggtaatgatgtccatgccctcctccccaccatccagggccgcggggtcttcatagctgcggatctcaggggccagctgctccatgtcctggtggaagacgtagggagggttgctgacaatcaggtccatggggccccagggcaggtgtgtccagctcctttctgaggtcatgtcgaggtggatgatccaaatcctgtcctgcaaccgaagcctctgagcattctcatgggtcagagagatagcagcttcccgcttatccacagcaatgactcggctctgggggagctggctcagcaggctgagggagatggctcctgatccgcagcccacctccagaatgagggggctgcctggggatcccacagcatgggacctctgggccacctcttccagcacccactcaaccagttcctctgtttctggccgaggaataaacactgggggcaccatccttaggctgagcccctggaagtcccactctccaaggatgtactgcaccggcatcctctgcaatcgacggctactcagctcccggatacactgtagttgctgagaggtcaagggctgggtccaaagtgccggcctcaggctctgaaatgttttggctccaaggacatgagccacgatgtactcactggattcccgggcctcagggatacccctcttctcaaagaccccagtccagtggctgaccagttctatggcactggataacccagccagaggtggttggggttgccatgagctgaaggcccagccccgggtacttcccctcctccctgggccagacaggagggcccacagcattcggccccaaagctccatgtctcagggaaaggttctccagagtgcttccaggttcccaagtctgctttatgatgtcagctgctgaggtgagtgctgagagtggcccctggacccagctgggtggagatggagaggtcacaagctctggtgccccaaaatggctctggtcctcagatatagttggttgccaccctgccggtcttccttaaaatcacagcagggatttggctccagcccaaggggattgctccgagctggcgtttaggaaccaggccgggaggtgtgt

SEQ ID NO: 13701 - RNA, 11270 nt, Homo sapiens
  source 1..11270: mol_type = other RNA
gctgggattacaggcatgagccaccatgcccagctaatttttgtatttttagtagagacagggtttcaccatgttggccaggctggtcttgaactcctgagctcgggtgatctgcctgcttcagcctcccaaagtgctgggattacaagtgtgagccaccctgcacggcccctttctttctggcttcctcctcccttcttccttttctttcatttttaaaacatttttttaaaattattatttttaaatttttttttttgagatggagtctagctctgtcgcccaggctggagtgcagtggcatgatcttggctcactgcaatctctgcctcccgggttcaagcaattctcctgcttcagcctcccgagtagctgggattacaggtgtccaccaccacacccagctaatttttgtatttttagtagacggggtttcactgtgttggccaggctggtcttgaactcctaaccttgtgatccttggcctcccaaagtgctgggattacaaacgtgagctactgcgcctggcctattattattatttttgagacagagttttgctcttgttgcctgggtgggagtacaatggcgtgatcttggctcactgcaacatctgcctctcggtttcaagcgattctcctgcctcagcctctcaagtagctgggattacaggcgtgagccaccacacccggctaatttttgtatttttagtacagacggattttcaccatgttggccaagctggcctcgaactcctgacctcaggtgatctgcctgcctcagcctcccagagtgctgggattacaggcgtgagccaccgcgcccggcctaaaattatttttttagagacagggtctgactctgatgtccaggctggagtgcagtggcgctattatagctcactgctgtcttaaactcttgtgctcaagtaatcctcctgcctcagcctcccgagtaggtgggaccacaggcatgtgccaccatgcccagctcatatttttaattattgaaaaaaaaaaaacccaattttaaaaaccacacacagactcaaatgggcacagcaccaaattatgacacattagaatccttcctatgtgctcagagaacagggtttgtgctgagcttgagataaggcttctcttgctgtccctgtcaatcaaagagactgcaaggtgggcttcagacacagtgctagcatttgtaaacaattatctgtgagaatcagcggtcactttgtcctgtgctaccaaaatcaaacactgaaagaaaatggacattgagaccaacataagactacaactaccatcccagcccccagttcaaacatttgtgttcattgctcttcgccctgatggactgtatgctaagaaagaatttgcacttgcaaaatacatttttgctaactagatgctcattttatctttttaaaaatatgtatttcagttgcacatgaaatgtactttgaaagaatgagctccaaagttctggggggctgagacaggcgggctgagtgaaatgatgaagaaacagtggctttcagtgcgggccaagagagtagtgagcaatggtcagttattgagctgtggagtgccttcaacaagggtttttagacacatccatctggtgcctcatcccagaacctcacaggcctagggacctgaaatgctccccatgacaaggcaaacttcatatcctcacatgctgagacagactcaactttcagtctggaactgggctgggtgtctgtcagtccacgccacccatatccggagtacatcagagtctgggttcagtggcagccactttcgctgccctctcctgccccacacctagcgctctgcctggcccctttgctgtgggcgtgaaaatctggcacccgggccgacagggagagagctcagtctgcgtctgctgctttctgtttgattcatcactttccccttcaccctggagcccacgttggctgtggggcacctaactggctcctgaggcccctctggggggttgaggccctgggctgcatttggcctcggcagcctgctcacgcctctcctgactgggatgtcagaggactaggttcaaactccagcatggccagctgctggctgtgtgaccttgggcatgttaagcctcagtcccttcatccatacagtgggccaaggaagggatccctgatgtgccaacagatggatttatgaccacgtgtgtgcagcacctggcactagtttacacactgcagatgcccggtactgttgtcgccagcactcaggtctaggagagtggtcttcacaactctacctcaagggttgcctttggactgtgtccccacatggtcacatttgcatctccagacgccccaatgctgcttctcggatattctgaaggcatcctacactgtcaagctccccgactgttccccccagcaccccagtctccaactcagggtggccccatttcccccaggtcccaatcagatccctgggcccactgtggtcctggccatctcacatccaaaccctcagcaatggttgtgagtcagttctgttccagaatatctgatgccactgctacagaccccagccacctccagaccctggacaagttgcagcctcctgccccagcccctttttcctggcagccagaaagagcagcctcaatgcttctctaaccctgtaactcagctcaaaaagctctttaggcccctggtccccagaaatgcattcagagctcagccaaggggacctctcggcaccacctcacccctacatatccctacccgcatgtctgcagaactccaggcttttgtccagactgtccctactgcctggtatattcctgtcctatccgcccctcctcaagcctggtgtgatgactaaggcctccagctccaggtcactcagcctatgccagaatcacagctcagccagcctatgagcaagtttcttagccccagtttgtttcttcgtcagtataacgagagggttcacagcctccatctctgaggatgtcatgaaggttgagtaagataatcctggaagtacttggcgcaggatgcaccatattctataggaccctccacttggtatcatctccctggtgcctgacacaaagtaggtcttgagagactgaggccctggccctatacctcaggagatgcacccaggagcagctgcaggtcttctagaaagccctctagggacagccctggaaacccttgctcctgctccaagggtccacaagcccaggtaacttctgcgctaagctctgcaggggacagcccaggacctagttatgctggcctcagcgtctctgatagtcaaatggacaccaatggcagcctcatcctcccttcctgtccagctatgcaacctgacctgcaactgcaccctgctgagccttggtgtcctcaactttgtaatgtggggacaactaaaaaccccatgtgccagccctggcaacatagcaagaccccgtttctaaaaaaaaaaaaaaattaaaaattagccaggcagggttgttcacacctgtagtcctagtttgctttgcttggtcacgtagctcagcctcacactgacttccaggaacagcagagggacttggacgcctctccaggcaggcaggcctgttcctggaaagccaggtggggtggggggtcttcaggtggcaaaggaaggactggcagctgtgagccagagaagagacctggctcgtgccccagccctgctcctgtcctgctaagcctcagtttcctcatctgtaccacagggatctctgtgagcgcttcaggcaccaacaatctgctccctgggctcagtaggggatatctgatcccaccatttccccagccacatgccccagaagagggccgcagacctagtacaagagggagcaataaggtgacatcctctgctctgagaggtagagtgtttggggaagaccccagcccctgggaagggggccacttagccaggcctgcctgccacggggcatggctactctaagctgtctcaccctccccctttaggcatagctggggcaggtggaggtcagcccagttcagggctttccatgaagctgaggtaggcttccctgcctttcccactttgtgagctgtaaaattagcctttcctgaccattttcctgcaggactgctgtatgtgtgagaggtagtctttggaagaaaaggggcctctagaatttgaagcttctgatttctggttatgaggccaaagatcccaaaggtccttccagacacctcaggagggccctggggggcagaggctgggggctgtacagccaattacctcagaggggaaggcacccactcattccgcaagcgggggaaatcctgctctcctcccacagctaccagagcttcagatgggactcagatctgtctgcacacccagggctacagttggcctaatgtgactcttacctgcccataaacctggcccagagggctttatgggccagaatccctgggtttagtagctacatggacagccatatgagcaccacctaattgacttaattaactaaccccaggcctttggaagcaataggagatgagagcatcatactgggagtcaggagtcaagtgctgtgttacttcaagtaagccccatccctctctgggaaaaaagatcagggattgaatataagtcttgccatgatccaccccttccagtataaacaggccctcctggcttcatccaaagcgtatccaggtgatttggggccaagctgacccttgaacccaggtgtccatgctctctgtcccccagcttctcagctctgaaacccagcatgaggcccatgtctggcctcccagtagctctccatgtggctcctgggttaggactggcttcaggagccccaagccttggctgggtgggatggtgtctccagagtcctttagtacccctggaaagggaggtcctagtcccagcttggacagggacagggctgagggcaccagttggccaattcagttttaggaaccaggaggttgagaaccccagggatagccccactccaccataggaacagaatggtgacacagctctgctcaggcctatggcttacatggaggggccaggcccattagctcaaagtcaggggctgctgtgctcatttcacagatgcagtacctgcaacccagagagtacagggcccctgctcatcctcacacacccaaggggtcctgggccagtcacataactccacaggagagcaggaacaggcttggtcccagtctctgaggtcctctctggacccagtctctggagatgggccatggaggccagccttgcactttctccccacatcccagtcccattcctcacccactcccttctgggacccatgctggtcagtctttcagtcttctcactctgggaaagggccacctctctccaaatatgagtaaaaaaagggggggcctgggcagtttaggtctgaaggttgaggaagagttcccctggccacatcacctatcagaagagaggtggttaaggcaatttatcatgactctcaaaattcttccagcctctgcccatttccacgttgcaattccaaagccacttcaatcagtaggcgtgtgttacagcagcactctaatttgggcaccacaatctatattcgtttcccgtggctgctgtaacaaattatcacacatgtgttttcacacatgtgaaaacaacacaaatttatgatcttactgttctggaggtcagcaatctgaaatcagtttcacagggcttaaaatcaaggtattggcaggactgcattcttcttgaggccccagaggagaagaggctgtctgcattcctcggctcatggctcttcctccagcaattgcatcactctgacctctgcttccattgttacatacattttcttccgtcactctgacactcctgcctcctttacagaggcccttgtgattatactcagtttacctgaaaaatccaggatactccttccatctcaagatccttaatcacatctgcaaagtccattttgctatgtgaaggtaatatagtcacatgttaaggtttaggtgattaagacactgccattttggggggtcactgttcagcctaccagagcaggggtagagttgctttgacagtcccaaatccagttcagggggcttgtccagggcagaaggtcatgaggaggagatcaggtcactgtcctagccaggactctggctgggggctggctgaagccaagagctccaggaaacctggcgcctgctcctactgccgccaaggacagcctgttctcctggtgtggctgttgcgcagggatcaggtgcacttgagtcttcgaagtggccattgctcaacttgaatggctgcctgggtcgggcagaaggccaggtcctcatggcttcccatccctaatgaccggaatacatgggctgccaggtcagatgtgggccacatgggaagtcccagctctattctagaaaatgcatgtaccatcagcttactgatagacatttactgaacttgggtatgccagatccacagggggccccagagatgagggggataagaaggtttctgaaggcatggtacagaaggtgccagcagaggtatgggctaggggaggcagggagagcacagagcaggcatcctaaaggaggcagcatttgtgttggagcttgaagaagtggattgtttgcaccgcctgggcaaagggaaggtgtgtgttcagggcatcgagagtactgcacaaaggctgaagcccagggcagtagagaagagaatccactaagaaggagccaatgaagaaaaaaaagagaaaagaatcgaaggtggatagggaaagacatgctgtcccgcagaggttaaaggggttctcacctcaagccagcagttctcaaaccttgtcagcagtggagccctttgttctgatgacagcctactcagagcactgatggggccttgggaggggcccccagggcttttcccacagttgtcctcccccacctcttcagaactggattccataggacacaagagaacacacttaagtcatggggagccagctaagtgtttggggcaaggattgggagcagccaatagcccagggtccaggtgggggtaaaggagcaaaaaagagtattttttgcatttagggggttcggggcctatttcaataaggcagctgtatgagacccatggagaaacccactgacaactgggaaaagcatccaactgtgagacaaggcctcagtttccccaactatcagaagaggagatagaattactctcccagagtacatcaaacagggactcctacactcctgtctatgctctgggctctggctgaaggaggctgcacgggcagtgggcacatctctcaagacctcaggggcttgcacagcctggactccatcagctccatgtcctcctcccattctgcctgcaagtgctccttgacatatgctggtggtggtggggaggctgttcgagtctctggctttggcctcaggagcaagggaggggatagggcaggtgggcctggctttccctgagctagagccactggctgccctggcctgggcctcaaggcactggggccatagtgaggagaggctgaggggagatgtaggctgccaggctaccagcctgctggctccatctctagacaacagtgaggagtcaagagcccaagactgaaactcctgccttcccttctttccagactgccttgtatccctgcctgccttatgttggtcccatgcatcagatggacgcctgagggcactgggtccttcctccctgtgtctgccctccgaggaaggcaaggaaaaatgccacaatgtgccaagccaggcacatcccatgggctcctcacatgcatcctataaaataaagcattaagtcccatttctcagccttagaagccaaggctgagtgaggtgaagtcatctgcccaaggtcacatcctcgtgaggggcagattctgggattgaaatccaggctggtgtggctccaacatctgggctcaacgtccagggcccaatcaagccagtggctgcaggcttgaggccccgcctgccagtcctcttggcttggaccttttcctcagcagagtcaagctgcacatttttctgggcagaaagttgtgcccgaggccggctcctgcttgtggccccagctgccccgacagtgtcactctccaacactgcactctcttctggtgcaacatccacaagctcgccaaggcccttcctcaggaatgggcctgaggccaggagggagagaccatcagggaagccaggactggctgaggtgtaggggggcgacagactgctccgaggtcagggcagctaccctgagatgctgctgaagacagcaagagccaaagggcacaaggagaaagacagaaagggcaatactggtgaggaccttagcaggcaaaggtctgtgagcatgggggactaaggaagtggggagccttgccctggttgtgcacccccttcgccctccccacccaggttccttctggagcagcctccttaaaggaagccaggggcagctcagagtccatgcagctggggctgggcacagggcaggacactggggcactgggagctgcagtgtgacctctaccaaatgtgtcctccagccatagtgcagggcaacacttaggctgggtatgactccagcaatataggctccccaaagggagggatctaacttactgtctccacttggtcactgtcatgtgacctcaggcagtacataccttctcttgctctccatgcctggcgaatggacattcagatgccagcatgcacattccacttgactaagagtaaagaggttgccagttggcgttggccctggactcagaagagccagcttctcatagggaaaggagttgcccaaggtcccactgcaggacacagccctggaactcagctctcccagctgcagcagaggatgctgcctattggaccatactgcccatcagaccatactgccaggccctgggaagtgccagggtggcagggggcagtctagtggaatgagacagcctggtttgccatgtttcttaggacccaccctgatgtaggctcacatcaccagcactcaccaacctagagatttcctgtcgctgttgacaggaaggctggatctgcaggcctcctggtggccatgagtctgcacagaccagagctggggtggaggccacaaccctgtgcccagtatctcagcttctcactctccccagccccaaccagggacacatgggttatttgaaaccccagggggtcaactcgggagggatgttttagctaaaagctatggggataaaaaggaaacacccctcactggctcaagccttcagttaaatgaacgtggatgtgcgacccaggaactgtgcagcaaagacctccagaccctcccctccagaaagcaggcagtcatccttgagccaaaacgcagatgagcttcctgtgctcgagccaggcttggccagggaattgtgtacgcatgcacccagggcagtggaggactaatcaatccctgggagtgagctgctctatgccaggacccatggtatccaaggccaggagtgaggactcacgtgccttcctccacactgcacccccacaccactaccaagcaggggactgacggccagccctgctggggcagaaggaaacccttgccccagtgctacctgggagtaagggggtcaggggacctgcaagtcatggacaaaacattaggtcaccatttgttagtctctcaatactttactggccatatcccccgatacccccacagcaatttcaccaacacagagcaactgccctcagccactctgatgtgatggagccaatccaggtgtcctagaaatatcctagaaatgcagagcatggggaaatcacagaaccctgggaaatgccataagaacctgggctctggaaagtgccatccacctcccctctggtcaggctggcggcactgacaaggcatccacagggcagccatgctatggcccagacctccggatatgcaggaaccggggcctcccacagaagtccctgcgcacagccacaagattaaggtacaggtcaggccggctctgaagccagctgctgacaagctccgggtgccttgggtccacttctaagaagatactaccagagtctttcaggagccggggtgccaaggccagaatgtgggtaatgatgtccatgccctcctccccaccatccagggccgcggggtcttcatagctgcggatctcaggggccagctgctccatgtcctggtggaagacgtagggagggttgctgacaatcaggtccatggggccccagggcaggtgtgtccagctcctttctgaggtcatgtcgaggtggatgatccaaatcctgtcctgcaaccgaagcctctgagcattctcatgggtcagagagatagcagcttcccgcttatccacagcaatgactcggctctgggggagctggctcagcaggctgagggagatggctcctgatccgcagcccacctccagaatgagggggctgcctggggatcccacagcatgggacctctgggccacctcttccagcacccactcaaccagttcctctgtttctggccgaggaataaacactgggggcaccatccttaggctgagcccctggaagtcccactctccaaggatgtactgcaccggcatcctctgcaatcgacggctactcagctcccggatacactgtagttgctgagaggtcaagggctgggtccaaagtgccggcctcaggctctgaaatgttttggctccaaggacatgagccacgatgtactcactggattcccgggcctcagggatacccctcttctcaaagaccccagtccagtggctgaccagttctatggcactggataacccagccagaggtggttggggttgccatgagctgaaggcccagccccgggtacttcccctcctccctgggccagacaggagggcccacagcattcggccccaaagctccatgtctcagggaaaggttctccagagtgcttccaggttcccaagtctgctttatgatgtcagctgctgaggtgagtgctgagagtggcccctggacccagctgggtggagatggagaggtcacaagctctggtgccccaaaatggctctggtcctcagatatagttggttgccaccctgcctgaaaggctgccccacccacccaccagccggagaagctgccccgaact

SEQ ID NO: 13702 - RNA, 11545 nt, Homo sapiens
  source 1..11545: mol_type = other RNA
gctgggattacaggcatgagccaccatgcccagctaatttttgtatttttagtagagacagggtttcaccatgttggccaggctggtcttgaactcctgagctcgggtgatctgcctgcttcagcctcccaaagtgctgggattacaagtgtgagccaccctgcacggcccctttctttctggcttcctcctcccttcttccttttctttcatttttaaaacatttttttaaaattattatttttaaatttttttttttgagatggagtctagctctgtcgcccaggctggagtgcagtggcatgatcttggctcactgcaatctctgcctcccgggttcaagcaattctcctgcttcagcctcccgagtagctgggattacaggtgtccaccaccacacccagctaatttttgtatttttagtagacggggtttcactgtgttggccaggctggtcttgaactcctaaccttgtgatccttggcctcccaaagtgctgggattacaaacgtgagctactgcgcctggcctattattattatttttgagacagagttttgctcttgttgcctgggtgggagtacaatggcgtgatcttggctcactgcaacatctgcctctcggtttcaagcgattctcctgcctcagcctctcaagtagctgggattacaggcgtgagccaccacacccggctaatttttgtatttttagtacagacggattttcaccatgttggccaagctggcctcgaactcctgacctcaggtgatctgcctgcctcagcctcccagagtgctgggattacaggcgtgagccaccgcgcccggcctaaaattatttttttagagacagggtctgactctgatgtccaggctggagtgcagtggcgctattatagctcactgctgtcttaaactcttgtgctcaagtaatcctcctgcctcagcctcccgagtaggtgggaccacaggcatgtgccaccatgcccagctcatatttttaattattgaaaaaaaaaaaacccaattttaaaaaccacacacagactcaaatgggcacagcaccaaattatgacacattagaatccttcctatgtgctcagagaacagggtttgtgctgagcttgagataaggcttctcttgctgtccctgtcaatcaaagagactgcaaggtgggcttcagacacagtgctagcatttgtaaacaattatctgtgagaatcagcggtcactttgtcctgtgctaccaaaatcaaacactgaaagaaaatggacattgagaccaacataagactacaactaccatcccagcccccagttcaaacatttgtgttcattgctcttcgccctgatggactgtatgctaagaaagaatttgcacttgcaaaatacatttttgctaactagatgctcattttatctttttaaaaatatgtatttcagttgcacatgaaatgtactttgaaagaatgagctccaaagttctggggggctgagacaggcgggctgagtgaaatgatgaagaaacagtggctttcagtgcgggccaagagagtagtgagcaatggtcagttattgagctgtggagtgccttcaacaagggtttttagacacatccatctggtgcctcatcccagaacctcacaggcctagggacctgaaatgctccccatgacaaggcaaacttcatatcctcacatgctgagacagactcaactttcagtctggaactgggctgggtgtctgtcagtccacgccacccatatccggagtacatcagagtctgggttcagtggcagccactttcgctgccctctcctgccccacacctagcgctctgcctggcccctttgctgtgggcgtgaaaatctggcacccgggccgacagggagagagctcagtctgcgtctgctgctttctgtttgattcatcactttccccttcaccctggagcccacgttggctgtggggcacctaactggctcctgaggcccctctggggggttgaggccctgggctgcatttggcctcggcagcctgctcacgcctctcctgactgggatgtcagaggactaggttcaaactccagcatggccagctgctggctgtgtgaccttgggcatgttaagcctcagtcccttcatccatacagtgggccaaggaagggatccctgatgtgccaacagatggatttatgaccacgtgtgtgcagcacctggcactagtttacacactgcagatgcccggtactgttgtcgccagcactcaggtctaggagagtggtcttcacaactctacctcaagggttgcctttggactgtgtccccacatggtcacatttgcatctccagacgccccaatgctgcttctcggatattctgaaggcatcctacactgtcaagctccccgactgttccccccagcaccccagtctccaactcagggtggccccatttcccccaggtcccaatcagatccctgggcccactgtggtcctggccatctcacatccaaaccctcagcaatggttgtgagtcagttctgttccagaatatctgatgccactgctacagaccccagccacctccagaccctggacaagttgcagcctcctgccccagcccctttttcctggcagccagaaagagcagcctcaatgcttctctaaccctgtaactcagctcaaaaagctctttaggcccctggtccccagaaatgcattcagagctcagccaaggggacctctcggcaccacctcacccctacatatccctacccgcatgtctgcagaactccaggcttttgtccagactgtccctactgcctggtatattcctgtcctatccgcccctcctcaagcctggtgtgatgactaaggcctccagctccaggtcactcagcctatgccagaatcacagctcagccagcctatgagcaagtttcttagccccagtttgtttcttcgtcagtataacgagagggttcacagcctccatctctgaggatgtcatgaaggttgagtaagataatcctggaagtacttggcgcaggatgcaccatattctataggaccctccacttggtatcatctccctggtgcctgacacaaagtaggtcttgagagactgaggccctggccctatacctcaggagatgcacccaggagcagctgcaggtcttctagaaagccctctagggacagccctggaaacccttgctcctgctccaagggtccacaagcccaggtaacttctgcgctaagctctgcaggggacagcccaggacctagttatgctggcctcagcgtctctgatagtcaaatggacaccaatggcagcctcatcctcccttcctgtccagctatgcaacctgacctgcaactgcaccctgctgagccttggtgtcctcaactttgtaatgtggggacaactaaaaaccccatgtgccagccctggcaacatagcaagaccccgtttctaaaaaaaaaaaaaaattaaaaattagccaggcagggttgttcacacctgtagtcctagtttgctttgcttggtcacgtagctcagcctcacactgacttccaggaacagcagagggacttggacgcctctccaggcaggcaggcctgttcctggaaagccaggtggggtggggggtcttcaggtggcaaaggaaggactggcagctgtgagccagagaagagacctggctcgtgccccagccctgctcctgtcctgctaagcctcagtttcctcatctgtaccacagggatctctgtgagcgcttcaggcaccaacaatctgctccctgggctcagtaggggatatctgatcccaccatttccccagccacatgccccagaagagggccgcagacctagtacaagagggagcaataaggtgacatcctctgctctgagaggtagagtgtttggggaagaccccagcccctgggaagggggccacttagccaggcctgcctgccacggggcatggctactctaagctgtctcaccctccccctttaggcatagctggggcaggtggaggtcagcccagttcagggctttccatgaagctgaggtaggcttccctgcctttcccactttgtgagctgtaaaattagcctttcctgaccattttcctgcaggactgctgtatgtgtgagaggtagtctttggaagaaaaggggcctctagaatttgaagcttctgatttctggttatgaggccaaagatcccaaaggtccttccagacacctcaggagggccctggggggcagaggctgggggctgtacagccaattacctcagaggggaaggcacccactcattccgcaagcgggggaaatcctgctctcctcccacagctaccagagcttcagatgggactcagatctgtctgcacacccagggctacagttggcctaatgtgactcttacctgcccataaacctggcccagagggctttatgggccagaatccctgggtttagtagctacatggacagccatatgagcaccacctaattgacttaattaactaaccccaggcctttggaagcaataggagatgagagcatcatactgggagtcaggagtcaagtgctgtgttacttcaagtaagccccatccctctctgggaaaaaagatcagggattgaatataagtcttgccatgatccaccccttccagtataaacaggccctcctggcttcatccaaagcgtatccaggtgatttggggccaagctgacccttgaacccaggtgtccatgctctctgtcccccagcttctcagctctgaaacccagcatgaggcccatgtctggcctcccagtagctctccatgtggctcctgggttaggactggcttcaggagccccaagccttggctgggtgggatggtgtctccagagtcctttagtacccctggaaagggaggtcctagtcccagcttggacagggacagggctgagggcaccagttggccaattcagttttaggaaccaggaggttgagaaccccagggatagccccactccaccataggaacagaatggtgacacagctctgctcaggcctatggcttacatggaggggccaggcccattagctcaaagtcaggggctgctgtgctcatttcacagatgcagtacctgcaacccagagagtacagggcccctgctcatcctcacacacccaaggggtcctgggccagtcacataactccacaggagagcaggaacaggcttggtcccagtctctgaggtcctctctggacccagtctctggagatgggccatggaggccagccttgcactttctccccacatcccagtcccattcctcacccactcccttctgggacccatgctggtcagtctttcagtcttctcactctgggaaagggccacctctctccaaatatgagtaaaaaaagggggggcctgggcagtttaggtctgaaggttgaggaagagttcccctggccacatcacctatcagaagagaggtggttaaggcaatttatcatgactctcaaaattcttccagcctctgcccatttccacgttgcaattccaaagccacttcaatcagtaggcgtgtgttacagcagcactctaatttgggcaccacaatctatattcgtttcccgtggctgctgtaacaaattatcacacatgtgttttcacacatgtgaaaacaacacaaatttatgatcttactgttctggaggtcagcaatctgaaatcagtttcacagggcttaaaatcaaggtattggcaggactgcattcttcttgaggccccagaggagaagaggctgtctgcattcctcggctcatggctcttcctccagcaattgcatcactctgacctctgcttccattgttacatacattttcttccgtcactctgacactcctgcctcctttacagaggcccttgtgattatactcagtttacctgaaaaatccaggatactccttccatctcaagatccttaatcacatctgcaaagtccattttgctatgtgaaggtaatatagtcacatgttaaggtttaggtgattaagacactgccattttggggggtcactgttcagcctaccagagcaggggtagagttgctttgacagtcccaaatccagttcagggggcttgtccagggcagaaggtcatgaggaggagatcaggtcactgtcctagccaggactctggctgggggctggctgaagccaagagctccaggaaacctggcgcctgctcctactgccgccaaggacagcctgttctcctggtgtggctgttgcgcagggatcaggtgcacttgagtcttcgaagtggccattgctcaacttgaatggctgcctgggtcgggcagaaggccaggtcctcatggcttcccatccctaatgaccggaatacatgggctgccaggtcagatgtgggccacatgggaagtcccagctctattctagaaaatgcatgtaccatcagcttactgatagacatttactgaacttgggtatgccagatccacagggggccccagagatgagggggataagaaggtttctgaaggcatggtacagaaggtgccagcagaggtatgggctaggggaggcagggagagcacagagcaggcatcctaaaggaggcagcatttgtgttggagcttgaagaagtggattgtttgcaccgcctgggcaaagggaaggtgtgtgttcagggcatcgagagtactgcacaaaggctgaagcccagggcagtagagaagagaatccactaagaaggagccaatgaagaaaaaaaagagaaaagaatcgaaggtggatagggaaagacatgctgtcccgcagaggttaaaggggttctcacctcaagccagcagttctcaaaccttgtcagcagtggagccctttgttctgatgacagcctactcagagcactgatggggccttgggaggggcccccagggcttttcccacagttgtcctcccccacctcttcagaactggattccataggacacaagagaacacacttaagtcatggggagccagctaagtgtttggggcaaggattgggagcagccaatagcccagggtccaggtgggggtaaaggagcaaaaaagagtattttttgcatttagggggttcggggcctatttcaataaggcagctgtatgagacccatggagaaacccactgacaactgggaaaagcatccaactgtgagacaaggcctcagtttccccaactatcagaagaggagatagaattactctcccagagtacatcaaacagggactcctacactcctgtctatgctctgggctctggctgaaggaggctgcacgggcagtgggcacatctctcaagacctcaggggcttgcacagcctggactccatcagctccatgtcctcctcccattctgcctgcaagtgctccttgacatatgctggtggtggtggggaggctgttcgagtctctggctttggcctcaggagcaagggaggggatagggcaggtgggcctggctttccctgagctagagccactggctgccctggcctgggcctcaaggcactggggccatagtgaggagaggctgaggggagatgtaggctgccaggctaccagcctgctggctccatctctagacaacagtgaggagtcaagagcccaagactgaaactcctgccttcccttctttccagactgccttgtatccctgcctgccttatgttggtcccatgcatcagatggacgcctgagggcactgggtccttcctccctgtgtctgccctccgaggaaggcaaggaaaaatgccacaatgtgccaagccaggcacatcccatgggctcctcacatgcatcctataaaataaagcattaagtcccatttctcagccttagaagccaaggctgagtgaggtgaagtcatctgcccaaggtcacatcctcgtgaggggcagattctgggattgaaatccaggctggtgtggctccaacatctgggctcaacgtccagggcccaatcaagccagtggctgcaggcttgaggccccgcctgccagtcctcttggcttggaccttttcctcagcagagtcaagctgcacatttttctgggcagaaagttgtgcccgaggccggctcctgcttgtggccccagctgccccgacagtgtcactctccaacactgcactctcttctggtgcaacatccacaagctcgccaaggcccttcctcaggaatgggcctgaggccaggagggagagaccatcagggaagccaggactggctgaggtgtaggggggcgacagactgctccgaggtcagggcagctaccctgagatgctgctgaagacagcaagagccaaagggcacaaggagaaagacagaaagggcaatactggtgaggaccttagcaggcaaaggtctgtgagcatgggggactaaggaagtggggagccttgccctggttgtgcacccccttcgccctccccacccaggttccttctggagcagcctccttaaaggaagccaggggcagctcagagtccatgcagctggggctgggcacagggcaggacactggggcactgggagctgcagtgtgacctctaccaaatgtgtcctccagccatagtgcagggcaacacttaggctgggtatgactccagcaatataggctccccaaagggagggatctaacttactgtctccacttggtcactgtcatgtgacctcaggcagtacataccttctcttgctctccatgcctggcgaatggacattcagatgccagcatgcacattccacttgactaagagtaaagaggttgccagttggcgttggccctggactcagaagagccagcttctcatagggaaaggagttgcccaaggtcccactgcaggacacagccctggaactcagctctcccagctgcagcagaggatgctgcctattggaccatactgcccatcagaccatactgccaggccctgggaagtgccagggtggcagggggcagtctagtggaatgagacagcctggtttgccatgtttcttaggacccaccctgatgtaggctcacatcaccagcactcaccaacctagagatttcctgtcgctgttgacaggaaggctggatctgcaggcctcctggtggccatgagtctgcacagaccagagctggggtggaggccacaaccctgtgcccagtatctcagcttctcactctccccagccccaaccagggacacatgggttatttgaaaccccagggggtcaactcgggagggatgttttagctaaaagctatggggataaaaaggaaacacccctcactggctcaagccttcagttaaatgaacgtggatgtgcgacccaggaactgtgcagcaaagacctccagaccctcccctccagaaagcaggcagtcatccttgagccaaaacgcagatgagcttcctgtgctcgagccaggcttggccagggaattgtgtacgcatgcacccagggcagtggaggactaatcaatccctgggagtgagctgctctatgccaggacccatggtatccaaggccaggagtgaggactcacgtgccttcctccacactgcacccccacaccactaccaagcaggggactgacggccagccctgctggggcagaaggaaacccttgccccagtgctacctgggagtaagggggtcaggggacctgcaagtcatggacaaaacattaggtcaccatttgttagtctctcaatactttactggccatatcccccgatacccccacagcaatttcaccaacacagagcaactgccctcagccactctgatgtgatggagccaatccaggtgtcctagaaatatcctagaaatgcagagcatggggaaatcacagaaccctgggaaatgccataagaacctgggctctggaaagtgccatccacctcccctctggtcaggctggcggcactgacaaggcatccacagggcagccatgctatggcccagacctccggatatgcaggaaccggggcctcccacagaagtccctgcgcacagccacaagattaaggtacaggtcaggccggctctgaagccagctgctgacaagctccgggtgccttgggtccacttctaagaagatactaccagagtctttcaggagccggggtgccaaggccagaatgtgggtaatgatgtccatgccctcctccccaccatccagggccgcggggtcttcatagctgcggatctcaggggccagctgctccatgtcctggtggaagacgtagggagggttgctgacaatcaggtccatggggccccagggcaggtgtgtccagctcctttctgaggtcatgtcgaggtggatgatccaaatcctgtcctgcaaccgaagcctctgagcattctcatgggtcagagagatagcagcttcccgcttatccacagcaatgactcggctctgggggagctggctcagcaggctgagggagatggctcctgatccgcagcccacctccagaatgagggggctgcctggggatcccacagcatgggacctctgggccacctcttccagcacccactcaaccagttcctctgtttctggccgaggaataaacactgggggcaccatccttaggctgagcccctggaagtcccactctccaaggatgtactgcaccggcatcctgcagagggggcagctgggtggtcatcagggacagagctctgcaatcgacggctactcagctcccggatacactgtagttgctgagaggtcaagggctgggtccaaagtgccggcctcaggctctgaaatgttttggctccaaggacatgagccacgatgtactcactggattcccgggcctcagggatacccctcttctcaaagaccccagtccagtggctgaccagttctatggcactggataacccagccagaggtggttggggttgccatgagctgaaggcccagccccgggtacttcccctcctccctgggccagacaggagggcccacagcattcggccccaaagctccatgtctcagggaaaggttctccagagtgcttccaggttcccaagtctgctttatgatgtcagctgctgaggtgagtgctgagagtggcccctggacccagctgggtggagatggagaggtcacaagctctggtgccccaaaatggctctggtcctcagatatagttggttgccaccccgagtccaccagactccagaagcggctcttgcaccagtgcgccgtcccaggagccaaggcccgaagtcagaagtgtaaactccctcacagctacgcaccgcattgttaacgacccagatgaggccccctctctccaaccctgtttccccatctgcactatggagaatggtaccggccaggtctccaggcggttgcagtcgaaacaccccgttccgatccccacctcccatgcatacctgcctgaaaggctgccccacccacccaccagccggagaagctgccccgaact

SEQ ID NO: 13703 - RNA, 11372 nt, Homo sapiens
  source 1..11372: mol_type = other RNA
gctgggattacaggcatgagccaccatgcccagctaatttttgtatttttagtagagacagggtttcaccatgttggccaggctggtcttgaactcctgagctcgggtgatctgcctgcttcagcctcccaaagtgctgggattacaagtgtgagccaccctgcacggcccctttctttctggcttcctcctcccttcttccttttctttcatttttaaaacatttttttaaaattattatttttaaatttttttttttgagatggagtctagctctgtcgcccaggctggagtgcagtggcatgatcttggctcactgcaatctctgcctcccgggttcaagcaattctcctgcttcagcctcccgagtagctgggattacaggtgtccaccaccacacccagctaatttttgtatttttagtagacggggtttcactgtgttggccaggctggtcttgaactcctaaccttgtgatccttggcctcccaaagtgctgggattacaaacgtgagctactgcgcctggcctattattattatttttgagacagagttttgctcttgttgcctgggtgggagtacaatggcgtgatcttggctcactgcaacatctgcctctcggtttcaagcgattctcctgcctcagcctctcaagtagctgggattacaggcgtgagccaccacacccggctaatttttgtatttttagtacagacggattttcaccatgttggccaagctggcctcgaactcctgacctcaggtgatctgcctgcctcagcctcccagagtgctgggattacaggcgtgagccaccgcgcccggcctaaaattatttttttagagacagggtctgactctgatgtccaggctggagtgcagtggcgctattatagctcactgctgtcttaaactcttgtgctcaagtaatcctcctgcctcagcctcccgagtaggtgggaccacaggcatgtgccaccatgcccagctcatatttttaattattgaaaaaaaaaaaacccaattttaaaaaccacacacagactcaaatgggcacagcaccaaattatgacacattagaatccttcctatgtgctcagagaacagggtttgtgctgagcttgagataaggcttctcttgctgtccctgtcaatcaaagagactgcaaggtgggcttcagacacagtgctagcatttgtaaacaattatctgtgagaatcagcggtcactttgtcctgtgctaccaaaatcaaacactgaaagaaaatggacattgagaccaacataagactacaactaccatcccagcccccagttcaaacatttgtgttcattgctcttcgccctgatggactgtatgctaagaaagaatttgcacttgcaaaatacatttttgctaactagatgctcattttatctttttaaaaatatgtatttcagttgcacatgaaatgtactttgaaagaatgagctccaaagttctggggggctgagacaggcgggctgagtgaaatgatgaagaaacagtggctttcagtgcgggccaagagagtagtgagcaatggtcagttattgagctgtggagtgccttcaacaagggtttttagacacatccatctggtgcctcatcccagaacctcacaggcctagggacctgaaatgctccccatgacaaggcaaacttcatatcctcacatgctgagacagactcaactttcagtctggaactgggctgggtgtctgtcagtccacgccacccatatccggagtacatcagagtctgggttcagtggcagccactttcgctgccctctcctgccccacacctagcgctctgcctggcccctttgctgtgggcgtgaaaatctggcacccgggccgacagggagagagctcagtctgcgtctgctgctttctgtttgattcatcactttccccttcaccctggagcccacgttggctgtggggcacctaactggctcctgaggcccctctggggggttgaggccctgggctgcatttggcctcggcagcctgctcacgcctctcctgactgggatgtcagaggactaggttcaaactccagcatggccagctgctggctgtgtgaccttgggcatgttaagcctcagtcccttcatccatacagtgggccaaggaagggatccctgatgtgccaacagatggatttatgaccacgtgtgtgcagcacctggcactagtttacacactgcagatgcccggtactgttgtcgccagcactcaggtctaggagagtggtcttcacaactctacctcaagggttgcctttggactgtgtccccacatggtcacatttgcatctccagacgccccaatgctgcttctcggatattctgaaggcatcctacactgtcaagctccccgactgttccccccagcaccccagtctccaactcagggtggccccatttcccccaggtcccaatcagatccctgggcccactgtggtcctggccatctcacatccaaaccctcagcaatggttgtgagtcagttctgttccagaatatctgatgccactgctacagaccccagccacctccagaccctggacaagttgcagcctcctgccccagcccctttttcctggcagccagaaagagcagcctcaatgcttctctaaccctgtaactcagctcaaaaagctctttaggcccctggtccccagaaatgcattcagagctcagccaaggggacctctcggcaccacctcacccctacatatccctacccgcatgtctgcagaactccaggcttttgtccagactgtccctactgcctggtatattcctgtcctatccgcccctcctcaagcctggtgtgatgactaaggcctccagctccaggtcactcagcctatgccagaatcacagctcagccagcctatgagcaagtttcttagccccagtttgtttcttcgtcagtataacgagagggttcacagcctccatctctgaggatgtcatgaaggttgagtaagataatcctggaagtacttggcgcaggatgcaccatattctataggaccctccacttggtatcatctccctggtgcctgacacaaagtaggtcttgagagactgaggccctggccctatacctcaggagatgcacccaggagcagctgcaggtcttctagaaagccctctagggacagccctggaaacccttgctcctgctccaagggtccacaagcccaggtaacttctgcgctaagctctgcaggggacagcccaggacctagttatgctggcctcagcgtctctgatagtcaaatggacaccaatggcagcctcatcctcccttcctgtccagctatgcaacctgacctgcaactgcaccctgctgagccttggtgtcctcaactttgtaatgtggggacaactaaaaaccccatgtgccagccctggcaacatagcaagaccccgtttctaaaaaaaaaaaaaaattaaaaattagccaggcagggttgttcacacctgtagtcctagtttgctttgcttggtcacgtagctcagcctcacactgacttccaggaacagcagagggacttggacgcctctccaggcaggcaggcctgttcctggaaagccaggtggggtggggggtcttcaggtggcaaaggaaggactggcagctgtgagccagagaagagacctggctcgtgccccagccctgctcctgtcctgctaagcctcagtttcctcatctgtaccacagggatctctgtgagcgcttcaggcaccaacaatctgctccctgggctcagtaggggatatctgatcccaccatttccccagccacatgccccagaagagggccgcagacctagtacaagagggagcaataaggtgacatcctctgctctgagaggtagagtgtttggggaagaccccagcccctgggaagggggccacttagccaggcctgcctgccacggggcatggctactctaagctgtctcaccctccccctttaggcatagctggggcaggtggaggtcagcccagttcagggctttccatgaagctgaggtaggcttccctgcctttcccactttgtgagctgtaaaattagcctttcctgaccattttcctgcaggactgctgtatgtgtgagaggtagtctttggaagaaaaggggcctctagaatttgaagcttctgatttctggttatgaggccaaagatcccaaaggtccttccagacacctcaggagggccctggggggcagaggctgggggctgtacagccaattacctcagaggggaaggcacccactcattccgcaagcgggggaaatcctgctctcctcccacagctaccagagcttcagatgggactcagatctgtctgcacacccagggctacagttggcctaatgtgactcttacctgcccataaacctggcccagagggctttatgggccagaatccctgggtttagtagctacatggacagccatatgagcaccacctaattgacttaattaactaaccccaggcctttggaagcaataggagatgagagcatcatactgggagtcaggagtcaagtgctgtgttacttcaagtaagccccatccctctctgggaaaaaagatcagggattgaatataagtcttgccatgatccaccccttccagtataaacaggccctcctggcttcatccaaagcgtatccaggtgatttggggccaagctgacccttgaacccaggtgtccatgctctctgtcccccagcttctcagctctgaaacccagcatgaggcccatgtctggcctcccagtagctctccatgtggctcctgggttaggactggcttcaggagccccaagccttggctgggtgggatggtgtctccagagtcctttagtacccctggaaagggaggtcctagtcccagcttggacagggacagggctgagggcaccagttggccaattcagttttaggaaccaggaggttgagaaccccagggatagccccactccaccataggaacagaatggtgacacagctctgctcaggcctatggcttacatggaggggccaggcccattagctcaaagtcaggggctgctgtgctcatttcacagatgcagtacctgcaacccagagagtacagggcccctgctcatcctcacacacccaaggggtcctgggccagtcacataactccacaggagagcaggaacaggcttggtcccagtctctgaggtcctctctggacccagtctctggagatgggccatggaggccagccttgcactttctccccacatcccagtcccattcctcacccactcccttctgggacccatgctggtcagtctttcagtcttctcactctgggaaagggccacctctctccaaatatgagtaaaaaaagggggggcctgggcagtttaggtctgaaggttgaggaagagttcccctggccacatcacctatcagaagagaggtggttaaggcaatttatcatgactctcaaaattcttccagcctctgcccatttccacgttgcaattccaaagccacttcaatcagtaggcgtgtgttacagcagcactctaatttgggcaccacaatctatattcgtttcccgtggctgctgtaacaaattatcacacatgtgttttcacacatgtgaaaacaacacaaatttatgatcttactgttctggaggtcagcaatctgaaatcagtttcacagggcttaaaatcaaggtattggcaggactgcattcttcttgaggccccagaggagaagaggctgtctgcattcctcggctcatggctcttcctccagcaattgcatcactctgacctctgcttccattgttacatacattttcttccgtcactctgacactcctgcctcctttacagaggcccttgtgattatactcagtttacctgaaaaatccaggatactccttccatctcaagatccttaatcacatctgcaaagtccattttgctatgtgaaggtaatatagtcacatgttaaggtttaggtgattaagacactgccattttggggggtcactgttcagcctaccagagcaggggtagagttgctttgacagtcccaaatccagttcagggggcttgtccagggcagaaggtcatgaggaggagatcaggtcactgtcctagccaggactctggctgggggctggctgaagccaagagctccaggaaacctggcgcctgctcctactgccgccaaggacagcctgttctcctggtgtggctgttgcgcagggatcaggtgcacttgagtcttcgaagtggccattgctcaacttgaatggctgcctgggtcgggcagaaggccaggtcctcatggcttcccatccctaatgaccggaatacatgggctgccaggtcagatgtgggccacatgggaagtcccagctctattctagaaaatgcatgtaccatcagcttactgatagacatttactgaacttgggtatgccagatccacagggggccccagagatgagggggataagaaggtttctgaaggcatggtacagaaggtgccagcagaggtatgggctaggggaggcagggagagcacagagcaggcatcctaaaggaggcagcatttgtgttggagcttgaagaagtggattgtttgcaccgcctgggcaaagggaaggtgtgtgttcagggcatcgagagtactgcacaaaggctgaagcccagggcagtagagaagagaatccactaagaaggagccaatgaagaaaaaaaagagaaaagaatcgaaggtggatagggaaagacatgctgtcccgcagaggttaaaggggttctcacctcaagccagcagttctcaaaccttgtcagcagtggagccctttgttctgatgacagcctactcagagcactgatggggccttgggaggggcccccagggcttttcccacagttgtcctcccccacctcttcagaactggattccataggacacaagagaacacacttaagtcatggggagccagctaagtgtttggggcaaggattgggagcagccaatagcccagggtccaggtgggggtaaaggagcaaaaaagagtattttttgcatttagggggttcggggcctatttcaataaggcagctgtatgagacccatggagaaacccactgacaactgggaaaagcatccaactgtgagacaaggcctcagtttccccaactatcagaagaggagatagaattactctcccagagtacatcaaacagggactcctacactcctgtctatgctctgggctctggctgaaggaggctgcacgggcagtgggcacatctctcaagacctcaggggcttgcacagcctggactccatcagctccatgtcctcctcccattctgcctgcaagtgctccttgacatatgctggtggtggtggggaggctgttcgagtctctggctttggcctcaggagcaagggaggggatagggcaggtgggcctggctttccctgagctagagccactggctgccctggcctgggcctcaaggcactggggccatagtgaggagaggctgaggggagatgtaggctgccaggctaccagcctgctggctccatctctagacaacagtgaggagtcaagagcccaagactgaaactcctgccttcccttctttccagactgccttgtatccctgcctgccttatgttggtcccatgcatcagatggacgcctgagggcactgggtccttcctccctgtgtctgccctccgaggaaggcaaggaaaaatgccacaatgtgccaagccaggcacatcccatgggctcctcacatgcatcctataaaataaagcattaagtcccatttctcagccttagaagccaaggctgagtgaggtgaagtcatctgcccaaggtcacatcctcgtgaggggcagattctgggattgaaatccaggctggtgtggctccaacatctgggctcaacgtccagggcccaatcaagccagtggctgcaggcttgaggccccgcctgccagtcctcttggcttggaccttttcctcagcagagtcaagctgcacatttttctgggcagaaagttgtgcccgaggccggctcctgcttgtggccccagctgccccgacagtgtcactctccaacactgcactctcttctggtgcaacatccacaagctcgccaaggcccttcctcaggaatgggcctgaggccaggagggagagaccatcagggaagccaggactggctgaggtgtaggggggcgacagactgctccgaggtcagggcagctaccctgagatgctgctgaagacagcaagagccaaagggcacaaggagaaagacagaaagggcaatactggtgaggaccttagcaggcaaaggtctgtgagcatgggggactaaggaagtggggagccttgccctggttgtgcacccccttcgccctccccacccaggttccttctggagcagcctccttaaaggaagccaggggcagctcagagtccatgcagctggggctgggcacagggcaggacactggggcactgggagctgcagtgtgacctctaccaaatgtgtcctccagccatagtgcagggcaacacttaggctgggtatgactccagcaatataggctccccaaagggagggatctaacttactgtctccacttggtcactgtcatgtgacctcaggcagtacataccttctcttgctctccatgcctggcgaatggacattcagatgccagcatgcacattccacttgactaagagtaaagaggttgccagttggcgttggccctggactcagaagagccagcttctcatagggaaaggagttgcccaaggtcccactgcaggacacagccctggaactcagctctcccagctgcagcagaggatgctgcctattggaccatactgcccatcagaccatactgccaggccctgggaagtgccagggtggcagggggcagtctagtggaatgagacagcctggtttgccatgtttcttaggacccaccctgatgtaggctcacatcaccagcactcaccaacctagagatttcctgtcgctgttgacaggaaggctggatctgcaggcctcctggtggccatgagtctgcacagaccagagctggggtggaggccacaaccctgtgcccagtatctcagcttctcactctccccagccccaaccagggacacatgggttatttgaaaccccagggggtcaactcgggagggatgttttagctaaaagctatggggataaaaaggaaacacccctcactggctcaagccttcagttaaatgaacgtggatgtgcgacccaggaactgtgcagcaaagacctccagaccctcccctccagaaagcaggcagtcatccttgagccaaaacgcagatgagcttcctgtgctcgagccaggcttggccagggaattgtgtacgcatgcacccagggcagtggaggactaatcaatccctgggagtgagctgctctatgccaggacccatggtatccaaggccaggagtgaggactcacgtgccttcctccacactgcacccccacaccactaccaagcaggggactgacggccagccctgctggggcagaaggaaacccttgccccagtgctacctgggagtaagggggtcaggggacctgcaagtcatggacaaaacattaggtcaccatttgttagtctctcaatactttactggccatatcccccgatacccccacagcaatttcaccaacacagagcaactgccctcagccactctgatgtgatggagccaatccaggtgtcctagaaatatcctagaaatgcagagcatggggaaatcacagaaccctgggaaatgccataagaacctgggctctggaaagtgccatccacctcccctctggtcaggctggcggcactgacaaggcatccacagggcagccatgctatggcccagacctccggatatgcaggaaccggggcctcccacagaagtccctgcgcacagccacaagattaaggtacaggtcaggccggctctgaagccagctgctgacaagctccgggtgccttgggtccacttctaagaagatactaccagagtctttcaggagccggggtgccaaggccagaatgtgggtaatgatgtccatgccctcctccccaccatccagggccgcggggtcttcatagctgcggatctcaggggccagctgctccatgtcctggtggaagacgtagggagggttgctgacaatcaggtccatggggccccagggcaggtgtgtccagctcctttctgaggtcatgtcgaggtggatgatccaaatcctgtcctgcaaccgaagcctctgagcattctcatgggtcagagagatagcagcttcccgcttatccacagcaatgactcggctctgggggagctggctcagcaggctgagggagatggctcctgatccgcagcccacctccagaatgagggggctgcctggggatcccacagcatgggacctctgggccacctcttccagcacccactcaaccagttcctctgtttctggccgaggaataaacactgggggcaccatccttaggctgagcccctggaagtcccactctccaaggatgtactgcaccggcatcctgcagagggggcagctgggtggtcatcagggacagagctctgcaatcgacggctactcagctcccggatacactgtagttgctgagaggtcaagggctgggtccaaagtgccggcctcaggctctgaaatgttttggctccaaggacatgagccacgatgtactcactggattcccgggcctcagggatacccctcttctcaaagaccccagtccagtggctgaccagttctatggcactggataacccagccagaggtggttggggttgccatgagctgaaggcccagccccgggtacttcccctcctccctgggccagacaggagggcccacagcattcggccccaaagctccatgtctcagggaaaggttctccagagtgcttccaggttcccaagtctgctttatgatgtcagctgctgaggtgagtgctgagagtggcccctggacccagctgggtggagatggagaggtcacaagctctggtgccccaaaatggctctggtcctcagatatagttggttgccacccggccaggtctccaggcggttgcagtcgaaacaccccgttccgatccccacctcccatgcatacctgcctgaaaggctgccccacccacccaccagccggagaagctgccccgaact
